European Patent Application EP 4 520 821 A1, published March 12, 2025. Title: microRNA-DERIVED RNAs AND POLYPEPTIDES AND USES THEREOF. Applicant: THE REGENTS OF THE UNIVERSITY OF MICHIGAN. Application CN. The sequence listing filed with the application follows.

SEQUENCE LISTING (19738 sequences)

SEQ ID NO: 1 - protein, 11 aa, Homo sapiens
MAACVRKWTLC

SEQ ID NO: 2 - protein, 13 aa, Homo sapiens
MACILPSQCPIPK

SEQ ID NO: 3 - protein, 18 aa, Homo sapiens
MACIWIGVGIWKPASRMF

SEQ ID NO: 4 - protein, 33 aa, Homo sapiens
MACSVLVICIFSVQGLLRFRQKGNTLNELINTI

SEQ ID NO: 5 - protein, 51 aa, Homo sapiens
MACTRSSGLICSSFKYHLTEVTSGTDTLHSSTALVPSITLTSFRGVITSTL

SEQ ID NO: 6 - protein, 16 aa, Homo sapiens
MAFHHVGQAGLELLTL

SEQ ID NO: 7 - protein, 64 aa, Homo sapiens
MAFHHVGQAGLELTSSDPPTLASQSVGITSVSHHAWPACFHYYLPVLSMQHGSTIDSEVLWHIR

SEQ ID NO: 8 - protein, 36 aa, Homo sapiens
MAFHHVGQASFKLLASSGLPALASQSAGITGDFWLF

SEQ ID NO: 9 - protein, 15 aa, Homo sapiens
MAFPYSLYLYNFSQG

SEQ ID NO: 10 - protein, 45 aa, Homo sapiens
MAFSQDKCWRRFGDTGSLIHCWWECKMARPLLESIKSPNHRTQST

SEQ ID NO: 11 - protein, 35 aa, Homo sapiens
MAFSQEALRTSSLCPSTPPNIATRVSVWIFHNRKA

SEQ ID NO: 12 - protein, 61 aa, Homo sapiens
MAGAASAPGGRAGSQGRTGRGSCALWLGHLSRCRGSQSSAPVAAAPRSGRGVISCVFVEFL

SEQ ID NO: 13 - protein, 19 aa, Homo sapiens
MAGIEGGIETRGLRLRFCS

SEQ ID NO: 14 - protein, 15 aa, Homo sapiens
MAGNHPEKVEIIIFS

SEQ ID NO: 15 - protein, 27 aa, Homo sapiens
MAGPAIGSSLGLGEGAVCSQHDLRRQG

SEQ ID NO: 16 - protein, 57 aa, Homo sapiens
MAGPAIGSSLSGRRVGGGGARGRAPAGAERSRGRAAERGRRGEVRGQPEDVPGLSGT

SEQ ID NO: 17 - protein, 11 aa, Homo sapiens
MAGPHLTVPFI

SEQ ID NO: 18 - protein, 18 aa, Homo sapiens
MAGQPRAAAEAEAGEPSR

SEQ ID NO: 19 - protein, 23 aa, Homo sapiens
MAGSSARSEGTSPSLLTIPTLAP

SEQ ID NO: 20 - protein, 45 aa, Homo sapiens
MAHCNLELQSSSDPLASASGVAGSTGAYHHAQLIFIFILLFIYLF

SEQ ID NO: 21 - protein, 12 aa, Homo sapiens
MAIIKKAGNNRC

SEQ ID NO: 22 - protein, 102 aa, Homo sapiens
MAIIKKSGNNTCWRGCGEIVTLLHRWWECKLVQPLWKTVWRFLKDLELEIPFDPLLGIYLKDYKSCYYKDTCTCMFIATLFTIAKTWNQPKCPSMIDRIKKM

SEQ ID NO: 23 - protein, 57 aa, Homo sapiens
MAISITNLDHVFFFFFFFFEIASHSSTQVGVQWCNHSLLQPQTSGLKQSSCLSLPST

SEQ ID NO: 24 - protein, 25 aa, Homo sapiens
MAISKLLNPSGPQMRITPATQVVVG

SEQ ID NO: 25 - protein, 12 aa, Homo sapiens
MAIYNLNSSPLL

SEQ ID NO: 26 - protein, 17 aa, Homo sapiens
MAKTKQGKVQKEYMIHL

SEQ ID NO: 27 - protein, 13 aa, Homo sapiens
MAKVVNPADRIAG

SEQ ID NO: 28 - protein, 99 aa, Homo sapiens
MALCWLTGSLGVCVAQELWASRDRAFSALGPTCQSPPGAGCMEKRKSNTKANMLTTFLCSSFKSKMFPMGHAGSCSELKGRDRSPTGQERRTTGRMPHV

SEQ ID NO: 29 - protein, 13 aa, Homo sapiens
MALEGSPDVHPFR

SEQ ID NO: 30 - protein, 59 aa, Homo sapiens
MALGGKQTGLWGPGVRQPVRRGPSMHLTAAVSCWVPKLEKSPWPRLGSGVDLGAGPGAG

SEQ ID NO: 31 - protein, 63 aa, Homo sapiens
MALGGKQTGLWGPGVRQPVRRGPSMHMTLEAQMIPTILQMRKQLRMATWLAQGGTASKRWSLK

SEQ ID NO: 32 - protein, 118 aa, Homo sapiens
MALGGKQTGLWGPGVRQPVRRGPSMHSGWVGVWGVQLGRAQPGLDSVALSACGHWSLRACGCRRRPGRAVRARLRSGPASPGSAASGPRSGLGSRSAGLGSAMVAAAASAAGRACVCA

SEQ ID NO: 33 - protein, 55 aa, Homo sapiens
MALGHTSQDCPPFAQCSSQATTWQFLAHLAFPSLFPCFSSANTLPLLLPPIQHPA

SEQ ID NO: 34 - protein, 14 aa, Homo sapiens
MALHKDSVACQVRV

SEQ ID NO: 35 - protein, 38 aa, Homo sapiens
MALIFRPCDPPTSASQSAGITGMSHCAQPRSAFIAAKI

SEQ ID NO: 36 - protein, 19 aa, Homo sapiens
MALLTISSPASSILITVNR

SEQ ID NO: 37 - protein, 106 aa, Homo sapiens
MALPERALLSLRNSAWTAWEVSHSHGPARNSDKNGCALPTTTSLKSPLSPDAAKSPPPAGQDHPQLDPPQTPSLEVTLEPLEEASLLRKVTTGLLLTTDFRRWLHA

SEQ ID NO: 38 - protein, 65 aa, Homo sapiens
MALQRELPVAFCYIPNSHSPIKPSRNEKRAVSGKVTGTDRTFMALHQSHTGSTVSKLPCVDVPYF

SEQ ID NO: 39 - protein, 20 aa, Homo sapiens
MALSTQLGHNTRQVVLVLLT

SEQ ID NO: 40 - protein, 85 aa, Homo sapiens
MALYCSYLTAGGQSTAPSRRPGRRRGRFCAELPPSPASPASRASQMASVPVQAANSVRRHPPPLGGAHGRRRPRPRRAGLSTSRL

SEQ ID NO: 41 - protein, 22 aa, Homo sapiens
MAMILRKKKMRTRAHEQSPILK

SEQ ID NO: 42 - protein, 18 aa, Homo sapiens
MAMPPPGSFFHSQFCCQL

SEQ ID NO: 43 - protein, 44 aa, Homo sapiens
MANAGALSSEYRKPKILSSWVLKQLSPRPNRKLQRMATSLLDLM

SEQ ID NO: 44 - protein, 21 aa, Homo sapiens
MANFYLLQTICQAPNLQLLFI

SEQ ID NO: 45 - protein, 15 aa, Homo sapiens
MANIFPVFAPVTFRT

SEQ ID NO: 46 - protein, 96 aa, Homo sapiens [sequence omitted]

SEQ ID NO: 47 - protein, 26 aa, Homo sapiens
MAPPRAAIWPKPTAVILSTVGKSSLL

SEQ ID NO: 48 - protein, 24 aa, Homo sapiens
MAPSWLTATSASWVQVILLPQPPE

SEQ ID NO: 49 - protein, 60 aa, Homo sapiens
MAQKGSEPLLPSSAPGMTYRQSWLWVSEKPAASPNDLLRWVANTKSSTWEVLLCFTTMKT

SEQ ID NO: 50 - protein, 16 aa, Homo sapiens
MAQKLFSQAGLERSLQ

SEQ ID NO: 51 - protein, 19 aa, Homo sapiens
MARRKHLLAEARLWSHTAA

SEQ ID NO: 52 - protein, 19 aa, Homo sapiens
MASEKLSLENYSRTFSYYI

SEQ ID NO: 53 - protein, 21 aa, Homo sapiens
MASFSVLIRPSWPPKVLELQA

SEQ ID NO: 54 - protein, 131 aa, Homo sapiens
MASISCSVTFIISCFRTLVSSSSMVVLVLSEDSFTPSLFLFPPLFPPEKFLVASIVVRMAPFSFLLALNFFRQSTVSCLCMQDATVERCEIQGCLRASAAVMRLDGLMVSILLIRSLASGVTVSHSGDGKS

SEQ ID NO: 55 - protein, 35 aa, Homo sapiens
MASISCSVTFIISCFRTLVSSSSMVVLVLSEDSIN

SEQ ID NO: 56 - protein, 17 aa, Homo sapiens
MATASMPRAQSASERPV

SEQ ID NO: 57 - protein, 25 aa, Homo sapiens
MATINNTKDNKCWQGCEEKGFLALL

SEQ ID NO: 58 - protein, 19 aa, Homo sapiens
MATIREYYSVFIFTYNFNI

SEQ ID NO: 59 - protein, 27 aa, Homo sapiens
MATLSRSWGGIFNKAHYHLPHPKWSYC

SEQ ID NO: 60 - protein, 11 aa, Homo sapiens
MATRLTYLGKT

SEQ ID NO: 61 - protein, 17 aa, Homo sapiens
MATSITQSLWPFKESFR

SEQ ID NO: 62 - protein, 25 aa, Homo sapiens
MAVHKVNVLYSGNWPNSSCHPKRGR

SEQ ID NO: 63 - protein, 118 aa, Homo sapiens
MAVRISFSRSCTILRRASSCCSRNRRGRDRPDRNACRTRRTSSSMAWSCRELHGPGALGSGRREACRCRPRLPSLRLPPGGVSTVNPQPQFTRPGLARSAATSTPAESHCQSEAPGED

SEQ ID NO: 64 - protein, 64 aa, Homo sapiens
MAVRISFSRSCTILRRASSCCSRNRRGRDRPDRNACRTRRTSSSMAWSCRELHGPGARPSSLES

SEQ ID NO: 65 - protein, 88 aa, Homo sapiens
MAVRISFSRSCTILRRASSCCSRNRRGRDRPDRNACRTRRTSSSMAWSCRELHGPGASHNSLAQGSLAQPRPPRPLSPTASRRRRGRT

SEQ ID NO: 66 - protein, 30 aa, Homo sapiens
MAVSAVFASSACFRFSRVDANRGLLMKCFI

SEQ ID NO: 67 - protein, 60 aa, Homo sapiens
MAWKPSRQGLLCDMTMLLSLLSLTAAPLRSKRRLSWVYDSYHSSSRTTEVPTLFWFCDQH

SEQ ID NO: 68 - protein, 24 aa, Homo sapiens
MAWSLFLRLDVGTRELIECSGSPT

SEQ ID NO: 69 - protein, 37 aa, Homo sapiens
MAYTKAASRLLLSMTRPKTVWSRSRVVQFQRWWRNWC

SEQ ID NO: 70 - protein, 13 aa, Homo sapiens
MCAKDSMLIWNAG

SEQ ID NO: 71 - protein, 21 aa, Homo sapiens
MCCCFHNKPLGLRTRLHLQSL

SEQ ID NO: 72 - protein, 12 aa, Homo sapiens
MCCLHQQSHFLR

SEQ ID NO: 73 - protein, 48 aa, Homo sapiens
MCCVLQLLYEGSLWNSASSGDGSLGGSLFFMLCRYGCNSDKFTSVSPN

SEQ ID NO: 74 - protein, 11 aa, Homo sapiens
MCDHASLILYF

SEQ ID NO: 75 - protein, 65 aa, Homo sapiens
MCEARNNKKSNNLIFKYLAGHLLASDSCHHVMIEAVGYLYRSVDLRVIHLGSSHSSIHGIHGILQ

SEQ ID NO: 76 - protein, 124 aa, Homo sapiens
MCEEWNSLSVKRHSRQVLPTPESPISSSRNSTSYCFAMTGASGAGNCGRAAGSALLRRCHRGPRPPGDAAGGEEDAGPGPRGCLARPPAHSLAGCREARLRREPGAAPARLGSARLGWREAVGG

SEQ ID NO: 77 - protein, 12 aa, Homo sapiens
MCFGVTIFPILY

SEQ ID NO: 78 - protein, 59 aa, Homo sapiens
MCHHAQLIFVCLVETGFRHVGQAGHEPLTSGGLPASASQIAGITGVSHCAQPMYFYFKS

SEQ ID NO: 79 - protein, 46 aa, Homo sapiens
MCHHARLIFVFYFVFLVETRFLHVGQAGLELPTSGICPPGPPKVLG

SEQ ID NO: 80 - protein, 11 aa, Homo sapiens
MCHHARQILYF

SEQ ID NO: 81 - protein, 11 aa, Homo sapiens
MCHHAWLILYF

SEQ ID NO: 82 - protein, 30 aa, Homo sapiens
MCHHDQLIFVFFVEMGFHHVGQDSLDPLTS

SEQ ID NO: 83 - protein, 57 aa, Homo sapiens
MCHHTKLIFVFLVETRFCHFGQAGLELLISGDPPASASKSAGITKHEPPRLTDCYNF

SEQ ID NO: 84 - protein, 25 aa, Homo sapiens
MCHYAWLIFVFLVETGFHQGLVSNP

SEQ ID NO: 85 - protein, 42 aa, Homo sapiens
MCICLFNPILLLYPYFTHFLIVIKWKTDLIIYKTLCQNRFND

SEQ ID NO: 86 - protein, 37 aa, Homo sapiens
MCIFLDFPEGTSFNVLAFLSFQHHCLEYFSCITLPFV

SEQ ID NO: 87 - protein, 21 aa, Homo sapiens
MCILLLLGGVPCRYLSSLVGL

SEQ ID NO: 88 - protein, 12 aa, Homo sapiens
MCISYCSTLGGT

SEQ ID NO: 89 - protein, 36 aa, Homo sapiens
MCLARHLILYFWDRHQCWAKANGQVIRVHHILIAVL

SEQ ID NO: 90 - protein, 13 aa, Homo sapiens
MCLMDALLDISIV

SEQ ID NO: 91 - protein, 24 aa, Homo sapiens
MCLSSFHSMYLISYDLLFFIITLT

SEQ ID NO: 92 - protein, 16 aa, Homo sapiens
MCLTCALKLSLYIMKL

SEQ ID NO: 93 - protein, 11 aa, Homo sapiens
MCLYSSALNIS

SEQ ID NO: 94 - protein, 19 aa, Homo sapiens
MCNDRMALHKDSVACQVRV

SEQ ID NO: 95 - protein, 32 aa, Homo sapiens
MCNGCSITENFVTIITLVKFPYTMDCLMVNKW

SEQ ID NO: 96 - protein, 54 aa, Homo sapiens
MCPKETEAELGEDNLNVSRCQPFQGRVHQEISLSSRASTCSLERLHFVPQAVHF

SEQ ID NO: 97 - protein, 22 aa, Homo sapiens
MCPKFNIAFLHLSSGQIFIIHL

SEQ ID NO: 98 - protein, 20 aa, Homo sapiens
MCPWSPGQCLAGIWLSVSVR

SEQ ID NO: 99 - protein, 46 aa, Homo sapiens
MCQCTWLIFFVFLVETAFHHVDQACLKLLTSGDTPPLAPQVLGLQV

SEQ ID NO: 100 - protein, 54 aa, Homo sapiens
MCRKLAIALIQEQPLSASVCLSLAQRKMDTEPTRASPSSVLWVLNGVFSANSEA

SEQ ID NO: 101 - protein, 29 aa, Homo sapiens
MCRPLGIKYSLRQHHCPHGAYIAALFLLY

SEQ ID NO: 102 - protein, 40 aa, Homo sapiens
MCRRTSSSVVCPKQTPDIKPFFFLDILEPSLLLSGESQCP

SEQ ID NO: 103 - protein, 13 aa, Homo sapiens
MCSCHDDIIIFFI

SEQ ID NO: 104 - protein, 26 aa, Homo sapiens
MCSEVKPIHYETLDVPALKIKNNSFK

SEQ ID NO: 105 - protein, 21 aa, Homo sapiens
MCSTNFGPEHQIYYSVIVDYR

SEQ ID NO: 106 - protein, 30 aa, Homo sapiens
MCSVRSISELDVTFMSLTSLDYPGPLPCIS

SEQ ID NO: 107 - protein, 16 aa, Homo sapiens
MCTAWKTRWSVTSLGG

SEQ ID NO: 108 - protein, 69 aa, Homo sapiens [sequence omitted]

SEQ ID NO: 109 - protein, 37 aa, Homo sapiens
MDCMFMSSQNSSVETLISKAMVLGGGANTISGPLGSE

SEQ ID NO: 110 - protein, 44 aa, Homo sapiens
MDEPLVISTPEPVLQMISLKKDAVIICAVQKPLIPRDRENNSFS

SEQ ID NO: 111 - protein, 25 aa, Homo sapiens
MDEPLVISTPEPVLQMISLLKHSEG

SEQ ID NO: 112 - protein, 25 aa, Homo sapiens
MDFSTKHPVFSLKHKCHHVTGSCLT

SEQ ID NO: 113 - protein, 90 aa, Homo sapiens
MDGQSTTSIHARKTRLILHHMAAHAITPRSYTRVTCHSSKSRGGCQGKLYLTSTLPDSLHSTQAGHSSHEGCNPPSPRLTTDSKNRKCVR

SEQ ID NO: 114 - protein, 35 aa, Homo sapiens
MDGRLLTRRLLTRVGSTRSLSPYLHKNCTGRISLM

SEQ ID NO: 115 - protein, 29 aa, Homo sapiens
MDIKKAYRPGAVVRVYNASTLGGRSGWIT

SEQ ID NO: 116 - protein, 23 aa, Homo sapiens
MDINGFSIFFIFVQFFSRIIAFL

SEQ ID NO: 117 - protein, 34 aa, Homo sapiens
MDKNEVSVQQIPINKIKWQGRGNPRKNILEHDHV

SEQ ID NO: 118 - protein, 24 aa, Homo sapiens
MDLHQSALGTSSSVTGGAPGADWP

SEQ ID NO: 119 - protein, 53 aa, Homo sapiens [sequence omitted]

SEQ ID NO: 120 - protein, 97 aa, Homo sapiens
MDNEPGHERKVFVPGLGLQENMALHILAGFTVCHTSFPHGILDLTDQLLPEGGAPPVGLLPGNVHACSPAPAARIPLGRHRRRLSHRARPKPGSRPQ

SEQ ID NO: 121 - protein, 14 aa, Homo sapiens
MDNQPLLFMHGRLV

SEQ ID NO: 122 - protein, 22 aa, Homo sapiens
MDPRHPVPQRAGFSPGSLRPCP

SEQ ID NO: 123 - protein, 48 aa, Homo sapiens
MDRSMLTMLGHSQKLLAMTTSMRLACRYRYSSLPRPRSMPSVRLRSRL

SEQ ID NO: 124 - protein, 65 aa, Homo sapiens [sequence omitted]

SEQ ID NO: 125 - protein, 90 aa, Homo sapiens [sequence omitted]

SEQ ID NO: 126 - protein, 12 aa, Homo sapiens
MDSWVFTRFLVL

SEQ ID NO: 127 - protein, 28 aa, Homo sapiens
MDTFGSAEQRPERYPSQRDIQGRTKLII

SEQ ID NO: 128 - protein, 11 aa, Homo sapiens
MDTFSDPSPGT

SEQ ID NO: 129 - protein, 13 aa, Homo sapiens
MDYLLLRFDRTYT

SEQ ID NO: 130 - protein, 28 aa, Homo sapiens
MEAKTDHLEVRDAMFSIGAISWGTVPCE

SEQ ID NO: 131 - protein, 18 aa, Homo sapiens
MECEAVLTFIIKMTSTSV

SEQ ID NO: 132 - protein, 74 aa, Homo sapiens [sequence omitted]

SEQ ID NO: 133 - protein, 14 aa, Homo sapiens
MEELGPGYVVILGL

SEQ ID NO: 134 - protein, 13 aa, Homo sapiens
MEEQIYTQGFLSD

SEQ ID NO: 135 - protein, 81 aa, Homo sapiens
MEESADDITAAETAPRPKKEIYTGQRYCRTIGKIMSASSVVLGSGSPYAVWFQSVDAPMAPMSMAGMAITRHPKAARKDST

SEQ ID NO: 136 - protein, 40 aa, Homo sapiens
MEFHHVGQADLKLLASSDSPALASQSAGITGPAYFCNNYE

SEQ ID NO: 137 - protein, 104 aa, Homo sapiens
MEFHHVGQAVLKLLISGDLPVSASQSAGITGVSHCAWPNVWLLLAMPFTELLFLTSYTYTCCKETNTKQDFSKTLKEERSSFLKNLIFLWHITMNSGVTSLLYN

SEQ ID NO: 138 - protein, 107 aa, Homo sapiens
MEFHHVVQAGFKLLTSGDPPALASQSARITGVSHCAQPEYIISLDSAGALDDQGIGHGCRSTFLLLFCFFLRQSLTCCPGWSAVTQSRLTVASTSGEQAILPPQPSE

SEQ ID NO: 139 - protein, 14 aa, Homo sapiens
MEFHPYEFPDILIQ

SEQ ID NO: 140 - protein, 19 aa, Homo sapiens
MEFLIHNRHSEMFGALTNE

SEQ ID NO: 141 - protein, 38 aa, Homo sapiens
MEFRHVGQVGLKLLGSSDSPTLASQSAGITGVSHCIQP

SEQ ID NO: 142 - protein, 34 aa, Homo sapiens
MEFRSLLPRLECTSRLIATPASQVQAILLPQSPE

SEQ ID NO: 143 - protein, 16 aa, Homo sapiens
MEFVSLSSLVCRSIGS

SEQ ID NO: 144 - protein, 33 aa, Homo sapiens
MEGASSCSCRKTFRVAGKAVTLYSSSINSNTLA

SEQ ID NO: 145 - protein, 171 aa, Homo sapiens
MEGCLHGGPQSQNFIHELKRPVSAARGSSYIQSCNTWSPRPDVHCVNNTRGAPICISDLLVRGWLIRSEGPQSEPFTHLHQLQEQSKTSRYVSSATNHSGNHSPSSFLCQSGGDLHLDSGSHHLGSLSCLYCCLLLLHLGLHWGLLHHHRSSDKFQWWLGIQHLSRESLRL

SEQ ID NO: 146 - protein, 24 aa, Homo sapiens
MEGGRKLSCRSLPFRHSSAFCVTA

SEQ ID NO: 147 - protein, 12 aa, Homo sapiens
MEGRLYYHVYRR

SEQ ID NO: 148 - protein, 30 aa, Homo sapiens
MEGTRQERNITWVLSPVACHNAPSTRFWVQ

SEQ ID NO: 149 - protein, 13 aa, Homo sapiens
MEHFHTAGGNVNY

SEQ ID NO: 150 - protein, 14 aa, Homo sapiens
MEHFYILITMAIKP

SEQ ID NO: 151 - protein, 77 aa, Homo sapiens
MEHSDTWNQMNTTSCFCNDPYCHAALGSWGHWTFGLVAYSPVLLVCSLAIPPEVAGRAGHWSLLWLQESLPVQSFSC

SEQ ID NO: 152 - protein, 11 aa, Homo sapiens
MEIPLFDIFSC

SEQ ID NO: 153 - protein, 18 aa, Homo sapiens
MEIYVFSDWFQKLPDYDI

SEQ ID NO: 154 - protein, 17 aa, Homo sapiens
MEKDLCLFGRNFCLLKF

SEQ ID NO: 155 - protein, 90 aa, Homo sapiens
MEKFWEAVWPLGILLSPNPFSSYTHHVITLGSFSVYLQEIHVGLFQWSPYIPGWSLWTASSLGSFLCFCPCLPFQRHLLWTFLPPCQKGN

SEQ ID NO: 156 - protein, 23 aa, Homo sapiens
MEKQLIKYLNPINLHVNDVNNTG

SEQ ID NO: 157 - protein, 87 aa, Homo sapiens
MELADKMEESADDITAAETAPRPKKEIYTGQRYCRTIGKIMSASSVVLGSGSPYAVWFQSVDAPMAPMSMAGMAITRHPKAARKDST

SEQ ID NO: 158 - protein, 13 aa, Homo sapiens
MELFRIPLKRNLS

SEQ ID NO: 159 - protein, 50 aa, Homo sapiens
MELILQPFFCYTEHSSRLNLRSVYWTCVGVYILFSHKCEMQRLNYLEHIK

SEQ ID NO: 160 - protein, 11 aa, Homo sapiens
MEMIESSCIKN

SEQ ID NO: 161 - protein, 25 aa, Homo sapiens
MENINVNKIHSIPESYSCYLKITYL

SEQ ID NO: 162 - protein, 31 aa, Homo sapiens
MENLKHISTSFSSNKITEINFNGFPQKENSF

SEQ ID NO: 163 - protein, 101 aa, Homo sapiens
MENLQRPVYDHLQVDAALRAPPAQLLPVDPRIHKQNAILQIYLQKASAALGRHPEQARHQLRQLQSQVLRDAAHEGAVFGLLGDRVVELTVPCLPGCEEKK

SEQ ID NO: 164 - protein, 224 aa, Homo sapiens [sequence omitted]

SEQ ID NO: 165 - protein, 12 aa, Homo sapiens
MENPVPLVWKQQ

SEQ ID NO: 166 - protein, 22 aa, Homo sapiens
MENQARMRFSFHYYIHTRVNQE

SEQ ID NO: 167 - protein, 40 aa, Homo sapiens
MEPMLLVMVTNVARARSSLLMESRFSLLIMLPKLDATADP

SEQ ID NO: 168 - protein, 40 aa, Homo sapiens
MEPMLLVMVTNVARARSSLLMESRFSLLIMLPKLVPVTLL

SEQ ID NO: 169 - protein, 33 aa, Homo sapiens
MEPQMVGKVGEVGVTNEVKLQQKGTDLQGIEKS

SEQ ID NO: 170 - protein, 17 aa, Homo sapiens
MEPTVCAYACRPSWPLR

SEQ ID NO: 171 - protein, 91 aa, Homo sapiens
MEQAPRADHAHCTLSEQLKFCLCMFILEGGMDARVQLLPPAPNKTVSQGSGPPGRGNCNERALSLSFVWHVPHCSHPCHCSCVTGLMLLFS

SEQ ID NO: 172 - protein, 45 aa, Homo sapiens
MEQHITTNTQVITGVTSTASSSCFSGPSSRLCFMYLFFTSRLPAQ

SEQ ID NO: 173 - protein, 17 aa, Homo sapiens
MERLLEKKKCWYDVFLP

SEQ ID NO: 174 - protein, 37 aa, Homo sapiens
MERSHKKMTPKGTTYVPQNCSSETFNGGEQGKASLRL

SEQ ID NO: 175 - protein, 49 aa, Homo sapiens
MESGPLDFKAPSATGCITSGKCLNLSEPLGNADFNLTGLGSWCPVRPLG

SEQ ID NO: 176 - protein, 15 aa, Homo sapiens
MESGSEMAFNTRALF

SEQ ID NO: 177 - protein, 27 aa, Homo sapiens
MESHSVTQAEVQWHHLGSLQPPPPGFK

SEQ ID NO: 178 - protein, 12 aa, Homo sapiens
MESSKFFSSSCS

SEQ ID NO: 179 - protein, 33 aa, Homo sapiens
METEFQYADGMKYRSLVQPISALTYTSGLCANA

SEQ ID NO: 180 - protein, 46 aa, Homo sapiens
METGFHHVDQAGLELLTSTDSPTSASQSAGITGMSHCAQPIFFFFF

SEQ ID NO: 181 - protein, 19 aa, Homo sapiens
MEVDTTHHDARMMGIIHYS

SEQ ID NO: 182 - protein, 53 aa, Homo sapiens
MEVTGRRQEVRRSKKNFILGVSYSFSVLLQQQQQLTLSLPSFSIPRTRLLTAS

SEQ ID NO: 183 - protein, 19 aa, Homo sapiens
MEWLCQQFLLPLLVSGSAG

SEQ ID NO: 184 - protein, 23 aa, Homo sapiens
MEWRVVESCHVGLSHSATPLPSV

SEQ ID NO: 185 - protein, 55 aa, Homo sapiens [sequence omitted]

SEQ ID NO: 186 - protein, 13 aa, Homo sapiens
MFCIFSRDGVSPC

SEQ ID NO: 187 - protein, 63 aa, Homo sapiens
MFFCACSIFFYLTASSPLAIKKFLKDVFFISFFSGGESFTLVAQAGVQRRDLGLLQPPPPRFK

SEQ ID NO: 188 - protein, 171 aa, Homo sapiens [sequence omitted]

SEQ ID NO: 189 - protein, 45 aa, Homo sapiens
MFFNIAVPSLGHHQTKLHFLFFNLWFIFFIITILWIFIISKGATW

SEQ ID NO: 190 - protein, 101 aa, Homo sapiens
MFFPQYQHLIDQQCVPRKRKLSWVKTILMSQGVSLSKEECTRRFLSAPGHPPAPSRGYTLYLRQSISRLPGGPGILAVHLPIPADNGVTEAGPLGAEYTEQ

SEQ ID NO: 191 - protein, 11 aa, Homo sapiens
MFFTFLYNSSC

SEQ ID NO: 192 - protein, 12 aa, Homo sapiens
MFFTFLYNSSCL

SEQ ID NO: 193 - protein, 37 aa, Homo sapiens
MFFTFLYNSSCSGTRPPFALRGPGILTPRSVAAAPGR

SEQ ID NO: 194 - protein, 85 aa, Homo sapiens
MFFTYIQASLSIVYCCIANHHTCSSFKRHKVISSQHPWTRSPGTVWRSCVLCSGTLKAKIHFGFQSVGWAGLSADSGEESTYKCI

SEQ ID NO: 195 - protein, 44 aa, Homo sapiens [sequence omitted]

SEQ ID NO: 196 - protein, 52 aa, Homo sapiens
MFHCYWFRCLSPQTLLCKCFSKGRTDWNCGSARSHSFQSHFFSAALSSCGTL

SEQ ID NO: 197 - protein, 18 aa, Homo sapiens
MFHQIQKQQVSVKLEQAF

SEQ ID NO: 198 - protein, 15 aa, Homo sapiens
MFHRRLQSVLLFGPE

SEQ ID NO: 199 - protein, 29 aa, Homo sapiens
MFHVHLRRMCILLLLGGVPCRYLSSLVGL

SEQ ID NO: 200 - protein, 52 aa, Homo sapiens
MFHVSQAGLQLLTSDYLPALASQSAGITGVSLHTRPMSDIFKTKKAWENLCQ

SEQ ID NO: 201 - protein, 23 aa, Homo sapiens
MFIFSTDGVSPCWSGWSRTPDLR

SEQ ID NO: 202 - protein, 15 aa, Homo sapiens
MFIIIDLKLLCRICQ

SEQ ID NO: 203 - protein, 37 aa, Homo sapiens
MFIVLRKSSLPLFIHHEEKFYHFSFLASIFPNTVQKL

SEQ ID NO: 204 - protein, 31 aa, Homo sapiens
MFIVYESDHFLKAAAICLGKGQDTMLGVHHS

SEQ ID NO: 205 - protein, 15 aa, Homo sapiens
MFKETYEHTSICYET

SEQ ID NO: 206 - protein, 17 aa, Homo sapiens
MFKSLCSYSQIYKNNFP

SEQ ID NO: 207 - protein, 98 aa, Homo sapiens
MFLETRFWRFALDRQGRARSTGLSGGPSRGPGRRTGGLPGAPHAPLTHWPRRLRCHGDRARTYSPPAAVRRLHEPRRQPASSPAGCACPGPEASLLRQ

SEQ ID NO: 208 - protein, 15 aa, Homo sapiens
MFLETRFWRLVRLQL

SEQ ID NO: 209 - protein, 14 aa, Homo sapiens
MFLFQLFRKIRQSL

SEQ ID NO: 210 - protein, 13 aa, Homo sapiens
MFLLEMGFHHVPC

SEQ ID NO: 211 - protein, 33 aa, Homo sapiens
MFLLTEVWTSESTVLECVCVPSQVCSTEGSSGK

SEQ ID NO: 212 - protein, 47 aa, Homo sapiens
MFLMLLLSKGYHLPIEIEDGQTLPEPNSVLEATLKCQLQIWSKIMYF

SEQ ID NO: 213 - protein, 34 aa, Homo sapiens
MFMSSQNSSVETLISKAMVLGGGANTISGPLGSE

SEQ ID NO: 214 - protein, 33 aa, Homo sapiens
MFNQVSVVRKTFSTLTTRIGLLTSMDPLMGYKV

SEQ ID NO: 215 - protein, 112 aa, Homo sapiens
MFPTSEMALPERALLSLRNSAWTAWEVSHSHGPARNSDKNGCALPTTTSLKSPLSPDAAKSPPPAGQDHPQLDPPQTPSLEVTLEPLEEASLLRKVTTGLLLTTDFRRWLHA

SEQ ID NO: 216 - protein, 50 aa, Homo sapiens
MFQCFRSTSSSASHLRVKKGCFLLIISPSKKVVRVGYSSVRPLIFKYPQR

SEQ ID NO: 217 - protein, 23 aa, Homo sapiens
MFQLNKILHKANIFPTNFFSSRS

SEQ ID NO: 218 - protein, 52 aa, Homo sapiens
MFQLSSNLEFILISPFEGEYNYRVNKSSTLVSGCNHTQTHTHTHTHTLSLSL

SEQ ID NO: 219 - protein, 18 aa, Homo sapiens
MFQNSEESFTFMKIKSLF

SEQ ID NO: 220 - protein, 19 aa, Homo sapiens
MFQRELLSFASGYLLERPF

SEQ ID NO: 221 - protein, 17 aa, Homo sapiens
MFQWWVFASSAQRQLEV

SEQ ID NO: 222 - protein, 92 aa, Homo sapiens
MFRANMELADKMEESADDITAAETAPRPKKEIYTGQRYCRTIGKIMSASSVVLGSGSPYAVWFQSVDAPMAPMSMAGMAITRHPKAARKDST

SEQ ID NO: 223 - protein, 46 aa, Homo sapiens
MFRCEDKSWQVTRKVQTSEIPNEVPENDWMLIDERRCMNHLITFIF

SEQ ID NO: 224 - protein, 42 aa, Homo sapiens
MFSDFCEERATTNAGSISQGNPAADDNSYTFIATFISVSLGM

SEQ ID NO: 225 - protein, 28 aa, Homo sapiens
MFSESKSMSGSVTCGRVVDTSHTHFFQS

SEQ ID NO: 226 - protein, 63 aa, Homo sapiens
MFSESTTPCPWANSLRESTVSLTTSLSKSKLNSLFRPRFSFLSLSSSRLLEVLLFISDSVLAR

SEQ ID NO: 227 - protein, 50 aa, Homo sapiens
MFSFNAHIRAMEPMLLVMVTNVARARSSLLMESRFSLLIMLPKLDATADP

SEQ ID NO: 228 - protein, 50 aa, Homo sapiens
MFSFNAHIRAMEPMLLVMVTNVARARSSLLMESRFSLLIMLPKLVPVTLL

SEQ ID NO: 229 - protein, 16 aa, Homo sapiens
MFSHVYMSGHMKMIPH

SEQ ID NO: 230 - protein, 30 aa, Homo sapiens
MFSICLIHTKVHMTFPVSSLVIIMQTALYY

SEQ ID NO: 231 - protein, 15 aa, Homo sapiens
MFSIGAISWGTVPCE

SEQ ID NO: 232 - protein, 15 aa, Homo sapiens
MFSLSSCQPILQFVH

SEQ ID NO: 233 - protein, 81 aa, Homo sapiens
MFSNRALSPFSVLDFVTVLGFPETFFPPVFSSFVILDAIFVPSFSFTSSCFRVLFILFLLVLDECPDAPNPSDFIFLLVER

SEQ ID NO: 234 - protein, 21 aa, Homo sapiens
MFSPRYVKMVKKYLKIQFSPL

SEQ ID NO: 235 - protein, 36 aa, Homo sapiens
MFSRDGVSPCWPGWSRTPDLRWSACLGLPNCWDYRR

SEQ ID NO: 236 - protein, 23 aa, Homo sapiens
MFSVKKGGTLPILREAGAPAGEE

SEQ ID NO: 237 - protein, 63 aa, Homo sapiens
MFSVKKGGTLPIRGPVPPPLASPRQALGGARSPARAVLGRDLEAGARAGEAAETPARRRQRRT

SEQ ID NO: 238 - protein, 60 aa, Homo sapiens
MFTAYLLLKEGERKAPAYITILLMERSHKKMTPKGTTYVPQNCSSETFNGGEQGKASLRL

SEQ ID NO: 239 - protein, 37 aa, Homo sapiens
MFTGGGGGGGGGRRGKLCMSNTGRGKGYCGIMGLFCL

SEQ ID NO: 240 - protein, 32 aa, Homo sapiens
MFTMIYSKNTLDILNEKIFFPKFRNLGYIQHI

SEQ ID NO: 241 - protein, 155 aa, Homo sapiens
MFTRLVLNSRLQVIRPPWPSNAGIIGMRHRTWLAFFLVRKFTIYPSLPPRSSFPVPTVDGSLGRGQNLPFRPSKIWSGFLCEVLKALWNQVHGTGSESQAVVSGGVGTFSGEQSRVPKRDLGCSLDGRLGICLEVAFALNAPYFTWGILKMLWRL

SEQ ID NO: 242 - protein, 16 aa, Homo sapiens
MFVHDFFFQRHNLTWS

SEQ ID NO: 243 - protein, 18 aa, Homo sapiens
MFVTQKWGWGGGMINKSA

SEQ ID NO: 244 - protein, 33 aa, Homo sapiens
MFVWFLDIGLAYFQPFYNFPAVSFLGEGDWLRF

SEQ ID NO: 245 - protein, 23 aa, Homo sapiens
MFWFSFNLTALVPPARHPSASNR

SEQ ID NO: 246 - protein, 15 aa, Homo sapiens
MFYIFRNKSDCIPFY

SEQ ID NO: 247 - protein, 18 aa, Homo sapiens
MFYLYTSNFYDTVYNKIL

SEQ ID NO: 248 - protein, 59 aa, Homo sapiens
MFYMYSMSILHWLQLQDDTRVELTPVGQDRINEWSEMGFCRQRGTSGCRCYHSMTSEHW

SEQ ID NO: 249 - protein, 13 aa, Homo sapiens
MGACLSYLSLCEG

SEQ ID NO: 250 - protein, 18 aa, Homo sapiens
MGAGGGGLTMLPRLVLNT

SEQ ID NO: 251 - protein, 55 aa, Homo sapiens
MGAPAWGPRARSPSARPTGGWAGSRPAETTLEVAKLGVQASSAGQSWVGEGSVPG

SEQ ID NO: 252 - protein, 19 aa, Homo sapiens
MGARERRLSGLLAVRSKLS

SEQ ID NO: 253 - protein, 32 aa, Homo sapiens
MGAVWMAGPAIGSSLGLGEGAVCSQHDLRRQG

SEQ ID NO: 254 - protein, 62 aa, Homo sapiens
MGAVWMAGPAIGSSLSGRRVGGGGARGRAPAGAERSRGRAAERGRRGEVRGQPEDVPGLSGT

SEQ ID NO: 255 - protein, 224 aa, Homo sapiens
MGCQQARRGLGMLLTPPASILLLTCISGAPSVRSARSPIACLSSRPDQAPAPAQPPPPFPPPPTPPPGSPRALAGLAVRLSAPRGREPSRSRGRGSGVGRREAAAPAGGWAGALRPRDRGCASLLLPPGPARSRRRRLCRWGRGRGRARSAAGPGPAGSGRACCSAPRVGRGAGAARVGTPRPPGPGPGPTAAAAACAVARRPLRLPRRLPLGLRALQRRGEGA

SEQ ID NO: 256 - protein, 57 aa, Homo sapiens
MGCQQARRGLGMLLTPPASILLLTLTAAVSCWVPKLEKSPWPRLGSGVDLGAGPGAG

SEQ ID NO: 257 - protein, 42 aa, Homo sapiens
MGCQQARRGLGMLLTPPASILLLTWASCCVPVQPKELSHPPG

SEQ ID NO: 258 - protein, 53 aa, Homo sapiens
MGCQQARRGLGMLLTPPASILLLTWVRWRWEANRLASGGLGCGSLSVAVPACT

SEQ ID NO: 259 - protein, 151 aa, Homo sapiens
MGCQQARRGLGMLLTPPASILLLTWVRWRWEANRLASGGLGCGSLSVAVPACTRVGWVSGEYSWAGLSLGWTQSPSLPVGTGASGPVGAGGVPGAPSARGSAPGRHPPARLPPVPAPASVPAPQGSAPRWWPRRRARQGGRVYARESAQRV

SEQ ID NO: 260 - protein, 16 aa, Homo sapiens
MGCWLVFNSWLSEKAK

SEQ ID NO: 261 - protein, 35 aa, Homo sapiens
MGDNVRASFRRLGTFSQEASTELRLKEANSVLKFL

SEQ ID NO: 262 - protein, 74 aa, Homo sapiens
MGEEFSTLTAFVPSYTSTTILAQMTITISSLSEGSSTFITFTAFTWSLHPWISAQMSLLGVVLVFNAMFFPIFS

SEQ ID NO: 263 - protein, 30 aa, Homo sapiens
MGFCHVGQAGLELLTSGDPLALPKVLGLQA

SEQ ID NO: 264 - protein, 16 aa, Homo sapiens
MGFHCVGQGGLDFLTP

SEQ ID NO: 265 - protein, 16 aa, Homo sapiens
MGFHCVSQDGLDLLTS

SEQ ID NO: 266 - protein, 16 aa, Homo sapiens
MGFHCVSQDGLHLLTS

SEQ ID NO: 267 - protein, 13 aa, Homo sapiens
MGFHHIGLKLLTS

SEQ ID NO: 268 - protein, 16 aa, Homo sapiens
MGFHHVCQDGLNLLTS

SEQ ID NO: 269 - protein, 42 aa, Homo sapiens
MGFHHVDQAGLELLTSGDLPTLASQSAGITGVSHRTQPKSCF

SEQ ID NO: 270 - protein, 16 aa, Homo sapiens
MGFHHVGQAGLDLLTS

SEQ ID NO: 271 - protein, 42 aa, Homo sapiens
MGFHHVGQAGLELLASGDPPTSASQSAWITGMSHCAQLAFVI

SEQ ID NO: 272 - protein, 16 aa, Homo sapiens
MGFHHVGQAGLELLTL

SEQ ID NO: 273 - protein, 50 aa, Homo sapiens
MGFHHVGQAGLELLTSGDPPTTASQSAGITGMSHCARPHFLLLCFFGFLF

SEQ ID NO: 274 - protein, 51 aa, Homo sapiens
MGFHHVGQAGLELLTSSDLPTTASQSAGITGMSHSAQSGNTFKCLILPYVE

SEQ ID NO: 275 - protein, 54 aa, Homo sapiens
MGFHHVGQAGLEPLTSGDPPASASQSAGITGISHRPQPIVKVFSINNSQMLSHR

SEQ ID NO: 276 - protein, 16 aa, Homo sapiens
MGFHHVGQAGLKLLTL

SEQ ID NO: 277 - protein, 28 aa, Homo sapiens
MGFHHVGQAGLKLLTSGDPLGHLSLPEC

SEQ ID NO: 278 - protein, 40 aa, Homo sapiens
MGFHHVGQAGLKLLTSRDPPTLASQNAGITGVSPDAWHVS

SEQ ID NO: 279 - protein, 29 aa, Homo sapiens
MGFHHVGQAGLKLPSSGNPPAVDSQSVGK

SEQ ID NO: 280 - protein, 15 aa, Homo sapiens
MGFHHVGQARLELLT

SEQ ID NO: 281 - protein, 38 aa, Homo sapiens
MGFHHVGQAVLERLTSSDLPTSASQSAGMSDMSPRAQP

SEQ ID NO: 282 - protein, 43 aa, Homo sapiens
MGFHHVGQDGLDLLTHDPPALASQSARITGVSHCAWPKITIYF

SEQ ID NO: 283 - protein, 16 aa, Homo sapiens
MGFHHVGQDGLDLLTL

SEQ ID NO: 284 - protein, 16 aa, Homo sapiens
MGFHHVGQDGLDLLTS

SEQ ID NO: 285 - protein, 16 aa, Homo sapiens
MGFHHVGQDGLELLTS

SEQ ID NO: 286 - protein, 44 aa, Homo sapiens
MGFHHVGQDGLELLTSGEPPHSASRSAGITGMSHCAQPGNTIDK

SEQ ID NO: 287 - protein, 16 aa, Homo sapiens
MGFHHVGQDSLDPLTS

SEQ ID NO: 288 - protein, 56 aa, Homo sapiens
MGFHHVGQTNLELLTSGDPPALASQSVGITGVSHHPSRLPFICNSHMYNVVRKTNN

SEQ ID NO: 289 - protein, 77 aa, Homo sapiens
MGFHHVGWAGLELLTSNDLPTPTSQIAGITGISPHTQPDHICFRKAPFHAFTSSSFFFVLFLFFFLRWGLAMLPKLV

SEQ ID NO: 290 - protein, 16 aa, Homo sapiens
MGFHHVSEDGLDLQTL

SEQ ID NO: 291 - protein, 11 aa, Homo sapiens
MGFHHVSQAAL

SEQ ID NO: 292 - protein, 16 aa, Homo sapiens
MGFHHVSQDGLDLLTS

SEQ ID NO: 293 - protein, 16 aa, Homo sapiens
MGFHHVSQDGLNLLIL

SEQ ID NO: 294 - protein, 39 aa, Homo sapiens
MGFHHVVKAGLKLLTSGDPPIWVGLPKCWDYRCEPLRPA

SEQ ID NO: 295 - protein, 37 aa, Homo sapiens
MGFHLAQAGWELLSSGNLPTSASQSAGITGVSHRARP

SEQ ID NO: 296 - protein, 16 aa, Homo sapiens
MGFHPLGQAGLELLTS

SEQ ID NO: 297 - protein, 16 aa, Homo sapiens
MGFHRVSQDFLDLLTS

SEQ ID NO: 298 - protein, 16 aa, Homo sapiens
MGFHRVSQDGLDLLTL

SEQ ID NO: 299 - protein, 16 aa, Homo sapiens
MGFHRVSQDGLNLLTS

SEQ ID NO: 300 - protein, 16 aa, Homo sapiens
MGFHRVSQNGLDLLTS

SEQ ID NO: 301 - protein, 13 aa, Homo sapiens
MGFHYVARLVSNS

SEQ ID NO: 302 - protein, 16 aa, Homo sapiens
MGFHYVGQAGLELLTS

SEQ ID NO: 303 - protein, 42 aa, Homo sapiens
MGFHYVGQDGLELLTSRSACLGLPQCWDYMREPLRPAFQLHF

SEQ ID NO: 304 - protein, 16 aa, Homo sapiens
MGFHYVGQTGLKLVTS

SEQ ID NO: 305 - protein, 31 aa, Homo sapiens
MGFLCVGQAGLRLQPQVICLPQPPKVLGLQA

SEQ ID NO: 306 - protein, 61 aa, Homo sapiens
MGFLHIGQAGLKLPTSGDPPASASQTAGITGVSHHAQPVLKILMNWPGAVADTCNPGTLGG

SEQ ID NO: 307 - protein, 43 aa, Homo sapiens
MGFLHVEAGLELLTSGDPPTSASQSAGITGVSHCAPLGANILK

SEQ ID NO: 308 - protein, 67 aa, Homo sapiens
MGFLHVGQAGLELPTSGDWPASASQSAEITGVSHHAWPLFPSLLPVSGTRMSAPVRASACSQLAPSY

SEQ ID NO: 309 - protein, 45 aa, Homo sapiens
MGFLHVGQAGLKLPTSGDPCLAYFFFSFSFSFSFLSFFSFFFFKR

SEQ ID NO: 310 - protein, 43 aa, Homo sapiens [sequence omitted]

SEQ ID NO: 311 - protein, 45 aa, Homo sapiens
MGFLLVGLAGLKLPTSGDLPASASQSAGITGVSHHAWLGIHSYSR

SEQ ID NO: 312 - protein, 47 aa, Homo sapiens
MGFLPVGQAGLELPTSGDPPTLASQSAGIIGVSHCARPLPGILTRGR

SEQ ID NO: 313 - protein, 16 aa, Homo sapiens
MGFPRVSQDGHDLLIS

SEQ ID NO: 314 - protein, 16 aa, Homo sapiens
MGFQHVGQDGLDLLTS

SEQ ID NO: 315 - protein, 16 aa, Homo sapiens
MGFQHVGQDGLHLLTS

SEQ ID NO: 316 - protein, 31 aa, Homo sapiens
MGFRHVGQAGLELLPSGDLPAWPPKVLRLQA

SEQ ID NO: 317 - protein, 57 aa, Homo sapiens
MGFRHVGQAGLELLTSGDPPASDSQSVGITGMSHCTQPVIAFSRNLSGINSLTLSKE

SEQ ID NO: 318 - protein, 38 aa, Homo sapiens
MGFRHVGQAGLELLTSGDPPTSASQNAGIIGMNHCAWP

SEQ ID NO: 319 - protein, 48 aa, Homo sapiens
MGFRHVGQAGLELLTSGYPSTLTSQSAGITGMSHHARPRFWSILNLGW

SEQ ID NO: 320 - protein, 38 aa, Homo sapiens
MGFRHVGQAGLKLLTSGDPPVSASQSAGITGVSHRARP

SEQ ID NO: 321 - protein, 31 aa, Homo sapiens
MGFRPEKILTIPIQILVARLILPCSVNIHPW

SEQ ID NO: 322 - protein, 77 aa, Homo sapiens [sequence omitted]

SEQ ID NO: 323 - protein, 68 aa, Homo sapiens [sequence omitted]

SEQ ID NO: 324 - protein, 16 aa, Homo sapiens
MGFYHVSQDGLDLLTL

SEQ ID NO: 325 - protein, 49 aa, Homo sapiens
MGFYNVGQDGLDLLTHDLPTSASQSAGITGVSHCAHSPKALDRCPIGEN

SEQ ID NO: 326 - protein, 30 aa, Homo sapiens
MGGCSVPGWVAGTAAGMLLVPRMAGAEMSM

SEQ ID NO: 327 - protein, 26 aa, Homo sapiens
MGGDTWRRLGRGNWELGLILLLFQHV

SEQ ID NO: 328 - protein, 13 aa, Homo sapiens
MGGNMVGSQLKLS

SEQ ID NO: 329 - protein, 29 aa, Homo sapiens
MGGWSAWGARRPLTAGPAQHKRAQAHTHT

SEQ ID NO: 330 - protein, 24 aa, Homo sapiens
MGIIWVHFRQTRMQMTASSYHFPP

SEQ ID NO: 331 - protein, 56 aa, Homo sapiens
MGILHVSQAGLELLTSGDPPALASQSAGITGLSYRAQPLLFFTQVGFPLVCHLPNS

SEQ ID NO: 332 - protein, 19 aa, Homo sapiens
MGILVLFLISVGKHSVFHH

SEQ ID NO: 333 - protein, 25 aa, Homo sapiens
MGKAGEHMSVVGLSLSSGATVFKGV

SEQ ID NO: 334 - protein, 24 aa, Homo sapiens
MGKKGLPHFGPQRRKGQRRWPERA

SEQ ID NO: 335 - protein, 45 aa, Homo sapiens
MGKRLSEGGRRDWVKLSRRGKNTQRTLQPMGIRRLGWFRRKVEQA

SEQ ID NO: 336 - protein, 48 aa, Homo sapiens
MGKTVKHKRNAIYSRNCLFQLLTAHIKLLFRKMENVSSTIQSTYNLFF

SEQ ID NO: 337 - protein, 15 aa, Homo sapiens
MGKYICIDVYLHIKN

SEQ ID NO: 338 - protein, 11 aa, Homo sapiens
MGLFSGLTEPD

SEQ ID NO: 339 - protein, 26 aa, Homo sapiens
MGLGSKVAITPKSSHTRCKMKRATQR

SEQ ID NO: 340 - protein, 81 aa, Homo sapiens
MGLHHAGHAGLELLTSSDRSASASQSIGLTGVSHHAWPNGRHLYFIFFILSVHTQPILLGSLFLICRRYNPHANYLPCWML

SEQ ID NO: 341 - protein, 11 aa, Homo sapiens
MGLQVPATKPG

SEQ ID NO: 342 - protein, 52 aa, Homo sapiens
MGLRDRAWRAACMGAPNPRISFMNSRGLFPQHAAAHTYKAATRGHHVLMSTV

SEQ ID NO: 343 - protein, 12 aa, Homo sapiens
MGLYISRVRIQN

SEQ ID NO: 344 - protein, 12 aa, Homo sapiens
MGNCWSWVDSLD

SEQ ID NO: 345 - protein, 116 aa, Homo sapiens
MGPKLKHASGNEAQEDNGEEGDIVDSVLGLHSWDEGRTPDIILDRRTHNDTDSLFLTLLGHGCLPLGPELGHRLMPRGAGHLRPGRIGPNRQPPLPGPSLGWRAASEGPVTGIRAV

SEQ ID NO: 346 - protein, 30 aa, Homo sapiens
MGQTWEIMRMIEFTNVAKLREFKSYPVSSF

SEQ ID NO: 347 - protein, 25 aa, Homo sapiens
MGQVSYLELLQNFFSSQELNASTSQ

SEQ ID NO: 348 - protein, 128 aa, Homo sapiens
MGRDDLNLRGGAGAVLLQVELHEVERELWDLADGPVLAPACAWPWSAWPAMRALGAQEALGQQALGQAAAAALGQELGQVLEVENEHDDSPVLVLHGHHIYQAAEAGGILAVVEDVHLALLSPQQGLR

SEQ ID NO: 349 - protein, 112 aa, Homo sapiens
MGRDDLNLRGGAGAVLLQVELHEVERELWDLADGPVLAPACAWPWSAWPAMRALGAQEALGQQALGQAAAAALGQELGQVLEVENEHDDSPVLVLHGHHIYQAAEAGGSTRE

SEQ ID NO: 350 - protein, 174 aa, Homo sapiens
MGRGARCGPRRPGCSPAGPSTRSPPPRPWNRGGAAPAGQGLRRPPAIVERRRAGPGPRRRAGGPGRLQPAPRSPGHLQPRAPAPLSPACQSRNPAAAAAADGAAGRRRRRRWRWRRRQAGEGVGVQGRPRGPRGGRAAQRGPGRGAAGRGAPGALPALLQCHGAPAEPPGLELG

SEQ ID NO: 351 - protein, 15 aa, Homo sapiens
MGSAGISPRKGMSIF

SEQ ID NO: 352 - protein, 15 aa, Homo sapiens
MGSCYVDQAGNLGLE

SEQ ID NO: 353 - protein, 54 aa, Homo sapiens
MGSFGILLWYSLSCSVVVKSVCTLGSLRKNFKSMLMPGNSRTIMITLSMELRNG

SEQ ID NO: 354 - protein, 67 aa, Homo sapiens [sequence omitted]

SEQ ID NO: 355 - protein, 43 aa, Homo sapiens
MGSRHVGQVGLGLLTSGDPPVSASQSAGITGISHCARPVFVVF

SEQ ID NO: 356 - protein, 28 aa, Homo sapiens
MGSTFNQAGHRLSLPSHGLEAQQAGFAL

SEQ ID NO: 357 - protein, 28 aa, Homo sapiens
MGTWEGSCITVEWWVSPAGAGGPRGRAL

SEQ ID NO: 358 - protein, 16 aa, Homo sapiens
MGVHHVAQNGLNLLAS

SEQ ID NO: 359 - protein, 11 aa, Homo sapiens
MGVSPCWSGWS

SEQ ID NO: 360 - protein, 17 aa, Homo sapiens
MGVSVDLTVYCILVLVV

SEQ ID NO: 361 - protein, 41 aa, Homo sapiens
MGWCPGWNWFQDPRKHQNPQMPLYKMATVFAYHQHTSPYIL

SEQ ID NO: 362 - protein, 13 aa, Homo sapiens
MGYRLFTLQTEYV

SEQ ID NO: 363 - protein, 18 aa, Homo sapiens
MHAAIMEHFHTAGGNVNY

SEQ ID NO: 364 - protein, 13 aa, Homo sapiens
MHATLITSRGSFS

SEQ ID NO: 365 - protein, 22 aa, Homo sapiens
MHCPSGWWPHSGRCPRRSGRGW

SEQ ID NO: 366 - protein, 16 aa, Homo sapiens
MHCRNMEIPLFDIFSC

SEQ ID NO: 367 - protein, 11 aa, Homo sapiens
MHFKSLFYQLN

SEQ ID NO: 368 - protein, 13 aa, Homo sapiens
MHFLCQSVLENIG

SEQ ID NO: 369 - protein, 11 aa, Homo sapiens
MHGCLNSDDKN

SEQ ID NO: 370 - protein, 11 aa, Homo sapiens
MHHHALLILYF

SEQ ID NO: 371 - protein, 11 aa, Homo sapiens
MHHHAQLILYF

SEQ ID NO: 372 - protein, 57 aa, Homo sapiens
MHHHARLIFVFLLETGFRHVHQAGLELLTSGDPPTSASQSAGITGMSHCALIIFYFF

SEQ ID NO: 373 - protein, 11 aa, Homo sapiens
MHHHARLILYF

SEQ ID NO: 374 - protein, 45 aa, Homo sapiens
MHHHAWLIFCIFSRDRVSPCWPGWSRTPDLVIRLLRPPKVLGLQA

SEQ ID NO: 375 - protein, 79 aa, Homo sapiens
MHHHAWLIFVFLVETGFLHVGQAGLKLLTSGDPPASASQSAGITGLSHCAWPFLAFKIAMSSLQNSPVARYDHETHVIK

SEQ ID NO: 376 - protein, 11 aa, Homo sapiens
MHHHAWLILYS

SEQ ID NO: 377 - protein, 58 aa, Homo sapiens
MHHHTQLIFVFFSRDGGRGEVSLCWPGWFQTPDLRCSTCLGLPKSWDYRHEPLCPAYL

SEQ ID NO: 378 - protein, 66 aa, Homo sapiens [sequence omitted]

SEQ ID NO: 379 - protein, 40 aa, Homo sapiens
MHHHTQVIFVFLVETGFHHVGQAGLKLLTSLSICLGLPKC

SEQ ID NO: 380 - protein, 11 aa, Homo sapiens
MHHHTRLILYF

SEQ ID NO: 381 - protein, 16 aa, Homo sapiens
MHHKSTFLKDKEHNKK

SEQ ID NO: 382 - protein, 11 aa, Homo sapiens
MHHQAWLILYF

SEQ ID NO: 383 - protein, 20 aa, Homo sapiens
MHHRARLIFCIFSRDGVSPC

SEQ ID NO: 384 - protein, 17 aa, Homo sapiens
MHIAFTMPYSQINIIFF

SEQ ID NO: 385 - protein, 21 aa, Homo sapiens
MHLRISAQINIHIPMRTGAFI

SEQ ID NO: 386 - protein, 14 aa, Homo sapiens
MHLYFSLCAVVMMT

SEQ ID NO: 387 - protein, 48 aa, Homo sapiens
MHPLAKHAVFSKERNRCSSYRHCFSGTIHIPYGEGHLGIPGQVRVFYW

SEQ ID NO: 388 - protein, 11 aa, Homo sapiens
MHQPWLIFLYF

SEQ ID NO: 389 - protein, 28 aa, Homo sapiens
MHRRTTKWSLVSLVYRLFNARYQGNIDF

SEQ ID NO: 390 - protein, 12 aa, Homo sapiens
MHSLGKSAKSRK

SEQ ID NO: 391 - protein, 12 aa, Homo sapiens
MHSYYRIDIIQI

SEQ ID NO: 392 - protein, 22 aa, Homo sapiens
MHTGFSTICSFRHPLGMLECIP

SEQ ID NO: 393 - protein, 59 aa, Homo sapiens
MHTISVPPRAQGGGGNTVSLDLLQQWSLTIVTWKYALVCDQVCLHSNLLFKVGALNPFM

SEQ ID NO: 394 - protein, 29 aa, Homo sapiens
MHTYIGFGTDSTPLKLEEKQGPLAGLNMM

SEQ ID NO: 395 - protein, 11 aa, Homo sapiens
MHVGCIIVSVK

SEQ ID NO: 396 - protein, 18 aa, Homo sapiens
MHWAHRCSQASSSCMWGK

SEQ ID NO: 397 - protein, 26 aa, Homo sapiens
MHWSPWLPKQDSQLGAHFLQRFLSAW

SEQ ID NO: 398 - protein, 16 aa, Homo sapiens
MHYNLKYIILHKQPKG

SEQ ID NO: 399 - protein, 123 aa, Homo sapiens
MHYSYKVPPLCELSDESELRSSDESYRQLHHIRTASYLCGFLDVYTSLISERSMLYRWSIDRGFLQVDFSCGKHTVSSNNKFLYIYYIHSTFLPLNLSVGLLDISPQHTVEGLPPLGYKNAEL

SEQ ID NO: 400 - protein, 30 aa, Homo sapiens
MIACPPSGKLASAVWPAAPLGSHVTSPMTS

SEQ ID NO: 401 - protein, 27 aa, Homo sapiens
MIATWLNQLKNSSQLWVLSNHALRKDR

SEQ ID NO: 402 - protein, 22 aa, Homo sapiens
MICLIIISLNFPQKTKRVRLPP

SEQ ID NO: 403 - protein, 13 aa, Homo sapiens
MICLLLGSRRKTF

SEQ ID NO: 404 - protein, 15 aa, Homo sapiens
MICLPQPPKVVGLQA

SEQ ID NO: 405 - protein, 15 aa, Homo sapiens
MICPPPPPKLLGLQA

SEQ ID NO: 406 - protein, 15 aa, Homo sapiens
MICPPQPPKVLGLQA

SEQ ID NO: 407 - protein, 15 aa, Homo sapiens
MICPPRPPKVLGLQV

SEQ ID NO: 408 - protein, 82 aa, Homo sapiens
MICSLCGSRSCLPPGLLLLHVGEVDLREVADDLQPLRVQLLLAAVPVAAVLLAQLAVVEELREEPVEEEDGKLACEEASCRN

SEQ ID NO: 409 - protein, 39 aa, Homo sapiens
MICSSWDEFISPKHWSPGLVICNQMMPSSALLFSSSLRL

SEQ ID NO: 410 - protein, 14 aa, Homo sapiens
MICVAKDRAVGQYS

SEQ ID NO: 411 - protein, 74 aa, Homo sapiens
MIDIYHSHLQRVKWNGCVSSFCFLCLFQVQQGRCKQRVIDEMLHIVLLTLLLGLGAHLIGYILPISKATVHHSF

SEQ ID NO: 412 - protein, 12 aa, Homo sapiens
MIDIYHSHLQSM

SEQ ID NO: 413 - protein, 21 aa, Homo sapiens
MIEFTNVAKLREFKSYPVSSF

SEQ ID NO: 414 - protein, 63 aa, Homo sapiens
MIFFFFFFFLRWSFALCCPGWSAHLGSLQPLPPRFKRFSCLSLPSSWDYRHAPSRLANFVFFF

SEQ ID NO: 415 - protein, 20 aa, Homo sapiens
MIFFIHSNGHMKKIFTFFHH

SEQ ID NO: 416 - protein, 12 aa, Homo sapiens
MIFHMLVAVTYI

SEQ ID NO: 417 - protein, 252 aa, Homo sapiens
MIFLSLVLFWCFGEPESSLPLKLGDWGAAPSHGRSDTNDGFLIYGVTSRMNLTSSSTSLPARFSACTAWSWVAWRRSVPFTDRMASPSRSARLWSAASPGKILEMRIGIRFSRPPLMLMPRPPASCFTTRTRRTGGDAPASPAGPRGGAGGLGGPRPRLGLPGSESPAPPPFGRPLKAAAAGPRAGSSSAAAASPVRLRLSPLSSATTRTQRSLRSSSTSPALVARVHTAMAGPAPAAAVAAATLIPVRQPR

SEQ ID NO: 418 - protein, 50 aa, Homo sapiens
MIGITYTKAAKRSVSVLKKLRISQDAKPRSGQEMSHPPRAASHKDRKCAY

SEQ ID NO: 419 - protein, 18 aa, Homo sapiens
MIGKGFVILITSVSLFPP

SEQ ID NO: 420 - protein, 134 aa, Homo sapiens [sequence omitted]

SEQ ID NO: 421 - protein, 15 aa, Homo sapiens
MIHLPRPPKVLGLQA

SEQ ID NO: 422 - protein, 15 aa, Homo sapiens
MIHLPRPPRVLRLQA

SEQ ID NO: 423 - protein, 15 aa, Homo sapiens
MIHLPWPPKVLGLQA

SEQ ID NO: 424 - protein, 15 aa, Homo sapiens
MIHLPWPPKVLGLQV

SEQ ID NO: 425 - protein, 15 aa, Homo sapiens
MIHPPQPPKMLGLQV

SEQ ID NO: 426 - protein, 15 aa, Homo sapiens
MIHPPQPPKVLGLQA

SEQ ID NO: 427 - protein, 15 aa, Homo sapiens
MIHPPWPPKVLGLQA

SEQ ID NO: 428 - protein, 69 aa, Homo sapiens
MIHPPWPPKVPPLPACVWYFSMACNFLYTPSFFLRLFCQQPKMEKAALCQGSPKTVKSCESQMFTFNFF

SEQ ID NO: 429 - protein, 12 aa, Homo sapiens
MIHWPSSDIITC

SEQ ID NO: 430 - protein, 56 aa, Homo sapiens
MIKGLLCLHVATRSPGNGESSKDAVFLPLLHPYKSKSRIKVQLMKRSLVLIYLAKF

SEQ ID NO: 431 - protein, 19 aa, Homo sapiens
MIKNPCSQRLRWLSLNEPC

SEQ ID NO: 432 - protein, 26 aa, Homo sapiens
MIKSLIIFTAFVRFLSCMDSLMNSKS

SEQ ID NO: 433 - protein, 13 aa, Homo sapiens
MIKSTYCKRESNI

SEQ ID NO: 434 - protein, 50 aa, Homo sapiens
MIKYHPTTYNVQNSKLRCFSFYCVWFCTKIKCIRQNTIKEWKSSYLFYPL

SEQ ID NO: 435 - protein, 16 aa, Homo sapiens
MILGWAWWLMTVILVL

SEQ ID NO: 436 - protein, 20 aa, Homo sapiens
MILRKKKMRTRAHEQSPILK

SEQ ID NO: 437 - protein, 31 aa, Homo sapiens
MILSVDVYPQAFQPGLLYVYILKICQNSSNN

SEQ ID NO: 438 - protein, 18 aa, Homo sapiens
MILVVFQQTLFMNTKYSC

SEQ ID NO: 439 - protein, 51 aa, Homo sapiens
MILYFFSRDEVSTGHVGQAGLKLPTSGDPPTSASQSAGITHLSHHAQTVNH

SEQ ID NO: 440 - protein, 44 aa, Homo sapiens
MILYLSSPPHPSLTSPFFPSLLLKKGKKRKKEVHCKMEKRGMEG

SEQ ID NO: 441 - protein, 33 aa, Homo sapiens
MINPRCSRNRKCSGGISYIIMIVKSMKLQGRRV

SEQ ID NO: 442 - protein, 64 aa, Homo sapiens
MIPCFVMLYEGFCWGGRRCQNKPQFIRNLWINVNKYFSPSLWCFLKFMHRKNIKKFMCKIKAVP

SEQ ID NO: 443 - protein, 95 aa, Homo sapiens
MIPCFVMLYEGFCWGGRRCQNKPQFIRNLWINVNKYFSPSLWCFLKFMHRKNIKKFMCKIKAVPFWNIVQISVPGNWNPRLSDTFHIHWGSSISL

SEQ ID NO: 444 - protein, 80 aa, Homo sapiens
MIPCFVMLYEGFCWGGRRCQNKPQFIRNLWINVNKYFSPSLWCFLKFMHRKNIKKFMCKIKAVPSTRCTEMSQFFSTDPS

SEQ ID NO: 445 - protein, 61 aa, Homo sapiens
MIPCFVMLYEGFCWGGRRCQNKPQFIRNLWINVNKYFSPSLWCFLLEHRADLGTRKLESQT

SEQ ID NO: 446 - protein, 49 aa, Homo sapiens
MIPCFVMLYEGFCWGGRRCQNKPQFIRNLWINVNKYFSPSLWCFLYQMY

SEQ ID NO: 447 - protein, 18 aa, Homo sapiens
MIPLGGFSKTNRLSQRPT

SEQ ID NO: 448 - protein, 19 aa, Homo sapiens
MIQFHPANTTCEHISGIFC

SEQ ID NO: 449 - protein, 87 aa, Homo sapiens [sequence omitted]

SEQ ID NO: 450 - protein, 25 aa, Homo sapiens
MIQMMPSAVSKATEHLKRFRSYLLI

SEQ ID NO: 451 - protein, 38 aa, Homo sapiens
MIQNFSMFTMIYSKNTLDILNEKIFFPKFRNLGYIQHI

SEQ ID NO: 452 - protein, 22 aa, Homo sapiens
MIQNLPGLLPVHCFYFSLDKKK

SEQ ID NO: 453 - protein, 12 aa, Homo sapiens
MIQYTIKYFKKI

SEQ ID NO: 454 - protein, 15 aa, Homo sapiens
MIRCLRPPKVLRLEA

SEQ ID NO: 455 - protein, 23 aa, Homo sapiens
MIRKNRGFKPLGGDEIIRPFIFM

SEQ ID NO: 456 - protein, 15 aa, Homo sapiens
MIRPPQPPKVLGLQA

SEQ ID NO: 457 - protein, 15 aa, Homo sapiens
MIRPPQPPKVLGLQV

SEQ ID NO: 458 - protein, 15 aa, Homo sapiens
MIRPPRLPKVLGLQA

SEQ ID NO: 459 - protein, 12 aa, Homo sapiens
MIRPPRPPKVLG

SEQ ID NO: 460 - protein, 15 aa, Homo sapiens
MIRPPWPPKMLGLQA

SEQ ID NO: 461 - protein, 15 aa, Homo sapiens
MIRPPWPPKVLGLQV

SEQ ID NO: 462 - protein, 21 aa, Homo sapiens
MISAHCNLHLLGSSNPPTSAS

SEQ ID NO: 463 - protein, 193 aa, Homo sapiens
MISASMLGSKGSVSVKSSSHTVSTHSSLRSSGHQGCRPLPRPRNATMIPGHRLAAAVLNFQSSLPRARRVVPRPARPGGAMSFFGFGQSVEVEILLNDAESRKRAEHKTEDGKKEKYFLFYDGETVSGKVSLALKNPNKRLEHQGIKIEFIGQIGESTPGTPSPSADSRPGSRVIQGPAPPARPVTVACQLQS

SEQ ID NO: 464 - protein, 119 aa, Homo sapiens
MISHADSFTRSNLKFPLGRHDLGISPRNLDSSIQAGPVMGLHDVPAIGSVCSHTTVIWTLGPWEAVGRPTKGVPICPHEGILLLHAKPGVLVAHHVHYPFTGVPQIGLCRPSIVLENFT

SEQ ID NO: 465 - protein, 16 aa, Homo sapiens
MISIRAPFISHTHLLE

SEQ ID NO: 466 - protein, 83 aa, Homo sapiens
MISIRAPFISSTVRRGRCSVPSSNLSFTADERPWKQRRMLSMTAAVSRDAMLGGAHSSSVAPSLLCSHRPVSLSRMDAILGES

SEQ ID NO: 467 - protein, 47 aa, Homo sapiens [sequence omitted]

SEQ ID NO: 468 - protein, 29 aa, Homo sapiens
MISLKKDAVIICAVQKPLIPRDRENNSFS

SEQ ID NO: 469 - protein, 12 aa, Homo sapiens
MISLLKFFDCPH

SEQ ID NO: 470 - protein, 20 aa, Homo sapiens
MITHTHSLQPSYQFPLECDP

SEQ ID NO: 471 - protein, 69 aa, Homo sapiens
MITNLRATSSYFLSASSAMCLASLSWISWSSIFSSSFKARFSITFIPLSLSSAAFSASSSFCRAVARRS

SEQ ID NO: 472 - protein, 11 aa, Homo sapiens
MITPASGHTST

SEQ ID NO: 473 - protein, 21 aa, Homo sapiens
MITPMKRFRVKNEPKMIKTTK

SEQ ID NO: 474 - protein, 14 aa, Homo sapiens
MITTSIFPTKGVRI

SEQ ID NO: 475 - protein, 15 aa, Homo sapiens
MITTSLVRTLQYSKD

SEQ ID NO: 476 - protein, 61 aa, Homo sapiens
MIVKTRDLAEALTTCITAIRYLPYVNSLMKVNSGALMKVTVNFITSVQLLTYVVSWMSIQV

SEQ ID NO: 477 - protein, 22 aa, Homo sapiens
MIVLSVCLLLHVLASLDAFALV

SEQ ID NO: 478 - protein, 18 aa, Homo sapiens
MIVLYISTLKYYRSVQKT

SEQ ID NO: 479 - protein, 61 aa, Homo sapiens
MIVYNTHRSRRGRWEEASWLRLAPAAAPNLSQPGRKQVEVSMETRLLRSQVRPLPRFRFPK

SEQ ID NO: 480 - protein, 24 aa, Homo sapiens
MIWSINTSFSCTCWTKRTTADQLS

SEQ ID NO: 481 - protein, 16 aa, Homo sapiens
MIWYCLYEQSSLIMTN

SEQ ID NO: 482 - protein, 15 aa, Homo sapiens
MIYLAHVLEAGAGIW

SEQ ID NO: 483 - protein, 29 aa, Homo sapiens
MIYSKNTLDILNEKIFFPKFRNLGYIQHI

SEQ ID NO: 484 - protein, 26 aa, Homo sapiens
MKADKSQDLQGELASRRSRRADGVPV

SEQ ID NO: 485 - protein, 20 aa, Homo sapiens
MKAELRAKETDPCLESWDAA

SEQ ID NO: 486 - protein, 26 aa, Homo sapiens
MKAIDMHLRISAQINIHIPMRTGAFI

SEQ ID NO: 487 - protein, 11 aa, Homo sapiens
MKALLFFNISF

SEQ ID NO: 488 - protein, 36 aa, Homo sapiens
MKASAGVAEGAKTNLSLSETCGSMSTNTSRHPCGVF

SEQ ID NO: 489 - protein, 67 aa, Homo sapiens
MKASAGVAEGAKTNLSLSETCGSMSTNTSRHPCGVFFWNIVQISVPGNWNPRLSDTFHIHWGSSISL

SEQ ID NO: 490 - protein, 52 aa, Homo sapiens
MKASAGVAEGAKTNLSLSETCGSMSTNTSRHPCGVFSTRCTEMSQFFSTDPS

SEQ ID NO: 491 - protein, 21 aa, Homo sapiens
MKAVGTISPKNNFIQNGEGLG

SEQ ID NO: 492 - protein, 75 aa, Homo sapiens
MKCGPRAPCLPRDCGAHTHGERPVPPRGTLWSLQPAAASWQTHGILIVLFAPCELKKNFFNCMVIFFFCKQSHPS

SEQ ID NO: 493 - protein, 19 aa, Homo sapiens
MKCSDRCHQLCQLALLSNL

SEQ ID NO: 494 - protein, 33 aa, Homo sapiens
MKDEFEIVQRDRVCKAGRIPSLGCGEGNLSGRS

SEQ ID NO: 495 - protein, 11 aa, Homo sapiens
MKDLENKGVNR

SEQ ID NO: 496 - protein, 11 aa, Homo sapiens
MKETEPFPVPG

SEQ ID NO: 497 - protein, 67 aa, Homo sapiens
MKEVSGIQPLVETAHWVDPFSSCYVDMDVIQTNSLLFLQTDCIPPKPDGSRCTGPLLEPSGISVALA

SEQ ID NO: 498 - protein, 104 aa, Homo sapiens
MKFAEEQLLKHGWTQGDPHGASSTSPSSLPTICPGESHHPGLPPHVVHLIKGGKASLKGNLQKKISNFPRKGKKGRNLTVDNEEVVVGRTRGGKKRYGLSTKRI

SEQ ID NO: 499 - protein, 37 aa, Homo sapiens
MKFALQNRLFQKINVTRILAWMFALKMYKRLKQWGKN

SEQ ID NO: 500 - protein, 15 aa, Homo sapiens
MKFQDPRCLSEKFII

SEQ ID NO: 501 - protein, 12 aa, Homo sapiens
MKFRYSKSPSTK

SEQ ID NO: 502 - protein, 68 aa, Homo sapiens
MKFSLSRNLRADEWGRAGGPREAEQDRGARRESRKRAAEATLSARTRARARAPFVDSRREPNPAAARH

SEQ ID NO: 503 - protein, 31 aa, Homo sapiens
MKFSLSRNLTNEKIEINSNRILPKKSFRMDC

SEQ ID NO: 504 - protein, 14 aa, Homo sapiens
MKFTGYMCVKLAHH

SEQ ID NO: 505 - protein, 49 aa, Homo sapiens [sequence omitted]

SEQ ID NO: 506 - protein, 25 aa, Homo sapiens
MKGQDLGSRPRTTGDGFLGGFRNLL

SEQ ID NO: 507 - protein, 48 aa, Homo sapiens
MKGSVTGEVGTIVSLWLKGDSLSRGRHHQRDLGNTALIGSSKAALQSW

SEQ ID NO: 508 - protein, 60 aa, Homo sapiens
MKGWWHPQSTFSPCSRFPNRRKKAPLPLHCQPLLLFLSYPPNQKYLSAALMLNEIQNYLE

SEQ ID NO: 509 - protein, 17 aa, Homo sapiens
MKIKSSLFEKGMVKFSM

SEQ ID NO: 510 - protein, 21 aa, Homo sapiens
MKIQKLHQRKKTIKEVYFQQN

SEQ ID NO: 511 - protein, 11 aa, Homo sapiens
MKKEVNCFNRI

SEQ ID NO: 512 - protein, 35 aa, Homo sapiens
MKKIININHGHPLKTVKKAMCTAWKTRWSVTSLGG

SEQ ID NO: 513 - protein, 14 aa, Homo sapiens
MKKLDVLGMYKFMN

SEQ ID NO: 514 - protein, 34 aa, Homo sapiens
MKKNKANKHAFRNVFACVHVRAHENDSSLELSTS

SEQ ID NO: 515 - protein, 82 aa, Homo sapiens [sequence omitted]

SEQ ID NO: 516 - protein, 18 aa, Homo sapiens
MKLDQILVLFLTTITSSV

SEQ ID NO: 517 - protein, 70 aa, Homo sapiens [sequence omitted]

SEQ ID NO: 518 - protein, 15 aa, Homo sapiens
MKMSICISLLFFLSS

SEQ ID NO: 519 - protein, 71 aa, Homo sapiens
MKNCSPKWLRSCFPRQVWNEASNEWRRMERTKIKPQSSQSWPLSLTPSCPVRHLDCCQVDYLPKPTLEKLL

SEQ ID NO: 520 - protein, 68 aa, Homo sapiens
MKPCLIVETSDDLSLTGQRTASSSTQTHATTHIHPCIPSQESRAYPSTSLTKGPAIKVLSHLAVICTP

SEQ ID NO: 521 - protein, 11 aa, Homo sapiens
MKPDTESEPKN

SEQ ID NO: 522 - protein, 33 aa, Homo sapiens
MKPLFPLVFNVEFFIGLQQPVPKTQASHSPLIY

SEQ ID NO: 523 - protein, 26 aa, Homo sapiens
MKQCAEGHLLVLCAPSRLLTLSPSFS

SEQ ID NO: 524 - protein, 15 aa, Homo sapiens
MKQILFSWFSTCLQK

SEQ ID NO: 525 - protein, 12 aa, Homo sapiens
MKQLGLVRIRKP

SEQ ID NO: 526 - protein, 38 aa, Homo sapiens
MKQPRTCEAKRRISNCFPHDFIVSWGPCFGRSGCLPWA

SEQ ID NO: 527 - protein, 17 aa, Homo sapiens
MKRFRVKNEPKMIKTTK

SEQ ID NO: 528 - protein, 29 aa, Homo sapiens
MKRQDHAERKYFQINHPTKDLYQEYEKNS

SEQ ID NO: 529 - protein, 33 aa, Homo sapiens
MKRTLKLNCRKTNNLKIVRRFEFVFYQRYLDGK

SEQ ID NO: 530 - protein, 17 aa, Homo sapiens
MKSCLLQQHRWDWKPFS

SEQ ID NO: 531 - protein, 35 aa, Homo sapiens
MKSVESNSPWSPICTISPIIIDTDQHILTGSLRSW

SEQ ID NO: 532 - protein, 100 aa, Homo sapiens [sequence omitted]

SEQ ID NO: 533 - protein, 20 aa, Homo sapiens
MKTGFSLSSMSKFNERQNLT

SEQ ID NO: 534 - protein, 13 aa, Homo sapiens
MKTKSFLPVIVAS

SEQ ID NO: 535 - protein, 127 aa, Homo sapiens [sequence omitted]

SEQ ID NO: 536 - protein, 11 aa, Homo sapiens
MKVGKLYLLNS

SEQ ID NO: 537 - protein, 27 aa, Homo sapiens
MKVLLLVLFCSYNFDSPQKLPQMKSSQ

SEQ ID NO: 538 - protein, 33 aa, Homo sapiens
MKVNSGALMKVTVNFITSVQLLTYVVSWMSIQV

SEQ ID NO: 539 - protein, 47 aa, Homo sapiens [sequence omitted]

SEQ ID NO: 540 - protein, 23 aa, Homo sapiens
MKYRSLVQPISALTYTSGLCANA

SEQ ID NO: 541 - protein, 65 aa, Homo sapiens
MLACHGHAPSRELFPFTILLPVMILLATCLPQQLLVSISEAALLISMSLMEAGTAFQDAMLFFNI

SEQ ID NO: 542 - protein, 18 aa, Homo sapiens
MLACMRQSWNTSTLLVGM

SEQ ID NO: 543 - protein, 33 aa, Homo sapiens
MLAGLELLSSICLPQSPKVLGLGATAPGQICLF

SEQ ID NO: 544 - protein, 18 aa, Homo sapiens
MLAIWSQTPQAIHPPRSP

SEQ ID NO: 545 - protein, 18 aa, Homo sapiens
MLAKIRRHWISHTLLVGM

SEQ ID NO: 546 - protein, 12 aa, Homo sapiens
MLALSSCSIYTF

SEQ ID NO: 547 - protein, 50 aa, Homo sapiens
MLANSMLHWPFFLTKRLRHLRRVCTLPLPKPLAPDMVTRCSPSSSDDTML

SEQ ID NO: 548 - protein, 27 aa, Homo sapiens
MLARLLFNSWPQVDMPALASQVLGLQA

SEQ ID NO: 549 - protein, 22 aa, Homo sapiens
MLARLVLNSCPQVICPLGLPKC

SEQ ID NO: 550 - protein, 44 aa, Homo sapiens
MLARLVLNSSPRDPPASASQSAGMTGVSHRARPKQLSYWYSWCW

SEQ ID NO: 551 - protein, 47 aa, Homo sapiens
MLARLVSNSCPQVIQPALAPQSAGITGMGHCVRPWTLFSNVKFEFWV

SEQ ID NO: 552 - protein, 27 aa, Homo sapiens
MLARLVSNSQPQAIHLPQPPKVLGLKA

SEQ ID NO: 553 - protein, 37 aa, Homo sapiens
MLARLVSNSQPQVIHLPWPSKVLGLQVCATASSPHSV

SEQ ID NO: 554 - protein, 27 aa, Homo sapiens
MLARLVSNSQPQVIHPPQPPRVPGLHT

SEQ ID NO: 555 - protein, 41 aa, Homo sapiens
MLARLVSNSRAQAIHQPWTPKVLGSKPLCLAGTTSNMRLTR

SEQ ID NO: 556 - protein, 27 aa, Homo sapiens
MLARLVSNSRPQVIRPLRPPKVLGLQV

SEQ ID NO: 557 - protein, 27 aa, Homo sapiens
MLARLVSNSWAQVIHLPWPPKVLGLQA

SEQ ID NO: 558 - protein, 19 aa, Homo sapiens
MLARLVSNSWPPKVLGLQA

SEQ ID NO: 559 - protein, 27 aa, Homo sapiens
MLARLVSNSWPQMIRPPWPPKMLGLQA

SEQ ID NO: 560 - protein, 27 aa, Homo sapiens
MLARLVSNSWPQVIRPPQPPKVLGLQA

SEQ ID NO: 561 - protein, 27 aa, Homo sapiens
MLARLVSNSYPQVIHPPRPPKVLGLQA

SEQ ID NO: 562 - protein, 25 aa, Homo sapiens
MLARMASFSVLIRPSWPPKVLELQA

SEQ ID NO: 563 - protein, 45 aa, Homo sapiens
MLARMVSISGPCDPPASASQSAGITGVSHHAQPGTSNFLSLCVCE

SEQ ID NO: 564 - protein, 50 aa, Homo sapiens
MLARPVSNSWPQVVCPPWPPKVLGLQVTSGYFKKSEMQGKKNISPTLFFS

SEQ ID NO: 565 - protein, 52 aa, Homo sapiens
MLASLVLNSRLTSDEPPASDSQSVRITGVSHRTWPAPSFYKMLIPNNLRAMC

SEQ ID NO: 566 - protein, 40 aa, Homo sapiens
MLCCLFVLFGLGFLTVCASVNPIYKVEIIIVPTSQGSCKD

SEQ ID NO: 567 - protein, 11 aa, Homo sapiens
MLCFPFKTECL

SEQ ID NO: 568 - protein, 14 aa, Homo sapiens
MLCLGFQLLEVVFV

SEQ ID NO: 569 - protein, 13 aa, Homo sapiens
MLCPHHQGLHMKH

SEQ ID NO: 570 - protein, 18 aa, Homo sapiens
MLCRYGCNSDKFTSVSPN

SEQ ID NO: 571 - protein, 25 aa, Homo sapiens
MLDFPASGTVRNNCCLSHLVYGNLV

SEQ ID NO: 572 - protein, 85 aa, Homo sapiens
MLDKLVLKDLLFMVSPNIHKLPIFIHFHRVLHKPIHVNELDSSLFCIKHHRWNHRELPHLFLIILLLREPINNFRNLMLTPSNGG

SEQ ID NO: 573 - protein, 20 aa, Homo sapiens
MLDSFPVNQPAILLCMQNGL

SEQ ID NO: 574 - protein, 21 aa, Homo sapiens
MLEFVLQFDHIIEPSGILNCT

SEQ ID NO: 575 - protein, 84 aa, Homo sapiens
MLELVLQLFFSFFKCCFFLLDSLHKSLFQLFFFPLTLIIELLSFGFKDFLKTNWLVVWTHICKAHFLQFLVPITFIVLSVGFFF

SEQ ID NO: 576 - protein, 11 aa, Homo sapiens
MLELYSFPIGC

SEQ ID NO: 577 - protein, 25 aa, Homo sapiens
MLEQLTAGKLGVRISVFEAHIHHLK

SEQ ID NO: 578 - protein, 65 aa, Homo sapiens
MLERMMRRDMRLSEAELRSRSKFLFMRYWRKAVWMVLAALRLRKEPPYFLSSISTFLSCRSVESS

SEQ ID NO: 579 - protein, 18 aa, Homo sapiens
MLERMWRNSNAFTPLVGV

SEQ ID NO: 580 - protein, 18 aa, Homo sapiens
MLERTWRNRNTFTLLVGL

SEQ ID NO: 581 - protein, 43 aa, Homo sapiens
MLETQTLRLVCQRITNQIKQAPFLNPVWKRATISTGHMSQGLF

SEQ ID NO: 582 - protein, 38 aa, Homo sapiens
MLFAENLWIRRAGLQPGPWHQEDVNNPEFQGLLMESTS

SEQ ID NO: 583 - protein, 49 aa, Homo sapiens
MLFEKVDLLVFVSNRYCFDRHMLIYSQQATSINTELDEEAHFLLQILHC

SEQ ID NO: 584 - protein, 11 aa, Homo sapiens
MLFGKEFGPFC

SEQ ID NO: 585 - protein, 13 aa, Homo sapiens
MLFHHFAETGIPL

SEQ ID NO: 586 - protein, 13 aa, Homo sapiens
MLFHRSLEGQRLE

SEQ ID NO: 587 - protein, 14 aa, Homo sapiens
MLFIKDSLYRYRYI

SEQ ID NO: 588 - protein, 101 aa, Homo sapiens
MLFLIPHLFSQVCALFLSPLCYDALQPTLHPHQVCRSQISPFHLSLLYSTTYHGLKNQTQIPQIPNTQPLPNFLQTHLPHPHPIPPTPTLTPAPNPALPAD

SEQ ID NO: 589 - protein, 12 aa, Homo sapiens
MLFLLTHSMCLL

SEQ ID NO: 590 - protein, 40 aa, Homo sapiens
MLFVKECMFLLTEVWTSESTVLECVCVPSQVCSTEGSSGK

SEQ ID NO: 591 - protein, 86 aa, Homo sapiens
MLGAGDLSAAEAALRSNRPRTTDKLVVSPHWGRPSAERSRGGRGSARVNQSAVSSPAAAAVGSAARLQGAGLKALAAAKQPRARPS

SEQ ID NO: 592 - protein, 28 aa, Homo sapiens
MLGAPWGPAARVIHAVETPPAVRRRAEP

SEQ ID NO: 593 - protein, 20 aa, Homo sapiens
MLGCLFWKSPAVMHSSELRK

SEQ ID NO: 594 - protein, 12 aa, Homo sapiens
MLGLHEENILFY

SEQ ID NO: 595 - protein, 24 aa, Homo sapiens
MLGQSKWPGYKGPSYSHRCTVIDD

SEQ ID NO: 596 - protein, 14 aa, Homo sapiens
MLGRCLQNTESPRY

SEQ ID NO: 597 - protein, 24 aa, Homo sapiens
MLGRRGAGSRCGVRAVRWAAAGSG

SEQ ID NO: 598 - protein, 188 aa, Homo sapiens
MLGSKGSVSVKSSSHTVSTHSSLRSSGHQGCRPLPRPRNATMIPGHRLAAAVLNFQSSLPRARRVVPRPARPGGAMSFFGFGQSVEVEILLNDAESRKRAEHKTEDGKKEKYFLFYDGETVSGKVSLALKNPNKRLEHQGIKIEFIGQIGESTPGTPSPSADSRPGSRVIQGPAPPARPVTVACQLQS

SEQ ID NO: 599 - protein, 24 aa, Homo sapiens
MLHECGRFPVSWGSGVLESVLFQE

SEQ ID NO: 600 - protein, 11 aa, Homo sapiens
MLHHAQLILYF

SEQ ID NO: 601 - protein, 12 aa, Homo sapiens
MLHHARLILYFW

SEQ ID NO: 602 - protein, 27 aa, Homo sapiens
MLHRLASNSWSQVIHPPQPLKVLRLQV

SEQ ID NO: 603 - protein, 71 aa, Homo sapiens
MLHSALRRHSSSRSIREFTNKMPFCRFTSRRPPRPLDATRNRRGTSSASSSPRSCAMRPTKVPCLASSETE

SEQ ID NO: 604 - protein, 45 aa, Homo sapiens
MLHWPFFLTKRLRHLRRVCTLPLPKPLAPDMVTRCSPSSSDDTML

SEQ ID NO: 605 - protein, 178 aa, Homo sapiens
MLIGRWVIIVSWGPVSSGTLSCGGRHGGRASLGLRLLEAYEQLESWLGHRVRHIVGDINLHQAAAVPLGTHKQPRGEAGDRCCLQNLLVGPVQLEGFLVVQVGGGQGDSEVDASSIGQDGIFSQGLQSHAGVLSGGEAPKCISLLGQPLHHRQGGSHVTQQSVGQKGVGCHFHLGRDH

SEQ ID NO: 606 - protein, 20 aa, Homo sapiens
MLILANFYRVGILSQRGIDE

SEQ ID NO: 607 - protein, 24 aa, Homo sapiens
MLILAQTCNVPTFFKFGVHSDFSF

SEQ ID NO: 608 - protein, 23 aa, Homo sapiens
MLIMNTQMPLLLLESTNTKEKMN

SEQ ID NO: 609 - protein, 116 aa, Homo sapiens
MLIRKFFHWWNYFSSLQNCITREYSGLLFNYAIWFFHFPPRGFILQKFIPEFLHRPHLLWGQHRLPRAQLLVLQPSPSQLSQLLQPQFLIRSVPRHVAAGTNAKGHGAPSNYGLVT

SEQ ID NO: 610 - protein, 147 aa, Homo sapiens [sequence omitted]

SEQ ID NO: 611 - protein, 132 aa, Homo sapiens
MLIRKFFHWWNYFSSLQNCITRNMILHVIMNNPDRYKYMSENKDTLFVYPMDHFPPRGFILQKFIPEFLHRPHLLWGQHRLPRAQLLVLQPSPSQLSQLLQPQFLIRSVPRHVAAGTNAKGHGAPSNYGLVT

SEQ ID NO: 612 - protein, 65 aa, Homo sapiens [sequence omitted]

SEQ ID NO: 613 - protein, 12 aa, Homo sapiens
MLIYCRVLFTLL

SEQ ID NO: 614 - protein, 28 aa, Homo sapiens
MLIYSQQATSINTELDEEAHFLLQILHC

SEQ ID NO: 615 - protein, 14 aa, Homo sapiens
MLKKKVRICLNSRI

SEQ ID NO: 616 - protein, 52 aa, Homo sapiens [sequence omitted]

SEQ ID NO: 617 - protein, 23 aa, Homo sapiens
MLKLHCNNHHSIYFCFILPLFYF

SEQ ID NO: 618 - protein, 11 aa, Homo sapiens
MLKLKMPRIQA

SEQ ID NO: 619 - protein, 43 aa, Homo sapiens
MLKLPPGLSRWRLTEALSTLWAVSSGQTWPVSSVSGLTAQAPA

SEQ ID NO: 620 - protein, 12 aa, Homo sapiens
MLKLSLQVSNLF

SEQ ID NO: 621 - protein, 11 aa, Homo sapiens
MLKNAIYQVKH

SEQ ID NO: 622 - protein, 21 aa, Homo sapiens
MLKNKSVDAHVNSTLYITHII

SEQ ID NO: 623 - protein, 30 aa, Homo sapiens
MLKTESSRERRGDGTCHEVILTLLSKMHEC

SEQ ID NO: 624 - protein, 11 aa, Homo sapiens
MLKVGIVTRVF

SEQ ID NO: 625 - protein, 17 aa, Homo sapiens
MLKWFSVQCVLKKCSLD

SEQ ID NO: 626 - protein, 19 aa, Homo sapiens
MLLCKKVIQNLPGEFHNAN

SEQ ID NO: 627 - protein, 35 aa, Homo sapiens
MLLCLSVVCSFSFLTFFCRDGGLAMLTRLLSNYWS

SEQ ID NO: 628 - protein, 35 aa, Homo sapiens [sequence omitted]

SEQ ID NO: 629 - protein, 23 aa, Homo sapiens
MLLFQARGKRDMEGRLYYHVYRR

SEQ ID NO: 630 - protein, 22 aa, Homo sapiens
MLLFRLLEQVSILLAINCPLLL

SEQ ID NO: 631 - protein, 12 aa, Homo sapiens
MLLGSLYHDEFQ

SEQ ID NO: 632 - protein, 22 aa, Homo sapiens
MLLILVPQLVTEVLMKSVTFQK

SEQ ID NO: 633 - protein, 198 aa, Homo sapiens
MLLITSNETADQQAPGSEERPSAHTVRSPEVGGPSWHRCRRMGVSTRLPGYLLCHPQHTAVHAKPVTSWSQDATMFQVSHHHTEALEAGSWGRCRKVFSLHAFVLYLKKNKSISWKPHQQACSVSRWPQLGCMPSLCHHRSVHTVVSSGRWTLSDLGVQAGLLSWLITELWLGHPAPDSSASAGCSSPGMAPNPLGSD

SEQ ID NO: 634 - protein, 44 aa, Homo sapiens
MLLLSKGYHLPIEIEDGQTLPEPNSVLEATLKCQLQIWSKIMYF

SEQ ID NO: 635 - protein, 16 aa, Homo sapiens
MLLLSPATYLEHDSHV

SEQ ID NO: 636 - protein, 34 aa, Homo sapiens
MLLLSPATYLELHECGRFPVSWGSGVLESVLFQE

SEQ ID NO: 637 - protein, 33 aa, Homo sapiens
MLLLSPATYLERSAARLIALGCRARDGEPGPAR

SEQ ID NO: 638 - protein, 30 aa, Homo sapiens
MLLPAPLEMENQARMRFSFHYYIHTRVNQE

SEQ ID NO: 639 - protein, 14 aa, Homo sapiens
MLLPRPPKVLGLQV

SEQ ID NO: 640 - protein, 13 aa, Homo sapiens
MLLQFNSSLSLCN

SEQ ID NO: 641 - protein, 38 aa, Homo sapiens
MLLRLVLNPWAQAILLPRPPKVLRFARIIGESHYAQPL

SEQ ID NO: 642 - protein, 108 aa, Homo sapiens
MLLRTIYVIACTSTSFLSTAESYPTVCAYHGLQFVYPFIHWIVCTFWLYFIIFRDEVSLCHPGWSAVAPPWFVAASTSLSSKDPPASATQVAGTTGMHYHAWLIFKFL

SEQ ID NO: 643 - protein, 11 aa, Homo sapiens
MLLSCSCFILQ

SEQ ID NO: 644 - protein, 34 aa, Homo sapiens
MLLSLFCRRAKYLLGKKNGKLSQASDQLWHHTGQ

SEQ ID NO: 645 - protein, 213 aa, Homo sapiens
MLLTPPASILLLTCISGAPSVRSARSPIACLSSRPDQAPAPAQPPPPFPPPPTPPPGSPRALAGLAVRLSAPRGREPSRSRGRGSGVGRREAAAPAGGWAGALRPRDRGCASLLLPPGPARSRRRRLCRWGRGRGRARSAAGPGPAGSGRACCSAPRVGRGAGAARVGTPRPPGPGPGPTAAAAACAVARRPLRLPRRLPLGLRALQRRGEGA

SEQ ID NO: 646 - protein, 46 aa, Homo sapiens
MLLTPPASILLLTLTAAVSCWVPKLEKSPWPRLGSGVDLGAGPGAG

SEQ ID NO: 647 - protein, 31 aa, Homo sapiens
MLLTPPASILLLTWASCCVPVQPKELSHPPG

SEQ ID NO: 648 - protein, 42 aa, Homo sapiens
MLLTPPASILLLTWVRWRWEANRLASGGLGCGSLSVAVPACT

SEQ ID NO: 649 - protein, 140 aa, Homo sapiens
MLLTPPASILLLTWVRWRWEANRLASGGLGCGSLSVAVPACTRVGWVSGEYSWAGLSLGWTQSPSLPVGTGASGPVGAGGVPGAPSARGSAPGRHPPARLPPVPAPASVPAPQGSAPRWWPRRRARQGGRVYARESAQRV

SEQ ID NO: 650 - protein, 37 aa, Homo sapiens
MLLVMVTNVARARSSLLMESRFSLLIMLPKLDATADP

SEQ ID NO: 651 - protein, 37 aa, Homo sapiens
MLLVMVTNVARARSSLLMESRFSLLIMLPKLVPVTLL

SEQ ID NO: 652 - protein, 16 aa, Homo sapiens
MLNCCHRLEKFTFPSM

SEQ ID NO: 653 - protein, 18 aa, Homo sapiens
MLNGSRCLYLVLTLVLFW

SEQ ID NO: 654 - protein, 66 aa, Homo sapiens
MLNRIPGLYSLNASSLLPACCDIKNVIHCQMSPRKSGAEGGQNPTHSLKPPPYLILTVTNHSNPRW

SEQ ID NO: 655 - protein, 25 aa, Homo sapiens
MLNRSAERGHPCLVPVLRKNAYNFC

SEQ ID NO: 656 - protein, 26 aa, Homo sapiens
MLNRSVIMGILVLFLISVGKHSVFHH

SEQ ID NO: 657 - protein, 29 aa, Homo sapiens
MLNTHEWSVCEQCLNAVELWWVPLGLLPN

SEQ ID NO: 658 - protein, 41 aa, Homo sapiens
MLPFVSWVIKCTERQREKKSLNYKALCIPRFVWEQAAEILG

SEQ ID NO: 659 - protein, 37 aa, Homo sapiens
MLPGWSQTPDLVIHPPRPPKVLGLQACATAPGQMWTL

SEQ ID NO: 660 - protein, 38 aa, Homo sapiens
MLPKMVSISWPRDPTISASQSAGFKGMSHCAWPRILYC

SEQ ID NO: 661 - protein, 15 aa, Homo sapiens
MLPLPKLNKLLLLFF

SEQ ID NO: 662 - protein, 34 aa, Homo sapiens
MLPRLVWNSWAQVICPPQPPKVLGLQVWATVPGL

SEQ ID NO: 663 - protein, 12 aa, Homo sapiens
MLPVTGQHFQFV

SEQ ID NO: 664 - protein, 18 aa, Homo sapiens
MLPVVEVLSVFVVIGADS

SEQ ID NO: 665 - protein, 16 aa, Homo sapiens
MLPYLEVRVGGTLQFH

SEQ ID NO: 666 - protein, 21 aa, Homo sapiens
MLQDLGEVVLLHEALLDRGNQ

SEQ ID NO: 667 - protein, 27 aa, Homo sapiens
MLQLVIHTLEHPNSTSQLPCHVLNLPL

SEQ ID NO: 668 - protein, 15 aa, Homo sapiens
MLQPAALALNIHCGA

SEQ ID NO: 669 - protein, 15 aa, Homo sapiens
MLQPPCDHEGESLAY

SEQ ID NO: 670 - protein, 24 aa, Homo sapiens
MLQTPYQKCMFSLSSCQPILQFVH

SEQ ID NO: 671 - protein, 19 aa, Homo sapiens
MLQVSSANLRCGCRSLELL

SEQ ID NO: 672 - protein, 16 aa, Homo sapiens
MLQYKLEKPTRINLSF

SEQ ID NO: 673 - protein, 11 aa, Homo sapiens
MLRCIPRYSHF

SEQ ID NO: 674 - protein, 12 aa, Homo sapiens
MLREIFPVHLFS

SEQ ID NO: 675 - protein, 52 aa, Homo sapiens
MLRENIFKLIIQQRTCIKNMKRTLKLNCRKTNNLKIVRRFEFVFYQRYLDGK

SEQ ID NO: 676 - protein, 265 aa, Homo sapiens
MLRFLAAKHILRGMIFLSLVLFWCFGEPESSLPLKLGDWGAAPSHGRSDTNDGFLIYGVTSRMNLTSSSTSLPARFSACTAWSWVAWRRSVPFTDRMASPSRSARLWSAASPGKILEMRIGIRFSRPPLMLMPRPPASCFTTRTRRTGGDAPASPAGPRGGAGGLGGPRPRLGLPGSESPAPPPFGRPLKAAAAGPRAGSSSAAAASPVRLRLSPLSSATTRTQRSLRSSSTSPALVARVHTAMAGPAPAAAVAAATLIPVRQPR

SEQ ID NO: 677 - protein, 26 aa, Homo sapiens
MLRIFFIPALKESLIRDKCLASIDII

SEQ ID NO: 678 - protein, 21 aa, Homo sapiens
MLRQGTVSPATARPYPWPVAG

SEQ ID NO: 679 - protein, 74 aa, Homo sapiens [sequence omitted]

SEQ ID NO: 680 - protein, 33 aa, Homo sapiens
MLSCRDMVAREGVAPGWPQLRGEHSKQSASDGE

SEQ ID NO: 681 - protein, 16 aa, Homo sapiens
MLSDIKGKCLLTTGDH

SEQ ID NO: 682 - protein, 16 aa, Homo sapiens
MLSIHLVRLLFKLFGF

SEQ ID NO: 683 - protein, 65 aa, Homo sapiens
MLSLRIFTLTSFCNTSSFALFISSTALSSSSGDLYSKSRSKYSSSAWVIHSCISAKSFFRFAAFS

SEQ ID NO: 684 - protein, 41 aa, Homo sapiens
MLSPVSLKFLSPWPAFLLLTWGSNWSSPNILGGGQRGINRA

SEQ ID NO: 685 - protein, 14 aa, Homo sapiens
MLSRASVCRQFVVA

SEQ ID NO: 686 - protein, 20 aa, Homo sapiens
MLSRMLNCCHRLEKFTFPSM

SEQ ID NO: 687 - protein, 125 aa, Homo sapiens
MLSSFCVSSLGRLSTLVNLKSTFTLFIHSSLRQTRHWSTTSTDRFWLVRAASILFRMVGPTRSAATGLPLVTTNSYLLRDWSSSHPTGWRVERAAAWTSTMTANSEESTWGGICTCGLSPRKLHR

SEQ ID NO: 688 - protein, 37 aa, Homo sapiens
MLSVSEPSSSCYQFRGHNSVHREGPQPPTQAPGVQSV

SEQ ID NO: 689 - protein, 20 aa, Homo sapiens
MLTHWSPVPQAITITLIGQD

SEQ ID NO: 690 - protein, 44 aa, Homo sapiens
MLTMLGHSQKLLAMTTSMRLACRYRYSSLPRPRSMPSVRLRSRL

SEQ ID NO: 691 - protein, 37 aa, Homo sapiens
MLTSFSKSYWPKIHLINSIFSEIEDSDDSDVSDVSSS

SEQ ID NO: 692 - protein, 44 aa, Homo sapiens
MLTSRRKKKQASSSILKQLLYLFLVGRNRMFHRRLQSVLLFGPE

SEQ ID NO: 693 - protein, 25 aa, Homo sapiens
MLTVHPNPKPPWAVYSKYCTLVRSY

SEQ ID NO: 694 - protein, 49 aa, Homo sapiens
MLVELYCRLHSSAGLMANSCRRFRARRSLPSQRSRRERLARSGKLLLLL

SEQ ID NO: 695 - protein, 36 aa, Homo sapiens
MLVGWEPILMEHSAWWGGWQAGGSAQMLAMPPLLSC

SEQ ID NO: 696 - protein, 27 aa, Homo sapiens
MLVKLVSNSRTLVIHPPWPPKVLGLQA

SEQ ID NO: 697 - protein, 13 aa, Homo sapiens
MLVLEVSCSDALF

SEQ ID NO: 698 - protein, 27 aa, Homo sapiens
MLVRLFSNALLQVICLPRPPRVLGCQT

SEQ ID NO: 699 - protein, 27 aa, Homo sapiens
MLVRLISNSQPQVIRLPQPPKVLGLQA

SEQ ID NO: 700 - protein, 27 aa, Homo sapiens
MLVRLVLNSQPQVICLPQPSKVLGLQV

SEQ ID NO: 701 - protein, 27 aa, Homo sapiens
MLVRLVLNSRPQVICLPWPPKVLGLQV

SEQ ID NO: 702 - protein, 27 aa, Homo sapiens
MLVRLVLNSRPQVNHPPRTSKVPRLQV

SEQ ID NO: 703 - protein, 53 aa, Homo sapiens
MLVRLVLNSRPQVSARPGLPKCWDDRCEPPHPACCKNFLNFKKKITHENGLIK

SEQ ID NO: 704 - protein, 27 aa, Homo sapiens
MLVRLVSNFCPQLFHLPQPPKVLGLHV

SEQ ID NO: 705 - protein, 27 aa, Homo sapiens
MLVRLVSNSQPQVIYPPWPPKELGLQV

SEQ ID NO: 706 - protein, 25 aa, Homo sapiens
MLVRLVSNSRPQVICPPPLPKVLGL

SEQ ID NO: 707 - protein, 67 aa, Homo sapiens
MLVRLVSNSRPQVIRAWPTFFFLFLFLFLFFLSFLFFFLRDRVLLCCPDWSQTPGLKWSSHLGLPKR

SEQ ID NO: 708 - protein, 12 aa, Homo sapiens
MLVRLVSNSRPR

SEQ ID NO: 709 - protein, 25 aa, Homo sapiens
MLVRLVWNSQPQVIRLPQPPKVLGL

SEQ ID NO: 710 - protein, 42 aa, Homo sapiens
MLVRMVLTSRPCDPPTSASQSAGITGVSHHAWPIIINQLLIK

SEQ ID NO: 711 - protein, 27 aa, Homo sapiens
MLVRVVLNSQPQVICPPQPPKVLGLQA

SEQ ID NO: 712 - protein, 34 aa, Homo sapiens
MLWRRRRLSGGARSRDPQRFRHTFNAAALSTRSF

SEQ ID NO: 713 - protein, 58 aa, Homo sapiens
MLYEGFCWGGRRCQNKPQFIRNLWINVNKYFSPSLWCFLKFMHRKNIKKFMCKIKAVP

SEQ ID NO: 714 - protein, 89 aa, Homo sapiens
MLYEGFCWGGRRCQNKPQFIRNLWINVNKYFSPSLWCFLKFMHRKNIKKFMCKIKAVPFWNIVQISVPGNWNPRLSDTFHIHWGSSISL

SEQ ID NO: 715 - protein, 74 aa, Homo sapiens
MLYEGFCWGGRRCQNKPQFIRNLWINVNKYFSPSLWCFLKFMHRKNIKKFMCKIKAVPSTRCTEMSQFFSTDPS

SEQ ID NO: 716 - protein, 55 aa, Homo sapiens
MLYEGFCWGGRRCQNKPQFIRNLWINVNKYFSPSLWCFLLEHRADLGTRKLESQT

SEQ ID NO: 717 - protein, 43 aa, Homo sapiens
MLYEGFCWGGRRCQNKPQFIRNLWINVNKYFSPSLWCFLYQMY

SEQ ID NO: 718 - protein, 11 aa, Homo sapiens
MLYKNLTSFYS

SEQ ID NO: 719 - protein, 18 aa, Homo sapiens
MLYSQIEFSFREPLSVLT

SEQ ID NO: 720 - protein, 26 aa, Homo sapiens
MLYTLRSITSHRSSHPERWATSSQVK

SEQ ID NO: 721 - protein, 33 aa, Homo sapiens
MMCNGCSITENFVTIITLVKFPYTMDCLMVNKW

SEQ ID NO: 722 - protein, 42 aa, Homo sapiens
MMGWCPGWNWFQDPRKHQNPQMPLYKMATVFAYHQHTSPYIL

SEQ ID NO: 723 - protein, 14 aa, Homo sapiens
MMHATLITSRGSFS

SEQ ID NO: 724 - protein, 23 aa, Homo sapiens
MMIQNLPGLLPVHCFYFSLDKKK

SEQ ID NO: 725 - protein, 16 aa, Homo sapiens
MMITTSLVRTLQYSKD

SEQ ID NO: 726 - protein, 62 aa, Homo sapiens
MMIVYNTHRSRRGRWEEASWLRLAPAAAPNLSQPGRKQVEVSMETRLLRSQVRPLPRFRFPK

SEQ ID NO: 727 - protein, 17 aa, Homo sapiens
MMIWYCLYEQSSLIMTN

SEQ ID NO: 728 - protein, 12 aa, Homo sapiens
MMKALLFFNISF

SEQ ID NO: 729 - protein, 35 aa, Homo sapiens
MMKKNKANKHAFRNVFACVHVRAHENDSSLELSTS

SEQ ID NO: 730 - protein, 117 aa, Homo sapiens
MMLIRKFFHWWNYFSSLQNCITREYSGLLFNYAIWFFHFPPRGFILQKFIPEFLHRPHLLWGQHRLPRAQLLVLQPSPSQLSQLLQPQFLIRSVPRHVAAGTNAKGHGAPSNYGLVT

SEQ ID NO: 731 - protein, 148 aa, Homo sapiens
MMLIRKFFHWWNYFSSLQNCITREYSGLLFNYAIWFFRNMILHVIMNNPDRYKYMSENKDTLFVYPMDHFPPRGFILQKFIPEFLHRPHLLWGQHRLPRAQLLVLQPSPSQLSQLLQPQFLIRSVPRHVAAGTNAKGHGAPSNYGLVT

SEQ ID NO: 732 - protein, 133 aa, Homo sapiens
MMLIRKFFHWWNYFSSLQNCITRNMILHVIMNNPDRYKYMSENKDTLFVYPMDHFPPRGFILQKFIPEFLHRPHLLWGQHRLPRAQLLVLQPSPSQLSQLLQPQFLIRSVPRHVAAGTNAKGHGAPSNYGLVT

SEQ ID NO: 733 - protein, 20 aa, Homo sapiens
MMLQVSSANLRCGCRSLELL

SEQ ID NO: 734 - protein, 16 aa, Homo sapiens
MMMVLIISFTCAWQDT

SEQ ID NO: 735 - protein, 11 aa, Homo sapiens
MMPASLFMWPY

SEQ ID NO: 736 - protein, 22 aa, Homo sapiens
MMPSAVSKATEHLKRFRSYLLI

SEQ ID NO: 737 - protein, 15 aa, Homo sapiens
MMPSSALLFSSSLRL

SEQ ID NO: 738 - protein, 12 aa, Homo sapiens
MMQLVQSFLDAG

SEQ ID NO: 739 - protein, 11 aa, Homo sapiens
MMRILVRISTQ

SEQ ID NO: 740 - protein, 61 aa, Homo sapiens
MMRRDMRLSEAELRSRSKFLFMRYWRKAVWMVLAALRLRKEPPYFLSSISTFLSCRSVESS

SEQ ID NO: 741 - protein, 19 aa, Homo sapiens
MMSFSKSNSTFIYLTCAFC

SEQ ID NO: 742 - protein, 42 aa, Homo sapiens
MMTLTFVKVCLPMVSSEARSFMLSFQHNMKMKEMHFAKQNRP

SEQ ID NO: 743 - protein, 15 aa, Homo sapiens
MMVLIISFTCAWQDT

SEQ ID NO: 744 - protein, 19 aa, Homo sapiens
MMVMSSEMTRMLSRIWNIL

SEQ ID NO: 745 - protein, 79 aa, Homo sapiens [sequence omitted]

SEQ ID NO: 746 - protein, 34 aa, Homo sapiens
MNEVATQGNVNQWYDFTLSCLICFVVVGSSRYYP

SEQ ID NO: 747 - protein, 12 aa, Homo sapiens
MNGPFFFFFFLF

SEQ ID NO: 748 - protein, 68 aa, Homo sapiens
MNHIKHLGKRLFQTHTDTGPVKKGILLCKAANSQYWKYSFWHSSTGKKSKSSLPNAHCRFFSLDMPHR

SEQ ID NO: 749 - protein, 59 aa, Homo sapiens
MNIFIIFNCLTLKAASSIVFSTLIFFSLKLYLGEFSTISLNVESFLFFLLLLSFSLSLF

SEQ ID NO: 750 - protein, 13 aa, Homo sapiens
MNIQRGKIYLNQL

SEQ ID NO: 751 - protein, 72 aa, Homo sapiens [sequence omitted]

SEQ ID NO: 752 - protein, 27 aa, Homo sapiens
MNLCVVRAEGWLKALPHSSHLKGFSPV

SEQ ID NO: 753 - protein, 19 aa, Homo sapiens
MNLLRSVCRRIFCGSSNHV

SEQ ID NO: 754 - protein, 19 aa, Homo sapiens
MNLREKNLIIWGKEIFFFA

SEQ ID NO: 755 - protein, 18 aa, Homo sapiens
MNLYPQSTGALDLSFVTR

SEQ ID NO: 756 - protein, 26 aa, Homo sapiens
MNMLHECGRFPVSWGSGVLESVLFQE

SEQ ID NO: 757 - protein, 12 aa, Homo sapiens
MNNRAWLFPGFF

SEQ ID NO: 758 - protein, 27 aa, Homo sapiens
MNNYVHLKVQIQDQYQNSDFLQPIIKL

SEQ ID NO: 759 - protein, 85 aa, Homo sapiens
MNQAQGPSLPVASHHHTHFAGPRALPGPYLAPRYFIHLCFEYFMGPSPPEASEHSQNWNGNTQCVLVSCPGRRVQRAGHSSFCSN

SEQ ID NO: 760 - protein, 19 aa, Homo sapiens
MNQKVSFCSGKEFLHSITA

SEQ ID NO: 761 - protein, 11 aa, Homo sapiens
MNQSLLAQTVF

SEQ ID NO: 762 - protein, 17 aa, Homo sapiens
MNRYNFNYSKANMPKER

SEQ ID NO: 763 - protein, 22 aa, Homo sapiens
MNSFTCSSCPSVSSMSRVGGCP

SEQ ID NO: 764 - protein, 31 aa, Homo sapiens
MNSHFLSTIFKVKIIDDSVMGNCWSWVDSLD

SEQ ID NO: 765 - protein, 11 aa, Homo sapiens
MNSLMFNEVST

SEQ ID NO: 766 - protein, 26 aa, Homo sapiens
MNSLVVFSSEPSTETNIGAPKYEVSK

SEQ ID NO: 767 - protein, 42 aa, Homo sapiens
MNSQTSSSSSDTPVQYTMSLTFSGILFLLLEIQSEISVDACW

SEQ ID NO: 768 - protein, 14 aa, Homo sapiens
MNTLQFAMKLNTYK

SEQ ID NO: 769 - protein, 20 aa, Homo sapiens
MNTQMPLLLLESTNTKEKMN

SEQ ID NO: 770 - protein, 68 aa, Homo sapiens
MNTTSCFCNDPYCHAALGSWGHWTFGLVAYSPVLLVCSLAIPPEVAGRAGHWSLLWLQESLPVQSFSC

SEQ ID NO: 771 - protein, 35 aa, Homo sapiens
MNTWSSSSKTKNFRPSMAAHACNPSTLGGRGRRVT

SEQ ID NO: 772 - protein, 62 aa, Homo sapiens
MNVEDSLFLGVLGSLSQSSSRSKLPFAQGTKPQCCPPHCARLPCARWRTGPRALVGGGKLRR

SEQ ID NO: 773 - protein, 28 aa, Homo sapiens
MNVLTSFALPCVSQHGQVTILFSHSSRL

SEQ ID NO: 774 - protein, 102 aa, Homo sapiens
MNVSKMDNEPGHERKVFVPGLGLQENMALHILAGFTVCHTSFPHGILDLTDQLLPEGGAPPVGLLPGNVHACSPAPAARIPLGRHRRRLSHRARPKPGSRPQ

SEQ ID NO: 775 - protein, 115 aa, Homo sapiens [sequence omitted]

SEQ ID NO: 776 - protein, 14 aa, Homo sapiens
MNYEIWKQTHFYIL

SEQ ID NO: 777 - protein, 21 aa, Homo sapiens
MPAFWEAEAGRSPEVRSARPA

SEQ ID NO: 778 - protein, 66 aa, Homo sapiens [sequence omitted]

SEQ ID NO: 779 - protein, 13 aa, Homo sapiens
MPALASQVLGLQA

SEQ ID NO: 780 - protein, 21 aa, Homo sapiens
MPALWEAEVGGSPEVSSSRSA

SEQ ID NO: 781 - protein, 99 aa, Homo sapiens [sequence omitted]

SEQ ID NO: 782 - protein, 11 aa, Homo sapiens
MPCKTSPNTDC

SEQ ID NO: 783 - protein, 43 aa, Homo sapiens
MPDFMPRSVWSSSSVSRRSRSPSTCCSRKLSQYLEKPICCSHV

SEQ ID NO: 784 - protein, 43 aa, Homo sapiens
MPFISLSCLIALARAFSTMLNRSAERGHPCLVPVLRKNAYNFC

SEQ ID NO: 785 - protein, 16 aa, Homo sapiens
MPFLGPNQDIQKPLAQ

SEQ ID NO: 786 - protein, 56 aa, Homo sapiens
MPFLGTALAAQAGLKERGLSLRGVPPLGELWAGSILLRGCQPPNLGQGQLLLLCVW

SEQ ID NO: 787 - protein, 13 aa, Homo sapiens
MPFRNRPYCIRPP

SEQ ID NO: 788 - protein, 19 aa, Homo sapiens
MPFRSQQVLCSLVVAQEKT

SEQ ID NO: 789 - protein, 12 aa, Homo sapiens
MPGFFFFFFLYF

SEQ ID NO: 790 - protein, 54 aa, Homo sapiens [sequence omitted]

SEQ ID NO: 791 - protein, 83 aa, Homo sapiens
MPGQEGTMPSSFCMTRVVQLCLGLQLQARLWAQLDLRLWVRSHWGPGSSSGSLTSARRGLPRPVLGRRPAAVSPPGSARSRGA

SEQ ID NO: 792 - protein, 43 aa, Homo sapiens
MPGQIFKGIKTMSYAFLHLQNTAKTFKWKWNFQMQNRISAIKR

SEQ ID NO: 793 - protein, 24 aa, Homo sapiens
MPGTRSILEFLDFQIFAILLVEYL

SEQ ID NO: 794 - protein, 42 aa, Homo sapiens
MPGYFFSNFSRDRVSPCWPGWSRTPDLVIHLPRPPKVLGLQA

SEQ ID NO: 795 - protein, 14 aa, Homo sapiens
MPGYLFLFLFFLYF

SEQ ID NO: 796 - protein, 119 aa, Homo sapiens
MPGYPASAGHCWPRCLSDRQHLLRIGWCRLWFLLGLSAYLLYVVVLAVIGHPFQICVAVEEGPAAPRDFLFQQHLQLRHLHILLLLLLIQVAEGAAAAAPRKPRTGRGGAAATAAVTRK

SEQ ID NO: 797 - protein, 16 aa, Homo sapiens
MPHATENVSNYVCFRA

SEQ ID NO: 798 - protein, 30 aa, Homo sapiens
MPHHAQLIFVFLVETGFHHVGQDGLDLWTL

SEQ ID NO: 799 - protein, 71 aa, Homo sapiens
MPHPERYPPSREPRPPPQGGGGSNLRRGDPSLFPRLSAQPRDPRRPGGKGKREGLQRLTGELLLQPLGWSA

SEQ ID NO: 800 - protein, 155 aa, Homo sapiens
MPHPERYPPSREPRPPPQGGGGSNLRRGDPSLFPRLSAQPRDPRRPGGKGKREGLQRLTGELLLQPLGWSAAGSGQEGVGGRRTREQRRRFPQGCGEEEAELRSVGAGGGVPSPGSGQRRRGPAGAHPTISRLAAGCPSTPGGVWVGPQAPAEQG

SEQ ID NO: 801 - protein, 60 aa, Homo sapiens
MPHPHLQVLGACREDPHDLGSPQGGPSSRRGPGEVGVGEALGQEVPALSLEAERFLPRPS

SEQ ID NO: 802 - protein, 61 aa, Homo sapiens
MPIFPLGFHSRGTKRTNRALTECNSLWCTTLSAFMFPAKVQMLSSCLYCFQLRPVSLNIRL

SEQ ID NO: 803 - protein, 24 aa, Homo sapiens
MPIRNKITHTYHSCSFISFSNDYY

SEQ ID NO: 804 - protein, 27 aa, Homo sapiens
MPIVLFVMCSFPTYLYVSLLSFLPMSA

SEQ ID NO: 805 - protein, 69 aa, Homo sapiens
MPKATWRADQRWLSIPELSFSAEQFLKLYFPLYVQDTQHLGCLFPVIRFPGPWALSVPIPSMLRGSVLR

SEQ ID NO: 806 - protein, 53 aa, Homo sapiens
MPKCSGFKQQSFITSCSSCRSEIREEQGWAAVAQDLSCAQSSWRARLGSVVPN

SEQ ID NO: 807 - protein, 26 aa, Homo sapiens
MPKKSSVEMGAGGGGLTMLPRLVLNT

SEQ ID NO: 808 - protein, 64 aa, Homo sapiens [sequence omitted]

SEQ ID NO: 809 - protein, 12 aa, Homo sapiens
MPLAPCSAIASR

SEQ ID NO: 810 - protein, 14 aa, Homo sapiens
MPLFTRCHISLNSL

SEQ ID NO: 811 - protein, 27 aa, Homo sapiens
MPLGLCKVLAELFSDFHIAQVTFYLCI

SEQ ID NO: 812 - protein, 16 aa, Homo sapiens
MPLLLLESTNTKEKMN

SEQ ID NO: 813 - protein, 25 aa, Homo sapiens
MPLLLPRCLSDDFPHACGRNLHLMT

SEQ ID NO: 814 - protein, 22 aa, Homo sapiens
MPLLWITLLKPRWFRLMFSLKS

SEQ ID NO: 815 - protein, 15 aa, Homo sapiens
MPLTTLESPLECFAA

SEQ ID NO: 816 - protein, 23 aa, Homo sapiens
MPLYNPISFRLGKTCDLLPINRI

SEQ ID NO: 817 - protein, 30 aa, Homo sapiens
MPPCPANFCIFSRDRVSLCWPGWSQTPDLK

SEQ ID NO: 818 - protein, 50 aa, Homo sapiens
MPPCPANLCIFSRDGVSSYWSGWSRAPDLPTSRLQMTRPPRPSKVLGLQV

SEQ ID NO: 819 - protein, 30 aa, Homo sapiens
MPPCPANTLHFCKDGVSPCWPGGSRTPDLK

SEQ ID NO: 820 - protein, 14 aa, Homo sapiens
MPPHPTNIYIFGIF

SEQ ID NO: 821 - protein, 19 aa, Homo sapiens
MPPIHTPTCLSVQRLATPG

SEQ ID NO: 822 - protein, 76 aa, Homo sapiens [sequence omitted]

SEQ ID NO: 823 - protein, 27 aa, Homo sapiens
MPPNPPQTPTICITSTGHPSNQSLSTF

SEQ ID NO: 824 - protein, 16 aa, Homo sapiens
MPPPGSFFHSQFCCQL

SEQ ID NO: 825 - protein, 153 aa, Homo sapiens
MPPRPAHFCIFSREEFHHVGQAGLELLTSGDPPASVSQSAGITGMSHQASPTPRLSVFWEIPQFPAPWALATRSPPFSRQTRPRRPKLQPRPPRPSTTRPAAQASAPSGPTSSSGWAFLPLSCQHTSKKGYTGLGRRSWKAKSGTSASASLAS

SEQ ID NO: 826 - protein, 24 aa, Homo sapiens
MPPRPANFCIFSRDGVSPCWPGWS

SEQ ID NO: 827 - protein, 30 aa, Homo sapiens
MPPRPANFCIFSTDGVSPCWPGWSRTPNLR

SEQ ID NO: 828 - protein, 12 aa, Homo sapiens
MPPRPANFFLYF

SEQ ID NO: 829 - protein, 13 aa, Homo sapiens
MPPVLSAKCSRNL

SEQ ID NO: 830 - protein, 15 aa, Homo sapiens
MPPVLSAKCSRNLSS

SEQ ID NO: 831 - protein, 59 aa, Homo sapiens
MPPVSLLKHNKSHLCSSSQQVLHFHLRLPHLGLCCPYCYQHFGKSHSTSLQEVPNLPTF

SEQ ID NO: 832 - protein, 100 aa, Homo sapiens
MPPVSLLNHNKSHLCSSSQQVPHLHLRPPQSRFHCPYHYQYFCQSHSTSLKEVPNFPIFLSSSEPSKLFQSLPVTKFQSCFHISRYLCSNTCSTGTNLLY

SEQ ID NO: 833 - protein, 71 aa, Homo sapiens
MPPYWPLANFSSICSRHMPCPGCCGKARPPRPPLRGPSATSSSAVATPPKGCRKGAVRPRCFSCRNSPRMR

SEQ ID NO: 834 - protein, 24 aa, Homo sapiens
MPQPLLHQQPGSAGVFLVSSLART

SEQ ID NO: 835 - protein, 12 aa, Homo sapiens
MPRAQSASERPV

SEQ ID NO: 836 - protein, 28 aa, Homo sapiens
MPRCPGRNRLSGVRPTYIRALMVSMCSA

SEQ ID NO: 837 - protein, 17 aa, Homo sapiens
MPRDTADYFREFAKETQ

SEQ ID NO: 838 - protein, 64 aa, Homo sapiens [sequence omitted]

SEQ ID NO: 839 - protein, 62 aa, Homo sapiens
MPRLRCPLTAPGAPPLLLLLLLFFSSSSSSFLSFSFFFSSASRSCSALALPESGAWAASGGA

SEQ ID NO: 840 - protein, 126 aa, Homo sapiens
MPRLRCPLTAPGAPPLLLLLLLFFSSSSSSFLSFSFFFSSASRSCSALALPESGAWAASGGALPPPHPPPRALSAAAAAAAAAAAAGPPAGAAAGAPTADAASRGAPGRIAWAGPPESHSHLQSAG

SEQ ID NO: 841 - protein, 19 aa, Homo sapiens
MPRMLPYLEVRVGGTLQFH

SEQ ID NO: 842 - protein, 39 aa, Homo sapiens
MPRSVWSSSSVSRRSRSPSTCCSRKLSQYLEKPICCSHV

SEQ ID NO: 843 - protein, 21 aa, Homo sapiens
MPSAVSKATEHLKRFRSYLLI

SEQ ID NO: 844 - protein, 15 aa, Homo sapiens
MPSGAPAAAMMIVYN

SEQ ID NO: 845 - protein, 71 aa, Homo sapiens
MPSGAPAAAMMIVYNTHRSRRGRWEEASWLRLAPAAAPNLSQPGRKQVEVSMETRLLRSQVRPLPRFRFPK

SEQ ID NO: 846 - protein, 30 aa, Homo sapiens
MPSHPADFLYFIVETGFHCVSQDCLDLLTS

SEQ ID NO: 847 - protein, 16 aa, Homo sapiens
MPSKTKESPNFSASVK

SEQ ID NO: 848 - protein, 15 aa, Homo sapiens
MPSLTSWHSRCTSGW

SEQ ID NO: 849 - protein, 97 aa, Homo sapiens
MPSQGVMEQAPRADHAHCTLSEQLKFCLCMFILEGGMDARVQLLPPAPNKTVSQGSGPPGRGNCNERALSLSFVWHVPHCSHPCHCSCVTGLMLLFS

SEQ ID NO: 850 - protein, 95 aa, Homo sapiens
MPSRLQTRSGTSWYSPTGTATSSSLLYVATPTRARESSLSTARTNRFTKTLARRKPSRVVPAELSSRKRRSTLHSRLSFRAQLASPPKASGQRHW

SEQ ID NO: 851 - protein, 14 aa, Homo sapiens
MPSSALLFSSSLRL

SEQ ID NO: 852 - protein, 76 aa, Homo sapiens
MPSSFCMTRVVQLCLGLQLQARLWAQLDLRLWVRSHWGPGSSSGSLTSARRGLPRPVLGRRPAAVSPPGSARSRGA

SEQ ID NO: 853 - protein, 50 aa, Homo sapiens
MPSVCPCACITVLSIRVILPLQGTSDSVWRHFFFACHNPEGGAVCYWPGK

SEQ ID NO: 854 - protein, 52 aa, Homo sapiens
MPSYFFVFLVDTGFCHVGQTGLELLTSGDPFALASQSAGITRMSHIWLFFIY

SEQ ID NO: 855 - protein, 21 aa, Homo sapiens
MPTIYYLIKSSQQSWEKSNNC

SEQ ID NO: 856 - protein, 20 aa, Homo sapiens
MPTPTLFFFFETESHSCHPG

SEQ ID NO: 857 - protein, 30 aa, Homo sapiens
MPTSCFPEAPWRRQKHLRMNGPFFFFFFLF

SEQ ID NO: 858 - protein, 73 aa, Homo sapiens [sequence omitted]

SEQ ID NO: 859 - protein, 36 aa, Homo sapiens
MPVAFFLPVVTSKMSYIAKCPQERVGLREDKILPTV

SEQ ID NO: 860 - protein, 16 aa, Homo sapiens
MPVAMRPRRTMEKRVI

SEQ ID NO: 861 - protein, 37 aa, Homo sapiens
MPVISALWEVKAGGSLEARSARRPGQHNETPSVQNVF

SEQ ID NO: 862 - protein, 24 aa, Homo sapiens
MPVMPAFWEAEAGRSPEVRSARPA

SEQ ID NO: 863 - protein, 43 aa, Homo sapiens [sequence omitted]

SEQ ID NO: 864 - protein, 16 aa, Homo sapiens
MPVRMAIIKKAGNNRC

SEQ ID NO: 865 - protein, 12 aa, Homo sapiens
MPWRHFPHCLGN

SEQ ID NO: 866 - protein, 57 aa, Homo sapiens
MPYFPKSETVVPPTGTAFPGPYTSHMVRATWAFLGRSGYFTGSFSHSFQFHLVLNAL

SEQ ID NO: 867 - protein, 61 aa, Homo sapiens
MPYFPKSETVVPPTGTAFPGPYTSHMVRATWAFLGRSGYFTGSFSHSFQILSWTLISRSQL

SEQ ID NO: 868 - protein, 25 aa, Homo sapiens
MPYIYETNIVFLVFNLLAEIIILIL

SEQ ID NO: 869 - protein, 11 aa, Homo sapiens
MPYSQINIIFF

SEQ ID NO: 870 - protein, 163 aa, Homo sapiens [sequence omitted]

SEQ ID NO: 871 - protein, 23 aa, Homo sapiens
MQCPCLLPIQVELYILPLYSFPH

SEQ ID NO: 872 - protein, 13 aa, Homo sapiens
MQCSNFLQIWSSF

SEQ ID NO: 873 - protein, 128 aa, Homo sapiens
MQDETGHPEMISHADSFTRSNLKFPLGRHDLGISPRNLDSSIQAGPVMGLHDVPAIGSVCSHTTVIWTLGPWEAVGRPTKGVPICPHEGILLLHAKPGVLVAHHVHYPFTGVPQIGLCRPSIVLENFT

SEQ ID NO: 874 - protein, 32 aa, Homo sapiens
MQDQSHKVIRQLMITHTHSLQPSYQFPLECDP

SEQ ID NO: 875 - protein, 13 aa, Homo sapiens
MQESDSESTRRIP

SEQ ID NO: 876 - protein, 42 aa, Homo sapiens
MQGISSQHLPRCDSTDQSAAAEGCGDSIYPWCVGTVWIASFL

SEQ ID NO: 877 - protein, 66 aa, Homo sapiens [sequence omitted]

SEQ ID NO: 878 - protein, 67 aa, Homo sapiens
MQHHTWLIFVFLVETRFHHIGQAGLELLTSGDLPTSASQSAGITGVSHHTQPNVSALKYNFKKSLIG

SEQ ID NO: 879 - protein, 12 aa, Homo sapiens
MQHLGHTKNKVQ

SEQ ID NO: 880 - protein, 53 aa, Homo sapiens
MQHLLHPGVVLVEDAHCWLVSSGIDSMIPAGLPFGSLFSAVSPRASWSLVCKT

SEQ ID NO: 881 - protein, 20 aa, Homo sapiens
MQHNWDGLHLDWRRHLETCI

SEQ ID NO: 882 - protein, 15 aa, Homo sapiens
MQHTPSRMKRKLPRR

SEQ ID NO: 883 - protein, 29 aa, Homo sapiens
MQISVGGKERLGQGEAWLPPILRYCQGRH

SEQ ID NO: 884 - protein, 11 aa, Homo sapiens
MQLFQKINFEK

SEQ ID NO: 885 - protein, 29 aa, Homo sapiens
MQLHLMPQPLLHQQPGSAGVFLVSSLART

SEQ ID NO: 886 - protein, 35 aa, Homo sapiens
MQLPPPAARPARQGGVPSSPRLPALAPAPLPFFSS

SEQ ID NO: 887 - protein, 134 aa, Homo sapiens
MQLQVSNHSEVLFEFESPASCGTEGGVKAREVLLAAHLNEPVHSTAGKADEVQVPFASTHGQVFQFQVDVSDPSFPISSIRSQILPDALQVLHFLLLLFGCNILRLEIHQFNQRSTDVHAKPWECLLFAIYKLH

SEQ ID NO: 888 - protein, 343 aa, Homo sapiens
MQLQVSNHSEVLFEFESPASCGTEGGVKAREVLLAAHLNEPVHSTAGKADEVQVPFASTHGQVFQFQVDVSDPSFPISSIRSQILPDALQVLHFLLLLFGCNILRLEIHQFNQRSTDVHAKPWEWRPVLSPRVHPPPQPAFLGRGVMLREQWLRLQLRQEREALGRRVAAAHWTPAADVRRLDWRRMEAVVQQPVHSGGAGAHGGPWRVRDRALLLPAAVAHAGGWRGCARAPAQAASLEVILRRLYFPGSSLRLPIQQPQSRRLGMANPALLPSSCRLPHLLCALPPARRPHGAGLEHASPGRGIGDPRAPPAGAPAARLPLIPRPRDFKRGFLASQTGPRH

SEQ ID NO: 889 - protein, 11 aa, Homo sapiens
MQLVQSFLDAG

SEQ ID NO: 890 - protein, 11 aa, Homo sapiens
MQMLPRLQTTL

SEQ ID NO: 891 - protein, 16 aa, Homo sapiens
MQNFLLLSISSSHLGE

SEQ ID NO: 892 - protein, 17 aa, Homo sapiens
MQNPGSRNLKDEMLLKV

SEQ ID NO: 893 - protein, 19 aa, Homo sapiens
MQPEKIKRNICEFVCYALI

SEQ ID NO: 894 - protein, 194 aa, Homo sapiens
MQPPGAHLQHHLVFLVMLIGRWVIIVSWGPVSSGTLSCGGRHGGRASLGLRLLEAYEQLESWLGHRVRHIVGDINLHQAAAVPLGTHKQPRGEAGDRCCLQNLLVGPVQLEGFLVVQVGGGQGDSEVDASSIGQDGIFSQGLQSHAGVLSGGEAPKCISLLGQPLHHRQGGSHVTQQSVGQKGVGCHFHLGRDH

SEQ ID NO: 895 - protein, 19 aa, Homo sapiens
MQPRTRHRAAKSCIQAQIL

SEQ ID NO: 896 - protein, 12 aa, Homo sapiens
MQPTGVQTDCLH

SEQ ID NO: 897 - protein, 17 aa, Homo sapiens
MQQKMCLIMFVLELKKC

SEQ ID NO: 898 - protein, 22 aa, Homo sapiens
MQRALPPNAKPWLPESKGRNVA

SEQ ID NO: 899 - protein, 12 aa, Homo sapiens
MQRIFHSIIQGY

SEQ ID NO: 900 - protein, 44 aa, Homo sapiens
MQTLALHALLFICVIWARFFNRLCLGESHLQSRDNNSTYLTGQL

SEQ ID NO: 901 - protein, 199 aa, Homo sapiens
MQVKAAPTPPSPSTAKAERRAPISWGTSVLARMQSPASNRDAASVGRRPRWLSSSRAPILAGMSTTPMNIWSRKMLLPRACRSRARPKKVKPKANQHNVEIQVRKRSPGMRSRVPRLAGGWPMLSSSRMAESKTSGVRVSCTAPFPLMAATLHSSCRPQSSLPVVRSHRADSASHQEYKKQRKKGTETTSCSSVQSRTP

SEQ ID NO: 902 - protein, 82 aa, Homo sapiens [sequence omitted]

SEQ ID NO: 903 - protein, 12 aa, Homo sapiens
MQYIVEIAYSNF

SEQ ID NO: 904 - protein, 116 aa, Homo sapiens
MQYKRINFLGFFHTQIRIMFLETRFWRFALDRQGRARSTGLSGGPSRGPGRRTGGLPGAPHAPLTHWPRRLRCHGDRARTYSPPAAVRRLHEPRRQPASSPAGCACPGPEASLLRQ

SEQ ID NO: 905 - protein, 33 aa, Homo sapiens
MQYKRINFLGFFHTQIRIMFLETRFWRLVRLQL

SEQ ID NO: 906 - protein, 24 aa, Homo sapiens
MQYYPFKIRAHSQTQNLSRILLGY

SEQ ID NO: 907 - protein, 16 aa, Homo sapiens
MRAKSWGFTLGLRLAS

SEQ ID NO: 908 - protein, 16 aa, Homo sapiens
MRALGAILIFLIRFLE

SEQ ID NO: 909 - protein, 14 aa, Homo sapiens
MRAPPSKTDTVVLI

SEQ ID NO: 910 - protein, 22 aa, Homo sapiens
MRCGIRVLLPSGHNLSDSAGLH

SEQ ID NO: 911 - protein, 88 aa, Homo sapiens
MRCLPWCRQPSEAPSQPGKDQAAGVTGRWGPGRSQAPLRAGAPPLSIAPHLRSTELGSALSPRGQGRFPWAGSLSLKIKMYPFLQWVT

SEQ ID NO: 912 - protein, 38 aa, Homo sapiens
MRCRRQSRQPAPSRLVTSRARRRTSEREGTAASTRRRA

SEQ ID NO: 913 - protein, 39 aa, Homo sapiens
MRCRRQSRQPAPSRLVTSRARRRTSEREGTAASTRRRAA

SEQ ID NO: 914 - protein, 41 aa, Homo sapiens
MRCRRQSRQPAPSRLVTSRARRRTSEREGTAASTRRRAAEN

SEQ ID NO: 915 - protein, 22 aa, Homo sapiens
MRDIAPGPAETGQMCIFPGPLC

SEQ ID NO: 916 - protein, 101 aa, Homo sapiens
MRDIAPGPALRSASAQVQRHSRGPAFCFPVWEKRVSGYFQEKKRKLSSHSRAGQSTSSSLPQLLCCCRLASNFASLWFSEKFYQEKRQEERSSLDYCLWGV

SEQ ID NO: 917 - protein, 100 aa, Homo sapiens
MRDIAPGPLRSASAQVQRHSRGPAFCFPVWEKRVSGYFQEKKRKLSSHSRAGQSTSSSLPQLLCCCRLASNFASLWFSEKFYQEKRQEERSSLDYCLWGV

SEQ ID NO: 918 - protein, 32 aa, Homo sapiens
MRFHHAGQASLKLLTSGDQPASASQSAENTGG

SEQ ID NO: 919 - protein, 40 aa, Homo sapiens
MRFHHIGQANLELLTSSHPPALASQSAGITGVSHCTQPCF

SEQ ID NO: 920 - protein, 16 aa, Homo sapiens
MRFHRVSQDGLDLLTS

SEQ ID NO: 921 - protein, 56 aa, Homo sapiens
MRFLSCSSSWSFASNSCIFFCFSKTDVLSISACFIIFRMYSNCFSNRLHLFSAANN

SEQ ID NO: 922 - protein, 44 aa, Homo sapiens
MRFLSCSSSWSFASNSCIFFSARACIVVSLLYSCSRRSNFSSWL

SEQ ID NO: 923 - protein, 51 aa, Homo sapiens
MRFMDRSMLTMLGHSQKLLAMTTSMRLACRYRYSSLPRPRSMPSVRLRSRL

SEQ ID NO: 924 - protein, 41 aa, Homo sapiens
MRFPHVGQAVLELLTSSYTPTLDSQSAGITGVSHGTSQKFL

SEQ ID NO: 925 - protein, 68 aa, Homo sapiens
MRFQHVGQAGIQFLTSSDPPASASLSAGITGISHRTRLRDTLYVSCVKVTRTSRRPICSSKWKKPCSN

SEQ ID NO: 926 - protein, 16 aa, Homo sapiens
MRFSFHYYIHTRVNQE

SEQ ID NO: 927 - protein, 39 aa, Homo sapiens
MRGEGRALGRSGLRLGQGWRARGPRAAPLPTAAAAAAAP

SEQ ID NO: 928 - protein, 50 aa, Homo sapiens
MRGGTDLCKRSQEKTDGASPIMRLLSRWSLSCVVALSLYKDTNFCERCHS

SEQ ID NO: 929 - protein, 18 aa, Homo sapiens
MRGVSGRRNSINGVLASV

SEQ ID NO: 930 - protein, 31 aa, Homo sapiens
MRHHARLSFYIFGRHGVSPRWPGWPRTPDLK

SEQ ID NO: 931 - protein, 25 aa, Homo sapiens
MRHHAWLIFCICSREGVSLYWSGWS

SEQ ID NO: 932 - protein, 11 aa, Homo sapiens
MRHHAWLILYF

SEQ ID NO: 933 - protein, 47 aa, Homo sapiens
MRHHAWLILYFFFSRDGGFSMLVRLVLNSRPQVNHPPRTSKVPRLQV

SEQ ID NO: 934 - protein, 11 aa, Homo sapiens
MRHHAWLILYY

SEQ ID NO: 935 - protein, 16 aa, Homo sapiens
MRHHAWPIFLCIFSRD

SEQ ID NO: 936 - protein, 12 aa, Homo sapiens
MRHHIWLILYFS

SEQ ID NO: 937 - protein, 11 aa, Homo sapiens
MRHHTWLILYF

SEQ ID NO: 938 - protein, 16 aa, Homo sapiens
MRHRWWRCARSGTRCR

SEQ ID NO: 939 - protein, 13 aa, Homo sapiens
MRHTEVLLVPDEG

SEQ ID NO: 940 - protein, 21 aa, Homo sapiens
MRKLLWPRGCETSLDFSSKYV

SEQ ID NO: 941 - protein, 13 aa, Homo sapiens
MRKLNLRVIRFQR

SEQ ID NO: 942 - protein, 27 aa, Homo sapiens
MRKNFIIFLSWPVFFQIQFKSYDKGWL

SEQ ID NO: 943 - protein, 11 aa, Homo sapiens
MRLARLWYTRL

SEQ ID NO: 944 - protein, 128 aa, Homo sapiens
MRLEGPWRPQSQCSSSEPSLQSGRPSHCGLGFFTQLRSSHWKVNVPHGTPSWHCSSSLPLRQSGCPSQTLGSEMHVLSSLHWNVALQTQFLSSRPLGQSLTPSQAGTQSPFTEQRNSPGQGSDWLYKP

SEQ ID NO: 945 - protein, 19 aa, Homo sapiens
MRLHHGPLNQSDFAPAGDI

SEQ ID NO: 946 - protein, 25 aa, Homo sapiens
MRLIVLSTVNLELTCSESNKLKYLY

SEQ ID NO: 947 - protein, 56 aa, Homo sapiens
MRLSEAELRSRSKFLFMRYWRKAVWMVLAALRLRKEPPYFLSSISTFLSCRSVESS

SEQ ID NO: 948 - protein, 18 aa, Homo sapiens
MRMCLTCALKLSLYIMKL

SEQ ID NO: 949 - protein, 23 aa, Homo sapiens
MRMIEFTNVAKLREFKSYPVSSF

SEQ ID NO: 950 - protein, 13 aa, Homo sapiens
MRNKFYCSASCYF

SEQ ID NO: 951 - protein, 41 aa, Homo sapiens
MRPETPRLRCCTFLAQSSKISCVLSFMRKLSPSCFSFCPST

SEQ ID NO: 952 - protein, 12 aa, Homo sapiens
MRPRRTMEKRVI

SEQ ID NO: 953 - protein, 14 aa, Homo sapiens
MRQSWNTSTLLVGM

SEQ ID NO: 954 - protein, 60 aa, Homo sapiens
MRRDMRLSEAELRSRSKFLFMRYWRKAVWMVLAALRLRKEPPYFLSSISTFLSCRSVESS

SEQ ID NO: 955 - protein, 23 aa, Homo sapiens
MRRTKEYLKQRRKPHVLITQETD

SEQ ID NO: 956 - protein, 24 aa, Homo sapiens
MRSFKIIISLENMSFIYLINKLQI

SEQ ID NO: 957 - protein, 37 aa, Homo sapiens
MRSLDRSSLCNQTPQLKVIFKAHLHLFFSYENILYIL

SEQ ID NO: 958 - protein, 22 aa, Homo sapiens
MRSLLLSPWRGVGGRSRGERWK

SEQ ID NO: 959 - protein, 14 aa, Homo sapiens
MRSNSFSKDHPGRS

SEQ ID NO: 960 - protein, 44 aa, Homo sapiens
MRTKAKAGALDKTTLSSRKLPMPLGGWDHHVLTMPRMAHSRNVW

SEQ ID NO: 961 - protein, 24 aa, Homo sapiens
MRVTAAGIMRAKSWGFTLGLRLAS

SEQ ID NO: 962 - protein, 13 aa, Homo sapiens
MRWHIQKLPLGYF

SEQ ID NO: 963 - protein, 21 aa, Homo sapiens
MRWLPSEMACCPSGWCLFGWT

SEQ ID NO: 964 - protein, 23 aa, Homo sapiens
MRYMVHLLRVTERSNNNLPRQRV

SEQ ID NO: 965 - protein, 20 aa, Homo sapiens
MSAEFHRLPLSPTSPWLSQS

SEQ ID NO: 966 - protein, 54 aa, Homo sapiens
MSAHCNLHLLGSSNYPASASQLAGITGVCHRAQLIFVFSVERSFTMLARLVLNS

SEQ ID NO: 967 - protein, 27 aa, Homo sapiens [sequence omitted]

SEQ ID NO: 968 - protein, 33 aa, Homo sapiens
MSATMSTQGSESRLASWMISIRAPFISHTHLLE

SEQ ID NO: 969 - protein, 100 aa, Homo sapiens
MSATMSTQGSESRLASWMISIRAPFISSTVRRGRCSVPSSNLSFTADERPWKQRRMLSMTAAVSRDAMLGGAHSSSVAPSLLCSHRPVSLSRMDAILGES

SEQ ID NO: 970 - protein, 25 aa, Homo sapiens
MSAVIIYHYIPIRKAEGGIPTEDKF

SEQ ID NO: 971 - protein, 46 aa, Homo sapiens
MSCIFSISYYHCLFKHLHGKYFPSICSCYFSYLKNLSIAPFTKYPK

SEQ ID NO: 972 - protein, 20 aa, Homo sapiens
MSCQDVLWSNNFPNIILSIY

SEQ ID NO: 973 - protein, 68 aa, Homo sapiens
MSCTLVTGPTRPVTQNGVDRDPRKHGRDTRRVTGLRWLCTQLPLQFPHTGFPFIPVIDAPGSAWKLCL

SEQ ID NO: 974 - protein, 67 aa, Homo sapiens
MSEEPPRRLDGILASAAGPTAFGGGPLGSPPSPPSAGSCQPGPAPQSSAVPTRNRSRLSSVSRGRQL

SEQ ID NO: 975 - protein, 26 aa, Homo sapiens
MSEKFATFITLVRSLHCGFSNDVQWL

SEQ ID NO: 976 - protein, 19 aa, Homo sapiens
MSERCMLFIKDSLYRYRYI

SEQ ID NO: 977 - protein, 17 aa, Homo sapiens
MSESSSTKSMSLKSHSA

SEQ ID NO: 978 - protein, 43 aa, Homo sapiens
MSFAATSMGLEAILLSKVVKKQSQMLHDLTYNWELNNVYAWAL

SEQ ID NO: 979 - protein, 62 aa, Homo sapiens
MSFAMSSDPTKHVKSQERTALDGTLEVQLLTMFRSALMMGLHCFTNSLASAKCLGVPPNSIR

SEQ ID NO: 980 - protein, 22 aa, Homo sapiens
MSFDHWRSLKSELHRGEGTCVF

SEQ ID NO: 981 - protein, 23 aa, Homo sapiens
MSFHSTSLSSRHTPEFHWVRTGK

SEQ ID NO: 982 - protein, 27 aa, Homo sapiens
MSFHWGHKHSLEALDFLPHQYTIFDHK

SEQ ID NO: 983 - protein, 12 aa, Homo sapiens
MSFIYLINKLQI

SEQ ID NO: 984 - protein, 32 aa, Homo sapiens
MSFLLSGAPFLVLPVRSILTRKSVRPCQHHFA

SEQ ID NO: 985 - protein, 11 aa, Homo sapiens
MSFLSFISCIR

SEQ ID NO: 986 - protein, 17 aa, Homo sapiens
MSFLTGFRNCQIMIYKK

SEQ ID NO: 987 - protein, 13 aa, Homo sapiens
MSFPSMRRSKIPS

SEQ ID NO: 988 - protein, 14 aa, Homo sapiens
MSFPSMRRSKIPSA

SEQ ID NO: 989 - protein, 20 aa, Homo sapiens
MSFQSTSPGSSGVSISHTGH

SEQ ID NO: 990 - protein, 18 aa, Homo sapiens
MSFSKSNSTFIYLTCAFC

SEQ ID NO: 991 - protein, 94 aa, Homo sapiens [sequence omitted]

SEQ ID NO: 992 - protein, 12 aa, Homo sapiens
MSGREKELKEYF

SEQ ID NO: 993 - protein, 65 aa, Homo sapiens
MSHHARLVFFFFFVFSVEMGFLPVGQAGLELPTSGDPPTLASQSAGIIGVSHCARPLPGILTRGR

SEQ ID NO: 994 - protein, 36 aa, Homo sapiens
MSHHLQLNFCGYFCTVISFWHNVLQYCCPISGTSPN

SEQ ID NO: 995 - protein, 11 aa, Homo sapiens
MSHHTRLILYF

SEQ ID NO: 996 - protein, 18 aa, Homo sapiens
MSHLHWSPPSSPQFPAAP

SEQ ID NO: 997 - protein, 13 aa, Homo sapiens
MSICISLLFFLSS

SEQ ID NO: 998 - protein, 28 aa, Homo sapiens
MSIHSDEELLPKMAQKLFSQAGLERSLQ

SEQ ID NO: 999 - protein, 75 aa, Homo sapiens [sequence omitted]

SEQ ID NO: 1000 - protein, 24 aa, Homo sapiens
MSILDSKNGKILGSRLASWNLAIP

SEQ ID NO: 1001 - protein, 53 aa, Homo sapiens
MSILHWLQLQDDTRVELTPVGQDRINEWSEMGFCRQRGTSGCRCYHSMTSEHW

SEQ ID NO: 1002 - protein, 11 aa, Homo sapiens
MSKFNERQNLT

SEQ ID NO: 1003 - protein, 11 aa, Homo sapiens
MSKGRAVAGNE

SEQ ID NO: 1004 - protein, 18 aa, Homo sapiens
MSKMKMSICISLLFFLSS

SEQ ID NO: 1005 - protein, 41 aa, Homo sapiens
MSLATRERYSSRVLAFRKTWLSISLLDLLCATPAFLMASSI

SEQ ID NO: 1006 - protein, 71 aa, Homo sapiens
MSLFRVSFSLRSTFCFFWSNSKCSTRPSSATSNGVWPSLFRISMSQSASARMEQASFTPQCAAAWRGVQPS

SEQ ID NO: 1007 - protein, 31 aa, Homo sapiens
MSLFTSNSGRIVYTSLIQLPTLSCLTISVDR

SEQ ID NO: 1008 - protein, 35 aa, Homo sapiens
MSLKVAWSLLSLLTWFRSKYQQFTGDNRFWSFLYC

SEQ ID NO: 1009 - protein, 96 aa, Homo sapiens
MSLLLPCGGGVIIWNRPCVPTRADPPGPSGKGTDGVCLRVQTLLAPQVKCLVYPLCHHCTSRGLHHSTSCLPLRVCPLHGEILEDRDSFPVCLPPP

SEQ ID NO: 1010 - protein, 37 aa, Homo sapiens
MSLRSRSFLQDTSWWSNRKNVRCWLLPCLVILVSSPE

SEQ ID NO: 1011 - protein, 25 aa, Homo sapiens
MSLSILLRLKLFLLSLNVWLLRTGT

SEQ ID NO: 1012 - protein, 21 aa, Homo sapiens
MSLSKCPAPGQDTGFSGPGAK

SEQ ID NO: 1013 - protein, 27 aa, Homo sapiens
MSLSQQHFEIKQRASGQAHFFKANFLI

SEQ ID NO: 1014 - protein, 37 aa, Homo sapiens
MSLTCPGDIFPIVLEINIQFLVTYANIYSQLEFLLRK

SEQ ID NO: 1015 - protein, 25 aa, Homo sapiens
MSLTFSGILFLLLEIQSEISVDACW

SEQ ID NO: 1016 - protein, 16 aa, Homo sapiens
MSLTSLDYPGPLPCIS

SEQ ID NO: 1017 - protein, 93 aa, Homo sapiens
MSLTSTSTWKTCSGLSTITSRWMLHSALRRHSSSRSIREFTNKMPFCRFTSRRPPRPLDATRNRRGTSSASSSPRSCAMRPTKVPCLASSETE

SEQ ID NO: 1018 - protein, 21 aa, Homo sapiens
MSMASEKLSLENYSRTFSYYI

SEQ ID NO: 1019 - protein, 19 aa, Homo sapiens
MSMNRYNFNYSKANMPKER

SEQ ID NO: 1020 - protein, 33 aa, Homo sapiens
MSNPRKHSIPTRDVNIILEELLAKDSFDKFNFF

SEQ ID NO: 1021 - protein, 25 aa, Homo sapiens
MSNSCPLSLLSLSSVWRTANMVSPF

SEQ ID NO: 1022 - protein, 36 aa, Homo sapiens
MSPIQTSNFIRAGYICFSARYRYQVMTDTYVRYTIN

SEQ ID NO: 1023 - protein, 66 aa, Homo sapiens
MSPMFFCACSIFFYLTASSPLAIKKFLKDVFFISFFSGGESFTLVAQAGVQRRDLGLLQPPPPRFK

SEQ ID NO: 1024 - protein, 42 aa, Homo sapiens
MSPSKDIFYKLIWKYNFTPEILIASHLHLKVWCFCTFLTNLI

SEQ ID NO: 1025 - protein, 12 aa, Homo sapiens
MSQGLVSAPEDQ

SEQ ID NO: 1026 - protein, 73 aa, Homo sapiens
MSQGVSLSKEECTRRFLSAPGHPPAPSRGYTLYLRQSISRLPGGPGILAVHLPIPADNGVTEAGPLGAEYTEQ

SEQ ID NO: 1027 - protein, 26 aa, Homo sapiens
MSQTLPTAAILRCLFSLLSSFELSSS

SEQ ID NO: 1028 - protein, 40 aa, Homo sapiens
MSRFSSFDNTSYASATSLNFLSASSLFSGFLSGCHLSATL

SEQ ID NO: 1029 - protein, 47 aa, Homo sapiens
MSRKWIMSLATRERYSSRVLAFRKTWLSISLLDLLCATPAFLMASSI

SEQ ID NO: 1030 - protein, 55 aa, Homo sapiens
MSRLECSGAIIAHCCLKLLCSSNPPASASRVGGTTGMCHHAQLIFLIIEKKKTQF

SEQ ID NO: 1031 - protein, 33 aa, Homo sapiens
MSRMVSASQPSGKIMQPRTRHRAAKSCIQAQIL

SEQ ID NO: 1032 - protein, 77 aa, Homo sapiens
MSRVEKGTYCDGVSTLLVAATLYLEGYLTLPPGWSSGYSWKHPSAHELTAEFQILGCPSAVACGSWALTPIPLGWTL

SEQ ID NO: 1033 - protein, 26 aa, Homo sapiens
MSRYNIVEMKLDQILVLFLTTITSSV

SEQ ID NO: 1034 - protein, 34 aa, Homo sapiens
MSSACLGLPKGREYRHEPPCLAPSSFFKPPRCKK

SEQ ID NO: 1035 - protein, 12 aa, Homo sapiens
MSSCHWVLFDLG

SEQ ID NO: 1036 - protein, 40 aa, Homo sapiens
MSSDLPVLASQSAAITGLSHYIWPPLHLFPLEGLQGQLYA

SEQ ID NO: 1037 - protein, 58 aa, Homo sapiens
MSSDPTKHVKSQERTALDGTLEVQLLTMFRSALMMGLHCFTNSLASAKCLGVPPNSIR

SEQ ID NO: 1038 - protein, 16 aa, Homo sapiens
MSSEMTRMLSRIWNIL

SEQ ID NO: 1039 - protein, 18 aa, Homo sapiens
MSSGWEQIQTNPAGIENG

SEQ ID NO: 1040 - protein, 52 aa, Homo sapiens
MSSHVWCSPTHVYRWGWWWGWRAEGKIMHVKHWKRKGVLWHNGIILSLRRKS

SEQ ID NO: 1041 - protein, 34 aa, Homo sapiens [sequence omitted]

SEQ ID NO: 1042 - protein, 23 aa, Homo sapiens
MSSLTDTSVLPFLLSLKEKPDSP

SEQ ID NO: 1043 - protein, 19 aa, Homo sapiens
MSSMYRQRMSTQVVNMSAR

SEQ ID NO: 1044 - protein, 32 aa, Homo sapiens
MSSQNSSVETLISKAMVLGGGANTISGPLGSE

SEQ ID NO: 1045 - protein, 13 aa, Homo sapiens
MSSRCWQCCRTAL

SEQ ID NO: 1046 - protein, 68 aa, Homo sapiens
MSSRPLSRTPPHGGGEMVRRPSGARGGGDPGRPGARAFSAASCQAGRPWRCGAAGGRAAAALWRAGST

SEQ ID NO: 1047 - protein, 32 aa, Homo sapiens
MSSSKLTAIIYLVYSLQLFFEVLLFSLYKSGT

SEQ ID NO: 1048 - protein, 29 aa, Homo sapiens
MSSSPRASYETLSPGTLGTVTISIICFCS

SEQ ID NO: 1049 - protein, 23 aa, Homo sapiens
MSSSRMVSVVLTSTLPSSSEHSR

SEQ ID NO: 1050 - protein, 14 aa, Homo sapiens
MSSSRSTSLLTGME

SEQ ID NO: 1051 - protein, 11 aa, Homo sapiens
MSSTLSISSIK

SEQ ID NO: 1052 - protein, 20 aa, Homo sapiens
MSSTWSRSQVESQGHQDEGD

SEQ ID NO: 1053 - protein, 62 aa, Homo sapiens
MSSVSTTALYCEYRSSRGSRRSRRSRRTVFSRWAPKYTLTLKACSRSKGSAAMTSSRNQVVT

SEQ ID NO: 1054 - protein, 21 aa, Homo sapiens
MSTCTLKIFRMAGPHLTVPFI

SEQ ID NO: 1055 - protein, 65 aa, Homo sapiens [sequence omitted]

SEQ ID NO: 1056 - protein, 29 aa, Homo sapiens
MSTQGSESRLASWMISIRAPFISHTHLLE

SEQ ID NO: 1057 - protein, 96 aa, Homo sapiens
MSTQGSESRLASWMISIRAPFISSTVRRGRCSVPSSNLSFTADERPWKQRRMLSMTAAVSRDAMLGGAHSSSVAPSLLCSHRPVSLSRMDAILGES

SEQ ID NO: 1058 - protein, 11 aa, Homo sapiens
MSTQVVNMSAR

SEQ ID NO: 1059 - protein, 77 aa, Homo sapiens
MSTSGLASDSEPHFRPVHLQRRPRGPILSLLTHIINIILDFLSKLGDNLQTPPLPVSQCLQGFRIWGRKQKISHMSC

SEQ ID NO: 1060 - protein, 16 aa, Homo sapiens
MSVFGRWPSTDFFCLF

SEQ ID NO: 1061 - protein, 15 aa, Homo sapiens
MSVFGRWPSTDFFLF

SEQ ID NO: 1062 - protein, 49 aa, Homo sapiens
MSVISASLLGRLRQENRWNPGGRGCSELRLHHYIPAGIPSFDSVPILSR

SEQ ID NO: 1063 - protein, 166 aa, Homo sapiens [sequence omitted]

SEQ ID NO: 1064 - protein, 27 aa, Homo sapiens
MSVRLVSNSRPQGIGPPRPPKVLRLQV

SEQ ID NO: 1065 - protein, 37 aa, Homo sapiens
MSVSPIPPLLCLLCDCIGKDSQDTLLPSRVVGPVLKT

SEQ ID NO: 1066 - protein, 18 aa, Homo sapiens
MSVVGLSLSSGATVFKGV

SEQ ID NO: 1067 - protein, 24 aa, Homo sapiens
MSVWREPAHVGMLVLEVSCSDALF

SEQ ID NO: 1068 - protein, 36 aa, Homo sapiens
MSWPPNFFCCWLKLSMITPMKRFRVKNEPKMIKTTK

SEQ ID NO: 1069 - protein, 14 aa, Homo sapiens
MSWTFHNLSHRNLN

SEQ ID NO: 1070 - protein, 18 aa, Homo sapiens
MSWVSPTPVKTPAKCPQN

SEQ ID NO: 1071 - protein, 23 aa, Homo sapiens
MSYCYVQNFWTMMKALLFFNISF

SEQ ID NO: 1072 - protein, 20 aa, Homo sapiens
MSYFFLRLKNNQYPSKVHTM

SEQ ID NO: 1073 - protein, 29 aa, Homo sapiens
MSYLLTIFTIHLLLPIFIYKFCSPVGQPM

SEQ ID NO: 1074 - protein, 21 aa, Homo sapiens
MSYQEQYMNYEIWKQTHFYIL

SEQ ID NO: 1075 - protein, 34 aa, Homo sapiens
MSYSWFAVGSKKQKSWYLCLVCEYKRWDSDCCNH

SEQ ID NO: 1076 - protein, 20 aa, Homo sapiens
MSYVYFNLKISDLFPLQLLY

SEQ ID NO: 1077 - protein, 58 aa, Homo sapiens
MTAAQGLEQSSPLPALGSPAFFAWSLPGKVAGVVLHTSKICNATRSPGPEPLMSQPLM

SEQ ID NO: 1078 - protein, 22 aa, Homo sapiens
MTACLPNESIFLLLMLCIYTHC

SEQ ID NO: 1079 - protein, 44 aa, Homo sapiens
MTAPNSLVFPILINSNSIFPITQAKTWSHSQHLSLYHSSHPIDQ

SEQ ID NO: 1080 - protein, 45 aa, Homo sapiens
MTCIVPLAYTSLDTAASKNPETGLKRWHGRQTWHSRWPRRSCSAW

SEQ ID NO: 1081 - protein, 19 aa, Homo sapiens
MTDYQIMVGKDATCNRKCV

SEQ ID NO: 1082 - protein, 65 aa, Homo sapiens
MTELPHPGQTFKRMANIFASCTPDPKPQATTHASALLVVPSQRPQPSRHLPDRRLAPSGLSGGLT

SEQ ID NO: 1083 - protein, 20 aa, Homo sapiens
MTEPSLTCSKQSPKCNMAQD

SEQ ID NO: 1084 - protein, 27 aa, Homo sapiens
MTFKCFIYTNNIANTNKSDALKHELLC

SEQ ID NO: 1085 - protein, 18 aa, Homo sapiens
MTFPVSSLVIIMQTALYY

SEQ ID NO: 1086 - protein, 46 aa, Homo sapiens
MTFVGFFSTVNSLMFNQVSVVRKTFSTLTTRIGLLTSMDPLMGYKV

SEQ ID NO: 1087 - protein, 13 aa, Homo sapiens
MTGCGHRQSQFLP

SEQ ID NO: 1088 - protein, 13 aa, Homo sapiens
MTGIYIDFRKVSV

SEQ ID NO: 1089 - protein, 32 aa, Homo sapiens
MTGWLYTKTRLHAKSGCNGASPQGRPCPLHSL

SEQ ID NO: 1090 - protein, 19 aa, Homo sapiens
MTHFVLIKMQLFQKINFEK

SEQ ID NO: 1091 - protein, 13 aa, Homo sapiens
MTIFSFCCLKKKK

SEQ ID NO: 1092 - protein, 43 aa, Homo sapiens
MTIFSFCSPSFPVLCCWAALQAFKLGPSERWPAPRVLGRSASP

SEQ ID NO: 1093 - protein, 36 aa, Homo sapiens
MTIFSFKHQPVVFKYYSYSIYREQSLLVWSKIMETS

SEQ ID NO: 1094 - protein, 26 aa, Homo sapiens
MTIIVSQLQQNGHCKSSAFSISKTIG

SEQ ID NO: 1095 - protein, 26 aa, Homo sapiens
MTITLDQFQFLFIFSENTPKINVNGK

SEQ ID NO: 1096 - protein, 16 aa, Homo sapiens
MTKLPNNTFLKTCLYC

SEQ ID NO: 1097 - protein, 12 aa, Homo sapiens
MTKMVIFPQGFM

SEQ ID NO: 1098 - protein, 71 aa, Homo sapiens [sequence omitted]

SEQ ID NO: 1099 - protein, 19 aa, Homo sapiens
MTLFGDQVFKLKGGHWEGP

SEQ ID NO: 1100 - protein, 27 aa, Homo sapiens
MTLHSGLSFSSEAQTLDVRIPFQRGVF

SEQ ID NO: 1101 - protein, 11 aa, Homo sapiens
MTLIIQVDLVK

SEQ ID NO: 1102 - protein, 91 aa, Homo sapiens [sequence omitted]

SEQ ID NO: 1103 - protein, 15 aa, Homo sapiens
MTLSGMLLKAGRLRN

SEQ ID NO: 1104 - protein, 41 aa, Homo sapiens
MTLTFVKVCLPMVSSEARSFMLSFQHNMKMKEMHFAKQNRP

SEQ ID NO: 1105 - protein, 18 aa, Homo sapiens
MTPDSCCSCPCITPSPSD

SEQ ID NO: 1106 - protein, 18 aa, Homo sapiens
MTPEQGFPPSTRLPLPAR

SEQ ID NO: 1107 - protein, 37 aa, Homo sapiens
MTPFTVVTISLSSEFTPSSITWSDQRMRLARLWYTRL

SEQ ID NO: 1108 - protein, 11 aa, Homo sapiens
MTQALVYGYLY

SEQ ID NO: 1109 - protein, 21 aa, Homo sapiens
MTQLDPFILQNISLKFSFVFH

SEQ ID NO: 1110 - protein, 40 aa, Homo sapiens [sequence omitted]

SEQ ID NO: 1111 - protein, 46 aa, Homo sapiens
MTQRASHKATWMIKLLCGPIAWHCGSKFQLFYIFSSCYLLPHPHVF

SEQ ID NO: 1112 - protein, 25 aa, Homo sapiens
MTQSNDAFVCDIPTGYYFHFQYGFL

SEQ ID NO: 1113 - protein, 26 aa, Homo sapiens
MTREPVKVVHREVKLPCFKVIVGNRK

SEQ ID NO: 1114 - protein, 51 aa, Homo sapiens
MTRKLSTRCGEKSILIQPFYFILFYFILFYFIFEKGSHSVTQAEVQWCHHR

SEQ ID NO: 1115 - protein, 12 aa, Homo sapiens
MTRMLSRIWNIL

SEQ ID NO: 1116 - protein, 24 aa, Homo sapiens
MTRPKTVWSRSRVVQFQRWWRNWC

SEQ ID NO: 1117 - protein, 70 aa, Homo sapiens
MTRVVQLCLGLQLQARLWAQLDLRLWVRSHWGPGSSSGSLTSARRGLPRPVLGRRPAAVSPPGSARSRGA

SEQ ID NO: 1118 - protein, 39 aa, Homo sapiens
MTSGDPPAPASQSAGIIGVSYHARPIMGISKMLIFNSTI

SEQ ID NO: 1119 - protein, 16 aa, Homo sapiens
MTSHNGQRQLRSGALS

SEQ ID NO: 1120 - protein, 61 aa, Homo sapiens
MTSRCLVPFTMACTRSSGLICSSFKYHLTEVTSGTDTLHSSTALVPSITLTSFRGVITSTL

SEQ ID NO: 1121 - protein, 28 aa, Homo sapiens
MTTAEITNEGKWNGFPVGYHMMQECSHP

SEQ ID NO: 1122 - protein, 69 aa, Homo sapiens [sequence omitted]

SEQ ID NO: 1123 - protein, 17 aa, Homo sapiens
MTTGVEVDRKTMSKISS

SEQ ID NO: 1124 - protein, 51 aa, Homo sapiens
MTTSTEAPLLGVCMKQPRTCEAKRRISNCFPHDFIVSWGPCFGRSGCLPWA

SEQ ID NO: 1125 - protein, 32 aa, Homo sapiens
MTVFSIVFYIASFIKPPQFFNGLWNFCTFFLC

SEQ ID NO: 1126 - protein, 18 aa, Homo sapiens
MTVPRKPMMRILVRISTQ

SEQ ID NO: 1127 - protein, 24 aa, Homo sapiens
MVAASSSVGAGTSERTGLQVTVRC

SEQ ID NO: 1128 - protein, 11 aa, Homo sapiens
MVAFCKICGCL

SEQ ID NO: 1129 - protein, 24 aa, Homo sapiens
MVAGGGAWGSSCQGRKAQCPAPSA

SEQ ID NO: 1130 - protein, 31 aa, Homo sapiens
MVAHDCYPSTLRGQGRRITLKLVQKPAWATK

SEQ ID NO: 1131 - protein, 27 aa, Homo sapiens
MVAREGVAPGWPQLRGEHSKQSASDGE

SEQ ID NO: 1132 - protein, 11 aa, Homo sapiens
MVARGRVSRAP

SEQ ID NO: 1133 - protein, 27 aa, Homo sapiens
MVAYHCNLSTEAGGSLGPKSSRPAWAT

SEQ ID NO: 1134 - protein, 14 aa, Homo sapiens
MVCGNDRNLKWQIY

SEQ ID NO: 1135 - protein, 24 aa, Homo sapiens
MVCIYICLYLYRYRGYIQWSTTQP

SEQ ID NO: 1136 - protein, 15 aa, Homo sapiens
MVCPPWPPKVLGLQA

SEQ ID NO: 1137 - protein, 26 aa, Homo sapiens
MVCTFFLNIIESRSFVILGIINLIKT

SEQ ID NO: 1138 - protein, 74 aa, Homo sapiens
MVDASPRTVPPQPGTPATPAGGWRQQPPPWRPQPLPPPQCPAKGSEEARWKGKKRGAAKADWRAAPPATGVERS

SEQ ID NO: 1139 - protein, 186 aa, Homo sapiens
MVDASPRTVPPQPGTPATPAGGWRQQPPPWRPQPLPPPQCPAKGSEEARWKGKKRGAAKADWRAAPPATGVERSGVRPGRSRRAENPGAEAALPSGMRRGGSRAPLGGGRRGGAEPRLRAAAARSCRSPPHHLPPRRRLPLNPRRRLGRSSGAGRAGLGAPRRRIPPDTLQPGLLLRGVEGAAGSV

SEQ ID NO: 1140 - protein, 48 aa, Homo sapiens
MVDDDGFDNFIHMCLARHLILYFWDRHQCWAKANGQVIRVHHILIAVL

SEQ ID NO: 1141 - protein, 36 aa, Homo sapiens
MVEDFQRDFNKSKIILNVLSPVDSKTIIIASYTSSW

SEQ ID NO: 1142 - protein, 127 aa, Homo sapiens
MVEMCEEWNSLSVKRHSRQVLPTPESPISSSRNSTSYCFAMTGASGAGNCGRAAGSALLRRCHRGPRPPGDAAGGEEDAGPGPRGCLARPPAHSLAGCREARLRREPGAAPARLGSARLGWREAVGG

SEQ ID NO: 1143 - protein, 38 aa, Homo sapiens [sequence omitted]

SEQ ID NO: 1144 - protein, 36 aa, Homo sapiens
MVETTTATRPEPAMSSSRMVSVVLTSTLPSSSEHSR

SEQ ID NO: 1145 - protein, 44 aa, Homo sapiens
MVFAFSPYLVQEQIPAVHWRQQVLVFLVLLMILSASCFCHEPFC

SEQ ID NO: 1146 - protein, 158 aa, Homo sapiens [sequence omitted]

SEQ ID NO: 1147 - protein, 13 aa, Homo sapiens
MVGKDATCNRKCV

SEQ ID NO: 1148 - protein, 29 aa, Homo sapiens [sequence omitted]

SEQ ID NO: 1149 - protein, 12 aa, Homo sapiens
MVGLMSETGLSD

SEQ ID NO: 1150 - protein, 27 aa, Homo sapiens
MVGMVVVFHQVPQFGACLLVRRNHGCP

SEQ ID NO: 1151 - protein, 39 aa, Homo sapiens
MVGTAPGLESGATLGRGRAQRGSFQSPVQGQASASEPSG

SEQ ID NO: 1152 - protein, 15 aa, Homo sapiens
MVGVIIEHSYSGKVR

SEQ ID NO: 1153 - protein, 20 aa, Homo sapiens
MVHLLRVTERSNNNLPRQRV

SEQ ID NO: 1154 - protein, 15 aa, Homo sapiens
MVHPPQPPKVLGLQA

SEQ ID NO: 1155 - protein, 27 aa, Homo sapiens
MVICIDRAHHQQIYHNRRFLLFYLTAS

SEQ ID NO: 1156 - protein, 68 aa, Homo sapiens
MVIFPLSQHLIKHIPLFLKSMKGSVTGEVGTIVSLWLKGDSLSRGRHHQRDLGNTALIGSSKAALQSW

SEQ ID NO: 1157 - protein, 21 aa, Homo sapiens
MVILTTCPVDAVCYFITVSRQ

SEQ ID NO: 1158 - protein, 11 aa, Homo sapiens
MVIWYSCPNGL

SEQ ID NO: 1159 - protein, 13 aa, Homo sapiens
MVKKYLKIQFSPL

SEQ ID NO: 1160 - protein, 22 aa, Homo sapiens
MVKLQFFFLIAAGCNHTDILPV

SEQ ID NO: 1161 - protein, 44 aa, Homo sapiens
MVKMRPETPRLRCCTFLAQSSKISCVLSFMRKLSPSCFSFCPST

SEQ ID NO: 1162 - protein, 14 aa, Homo sapiens
MVLIISFTCAWQDT

SEQ ID NO: 1163 - protein, 16 aa, Homo sapiens
MVLPCWPGWSQTPDLR

SEQ ID NO: 1164 - protein, 33 aa, Homo sapiens
MVLSLEADRIHFLLLLMATSITQSLWPFKESFR

SEQ ID NO: 1165 - protein, 38 aa, Homo sapiens
MVLTSRPCDPPTSASQSAGITGVSHHAWPIIINQLLIK

SEQ ID NO: 1166 - protein, 40 aa, Homo sapiens
MVLWTSPNPKQPQQFVPSTKISSFTVVYKTSLPALPKTQA

SEQ ID NO: 1167 - protein, 201 aa, Homo sapiens
MVMQVKAAPTPPSPSTAKAERRAPISWGTSVLARMQSPASNRDAASVGRRPRWLSSSRAPILAGMSTTPMNIWSRKMLLPRACRSRARPKKVKPKANQHNVEIQVRKRSPGMRSRVPRLAGGWPMLSSSRMAESKTSGVRVSCTAPFPLMAATLHSSCRPQSSLPVVRSHRADSASHQEYKKQRKKGTETTSCSSVQSRTP

SEQ ID NO: 1168 - protein, 18 aa, Homo sapiens
MVMSSEMTRMLSRIWNIL

SEQ ID NO: 1169 - protein, 13 aa, Homo sapiens
MVNHKGMILKRPL

SEQ ID NO: 1170 - protein, 21 aa, Homo sapiens
MVPGSRTSLRLIYQRMFKSLR

SEQ ID NO: 1171 - protein, 43 aa, Homo sapiens
MVRIGCPLLLSLRVPGGSGTKGQTGRELEQGRQETRRRPRAVA

SEQ ID NO: 1172 - protein, 13 aa, Homo sapiens
MVRILITRCQHTD

SEQ ID NO: 1173 - protein, 52 aa, Homo sapiens
MVRRPSGARGGGDPGRPGARAFSAASCQAGRPWRCGAAGGRAAAALWRAGST

SEQ ID NO: 1174 - protein, 30 aa, Homo sapiens
MVSASQPSGKIMQPRTRHRAAKSCIQAQIL

SEQ ID NO: 1175 - protein, 95 aa, Homo sapiens
MVSATRPARPVPALPAANDPAARVRPLVRRRRPRALSARLAAPARRQPLPRVILAARRPLAAAPEPRSPLRAAAAAGEEPRGVSAWRAPSLPRTS

SEQ ID NO: 1176 - protein, 41 aa, Homo sapiens
MVSISGPCDPPASASQSAGITGVSHHAQPGTSNFLSLCVCE

SEQ ID NO: 1177 - protein, 34 aa, Homo sapiens
MVSISWPRDPTISASQSAGFKGMSHCAWPRILYC

SEQ ID NO: 1178 - protein, 52 aa, Homo sapiens
MVSLPFSNSYMLMLLVQTLPFFLSLTKSFRTIFFSLLVLSLQCRLPSGGIPN

SEQ ID NO: 1179 - protein, 26 aa, Homo sapiens
MVSPVCGCSYYLPQLISNAVLPASLR

SEQ ID NO: 1180 - protein, 81 aa, Homo sapiens
MVSPVCGCSYYLPQLISNFMNVEDSLFLGVLGSLSQSSSRSKLPFAQGTKPQCCPPHCARLPCARWRTGPRALVGGGKLRR

SEQ ID NO: 1181 - protein, 24 aa, Homo sapiens
MVSPVCGCSYYLPQLISNMIHMYR

SEQ ID NO: 1182 - protein, 18 aa, Homo sapiens
MVSVVLTSTLPSSSEHSR

SEQ ID NO: 1183 - protein, 31 aa, Homo sapiens
MVTDPSRGNALLIDTSKLALCALPGSTVFLI

SEQ ID NO: 1184 - protein, 33 aa, Homo sapiens
MVTNVARARSSLLMESRFSLLIMLPKLDATADP

SEQ ID NO: 1185 - protein, 33 aa, Homo sapiens
MVTNVARARSSLLMESRFSLLIMLPKLVPVTLL

SEQ ID NO: 1186 - protein, 22 aa, Homo sapiens
MVVCISVGSVVISPLSFFIASI

SEQ ID NO: 1187 - protein, 14 aa, Homo sapiens
MVVFVCFVLLKQNT

SEQ ID NO: 1188 - protein, 16 aa, Homo sapiens
MVVMTGCGHRQSQFLP

SEQ ID NO: 1189 - protein, 11 aa, Homo sapiens
MVVMTGIFSGI

SEQ ID NO: 1190 - protein, 24 aa, Homo sapiens
MVVVFHQVPQFGACLLVRRNHGCP

SEQ ID NO: 1191 - protein, 12 aa, Homo sapiens
MVWLSSPIQISS

SEQ ID NO: 1192 - protein, 24 aa, Homo sapiens
MVYLAPVKHHILYPFHHRGQPQHH

SEQ ID NO: 1193 - protein, 22 aa, Homo sapiens
MVYLVTNPVLKLLWNLLHECLR

SEQ ID NO: 1194 - protein, 124 aa, Homo sapiens
MWCGKGAGAPSRVCPSPTALPGGQSAPSLQPPRPALPWSPADSSTPGSCAQSSSAAPPVAGSEGSGCMFTSATPNAPQLWGAQVRGGRRYGPSPAREYPLSFFASRWRPSLYSPTLPRSPRQPL

SEQ ID NO: 1195 - protein, 30 aa, Homo sapiens
MWDDTCWKNWILTHCWYSLFPSHESVKAGS

SEQ ID NO: 1196 - protein, 24 aa, Homo sapiens
MWDIIKLSTYPPTHLLTYLQAIYL

SEQ ID NO: 1197 - protein, 34 aa, Homo sapiens
MWDIQINVRNFIVNSLITSFHLVYSNGRRLPKGL

SEQ ID NO: 1198 - protein, 28 aa, Homo sapiens
MWEQTTLSSFCLSSSRMIGVLFTKRNPP

SEQ ID NO: 1199 - protein, 25 aa, Homo sapiens
MWFCHVGQAGLELLTSSDLPTIHNI

SEQ ID NO: 1200 - protein, 58 aa, Homo sapiens
MWHHTQLIFVFVVETRFHHVGQAGVEPLTSGDPPTLASQSATITGMSHCAWPIFRFLT

SEQ ID NO: 1201 - protein, 13 aa, Homo sapiens
MWKIPCFLGFWGP

SEQ ID NO: 1202 - protein, 13 aa, Homo sapiens
MWLKFLYAQAENA

SEQ ID NO: 1203 - protein, 34 aa, Homo sapiens
MWLLEPDFSMLEQLTAGKLGVRISVFEAHIHHLK

SEQ ID NO: 1204 - protein, 18 aa, Homo sapiens
MWLVLKEISSSLSTCVDS

SEQ ID NO: 1205 - protein, 47 aa, Homo sapiens
MWNRTSGEDRVKAPFSILLFFRILASLFSPRRLVVISSFMFAESILN

SEQ ID NO: 1206 - protein, 14 aa, Homo sapiens
MWRNSNAFTPLVGV

SEQ ID NO: 1207 - protein, 37 aa, Homo sapiens
MWRNWNPHLPLVGISNGAASVGNNLAVPQIVKHGVTV

SEQ ID NO: 1208 - protein, 34 aa, Homo sapiens
MWSFSCALMGGDTWRRLGRGNWELGLILLLFQHV

SEQ ID NO: 1209 - protein, 21 aa, Homo sapiens
MWSKLILNSWAQVILPPQPPE

SEQ ID NO: 1210 - protein, 31 aa, Homo sapiens
MYDLILFLSPSPPPLCSSHTGLLVLNTPNTY

SEQ ID NO: 1211 - protein, 18 aa, Homo sapiens
MYFFVCLISLGRTSSQIE

SEQ ID NO: 1212 - protein, 37 aa, Homo sapiens
MYFIKAGTFSTIISSNIMSLSLFLLLLGLPSCIYWYA

SEQ ID NO: 1213 - protein, 25 aa, Homo sapiens
MYFKTFILQITYVHKNTYIHIHKDT

SEQ ID NO: 1214 - protein, 15 aa, Homo sapiens
MYFWELLSNPRTKEC

SEQ ID NO: 1215 - protein, 24 aa, Homo sapiens
MYGKYMYLLCFVIIFSVTKNFQFC

SEQ ID NO: 1216 - protein, 45 aa, Homo sapiens [sequence omitted]

SEQ ID NO: 1217 - protein, 61 aa, Homo sapiens
MYHKISTRGKDFPTYMTFVGFFSTVNSLMFNQVSVVRKTFSTLTTRIGLLTSMDPLMGYKV

SEQ ID NO: 1218 - protein, 24 aa, Homo sapiens
MYIKIHTYIFIKIHRDFSLQQCPY

SEQ ID NO: 1219 - protein, 13 aa, Homo sapiens
MYINKNVSHFLIY

SEQ ID NO: 1220 - protein, 23 aa, Homo sapiens
MYKAEQLIKRHLETAKTHSFHVT

SEQ ID NO: 1221 - protein, 21 aa, Homo sapiens
MYKFWLRLAVVSSHRTAVQNT

SEQ ID NO: 1222 - protein, 13 aa, Homo sapiens
MYKKKKVQMCLAN

SEQ ID NO: 1223 - protein, 18 aa, Homo sapiens
MYLANFFCIFSRDGVSPC

SEQ ID NO: 1224 - protein, 16 aa, Homo sapiens
MYLISYDLLFFIITLT

SEQ ID NO: 1225 - protein, 19 aa, Homo sapiens
MYLLCFVIIFSVTKNFQFC

SEQ ID NO: 1226 - protein, 20 aa, Homo sapiens
MYLLDKAHNCRSALLISKGN

SEQ ID NO: 1227 - protein, 33 aa, Homo sapiens
MYLPLPVNVVVRTRFQHAGAANGREVRSQNICV

SEQ ID NO: 1228 - protein, 11 aa, Homo sapiens
MYNWTWMSLSG

SEQ ID NO: 1229 - protein, 20 aa, Homo sapiens
MYPDLILCSVRVTVNFNFHA

SEQ ID NO: 1230 - protein, 113 aa, Homo sapiens
MYRAEVERGRRVGEQEHLEKNRGAQAHLIKMLKCFNSSILQSSQKRGMQAQKAKAGAYGHMPPAAGSGASGTERECHPNMPQLSPPRKRKARYTSHHSKTSLTGENRFTCFVH

SEQ ID NO: 1231 - protein, 32 aa, Homo sapiens [sequence omitted]

SEQ ID NO: 1232 - protein, 43 aa, Homo sapiens
MYRKKQCIQGSVLSAVLDIHWECWNVFPKDKGRLQYKHPKRLF

SEQ ID NO: 1233 - protein, 16 aa, Homo sapiens
MYRQRMSTQVVNMSAR

SEQ ID NO: 1234 - protein, 56 aa, Homo sapiens
MYSMSILHWLQLQDDTRVELTPVGQDRINEWSEMGFCRQRGTSGCRCYHSMTSEHW

SEQ ID NO: 1235 - protein, 80 aa, Homo sapiens
MYSTVLAFLINPYCLEETSFQLSDILSRISRGARILALLVSTMQPFNTISSKMMCTLSKLNIISNSLTRLKYSSKTSTKL

SEQ ID NO: 1236 - protein, 22 aa, Homo sapiens
MYTFEKIYTIFQNKPFKTIFKQ

SEQ ID NO: 1237 - protein, 19 aa, Homo sapiens
MYVCIGKNNAYRVQYYLQF

SEQ ID NO: 1238 - protein, 18 aa, Homo sapiens
MYVLHVFNVNSTLVTATR

SEQ ID NO: 1239 - protein, 26 aa, Homo sapiens
MYVLMIVLSVCLLLHVLASLDAFALV

SEQ ID NO: 1240 - protein, 102 aa, Homo sapiens [sequence omitted]

SEQ ID NO: 1241 - protein, 37 aa, Homo sapiens
MAAAARRLQTTTPPYRKLQTAADLCSRRAGTTQERRT

SEQ ID NO: 1242 - protein, 51 aa, Homo sapiens
MAAQLDPRWRRSVEAPGCPYLPVWGTCHLLLSRNGARCFLPWGLHLLSLLG

SEQ ID NO: 1243 - protein, 45 aa, Homo sapiens
MAARAPSPPCQARALGSCCRFPLGLGRGKEGTALRLRNLYCDFGR

SEQ ID NO: 1244 - protein, 14 aa, Homo sapiens
MACLFIILAVFFKE

SEQ ID NO: 1245 - protein, 71 aa, Homo sapiens
MACTQSSMSRWELAMSRSASGLAGTFSRSPAPPGLISKRCFPGSSGPGGSSVTCVPCREINPWGLISSLSL

SEQ ID NO: 1246 - protein, 14 aa, Homo sapiens
MADPMSPVPIQCLL

SEQ ID NO: 1247 - protein, 15 aa, Homo sapiens
MAFLMDGKQERERGS

SEQ ID NO: 1248 - protein, 81 aa, Homo sapiens
MAGAASCARGRGRGAPQAGRGRGRCRRLSRQPGPERGGSCGADPDRPRGAVVLQLARGGERPFGAQLAAAAAAASAAAAAR

SEQ ID NO: 1249 - protein, 24 aa, Homo sapiens
MAGGHGSLVLIHLRVWRLTGGLAL

SEQ ID NO: 1250 - protein, 32 aa, Homo sapiens
MAGRGRSAGALSGRASAPRPTQGLGTPRRQGG

SEQ ID NO: 1251 - protein, 127 aa, Homo sapiens
MAGRGRSAGALSGRASAPRPTQGLGTPRRQGGWARRAAGGGAGRDGRRPRPQRGPWSARRATPVLAPGREDADATASRPGLLCGLGLSANPSVAAVPASPAVAAVRAAQGRWASSCSHPLGAVPASP

SEQ ID NO: 1252 - protein, 13 aa, Homo sapiens
MAGRSISVSALKK

SEQ ID NO: 1253 - protein, 157 aa, Homo sapiens
MAIIEKSGNNRCWRGCGEIGTLLHCWWDCKLVQPLWKTVWQFLKDPELEIPFDSAIPLLGIYPKDYKSCCYKDTCTRYVYCDTVHNSKDLEPIQMSTMIDWIKKMWHIYTMEYYAAIKKDEFMSFVGTWMKVETIILSKLSQGRKTKHLMFSLIGGN

SEQ ID NO: 1254 - protein, 42 aa, Homo sapiens
MAIKAKTDKWDLIKELLHGKRNYDQSEQATYRMGETFCNLSI

SEQ ID NO: 1255 - protein, 18 aa, Homo sapiens
MAIYLGETSFRWKLIVIL

SEQ ID NO: 1256 - protein, 62 aa, Homo sapiens
MAKARVFPLPVSAAPRMSSLSRMAGAKVRAWIGVGAEKPRKLSARRTGLGTNRSFQADTSAF

SEQ ID NO: 1257 - protein, 45 aa, Homo sapiens
MAKETMIRVNRQPTEWEKLFAIYPSDKGLISRIYKELKFTRKKSH

SEQ ID NO: 1258 - protein, 22 aa, Homo sapiens
MAKSHHFSVWSYSIVALCKLFK

SEQ ID NO: 1259 - protein, 49 aa, Homo sapiens
MALGRDAALAHPFALSGQTGRERNSGAGSRSSWVPIQAPHSPALRFGTT

SEQ ID NO: 1260 - protein, 36 aa, Homo sapiens
MALRERRMKVTNEDFKKSKENVLYKKQEGTPEGLYL

SEQ ID NO: 1261 - protein, 41 aa, Homo sapiens
MALRGTDAKPGTGLPSSWNLPVRPRTSVQLEWAPQKEKQYS

SEQ ID NO: 1262 - protein, 85 aa, Homo sapiens
MALSLNATGQQSPPLCLVLPQDSPECPIESPGTAPRDGWQGLPAHRRQERTFPLPIPAITSDATVAIPTNPSSQLPLSTFPKHLA

SEQ ID NO: 1263 - protein, 19 aa, Homo sapiens
MALSRLVSSLQSESKKMSL

SEQ ID NO: 1264 - protein, 26 aa, Homo sapiens
MALYRSPLASQNWGVQLAYSQAPTAP

SEQ ID NO: 1265 - protein, 86 aa, Homo sapiens
MALYRSPLASQNWGVQLAYSQAPTAPSSTMRSPSFREAPCPAQVLFIWATRARLLFSLVSSSSLAAGLSSSSNSSRTVMLATMVMA

SEQ ID NO: 1266 - protein, 55 aa, Homo sapiens
MAMFYHLAKKGKLPSDSNLHGPSVSSLNMWYEDRKCWSCLIQTWVQISFPPCLAM

SEQ ID NO: 1267 - protein, 23 aa, Homo sapiens
MAMSSGISSLSMSSSLSSANCGS

SEQ ID NO: 1268 - protein, 89 aa, Homo sapiens
MAMVITTIIAIIKLLIVTGCPTFLRFSSAICDSFLICPQVGGCVRWVLLVTVGVPLSVSLNMAATRGSSGSSQNLFLSIRLMIRFQVPR

SEQ ID NO: 1269 - protein, 19 aa, Homo sapiens
MANIKNSDSVNVDRHVKQL

SEQ ID NO: 1270 - protein, 34 aa, Homo sapiens
MANLMENSLNSLYNFFFVSNSSSALHTVSSRNCP

SEQ ID NO: 1271 - protein, 14 aa, Homo sapiens
MANRREKGVLKEYN

SEQ ID NO: 1272 - protein, 27 aa, Homo sapiens
MAPQMQQWRKIPPKTRKVPLQPRFSRR

SEQ ID NO: 1273 - protein, 22 aa, Homo sapiens
MAQQRVGTQEAQADVGGLGELT

SEQ ID NO: 1274 - protein, 52 aa, Homo sapiens
MAQQSTGRPYRCRPTTSGARYSGVPQGSLMRPFSSLARWKSLMTIFEFFSRL

SEQ ID NO: 1275 - protein, 14 aa, Homo sapiens
MARAHIAQGRTHPL

SEQ ID NO: 1276 - protein, 29 aa, Homo sapiens
MARLTRAFLLGSCISLNRAASLSQGNILY

SEQ ID NO: 1277 - protein, 24 aa, Homo sapiens
MARNCSNISSSRICSLECTSGLNH

SEQ ID NO: 1278 - protein, 22 aa, Homo sapiens
MARRSPLSRSSWKKCRMSPSTI

SEQ ID NO: 1279 - protein, 89 aa, Homo sapiens
MASCFFLAASTAARSYPKLSWATRRWFSLSQVSLIAAFRSKRRASCSSFSCRMSSFLRASSRRYSASSRLSQALLMSDTSFPSWGVYTF

SEQ ID NO: 1280 - protein, 13 aa, Homo sapiens
MASCSSWKHFTIL

SEQ ID NO: 1281 - protein, 20 aa, Homo sapiens
MASIKLGPWFRLFSVSETCS

SEQ ID NO: 1282 - protein, 14 aa, Homo sapiens
MASIRSSVHSRSFS

SEQ ID NO: 1283 - protein, 136 aa, Homo sapiens [sequence omitted]

SEQ ID NO: 1284 - protein, 39 aa, Homo sapiens
MASPPPPSAGWSLRGAARTGWAAGAAEAPSPRSPRSSRG

SEQ ID NO: 1285 - protein, 151 aa, Homo sapiens
MASRSSRLSMSSRKSLSSLKSIASKKSGSSRKSVSSSKSTSSNKAMSSRLSMSSRKSLSSLKSIASEKSRSSRKSVSSSKSTSSNKAMSSIKLMSSSLLVSSNKGTSSNKGTSSNKGMSSNKGTSSRKSTSSNQAMSSRKSTSSRKYMSSN

SEQ ID NO: 1286 - protein, 13 aa, Homo sapiens
MASVRWSSCLSRS

SEQ ID NO: 1287 - protein, 47 aa, Homo sapiens
MASWKRCIRSQYVSGSKLSNRCSLPSLSKQLMLSGMKSWARRGSPYR

SEQ ID NO: 1288 - protein, 32 aa, Homo sapiens
MASWKRCIRSQYVSGSKPSRRVLLRSPPSSAA

SEQ ID NO: 1289 - protein, 69 aa, Homo sapiens
MATEAKIDKWDLIKLKSFCTAKETTIRVNRQPTKWEKIFAIYSSDKGLISRIYKELKQTYKKKTNPIKK

SEQ ID NO: 1290 - protein, 34 aa, Homo sapiens
MATKAKIDKWDLIKLKSFCTAKETTIRVNRQHTE

SEQ ID NO: 1291 - protein, 74 aa, Homo sapiens
MATSLLQQPVGCGAADEARVPRFFHVQHSAFSITGTRGDFRKQAPRCHHQAQKYLSHFADFLQTQYSLFHGLSF

SEQ ID NO: 1292 - protein, 151 aa, Homo sapiens
MAVAALGAEPGRAGPGRAGGAAGTRERVRSAGSGAGSRRVPGDPGEEGMQSRRAAPGPRRCTEPGGPGDADRSVPRESGRTGPGGSGAPGSWVPEDLGGGPGQEGAGGRDSGCTVIWRSAAGPTGIRGFGGARRPGSELGSCCAAHVLTSA

SEQ ID NO: 1293 - protein, 17 aa, Homo sapiens
MAVKYSPNSCSSFMALS

SEQ ID NO: 1294 - protein, 49 aa, Homo sapiens
MAVLDLKARCPNFLFCALFIMQGYTGYKFEIKCVNPFTAIKKYLRLGNL

SEQ ID NO: 1295 - protein, 12 aa, Homo sapiens
MAYRPGLFMTSS

SEQ ID NO: 1296 - protein, 22 aa, Homo sapiens
MCALALISVQFHLKQKSLLQIF

SEQ ID NO: 1297 - protein, 77 aa, Homo sapiens
MCCSCVYSTSVISTRLRSVVVKLSPGSPSAASPPPAPSTAASPPAAPASGGGSRGPGPDMAARRGPTAARATRAAGG

SEQ ID NO: 1298 - protein, 110 aa, Homo sapiens
MCCSCVYSTSVISTRLRSVVVKLSPGSPSAASPPPAPSTAASPPAAPASGGGSRGPGPDMAARRGPTAARATRAAGGGRREAGGGRRPPARALLCAGHSRRAVGGGKTAE

SEQ ID NO: 1299 - protein, 51 aa, Homo sapiens
MCENIIFFTTRGKQKSFTVVRILTITSSDLTFFLRFDIFLRSYLSFYFHSE

SEQ ID NO: 1300 - protein, 82 aa, Homo sapiens
MCEQRMCCSCVYSTSVISTRLRSVVVKLSPGSPSAASPPPAPSTAASPPAAPASGGGSRGPGPDMAARRGPTAARATRAAGG

SEQ ID NO: 1301 - protein, 115 aa, Homo sapiens
MCEQRMCCSCVYSTSVISTRLRSVVVKLSPGSPSAASPPPAPSTAASPPAAPASGGGSRGPGPDMAARRGPTAARATRAAGGGRREAGGGRRPPARALLCAGHSRRAVGGGKTAE

SEQ ID NO: 1302 - protein, 60 aa, Homo sapiens [sequence omitted]

SEQ ID NO: 1303 - protein, 14 aa, Homo sapiens
MCFNSSFLNAGSDC

SEQ ID NO: 1304 - protein, 77 aa, Homo sapiens
MCGDAKATSGAAGRTGGVNVGVGVGERESRRGAGWLPAADGGRDGLAGRSQEQQRDTERKRRDLRRRHTFYSPRKRA

SEQ ID NO: 1305 - protein, 19 aa, Homo sapiens
MCGSRGRKRLPASPNRPDA

SEQ ID NO: 1306 - protein, 42 aa, Homo sapiens
MCHHAQLIFVLLLVSHVSQAGLELLTSGDCLPWPPKVLGLQV

SEQ ID NO: 1307 - protein, 11 aa, Homo sapiens
MCHHAQLILYF

SEQ ID NO: 1308 - protein, 59 aa, Homo sapiens
MCHHAQLIVVFLVETGFHHGGQATLKLLTSSDPPASAFECWDYRCEPLHLAPISLFCLS

SEQ ID NO: 1309 - protein, 14 aa, Homo sapiens
MCHHARLIYILYIY

SEQ ID NO: 1310 - protein, 45 aa, Homo sapiens
MCHHTQLIFVFLEETRFAMLDRLVSNSQSQVIRLPRPPKVQGLEV

SEQ ID NO: 1311 - protein, 66 aa, Homo sapiens [sequence omitted]

SEQ ID NO: 1312 - protein, 92 aa, Homo sapiens
MCKTLNLSSSCSFSQESTRAYALSLTKFQMSGLQIPVPSRCSATVLRLHGGLPHTALVRHPTGANAYPEALSGSTSLRLVRVPCRDVPQGRL

SEQ ID NO: 1313 - protein, 43 aa, Homo sapiens
MCLIFPLKATLTSLSGSSIKFNKVPRTAFTSVSSSLKSRCLQR

SEQ ID NO: 1314 - protein, 22 aa, Homo sapiens
MCLMKIMIFHSQMAEDVFDRYV

SEQ ID NO: 1315 - protein, 142 aa, Homo sapiens
MCLMWERMRRSWASRWCCCCRVRPALAIRWIKVSVILSRTRWIWSFSSRDFRVLDRNVYTPELSKIIDLRHTNSSPCRFIMRNRDDVASSMSKISTMPSTHFPWFLSKSKLGANSSFPGCSMERQTRPIIRISSQAHSRRWT

SEQ ID NO: 1316 - protein, 34 aa, Homo sapiens
MCLPWALIKRSLYACELESCQFCYCHNQRQVNLC

SEQ ID NO: 1317 - protein, 68 aa, Homo sapiens
MCLRLILLKHNKWSLSLLPCQRNKLWWVACCEFDKEGSGTAIVYCYLYQAVHPPPPTHHFLSAPVPAH

SEQ ID NO: 1318 - protein, 50 aa, Homo sapiens
MCLVRRKLKKSALKRHLSPFQMPPICRLHFISSSSLKPFTPWLFLANTHI

SEQ ID NO: 1319 - protein, 18 aa, Homo sapiens
MCPTPWMDRRTFLPPGSS

SEQ ID NO: 1320 - protein, 31 aa, Homo sapiens
MCSGPPCPRGVGMGVVEAQSGVGLACRTPVQ

SEQ ID NO: 1321 - protein, 20 aa, Homo sapiens
MCSQSVRAAALSSRGLTAHC

SEQ ID NO: 1322 - protein, 13 aa, Homo sapiens
MCTEHRLLVEWEW

SEQ ID NO: 1323 - protein, 25 aa, Homo sapiens
MCVCLLQRHHMAFLMDGKQERERGS

SEQ ID NO: 1324 - protein, 57 aa, Homo sapiens
MCVPTAFLHIYKRLNICSGREKKGILTSPFFTPDSCLETSLALPVLQVYLKSPTHLF

SEQ ID NO: 1325 - protein, 16 aa, Homo sapiens
MDAPRSWNTFSSSAER

SEQ ID NO: 1326 - protein, 11 aa, Homo sapiens
MDESDGVVSSV

SEQ ID NO: 1327 - protein, 32 aa, Homo sapiens
MDFISPPKAEAQSFTTESGICCSERTTSPSAA

SEQ ID NO: 1328 - protein, 11 aa, Homo sapiens
MDFLNRMGYQC

SEQ ID NO: 1329 - protein, 11 aa, Homo sapiens
MDGKQERERGS

SEQ ID NO: 1330 - protein, 15 aa, Homo sapiens
MDGQSSSSGAIRKGS

SEQ ID NO: 1331 - protein, 23 aa, Homo sapiens
MDHNFVWWIYLSKFTIQGLLVLG

SEQ ID NO: 1332 - protein, 26 aa, Homo sapiens
MDIFLSEVDTPSRNGIPVASLLPLIL

SEQ ID NO: 1333 - protein, 29 aa, Homo sapiens
MDKSMLTGFKISMSFCGKLACKIVLDSFN

SEQ ID NO: 1334 - protein, 16 aa, Homo sapiens
MDLITSHSSPDWILPT

SEQ ID NO: 1335 - protein, 107 aa, Homo sapiens
MDLNPPVPATHPHADLHPTPRPFPTSPGGRSPAVSAEAWTRAREAGGTSHLLSTSFSRGKEVPAHPAHSSSAKPRLVQGQPPLCWFQFLLYPFINVEQKRSFPSRYL

SEQ ID NO: 1336 - protein, 11 aa, Homo sapiens
MDLSPFPCCLC

SEQ ID NO: 1337 - protein, 53 aa, Homo sapiens
MDMFWKPVPFSQLSKTGIVQGPYTELLTERESSTRRAGAPQPSTPSLNTYLRM

SEQ ID NO: 1338 - protein, 55 aa, Homo sapiens
MDMTDWAKLLLAGPSGEEIVDDRGVPVQDDWSIAPDDDKVRFSLSGVTPHSSPRC

SEQ ID NO: 1339 - protein, 28 aa, Homo sapiens
MDPGRAERAEVVGLGQGGPVGTLSHPRV

SEQ ID NO: 1340 - protein, 34 aa, Homo sapiens
MDPGRAGGGSGSAGVAGGLGPGGMQRRRRWQWHS

SEQ ID NO: 1341 - protein, 12 aa, Homo sapiens
MDPGRASRGWSG

SEQ ID NO: 1342 - protein, 11 aa, Homo sapiens
MDPGSSLVVRP

SEQ ID NO: 1343 - protein, 87 aa, Homo sapiens
MDRAEPKKDIATANSKKHRAGRSDGPSTNIGMPGLGKGSDGDSTGLDVGLGAVNQSPVRSWRLAAGSAEVQGHLIQKGPFIGPLWLK

SEQ ID NO: 1344 - protein, 71 aa, Homo sapiens
MDRAEPKKDIATANSKKHRAGRSDGPSTNIGMPGLGKGSDGDSTGLGTAPETEGCLLSAPASVQSTGKAHQ

SEQ ID NO: 1345 - protein, 60 aa, Homo sapiens
MDRAEPKKDIATANSKKHRAGRSDGPSTNIGMPGLGTAPETEGCLLSAPASVQSTGKAHQ

SEQ ID NO: 1346 - protein, 16 aa, Homo sapiens
MDRAGCGVGSGESEPS

SEQ ID NO: 1347 - protein, 11 aa, Homo sapiens
MDRPKILHKIS

SEQ ID NO: 1348 - protein, 12 aa, Homo sapiens
MDRRTFLPPGSS

SEQ ID NO: 1349 - protein, 25 aa, Homo sapiens
MDSHLPLELLGRDPNRKMKSGANRL

SEQ ID NO: 1350 - protein, 14 aa, Homo sapiens
MDSKEEGILSALCS

SEQ ID NO: 1351 - protein, 13 aa, Homo sapiens
MDSKWRSPMKMIN

SEQ ID NO: 1352 - protein, 83 aa, Homo sapiens
MDVCCLPSGILPVFHIFISEFSKYCYDIYQKTCSIEGLDHVFVKSSSTIFIVCIQKHFQSIILQMGTAHYFLSNSFIITQLLL

SEQ ID NO: 1353 - protein, 30 aa, Homo sapiens
MEACKNVCSFFPRKRMELGICRIGYMSSLF

SEQ ID NO: 1354 - protein, 21 aa, Homo sapiens
MEADFLIPKMFSFPHMRGKQK

SEQ ID NO: 1355 - protein, 60 aa, Homo sapiens
MEALLCFLSQSQHRRQIAVFRTCLLLQQQAGWPGCRPPCPGGRLWASPYTAAPAPDPSPP

SEQ ID NO: 1356 - protein, 26 aa, Homo sapiens
MEAVWNEAKPHELMDSKWRSPMKMIN

SEQ ID NO: 1357 - protein, 15 aa, Homo sapiens
MECVSAFSKGIIWLS

SEQ ID NO: 1358 - protein, 40 aa, Homo sapiens
MEDCCSFQLSSPISCLPNHPVPTPNFVSVYVTTIHPSMTN

SEQ ID NO: 1359 - protein, 17 aa, Homo sapiens
MEDVGLLRKQVKHGHSE

SEQ ID NO: 1360 - protein, 31 aa, Homo sapiens
MEEKNYSHTKLDSLSMTIFVTLRNVALTFFL

SEQ ID NO: 1361 - protein, 68 aa, Homo sapiens
MEETVSVLIWEDAMDMTDWAKLLLAGPSGEEIVDDRGVPVQDDWSIAPDDDKVRFSLSGVTPHSSPRC

SEQ ID NO: 1362 - protein, 98 aa, Homo sapiens
MEFAAASHFFQRSCEFFWFSWYVHAVLLGGKFHCVSLHMLFCLSSFSGGSSRFLHSIPHTVPHTAPHMGHQLGAGLLSRGHQLWGVCPLQTPDPMTGE

SEQ ID NO: 1363 - protein, 17 aa, Homo sapiens
MEFFICNKFFFSFHNWV

SEQ ID NO: 1364 - protein, 16 aa, Homo sapiens
MEFHRVSQDGLDLLTS

SEQ ID NO: 1365 - protein, 62 aa, Homo sapiens
MEFITTRPALQEMLNTSEGKKMIITIMKTYKSIKCTSVIDTQRRKIKKTYLHRKSQNHSDKH

SEQ ID NO: 1366 - protein, 76 aa, Homo sapiens
MEFLPFGQAVLQLLTSGDPPVSASQSAGITGVSHCARPVCDFLKYKIKFILSVPFIVFYYIYNVLQPLPLPNSRTF

SEQ ID NO: 1367 - protein, 42 aa, Homo sapiens
MEGAKSLIMCLPWALIKRSLYACELESCQFCYCHNQRQVNLC

SEQ ID NO: 1368 - protein, 113 aa, Homo sapiens
MEGGLPRFLLGSLKFSCGLFTMSFSGFLSTWASPEYSLSFSEMFSLSSFSFLGRLFSDTFPFSEQINFPSLSGCLGRFSVFKGLSSLSFFTFTVAFLCSLNFSRLSGDDERLL

SEQ ID NO: 1369 - protein, 39 aa, Homo sapiens
MEHILPLWSVTRSGNSASDHSRGAHCSIFLCFSMPGKPP

SEQ ID NO: 1370 - protein, 11 aa, Homo sapiens
MEHQLGDRQHI

SEQ ID NO: 1371 - protein, 29 aa, Homo sapiens
MEIGKDFETHVPDNIIDISIPIVAYRCVI

SEQ ID NO: 1372 - protein, 21 aa, Homo sapiens
MEIKPASFSNVYYNSKIIFYS

SEQ ID NO: 1373 - protein, 184 aa, Homo sapiens
MEIPNENDKLNDMEPSKAVPLNASKQDGPTPQPHSASLHDTETRKLTEECKRLQGEMMKLSEANQHLRDEGLRLRKVAYSDKPGSTSTASFRDVTSLLPSLLVVIAAIFTGFLFFFWRRSLTLVAQAGVQRRDLGSLQPPSPGFKQFSHLSLPSSWDYRRPPPHPANFCIFSREGVSPCWPGWS

SEQ ID NO: 1374 - protein, 13 aa, Homo sapiens
MEKSHMRWILALH

SEQ ID NO: 1375 - protein, 35 aa, Homo sapiens
MELDMCSGPPCPRGVGMGVVEAQSGVGLACRTPVQ

SEQ ID NO: 1376 - protein, 15 aa, Homo sapiens
MELGICRIGYMSSLF

SEQ ID NO: 1377 - protein, 19 aa, Homo sapiens
MELGVEPRYWSPDMQNTCV

SEQ ID NO: 1378 - protein, 14 aa, Homo sapiens
MELLFRSGYPNALQ

SEQ ID NO: 1379 - protein, 19 aa, Homo sapiens
MELMLISSSLCSLVSVQRS

SEQ ID NO: 1380 - protein, 33 aa, Homo sapiens
MELPLLLVSSHPMLEVGKAGLPHLPPHQYSTFF

SEQ ID NO: 1381 - protein, 57 aa, Homo sapiens
MELTQLGRGVVSIFHGNSGIHDALFRAGLSVPQVSELKSWTSQAQYPLLGPFCHILV

SEQ ID NO: 1382 - protein, 19 aa, Homo sapiens
MENHKLSVPCSRSFHEDFA

SEQ ID NO: 1383 - protein, 22 aa, Homo sapiens
MENSINKFNRLTLESIKKLKDG

SEQ ID NO: 1384 - protein, 30 aa, Homo sapiens
MENSLNSLYNFFFVSNSSSALHTVSSRNCP

SEQ ID NO: 1385 - protein, 12 aa, Homo sapiens
MEPMFPWFQWQG

SEQ ID NO: 1386 - protein, 172 aa, Homo sapiens
MEPSKAVPLNASKQDGPTPQPHSASLHDTETRKLTEECKRLQGEMMKLSEANQHLRDEGLRLRKVAYSDKPGSTSTASFRDVTSLLPSLLVVIAAIFTGFLFFFWRRSLTLVAQAGVQRRDLGSLQPPSPGFKQFSHLSLPSSWDYRRPPPHPANFCIFSREGVSPCWPGWS

SEQ ID NO: 1387 - protein, 14 aa, Homo sapiens
MEPSNTCWWKCKML

SEQ ID NO: 1388 - protein, 19 aa, Homo sapiens
MEPSWKTLCRILSRRTSPI

SEQ ID NO: 1389 - protein, 15 aa, Homo sapiens
MEQTKPAAWEIRNHS

SEQ ID NO: 1390 - protein, 18 aa, Homo sapiens
MEQWQDHTEQGRGKCSYS

SEQ ID NO: 1391 - protein, 73 aa, Homo sapiens
MERTDPAPRGGRERGACAGRRRDPGGCNMAARAPSPPCQARALGSCCRFPLGLGRGKEGTALRLRNLYCDFGR

SEQ ID NO: 1392 - protein, 68 aa, Homo sapiens
MESAVAAFLSGSAGLGVNGTLPSRCPPGAGPLTPKTLPKTRPPGQGQKTDPGRPAPAGWWRRWRAGRC

SEQ ID NO: 1393 - protein, 23 aa, Homo sapiens
MESFLMSLNVVKAIYKAETVGSW

SEQ ID NO: 1394 - protein, 75 aa, Homo sapiens
MESGSVAQAGVQWRHLSSLQALPPGFTPLPFSRLSLPSSWGYRRPPPRPANFLYFFSRDRVSPCWPGWSRTPDLK

SEQ ID NO: 1395 - protein, 11 aa, Homo sapiens
MESIFIALSEK

SEQ ID NO: 1396 - protein, 28 aa, Homo sapiens
MESPNLHKRPGERPSPLSSAPPPAPSVR

SEQ ID NO: 1397 - protein, 17 aa, Homo sapiens
METASFLDKHHPGTHKQ

SEQ ID NO: 1398 - protein, 34 aa, Homo sapiens
METNCNSLSFMYLDVHQSGKSPRYGKFSAIISLN

SEQ ID NO: 1399 - protein, 24 aa, Homo sapiens
METRKELPHPHSKRLPELPQASKR

SEQ ID NO: 1400 - protein, 122 aa, Homo sapiens
MEVGSPGAERSPRNQVFLGTGEKGCMSRMEGGWAGPRPPRPPLNRFHGGHSRFRTLPMCSGFSNAREVSCRERVLVGHGGLAGAPLGGWLCACAELHPAHRLSFCKLSRGPTCVFAPLQLTF

SEQ ID NO: 1401 - protein, 22 aa, Homo sapiens
MEVQINCNWMSNSFTMLWSSPS

SEQ ID NO: 1402 - protein, 35 aa, Homo sapiens
MEVVIARALMVSCWLCHAVGTAILKVNRHSGSYFH

SEQ ID NO: 1403 - protein, 38 aa, Homo sapiens
MEYVQFFCREVAAVCHHCLICQKIVFIIHRCVVFITGV

SEQ ID NO: 1404 - protein, 40 aa, Homo sapiens
MFAPRSFPCPSLQAVFPSLLCHLASCWVQLVARLKYRRKG

SEQ ID NO: 1405 - protein, 24 aa, Homo sapiens
MFCIFNRDGVSSFWPDWSQTPDLR

SEQ ID NO: 1406 - protein, 23 aa, Homo sapiens
MFCIMWGILFHSETRDCNYKTSN

SEQ ID NO: 1407 - protein, 37 aa, Homo sapiens
MFCLFMFLVCLHWYLHIWCNSSFFQFFDLSFLRESCS

SEQ ID NO: 1408 - protein, 21 aa, Homo sapiens
MFCLSPEVQIKGCSEVRPSVH

SEQ ID NO: 1409 - protein, 22 aa, Homo sapiens
MFDHTTYLKCCWLKVFLLYSFL

SEQ ID NO: 1410 - protein, 62 aa, Homo sapiens
MFDSLNYSIIKFHSVSTILVNSSDFGRVKTTIRPASKDLLIYLKFRRSILFMQALFPQLYFL

SEQ ID NO: 1411 - protein, 21 aa, Homo sapiens
MFFHFSCSLNMNLLPTQKDLR

SEQ ID NO: 1412 - protein, 16 aa, Homo sapiens
MFFLLLHNFELEVAAK

SEQ ID NO: 1413 - protein, 90 aa, Homo sapiens
MFFSLIQSIPNKLLSKALLSCISMSNILSPETPFCMCACWVIPGAGYAIPGTVRVSSQAAVSTSTSIHVTVMESDLSHSRSRSNIQLLPL

SEQ ID NO: 1414 - protein, 21 aa, Homo sapiens
MFFSRDRVSRVSQDGLDLLTS

SEQ ID NO: 1415 - protein, 17 aa, Homo sapiens
MFGLIPLKVEEHTVIIT

SEQ ID NO: 1416 - protein, 23 aa, Homo sapiens
MFHFQCFRNNHFEESSHCPCFWK

SEQ ID NO: 1417 - protein, 12 aa, Homo sapiens
MFHPPSPPKVLG

SEQ ID NO: 1418 - protein, 31 aa, Homo sapiens
MFHRSCHIFPRQDIPVNTFFVIHIPTVYFFI

SEQ ID NO: 1419 - protein, 16 aa, Homo sapiens
MFHSNLAPEYLYFSQW

SEQ ID NO: 1420 - protein, 19 aa, Homo sapiens
MFIFFKILLINKHMKTSKF

SEQ ID NO: 1421 - protein, 21 aa, Homo sapiens
MFIFKIYKYICTYIWQVYCSY

SEQ ID NO: 1422 - protein, 14 aa, Homo sapiens
MFILMMCLCLGLMS

SEQ ID NO: 1423 - protein, 12 aa, Homo sapiens
MFKRYVSIHLFS

SEQ ID NO: 1424 - protein, 14 aa, Homo sapiens
MFLHMVVQYTTHLY

SEQ ID NO: 1425 - protein, 11 aa, Homo sapiens
MFLKCFLSVRH

SEQ ID NO: 1426 - protein, 13 aa, Homo sapiens
MFLKSSAESLTKQ

SEQ ID NO: 1427 - protein, 11 aa, Homo sapiens
MFLTVCNSFLY

SEQ ID NO: 1428 - protein, 32 aa, Homo sapiens
MFLVCLHWYLHIWCNSSFFQFFDLSFLRESCS

SEQ ID NO: 1429 - protein, 14 aa, Homo sapiens
MFNIMAKMRILLYS

SEQ ID NO: 1430 - protein, 19 aa, Homo sapiens
MFNIYYLSLLFSIHKTLPD

SEQ ID NO: 1431 - protein, 15 aa, Homo sapiens
MFPITVPAPCSSGTE

SEQ ID NO: 1432 - protein, 22 aa, Homo sapiens
MFRMMSLWVESFKCPIRKGIHF

SEQ ID NO: 1433 - protein, 27 aa, Homo sapiens
MFSCIFQILSNEQVLLYNWRRVKLIFK

SEQ ID NO: 1434 - protein, 12 aa, Homo sapiens
MFSFPHMRGKQK

SEQ ID NO: 1435 - protein, 19 aa, Homo sapiens
MFSLNKCVYPLHSYTFIKG

SEQ ID NO: 1436 - protein, 51 aa, Homo sapiens
MFSPSRQFTRAHTRAGTGMNLYPRDRFTPPQERDRGEGTMKEPGTEAGILF

SEQ ID NO: 1437 - protein, 77 aa, Homo sapiens
MFSRVSTGAAQRVCVNLLNSGFRSSCRFWSRVSKPWLLSSPRGPSRRLRVSWGTCQFCSMDIRKDRQLLMLAITLAL

SEQ ID NO: 1438 - protein, 15 aa, Homo sapiens
MFSRVTMLARLVLNS

SEQ ID NO: 1439 - protein, 25 aa, Homo sapiens
MFSTSLKSLRSCLFLLLVPSISSSA

SEQ ID NO: 1440 - protein, 12 aa, Homo sapiens
MFVEKNCNGTIF

SEQ ID NO: 1441 - protein, 12 aa, Homo sapiens
MFVFFLGFLFLY

SEQ ID NO: 1442 - protein, 23 aa, Homo sapiens
MFVSLLRDFWCCGSTTKPGCLWL

SEQ ID NO: 1443 - protein, 12 aa, Homo sapiens
MFVVSFLEREWN

SEQ ID NO: 1444 - protein, 13 aa, Homo sapiens
MFWITGSKIHLRY

SEQ ID NO: 1445 - protein, 51 aa, Homo sapiens
MFWKPVPFSQLSKTGIVQGPYTELLTERESSTRRAGAPQPSTPSLNTYLRM

SEQ ID NO: 1446 - protein, 18 aa, Homo sapiens
MFYFCLNTDHLFSYTQCM

SEQ ID NO: 1447 - protein, 77 aa, Homo sapiens
MFYFKLDFSSGLISSLNPASHFLNRCSDAMKHPAELLLLILCLRHHLVFVEAVSQLLLFLLSLFHIGILFLSNDSVH

SEQ ID NO: 1448 - protein, 35 aa, Homo sapiens
MFYFKLLCVAFHLLSTSYSSCKLILYFLKLTSHLV

SEQ ID NO: 1449 - protein, 53 aa, Homo sapiens
MFYHLAKKGKLPSDSNLHGPSVSSLNMWYEDRKCWSCLIQTWVQISFPPCLAM

SEQ ID NO: 1450 - protein, 18 aa, Homo sapiens
MGAAMTDGGIRPAGLRGA

SEQ ID NO: 1451 - protein, 20 aa, Homo sapiens
MGAAMTDGGIRPAGLRGACE

SEQ ID NO: 1452 - protein, 25 aa, Homo sapiens
MGACLPPGPSLVLLCRLYFPHFSAT

SEQ ID NO: 1453 - protein, 13 aa, Homo sapiens
MGAGVGWGGVGVL

SEQ ID NO: 1454 - protein, 11 aa, Homo sapiens
MGALPRLVSNS

SEQ ID NO: 1455 - protein, 44 aa, Homo sapiens
MGALTQGHTLKVENPGQLFGECGTLNPSFRYSSLSPGLFLSRTR

SEQ ID NO: 1456 - protein, 105 aa, Homo sapiens
MGATASGSLLVVQHSLEEVLLHPTDLGISFSSSSCPSTQSSQHPCHWPRHRVARPARPCPCAVPETFLPPAGTRGSLKCTHSFQRSCYRSHCSPAQTGSRTARHP

SEQ ID NO: 1457 - protein, 17 aa, Homo sapiens
MGEASPLFGRGWPWSKA

SEQ ID NO: 1458 - protein, 43 aa, Homo sapiens
MGEDQDPRGWAEGVERRQRESCRDPHQVTVSTSLASMCLPGLL

SEQ ID NO: 1459 - protein, 49 aa, Homo sapiens
MGELLLLAAEHVNRMSLPTIAMVVSGWVMICGFRKSSHTKLSGGTEKML

SEQ ID NO: 1460 - protein, 19 aa, Homo sapiens
MGELTRYSTDTQERALGMW

SEQ ID NO: 1461 - protein, 17 aa, Homo sapiens
MGEVGNYSNLITSSSST

SEQ ID NO: 1462 - protein, 48 aa, Homo sapiens [sequence omitted]

SEQ ID NO: 1463 - protein, 16 aa, Homo sapiens
MGFHCVRQDGLDLLTS

SEQ ID NO: 1464 - protein, 16 aa, Homo sapiens
MGFHCVSHDGLNLLTS

SEQ ID NO: 1465 - protein, 16 aa, Homo sapiens
MGFHHAGQAGLEFLTL

SEQ ID NO: 1466 - protein, 16 aa, Homo sapiens
MGFHHAGQAGLELLIS

SEQ ID NO: 1467 - protein, 36 aa, Homo sapiens
MGFHHFGQTGLKLLTSGDPPASASQSAGITGVSHCI

SEQ ID NO: 1468 - protein, 47 aa, Homo sapiens
MGFHHLDQAGLELLASSDPPASASQRAGITSGVSHPTQLRISYAGKL

SEQ ID NO: 1469 - protein, 16 aa, Homo sapiens
MGFHHLGQAGLELLTS

SEQ ID NO: 1470 - protein, 36 aa, Homo sapiens
MGFHHLGQAGLQLLTSSDLPMLASQSGGSHSNITVF

SEQ ID NO: 1471 - protein, 16 aa, Homo sapiens
MGFHHRGQAGLELLTS

SEQ ID NO: 1472 - protein, 16 aa, Homo sapiens
MGFHHVGQAALKLLTS

SEQ ID NO: 1473 - protein, 144 aa, Homo sapiens
MGFHHVGQAGFKLLTSNDPPASASQSAGITGVSHRAWPECLFFINYPVLGVLSQRPILPEPRLSALNAVLKSPALAPEAAPKAGTAVHELRHLGHVITSLSPEAPRQKWNQQCPFHSSCPGEENGKSCPLSAIPGKKSHTELRP

SEQ ID NO: 1474 - protein, 67 aa, Homo sapiens
MGFHHVGQAGLELLSSGNLPTSASQSAGITGMSHCAWPCFSNFDGYLFKTSRVSLKFGKKKKVVLKN

SEQ ID NO: 1475 - protein, 46 aa, Homo sapiens
MGFHHVGQAGLELLTSSDPPTSASQGAGITGVSYCDRPVVYFLEQF

SEQ ID NO: 1476 - protein, 38 aa, Homo sapiens
MGFHHVGQAGLKLLTSGDLPTSASQSAGITGVSHHARP

SEQ ID NO: 1477 - protein, 80 aa, Homo sapiens [sequence omitted]

SEQ ID NO: 1478 - protein, 70 aa, Homo sapiens
MGFHHVGQAGLKLLTSGDPPTSTSQSAGITGVSHRAQPVFSFLLSLGKRVGRTDPGVAGMGDCCREVTGP

SEQ ID NO: 1479 - protein, 61 aa, Homo sapiens [sequence omitted]

SEQ ID NO: 1480 - protein, 57 aa, Homo sapiens [sequence omitted]

SEQ ID NO: 1481 - protein, 35 aa, Homo sapiens
MGFHHVGQASLNLLTSSDPPALNSQSSGITQKHNF

SEQ ID NO: 1482 - protein, 16 aa, Homo sapiens
MGFHHVGQDGLDFLTS

SEQ ID NO: 1483 - protein, 29 aa, Homo sapiens
MGFHHVGQVGLELLILVIRPPQPPKVLRL

SEQ ID NO: 1484 - protein, 14 aa, Homo sapiens
MGFHHVLVRMVLIS

SEQ ID NO: 1485 - protein, 16 aa, Homo sapiens
MGFHHVSQDVLDLLTS

SEQ ID NO: 1486 - protein, 45 aa, Homo sapiens
MGFHIGQVGLELLTSGDLPTLASQSAGITGMSHRAWPVSIFIMQK

SEQ ID NO: 1487 - protein, 16 aa, Homo sapiens
MGFHPSGWSRTFDDLR

SEQ ID NO: 1488 - protein, 29 aa, Homo sapiens
MGFHRAGWSRSPDLVSCLPQPPKVLGLQA

SEQ ID NO: 1489 - protein, 16 aa, Homo sapiens
MGFHRIGQAGLELLTL

SEQ ID NO: 1490 - protein, 47 aa, Homo sapiens
MGFHRVGQAGLELLTLGDPPASASQSAGITGVSHRAWPQNRFFGIPC

SEQ ID NO: 1491 - protein, 16 aa, Homo sapiens
MGFHRVSQDGLDLLTS

SEQ ID NO: 1492 - protein, 15 aa, Homo sapiens
MGFHYVGQAGLELPT

SEQ ID NO: 1493 - protein, 31 aa, Homo sapiens
MGFIMLARLVLNSSPQVICPPQPPKVLGLQV

SEQ ID NO: 1494 - protein, 38 aa, Homo sapiens
MGFKHMKCSFCCHNFGRIQLLLNAQLKIFFLFKWDCEN

SEQ ID NO: 1495 - protein, 22 aa, Homo sapiens
MGFKVPTPPADQARGPQGPALQ

SEQ ID NO: 1496 - protein, 68 aa, Homo sapiens
MGFLHVGQAGLKLPTSGDLPALASQSVGITGVSHHTRPRFLFKIGPLFLFSKSMSQDEPGFKYTNINF

SEQ ID NO: 1497 - protein, 13 aa, Homo sapiens
MGFRHGPRLVSNS

SEQ ID NO: 1498 - protein, 15 aa, Homo sapiens
MGFRSVGQAGLKLLA

SEQ ID NO: 1499 - protein, 11 aa, Homo sapiens
MGFYHVGQVGL

SEQ ID NO: 1500 - protein, 70 aa, Homo sapiens
MGGLSVEESFFHPAKMLIAERQDARFQLNTPFVSLSLKEHLSIIHQSLPTFPSHPRQAITPNPDLVQNQT

SEQ ID NO: 1501 - protein, 22 aa, Homo sapiens
MGGSRGQEIETILANMVKPRLY

SEQ ID NO: 1502 - protein, 28 aa, Homo sapiens
MGHPLPQLCHPGKIGPTSPRASSEAAGA

SEQ ID NO: 1503 - protein, 11 aa, Homo sapiens
MGHPPTSGCLD

SEQ ID NO: 1504 - protein, 37 aa, Homo sapiens
MGHPPTSGCLDSEQLQKLRAVCSAPQHLCRAPEKLTN

SEQ ID NO: 1505 - protein, 114 aa, Homo sapiens [sequence omitted]

SEQ ID NO: 1506 - protein, 18 aa, Homo sapiens
MGHSHLCLINTSAFALVQ

SEQ ID NO: 1507 - protein, 21 aa, Homo sapiens
MGHVPGRTTWARLEEGVGIQK

SEQ ID NO: 1508 - protein, 31 aa, Homo sapiens
MGITPPHRRSASFMVGTTTVSDRLRTSDFRS

SEQ ID NO: 1509 - protein, 42 aa, Homo sapiens
MGKCFFFSFTPGNGEVLFFFFFFLLWTTVWEGRGGPQQGDLR

SEQ ID NO: 1510 - protein, 63 aa, Homo sapiens [sequence omitted]

SEQ ID NO: 1511 - protein, 18 aa, Homo sapiens
MGLCNINPAKTVYNSVWV

SEQ ID NO: 1512 - protein, 30 aa, Homo sapiens
MGLFLVCELMKTSIFLTHFPCHSLPCGFFI

SEQ ID NO: 1513 - protein, 31 aa, Homo sapiens
MGLGRAHTPGLVADLTQVAELPELKSGRAAA

SEQ ID NO: 1514 - protein, 21 aa, Homo sapiens
MGLGSFAAGAFPRGSMVLPDP

SEQ ID NO: 1515 - protein, 24 aa, Homo sapiens
MGLLSRIARSTQDVFSFKDNSKDC

SEQ ID NO: 1516 - protein, 45 aa, Homo sapiens
MGMGEDQDPRGWAEGVERRQRESCRDPHQVTVSTSLASMCLPGLL

SEQ ID NO: 1517 - protein, 25 aa, Homo sapiens
MGNVYALGLFRIFIILKSILVDICS

SEQ ID NO: 1518 - protein, 19 aa, Homo sapiens
MGPAHPAVRVGGQADGVLG

SEQ ID NO: 1519 - protein, 17 aa, Homo sapiens
MGPGAHRHSRQTRREGI

SEQ ID NO: 1520 - protein, 90 aa, Homo sapiens
MGPSLRINRLGGITWGPRAGSEAGKLSGGGGLRPERAHTDWRGRIQGCGWTAFPHLPRRALPLVQSPHPAPARLQRALALTGGRNFPAST

SEQ ID NO: 1521 - protein, 50 aa, Homo sapiens
MGPSSRASTVVEVPHGWQSRNGPAEQSRGPRPHPHLLPCGSVRPGARAPL

SEQ ID NO: 1522 - protein, 14 aa, Homo sapiens
MGPVLHTRQLGPGL

SEQ ID NO: 1523 - protein, 14 aa, Homo sapiens
MGQGGEVIIAAGNL

SEQ ID NO: 1524 - protein, 88 aa, Homo sapiens
MGQHGEQAAIADTQAHAVWLQHGPQSLDVSISSVLVIDLSKPRPVPEQVSLAVTHGAHLADSLILFRAGPLQAVPYAVVIVVGYQIER

SEQ ID NO: 1525 - protein, 23 aa, Homo sapiens
MGQRQLKSVNTLQIQRFSHSPVG

SEQ ID NO: 1526 - protein, 29 aa, Homo sapiens
MGQSPHAAEDRSVSAPVVTVESSKQFTTN

SEQ ID NO: 1527 - protein, 16 aa, Homo sapiens
MGQTDCRHTNFRFTFH

SEQ ID NO: 1528 - protein, 40 aa, Homo sapiens
MGRGHRAGGSGCNNVLSLSSLVPGNIAWDMLSQQLKSNAT

SEQ ID NO: 1529 - protein, 44 aa, Homo sapiens
MGRQRAGGEQGISLGTVPVSFQVLLHLLLLLFLLFIISQDPWLE

SEQ ID NO: 1530 - protein, 19 aa, Homo sapiens
MGRRGWSSAPWGHLLKATH

SEQ ID NO: 1531 - protein, 56 aa, Homo sapiens
MGRTSSFSVYYFVVLGLVYYLYKKPLLKLICTQIWKTQKIWKTQNHSLPPPRDNHC

SEQ ID NO: 1532 - protein, 13 aa, Homo sapiens
MGSALSQLLALGS

SEQ ID NO: 1533 - protein, 29 aa, Homo sapiens
MGSFVYLILKPVHCINLSFVSYLPLFPST

SEQ ID NO: 1534 - protein, 15 aa, Homo sapiens
MGSQKRTEHRVCICM

SEQ ID NO: 1535 - protein, 53 aa, Homo sapiens
MGSSASGPLSLSISKGLIQVGSSKGLPGTRGLESLCWGCSSSSLKGLGAGLSG

SEQ ID NO: 1536 - protein, 209 aa, Homo sapiens
MGSWLFPRVSGRQRVASGLSDSSLGNVCTFRRRLLLRASLSSSPRVRSASRTRPASPSRLWLSPFLTGVDSRALVGEALGPRLVSDSGPSGVGRTSGSVLGSPGGLLGPAFPGAGLSRQLLSLTSCSAPKDSMERTLLPTAERLRHTRQEDVSCSFSSHSAMMLSRSGRSPGSSACIRLSSASRSWLSLGSSVGSATYSRAAFSVAPRE

SEQ ID NO: 1537 - protein, 23 aa, Homo sapiens
MHFPICPAELPHAVCGILLPIMP

SEQ ID NO: 1538 - protein, 23 aa, Homo sapiens
MHHHAQLIFIFLVEKGVSSCWPG

SEQ ID NO: 1539 - protein, 11 aa, Homo sapiens
MHHHPQLVLFF

SEQ ID NO: 1540 - protein, 49 aa, Homo sapiens
MHHHRLIFVFLVEMGFHHLGQAGLQLLTSSDLPMLASQSGGSHSNITVF

SEQ ID NO: 1541 - protein, 60 aa, Homo sapiens [sequence omitted]

SEQ ID NO: 1542 - protein, 39 aa, Homo sapiens
MHHRLEFINSLLGISLSDFPIGYCIVSGISISGDITLLP

SEQ ID NO: 1543 - protein, 11 aa, Homo sapiens
MHIIVGNTKRV

SEQ ID NO: 1544 - protein, 11 aa, Homo sapiens
MHLFKKLVNFM

SEQ ID NO: 1545 - protein, 87 aa, Homo sapiens
MHLGRKHRGLRKAKNKNKKAPPQPLPLSRRSRSCQPMQQSWSGAQVHIPQPPHTTCITWAGSPNTSVSSSATWVRWECPPPGELRTR

SEQ ID NO: 1546 - protein, 99 aa, Homo sapiens
MHLPNNVLPVPRGPNKRMLRGKAVSPLNASDLNTGHKTSSLMTAFTRSRPAMSFQSTGGPWVIISLVTRSMRCVSVFFSCSSTEWLDEVAARSPGPCIG

SEQ ID NO: 1547 - protein, 26 aa, Homo sapiens
MHLSVFICNVGKMGMPTSWGTQDSLS

SEQ ID NO: 1548 - protein, 26 aa, Homo sapiens
MHLVRLPFALLNSIFSLYNLVKFHFF

SEQ ID NO: 1549 - protein, 52 aa, Homo sapiens
MHLWAWGGLQITPALRDGDAEKCYFYSSPSLARLHCQGQHFGDISLVSQFTQ

SEQ ID NO: 1550 - protein, 36 aa, Homo sapiens
MHLYHLGRFSQYLSVFICNVGKMGMPTSWGTQDSLS

SEQ ID NO: 1551 - protein, 15 aa, Homo sapiens
MHPLKQRIMRNSSRL

SEQ ID NO: 1552 - protein, 22 aa, Homo sapiens
MHTFSHSNMNLSVAAESFCGCN

SEQ ID NO: 1553 - protein, 127 aa, Homo sapiens
MHTHVHTHPHTVSHPGSHPHMDLNPPVPATHPHADLHPTPRPFPTSPGGRSPAVSAEAWTRAREAGGTSHLLSTSFSRGKEVPAHPAHSSSAKPRLVQGQPPLCWFQFLLYPFINVEQKRSFPSRYL

SEQ ID NO: 1554 - protein, 11 aa, Homo sapiens
MHTNKRPTKWS

SEQ ID NO: 1555 - protein, 11 aa, Homo sapiens
MHVISLSGNLI

SEQ ID NO: 1556 - protein, 19 aa, Homo sapiens
MHVIVDQEILHYKNKSQLY

SEQ ID NO: 1557 - protein, 22 aa, Homo sapiens
MHVYLAIKPYGRTVITKSLSQT

SEQ ID NO: 1558 - protein, 20 aa, Homo sapiens
MHYHSWLIFCIFSRNGVSPC

SEQ ID NO: 1559 - protein, 39 aa, Homo sapiens
MHYILHLQNVCFFFRISISLLNVSFCVLMISLGCLSVLW

SEQ ID NO: 1560 - protein, 42 aa, Homo sapiens
MIAKKNHLTINYMWLVASWELVFLMADVQESNPGEYNSKLGN

SEQ ID NO: 1561 - protein, 11 aa, Homo sapiens
MIANMLLIPCS

SEQ ID NO: 1562 - protein, 21 aa, Homo sapiens
MICGFRKSSHTKLSGGTEKML

SEQ ID NO: 1563 - protein, 15 aa, Homo sapiens
MICPRQPPKVLELQV

SEQ ID NO: 1564 - protein, 13 aa, Homo sapiens
MIDIKIDYLPPLL

SEQ ID NO: 1565 - protein, 26 aa, Homo sapiens
MIEKDKMLAQYKRETNRKLFRLSGQQ

SEQ ID NO: 1566 - protein, 53 aa, Homo sapiens
MIFFGTRHAPLPSRPPLLFPYVHILIQCKYEDALEALWGTFPNPGSSVCTVDS

SEQ ID NO: 1567 - protein, 16 aa, Homo sapiens
MIFHSQMAEDVFDRYV

SEQ ID NO: 1568 - protein, 72 aa, Homo sapiens
MIGILSASHEERFQRTPVTSSRISRSVVLRSNLTSAGMPPQFFRAILLSSLAFPYTRFLRAPQALRWTSVIR

SEQ ID NO: 1569 - protein, 15 aa, Homo sapiens
MIHLPWAPKVLGLQV

SEQ ID NO: 1570 - protein, 15 aa, Homo sapiens
MIHPPLPPKVQRLQA

SEQ ID NO: 1571 - protein, 15 aa, Homo sapiens
MIHPPPSPKVLGLQA

SEQ ID NO: 1572 - protein, 15 aa, Homo sapiens
MIHPPRPPKVLGLQA

SEQ ID NO: 1573 - protein, 15 aa, Homo sapiens
MIHPPRPPKVLGLQL

SEQ ID NO: 1574 - protein, 26 aa, Homo sapiens
MIHPPRPPKVLGRQAKSPRPATPSLF

SEQ ID NO: 1575 - protein, 11 aa, Homo sapiens
MIHQNLVKQSE

SEQ ID NO: 1576 - protein, 38 aa, Homo sapiens
MIHSAQCDRNEQKACALQNMTLKREVMPFSFVGWKDCL

SEQ ID NO: 1577 - protein, 13 aa, Homo sapiens
MIHSRQPPKVLGL

SEQ ID NO: 1578 - protein, 41 aa, Homo sapiens
MIITIMKTYKSIKCTSVIDTQRRKIKKTYLHRKSQNHSDKH

SEQ ID NO: 1579 - protein, 36 aa, Homo sapiens
MIIVEAVDTRLFTVICCISYSVSSLLSCRHRYRYLV

SEQ ID NO: 1580 - protein, 63 aa, Homo sapiens
MIKQRNLNESEENKPCFHYIHGGMFAPRSFPCPSLQAVFPSLLCHLASCWVQLVARLKYRRKG

SEQ ID NO: 1581 - protein, 28 aa, Homo sapiens
MILFSLLSYRKRKGRKNNKQLETDWYQI

SEQ ID NO: 1582 - protein, 19 aa, Homo sapiens
MILLLWPQCTGLLSICHSD

SEQ ID NO: 1583 - protein, 64 aa, Homo sapiens
MILNRFPGNANFMLTISHLKYSPASHRVPMTSLQICRNLGFSVYHKLATGAWQITLSFYSSSLK

SEQ ID NO: 1584 - protein, 15 aa, Homo sapiens
MILPPQPPKVLGLQA

SEQ ID NO: 1585 - protein, 56 aa, Homo sapiens
MILRGSLASPPGRRERSGQAHLCEALLQAEAEAEPKPMAKPEPENLRALSIAPLSL

SEQ ID NO: 1586 - protein, 130 aa, Homo sapiens
MILRGSLASPPGRRERSGQAHLCEALLQAEAEAEPKPMAKPEPENLRALSIAPLSLPWLPTLPAPLLPARQPLGPHPANLSPGTPAGPTSSRPRAAAAAAAAASGAGPLPARPPGRSESRQPHRLNCFLL

SEQ ID NO: 1587 - protein, 22 aa, Homo sapiens
MILRGSLSPGTPAGPTSSRPRA

SEQ ID NO: 1588 - protein, 21 aa, Homo sapiens
MILRGSLVKSSSASMCLGIGE

SEQ ID NO: 1589 - protein, 11 aa, Homo sapiens
MILRLILTELH

SEQ ID NO: 1590 - protein, 24 aa, Homo sapiens
MIMFDHTTYLKCCWLKVFLLYSFL

SEQ ID NO: 1591 - protein, 66 aa, Homo sapiens
MIPMIKQRNLNESEENKPCFHYIHGGMFAPRSFPCPSLQAVFPSLLCHLASCWVQLVARLKYRRKG

SEQ ID NO: 1592 - protein, 22 aa, Homo sapiens
MIQKRFLAPEAVGIEMVFPAAS

SEQ ID NO: 1593 - protein, 50 aa, Homo sapiens
MIQKRFLAPEAVGIEMVFPAAVLSLPTGVLEQLRSMVDDSEDMAPGLQPV

SEQ ID NO: 1594 - protein, 15 aa, Homo sapiens
MIRLPQPPKVLGLQA

SEQ ID NO: 1595 - protein, 15 aa, Homo sapiens
MIRLPRAPKVLGLQA

SEQ ID NO: 1596 - protein, 15 aa, Homo sapiens
MIRPPRPPKVLGLQA

SEQ ID NO: 1597 - protein, 34 aa, Homo sapiens
MIRQTTEFVHLLLLKFVYLLCAHILLHCFSAVKN

SEQ ID NO: 1598 - protein, 15 aa, Homo sapiens
MIRRAQPLFLKNRKL

SEQ ID NO: 1599 - protein, 40 aa, Homo sapiens
MIRVNRQPTEWEKLFAIYPSDKGLISRIYKELKFTRKKSH

SEQ ID NO: 1600 - protein, 16 aa, Homo sapiens
MISKKIPGHSPDSQVL

SEQ ID NO: 1601 - protein, 25 aa, Homo sapiens
MISNIEPPLSNFMTSQSSSLTTKEV

SEQ ID NO: 1602 - protein, 84 aa, Homo sapiens
MISPSRTEGDPLPLPPGVRVRRSEALEEALRRRRPRDIAGQVFPSSACVGPGRARQDLPGSRCGGRIRAGSESRHRRLRRCRRQ

SEQ ID NO: 1603 - protein, 83 aa, Homo sapiens
MISPSRTEGDPLPLPPGVRVRRSEALEEALRRRRPRDIAGQVFPSSACVGPGRARQDPGPAAGAGFAPAPRAATVASAAAAAS

SEQ ID NO: 1604 - protein, 13 aa, Homo sapiens
MITAFCTPGELTF

SEQ ID NO: 1605 - protein, 16 aa, Homo sapiens
MITPKIKFRTIMITMK

SEQ ID NO: 1606 - protein, 13 aa, Homo sapiens
MITSCWLVFNVHL

SEQ ID NO: 1607 - protein, 44 aa, Homo sapiens
MITTPPRKQRLSSSGSPQNPLSFGTYSTIYYIFVILKFVLFQRW

SEQ ID NO: 1608 - protein, 23 aa, Homo sapiens
MIVTSHKMPRMRCSFKMESTVSL

SEQ ID NO: 1609 - protein, 26 aa, Homo sapiens
MIWEFQERVFCRADDIHRDGYFSLRG

SEQ ID NO: 1610 - protein, 37 aa, Homo sapiens
MIYYKQLPWRSLLKDSSESIGLHLEPPKGWGQGRKET

SEQ ID NO: 1611 - protein, 82 aa, Homo sapiens
MKAFTLSTRSCPIAPVSRAKSRNLSRRRVTWSKSCPISGEEATSSFSEIHCSRSSVSRLSWNRWYMFSSLRLRSSATSFSPA

SEQ ID NO: 1612 - protein, 36 aa, Homo sapiens
MKALAGWRVGRLRNLLSRLRIHSRQQLLPRSARRRR

SEQ ID NO: 1613 - protein, 42 aa, Homo sapiens
MKALAGWRVGRLRNLLSRLRIHSRQQLLPRSARRRRQWRAVM

SEQ ID NO: 1614 - protein, 131 aa, Homo sapiens
MKAQGAPSRERTVQELDALPPRCHLWDKHLISESSLGYLSTRLMTSSTTSPTHRICFSSMRLLPELPARPADGVPPGLCLLSRRMVSPLPAALAPPPRGSSSSREPPAAARGAGNERSRALPRDTRRPERV

SEQ ID NO: 1615 - protein, 33 aa, Homo sapiens
MKCSFCCHNFGRIQLLLNAQLKIFFLFKWDCEN

SEQ ID NO: 1616 - protein, 72 aa, Homo sapiens
MKEEKRRFPISAQLTIRDPSCSALSPHPGLPFLPCSKASRLRSHKAATWPLSPMCGFDLHSLLGHSPRLHLV

SEQ ID NO: 1617 - protein, 14 aa, Homo sapiens
MKEKGFHHPCQYLG

SEQ ID NO: 1618 - protein, 12 aa, Homo sapiens
MKETGTLLMQFS

SEQ ID NO: 1619 - protein, 82 aa, Homo sapiens
MKETKMPSPSSPPTMLKPRPVEPLCRMILRGSLASPPGRRERSGQAHLCEALLQAEAEAEPKPMAKPEPENLRALSIAPLSL

SEQ ID NO: 1620 - protein, 156 aa, Homo sapiens
MKETKMPSPSSPPTMLKPRPVEPLCRMILRGSLASPPGRRERSGQAHLCEALLQAEAEAEPKPMAKPEPENLRALSIAPLSLPWLPTLPAPLLPARQPLGPHPANLSPGTPAGPTSSRPRAAAAAAAAASGAGPLPARPPGRSESRQPHRLNCFLL

SEQ ID NO: 1621 - protein, 48 aa, Homo sapiens
MKETKMPSPSSPPTMLKPRPVEPLCRMILRGSLSPGTPAGPTSSRPRA

SEQ ID NO: 1622 - protein, 47 aa, Homo sapiens
MKETKMPSPSSPPTMLKPRPVEPLCRMILRGSLVKSSSASMCLGIGE

SEQ ID NO: 1623 - protein, 47 aa, Homo sapiens
MKEWSCRWSNGKIILNKGGESVLIPNAASPYCCVFSLLDRVGLHTLS

SEQ ID NO: 1624 - protein, 13 aa, Homo sapiens
MKFLKEYFLAKEN

SEQ ID NO: 1625 - protein, 12 aa, Homo sapiens
MKFLPPERRSCP

SEQ ID NO: 1626 - protein, 23 aa, Homo sapiens
MKFLWNSSSHSQLLPLSRNVLIR

SEQ ID NO: 1627 - protein, 19 aa, Homo sapiens
MKFQLYHDLWVKLEIIVTL

SEQ ID NO: 1628 - protein, 48 aa, Homo sapiens
MKHPAELLLLILCLRHHLVFVEAVSQLLLFLLSLFHIGILFLSNDSVH

SEQ ID NO: 1629 - protein, 57 aa, Homo sapiens
MKIIPCFHHYLYSSHHYLYSSSLCLFFFPKKDITSLSSPPLCSCPSLPLARSRQSWR

SEQ ID NO: 1630 - protein, 21 aa, Homo sapiens
MKILLENYEKKTIFCFQKVKD

SEQ ID NO: 1631 - protein, 19 aa, Homo sapiens
MKIMIFHSQMAEDVFDRYV

SEQ ID NO: 1632 - protein, 37 aa, Homo sapiens
MKINNTDPTYTVEPYLGCHGRKRERKKEREREETTLC

SEQ ID NO: 1633 - protein, 11 aa, Homo sapiens
MKIRISSDGGR

SEQ ID NO: 1634 - protein, 21 aa, Homo sapiens
MKKPSDFFFFLDKVSLLLPRL

SEQ ID NO: 1635 - protein, 57 aa, Homo sapiens
MKLDVFLPCRDNNGVDLAAQIYVVITATQDTARCAPGTERCKQSEERSLLLCCLCFQ

SEQ ID NO: 1636 - protein, 49 aa, Homo sapiens
MKLKSWGIFRNFCNYALKGPFIMVTVPDSRNIIVFLYIIESDTHTVRQG

SEQ ID NO: 1637 - protein, 41 aa, Homo sapiens
MKLRFKAASLPEDCKPATSPGFGSSEDLKVPDYLAQECRRF

SEQ ID NO: 1638 - protein, 57 aa, Homo sapiens
MKMAMFYHLAKKGKLPSDSNLHGPSVSSLNMWYEDRKCWSCLIQTWVQISFPPCLAM

SEQ ID NO: 1639 - protein, 15 aa, Homo sapiens
MKMIDIKIDYLPPLL

SEQ ID NO: 1640 - protein, 186 aa, Homo sapiens [sequence omitted]

SEQ ID NO: 1641 - protein, 47 aa, Homo sapiens
MKNCPRFVRVISFFNKSIYMSDGLLPKMCLLVYKLPLKQVFTFPVFP

SEQ ID NO: 1642 - protein, 23 aa, Homo sapiens
MKNFSRGGISTVGAWQGVTDPWF

SEQ ID NO: 1643 - protein, 77 aa, Homo sapiens
MKPCLIWLTSTGQVLWLERSMSRSHTSARSSCSRATVGLLSSQQSSLSSGMKGHQMILRKWFSGVPSGCRIWTKISS

SEQ ID NO: 1644 - protein, 20 aa, Homo sapiens
MKPYKPWQILHSSSSMQKKN

SEQ ID NO: 1645 - protein, 23 aa, Homo sapiens
MKPYKPWQILHSSSSMQKKNLSF

SEQ ID NO: 1646 - protein, 31 aa, Homo sapiens
MKRCSASLLIREMQIKTTMKCHLTPTMMAAI

SEQ ID NO: 1647 - protein, 19 aa, Homo sapiens
MKSHYQQKDYNLWSSYCYL

SEQ ID NO: 1648 - protein, 100 aa, Homo sapiens
MKSITVVASGERPGAIGASCSTRATLGAEKRESSLGTRATPPAAAPGGTAAAPPPAAAPPRARGLPFRSGPADSSDSEPSSSSTSTAAACGDGFTGAPDQ

SEQ ID NO: 1649 - protein, 31 aa, Homo sapiens
MKTARRFLSHEENGLISLENCTMCFHHNGEP

SEQ ID NO: 1650 - protein, 53 aa, Homo sapiens
MKTMCLVRRKLKKSALKRHLSPFQMPPICRLHFISSSSLKPFTPWLFLANTHI

SEQ ID NO: 1651 - protein, 28 aa, Homo sapiens
MKTSATMRKSWSESASGLFSQLDLLLST

SEQ ID NO: 1652 - protein, 21 aa, Homo sapiens
MKTSIFLTHFPCHSLPCGFFI

SEQ ID NO: 1653 - protein, 22 aa, Homo sapiens
MKTVAHEMHPLKQRIMRNSSRL

SEQ ID NO: 1654 - protein, 12 aa, Homo sapiens
MKTVYNGDQGWR

SEQ ID NO: 1655 - protein, 36 aa, Homo sapiens
MKTYKSIKCTSVIDTQRRKIKKTYLHRKSQNHSDKH

SEQ ID NO: 1656 - protein, 53 aa, Homo sapiens
MKVWPEILVVFPLRVVLGSWMSRMGLFLVCELMKTSIFLTHFPCHSLPCGFFI

SEQ ID NO: 1657 - protein, 27 aa, Homo sapiens
MLACMVRKSRPKSTRQPTSPKCHSLVT

SEQ ID NO: 1658 - protein, 26 aa, Homo sapiens
MLAKMVSSPDLVIHLPRPPRVLGFQV

SEQ ID NO: 1659 - protein, 20 aa, Homo sapiens
MLAQYKRETNRKLFRLSGQQ

SEQ ID NO: 1660 - protein, 77 aa, Homo sapiens [sequence omitted]

SEQ ID NO: 1661 - protein, 14 aa, Homo sapiens
MLARLVLNLTPDVK

SEQ ID NO: 1662 - protein, 27 aa, Homo sapiens
MLARLVLNSRPEVVQPPQPRKVLGLQA

SEQ ID NO: 1663 - protein, 27 aa, Homo sapiens
MLARLVLNSSPQVICPPQPPKVLGLQV

SEQ ID NO: 1664 - protein, 11 aa, Homo sapiens
MLARLVSNCCP

SEQ ID NO: 1665 - protein, 54 aa, Homo sapiens [sequence omitted]

SEQ ID NO: 1666 - protein, 37 aa, Homo sapiens [sequence omitted]

SEQ ID NO: 1667 - protein, 33 aa, Homo sapiens
MLCSLSPGPATLGSSAKGTWHCSGTSCRAWISR

SEQ ID NO: 1668 - protein, 27 aa, Homo sapiens
MLDRLVSNSQSQVIRLPRPPKVQGLEV

SEQ ID NO: 1669 - protein, 27 aa, Homo sapiens
MLDSARQPLQKTPPGRRLGAPSRGEAD

SEQ ID NO: 1670 - protein, 114 aa, Homo sapiens [sequence omitted]

SEQ ID NO: 1671 - protein, 19 aa, Homo sapiens
MLEIKILEMNNSVQLCIHK

SEQ ID NO: 1672 - protein, 18 aa, Homo sapiens
MLERMWRNRNAFTLLVGV

SEQ ID NO: 1673 - protein, 12 aa, Homo sapiens
MLESVFIQIWKR

SEQ ID NO: 1674 - protein, 28 aa, Homo sapiens
MLEVGSCGRCLGHGDRFLITWCCPTDNE

SEQ ID NO: 1675 - protein, 18 aa, Homo sapiens
MLFHRCKLHCHLKSLCLQ

SEQ ID NO: 1676 - protein, 18 aa, Homo sapiens
MLFLHCGPADVLKDMRTT

SEQ ID NO: 1677 - protein, 134 aa, Homo sapiens
MLFNRKIRCDEDLYSCSRFRPDRTSNKAIRILPSCISTNKSLTSRGGLHFSRCRFIHRVKVLFCTFSLSTCRFCTRMSLICPMSSSRWNQSHSCAAMKRGRESPGQRGAGGGRGEPGWRARERHAPGEGAAELE

SEQ ID NO: 1678 - protein, 135 aa, Homo sapiens
MLFNRKIRCDEDLYSCSRFRPDRTSNKAIRILPSCISTNKSLTSRGGLHFSRCRFIHRVKVLFCTFSLSTCRFCTRMSLICPMSSSRWNQSHSCAAMKRGRESPGQRGAGGGRGEPGWRARERHAPGEGAAELES

SEQ ID NO: 1679 - protein, 112 aa, Homo sapiens
MLFNRKIRCDEDLYSCSRFRPDRTSNKAIRILPSCISTNKSLTSRGGLHFSRCRFIHRVKVLFCTFSLSTPEAPPTIQFPLPRRYLGSARTHTHTHTHTHTHTQSRTVSSPP

SEQ ID NO: 1680 - protein, 42 aa, Homo sapiens
MLFSLICTFNFFEFILDNFQISNSFCLTGLLYLQSSFKVSNP

SEQ ID NO: 1681 - protein, 473 aa, Homo sapiens
MLGHNEVAAAVDAGYEGGKVAVLAAGRLSERDVHVPVGVDSSLHDTDVRTILLLQAWPPPTGGATPVAVTIAGREAGSSLLLQVPGGRQGDCPLVCQPPPVHRGGYSAARAVADRRMHLQDPLGHKRLQTFPFVADAALPVLGRLAAADELELVGREPLAAVADGRALAALAEFAHVEQRAVGAALHLDARLAVVQQRLEIRGRGRGGREALEGQRVPGQVEVRGGLVQAEVGARGAERRGQQSLVTGGRGGQRGGRGEGGRRGQWRQVAWQRRQRQRGQGRVERGQSQGQVLAARELLLDRRHGAPVAPQPRSPPAAATYSGPGWSWVAGAGEAPGRAPTPSASAPRRPQPPPTRRPPGLPGLPSRPAGPQRPETWSCYRSRIDSPSAAVPGPRGSPGRLESRAPATSARARGSPTPGSPTHPPGRARQRGVAESPPLSGVPSPRPAARAASVVHPRPLARARPAGTWETPP

SEQ ID NO: 1682 - protein, 155 aa, Homo sapiens
MLGHNEVAAAVDAGYEGGKVAVLAAGRLSERDVHVPVGVDSSLHDTDVRTILLLQAWPPPTGGATPVAVTIAGREAGSSLLLQVPGGRQGDCPLVCQPPPVHRGGYSAARAVADRRMHLQDPLGHKRLQTFPSARLPSPLPVPPSRTPQGSAGLC

SEQ ID NO: 1683 - protein, 80 aa, Homo sapiens
MLGLDSKRDSQELNWVFDFSGSRVVPPTPSEEMHLRLVDLKRPPAAPSISRGDFAPTLSERFPSSLPALPLLSVEAPVVW

SEQ ID NO: 1684 - protein, 94 aa, Homo sapiens
MLGQAAWVLKVLKKAAAVASTTPLRVRKSSAWMLLKFPQRPQVCPRSLGASCMNSCMVGTSCRFSCRPRLVWAMMKKVEGLKMVTLAAEMGSWV

SEQ ID NO: 1685 - protein, 71 aa, Homo sapiens
MLGQSCSLTEPLSPCISLGRDPCPGTYLRFTHRKVLRRVSKPLMPQRALVPMTDGSMPPFHSHFLSIYYEP

SEQ ID NO: 1686 - protein, 16 aa, Homo sapiens
MLGSYEETAWYVRERK

SEQ ID NO: 1687 - protein, 88 aa, Homo sapiens
MLHAFVTELSKIIDLRHTNSSPCRFIMRNRDDVASSMSKISTMPSTHFPWFLSKSKLGANSSFPGCSMERQTRPIIRISSQAHSRRWT

SEQ ID NO: 1688 - protein, 92 aa, Homo sapiens
MLHAFVTHVPDVGEDEEELGQPLVLLLQGQACLGHQVDQSVCDLVQDSVDMVLLFQRLQGAGQKCVHSRIKQNNRFEAHKLLSLQIHHAEPR

SEQ ID NO: 1689 - protein, 12 aa, Homo sapiens
MLIIKKSRNNRC

SEQ ID NO: 1690 - protein, 16 aa, Homo sapiens
MLISSSLCSLVSVQRS

SEQ ID NO: 1691 - protein, 21 aa, Homo sapiens
MLISYHPTFHPFAGRSILFQC

SEQ ID NO: 1692 - protein, 36 aa, Homo sapiens
MLKGNWEVTSLIEFSKCCGLGWSFFKCPCSWRASHD

SEQ ID NO: 1693 - protein, 50 aa, Homo sapiens
MLKIFTEKLCFLFWNPVTSQVVSALTTALSCLNCVNQNDCSKISQDLFHV

SEQ ID NO: 1694 - protein, 15 aa, Homo sapiens
MLKLQCVPGLGDISP

SEQ ID NO: 1695 - protein, 64 aa, Homo sapiens
MLKPLIKGFMGFQISSDAQMFSDSIIIFSRKWTFHSLFLALIIDFCYRILRNFHKYFFCSFVLF

SEQ ID NO: 1696 - protein, 68 aa, Homo sapiens
MLKPRPVEPLCRMILRGSLASPPGRRERSGQAHLCEALLQAEAEAEPKPMAKPEPENLRALSIAPLSL

SEQ ID NO: 1697 - protein, 142 aa, Homo sapiens
MLKPRPVEPLCRMILRGSLASPPGRRERSGQAHLCEALLQAEAEAEPKPMAKPEPENLRALSIAPLSLPWLPTLPAPLLPARQPLGPHPANLSPGTPAGPTSSRPRAAAAAAAAASGAGPLPARPPGRSESRQPHRLNCFLL

SEQ ID NO: 1698 - protein, 34 aa, Homo sapiens
MLKPRPVEPLCRMILRGSLSPGTPAGPTSSRPRA

SEQ ID NO: 1699 - protein, 33 aa, Homo sapiens
MLKPRPVEPLCRMILRGSLVKSSSASMCLGIGE

SEQ ID NO: 1700 - protein, 40 aa, Homo sapiens
MLKSKHWYKITAFSHHQNMCLMKIMIFHSQMAEDVFDRYV

SEQ ID NO: 1701 - protein, 77 aa, Homo sapiens
MLKTLNELGIDGTYLKIIRAIYDKPTANIRLNGQKLEAFPLKTGTRQGCPLSPLLFNIVLEVLARAIRQEKEIKGIQ

SEQ ID NO: 1702 - protein, 11 aa, Homo sapiens
MLLDLSISVSP

SEQ ID NO: 1703 - protein, 18 aa, Homo sapiens
MLLFFALNGQVSFKIFKK

SEQ ID NO: 1704 - protein, 42 aa, Homo sapiens
MLLHCWWEYKLVQPLWKTVWQFLEDLEPEIPFNPAIPLLGIP

SEQ ID NO: 1705 - protein, 12 aa, Homo sapiens
MLLILSIEVSPS

SEQ ID NO: 1706 - protein, 13 aa, Homo sapiens
MLLIQEKNEREQN

SEQ ID NO: 1707 - protein, 44 aa, Homo sapiens
MLLLGGLHSCQVIPKVILGHEALVFTEPGLSHCGLPVKAPGQLL

SEQ ID NO: 1708 - protein, 13 aa, Homo sapiens
MLLLSFAVWTKAC

SEQ ID NO: 1709 - protein, 20 aa, Homo sapiens
MLLTILAEDFSCLASPSIIL

SEQ ID NO: 1710 - protein, 85 aa, Homo sapiens
MLLVAKFESLNPQLIFGKSFDMNMFDSLNYSIIKFHSVSTILVNSSDFGRVKTTIRPASKDLLIYLKFRRSILFMQALFPQLYFL

SEQ ID NO: 1711 - protein, 14 aa, Homo sapiens
MLLVAKFESLNPQQ

SEQ ID NO: 1712 - protein, 66 aa, Homo sapiens
MLLVHGIRSVLLQRGSSRVPSLSYLSKDCFYHTQMCSFYNWGISFSQLQLHHDFHLYGSECANHGF

SEQ ID NO: 1713 - protein, 39 aa, Homo sapiens
MLLVKSFSALLIPLTALICEHLYSVQLYLWHKISFPKWH

SEQ ID NO: 1714 - protein, 30 aa, Homo sapiens
MLLVVSYLSSPPDGNLLQNMDLSPFPCCLC

SEQ ID NO: 1715 - protein, 44 aa, Homo sapiens
MLNKHICWASWAFESVNLAAVQGAPEGYPWCMLETGGREIVAKM

SEQ ID NO: 1716 - protein, 20 aa, Homo sapiens
MLNPTSSGKDSKTILREGNG

SEQ ID NO: 1717 - protein, 50 aa, Homo sapiens
MLNTSEGKKMIITIMKTYKSIKCTSVIDTQRRKIKKTYLHRKSQNHSDKH

SEQ ID NO: 1718 - protein, 29 aa, Homo sapiens
MLNVVLAVLLKSLYYRKRKCSVYFLENSS

SEQ ID NO: 1719 - protein, 11 aa, Homo sapiens
MLPAPASCGHM

SEQ ID NO: 1720 - protein, 15 aa, Homo sapiens
MLPAPASCGHMSQHG

SEQ ID NO: 1721 - protein, 18 aa, Homo sapiens
MLPAPASCGHMSQHGSCS

SEQ ID NO: 1722 - protein, 20 aa, Homo sapiens
MLPAPASCGHMSQHGSCSRS

SEQ ID NO: 1723 - protein, 29 aa, Homo sapiens
MLPGCPGVLAVDLPIPAGHRATEAGPPGE

SEQ ID NO: 1724 - protein, 19 aa, Homo sapiens
MLPLTLDICSCSPALWKEH

SEQ ID NO: 1725 - protein, 17 aa, Homo sapiens
MLPLYVTVPWSEMVTVL

SEQ ID NO: 1726 - protein, 27 aa, Homo sapiens
MLPRLVLNSWPQAIFPPWPPKVPGLQA

SEQ ID NO: 1727 - protein, 12 aa, Homo sapiens
MLPSDDLKNVYF

SEQ ID NO: 1728 - protein, 16 aa, Homo sapiens
MLPSIWHTSCVSHFHQ

SEQ ID NO: 1729 - protein, 37 aa, Homo sapiens [sequence omitted]

SEQ ID NO: 1730 - protein, 71 aa, Homo sapiens
MLQGSRAPHYVWCCHRTPQSALLRALGLLPGMAGRACQHTGGRSGLFLFPFLLSQVMQQSPSQLIRVHSSH

SEQ ID NO: 1731 - protein, 25 aa, Homo sapiens
MLRCNPQCWRWGLVGGVWVMGTDSS

SEQ ID NO: 1732 - protein, 51 aa, Homo sapiens
MLRGCGEIGMLLHCWWEYKLVQPLWKTVWQFLEDLEPEIPFNPAIPLLGIP

SEQ ID NO: 1733 - protein, 11 aa, Homo sapiens
MLRKIAASLLQ

SEQ ID NO: 1734 - protein, 39 aa, Homo sapiens
MLRLMTTHCILFLYCNLEGSGKFQKVLKGSHPVKCCTPM

SEQ ID NO: 1735 - protein, 34 aa, Homo sapiens
MLSADMGQSPHAAEDRSVSAPVVTVESSKQFTTN

SEQ ID NO: 1736 - protein, 25 aa, Homo sapiens
MLSAGLRKVRHRACMSSARTGWMWS

SEQ ID NO: 1737 - protein, 65 aa, Homo sapiens
MLSICCRRSSSSMGSSASGPLSLSISKGLIQVGSSKGLPGTRGLESLCWGCSSSSLKGLGAGLSG

SEQ ID NO: 1738 - protein, 29 aa, Homo sapiens
MLSISLFISCTIFFTSKMFVFFLGFLFLY

SEQ ID NO: 1739 - protein, 21 aa, Homo sapiens
MLSLKYQHHLEVEQVDKGGEV

SEQ ID NO: 1740 - protein, 61 aa, Homo sapiens
MLSPPGLPCRIRLTCLPWDLSNLILTGVFSLSSLAPYTPFLVSLRSTSLIIHFPTVLRVCF

SEQ ID NO: 1741 - protein, 36 aa, Homo sapiens
MLSPSKTEEGATRVSESACSVTASKMTSNDHSSMRT

SEQ ID NO: 1742 - protein, 91 aa, Homo sapiens
MLSQPSLQLLRKDGQELLQHQQLQDLLLGVHLRPQPLTAKLSQPAQSLPRASGVRVTKLPELLPEYLLAPGVFLKAKVLVQNIIFFFNLDN

SEQ ID NO: 1743 - protein, 35 aa, Homo sapiens
MLSRMRRKWNPQTHAGGNAKCCSHFGKQPGSSSKG

SEQ ID NO: 1744 - protein, 83 aa, Homo sapiens [sequence omitted]

SEQ ID NO: 1745 - protein, 18 aa, Homo sapiens
MLSSSSSRLKQCKDTFTG

SEQ ID NO: 1746 - protein, 13 aa, Homo sapiens
MLTATESWNPTLD

SEQ ID NO: 1747 - protein, 14 aa, Homo sapiens
MLTDLGLGQGLMEL

SEQ ID NO: 1748 - protein, 25 aa, Homo sapiens
MLTGFKISMSFCGKLACKIVLDSFN

SEQ ID NO: 1749 - protein, 52 aa, Homo sapiens
MLTISHLKYSPASHRVPMTSLQICRNLGFSVYHKLATGAWQITLSFYSSSLK

SEQ ID NO: 1750 - protein, 14 aa, Homo sapiens
MLVDFLMGPEMSFT

SEQ ID NO: 1751 - protein, 32 aa, Homo sapiens [sequence omitted]

SEQ ID NO: 1752 - protein, 17 aa, Homo sapiens
MLVFWCFLLTFENLVHC

SEQ ID NO: 1753 - protein, 171 aa, Homo sapiens
MLVGTLDGTMPARVELMGNLDGAGLVSALEGTAPGGFELVGNLEGTVLTDAGLAGTFRATVFTGIKVVGTLEGRELAGASAPLEQMIGSAWSLSAPCLPSAAPAEAKPGDEEEKEVPVDTTDPVGPGKRLALGVERARGWKETDGDTGPRDGVRLEVAPAVWVLPSSVSCS

SEQ ID NO: 1754 - protein, 73 aa, Homo sapiens
MLVKLVSNSGPQVIHLPRPPKVLGLQARATAPGQFPCISSLLRVLANCSFLYLSKLPHVIYHFFLINETDYND

SEQ ID NO: 1755 - protein, 25 aa, Homo sapiens
MLVQIARIGVPALPFVVYICTCYFI

SEQ ID NO: 1756 - protein, 27 aa, Homo sapiens
MLVRLVLNSWPQVIRPPQPPEVLGLQA

SEQ ID NO: 1757 - protein, 27 aa, Homo sapiens
MLVRLVSNSQPQVICLPWPPKVLGLQV

SEQ ID NO: 1758 - protein, 48 aa, Homo sapiens
MLVRVVSNSRPQIIRPPPNPGLPKCWDYRREPPRPASFLFCKFFLIPS

SEQ ID NO: 1759 - protein, 27 aa, Homo sapiens
MLVYPHQVLHIKSPYPKLSRKYRQGRE

SEQ ID NO: 1760 - protein, 11 aa, Homo sapiens
MLYMLEIMQIN

SEQ ID NO: 1761 - protein, 153 aa, Homo sapiens
MLYRCSMPLLLMCLMWERMRRSWASRWCCCCRVRPALAIRWIKVSVILSRTRWIWSFSSRDFRVLDRNVYTPELSKIIDLRHTNSSPCRFIMRNRDDVASSMSKISTMPSTHFPWFLSKSKLGANSSFPGCSMERQTRPIIRISSQAHSRRWT

SEQ ID NO: 1762 - protein, 12 aa, Homo sapiens
MLYRCSMPLLQN

SEQ ID NO: 1763 - protein, 70 aa, Homo sapiens
MLYSISAFSPTSASLALILPIGVPGGEDSGVLNWYVLWGNRGGLSLTSVSVMFTVVVPDNPPIWPPISLA

SEQ ID NO: 1764 - protein, 28 aa, Homo sapiens
MLYTSKHTEHKFNFIRHIHSLLLPTYTL

SEQ ID NO: 1765 - protein, 23 aa, Homo sapiens
MMAKSHHFSVWSYSIVALCKLFK

SEQ ID NO: 1766 - protein, 28 aa, Homo sapiens
MMAPQMQQWRKIPPKTRKVPLQPRFSRR

SEQ ID NO: 1767 - protein, 14 aa, Homo sapiens
MMCTEHRLLVEWEW

SEQ ID NO: 1768 - protein, 78 aa, Homo sapiens
MMFSRVSTGAAQRVCVNLLNSGFRSSCRFWSRVSKPWLLSSPRGPSRRLRVSWGTCQFCSMDIRKDRQLLMLAITLAL

SEQ ID NO: 1769 - protein, 25 aa, Homo sapiens
MMGLLSRIARSTQDVFSFKDNSKDC

SEQ ID NO: 1770 - protein, 29 aa, Homo sapiens
MMNCVAGAEELLSLESGSKPSFSSLAFSK

SEQ ID NO: 1771 - protein, 56 aa, Homo sapiens
MMNCVAGAEELLSLESLMTVTTDTLSPTWGWGTARLPVGRSGEPFTKVSSITRLVW

SEQ ID NO: 1772 - protein, 18 aa, Homo sapiens
MMPLFLFHILWLESHYYV

SEQ ID NO: 1773 - protein, 15 aa, Homo sapiens
MMRPPQPPKVLGLQA

SEQ ID NO: 1774 - protein, 19 aa, Homo sapiens
MMSLWVESFKCPIRKGIHF

SEQ ID NO: 1775 - protein, 56 aa, Homo sapiens
MMTPMAQQSTGRPYRCRPTTSGARYSGVPQGSLMRPFSSLARWKSLMTIFEFFSRL

SEQ ID NO: 1776 - protein, 12 aa, Homo sapiens
MMTVAMGTEPVV

SEQ ID NO: 1777 - protein, 84 aa, Homo sapiens
MMVSPFPGSLQAPCLGSIFFFSSPILTRKMSELTSRKRVFRLCQKYMQFFKNQLKNLAFIFICKKKVVGSVGFSKNGLSYGCGS

SEQ ID NO: 1778 - protein, 139 aa, Homo sapiens
MMVSTVSNRTAFPAFRLVSVLVATWASKSFMVSLLSSWFRPRIRSRRSIWTCRKGSLTPDMLCSVEYPIVTRVRRMCTSWGTTFRKCLRAAGLRSQSSVISVMVPSRMPGVSVGEVNGGGQGQESLLRVCLCVCTTLLL

SEQ ID NO: 1779 - protein, 110 aa, Homo sapiens
MMVSTVSNRTAFPAFRLVSVLVATWASKSFMVSLLSSWFRPRIRSRRSIWTCRKGSLTPDMLCSVEYPIVTRVRRMCTSWGTTFRKCLRAAGLRSQSSVISVMVPSRMPW

SEQ ID NO: 1780 - protein, 47 aa, Homo sapiens
MMWKEYKLLNSFQRVIWQESSNVKIRYHLQPICLASRSRHLCSEKHI

SEQ ID NO: 1781 - protein, 28 aa, Homo sapiens
MNCVAGAEELLSLESGSKPSFSSLAFSK

SEQ ID NO: 1782 - protein, 55 aa, Homo sapiens
MNCVAGAEELLSLESLMTVTTDTLSPTWGWGTARLPVGRSGEPFTKVSSITRLVW

SEQ ID NO: 1783 - protein, 21 aa, Homo sapiens
MNDLKNLVLLNTECKSVVFHL

SEQ ID NO: 1784 - protein, 15 aa, Homo sapiens
MNFSIAPHMGLVIKL

SEQ ID NO: 1785 - protein, 43 aa, Homo sapiens
MNHWDGKGKSFPTSCLSSPKDVQFVTDGRCQGQGLDWCGCREA

SEQ ID NO: 1786 - protein, 11 aa, Homo sapiens
MNKYYFIIGEE

SEQ ID NO: 1787 - protein, 21 aa, Homo sapiens
MNLKEHGTPLQVWLSQCAPIA

SEQ ID NO: 1788 - protein, 11 aa, Homo sapiens
MNLLPTQKDLR

SEQ ID NO: 1789 - protein, 33 aa, Homo sapiens [sequence omitted]

SEQ ID NO: 1790 - protein, 64 aa, Homo sapiens
MNMFDSLNYSIIKFHSVSTILVNSSDFGRVKTTIRPASKDLLIYLKFRRSILFMQALFPQLYFL

SEQ ID NO: 1791 - protein, 11 aa, Homo sapiens
MNNSVQLCIHK

SEQ ID NO: 1792 - protein, 38 aa, Homo sapiens
MNQKRISLVFIIYMGACLPPGPSLVLLCRLYFPHFSAT

SEQ ID NO: 1793 - protein, 24 aa, Homo sapiens
MNQKVEKTCHGSSLGGGQTRGHWQ

SEQ ID NO: 1794 - protein, 11 aa, Homo sapiens
MNRKSLLVRKI

SEQ ID NO: 1795 - protein, 14 aa, Homo sapiens
MNSACSGSQEARYI

SEQ ID NO: 1796 - protein, 18 aa, Homo sapiens
MNSESFNPPDDLIFPSKL

SEQ ID NO: 1797 - protein, 79 aa, Homo sapiens
MNSGRNNTTKYSFSGSVISGASPNRAWFSKIRPAEPPQLCSWPKLKKPSHYQMYLSICSLCESYHVAFTKKKAFKEWQK

SEQ ID NO: 1798 - protein, 60 aa, Homo sapiens
MNSSFYLIKSAADAFYFTFHFMHYILHLQNVCFFFRISISLLNVSFCVLMISLGCLSVLW

SEQ ID NO: 1799 - protein, 38 aa, Homo sapiens
MNSYNSKFQPLSLGNNLGLAATDVLVGIHFLRRKSANS

SEQ ID NO: 1800 - protein, 116 aa, Homo sapiens
MNSYNSKFQPLSLGNNLGLAATDVLVGIHFLRRKSVHIHHGTFGYPLNDYNTMHPHCPEPGPLPPPRPPPRPAEGAAHLAERPGRSPCPGRAAPEPRDARTQLGRSRCRRYRRRSR

SEQ ID NO: 1801 - protein, 118 aa, Homo sapiens
MNSYNSKFQPLSLGNNLGLAATDVLVGIHFLRRKSVHIHHGTFGYPLNDYNTMHPHCPEPGPLPPPRPPPRPAEGAAHLAERPGRSPCPGRAAPEPRDARTQLGRSRCRRYRRRSREA

SEQ ID NO: 1802 - protein, 30 aa, Homo sapiens
MNTECLVSLCKTCKCPSADNFWPFLYPGWS

SEQ ID NO: 1803 - protein, 12 aa, Homo sapiens
MNVFDASNKIVN

SEQ ID NO: 1804 - protein, 65 aa, Homo sapiens [sequence omitted]

SEQ ID NO: 1805 - protein, 47 aa, Homo sapiens
MNYFLNKPICYIWKSCFLETNKNIIYISFTRMVSNGNTRQMAKSIIK

SEQ ID NO: 1806 - protein, 21 aa, Homo sapiens
MNYFLNKPICYIWKSCFRFFH

SEQ ID NO: 1807 - protein, 79 aa, Homo sapiens
MPAAAAGSGTPGPPWPRGARPAVPRPAVTAPCPRTRTGPPGPAAPAGSPSCDAWGPPRARRRRTGGTALWCCLPPPPPG

SEQ ID NO: 1808 - protein, 50 aa, Homo sapiens
MPAAAGTRPEEWAGCGAGAPGSALRRQRQRAERKAERTRRRRRRRLRSWP

SEQ ID NO: 1809 - protein, 12 aa, Homo sapiens
MPESSIQQANSR

SEQ ID NO: 1810 - protein, 77 aa, Homo sapiens [sequence omitted]

SEQ ID NO: 1811 - protein, 48 aa, Homo sapiens
MPFQHRWVGACDSQAANAGNSVSSEMLEPGRLLESSRPRRRTTGPGDP

SEQ ID NO: 1812 - protein, 12 aa, Homo sapiens
MPFSFVGWKDCL

SEQ ID NO: 1813 - protein, 59 aa, Homo sapiens
MPGANVMKTMCLVRRKLKKSALKRHLSPFQMPPICRLHFISSSSLKPFTPWLFLANTHI

SEQ ID NO: 1814 - protein, 29 aa, Homo sapiens
MPGKLCTKYNDVLSTQRLLNSFSLSFVPL

SEQ ID NO: 1815 - protein, 27 aa, Homo sapiens
MPGLLLYFCREGVSPCWPGWSQTPDLK

SEQ ID NO: 1816 - protein, 72 aa, Homo sapiens
MPGLLNGAAFAPGLFPSNVRSGKGWSPPSASAPVLHIFLTLLLLLGFVSLGFPSVILFFYLFIGIRGGPLTF

SEQ ID NO: 1817 - protein, 35 aa, Homo sapiens
MPGLLNGADAHFIKSLFSRLCSTQLGRSEGAAESI

SEQ ID NO: 1818 - protein, 26 aa, Homo sapiens
MPGLLNGAHSARPRSRFHISWQLRNS

SEQ ID NO: 1819 - protein, 16 aa, Homo sapiens
MPGLLNGAHSSFVECD

SEQ ID NO: 1820 - protein, 27 aa, Homo sapiens
MPGLLNGVCWPALDSFLLQSCQCAGTV

SEQ ID NO: 1821 - protein, 12 aa, Homo sapiens
MPGRRSVHCGSH

SEQ ID NO: 1822 - protein, 14 aa, Homo sapiens
MPKIKGLVFDGVRS

SEQ ID NO: 1823 - protein, 23 aa, Homo sapiens
MPKRPKNLILLRQWYRQPIMWPL

SEQ ID NO: 1824 - protein, 17 aa, Homo sapiens
MPLFLFHILWLESHYYV

SEQ ID NO: 1825 - protein, 20 aa, Homo sapiens
MPLGVDFPQLVGTHDQAPGM

SEQ ID NO: 1826 - protein, 147 aa, Homo sapiens
MPLLLMCLMWERMRRSWASRWCCCCRVRPALAIRWIKVSVILSRTRWIWSFSSRDFRVLDRNVYTPELSKIIDLRHTNSSPCRFIMRNRDDVASSMSKISTMPSTHFPWFLSKSKLGANSSFPGCSMERQTRPIIRISSQAHSRRWT

SEQ ID NO: 1827 - protein, 44 aa, Homo sapiens
MPLRLANFCIFSRDGVSPCWPGWSRFPDLVIRPPRPPKVVGLQA

SEQ ID NO: 1828 - protein, 17 aa, Homo sapiens
MPLSLPGPHSCSHMFTS

SEQ ID NO: 1829 - protein, 28 aa, Homo sapiens
MPPAAPETGQVTGCTSPSGVTSQCNALF

SEQ ID NO: 1830 - protein, 46 aa, Homo sapiens
MPPAAPETGQVTGCTSPSGVTSQCNALFPCGIRQMSNFSSLSQTSA

SEQ ID NO: 1831 - protein, 39 aa, Homo sapiens
MPPAAPETGQVTGCTSPSGVTSQCNALFPLCTGISGHRK

SEQ ID NO: 1832 - protein, 70 aa, Homo sapiens
MPPCLANFCIFSRDGVSPCWPGWSQTPDLKRSAHLGLPKCWDYRREPLQPARVHILKFGMRIALVLEHAL

SEQ ID NO: 1833 - protein, 78 aa, Homo sapiens
MPPCPANFFSFRDGSLAQASLKLLASSDPPISASQSDRITGVSHHAWLLCKCLNFILYLSVCLDFLSLLGSVRPLVSF

SEQ ID NO: 1834 - protein, 19 aa, Homo sapiens
MPPCPANFLYFSRDGVSPC

SEQ ID NO: 1835 - protein, 13 aa, Homo sapiens
MPPFLRHLPSVPS

SEQ ID NO: 1836 - protein, 35 aa, Homo sapiens
MPPQFFRAILLSSLAFPYTRFLRAPQALRWTSVIR

SEQ ID NO: 1837 - protein, 42 aa, Homo sapiens
MPPQPSRPNAQFCLCVCNNNPSIYDKLSDSFLKTGFLRLSTL

SEQ ID NO: 1838 - protein, 24 aa, Homo sapiens
MPPRPAYFCIFSRDGVSSYRSGWS

SEQ ID NO: 1839 - protein, 117 aa, Homo sapiens
MPQGQATQCLGAAGCQAHLLRLGAAGCVLQLLLQAPDDLLRLLVELLQVGLLTLQHADLAPASLLHVLPLLLKVPFQCRNFPFVVIYHSTMGGQGSPELPVNPSGIPRAWPQAAPPS

SEQ ID NO: 1840 - protein, 120 aa, Homo sapiens
MPQGQATQCLGAAGCQAHLLRLGAAGCVLQLLLQAPDDLLRLLVELLQVGLLTLQHADLAPASLLHVLPLLLKVPFQCRNFPFVVIYLGLQLGPEVLVMLLYLLHHQLRFYTHWSRITQE

SEQ ID NO: 1841 - protein, 23 aa, Homo sapiens
MPQTENFTHTMGAGVGWGGVGVL

SEQ ID NO: 1842 - protein, 16 aa, Homo sapiens
MPRMRCSFKMESTVSL

SEQ ID NO: 1843 - protein, 69 aa, Homo sapiens
MPRSAAGAPPPPLGPSAAAAPDLEAPGVTRSLAKAVTVVAPESGSATGRTGLRGPWAGRTVAPGCSPEC

SEQ ID NO: 1844 - protein, 37 aa, Homo sapiens
MPRVHFFFFLSHPNKEDVRANIQEKGLSSLSKVHAIF

SEQ ID NO: 1845 - protein, 50 aa, Homo sapiens
MPSAVSKTFLASSVLPSNHSRCAYCFHRQKLLQFSGSLRRFLASFLQFFP

SEQ ID NO: 1846 - protein, 24 aa, Homo sapiens
MPSCPANFCIFSRDRVLPHWPGWS

SEQ ID NO: 1847 - protein, 16 aa, Homo sapiens
MPSPHSFSAPRYSMYL

SEQ ID NO: 1848 - protein, 77 aa, Homo sapiens
MPSPSSPPTMLKPRPVEPLCRMILRGSLASPPGRRERSGQAHLCEALLQAEAEAEPKPMAKPEPENLRALSIAPLSL

SEQ ID NO: 1849 - protein, 151 aa, Homo sapiens
MPSPSSPPTMLKPRPVEPLCRMILRGSLASPPGRRERSGQAHLCEALLQAEAEAEPKPMAKPEPENLRALSIAPLSLPWLPTLPAPLLPARQPLGPHPANLSPGTPAGPTSSRPRAAAAAAAAASGAGPLPARPPGRSESRQPHRLNCFLL

SEQ ID NO: 1850 - protein, 43 aa, Homo sapiens
MPSPSSPPTMLKPRPVEPLCRMILRGSLSPGTPAGPTSSRPRA

SEQ ID NO: 1851 - protein, 42 aa, Homo sapiens
MPSPSSPPTMLKPRPVEPLCRMILRGSLVKSSSASMCLGIGE

SEQ ID NO: 1852 - protein, 28 aa, Homo sapiens
MPSQFFCIFSRDGVSSCWPGWSQTPDLR

SEQ ID NO: 1853 - protein, 12 aa, Homo sapiens
MPSSLSLIISSF

SEQ ID NO: 1854 - protein, 38 aa, Homo sapiens
MPSTMRLVPKVLGTQILSERRNSLENLGHSAWLLTTTQ

SEQ ID NO: 1855 - protein, 15 aa, Homo sapiens
MPTGSIFQSWMMNVT

SEQ ID NO: 1856 - protein, 169 aa, Homo sapiens
MPTQILSTAGFRFLLYIFVNSLISKMSFWPPPSRILCLSRLTSSSSSFRGDSFAFTGLGLMKNLYWIRTVMRKNTTPSTAMAKRFRPTKSQDNGDTKRFSPNLSRASAIAWFFTMSMSPRPRQKCGKIKNTDFRISLILFSLLSVNSSSTKVATLPLMPMKRFTLVSTT

SEQ ID NO: 1857 - protein, 77 aa, Homo sapiens
MPVIPALWEAEVGGLPEVRSSRPACPSWQNPISTKNTKLRWAWWCMPVVPATGEAEAGELLDTYNPSTLGGQGRRTA

SEQ ID NO: 1858 - protein, 22 aa, Homo sapiens
MPVYNSVSKIKNLKIKSQVEEK

SEQ ID NO: 1859 - protein, 18 aa, Homo sapiens
MQACAKWGMCLAGLLGQD

SEQ ID NO: 1860 - protein, 26 aa, Homo sapiens
MQASSLTGHATPSRLLTSLCLSFPHL

SEQ ID NO: 1861 - protein, 22 aa, Homo sapiens
MQCPVPLETQGSPEACHQDTAQ

SEQ ID NO: 1862 - protein, 82 aa, Homo sapiens
MQEAGLPTSNSSLHLNSAMVRLRLYRFSERKVLRELLMKTVTVGADTPVTSILPRPADACSAVQPPHTRSAAAAAAAAAGLS

SEQ ID NO: 1863 - protein, 209 aa, Homo sapiens
MQEAGLPTSNSSLHLNSAMVRLRLYRFSERKVLRELLMKTVTVGADTPVTSILPRPADACSAVQPPHTRSAAAAAAAAAGLSAPPPAPCLTNPRSPARSVRQSPPSLPHRQEEGSPYSWASPANPEGPSIVHGSSNSGPGKDQNRRRRLKPGGRSGKSSPSPRRVNSRMRTGLQPSQAPWLLSWMLSVLRFTMRIVFPALAPDPYYSVN

SEQ ID NO: 1864 - protein, 66 aa, Homo sapiens
MQEAGLPTSNSSLQGPQSSPSPLAPALWTVGFFAGPGPHLCTLEFSPDPPRRDRVPSLRSLGSPPG

SEQ ID NO: 1865 - protein, 25 aa, Homo sapiens
MQETQYNGCLKNDFKESEADSSRPC

SEQ ID NO: 1866 - protein, 56 aa, Homo sapiens
MQGTRWSHGTPKSWWRAGNLSRHSARQFPSPPPPPPPPLPPLHHLPGSLAGVAPVP

SEQ ID NO: 1867 - protein, 23 aa, Homo sapiens
MQGVIVCFLGITILKGSSWTVKK

SEQ ID NO: 1868 - protein, 19 aa, Homo sapiens
MQIKTTMKCHLTPTMMAAI

SEQ ID NO: 1869 - protein, 38 aa, Homo sapiens
MQKLLAALPQNLVALPDGISELLILLQAALEGLRSALF

SEQ ID NO: 1870 - protein, 29 aa, Homo sapiens
MQKRGNKKCWQVCREKGTFVPCWWECRLA

SEQ ID NO: 1871 - protein, 31 aa, Homo sapiens
MQKYPVHRKRKIEVNVRLAKGLVTGLTQFIE

SEQ ID NO: 1872 - protein, 38 aa, Homo sapiens
MQLSQKRCPHSVCFGLHSTRWHFSHLYLSSTVFTNFSL

SEQ ID NO: 1873 - protein, 31 aa, Homo sapiens
MQPDATGSPRDRSGDRLHLTQRSYLPVQRSV

SEQ ID NO: 1874 - protein, 40 aa, Homo sapiens
MQPDATGSPRDRSGDRLHLTQRSYLPVQRSVSSLHRNLWS

SEQ ID NO: 1875 - protein, 39 aa, Homo sapiens
MQPDATGSPRDRSGDRLHLTQRSYLPVQRSVSVRNQANE

SEQ ID NO: 1876 - protein, 246 aa, Homo sapiens
MQPHGDVLRDLDILLQTTDKLAVHLAGLGGTETAALGFAQPVLQDAAGLAGLVQLLSQLLQLIHVLLHIDVPHLQHLGPQLLNLVLEIVVLRAQLLQLPHQAAGPAVQHLLGEVGEGKRGAERQAAAAHRRRGHRRLVRGGGRPRGLLRGGRGLGRLPRTDPRRAPGRGLGVAAQRQLQAQQARLLRRAVRHLRAAIREAGGRRWRSRPRTRARTALGTDPGADPGHPHTRTARPGSHCAPLLVRP

SEQ ID NO: 1877 - protein, 16 aa, Homo sapiens
MQPLGRHELGSGCPQP

SEQ ID NO: 1878 - protein, 29 aa, Homo sapiens
MQPPCPMQGVIVCFLGITILKGSSWTVKK

SEQ ID NO: 1879 - protein, 46 aa, Homo sapiens
MQPVSLLKYSKSHLYSSTKQVPHRYLRPTQPGFHVPIIISILVKAI

SEQ ID NO: 1880 - protein, 62 aa, Homo sapiens
MQQATCTLRVRALQPVCVQLLNPRRVLGRLSPDHAVQSLHVLEELSAGPVWGLELAPAVQAA

SEQ ID NO: 1881 - protein, 24 aa, Homo sapiens
MQQVMCSQSVRAAALSSRGLTAHC

SEQ ID NO: 1882 - protein, 23 aa, Homo sapiens
MQQWRKIPPKTRKVPLQPRFSRR

SEQ ID NO: 1883 - protein, 33 aa, Homo sapiens
MQRKGNFCTLLVGMQVSITTVENSLEAPQNTKN

SEQ ID NO: 1884 - protein, 73 aa, Homo sapiens
MQRQRVERLAGLEVSMWVSVLVKGSRGEGQAGYQLRTVDGTDSPGAHRSSSGTRSERDAISAAATRSTRRASV

SEQ ID NO: 1885 - protein, 32 aa, Homo sapiens
MQSSGWEVEVSLSCSLEFLCWQICPAYHPSVS

SEQ ID NO: 1886 - protein, 126 aa, Homo sapiens
MQSSGWEVEVSLSCSLEFLCWQICPETWGASPQAPRGHWAAEGVGGPSCAASCFPGSRGERLRKGRESQRLSLGPGGAAAAGAVPSFPAAPGTGKKVATQQAASWKLRDRQQVLLPGSATQTVSTA

SEQ ID NO: 1887 - protein, 12 aa, Homo sapiens
MQTLLKATERSW

SEQ ID NO: 1888 - protein, 86 aa, Homo sapiens [sequence omitted]

SEQ ID NO: 1889 - protein, 91 aa, Homo sapiens
MQVWHGFDPGAMFGNWFPAIGGFKTLIIGVIIVIGTCLLLPCLLPVLLQMIKSFIITLVHQNASAQVYYMNHYQSIAREDISSENESENSH

SEQ ID NO: 1890 - protein, 21 aa, Homo sapiens
MQYLINVVSDIAYQPQSLGSM

SEQ ID NO: 1891 - protein, 28 aa, Homo sapiens
MQYLINVVSDIAYQPQSLGSNLSRAAPQ

SEQ ID NO: 1892 - protein, 21 aa, Homo sapiens
MQYLINVVSDIAYQPQSLGST

SEQ ID NO: 1893 - protein, 23 aa, Homo sapiens
MQYLINVVSDIAYQPQSLGSTEP

SEQ ID NO: 1894 - protein, 43 aa, Homo sapiens
MQYLINVVSDIAYQPQSLGSTVGKDWAASLVDQTGVTLQERAN

SEQ ID NO: 1895 - protein, 84 aa, Homo sapiens [sequence omitted]

SEQ ID NO: 1896 - protein, 49 aa, Homo sapiens
MRCFTDAFCKILQQTIKYFQEILNRFFISFHYIFSCYVRQADLQVVQGQ

SEQ ID NO: 1897 - protein, 47 aa, Homo sapiens
MRCFTDAFCKILQQTIKYFQEILNRFFISFHYIFSWRQNIELLCETS

SEQ ID NO: 1898 - protein, 13 aa, Homo sapiens
MRCSFKMESTVSL

SEQ ID NO: 1899 - protein, 56 aa, Homo sapiens
MRDSGPQPPRYITPKSPTDTDCERVNVRCFKPLRVGDLLRQQRMNTLQILLMSHFK

SEQ ID NO: 1900 - protein, 64 aa, Homo sapiens
MRERSAWSTRFEFALYSYCRLRAVTSAMAAAARRLQTTTPPYRKLQTAADLCSRRAGTTQERRT

SEQ ID NO: 1901 - protein, 24 aa, Homo sapiens
MRFHHVGQAGLELLASSDPSASAS

SEQ ID NO: 1902 - protein, 171 aa, Homo sapiens
MRFTPQNEDFCHHAEELVRISIRTFQPVRSVVVHVADQHGVEGIEISAEDRELVQDEEFCLLGVPFAIGFQLLLLLHRLDSLFLQLLQSWDEVASQQVGPGFADDGLCIHCNALHPGGLIDAQVVVDDFQNVAQDETEVFRGDLGAAWPCAGGQVLRTPLPPVGQVVAEHG

SEQ ID NO: 1903 - protein, 52 aa, Homo sapiens
MRGGPEHPKRQQRPGPGPGHRYAPRGKRRRDGSPGPLPGRSRRQGRGGRSPS

SEQ ID NO: 1904 - protein, 91 aa, Homo sapiens
MRGGPEHPKRQQRPGPGPGHRYAPRGKRRRDGSPGPLPGRSRRQGRGGRSPSLHAGPRVWGPPLLGGHLWSGTLGGTEGRGTRRRMRHDLF

SEQ ID NO: 1905 - protein, 27 aa, Homo sapiens
MRGLWSSTPSRAAFIMSSRWASDALSL

SEQ ID NO: 1906 - protein, 11 aa, Homo sapiens
MRHHSRLILYF

SEQ ID NO: 1907 - protein, 27 aa, Homo sapiens
MRHHTWLIFVFSVEKGFTMLARLVVNS

SEQ ID NO: 1908 - protein, 29 aa, Homo sapiens
MRKELLLAPFYRRGNRHREIKQFAQDQDV

SEQ ID NO: 1909 - protein, 11 aa, Homo sapiens
MRKKLFFVFKK

SEQ ID NO: 1910 - protein, 24 aa, Homo sapiens
MRKLSCSTLYSLPAPKNAWHMVNP

SEQ ID NO: 1911 - protein, 22 aa, Homo sapiens
MRKSWSESASGLFSQLDLLLST

SEQ ID NO: 1912 - protein, 69 aa, Homo sapiens
MRLASSRKRFVCSCSRRSIVCFCCFSRFSISWSYCRFLLIISCSKRRKICSRCCCSLLLSCCWALCSSF

SEQ ID NO: 1913 - protein, 32 aa, Homo sapiens
MRLSEPLFFLCLLLPYPRLEGKYLFLSPFPDH

SEQ ID NO: 1914 - protein, 34 aa, Homo sapiens
MRLVPKVLGTQILSERRNSLENLGHSAWLLTTTQ

SEQ ID NO: 1915 - protein, 24 aa, Homo sapiens
MRMFRMMSLWVESFKCPIRKGIHF

SEQ ID NO: 1916 - protein, 35 aa, Homo sapiens
MRNSFSSLWLAWKCRSSSQRSRRIWLLCRMASRSS

SEQ ID NO: 1917 - protein, 22 aa, Homo sapiens
MRPCPQTRKKCPAGAACTAEVT

SEQ ID NO: 1918 - protein, 74 aa, Homo sapiens [sequence omitted]

SEQ ID NO: 1919 - protein, 15 aa, Homo sapiens
MRPTKVPCSASSGTE

SEQ ID NO: 1920 - protein, 17 aa, Homo sapiens
MRQEDCLIPGAPGYNVL

SEQ ID NO: 1921 - protein, 17 aa, Homo sapiens
MRRGFVFVQQIPPRQDF

SEQ ID NO: 1922 - protein, 18 aa, Homo sapiens
MRRHGGGSLRSGDLRRKE

SEQ ID NO: 1923 - protein, 31 aa, Homo sapiens
MRRKWNPQTHAGGNAKCCSHFGKQPGSSSKG

SEQ ID NO: 1924 - protein, 14 aa, Homo sapiens
MRRQPGMFGKENKG

SEQ ID NO: 1925 - protein, 26 aa, Homo sapiens
MRRRFRSFSREPESRRTPRSRRIMRL

SEQ ID NO: 1926 - protein, 14 aa, Homo sapiens
MRRRTVPRSSLLTH

SEQ ID NO: 1927 - protein, 76 aa, Homo sapiens
MRRSRTRSLSADKPVESAILERVPEAPGFQFRLLTRQPCDLGQLNVRMLGSVFSIGLMSVRGSRKGGWPAGNLRSM

SEQ ID NO: 1928 - protein, 135 aa, Homo sapiens
MRRSWASRWCCCCRVRPALAIRWIKVSVILSRTRWIWSFSSRDFRVLDRNVYTPELSKIIDLRHTNSSPCRFIMRNRDDVASSMSKISTMPSTHFPWFLSKSKLGANSSFPGCSMERQTRPIIRISSQAHSRRWT

SEQ ID NO: 1929 - protein, 31 aa, Homo sapiens
MRRVIISTYRLKNVKKKSKGKEQCLRPSCIQ

SEQ ID NO: 1930 - protein, 215 aa, Homo sapiens
MRSLSAFFTADRSSSLERRRASRSLAPSPRLRRSSPASWRCTSRPSWLSRSLRWASSSSRRSPSRASSSRRSWVRSSSASRRQESRCLPRSRACSCSLLTSWAWAAAASSRWARRSRSSDVRAFTVLRSCSCRLWASRFCRSISREMVARLCRVPINFSDSAVFSDSFRDKACCFSLSARRRPSSRSCCRAAISSLSSSFSASSRASSSSCSRCS

SEQ ID NO: 1931 - protein, 34 aa, Homo sapiens
MRSVRYSNKPSNISRRFLIDSLSPFTIFSPGDRI

SEQ ID NO: 1932 - protein, 32 aa, Homo sapiens
MRSVRYSNKPSNISRRFLIDSLSPFTIFSPVM

SEQ ID NO: 1933 - protein, 162 aa, Homo sapiens [sequence omitted]

SEQ ID NO: 1934 - protein, 140 aa, Homo sapiens
MRVGRLPSWLQDASRKEMFTSQWVWTLLFMIRMCGPSSCFKPGRRPQVGPLPSLSPSLAEKLGVRSFFRFRAAGRATVLLSASRPRFTGEDIRQPGQSQIGGCTCRIPLDISVFRLFPRPDFPARFPSHPRERRRDLLGS

SEQ ID NO: 1935 - protein, 63 aa, Homo sapiens
MRVTAIKHGGLLFLPTQLTHLMPPQPSRPNAQFCLCVCNNNPSIYDKLSDSFLKTGFLRLSTL

SEQ ID NO: 1936 - protein, 28 aa, Homo sapiens
MRWPSSVLVRRKRRRTLVALVNSRSSGE

SEQ ID NO: 1937 - protein, 12 aa, Homo sapiens
MRYHARLIFVFY

SEQ ID NO: 1938 - protein, 21 aa, Homo sapiens
MRYHLTPVRMVIIKKSGNNKC

SEQ ID NO: 1939 - protein, 24 aa, Homo sapiens
MSAFIGSLPGFNFVRIPYIGVQMF

SEQ ID NO: 1940 - protein, 15 aa, Homo sapiens
MSCIWIQSHTNLMTP

SEQ ID NO: 1941 - protein, 12 aa, Homo sapiens
MSCPCHPWFLGT

SEQ ID NO: 1942 - protein, 28 aa, Homo sapiens
MSDGLLPKMCLLVYKLPLKQVFTFPVFP

SEQ ID NO: 1943 - protein, 32 aa, Homo sapiens
MSDPGRLTTMKNFSRGGISTVGAWQGVTDPWF

SEQ ID NO: 1944 - protein, 15 aa, Homo sapiens
MSEMQTLLKATERSW

SEQ ID NO: 1945 - protein, 41 aa, Homo sapiens
MSENIYTLRKIHTQRIKQLSHLLLTSDPQFRVNHSNTELLY

SEQ ID NO: 1946 - protein, 11 aa, Homo sapiens
MSESRTLKTKN

SEQ ID NO: 1947 - protein, 17 aa, Homo sapiens
MSFCGKLACKIVLDSFN

SEQ ID NO: 1948 - protein, 56 aa, Homo sapiens
MSFKGSTTSHFGSDRKNMETCCKAISCGTAGSGSPRWLLSAAPCRPAAPCRLAASP

SEQ ID NO: 1949 - protein, 27 aa, Homo sapiens
MSFKGSTTSHFGSDRKNMETCCKAISV

SEQ ID NO: 1950 - protein, 30 aa, Homo sapiens
MSFKGSTTSHFGSDRKNMETCCKAISVSCC

SEQ ID NO: 1951 - protein, 11 aa, Homo sapiens
MSFNVGKYLYT

SEQ ID NO: 1952 - protein, 27 aa, Homo sapiens
MSFRDLFRFSCSPSSMAYRPGLFMTSS

SEQ ID NO: 1953 - protein, 144 aa, Homo sapiens
MSFWPPPSRILCLSRLTSSSSSFRGDSFAFTGLGLMKNLYWIRTVMRKNTTPSTAMAKRFRPTKSQDNGDTKRFSPNLSRASAIAWFFTMSMSPRPRQKCGKIKNTDFRISLILFSLLSVNSSSTKVATLPLMPMKRFTLVSTT

SEQ ID NO: 1954 - protein, 13 aa, Homo sapiens
MSGAATGLPRVPY

SEQ ID NO: 1955 - protein, 57 aa, Homo sapiens
MSGFVAGEAITALGHVAVTEPSGVIDLVGSHVLSLRPLPKLGRCLKLPVVKAEQEHL

SEQ ID NO: 1956 - protein, 68 aa, Homo sapiens
MSGGWSGTMEALLCFLSQSQHRRQIAVFRTCLLLQQQAGWPGCRPPCPGGRLWASPYTAAPAPDPSPP

SEQ ID NO: 1957 - protein, 76 aa, Homo sapiens
MSGHPSSDGGGAAPPGLRLQCPPRGPGAARAGRPTPTRLPGSAAGAGWAGERSRGGGGGGGGEAARGGNGAGPGRG

SEQ ID NO: 1958 - protein, 38 aa, Homo sapiens
MSGKLCVPFSHGTFLKCYRAAEPPTMSGAATGLPRVPY

SEQ ID NO: 1959 - protein, 28 aa, Homo sapiens
MSGVTLKFNDEVSKVFLNPSPSTACSGG

SEQ ID NO: 1960 - protein, 71 aa, Homo sapiens
MSGVTLKFNDEVSKVFLNPSPSTYSMLWGLSRELSQLCSHVFFTITKGIEKAVRAILPKIWSTAIRHFSFV

SEQ ID NO: 1961 - protein, 19 aa, Homo sapiens
MSHFLSKSWLRYQSRFLWN

SEQ ID NO: 1962 - protein, 24 aa, Homo sapiens
MSHQLEWRSLKSEETTDAGEDVEK

SEQ ID NO: 1963 - protein, 157 aa, Homo sapiens
MSIIKKSGNNRCWRGCGEIGTLLHWWWDCKLVQPLWKTVWRFLRDLELEIPFDPAIPLLGIYPKDYKSCCYKDTCTRIFIVALFTIAKTWNQPKCPSMIDWFKKMWHIYTMEYYAAIKKEEFMSFIGTWMKLETILLSKLFQGQKNKHRMFSLIDGN

SEQ ID NO: 1964 - protein, 19 aa, Homo sapiens
MSINLGRAPDMGSFQPLFL

SEQ ID NO: 1965 - protein, 23 aa, Homo sapiens
MSKNIRNIKEKKESGESYRELAI

SEQ ID NO: 1966 - protein, 76 aa, Homo sapiens
MSKTPKAMATEAKIDKWDLIKLKSFCTAKETTIRVNRQPTKWEKIFAIYSSDKGLISRIYKELKQTYKKKTNPIKK

SEQ ID NO: 1967 - protein, 41 aa, Homo sapiens
MSKTPKAMATKAKIDKWDLIKLKSFCTAKETTIRVNRQHTE

SEQ ID NO: 1968 - protein, 43 aa, Homo sapiens
MSKYVDKLPSHIPSLCWQIHFISMLNPTSSGKDSKTILREGNG

SEQ ID NO: 1969 - protein, 93 aa, Homo sapiens
MSLGVVGELSFLPMLGLDSKRDSQELNWVFDFSGSRVVPPTPSEEMHLRLVDLKRPPAAPSISRGDFAPTLSERFPSSLPALPLLSVEAPVVW

SEQ ID NO: 1970 - protein, 18 aa, Homo sapiens
MSLNVVKAIYKAETVGSW

SEQ ID NO: 1971 - protein, 19 aa, Homo sapiens
MSLPLVNYHLTWTTDSLWF

SEQ ID NO: 1972 - protein, 35 aa, Homo sapiens
MSLPTIAMVVSGWVMICGFRKSSHTKLSGGTEKML

SEQ ID NO: 1973 - protein, 15 aa, Homo sapiens
MSLQYVLVKLSEHLD

SEQ ID NO: 1974 - protein, 19 aa, Homo sapiens
MSLSEHTLLSYRQSVQKLV

SEQ ID NO: 1975 - protein, 129 aa, Homo sapiens
MSLTIILAIFQASSSWASSVFPCTHFFIACENMDPFDFLTSGSGSDSRMNCPKSLTLPNVIFLRRRAVRTPWVRLIRRANRARSSQRHVPAQKFISSNRMDEIIQIFIIKIAGQKARQKDLLHGCPGLT

SEQ ID NO: 1976 - protein, 67 aa, Homo sapiens
MSLTIILAIFQASSSWASSVFPCTHFFIACENMDPFDFLTSGSGSDSRMNCPKSLTLPNVIFPAYVR

SEQ ID NO: 1977 - protein, 18 aa, Homo sapiens
MSLWVESFKCPIRKGIHF

SEQ ID NO: 1978 - protein, 21 aa, Homo sapiens
MSMSLSEHTLLSYRQSVQKLV

SEQ ID NO: 1979 - protein, 12 aa, Homo sapiens
MSNNLRITQRLK

SEQ ID NO: 1980 - protein, 13 aa, Homo sapiens
MSNSFTMLWSSPS

SEQ ID NO: 1981 - protein, 152 aa, Homo sapiens
MSPCKEKDNENCVQRGSGLEIRGCGSWNILGHRRESRVNLLPSLLGLPCLGKGEEMEGRRWDGWCWHDRLEPLAARHTLSVRKHRLCMCDSLEEGIQSYLWGSGLERVSSGLDRPCDCLTPDTRSSRWTLTKPLPGSETSRDHGSQHCRWPP

SEQ ID NO: 1982 - protein, 83 aa, Homo sapiens
MSPDQEPVSEARAECGTQAPHPCYCRHLSLRMSVFHLGHPTASSLQAETGRMRGWDGEEEERERSGEEVWRDQERGWVRKDGR

SEQ ID NO: 1983 - protein, 75 aa, Homo sapiens
MSPHLANLCIFSRDGVSPWAQASLKLLTSKDPPSSASHSAGITSVSHHSWLQVLKMSATFLGWVYTQVASPPWHY

SEQ ID NO: 1984 - protein, 34 aa, Homo sapiens
MSPHTHYDGCNLKKAENNKCWGGCGNLGTLVHSW

SEQ ID NO: 1985 - protein, 89 aa, Homo sapiens [sequence omitted]

SEQ ID NO: 1986 - protein, 17 aa, Homo sapiens
MSQCHGLKWLQFYKFYL

SEQ ID NO: 1987 - protein, 15 aa, Homo sapiens
MSRILYIARCQGSCL

SEQ ID NO: 1988 - protein, 26 aa, Homo sapiens
MSRKKFSTVIDTKALTRTMMSIVTRH

SEQ ID NO: 1989 - protein, 33 aa, Homo sapiens
MSRMGLFLVCELMKTSIFLTHFPCHSLPCGFFI

SEQ ID NO: 1990 - protein, 57 aa, Homo sapiens
MSRSHTSARSSCSRATVGLLSSQQSSLSSGMKGHQMILRKWFSGVPSGCRIWTKISS

SEQ ID NO: 1991 - protein, 86 aa, Homo sapiens
MSRSMKAFTLSTRSCPIAPVSRAKSRNLSRRRVTWSKSCPISGEEATSSFSEIHCSRSSVSRLSWNRWYMFSSLRLRSSATSFSPA

SEQ ID NO: 1992 - protein, 64 aa, Homo sapiens
MSRWELAMSRSASGLAGTFSRSPAPPGLISKRCFPGSSGPGGSSVTCVPCREINPWGLISSLSL

SEQ ID NO: 1993 - protein, 11 aa, Homo sapiens
MSSARTGWMWS

SEQ ID NO: 1994 - protein, 48 aa, Homo sapiens [sequence omitted]

SEQ ID NO: 1995 - protein, 26 aa, Homo sapiens
MSSDPPISASQSAGIIGMSHCAQPKC

SEQ ID NO: 1996 - protein, 53 aa, Homo sapiens
MSSFSFLFLEKYSFSNKFSFAKLSCALCFSRSYALSTSLNSFLIISKSATASA

SEQ ID NO: 1997 - protein, 21 aa, Homo sapiens
MSSGISSLSMSSSLSSANCGS

SEQ ID NO: 1998 - protein, 47 aa, Homo sapiens
MSSILLSASREREVISVSRLQGATTKPRSIFPTLQISYRPSILSSMG

SEQ ID NO: 1999 - protein, 25 aa, Homo sapiens
MSSMIQKRFLAPEAVGIEMVFPAAS

SEQ ID NO: 2000 - protein, 53 aa, Homo sapiens
MSSMIQKRFLAPEAVGIEMVFPAAVLSLPTGVLEQLRSMVDDSEDMAPGLQPV

SEQ ID NO: 2001 - protein, 21 aa, Homo sapiens
MSSNFPMNFSIAPHMGLVIKL

SEQ ID NO: 2002 - protein, 44 aa, Homo sapiens
MSSPQPPDHHKPCHLPGPPAQDLSLQILSGYWFLQLLHFYFSST

SEQ ID NO: 2003 - protein, 76 aa, Homo sapiens
MSSPWASSSGSFTSNSFWVLVPSVATFLLFFNLIFFFGELDFPSSSSSSSETACAFLLGASFEKRLEGFLAGETNW

SEQ ID NO: 2004 - protein, 142 aa, Homo sapiens
MSSRKSLSSLKSIASKKSGSSRKSVSSSKSTSSNKAMSSRLSMSSRKSLSSLKSIASEKSRSSRKSVSSSKSTSSNKAMSSIKLMSSSLLVSSNKGTSSNKGTSSNKGMSSNKGTSSRKSTSSNQAMSSRKSTSSRKYMSSN

SEQ ID NO: 2005 - protein, 28 aa, Homo sapiens
MSSRKSTSSNGLQVFQTIHVFQKILVFP

SEQ ID NO: 2006 - protein, 63 aa, Homo sapiens [sequence omitted]

SEQ ID NO: 2007 - protein, 12 aa, Homo sapiens
MSSSLSSANCGS

SEQ ID NO: 2008 - protein, 180 aa, Homo sapiens
MSTTRWAEAPRPDACSSCRKRHARSPVAARGSPSSSQASCDSAVPPHAYRSARASCTSRKSILRRLGPAQGPPPPHRRHSTVVLPATATTRMTPRNTRRTRRLGGPEAGAPCPKVRLRPQPSKMGTEMLGAGGRIEGLKRSSILVPEEEEAPKRAGRTRETKVEARRRGERRWVYTSSQS

SEQ ID NO: 2009 - protein, 13 aa, Homo sapiens
MSVKHIYTILGIL

SEQ ID NO: 2010 - protein, 30 aa, Homo sapiens
MSVSIQFLNCMFAINSLYITWNLLNINSCH

SEQ ID NO: 2011 - protein, 91 aa, Homo sapiens
MSWGRGVPSPRAQSCHHSPPPTWVGAGRALLGTNPKTMRSGPGWSPGSRHPLCQGEKLGPHVRLEGGSPGGEKEQEGTGPSLEGPRTQAAP

SEQ ID NO: 2012 - protein, 26 aa, Homo sapiens
MSWHFHGGRRPFKKTGQARSFRVGYE

SEQ ID NO: 2013 - protein, 34 aa, Homo sapiens
MSWLSCQNIWTSRICFFVRGRGIRQAVELKPDVG

SEQ ID NO: 2014 - protein, 11 aa, Homo sapiens
MSYLKQCNSLS

SEQ ID NO: 2015 - protein, 18 aa, Homo sapiens
MSYRPLKEVLSPPSPYFA

SEQ ID NO: 2016 - protein, 21 aa, Homo sapiens
MTAPKTSHPVGWLSNSSDHCS

SEQ ID NO: 2017 - protein, 12 aa, Homo sapiens
MTCIWYKGKNSS

SEQ ID NO: 2018 - protein, 14 aa, Homo sapiens
MTDGGIRPAGLRGA

SEQ ID NO: 2019 - protein, 16 aa, Homo sapiens
MTDGGIRPAGLRGACE

SEQ ID NO: 2020 - protein, 53 aa, Homo sapiens
MTDWAKLLLAGPSGEEIVDDRGVPVQDDWSIAPDDDKVRFSLSGVTPHSSPRC

SEQ ID NO: 2021 - protein, 12 aa, Homo sapiens
MTELIFSPSLTH

SEQ ID NO: 2022 - protein, 13 aa, Homo sapiens
MTELTSGNCKFVS

SEQ ID NO: 2023 - protein, 61 aa, Homo sapiens
MTFLFTVFDLKSILSHVSIVISALFWLPFVCNIFLHTFTFGLSLQVRFLVGSIQSSHDGGF

SEQ ID NO: 2024 - protein, 15 aa, Homo sapiens
MTFLIFNEGLLREII

SEQ ID NO: 2025 - protein, 26 aa, Homo sapiens
MTFPMRPCPQTRKKCPAGAACTAEVT

SEQ ID NO: 2026 - protein, 24 aa, Homo sapiens
MTFSTSSFCASPSISLVHLIVAVS

SEQ ID NO: 2027 - protein, 24 aa, Homo sapiens
MTFTFYEREGVSPSLPISWVIVQQ

SEQ ID NO: 2028 - protein, 187 aa, Homo sapiens
MTFYHNEALLDLANIHRPGTVAGAEHVQVPHLSPVFMQQGHCWAALLTAVFALLRDEGAPDDPAKVVQWRALWLPNMDQDLFLNFAINQSQAPHEQVACLIQAGQLWRVEVRESQISHTACEALEQGPLRSADADHPHHGRAIVGSPNGIGQEGVRHSNQVAIVVLLFPVILGDRLNFHLVASPGLA

SEQ ID NO: 2029 - protein, 31 aa, Homo sapiens
MTGVQTLCDTLWRRVNDFSLQNVESEISTSS

SEQ ID NO: 2030 - protein, 53 aa, Homo sapiens
MTGVQTLCDTTQWRCRGWCHLCSLNPRRCPCRSSHTGRTCRGPGDHSSAEPGA

SEQ ID NO: 2031 - protein, 16 aa, Homo sapiens
MTIFVTLRNVALTFFL

SEQ ID NO: 2032 - protein, 41 aa, Homo sapiens
MTIGTNCWPLLSTSSEVSVVKFIRTVFTHYSKGKIKVSRRV

SEQ ID NO: 2033 - protein, 20 aa, Homo sapiens
MTILSHSVLPCLPPSLFLSS

SEQ ID NO: 2034 - protein, 20 aa, Homo sapiens
MTIVFFRHNAIAPLIDYSIV

SEQ ID NO: 2035 - protein, 30 aa, Homo sapiens
MTKVKAGGILNTWRGGQFPFLLLKSKKITI

SEQ ID NO: 2036 - protein, 19 aa, Homo sapiens
MTLKREVMPFSFVGWKDCL

SEQ ID NO: 2037 - protein, 40 aa, Homo sapiens [sequence omitted]

SEQ ID NO: 2038 - protein, 43 aa, Homo sapiens
MTMALRGTDAKPGTGLPSSWNLPVRPRTSVQLEWAPQKEKQYS

SEQ ID NO: 2039 - protein, 42 aa, Homo sapiens
MTNSLWSTVFLKKETASWLQVFPKGQISARVHFTANIGSCLN

SEQ ID NO: 2040 - protein, 59 aa, Homo sapiens
MTPATVPLQAQYGERSSNRRSKPALTNAAQRCSWVRMFSTLRGASGGRLEVWGDSGFSS

SEQ ID NO: 2041 - protein, 55 aa, Homo sapiens
MTPMAQQSTGRPYRCRPTTSGARYSGVPQGSLMRPFSSLARWKSLMTIFEFFSRL

SEQ ID NO: 2042 - protein, 71 aa, Homo sapiens
MTQDTRQLLVNSGLCQRSITQAILHPRLSYSLLWSLSITSLPSTSWVSIAPPPPVIIPFHHLPNLAASTYP

SEQ ID NO: 2043 - protein, 42 aa, Homo sapiens
MTQNGQLLNCSQTFQVIRNMFIFVFRDRVSLCTQTGVQWHNH

SEQ ID NO: 2044 - protein, 29 aa, Homo sapiens
MTRKQMVIVWSIRNKASPQELNGKLLVML

SEQ ID NO: 2045 - protein, 41 aa, Homo sapiens
MTRKQMVIVWSIRNKASPQELQSQELGGRKAGLNGKLLVML

SEQ ID NO: 2046 - protein, 26 aa, Homo sapiens
MTRMAMSSGISSLSMSSSLSSANCGS

SEQ ID NO: 2047 - protein, 39 aa, Homo sapiens
MTRPSGSLAVPSWESEGKPDRPPQGMGEVHRPGGTCSHF

SEQ ID NO: 2048 - protein, 43 aa, Homo sapiens
MTRPSGSLAVPSWESEGKPDRPPQGMGEVHRPGGTCSSSLSSS

SEQ ID NO: 2049 - protein, 75 aa, Homo sapiens
MTRRMACTQSSMSRWELAMSRSASGLAGTFSRSPAPPGLISKRCFPGSSGPGGSSVTCVPCREINPWGLISSLSL

SEQ ID NO: 2050 - protein, 67 aa, Homo sapiens
MTRTLCTTGLRTQHMDMFWKPVPFSQLSKTGIVQGPYTELLTERESSTRRAGAPQPSTPSLNTYLRM

SEQ ID NO: 2051 - protein, 49 aa, Homo sapiens
MTRTPKAMAIKAKTDKWDLIKELLHGKRNYDQSEQATYRMGETFCNLSI

SEQ ID NO: 2052 - protein, 27 aa, Homo sapiens
MTSAFKMLSLKYQHHLEVEQVDKGGEV

SEQ ID NO: 2053 - protein, 67 aa, Homo sapiens
MTSAGCGIRRIISTAFSPACLGAAFSPACLGATFSPACLGAPWGQEPCPLLLHLVRAQFGIWPQYSC

SEQ ID NO: 2054 - protein, 36 aa, Homo sapiens
MTSKHMKRCSASLLIREMQIKTTMKCHLTPTMMAAI

SEQ ID NO: 2055 - protein, 82 aa, Homo sapiens
MTSNISSPSPSVMLYSISAFSPTSASLALILPIGVPGGEDSGVLNWYVLWGNRGGLSLTSVSVMFTVVVPDNPPIWPPISLA

SEQ ID NO: 2056 - protein, 13 aa, Homo sapiens
MTSQSSSLTTKEV

SEQ ID NO: 2057 - protein, 31 aa, Homo sapiens
MTSTEMDIFLSEVDTPSRNGIPVASLLPLIL

SEQ ID NO: 2058 - protein, 21 aa, Homo sapiens
MTSTGTMKEKRKMQMANTGPQ

SEQ ID NO: 2059 - protein, 35 aa, Homo sapiens
MTTHCILFLYCNLEGSGKFQKVLKGSHPVKCCTPM

SEQ ID NO: 2060 - protein, 17 aa, Homo sapiens
MTTLQHRPLHLSGWGPP

SEQ ID NO: 2061 - protein, 18 aa, Homo sapiens
MTTSMDSKEEGILSALCS

SEQ ID NO: 2062 - protein, 11 aa, Homo sapiens
MTVAMGTEPVV

SEQ ID NO: 2063 - protein, 53 aa, Homo sapiens
MTVSSSKRKCLLMSENIYTLRKIHTQRIKQLSHLLLTSDPQFRVNHSNTELLY

SEQ ID NO: 2064 - protein, 33 aa, Homo sapiens
MTVSVKMLACMVRKSRPKSTRQPTSPKCHSLVT

SEQ ID NO: 2065 - protein, 25 aa, Homo sapiens
MTYCILSAFHITHAAPTSSRLQALA

SEQ ID NO: 2066 - protein, 96 aa, Homo sapiens
MVAASLWPASMSRSMKAFTLSTRSCPIAPVSRAKSRNLSRRRVTWSKSCPISGEEATSSFSEIHCSRSSVSRLSWNRWYMFSSLRLRSSATSFSPA

SEQ ID NO: 2067 - protein, 29 aa, Homo sapiens
MVAGENKSCCLPLQFLKSNIRNISIEGHR

SEQ ID NO: 2068 - protein, 22 aa, Homo sapiens
MVDIMCPTPWMDRRTFLPPGSS

SEQ ID NO: 2069 - protein, 15 aa, Homo sapiens
MVDMRKVSVLLSSRQ

SEQ ID NO: 2070 - protein, 43 aa, Homo sapiens
MVDPPIILSSGGATGSWATLCLSSVILGKSARRRRELAAKPPE

SEQ ID NO: 2071 - protein, 43 aa, Homo sapiens
MVEVLSTGRIFIHHCPSGISLRGAIGVQLSLFVLCLHILQNPL

SEQ ID NO: 2072 - protein, 35 aa, Homo sapiens
MVFPAAVLSLPTGVLEQLRSMVDDSEDMAPGLQPV

SEQ ID NO: 2073 - protein, 36 aa, Homo sapiens
MVGFGSAIWANDLTSLNLSFCFYEVGIVIPTFFRLL

SEQ ID NO: 2074 - protein, 13 aa, Homo sapiens
MVGKLMGKSFARG

SEQ ID NO: 2075 - protein, 18 aa, Homo sapiens
MVGTTTVSDRLRTSDFRS

SEQ ID NO: 2076 - protein, 62 aa, Homo sapiens
MVGVVTSAVYLWSSTSLTDIPEISLANQELPGSGVHRWADCCLHYWLLGPRRLRVQVKSQER

SEQ ID NO: 2077 - protein, 81 aa, Homo sapiens
MVGVVTSAVYLWSSTSLTDIPEISLANQELPGSGVHRWADCCLHYWLLGPRRLRVQVKSQERRQFTSRPALKAACPPSLLP

SEQ ID NO: 2078 - protein, 23 aa, Homo sapiens
MVICFRTWTFLLFPAVSANSTAP

SEQ ID NO: 2079 - protein, 12 aa, Homo sapiens
MVIIKKSGNNKC

SEQ ID NO: 2080 - protein, 27 aa, Homo sapiens
MVILKEGAFLLSFLVPIVLFGNTLSGL

SEQ ID NO: 2081 - protein, 13 aa, Homo sapiens
MVISCPNRTFHYF

SEQ ID NO: 2082 - protein, 87 aa, Homo sapiens
MVITTIIAIIKLLIVTGCPTFLRFSSAICDSFLICPQVGGCVRWVLLVTVGVPLSVSLNMAATRGSSGSSQNLFLSIRLMIRFQVPR

SEQ ID NO: 2083 - protein, 24 aa, Homo sapiens
MVIVWSIRNKASPQELNGKLLVML

SEQ ID NO: 2084 - protein, 36 aa, Homo sapiens
MVIVWSIRNKASPQELQSQELGGRKAGLNGKLLVML

SEQ ID NO: 2085 - protein, 14 aa, Homo sapiens
MVKEQGDFPFLAGI

SEQ ID NO: 2086 - protein, 22 aa, Homo sapiens
MVKFQPRFSGCGTSSDSAVSLT

SEQ ID NO: 2087 - protein, 50 aa, Homo sapiens [sequence omitted]

SEQ ID NO: 2088 - protein, 45 aa, Homo sapiens [sequence omitted]

SEQ ID NO: 2089 - protein, 50 aa, Homo sapiens
MVLISWPRDPPASASQSAGITGVSHRAWPHFVFLLLFAYLYDVACVQSFD

SEQ ID NO: 2090 - protein, 24 aa, Homo sapiens
MVLLGSEDYLQVSSICSMGIHGSK

SEQ ID NO: 2091 - protein, 39 aa, Homo sapiens
MVLQALGVSSSWHRAAGRAKPEKPLWSSCSLCHHHHQPQ

SEQ ID NO: 2092 - protein, 27 aa, Homo sapiens
MVLRAWTYRSVLSWSLISPNRGRFQSR

SEQ ID NO: 2093 - protein, 57 aa, Homo sapiens
MVPTTCPVGSSLFMLNKHICWASWAFESVNLAAVQGAPEGYPWCMLETGGREIVAKM

SEQ ID NO: 2094 - protein, 31 aa, Homo sapiens
MVQYFKDGFHQAGSLVQVIFCVGNLFLKGTF

SEQ ID NO: 2095 - protein, 25 aa, Homo sapiens
MVRCLLKFLRNKTESFIFIHIFTIY

SEQ ID NO: 2096 - protein, 147 aa, Homo sapiens
MVRDNGGSFVFFITIAASSTDCSISYLSSVTAASWMARLSATLSRRAVVGFSLHSSTSSRSKSPLSRRPFATRPTRITPRRVLVMCSVFCSPAPSLLSSSGGTSMLSDSACSLLPFSCSSIQSDTALSARSVWDTMFWTASSSSCVG

SEQ ID NO: 2097 - protein, 23 aa, Homo sapiens
MVRKSRPKSTRQPTSPKCHSLVT

SEQ ID NO: 2098 - protein, 21 aa, Homo sapiens
MVRLPLASLMMTVAMGTEPVV

SEQ ID NO: 2099 - protein, 64 aa, Homo sapiens
MVRLRLYRFSERKVLRELLMKTVTVGADTPVTSILPRPADACSAVQPPHTRSAAAAAAAAAGLS

SEQ ID NO: 2100 - protein, 191 aa, Homo sapiens [sequence omitted]

SEQ ID NO: 2101 - protein, 47 aa, Homo sapiens
MVSHLLNFPVLFSLAFQNDAVSFEDRRGRHKGQRICLFSDCIKDDQQ

SEQ ID NO: 2102 - protein, 109 aa, Homo sapiens
MVSLLSSWFRPRIRSRRSIWTCRKGSLTPDMLCSVEYPIVTRVRRMCTSWGTTFRKCLRAAGLRSQSSVISVMVPSRMPGVSVGEVNGGGQGQESLLRVCLCVCTTLLL

SEQ ID NO: 2103 - protein, 80 aa, Homo sapiens
MVSLLSSWFRPRIRSRRSIWTCRKGSLTPDMLCSVEYPIVTRVRRMCTSWGTTFRKCLRAAGLRSQSSVISVMVPSRMPW

SEQ ID NO: 2104 - protein, 11 aa, Homo sapiens
MVSPCCCRGWS

SEQ ID NO: 2105 - protein, 83 aa, Homo sapiens [sequence omitted]

SEQ ID NO: 2106 - protein, 40 aa, Homo sapiens
MVSQALGVSSSSWHRAAGRAKPEKPLWSSCSLCHHHHQPQ

SEQ ID NO: 2107 - protein, 22 aa, Homo sapiens
MVSSPDLVIHLPRPPRVLGFQV

SEQ ID NO: 2108 - protein, 138 aa, Homo sapiens
MVSTVSNRTAFPAFRLVSVLVATWASKSFMVSLLSSWFRPRIRSRRSIWTCRKGSLTPDMLCSVEYPIVTRVRRMCTSWGTTFRKCLRAAGLRSQSSVISVMVPSRMPGVSVGEVNGGGQGQESLLRVCLCVCTTLLL

SEQ ID NO: 2109 - protein, 109 aa, Homo sapiens
MVSTVSNRTAFPAFRLVSVLVATWASKSFMVSLLSSWFRPRIRSRRSIWTCRKGSLTPDMLCSVEYPIVTRVRRMCTSWGTTFRKCLRAAGLRSQSSVISVMVPSRMPW

SEQ ID NO: 2110 - protein, 52 aa, Homo sapiens
MVSVLYRCTIFYFLDCIFTVPFLCLYCFNIQILAIVLQLPTIFNKVTCRTGL

SEQ ID NO: 2111 - protein, 78 aa, Homo sapiens
MVTARQVKLRVSDISAEYLTVNKCFFKKRNVTIDVKSRGLNVQMNSAIKNIYYFQYLRIHVCIISKINFHTKVFEQCC

SEQ ID NO: 2112 - protein, 11 aa, Homo sapiens
MVTISLYHYLK

SEQ ID NO: 2113 - protein, 14 aa, Homo sapiens
MVTSALLISGGASL

SEQ ID NO: 2114 - protein, 27 aa, Homo sapiens
MVTVPDSRNIIVFLYIIESDTHTVRQG

SEQ ID NO: 2115 - protein, 22 aa, Homo sapiens
MVVFLVETGFCHVGQAGHELLT

SEQ ID NO: 2116 - protein, 13 aa, Homo sapiens
MVVLICSPSSSGG

SEQ ID NO: 2117 - protein, 28 aa, Homo sapiens
MVVSGWVMICGFRKSSHTKLSGGTEKML

SEQ ID NO: 2118 - protein, 35 aa, Homo sapiens
MVYPCYSMYQYFISFYGQVIFHYMAIIYFLFPFVS

SEQ ID NO: 2119 - protein, 82 aa, Homo sapiens
MWDLGRVEVSHIMEVFHPLNSEQGVYHLFVVSAVVQEGSLETHLDEKYFHRLHCSPHVTMAPDFCVAQRTGHHCGLLCPPGH

SEQ ID NO: 2120 - protein, 14 aa, Homo sapiens
MWEPRNPCALLVRT

SEQ ID NO: 2121 - protein, 139 aa, Homo sapiens
MWERMRRSWASRWCCCCRVRPALAIRWIKVSVILSRTRWIWSFSSRDFRVLDRNVYTPELSKIIDLRHTNSSPCRFIMRNRDDVASSMSKISTMPSTHFPWFLSKSKLGANSSFPGCSMERQTRPIIRISSQAHSRRWT

SEQ ID NO: 2122 - protein, 19 aa, Homo sapiens
MWGILFHSETRDCNYKTSN

SEQ ID NO: 2123 - protein, 12 aa, Homo sapiens
MWHGIQKLQLAS

SEQ ID NO: 2124 - protein, 24 aa, Homo sapiens
MWKIQGSEASVGLNAELNQAHWIV

SEQ ID NO: 2125 - protein, 30 aa, Homo sapiens [sequence omitted]

SEQ ID NO: 2126 - protein, 14 aa, Homo sapiens
MWRNRNAFTLLVGV

SEQ ID NO: 2127 - protein, 14 aa, Homo sapiens
MWRNRNTFALLVGL

SEQ ID NO: 2128 - protein, 14 aa, Homo sapiens
MWRNRNTFTLLVGL

SEQ ID NO: 2129 - protein, 14 aa, Homo sapiens
MWRNRNTFTLVVGL

SEQ ID NO: 2130 - protein, 22 aa, Homo sapiens
MWSFKCMLGSYEETAWYVRERK

SEQ ID NO: 2131 - protein, 11 aa, Homo sapiens
MWSKLSTKQRQ

SEQ ID NO: 2132 - protein, 68 aa, Homo sapiens
MWSTLNSHHQNGNKSMEVRAYHINLPGYDLQMNCLLAYKSKHHKFSPPYQWLPPGPVSEQILTNFYSS

SEQ ID NO: 2133 - protein, 27 aa, Homo sapiens
MWSVPSFALLFALSFFVTRATVTVLIK

SEQ ID NO: 2134 - protein, 58 aa, Homo sapiens
MWVSVLVKGSRGEGQAGYQLRTVDGTDSPGAHRSSSGTRSERDAISAAATRSTRRASV

SEQ ID NO: 2135 - protein, 27 aa, Homo sapiens
MWYEDRKCWSCLIQTWVQISFPPCLAM

SEQ ID NO: 2136 - protein, 30 aa, Homo sapiens
MWYMRGLWSSTPSRAAFIMSSRWASDALSL

SEQ ID NO: 2137 - protein, 46 aa, Homo sapiens
MYAAGSSCFVRRWCGHQCLQLQKAGTQLWIETFLHNLHGSLQKHVS

SEQ ID NO: 2138 - protein, 69 aa, Homo sapiens
MYALMLSICCRRSSSSMGSSASGPLSLSISKGLIQVGSSKGLPGTRGLESLCWGCSSSSLKGLGAGLSG

SEQ ID NO: 2139 - protein, 28 aa, Homo sapiens
MYFMISNIEPPLSNFMTSQSSSLTTKEV

SEQ ID NO: 2140 - protein, 49 aa, Homo sapiens
MYHHTWLIFIFLVKMGFHHVGQASLNLLTSSDPPALNSQSSGITQKHNF

SEQ ID NO: 2141 - protein, 40 aa, Homo sapiens
MYICSTRQHFLCQLIPGTRTLNTASHETAGTFPPFLRSSE

SEQ ID NO: 2142 - protein, 32 aa, Homo sapiens
MYIYLASLLLVLRVQQFCFCFSGLMLWFFSYP

SEQ ID NO: 2143 - protein, 24 aa, Homo sapiens
MYLDVHQSGKSPRYGKFSAIISLN

SEQ ID NO: 2144 - protein, 38 aa, Homo sapiens [sequence omitted]

SEQ ID NO: 2145 - protein, 58 aa, Homo sapiens
MYMMTPMAQQSTGRPYRCRPTTSGARYSGVPQGSLMRPFSSLARWKSLMTIFEFFSRL

SEQ ID NO: 2146 - protein, 22 aa, Homo sapiens
MYPCKCGTDLILGPCLEIGSQQ

SEQ ID NO: 2147 - protein, 36 aa, Homo sapiens
MYPSRAVGYSSVQEALSLCGRVRLYLYDPLWILACI

SEQ ID NO: 2148 - protein, 28 aa, Homo sapiens
MYQYFISFYGQVIFHYMAIIYFLFPFVS

SEQ ID NO: 2149 - protein, 11 aa, Homo sapiens
MYRLYSPTLSL

SEQ ID NO: 2150 - protein, 11 aa, Homo sapiens
MYSDEKLSQIC

SEQ ID NO: 2151 - protein, 11 aa, Homo sapiens
MYTCSPSYSRG

SEQ ID NO: 2152 - protein, 42 aa, Homo sapiens
MYTTTAKLFFIHDLYYCRMASRGEVNGGRGWWEQNARTKPNT

SEQ ID NO: 2153 - protein, 54 aa, Homo sapiens
MYTTTAKLFFIHDLYYCRMASRGEVNGGRGWWEQNARTKPQILEQHPLQKQNNE

SEQ ID NO: 2154 - protein, 33 aa, Homo sapiens
MYVAFHLAYFLCFTFSSVSSPNTVMTSIKRLAV

SEQ ID NO: 2155 - protein, 40 aa, Homo sapiens
MAAAQLSPPSMVFLSMVSVTRGKVGSDSVLRPRPLVFSLE

SEQ ID NO: 2156 - protein, 56 aa, Homo sapiens
MAAIFCSAFLFNSANFAALSDSSLSSNAFNSSSLLFTLKFTCSNSFFLVSSSAFME

SEQ ID NO: 2157 - protein, 11 aa, Homo sapiens
MAAKARLVLNS

SEQ ID NO: 2158 - protein, 42 aa, Homo sapiens
MAALAGCPGQDSGLLWQGVRLQWEILRLGNALPPQSLSSDAC

SEQ ID NO: 2159 - protein, 42 aa, Homo sapiens
MAASSCFCCTRWSPHASSSFTTSTGKANRASSTAFMNALPLR

SEQ ID NO: 2160 - protein, 32 aa, Homo sapiens
MAASSTDKEVGSRGAISTHVPELMASSTDAST

SEQ ID NO: 2161 - protein, 29 aa, Homo sapiens
MACISCPFITCPKSRDPNYQRETLVNHRL

SEQ ID NO: 2162 - protein, 91 aa, Homo sapiens
MACLISRVAAFWSASWSPLAFLCSSRLCMSPKLAGLWARSVLCQSASARCPTTSLTTSSLLSMSHRPSEASTRNLSWGLSLWYVTSGSAVR

SEQ ID NO: 2163 - protein, 12 aa, Homo sapiens
MAEGSPTPECLR

SEQ ID NO: 2164 - protein, 12 aa, Homo sapiens
MAEPCPLTSGAS

SEQ ID NO: 2165 - protein, 66 aa, Homo sapiens
MAEPQRDQGAPVQPAEHQEAQDDQQQESQRAGRPPPEAPRGHRVFSKRGDPGSHSSPHSAARGSLA

SEQ ID NO: 2166 - protein, 28 aa, Homo sapiens
MAETIYLQMPSHSLINLLCAVTEICDSI

SEQ ID NO: 2167 - protein, 17 aa, Homo sapiens
MAFAKFGTPSISVVFCP

SEQ ID NO: 2168 - protein, 17 aa, Homo sapiens
MAFCTFFILFFFLFHLR

SEQ ID NO: 2169 - protein, 18 aa, Homo sapiens
MAFFFPEAYPSELLVKNS

SEQ ID NO: 2170 - protein, 12 aa, Homo sapiens
MAFFKGVLLRLN

SEQ ID NO: 2171 - protein, 40 aa, Homo sapiens
MAFGWAKKLYMCERSSPRRTFPERSRWTRVEAVNGLALSD

SEQ ID NO: 2172 - protein, 41 aa, Homo sapiens
MAFHHVGQAGFELLTSSNQPALASQSVGITGVSHHAQEKCF

SEQ ID NO: 2173 - protein, 31 aa, Homo sapiens
MAFINRCRDFCYTHNPKERSRFPAFIWHLVT

SEQ ID NO: 2174 - protein, 69 aa, Homo sapiens
MAFLCVGQADLELPTSGDLPALASQSAGITGLSHQAQPTVLFFLNTMVTFRTFNGPKILCDECIILHSN

SEQ ID NO: 2175 - protein, 112 aa, Homo sapiens
MAFPTPSLRASPRPCPRASPIFVPVLSSPLCRGPASPLPRQRASRRQARGPWNFISAQPPLSPECLPPTRVSSLPPLLCVSVPSSVLLLPTPCPPSLWVCSLLSPVLNCLGF

SEQ ID NO: 2176 - protein, 122 aa, Homo sapiens
MAFPTPSLRASPRPCPRASPIFVPVLSSPLCRGPASPLPRQRASRRQARGPWNFISAQPPLSPECLPPTRVSSLPPLLCVSVPSSVLLLPTPCPPSLWVCSLLSPVLNCLGFSESTSLSLLL

SEQ ID NO: 2177 - protein, 79 aa, Homo sapiens
MAFTSISLIITDTSLLSPPCLGARSPPRTDARCRAPWTSLSMQEKCQGKVHGSFLLSTQGPDRSGFLPRTQLQVVQKPP

SEQ ID NO: 2178 - protein, 44 aa, Homo sapiens
MAGAALSLAAPSPPGARRTRRTLGARRTFRGTQRCCAPCFGRGT

SEQ ID NO: 2179 - protein, 11 aa, Homo sapiens
MAGAHQSFSRM

SEQ ID NO: 2180 - protein, 19 aa, Homo sapiens
MAGASCSSLSSFLFLNCIS

SEQ ID NO: 2181 - protein, 87 aa, Homo sapiens
MAGEPGGAAGEVSWWADGQARRRERCGGSGVRVAPGGSRRGRHGRRGAARAGGTQVRGGGPGPELVAARCPPRRLDSELPGSPAANK

SEQ ID NO: 2182 - protein, 37 aa, Homo sapiens
MAGERVRPTPRTQERRGAAASPVQETRPHGSPPVPQP

SEQ ID NO: 2183 - protein, 58 aa, Homo sapiens
MAGGLWPLGFPLLAWGVRLTVERMPDPRSSFRYLLLTTYRNNWAVTREVIPYILRPRI

SEQ ID NO: 2184 - protein, 38 aa, Homo sapiens
MAGQRLGPSLALVQKCCWLELVQSCCKVHRVSRAHQPQ

SEQ ID NO: 2185 - protein, 23 aa, Homo sapiens
MAGTPGAGAGGSSGGGARAAASP

SEQ ID NO: 2186 - protein, 98 aa, Homo sapiens
MAGTPGAGAGGSSGGGARAAASPRRSGLPPSLYGGPDRSRQPSQLLRGASRPLGLTRSRPEMRPRPPRGRGRGRSPSRLPCMRGWDRGPRAPSPEPRL

SEQ ID NO: 2187 - protein, 15 aa, Homo sapiens
MAHHLSLLPFHYLQH

SEQ ID NO: 2188 - protein, 17 aa, Homo sapiens
MAIIKKDTTEAGEDVEK

SEQ ID NO: 2189 - protein, 13 aa, Homo sapiens
MAIIKKLKNNRCW

SEQ ID NO: 2190 - protein, 25 aa, Homo sapiens
MAIIKKQKKKSRCWRSYGAIGTHIH

SEQ ID NO: 2191 - protein, 168 aa, Homo sapiens
MAIIKKSGNNRCWKGCGEIGTLLHFWWECKLVQPLWKTVWQFLRDLELEIPFDPAIPLLGIYPKDYKSCCYKDTCTRIFIAALFTIAKTWNQPKCPSMIDWIKKMWHIYTIEYCAAIKNDEFMSFVGTWIKLETILFSKLLQEQKNQTPHVLSHWWELNDENTWTQER

SEQ ID NO: 2192 - protein, 119 aa, Homo sapiens
MAIIKKSGNNRCWRGCGEIRTLLHCWWDCELVQPLWKSVWRFLRDLELEIPFDPAIPLLGIYPKDYKSCCYKDTCTLMFIAALFTIAKTWNQPKCPTMIDWIKKRWHIYTMEVRHFSSL

SEQ ID NO: 2193 - protein, 34 aa, Homo sapiens
MAIIQKSKNNRYWQGCGGKGKLLNSWLEYKSVHH

SEQ ID NO: 2194 - protein, 26 aa, Homo sapiens
MAILCGEDTGNGLLNTKSLVYPLLPF

SEQ ID NO: 2195 - protein, 50 aa, Homo sapiens
MAIPMIGTNFSSSAKESSLLLIPRPPTLLHTNQDVFCASLVLSSSKTIFT

SEQ ID NO: 2196 - protein, 106 aa, Homo sapiens
MAIWEYPRQTQNVQLMTSPPSWWSHRSHTPPSQPAASSLKVFRSLWPRCFHPILLLPFQLFLHLSEWGGLTCKLEHTFATSRVPRKGGVETKATMVLHVHKRLAGV

SEQ ID NO: 2197 - protein, 54 aa, Homo sapiens
MAKAKLSKLVMPCLGPSQPGLHTVPFWHCRPWPVSSAQGEGSSSAGTSAMPSWL

SEQ ID NO: 2198 - protein, 16 aa, Homo sapiens
MAKEGNQHILEYLSYT

SEQ ID NO: 2199 - protein, 11 aa, Homo sapiens
MAKGLSKENEE

SEQ ID NO: 2200 - protein, 44 aa, Homo sapiens
MAKIHYIFAFYSFLCVKFISLNQDNLERVVIFPNMRNNSCFLWW

SEQ ID NO: 2201 - protein, 170 aa, Homo sapiens
MALAMGSIMAVEAVLLSHMDKNEVVTIIPRMSLAGWTPTSIRILRAIRRCRFHSSMALAMISPLRKRKLVSRKYWGQTLLEGKMPMKGKRTMGSSAVTESGRASVHQYTAMSRMTNKQRPSLGGRAKTTGSSASGVNSSTSSRRALHTFLAAAASAAISAIAWRYGPARD

SEQ ID NO: 2202 - protein, 11 aa, Homo sapiens
MALGQGCPACL

SEQ ID NO: 2203 - protein, 33 aa, Homo sapiens
MALIFVEKDLLLALLLEKGRAAFEAAEPSPALG

SEQ ID NO: 2204 - protein, 37 aa, Homo sapiens
MALIFVEKDLLLALLLEKGRAQALPAFEAAEPSPALG

SEQ ID NO: 2205 - protein, 23 aa, Homo sapiens
MALISGELFSDKYAQNFVRTDPT

SEQ ID NO: 2206 - protein, 74 aa, Homo sapiens
MALRAPPCNKGDLTSPISSLRMDPLIFEREEGYTFAKVVRKLMAICETCISLSLIRGGSSSRTASIMAAVKLSL

SEQ ID NO: 2207 - protein, 28 aa, Homo sapiens
MALSKVTQLISGRAGLQPSSVAPVSRRA

SEQ ID NO: 2208 - protein, 21 aa, Homo sapiens
MALSLSLQLMTQLYLIHQLMV

SEQ ID NO: 2209 - protein, 71 aa, Homo sapiens
MALSTPQSRKHGYAAKCLTAQFRRILPSILGILNAVQWQPVSASIFSSAPQAQCRGNRFGFQLFLLPLSTL

SEQ ID NO: 2210 - protein, 40 aa, Homo sapiens
MALSTPQSRKHGYAAKCLTAQFRRILPSILGIWYILHGFQ

SEQ ID NO: 2211 - protein, 33 aa, Homo sapiens
MAMLASSVNVSEKLILPGWVSGAGVPGVLKDKG

SEQ ID NO: 2212 - protein, 37 aa, Homo sapiens
MANEQRIADLAADDVMKAPGKLHSDPRVELWARLQHL

SEQ ID NO: 2213 - protein, 27 aa, Homo sapiens
MANFIIERMSFINTSVVQSCACKSQQS

SEQ ID NO: 2214 - protein, 13 aa, Homo sapiens
MANLCRDSLCRTK

SEQ ID NO: 2215 - protein, 21 aa, Homo sapiens
MANLLKMASIIAFKNEYKTKQ

SEQ ID NO: 2216 - protein, 16 aa, Homo sapiens
MANMMVAGKAVGCVAI

SEQ ID NO: 2217 - protein, 19 aa, Homo sapiens
MANSPVFLTAPPTRRKTVP

SEQ ID NO: 2218 - protein, 25 aa, Homo sapiens
MANTEKKVSSSRKSGPKFSLNISDL

SEQ ID NO: 2219 - protein, 63 aa, Homo sapiens [sequence omitted]

SEQ ID NO: 2220 - protein, 34 aa, Homo sapiens
MAPASYRSLEPNHRRSACHQQASLRFEGMLFIPT

SEQ ID NO: 2221 - protein, 17 aa, Homo sapiens
MAPNPYHWPFTSPTSDT

SEQ ID NO: 2222 - protein, 29 aa, Homo sapiens
MAPPPTPRSPTGSASLPRHSRRAQGTAGS

SEQ ID NO: 2223 - protein, 79 aa, Homo sapiens
MAPTSPFGVLPAVGSWNTGSCMALEVTCDSLTESASACNGPRSLSRSSCSATTAASSALRVLRASSSACSWCICSRAEL

SEQ ID NO: 2224 - protein, 92 aa, Homo sapiens
MAQALATASDTAPMAILPLSTGSTGSAGAIGFSVIVSFLPGFCPFFLVGGGGGGGGGTGGRGVGTVEYSRLFSNSFLPLSSCTLLAKNILSR

SEQ ID NO: 2225 - protein, 32 aa, Homo sapiens [sequence omitted]

SEQ ID NO: 2226 - protein, 20 aa, Homo sapiens
MAQNMRRCKVPCLVKSHLEQ

SEQ ID NO: 2227 - protein, 22 aa, Homo sapiens
MAQPLCLSPGGGVETAPSASVL

SEQ ID NO: 2228 - protein, 11 aa, Homo sapiens
MAQRTARTVST

SEQ ID NO: 2229 - protein, 13 aa, Homo sapiens
MAQVRKQLRKKYL

SEQ ID NO: 2230 - protein, 16 aa, Homo sapiens
MARAPAAATWRPAAAV

SEQ ID NO: 2231 - protein, 22 aa, Homo sapiens
MARAPAAATWRPAAAVGARVSR

SEQ ID NO: 2232 - protein, 95 aa, Homo sapiens
MARASSLTTASSIKKQFTIYDRKLGRKSCSNCFMANMTSEKLKIKRFSNLLSNIFSMVSLMRVSGKETFSPRIKAEITSKRVSQQDVERLATCSV

SEQ ID NO: 2233 - protein, 26 aa, Homo sapiens
MARHLHPLWHTQVSMRLVLWVKCGRK

SEQ ID NO: 2234 - protein, 46 aa, Homo sapiens
MARLLISWPSLVHLHIGNGFPLIGMVSLMTPPCLTKIPSWYLSSSS

SEQ ID NO: 2235 - protein, 42 aa, Homo sapiens
MARPLFLKIRQLWFTTGDSQQIAPVSAHPRPFCCGQGLERVP

SEQ ID NO: 2236 - protein, 24 aa, Homo sapiens
MARSRLIATSASQIQVILPFQPPE

SEQ ID NO: 2237 - protein, 24 aa, Homo sapiens
MARSRLTTTSSSWVQAILLPQPPK

SEQ ID NO: 2238 - protein, 18 aa, Homo sapiens
MASADVPPSVGTCSSSSS

SEQ ID NO: 2239 - protein, 19 aa, Homo sapiens
MASADVPPSVGTCSSSSSS

SEQ ID NO: 2240 - protein, 23 aa, Homo sapiens
MASALSLRDERNREKGVKSRSMV

SEQ ID NO: 2241 - protein, 30 aa, Homo sapiens
MASFEKKLTVQVWSSRGESTSSRSLMSSGL

SEQ ID NO: 2242 - protein, 19 aa, Homo sapiens
MASGARGAGGARGSKRRRR

SEQ ID NO: 2243 - protein, 15 aa, Homo sapiens
MASGGVRDLNTFVQG

SEQ ID NO: 2244 - protein, 34 aa, Homo sapiens
MASGISPSCLGCEVDGREDARSKELLQISPSNYI

SEQ ID NO: 2245 - protein, 15 aa, Homo sapiens
MASIIAFKNEYKTKQ

SEQ ID NO: 2246 - protein, 18 aa, Homo sapiens
MASPFLVGAARRLWARPP

SEQ ID NO: 2247 - protein, 22 aa, Homo sapiens
MASPFLVGAARRLWARPPGAGL

SEQ ID NO: 2248 - protein, 25 aa, Homo sapiens
MASSTSPVIFSTLSIHWFFMVSKCS

SEQ ID NO: 2249 - protein, 20 aa, Homo sapiens
MASTTGSGKGPLLPMQVMQP

SEQ ID NO: 2250 - protein, 32 aa, Homo sapiens
MATARGHLKGGALSTSTAPQQAVGEREGSSWP

SEQ ID NO: 2251 - protein, 17 aa, Homo sapiens
MATEPQLSGHSPYLSMF

SEQ ID NO: 2252 - protein, 35 aa, Homo sapiens
MATKAKIDKRDLIKLKSFCTAKETTIRAGHSGSCL

SEQ ID NO: 2253 - protein, 74 aa, Homo sapiens
MATKAKIDKWDLIKLKSFCTAKETTISVNRQPTEWEKIFAIYSSDKGLISRIYKELKQIYKKKKTTPSTSVQRI

SEQ ID NO: 2254 - protein, 44 aa, Homo sapiens
MATNHSSRTACAEVTTDHHLLCWTPADSSRAGTMSERPKKRPWF

SEQ ID NO: 2255 - protein, 21 aa, Homo sapiens
MATPESSGSWVCPILPLFHSN

SEQ ID NO: 2256 - protein, 27 aa, Homo sapiens
MATSGSVGAGVLRWIVRCLAASLTSAD

SEQ ID NO: 2257 - protein, 12 aa, Homo sapiens
MATSTKYFLLCR

SEQ ID NO: 2258 - protein, 16 aa, Homo sapiens
MATYRKWRNGPLLHFL

SEQ ID NO: 2259 - protein, 20 aa, Homo sapiens
MAVAPLLKMNRQCQDLLLDF

SEQ ID NO: 2260 - protein, 13 aa, Homo sapiens
MAVAYFLTCMSLA

SEQ ID NO: 2261 - protein, 30 aa, Homo sapiens
MAVIKKSKNNRCWGGCREKGMLYTADGNIN

SEQ ID NO: 2262 - protein, 27 aa, Homo sapiens
MAVLCYQIPFFSKLQIMYFRDFFKVAK

SEQ ID NO: 2263 - protein, 63 aa, Homo sapiens
MAVPINMLMENNSQKGEGRTNKPTGVSYRRGWTPPLRGRRQLLASFLPDSSQLFCRLLCPEGS

SEQ ID NO: 2264 - protein, 47 aa, Homo sapiens
MAVPINMLMENNSQKGEGRTNKPTGVSYRRGWTPPLRGRRQLMVGSC

SEQ ID NO: 2265 - protein, 28 aa, Homo sapiens
MAVRTFGTLGESEQRSPACGRVCGTSST

SEQ ID NO: 2266 - protein, 113 aa, Homo sapiens
MAVRTFLPLWLLEASLAEREGNWPREGGFRPRSSWAPLVASSSLSSGSRPVSAAELRELSVQHSLGPPWPVPSLSGAAVISSPSLSARDSSSSVTAWLSSFCRRGRVRSTVMR

SEQ ID NO: 2267 - protein, 112 aa, Homo sapiens
MAVRTFLPLWLLEASLAEREGNWPREGGFRPRSSWAPVASSSLSSGSRPVSAAELRELSVQHSLGPPWPVPSLSGAAVISSPSLSARDSSSSVTAWLSSFCRRGRVRSTVMR

SEQ ID NO: 2268 - protein, 16 aa, Homo sapiens
MAVSCCCLLAKAFLAK

SEQ ID NO: 2269 - protein, 41 aa, Homo sapiens
MAVTNGLKSTAPTQLTFIKPYQGQTLYIPIHHPHLILPLTL

SEQ ID NO: 2270 - protein, 57 aa, Homo sapiens [sequence omitted]

SEQ ID NO: 2271 - protein, 42 aa, Homo sapiens
MCAGQGEGLFFPPLFKGLQPLCDYKSQSSDLFTQCQFPKFNS

SEQ ID NO: 2272 - protein, 18 aa, Homo sapiens
MCCENVVSFACGLPFLRS

SEQ ID NO: 2273 - protein, 30 aa, Homo sapiens
MCERSSPRRTFPERSRWTRVEAVNGLALSD

SEQ ID NO: 2274 - protein, 22 aa, Homo sapiens
MCFDQWNVAEVILSPECLLSPS

SEQ ID NO: 2275 - protein, 15 aa, Homo sapiens
MCFPYWCNNKQMMQQ

SEQ ID NO: 2276 - protein, 39 aa, Homo sapiens
MCGGFESRASAFFLSFFFLFFFLRQRFALSPRLECSAVM

SEQ ID NO: 2277 - protein, 25 aa, Homo sapiens
MCGKLIFLISRLCFTAVSGSSKLCL

SEQ ID NO: 2278 - protein, 21 aa, Homo sapiens
MCHDIWLIFEFLVETGFLHVS

SEQ ID NO: 2279 - protein, 38 aa, Homo sapiens
MCHGGLLHLWEQFFLNKNIFFNTELRPQAYISHLKTVL

SEQ ID NO: 2280 - protein, 31 aa, Homo sapiens
MCHHAQLIFCIFSRDGVSPCWSGWSRIPDLR

SEQ ID NO: 2281 - protein, 30 aa, Homo sapiens
MCHHARLIFVFLVEKGFHCVGQAGLELLTL

SEQ ID NO: 2282 - protein, 11 aa, Homo sapiens
MCHHARLILYF

SEQ ID NO: 2283 - protein, 12 aa, Homo sapiens
MCHHAWLIFLYL

SEQ ID NO: 2284 - protein, 31 aa, Homo sapiens
MCHHAWLIFVFLVEMGFHHVGQAGSRTPDLR

SEQ ID NO: 2285 - protein, 29 aa, Homo sapiens
MCHHAWLIFVFLVETAFHHVGQAGLELLT

SEQ ID NO: 2286 - protein, 94 aa, Homo sapiens
MCHHAWLIFVFLVETGFCHVGQAGLKLLTSSDLPTLVSQSAGITGVSHRAQPQVDSSSGTKRTCLTSFWPPWFPERNPLSSELLFPLAKISLLS

SEQ ID NO: 2287 - protein, 45 aa, Homo sapiens
MCHHAWLIFVFLVETGFHHVGQAGLKLLTSMICPPQPAKVLGLQV

SEQ ID NO: 2288 - protein, 11 aa, Homo sapiens
MCHHAWLTLYF

SEQ ID NO: 2289 - protein, 87 aa, Homo sapiens [sequence omitted]

SEQ ID NO: 2290 - protein, 44 aa, Homo sapiens
MCHHIQLIVVFLVETGFHHVGQAGLEFLISGDPPRSASQSWSYF

SEQ ID NO: 2291 - protein, 31 aa, Homo sapiens
MCHHIWLIFVFLIETRVSSCWPGWSQTPDLR

SEQ ID NO: 2292 - protein, 24 aa, Homo sapiens
MCHHLHINYTSVKHRLESFAFLCI

SEQ ID NO: 2293 - protein, 57 aa, Homo sapiens
MCHHTQLIFVFLVEMGFHHVDQTSLELLTSGDPPASASQSVGITGMSHCTQPSTAYF

SEQ ID NO: 2294 - protein, 56 aa, Homo sapiens
MCHHTRLIFVFLIETGFHHVGQAGFELLTSGDPPTSASQSAEVTGMSHRTWPVFAY

SEQ ID NO: 2295 - protein, 20 aa, Homo sapiens
MCHHTRLMFSIFSRDGVLPC

SEQ ID NO: 2296 - protein, 12 aa, Homo sapiens
MCHHTWLILYFF

SEQ ID NO: 2297 - protein, 56 aa, Homo sapiens
MCHYTRLIFLFLVEMGFCHVGQAGLELLTSSHLPASASQSAGITGMSHCARLERFF

SEQ ID NO: 2298 - protein, 14 aa, Homo sapiens
MCIKSFFISTALHF

SEQ ID NO: 2299 - protein, 25 aa, Homo sapiens
MCIPHSFVLVILFSLLQSNFNNESA

SEQ ID NO: 2300 - protein, 20 aa, Homo sapiens
MCITGLYLLKELLCYLSTLL

SEQ ID NO: 2301 - protein, 14 aa, Homo sapiens
MCKGEEAQCFTGLA

SEQ ID NO: 2302 - protein, 33 aa, Homo sapiens
MCLFSRYIVHLVPCASPFNPCPRFFGWVHGPDY

SEQ ID NO: 2303 - protein, 47 aa, Homo sapiens
MCLHQWAPALLLLLEKTQWVAGNQECILFFPLHLYFQVEETEVHCSC

SEQ ID NO: 2304 - protein, 48 aa, Homo sapiens
MCLHQWAPALLLLLLEKTQWVAGNQECILFFPLHLYFQVEETEVHCSC

SEQ ID NO: 2305 - protein, 15 aa, Homo sapiens
MCLSAGIPMRHLSYR

SEQ ID NO: 2306 - protein, 63 aa, Homo sapiens
MCLVPESDKLVMYSGNVSTLGSLSRSSDSSDGELPLLMSSYSSQSRRWTCLFGYQIEQDSSKP

SEQ ID NO: 2307 - protein, 30 aa, Homo sapiens
MCNINTEAMNRRLITNTGTGPTLSPGESSV

SEQ ID NO: 2308 - protein, 73 aa, Homo sapiens
MCNPRPISKSLPKINIFLLLHLTAALRKTVPMTYLTGGVNTTNIFYSFLQFFQFLYQQYLNFSFRKHHSSWCL

SEQ ID NO: 2309 - protein, 44 aa, Homo sapiens
MCPLRFSKPPILDTDVVWLCPHPNLNLNCISQNFHMLWEGPRRS

SEQ ID NO: 2310 - protein, 30 aa, Homo sapiens
MCQDYDLFQIVVSHLIYFFLLVLLLSSFSF

SEQ ID NO: 2311 - protein, 13 aa, Homo sapiens
MCQTLFPDSFCAL

SEQ ID NO: 2312 - protein, 31 aa, Homo sapiens
MCQWKWHWQKTSPSRNSYRYFVTLQEQRIKH

SEQ ID NO: 2313 - protein, 83 aa, Homo sapiens
MCRGVPLLRGGGAGRAAPGAWLQSSSPLPIWGGGGRGQRRGEPPPLPPRLRFPETGSSGHTQAWGWGSAVEPGCAGWGEGKTD

SEQ ID NO: 2314 - protein, 59 aa, Homo sapiens [sequence omitted]

SEQ ID NO: 2315 - protein, 20 aa, Homo sapiens
MCRHSMLPSHTLTSLSCAIT

SEQ ID NO: 2316 - protein, 20 aa, Homo sapiens
MCRSAAGARPAGAGPQGSGR

SEQ ID NO: 2317 - protein, 128 aa, Homo sapiens
MCSARSRLASSMNGRFSASDMTFHSAPRRLLISELCILGFSWAILRRCPRDHTMKAFMGRLTRSWLALAPPPPPPPPPPPPPPPAPAGPERFVGAWAPPGECRSVSIIMLYIGAAGGFTGTARRGPGA

SEQ ID NO: 2318 - protein, 21 aa, Homo sapiens
MCSCFLHNIGLTFATNRILWK

SEQ ID NO: 2319 - protein, 55 aa, Homo sapiens
MCSKMPCSRRCRALKFSTPHCGMAMLASSVNVSEKLILPGWVSGAGVPGVLKDKG

SEQ ID NO: 2320 - protein, 31 aa, Homo sapiens
MCSKQLSVPGPAQQWEAAALLQHLTQGIICT

SEQ ID NO: 2321 - protein, 154 aa, Homo sapiens [sequence omitted]

SEQ ID NO: 2322 - protein, 22 aa, Homo sapiens
MCTETYNVYSYHQWSNLMNHTD

SEQ ID NO: 2323 - protein, 103 aa, Homo sapiens
MCTQPVTNTKEVKWQRVLYEQQPFPDNFVDRRFLEELWKNIHARKYQYWAMVFESSVVIPQLCSVFVFLVIWWYMDEGLLAPQWLFGTGLASSLIGYVLFDLT

SEQ ID NO: 2324 - protein, 138 aa, Homo sapiens [sequence omitted]

SEQ ID NO: 2325 - protein, 16 aa, Homo sapiens
MCVCTYIYFFYYFFLL

SEQ ID NO: 2326 - protein, 25 aa, Homo sapiens
MCYRICKEDRLQDQGEGSSPQVRGV

SEQ ID NO: 2327 - protein, 23 aa, Homo sapiens
MCYYNLCWKSLYGVRKNKPFISS

SEQ ID NO: 2328 - protein, 14 aa, Homo sapiens
MDAILKYKCQSSAW

SEQ ID NO: 2329 - protein, 17 aa, Homo sapiens
MDDPFYYLSLDPLYTLN

SEQ ID NO: 2330 - protein, 14 aa, Homo sapiens
MDFEVVTVLEPVLL

SEQ ID NO: 2331 - protein, 24 aa, Homo sapiens
MDFPILLANMHKFFILKKLCLSSY

SEQ ID NO: 2332 - protein, 41 aa, Homo sapiens
MDFRTSMPSFGAISSLTTVTLGKFLLLFFSTKQPSEKNVSL

SEQ ID NO: 2333 - protein, 44 aa, Homo sapiens
MDFSISLSKSSRSLISALKPIISLSSFKPMNKYPPSVFANAETY

SEQ ID NO: 2334 - protein, 25 aa, Homo sapiens
MDFSTLVTYVTWSSLDLSSFCCILS

SEQ ID NO: 2335 - protein, 36 aa, Homo sapiens
MDHCCISFRRQCSPWYFSSSHTRVVASGSLESIMKS

SEQ ID NO: 2336 - protein, 27 aa, Homo sapiens
MDIWTETVEAAAGCLLVSEAAEHHNRD

SEQ ID NO: 2337 - protein, 12 aa, Homo sapiens
MDKIARCQLIHL

SEQ ID NO: 2338 - protein, 28 aa, Homo sapiens
MDLFKLQKQSLLVLLGFFGLSYYKYIKL

SEQ ID NO: 2339 - protein, 18 aa, Homo sapiens
MDLFYIKTQLFPNLRDGY

SEQ ID NO: 2340 - protein, 191 aa, Homo sapiens
MDLLQEFPEAWDLPSLQSESNGAANHVEVLRHGDQGGAGPGLAGQPDLARDIAPDNLLDEGLKIWATGENHDDFGRGILNHLYHMLDLFLIRVLGDEFTEVDADIPFLSFLSEFLNPRPPIVVISCNCAHPVPAEILDDVCHGSGLVLIIGDGSEERLELILVAEESAGGGITDLGNVEEPQQICHCRGDA

SEQ ID NO: 2341 - protein, 44 aa, Homo sapiens
MDLPMMFSSPKLKNACEMIFLNPCNRPFRCCPQEKRFLKKQIEK

SEQ ID NO: 2342 - protein, 17 aa, Homo sapiens
MDLSVNFSLKQQKNTVY

SEQ ID NO: 2343 - protein, 30 aa, Homo sapiens
MDMNSSMLSLARRSLSRLSCTASSSRGASS

SEQ ID NO: 2344 - protein, 35 aa, Homo sapiens [sequence omitted]

SEQ ID NO: 2345 - protein, 22 aa, Homo sapiens
MDMRICIICKGHPTVITWERLW

SEQ ID NO: 2346 - protein, 20 aa, Homo sapiens
MDPCQYYFQPQFGKSRLFLE

SEQ ID NO: 2347 - protein, 31 aa, Homo sapiens
MDPCRVLEMWFPIRLSKAELQARATLAVPMT

SEQ ID NO: 2348 - protein, 51 aa, Homo sapiens [sequence omitted]

SEQ ID NO: 2349 - protein, 123 aa, Homo sapiens
MDPIIPIHALLFGQGLIKSLLCFFKCVPVPLRLLHLLRLTLGCENQTGTKGGYSSLTDGLFGVPHGHKNVVKEGLHLLEEEGRDADGQLTENQDLWPRCHLSSHWHLSWKPIQKCDGSVGHRS

SEQ ID NO: 2350 - protein, 184 aa, Homo sapiens
MDPIIPIHALLFGQGLIKSLLCFFKCVPVPLRLLHLLRLTLGCENQTGTKGGYSSLTDGLFGVPHGHKNVVKEGLHLLEEEGRDADGQLTENQDSCMSPALIAVSTQPFQGSLHLKFHVLSGKSVPCHGKTANGLGCHFHDNWVIGGEEVPKIVGKSANSGGIPTFHSYEASYGQDATFPLIGI

SEQ ID NO: 2351 - protein, 19 aa, Homo sapiens
MDPPPNTLLPLFRGTSVSL

SEQ ID NO: 2352 - protein, 42 aa, Homo sapiens
MDQCCFSNSCDYQQKLDISTSHRGCRRSLEIPFVQTTTSTLQ

SEQ ID NO: 2353 - protein, 13 aa, Homo sapiens
MDQCCFSNSWGPR

SEQ ID NO: 2354 - protein, 14 aa, Homo sapiens
MDSICSKSCKPFSW

SEQ ID NO: 2355 - protein, 27 aa, Homo sapiens
MDSIRSLKNLVSMKRRMSSGLRHFSCW

SEQ ID NO: 2356 - protein, 41 aa, Homo sapiens
MDSLHLFSTLQCVKPFHITLLMSCHKQLCEARRARGVQSPF

SEQ ID NO: 2357 - protein, 144 aa, Homo sapiens
MDSSTNNRPAAIQFSPLLKNTAPMPIRTALSSSQSLNIISGDLPPSSRETFFKLLTAQLFMICLPIGVDPVKPSLRMSGCSDRRCPAMPPEPGMMLMTPFGKPAFTDSSANFKAVKGVTCAGLSTKVLPAAKHAALFHASIISG

SEQ ID NO: 2358 - protein, 26 aa, Homo sapiens
MDTEAWRSPEQSLGTLEKTLPVEGRA

SEQ ID NO: 2359 - protein, 24 aa, Homo sapiens
MDTPFSMIRLFHIAYLYQNISCTP

SEQ ID NO: 2360 - protein, 76 aa, Homo sapiens
MDTQDTIWPRRPILTQGLCSPGTSVLTAGVSRALLLVGAQARTAPATTRHPSAQGQGPVVSLLRRLWNNPVPFSSF

SEQ ID NO: 2361 - protein, 16 aa, Homo sapiens
MDVSQEGKRQRGGYRV

SEQ ID NO: 2362 - protein, 17 aa, Homo sapiens
MDVTESTNECTCPKCAT

SEQ ID NO: 2363 - protein, 20 aa, Homo sapiens
MDWSCRSHSPPWSQIGQSNG

SEQ ID NO: 2364 - protein, 67 aa, Homo sapiens [sequence omitted]

SEQ ID NO: 2365 - protein, 63 aa, Homo sapiens
MEACKVLPRICSPLEWRESLKMRNTRTRRMTRRMARDMACCPFWPPPPPPGCCSASSVPRVMK

SEQ ID NO: 2366 - protein, 41 aa, Homo sapiens
MEALHRTGVQSRSKRLYNSGISANRMNRHTPSCIISTRTNI

SEQ ID NO: 2367 - protein, 66 aa, Homo sapiens [sequence omitted]

SEQ ID NO: 2368 - protein, 14 aa, Homo sapiens
MECNFSQIQNYFIF

SEQ ID NO: 2369 - protein, 94 aa, Homo sapiens
MEDERLVRLKDPRMTSNAGAKKVWKDGSCRSHWYWTAGLLLGDWQLRVTFAPTWGTPWRRQDGGAGGTSTLSSKVLMLWPLDLPCLSCTFTEQL

SEQ ID NO: 2370 - protein, 23 aa, Homo sapiens
MEDIAPQMVVCNTGGFLKWHIFP

SEQ ID NO: 2371 - protein, 11 aa, Homo sapiens
MEDNETRDFTL

SEQ ID NO: 2372 - protein, 17 aa, Homo sapiens
MEEKEHMIRMQESSLVG

SEQ ID NO: 2373 - protein, 37 aa, Homo sapiens
MEELFINFFIFFNRQFCCFLGILKYTVLLLQGYNPFS

SEQ ID NO: 2374 - protein, 33 aa, Homo sapiens
MEEPLGPIAVLRFTGHSMFLWFSLKLFVMLDRG

SEQ ID NO: 2375 - protein, 13 aa, Homo sapiens
MEESESLSGQPVN

SEQ ID NO: 2376 - protein, 26 aa, Homo sapiens
MEEWTTAAFPLGDSALLGTSVVHIHE

SEQ ID NO: 2377 - protein, 34 aa, Homo sapiens
MEFHHVFQAGLDLPGSSDPPAVAFQSARITSVTH

SEQ ID NO: 2378 - protein, 18 aa, Homo sapiens
MEFKLSHFQKEPKDIFGS

SEQ ID NO: 2379 - protein, 31 aa, Homo sapiens
MEFLHVGHLVSNSRPQVIRPPWPPKVLGLQA

SEQ ID NO: 2380 - protein, 25 aa, Homo sapiens
MEFRAPLLKGQEGEKSMPADKESVH

SEQ ID NO: 2381 - protein, 61 aa, Homo sapiens
MEFRAPLLSGRVCPGFHASVFAGMSFCPLFPSPPSKPDRMLLEGRASSASSLKAQMQSGSW

SEQ ID NO: 2382 - protein, 35 aa, Homo sapiens
MEFRAPLSAFILFFPFSLFQQNIYLLSQVGCTGKQ

SEQ ID NO: 2383 - protein, 108 aa, Homo sapiens
MEFRHVGQAGLKLLTSGDPPALASQSAGITGMSHCTRPRRVHFITAITTITACGNYKVKSTVPRTLHKLSHLILTTTLLGRHSLSAVKKARSERSRCTATMLSHTSIW

SEQ ID NO: 2384 - protein, 12 aa, Homo sapiens
MEGLSTWLTPTV

SEQ ID NO: 2385 - protein, 26 aa, Homo sapiens
MEGPHFHILRLSMFSIHSSTHKVRIH

SEQ ID NO: 2386 - protein, 23 aa, Homo sapiens
MEGPWVNSCVRKETEAGLGRGRS

SEQ ID NO: 2387 - protein, 87 aa, Homo sapiens
MEGTGTGRGGHSLQANKLPLLKIHNVQRGGGPMFHGLSVAAIAGDKDSQCSHEFPDYGLIFPQDHKCPPTEQGVDGWVGKGVLADEF

SEQ ID NO: 2388 - protein, 26 aa, Homo sapiens
MEHRVTLRPGPQGWEGSPASDRTHQG

SEQ ID NO: 2389 - protein, 53 aa, Homo sapiens
MEKAEPAATCIHHGAPPLSPSADFETGLCWWVPAGKHGPLPGAALPVWPHPQS

SEQ ID NO: 2390 - protein, 23 aa, Homo sapiens
MEKEESISNPLWAEQKFINIYIF

SEQ ID NO: 2391 - protein, 12 aa, Homo sapiens
MEKIKLSHKASL

SEQ ID NO: 2392 - protein, 53 aa, Homo sapiens [sequence omitted]

SEQ ID NO: 2393 - protein, 49 aa, Homo sapiens
MEKTYIVSLKLPKSLAIMVSSFLKTESMAGAVAHACNPSNLGHRGRRIT

SEQ ID NO: 2394 - protein, 15 aa, Homo sapiens
MELERINHLLVVNIY

SEQ ID NO: 2395 - protein, 17 aa, Homo sapiens
MELFFFRNFFHFCFYYF

SEQ ID NO: 2396 - protein, 42 aa, Homo sapiens
MELHRVSQAGCELLSSGNPPASASQSAGITSVSHCAQPEFES

SEQ ID NO: 2397 - protein, 24 aa, Homo sapiens
MELLLIELCPELRVHLDQLKAGQV

SEQ ID NO: 2398 - protein, 13 aa, Homo sapiens
MELLSDTSLNFHK

SEQ ID NO: 2399 - protein, 17 aa, Homo sapiens
MELLWLKQFICRCLATH

SEQ ID NO: 2400 - protein, 45 aa, Homo sapiens
MELQIGNRVAPWLRTLELEPQVALSPGALALAKLCSLGEPGFLHL

SEQ ID NO: 2401 - protein, 11 aa, Homo sapiens
MELRSRHCTPA

SEQ ID NO: 2402 - protein, 18 aa, Homo sapiens
MELSRAWRQSKGGGLFGR

SEQ ID NO: 2403 - protein, 62 aa, Homo sapiens
MELWVTRVSASSSTGSVSSRGSGARKTLKVKLAAASRRTPKPAMNFRWRRGTWTFRIRILVG

SEQ ID NO: 2404 - protein, 29 aa, Homo sapiens
MEMAVLCYQIPFFSKLQIMYFRDFFKVAK

SEQ ID NO: 2405 - protein, 12 aa, Homo sapiens
MEMFRPPSAQAG

SEQ ID NO: 2406 - protein, 40 aa, Homo sapiens
MEMINQLCPACRPYLLSRSNHPLIICPSSSGVAGLNPRTM

SEQ ID NO: 2407 - protein, 19 aa, Homo sapiens
MEMYNGTVSLEKLCRFFKN

SEQ ID NO: 2408 - protein, 50 aa, Homo sapiens
MENLVKPVTNSGIIQVNNPMNTSLNRVSVFWKFKLNSVKTICAQRLAKKQ

SEQ ID NO: 2409 - protein, 55 aa, Homo sapiens
MENNSQKGEGRTNKPTGVSYRRGWTPPLRGRRQLLASFLPDSSQLFCRLLCPEGS

SEQ ID NO: 2410 - protein, 39 aa, Homo sapiens
MENNSQKGEGRTNKPTGVSYRRGWTPPLRGRRQLMVGSC

SEQ ID NO: 2411 - protein, 18 aa, Homo sapiens
MENVIFERQVSITNQIDV

SEQ ID NO: 2412 - protein, 47 aa, Homo sapiens
MEPAELGWRRSPFPRAGLGVRVGGLECALSPSSCPCGKQREPPALQL

SEQ ID NO: 2413 - protein, 90 aa, Homo sapiens
MEPHPSAPQLTLKLASVGGSPLGNMAPYLELLFQSGLIHSPKGLGANGSPKEATSNGNEGPTWPPGPGHMSSFACSPGFPSVPWNAQSSL

SEQ ID NO: 2414 - protein, 64 aa, Homo sapiens
MEPSSATFTRGTSNGPSSVSSSISLSSALGVLLPSCSLVWTGVDGFSVFFSCSSEEVIGLLSGR

SEQ ID NO: 2415 - protein, 19 aa, Homo sapiens
MEPSWKTHFWISSRKTSPT

SEQ ID NO: 2416 - protein, 15 aa, Homo sapiens
MEQEFFIKCISSILV

SEQ ID NO: 2417 - protein, 44 aa, Homo sapiens
MEQHITTNTQVITGVTSTASSSCFSGPSSRLCFMYFFTSRLPAQ

SEQ ID NO: 2418 - protein, 66 aa, Homo sapiens
MEQHITTNTQVITGVTSTASSSCFSGPSSRLCFMYLCCSGRLAVPARVRAARPRHSTRTMRNSLLH

SEQ ID NO: 2419 - protein, 250 aa, Homo sapiens [sequence omitted]

SEQ ID NO: 2420 - protein, 17 aa, Homo sapiens
MEQIWSLSCILPFSTSI

SEQ ID NO: 2421 - protein, 15 aa, Homo sapiens
MEQLERIYTDTGSVN

SEQ ID NO: 2422 - protein, 259 aa, Homo sapiens
MEQRCLCVRVELTFTHLDCTSDDHKERGLHEIPQAPGFLNLEQQAFSKLLDQHFSDESLGAVFCHIPHLSSQGTKLPYVPQALSGSGDDDHVLEAVVFLYQGFDFWAVLGLEFIVAIKKEKNPLPQLQQHGHECLLPDCARYIQELITEGFKKSTLGPAETEEEDEFELGQSLALSGAPEHGNSLQQSGLAFARFPFNDAGALKSLQEAIQGQLLHAVMVLVLPPQDRFCEGAFQVKNNVNIFTKGIKVQKRWGMVQVL

SEQ ID NO: 2423 - protein, 19 aa, Homo sapiens
MEQSLMSATHGGRAGEANP

SEQ ID NO: 2424 - protein, 22 aa, Homo sapiens
MERNVENPWGVKSCLKHHLSNF

SEQ ID NO: 2425 - protein, 33 aa, Homo sapiens
MERQLPPWNFLESGQKTGFLELGRPRFYKEIRI

SEQ ID NO: 2426 - protein, 34 aa, Homo sapiens
MESCHRSFQRQNQNTWALELGKIFLLDLAQEKDG

SEQ ID NO: 2427 - protein, 52 aa, Homo sapiens
MESCSVTQAGMQWSAAQYNLCLPGSSDSPASASRVAGTTGTCHHVRLIFCTF

SEQ ID NO: 2428 - protein, 52 aa, Homo sapiens [sequence omitted]

SEQ ID NO: 2429 - protein, 18 aa, Homo sapiens
MESELVPSYRNLSCCLAA

SEQ ID NO: 2430 - protein, 11 aa, Homo sapiens
MESFCSLDPSI

SEQ ID NO: 2431 - protein, 32 aa, Homo sapiens
MESHSVARLEGTISAHCNLHLLGSSTSPSSAS

SEQ ID NO: 2432 - protein, 91 aa, Homo sapiens
MESHSVTQAGVQWHDLGSPQPPPPGFKRFSCLSLLSSWDYRHVPPRLANFVFLVETGFLHVGQAGLELPNSGDPPALASQSAGITGVSHRT

SEQ ID NO: 2433 - protein, 34 aa, Homo sapiens
MESHWLPRLECSSVISAHCSLHLPSSRDSPASAS

SEQ ID NO: 2434 - protein, 16 aa, Homo sapiens
MESIIVTIKLPRVFRI

SEQ ID NO: 2435 - protein, 12 aa, Homo sapiens
MESRSVALAGVQ

SEQ ID NO: 2436 - protein, 31 aa, Homo sapiens
MESSARFHTSRYSAGVLMILLTKGTFRFCEA

SEQ ID NO: 2437 - protein, 11 aa, Homo sapiens
MESSWKAQFRI

SEQ ID NO: 2438 - protein, 16 aa, Homo sapiens
MESVRFVKVCGGHFSH

SEQ ID NO: 2439 - protein, 19 aa, Homo sapiens
METDDSFIFWHFVVFFFRI

SEQ ID NO: 2440 - protein, 80 aa, Homo sapiens
METELSHTSRKESFLQFRFMVFGAEVVLKRKENAGNCGLLLSPWRMVTINTDIFAKLCWDMLHVAPLLFPDHLESSAIQQ

SEQ ID NO: 2441 - protein, 12 aa, Homo sapiens
METLKAEKGGRS

SEQ ID NO: 2442 - protein, 16 aa, Homo sapiens
METLQLLHLPCHLHLC

SEQ ID NO: 2443 - protein, 40 aa, Homo sapiens
METSSYLRRDRTAGLPTQHLQLSLLSMRQRALSLQDSRKS

SEQ ID NO: 2444 - protein, 17 aa, Homo sapiens
MEVIHPPWPPKVLGLQA

SEQ ID NO: 2445 - protein, 11 aa, Homo sapiens
MEVKTKITDPF

SEQ ID NO: 2446 - protein, 11 aa, Homo sapiens
MEVPQSMTSMT

SEQ ID NO: 2447 - protein, 30 aa, Homo sapiens
MEVRLAVSCPNSKVKYDQRTLRLISLDTCI

SEQ ID NO: 2448 - protein, 14 aa, Homo sapiens
MEVSLWETEVAGWR

SEQ ID NO: 2449 - protein, 21 aa, Homo sapiens
MEWISLHASKTAPLASPSHFQ

SEQ ID NO: 2450 - protein, 68 aa, Homo sapiens [sequence omitted]

SEQ ID NO: 2451 - protein, 30 aa, Homo sapiens
MFASPSAMIVSFLRPPQPYRTVIQFNLFSL

SEQ ID NO: 2452 - protein, 42 aa, Homo sapiens
MFAVPAAATGRRFSLLFWLFLFFFLFFFFFFLRLGFLKVFFF

SEQ ID NO: 2453 - protein, 12 aa, Homo sapiens
MFAVTIICRTLN

SEQ ID NO: 2454 - protein, 13 aa, Homo sapiens
MFCIFSRDGVSLC

SEQ ID NO: 2455 - protein, 29 aa, Homo sapiens
MFCKLPPTPLQIILFKNIRLPLASTYVHL

SEQ ID NO: 2456 - protein, 194 aa, Homo sapiens [sequence omitted]

SEQ ID NO: 2457 - protein, 15 aa, Homo sapiens
MFCRDEVSLCCPGWS

SEQ ID NO: 2458 - protein, 48 aa, Homo sapiens
MFCRDGGRPVLPKLVWNSWPQGFVCPSLASESVGIIGVSHHAQPKLIF

SEQ ID NO: 2459 - protein, 40 aa, Homo sapiens
MFCRVRNLAGLVSYTALIFLYDPGGKPDVAVIIPFYRQRH

SEQ ID NO: 2460 - protein, 124 aa, Homo sapiens
MFCRVRNLAGLVSYTALIFVMLPLMSALMGVNTGDPRQSKKGGRWDTASRKGPVSICLSAGSGFSKCSASSAISGSRPAVMPQPAPRASTPPPRPPPSAPGPSQPPAAGSGDASVATSARTAPS

SEQ ID NO: 2461 - protein, 88 aa, Homo sapiens
MFDSEQVSGDDVPAGCIQLLPVFAQETAQGQVARQKLLIELHSTTGIGCREGGRAAVQPGLHGMSERILGEGVGHKACHCCHQAEGSP

SEQ ID NO: 2462 - protein, 12 aa, Homo sapiens
MFFAFDHGHHRN

SEQ ID NO: 2463 - protein, 59 aa, Homo sapiens
MFFNSEMYILATVSSLSSFSMDFIRCWKRALQASTSSSKRKRSATENSTESRLSCRKSS

SEQ ID NO: 2464 - protein, 15 aa, Homo sapiens
MFFPTLAFSSLSMAP

SEQ ID NO: 2465 - protein, 23 aa, Homo sapiens
MFFPYFVFVNPLMKSRRLVLLFI

SEQ ID NO: 2466 - protein, 47 aa, Homo sapiens
MFFSGGELPIAINRRDYYGSIIDKKSARFRSTCNNTETNLKIIKYLG

SEQ ID NO: 2467 - protein, 35 aa, Homo sapiens
MFGCLLQSQERESFILILDWIYCQSNSFLKKDASL

SEQ ID NO: 2468 - protein, 44 aa, Homo sapiens
MFGTVFQVSEVFHLSSILKVFINAYFLFEWKNCRRLATSLINCF

SEQ ID NO: 2469 - protein, 37 aa, Homo sapiens
MFHCLLASVDSVEKLVCHLFGDQSIHAQPKSIFSGRF

SEQ ID NO: 2470 - protein, 49 aa, Homo sapiens
MFHHTQLIFGKDGVLPYCPGWSRTPGFKQSTQRSKVLGLCCEKLSVGRS

SEQ ID NO: 2471 - protein, 29 aa, Homo sapiens
MFHLLDLSSYFLWHHLVCSSICCIFYKLC

SEQ ID NO: 2472 - protein, 37 aa, Homo sapiens
MFIIFKASSSSIIYIHIGSCPISMDSICSKSCKPFSW

SEQ ID NO: 2473 - protein, 16 aa, Homo sapiens
MFIMAQVRKQLRKKYL

SEQ ID NO: 2474 - protein, 29 aa, Homo sapiens
MFINLLSSWLITPLGSEDIPKHFHLKYLL

SEQ ID NO: 2475 - protein, 12 aa, Homo sapiens
MFISSLISRVPK

SEQ ID NO: 2476 - protein, 17 aa, Homo sapiens
MFIVKKDTPDLSGHQNI

SEQ ID NO: 2477 - protein, 29 aa, Homo sapiens
MFKERNKMERNVENPWGVKSCLKHHLSNF

SEQ ID NO: 2478 - protein, 15 aa, Homo sapiens
MFKHKRYICQIASPP

SEQ ID NO: 2479 - protein, 16 aa, Homo sapiens
MFKLYIYSLKHSVKSG

SEQ ID NO: 2480 - protein, 18 aa, Homo sapiens
MFKVCLFKPSILQTISLE

SEQ ID NO: 2481 - protein, 12 aa, Homo sapiens
MFKVVQTIFLVK

SEQ ID NO: 2482 - protein, 50 aa, Homo sapiens
MFLDFFHYLFFKLLAFLWCECVCFGNKWDDIHFFMQTLHKLNIQWFKSMS

SEQ ID NO: 2483 - protein, 36 aa, Homo sapiens
MFLEFSNQIHLQGTACLGMFLISLLSSLVLHTGTIS

SEQ ID NO: 2484 - protein, 83 aa, Homo sapiens
MFLFIFNLWQHRTDCGPPMHFWCRELPFSTSPSPIAIPTSCPIKEYFRCKLNMPRGLLFMKCLVGLRMGGRLDTAESSFWVTL

SEQ ID NO: 2485 - protein, 15 aa, Homo sapiens
MFLFIILLFLVILKI

SEQ ID NO: 2486 - protein, 22 aa, Homo sapiens
MFLHPLEVRPLAWVLTTLQRMK

SEQ ID NO: 2487 - protein, 52 aa, Homo sapiens [sequence omitted]

SEQ ID NO: 2488 - protein, 25 aa, Homo sapiens
MFLIFLLIFLLIDFGEFLHLKVVYF

SEQ ID NO: 2489 - protein, 28 aa, Homo sapiens
MFLNLYYQPRESLYQTGRKPLTTTEEVN

SEQ ID NO: 2490 - protein, 55 aa, Homo sapiens
MFLPMAFIMEFKRGSPGPPHDSCELIKNSNDGGEDGGGDDGNDRCSPQKALMPGD

SEQ ID NO: 2491 - protein, 40 aa, Homo sapiens
MFLQGPPFLHLPDEKLPAGISGNRQEVESWKLVSLLTSVE

SEQ ID NO: 2492 - protein, 20 aa, Homo sapiens
MFLSPQQLKTSLGNSLGNRF

SEQ ID NO: 2493 - protein, 18 aa, Homo sapiens
MFLWFFLLLFFFFFFDLR

SEQ ID NO: 2494 - protein, 16 aa, Homo sapiens
MFLWFSLKLFVMLDRG

SEQ ID NO: 2495 - protein, 65 aa, Homo sapiens
MFNECLLCARHCSQTVFVLYDNQYHTAFIHSFIQHIFNECLLCARHCSQTLIVLRYNQYYTAFIH

SEQ ID NO: 2496 - protein, 11 aa, Homo sapiens
MFNIFLSLAFL

SEQ ID NO: 2497 - protein, 12 aa, Homo sapiens
MFNRDYILFCFY

SEQ ID NO: 2498 - protein, 11 aa, Homo sapiens
MFNSCFENFIV

SEQ ID NO: 2499 - protein, 19 aa, Homo sapiens
MFNWSFEWKLMTVLYSGTL

SEQ ID NO: 2500 - protein, 18 aa, Homo sapiens
MFPAVEGEKDTNVFLCLN

SEQ ID NO: 2501 - protein, 62 aa, Homo sapiens
MFPDARLATCWQKGRSHCPKPHSLGKCMIITIGVKGSAWNCWCPVQGLPEKVRPNPRPLPTT

SEQ ID NO: 2502 - protein, 27 aa, Homo sapiens
MFPFIVVKCTLHKFTILAVSKCIVLWH

SEQ ID NO: 2503 - protein, 82 aa, Homo sapiens
MFPGAAGQGLGGLRGTGRAVLQVGRGGPCPWKAPEEGQWVPQSTQPWAQGLPVLSTQKRSSREAGQWLRRFPGTTPTVRAGE

SEQ ID NO: 2504 - protein, 28 aa, Homo sapiens
MFPLGVYSFSPSLPKRLRRARLPDRSFS

SEQ ID NO: 2505 - protein, 11 aa, Homo sapiens
MFPRLKYHRLK

SEQ ID NO: 2506 - protein, 17 aa, Homo sapiens
MFPRLVLNPWIQVILLP

SEQ ID NO: 2507 - protein, 13 aa, Homo sapiens
MFPTLTSASINFV

SEQ ID NO: 2508 - protein, 32 aa, Homo sapiens [sequence omitted]

SEQ ID NO: 2509 - protein, 12 aa, Homo sapiens
MFQGLACPNTAR

SEQ ID NO: 2510 - protein, 17 aa, Homo sapiens
MFQQTVNLELLCWMILL

SEQ ID NO: 2511 - protein, 15 aa, Homo sapiens
MFRPPWPPKVLGLQA

SEQ ID NO: 2512 - protein, 67 aa, Homo sapiens [sequence omitted]

SEQ ID NO: 2513 - protein, 49 aa, Homo sapiens
MFRTTFLSPQTPHQIQKMSPQHASWAVSDFSLDAFWSATAVLSPVRGRQ

SEQ ID NO: 2514 - protein, 12 aa, Homo sapiens
MFSAGSMRSKMS

SEQ ID NO: 2515 - protein, 15 aa, Homo sapiens
MFSAWDDPEEKSKNS

SEQ ID NO: 2516 - protein, 21 aa, Homo sapiens
MFSFCDSTEQNYLSWFLLQFT

SEQ ID NO: 2517 - protein, 15 aa, Homo sapiens
MFSHKKCSLMPSHNL

SEQ ID NO: 2518 - protein, 27 aa, Homo sapiens
MFSHTAHIHMVSLQCEFFDVEQGMNYD

SEQ ID NO: 2519 - protein, 13 aa, Homo sapiens
MFSIFSRDGVLPC

SEQ ID NO: 2520 - protein, 14 aa, Homo sapiens
MFSIHSSTHKVRIH

SEQ ID NO: 2521 - protein, 66 aa, Homo sapiens
MFSKNVFCGATSPLLPPGILGLESSGQDPRRGRGGCRQRRWRKRRKRWKRRLSRKKRGRGGGDGVP

SEQ ID NO: 2522 - protein, 87 aa, Homo sapiens
MFSLFYWITVINHSIAPSIPLNSTNSEEDSINHIFTLDLLSGECQLNLISSKKLNIPFHIHHRSIFHEAELLNQMFENQSGGKLFIS

SEQ ID NO: 2523 - protein, 23 aa, Homo sapiens
MFSLLHQLATLPSLLLFPGLLIP

SEQ ID NO: 2524 - protein, 23 aa, Homo sapiens
MFSNFFFSTLNCFIQQCRFSSSS

SEQ ID NO: 2525 - protein, 34 aa, Homo sapiens
MFSPESEFPIAICMCIDGHGKRGHYRTEDIAEMQ

SEQ ID NO: 2526 - protein, 21 aa, Homo sapiens
MFSRDGVSPCWPGWSRTPDLR

SEQ ID NO: 2527 - protein, 71 aa, Homo sapiens
MFSRFIYVVACISISFPFYCHIVFHCVDRKHFFFFLRQGLTLSPSWSAVVQPLTTASTSRAQVIIPPQLPE

SEQ ID NO: 2528 - protein, 27 aa, Homo sapiens
MFSRLVSTSQAQVILLLWPSKVLGLQV

SEQ ID NO: 2529 - protein, 39 aa, Homo sapiens
MFSSPKLKNACEMIFLNPCNRPFRCCPQEKRFLKKQIEK

SEQ ID NO: 2530 - protein, 11 aa, Homo sapiens
MFSSTFFTKEP

SEQ ID NO: 2531 - protein, 20 aa, Homo sapiens
MFSTDGVSPCWSGWLDAHFL

SEQ ID NO: 2532 - protein, 15 aa, Homo sapiens
MFSTFFHVFILSSFA

SEQ ID NO: 2533 - protein, 42 aa, Homo sapiens
MFTTSIETILSNLSNMRKALLAKASCQSRREAPLFCWQKQTS

SEQ ID NO: 2534 - protein, 19 aa, Homo sapiens
MFVCCISVRISEFVSNKVF

SEQ ID NO: 2535 - protein, 16 aa, Homo sapiens
MFVEDNDGGSDHTAPL

SEQ ID NO: 2536 - protein, 20 aa, Homo sapiens
MFVNLMSLSFKTTKKYIIQL

SEQ ID NO: 2537 - protein, 21 aa, Homo sapiens
MFVPCPRPQVRAQLRNFSRWC

SEQ ID NO: 2538 - protein, 22 aa, Homo sapiens
MFVTLFITVVFSSMSYLTYNQV

SEQ ID NO: 2539 - protein, 15 aa, Homo sapiens
MFVTVLYRAFFFLVA

SEQ ID NO: 2540 - protein, 44 aa, Homo sapiens
MFWGKKGMNNFWSRRSNTCVHPFKWVRRHPLSHRVRLPPMLYII

SEQ ID NO: 2541 - protein, 57 aa, Homo sapiens
MFWKCQHLGIPTVPPRLSSSWKWYNCLCETLCPDLGFRKRSLYPRDSKKSCPVSLGR

SEQ ID NO: 2542 - protein, 39 aa, Homo sapiens [sequence omitted]

SEQ ID NO: 2543 - protein, 28 aa, Homo sapiens
MFYTCIFIFIHVLIHSKNIYGMPTMYQH

SEQ ID NO: 2544 - protein, 48 aa, Homo sapiens
MGAAAIMFAVPAAATGRRFSLLFWLFLFFFLFFFFFFLRLGFLKVFFF

SEQ ID NO: 2545 - protein, 22 aa, Homo sapiens
MGAAMTDGGIRPAGLRGACEPG

SEQ ID NO: 2546 - protein, 35 aa, Homo sapiens
MGANIYNLDCNDSKIPNISQCHSQNAFPYLVHPGL

SEQ ID NO: 2547 - protein, 45 aa, Homo sapiens
MGAPRRALAGEDVSVGRVGRCGDHPDHGDGGGLLHDVDGVARGLL

SEQ ID NO: 2548 - protein, 24 aa, Homo sapiens
MGCGICRDWLTRDIVPSKEEVSSA

SEQ ID NO: 2549 - protein, 15 aa, Homo sapiens
MGCNKMPTREIMTLP

SEQ ID NO: 2550 - protein, 40 aa, Homo sapiens
MGCQIHHVPLMSMKLVFHHFHIIRNLSLCLQCVLSRKKPR

SEQ ID NO: 2551 - protein, 16 aa, Homo sapiens
MGDFYFVVSISLYIFF

SEQ ID NO: 2552 - protein, 24 aa, Homo sapiens
MGDGGLGVKAASGVCRSQPQRGKA

SEQ ID NO: 2553 - protein, 21 aa, Homo sapiens
MGDRGCWLEVKGVALGLYSSM

SEQ ID NO: 2554 - protein, 65 aa, Homo sapiens
MGEGEWDYLASTCQPWYSGLELPCWNGFESFSTTLKIRSMWWHQREADNWSLWQPQRLLILHQCH

SEQ ID NO: 2555 - protein, 18 aa, Homo sapiens
MGENIPNRGNIKGKGFIY

SEQ ID NO: 2556 - protein, 140 aa, Homo sapiens
MGERGASSSWTSSNSVLAMMGDRRPLTVLALELVRERKSVHASSSSLLRDVGLPDHLESWEGLSSADSGAVCRAAFFLAVRPRLLVYLLLLSMETARRRGAFPLFPPSGLMIHQELLPVPSFWTRMNRLCSDRLCRMEFF

SEQ ID NO: 2557 - protein, 151 aa, Homo sapiens
MGERGASSSWTSSNSVLAMMGDRRPLTVLALELVRERKSVHASSSSLLRDVGLPGHLESWEGLSSADSGAVCRAAFFLAARPRLLVYLLLLSMETARRRGAFPLFPPSGLMIHQELLPVPSFWTRMNRLCSDRLCRMEFCLRQGPPPLAPF

SEQ ID NO: 2558 - protein, 153 aa, Homo sapiens
MGERGASSSWTSSNSVLAMMGDRRPLTVLALELVRERKSVHASSSSLLRDVGLPGHLESWEGLSSADSGAVCRAAFFLAARPRLLVYLLLLSMETARRRGAFPLFPPSGLMIHQELLPVPSFWTRMNRLCSDRLCRMEFFQPAELLLSPLSLK

SEQ ID NO: 2559 - protein, 191 aa, Homo sapiens
MGERGASSSWTSSNSVLAMMGDRRPLTVLALELVRERKSVHASSSSLLRDVGLPGHLESWEGLSSADSGAVCRAAFFLAARPRLLVYLLLLSMETARRRGAFPLFPPSGLMIHQELLPVPSFWTRMNRLCSDRLCRMEFLWRLSTHPDTSCMCFPWNTERFLSGSNMWYQFIFLSNDNKKSAHFKNKKRVV

SEQ ID NO: 2560 - protein, 144 aa, Homo sapiens
MGERGASSSWTSSNSVLAMMGDRRPLTVLALELVRERKSVHASSSSLLRDVGLPGHLESWEGLSSADSGAVCRAAFFLAARPRLLVYLLLLSMETARRRGAFPLFPPSGLMIHQELLPVPSFWTRMNRLCSDRLCRMEFSPLQS

SEQ ID NO: 2561 - protein, 195 aa, Homo sapiens
MGERGASSSWTSSNSVLAMMGDRRPLTVLALELVRERKSVHASSSSLLRDVGLPGHLESWEGLSSADSGAVCRAAFFLAARPRLLVYLLLLSMETARRRGAFPLFPPSGLMIHQELLPVPSFWTRMNRLCSDRLCRMEFSSVLSGESSKCTPVRSPFPRRRPLPPLLTWPCPKLLGSLIHPSETVPRCPDSGDQR

SEQ ID NO: 2562 - protein, 163 aa, Homo sapiens
MGERGASSSWTSSNSVLAMMGDRRPLTVLALELVRERKSVHASSSSLLRDVGLPGHLESWEGLSSADSGAVCRAAFFLAARPRLLVYLLLLSMETARRRGAFPLFPPSGLMIHQELLPVPSFWTRMNRLCSDRLCRMEFVFRASYTLSQKVPGRPLPGKDFKL

SEQ ID NO: 2563 - protein, 165 aa, Homo sapiens
MGERGASSSWTSSNSVLAMMGDRRPLTVLALELVRERKSVHASSSSLLRDVGLPGHLESWEGLSSADSGAVCRAAFFLAARPRLLVYLLLLSMETARRRGAFPLFPPSGLMIHQELLPVPSFWTRMNRLCSDRLCRMELIGRLYLRISKRQHCVIQKSPKFPIRI

SEQ ID NO: 2564 - protein, 24 aa, Homo sapiens
MGERQGPDLSAFRDPPPSQGQGPS

SEQ ID NO: 2565 - protein, 24 aa, Homo sapiens
MGEVIHCMHLSFCKPNKSTGPCCL

SEQ ID NO: 2566 - protein, 31 aa, Homo sapiens
MGFAMLTRLVSNFRPQVICPPRPLKVLGLQT

SEQ ID NO: 2567 - protein, 32 aa, Homo sapiens
MGFCHIAQDGLELLGSSNPPSVPKCWDYVAKS

SEQ ID NO: 2568 - protein, 42 aa, Homo sapiens
MGFCHVGQAGLELLTSSHLPASASQSAGITGMSHCARLERFF

SEQ ID NO: 2569 - protein, 30 aa, Homo sapiens
MGFCHVGQAGLKLLTSSDPPASASSNVLEL

SEQ ID NO: 2570 - protein, 13 aa, Homo sapiens
MGFCHVGQGGLES

SEQ ID NO: 2571 - protein, 67 aa, Homo sapiens
MGFCHVGWAGLELLTSGDPPTSASQSAGIIGVSHHTGPTAFLKDLPKPSTLKCPGLLLTSWLIPLII

SEQ ID NO: 2572 - protein, 37 aa, Homo sapiens
MGFCLARASFILRVNIRFITGFLLGVPCLLGKVFVCL

SEQ ID NO: 2573 - protein, 31 aa, Homo sapiens
MGFCMLPRLVSNFWAQVICPPWPPKVLGLRA

SEQ ID NO: 2574 - protein, 12 aa, Homo sapiens
MGFCPFLLNRWR

SEQ ID NO: 2575 - protein, 67 aa, Homo sapiens [sequence omitted]

SEQ ID NO: 2576 - protein, 41 aa, Homo sapiens
MGFFHVVQAGLKLLGSSNPLALASQSWDYRCEPPLLAYNEV

SEQ ID NO: 2577 - protein, 61 aa, Homo sapiens
MGFGYQQHAAHEVCGGHPLRALAFSVPPSLLYFLIGVPAIYSQGDVIAVNTEVTVVFVQGL

SEQ ID NO: 2578 - protein, 15 aa, Homo sapiens
MGFHCISQASLELTS

SEQ ID NO: 2579 - protein, 46 aa, Homo sapiens
MGFHCVGQAGLELLTSSDLPASASQSAGIMGMSHHTQLIYCILTIK

SEQ ID NO: 2580 - protein, 16 aa, Homo sapiens
MGFHCVSHVGLDLLTL

SEQ ID NO: 2581 - protein, 16 aa, Homo sapiens
MGFHCVSQDDLDLLTS

SEQ ID NO: 2582 - protein, 16 aa, Homo sapiens
MGFHCVSQDGLNLLTL

SEQ ID NO: 2583 - protein, 16 aa, Homo sapiens
MGFHCVSQNGLDLLTS

SEQ ID NO: 2584 - protein, 45 aa, Homo sapiens
MGFHHIAQAGLKLLTLGNPLASASQSAGITGVSHCTRPTPYTFIL

SEQ ID NO: 2585 - protein, 40 aa, Homo sapiens
MGFHHIGQAGLDLLTSGGPTASASQNAEIVGVSHRSWQLR

SEQ ID NO: 2586 - protein, 56 aa, Homo sapiens
MGFHHIGQAGLELLTLGDPPASASQSAGITGVSHHAQPLFGIFIYKFTYICRKTRT

SEQ ID NO: 2587 - protein, 16 aa, Homo sapiens
MGFHHIGQAGLNLLAL

SEQ ID NO: 2588 - protein, 54 aa, Homo sapiens
MGFHHISQAGLELLTSGDPPALASQSAGITGVSHRTWPQADVSDWITFSLILYS

SEQ ID NO: 2589 - protein, 11 aa, Homo sapiens
MGFHHLGQAGL

SEQ ID NO: 2590 - protein, 46 aa, Homo sapiens
MGFHHVALAGLELLSSGNLPTLASQNARVTGVSHRAWPRLLPFNHE

SEQ ID NO: 2591 - protein, 43 aa, Homo sapiens
MGFHHVDQTSLELLTSGDPPASASQSVGITGMSHCTQPSTAYF

SEQ ID NO: 2592 - protein, 23 aa, Homo sapiens
MGFHHVGLAGFEPQPPKVLRLQV

SEQ ID NO: 2593 - protein, 76 aa, Homo sapiens
MGFHHVGPDLELLTSSDLPTLASQSAGIIGVSHAPGRFAILAGLPGLTTYCACVCVNTYVYVFVCIHRHTHIYINA

SEQ ID NO: 2594 - protein, 34 aa, Homo sapiens
MGFHHVGQADLELLASSDLPSSASLSAGIIDVSH

SEQ ID NO: 2595 - protein, 62 aa, Homo sapiens
MGFHHVGQAGIKFLTSGDPSASASQSARITGVSHCAQPFLITLNKDWLWWLIAVPTGIIVFR

SEQ ID NO: 2596 - protein, 11 aa, Homo sapiens
MGFHHVGQAGL

SEQ ID NO: 2597 - protein, 16 aa, Homo sapiens
MGFHHVGQAGLEFLTS

SEQ ID NO: 2598 - protein, 15 aa, Homo sapiens
MGFHHVGQAGLELLT

SEQ ID NO: 2599 - protein, 16 aa, Homo sapiens
MGFHHVGQAGLELLTS

SEQ ID NO: 2600 - protein, 44 aa, Homo sapiens
MGFHHVGQAGLELLTSGDLPALTSQSVGITGVSHHAWPDIPTFL

SEQ ID NO: 2601 - protein, 43 aa, Homo sapiens
MGFHHVGQAGLELLTSGDLPASASQSGGITGMSHRIRPDFRCF

SEQ ID NO: 2602 - protein, 33 aa, Homo sapiens
MGFHHVGQAGLELLTSGDPPSLASQSAGINLCI

SEQ ID NO: 2603 - protein, 38 aa, Homo sapiens
MGFHHVGQAGLELLTSSDLPTSAPQSAGITGMSHRVQP

SEQ ID NO: 2604 - protein, 45 aa, Homo sapiens
MGFHHVGQAGLEPLTSNVSPALASQSAGITGVSHHTQPRHLLCGI

SEQ ID NO: 2605 - protein, 43 aa, Homo sapiens
MGFHHVGQAGLKLLKSGDPPASASQNVGITGVSHRTWPFICFK

SEQ ID NO: 2606 - protein, 56 aa, Homo sapiens
MGFHHVGQAGLKLLTSGDSPTSASQSARITGVNHCARPSTFLRLQRKAGRCSSSRL

SEQ ID NO: 2607 - protein, 41 aa, Homo sapiens
MGFHHVGQAGLKLLTSGNSPASASQSAGITGVSHHSQPNNL

SEQ ID NO: 2608 - protein, 43 aa, Homo sapiens [sequence omitted]

SEQ ID NO: 2609 - protein, 41 aa, Homo sapiens
MGFHHVGQAGLMHISYRYIGKLLPNHNKHCVQVFKMSLDTH

SEQ ID NO: 2610 - protein, 17 aa, Homo sapiens
MGFHHVGQAGSRTPDLR

SEQ ID NO: 2611 - protein, 16 aa, Homo sapiens
MGFHHVGQDGLNLLIS

SEQ ID NO: 2612 - protein, 11 aa, Homo sapiens
MGFHHVGQSGL

SEQ ID NO: 2613 - protein, 65 aa, Homo sapiens
MGFHHVGQSGLEPLTSSDPPALASQSAGIVGVSHCTHLLSVSNPQDIYLGMKLLSHRVCEYSLLI

SEQ ID NO: 2614 - protein, 44 aa, Homo sapiens
MGFHHVGQTGLELLTSSDPPTLASQSAGITGVSHCTRPILAFSM

SEQ ID NO: 2615 - protein, 16 aa, Homo sapiens
MGFHHVSQDGLDLLNL

SEQ ID NO: 2616 - protein, 59 aa, Homo sapiens
MGFHPVGQAGLELLTSSDPPALAFQSAGITGVSHRTRPGTPQILISDPAKNIVTCLNGH

SEQ ID NO: 2617 - protein, 38 aa, Homo sapiens
MGFHRLGQAGLELLTSGDLPALASQSAGITGMSHHALP

SEQ ID NO: 2618 - protein, 45 aa, Homo sapiens
MGFHRVGQAGLELLTSGDPPTLASQSAGIIGMSHRAWRNSFLEAF

SEQ ID NO: 2619 - protein, 36 aa, Homo sapiens
MGFHRVGQAGLELLTSSDPPASASQSAGITGMSHRA

SEQ ID NO: 2620 - protein, 13 aa, Homo sapiens
MGFHTLVRLVSNS

SEQ ID NO: 2621 - protein, 47 aa, Homo sapiens
MGFHYVGQGRSQSLDLVIHPPWPPKMLGLQVSATTPNQKRFFLLILP

SEQ ID NO: 2622 - protein, 16 aa, Homo sapiens
MGFHYVGQNGLDLLTS

SEQ ID NO: 2623 - protein, 36 aa, Homo sapiens
MGFLFYHIVKLHIFQTFMHCYFLNTLLLRNFFYQIP

SEQ ID NO: 2624 - protein, 48 aa, Homo sapiens
MGFLHVGQAGLEFPTSGDPPALASQSAGITGVSYHARPGKLIFYDIIL

SEQ ID NO: 2625 - protein, 42 aa, Homo sapiens
MGFLHVGQAGLELPTSGDPPTSASQSAGITGVSHRTRPQTFF

SEQ ID NO: 2626 - protein, 40 aa, Homo sapiens
MGFLHVGQAGLERAISGDPPAKASQSPGITGVSHHARLAL

SEQ ID NO: 2627 - protein, 38 aa, Homo sapiens
MGFLHVGWAGLELPTSGNPPASACQSAGITGVSHHTQP

SEQ ID NO: 2628 - protein, 65 aa, Homo sapiens
MGFRHVGQAGLELLASSGPPTSASQSAGIIGVSHHTQPRVTCKRSLASVPSNPVPPHPTSPQFSW

SEQ ID NO: 2629 - protein, 93 aa, Homo sapiens [sequence omitted]

SEQ ID NO: 2630 - protein, 16 aa, Homo sapiens
MGFRHVGQAGLELLTS

SEQ ID NO: 2631 - protein, 38 aa, Homo sapiens [sequence omitted]

SEQ ID NO: 2632 - protein, 42 aa, Homo sapiens
MGFRHVGQAGLELLTSSDLPTPAHQSAGITGVSHHTWPRTGF

SEQ ID NO: 2633 - protein, 16 aa, Homo sapiens
MGFRHVGQVGLKLLTS

SEQ ID NO: 2634 - protein, 42 aa, Homo sapiens
MGFRPKPCSPVHFLQKSLELRVIGYLHRLIKFLPMSHLNSNH

SEQ ID NO: 2635 - protein, 58 aa, Homo sapiens
MGFSARARACAGLYLQRIPRVTWTPASQPPAPLGPFLPLIPPAASHRQPSSSFFRRHR

SEQ ID NO: 2636 - protein, 15 aa, Homo sapiens
MGFSRDRVSSCCPGW

SEQ ID NO: 2637 - protein, 13 aa, Homo sapiens
MGFSRVAHRFFCP

SEQ ID NO: 2638 - protein, 13 aa, Homo sapiens
MGFTILARMVSIS

SEQ ID NO: 2639 - protein, 58 aa, Homo sapiens
MGFTMLARLISNSWTQVNHPFWPPKVLGLQEWATMPSLNFSKVLLNKGFAAYLQVLFT

SEQ ID NO: 2640 - protein, 49 aa, Homo sapiens
MGFYHVGQAGLELLTSGDPPASASQSAGIIGVSHCTWPEVMLSKPPELT

SEQ ID NO: 2641 - protein, 48 aa, Homo sapiens
MGFYHVGQTDLQLVTSGDLPASASQSAGITVAHAWPGIAILMRYPFSL

SEQ ID NO: 2642 - protein, 58 aa, Homo sapiens
MGFYYVGRAGLKLLTSGDPPASTSQSAGITGMSHHTRPGLLIYEVLYIILHINIYIYV

SEQ ID NO: 2643 - protein, 13 aa, Homo sapiens
MGGECSLRFVVRG

SEQ ID NO: 2644 - protein, 27 aa, Homo sapiens
MGGLSSFQKSVLISKGSGYLLPHKYEN

SEQ ID NO: 2645 - protein, 81 aa, Homo sapiens [sequence omitted]

SEQ ID NO: 2646 - protein, 39 aa, Homo sapiens
MGGQPDSRVLPPHAGLWQTLGGKAGHTLLAASCKHPWLK

SEQ ID NO: 2647 - protein, 61 aa, Homo sapiens [sequence omitted]

SEQ ID NO: 2648 - protein, 24 aa, Homo sapiens
MGGSCSPSTSHTGNYLYLKRMVFK

SEQ ID NO: 2649 - protein, 23 aa, Homo sapiens
MGGTPGEPVRSSGHFVTVHHQEP

SEQ ID NO: 2650 - protein, 86 aa, Homo sapiens
MGHCSSPHMEMKTKAWVLSLPSEDFKTSGKAAGIPICRSSRILEREDQAVLFIPDIVPQGYRGHHFSVDYLHPSPSNACSWGTDRH

SEQ ID NO: 2651 - protein, 61 aa, Homo sapiens [sequence omitted]

SEQ ID NO: 2652 - protein, 17 aa, Homo sapiens
MGHSSEYQLYRATCLHF

SEQ ID NO: 2653 - protein, 40 aa, Homo sapiens
MGHVGQAGLELLAPSDLPSSAYQNAGITGMSHCTWPAYTL

SEQ ID NO: 2654 - protein, 105 aa, Homo sapiens
MGHVQCNGPLQSLRDVVPNQVVKSRAPGPGHTGCTNDIGEDEVPASGEGPEFTHSDIAVEICRTRTGNPGTKLRIAQPSQHRRQGSHQKADHNGWPCFIFGHLAS

SEQ ID NO: 2655 - protein, 12 aa, Homo sapiens
MGICKNIAINDR

SEQ ID NO: 2656 - protein, 11 aa, Homo sapiens
MGIPIPNFHIG

SEQ ID NO: 2657 - protein, 69 aa, Homo sapiens
MGIPKTDPERAADDQSSKLVVSPEPHTSFSASSFFSKGFQVTLAQMLSSHLAPPFSAFLAFIRVGWADL

SEQ ID NO: 2658 - protein, 12 aa, Homo sapiens
MGIRKILGPRVL

SEQ ID NO: 2659 - protein, 48 aa, Homo sapiens
MGKAVVIHGPHYVFQPLISYPSFSHSWDVYQGPLLYILGTHDDHMRSN

SEQ ID NO: 2660 - protein, 24 aa, Homo sapiens
MGKETPVVSSCKTATHALYNLRNK

SEQ ID NO: 2661 - protein, 66 aa, Homo sapiens [sequence omitted]

SEQ ID NO: 2662 - protein, 28 aa, Homo sapiens
MGKLPENFNFSNCCNWKAFLFIIQTYFF

SEQ ID NO: 2663 - protein, 30 aa, Homo sapiens
MGKPRRTLGTAGINAHTLPSPCSHRESLSR

SEQ ID NO: 2664 - protein, 70 aa, Homo sapiens
MGKRTSLEVSLGELGGEKCRGGRRSFPPLAASRPARPGGWRWARRDLCKTASRAENNSQACRPQSHETKI

SEQ ID NO: 2665 - protein, 12 aa, Homo sapiens
MGKVRSGRLGWA

SEQ ID NO: 2666 - protein, 24 aa, Homo sapiens
MGLCLMPRNVRHALILSSSVPGSN

SEQ ID NO: 2667 - protein, 42 aa, Homo sapiens
MGLGGRKDLGQGNRWSYRAEPDQQRAFPETLRPSLLLPQRLW

SEQ ID NO: 2668 - protein, 52 aa, Homo sapiens
MGLHHVGQAGLELLTSSDPPTSASQSVGITGVSHHAQPGLFLFIVVSCYLNA

SEQ ID NO: 2669 - protein, 13 aa, Homo sapiens
MGLIPLGDHASQT

SEQ ID NO: 2670 - protein, 35 aa, Homo sapiens
MGLLTPVSFPQPSFWAQAWSRASRAITRCCRSSYP

SEQ ID NO: 2671 - protein, 11 aa, Homo sapiens
MGLNWPSPPLV

SEQ ID NO: 2672 - protein, 53 aa, Homo sapiens
MGLQKALPGLRVSASRSRSKGTNASVSSREPWTPGRGLLSLSWDSAGMPSGPY

SEQ ID NO: 2673 - protein, 11 aa, Homo sapiens
MGLRPSTHPAH

SEQ ID NO: 2674 - protein, 29 aa, Homo sapiens
MGLSSMMHFHPWQALSFSVDQEESLIITC

SEQ ID NO: 2675 - protein, 83 aa, Homo sapiens
MGLVGDIGCSLHSLRAPGRMDAEEAGERRRLRNELLPQPLRSSPSRLRPQLTQFCALLLSLTFLHRLPGISMTAERAEQPGFS

SEQ ID NO: 2676 - protein, 37 aa, Homo sapiens
MGLVGDIGCSLHSLSGGAGEGGRSSHERWLGPHAAPS

SEQ ID NO: 2677 - protein, 38 aa, Homo sapiens
MGLVGDIGCSLHSPVLRVIAQFDFLAQAPGDLHDRGAR

SEQ ID NO: 2678 - protein, 21 aa, Homo sapiens
MGLWVAGPAMGLGGAGLQAPG

SEQ ID NO: 2679 - protein, 101 aa, Homo sapiens
MGMGQPWGGGGPRGDNGAIRGEEGTLQKAWVGQCWALVGGSGGAGGRQEALGSGWRAAGPGLQAPWRAEGARRGPGGNPRLEAGPKSASLAAPAGKEENKV

SEQ ID NO: 2680 - protein, 89 aa, Homo sapiens
MGMLDTKYANLSSNFKKSSLSSLINLLLSQTITFPYIVVNVISNIIELQNGYSSAVSQLVVFNSWGSKTCFRFCIMLSKSMSKDLPCKN

SEQ ID NO: 2681 - protein, 38 aa, Homo sapiens
MGMTMLVPHWILRGLNEKIHAKQSLAWHVLRGSHYCYF

SEQ ID NO: 2682 - protein, 76 aa, Homo sapiens
MGPKLKHASGNEAQEDNGEEGDIVDSVLGLHSWDEGRTPDIILDRRTHNDTDSLFLTLLVPRLLAPQGMPQATTGP

SEQ ID NO: 2683 - protein, 68 aa, Homo sapiens
MGPKLKHASGNEAQEDNGEEGDIVDSVLGLHSWDEGRTPDIILDRRTHNDTDSLFLTLQKHLKEKQQL

SEQ ID NO: 2684 - protein, 49 aa, Homo sapiens
MGPLPACLDWPQPGWTQAGTASPPGGAMWAPEPIPGWAWRVWPALPGEK

SEQ ID NO: 2685 - protein, 19 aa, Homo sapiens
MGPLSQRMKVIGNLSPVIY

SEQ ID NO: 2686 - protein, 54 aa, Homo sapiens
MGPRHPIGRPGPPRSVRSWNSFLSDFTYSDHFFFHFSLDLFMADSPSLSRKIVA

SEQ ID NO: 2687 - protein, 68 aa, Homo sapiens
MGPRHPIGRPGPPRSVRSWNSGAGKPERGAVCQELPDGSIPCLDPCRNQNRTLNKLLSAPLPAVTSST

SEQ ID NO: 2688 - protein, 45 aa, Homo sapiens
MGPRHPIGRPGPPRSVRSWNSSLQFCDYSRGQTGNLHGGSLFESV

SEQ ID NO: 2689 - protein, 55 aa, Homo sapiens
MGPSSGSRQLWPRPSPPLSSPGLRSQPPNWTPCPQPLPDPAPPHGSQSARSKTQT

SEQ ID NO: 2690 - protein, 74 aa, Homo sapiens
MGPSSGSRQLWPRPSPPLSSPGLRSQPPNWTPCPQPLPDPAPPHGSQSARSWPGLPQWRPLSLTGSGSHFSVAY

SEQ ID NO: 2691 - protein, 58 aa, Homo sapiens
MGPSSGSRQLWPRPSPPLSSPGLRSQPPNWTPCPQPLPDPAPPHGSQSARYSPHNAAT

SEQ ID NO: 2692 - protein, 14 aa, Homo sapiens
MGPSWPTQCWSFTQ

SEQ ID NO: 2693 - protein, 74 aa, Homo sapiens
MGPYVERRGPYRRPGLGSAGLSSEGQVALAAGRKPWVAGGGQQVPGCRPRGERKARGEARAGTQGWRPALRVLP

SEQ ID NO: 2694 - protein, 36 aa, Homo sapiens
MGQLSCRMFHLLDLSSYFLWHHLVCSSICCIFYKLC

SEQ ID NO: 2695 - protein, 35 aa, Homo sapiens
MGQPSRGAREGTSGSGQGMVRVNGVRRKKGPGTGK

SEQ ID NO: 2696 - protein, 99 aa, Homo sapiens
MGQPWGGGGPRGDNGAIRGEEGTLQKAWVGQCWALVGGSGGAGGRQEALGSGWRAAGPGLQAPWRAEGARRGPGGNPRLEAGPKSASLAAPAGKEENKV

SEQ ID NO: 2697 - protein, 24 aa, Homo sapiens
MGQSCQPTYKTPPIPHPLPWVINW

SEQ ID NO: 2698 - protein, 43 aa, Homo sapiens
MGQWQLLLWNGLQKICKQDQTSHPYQPAGKCAQNLTSNHGFPF

SEQ ID NO: 2699 - protein, 117 aa, Homo sapiens
MGRARQACRQLGEQGEVTPLCEWQKVLAGSILFPLSLTFIKPCHARTVKGKARDTTIRLRQQWGAAAPWLGDSSRLRRGRAPQHYLSVNERVKTTPWSSHRASFTLTSYLLANINLS

SEQ ID NO: 2700 - protein, 28 aa, Homo sapiens
MGRHVMFFPYFVFVNPLMKSRRLVLLFI

SEQ ID NO: 2701 - protein, 14 aa, Homo sapiens
MGRMESSWKAQFRI

SEQ ID NO: 2702 - protein, 43 aa, Homo sapiens
MGRQGASAELGSPEGSSRTLGLECSGLGAGTASRGLAIPRAPG

SEQ ID NO: 2703 - protein, 41 aa, Homo sapiens
MGRQGASAELRAAAARSGSSAQGSVQAPPAEGWRSPGLLAD

SEQ ID NO: 2704 - protein, 135 aa, Homo sapiens
MGRRVDGSAAGAQASGWLRGAPGGGAMGGVVRPGPAGLKCGAGAQGPSWWRRAVPLGASTLSCRARRPPINRPARLFWQRGGGGGRRAAGLRAAGLGWAGRAGGLQGPAVSTPARRSGGSGGAGAAAVCGAARGR

SEQ ID NO: 2705 - protein, 37 aa, Homo sapiens
MGRSWRHCTPDSPRRQKTRSRCRSRMVGTCPTDIQIY

SEQ ID NO: 2706 - protein, 104 aa, Homo sapiens [sequence omitted]

SEQ ID NO: 2707 - protein, 84 aa, Homo sapiens
MGSATEMRIRVRYWSSMTLKREFRSALGNWIFISCRTLFRKIHFCWKVSHTSSRAPRPCMMATHSKAILFKSPDFSMAKILDNT

SEQ ID NO: 2708 - protein, 21 aa, Homo sapiens
MGSCYVAQAGLELLGSSDPPT

SEQ ID NO: 2709 - protein, 36 aa, Homo sapiens [sequence omitted]

SEQ ID NO: 2710 - protein, 32 aa, Homo sapiens
MGSFDICTHCETVTTVKVINIHHLHSYWFFLW

SEQ ID NO: 2711 - protein, 17 aa, Homo sapiens
MGSFFFLKLLVLGEMSF

SEQ ID NO: 2712 - protein, 16 aa, Homo sapiens
MGSHRVSQDGLNLLTL

SEQ ID NO: 2713 - protein, 42 aa, Homo sapiens
MGSLVTRLAQFVHISATDKEGFFDQNQCHRERSQRLCSHARK

SEQ ID NO: 2714 - protein, 40 aa, Homo sapiens
MGSPPCRHVILLHIWQLPMRQVGFRVASSPIAASPEDYIW

SEQ ID NO: 2715 - protein, 13 aa, Homo sapiens
MGSPSFVVHQTFL

SEQ ID NO: 2716 - protein, 54 aa, Homo sapiens
MGSSSVGLGQAEHTRPSASCPLAPRAPCLPTSAQLQTLASNSRPRSLERNLLPN

SEQ ID NO: 2717 - protein, 66 aa, Homo sapiens
MGSWDPGGPHTRRLPTSSGSGSTSATWCSSSSGGRGPRSPRPAAGRSRAQPSSAPLSAGLQGPRQL

SEQ ID NO: 2718 - protein, 100 aa, Homo sapiens
MGSWDPGGPHTRRLPTSSGSGSTSATWCSSSSGGRGPRSPRPAAGRSRAQPSSAPLSAGLQGPRQLRAANFDSFAFVSWKTPRPWFPFAFSLTQRTQEWQ

SEQ ID NO: 2719 - protein, 101 aa, Homo sapiens
MGSWDPGGPHTRRLPTSSGSGSTSATWCSSSSGGRGPRSPRPAAGRSRAQPSSAPLSAGLQGPRQLRAANFDSFAFVSWKTPRPWFPFAFSLTQRTQEWQS

SEQ ID NO: 2720 - protein, 32 aa, Homo sapiens
MGSWVFAYVQTHQILHIIYVPSFAYQLYFSKA

SEQ ID NO: 2721 - protein, 33 aa, Homo sapiens
MGTGTGQDFFTGPCSRKGWLKNASKSILSFWFL

SEQ ID NO: 2722 - protein, 12 aa, Homo sapiens
MGTISVATDSEL

SEQ ID NO: 2723 - protein, 59 aa, Homo sapiens
MGTPVWVPFCWMGAAAIMFAVPAAATGRRFSLLFWLFLFFFLFFFFFFLRLGFLKVFFF

SEQ ID NO: 2724 - protein, 30 aa, Homo sapiens
MGTRARRKKLKLSVGNSGLENRPLSPAFAV

SEQ ID NO: 2725 - protein, 17 aa, Homo sapiens
MGTTKAGSTLASISSGL

SEQ ID NO: 2726 - protein, 23 aa, Homo sapiens
MGTTQMPPTLEWMSKLQCLCTVE

SEQ ID NO: 2727 - protein, 51 aa, Homo sapiens
MGTVIPALQNSCEDESDCASPPFLPSFLPPLSLYIFSLILHNPVAHKGSHS

SEQ ID NO: 2728 - protein, 11 aa, Homo sapiens
MGTVQSTFSSG

SEQ ID NO: 2729 - protein, 155 aa, Homo sapiens
MGVAGLRSLKGTFGDKVYLRVHALQQALHLGPSDSLEPLHPALCQDQPPEAPAELLVLQVGGHGDWVILKQVVRQLTDFDSEVGGDGAVLEGAVLGPTESRAQQQQQEEIGCWAPGWRQHCHFGRGPLMPPVAGSWKGQKNKSRTLMPQPLPCPP

SEQ ID NO: 2730 - protein, 27 aa, Homo sapiens
MGVCICPNSSNFTHYICAIICISIILQ

SEQ ID NO: 2731 - protein, 139 aa, Homo sapiens [sequence omitted]

SEQ ID NO: 2732 - protein, 27 aa, Homo sapiens
MGVGVKVAVFEQPRRCYEHCSGAPAAS

SEQ ID NO: 2733 - protein, 76 aa, Homo sapiens
MGVLILPRSARMSGILSATATVTVKVADRGGWPWSSTATTRLCLSASLSSRARAVRTSPVCSPTAKSPGSLALSRR

SEQ ID NO: 2734 - protein, 96 aa, Homo sapiens
MGVNTGDPRQSKKGGRWDTASRKGPVSICLSAGSGFSKCSASSAISGSRPAVMPQPAPRASTPPPRPPPSAPGPSQPPAAGSGDASVATSARTAPS

SEQ ID NO: 2735 - protein, 13 aa, Homo sapiens
MGVRNTKIPPHRR

SEQ ID NO: 2736 - protein, 137 aa, Homo sapiens
MGVSCGGRPPACEERWSDRSLQMPEGGGCWAGKTSELVPVTCSLGEEILLAQDKGSLRTVTCPGRLEGPCSLAWGCCALPFSSSSRFLLLKNCCSRALWSCSLCWILSVFPTWRQVVTLGRQRRLSRISCLRSHLAS

SEQ ID NO: 2737 - protein, 17 aa, Homo sapiens
MGVSPCWSGRSRTPNLR

SEQ ID NO: 2738 - protein, 11 aa, Homo sapiens
MGVSPCWTGWS

SEQ ID NO: 2739 - protein, 20 aa, Homo sapiens
MGWACSLDAEDSAGALGMEL

SEQ ID NO: 2740 - protein, 33 aa, Homo sapiens
MGWAHGVRVLFSELLLVLIDVSEGGGALQSSTR

SEQ ID NO: 2741 - protein, 18 aa, Homo sapiens
MGWGSGRFWDPEFCSREA

SEQ ID NO: 2742 - protein, 23 aa, Homo sapiens
MGYQLVMILLTTQMFRPQNQDLS

SEQ ID NO: 2743 - protein, 24 aa, Homo sapiens
MHAWPHAGRKGDPTVQSPTAWESA

SEQ ID NO: 2744 - protein, 38 aa, Homo sapiens
MHCEQIVSFDEDHLPSNPNARNHAIGYEKLLPKHHVYL

SEQ ID NO: 2745 - protein, 19 aa, Homo sapiens
MHCYFLNTLLLRNFFYQIP

SEQ ID NO: 2746 - protein, 34 aa, Homo sapiens [sequence omitted]

SEQ ID NO: 2747 - protein, 14 aa, Homo sapiens
MHFFHQQFYNNHNS

SEQ ID NO: 2748 - protein, 23 aa, Homo sapiens
MHFHPWQALSFSVDQEESLIITC

SEQ ID NO: 2749 - protein, 70 aa, Homo sapiens
MHFICRTLILVIIIILRRSFTLVAQAGVQWCDLGSPQPLPPGFKRFSCLCLLSIWDYRHAPPCLANFLYL

SEQ ID NO: 2750 - protein, 12 aa, Homo sapiens
MHFMSIYHMSQV

SEQ ID NO: 2751 - protein, 26 aa, Homo sapiens
MHFQSNCNPWSQFPFPSAKTFSEQTT

SEQ ID NO: 2752 - protein, 15 aa, Homo sapiens
MHFTRPEISSDIRKP

SEQ ID NO: 2753 - protein, 65 aa, Homo sapiens
MHFWCRELPFSTSPSPIAIPTSCPIKEYFRCKLNMPRGLLFMKCLVGLRMGGRLDTAESSFWVTL

SEQ ID NO: 2754 - protein, 16 aa, Homo sapiens
MHGISIKIFSGQRGLD

SEQ ID NO: 2755 - protein, 67 aa, Homo sapiens
MHGPGLGAGPELPAWLQLLGRRRGRRRPGARRSSGLRIGGRDCGLSPTAETQAPSPGPGQQPWQRWQ

SEQ ID NO: 2756 - protein, 16 aa, Homo sapiens
MHHARRDNQSKRSSRE

SEQ ID NO: 2757 - protein, 12 aa, Homo sapiens
MHHHAQLIFLYF

SEQ ID NO: 2758 - protein, 27 aa, Homo sapiens
MHHHAQLIFVFLVETGFTILARLVLNS

SEQ ID NO: 2759 - protein, 204 aa, Homo sapiens [sequence omitted]

SEQ ID NO: 2760 - protein, 11 aa, Homo sapiens
MHHHAWLILYF

SEQ ID NO: 2761 - protein, 56 aa, Homo sapiens
MHHHTWLIFVFLVEARFHYVRQDGLELLTSGVLPTLASQSVGITGVSHRARPFCIF

SEQ ID NO: 2762 - protein, 68 aa, Homo sapiens [sequence omitted]

SEQ ID NO: 2763 - protein, 66 aa, Homo sapiens
MHHHVRLIFVFLVATGFHYFGQTGLKLLTSGDPPASASQSAGMTGVSHDTRPWLLLIIQIPRLRRL

SEQ ID NO: 2764 - protein, 11 aa, Homo sapiens
MHHRAQLILYF

SEQ ID NO: 2765 - protein, 69 aa, Homo sapiens
MHHSCHLPSQRYSYQSSFFTIINLCHTSRLYPQHVCCQIPCMWSTFAASTSFLTISIAPSSIASLLPIS

SEQ ID NO: 2766 - protein, 20 aa, Homo sapiens
MHIDRLLCKCQCYFSFLKAK

SEQ ID NO: 2767 - protein, 51 aa, Homo sapiens
MHIFNSGLKGSKTYNSTQRKKAFFINGGEILILIVIIISDMNSFLLHSSKM

SEQ ID NO: 2768 - protein, 32 aa, Homo sapiens
MHIHIHSCAHPLEKYLWNAYYVPALIFLGAYI

SEQ ID NO: 2769 - protein, 23 aa, Homo sapiens
MHISRDDVSFTNSTFNQRLPFLQ

SEQ ID NO: 2770 - protein, 30 aa, Homo sapiens
MHISYRYIGKLLPNHNKHCVQVFKMSLDTH

SEQ ID NO: 2771 - protein, 15 aa, Homo sapiens
MHKFFILKKLCLSSY

SEQ ID NO: 2772 - protein, 16 aa, Homo sapiens
MHKSCQVKTLSLFYRN

SEQ ID NO: 2773 - protein, 11 aa, Homo sapiens
MHKTHRSGTVC

SEQ ID NO: 2774 - protein, 35 aa, Homo sapiens
MHKYFKENQIFLKHDVTNLLVGGRHFKWLTFTSAQ

SEQ ID NO: 2775 - protein, 18 aa, Homo sapiens
MHLEGISIMCIIRKLYKL

SEQ ID NO: 2776 - protein, 19 aa, Homo sapiens
MHLGGQHVVKGSGEVRQGG

SEQ ID NO: 2777 - protein, 15 aa, Homo sapiens
MHLQIANLFQWILLI

SEQ ID NO: 2778 - protein, 18 aa, Homo sapiens
MHLSIVLYQAQGNSLTVS

SEQ ID NO: 2779 - protein, 44 aa, Homo sapiens
MHLSVIPPTATYAQVPLTIQSYSMSLIFLRTKLDLQNKQAMKMT

SEQ ID NO: 2780 - protein, 14 aa, Homo sapiens
MHLVTMFQSTMMVP

SEQ ID NO: 2781 - protein, 30 aa, Homo sapiens
MHMSILSIHKCDIFRLEFRKHTCVCTHTHI

SEQ ID NO: 2782 - protein, 25 aa, Homo sapiens
MHNIFGNVTLLIDTNIIIDLGSELL

SEQ ID NO: 2783 - protein, 85 aa, Homo sapiens
MHNLQNRLTSRRGAFRSREDSNRLLSSPRIFFTVDIDFRLGLFGDVPNGGTFFSYDGSNKLGGNQQAQRQITWFLLGYGSWRPLP

SEQ ID NO: 2784 - protein, 14 aa, Homo sapiens
MHPIKGGPLQSCHL

SEQ ID NO: 2785 - protein, 24 aa, Homo sapiens
MHPITQGHSQQREVKQPASCPSTG

SEQ ID NO: 2786 - protein, 21 aa, Homo sapiens
MHPKGLQPVGLGLIESPPLAL

SEQ ID NO: 2787 - protein, 16 aa, Homo sapiens
MHQECATLQGIMKPSL

SEQ ID NO: 2788 - protein, 11 aa, Homo sapiens
MHQLLNRSLGC

SEQ ID NO: 2789 - protein, 69 aa, Homo sapiens
MHQRCCPGQNIQWRLHSWLEPEGTGHTGCGRGCSAPLRSERPRRSRALRRRWVSSHYSMLHSSAALHTR

SEQ ID NO: 2790 - protein, 30 aa, Homo sapiens
MHQRCCPGQNIQWRLHSWLEPPGGSGRARL

SEQ ID NO: 2791 - protein, 33 aa, Homo sapiens
MHQRCCPGQNIQWRLHSWLEPPGGSGRARLGPA

SEQ ID NO: 2792 - protein, 35 aa, Homo sapiens
MHRAQELRVCWCRLHPWQREHGDPGIRTPGFSSHL

SEQ ID NO: 2793 - protein, 30 aa, Homo sapiens
MHREGVGEGGGLGRWGLVHSDQTEVSQPVM

SEQ ID NO: 2794 - protein, 14 aa, Homo sapiens
MHRHLPNGLFDFSF

SEQ ID NO: 2795 - protein, 11 aa, Homo sapiens
MHRRKVGAGTG

SEQ ID NO: 2796 - protein, 12 aa, Homo sapiens
MHSKVISNWNGL

SEQ ID NO: 2797 - protein, 13 aa, Homo sapiens
MHSLPSIQNPAAS

SEQ ID NO: 2798 - protein, 29 aa, Homo sapiens
MHSQVWKSGSEMNREPGDTGKRVFQQQVE

SEQ ID NO: 2799 - protein, 22 aa, Homo sapiens
MHSSSFKMQILPRDVVVIKISA

SEQ ID NO: 2800 - protein, 12 aa, Homo sapiens
MHSWYLVMFRGS

SEQ ID NO: 2801 - protein, 36 aa, Homo sapiens
MHTIFKFRFFNFWIEFDDTHKSASIIQLVLLGPISL

SEQ ID NO: 2802 - protein, 14 aa, Homo sapiens
MHTQTHIYTRIHTH

SEQ ID NO: 2803 - protein, 75 aa, Homo sapiens [sequence omitted]

SEQ ID NO: 2804 - protein, 40 aa, Homo sapiens
MHVAGTETAAGTPGICSVFLPYRRTPGRQFSATPPPSTPW

SEQ ID NO: 2805 - protein, 23 aa, Homo sapiens
MHVAWASLASLGFCKERGRGYGV

SEQ ID NO: 2806 - protein, 19 aa, Homo sapiens
MHWNICVGQTKPEQKGKNK

SEQ ID NO: 2807 - protein, 61 aa, Homo sapiens
MHWNTVSMAKAKLSKLVMPCLGPSQPGLHTVPFWHCRPWPVSSAQGEGSSSAGTSAMPSWL

SEQ ID NO: 2808 - protein, 76 aa, Homo sapiens
MHYRILDEVLDQTLVNGYYQSWFHFSFNFLWTVKTIEFTSSQNTIQPSPTNQTFYHLLLIKKSCKCILSHTSWLGN

SEQ ID NO: 2809 - protein, 20 aa, Homo sapiens
MICCRMVRSWIIFPFFHWSM

SEQ ID NO: 2810 - protein, 15 aa, Homo sapiens
MICLLWPPKVLGLQA

SEQ ID NO: 2811 - protein, 15 aa, Homo sapiens
MICLPQPPKVLGLQV

SEQ ID NO: 2812 - protein, 13 aa, Homo sapiens
MICLQYKMLHLEI

SEQ ID NO: 2813 - protein, 15 aa, Homo sapiens
MICLRWPPKVLGLQE

SEQ ID NO: 2814 - protein, 15 aa, Homo sapiens
MICPPQPAKVLGLQV

SEQ ID NO: 2815 - protein, 15 aa, Homo sapiens
MICPPQPPKVLGLQT

SEQ ID NO: 2816 - protein, 15 aa, Homo sapiens
MICPPRPPKVLGLQA

SEQ ID NO: 2817 - protein, 15 aa, Homo sapiens
MICPPRPPNVLGLQV

SEQ ID NO: 2818 - protein, 27 aa, Homo sapiens
MICPPWPPKAPFLIFFCRDEVSLCCPG

SEQ ID NO: 2819 - protein, 15 aa, Homo sapiens
MICPPWPPKVLGLQA

SEQ ID NO: 2820 - protein, 51 aa, Homo sapiens
MICSWVSLLSMMLYSSIKHRISTMVWFPLSARSMQGPSLFSARESRNFLVL

SEQ ID NO: 2821 - protein, 32 aa, Homo sapiens
MIDIEMFSHTAHIHMVSLQCEFFDVEQGMNYD

SEQ ID NO: 2822 - protein, 27 aa, Homo sapiens
MIFLNPCNRPFRCCPQEKRFLKKQIEK

SEQ ID NO: 2823 - protein, 55 aa, Homo sapiens
MIFLVAMACMTAPSSGVSSGYTSRGTTHWAAISQGDCKVWSSLGASSTRKPVIIR

SEQ ID NO: 2824 - protein, 12 aa, Homo sapiens
MIFQKCSRSSLS

SEQ ID NO: 2825 - protein, 21 aa, Homo sapiens
MIFQKESQKKLKTTNKGTELL

SEQ ID NO: 2826 - protein, 16 aa, Homo sapiens
MIFQQVESTYPSFLDT

SEQ ID NO: 2827 - protein, 15 aa, Homo sapiens
MIFQSQSDHKQKDRY

SEQ ID NO: 2828 - protein, 18 aa, Homo sapiens
MIFTPPSAPFIVTLIHLF

SEQ ID NO: 2829 - protein, 25 aa, Homo sapiens
MIGGDALGLRCSPAAAFSPSSLALG

SEQ ID NO: 2830 - protein, 46 aa, Homo sapiens
MIGTNFSSSAKESSLLLIPRPPTLLHTNQDVFCASLVLSSSKTIFT

SEQ ID NO: 2831 - protein, 15 aa, Homo sapiens
MIHAPQPPKVLGLQA

SEQ ID NO: 2832 - protein, 30 aa, Homo sapiens
MIHHSHFHSNLTFAILLQPPVEDTASDLTY

SEQ ID NO: 2833 - protein, 15 aa, Homo sapiens
MIHLPCPPKVLGLQV

SEQ ID NO: 2834 - protein, 15 aa, Homo sapiens
MIHLPRPPKVLGLPV

SEQ ID NO: 2835 - protein, 22 aa, Homo sapiens
MIHLPRPPRVLGLQAGATTPCW

SEQ ID NO: 2836 - protein, 15 aa, Homo sapiens
MIHPPQPPKVLGFQA

SEQ ID NO: 2837 - protein, 12 aa, Homo sapiens
MIHPPQPPRALR

SEQ ID NO: 2838 - protein, 15 aa, Homo sapiens
MIHPPRAPKVLELQA

SEQ ID NO: 2839 - protein, 131 aa, Homo sapiens
MIHPPRPPKCWDHRHESLRQAWEPFLEEVLVCCSNLSLFSSQTPAWVNSSNSPTAWTRYKVRTLWIYFTKVCSLLEGQRATDPGHCNAEAGTWNSGPPKAGPRTLELGSPEGRAQNPGTGVPPRQGPEPAL

SEQ ID NO: 2840 - protein, 15 aa, Homo sapiens
MIHPPRPPKMLGSQA

SEQ ID NO: 2841 - protein, 13 aa, Homo sapiens
MIHPPRPPKVLGL

SEQ ID NO: 2842 - protein, 15 aa, Homo sapiens
MIHPPWPPKLLGLQA

SEQ ID NO: 2843 - protein, 11 aa, Homo sapiens
MIHTNLPQLFN

SEQ ID NO: 2844 - protein, 73 aa, Homo sapiens [sequence omitted]

SEQ ID NO: 2845 - protein, 22 aa, Homo sapiens
MIILYNILQAFSSFPGFEYWTL

SEQ ID NO: 2846 - protein, 31 aa, Homo sapiens
MIIQQLSLKSKFTKICQYIICFISIDYNYQL

SEQ ID NO: 2847 - protein, 69 aa, Homo sapiens
MIIQSKILSNKISGRAWWLMSVIPALWEAEAGGSPEVGSSRPAWPTWRNPVSTKNKKKKTLAGFGGTRL

SEQ ID NO: 2848 - protein, 84 aa, Homo sapiens
MIISIIQHLYIHLFSTYLTSAYYVPDTVPRHLLFCAIISIIQHLYINLFNRYLISAYYVLGTVPRHLLYCTIISIIQSACQLPH

SEQ ID NO: 2849 - protein, 35 aa, Homo sapiens
MIITIGVKGSAWNCWCPVQGLPEKVRPNPRPLPTT

SEQ ID NO: 2850 - protein, 67 aa, Homo sapiens
MIKKGFNCHPFNWNPTLAPLHVGILFINISGQAEIRNLHLPPLSYQDVSGCQVPMNELHLGQILHPL

SEQ ID NO: 2851 - protein, 19 aa, Homo sapiens
MIKLKVIHHIFFDLSNHVL

SEQ ID NO: 2852 - protein, 40 aa, Homo sapiens
MIKSIIPQLFDKFNVITIKFSGHSFSCNNLVYQYLVSSKE

SEQ ID NO: 2853 - protein, 39 aa, Homo sapiens
MILANCNLRLPGSNNPPTSTSQVAGTIGTHRHSWFLYFL

SEQ ID NO: 2854 - protein, 22 aa, Homo sapiens
MILDQESKEVNKIFFLSYFVLN

SEQ ID NO: 2855 - protein, 14 aa, Homo sapiens
MILFSLKGNGVSRN

SEQ ID NO: 2856 - protein, 14 aa, Homo sapiens
MILGGFLISFPSAP

SEQ ID NO: 2857 - protein, 32 aa, Homo sapiens
MILILCRPKLMCVFVSSFLTKHLKSKIKIKKR

SEQ ID NO: 2858 - protein, 12 aa, Homo sapiens
MILIVPKANSLS

SEQ ID NO: 2859 - protein, 22 aa, Homo sapiens
MILKRPLAGGEEKMCSLDAKDR

SEQ ID NO: 2860 - protein, 24 aa, Homo sapiens
MILKRSQKTHDLSEIWGPFQKLFA

SEQ ID NO: 2861 - protein, 52 aa, Homo sapiens [sequence omitted]

SEQ ID NO: 2862 - protein, 16 aa, Homo sapiens
MILLAHHGKIADMLHF

SEQ ID NO: 2863 - protein, 14 aa, Homo sapiens
MILLTKGTFRFCEA

SEQ ID NO: 2864 - protein, 17 aa, Homo sapiens
MILLTTQMFRPQNQDLS

SEQ ID NO: 2865 - protein, 21 aa, Homo sapiens
MILNGQALETFPLRTGTRQGC

SEQ ID NO: 2866 - protein, 12 aa, Homo sapiens
MILNLETFKKKT

SEQ ID NO: 2867 - protein, 20 aa, Homo sapiens
MILSLFFPPPKQITLESQDF

SEQ ID NO: 2868 - protein, 12 aa, Homo sapiens
MILTYCLCWVLW

SEQ ID NO: 2869 - protein, 53 aa, Homo sapiens
MILVANLMLLSLSHFTGRDTEAHRGARTCPRSHSWYRVHVLQPLLTLPQTPSI

SEQ ID NO: 2870 - protein, 32 aa, Homo sapiens
MILVTVATNSLHLSSGTKGPLSVTRKVCLCPE

SEQ ID NO: 2871 - protein, 26 aa, Homo sapiens
MIMSFASKMLGRISTSIMLNRSNYIF

SEQ ID NO: 2872 - protein, 15 aa, Homo sapiens
MINLPRPPKVLGLQV

SEQ ID NO: 2873 - protein, 38 aa, Homo sapiens
MINQLCPACRPYLLSRSNHPLIICPSSSGVAGLNPRTM

SEQ ID NO: 2874 - protein, 11 aa, Homo sapiens
MINSILVLSAE

SEQ ID NO: 2875 - protein, 28 aa, Homo sapiens
MINWILFLHSIIHVDNIHYKIFSLQFHV

SEQ ID NO: 2876 - protein, 31 aa, Homo sapiens
MIPLKPQRIFSSSVFTSALDLDTRRGEHLLR

SEQ ID NO: 2877 - protein, 19 aa, Homo sapiens
MIPTTKTFSTFFTLMSFFT

SEQ ID NO: 2878 - protein, 12 aa, Homo sapiens
MIQAKPEIIIIP

SEQ ID NO: 2879 - protein, 18 aa, Homo sapiens
MIQDQYTKVSCIIIIHKQ

SEQ ID NO: 2880 - protein, 52 aa, Homo sapiens
MIQFSLSPQLIVQLSLSPRLIFQLSLSLQLMVQLSLSLQLVVHLYPLFQLMV

SEQ ID NO: 2881 - protein, 62 aa, Homo sapiens
MIQFSLSPQLMIQFSLSPQLIVQLSLSPRLIFQLSLSLQLMVQLSLSLQLVVHLYPLFQLMV

SEQ ID NO: 2882 - protein, 11 aa, Homo sapiens
MIQLLGLSIFN

SEQ ID NO: 2883 - protein, 12 aa, Homo sapiens
MIQLLLSLQLII

SEQ ID NO: 2884 - protein, 52 aa, Homo sapiens
MIQLSLSLQLIVQLSLSLQQIVQFSLSPQPIVQLSLLLQLIVHLSLLLQLIW

SEQ ID NO: 2885 - protein, 42 aa, Homo sapiens
MIQLSLSPQLIVHLSLSFQLIVHLYLLFQLMVQLSLILQLMF

SEQ ID NO: 2886 - protein, 62 aa, Homo sapiens
MIQLSLSPQLIVQLFLSLQQIVQLSLSPQLMVELSLLLQLIVQLSLLLQLILWLSLSLQLMV

SEQ ID NO: 2887 - protein, 42 aa, Homo sapiens
MIQLSLSPQLMVQLSLSPQLIFQLSLSLQLIVLLSLLPQLMV

SEQ ID NO: 2888 - protein, 52 aa, Homo sapiens
MIQLSLSPQLRVQLSLSPQLIVQLSLSPQLIVQLSLLLQLIVQLSLLLRLIL

SEQ ID NO: 2889 - protein, 62 aa, Homo sapiens
MIQLSLSPQVMIQLSLSLQLIVQLSLSLQQIVQFSLSPQPIVQLSLLLQLIVHLSLLLQLIW

SEQ ID NO: 2890 - protein, 166 aa, Homo sapiens
MIQLSLSTQLMVQLSLSLQLIVQLSLSLQLMVWLSLSPQLIVQLSLSPQLIVQLSLSPQLIVQLSLSPQLIVQLSLSPQLIVQLSLSPQLIAELSLSLQLVIQLSLSPQLILQVALLLQLMGQLSLSLQLIVYLSLSPQLMVQLSLSLRLMVQLPLSLQLMVQLSL

SEQ ID NO: 2891 - protein, 30 aa, Homo sapiens
MIQRMPPSCVPSGGPWAASPWQPRHSFGSG

SEQ ID NO: 2892 - protein, 13 aa, Homo sapiens
MIRDGRLCPKTLG

SEQ ID NO: 2893 - protein, 18 aa, Homo sapiens
MIRLFHIAYLYQNISCTP

SEQ ID NO: 2894 - protein, 15 aa, Homo sapiens
MIRLPRPAKVLGLQA

SEQ ID NO: 2895 - protein, 15 aa, Homo sapiens
MIRLPRPPKVLELPV

SEQ ID NO: 2896 - protein, 15 aa, Homo sapiens
MIRLPRPPKVLGLQA

SEQ ID NO: 2897 - protein, 11 aa, Homo sapiens
MIRMQESSLVG

SEQ ID NO: 2898 - protein, 22 aa, Homo sapiens
MIRPPQPPKVLALQALNHHVWP

SEQ ID NO: 2899 - protein, 15 aa, Homo sapiens
MIRPPRPPKVLGLHG

SEQ ID NO: 2900 - protein, 15 aa, Homo sapiens
MIRPPWPPKVLGLQA

SEQ ID NO: 2901 - protein, 15 aa, Homo sapiens
MIRPSWPPKVLGSQA

SEQ ID NO: 2902 - protein, 17 aa, Homo sapiens
MIRSGLGAAIPRKTRFL

SEQ ID NO: 2903 - protein, 17 aa, Homo sapiens
MIRSGLKAAIPRKTRFL

SEQ ID NO: 2904 - protein, 61 aa, Homo sapiens
MIRSPRPPKVLDYRHEPPRPAHFLTFLRSLSTSQIKGVYCSWVSYWGRHEATQQLSERSVF

SEQ ID NO: 2905 - protein, 19 aa, Homo sapiens
MISAHCSLYLPGSGSSPTG

SEQ ID NO: 2906 - protein, 28 aa, Homo sapiens
MISGTYGLHNLKACEYSSLTNFPSQGKY

SEQ ID NO: 2907 - protein, 35 aa, Homo sapiens
MISLDGRAPRAHCSSQIHRTLDVPMVLIEVICDAG

SEQ ID NO: 2908 - protein, 13 aa, Homo sapiens
MISLLWYSEISKQ

SEQ ID NO: 2909 - protein, 30 aa, Homo sapiens
MISLMNCQGELVPKSFVTFFTFVRFLSSVD

SEQ ID NO: 2910 - protein, 43 aa, Homo sapiens [sequence omitted]

SEQ ID NO: 2911 - protein, 16 aa, Homo sapiens
MISSCISCDLCKRKAS

SEQ ID NO: 2912 - protein, 27 aa, Homo sapiens
MISTHSNRVFDPGILDSGRSTLWLLHS

SEQ ID NO: 2913 - protein, 119 aa, Homo sapiens
MISTKWPDWPANTQQRRGLHKVRTKMSSEIPSYEAKRGPTSGPTRPGAVRGDRSRAQRRGRGLGEPPGAAKPGSSCTRTGRTRGGGAAAHGADPANRPPPYTPRCLCAPDRQTEISKDQ

SEQ ID NO: 2914 - protein, 32 aa, Homo sapiens
MITFCFLSKAIRLKSRGIFSLLSPPLVSSCCG

SEQ ID NO: 2915 - protein, 28 aa, Homo sapiens
MITFKRHNIYCKCFLLLWLNVHYINLPF

SEQ ID NO: 2916 - protein, 14 aa, Homo sapiens
MITPPTVECSFQAL

SEQ ID NO: 2917 - protein, 21 aa, Homo sapiens
MITSPGIFVCENHESTLLSSV

SEQ ID NO: 2918 - protein, 33 aa, Homo sapiens
MITSVNKRLSRNSLNIWSMFSAWDDPEEKSKNS

SEQ ID NO: 2919 - protein, 25 aa, Homo sapiens
MITTILSLLYSEARSLFGPTWAPPR

SEQ ID NO: 2920 - protein, 31 aa, Homo sapiens
MITVGIIFQHYSLVITLIFLSQKYITNRELP

SEQ ID NO: 2921 - protein, 17 aa, Homo sapiens
MIVEINNYYLEYLSYSH

SEQ ID NO: 2922 - protein, 42 aa, Homo sapiens [sequence omitted]

SEQ ID NO: 2923 - protein, 98 aa, Homo sapiens
MIVGGVEHFEPVLIVVVSKQVLEAPQADDLLLTGLRQGHPPSAASCKLLGLVQQSIHGEDVGVGPDHHGVGWYLCQVAGCKLGHLGSGPVGAQQFIVL

SEQ ID NO: 2924 - protein, 71 aa, Homo sapiens
MIVGGVEHFEPVLIVVVSKQVLGLVQQSIHGEDVGVGPDHHGVGWYLCQVAGCKLGHLGSGPVGAQQFIVL

SEQ ID NO: 2925 - protein, 11 aa, Homo sapiens
MIVHLILRFSR

SEQ ID NO: 2926 - protein, 22 aa, Homo sapiens
MIVMQQFNDKNILIFYYTAARS

SEQ ID NO: 2927 - protein, 16 aa, Homo sapiens
MIVPSFLDPFLYELPC

SEQ ID NO: 2928 - protein, 23 aa, Homo sapiens
MIVSFLRPPQPYRTVIQFNLFSL

SEQ ID NO: 2929 - protein, 56 aa, Homo sapiens
MIVSSIYWPFVSGFFLLLRTAETSINIFKMQGMFFSVKATVLMCFSFALYHQILYI

SEQ ID NO: 2930 - protein, 15 aa, Homo sapiens
MIVYKFVPFRKKCFM

SEQ ID NO: 2931 - protein, 34 aa, Homo sapiens
MIVYRSCPVSPRASAFSPGRYSSGITPIPTRLLR

SEQ ID NO: 2932 - protein, 12 aa, Homo sapiens
MIWLTVSTTCPG

SEQ ID NO: 2933 - protein, 48 aa, Homo sapiens
MIYCLSLSKWWDYRREPQCLAFFFFWRQPHRSVARLECSGAISAHCNL

SEQ ID NO: 2934 - protein, 13 aa, Homo sapiens
MIYLIKGLYLEYF

SEQ ID NO: 2935 - protein, 15 aa, Homo sapiens
MIYPPWPPKVLRLQA

SEQ ID NO: 2936 - protein, 113 aa, Homo sapiens [sequence omitted]

SEQ ID NO: 2937 - protein, 37 aa, Homo sapiens
MIYYFSTFISIRVSHFIVTYFPCEKQLKDPFKIYPKA

SEQ ID NO: 2938 - protein, 53 aa, Homo sapiens
MKAAWVWELRSLSSNSPGGVTSTAPERLLLADSCSSSQYAQLAAGTLAPHRAP

SEQ ID NO: 2939 - protein, 51 aa, Homo sapiens
MKAHAGCKHFQQCRNEQGESGTCCGHGHRTTLLFLLGCLGRFHRSPRSPAG

SEQ ID NO: 2940 - protein, 22 aa, Homo sapiens
MKAPGKLHSDPRVELWARLQHL

SEQ ID NO: 2941 - protein, 44 aa, Homo sapiens
MKAQLSGAPHSLILTEAFPMTAFSGSGYNYFMSYITNHCSSFLS

SEQ ID NO: 2942 - protein, 43 aa, Homo sapiens
MKARTSKFRLSNTIREYTFDPGRLQSSSAAIQDFSPLGNVSRR

SEQ ID NO: 2943 - protein, 17 aa, Homo sapiens
MKATAGCSSQNGTHARS

SEQ ID NO: 2944 - protein, 42 aa, Homo sapiens
MKCCFIFLPHFLSKVYAFVMNSEMIPTTKTFSTFFTLMSFFT

SEQ ID NO: 2945 - protein, 12 aa, Homo sapiens
MKCFTQPTNLII

SEQ ID NO: 2946 - protein, 44 aa, Homo sapiens
MKDSRFYLENSQNNLVILNKCYHLLNSQDMYVPIYFFAICILVQ

SEQ ID NO: 2947 - protein, 40 aa, Homo sapiens
MKFCYFVNCLYICIYVFYLPPNFMRSEIFICFLFTAGFFF

SEQ ID NO: 2948 - protein, 50 aa, Homo sapiens
MKFKLSMMTMEALHRTGVQSRSKRLYNSGISANRMNRHTPSCIISTRTNI

SEQ ID NO: 2949 - protein, 12 aa, Homo sapiens
MKFLKPHHSGCI

SEQ ID NO: 2950 - protein, 20 aa, Homo sapiens
MKFLKPHHSGCISNFILIIL

SEQ ID NO: 2951 - protein, 24 aa, Homo sapiens
MKFLWNSSSHSQLLPLSRNVLIRL

SEQ ID NO: 2952 - protein, 25 aa, Homo sapiens
MKFLWNSSSHSQLLPLSRNVLIRLH

SEQ ID NO: 2953 - protein, 26 aa, Homo sapiens
MKFLWNSSSHSQLLPLSRNVLIRLHD

SEQ ID NO: 2954 - protein, 27 aa, Homo sapiens
MKFLWNSSSHSQLLPLSRNVLIRLHDL

SEQ ID NO: 2955 - protein, 28 aa, Homo sapiens
MKFLWNSSSHSQLLPLSRNVLIRLHDLC

SEQ ID NO: 2956 - protein, 29 aa, Homo sapiens
MKFLWNSSSHSQLLPLSRNVLIRLHDLCI

SEQ ID NO: 2957 - protein, 30 aa, Homo sapiens
MKFLWNSSSHSQLLPLSRNVLIRLHDLCIW

SEQ ID NO: 2958 - protein, 31 aa, Homo sapiens
MKFLWNSSSHSQLLPLSRNVLIRLHDLCIWF

SEQ ID NO: 2959 - protein, 32 aa, Homo sapiens
MKFLWNSSSHSQLLPLSRNVLIRLHDLCIWFV

SEQ ID NO: 2960 - protein, 33 aa, Homo sapiens
MKFLWNSSSHSQLLPLSRNVLIRLHDLCIWFVF

SEQ ID NO: 2961 - protein, 36 aa, Homo sapiens
MKFRDCCVLLRSSPWEGKSGACCWVPHSTGKSQTSK

SEQ ID NO: 2962 - protein, 11 aa, Homo sapiens
MKFRQYRQART

SEQ ID NO: 2963 - protein, 11 aa, Homo sapiens
MKGEGRTMRGE

SEQ ID NO: 2964 - protein, 30 aa, Homo sapiens
MKGHQARRRAGILLRHRLVTRSVLQITSLL

SEQ ID NO: 2965 - protein, 15 aa, Homo sapiens
MKGLLKVVITFFFPP

SEQ ID NO: 2966 - protein, 11 aa, Homo sapiens
MKGVLCRRYSL

SEQ ID NO: 2967 - protein, 63 aa, Homo sapiens [sequence omitted]

SEQ ID NO: 2968 - protein, 13 aa, Homo sapiens
MKHLTLWTYAGLG

SEQ ID NO: 2969 - protein, 75 aa, Homo sapiens
MKICLWRTMMEAQITLHLFSLPTCICIIPKCLDPQRTIFQRSISGQLTCHHYGIFILNWRLQLSACGTREQGKIG

SEQ ID NO: 2970 - protein, 13 aa, Homo sapiens
MKILGCVDESYKS

SEQ ID NO: 2971 - protein, 187 aa, Homo sapiens
MKIMSKRDKMVGMKSMLSSPFVSSQRPNTELAAARTEQREFRVVVIPALAIEMVCCSMASWIATRSSSRILSNSSIQTTPPSARTMAPPSMMKFRDEGSLITEAVSPAALLPFPDVYTPMGEHFSTNFRSWDLAVPGSPSISRLMSPRRVSPSGSLFREPPKSRQAMAFFMSVPPKMEGAMLLEMTS

SEQ ID NO: 2972 - protein, 19 aa, Homo sapiens
MKISEIWSSNGQDLTGLGQ

SEQ ID NO: 2973 - protein, 11 aa, Homo sapiens
MKIYFISKASV

SEQ ID NO: 2974 - protein, 24 aa, Homo sapiens
MKKFYPYLLPSPNFSAIPRTSLLD

SEQ ID NO: 2975 - protein, 19 aa, Homo sapiens
MKKLNLCIFSHLSFCHKVC

SEQ ID NO: 2976 - protein, 47 aa, Homo sapiens
MKKLVHFKEPPSLWTSLLFSHLNQLLIQLKFLPIAREVRSLSPSFQS

SEQ ID NO: 2977 - protein, 29 aa, Homo sapiens
MKLAFFKIFFNFMELFFFRNFFHFCFYYF

SEQ ID NO: 2978 - protein, 24 aa, Homo sapiens
MKLDNCLYNITSDKTSKEGWFAVI

SEQ ID NO: 2979 - protein, 18 aa, Homo sapiens
MKLEFFQMVLQALYMIIS

SEQ ID NO: 2980 - protein, 55 aa, Homo sapiens
MKLIGFLLMTVMLEAVVDIQLTDTTLQDRGQVTHSLPTDHTLLPIHQNVSSRDDE

SEQ ID NO: 2981 - protein, 53 aa, Homo sapiens
MKLLAHVSMQLGNLHPDSKKMKMCQWKWHWQKTSPSRNSYRYFVTLQEQRIKH

SEQ ID NO: 2982 - protein, 16 aa, Homo sapiens
MKLLILPIYGQVSLLQ

SEQ ID NO: 2983 - protein, 22 aa, Homo sapiens
MKLPHSYCFGLFKLFQWSPLIY

SEQ ID NO: 2984 - protein, 28 aa, Homo sapiens
MKLVFHHFHIIRNLSLCLQCVLSRKKPR

SEQ ID NO: 2985 - protein, 28 aa, Homo sapiens
MKLWLAIYVRSIKDGDIQTVEEIKYVCI

SEQ ID NO: 2986 - protein, 42 aa, Homo sapiens
MKLWQIQQLLRWFPEAIILEKLTREFSFHCACESRGMGRRER

SEQ ID NO: 2987 - protein, 25 aa, Homo sapiens
MKLYSCEDGQNCQMSTNSSVAKFYL

SEQ ID NO: 2988 - protein, 33 aa, Homo sapiens
MKMCQWKWHWQKTSPSRNSYRYFVTLQEQRIKH

SEQ ID NO: 2989 - protein, 25 aa, Homo sapiens
MKMLPCCKIYLFIFLETMNGMKILI

SEQ ID NO: 2990 - protein, 26 aa, Homo sapiens
MKNVLAIEIRKYGHKINLENIQLQLY

SEQ ID NO: 2991 - protein, 38 aa, Homo sapiens
MKPAFSQTEADTLVLSGGGGTCGQSGTVAGSARPVGLG

SEQ ID NO: 2992 - protein, 97 aa, Homo sapiens
MKPAPHSLEGTPGLSRPLWRVWAGFIPMRQCPWVTRNFAGAQGRGLSRLITFTTLFRLRFFIRTNTPISPNLLRVSSLPATVPLLSKAPVLSPTCRG

SEQ ID NO: 2993 - protein, 26 aa, Homo sapiens
MKPPFRGRICTVQRIFKLNDISILLF

SEQ ID NO: 2994 - protein, 23 aa, Homo sapiens
MKPQLNSQKHQHNTVYSNLSPVH

SEQ ID NO: 2995 - protein, 15 aa, Homo sapiens
MKPTVPSFLLLELSE

SEQ ID NO: 2996 - protein, 44 aa, Homo sapiens [sequence omitted]

SEQ ID NO: 2997 - protein, 17 aa, Homo sapiens
MKQEQNVHIYIYIYIYG

SEQ ID NO: 2998 - protein, 35 aa, Homo sapiens
MKQTGVGSQGLTPKLCSIDILLYFFLCLPAIDISL

SEQ ID NO: 2999 - protein, 33 aa, Homo sapiens
MKRGGRLDSGCGLQFAGICSRATLSVTKTCIRL

SEQ ID NO: 3000 - protein, 22 aa, Homo sapiens
MKRKHHMWKTCKLEKHKENELT

SEQ ID NO: 3001 - protein, 32 aa, Homo sapiens
MKRKHHMWKTCKLIIWQKAFQRKTKSSRIQFP

SEQ ID NO: 3002 - protein, 21 aa, Homo sapiens
MKRKHHMWKTCKLSNVQGLLI

SEQ ID NO: 3003 - protein, 75 aa, Homo sapiens
MKRKKMSSPSSLMEACKVLPRICSPLEWRESLKMRNTRTRRMTRRMARDMACCPFWPPPPPPGCCSASSVPRVMK

SEQ ID NO: 3004 - protein, 62 aa, Homo sapiens
MKRNTLLLDDRAESHQHTEYLKALRIMGKKRTRIHPPPHQPHTHKSTKEQAPTCCTLGPFQP

SEQ ID NO: 3005 - protein, 15 aa, Homo sapiens
MKRRMSSGLRHFSCW

SEQ ID NO: 3006 - protein, 54 aa, Homo sapiens
MKSCYFAKYAVTPCNQFALCLQIILNMGEPVRDWSTRMMRTYIILKWRRSLSKN

SEQ ID NO: 3007 - protein, 31 aa, Homo sapiens
MKSINTSHKYIFMSLFLRLLMHFQNLFISLQ

SEQ ID NO: 3008 - protein, 12 aa, Homo sapiens
MKSLGTPFLSGW

SEQ ID NO: 3009 - protein, 25 aa, Homo sapiens
MKSLPTFTTFIGFLSSMNSLMLIKI

SEQ ID NO: 3010 - protein, 175 aa, Homo sapiens
MKSMLSSPFVSSQRPNTELAAARTEQREFRVVVIPALAIEMVCCSMASWIATRSSSRILSNSSIQTTPPSARTMAPPSMMKFRDEGSLITEAVSPAALLPFPDVYTPMGEHFSTNFRSWDLAVPGSPSISRLMSPRRVSPSGSLFREPPKSRQAMAFFMSVPPKMEGAMLLEMTS

SEQ ID NO: 3011 - protein, 17 aa, Homo sapiens
MKSQKQLQQKQNLTNGI

SEQ ID NO: 3012 - protein, 17 aa, Homo sapiens
MKSSNLCSLFLQAQCLL

SEQ ID NO: 3013 - protein, 26 aa, Homo sapiens
MKTDFLRKGGHKDAPLMLLLLINPFL

SEQ ID NO: 3014 - protein, 15 aa, Homo sapiens
MKTDFMTIGHLAKEP

SEQ ID NO: 3015 - protein, 33 aa, Homo sapiens
MKTVSSFKSFLKAFQVKGEKTKELFKFAILSSS

SEQ ID NO: 3016 - protein, 72 aa, Homo sapiens [sequence omitted]

SEQ ID NO: 3017 - protein, 36 aa, Homo sapiens
MKVGIVRERDGRFSGRKKTERWLQSLGKHTILPGLL

SEQ ID NO: 3018 - protein, 14 aa, Homo sapiens
MKVMEVKTKITDPF

SEQ ID NO: 3019 - protein, 43 aa, Homo sapiens
MKVRFFLLFKSSLCASFKCVLQVQLFLPGGKKACFSLQCPFII

SEQ ID NO: 3020 - protein, 14 aa, Homo sapiens
MKWCCLSQTQSHCC

SEQ ID NO: 3021 - protein, 17 aa, Homo sapiens
MKWICTPSRRATPSRGK

SEQ ID NO: 3022 - protein, 32 aa, Homo sapiens
MKYKINFVFKFLSLKNVLSLIIFPHTYPIQSQ

SEQ ID NO: 3023 - protein, 153 aa, Homo sapiens
MLAAATPPVRGSERGLLARPPPLLLRPPTARSALPFNSPRGDPSMRFLLPLFVRLLLRRHRPYYAHRSDLRSHFTHKHTFKWPDRPPVRASRKRRPRTARWALESLLRPPLVGRSSSRDEHAGSGRSQLFSAGLSNRASIVKHPMPRKASWEL

SEQ ID NO: 3024 - protein, 32 aa, Homo sapiens
MLAASSSWNRAWTCCRLPEKRAWWTAGSRQER

SEQ ID NO: 3025 - protein, 81 aa, Homo sapiens
MLACACDYWNSFLALFMPQTKIILPSWETCHGSRMSWEERARGWDSWGHTRASAHPDYTQGQGGDRQMPGSYSLRARSELG

SEQ ID NO: 3026 - protein, 21 aa, Homo sapiens
MLAEPLQRKALLGLNCDWVKL

SEQ ID NO: 3027 - protein, 40 aa, Homo sapiens
MLAERAIPLSKAPQPGKVHDNNHRGKRISMELLVPCAGPT

SEQ ID NO: 3028 - protein, 18 aa, Homo sapiens
MLAFYVRRISLGSYAHKH

SEQ ID NO: 3029 - protein, 27 aa, Homo sapiens
MLAGLVSNSWPQVISPPQPPKVLGLQT

SEQ ID NO: 3030 - protein, 25 aa, Homo sapiens
MLAKLVLNSWPQVVHPPQPPKVLGL

SEQ ID NO: 3031 - protein, 143 aa, Homo sapiens [sequence omitted]

SEQ ID NO: 3032 - protein, 18 aa, Homo sapiens
MLAKLWSNWNAYTLILGV

SEQ ID NO: 3033 - protein, 20 aa, Homo sapiens
MLAKQPLSHPPVTSNDTNLF

SEQ ID NO: 3034 - protein, 50 aa, Homo sapiens
MLANAMLHWPFFLTKRLRHLRRVCTLPLPKPLAPDMVTRCSPSSSNDTML

SEQ ID NO: 3035 - protein, 12 aa, Homo sapiens
MLAREGLNLLTS

SEQ ID NO: 3036 - protein, 27 aa, Homo sapiens
MLARLGLELLTSGDLPASPPKVLGLQP

SEQ ID NO: 3037 - protein, 20 aa, Homo sapiens
MLARLISNSWPQVICLPQPP

SEQ ID NO: 3038 - protein, 54 aa, Homo sapiens
MLARLISNSWTQVNHPFWPPKVLGLQEWATMPSLNFSKVLLNKGFAAYLQVLFT

SEQ ID NO: 3039 - protein, 17 aa, Homo sapiens
MLARLVLNSQPQAICPP

SEQ ID NO: 3040 - protein, 54 aa, Homo sapiens
MLARLVLNSWPRDPPVSASQSEPPRPAQPSLCNFYLKLCSPLFSTLTDEQHHCF

SEQ ID NO: 3041 - protein, 125 aa, Homo sapiens
MLARLVLTSGDPPSSASQSVGITGMSHHARPDSIFKYQNNKNPQASVQWKVQVCLEMVYGILHQSEEDNTADSRHRQMSFQSWIQLVHLASDACSHMCGTVQSQLQKVEVTERHRTSKISHGLVV

SEQ ID NO: 3042 - protein, 80 aa, Homo sapiens
MLARLVSISWPRDLPSSASQSAGITGVSRCAQPGNFLRLYHVYIHRIYFFQVSECDKTNECFPTFHTLIEYPSSVSFYVY

SEQ ID NO: 3043 - protein, 21 aa, Homo sapiens
MLARLVSNSRPQPPKVLGLQA

SEQ ID NO: 3044 - protein, 27 aa, Homo sapiens
MLARLVSNSRPQVIHPPQPPKVLGLQA

SEQ ID NO: 3045 - protein, 26 aa, Homo sapiens
MLARLVSNSSKYHNVPHQYVQLCQLK

SEQ ID NO: 3046 - protein, 173 aa, Homo sapiens [sequence omitted]

SEQ ID NO: 3047 - protein, 27 aa, Homo sapiens
MLARLVSNSSRQVIHLPRPPKVLGLQV

SEQ ID NO: 3048 - protein, 27 aa, Homo sapiens
MLARLVSNSWSQMIRPPRPPKVLGLHG

SEQ ID NO: 3049 - protein, 26 aa, Homo sapiens
MLARLVSTPDLVIHPPQPPEVLQLQA

SEQ ID NO: 3050 - protein, 12 aa, Homo sapiens
MLARMVSISLTL

SEQ ID NO: 3051 - protein, 48 aa, Homo sapiens
MLARNPGFRSRSQMPGTASVTSTHDVGPKYACVEVFWQLLQALTAGAG

SEQ ID NO: 3052 - protein, 28 aa, Homo sapiens
MLARRVSISCPHDLPALASQSPLFNFFL

SEQ ID NO: 3053 - protein, 22 aa, Homo sapiens
MLARTSLIGKMKSLGTPFLSGW

SEQ ID NO: 3054 - protein, 12 aa, Homo sapiens
MLARVVSNPDLR

SEQ ID NO: 3055 - protein, 12 aa, Homo sapiens
MLARWSQTPDLK

SEQ ID NO: 3056 - protein, 31 aa, Homo sapiens
MLASSVNVSEKLILPGWVSGAGVPGVLKDKG

SEQ ID NO: 3057 - protein, 19 aa, Homo sapiens
MLAVKPHPPNQPTQVNSPE

SEQ ID NO: 3058 - protein, 14 aa, Homo sapiens
MLAWLVLNLSLPKC

SEQ ID NO: 3059 - protein, 14 aa, Homo sapiens
MLCFSHILSLLILL

SEQ ID NO: 3060 - protein, 71 aa, Homo sapiens
MLCGNRNVWATALKHILFLGEHGNRAPAVRPFSLSQHVLVIPAVLVIIENYKQEGRWGKVSSMLSGELSFQ

SEQ ID NO: 3061 - protein, 34 aa, Homo sapiens
MLCNNFQISGTCKNKGHLLLKFHVRSWLAATVWF

SEQ ID NO: 3062 - protein, 22 aa, Homo sapiens
MLCSHCSTNWPLSPLSSSSQAS

SEQ ID NO: 3063 - protein, 65 aa, Homo sapiens
MLCSLFCSSAEAASGTSADIVLPLQTRRREKMQLAGGRGHPAAARPSSPRARRAASARENGRRLM

SEQ ID NO: 3064 - protein, 62 aa, Homo sapiens
MLCSLFCSSAEAASGTSADIVLPLTPLLPLAVVQTLPFFLQRSPLLPHLTSVCGCRVLPILA

SEQ ID NO: 3065 - protein, 46 aa, Homo sapiens
MLDDCCTLHQLFLKKNNHIRCSCRVPLSFIFQMRSCQQGYQGIGRR

SEQ ID NO: 3066 - protein, 15 aa, Homo sapiens
MLDIRDIKMQKRPSP

SEQ ID NO: 3067 - protein, 15 aa, Homo sapiens
MLDLVNFGVIPSILF

SEQ ID NO: 3068 - protein, 46 aa, Homo sapiens
MLDPEKSGEGAQWNWGLPAPARAHRPWHPGLCPGLCPDRLQGHPDS

SEQ ID NO: 3069 - protein, 20 aa, Homo sapiens
MLDQRGSSLHFTASNSSMVV

SEQ ID NO: 3070 - protein, 87 aa, Homo sapiens
MLDTKYANLSSNFKKSSLSSLINLLLSQTITFPYIVVNVISNIIELQNGYSSAVSQLVVFNSWGSKTCFRFCIMLSKSMSKDLPCKN

SEQ ID NO: 3071 - protein, 22 aa, Homo sapiens
MLEAGASTAQPRPRQGAGSRHF

SEQ ID NO: 3072 - protein, 28 aa, Homo sapiens
MLEGMDTPFSMIRLFHIAYLYQNISCTP

SEQ ID NO: 3073 - protein, 22 aa, Homo sapiens
MLEILFSTHSMAFFKGVLLRLN

SEQ ID NO: 3074 - protein, 11 aa, Homo sapiens
MLERTQNLEPT

SEQ ID NO: 3075 - protein, 17 aa, Homo sapiens
MLESGGTDLAGFPAATS

SEQ ID NO: 3076 - protein, 19 aa, Homo sapiens
MLESGGTDLAGFPAATSGA

SEQ ID NO: 3077 - protein, 43 aa, Homo sapiens
MLFATELPIVLTEDMELSDAWRSCSVAILGLGGTLLCFQEVSV

SEQ ID NO: 3078 - protein, 84 aa, Homo sapiens
MLFDCLQLFPGCGICVCFPDTLYIWSHVLLHSTPVPASLAGSMAQIIRLYCEFFYLLPSYIYTHKHTQRHMQNIAPQTFHLHIN

SEQ ID NO: 3079 - protein, 50 aa, Homo sapiens
MLFFQLLGAPLGTRAGPYWWAGVGVAVRGAVQVGVAIQVRSGPGSRLRTR

SEQ ID NO: 3080 - protein, 110 aa, Homo sapiens
MLFLLNYTYLCVQRHNYSLTGRKESSLHSPQGPERRFRLSRRPSVLNAHCKHLESFINTELWVLGPPPPSDCIGVGFFKAHQVAACSRSQCAASFLQGAPNTSRAGVALL

SEQ ID NO: 3081 - protein, 29 aa, Homo sapiens
MLFPSYSTLPTPISFLTLRVYSYSVVLQG

SEQ ID NO: 3082 - protein, 13 aa, Homo sapiens
MLFVCSFKIWQDN

SEQ ID NO: 3083 - protein, 15 aa, Homo sapiens
MLGFFLLLQMTDGCN

SEQ ID NO: 3084 - protein, 33 aa, Homo sapiens
MLGLILPLKATKRTMNSGAPPLEFGFLQIYTST

SEQ ID NO: 3085 - protein, 45 aa, Homo sapiens
MLGQHHIPLLIVLILDDEDHVEARQDGGHEVNVVLPLRLIPAAEH

SEQ ID NO: 3086 - protein, 18 aa, Homo sapiens
MLGRISTSIMLNRSNYIF

SEQ ID NO: 3087 - protein, 14 aa, Homo sapiens
MLGRLQRKGNAIHC

SEQ ID NO: 3088 - protein, 28 aa, Homo sapiens
MLGWRATVKTFLIPTSNRAVQQWYRRSM

SEQ ID NO: 3089 - protein, 29 aa, Homo sapiens
MLHGILIVLLLCQQVVECLIHTLVVVALD

SEQ ID NO: 3090 - protein, 60 aa, Homo sapiens
MLHGILVEMILLAELHALGPPVIALVQIGRNAPELHQLMLLQLLSQADVVKVVIGIDRCP

SEQ ID NO: 3091 - protein, 20 aa, Homo sapiens
MLHHSAPKALSYMLYSQHPG

SEQ ID NO: 3092 - protein, 74 aa, Homo sapiens
MLHIWKGWWRSKTTRWRAATGASRDRTRIHGHWNWARFFYWTLLKKRMAKKCFKVHSIFLVSLKQTQKEISQIR

SEQ ID NO: 3093 - protein, 66 aa, Homo sapiens [sequence omitted]

SEQ ID NO: 3094 - protein, 17 aa, Homo sapiens
MLHNSNQSCNELFRRQE

SEQ ID NO: 3095 - protein, 31 aa, Homo sapiens
MLHRGNAVVALPELALVPSTDLLIIIQHPHS

SEQ ID NO: 3096 - protein, 92 aa, Homo sapiens
MLHSVRNSQNRQDRMQWTQQSSCAWRGIWEVVDLLLLLLFLLPWLARDGCVCNFRWALGPPRAPFPARLVPPSSEGWPESFGRSGVQPKGFP

SEQ ID NO: 3097 - protein, 12 aa, Homo sapiens
MLHTAYKSDHLK

SEQ ID NO: 3098 - protein, 45 aa, Homo sapiens
MLHWPFFLTKRLRHLRRVCTLPLPKPLAPDMVTRCSPSSSNDTML

SEQ ID NO: 3099 - protein, 26 aa, Homo sapiens
MLICHPIKGRVYFLCPLNFGWHYDVL

SEQ ID NO: 3100 - protein, 15 aa, Homo sapiens
MLIFKLPARYLLPPQ

SEQ ID NO: 3101 - protein, 46 aa, Homo sapiens
MLIFVFFLVETGFHHFGQAGLELLASSDLPTSASQIAGLQGVSHCT

SEQ ID NO: 3102 - protein, 103 aa, Homo sapiens
MLIGEIPCSPLYTSKILPDNVLCISRGESAPSSLKLDSIPIISSITSSICHCALSSSFPIASNLVSGFSVRPASLSRVVCACCTRGPPLGTAGCDHLRVGLMI

SEQ ID NO: 3103 - protein, 83 aa, Homo sapiens
MLIIIFNQEFFLIFSLPIHMSVSSIWVQVCETKGRNPPDTASLRQVELLQFLSSYVNSVMAMRSFCLNAFSNKSRASWPNCFE

SEQ ID NO: 3104 - protein, 13 aa, Homo sapiens
MLIKDSASFSLSN

SEQ ID NO: 3105 - protein, 25 aa, Homo sapiens
MLIRVILSVPKYEAWIVEELTALIS

SEQ ID NO: 3106 - protein, 26 aa, Homo sapiens
MLIRVILSVPKYEAWIVEELTALISS

SEQ ID NO: 3107 - protein, 29 aa, Homo sapiens
MLIRVILSVPKYEAWIVEELTALISWFHP

SEQ ID NO: 3108 - protein, 21 aa, Homo sapiens
MLISKLGTTLSQVSMSPKCVL

SEQ ID NO: 3109 - protein, 27 aa, Homo sapiens
MLKDIPGVERKIQNEHKNRLQTRQYES

SEQ ID NO: 3110 - protein, 31 aa, Homo sapiens
MLKFRIGPVQLFTGCLQTSCFCCRLLKAGIL

SEQ ID NO: 3111 - protein, 18 aa, Homo sapiens
MLKGRKRSSRLEVPFTPR

SEQ ID NO: 3112 - protein, 25 aa, Homo sapiens
MLKIPRHLSPGAYQGPEERGEDARR

SEQ ID NO: 3113 - protein, 24 aa, Homo sapiens
MLKKAFQRKVEFNLLHCVHLNISK

SEQ ID NO: 3114 - protein, 18 aa, Homo sapiens
MLKLKTRKKTRNLNITSQ

SEQ ID NO: 3115 - protein, 12 aa, Homo sapiens
MLKLLRSIVTPT

SEQ ID NO: 3116 - protein, 11 aa, Homo sapiens
MLKREMKGVIL

SEQ ID NO: 3117 - protein, 152 aa, Homo sapiens [sequence omitted]

SEQ ID NO: 3118 - protein, 30 aa, Homo sapiens
MLKTLNKLGIDGTYLKIIRAVMTNPQPISH

SEQ ID NO: 3119 - protein, 48 aa, Homo sapiens
MLKTLNKLGIEGTYFKIIRAIYDRLTANIIPNGQKLEALPLKTSTRQG

SEQ ID NO: 3120 - protein, 16 aa, Homo sapiens
MLKTLNKLGIEGTYLK

SEQ ID NO: 3121 - protein, 77 aa, Homo sapiens
MLKVLCSLPLALRTNSNFLPQLTCPCVVWLHPHSCLLPPCCSHPVLFWFFQTAGPLHLLSLCLEYTFCSWFIGLTPS

SEQ ID NO: 3122 - protein, 394 aa, Homo sapiens
MLLAGIGAVLLQGAPRLQGTPAAVGVRRTHAVPTGGVHVAGGDLHPGHLVGRHQVKVTGVCWVKLHDMVHGLPIGHSHHPPAHHLHALVQVDLEKPPVDRAQEDRCVVVDAGHGHGGEARGAEHGRGLQGLQDGQRVLQVSSSTVQLLWLELDVELALTGRSRALHHAVEHRHHVGRRFHEAGGARSSDGGSHVGEAEGAECGRSSAGRGGPLGPLEDSKEPLPGWEDRHQAAVEVAAARAARALQAQLDVGLGELLGVAAGAVGQADARQQAPRLALLVARARLAVERQVRVGLCTRRRVGRVQEGAHEAQLVLLLGALLDLEDVVVGGVEVEGEELGQVAARVQGADGDLGRVLEAVVLQAAVAREEGAAVTGVRGAHEQAAAPRARGGRQN

SEQ ID NO: 3123 - protein, 17 aa, Homo sapiens
MLLALGAHLLRLSVPPL

SEQ ID NO: 3124 - protein, 27 aa, Homo sapiens
MLLCNVNLSSNKRQSLFPLPLEFWLAL

SEQ ID NO: 3125 - protein, 45 aa, Homo sapiens
MLLIRTSSLRINKAPWIRSSRFMPFSLAKVSSNPFSASSNVCLYH

SEQ ID NO: 3126 - protein, 14 aa, Homo sapiens
MLLKLCDSKTLELD

SEQ ID NO: 3127 - protein, 16 aa, Homo sapiens
MLLLCNLSINAALLHL

SEQ ID NO: 3128 - protein, 28 aa, Homo sapiens
MLLLEHFSTTVTLTALFSSVNFPKFNEN

SEQ ID NO: 3129 - protein, 34 aa, Homo sapiens
MLLLLLLLLLLLVTATLAGPGSCGVGGSTFRFFF

SEQ ID NO: 3130 - protein, 58 aa, Homo sapiens
MLLLPAHPSTVCFENLQSLVFNSVATWCVKEKFPNSSLSASTPRSGKGPESVLHGFSF

SEQ ID NO: 3131 - protein, 54 aa, Homo sapiens
MLLLPAHPSTVCFENLQSLVFNWCVKEKFPNSSLSASTPRSGKGPESVLHGFSF

SEQ ID NO: 3132 - protein, 35 aa, Homo sapiens
MLLLQLLLREESQVAENNILCFIVKSQRHSRRGRH

SEQ ID NO: 3133 - protein, 24 aa, Homo sapiens
MLLLRSPKFQFLFYLTPTFLSTSF

SEQ ID NO: 3134 - protein, 11 aa, Homo sapiens
MLLLSSFLLIS

SEQ ID NO: 3135 - protein, 64 aa, Homo sapiens [sequence omitted]

SEQ ID NO: 3136 - protein, 33 aa, Homo sapiens
MLLNILQCTGQPHAPLPRIICPYVSLVLRWRSP

SEQ ID NO: 3137 - protein, 27 aa, Homo sapiens
MLLRLVSNSRPQVIHPPQPPKVPGLQA

SEQ ID NO: 3138 - protein, 49 aa, Homo sapiens
MLLSDCVREMAAAQLSPPSMVFLSMVSVTRGKVGSDSVLRPRPLVFSLE

SEQ ID NO: 3139 - protein, 14 aa, Homo sapiens
MLLSDLIQFSGPGL

SEQ ID NO: 3140 - protein, 26 aa, Homo sapiens
MLLSDLTKSQILVCPELLIPFLCFLS

SEQ ID NO: 3141 - protein, 35 aa, Homo sapiens
MLLSFSSVLCQKYSLSRRWRKGKKKITYIFINTSA

SEQ ID NO: 3142 - protein, 171 aa, Homo sapiens [sequence omitted]

SEQ ID NO: 3143 - protein, 26 aa, Homo sapiens
MLLSLGWLTSPWPPEVPQLWLLFYGK

SEQ ID NO: 3144 - protein, 46 aa, Homo sapiens
MLLSLSHFTGRDTEAHRGARTCPRSHSWYRVHVLQPLLTLPQTPSI

SEQ ID NO: 3145 - protein, 71 aa, Homo sapiens
MLLSNLGWTKCDLDFSSVFSSKSSVGLFLPSICCKACNFSYFEVNSSISTLCTSFCLTKQESSSFIFCSKI

SEQ ID NO: 3146 - protein, 64 aa, Homo sapiens
MLLSPTHVLPHGFVIFDLLSIDSPLQAFQSENPPSPGKQHPFPQGEDSPMDSSPHSIMPRISPR

SEQ ID NO: 3147 - protein, 25 aa, Homo sapiens
MLLSSVTGLRPCIRPTITHRLSGQL

SEQ ID NO: 3148 - protein, 37 aa, Homo sapiens
MLLTLIRASQAMVVCFSSGVSSNNCMISSCRGLQIFA

SEQ ID NO: 3149 - protein, 92 aa, Homo sapiens
MLLTPRWSACPQPPGRMDTQDTIWPRRPILTQGLCSPGTSVLTAGVSRALLLVGAQARTAPATTRHPSAQGQGPVVSLLRRLWNNPVPFSSF

SEQ ID NO: 3150 - protein, 31 aa, Homo sapiens
MLLWLCRRRRSPRHAARPRSAPQLRPLRCRR

SEQ ID NO: 3151 - protein, 33 aa, Homo sapiens
MLLWLCRRRRSPRHAARPRSAPQLRPLRCRRAN

SEQ ID NO: 3152 - protein, 20 aa, Homo sapiens
MLLYIFATLSLQGVRFCNEQ

SEQ ID NO: 3153 - protein, 57 aa, Homo sapiens
MLMENNSQKGEGRTNKPTGVSYRRGWTPPLRGRRQLLASFLPDSSQLFCRLLCPEGS

SEQ ID NO: 3154 - protein, 41 aa, Homo sapiens
MLMENNSQKGEGRTNKPTGVSYRRGWTPPLRGRRQLMVGSC

SEQ ID NO: 3155 - protein, 38 aa, Homo sapiens
MLMLQVHRPLRITRRLEALESWFSQSDWSHQRASPRTG

SEQ ID NO: 3156 - protein, 15 aa, Homo sapiens
MLMSPGTHCSRSRRC

SEQ ID NO: 3157 - protein, 66 aa, Homo sapiens
MLNDRYPEAVNSSGDVRLLMAIRTSTATRIQKNVTERCGPETESSTFRAMIPPRTAEMPAITSTTE

SEQ ID NO: 3158 - protein, 36 aa, Homo sapiens
MLNDRYPEAVNSSGDVRLLMAIRTSTRHLLGHSAAT

SEQ ID NO: 3159 - protein, 29 aa, Homo sapiens [sequence omitted]

SEQ ID NO: 3160 - protein, 16 aa, Homo sapiens
MLNLGQSSLSFGHTFT

SEQ ID NO: 3161 - protein, 28 aa, Homo sapiens
MLNLLALFVSSFCEIFLLLESRFPVPFH

SEQ ID NO: 3162 - protein, 103 aa, Homo sapiens
MLNVCAKASHLQLLEGRCRSNSWKHWSLQCRCGPSPQCSWSMLTWSEAVTLGVYLQLNRGGGPCNKASTWAGLLFHGHSFKVWSIRSSLELQPRPDNSQEFSR

SEQ ID NO: 3163 - protein, 23 aa, Homo sapiens
MLPCCKIYLFIFLETMNGMKILI

SEQ ID NO: 3164 - protein, 25 aa, Homo sapiens
MLPGQEAASRTLALPLLDGAGEGRG

SEQ ID NO: 3165 - protein, 16 aa, Homo sapiens
MLPHLKRCPRFYSLKL

SEQ ID NO: 3166 - protein, 27 aa, Homo sapiens
MLPKLLSKSLAQAIFPPWLLKVLGLQA

SEQ ID NO: 3167 - protein, 14 aa, Homo sapiens
MLPLLPLQTSSCES

SEQ ID NO: 3168 - protein, 104 aa, Homo sapiens
MLPLMSALMGVNTGDPRQSKKGGRWDTASRKGPVSICLSAGSGFSKCSASSAISGSRPAVMPQPAPRASTPPPRPPPSAPGPSQPPAAGSGDASVATSARTAPS

SEQ ID NO: 3169 - protein, 14 aa, Homo sapiens
MLPLYFLLHSVKRM

SEQ ID NO: 3170 - protein, 42 aa, Homo sapiens
MLPQELACSPIVKLLLGLRSLHGINNQIHQLVLQHRAALLVL

SEQ ID NO: 3171 - protein, 61 aa, Homo sapiens
MLPQELACSPIVKLLLGLRSLHGINNQIHQLVLQHRAALLVLIIWQKAFQRKTKSSRIQFP

SEQ ID NO: 3172 - protein, 44 aa, Homo sapiens
MLPQELACSPIVKLLLGLRSLHGINNQIHQLVLQHRAALLVLLI

SEQ ID NO: 3173 - protein, 50 aa, Homo sapiens
MLPQELACSPIVKLLLGLRSLHGINNQIHQLVLQHRAALLVLSNVQGLLI

SEQ ID NO: 3174 - protein, 15 aa, Homo sapiens
MLPQQLSLDKFITNL

SEQ ID NO: 3175 - protein, 27 aa, Homo sapiens
MLPRLVLNAWVQAIPPASPPKVLGLQV

SEQ ID NO: 3176 - protein, 27 aa, Homo sapiens
MLPRLVSNFWAQVICPPWPPKVLGLRA

SEQ ID NO: 3177 - protein, 30 aa, Homo sapiens
MLPRPVNFCIFSRDGVSPCWSGWPQTPDLR

SEQ ID NO: 3178 - protein, 27 aa, Homo sapiens
MLPSFKFTGHVRPHLLLCHLYLGAISL

SEQ ID NO: 3179 - protein, 15 aa, Homo sapiens
MLPSHTLTSLSCAIT

SEQ ID NO: 3180 - protein, 17 aa, Homo sapiens
MLPWTKHPMASPFLVGA

SEQ ID NO: 3181 - protein, 26 aa, Homo sapiens
MLPWTKHPMASPFLVGAARRLWARPP

SEQ ID NO: 3182 - protein, 30 aa, Homo sapiens
MLPWTKHPMASPFLVGAARRLWARPPGAGL

SEQ ID NO: 3183 - protein, 11 aa, Homo sapiens
MLPYQKQETAS

SEQ ID NO: 3184 - protein, 13 aa, Homo sapiens
MLQFCLWFSFVLL

SEQ ID NO: 3185 - protein, 28 aa, Homo sapiens
MLQGGLLGAPESGACGGVRPALLALGGC

SEQ ID NO: 3186 - protein, 38 aa, Homo sapiens
MLQKGFVSAADATTSPAQRSPGGRAAAPGALGRVSLRG

SEQ ID NO: 3187 - protein, 65 aa, Homo sapiens
MLQKILPLGRENWRTTKIAYFSSPTASFKTSPCRAHNPKLLLITLPSAYSAQSLPCLTKPCFFKF

SEQ ID NO: 3188 - protein, 14 aa, Homo sapiens
MLQLISLYPLFTFI

SEQ ID NO: 3189 - protein, 37 aa, Homo sapiens
MLQLLVSCHLISQSLLHETVLGRCDQEHLQGCLLQQR

SEQ ID NO: 3190 - protein, 36 aa, Homo sapiens
MLQVHRPLRITRRLEALESWFSQSDWSHQRASPRTG

SEQ ID NO: 3191 - protein, 103 aa, Homo sapiens
MLRLPPLPPGAKIRRAPRGLVPPARPGGAHKRVWGDAQQVPLLGSRSKMQKRSLLPLGERAAATKWCLSGPELQWRDGRDRIQACLAGMRVLVPREGGSGRRG

SEQ ID NO: 3192 - protein, 62 aa, Homo sapiens
MLRMREKPLPSWLALSWGSRKSVCRSGPSAFKSKLSLWHRKLPNFSLRGLLSLGIPGRGPHW

SEQ ID NO: 3193 - protein, 11 aa, Homo sapiens
MLRQPIAEKND

SEQ ID NO: 3194 - protein, 11 aa, Homo sapiens
MLSEHSSSCCL

SEQ ID NO: 3195 - protein, 38 aa, Homo sapiens
MLSFAIRHEHWLNVCHIVYYSSFLQYELSYLQSSVTAT

SEQ ID NO: 3196 - protein, 16 aa, Homo sapiens
MLSFQIQEYLSVLLVF

SEQ ID NO: 3197 - protein, 22 aa, Homo sapiens
MLSHHTLSLFNMAFKQLFLLAK

SEQ ID NO: 3198 - protein, 13 aa, Homo sapiens
MLSLARRCTGDLV

SEQ ID NO: 3199 - protein, 24 aa, Homo sapiens
MLSLARRSLSRLSCTASSSRGASS

SEQ ID NO: 3200 - protein, 39 aa, Homo sapiens
MLSMCSRICKSKHLGLKNKIEKILFLSLHKIVCPNKRKS

SEQ ID NO: 3201 - protein, 21 aa, Homo sapiens
MLSNFTLKRKMLSEHSSSCCL

SEQ ID NO: 3202 - protein, 13 aa, Homo sapiens
MLSNIQWNQSSLQ

SEQ ID NO: 3203 - protein, 37 aa, Homo sapiens
MLSNLVCPLLGRLRADSRLSPLSSHFSSRTILDAGHT

SEQ ID NO: 3204 - protein, 27 aa, Homo sapiens
MLSRLVSNSWAQAIHRPQPPKMLRLQA

SEQ ID NO: 3205 - protein, 74 aa, Homo sapiens
MLSRTTREMTLYVPNMVAPTNSVNSCCALTLVTYKLMSPNIDQNRDCSVSNNVENALFCFSHLMPLQVNPFVSS

SEQ ID NO: 3206 - protein, 18 aa, Homo sapiens
MLSTVPTQILIFFWLVGI

SEQ ID NO: 3207 - protein, 18 aa, Homo sapiens
MLSYLKPSLTKSCRFKAA

SEQ ID NO: 3208 - protein, 24 aa, Homo sapiens
MLTEPKASKMPIWPVHVSLKINSI

SEQ ID NO: 3209 - protein, 17 aa, Homo sapiens
MLTFFLSGKTVDVWQPV

SEQ ID NO: 3210 - protein, 39 aa, Homo sapiens
MLTFPPLIYCLMLNLLALFVSSFCEIFLLLESRFPVPFH

SEQ ID NO: 3211 - protein, 16 aa, Homo sapiens
MLTFQTKARSASLRGR

SEQ ID NO: 3212 - protein, 14 aa, Homo sapiens
MLTLATPFLLLLTV

SEQ ID NO: 3213 - protein, 12 aa, Homo sapiens
MLTPRNRCARPP

SEQ ID NO: 3214 - protein, 27 aa, Homo sapiens
MLTRLVSNFRPQVICPPRPLKVLGLQT

SEQ ID NO: 3215 - protein, 14 aa, Homo sapiens
MLTSSSSNQLLRDL

SEQ ID NO: 3216 - protein, 69 aa, Homo sapiens
MLTTGVLMELWVTRVSASSSTGSVSSRGSGARKTLKVKLAAASRRTPKPAMNFRWRRGTWTFRIRILVG

SEQ ID NO: 3217 - protein, 18 aa, Homo sapiens
MLVARQNSSDSLPRCYRF

SEQ ID NO: 3218 - protein, 23 aa, Homo sapiens
MLVDLENFCQDYTYQFFFNEKVF

SEQ ID NO: 3219 - protein, 21 aa, Homo sapiens
MLVFQLGKILGLFFLFCKICR

SEQ ID NO: 3220 - protein, 20 aa, Homo sapiens
MLVILNIVRLILINLDWRHF

SEQ ID NO: 3221 - protein, 22 aa, Homo sapiens
MLVINSSKYLQDFSKCVVLIII

SEQ ID NO: 3222 - protein, 46 aa, Homo sapiens
MLVITDSSSWMMSFVKGSVMILSRSGASRPPWMLKEATTSRVMWCR

SEQ ID NO: 3223 - protein, 17 aa, Homo sapiens
MLVLNPGAQRPKTAATV

SEQ ID NO: 3224 - protein, 22 aa, Homo sapiens
MLVLRCSIDVGIFSTQGYAWVK

SEQ ID NO: 3225 - protein, 54 aa, Homo sapiens
MLVLSREKYFCPMFTTSIETILSNLSNMRKALLAKASCQSRREAPLFCWQKQTS

SEQ ID NO: 3226 - protein, 34 aa, Homo sapiens
MLVPHWILRGLNEKIHAKQSLAWHVLRGSHYCYF

SEQ ID NO: 3227 - protein, 11 aa, Homo sapiens
MLVPVPQPPCY

SEQ ID NO: 3228 - protein, 42 aa, Homo sapiens
MLVRLVLNSRPQVICLPWPPKVLGLQVSATTPGQFCCCCCCC

SEQ ID NO: 3229 - protein, 27 aa, Homo sapiens
MLVRLVSDSRPQVIHPPQPPKVLGLQA

SEQ ID NO: 3230 - protein, 27 aa, Homo sapiens
MLVRLVSNFRPQVIRLPRPPKVLGLQA

SEQ ID NO: 3231 - protein, 27 aa, Homo sapiens
MLVRLVSNSQTQVIRPPWPPKVLGLQA

SEQ ID NO: 3232 - protein, 27 aa, Homo sapiens
MLVRLVSNSRPQVIHLPRPPKLLGLQA

SEQ ID NO: 3233 - protein, 27 aa, Homo sapiens
MLVRLVSNSRPQVIHLPWPPKVLGLQV

SEQ ID NO: 3234 - protein, 27 aa, Homo sapiens
MLVRLVSNSWPQVIRLPQPPKALGLQV

SEQ ID NO: 3235 - protein, 27 aa, Homo sapiens
MLVRLVSNVRSQVIHLPRPPKALGLRA

SEQ ID NO: 3236 - protein, 27 aa, Homo sapiens
MLVRQVSNSQPQVICLPQPPKVLALQA

SEQ ID NO: 3237 - protein, 31 aa, Homo sapiens
MLVSSPLQAANTEACQRNILIGGSVLLLGKP

SEQ ID NO: 3238 - protein, 15 aa, Homo sapiens
MLVTKLRVQECPGNE

SEQ ID NO: 3239 - protein, 12 aa, Homo sapiens
MLVTWSQTPDLK

SEQ ID NO: 3240 - protein, 12 aa, Homo sapiens
MLVVKASVVIIY

SEQ ID NO: 3241 - protein, 124 aa, Homo sapiens [sequence omitted]

SEQ ID NO: 3242 - protein, 27 aa, Homo sapiens
MLVWVVLNSRPQVIHLPWPPKVLGLQA

SEQ ID NO: 3243 - protein, 13 aa, Homo sapiens
MLYCYQFKNSNQK

SEQ ID NO: 3244 - protein, 11 aa, Homo sapiens
MLYFPFKTECL

SEQ ID NO: 3245 - protein, 11 aa, Homo sapiens
MLYQTWIRLPK

SEQ ID NO: 3246 - protein, 18 aa, Homo sapiens
MLYSFARNFVIASSLFFS

SEQ ID NO: 3247 - protein, 16 aa, Homo sapiens
MLYSFCIKMTKEIKPK

SEQ ID NO: 3248 - protein, 40 aa, Homo sapiens
MLYSSIKHRISTMVWFPLSARSMQGPSLFSARESRNFLVL

SEQ ID NO: 3249 - protein, 22 aa, Homo sapiens
MMALSLSLQLMTQLYLIHQLMV

SEQ ID NO: 3250 - protein, 23 aa, Homo sapiens
MMCFDQWNVAEVILSPECLLSPS

SEQ ID NO: 3251 - protein, 67 aa, Homo sapiens [sequence omitted]

SEQ ID NO: 3252 - protein, 72 aa, Homo sapiens
MMFSRFIYVVACISISFPFYCHIVFHCVDRKHFFFFLRQGLTLSPSWSAVVQPLTTASTSRAQVIIPPQLPE

SEQ ID NO: 3253 - protein, 40 aa, Homo sapiens
MMFSSPKLKNACEMIFLNPCNRPFRCCPQEKRFLKKQIEK

SEQ ID NO: 3254 - protein, 29 aa, Homo sapiens
MMFYTCIFIFIHVLIHSKNIYGMPTMYQH

SEQ ID NO: 3255 - protein, 14 aa, Homo sapiens
MMGFLSVKNQNHWS

SEQ ID NO: 3256 - protein, 84 aa, Homo sapiens
MMGLVGDIGCSLHSLRAPGRMDAEEAGERRRLRNELLPQPLRSSPSRLRPQLTQFCALLLSLTFLHRLPGISMTAERAEQPGFS

SEQ ID NO: 3257 - protein, 38 aa, Homo sapiens
MMGLVGDIGCSLHSLSGGAGEGGRSSHERWLGPHAAPS

SEQ ID NO: 3258 - protein, 39 aa, Homo sapiens
MMGLVGDIGCSLHSPVLRVIAQFDFLAQAPGDLHDRGAR

SEQ ID NO: 3259 - protein, 453 aa, Homo sapiens
MMGMSLFPVSFKSISFSLIALNSASTFSLWEISSLISFKSVSILPTGLTSSGPFSCGDISLSVSSKSVSITSAASITSRVFSLEEPSLPVVFKSVSISSTGLTSSGPFSSGDISLLPVSSRSLSISSVASITSGVFSLGEISLPVAFKSVCISPRGLTSSRPFSCGDISLSVSSKSISISSMASITSGVFPLGKLSLPVAFKSVSISPRGLTSSSPFSCGDTSLSVSSKSISSVASITSGVFSLGELSLPVAFKSVSISSTGLTSSGPFSLGDIFLLPVSSKFLSISSVASVTSGVFSLGELSFPVAFKSVSTSPRGLTSSGPFFCGDISLLPASSKSLSISSVASITSGVFSLRQISLPIAFRPVSISMVSSITSRIFSLGEMALLPVSFKSDCISLVLISAGTISFGEVSSLTVSLNAAAISPETRIFSSTSSFEEISLLPVPLPIFGFGF

SEQ ID NO: 3260 - protein, 24 aa, Homo sapiens
MMHFHPWQALSFSVDQEESLIITC

SEQ ID NO: 3261 - protein, 24 aa, Homo sapiens
MMKPQLNSQKHQHNTVYSNLSPVH

SEQ ID NO: 3262 - protein, 32 aa, Homo sapiens
MMKSINTSHKYIFMSLFLRLLMHFQNLFISLQ

SEQ ID NO: 3263 - protein, 18 aa, Homo sapiens
MMKSQKQLQQKQNLTNGI

SEQ ID NO: 3264 - protein, 29 aa, Homo sapiens
MMLGWRATVKTFLIPTSNRAVQQWYRRSM

SEQ ID NO: 3265 - protein, 67 aa, Homo sapiens
MMLNDRYPEAVNSSGDVRLLMAIRTSTATRIQKNVTERCGPETESSTFRAMIPPRTAEMPAITSTTE

SEQ ID NO: 3266 - protein, 37 aa, Homo sapiens
MMLNDRYPEAVNSSGDVRLLMAIRTSTRHLLGHSAAT

SEQ ID NO: 3267 - protein, 22 aa, Homo sapiens
MMLSNFTLKRKMLSEHSSSCCL

SEQ ID NO: 3268 - protein, 24 aa, Homo sapiens
MMLVDLENFCQDYTYQFFFNEKVF

SEQ ID NO: 3269 - protein, 41 aa, Homo sapiens
MMLYSSIKHRISTMVWFPLSARSMQGPSLFSARESRNFLVL

SEQ ID NO: 3270 - protein, 23 aa, Homo sapiens
MMMALSLSLQLMTQLYLIHQLMV

SEQ ID NO: 3271 - protein, 25 aa, Homo sapiens
MMNFLRSETIFYFEFQMLWHILEAK

SEQ ID NO: 3272 - protein, 26 aa, Homo sapiens
MMNILRLVINSMNKVVHSRHIGFLMF

SEQ ID NO: 3273 - protein, 35 aa, Homo sapiens
MMPCSKVQASAGDHPDFLWTSALSFHPPALSIESK

SEQ ID NO: 3274 - protein, 52 aa, Homo sapiens
MMSVSLTVRSTRDCLFFSNSFVPSTSPPMISFSPSCFLAVSVSFDSVWSCFR

SEQ ID NO: 3275 - protein, 26 aa, Homo sapiens
MMSVVHRSDQRVNEPSTYAGPDITDR

SEQ ID NO: 3276 - protein, 26 aa, Homo sapiens
MMSVVHRSDQRVNEPSVCADPDITDR

SEQ ID NO: 3277 - protein, 36 aa, Homo sapiens
MMTKASVEPLNCSSWWPAIQCCSCLVRDATWREGFL

SEQ ID NO: 3278 - protein, 44 aa, Homo sapiens
MMTMEALHRTGVQSRSKRLYNSGISANRMNRHTPSCIISTRTNI

SEQ ID NO: 3279 - protein, 21 aa, Homo sapiens
MMTPINRFKVKKDPKMMKITK

SEQ ID NO: 3280 - protein, 37 aa, Homo sapiens
MMTRTVALLCSEGRPPSLASTLNSNALVCSWLKDRSA

SEQ ID NO: 3281 - protein, 13 aa, Homo sapiens
MMVAGKAVGCVAI

SEQ ID NO: 3282 - protein, 65 aa, Homo sapiens
MMVCQLFLGLGQFALSGFFGHHRMGREVGMGREVGMGREVGLGPHQHDPGEDKYIPPVTSTSLCD

SEQ ID NO: 3283 - protein, 71 aa, Homo sapiens
MMVCQLFLGLGQFALSGFFGHHRMGREVGMGREVGMGREVGMGREVGLGPHQHDPGEDKYIPPVTSTSLCD

SEQ ID NO: 3284 - protein, 76 aa, Homo sapiens
MMVCQLFLGLGQFALSGFFGHHRMGREVGMGREVGMGREVGMGREVGMGREVGLGPHQHDPGEDKYIPPVTSTSLC

SEQ ID NO: 3285 - protein, 77 aa, Homo sapiens
MMVCQLFLGLGQFALSGFFGHHRMGREVGMGREVGMGREVGMGREVGMGREVGLGPHQHDPGEDKYIPPVTSTSLCD

SEQ ID NO: 3286 - protein, 83 aa, Homo sapiens
MMVCQLFLGLGQFALSGFFGHHRMGREVGMGREVGMGREVGMGREVGMGREVGMGREVGLGPHQHDPGEDKYIPPVTSTSLCD

SEQ ID NO: 3287 - protein, 89 aa, Homo sapiens
MMVCQLFLGLGQFALSGFFGHHRMGREVGMGREVGMGREVGMGREVGMGREVGMGREVGMGREVGLGPHQHDPGEDKYIPPVTSTSLCD

SEQ ID NO: 3288 - protein, 18 aa, Homo sapiens
MMVSFHKPSSFSPSLSII

SEQ ID NO: 3289 - protein, 24 aa, Homo sapiens
MMVSTVSNRTAFPAFRLVSVLVAT

SEQ ID NO: 3290 - protein, 179 aa, Homo sapiens
MMVSTVSNRTAFPAFRLVSVLVATWASKSFMVSLLSSWFRPRIRSRRSIWTCRKGSLTPDMLCSVEYPIVTRVRRMCTSWGTTMVTLMKQLGTGWEEDTGEFRDLPDHVHCSQNSLLAHVGTGLQEQFLHLWGQVSAHLSRAHGAQSAQGQALYWLNPLAQVILDAVGNEQVGIVPLIQ

SEQ ID NO: 3291 - protein, 219 aa, Homo sapiens
MMVSTVSNRTAFPAFRLVSVLVATWASKSFMVSLLSSWFRPRIRSRRSIWTCRKGSLTPDMLCSVEYPIVTRVRRMCTSWGTTMVTLMKQLGTGWEEDTGEFRDLPDHVHCSQNSLLAHVGTGLQEQFLHLWGQVSAHLSRAHGAQSAQGQALYWLNPLAQVTVQSGRGSPTCGRRAVWPAAGACALGPRRGRRPGCGHTPFGSPPAPGPESWPRESLR

SEQ ID NO: 3292 - protein, 14 aa, Homo sapiens
MMYFSPSIIFMLEF

SEQ ID NO: 3293 - protein, 46 aa, Homo sapiens
MNAGCPRTLPFYKLPLLISPHNIFMSDAVIMPFNRMKSFVCEAHSS

SEQ ID NO: 3294 - protein, 16 aa, Homo sapiens
MNAKIEARKQRENIPE

SEQ ID NO: 3295 - protein, 115 aa, Homo sapiens
MNAKSSSSAKDHDSPLNAGPGSPPLPKAGCCTQQVILRSPASCEKSCAGRGGGAPGSAPGTQGRQGPLLSASENVGQAPHAPFCGGIACERPGRTLGERTGCTLHTSSGWTSPGR

SEQ ID NO: 3296 - protein, 101 aa, Homo sapiens [sequence omitted]

SEQ ID NO: 3297 - protein, 26 aa, Homo sapiens
MNCQGELVPKSFVTFFTFVRFLSSVD

SEQ ID NO: 3298 - protein, 13 aa, Homo sapiens
MNCSEDKSNCNLP

SEQ ID NO: 3299 - protein, 11 aa, Homo sapiens
MNESDSFPKGK

SEQ ID NO: 3300 - protein, 24 aa, Homo sapiens
MNFLRSETIFYFEFQMLWHILEAK

SEQ ID NO: 3301 - protein, 22 aa, Homo sapiens
MNFNFTNCHLYASFAPFANIIL

SEQ ID NO: 3302 - protein, 44 aa, Homo sapiens
MNGCDQWFEKHSSNTANIYKAIPGPDAIHSYSSPSFNPSINFVI

SEQ ID NO: 3303 - protein, 181 aa, Homo sapiens [sequence omitted]

SEQ ID NO: 3304 - protein, 30 aa, Homo sapiens
MNGLFSVVQSATQRSSFIFDLLWPILSLNE

SEQ ID NO: 3305 - protein, 11 aa, Homo sapiens
MNHSKCFNKFG

SEQ ID NO: 3306 - protein, 23 aa, Homo sapiens
MNHTRAELKSNFDLIRKQKLANQ

SEQ ID NO: 3307 - protein, 23 aa, Homo sapiens
MNIFFLFFLRWNLTGCPGWSAVA

SEQ ID NO: 3308 - protein, 16 aa, Homo sapiens
MNIFSVNDKNKHGLDI

SEQ ID NO: 3309 - protein, 18 aa, Homo sapiens
MNIFVHITATKRKFTLKT

SEQ ID NO: 3310 - protein, 127 aa, Homo sapiens [sequence omitted]

SEQ ID NO: 3311 - protein, 31 aa, Homo sapiens [sequence omitted]

SEQ ID NO: 3312 - protein, 25 aa, Homo sapiens
MNILRLVINSMNKVVHSRHIGFLMF

SEQ ID NO: 3313 - protein, 35 aa, Homo sapiens
MNINYIYICVCVHIYIFFIIFFCYRLNHTAPQKDS

SEQ ID NO: 3314 - protein, 18 aa, Homo sapiens
MNIRTRQYFAYQVGNDFK

SEQ ID NO: 3315 - protein, 36 aa, Homo sapiens
MNISAAWRLLGSPPSTSLGHTQTHWYFDEPCCPLKC

SEQ ID NO: 3316 - protein, 27 aa, Homo sapiens
MNKPKPAIKNDMNIFSVNDKNKHGLDI

SEQ ID NO: 3317 - protein, 15 aa, Homo sapiens
MNKVVHSRHIGFLMF

SEQ ID NO: 3318 - protein, 33 aa, Homo sapiens
MNLAVLPFKLHLLMSSFFNIVENLLLSPTTEPK

SEQ ID NO: 3319 - protein, 38 aa, Homo sapiens
MNLESFCQIPKQNFIVIHWKKHICQGRIGRVWKKCELL

SEQ ID NO: 3320 - protein, 12 aa, Homo sapiens
MNLFLCTVFGIS

SEQ ID NO: 3321 - protein, 13 aa, Homo sapiens
MNLHTKILQTVPS

SEQ ID NO: 3322 - protein, 24 aa, Homo sapiens
MNLIVHLLPSCLPFFLLSLSTYFH

SEQ ID NO: 3323 - protein, 13 aa, Homo sapiens
MNLLCPALAKDLG

SEQ ID NO: 3324 - protein, 15 aa, Homo sapiens
MNLNKYKYLRRVNPN

SEQ ID NO: 3325 - protein, 37 aa, Homo sapiens
MNLPQVHSGLCHLMLTEPKASKMPIWPVHVSLKINSI

SEQ ID NO: 3326 - protein, 23 aa, Homo sapiens
MNLRCSRGPALARSSFTTTWAGV

SEQ ID NO: 3327 - protein, 14 aa, Homo sapiens
MNMVLERCSGKGMS

SEQ ID NO: 3328 - protein, 16 aa, Homo sapiens
MNMYFFLISKDKRIGT

SEQ ID NO: 3329 - protein, 37 aa, Homo sapiens
MNNFWSRRSNTCVHPFKWVRRHPLSHRVRLPPMLYII

SEQ ID NO: 3330 - protein, 14 aa, Homo sapiens
MNNGIWLGQKIIHV

SEQ ID NO: 3331 - protein, 16 aa, Homo sapiens
MNNIKMNESDSFPKGK

SEQ ID NO: 3332 - protein, 74 aa, Homo sapiens [sequence omitted]

SEQ ID NO: 3333 - protein, 17 aa, Homo sapiens
MNNTDCTPDGCIPQTQH

SEQ ID NO: 3334 - protein, 27 aa, Homo sapiens
MNPAPMLARTSLIGKMKSLGTPFLSGW

SEQ ID NO: 3335 - protein, 27 aa, Homo sapiens
MNPASVLTRTSLIGKMKSLGTPFLSGW

SEQ ID NO: 3336 - protein, 18 aa, Homo sapiens
MNPCSIACAGGVFGISQR

SEQ ID NO: 3337 - protein, 39 aa, Homo sapiens
MNPLTEQSQVPWLSVLASFGLFSFGCLRPGMKQSKITHK

SEQ ID NO: 3338 - protein, 11 aa, Homo sapiens
MNPVCTSAHLN

SEQ ID NO: 3339 - protein, 40 aa, Homo sapiens
MNQDSDLFVKLMLYFHHFLAVPPPPLPRPLRYPHPPLQPP

SEQ ID NO: 3340 - protein, 32 aa, Homo sapiens
MNQDSDLFVKLMLYFHHFSGLVRSRSCSSYCR

SEQ ID NO: 3341 - protein, 14 aa, Homo sapiens
MNQLCTLPLRRRTG

SEQ ID NO: 3342 - protein, 23 aa, Homo sapiens
MNRAMTIKPCPWDRTMAQHMLTE

SEQ ID NO: 3343 - protein, 18 aa, Homo sapiens
MNREPGDTGKRVFQQQVE

SEQ ID NO: 3344 - protein, 40 aa, Homo sapiens
MNRIYASNQGWSPPKLSPLISQTAIFMLPLLPLQTSSCES

SEQ ID NO: 3345 - protein, 30 aa, Homo sapiens
MNRNCPCFSLLTTGTIGTELTNIRKISLHF

SEQ ID NO: 3346 - protein, 12 aa, Homo sapiens
MNRQCQDLLLDF

SEQ ID NO: 3347 - protein, 23 aa, Homo sapiens
MNSEMIPTTKTFSTFFTLMSFFT

SEQ ID NO: 3348 - protein, 20 aa, Homo sapiens
MNSFLINYYYKRIHIYCGKF

SEQ ID NO: 3349 - protein, 19 aa, Homo sapiens
MNSGAPPLEFGFLQIYTST

SEQ ID NO: 3350 - protein, 36 aa, Homo sapiens
MNSKVQNKHCIFSTIEYRSSPNCCSLEIDKIHEIAT

SEQ ID NO: 3351 - protein, 19 aa, Homo sapiens
MNSSDKCICMFGKKGRAAD

SEQ ID NO: 3352 - protein, 15 aa, Homo sapiens
MNSSICCLSYFLVFY

SEQ ID NO: 3353 - protein, 28 aa, Homo sapiens
MNSSMLSLARRSLSRLSCTASSSRGASS

SEQ ID NO: 3354 - protein, 14 aa, Homo sapiens
MNSSVASPSSPRIR

SEQ ID NO: 3355 - protein, 91 aa, Homo sapiens
MNSVPVRWARMRKERDWPVPGRGRQSSVFSISRCLLASGTSGRSGCPFCCGALSAGGGAPKGRAVLLRETLGAKVYRGGSAAGAEAFCGLL

SEQ ID NO: 3356 - protein, 12 aa, Homo sapiens
MNTLILHLDDKV

SEQ ID NO: 3357 - protein, 48 aa, Homo sapiens [sequence omitted]

SEQ ID NO: 3358 - protein, 46 aa, Homo sapiens
MNTSFHGWLLSWLLSIHQLLPTIILASPCSPRLSPLLLTSPPPAQP

SEQ ID NO: 3359 - protein, 47 aa, Homo sapiens
MNVSCLITQGRIITYKSQILRHILPPIVIPKQNESRSQVTSLPNTIY

SEQ ID NO: 3360 - protein, 13 aa, Homo sapiens
MNVTFMFALPLAP

SEQ ID NO: 3361 - protein, 32 aa, Homo sapiens
MNVYYCPPQVFSKITLKSCFETLSFLGNKIHL

SEQ ID NO: 3362 - protein, 12 aa, Homo sapiens
MNWMLQQLPSWV

SEQ ID NO: 3363 - protein, 22 aa, Homo sapiens
MNYKIPRTQLAGGRSGGGCEKP

SEQ ID NO: 3364 - protein, 79 aa, Homo sapiens
MPAHSFVPHARKTRPPMSFPHCHLQLQIKVCILRNDPLRSSSGQSLLLEPTAATPQDRVCRRLDRGSLGLLCSIQCQRS

SEQ ID NO: 3365 - protein, 33 aa, Homo sapiens
MPAKSVSPLFPGVLGQKAQIPQKLMTFHLPHLG

SEQ ID NO: 3366 - protein, 30 aa, Homo sapiens
MPAMEPRAIMKIKDKFTEPIDSWASRAGDK

SEQ ID NO: 3367 - protein, 19 aa, Homo sapiens
MPAPAPAAPLPARGAPGRA

SEQ ID NO: 3368 - protein, 16 aa, Homo sapiens
MPARPQVVWTNACLCP

SEQ ID NO: 3369 - protein, 43 aa, Homo sapiens
MPARPVGRQSSCLPNSQPTIQAPELKINLLLRDPSDPVGIRVK

SEQ ID NO: 3370 - protein, 11 aa, Homo sapiens
MPASHSTGGFQ

SEQ ID NO: 3371 - protein, 16 aa, Homo sapiens
MPCDEPTALHQKHLFQ

SEQ ID NO: 3372 - protein, 28 aa, Homo sapiens
MPCKRTSLLVIYICTRLMINTDHYIFLF

SEQ ID NO: 3373 - protein, 44 aa, Homo sapiens
MPCLGPSQPGLHTVPFWHCRPWPVSSAQGEGSSSAGTSAMPSWL

SEQ ID NO: 3374 - protein, 34 aa, Homo sapiens
MPCSKVQASAGDHPDFLWTSALSFHPPALSIESK

SEQ ID NO: 3375 - protein, 51 aa, Homo sapiens
MPCSRRCRALKFSTPHCGMAMLASSVNVSEKLILPGWVSGAGVPGVLKDKG

SEQ ID NO: 3376 - protein, 11 aa, Homo sapiens
MPCTGQRSWVK

SEQ ID NO: 3377 - protein, 20 aa, Homo sapiens
MPDAAADHSSVQETRMPGRA

SEQ ID NO: 3378 - protein, 33 aa, Homo sapiens
MPDAGPHLHGPAQQRGQRRDLRLWAGDGQSQWG

SEQ ID NO: 3379 - protein, 17 aa, Homo sapiens
MPDLLNVNESVAGQYHG

SEQ ID NO: 3380 - protein, 21 aa, Homo sapiens
MPDLSCIFSRDGVPPCWSGWS

SEQ ID NO: 3381 - protein, 16 aa, Homo sapiens
MPEGTTKVNDLAVSNE

SEQ ID NO: 3382 - protein, 22 aa, Homo sapiens
MPEGTTKVNDLAVSNEYFGLVG

SEQ ID NO: 3383 - protein, 18 aa, Homo sapiens
MPELFIYECQKQQLCKGP

SEQ ID NO: 3384 - protein, 16 aa, Homo sapiens
MPETTLLPADTKKKSR

SEQ ID NO: 3385 - protein, 36 aa, Homo sapiens
MPEVLLSTGICYTAAQYVLPRERVSHCHLYVHRWSW

SEQ ID NO: 3386 - protein, 11 aa, Homo sapiens
MPFLLSSFQMF

SEQ ID NO: 3387 - protein, 23 aa, Homo sapiens
MPFSLAKVSSNPFSASSNVCLYH

SEQ ID NO: 3388 - protein, 18 aa, Homo sapiens
MPFSSLQAPHQSSTRSQK

SEQ ID NO: 3389 - protein, 25 aa, Homo sapiens
MPGFKPFPLPRLPKCWDYRCEPLPS

SEQ ID NO: 3390 - protein, 65 aa, Homo sapiens
MPGPWRDRSWPEAVAGWGAWRKGSVVLTILPLDSRLACAHCMTSGLRSDGPSLEISPLRRSWTRP

SEQ ID NO: 3391 - protein, 39 aa, Homo sapiens
MPGQAALPSWAKTLTHQLHGALGGRSSHGSGWGWAAGSG

SEQ ID NO: 3392 - protein, 54 aa, Homo sapiens
MPGSQAGVPDRPPALACSALRAARDASAPLLPDRGGSGETATLPSPRTALHPQQ

SEQ ID NO: 3393 - protein, 110 aa, Homo sapiens
MPGSRGSSLVVPILSWLLHVGFALCGCYLHSGVHLPCGGRMIAGSPRLPLSNPHGKRESFLPRASRSPGIGSMPVHNCGPWGGIHRLDRSDKWSHSLIISPWLDRKEGPF

SEQ ID NO: 3394 - protein, 28 aa, Homo sapiens
MPGSSFPLTMANSPVFLTAPPTRRKTVP

SEQ ID NO: 3395 - protein, 35 aa, Homo sapiens
MPGTASVTSTHDVGPKYACVEVFWQLLQALTAGAG

SEQ ID NO: 3396 - protein, 27 aa, Homo sapiens
MPGYFCSFSRDWVSPYSSGWSQTPDLR

SEQ ID NO: 3397 - protein, 32 aa, Homo sapiens
MPGYFFFFFFCIFNRDRVSPCWSGWSRTPDLR

SEQ ID NO: 3398 - protein, 11 aa, Homo sapiens
MPGYFFFFPYF

SEQ ID NO: 3399 - protein, 23 aa, Homo sapiens
MPHALSEQLQSLEPIPFSFCKDI

SEQ ID NO: 3400 - protein, 47 aa, Homo sapiens [sequence omitted]

SEQ ID NO: 3401 - protein, 18 aa, Homo sapiens
MPHLMKWCCLSQTQSHCC

SEQ ID NO: 3402 - protein, 12 aa, Homo sapiens
MPIISMVKGREQ

SEQ ID NO: 3403 - protein, 12 aa, Homo sapiens
MPILFSAAIRKK

SEQ ID NO: 3404 - protein, 121 aa, Homo sapiens
MPIRTALSSSQSLNIISGDLPPSSRETFFKLLTAQLFMICLPIGVDPVKPSLRMSGCSDRRCPAMPPEPGMMLMTPFGKPAFTDSSANFKAVKGVTCAGLSTKVLPAAKHAALFHASIISG

SEQ ID NO: 3405 - protein, 15 aa, Homo sapiens
MPIWPVHVSLKINSI

SEQ ID NO: 3406 - protein, 94 aa, Homo sapiens [sequence omitted]

SEQ ID NO: 3407 - protein, 11 aa, Homo sapiens
MPKLGSPVQWE

SEQ ID NO: 3408 - protein, 16 aa, Homo sapiens
MPKRFRSLRQRLRYLW

SEQ ID NO: 3409 - protein, 35 aa, Homo sapiens
MPKVINQSRAPPLPPPPTPSQQADISQLQKQACWR

SEQ ID NO: 3410 - protein, 16 aa, Homo sapiens
MPLCSFVFMPFVFPAG

SEQ ID NO: 3411 - protein, 29 aa, Homo sapiens
MPLFFFPLQAALPHPSSSWQLNTRASFWC

SEQ ID NO: 3412 - protein, 15 aa, Homo sapiens
MPLIATKSPLECFAA

SEQ ID NO: 3413 - protein, 50 aa, Homo sapiens
MPLKAYFAKLLLQVFLFGKSITVGHSCLLDEQKRKICLWQPESFTVFQVV

SEQ ID NO: 3414 - protein, 19 aa, Homo sapiens
MPLKKVCLILLVKYNFELF

SEQ ID NO: 3415 - protein, 23 aa, Homo sapiens
MPLKKVCLILLVKYNFELFLFFS

SEQ ID NO: 3416 - protein, 34 aa, Homo sapiens
MPLLLAKMLFQTDLGRKVLILPLAISIQGNFFPS

SEQ ID NO: 3417 - protein, 11 aa, Homo sapiens
MPLLSLMSTVA

SEQ ID NO: 3418 - protein, 20 aa, Homo sapiens
MPLNVLRSGIVYNSSLFPHI

SEQ ID NO: 3419 - protein, 25 aa, Homo sapiens
MPLQTTAQCRRPGCQEGPELQLTRC

SEQ ID NO: 3420 - protein, 60 aa, Homo sapiens [sequence omitted]

SEQ ID NO: 3421 - protein, 13 aa, Homo sapiens
MPLSHVFLRTGLN

SEQ ID NO: 3422 - protein, 28 aa, Homo sapiens
MPLTPGSGALRPAVAARRAWARRPGALG

SEQ ID NO: 3423 - protein, 44 aa, Homo sapiens
MPLTQHPTSSRTAEASPQPFSLQRGLPGSGVRRQSQCFAAKVMG

SEQ ID NO: 3424 - protein, 36 aa, Homo sapiens
MPLVLLSKVPGPSNMNYKIPRTQLAGGRSGGGCEKP

SEQ ID NO: 3425 - protein, 16 aa, Homo sapiens
MPLVREILGQFLWDHK

SEQ ID NO: 3426 - protein, 38 aa, Homo sapiens
MPNKVDCPIGSIANQFNRFKITFPRFPSKFQGGIRATH

SEQ ID NO: 3427 - protein, 37 aa, Homo sapiens
MPPAIFFPQKSGGKYLLSLAEQYQCWLFCDHLGFSSW

SEQ ID NO: 3428 - protein, 30 aa, Homo sapiens
MPPCPANFCIFSRDGISPRWPGWSRAPDLR

SEQ ID NO: 3429 - protein, 118 aa, Homo sapiens
MPPCPANFLYFLVETGFRHVGQAGLKLLTSGDPPALASQSAGITDVNHCAQPGPSLSKQKPGSCYRIGQCVCYYRGRSEHFFSVSGRSQLVWRLPALPLPPALAFLLGTARRSTTCVY

SEQ ID NO: 3430 - protein, 27 aa, Homo sapiens
MPPCPANFYIFSKDGVFIILDRLVWNT

SEQ ID NO: 3431 - protein, 46 aa, Homo sapiens
MPPHLANFCIFSRDGVSPWPGWSRTPDLRGSRCEPLRPAKNKILSS

SEQ ID NO: 3432 - protein, 64 aa, Homo sapiens
MPPHLANFYFCRHLYVAQAGLKLLDSSDPPALVSQSVATTGMSRRAWQDIILQQKQAATAAVCL

SEQ ID NO: 3433 - protein, 22 aa, Homo sapiens
MPPHLATFLYFSRDRVSPCCSG

SEQ ID NO: 3434 - protein, 22 aa, Homo sapiens
MPPHPANFCIFSRVGVSPCGPG

SEQ ID NO: 3435 - protein, 12 aa, Homo sapiens
MPPHPANFLYFW

SEQ ID NO: 3436 - protein, 51 aa, Homo sapiens
MPPHPANFYTFSRDSVSPCFPEWSLSPDLMIRPPQPPKVLALQALNHHVWP

SEQ ID NO: 3437 - protein, 12 aa, Homo sapiens
MPPPHPANFLYF

SEQ ID NO: 3438 - protein, 45 aa, Homo sapiens
MPPRLANFCIFSRDGISPYWPCWSRTADLKIHSLAQPVKVLGLQT

SEQ ID NO: 3439 - protein, 11 aa, Homo sapiens
MPPRPANFLYF

SEQ ID NO: 3440 - protein, 11 aa, Homo sapiens
MPPRPATFLYF

SEQ ID NO: 3441 - protein, 30 aa, Homo sapiens
MPPRSGNFCIFSRDGVSPSWPGWSRTPDLR

SEQ ID NO: 3442 - protein, 26 aa, Homo sapiens
MPPSCVPSGGPWAASPWQPRHSFGSG

SEQ ID NO: 3443 - protein, 18 aa, Homo sapiens
MPPTLEWMSKLQCLCTVE

SEQ ID NO: 3444 - protein, 27 aa, Homo sapiens
MPPWLANFVFLVETEFHHVGQAGLENS

SEQ ID NO: 3445 - protein, 74 aa, Homo sapiens
MPQKNTGIFCSWTWSLPCLPFQKREQKAWGQPAEARSSSLLLDDLSVKHVVPAGPGTAMSQNNERERKTKKERK

SEQ ID NO: 3446 - protein, 52 aa, Homo sapiens
MPQSLFPDKSLFFKLLFSFWRSRIILLFLSTSVFKKLIVAWCFSAFSDVSLS

SEQ ID NO: 3447 - protein, 65 aa, Homo sapiens
MPQTKIILPSWETCHGSRMSWEERARGWDSWGHTRASAHPDYTQGQGGDRQMPGSYSLRARSELG

SEQ ID NO: 3448 - protein, 11 aa, Homo sapiens
MPQVLGPHLEK

SEQ ID NO: 3449 - protein, 25 aa, Homo sapiens
MPQVSCMTSAGNQPQKQSFHIFLPA

SEQ ID NO: 3450 - protein, 11 aa, Homo sapiens
MPREIHPAECS

SEQ ID NO: 3451 - protein, 64 aa, Homo sapiens
MPRMTVGWEAGRPLRWTCLCRGRCDFTTSGRARGRVCRSSMELICWDTVSSCRNRSSYCSSGWA

SEQ ID NO: 3452 - protein, 19 aa, Homo sapiens
MPRNVRHALILSSSVPGSN

SEQ ID NO: 3453 - protein, 39 aa, Homo sapiens
MPRRGGGVATYEKQLKINLKSTTMSCAGLHSPEVSAQEG

SEQ ID NO: 3454 - protein, 22 aa, Homo sapiens
MPRTLSGQTLHRKNTFQDLYSM

SEQ ID NO: 3455 - protein, 54 aa, Homo sapiens
MPSAGGGLLRTAQTARWGCQGWPQAAQGEWPVLGGRGVRPGASGSPGCWPSLGW

SEQ ID NO: 3456 - protein, 20 aa, Homo sapiens
MPSARHFWKRQYWHLLRFFF

SEQ ID NO: 3457 - protein, 35 aa, Homo sapiens
MPSFGAISSLTTVTLGKFLLLFFSTKQPSEKNVSL

SEQ ID NO: 3458 - protein, 28 aa, Homo sapiens
MPSGLELAFLGKPRDGFVSEAETVPRAY

SEQ ID NO: 3459 - protein, 20 aa, Homo sapiens
MPSHSLINLLCAVTEICDSI

SEQ ID NO: 3460 - protein, 28 aa, Homo sapiens
MPSLAWAFLTKKRCKRGCTLTLQHSRLS

SEQ ID NO: 3461 - protein, 71 aa, Homo sapiens [sequence omitted]

SEQ ID NO: 3462 - protein, 38 aa, Homo sapiens
MPSLLEVTASTSFQLGWKNKLDQREVGGGPVGGPEAGH

SEQ ID NO: 3463 - protein, 32 aa, Homo sapiens
MPSLVLNSLSVIPATREAEAGESLEPRRWRSQ

SEQ ID NO: 3464 - protein, 11 aa, Homo sapiens
MPSQYPESYVF

SEQ ID NO: 3465 - protein, 64 aa, Homo sapiens
MPSRDGLGEPHQEGHPMWTGGGSFPIQQKVRRWLKCPFFHVTHAFFFFFFETESHSGPGWSAVA

SEQ ID NO: 3466 - protein, 31 aa, Homo sapiens
MPSSPAEAIWQHLQLIKKWVAEVQYQPMFQS

SEQ ID NO: 3467 - protein, 12 aa, Homo sapiens
MPSVPIKMDIVM

SEQ ID NO: 3468 - protein, 40 aa, Homo sapiens
MPSVPRPFVVLIPAATDKDTSLTPKLCTQHTQKWDVLHKN

SEQ ID NO: 3469 - protein, 27 aa, Homo sapiens
MPSYFFVFLVEMGFHHVSQDGLDLLNL

SEQ ID NO: 3470 - protein, 33 aa, Homo sapiens
MPTAAPAPPGPRPPLRLQSRGRMGREGAGRSPR

SEQ ID NO: 3471 - protein, 13 aa, Homo sapiens
MPTFKRSLKLTGQ

SEQ ID NO: 3472 - protein, 51 aa, Homo sapiens
MPTFLMSWPLTGNGGMDHCCISFRRQCSPWYFSSSHTRVVASGSLESIMKS

SEQ ID NO: 3473 - protein, 20 aa, Homo sapiens
MPTGQGQRLVSCLMIHYNTV

SEQ ID NO: 3474 - protein, 16 aa, Homo sapiens
MPTMCQTLFPDSFCAL

SEQ ID NO: 3475 - protein, 28 aa, Homo sapiens
MPTMDFSTLVTYVTWSSLDLSSFCCILS

SEQ ID NO: 3476 - protein, 55 aa, Homo sapiens
MPTQLTIVFLNEYYCIVFAYLVGQKMQRVTDSRFRSRDSGLFLLSNGPRFRSSHS

SEQ ID NO: 3477 - protein, 11 aa, Homo sapiens
MPTRLANFFVF

SEQ ID NO: 3478 - protein, 14 aa, Homo sapiens
MPTSGHSNCASQTV

SEQ ID NO: 3479 - protein, 96 aa, Homo sapiens
MPVFLPGSPGLQEGVFSLSPGTRRGCHQAPTRVGHFTPRVVLKAPHTPSCRRKGTLPRRPNSEMGTGARRLGARYCRDTSFGALRLGFSPPRLLTC

SEQ ID NO: 3480 - protein, 92 aa, Homo sapiens
MPVGVKPFSVSTLSLSSLSTENTLAILPIARILFLITSFRAAAVAPSNPSSSDPSSSSEQMLRTFTSISVTFSPTNGRDQVKTSMKFGSQYG

SEQ ID NO: 3481 - protein, 78 aa, Homo sapiens
MPVGVKPFSVSTLSLSSLSTENTLAILPIARILFLITSFRAAAVAPSNPSSSDPSSSSEQMLRTFTSISVTLLLYTSK

SEQ ID NO: 3482 - protein, 24 aa, Homo sapiens
MPVHSTQRQNLLVEVVGDLLSLFS

SEQ ID NO: 3483 - protein, 11 aa, Homo sapiens
MPWESPRQMPA

SEQ ID NO: 3484 - protein, 60 aa, Homo sapiens
MPWRSERGVLGFFRVILYFSSLHLCRISKLLWWTGCWRKLKLSILFKIAHGAVSSCPVFL

SEQ ID NO: 3485 - protein, 20 aa, Homo sapiens
MPWRSERGVLGFFRVIPVFL

SEQ ID NO: 3486 - protein, 24 aa, Homo sapiens
MPWSALHALNVLKNLQKQTSGAEK

SEQ ID NO: 3487 - protein, 87 aa, Homo sapiens
MPWSLFWGHPTLNLFRGRKTAQLLSVEQAPPGPPWSCPRQQKGLTNPAIPHLQRGHRTAHICLACQLVGNRPSRFTLLLSSQGSLQR

SEQ ID NO: 3488 - protein, 36 aa, Homo sapiens
MPWVVEPIGTSGSSPSLQQSLLEATRWTSVPLRTTV

SEQ ID NO: 3489 - protein, 23 aa, Homo sapiens
MPYHGNSRVIRVLGLSYSSAFPF

SEQ ID NO: 3490 - protein, 49 aa, Homo sapiens
MPYTPCCSSEWEVQVGLLPGGGAVSDNHCHLGLPTARGTRPLSKQHTGI

SEQ ID NO: 3491 - protein, 33 aa, Homo sapiens
MQAAAGATDTARGDTLTTKEQPQAQKHTCSLRT

SEQ ID NO: 3492 - protein, 23 aa, Homo sapiens
MQAADSAQQDRSNTQMQFLYVEH

SEQ ID NO: 3493 - protein, 15 aa, Homo sapiens
MQAAPGHFHFINFHF

SEQ ID NO: 3494 - protein, 29 aa, Homo sapiens
MQARRSPRPGHLGPLVYRSNLFMDNLVTT

SEQ ID NO: 3495 - protein, 27 aa, Homo sapiens
MQCHSRGLMDPPPNTLLPLFRGTSVSL

SEQ ID NO: 3496 - protein, 27 aa, Homo sapiens
MQDAFSKHDTALGEMQMKGVLCRRYSL

SEQ ID NO: 3497 - protein, 18 aa, Homo sapiens
MQDLTVKALKHSTQNETI

SEQ ID NO: 3498 - protein, 81 aa, Homo sapiens [sequence omitted]

SEQ ID NO: 3499 - protein, 89 aa, Homo sapiens
MQDPEILVVVELLSVGRGKLPSKDPQLSATLRHYHRLVSTAPRRWTGDVNFGPGVLSGIVDIELVIQKSFTFWPLKYSPPKRINSSFSG

SEQ ID NO: 3500 - protein, 81 aa, Homo sapiens
MQDPEILVVVELLSVGRGKLPSKDPQLSATLRHYHRLVSTAPRRWTGDVNFGPGVLSGIVDIELVIQKSLGEGGGHGSSTV

SEQ ID NO: 3501 - protein, 112 aa, Homo sapiens
MQDPEILVVVELLSVGRGKLPSKDPQLSATLRHYHRLVSTAPRRWTGDVNFGPGVLSGIVDIELVIQKSLQKGLTHLSQDEPRGRHLTLVRVGGTEVPQSESSWHRVSGNGL

SEQ ID NO: 3502 - protein, 20 aa, Homo sapiens
MQDSEYHNSIHTALIVNSPA

SEQ ID NO: 3503 - protein, 52 aa, Homo sapiens [sequence omitted]

SEQ ID NO: 3504 - protein, 20 aa, Homo sapiens
MQEYGSILANPMLVIHPVTL

SEQ ID NO: 3505 - protein, 18 aa, Homo sapiens
MQFFTRVLVRTSSLLDAL

SEQ ID NO: 3506 - protein, 47 aa, Homo sapiens
MQFKCRGWNEPLFCSLPAAAWANLGVHWARQVSMHTPCPPHAVTVRA

SEQ ID NO: 3507 - protein, 25 aa, Homo sapiens
MQGLSYNMELSRAWRQSKGGGLFGR

SEQ ID NO: 3508 - protein, 43 aa, Homo sapiens
MQGLWVLREPPEALSPASTAGGKTPTSPPSTAHTAHLLSSLLH

SEQ ID NO: 3509 - protein, 27 aa, Homo sapiens
MQGMFFSVKATVLMCFSFALYHQILYI

SEQ ID NO: 3510 - protein, 43 aa, Homo sapiens
MQGPSYLLSKVQSKGLGVGWWTSKCMLFSKNSNLTMNLLAKGI

SEQ ID NO: 3511 - protein, 77 aa, Homo sapiens
MQGRQSTICWRYFSSLGGKEMQLSWPACSPVSATSPAGPRSAPPPPVREERQVWLWEHLMSRKNFWVSRRFCRSRPR

SEQ ID NO: 3512 - protein, 29 aa, Homo sapiens
MQGSKVKWKRKSNSSLLILKLSTAKVSPF

SEQ ID NO: 3513 - protein, 13 aa, Homo sapiens
MQGWAGARGSQTG

SEQ ID NO: 3514 - protein, 20 aa, Homo sapiens
MQILLLALQICDAGLSAMWN

SEQ ID NO: 3515 - protein, 15 aa, Homo sapiens
MQILPRDVVVIKISA

SEQ ID NO: 3516 - protein, 30 aa, Homo sapiens
MQILVLQPSPPLRCRLEDAAAASRAALPRF

SEQ ID NO: 3517 - protein, 17 aa, Homo sapiens
MQIQNISVFADTSIKHH

SEQ ID NO: 3518 - protein, 16 aa, Homo sapiens
MQIRRVQSAISTGQRG

SEQ ID NO: 3519 - protein, 87 aa, Homo sapiens
MQISDTFNVIFLKFILNLFIYLFFETESRSVAQAGVQWHDLGSLQAPPPGFTPFSCLSLPSSWDYRHPPPCLANFFCIFSRDGVSPC

SEQ ID NO: 3520 - protein, 21 aa, Homo sapiens
MQITILSSCKLQLITFLLIFC

SEQ ID NO: 3521 - protein, 16 aa, Homo sapiens
MQKGHCFFFFFNFILF

SEQ ID NO: 3522 - protein, 62 aa, Homo sapiens
MQKGPSQMFLPMAFIMEFKRGSPGPPHDSCELIKNSNDGGEDGGGDDGNDRCSPQKALMPGD

SEQ ID NO: 3523 - protein, 58 aa, Homo sapiens
MQLAMRNCSPSTMFICENIENLLFQLICCYMISMFSSTDKMVTHLFFLSSISSILGTL

SEQ ID NO: 3524 - protein, 45 aa, Homo sapiens
MQLGNLHPDSKKMKMCQWKWHWQKTSPSRNSYRYFVTLQEQRIKH

SEQ ID NO: 3525 - protein, 16 aa, Homo sapiens
MQLHRAINLHCVCKLS

SEQ ID NO: 3526 - protein, 13 aa, Homo sapiens
MQLLKMTVLYTLI

SEQ ID NO: 3527 - protein, 24 aa, Homo sapiens
MQLLLNGNWLCLCGRLRWDLFLRE

SEQ ID NO: 3528 - protein, 234 aa, Homo sapiens
MQLLTEELGAVRPHLLVKGHFQQLECAGAQLEPVLQELVHRGLDADALLLGQRSHREGADHHLLPNQGVRGHPREDDPVRGEEDGALSWEQCWSPSTAPRALLTPIRQQVDAQAVQHTLLTRQQARPQQLGLLDGRQPPALPLHGLQGLDVHLDNVWHHDMQPLEVVAGDPTLRADLVHKAVDEADHSPSYVAGLCILEAALRVIALGHTASHAVGDQAVAGALQVAQPGTLPK

SEQ ID NO: 3529 - protein, 26 aa, Homo sapiens
MQLPSQTQVLSGDCRHLLHSGLHFYY

SEQ ID NO: 3530 - protein, 13 aa, Homo sapiens
MQMKGVLCRRYSL

SEQ ID NO: 3531 - protein, 56 aa, Homo sapiens [sequence omitted]

SEQ ID NO: 3532 - protein, 37 aa, Homo sapiens
MQPLCLACSSATAQAAAPAHSSEALPCAQEAPGLVQL

SEQ ID NO: 3533 - protein, 25 aa, Homo sapiens
MQPLGAPWLRDQSVSTKHNRCQPRR

SEQ ID NO: 3534 - protein, 19 aa, Homo sapiens
MQQFNDKNILIFYYTAARS

SEQ ID NO: 3535 - protein, 19 aa, Homo sapiens
MQQNRGLRNNTTHLQPSDL

SEQ ID NO: 3536 - protein, 101 aa, Homo sapiens [sequence omitted]

SEQ ID NO: 3537 - protein, 19 aa, Homo sapiens
MQQTLQMLSPREEIFEKTN

SEQ ID NO: 3538 - protein, 22 aa, Homo sapiens
MQRGISNLGLIVSHPVKCSLTS

SEQ ID NO: 3539 - protein, 55 aa, Homo sapiens
MQRLGDGEGAFWPDAAGAGSSVSDTCPPTARRGWGRTRVNPAATAASPHCVFGVR

SEQ ID NO: 3540 - protein, 25 aa, Homo sapiens
MQRLKLGSREKTFQNDTTLLNTYNT

SEQ ID NO: 3541 - protein, 30 aa, Homo sapiens
MQRVTDSRFRSRDSGLFLLSNGPRFRSSHS

SEQ ID NO: 3542 - protein, 11 aa, Homo sapiens
MQSALRKRRIL

SEQ ID NO: 3543 - protein, 18 aa, Homo sapiens
MQSCIIKWIYLNCRNNHC

SEQ ID NO: 3544 - protein, 34 aa, Homo sapiens
MQSGPAVRPVPPPSAPAPSRTEPTRAGCSAVSPG

SEQ ID NO: 3545 - protein, 15 aa, Homo sapiens
MQTCHQILKNHLLAH

SEQ ID NO: 3546 - protein, 28 aa, Homo sapiens
MQTKLLLHYTQRKEKKGILLNFTWSTKS

SEQ ID NO: 3547 - protein, 184 aa, Homo sapiens [sequence omitted]

SEQ ID NO: 3548 - protein, 45 aa, Homo sapiens [sequence omitted]

SEQ ID NO: 3549 - protein, 45 aa, Homo sapiens [sequence omitted]

SEQ ID NO: 3550 - protein, 87 aa, Homo sapiens [sequence omitted]

SEQ ID NO: 3551 - protein, 78 aa, Homo sapiens
MQWTQQSSCAWRGIWEVVDLLLLLLFLLPWLARDGCVCNFRWALGPPRAPFPARLVPPSSEGWPESFGRSGVQPKGFP

SEQ ID NO: 3552 - protein, 27 aa, Homo sapiens
MQYISLHSKSDLYSSFQQIPHLNLRPP

SEQ ID NO: 3553 - protein, 16 aa, Homo sapiens
MQYSLTHNHMKSTHIH

SEQ ID NO: 3554 - protein, 92 aa, Homo sapiens
MQYSPIAERVVESVRQANKLGLGGINHLRSWISANMQQNRGWDGRTEGRRPSCSPHRLYGVGRNLCKEGRYWLRGGLWGLLFVAPESREVKI

SEQ ID NO: 3555 - protein, 67 aa, Homo sapiens
MRAERQLKGEEHHLQKLATTPGAWSNINKLFSFCHPGKCLGIFTVFLQNSVSSSQPGMLCVQAEPSR

SEQ ID NO: 3556 - protein, 54 aa, Homo sapiens
MRAPRPWTSSLQNCEKQISVVYQPHTLWKFFIERVFSRKMRTRRRNAQGKGKKR

SEQ ID NO: 3557 - protein, 17 aa, Homo sapiens
MRASILMSGRKGISNPG

SEQ ID NO: 3558 - protein, 57 aa, Homo sapiens
MRCYGKKIDLVGQPLGGLHCGNIGVDQQRLDVFLLQGLNCLRARVVKFSSLANGEAP

SEQ ID NO: 3559 - protein, 31 aa, Homo sapiens
MREEMYLLKALLRSPFFDTGSHSVAQSSLQP

SEQ ID NO: 3560 - protein, 59 aa, Homo sapiens
MREKPLPSWLALSWGSRKSVCRSGPSAFKSKLSLWHRKLPNFSLRGLLSLGIPGRGPHW

SEQ ID NO: 3561 - protein, 30 aa, Homo sapiens
MRELDFPVHSHTLSLPRPETEQALVLGLQR

SEQ ID NO: 3562 - protein, 24 aa, Homo sapiens
MRELLHLKWTLDLLLGNFLKKVTF

SEQ ID NO: 3563 - protein, 55 aa, Homo sapiens
MRESKCQRFCFQQEFAIQLPSMFSPESEFPIAICMCIDGHGKRGHYRTEDIAEMQ

SEQ ID NO: 3564 - protein, 21 aa, Homo sapiens
MREVCKGEGLPQENTKALPQI

SEQ ID NO: 3565 - protein, 87 aa, Homo sapiens
MRFFSRMRQDLLSHFTCMVLTGHSSLELPWPQLIAARGIQLHRSCYSLFVLTSHIFWLSQHPVFILWRNKEFFHFCFFDIRRLGCHK

SEQ ID NO: 3566 - protein, 31 aa, Homo sapiens
MRFHHVGQAGLELLTSSDPPASASKVLGLQM

SEQ ID NO: 3567 - protein, 63 aa, Homo sapiens
MRFPTSVLSRVEMICSWVSLLSMMLYSSIKHRISTMVWFPLSARSMQGPSLFSARESRNFLVL

SEQ ID NO: 3568 - protein, 18 aa, Homo sapiens
MRGFFFHSFTNTWYYLIL

SEQ ID NO: 3569 - protein, 41 aa, Homo sapiens
MRGLTCMGQPSRGAREGTSGSGQGMVRVNGVRRKKGPGTGK

SEQ ID NO: 3570 - protein, 18 aa, Homo sapiens
MRGPHMLSLARRCTGDLV

SEQ ID NO: 3571 - protein, 63 aa, Homo sapiens
MRGPVSPEDSSGHLDASISATCPSGSLLALDSPCCFSSPALLLLLPQAPLDPAAAARRHPSFH

SEQ ID NO: 3572 - protein, 25 aa, Homo sapiens
MRGRARACHAPRVWPVPRPQRPSFF

SEQ ID NO: 3573 - protein, 35 aa, Homo sapiens
MRGRTVRILVFTMSKTFRCFTESNFMSQYEATLVL

SEQ ID NO: 3574 - protein, 138 aa, Homo sapiens
MRGWEAAPLGLGKQEVLQELGPEGAGCSDITQDHGLQAQSCRREGSKGHIYFGFPLHVLQAPQLILQPLHGISERMLLSSHGPSLGPEEESSTLGVLSVLTCLLHGRVLSLSVSLHQLQALVEFLDFCPQAGHSSFQL

SEQ ID NO: 3575 - protein, 12 aa, Homo sapiens
MRGWWQRWKTEI

SEQ ID NO: 3576 - protein, 13 aa, Homo sapiens
MRHDTWLIFFFYF

SEQ ID NO: 3577 - protein, 38 aa, Homo sapiens
MRHEGDEVTTSSHCVTARPQPKAGLRPPSSSAPAAGIT

SEQ ID NO: 3578 - protein, 30 aa, Homo sapiens
MRHHAQLIFVFLIETGFHHVGQDGLDLLTL

SEQ ID NO: 3579 - protein, 12 aa, Homo sapiens
MRHHAQLILYFW

SEQ ID NO: 3580 - protein, 30 aa, Homo sapiens
MRHHARLIFALLVETGFHRVSQDGLDLLIS

SEQ ID NO: 3581 - protein, 21 aa, Homo sapiens
MRHHARLIFVFLVETGFHHIG

SEQ ID NO: 3582 - protein, 11 aa, Homo sapiens
MRHHARLILYF

SEQ ID NO: 3583 - protein, 13 aa, Homo sapiens
MRHHPRLLFFLYF

SEQ ID NO: 3584 - protein, 45 aa, Homo sapiens
MRHHTGLILYFLVEMEFLHVGHLVSNSRPQVIRPPWPPKVLGLQA

SEQ ID NO: 3585 - protein, 13 aa, Homo sapiens
MRHHTRLIFVFFF

SEQ ID NO: 3586 - protein, 73 aa, Homo sapiens
MRHHTWLIFVFWGEMGFHPVGQAGLELLTSSDPPALAFQSAGITGVSHRTRPGTPQILISDPAKNIVTCLNGH

SEQ ID NO: 3587 - protein, 83 aa, Homo sapiens
MRHKEFKPQISPSWFVPPLEPSPLGGRAKVTGKVSGRLFLKCRQVICSARSVSLVPRACSAGGSGLRYPLPSRGCRRRWARAR

SEQ ID NO: 3588 - protein, 23 aa, Homo sapiens
MRHQCQLSFKFFCRDRVLLCCPH

SEQ ID NO: 3589 - protein, 18 aa, Homo sapiens
MRHQQCIMLTFCKTFHTF

SEQ ID NO: 3590 - protein, 20 aa, Homo sapiens
MRICIICKGHPTVITWERLW

SEQ ID NO: 3591 - protein, 13 aa, Homo sapiens
MRIDFSFVSPKLF

SEQ ID NO: 3592 - protein, 19 aa, Homo sapiens
MRILFAFDQRMLLLSLYSR

SEQ ID NO: 3593 - protein, 11 aa, Homo sapiens
MRILGEVCLLK

SEQ ID NO: 3594 - protein, 31 aa, Homo sapiens
MRIQTDSLMALISGELFSDKYAQNFVRTDPT

SEQ ID NO: 3595 - protein, 78 aa, Homo sapiens
MRIRVRYWSSMTLKREFRSALGNWIFISCRTLFRKIHFCWKVSHTSSRAPRPCMMATHSKAILFKSPDFSMAKILDNT

SEQ ID NO: 3596 - protein, 56 aa, Homo sapiens
MRIRWHSAVKICSFSSDVSSKNSEVSSFSRNSSCTSLSSNAAESLLSSVSEPSLSS

SEQ ID NO: 3597 - protein, 27 aa, Homo sapiens
MRKALLAKASCQSRREAPLFCWQKQTS

SEQ ID NO: 3598 - protein, 81 aa, Homo sapiens [sequence omitted]

SEQ ID NO: 3599 - protein, 41 aa, Homo sapiens
MRKKNSCSTKNLRYIHSYLSRWLVQSKHYIIGHGGCHLAAC

SEQ ID NO: 3600 - protein, 53 aa, Homo sapiens [sequence omitted]

SEQ ID NO: 3601 - protein, 38 aa, Homo sapiens
MRKTLVSIPPQTTPENSSFHINTTQFLPIPIICFTKIH

SEQ ID NO: 3602 - protein, 20 aa, Homo sapiens
MRLGASSILEARWTQAIDTC

SEQ ID NO: 3603 - protein, 30 aa, Homo sapiens
MRLGASSILEARWTQAIDTCSMECFTKDLV

SEQ ID NO: 3604 - protein, 25 aa, Homo sapiens
MRLHSLLASHVILRVSSDVRIKASE

SEQ ID NO: 3605 - protein, 52 aa, Homo sapiens
MRLKGRCGHRWTCRQLQAPQTRLVGTPSLPRSSLRPRNTPAPSGPDVRPTFL

SEQ ID NO: 3606 - protein, 66 aa, Homo sapiens
MRLSDASQVSFSIVSWSSGTESTDSSEADDISSSSSWVRSSKSSSSSSSGPFFSPPVSGPTGVPTD

SEQ ID NO: 3607 - protein, 106 aa, Homo sapiens
MRLSWGASHRYSPASPLRAPCTRSTCLAPACSSCTRPWLASRSPSLYQRTGPPGPERCTTSSRSPPGVLRTLVWAASGATTRTGGSATWTVKLRLGAPGAAPDWQV

SEQ ID NO: 3608 - protein, 59 aa, Homo sapiens
MRLWFLRDSSPVAMLVITDSSSWMMSFVKGSVMILSRSGASRPPWMLKEATTSRVMWCR

SEQ ID NO: 3609 - protein, 112 aa, Homo sapiens
MRLWLSFFCLSFAKALVSVSVISLFIGRLLGQEALVSPMLIGEIPCSPLYTSKILPDKCHCALSSSFPIASNLVSGFSVRPASLSRVVCACCTRGPPLGTAGCDHLRVGLMI

SEQ ID NO: 3610 - protein, 58 aa, Homo sapiens
MRLWLSFFCLSFAKALVSVSVISLFIGRLLGQEALVSPMLIGEIPCSPLYTSKILPDN

SEQ ID NO: 3611 - protein, 61 aa, Homo sapiens
MRLWLSFFCLSFAKALVSVSVISLFIGRLLGQEALVSPMLIGEIPCSPLYTSKILPDNLFY

SEQ ID NO: 3612 - protein, 68 aa, Homo sapiens
MRLWLSFFCLSFAKALVSVSVISLFIGRLLGQEALVSPMLIGEIPCSPLYTSKILPDNMYKEEKAAGN

SEQ ID NO: 3613 - protein, 99 aa, Homo sapiens
MRLWLSFFCLSFAKALVSVSVISLFIGRLLGQEALVSPMLIGEIPCSPLYTSKILPDNSFNFEVSITFTIAMVFSFSFIIFFSLNLQTITKRTVWKLLH

SEQ ID NO: 3614 - protein, 141 aa, Homo sapiens
MRLWLSFFCLSFAKALVSVSVISLFIGRLLGQEALVSPMLIGEIPCSPLYTSKILPDNVLCISRGESAPSSLKLDSIPIISSITSSICHCALSSSFPIASNLVSGFSVRPASLSRVVCACCTRGPPLGTAGCDHLRVGLMI

SEQ ID NO: 3615 - protein, 136 aa, Homo sapiens
MRLWLSFFCLSFAKALVSVSVISLFIGRLLGQEALVSPMLIGEIPCSPLYTSKILPDNVLCISRGESAPSSLKLDSIPIISSITSSISNEWILSVLSSLQTAPNYNPSSHNICTMPEGTTKVNDLAVSNEYFGLVG

SEQ ID NO: 3616 - protein, 19 aa, Homo sapiens
MRLYIMLQLISLYPLFTFI

SEQ ID NO: 3617 - protein, 11 aa, Homo sapiens
MRMGGSSLSFL

SEQ ID NO: 3618 - protein, 54 aa, Homo sapiens
MRNCSPSTMFICENIENLLFQLICCYMISMFSSTDKMVTHLFFLSSISSILGTL

SEQ ID NO: 3619 - protein, 26 aa, Homo sapiens
MRNLSSDRHFMANMMVAGKAVGCVAI

SEQ ID NO: 3620 - protein, 31 aa, Homo sapiens
MRNNCCDRDDHSDTHSCLQGHIVTSSCFAYN

SEQ ID NO: 3621 - protein, 12 aa, Homo sapiens
MRNTSNSTYSGG

SEQ ID NO: 3622 - protein, 12 aa, Homo sapiens
MRPDSIMEKRHW

SEQ ID NO: 3623 - protein, 27 aa, Homo sapiens
MRPTRSVVDTPCVRLHSLYLPACFTSS

SEQ ID NO: 3624 - protein, 27 aa, Homo sapiens
MRPVILILKLAKTIQKMRTIDQYLTNT

SEQ ID NO: 3625 - protein, 70 aa, Homo sapiens
MRQCPWVTRNFAGAQGRGLSRLITFTTLFRLRFFIRTNTPISPNLLRVSSLPATVPLLSKAPVLSPTCRG

SEQ ID NO: 3626 - protein, 81 aa, Homo sapiens
MRQDLLSHFTCMVLTGHSSLELPWPQLIAARGIQLHRSCYSLFVLTSHIFWLSQHPVFILWRNKEFFHFCFFDIRRLGCHK

SEQ ID NO: 3627 - protein, 11 aa, Homo sapiens
MRQHTWLILYF

SEQ ID NO: 3628 - protein, 12 aa, Homo sapiens
MRQISCLHVKKY

SEQ ID NO: 3629 - protein, 11 aa, Homo sapiens
MRQSSEFASLT

SEQ ID NO: 3630 - protein, 16 aa, Homo sapiens
MRRCKVPCLVKSHLEQ

SEQ ID NO: 3631 - protein, 26 aa, Homo sapiens
MRRHLRNLCPSVLQISLNQTLSTPHL

SEQ ID NO: 3632 - protein, 29 aa, Homo sapiens
MRRNCSAVGKTGRPRRRHSPSGLQSPLSR

SEQ ID NO: 3633 - protein, 33 aa, Homo sapiens
MRRQSRKYTILQNKCLLLKHRKQKTHRAASVGL

SEQ ID NO: 3634 - protein, 17 aa, Homo sapiens
MRSEIFICFLFTAGFFF

SEQ ID NO: 3635 - protein, 30 aa, Homo sapiens
MRSGFTCAVFFGLFLSPLISLCSTDFSHIC

SEQ ID NO: 3636 - protein, 34 aa, Homo sapiens
MRSGFTCAVFFGLFLSPSLINLISLCSTDFSHIC

SEQ ID NO: 3637 - protein, 12 aa, Homo sapiens
MRSRARRRSPGP

SEQ ID NO: 3638 - protein, 35 aa, Homo sapiens
MRSRVRGSMISTHSNRVFDPGILDSGRSTLWLLHS

SEQ ID NO: 3639 - protein, 21 aa, Homo sapiens
MRSSVAYFCSKRSWRCDWPNF

SEQ ID NO: 3640 - protein, 14 aa, Homo sapiens
MRSTWGEMSSRQPS

SEQ ID NO: 3641 - protein, 26 aa, Homo sapiens
MRSWIRHLLMGTTKAGSTLASISSGL

SEQ ID NO: 3642 - protein, 24 aa, Homo sapiens
MRTAPFIAGECRRSVDISSCMFHL

SEQ ID NO: 3643 - protein, 41 aa, Homo sapiens
MRTHTISRLQGCRRVLATNHPIPAGHRATEAEAVAESLRPP

SEQ ID NO: 3644 - protein, 11 aa, Homo sapiens
MRTIDQYLTNT

SEQ ID NO: 3645 - protein, 20 aa, Homo sapiens
MRTKAGRKRSTLPMMLMSLG

SEQ ID NO: 3646 - protein, 19 aa, Homo sapiens
MRTMSLCCPSTAWLGGCRV

SEQ ID NO: 3647 - protein, 69 aa, Homo sapiens
MRTPAAMCLVPESDKLVMYSGNVSTLGSLSRSSDSSDGELPLLMSSYSSQSRRWTCLFGYQIEQDSSKP

SEQ ID NO: 3648 - protein, 29 aa, Homo sapiens
MRTRLSPTATLATGSGASEAPVSGDRKPA

SEQ ID NO: 3649 - protein, 11 aa, Homo sapiens
MRTTDSSMACW

SEQ ID NO: 3650 - protein, 14 aa, Homo sapiens
MRTTTLKSWRVSAC

SEQ ID NO: 3651 - protein, 17 aa, Homo sapiens
MRVDEGLHPDVWKEGHF

SEQ ID NO: 3652 - protein, 17 aa, Homo sapiens
MRVESPCWERRHKGEVS

SEQ ID NO: 3653 - protein, 36 aa, Homo sapiens
MRVILSQKENKRYQGRKLCLSRKFDVEKGSLYQGFG

SEQ ID NO: 3654 - protein, 123 aa, Homo sapiens
MRVRVREVCSSGYSCISPKRLGDIIAGQRKRRKSEALISLSAMSSRPRSAQRSRHEANTSFSSLGNTQWELTTLHRANSQHIRRLAWCSAKLDAVHLIGSTSQFSSDSYRARMNSPMASLRYF

SEQ ID NO: 3655 - protein, 24 aa, Homo sapiens
MRWHLHSSGLLEATYRKVSIKPSC

SEQ ID NO: 3656 - protein, 13 aa, Homo sapiens
MRWVSLTCSFYLS

SEQ ID NO: 3657 - protein, 128 aa, Homo sapiens
MRYHLTPVRMAIIKKSGNNRCWRGCGEIRTLLHCWWDCELVQPLWKSVWRFLRDLELEIPFDPAIPLLGIYPKDYKSCCYKDTCTLMFIAALFTIAKTWNQPKCPTMIDWIKKRWHIYTMEVRHFSSL

SEQ ID NO: 3658 - protein, 36 aa, Homo sapiens
MRYMCLFSRYIVHLVPCASPFNPCPRFFGWVHGPDY

SEQ ID NO: 3659 - protein, 25 aa, Homo sapiens
MSAGPAGPWPLGDEKLRGLSSHRCR

SEQ ID NO: 3660 - protein, 100 aa, Homo sapiens
MSALMGVNTGDPRQSKKGGRWDTASRKGPVSICLSAGSGFSKCSASSAISGSRPAVMPQPAPRASTPPPRPPPSAPGPSQPPAAGSGDASVATSARTAPS

SEQ ID NO: 3661 - protein, 22 aa, Homo sapiens
MSALNIFPSLQQEEKLVHLIPV

SEQ ID NO: 3662 - protein, 35 aa, Homo sapiens
MSARLVLNSRPCDLLALASQSSGITGMSHYAWPRN

SEQ ID NO: 3663 - protein, 123 aa, Homo sapiens
MSASALRCSPTNPVSGRVLAGCTGVLRGLRGSATAQRRGAGAAHAARGRVSRAARPERQGGGGGGAGSGPAELRGTAGGEPAPRARPRLGREPRLPVRTLLMGRLAAGSAAAPPRLGPSVHRA

SEQ ID NO: 3664 - protein, 25 aa, Homo sapiens
MSASALRCSPTNPVSGRVLAGCTGW

SEQ ID NO: 3665 - protein, 22 aa, Homo sapiens
MSASPPAALPPSPHTHCSRWHV

SEQ ID NO: 3666 - protein, 20 aa, Homo sapiens
MSASSWPQNGMPPSVGVCRA

SEQ ID NO: 3667 - protein, 27 aa, Homo sapiens
MSATDIWNSRLITKALCFIEKDAESRF

SEQ ID NO: 3668 - protein, 14 aa, Homo sapiens
MSATHGGRAGEANP

SEQ ID NO: 3669 - protein, 16 aa, Homo sapiens
MSCAGLHSPEVSAQEG

SEQ ID NO: 3670 - protein, 20 aa, Homo sapiens
MSCHKQLCEARRARGVQSPF

SEQ ID NO: 3671 - protein, 34 aa, Homo sapiens
MSCIHECFLLDNPRKNYHIQISDPKTHFATNSHP

SEQ ID NO: 3672 - protein, 31 aa, Homo sapiens
MSCKCGALVGLLTSLLPSPSCTTAMLTSPGP

SEQ ID NO: 3673 - protein, 24 aa, Homo sapiens
MSCLSCKTNRYLVNSSRRLFGSEE

SEQ ID NO: 3674 - protein, 47 aa, Homo sapiens [sequence omitted]

SEQ ID NO: 3675 - protein, 22 aa, Homo sapiens
MSDAVIMPFNRMKSFVCEAHSS

SEQ ID NO: 3676 - protein, 15 aa, Homo sapiens
MSDLKESTRCSGKLV

SEQ ID NO: 3677 - protein, 12 aa, Homo sapiens
MSDLKNNKHFQF

SEQ ID NO: 3678 - protein, 12 aa, Homo sapiens
MSDMEVQVCYRS

SEQ ID NO: 3679 - protein, 13 aa, Homo sapiens
MSDRLVSKTPDLR

SEQ ID NO: 3680 - protein, 54 aa, Homo sapiens
MSDTLLSCPSSLFSGSKSLLSCPSSSWGIRSVFSSSSPEGCLSGELICCSSGLI

SEQ ID NO: 3681 - protein, 53 aa, Homo sapiens
MSEFPESEAPKAKKGGEGRDSFPYTTPPPQNTRAGSRPDGGGDGGDRSPGPQV

SEQ ID NO: 3682 - protein, 49 aa, Homo sapiens [sequence omitted]

SEQ ID NO: 3683 - protein, 24 aa, Homo sapiens
MSFASKMLGRISTSIMLNRSNYIF

SEQ ID NO: 3684 - protein, 51 aa, Homo sapiens
MSFDGFHLNKGGEKACETFKGITLLQIGTQGSLLQGQQTSYFLGDEVAHIG

SEQ ID NO: 3685 - protein, 16 aa, Homo sapiens
MSFHTNVLCLAKEHHY

SEQ ID NO: 3686 - protein, 19 aa, Homo sapiens
MSFINTSVVQSCACKSQQS

SEQ ID NO: 3687 - protein, 47 aa, Homo sapiens [sequence omitted]

SEQ ID NO: 3688 - protein, 54 aa, Homo sapiens
MSFLVVSKVKNILQDEATHFTGVSLLRRNTCPRSPALRLSLYRNSLLTRCLLIF

SEQ ID NO: 3689 - protein, 63 aa, Homo sapiens
MSFPHCHLQLQIKVCILRNDPLRSSSGQSLLLEPTAATPQDRVCRRLDRGSLGLLCSIQCQRS

SEQ ID NO: 3690 - protein, 12 aa, Homo sapiens
MSFPPSVLCDVT

SEQ ID NO: 3691 - protein, 36 aa, Homo sapiens
MSFVLCTLISFYIFKLFLETVSLSITWAGVQCHDHS

SEQ ID NO: 3692 - protein, 14 aa, Homo sapiens
MSFVLLGLSLFLLF

SEQ ID NO: 3693 - protein, 25 aa, Homo sapiens
MSFWENNLRKLKTDEFIFSLFFFWW

SEQ ID NO: 3694 - protein, 37 aa, Homo sapiens
MSGAGLGIRRVYRALGLDTVSGVCAFRAWWSSQATGH

SEQ ID NO: 3695 - protein, 22 aa, Homo sapiens
MSGAGWLQLCGSEAVLQGAGGE

SEQ ID NO: 3696 - protein, 22 aa, Homo sapiens
MSGGRWNKGTMGGGLGSCRWHH

SEQ ID NO: 3697 - protein, 80 aa, Homo sapiens
MSGKLRRLFSCVLVESANMLRMREKPLPSWLALSWGSRKSVCRSGPSAFKSKLSLWHRKLPNFSLRGLLSLGIPGRGPHW

SEQ ID NO: 3698 - protein, 51 aa, Homo sapiens
MSGLASCGETRTRSSCAETWRRSSSSARVSFSNWASCSFTEAKMLAVDSTC

SEQ ID NO: 3699 - protein, 107 aa, Homo sapiens
MSGLASCGETRTRSSCAETWRRSSSSARVSFSNWASCSFTEAKMLAVDSTSESSMKVRGGAAAGQGKKEGESQRKEKEGERPPHFTLKCGVLKISPLRKKPKASPRC

SEQ ID NO: 3700 - protein, 93 aa, Homo sapiens
MSGLASCGETRTRSSCAETWRRSSSSARVSFSNWASCSFTEAKMLAVDSTSESSMKVRGGAAAGQGKKEGESQRKEKEGERPPHFTLLREGRN

SEQ ID NO: 3701 - protein, 55 aa, Homo sapiens
MSGLASCGETRTRSSCAETWRRSSSSARVSFSNWASCSFTEAKMLAVDSTSNVEF

SEQ ID NO: 3702 - protein, 39 aa, Homo sapiens
MSGLGQGAALQSLPGEHSLLQNWLGPPAHHTELFSHKVP

SEQ ID NO: 3703 - protein, 28 aa, Homo sapiens
MSGPTSRERGRGCGGTQTSPQSAPQFAP

SEQ ID NO: 3704 - protein, 11 aa, Homo sapiens
MSGRKGISNPG

SEQ ID NO: 3705 - protein, 14 aa, Homo sapiens
MSGSEITINIRRPR

SEQ ID NO: 3706 - protein, 109 aa, Homo sapiens
MSGSLQMLNVCAKASHLQLLEGRCRSNSWKHWSLQCRCGPSPQCSWSMLTWSEAVTLGVYLQLNRGGGPCNKASTWAGLLFHGHSFKVWSIRSSLELQPRPDNSQEFSR

SEQ ID NO: 3707 - protein, 76 aa, Homo sapiens
MSGSSPLRQFPQSHTHGIRQCSDLSLAHARPRSQPRPSPRSGDLRASKIPADSLHRMPTPETLCARAGFHPRRPPA

SEQ ID NO: 3708 - protein, 13 aa, Homo sapiens
MSGTVGLVPGADF

SEQ ID NO: 3709 - protein, 17 aa, Homo sapiens
MSHDALFQGPGLGRRPP

SEQ ID NO: 3710 - protein, 35 aa, Homo sapiens
MSHDTGGRTRGIVPCCGTPCGLQPPCAWCRSLTSW

SEQ ID NO: 3711 - protein, 57 aa, Homo sapiens
MSHITRQEFPIVAAGGGLRAERAVAGHAGPQVVLAHDPQRAALEGPQQQHLLPLLQH

SEQ ID NO: 3712 - protein, 56 aa, Homo sapiens
MSHKSLGQGQNASSLFALCLKHNKSHLCSSSQEVPYLCLRPPQPGLHCSYYYQHFG

SEQ ID NO: 3713 - protein, 25 aa, Homo sapiens
MSHLENAQRGSWGGGWAREMGVGSQ

SEQ ID NO: 3714 - protein, 25 aa, Homo sapiens
MSHQAQLIFIFLVETGFCLVGQAGL

SEQ ID NO: 3715 - protein, 17 aa, Homo sapiens
MSHYHWKCVGRVGVIIF

SEQ ID NO: 3716 - protein, 14 aa, Homo sapiens
MSIIVPPKSSQKSL

SEQ ID NO: 3717 - protein, 31 aa, Homo sapiens
MSIKLIHNISFIVIVFTLSCFTSKNNVFPLF

SEQ ID NO: 3718 - protein, 22 aa, Homo sapiens
MSIKLWCFLLIPYLSSPTLFSV

SEQ ID NO: 3719 - protein, 28 aa, Homo sapiens
MSILSIHKCDIFRLEFRKHTCVCTHTHI

SEQ ID NO: 3720 - protein, 12 aa, Homo sapiens
MSISRVIIHFPF

SEQ ID NO: 3721 - protein, 13 aa, Homo sapiens
MSKCVVSDVKATS

SEQ ID NO: 3722 - protein, 31 aa, Homo sapiens
MSKEYFNRRICVAFGETVTIMNRAPSMPTSL

SEQ ID NO: 3723 - protein, 11 aa, Homo sapiens
MSKLFGVLNNF

SEQ ID NO: 3724 - protein, 35 aa, Homo sapiens
MSKLIKFYTLYMCHHLHINYTSVKHRLESFAFLCI

SEQ ID NO: 3725 - protein, 11 aa, Homo sapiens
MSKLQCLCTVE

SEQ ID NO: 3726 - protein, 45 aa, Homo sapiens
MSKQPWVSTWSSVFSSGTDTLSFRRLSSKICRRVPLKLPRACGSL

SEQ ID NO: 3727 - protein, 184 aa, Homo sapiens
MSKRDKMVGMKSMLSSPFVSSQRPNTELAAARTEQREFRVVVIPALAIEMVCCSMASWIATRSSSRILSNSSIQTTPPSARTMAPPSMMKFRDEGSLITEAVSPAALLPFPDVYTPMGEHFSTNFRSWDLAVPGSPSISRLMSPRRVSPSGSLFREPPKSRQAMAFFMSVPPKMEGAMLLEMTS

SEQ ID NO: 3728 - protein, 84 aa, Homo sapiens
MSKSLLLSHSIPRNAHVLWPSCVGDPSSSSITSFPSASCSPAGRPAKLLSGDSAGSPSPSSEGALLAGWGEERASPSSSVPGAM

SEQ ID NO: 3729 - protein, 23 aa, Homo sapiens
MSKTFRCFTESNFMSQYEATLVL

SEQ ID NO: 3730 - protein, 81 aa, Homo sapiens
MSKTPKAMATKAKIDKWDLIKLKSFCTAKETTISVNRQPTEWEKIFAIYSSDKGLISRIYKELKQIYKKKKTTPSTSVQRI

SEQ ID NO: 3731 - protein, 113 aa, Homo sapiens
MSKVKVELAVDTATGPRFCSCWDAWVGFTGRLAVLQAEPVCLGAPRCLPPGHSGATWMDARLSTVRCVQSGICTKNGPSMRESPPWEGLPCLPFWALLDFLQEVLSLSHSVLS

SEQ ID NO: 3732 - protein, 100 aa, Homo sapiens
MSLARMARASSLTTASSIKKQFTIYDRKLGRKSCSNCFMANMTSEKLKIKRFSNLLSNIFSMVSLMRVSGKETFSPRIKAEITSKRVSQQDVERLATCSV

SEQ ID NO: 3733 - protein, 16 aa, Homo sapiens
MSLCCPSTAWLGGCRV

SEQ ID NO: 3734 - protein, 38 aa, Homo sapiens
MSLCHLPSVFHPAMLIRVILSVPKYEAWIVEELTALIS

SEQ ID NO: 3735 - protein, 39 aa, Homo sapiens
MSLCHLPSVFHPAMLIRVILSVPKYEAWIVEELTALISS

SEQ ID NO: 3736 - protein, 42 aa, Homo sapiens
MSLCHLPSVFHPAMLIRVILSVPKYEAWIVEELTALISWFHP

SEQ ID NO: 3737 - protein, 57 aa, Homo sapiens
MSLEYLSLLKVLQPSHMCRHHTLLGPGASELWTQPACAEQQQGLAEQGPQQASWEAP

SEQ ID NO: 3738 - protein, 11 aa, Homo sapiens
MSLFFLYLFVA

SEQ ID NO: 3739 - protein, 14 aa, Homo sapiens
MSLFSLYSWRIFFT

SEQ ID NO: 3740 - protein, 11 aa, Homo sapiens
MSLHKNVPASW

SEQ ID NO: 3741 - protein, 14 aa, Homo sapiens
MSLHMNFHLINLVY

SEQ ID NO: 3742 - protein, 21 aa, Homo sapiens
MSLILCSSNLGFSSRTTSLNN

SEQ ID NO: 3743 - protein, 11 aa, Homo sapiens
MSLKSSQYLAH

SEQ ID NO: 3744 - protein, 14 aa, Homo sapiens
MSLLCLHCLWLHRH

SEQ ID NO: 3745 - protein, 33 aa, Homo sapiens
MSLLLSLPLVDLWVSIELEANFCDPPSLYHSGS

SEQ ID NO: 3746 - protein, 55 aa, Homo sapiens
MSLLLSLPLVDPCSTCTNTRMHRAQELRVCWCRLHPWQREHGDPGIRTPGFSSHL

SEQ ID NO: 3747 - protein, 27 aa, Homo sapiens
MSLQLIVHLYLLFLLMVWLPLILQPMF

SEQ ID NO: 3748 - protein, 15 aa, Homo sapiens
MSLSFKTTKKYIIQL

SEQ ID NO: 3749 - protein, 44 aa, Homo sapiens
MSLSSSKVMMTKASVEPLNCSSWWPAIQCCSCLVRDATWREGFL

SEQ ID NO: 3750 - protein, 12 aa, Homo sapiens
MSLWLMVGLQTF

SEQ ID NO: 3751 - protein, 30 aa, Homo sapiens
MSMKLVFHHFHIIRNLSLCLQCVLSRKKPR

SEQ ID NO: 3752 - protein, 28 aa, Homo sapiens
MSMKPPFRGRICTVQRIFKLNDISILLF

SEQ ID NO: 3753 - protein, 102 aa, Homo sapiens [sequence omitted]

SEQ ID NO: 3754 - protein, 14 aa, Homo sapiens
MSNAMIFSNNWFRA

SEQ ID NO: 3755 - protein, 12 aa, Homo sapiens
MSNISNEILNYS

SEQ ID NO: 3756 - protein, 39 aa, Homo sapiens
MSNSPFLITLWTGGSWKSSGKTSMLGNTNIGLWYLSPVW

SEQ ID NO: 3757 - protein, 64 aa, Homo sapiens [sequence omitted]

SEQ ID NO: 3758 - protein, 13 aa, Homo sapiens
MSPGTHCSRSRRC

SEQ ID NO: 3759 - protein, 47 aa, Homo sapiens
MSPPAHCVPLLICSGKIAALPSLFPPSSLVFPVTITLTSPVLPPQSS

SEQ ID NO: 3760 - protein, 27 aa, Homo sapiens
MSPRLISNSCPQAILPPWPPKVLRLQV

SEQ ID NO: 3761 - protein, 18 aa, Homo sapiens
MSPRTRPGVLSCTISHSS

SEQ ID NO: 3762 - protein, 27 aa, Homo sapiens
MSPSDAQRNFWCRGAGGTRPARGSLPR

SEQ ID NO: 3763 - protein, 55 aa, Homo sapiens
MSPSFSKVFLPKQLLYYHQSLPYFKALSSACLLSDSLYVVYICCFYLLSNHFHSS

SEQ ID NO: 3764 - protein, 17 aa, Homo sapiens
MSPSKNKYIFILVLLFL

SEQ ID NO: 3765 - protein, 15 aa, Homo sapiens
MSQAWWLMPPSTLGG

SEQ ID NO: 3766 - protein, 62 aa, Homo sapiens
MSQHLQGVGSSGSIWAPWSLISMFCNASGISTLLCSVFSVLHSARHSLCLVFGSGSSEAGGN

SEQ ID NO: 3767 - protein, 33 aa, Homo sapiens
MSQHVDLIFQRLSFICQSGQFIILLPKFRDLLF

SEQ ID NO: 3768 - protein, 64 aa, Homo sapiens
MSQIISEPQHHFVNNRAKSSDCTADWFLLLEQGLNHAWNPSCYRGGGREGLLTCSHCEGVRKPR

SEQ ID NO: 3769 - protein, 24 aa, Homo sapiens
MSQQMDPCQYYFQPQFGKSRLFLE

SEQ ID NO: 3770 - protein, 11 aa, Homo sapiens
MSQQRSNGPTT

SEQ ID NO: 3771 - protein, 11 aa, Homo sapiens
MSQTWWHQQTQ

SEQ ID NO: 3772 - protein, 11 aa, Homo sapiens
MSRCSIAGVIG

SEQ ID NO: 3773 - protein, 30 aa, Homo sapiens
MSRDLYSFSAELCFKLSARHAVRPGRTKPY

SEQ ID NO: 3774 - protein, 53 aa, Homo sapiens
MSRDLYSFSAELCFKLSARHAVRPGRTKPYGMSMQLGDNGTLFPSWDCKPFIH

SEQ ID NO: 3775 - protein, 12 aa, Homo sapiens
MSRGLLTWLQMM

SEQ ID NO: 3776 - protein, 43 aa, Homo sapiens
MSRHLIYSFGKLKGSVSGNYLDDFSRKTRLCRCLFCLHRRFPA

SEQ ID NO: 3777 - protein, 78 aa, Homo sapiens [sequence omitted]

SEQ ID NO: 3778 - protein, 36 aa, Homo sapiens
MSRLPVMDMNSSMLSLARRSLSRLSCTASSSRGASS

SEQ ID NO: 3779 - protein, 16 aa, Homo sapiens
MSRMMSDLKNNKHFQF

SEQ ID NO: 3780 - protein, 20 aa, Homo sapiens
MSRPPSLCSFSFALSCNNPK

SEQ ID NO: 3781 - protein, 30 aa, Homo sapiens
MSRSGSPLHLHAAEKRPSNNVCTQTQSSEP

SEQ ID NO: 3782 - protein, 20 aa, Homo sapiens
MSSDVRSFMILTYCLCWVLW

SEQ ID NO: 3783 - protein, 20 aa, Homo sapiens
MSSFFNIVENLLLSPTTEPK

SEQ ID NO: 3784 - protein, 11 aa, Homo sapiens
MSSFFTSGSFR

SEQ ID NO: 3785 - protein, 121 aa, Homo sapiens
MSSGARLLVAAEGLRSGRNGRRRTQRPLERAGSERQPHTRLAAVAPGHDALKLTCSRTGLRATSKGTEDGPCPMCAACKPENFPGNYLLQLQRQREERRISSRKTRGQKSSSSSPVEPETT

SEQ ID NO: 3786 - protein, 11 aa, Homo sapiens
MSSGLRHFSCW

SEQ ID NO: 3787 - protein, 15 aa, Homo sapiens
MSSGPCRSRSSPSSS

SEQ ID NO: 3788 - protein, 17 aa, Homo sapiens
MSSGPWSSGLSVNLHGR

SEQ ID NO: 3789 - protein, 12 aa, Homo sapiens
MSSIEFVVGFSS

SEQ ID NO: 3790 - protein, 70 aa, Homo sapiens
MSSILKSCGAIELGSVNCLWKHISDVGDKFFQVLTGFLQMCCIDNNLNKLSKPNILPFNYILQRVAQSPG

SEQ ID NO: 3791 - protein, 25 aa, Homo sapiens
MSSILSKPNILPFNYILQRVAQSPG

SEQ ID NO: 3792 - protein, 15 aa, Homo sapiens
MSSKSFFVFSNFLNI

SEQ ID NO: 3793 - protein, 70 aa, Homo sapiens
MSSPSSLMEACKVLPRICSPLEWRESLKMRNTRTRRMTRRMARDMACCPFWPPPPPPGCCSASSVPRVMK

SEQ ID NO: 3794 - protein, 12 aa, Homo sapiens
MSSRGWVSKIHF

SEQ ID NO: 3795 - protein, 16 aa, Homo sapiens
MSSSFLCKEMITWQSI

SEQ ID NO: 3796 - protein, 24 aa, Homo sapiens
MSSSSVLNHISSSSSSVLASLRYL

SEQ ID NO: 3797 - protein, 16 aa, Homo sapiens
MSSVTISLRTQKAEPL

SEQ ID NO: 3798 - protein, 13 aa, Homo sapiens
MSTGHSNNFGFFH

SEQ ID NO: 3799 - protein, 16 aa, Homo sapiens
MSTIELLLSAEDILLL

SEQ ID NO: 3800 - protein, 107 aa, Homo sapiens
MSTKAKIDKWDLIKLRSFCAAKETIIRVNRQPTEWEKIFATYPSDKGLISRIYKELKQIYKKKNNSIKKWVKDMNRHFLKEDIYAANKRKKKSHHHWSLEKCKSKRQ

SEQ ID NO: 3801 - protein, 29 aa, Homo sapiens
MSTLFLANSFSKLHLSCTISFSVLLTLQR

SEQ ID NO: 3802 - protein, 28 aa, Homo sapiens
MSTLFLANSFSKLHLSCTISFSVLLTSL

SEQ ID NO: 3803 - protein, 21 aa, Homo sapiens
MSTMQFFTRVLVRTSSLLDAL

SEQ ID NO: 3804 - protein, 12 aa, Homo sapiens
MSTNSSVAKFYL

SEQ ID NO: 3805 - protein, 76 aa, Homo sapiens
MSTRCCPTWYVHSWADSGQIADCPHSPPILAPGLSWTPGTLKLVHSQLGQEAPFTYTQRRSAQATTSAPKPSPQNR

SEQ ID NO: 3806 - protein, 60 aa, Homo sapiens
MSTRCCPTWYVHSWADSGQIADCPHSPPILAPGLSWTPGTLKLVHSQPYPGSLGAEASES

SEQ ID NO: 3807 - protein, 12 aa, Homo sapiens
MSTRWTMMQFFK

SEQ ID NO: 3808 - protein, 27 aa, Homo sapiens
MSTTHLSRTRPEGNQADMGDVPSSRPS

SEQ ID NO: 3809 - protein, 103 aa, Homo sapiens [sequence omitted]

SEQ ID NO: 3810 - protein, 27 aa, Homo sapiens
MSTWEGIFIYLFILFYFIYFLRQSLAL

SEQ ID NO: 3811 - protein, 14 aa, Homo sapiens
MSVAIKHPHRSVME

SEQ ID NO: 3812 - protein, 50 aa, Homo sapiens
MSVIPALWEAEAGGSPEVGSSRPAWPTWRNPVSTKNKKKKTLAGFGGTRL

SEQ ID NO: 3813 - protein, 18 aa, Homo sapiens
MSVLFFIFKSKVKIYSFS

SEQ ID NO: 3814 - protein, 16 aa, Homo sapiens
MSVPLGIRFPRMAYIT

SEQ ID NO: 3815 - protein, 65 aa, Homo sapiens
MSVPTPPSSGAKCIIDLRVKSLSDLEATRHCYVCGRLGSRDPGPRDVPSIPEPTPTQATTLWDSS

SEQ ID NO: 3816 - protein, 51 aa, Homo sapiens
MSVSLTVRSTRDCLFFSNSFVPSTSPPMISFSPSCFLAVSVSFDSVWSCFR

SEQ ID NO: 3817 - protein, 24 aa, Homo sapiens
MSVSRSSSTVHGLLTEGDRLAELL

SEQ ID NO: 3818 - protein, 64 aa, Homo sapiens
MSVSSIWVQVCETKGRNPPDTASLRQVELLQFLSSYVNSVMAMRSFCLNAFSNKSRASWPNCFE

SEQ ID NO: 3819 - protein, 14 aa, Homo sapiens
MSVTTGIKVTELCS

SEQ ID NO: 3820 - protein, 25 aa, Homo sapiens
MSVVHRSDQRVNEPSTYAGPDITDR

SEQ ID NO: 3821 - protein, 25 aa, Homo sapiens
MSVVHRSDQRVNEPSVCADPDITDR

SEQ ID NO: 3822 - protein, 12 aa, Homo sapiens
MSWFYRATIEVF

SEQ ID NO: 3823 - protein, 53 aa, Homo sapiens
MSWGVAPRAPRTPGGAISDTYTGMQAAVSPPAKPVSVLPSSSIQRPCAPAMSA

SEQ ID NO: 3824 - protein, 58 aa, Homo sapiens
MSWMGPSSGSRQLWPRPSPPLSSPGLRSQPPNWTPCPQPLPDPAPPHGSQSARSKTQT

SEQ ID NO: 3825 - protein, 77 aa, Homo sapiens
MSWMGPSSGSRQLWPRPSPPLSSPGLRSQPPNWTPCPQPLPDPAPPHGSQSARSWPGLPQWRPLSLTGSGSHFSVAY

SEQ ID NO: 3826 - protein, 61 aa, Homo sapiens
MSWMGPSSGSRQLWPRPSPPLSSPGLRSQPPNWTPCPQPLPDPAPPHGSQSARYSPHNAAT

SEQ ID NO: 3827 - protein, 46 aa, Homo sapiens
MSWPLTGNGGMDHCCISFRRQCSPWYFSSSHTRVVASGSLESIMKS

SEQ ID NO: 3828 - protein, 14 aa, Homo sapiens
MSWTRDTCLIIACL

SEQ ID NO: 3829 - protein, 17 aa, Homo sapiens
MSYHAQPSLGLSNQEAL

SEQ ID NO: 3830 - protein, 17 aa, Homo sapiens
MTAIISLLNLSFHMLFL

SEQ ID NO: 3831 - protein, 36 aa, Homo sapiens
MTALPLRCGRDFLPPQHLQPGRERARPQSQGTGSQR

SEQ ID NO: 3832 - protein, 64 aa, Homo sapiens
MTALRLLWAVASGFLPRRTLSPSFWSRGGRADRAGRDKPGRLPLPPQTHQGRLPASPWEDWSVG

SEQ ID NO: 3833 - protein, 84 aa, Homo sapiens
MTAPSTQAQGAPLCQRLAAAPSRSFCGHLLAVRSHVPGEVVALPEVLLAHRAGKGLFSPLLRMWVRPRMLLFVVGSHVKDQVGR

SEQ ID NO: 3834 - protein, 46 aa, Homo sapiens
MTARFLTLVSVIPKMPFLILSILAFNSSNTGSVMILSLRVKIRIWA

SEQ ID NO: 3835 - protein, 59 aa, Homo sapiens
MTAWKVLPVSSLTWTFICGLRFSGIMIVYRSCPVSPRASAFSPGRYSSGITPIPTRLLR

SEQ ID NO: 3836 - protein, 22 aa, Homo sapiens
MTCATLENKYYHINISLLLQKH

SEQ ID NO: 3837 - protein, 11 aa, Homo sapiens
MTCFPQFPLRS

SEQ ID NO: 3838 - protein, 25 aa, Homo sapiens
MTCKHIKDKIIYQLHDNTIELQNKN

SEQ ID NO: 3839 - protein, 205 aa, Homo sapiens
MTCLASITSLSSLCSSLTMKIMSKRDKMVGMKSMLSSPFVSSQRPNTELAAARTEQREFRVVVIPALAIEMVCCSMASWIATRSSSRILSNSSIQTTPPSARTMAPPSMMKFRDEGSLITEAVSPAALLPFPDVYTPMGEHFSTNFRSWDLAVPGSPSISRLMSPRRVSPSGSLFREPPKSRQAMAFFMSVPPKMEGAMLLEMTS

SEQ ID NO: 3840 - protein, 28 aa, Homo sapiens
MTCQRFGVHFKNFSLSCWGITHPKILSV

SEQ ID NO: 3841 - protein, 18 aa, Homo sapiens
MTDGGIRPAGLRGACEPG

SEQ ID NO: 3842 - protein, 37 aa, Homo sapiens
MTDMPLLLAKMLFQTDLGRKVLILPLAISIQGNFFPS

SEQ ID NO: 3843 - protein, 19 aa, Homo sapiens
MTDSQPISYRMGKSWKHSP

SEQ ID NO: 3844 - protein, 33 aa, Homo sapiens
MTEDTENRKRGTFTCCTEVFKTQKLVVRVRLYR

SEQ ID NO: 3845 - protein, 114 aa, Homo sapiens
MTETPKAMSTKAKIDKWDLIKLRSFCAAKETIIRVNRQPTEWEKIFATYPSDKGLISRIYKELKQIYKKKNNSIKKWVKDMNRHFLKEDIYAANKRKKKSHHHWSLEKCKSKRQ

SEQ ID NO: 3846 - protein, 22 aa, Homo sapiens
MTEYTSYDRLYDIQDTAFWEAV

SEQ ID NO: 3847 - protein, 18 aa, Homo sapiens
MTFAASSEKASLVHRHHV

SEQ ID NO: 3848 - protein, 26 aa, Homo sapiens
MTFKSLKISDTFKCLVLPTFPFVLLS

SEQ ID NO: 3849 - protein, 109 aa, Homo sapiens
MTFPEKQGCADVFFASIEDSQHRTGATESFCSSRHCPWKQREPPRPGCCWFYSGRPAEAQGCPNCSLSCISGCAGLWESLPCLPGGFRAMTTPHGSDPGRASSKTADVY

SEQ ID NO: 3850 - protein, 14 aa, Homo sapiens
MTFPTALSSRSLTQ

SEQ ID NO: 3851 - protein, 30 aa, Homo sapiens
MTFRIVSSWAVAQTRVVQHYFTQEESKPRA

SEQ ID NO: 3852 - protein, 30 aa, Homo sapiens
MTGAACTGGQRETEQDREFHNVLLYNVWNL

SEQ ID NO: 3853 - protein, 100 aa, Homo sapiens
MTGAQKNCGPRTFELCLKVTAVLSAGPASNRPSGGFTMKVMKFKHQDPSLVLVLGAAPEILHFCFCILKAAKSRKPQTPQNICSYTVWTWASQPDGHNFT

SEQ ID NO: 3854 - protein, 23 aa, Homo sapiens
MTGFPSLPGASWRPEHSSHSLLS

SEQ ID NO: 3855 - protein, 30 aa, Homo sapiens
MTGFPSLPGASWRPEHSSHSLLSKLGGFYP

SEQ ID NO: 3856 - protein, 38 aa, Homo sapiens
MTGFPSLPGASWRPEHSSHSLLSKLGGFYPRGQTNSGV

SEQ ID NO: 3857 - protein, 26 aa, Homo sapiens
MTGGFCCPQKRPIIGEKPKGPSRTSI

SEQ ID NO: 3858 - protein, 18 aa, Homo sapiens
MTGLSERSPMVSWSVLYL

SEQ ID NO: 3859 - protein, 17 aa, Homo sapiens
MTGLSLTNTLSTLRLSG

SEQ ID NO: 3860 - protein, 21 aa, Homo sapiens
MTGPRRLWHCHSVGQGMLRLN

SEQ ID NO: 3861 - protein, 47 aa, Homo sapiens
MTGVLSLTSRMMTRTVALLCSEGRPPSLASTLNSNALVCSWLKDRSA

SEQ ID NO: 3862 - protein, 71 aa, Homo sapiens
MTHFRYPQIHMFTIFFGVSFFSYCVLKISPFQMQKFSPSDVMTDEDIFVLSQIEQIQPSSNFLCAPFLNRL

SEQ ID NO: 3863 - protein, 55 aa, Homo sapiens
MTHFRYPQILKISPFQMQKFSPSDVMTDEDIFVLSQIEQIQPSSNFLCAPFLNRL

SEQ ID NO: 3864 - protein, 56 aa, Homo sapiens
MTHFRYPQILKISPFQMQKFSPSDVMTDEDIFVLSQIEQIQPSSNFLCAPFLNYQS

SEQ ID NO: 3865 - protein, 23 aa, Homo sapiens
MTHFRYPQIQAVNLSSASEPFPF

SEQ ID NO: 3866 - protein, 67 aa, Homo sapiens
MTHIYLSSQEDIFQFYKTEARNAENQRFLRSLLSNDIMCSLEHSGHSLDGWLLPLHSRISYWKLTMW

SEQ ID NO: 3867 - protein, 41 aa, Homo sapiens
MTHNPGKEVNPTLSRLFFFFFAKIRTCKIGQLQVTSGRSCF

SEQ ID NO: 3868 - protein, 14 aa, Homo sapiens
MTHQTSVDFFQFFS

SEQ ID NO: 3869 - protein, 19 aa, Homo sapiens
MTIKPCPWDRTMAQHMLTE

SEQ ID NO: 3870 - protein, 25 aa, Homo sapiens
MTITCPSAVPNSTCWSSGVHMPHVI

SEQ ID NO: 3871 - protein, 35 aa, Homo sapiens
MTKASVEPLNCSSWWPAIQCCSCLVRDATWREGFL

SEQ ID NO: 3872 - protein, 18 aa, Homo sapiens
MTKCKLSSSCSQNWLGLP

SEQ ID NO: 3873 - protein, 61 aa, Homo sapiens
MTKGSRTEELRPARITKLPLYHPRHTHTKKDQIPVTESFANSSQWLYMPINLTLHRKCKMA

SEQ ID NO: 3874 - protein, 55 aa, Homo sapiens [sequence omitted]

SEQ ID NO: 3875 - protein, 20 aa, Homo sapiens
MTKTIAGGIQRDTFHYSIPN

SEQ ID NO: 3876 - protein, 42 aa, Homo sapiens
MTKTPKAMATKAKIDKRDLIKLKSFCTAKETTIRAGHSGSCL

SEQ ID NO: 3877 - protein, 127 aa, Homo sapiens
MTLAMRVRVREVCSSGYSCISPKRLGDIIAGQRKRRKSEALISLSAMSSRPRSAQRSRHEANTSFSSLGNTQWELTTLHRANSQHIRRLAWCSAKLDAVHLIGSTSQFSSDSYRARMNSPMASLRYF

SEQ ID NO: 3878 - protein, 24 aa, Homo sapiens
MTLFFALCSPIWVPVLCWVSLFIC

SEQ ID NO: 3879 - protein, 15 aa, Homo sapiens
MTLKRVKMSFHSSVK

SEQ ID NO: 3880 - protein, 35 aa, Homo sapiens
MTLNHKHIPLNTNKSPNHKMPETTLLPADTKKKSR

SEQ ID NO: 3881 - protein, 52 aa, Homo sapiens
MTLRCSSTAPRSSSLWSHVSSISSSAFISSGSLANSPDSATGCSSGTATGLL

SEQ ID NO: 3882 - protein, 44 aa, Homo sapiens
MTLYIFLCFLASSISSRFNSPTTLFVNGSGMQLGLCELTVKSSL

SEQ ID NO: 3883 - protein, 66 aa, Homo sapiens
MTLYVPNMVAPTNSVNSCCALTLVTYKLMSPNIDQNRDCSVSNNVENALFCFSHLMPLQVNPFVSS

SEQ ID NO: 3884 - protein, 43 aa, Homo sapiens
MTMEALHRTGVQSRSKRLYNSGISANRMNRHTPSCIISTRTNI

SEQ ID NO: 3885 - protein, 36 aa, Homo sapiens
MTMLVPHWILRGLNEKIHAKQSLAWHVLRGSHYCYF

SEQ ID NO: 3886 - protein, 28 aa, Homo sapiens
MTNEILQQNAAGPAFSLHMYGPYWTQQP

SEQ ID NO: 3887 - protein, 19 aa, Homo sapiens
MTNHQPISYCMGKTWKHSL

SEQ ID NO: 3888 - protein, 34 aa, Homo sapiens
MTNRRNSQEGEASGGREGKAGQGLLLPHKPFSTS

SEQ ID NO: 3889 - protein, 15 aa, Homo sapiens
MTPGPGPCFSCLSVP

SEQ ID NO: 3890 - protein, 20 aa, Homo sapiens
MTPINRFKVKKDPKMMKITK

SEQ ID NO: 3891 - protein, 52 aa, Homo sapiens
MTPIPESQRRKQGPESRSNLPKVTQQDLAAIASKSRPLNIPSWACGTLGSRP

SEQ ID NO: 3892 - protein, 78 aa, Homo sapiens
MTPMKRKKMSSPSSLMEACKVLPRICSPLEWRESLKMRNTRTRRMTRRMARDMACCPFWPPPPPPGCCSASSVPRVMK

SEQ ID NO: 3893 - protein, 153 aa, Homo sapiens
MTPPPHPSGTSISASSVCPPGHSQWHTSPGLLQRGRVGGRKQQQPVPGQGQRSGCLLFPEVLSEKYLAGLRTREGAEGYIWIAQLLAPHPCKSEGLSGPLISLFSTKPALRGEWTEQRPGRPWPETASLWRQAIWVGPSAALGLSLPLCWGLR

SEQ ID NO: 3894 - protein, 165 aa, Homo sapiens
MTPPPHPSGTSISASSVCPPGHSQWHTSPGLLQRGRVGGRKQQQPVPGQGQRSGCLLFPEVLSEKYLAGLRTREGAEGYIWIAQLLAPHPCKSEGLSGPLISLFSTKPALRGEWTEQRPGRPWPETASLWRQAIWVGPSAALGLSLPLSLPPAGDSDDHRLGGSG

SEQ ID NO: 3895 - protein, 16 aa, Homo sapiens
MTPPYLTPIILNSNDN

SEQ ID NO: 3896 - protein, 12 aa, Homo sapiens
MTPSSQHCSKGL

SEQ ID NO: 3897 - protein, 13 aa, Homo sapiens
MTPVSGCMEKCFG

SEQ ID NO: 3898 - protein, 17 aa, Homo sapiens
MTQARLSVPGWLGCQRE

SEQ ID NO: 3899 - protein, 29 aa, Homo sapiens
MTQGAGRGASSLAVALHADSSRHVLGAGV

SEQ ID NO: 3900 - protein, 12 aa, Homo sapiens
MTQLYLIHQLMV

SEQ ID NO: 3901 - protein, 14 aa, Homo sapiens
MTQNTLKQCSVTIH

SEQ ID NO: 3902 - protein, 53 aa, Homo sapiens
MTQSFAWLRELPELLAPRPSAGVHRCKFCCLHSKSVMQDCLLCGINSGLEESL

SEQ ID NO: 3903 - protein, 39 aa, Homo sapiens
MTRHGIQGASLCFYSFFSFFSFSAEHIPSITSWVHWETD

SEQ ID NO: 3904 - protein, 124 aa, Homo sapiens [sequence omitted]

SEQ ID NO: 3905 - protein, 41 aa, Homo sapiens
MTRHGIQGASPEWESVPWFPCISLCRNVFLPTLPFSTLQTR

SEQ ID NO: 3906 - protein, 36 aa, Homo sapiens
MTRRIANSTTRCFSFMLTSFPSPLTHSCSCIKESWW

SEQ ID NO: 3907 - protein, 51 aa, Homo sapiens
MTRSQKDFRLCWASLRLVPPNPPSVDISTNASSGSPGRAGAALALLRSRAL

SEQ ID NO: 3908 - protein, 36 aa, Homo sapiens
MTRTVALLCSEGRPPSLASTLNSNALVCSWLKDRSA

SEQ ID NO: 3909 - protein, 19 aa, Homo sapiens
MTSAGNQPQKQSFHIFLPA

SEQ ID NO: 3910 - protein, 37 aa, Homo sapiens
MTSGDPPASASQSAGIPGVSPHSQPRMYNYMCGYLLL

SEQ ID NO: 3911 - protein, 116 aa, Homo sapiens
MTSGSCLLSSLSPSSLTRVVPSGCSCCPRAPGLGRSSSGLILDLLLCIGSPVLLTADSLVGLFCEDSEGPELTWTGFRTVGIPGIGLCVGKVGAGWMSGGLCPKAEPKLCCRLRIC

SEQ ID NO: 3912 - protein, 65 aa, Homo sapiens
MTSHSPLSNFISLRHCFICLYSGRATSKRRVDSCICNISSSKASSSSFALSSAVYGFSALNPRGA

SEQ ID NO: 3913 - protein, 64 aa, Homo sapiens
MTSKIPRSTKEPLFAAYICVPLIITAWAGRLTPQANVAVHTRTLICPLENKFSTKFLSCRSIPA

SEQ ID NO: 3914 - protein, 11 aa, Homo sapiens
MTSPFFSFNCP

SEQ ID NO: 3915 - protein, 91 aa, Homo sapiens
MTSPPSWWSHRSHTPPSQPAASSLKVFRSLWPRCFHPILLLPFQLFLHLSEWGGLTCKLEHTFATSRVPRKGGVETKATMVLHVHKRLAGV

SEQ ID NO: 3916 - protein, 40 aa, Homo sapiens
MTSQRFCKYFNYEKKVSSLKESKILKACWDGVTYLLGLGS

SEQ ID NO: 3917 - protein, 24 aa, Homo sapiens
MTSRMRLGASSILEARWTQAIDTC

SEQ ID NO: 3918 - protein, 34 aa, Homo sapiens
MTSRMRLGASSILEARWTQAIDTCSMECFTKDLV

SEQ ID NO: 3919 - protein, 13 aa, Homo sapiens
MTSSSSFSLDEDF

SEQ ID NO: 3920 - protein, 82 aa, Homo sapiens
MTSVFEGPVRSCSLSSRIWGRTGRKPVRSPIILAFFSVGSSLQQPSQMVLWSWILFSSLQFPNWKMPPRVTVWVPGMMYGEL

SEQ ID NO: 3921 - protein, 24 aa, Homo sapiens
MTTGSFSVFWVEICMSGRPDGHKR

SEQ ID NO: 3922 - protein, 17 aa, Homo sapiens
MTTKRGVFMRFLKHLDF

SEQ ID NO: 3923 - protein, 15 aa, Homo sapiens
MTTLYGSFITVSISS

SEQ ID NO: 3924 - protein, 61 aa, Homo sapiens
MTVGWEAGRPLRWTCLCRGRCDFTTSGRARGRVCRSSMELICWDTVSSCRNRSSYCSSGWA

SEQ ID NO: 3925 - protein, 35 aa, Homo sapiens
MTVSCLALTGLCPSVLVMIFTPPSAPFIVTLIHLF

SEQ ID NO: 3926 - protein, 25 aa, Homo sapiens
MVAEQKINLVRSKRRNSSPKNWRNA

SEQ ID NO: 3927 - protein, 27 aa, Homo sapiens
MVAETKGACCVHSSAPPRRLPRGLPQT

SEQ ID NO: 3928 - protein, 12 aa, Homo sapiens
MVAGKAVGCVAI

SEQ ID NO: 3929 - protein, 27 aa, Homo sapiens
MVAHASQHFGRLRQADHFRSGVRDQPG

SEQ ID NO: 3930 - protein, 59 aa, Homo sapiens
MVAPTNSVNSCCALTLVTYKLMSPNIDQNRDCSVSNNVENALFCFSHLMPLQVNPFVSS

SEQ ID NO: 3931 - protein, 16 aa, Homo sapiens
MVAQTPALWEAEAGGS

SEQ ID NO: 3932 - protein, 43 aa, Homo sapiens
MVAVPCSAWVTARAPSGRMLPGQEAASRTLALPLLDGAGEGRG

SEQ ID NO: 3933 - protein, 26 aa, Homo sapiens
MVAVPGPLALVLVSPLVSQRAARAVA

SEQ ID NO: 3934 - protein, 13 aa, Homo sapiens
MVAVPLRVFKCWS

SEQ ID NO: 3935 - protein, 40 aa, Homo sapiens
MVAVPSRRDAPDGVQSLQGTRGPYNGQAAARACSGRWSSA

SEQ ID NO: 3936 - protein, 42 aa, Homo sapiens
MVCIHYLPFKIQLLHSSVNFSHNVIRFALTSDSKMPLGFFHS

SEQ ID NO: 3937 - protein, 13 aa, Homo sapiens
MVCPPVKTNTFLS

SEQ ID NO: 3938 - protein, 64 aa, Homo sapiens
MVCQLFLGLGQFALSGFFGHHRMGREVGMGREVGMGREVGLGPHQHDPGEDKYIPPVTSTSLCD

SEQ ID NO: 3939 - protein, 70 aa, Homo sapiens
MVCQLFLGLGQFALSGFFGHHRMGREVGMGREVGMGREVGMGREVGLGPHQHDPGEDKYIPPVTSTSLCD

SEQ ID NO: 3940 - protein, 75 aa, Homo sapiens
MVCQLFLGLGQFALSGFFGHHRMGREVGMGREVGMGREVGMGREVGMGREVGLGPHQHDPGEDKYIPPVTSTSLC

SEQ ID NO: 3941 - protein, 76 aa, Homo sapiens
MVCQLFLGLGQFALSGFFGHHRMGREVGMGREVGMGREVGMGREVGMGREVGLGPHQHDPGEDKYIPPVTSTSLCD

SEQ ID NO: 3942 - protein, 82 aa, Homo sapiens
MVCQLFLGLGQFALSGFFGHHRMGREVGMGREVGMGREVGMGREVGMGREVGMGREVGLGPHQHDPGEDKYIPPVTSTSLCD

SEQ ID NO: 3943 - protein, 88 aa, Homo sapiens
MVCQLFLGLGQFALSGFFGHHRMGREVGMGREVGMGREVGMGREVGMGREVGMGREVGMGREVGLGPHQHDPGEDKYIPPVTSTSLCD

SEQ ID NO: 3944 - protein, 12 aa, Homo sapiens
MVCVSARISHFK

SEQ ID NO: 3945 - protein, 21 aa, Homo sapiens
MVDSIMLPHLKRCPRFYSLKL

SEQ ID NO: 3946 - protein, 23 aa, Homo sapiens
MVDVLCEAIFLEQFMGRMLELGQ

SEQ ID NO: 3947 - protein, 42 aa, Homo sapiens
MVEKQNDKMESCHRSFQRQNQNTWALELGKIFLLDLAQEKDG

SEQ ID NO: 3948 - protein, 32 aa, Homo sapiens
MVELSLLLQLIVQLSLLLQLILWLSLSLQLMV

SEQ ID NO: 3949 - protein, 27 aa, Homo sapiens
MVETGFHHVGWAGLELLASGDLPSSAS

SEQ ID NO: 3950 - protein, 51 aa, Homo sapiens
MVFAFVFNHIKRGKCHNSSNVKTAQVYSDTNLIVHFQAFTFNSSMTTNSIN

SEQ ID NO: 3951 - protein, 14 aa, Homo sapiens
MVFFCSSVNSELLC

SEQ ID NO: 3952 - protein, 61 aa, Homo sapiens
MVFGAEVVLKRKENAGNCGLLLSPWRMVTINTDIFAKLCWDMLHVAPLLFPDHLESSAIQQ

SEQ ID NO: 3953 - protein, 26 aa, Homo sapiens
MVFGDVSRLLGTLSIVLNNSQLILSK

SEQ ID NO: 3954 - protein, 16 aa, Homo sapiens
MVFHHIGQAGLKLLTL

SEQ ID NO: 3955 - protein, 41 aa, Homo sapiens
MVFHHVGQAGLELLTSGDLPTSASQSAGITGMSHRARPNCF

SEQ ID NO: 3956 - protein, 30 aa, Homo sapiens
MVFLSMVSVTRGKVGSDSVLRPRPLVFSLE

SEQ ID NO: 3957 - protein, 31 aa, Homo sapiens
MVFNTSSKKATKSSVLGNHINIYYKCRKQGG

SEQ ID NO: 3958 - protein, 16 aa, Homo sapiens
MVFVMYSSFFNKHLKI

SEQ ID NO: 3959 - protein, 17 aa, Homo sapiens
MVGCCPGCCPFTNSSPP

SEQ ID NO: 3960 - protein, 89 aa, Homo sapiens
MVGGKIMLIIIFNQEFFLIFSLPIHMSVSSIWVQVCETKGRNPPDTASLRQVELLQFLSSYVNSVMAMRSFCLNAFSNKSRASWPNCFE

SEQ ID NO: 3961 - protein, 178 aa, Homo sapiens
MVGMKSMLSSPFVSSQRPNTELAAARTEQREFRVVVIPALAIEMVCCSMASWIATRSSSRILSNSSIQTTPPSARTMAPPSMMKFRDEGSLITEAVSPAALLPFPDVYTPMGEHFSTNFRSWDLAVPGSPSISRLMSPRRVSPSGSLFREPPKSRQAMAFFMSVPPKMEGAMLLEMTS

SEQ ID NO: 3962 - protein, 39 aa, Homo sapiens
MVGTYSYESLPLYCFWHIISFGILCLHYHLFHEIFQFPS

SEQ ID NO: 3963 - protein, 48 aa, Homo sapiens
MVHHKPSILHLHEITLSPTEFPSPSFLGLLLFVFLQACALLQLLHQCL

SEQ ID NO: 3964 - protein, 87 aa, Homo sapiens
MVHKLLLGVELPRAAFPVAVCLIDDFRLLFAFIFVPFLLDKGCSFGLFLLPPSPWAGEVFIGFDLGPLVVHRVTSAAHCRLTRGLVL

SEQ ID NO: 3965 - protein, 16 aa, Homo sapiens
MVIKLILKTYSYSYID

SEQ ID NO: 3966 - protein, 33 aa, Homo sapiens
MVILLKWRSDHVIPLLTFLLSPLIPIFFPKYIV

SEQ ID NO: 3967 - protein, 28 aa, Homo sapiens
MVISLFRFFEPMFQQTVNLELLCWMILL

SEQ ID NO: 3968 - protein, 35 aa, Homo sapiens
MVKDGSSHSSVFHVMICTVVPAAQELFVPDFLVIL

SEQ ID NO: 3969 - protein, 47 aa, Homo sapiens
MVKMKAQLSGAPHSLILTEAFPMTAFSGSGYNYFMSYITNHCSSFLS

SEQ ID NO: 3970 - protein, 22 aa, Homo sapiens
MVKTLMTQARLSVPGWLGCQRE

SEQ ID NO: 3971 - protein, 18 aa, Homo sapiens
MVKTVQRKAILLLLKTIS

SEQ ID NO: 3972 - protein, 38 aa, Homo sapiens
MVLALCPNISVDLVSASLKTEGEQQMTMVVLQFPPKES

SEQ ID NO: 3973 - protein, 42 aa, Homo sapiens
MVLEQYKHQDVNNLNERAGWNAIADGQPCHKTGPVCAYFCYR

SEQ ID NO: 3974 - protein, 12 aa, Homo sapiens
MVLERCSGKGMS

SEQ ID NO: 3975 - protein, 29 aa, Homo sapiens
MVLESHIRKAIPCGREEALSQFNRKSGDG

SEQ ID NO: 3976 - protein, 11 aa, Homo sapiens
MVLIEVICDAG

SEQ ID NO: 3977 - protein, 12 aa, Homo sapiens
MVLIRKGIMNKR

SEQ ID NO: 3978 - protein, 15 aa, Homo sapiens
MVLISSPRDPPASAS

SEQ ID NO: 3979 - protein, 23 aa, Homo sapiens
MVLLLAGLFSFWLKVRVEADQLV

SEQ ID NO: 3980 - protein, 50 aa, Homo sapiens [sequence omitted]

SEQ ID NO: 3981 - protein, 28 aa, Homo sapiens
MVLLVTDTVTLLLRSPDILHSSPSSSLR

SEQ ID NO: 3982 - protein, 11 aa, Homo sapiens
MVLQALYMIIS

SEQ ID NO: 3983 - protein, 13 aa, Homo sapiens
MVLRNLRKKPTIF

SEQ ID NO: 3984 - protein, 34 aa, Homo sapiens
MVLSIFSSSASSPWEKEGVPDSGGSGLQMGYSPC

SEQ ID NO: 3985 - protein, 20 aa, Homo sapiens
MVLSKVQGIRPFSVLQDESR

SEQ ID NO: 3986 - protein, 63 aa, Homo sapiens
MVMHWNTVSMAKAKLSKLVMPCLGPSQPGLHTVPFWHCRPWPVSSAQGEGSSSAGTSAMPSWL

SEQ ID NO: 3987 - protein, 28 aa, Homo sapiens
MVNHKGMILKRPLAGGEEKMCSLDAKDR

SEQ ID NO: 3988 - protein, 20 aa, Homo sapiens
MVPALSSLPEAGAEGMGTAS

SEQ ID NO: 3989 - protein, 18 aa, Homo sapiens
MVPDFFLHFLEVSLCQIR

SEQ ID NO: 3990 - protein, 23 aa, Homo sapiens
MVPLMIKLKVIHHIFFDLSNHVL

SEQ ID NO: 3991 - protein, 86 aa, Homo sapiens
MVPQLLGQGLPIQQGPGELAHQLVLLYQLPYQPQGLQQLQQVVPEQCQYLWGVAPPQSWIPSSPHAATPDPKPAFLHALVASHSLA

SEQ ID NO: 3992 - protein, 72 aa, Homo sapiens
MVQFFLSLLLMIQFSLSPQLMIQFSLSPQLIVQLSLSPRLIFQLSLSLQLMVQLSLSLQLVVHLYPLFQLMV

SEQ ID NO: 3993 - protein, 15 aa, Homo sapiens
MVQFNESHRLKGFKS

SEQ ID NO: 3994 - protein, 72 aa, Homo sapiens
MVQFSLLLQLIVHLYLSPQLMIQLSLSPQLRVQLSLSPQLIVQLSLSPQLIVQLSLLLQLIVQLSLLLRLIL

SEQ ID NO: 3995 - protein, 32 aa, Homo sapiens
MVQLLLILLMMMALSLSLQLMTQLYLIHQLMV

SEQ ID NO: 3996 - protein, 28 aa, Homo sapiens
MVQLSLSLLLIVQLSLSPQLIVLYSLSP

SEQ ID NO: 3997 - protein, 12 aa, Homo sapiens
MVQLSLSLQLIV

SEQ ID NO: 3998 - protein, 156 aa, Homo sapiens
MVQLSLSLQLIVQLSLSLQLMVWLSLSPQLIVQLSLSPQLIVQLSLSPQLIVQLSLSPQLIVQLSLSPQLIVQLSLSPQLIAELSLSLQLVIQLSLSPQLILQVALLLQLMGQLSLSLQLIVYLSLSPQLMVQLSLSLRLMVQLPLSLQLMVQLSL

SEQ ID NO: 3999 - protein, 82 aa, Homo sapiens
MVQLSLSLQLTVQLSLSLQLIVQLSLSLQLIVLLSLPLQLMIQLSLSPQLMVQLSLSPQLIFQLSLSLQLIVLLSLLPQLMV

SEQ ID NO: 4000 - protein, 32 aa, Homo sapiens
MVQLSLSPQLIFQLSLSLQLIVLLSLLPQLMV

SEQ ID NO: 4001 - protein, 12 aa, Homo sapiens
MVQSHCNLCLPD

SEQ ID NO: 4002 - protein, 152 aa, Homo sapiens
MVRAWARGPSSPLGSSSWGGGAGGGGPAPGGAAASGSGGGTAGSAPLQRLKPPARARASSRGSGGSSSSSSRGHRRCRARHRRPRPRPRAGSGLGGAGGPLGSAVYAAAVGRGLEGYARRGLSGGRRATSVAPGREVGRIQVRGLFFLPEWE

SEQ ID NO: 4003 - protein, 26 aa, Homo sapiens
MVRGAGKNGVELALASACLRLSLERA

SEQ ID NO: 4004 - protein, 18 aa, Homo sapiens
MVRSCALGASSEEGCGCW

SEQ ID NO: 4005 - protein, 15 aa, Homo sapiens
MVRSWIIFPFFHWSM

SEQ ID NO: 4006 - protein, 17 aa, Homo sapiens
MVRVNGVRRKKGPGTGK

SEQ ID NO: 4007 - protein, 25 aa, Homo sapiens
MVSACCNLCSSFWSCLCSQVSNFTW

SEQ ID NO: 4008 - protein, 24 aa, Homo sapiens
MVSCCNLCSSFWSCLCSQVSNFTW

SEQ ID NO: 4009 - protein, 17 aa, Homo sapiens
MVSFHKPSSFSPSLSII

SEQ ID NO: 4010 - protein, 14 aa, Homo sapiens
MVSFHYLVLAEFQE

SEQ ID NO: 4011 - protein, 54 aa, Homo sapiens
MVSFHYLVLAEWWRVWSLSLLMFRCVQSFFLLVGSWSRWLGSEAADLHGECYSS

SEQ ID NO: 4012 - protein, 52 aa, Homo sapiens
MVSFKEGAFLDIWQSKLGEGSKETLFLSTEGWIFFTFPKRTLKIKILSTVML

SEQ ID NO: 4013 - protein, 28 aa, Homo sapiens
MVSIHLIIEFQFCLSWEEHKEMRVSLLT

SEQ ID NO: 4014 - protein, 39 aa, Homo sapiens
MVSISLPCDPPASASQSAGITGVSHCARPISSCFLFFFF

SEQ ID NO: 4015 - protein, 47 aa, Homo sapiens
MVSISRPSDPPRALASQSAGIAGVSHRALPYICRFLRDKNSIRFVEI

SEQ ID NO: 4016 - protein, 33 aa, Homo sapiens
MVSISSPRDLPASASQRAGITGMSHCAWPCFTF

SEQ ID NO: 4017 - protein, 29 aa, Homo sapiens
MVSISSPRDPPASASQSCWDYRREPPRPA

SEQ ID NO: 4018 - protein, 12 aa, Homo sapiens
MVSKNIMLLSNK

SEQ ID NO: 4019 - protein, 149 aa, Homo sapiens
MVSLLSSWFRPRIRSRRSIWTCRKGSLTPDMLCSVEYPIVTRVRRMCTSWGTTMVTLMKQLGTGWEEDTGEFRDLPDHVHCSQNSLLAHVGTGLQEQFLHLWGQVSAHLSRAHGAQSAQGQALYWLNPLAQVILDAVGNEQVGIVPLIQ

SEQ ID NO: 4020 - protein, 189 aa, Homo sapiens
MVSLLSSWFRPRIRSRRSIWTCRKGSLTPDMLCSVEYPIVTRVRRMCTSWGTTMVTLMKQLGTGWEEDTGEFRDLPDHVHCSQNSLLAHVGTGLQEQFLHLWGQVSAHLSRAHGAQSAQGQALYWLNPLAQVTVQSGRGSPTCGRRAVWPAAGACALGPRRGRRPGCGHTPFGSPPAPGPESWPRESLR

SEQ ID NO: 4021 - protein, 18 aa, Homo sapiens
MVSLQCEFFDVEQGMNYD

SEQ ID NO: 4022 - protein, 27 aa, Homo sapiens
MVSNLCQVNKRWRYTNSRGNKVCVYLI

SEQ ID NO: 4023 - protein, 70 aa, Homo sapiens
MVSNSRPQVIRPPRPPKALGLQVRATVPTPIFLNLCLMPPAWVDEPGLLPSSPDGHRQNLVGALQFTPRG

SEQ ID NO: 4024 - protein, 39 aa, Homo sapiens
MVSNSWVQAIHPAFQSAGIMLRKAECWEKLRQGLHSDIM

SEQ ID NO: 4025 - protein, 22 aa, Homo sapiens
MVSQEYNCSLALCVKIGGEDVN

SEQ ID NO: 4026 - protein, 181 aa, Homo sapiens
MVSRRSVVACSRPCFSLCRLCSSSCWALSWHCPCSRSLCSCSSTRARWASASSRLPRSSSRSWSRLSSCFSRARCLACRDSWWRTMLSTRAFSLSSSVLAQQTCWPAPSSRPTNSCTCASNCCTCSSSCCTCLSAAALRSPSSCSCWAFASTACVDSRCCFSSLSRVAIFVFRSLVSRFPH

SEQ ID NO: 4027 - protein, 282 aa, Homo sapiens
MVSRRSVVACSRPCFSLCRLCSSSCWALSWHCPCSRSLCSCSSTRARWASASSRLPRSSSRSWSRLSSCFSRARCLACRDSWWRTMLSTRAFSLSSSVLAQQTCWPAPSSRPTNSCTCASNCCTCSSSCCTCLSAAALRSPSSCSCWAFASTACVDSRCCFSSLSRVAIFVFRSLVSVSSCCLSCSHSDRHCSSSSACRRRAPCSCFSACSSLPACFLRPSFCPSASSSWALRASTCLLRRVRSFLCSAAQRPTVAAGSGLSPMLSCTSCWNWPKDEGRFWL

SEQ ID NO: 4028 - protein, 21 aa, Homo sapiens
MVSRSNYFGKTDKGIFIPLCL

SEQ ID NO: 4029 - protein, 23 aa, Homo sapiens
MVSTVSNRTAFPAFRLVSVLVAT

SEQ ID NO: 4030 - protein, 178 aa, Homo sapiens
MVSTVSNRTAFPAFRLVSVLVATWASKSFMVSLLSSWFRPRIRSRRSIWTCRKGSLTPDMLCSVEYPIVTRVRRMCTSWGTTMVTLMKQLGTGWEEDTGEFRDLPDHVHCSQNSLLAHVGTGLQEQFLHLWGQVSAHLSRAHGAQSAQGQALYWLNPLAQVILDAVGNEQVGIVPLIQ

SEQ ID NO: 4031 - protein, 218 aa, Homo sapiens
MVSTVSNRTAFPAFRLVSVLVATWASKSFMVSLLSSWFRPRIRSRRSIWTCRKGSLTPDMLCSVEYPIVTRVRRMCTSWGTTMVTLMKQLGTGWEEDTGEFRDLPDHVHCSQNSLLAHVGTGLQEQFLHLWGQVSAHLSRAHGAQSAQGQALYWLNPLAQVTVQSGRGSPTCGRRAVWPAAGACALGPRRGRRPGCGHTPFGSPPAPGPESWPRESLR

SEQ ID NO: 4032 - protein, 15 aa, Homo sapiens
MVTGQQFKNQMCFMC

SEQ ID NO: 4033 - protein, 57 aa, Homo sapiens
MVTRIARASGSKSKENSGPPCLCESNLGRLSHVSGSEGWVLLERSPLWEMSGEGMEM

SEQ ID NO: 4034 - protein, 15 aa, Homo sapiens
MVTYHQLCKEKYINI

SEQ ID NO: 4035 - protein, 16 aa, Homo sapiens
MVVCNTGGFLKWHIFP

SEQ ID NO: 4036 - protein, 25 aa, Homo sapiens
MVVFWVPPRWLEDYGLWDFPFLPGV

SEQ ID NO: 4037 - protein, 40 aa, Homo sapiens
MVVHLVLTLKPNILPSGDFHQPCRLSYRNTKEEAQPSPVP

SEQ ID NO: 4038 - protein, 13 aa, Homo sapiens
MVVHRGPCPRSPT

SEQ ID NO: 4039 - protein, 92 aa, Homo sapiens
MVVIYMVHKLLLGVELPRAAFPVAVCLIDDFRLLFAFIFVPFLLDKGCSFGLFLLPPSPWAGEVFIGFDLGPLVVHRVTSAAHCRLTRGLVL

SEQ ID NO: 4040 - protein, 40 aa, Homo sapiens
MVVPGDHICTSKFSVNIKCSHFRFKSIFQFFSCFEIPNKV

SEQ ID NO: 4041 - protein, 82 aa, Homo sapiens
MVVSFGRSGGSAVRFLLSQFTSRWLATLETSQMGWGCKGLGSRSSKRRRGMRTGRQKDLRRHRASSRVPLDSVLLSSSPMED

SEQ ID NO: 4042 - protein, 812 aa, Homo sapiens
MVVVPVIPADGPVIPVTPAESPAIPVTPTDSPVVPVTSADSPVIPVTADSPFVPVTPADSPVIPVTPPDDLVVPVTPTDCPVVPVTLADCPVVSVTPANSPVDPVTPADGPVVPVTPADSPVIPVTPADDLIVPVTPADSLIVSVTPADSPVVPVTPADSPVISVASADSPVVPVTPADTVVVPVTPADGPVIPVTPAESPAIPVTPADSPVVPVTPADDPVVPVTPADSPIVPVPPASDPVVPVTPADTPGSPVASADGPVVPVTSADSPLVPVTPGDSPVVPVTPADSPVFPVTSADGPVFPVTLADDPVFPVTPADDPIFPVSPADSPVVPVTPANIPVVPVPPANGSVVPVTSAGSPFVPIIPADGLVVLDSSTDVLVVLVSPTDGIPVPDLADDPVVSVTTSDSPVIPVTPTDSPVVPVAPADGPVVPVTSVDSPVVPVTPADSPVIPVTPADSLVVPATPADDPVVSVTPADGPVVPVTTADIPVISVTSADSPVVPVTPADGLVVPVTSADSVVVPATPADCPLVPVDPADSPIVLFTPYDNPVVSVTSDDSPVFPVTPADSSVVPVTPAGVPVVPVTPGDGPVVPVTPADSLVVPVTSADSPVFPVTPADSPVFPVSPADDLVVLVTPGDSPVVPVSPADSPVVLVTPADGPVVPVTPANGPVVPVTSADSPFVPVIPADGLVVLDSSTDVLVVPVFPTDGILVPDLADDPVVPVTPGDDPVVPVTPGDDPVIPVTPADDGPFVPVTPAVGPVVPDLTADDSVVPDSLTDDPVISVCPDDGLVVPDTVRDCTVVPDTAADDPVV

SEQ ID NO: 4043 - protein, 12 aa, Homo sapiens
MVWLPLILQPMF

SEQ ID NO: 4044 - protein, 17 aa, Homo sapiens
MVYLKFFFCLDGRHLQL

SEQ ID NO: 4045 - protein, 41 aa, Homo sapiens
MWAEAWDGDQEDSGTQSFVVERLEEPLHQFDFSSQVTCKHT

SEQ ID NO: 4046 - protein, 34 aa, Homo sapiens
MWAEAWDGDQEDSGTQSFVVERLEEPSALPHSFA

SEQ ID NO: 4047 - protein, 12 aa, Homo sapiens
MWAYFQPRDMHG

SEQ ID NO: 4048 - protein, 12 aa, Homo sapiens
MWFGCAPTQIST

SEQ ID NO: 4049 - protein, 16 aa, Homo sapiens
MWFHRVSQDGLDLLTS

SEQ ID NO: 4050 - protein, 23 aa, Homo sapiens
MWFPIRLSKAELQARATLAVPMT

SEQ ID NO: 4051 - protein, 29 aa, Homo sapiens
MWGFSWASHFPPAVPILYHGNADKSRSIG

SEQ ID NO: 4052 - protein, 39 aa, Homo sapiens
MWHPMVKDGSSHSSVFHVMICTVVPAAQELFVPDFLVIL

SEQ ID NO: 4053 - protein, 21 aa, Homo sapiens
MWKDAERNLKSGTDCFSSSKM

SEQ ID NO: 4054 - protein, 24 aa, Homo sapiens
MWKLRSPPFISVSTRHSASLVSQV

SEQ ID NO: 4055 - protein, 16 aa, Homo sapiens
MWKTCKLEKHKENELT

SEQ ID NO: 4056 - protein, 26 aa, Homo sapiens
MWKTCKLIIWQKAFQRKTKSSRIQFP

SEQ ID NO: 4057 - protein, 15 aa, Homo sapiens
MWKTCKLSNVQGLLI

SEQ ID NO: 4058 - protein, 17 aa, Homo sapiens
MWLFHSGSLMINWVFLK

SEQ ID NO: 4059 - protein, 57 aa, Homo sapiens
MWMCSKMPCSRRCRALKFSTPHCGMAMLASSVNVSEKLILPGWVSGAGVPGVLKDKG

SEQ ID NO: 4060 - protein, 39 aa, Homo sapiens
MWPGPAWLLWASARREGEAMECRWRGFRATKLCDFESPC

SEQ ID NO: 4061 - protein, 15 aa, Homo sapiens
MWPGSGLPAPCDCQP

SEQ ID NO: 4062 - protein, 121 aa, Homo sapiens
MWQELKPQLVHLEFVLFFFHTEGLLDVNFLQHLPQAHPGELLLQAFHSLQGFLGVEHGHAHHGCLDVGAGHHENLPQPWNAQGDVHLASACKVEGVEGHLGGGLSDALGSQQAHSLARLTQ

SEQ ID NO: 4063 - protein, 27 aa, Homo sapiens
MWQMWKLRSPPFISVSTRHSASLVSQV

SEQ ID NO: 4064 - protein, 40 aa, Homo sapiens
MWQPRSSFHTGASPPRMGDGGLGVKAASGVCRSQPQRGKA

SEQ ID NO: 4065 - protein, 14 aa, Homo sapiens
MWRNKNTFTLLVGL

SEQ ID NO: 4066 - protein, 22 aa, Homo sapiens
MWRNRNAFNTVGGSVIYFNHCG

SEQ ID NO: 4067 - protein, 14 aa, Homo sapiens
MWRNRNTFTLLVGV

SEQ ID NO: 4068 - protein, 69 aa, Homo sapiens [sequence omitted]

SEQ ID NO: 4069 - protein, 64 aa, Homo sapiens
MWSCTEYVMRIRWHSAVKICSFSSDVSSKNSEVSSFSRNSSCTSLSSNAAESLLSSVSEPSLSS

SEQ ID NO: 4070 - protein, 15 aa, Homo sapiens
MWSYKCKHTGTMRNR

SEQ ID NO: 4071 - protein, 39 aa, Homo sapiens [sequence omitted]

SEQ ID NO: 4072 - protein, 11 aa, Homo sapiens
MWTRLTPFEQR

SEQ ID NO: 4073 - protein, 39 aa, Homo sapiens
MWTSLVDWTVRLPPVKEFMLAEPLQRKALLGLNCDWVKL

SEQ ID NO: 4074 - protein, 14 aa, Homo sapiens
MWTYWGRGALFCLL

SEQ ID NO: 4075 - protein, 20 aa, Homo sapiens
MWVNQQWPLLAILDQDGILY

SEQ ID NO: 4076 - protein, 11 aa, Homo sapiens
MWWEHAHLIII

SEQ ID NO: 4077 - protein, 32 aa, Homo sapiens
MWYKELETSHSQEMDRAGGVLNENTVSVIFVA

SEQ ID NO: 4078 - protein, 12 aa, Homo sapiens
MYCSNLTFMYFG

SEQ ID NO: 4079 - protein, 59 aa, Homo sapiens
MYETHKTRDCGTWENTTYTQYIIRNSAFHYNIRTELLGNNIPLLHVTLYIVQYLLFPGQ

SEQ ID NO: 4080 - protein, 14 aa, Homo sapiens
MYFFLISKDKRIGT

SEQ ID NO: 4081 - protein, 11 aa, Homo sapiens
MYFNNIIVFGT

SEQ ID NO: 4082 - protein, 13 aa, Homo sapiens
MYFSPSIIFMLEF

SEQ ID NO: 4083 - protein, 39 aa, Homo sapiens
MYGKYHLLGQKSRTRSLSLIIGRTQYIFCSTYKKDVYYL

SEQ ID NO: 4084 - protein, 13 aa, Homo sapiens
MYGLFEVFLLFGW

SEQ ID NO: 4085 - protein, 18 aa, Homo sapiens
MYGNPQSRKGRKILKILL

SEQ ID NO: 4086 - protein, 11 aa, Homo sapiens
MYGTLLETLYT

SEQ ID NO: 4087 - protein, 68 aa, Homo sapiens
MYGVWMKHDHRLKQEGRVPWRRTVADKYNGLHLQNIYPDPLGSFFLTTLEHKFDQKVSLDLKASLIYK

SEQ ID NO: 4088 - protein, 30 aa, Homo sapiens
MYHHAWLICVFSRDGVSPCWSGWSRTCDLR

SEQ ID NO: 4089 - protein, 54 aa, Homo sapiens
MYHHDRLILVFLIEMGFHHIGQAGLDLLTSGGPTASASQNAEIVGVSHRSWQLR

SEQ ID NO: 4090 - protein, 51 aa, Homo sapiens
MYHVGFFHLEHSCPGDQKEVFWDFSGLYCTSLPCISAESLSSSGGLGVGES

SEQ ID NO: 4091 - protein, 40 aa, Homo sapiens
MYHVGFFHLEHSCPGDQKEVFWDFSGLYQFFCECFFSQLP

SEQ ID NO: 4092 - protein, 39 aa, Homo sapiens
MYHYFRFIEQMVYENIIHLNINPLKILAGFINVYSIFFT

SEQ ID NO: 4093 - protein, 37 aa, Homo sapiens
MYICILSPTKLHEIRDFHLFSVHCWFFFLVPRIVPGT

SEQ ID NO: 4094 - protein, 25 aa, Homo sapiens
MYIKKNLTFPTKSTILLSQKKSSSS

SEQ ID NO: 4095 - protein, 53 aa, Homo sapiens
MYILATVSSLSSFSMDFIRCWKRALQASTSSSKRKRSATENSTESRLSCRKSS

SEQ ID NO: 4096 - protein, 42 aa, Homo sapiens
MYIVSIFTVNIYLLVRENPMNIFFLFFLRWNLTGCPGWSAVA

SEQ ID NO: 4097 - protein, 26 aa, Homo sapiens
MYKHWQGTVAHACNPSTLGGRGGWIT

SEQ ID NO: 4098 - protein, 24 aa, Homo sapiens
MYKRAKLPLSAGRPHVTERLRLCC

SEQ ID NO: 4099 - protein, 57 aa, Homo sapiens
MYLHVGSKNVISISSLNSLNNYFLIRKKSQILCVQKQKHPPSTHTHTHTLLITKSKL

SEQ ID NO: 4100 - protein, 140 aa, Homo sapiens [sequence omitted]

SEQ ID NO: 4101 - protein, 25 aa, Homo sapiens
MYLNEKVTCLDVLFHVLVSSSQPPE

SEQ ID NO: 4102 - protein, 11 aa, Homo sapiens
MYLSCQSGKLW

SEQ ID NO: 4103 - protein, 17 aa, Homo sapiens
MYPESPRLRKLTGFHFE

SEQ ID NO: 4104 - protein, 26 aa, Homo sapiens
MYPFQTGFFHLAKCLCFFCIFLWLDS

SEQ ID NO: 4105 - protein, 11 aa, Homo sapiens
MYPINMYNYVN

SEQ ID NO: 4106 - protein, 42 aa, Homo sapiens
MYPLAELADVVTTLTMVTVGACCTTWMAWPAGCCEVTMEAGM

SEQ ID NO: 4107 - protein, 88 aa, Homo sapiens
MYPLSHHLHLFLQAPSLIVQILQQAALLGLPPAYSDQLQRAGQLHFYSGLIKISLVLTTRLSFLKAMSPSDVMHAVTGEYESSHLSSS

SEQ ID NO: 4108 - protein, 68 aa, Homo sapiens
MYPLSSRSICCCRLSFRKARRFSTRSLSLANSPDSTPSTRFSIKKEPMMMRGMKYNQFQVFPEASLLL

SEQ ID NO: 4109 - protein, 27 aa, Homo sapiens
MYQKWNPYNTDGNVQWHSLFGKTLQIL

SEQ ID NO: 4110 - protein, 13 aa, Homo sapiens
MYQLISASKSILS

SEQ ID NO: 4111 - protein, 18 aa, Homo sapiens
MYQYFIPFLLPHSIPLCR

SEQ ID NO: 4112 - protein, 27 aa, Homo sapiens
MYRTASRPAPENHLPLCVISAEVEKSW

SEQ ID NO: 4113 - protein, 16 aa, Homo sapiens
MYSCDNFNLTCILICL

SEQ ID NO: 4114 - protein, 107 aa, Homo sapiens
MYSGKTEKHLWFFSWSICSFKKIFFIQWKIYNLFTCPAGRASRQLFGGPCGGPSGGQGAGGGKARAASGGPHTHGPGRGRSAYGHRHGRPAARDRLGAAGGTPIAPK

SEQ ID NO: 4115 - protein, 92 aa, Homo sapiens
MYSISAMNFFCSLQNACHWCMFTMFSIGSVLGDADDALLFGHDHGHIHHLLGPLHPLQQDRLAGQRLGLDLRRHRRRGRAWGAAANRAAGPG

SEQ ID NO: 4116 - protein, 35 aa, Homo sapiens
MYSITFPSVTKILIKYMNASYQIILKVYFLSLIIR

SEQ ID NO: 4117 - protein, 12 aa, Homo sapiens
MYSSFFNKHLKI

SEQ ID NO: 4118 - protein, 32 aa, Homo sapiens
MYSTDAFRMVPLFQRISGSLDFGIRVPSSLIR

SEQ ID NO: 4119 - protein, 31 aa, Homo sapiens
MYTAVKVTTLLNCTAHYRTNYWKFSSHTGIF

SEQ ID NO: 4120 - protein, 20 aa, Homo sapiens
MYTKYLTKFTTYMVNFTYKL

SEQ ID NO: 4121 - protein, 26 aa, Homo sapiens
MYTLQKGRIRKTEIKFNRATPMEQNL

SEQ ID NO: 4122 - protein, 25 aa, Homo sapiens
MYVHTHTLSCAQKHTMCILIINGPI

SEQ ID NO: 4123 - protein, 26 aa, Homo sapiens
MYVHYLQSVVFLHHLYSYWILSHQHG

SEQ ID NO: 4124 - protein, 11 aa, Homo sapiens
MYVLRQAICSC

SEQ ID NO: 4125 - protein, 15 aa, Homo sapiens
MYVPIYFFAICILVQ

SEQ ID NO: 4126 - protein, 25 aa, Homo sapiens
MAADVLSRSLLGSPLAPVEETPLAF

SEQ ID NO: 4127 - protein, 51 aa, Homo sapiens
MAADVLSRSLLGSPLAPVEETPLAFPPRLPLRTPRGWPAGGWRPATAEHRA

SEQ ID NO: 4128 - protein, 27 aa, Homo sapiens
MAAFGAKRMQKSSFSVGTPVIASLMKW

SEQ ID NO: 4129 - protein, 23 aa, Homo sapiens
MAALIVNTPFQLDVPPFQLDVPS

SEQ ID NO: 4130 - protein, 54 aa, Homo sapiens
MAAPAAGLRAPGILESGEGTAARRSLCVLPADLCVPRRERASQPGRQLQRVSPH

SEQ ID NO: 4131 - protein, 29 aa, Homo sapiens
MAAPAAGLRAPGILESGEGTALRRGGRKS

SEQ ID NO: 4132 - protein, 65 aa, Homo sapiens [sequence omitted]

SEQ ID NO: 4133 - protein, 23 aa, Homo sapiens
MAASLLFSDLGFLASRIPRNGTL

SEQ ID NO: 4134 - protein, 119 aa, Homo sapiens
MAATISTLLLGLGTSRLPTYLASKQMPCWKASSLCKGIRRSCPSSTRLYLVLLGMVTRGGPAPSEAAAAGRGWRDPGEGRLELGAATRGGAWERWAGGALAARRPDPERCRGPSGSGLS

SEQ ID NO: 4135 - protein, 13 aa, Homo sapiens
MAATVITKRGRAL

SEQ ID NO: 4136 - protein, 16 aa, Homo sapiens
MACCFPLHHRRPRRGE

SEQ ID NO: 4137 - protein, 24 aa, Homo sapiens
MACSRLTATSTSQVQAILLPQPPE

SEQ ID NO: 4138 - protein, 34 aa, Homo sapiens
MADLKLLTSDDLPASASQSAGLTSVSHHTWLTPS

SEQ ID NO: 4139 - protein, 171 aa, Homo sapiens
MAEGRCFPLPPLSDMMVPTASSWAQPQAQDSSYRSCSGRGKHSLGRLHGSHPQLCLPWGTFPATGWCGLAGTSSPMGKLDLHWLGGFVSQLIRDKVLKDKAPSKHLSFCPILFLPDKIPEIFVGDRKYVDGKGFHCRLPHRPVTISAVWRICSHQESPTLQLDHASSLSIS

SEQ ID NO: 4140 - protein, 30 aa, Homo sapiens
MAEKGQETKKSCGRTDWQRHREGTATALHR

SEQ ID NO: 4141 - protein, 38 aa, Homo sapiens [sequence omitted]

SEQ ID NO: 4142 - protein, 34 aa, Homo sapiens
MAFSTAALICCSSLTSTIHGKAFPPTASISSAAV

SEQ ID NO: 4143 - protein, 32 aa, Homo sapiens
MAFSTAALICCSSLTSTIHGKAFPPTASTGVG

SEQ ID NO: 4144 - protein, 43 aa, Homo sapiens
MAFTSTSLVMLSTMPEANSSGIFPSVCPLTHWFMVFLASSEAC

SEQ ID NO: 4145 - protein, 36 aa, Homo sapiens
MAGFPWVPNISMCKCARPLAMDSTIRRQLTVSRVVS

SEQ ID NO: 4146 - protein, 38 aa, Homo sapiens
MAGHKIPNVQAYMISVHTQVASVLSNLCQSTNSLCEAK

SEQ ID NO: 4147 - protein, 19 aa, Homo sapiens
MAGIATKASFRKFIVFDYG

SEQ ID NO: 4148 - protein, 34 aa, Homo sapiens
MAGPPLVPRNPFRKSTTPQKVSGGENLNLMLEGC

SEQ ID NO: 4149 - protein, 12 aa, Homo sapiens
MAGQEAQIFKPD

SEQ ID NO: 4150 - protein, 26 aa, Homo sapiens
MAHRSDKSTPGTREANVSRLTESGKQ

SEQ ID NO: 4151 - protein, 18 aa, Homo sapiens
MAHVCNPKTLGGRGGKIA

SEQ ID NO: 4152 - protein, 60 aa, Homo sapiens
MAIIKKSGNNRCRRGCGEIGTLLHCWWDCKLVQPLCKSMWRFLRDLEPSHPITGYIPKGL

SEQ ID NO: 4153 - protein, 194 aa, Homo sapiens
MAIIKKSGNNRCWRGCGEIGTLLHCWWDCKLVQPLWKSVWRFLRDLELEIPFDPAIPLLGIYPKDYKSCCYKDTCTRMFIAALFTIAKTWNQPKSPTRIDWIKKMWHIYTMEYYAAIKNDEFMSFVGTWMKLEIIILSKLSQGQKNQTLHVLTHRWELNNENTWTQEGEHHTLGTVVGWGEGGGIALGDIANAK

SEQ ID NO: 4154 - protein, 33 aa, Homo sapiens
MAIINQTIIDAGVDAVKRELLHCWWECKLVQPL

SEQ ID NO: 4155 - protein, 16 aa, Homo sapiens
MAIPVLMFCGSSYSGG

SEQ ID NO: 4156 - protein, 31 aa, Homo sapiens
MAIPVLMFCNPNTLGGRGRQITRPGDRDHPD

SEQ ID NO: 4157 - protein, 16 aa, Homo sapiens
MAIPVLMFCNPSYSGG

SEQ ID NO: 4158 - protein, 54 aa, Homo sapiens
MAIPVLMFRTRRRWSSAHCEIRATTLGSIPSLSADGEPVAAGCPAMFPASCERP

SEQ ID NO: 4159 - protein, 55 aa, Homo sapiens
MAIQTEAWLAANSRMLAVRTTAWGTWRASTAPCRRKPANTMTTWMMISEAVSARR

SEQ ID NO: 4160 - protein, 26 aa, Homo sapiens
MAITKIPRNNRYWQGCGEKGTFIHRY

SEQ ID NO: 4161 - protein, 13 aa, Homo sapiens
MAITKKSKNNRCS

SEQ ID NO: 4162 - protein, 13 aa, Homo sapiens
MAKHKTAMATKIR

SEQ ID NO: 4163 - protein, 12 aa, Homo sapiens
MAKIQNTGNIKC

SEQ ID NO: 4164 - protein, 18 aa, Homo sapiens
MAKPRLSDNSKSHGLTEH

SEQ ID NO: 4165 - protein, 20 aa, Homo sapiens
MAKQGKHPHQNNLNNKDPHY

SEQ ID NO: 4166 - protein, 11 aa, Homo sapiens
MAKQSAYLFPP

SEQ ID NO: 4167 - protein, 17 aa, Homo sapiens
MAKSTRCAKGLLSPSYF

SEQ ID NO: 4168 - protein, 18 aa, Homo sapiens
MALCHLSLVWLSLAHIPP

SEQ ID NO: 4169 - protein, 170 aa, Homo sapiens
MALELQCVQIRYLHNLPVFLALLFHVLGLSLFSLCRSKSRPLSFPSLVFSSILSFTLYFSLYFFPRAISSGIGGGGLGVRGPFFLLWLVFEFLCWSNRGEDTADVFLSFLLAEDDFGLDFRFGDLLDFLREGDGDNFDLTTSGETSFLMIISSLFSMFSCSSFINSLCIF

SEQ ID NO: 4170 - protein, 32 aa, Homo sapiens
MALENCRLYEIYSNWHRKTPITTTIFLKKQIT

SEQ ID NO: 4171 - protein, 36 aa, Homo sapiens
MALFSVHLQVKELMRCGVTKGQKTRGRNKGPKNPKP

SEQ ID NO: 4172 - protein, 18 aa, Homo sapiens
MALLMIIHSPSKLTAYSA

SEQ ID NO: 4173 - protein, 94 aa, Homo sapiens
MALLRAQPPQPLRPHAHFPWGHCPAPGMQTQAPCRPQWCPHALTGHRPACLVRWEARRERGVRPGLGFRAGSSNGIRTVLASELCLPKIRMLMS

SEQ ID NO: 4174 - protein, 11 aa, Homo sapiens
MALPKQVEITE

SEQ ID NO: 4175 - protein, 109 aa, Homo sapiens
MALPPAQDGKSQQALEMDILRRCPLGPLHPELPEEPSTRVFPLAPAGKSEPVWEMEMLPGKPQPHNSPASHPCTGLSEQGPGRSIRSQRSRRPHPRRSLTPARPQHPGG

SEQ ID NO: 4176 - protein, 20 aa, Homo sapiens
MALSPIAGSGTQMQRLLLLS

SEQ ID NO: 4177 - protein, 18 aa, Homo sapiens
MAMSSTISTPPMTWMKKI

SEQ ID NO: 4178 - protein, 18 aa, Homo sapiens
MAMSSTISTPPTTWMKKI

SEQ ID NO: 4179 - protein, 25 aa, Homo sapiens
MANALDSFSSQKLEFLLNSKLNNVL

SEQ ID NO: 4180 - protein, 14 aa, Homo sapiens
MANNKNMIYIMKWD

SEQ ID NO: 4181 - protein, 100 aa, Homo sapiens
MANPIFNSMTRTIMIELGPELASFSKAGHESLLAGFFGIASSDFLAFGSALLSLATGFVTDLEGLHLLADGLCTSAEEDWLDPSPSSTSTGGCWGAFSFT

SEQ ID NO: 4182 - protein, 92 aa, Homo sapiens
MANSLAELKVLGLERFLDLRLPVPRRMLLLLLLRRRGRAGGQAVQHLPDVEFPHGLGGAPPQPGRGGTGGPRAGETTRGRRQLRPRKRRSGS

SEQ ID NO: 4183 - protein, 104 aa, Homo sapiens [sequence omitted]

SEQ ID NO: 4184 - protein, 16 aa, Homo sapiens
MAPRKLCLNKYSRFSF

SEQ ID NO: 4185 - protein, 31 aa, Homo sapiens
MAQGDLGVQRGLGGLVLHLGLVARGHQAVLL

SEQ ID NO: 4186 - protein, 20 aa, Homo sapiens
MAQNLGPGLHPPVLGGGRLC

SEQ ID NO: 4187 - protein, 28 aa, Homo sapiens
MAQNLGPGLHPPVLGGGRLCPDPGRGGG

SEQ ID NO: 4188 - protein, 30 aa, Homo sapiens
MAQNLGPGLHPPVLGGGRLCPDPGRGGGGA

SEQ ID NO: 4189 - protein, 24 aa, Homo sapiens
MAQSQLTATSASQVQVILLPQPPE

SEQ ID NO: 4190 - protein, 29 aa, Homo sapiens
MAQSTSISVPHSGYKMHQHSFFLKKKNPL

SEQ ID NO: 4191 - protein, 14 aa, Homo sapiens
MARITLDTQGFHTD

SEQ ID NO: 4192 - protein, 24 aa, Homo sapiens
MARMVSRSRVSFSRTTAFTVSVTE

SEQ ID NO: 4193 - protein, 31 aa, Homo sapiens
MARPAPLSRSLAPRRPLRAARSRPLAGQLGT

SEQ ID NO: 4194 - protein, 26 aa, Homo sapiens
MARPASVRAEAGTGPGLAAAAQTSAT

SEQ ID NO: 4195 - protein, 14 aa, Homo sapiens
MARPPPPGPPRGPP

SEQ ID NO: 4196 - protein, 24 aa, Homo sapiens
MARPRLIATSASQVQAILLSQPSK

SEQ ID NO: 4197 - protein, 94 aa, Homo sapiens
MARRKARRMAKSSEQRIERTWTGHRRGWALLPAAAGKIPLRLSGRTGDPFPSGGSTERFLGSDHAPAENSARRSRATWSHPSSSSTSPSPQLSP

SEQ ID NO: 4198 - protein, 18 aa, Homo sapiens
MARRRRLLARLPAPPPPP

SEQ ID NO: 4199 - protein, 26 aa, Homo sapiens
MARRRRLLARLPAPPPPPSGAADQDD

SEQ ID NO: 4200 - protein, 26 aa, Homo sapiens
MARVSRTITRTLSSEGCISEATCPDP

SEQ ID NO: 4201 - protein, 27 aa, Homo sapiens
MARVSRTITRTLSSEGCISEATCPDPP

SEQ ID NO: 4202 - protein, 38 aa, Homo sapiens
MARVSRTITRTLSSEGCISEATCPDPPSLQPEPDGYPG

SEQ ID NO: 4203 - protein, 17 aa, Homo sapiens
MASFEKDFINAIIPSLS

SEQ ID NO: 4204 - protein, 28 aa, Homo sapiens
MASGEQDRGLAPDHMVQKFSSTSRISST

SEQ ID NO: 4205 - protein, 28 aa, Homo sapiens
MASGEQDRSLAPDHMVQKFSSTSRISST

SEQ ID NO: 4206 - protein, 32 aa, Homo sapiens
MASIKLGPWFRLFSVSETCFELFSKILSKSPS

SEQ ID NO: 4207 - protein, 19 aa, Homo sapiens
MASNWKQIPHKRQSESLGY

SEQ ID NO: 4208 - protein, 20 aa, Homo sapiens
MASRPAAAAGGLARRRQTQC

SEQ ID NO: 4209 - protein, 52 aa, Homo sapiens
MASSFFLSTRKRSSLHSGLCRVAPATKSSSEPGTGESVLRSLLEPGSDCAAR

SEQ ID NO: 4210 - protein, 37 aa, Homo sapiens
MASSTLCTFTMGRMGPKISSCITGSVSCTSTSTVGAM

SEQ ID NO: 4211 - protein, 44 aa, Homo sapiens
MASSVASLSSAQLSDFSILASPTLRLSFPFLFFSIFTFFSEFPL

SEQ ID NO: 4212 - protein, 24 aa, Homo sapiens
MASVIFFLYFNSYVLDLLLFVFYS

SEQ ID NO: 4213 - protein, 18 aa, Homo sapiens
MATKAQIEKWDLIKLKSF

SEQ ID NO: 4214 - protein, 50 aa, Homo sapiens
MATTQTDGLSNCFVESLSANWAGEEIRPLWSLYRHCFWSYNSRTQTHTQI

SEQ ID NO: 4215 - protein, 63 aa, Homo sapiens
MATVDWKITHCGWNRGASVCHSPHHSLLLTQTKYINYHLSSHCCFPYTSPAILVTTEGIRSAK

SEQ ID NO: 4216 - protein, 48 aa, Homo sapiens
MATWPCFSFLFFGDGVLLLLPRLEFSGAILAHCNFRLPDLSNSPASAS

SEQ ID NO: 4217 - protein, 25 aa, Homo sapiens
MAVFDLPMFLQLCNELAKLLVRWIQ

SEQ ID NO: 4218 - protein, 33 aa, Homo sapiens
MAVFSSLLTSSIFSCISASNILSSKYSFLNLFS

SEQ ID NO: 4219 - protein, 34 aa, Homo sapiens
MAVIGKPSFSLSSLTFFRATSSPVSLSLALYTWP

SEQ ID NO: 4220 - protein, 51 aa, Homo sapiens [sequence omitted]

SEQ ID NO: 4221 - protein, 32 aa, Homo sapiens
MAVKVVQVNYLFIVVSLFHFQMQTCTYGTANI

SEQ ID NO: 4222 - protein, 64 aa, Homo sapiens
MAVQYRLCSKTWIQSLAPSLRCGVRGMKVNSCTLVSSLCENIKSDTPSRGLPHSVLLLPVNGTT

SEQ ID NO: 4223 - protein, 33 aa, Homo sapiens
MAVRVLPKPISSAKIPPWTFSGRSFSEKFVIVL

SEQ ID NO: 4224 - protein, 20 aa, Homo sapiens
MAVVFPWSICTNQGIFIQVS

SEQ ID NO: 4225 - protein, 52 aa, Homo sapiens
MAVVTVGPHSSPIPDFNGHSLNTSSFNIKIIIICGYRIHQNQKSYKIIKSFS

SEQ ID NO: 4226 - protein, 23 aa, Homo sapiens
MAVVWYLASNSLLNELINEHPPN

SEQ ID NO: 4227 - protein, 66 aa, Homo sapiens
MAWGSGVLPTGRGSGGCTRRPHPRRARSCGCPRRCAGTPAGSAPSPRSAHRPAEWAASRPGRTRLS

SEQ ID NO: 4228 - protein, 40 aa, Homo sapiens
MAWLIQCSILMLPWLEVGVPWESPCTEPSSSEPEEVSGGV

SEQ ID NO: 4229 - protein, 12 aa, Homo sapiens
MAWQRLLSSFIV

SEQ ID NO: 4230 - protein, 12 aa, Homo sapiens
MAWRPWFLVLVE

SEQ ID NO: 4231 - protein, 15 aa, Homo sapiens
MAWTYQKKKTGVKAF

SEQ ID NO: 4232 - protein, 15 aa, Homo sapiens
MAYNLIQTASFSLHY

SEQ ID NO: 4233 - protein, 11 aa, Homo sapiens
MAYSSISASFV

SEQ ID NO: 4234 - protein, 21 aa, Homo sapiens
MCAHICIYIIYIHIYILYVYI

SEQ ID NO: 4235 - protein, 26 aa, Homo sapiens
MCFLMCTKRDTTPLMRYSCQKCITSI

SEQ ID NO: 4236 - protein, 18 aa, Homo sapiens
MCFVLRNGGRFRIVLPLL

SEQ ID NO: 4237 - protein, 18 aa, Homo sapiens
MCFYCCFPLSERHLVLGH

SEQ ID NO: 4238 - protein, 20 aa, Homo sapiens
MCGRTWALPAASSPSGPCSP

SEQ ID NO: 4239 - protein, 20 aa, Homo sapiens
MCHHAHLIFCIFSSDGVLPC

SEQ ID NO: 4240 - protein, 43 aa, Homo sapiens
MCHHAQLIFCIFSRDGLLPCWPGCTLIFSVSYLDQAFLAVPCI

SEQ ID NO: 4241 - protein, 21 aa, Homo sapiens
MCHHAQLIFCIGQLILNKDAQ

SEQ ID NO: 4242 - protein, 30 aa, Homo sapiens
MCHHAQLIFVFLVEMRFHHVGQDGLDLLTS

SEQ ID NO: 4243 - protein, 45 aa, Homo sapiens
MCHHAQLIFVLLLFFFLRQNFALVAQAGVQWRNLSSLQPPPPRFK

SEQ ID NO: 4244 - protein, 56 aa, Homo sapiens
MCHHARLIFCILVETGFHHVAQVGLKLLSSSNPLASASQSARITGVSHCTRPPNLI

SEQ ID NO: 4245 - protein, 106 aa, Homo sapiens
MCHHARLIFVFLIQKGFHHISQTGLELLTLNDPLAVASQSAGIIGVSHRGQPTTFFFFWDRVSLCRQPGVQWHNLGSLQPSHPGFKRFSCLSLPSSWDYRHTTTPS

SEQ ID NO: 4246 - protein, 79 aa, Homo sapiens
MCHHARLIFVILVEMRFRHVGQTVLELLASSNLPASASQSVGITGEPLRPAMGTYFMWIKLRREKDMFFSTWKVFFKLV

SEQ ID NO: 4247 - protein, 25 aa, Homo sapiens
MCHHARLILYFLSRDRISPCWSGWS

SEQ ID NO: 4248 - protein, 27 aa, Homo sapiens
MCHHAWLCFFGRDRVLLCCQAGLKPIA

SEQ ID NO: 4249 - protein, 27 aa, Homo sapiens
MCHHAWLIFVFLVEMGFHHIVKMVSTS

SEQ ID NO: 4250 - protein, 12 aa, Homo sapiens
MCHHAWLILYFQ

SEQ ID NO: 4251 - protein, 11 aa, Homo sapiens
MCHHTLPILYF

SEQ ID NO: 4252 - protein, 24 aa, Homo sapiens
MCHHTQLILYFSGDGVSPRWSGWS

SEQ ID NO: 4253 - protein, 11 aa, Homo sapiens
MCHHTRLILYL

SEQ ID NO: 4254 - protein, 11 aa, Homo sapiens
MCHHTRLLLYF

SEQ ID NO: 4255 - protein, 75 aa, Homo sapiens [sequence omitted]

SEQ ID NO: 4256 - protein, 65 aa, Homo sapiens
MCHHTWLIFVFLVEIGFHHAGQAGHELLTSSDPPASASQRAGITGVSTDGRGPGIGGGEGGSYSL

SEQ ID NO: 4257 - protein, 52 aa, Homo sapiens [sequence omitted]

SEQ ID NO: 4258 - protein, 11 aa, Homo sapiens
MCHHTWLILYF

SEQ ID NO: 4259 - protein, 48 aa, Homo sapiens
MCHYARLTFVFLAEMGFHNVGQAGRELLTSSNRPALASQSAGITGVSH

SEQ ID NO: 4260 - protein, 14 aa, Homo sapiens
MCIIFIIRKKCVLF

SEQ ID NO: 4261 - protein, 21 aa, Homo sapiens
MCIPTYSTAMRNKEHILFFFF

SEQ ID NO: 4262 - protein, 26 aa, Homo sapiens
MCKAFAFSINCFAFDMFFEVLLAFLI

SEQ ID NO: 4263 - protein, 25 aa, Homo sapiens
MCKCARPLAMDSTIRRQLTVSRVVS

SEQ ID NO: 4264 - protein, 16 aa, Homo sapiens
MCKFCISVGYFITEQT

SEQ ID NO: 4265 - protein, 37 aa, Homo sapiens
MCKTTSYGQHYSKAANCIQSSKLKIVVQRSHFMIMCN

SEQ ID NO: 4266 - protein, 39 aa, Homo sapiens
MCLCPFMKSKVLDISEGFPTFLTFIGFLSSVNPTMDSKL

SEQ ID NO: 4267 - protein, 134 aa, Homo sapiens
MCLSAAASPCAPGCQPVPAPAVAPVGAPRGAVAPVGAPRGAVAPVGVPRGAVVLVAAPSPAVVSPVAAPQAVDHPAASPAAASPAAASPAAVSPCAASPAAASPVAASPTVVSLCAASVRSEALDPDLQVSPVW

SEQ ID NO: 4268 - protein, 31 aa, Homo sapiens
MCLSLKPLLKMKNLLKEAKINCFILREHIIE

SEQ ID NO: 4269 - protein, 13 aa, Homo sapiens
MCLSLSNQYEDIG

SEQ ID NO: 4270 - protein, 18 aa, Homo sapiens
MCNCFFFSPLSITLCFFH

SEQ ID NO: 4271 - protein, 37 aa, Homo sapiens
MCPFFYFPYPTPSLPNFSLPLCLYLCTVFCSHPLTRH

SEQ ID NO: 4272 - protein, 83 aa, Homo sapiens
MCPPPAATAGTFPPRGCALFAKPELPPSQLSGPRARERRGGAQGGSAGREAAADPGPGLVRLEPRGPWLRASPRGKGFSLSPS

SEQ ID NO: 4273 - protein, 29 aa, Homo sapiens
MCPPRPPKVLRLQARGTAPSPWFPNTASL

SEQ ID NO: 4274 - protein, 18 aa, Homo sapiens
MCPYLIEISHNSQFIRNC

SEQ ID NO: 4275 - protein, 38 aa, Homo sapiens
MCPYMGALEDTLGSKSKSNQRDGPESSPQHRARPGAPC

SEQ ID NO: 4276 - protein, 14 aa, Homo sapiens
MCQFDWAKGCPNIW

SEQ ID NO: 4277 - protein, 41 aa, Homo sapiens
MCQKYPYCFENQNNFPQALALLYQYWLKKDHLYPDEFHFQL

SEQ ID NO: 4278 - protein, 11 aa, Homo sapiens
MCRILYIPNSY

SEQ ID NO: 4279 - protein, 12 aa, Homo sapiens
MCRKRTRFTFNT

SEQ ID NO: 4280 - protein, 51 aa, Homo sapiens
MCSKLSSTKKTKSSVTIKKVVFRSIFNGSGVIDNSYIKSFFGKLFISFHFH

SEQ ID NO: 4281 - protein, 18 aa, Homo sapiens
MCSPKFRMNFSRSPTVFW

SEQ ID NO: 4282 - protein, 14 aa, Homo sapiens
MCSSWRSWISAFTA

SEQ ID NO: 4283 - protein, 27 aa, Homo sapiens
MCTPMAVVWYLASNSLLNELINEHPPN

SEQ ID NO: 4284 - protein, 15 aa, Homo sapiens
MCVCIYMCIHIHIYI

SEQ ID NO: 4285 - protein, 33 aa, Homo sapiens
MCVCVCAQLSPLTPGVTPNKNRNFAAFVFTHSF

SEQ ID NO: 4286 - protein, 18 aa, Homo sapiens
MCVGYKLLQMLYGKRKWV

SEQ ID NO: 4287 - protein, 20 aa, Homo sapiens
MCVWEVSSFLSFLLLVSVVL

SEQ ID NO: 4288 - protein, 37 aa, Homo sapiens [sequence omitted]

SEQ ID NO: 4289 - protein, 71 aa, Homo sapiens
MCYHPQLIFMFLVETGFCHVGQAGLKLLTLSDPPSLASQSVGITGMSHHARPAFSVWIFKLQPQKHESHTC

SEQ ID NO: 4290 - protein, 271 aa, Homo sapiens
MDAAVGQVVCVLLQVDVSNPLEHPLVGPHHGVNVLRLAAGPALLEGLPAEVHLVQQLDPQQDADLVELLGHVQVLLQVSLHQGIQHPPINQVVLKGLGVLGQANVIQPGLGHPVMVQLGSFGQAAACLGITVVLDGQAQLAPVQGAAHPKAQLQVLVTQAQQHLPALHVLRAGLDVHRHGHHHLQPGLDGARLPVGHRGGPHQLHLLQPVHLLLAFRQAEALPRGAALAVRVIKEAGVEGLPLLPSGEDAGDGAESHLLFLLFPFLVFKIL

SEQ ID NO: 4291 - protein, 16 aa, Homo sapiens
MDAGGVVWMICCRMLI

SEQ ID NO: 4292 - protein, 20 aa, Homo sapiens
MDCFCASSKDFTDCANSDGF

SEQ ID NO: 4293 - protein, 18 aa, Homo sapiens
MDCSVVPAQVRPVDLLGT

SEQ ID NO: 4294 - protein, 33 aa, Homo sapiens
MDCVSNSRSVLGASAGSSGVELPPPPSSMMGME

SEQ ID NO: 4295 - protein, 16 aa, Homo sapiens
MDDMLPMGSRRSAICR

SEQ ID NO: 4296 - protein, 26 aa, Homo sapiens
MDEGRLFNEKWTNDFFLLRQIAKHSA

SEQ ID NO: 4297 - protein, 37 aa, Homo sapiens
MDEIHLLYWFCIQCAGKKLPRMDVQYPHVRSHLRLLI

SEQ ID NO: 4298 - protein, 23 aa, Homo sapiens
MDEVHSSSFKNIVQGEAVGMRPR

SEQ ID NO: 4299 - protein, 42 aa, Homo sapiens
MDFHQFEVLKNFLLPPPAVVLARPPFPDASLTSRDSSWPFLS

SEQ ID NO: 4300 - protein, 13 aa, Homo sapiens
MDFIYNQKKKKLF

SEQ ID NO: 4301 - protein, 27 aa, Homo sapiens
MDFNTKKKKKKSYQAMKRHERNLNAYY

SEQ ID NO: 4302 - protein, 23 aa, Homo sapiens
MDGFQIHTLETHGASLRQLCTVS

SEQ ID NO: 4303 - protein, 85 aa, Homo sapiens
MDGSFLRSANIFLGWSSQRRVQAAIFAVSQPSLVRHPGTGKFEVTRDWSRPLGYYSSHFWRQGVQDQVFSQFDYWSGLSSWLADS

SEQ ID NO: 4304 - protein, 11 aa, Homo sapiens
MDHCKQQILYS

SEQ ID NO: 4305 - protein, 26 aa, Homo sapiens
MDHCPEGSRQRAHRREHGSDVLLLFC

SEQ ID NO: 4306 - protein, 25 aa, Homo sapiens
MDHLSCSMQEDSPTTVPVLQVLSPS

SEQ ID NO: 4307 - protein, 44 aa, Homo sapiens
MDHSLLTPFYNISKVTLSINSLFLLSAIFFHCSQSFTPQIVFFS

SEQ ID NO: 4308 - protein, 57 aa, Homo sapiens
MDISVNHAKGLDFPPEGFWERHDHADSTQDAWGFIRGSNSVHTSRVPKKFVFIVTSA

SEQ ID NO: 4309 - protein, 25 aa, Homo sapiens
MDKFIILIMMMVSPLYTEANQISPT

SEQ ID NO: 4310 - protein, 11 aa, Homo sapiens
MDKQHLKVIGE

SEQ ID NO: 4311 - protein, 36 aa, Homo sapiens
MDLASESPHLFPEVLYFFTKNFHLFAKSLFLLQLVH

SEQ ID NO: 4312 - protein, 23 aa, Homo sapiens
MDLEGSFRPFLQFRKRIYSSRIR

SEQ ID NO: 4313 - protein, 33 aa, Homo sapiens
MDLISLDKKVCLSVPKLNSISLLERLVVLVYRS

SEQ ID NO: 4314 - protein, 12 aa, Homo sapiens
MDLLSINFLICT

SEQ ID NO: 4315 - protein, 40 aa, Homo sapiens
MDLPEDPRQANSNCFLLVASAAQDLAIPTWKKLKRTYELK

SEQ ID NO: 4316 - protein, 43 aa, Homo sapiens
MDLPEIQGHPVSRFVSSSLSKTLQVGPALSASGFSLARLRSAP

SEQ ID NO: 4317 - protein, 25 aa, Homo sapiens
MDLPGPSGLSIGVLRGAQVAVRGWL

SEQ ID NO: 4318 - protein, 66 aa, Homo sapiens [sequence omitted]

SEQ ID NO: 4319 - protein, 32 aa, Homo sapiens
MDLSEEEDRSEGFLRASIFCIKYEKDFLISIV

SEQ ID NO: 4320 - protein, 16 aa, Homo sapiens
MDMDSASAGLNLDFLS

SEQ ID NO: 4321 - protein, 13 aa, Homo sapiens
MDNEPGHERKVFV

SEQ ID NO: 4322 - protein, 65 aa, Homo sapiens
MDNEPGHERKVFVPGLGLQENMALHILAGFTVCHTSFPHGILAVVPATWEADVGGSLEPRRWRLQ

SEQ ID NO: 4323 - protein, 85 aa, Homo sapiens
MDNEPGHERKVFVPGLGLQENMALHILAGFTVCHTSFPHGILDLTDQLLPEGGAPPVGLLPGNVHACSPAPAARIPLGRHRRRLS

SEQ ID NO: 4324 - protein, 67 aa, Homo sapiens
MDNEPGHERKVFVRAEAHPARQIQTLARPPLESASRKRAVSAQLGWPITGTKKQEGDREPPTATPLP

SEQ ID NO: 4325 - protein, 18 aa, Homo sapiens
MDNFLQVQMVQDLETNRG

SEQ ID NO: 4326 - protein, 15 aa, Homo sapiens
MDPLFWEEQIAMIFK

SEQ ID NO: 4327 - protein, 26 aa, Homo sapiens
MDPLLRPLPYCPMNFKVDSRFLDRPK

SEQ ID NO: 4328 - protein, 16 aa, Homo sapiens
MDPQGSCHIHHPGNTT

SEQ ID NO: 4329 - protein, 19 aa, Homo sapiens
MDQTSKSGFHSFQRGDRVG

SEQ ID NO: 4330 - protein, 15 aa, Homo sapiens
MDQTSKYGFHSSQGR

SEQ ID NO: 4331 - protein, 41 aa, Homo sapiens
MDRGRGAAVSNTMQGNLAHHMVSYIQTPLQMKTSHPWAVSR

SEQ ID NO: 4332 - protein, 50 aa, Homo sapiens
MDRSDSDCRKEADVLSSSPSPARSPPGSGSATASSSSSSGDSGVTSTAST

SEQ ID NO: 4333 - protein, 17 aa, Homo sapiens
MDRVESTDSLIILRSQI

SEQ ID NO: 4334 - protein, 12 aa, Homo sapiens
MDRVLPYWPGWS

SEQ ID NO: 4335 - protein, 14 aa, Homo sapiens
MDSASAGLNLDFLS

SEQ ID NO: 4336 - protein, 18 aa, Homo sapiens
MDSDFRGAGLLHCSRAAT

SEQ ID NO: 4337 - protein, 49 aa, Homo sapiens [sequence omitted]

SEQ ID NO: 4338 - protein, 44 aa, Homo sapiens
MDSRTVSCCMLMFKKLICSTHTFKIYCNSYSSLDIFLPLKKKSF

SEQ ID NO: 4339 - protein, 16 aa, Homo sapiens
MDSTIRRQLTVSRVVS

SEQ ID NO: 4340 - protein, 11 aa, Homo sapiens
MDTGPLPGIPT

SEQ ID NO: 4341 - protein, 22 aa, Homo sapiens
MDTLVVAHSEGEPPSRAVTTSS

SEQ ID NO: 4342 - protein, 36 aa, Homo sapiens
MDVISSIIFLSIQNIHKVLVRLYISSGINIYIYPNS

SEQ ID NO: 4343 - protein, 80 aa, Homo sapiens
MDVKEMLLSLILGWRSLMIPRKIQYVLFFLWLFLFYTFILAKHPIWLDYEHRELSFLLILSQGSFPFVLAVFLGSVKHEL

SEQ ID NO: 4344 - protein, 22 aa, Homo sapiens
MDVLIQITFRTSGVLQSGTLLP

SEQ ID NO: 4345 - protein, 16 aa, Homo sapiens
MDVQYPHVRSHLRLLI

SEQ ID NO: 4346 - protein, 12 aa, Homo sapiens
MDVSKICSYLPA

SEQ ID NO: 4347 - protein, 12 aa, Homo sapiens
MDWSSRSCSMLR

SEQ ID NO: 4348 - protein, 12 aa, Homo sapiens
MDYTSLSLLHLP

SEQ ID NO: 4349 - protein, 92 aa, Homo sapiens
MEADPNSNLHFGTYCCVTLGKSLESLCLPLEVWRHPLMQMLLEELSPSHALSCLSLNSQFLDPTGLGCTQGLRDVSTPPWMAFAAGHNCCGS

SEQ ID NO: 4350 - protein, 22 aa, Homo sapiens
MEAEAGGRRRCLCELFCFILPV

SEQ ID NO: 4351 - protein, 121 aa, Homo sapiens [sequence omitted]

SEQ ID NO: 4352 - protein, 26 aa, Homo sapiens
MECSGMISAHCNLCLLGSSDSPASAS

SEQ ID NO: 4353 - protein, 49 aa, Homo sapiens
MECSSRCIPRGSSPRAGLFQAAPSGRRGGPRTVSDADGHPRPGTDPPSG

SEQ ID NO: 4354 - protein, 21 aa, Homo sapiens
MEDVSPSCLSSPLTLSQSFSL

SEQ ID NO: 4355 - protein, 45 aa, Homo sapiens
MEEKNIYASVSESQVVVLALPFSKVYSQKQVAFLLRCRAHWNPRG

SEQ ID NO: 4356 - protein, 40 aa, Homo sapiens
MEEPDSLSLSRFWGVYAGDLLWLGEPRSCFGVEPLMSGEP

SEQ ID NO: 4357 - protein, 15 aa, Homo sapiens
MEERTKSQGIHGMQL

SEQ ID NO: 4358 - protein, 64 aa, Homo sapiens
MEFCHVGQAGLELLTPGDPPSSASQSARITGVSHPVRPVFKALISIVRKAVTMQTPLFSSQRSP

SEQ ID NO: 4359 - protein, 26 aa, Homo sapiens
MEFCSCCLGWSSVARSWLTATSASQI

SEQ ID NO: 4360 - protein, 72 aa, Homo sapiens
MEFCSVAQAGVQWRNLSSVQPPPPWFNQFSCLSLLSSWDYRHTPQCPANFFVLLVDMGFHHVGQAGLKLLTL

SEQ ID NO: 4361 - protein, 78 aa, Homo sapiens
MEFFHVGQAGLELLTSGDPAPSVSQSVGITGMSHRAQPEKNLLLETVPMLTFPTWKAKQNKTKQTNKCNKTTSHYYCA

SEQ ID NO: 4362 - protein, 16 aa, Homo sapiens
MEFHHVGQAGLELLTS

SEQ ID NO: 4363 - protein, 29 aa, Homo sapiens
MEFHHVGQAGLELPTSGDPLSLASLRFQA

SEQ ID NO: 4364 - protein, 31 aa, Homo sapiens
MEFHHVGQAGLKLLTSSDPPASASKELGLQV

SEQ ID NO: 4365 - protein, 12 aa, Homo sapiens
MEFPSCCQAGVQ

SEQ ID NO: 4366 - protein, 12 aa, Homo sapiens
MEFSAYFNMVCM

SEQ ID NO: 4367 - protein, 21 aa, Homo sapiens
MEFTFSNNTYIKTNNKQTNKP

SEQ ID NO: 4368 - protein, 57 aa, Homo sapiens
MEGASCPGEGGGEWNPYPDWETETSGGTRQQDWTKKCRPDWLPGVPEVTDLHNVSLG

SEQ ID NO: 4369 - protein, 26 aa, Homo sapiens
MEGHCIPQFYFLPQGEKGQQVSGPQG

SEQ ID NO: 4370 - protein, 64 aa, Homo sapiens
MEGNWNPHIAWWECKIVQLLSVSLAVPQKVITAPNNSIPCMCPRETKTHIHSKTYHKCLWQHYS

SEQ ID NO: 4371 - protein, 27 aa, Homo sapiens
MEGSGAISAHCNLRLQVQAILLPQPPK

SEQ ID NO: 4372 - protein, 16 aa, Homo sapiens
MEHFCSLLQKITLPPD

SEQ ID NO: 4373 - protein, 16 aa, Homo sapiens
MEHLKSPYPLPAPNHS

SEQ ID NO: 4374 - protein, 39 aa, Homo sapiens
MEHLRDMRGGNTWSYMTICHRGQERGHQGTRADRKEMWI

SEQ ID NO: 4375 - protein, 16 aa, Homo sapiens
MEIHLPLSTAPLPAPT

SEQ ID NO: 4376 - protein, 13 aa, Homo sapiens
MEIILLVTLGNTS

SEQ ID NO: 4377 - protein, 43 aa, Homo sapiens
MEIKLLRDQLELRSSTPGSRLPPTTPHWHRLKQRLVNYNQVDR

SEQ ID NO: 4378 - protein, 11 aa, Homo sapiens
MEIRPLPFTMH

SEQ ID NO: 4379 - protein, 46 aa, Homo sapiens
MEKGNGYNYVCLGAPLISLSLSLSLSLSHTHTHTHTHTHTHTHNGI

SEQ ID NO: 4380 - protein, 25 aa, Homo sapiens
MEKIMEDVSPSCLSSPLTLSQSFSL

SEQ ID NO: 4381 - protein, 29 aa, Homo sapiens
MEKKGHVRTQREGGHLQAKERGLRRDETC

SEQ ID NO: 4382 - protein, 50 aa, Homo sapiens
MEKQKVNLYRLDSGVSHSFLLNSEPTFKILKVFGNVFLDIVTASNLCVVL

SEQ ID NO: 4383 - protein, 146 aa, Homo sapiens
MEKRGSGLGSNEGQRKGPKEKTRGLLRLCQAARPRTPWLPTLPQEKAFCPCLCPVPWADLRDQGWVGCVAPDRLLSQGTGCPLLPKGPQQRLGPGGSCANPSLISQEPLDGRKSECSLQARVGTGWGWGPSSEPPPGPPQPGHSSR

SEQ ID NO: 4384 - protein, 18 aa, Homo sapiens
MEKVSVCFLDTTLKFTTW

SEQ ID NO: 4385 - protein, 19 aa, Homo sapiens
MEKYAEILSSSFSELMWQN

SEQ ID NO: 4386 - protein, 26 aa, Homo sapiens
MEKYRQDMAGIATKASFRKFIVFDYG

SEQ ID NO: 4387 - protein, 18 aa, Homo sapiens
MELILWTSCVGGLLYFLS

SEQ ID NO: 4388 - protein, 40 aa, Homo sapiens
MELILWTSLGMRRARRLDSSSLVVLRLSSLRLEGEDGRLS

SEQ ID NO: 4389 - protein, 163 aa, Homo sapiens
MELKFKLPAGQALLSFIPGTALPLVCSRALSSEGPRKRQPSPTLGSSSLLMFLSHFIFQISEGSLKRRDLALILPVLTGTPCGWQPLESRWLSPSRATWNWPLSQAYCSISVQHQPRIHKNMNRAWVTCFEFATLPHCDEHHKKCISTYQSTMVLVLTWMIQL

SEQ ID NO: 4390 - protein, 35 aa, Homo sapiens
MELPEEGAGCHFCCFTTFTGETSRDWKIRGNQGLE

SEQ ID NO: 4391 - protein, 37 aa, Homo sapiens
MELTFKNSNAICWIHWYKTGPCHSKTVMVCQYSKNWI

SEQ ID NO: 4392 - protein, 35 aa, Homo sapiens
MEMGIFRVTCCIKNCPCPCPLGPLSSHFRDPGKPR

SEQ ID NO: 4393 - protein, 16 aa, Homo sapiens
MENFENFTEKIVLKIF

SEQ ID NO: 4394 - protein, 32 aa, Homo sapiens
MENIDIMCFLMCTKRDTTPLMRYSCQKCITSI

SEQ ID NO: 4395 - protein, 104 aa, Homo sapiens [sequence omitted]

SEQ ID NO: 4396 - protein, 121 aa, Homo sapiens
MENLQRPVHDHLQVDTALRAPPAQLLAVDPRIHKQNAILQIYLQKVPVSFGRHPEQARHQLRQLQPQVLSDAAHEGAVFGLLVDGVVELAAPHLPGCKEQKREQQTLGSRASWSDNHHCRK

SEQ ID NO: 4397 - protein, 52 aa, Homo sapiens [sequence omitted]

SEQ ID NO: 4398 - protein, 25 aa, Homo sapiens
MEPDSMDCFCASSKDFTDCANSDGF

SEQ ID NO: 4399 - protein, 15 aa, Homo sapiens
MEPFPCRLPLHQWPM

SEQ ID NO: 4400 - protein, 50 aa, Homo sapiens
MEPNMNYYPGLSLIKHFINMQVCLGISCLFHRCCTLFLYRYHPVLITVAT

SEQ ID NO: 4401 - protein, 125 aa, Homo sapiens [sequence omitted]

SEQ ID NO: 4402 - protein, 25 aa, Homo sapiens
MEPSCSCPSTQPCSAAFWKYLRARS

SEQ ID NO: 4403 - protein, 23 aa, Homo sapiens
MEQFDFNCLGTKTTRAALKINIC

SEQ ID NO: 4404 - protein, 60 aa, Homo sapiens
MEQNPIHAIKKGKKTEDRSYTALNTACYALRGSRVDAGWAWRQEGPQQGQGRQEAAFPSL

SEQ ID NO: 4405 - protein, 13 aa, Homo sapiens
MEQRDMHLKPSVK

SEQ ID NO: 4406 - protein, 23 aa, Homo sapiens
MEQRIYILSIRGPLSLMSMSNNV

SEQ ID NO: 4407 - protein, 29 aa, Homo sapiens
MERGLPSQNWVHVQAQSLLVVPGPQFPFQ

SEQ ID NO: 4408 - protein, 17 aa, Homo sapiens
MERKIIGSHYNCLYLGK

SEQ ID NO: 4409 - protein, 96 aa, Homo sapiens
MERSSKKMTDLRQNHSQYHTEWVNLEAFPLKAGTRQGCPLSPLLFKIVLKVLARAIRQEKEIKGIQIGKQEVKLSLFADDMNCIYREPHHLSPKSP

SEQ ID NO: 4410 - protein, 37 aa, Homo sapiens
MESCSAAQAGVQWHDLGSLQPPPPGFKQFSCLRLPNS

SEQ ID NO: 4411 - protein, 11 aa, Homo sapiens
MESHSLTQAGM

SEQ ID NO: 4412 - protein, 36 aa, Homo sapiens
MESMQTLSMLWASSKTTTALRASSLDTRSAILGSRR

SEQ ID NO: 4413 - protein, 120 aa, Homo sapiens [sequence omitted]

SEQ ID NO: 4414 - protein, 27 aa, Homo sapiens
METHIKYFDNSSSLLKSLHQFWISQVL

SEQ ID NO: 4415 - protein, 85 aa, Homo sapiens [sequence omitted]

SEQ ID NO: 4416 - protein, 33 aa, Homo sapiens
METSSYLRRDRTAGLPTQHLQLSLLSMRQRALS

SEQ ID NO: 4417 - protein, 37 aa, Homo sapiens
METSSYLRRDRTAGLPTQHLQLSLLSMRQRALSLQDS

SEQ ID NO: 4418 - protein, 41 aa, Homo sapiens
METSSYLRRDRTAGLPTQHLQLSLLSMRQRALSLQDSRKSI

SEQ ID NO: 4419 - protein, 18 aa, Homo sapiens
METYSSVIFLIVDIAIVQ

SEQ ID NO: 4420 - protein, 21 aa, Homo sapiens
MEVGKDYCNGRKSFTQTHIIS

SEQ ID NO: 4421 - protein, 12 aa, Homo sapiens
MEVHSDNTVPVS

SEQ ID NO: 4422 - protein, 12 aa, Homo sapiens
MEVKWPYPNRWK

SEQ ID NO: 4423 - protein, 29 aa, Homo sapiens
MEVNTSTLNCTNPCIIFLVLLSLKSVELD

SEQ ID NO: 4424 - protein, 14 aa, Homo sapiens
MEVSVSENSNNAQS

SEQ ID NO: 4425 - protein, 21 aa, Homo sapiens
MEYYHFIEKQYEITLRNENSH

SEQ ID NO: 4426 - protein, 23 aa, Homo sapiens
MFAFLVETGFHHVGQDGLDLLTS

SEQ ID NO: 4427 - protein, 15 aa, Homo sapiens
MFAKPPQGWVASASV

SEQ ID NO: 4428 - protein, 14 aa, Homo sapiens
MFALASILAEFMLL

SEQ ID NO: 4429 - protein, 87 aa, Homo sapiens
MFANTATSLLDSSLSLLDILEMLISLITYCLPSSVDLTRMAFPNEPSPIFCSLTYFSMILFLRHLYRYARHLKNSVTQDVSRNNGDD

SEQ ID NO: 4430 - protein, 103 aa, Homo sapiens
MFAQEAEPSVVGKASSRWRETLPGLSAPLTTVRVSLITWVALPLPAAEPAPPGASRRVRRCQTGLIVPASCPFLLQTCEGAGVIFIWGHWRGRYLLTSSGKRS

SEQ ID NO: 4431 - protein, 15 aa, Homo sapiens
MFATQEAQVMPVTCM

SEQ ID NO: 4432 - protein, 24 aa, Homo sapiens
MFCIFSTDGVSPCWPGWSQTPDLK

SEQ ID NO: 4433 - protein, 39 aa, Homo sapiens
MFCIVIDPDAASFPTNPNALYPNCSYNKDPPSLAVFKRR

SEQ ID NO: 4434 - protein, 30 aa, Homo sapiens
MFCLFSPYSKIQSCQSRQTSNCFSPLETFH

SEQ ID NO: 4435 - protein, 24 aa, Homo sapiens
MFCLLCILNLFQGSRPFFLSKTLS

SEQ ID NO: 4436 - protein, 53 aa, Homo sapiens
MFCLSYLFDMASSVASLSSAQLSDFSILASPTLRLSFPFLFFSIFTFFSEFPL

SEQ ID NO: 4437 - protein, 25 aa, Homo sapiens
MFCNPNTLGGRGRQITRPGDRDHPD

SEQ ID NO: 4438 - protein, 19 aa, Homo sapiens
MFCPPITISPLGFGLSLIV

SEQ ID NO: 4439 - protein, 14 aa, Homo sapiens
MFCTQSPSYQHVPS

SEQ ID NO: 4440 - protein, 61 aa, Homo sapiens
MFCVSQRARRSWRASLLKFTWYSSSIPSRMLTWWNFLDTFRCFSRSRFIREFSIRPSTRWF

SEQ ID NO: 4441 - protein, 53 aa, Homo sapiens
MFFGYCFQLLVPLNSLLLLKFFHFLQSLLFSFSFKLCLLFFCLPFLTFLLLGL

SEQ ID NO: 4442 - protein, 29 aa, Homo sapiens
MFFINVLGLGLRRWNQIIIMKFCLSGSLT

SEQ ID NO: 4443 - protein, 13 aa, Homo sapiens
MFFLFPFGDDNYT

SEQ ID NO: 4444 - protein, 106 aa, Homo sapiens
MFFSPSKASFSFSTIFTLFNFSPLCSFNISTLRHKTLIGSFSRPQPIISSKYSSIPSSCSVWPFGFIIAICSTSPCKIKNLLWSKSIPWLRRRFPTSLNVFFFPLM

SEQ ID NO: 4445 - protein, 21 aa, Homo sapiens
MFGRDRVSPCWSGWSRTPDLR

SEQ ID NO: 4446 - protein, 33 aa, Homo sapiens
MFGWGIVSKSNVCASILSGDNSSKGQTAGHKGS

SEQ ID NO: 4447 - protein, 25 aa, Homo sapiens
MFHLGNKYLDSKDSKTFQHYKKTVI

SEQ ID NO: 4448 - protein, 15 aa, Homo sapiens
MFHPPWPPKVLGLQA

SEQ ID NO: 4449 - protein, 64 aa, Homo sapiens
MFIKQSRRAGFAGGVTCKALPGAFIVTERSHAFGKPGRIRIAWLVLSHTLLLAIEGHFASLKCG

SEQ ID NO: 4450 - protein, 32 aa, Homo sapiens
MFIKYFGFIIIFLLSILFLYSSCSYTPLVSLH

SEQ ID NO: 4451 - protein, 98 aa, Homo sapiens [sequence omitted]

SEQ ID NO: 4452 - protein, 19 aa, Homo sapiens
MFKAPQISRTEAKCHQSLC

SEQ ID NO: 4453 - protein, 33 aa, Homo sapiens
MFKKLICSTHTFKIYCNSYSSLDIFLPLKKKSF

SEQ ID NO: 4454 - protein, 13 aa, Homo sapiens
MFKNKNSLVLDCM

SEQ ID NO: 4455 - protein, 131 aa, Homo sapiens
MFLALNSYRIRRMAATISTLLLGLGTSRLPTYLASKQMPCWKASSLCKGIRRSCPSSTRLYLVLLGMVTRGGPAPSEAAAAGRGWRDPGEGRLELGAATRGGAWERWAGGALAARRPDPERCRGPSGSGLS

SEQ ID NO: 4456 - protein, 15 aa, Homo sapiens
MFLCAVFWKWSDTIV

SEQ ID NO: 4457 - protein, 48 aa, Homo sapiens
MFLCSRATRVAHFRASLFRLCSSVVPVSDSNCRLVSLSQGWNWKGWGL

SEQ ID NO: 4458 - protein, 63 aa, Homo sapiens
MFLETRFWRFALDRQGRARSTGLSGGPSRGPGRRTGGLPGAPHAPLTHWPRRLRCHGDRARTY

SEQ ID NO: 4459 - protein, 24 aa, Homo sapiens
MFLFFIMVPIISIRINNTCKSPTI

SEQ ID NO: 4460 - protein, 15 aa, Homo sapiens
MFLHLLFIILCVSFA

SEQ ID NO: 4461 - protein, 12 aa, Homo sapiens
MFLKILLFFNCD

SEQ ID NO: 4462 - protein, 22 aa, Homo sapiens
MFLKLSCRASKRQMVVCENTLP

SEQ ID NO: 4463 - protein, 39 aa, Homo sapiens
MFLLFKASLVDFVNRVRASGKLKSGGVGDIFSAARARHC

SEQ ID NO: 4464 - protein, 14 aa, Homo sapiens
MFLLNQRASPKPRR

SEQ ID NO: 4465 - protein, 25 aa, Homo sapiens
MFLMFTSVFMLLFFVTTVLILRLVF

SEQ ID NO: 4466 - protein, 27 aa, Homo sapiens
MFLNTTHYSNSGFQHYSEIEYFIIQEL

SEQ ID NO: 4467 - protein, 18 aa, Homo sapiens
MFLQLCNELAKLLVRWIQ

SEQ ID NO: 4468 - protein, 16 aa, Homo sapiens
MFLRNGRAAPCSQKPF

SEQ ID NO: 4469 - protein, 12 aa, Homo sapiens
MFLSKEVIQRRS

SEQ ID NO: 4470 - protein, 25 aa, Homo sapiens
MFLTLHLCQGKYIANSTILLIILIL

SEQ ID NO: 4471 - protein, 62 aa, Homo sapiens
MFLVETGFCHVGQAGLKLLTLSDPPSLASQSVGITGMSHHARPAFSVWIFKLQPQKHESHTC

SEQ ID NO: 4472 - protein, 27 aa, Homo sapiens
MFMFLMFTSVFMLLFFVTTVLILRLVF

SEQ ID NO: 4473 - protein, 37 aa, Homo sapiens
MFMTNYLELYRLHGSSIPVVNLYKSGHLHTSLIRTTA

SEQ ID NO: 4474 - protein, 13 aa, Homo sapiens
MFNFNLRTSDMVR

SEQ ID NO: 4475 - protein, 22 aa, Homo sapiens
MFNFNLRTSDMVRMLTVHRTLQ

SEQ ID NO: 4476 - protein, 24 aa, Homo sapiens
MFNFNLRTSDMVRMLTVHRTLQLT

SEQ ID NO: 4477 - protein, 25 aa, Homo sapiens
MFNFNLRTSDMVRMLTVHRTLQLTM

SEQ ID NO: 4478 - protein, 27 aa, Homo sapiens
MFNFNLRTSDMVRMLTVHRTLQLTMRM

SEQ ID NO: 4479 - protein, 22 aa, Homo sapiens
MFQAMYLYSRSTMEYMPMSLLL

SEQ ID NO: 4480 - protein, 71 aa, Homo sapiens
MFQEDENHLAQSFRHHSAGNSPLCIHKTIPSCRQHLTTDTGNSWEVPYIAPETLWCHAHPPEATQIKRMGL

SEQ ID NO: 4481 - protein, 15 aa, Homo sapiens
MFQVSKCIRRPVLLP

SEQ ID NO: 4482 - protein, 31 aa, Homo sapiens
MFRIGITEVHSSTGSSFWEWEHVAVCNSFFA

SEQ ID NO: 4483 - protein, 18 aa, Homo sapiens
MFRLNIADKSKIITYKNI

SEQ ID NO: 4484 - protein, 46 aa, Homo sapiens
MFRRDGVSPCCPGWSQTPGLEQSTCLSLPKCWDYRCEPLHLASLKS

SEQ ID NO: 4485 - protein, 48 aa, Homo sapiens
MFRTRRRWSSAHCEIRATTLGSIPSLSADGEPVAAGCPAMFPASCERP

SEQ ID NO: 4486 - protein, 72 aa, Homo sapiens [sequence omitted]

SEQ ID NO: 4487 - protein, 21 aa, Homo sapiens
MFSAHCNLHLPGSSDSLASAS

SEQ ID NO: 4488 - protein, 27 aa, Homo sapiens
MFSIIKKFAVNVIVFRSLHTSMIIFFW

SEQ ID NO: 4489 - protein, 22 aa, Homo sapiens
MFSISSWALFCRMSMLESREEK

SEQ ID NO: 4490 - protein, 70 aa, Homo sapiens
MFSNPRCLCPSSGHHYFSSGSNSPPRLLASRLAYLQNVFQVADRGIFLKCNADQLTLLFQPFDGFTFLSG

SEQ ID NO: 4491 - protein, 52 aa, Homo sapiens
MFSSCSESMGSSFFSHSTSAAGTPSGGRQCSTIMPSMGTSLPCGSCSKFFRK

SEQ ID NO: 4492 - protein, 15 aa, Homo sapiens
MFSSMVSIVCWTQRS

SEQ ID NO: 4493 - protein, 16 aa, Homo sapiens
MFSWALRSCPTWHITI

SEQ ID NO: 4494 - protein, 36 aa, Homo sapiens
MFSWLSEEYGGAIDESKETWVPVPALLLTGCVTLGN

SEQ ID NO: 4495 - protein, 41 aa, Homo sapiens
MFTDKYFKLLHEHLIHLSVYVWGQTFTAGTQFVPLSSSLCW

SEQ ID NO: 4496 - protein, 77 aa, Homo sapiens [sequence omitted]

SEQ ID NO: 4497 - protein, 14 aa, Homo sapiens
MFTLNISYIHFMTL

SEQ ID NO: 4498 - protein, 22 aa, Homo sapiens
MFTSVFMLLFFVTTVLILRLVF

SEQ ID NO: 4499 - protein, 50 aa, Homo sapiens
MFTWTNGCTNSEYTLSARCATLSARCALVTKLGHMGCVQRWECKLRSFPV

SEQ ID NO: 4500 - protein, 89 aa, Homo sapiens
MFVCLCLCVSVSVYVMVRLCGKKRVCVIVCMCVFLCVSVCVMVCLCGGEGMCVIVCLCVCLCMSVCVCVCNGVSLWQGGAVCVFLCMCV

SEQ ID NO: 4501 - protein, 65 aa, Homo sapiens
MFVFGHQVIPDNKEDGSHGDHKKRKGSVKVQHTGRNHHNQITLFVASPHHHPPCVLCFLENPAQL

SEQ ID NO: 4502 - protein, 68 aa, Homo sapiens
MFVFLVETGFYHVGQAGLKVLTSSDLPALASQSAGITGVSHDAWPRALLFLPQCSLGFCPPSCLDLCI

SEQ ID NO: 4503 - protein, 18 aa, Homo sapiens
MFVNAWITKGNSYFTMKR

SEQ ID NO: 4504 - protein, 27 aa, Homo sapiens
MFVRLVLNSRPQVIHPPRPPKVLGLQE

SEQ ID NO: 4505 - protein, 17 aa, Homo sapiens
MFVSPKQMSRECGSPRH

SEQ ID NO: 4506 - protein, 33 aa, Homo sapiens
MFVWFLDIGLAYFQPFYNFPAVSFLPTVPLGGC

SEQ ID NO: 4507 - protein, 11 aa, Homo sapiens
MFWALVCGSEF

SEQ ID NO: 4508 - protein, 12 aa, Homo sapiens
MFYAFLENDCNA

SEQ ID NO: 4509 - protein, 21 aa, Homo sapiens
MFYALQLWLYSKLQRFHILLL

SEQ ID NO: 4510 - protein, 24 aa, Homo sapiens
MFYRIPCRSTVHILLESFLDIYYY

SEQ ID NO: 4511 - protein, 40 aa, Homo sapiens
MGAGSKGFGMNCAVASVNSSTALAGISTRVKIKACSSSPS

SEQ ID NO: 4512 - protein, 34 aa, Homo sapiens
MGALEDTLGSKSKSNQRDGPESSPQHRARPGAPC

SEQ ID NO: 4513 - protein, 21 aa, Homo sapiens
MGAPSRKNALGQGRVGESDAS

SEQ ID NO: 4514 - protein, 13 aa, Homo sapiens
MGARASNLALECW

SEQ ID NO: 4515 - protein, 16 aa, Homo sapiens
MGCHQVGQDGLDLLTS

SEQ ID NO: 4516 - protein, 27 aa, Homo sapiens
MGCICKCLISIYIVKILMASPSNPDTL

SEQ ID NO: 4517 - protein, 48 aa, Homo sapiens
MGCKSLNIHGISSRFTHLQTRVQALALTHKGCATLHIHRVCHFGIQAV

SEQ ID NO: 4518 - protein, 18 aa, Homo sapiens
MGCSCKRSIRMSKLTFFF

SEQ ID NO: 4519 - protein, 103 aa, Homo sapiens
MGCWAPYIFTKNSSRRSLLREGCDESRPMSSSSLVNSLRCRFMLAGDAGCLDVLDLWFFPSVNFCFCLGFGERGMQHCNQPLCRRASLSSERSCSEVSHCRSF

SEQ ID NO: 4520 - protein, 71 aa, Homo sapiens
MGCWAPYIFTKNSSRRSLLREGCDESRPMSSSSLVNSLRCRFMLALCLSRLRREGNAALQPATVQTCISFK

SEQ ID NO: 4521 - protein, 58 aa, Homo sapiens
MGDLGTCFSVILFSYYQYDKLFYRICCHGRLRTSVSKSKSQSCLSDEIVSPSFQAQAL

SEQ ID NO: 4522 - protein, 64 aa, Homo sapiens
MGEHLSISFFNPYKCCRISSIRATVRMILLGKLMKRFPDFICRASFLHVQQSIIFSDLLFGFMG

SEQ ID NO: 4523 - protein, 13 aa, Homo sapiens
MGFAMLVRLVSNS

SEQ ID NO: 4524 - protein, 15 aa, Homo sapiens
MGFCHVGQAGLKLLT

SEQ ID NO: 4525 - protein, 54 aa, Homo sapiens
MGFCHVSQAGLELLTSGDLPALVSQSAGITGVNHRAGPLLFFSDGVSLCWGTVA

SEQ ID NO: 4526 - protein, 24 aa, Homo sapiens
MGFHCVAQAGLELLTSNNPPVSAS

SEQ ID NO: 4527 - protein, 38 aa, Homo sapiens
MGFHHAGQAGLEFLTSNDSPASASQSAGITGVSHRTQS

SEQ ID NO: 4528 - protein, 36 aa, Homo sapiens
MGFHHAGQAGLELLTSSDPSTSTSQSARITGVSHHT

SEQ ID NO: 4529 - protein, 16 aa, Homo sapiens
MGFHHDSQDGLDLLTS

SEQ ID NO: 4530 - protein, 16 aa, Homo sapiens
MGFHHIGQAGLELLTL

SEQ ID NO: 4531 - protein, 64 aa, Homo sapiens
MGFHHIGQAGLELLTLADPPALASQSAGIIGVSHCPWPNSAYKRLKTRKPLTFNINMHILHTIC

SEQ ID NO: 4532 - protein, 21 aa, Homo sapiens
MGFHHIGQAGLELLTSRDPPT

SEQ ID NO: 4533 - protein, 43 aa, Homo sapiens
MGFHHIGQSGLKLLTSSDSPISVSRSAGITGVSHCARHGPVFK

SEQ ID NO: 4534 - protein, 13 aa, Homo sapiens
MGFHHIVKMVSTS

SEQ ID NO: 4535 - protein, 44 aa, Homo sapiens
MGFHHVARGGLELLNSGDTPTSAPQSAGINRREPPQPALVIFSK

SEQ ID NO: 4536 - protein, 61 aa, Homo sapiens
MGFHHVCQAGLELLTSGDLPALASHSAGITDMSHAPSLIFVFLVETGFHHVGQDGLDILTS

SEQ ID NO: 4537 - protein, 24 aa, Homo sapiens
MGFHHVCQTGFKHLTSGDLPALAS

SEQ ID NO: 4538 - protein, 37 aa, Homo sapiens
MGFHHVGKAGFELLTSGDSPALASQSAGIIGVSHLTC

SEQ ID NO: 4539 - protein, 16 aa, Homo sapiens
MGFHHVGPDGLDLLTL

SEQ ID NO: 4540 - protein, 54 aa, Homo sapiens [sequence omitted]

SEQ ID NO: 4541 - protein, 48 aa, Homo sapiens
MGFHHVGQADLQFLTSGDLSTLAPKVLGLQEILEMSFKNRKPYCWLSS

SEQ ID NO: 4542 - protein, 60 aa, Homo sapiens
MGFHHVGQAGLELLMSSDPPTSASQSAGITGVSHRAWPVLTLKVGIQRQKRGGRLRGSWG

SEQ ID NO: 4543 - protein, 42 aa, Homo sapiens
MGFHHVGQAGLELLTSGDPPTLASQSAGITGVSHHTWPAKPL

SEQ ID NO: 4544 - protein, 49 aa, Homo sapiens
MGFHHVGQAGLELLTSGDPPTLASQSAGITGVSHRARPTSIFLNQQNAC

SEQ ID NO: 4545 - protein, 116 aa, Homo sapiens
MGFHHVGQAGLELLTSGDPPTSASQCAEITGVSHCAWPDSFNTGSSTSAHTYTVGTTFFFFLRRSLTLSPRLECSGAILAHCKLRLLGSRHSPASASRVAGTTGACHHVRLIFLYF

SEQ ID NO: 4546 - protein, 42 aa, Homo sapiens
MGFHHVGQAGLELLTSGDSPILASQSAGVTGVSHCTWPIDIF

SEQ ID NO: 4547 - protein, 38 aa, Homo sapiens
MGFHHVGQAGLELLTSSGLPASASQSAEINRRDPPCLA

SEQ ID NO: 4548 - protein, 48 aa, Homo sapiens
MGFHHVGQAGLELLTSTDLPTSASHSARITGMSQHAWPGSSFKASKPK

SEQ ID NO: 4549 - protein, 42 aa, Homo sapiens
MGFHHVGQAGLEPLTSSDLPASASQSAGTTGVSQHARQFCDS

SEQ ID NO: 4550 - protein, 16 aa, Homo sapiens
MGFHHVGQAGLKLLAS

SEQ ID NO: 4551 - protein, 63 aa, Homo sapiens
MGFHHVGQAGLKLLASSDPPASASPKCWDYRHEPPHATFTSPSCIPLTKGVLLEKSSLFSKHQ

SEQ ID NO: 4552 - protein, 49 aa, Homo sapiens
MGFHHVGQAGLKLLTSGDLLTSASQSAGITGMSHRTQPIFLSLLNGYFC

SEQ ID NO: 4553 - protein, 54 aa, Homo sapiens
MGFHHVGQAGLKLLTSGDLPASASQSAGITGVSYHAWPWPCRFLSHLPYSFFRS

SEQ ID NO: 4554 - protein, 21 aa, Homo sapiens
MGFHHVGQAGLKLLTSGDLPT

SEQ ID NO: 4555 - protein, 44 aa, Homo sapiens
MGFHHVGQAGLKLLTSGDPPASASQIAGITGVSHRTWPRISIFK

SEQ ID NO: 4556 - protein, 58 aa, Homo sapiens
MGFHHVGQAGLKLLTSGDPPDLASQSAGITGVSHCARPVSGLFYSASIEDGVTWSKCF

SEQ ID NO: 4557 - protein, 31 aa, Homo sapiens
MGFHHVGQAGLKLLTSGIYPPRPPKVLGLQA

SEQ ID NO: 4558 - protein, 60 aa, Homo sapiens
MGFHHVGQAGLKLLTSRDPPTSTSQSAGIPGMSHRTRPARAVFKRIYPGLLLCSFPKVSI

SEQ ID NO: 4559 - protein, 21 aa, Homo sapiens
MGFHHVGQAGLKTPDLVIRPP

SEQ ID NO: 4560 - protein, 43 aa, Homo sapiens
MGFHHVGQASLELLASGVPPTSVSQSAGITGVSHCAWPPCCFS

SEQ ID NO: 4561 - protein, 40 aa, Homo sapiens
MGFHHVGQASLELLTSGNPPTSASQSAGITGMSHRARPIF

SEQ ID NO: 4562 - protein, 39 aa, Homo sapiens
MGFHHVGQASLELLTSSDPPASASQSAGCEPPHPANKCF

SEQ ID NO: 4563 - protein, 42 aa, Homo sapiens
MGFHHVGQAVLELLTSGDPPASASQSAGIIGMSYRAPPSHCF

SEQ ID NO: 4564 - protein, 16 aa, Homo sapiens
MGFHHVGQDGFHLLTL

SEQ ID NO: 4565 - protein, 16 aa, Homo sapiens
MGFHHVGQDGLHLLTS

SEQ ID NO: 4566 - protein, 16 aa, Homo sapiens
MGFHHVGQDGPDLLTS

SEQ ID NO: 4567 - protein, 29 aa, Homo sapiens
MGFHHVGQGGLKLPTSSDLPALASQSAVI

SEQ ID NO: 4568 - protein, 13 aa, Homo sapiens
MGFHHVGQMVSIS

SEQ ID NO: 4569 - protein, 16 aa, Homo sapiens
MGFHHVGQTGLELLTL

SEQ ID NO: 4570 - protein, 24 aa, Homo sapiens
MGFHHVGQVGLELLASSDLPALAS

SEQ ID NO: 4571 - protein, 16 aa, Homo sapiens
MGFHHVRQAGLELLTS

SEQ ID NO: 4572 - protein, 42 aa, Homo sapiens
MGFHHVSQAGLELLTSGDLPTSASQSAEITGVSHHTWPTNAF

SEQ ID NO: 4573 - protein, 53 aa, Homo sapiens
MGFHHVSQAGLKLLTPGDPPALAAQSVGIIGVSHGTQPTPPFNDESLRDEMTW

SEQ ID NO: 4574 - protein, 41 aa, Homo sapiens
MGFHHVSQDGLDLLTLGSGHLSLPKCWDYRCEPPHPSSPSY

SEQ ID NO: 4575 - protein, 66 aa, Homo sapiens
MGFHHVSQDGLDLLTSWSAHLGLPKCWDYRCEPPRPAENKIFKWVLQNSGFIIQGSRWIETQNFGN

SEQ ID NO: 4576 - protein, 25 aa, Homo sapiens
MGFHHVSQDGLDRPPRSPKVLGLQA

SEQ ID NO: 4577 - protein, 13 aa, Homo sapiens
MGFHMLARLVLNS

SEQ ID NO: 4578 - protein, 34 aa, Homo sapiens
MGFHNVGQAGRELLTSSNRPALASQSAGITGVSH

SEQ ID NO: 4579 - protein, 16 aa, Homo sapiens
MGFHRVGQAGLELLTS

SEQ ID NO: 4580 - protein, 16 aa, Homo sapiens
MGFHRVRQDGLELLTL

SEQ ID NO: 4581 - protein, 16 aa, Homo sapiens
MGFHRVSHDGLDLLIS

SEQ ID NO: 4582 - protein, 16 aa, Homo sapiens
MGFHRVSQDGLDLLNL

SEQ ID NO: 4583 - protein, 21 aa, Homo sapiens
MGFHRVSQIGLELLTSGDPPA

SEQ ID NO: 4584 - protein, 57 aa, Homo sapiens
MGFHYVAQAGLELLTSGDLPASASQSAEITGMSHRAWPPKEFSKMVILPLRQTVMGT

SEQ ID NO: 4585 - protein, 45 aa, Homo sapiens
MGFHYVGQAGLELLTSGDPPALASQSVGITGVSHCTRLNKPTTRS

SEQ ID NO: 4586 - protein, 90 aa, Homo sapiens [sequence omitted]

SEQ ID NO: 4587 - protein, 16 aa, Homo sapiens
MGFHYVGQAGLKLLTS

SEQ ID NO: 4588 - protein, 27 aa, Homo sapiens
MGFLHVGQAGLELPASGDPPISASQSA

SEQ ID NO: 4589 - protein, 150 aa, Homo sapiens
MGFLHVGQAGLELPTSGDLPASAFQSAGITDVSHRAWPAQALFNNQLSPWASPDCHTQEAGLGLLLHRLLGVAKVGFFGHHFLGDSSWWLEKIYPARDAPSLGGELLRRGGGGSASRLGRKELASVSFLAVFEPLSSYSVFPCLHPHHFQ

SEQ ID NO: 4590 - protein, 99 aa, Homo sapiens
MGFLHVGQAGLELPTSGDLPASAFQSAGITDVSHRAWPAQALFNNQLSPWASPDCHTQEAGLGLLLHRLLGVAKVGFFGHHFLGDSSWWLFLSWLSSNL

SEQ ID NO: 4591 - protein, 64 aa, Homo sapiens
MGFLHVGQAGLELPTSGDPPASASQSAGITGVSHCARPFYKTHSPQTSEIDYSLLRGIPSNFTK

SEQ ID NO: 4592 - protein, 96 aa, Homo sapiens
MGFLHVGQAGLELPTSGNPPASASQSIRITGVSYCSRPFLSLETGSLSVTLTGVQWHDHDSLQLRPPGFKRSSHLSVLSIWDHHASLIFVFFFFFL

SEQ ID NO: 4593 - protein, 44 aa, Homo sapiens
MGFLHVGQAGLGLLTSGDPPTLASQSVGITGVSHHARPNFFSNG

SEQ ID NO: 4594 - protein, 50 aa, Homo sapiens
MGFLHVGQASLDLLTSGDPPTLASQSAGITGVSHRNQANYNFGCDCSFVL

SEQ ID NO: 4595 - protein, 40 aa, Homo sapiens
MGFLHVGQTGLELQPQVTHPPWPPKVLGFISMSHHAQPVM

SEQ ID NO: 4596 - protein, 39 aa, Homo sapiens
MGFLYVGQAGLKLPTSGDLPTSASQSAGITGVSHCTWPR

SEQ ID NO: 4597 - protein, 16 aa, Homo sapiens
MGFPHVGQAGLKLLTS

SEQ ID NO: 4598 - protein, 47 aa, Homo sapiens
MGFQHVSQAGLELLISGDPPISASQSAGITGVSHCAQPQYVLKGVWD

SEQ ID NO: 4599 - protein, 38 aa, Homo sapiens
MGFQPFAQAALELLTSGDPPTLASQSAGITGMSHCAWP

SEQ ID NO: 4600 - protein, 38 aa, Homo sapiens
MGFRHVGQAGLELLTSGDSPTSTSQNAGITGMSHHAGP

SEQ ID NO: 4601 - protein, 88 aa, Homo sapiens
MGFRHVGQAGLKLLTSSDPLALASQSAGITDVSHCAWPLLYFFRGPWKRTLRDTAEAHDPHLPWVLGILNINQKNTFKMSRKVKKKNQ

SEQ ID NO: 4602 - protein, 28 aa, Homo sapiens
MGFRHVSHAGLELLTSGDPPTSASKHVL

SEQ ID NO: 4603 - protein, 13 aa, Homo sapiens
MGFSMLARLFLNS

SEQ ID NO: 4604 - protein, 11 aa, Homo sapiens
MGFSPCWSGWS

SEQ ID NO: 4605 - protein, 31 aa, Homo sapiens
MGFSPCWSGWSRTPDLVICLPQPPKVLGLQA

SEQ ID NO: 4606 - protein, 16 aa, Homo sapiens
MGFTMLARLVLNSDLK

SEQ ID NO: 4607 - protein, 43 aa, Homo sapiens
MGFWFYTTPLARDKNLEASFLPSRLDSPLLCCFLQTDHSGICQ

SEQ ID NO: 4608 - protein, 38 aa, Homo sapiens
MGFYCVGQAGLKLLTSGDPPALASPSAGIIGMNHRGQP

SEQ ID NO: 4609 - protein, 16 aa, Homo sapiens
MGFYHIGQAGIELLTS

SEQ ID NO: 4610 - protein, 46 aa, Homo sapiens
MGFYHVDQAGLELLTSGDPPASAFQSAGITGMSHCAWPILFIFIII

SEQ ID NO: 4611 - protein, 50 aa, Homo sapiens
MGFYHVGQAGLEFLTSGYPPGSASQSVEITGMSHRARPWLFSYALWRPAS

SEQ ID NO: 4612 - protein, 16 aa, Homo sapiens
MGFYHVGQASLKLLAL

SEQ ID NO: 4613 - protein, 11 aa, Homo sapiens
MGFYHVGQAVH

SEQ ID NO: 4614 - protein, 16 aa, Homo sapiens
MGFYHVSQDGLNLLTL

SEQ ID NO: 4615 - protein, 41 aa, Homo sapiens
MGFYRVGQAGLEFLTSCNPPASASQSAGITGMSFCAHHFFF

SEQ ID NO: 4616 - protein, 18 aa, Homo sapiens
MGGAQVGHQLVQIFPVQS

SEQ ID NO: 4617 - protein, 60 aa, Homo sapiens
MGGGQLLREGTCRAHSWPSLRYQVLQPSLQLTAEEATVSQFKEFLGSFLHSQSLKAQTGP

SEQ ID NO: 4618 - protein, 14 aa, Homo sapiens
MGGGSGLFFPFYRL

SEQ ID NO: 4619 - protein, 13 aa, Homo sapiens
MGGLLEPRRLGLQ

SEQ ID NO: 4620 - protein, 21 aa, Homo sapiens
MGHFLWKSIQQSMSLAQQIAC

SEQ ID NO: 4621 - protein, 45 aa, Homo sapiens
MGHHTLVILVFLVEMGFHHVGQAGLKLLTSGIYPPRPPKVLGLQA

SEQ ID NO: 4622 - protein, 15 aa, Homo sapiens
MGHLQMNLPRCPSLT

SEQ ID NO: 4623 - protein, 13 aa, Homo sapiens
MGIFLGFGSDLQF

SEQ ID NO: 4624 - protein, 33 aa, Homo sapiens
MGIFRVTCCIKNCPCPCPLGPLSSHFRDPGKPR

SEQ ID NO: 4625 - protein, 11 aa, Homo sapiens
MGIIYFLLNVD

SEQ ID NO: 4626 - protein, 17 aa, Homo sapiens
MGIKFQHEICRGQTNHI

SEQ ID NO: 4627 - protein, 15 aa, Homo sapiens
MGKCLSELYKHYLLA

SEQ ID NO: 4628 - protein, 29 aa, Homo sapiens
MGKEEGLGQVARLQNLRSTRCCHLISQGN

SEQ ID NO: 4629 - protein, 18 aa, Homo sapiens
MGKGEEHVAMATVSPVTE

SEQ ID NO: 4630 - protein, 22 aa, Homo sapiens
MGKPCGGVYSGTSCRQYGHNPN

SEQ ID NO: 4631 - protein, 11 aa, Homo sapiens
MGKQSLLRLNS

SEQ ID NO: 4632 - protein, 33 aa, Homo sapiens
MGKRKGGRRRRRRHKPTAAPPDHDQTRQLAARA

SEQ ID NO: 4633 - protein, 37 aa, Homo sapiens
MGKRKGGRRRRRRHKPTAAPPDHDQTRQLAARAAFVR

SEQ ID NO: 4634 - protein, 16 aa, Homo sapiens
MGKRRGRKCTGQLLLG

SEQ ID NO: 4635 - protein, 13 aa, Homo sapiens
MGKSLRDTTTHCT

SEQ ID NO: 4636 - protein, 22 aa, Homo sapiens
MGKVVGTYSLPPPVSLSPIHYL

SEQ ID NO: 4637 - protein, 19 aa, Homo sapiens
MGKYFSAKASSLPHIFLME

SEQ ID NO: 4638 - protein, 23 aa, Homo sapiens
MGLGERLWWSWQKEVWNVTSTPL

SEQ ID NO: 4639 - protein, 30 aa, Homo sapiens [sequence omitted]

SEQ ID NO: 4640 - protein, 83 aa, Homo sapiens [sequence omitted]

SEQ ID NO: 4641 - protein, 69 aa, Homo sapiens
MGLGLEAALPFLLSGQERGLSIRRLLLKTLSPAPAPTPAAEKRSRLAPLLVGGQGKLEGGAGTKCCISL

SEQ ID NO: 4642 - protein, 19 aa, Homo sapiens
MGLGRSRGLLWPPGGPATP

SEQ ID NO: 4643 - protein, 20 aa, Homo sapiens
MGLIPSLTPAALRTSPIQSE

SEQ ID NO: 4644 - protein, 13 aa, Homo sapiens
MGLLQQILKKNYY

SEQ ID NO: 4645 - protein, 13 aa, Homo sapiens
MGLLWPPGGPATP

SEQ ID NO: 4646 - protein, 25 aa, Homo sapiens
MGLTYFILNILEYVKNNLNFPYTLY

SEQ ID NO: 4647 - protein, 44 aa, Homo sapiens
MGLWEKGTPHGVGPSPQWVQMAVGHEPGQSQPTVFPPIPAPAFL

SEQ ID NO: 4648 - protein, 53 aa, Homo sapiens
MGNGWFPLGPKYLYVQMCKTTSYGQHYSKAANCIQSSKLKIVVQRSHFMIMCN

SEQ ID NO: 4649 - protein, 59 aa, Homo sapiens
MGNNRGHEVLWMTLCLAGLFCLFKARSEILAFPTVEVSPSPCHKLTQLLHSEVLALEAP

SEQ ID NO: 4650 - protein, 17 aa, Homo sapiens
MGNSFKIKRMCINTIWR

SEQ ID NO: 4651 - protein, 12 aa, Homo sapiens
MGNTETDFTARI

SEQ ID NO: 4652 - protein, 14 aa, Homo sapiens
MGPELSSGRLWTSL

SEQ ID NO: 4653 - protein, 58 aa, Homo sapiens
MGPGKAKWWGRDQDQVFHYSKCGWLCDGPHVALFVHTCGLSLQGAVCFQEAKICLPHF

SEQ ID NO: 4654 - protein, 47 aa, Homo sapiens
MGPINFELVYLVTALVPSDTACLASSPGSSRRTAVWISRDVMVERLL

SEQ ID NO: 4655 - protein, 77 aa, Homo sapiens
MGPLSSLCKGDGRLRAFSPSQLKPFNHLCFLMSFIPFFRFPSLSVGFCLQSLRIKSSGRRVIFLGKSIFSIPLRIKL

SEQ ID NO: 4656 - protein, 13 aa, Homo sapiens
MGPSCCFISFRTL

SEQ ID NO: 4657 - protein, 25 aa, Homo sapiens
MGPVLWDEDVVHVFPGEAVKVFQFG

SEQ ID NO: 4658 - protein, 19 aa, Homo sapiens
MGQLHSSRWHLRLLSLSSL

SEQ ID NO: 4659 - protein, 41 aa, Homo sapiens
MGQLPAVHTQNRLSMDASVCPDRLSGLKCGFQQLAFLFGDS

SEQ ID NO: 4660 - protein, 17 aa, Homo sapiens
MGQSGRPPCLQPKFPPK

SEQ ID NO: 4661 - protein, 30 aa, Homo sapiens
MGRAAPKMAASLLFSDLGFLASRIPRNGTL

SEQ ID NO: 4662 - protein, 12 aa, Homo sapiens
MGREQWLTLVIP

SEQ ID NO: 4663 - protein, 13 aa, Homo sapiens
MGREQWLTLVIPA

SEQ ID NO: 4664 - protein, 78 aa, Homo sapiens
MGRGPGSLAGRLGPPRGRRTEPWAGHRLSCLPAATLEPLPGLAEAVWEACLALPPSVVCPAPTGLPGTAVKGHSLRER

SEQ ID NO: 4665 - protein, 17 aa, Homo sapiens
MGRKSKTSRYSFASVLC

SEQ ID NO: 4666 - protein, 50 aa, Homo sapiens
MGRLGCEEPLPLSSSLCPQSWRHSREGQDVHSHQAGLFLSPSLMSCPSLS

SEQ ID NO: 4667 - protein, 27 aa, Homo sapiens
MGRMGPKISSCITGSVSCTSTSTVGAM

SEQ ID NO: 4668 - protein, 36 aa, Homo sapiens
MGRSGSTSWPQSTGKLPTVGGTGALQFATVPTIPYC

SEQ ID NO: 4669 - protein, 33 aa, Homo sapiens
MGRVSRSNSAVTVICPVCGLIEKAPFSFPDPMK

SEQ ID NO: 4670 - protein, 68 aa, Homo sapiens
MGSHYIAQAGLELLASSDLPASASQSAGITGVSPCIRPKVSLSSPVVWKVCSHLSASPIGLCGWPGGC

SEQ ID NO: 4671 - protein, 31 aa, Homo sapiens
MGSIKLCIIIGNMYSSNHQMILLIRRMSPQH

SEQ ID NO: 4672 - protein, 17 aa, Homo sapiens
MGSNARPCMSLRAPELH

SEQ ID NO: 4673 - protein, 54 aa, Homo sapiens
MGSSASCLCNSAIFCSYIIFLSDTMAIKLNRISPSLYFCILFSMTGLTALIQSS

SEQ ID NO: 4674 - protein, 52 aa, Homo sapiens
MGSSASCLCNSAIFCSYIIFLSDTMAIKLNRISPSLYHFGRSRQADGLSSGV

SEQ ID NO: 4675 - protein, 44 aa, Homo sapiens
MGSSFFSHSTSAAGTPSGGRQCSTIMPSMGTSLPCGSCSKFFRK

SEQ ID NO: 4676 - protein, 55 aa, Homo sapiens
MGSSSASCLCNSAIFCSYIIFLSDTMAIKLNRISPSLYFCILFSMTGLTALIQSS

SEQ ID NO: 4677 - protein, 53 aa, Homo sapiens
MGSSSASCLCNSAIFCSYIIFLSDTMAIKLNRISPSLYHFGRSRQADGLSSGV

SEQ ID NO: 4678 - protein, 37 aa, Homo sapiens
MGSSSVTGNRIGAEVGPCHTYFFHLIPVKSARQKRLQ

SEQ ID NO: 4679 - protein, 12 aa, Homo sapiens
MGSTLPRGGDRV

SEQ ID NO: 4680 - protein, 224 aa, Homo sapiens
MGTFKTVRWGVARQAWVEERSFPSLAFLVDFVNVLFREPILLRDRIPQPLQVWGLQHERVKHLLSLPPHIQQNSLKVAFLGLLGGQRLKLLSEGRAGTLQRQPVGAAGSCRGGCPSRALQAGEVHIGDEQHGWRLQVSLWPKVGRLIAPEARQQAALDATVAGVRALDLPPELLPLVIAHLPLSSLVTEDLDLADSTVYQALSAQATVIGVNLQVQGDTLHPLL

SEQ ID NO: 4681 - protein, 84 aa, Homo sapiens
MGTSTSSPGISSIKTELLTATIVPGTNIGPFLSYSVKYFNLLQVDSKAGSHGYRFCGIILVAPSDRPVCMCSVRPVDVSPKDCN

SEQ ID NO: 4682 - protein, 23 aa, Homo sapiens
MGVAGLRSRADTAAPGTGRSSGE

SEQ ID NO: 4683 - protein, 63 aa, Homo sapiens
MGVKMSFPSFKNLHFLPIAESLLSDSDSLRDTEDSPGSGPISSCQPSPQPQPSMFPTHVLQPY

SEQ ID NO: 4684 - protein, 20 aa, Homo sapiens
MGVLDGQSPSSDKNRLWYAS

SEQ ID NO: 4685 - protein, 26 aa, Homo sapiens
MGVLDGQSPYFSEMKILSASFFPNSL

SEQ ID NO: 4686 - protein, 14 aa, Homo sapiens
MGVSFFSKLHLLVN

SEQ ID NO: 4687 - protein, 11 aa, Homo sapiens
MGVSPCCPGWS

SEQ ID NO: 4688 - protein, 17 aa, Homo sapiens
MGVSPCWSGWSRTLDLR

SEQ ID NO: 4689 - protein, 65 aa, Homo sapiens
MGVWRLRSLQTVAMMSRLPSSVNRYISRNSRKSISWRWGKAEKPTRMNSDMEVWFSPSMTATPSW

SEQ ID NO: 4690 - protein, 16 aa, Homo sapiens
MGWMYGNHIASVKKMF

SEQ ID NO: 4691 - protein, 153 aa, Homo sapiens [sequence omitted]

SEQ ID NO: 4692 - protein, 84 aa, Homo sapiens
MGWSPAETFGRQWETPQVVSHPGVKKSRDKHFPCPSHSNSWCNPLGVVLVHSWSFVWELGGKHLQFFCDVPISGRSASNAQRTG

SEQ ID NO: 4693 - protein, 53 aa, Homo sapiens
MGYGCQRDAAVPYSWMEKFDDTQKDPVCPVLSLVVPFLYLHFGQASYMAGLRT

SEQ ID NO: 4694 - protein, 76 aa, Homo sapiens
MGYPCILSFHLMSPVTSWALSVGCLGTAHGRNVSRKRRGLVFNPLLMHFITFGFSGSLMFLRDPLVQDPVISAHVW

SEQ ID NO: 4695 - protein, 53 aa, Homo sapiens
MHAHGEKRPREDTARRRPSASQGERPQKRRNLLTPCASASPICLYAGSHALYC

SEQ ID NO: 4696 - protein, 30 aa, Homo sapiens
MHCLGVVAGVEQAICLQQHREACHWPDPGV

SEQ ID NO: 4697 - protein, 45 aa, Homo sapiens
MHCLGVVAGVEQAICLQQHREACLEEMERDKRSPWNYRARASSRG

SEQ ID NO: 4698 - protein, 57 aa, Homo sapiens
MHCLGVVAGVEQAICLQQHREACLGTTGQELLPGGEVFGADHLPRQHSIAQKVVVSV

SEQ ID NO: 4699 - protein, 86 aa, Homo sapiens [sequence omitted]

SEQ ID NO: 4700 - protein, 124 aa, Homo sapiens
MHCLGVVAGVEQAICLQQHREACLGTTGQELLPGGEVFGADHLPRQHSIAQKVVVSVSFPLKLRIPARAELECGGYVPGRQRGDDKFLPQAVAWGFCKAPAAGPQEQQDEQSKRHSRRHACGYF

SEQ ID NO: 4701 - protein, 49 aa, Homo sapiens
MHCLGVVAGVEQAICLQQHREACLLPAEAPNPSACGTGMWRLRPRKAAG

SEQ ID NO: 4702 - protein, 17 aa, Homo sapiens
MHCLYFIFSINFPVFII

SEQ ID NO: 4703 - protein, 12 aa, Homo sapiens
MHCTILNDQDTF

SEQ ID NO: 4704 - protein, 15 aa, Homo sapiens
MHDSYVNKLPQVEQT

SEQ ID NO: 4705 - protein, 16 aa, Homo sapiens
MHEIVALQVFHGLADI

SEQ ID NO: 4706 - protein, 36 aa, Homo sapiens
MHFAAYHPICLAWVHSLICCQTGLSCQDVVQMSPAA

SEQ ID NO: 4707 - protein, 25 aa, Homo sapiens
MHFLLLWLQEAFSFHFVDVKSSWLG

SEQ ID NO: 4708 - protein, 17 aa, Homo sapiens
MHFSKTTVTPEYSPCLI

SEQ ID NO: 4709 - protein, 27 aa, Homo sapiens
MHGFHLQSEKKKTILKVRSPKLETAGL

SEQ ID NO: 4710 - protein, 32 aa, Homo sapiens
MHGTVYSLSLYNFLFTRKLTSKNIGKLGQDLI

SEQ ID NO: 4711 - protein, 22 aa, Homo sapiens
MHGVWLLKVNTDRLVLSLFSPL

SEQ ID NO: 4712 - protein, 60 aa, Homo sapiens
MHHHAQLIFVFLVEMGFYHVDQAGLELLTSGDPPASAFQSAGITGMSHCAWPILFIFIII

SEQ ID NO: 4713 - protein, 45 aa, Homo sapiens
MHHHARLIFIFLVEMEFHHVGQAGLKLLTSSDPPASASKELGLQV

SEQ ID NO: 4714 - protein, 30 aa, Homo sapiens
MHHHARLIFLILVETGFHHVGKDGLYLLTL

SEQ ID NO: 4715 - protein, 61 aa, Homo sapiens [sequence omitted]

SEQ ID NO: 4716 - protein, 53 aa, Homo sapiens
MHHHAWLIFVFLVETGFHHVGQAGLKLLTSSDPPASASQSAGITGVSHLTQCK

SEQ ID NO: 4717 - protein, 54 aa, Homo sapiens
MHHHAWLIFVFLVETRFHHVGQAGLKLLTSGDPPASASQNARITGASHCAQPLS

SEQ ID NO: 4718 - protein, 130 aa, Homo sapiens
MHHHSQLIFKIFCRDKVSLCCIGWSSTPAIKQSSRPGLPKCWDYGRESPHPGFIHFQKVISIHLNIALDSILCQFFKKIFQELVGEKKNMRNKDINSFCKELYKKNLFTYGGNMRAPQSLGGDQSIKTSF

SEQ ID NO: 4719 - protein, 31 aa, Homo sapiens
MHHHTGPIFFFFFFFFFVEIGSMLPRLVSNC

SEQ ID NO: 4720 - protein, 38 aa, Homo sapiens
MHHHTKLIFVFLVEMRFHHAGQAGLELLTSSDPPTTAS

SEQ ID NO: 4721 - protein, 52 aa, Homo sapiens
MHHHTQIIFVFLVETGFRHVGQAGLELLTSDDPPASVSQSAGITGVSHRTRL

SEQ ID NO: 4722 - protein, 12 aa, Homo sapiens
MHHHTWLILYFF

SEQ ID NO: 4723 - protein, 11 aa, Homo sapiens
MHHSTQLILYC

SEQ ID NO: 4724 - protein, 75 aa, Homo sapiens
MHHYAQLILYFLVETGFLHVGQAGLKLLTSGDLPTSVSQSAGIIGVSHCAWPIQWMLYSTFVANNFSRVNINDIY

SEQ ID NO: 4725 - protein, 12 aa, Homo sapiens
MHHYTQLTFLYF

SEQ ID NO: 4726 - protein, 26 aa, Homo sapiens
MHICFQRANDSKNCFRIREFGKQKEP

SEQ ID NO: 4727 - protein, 25 aa, Homo sapiens
MHIEGEYNSSHNLRENLQLAFDNRR

SEQ ID NO: 4728 - protein, 37 aa, Homo sapiens
MHIILILLLDSSCFQSAVFFQQESFVIFQTQHKFICL

SEQ ID NO: 4729 - protein, 13 aa, Homo sapiens
MHIKTLRPLEDPK

SEQ ID NO: 4730 - protein, 12 aa, Homo sapiens
MHKGSSSWKPVL

SEQ ID NO: 4731 - protein, 17 aa, Homo sapiens
MHLCIHFPIFTSKPKVV

SEQ ID NO: 4732 - protein, 90 aa, Homo sapiens
MHLENGALEGYEGGKYLELHDNMSQGPGKGAPGDQGGQKRNVDLMVSNRGTADKRVIVHLLDGHFCGLFFFFFFFEIEICSCCPGWSVVP

SEQ ID NO: 4733 - protein, 11 aa, Homo sapiens
MHLFYIFSVLA

SEQ ID NO: 4734 - protein, 11 aa, Homo sapiens
MHLIFAGTLEL

SEQ ID NO: 4735 - protein, 22 aa, Homo sapiens
MHLPWPSGVAETILLSLECTPG

SEQ ID NO: 4736 - protein, 23 aa, Homo sapiens
MHLQHSPLHLPFSAISQCFLLPL

SEQ ID NO: 4737 - protein, 17 aa, Homo sapiens
MHLTYKAMDKLKFSSTQ

SEQ ID NO: 4738 - protein, 16 aa, Homo sapiens
MHMFLLNQRASPKPRR

SEQ ID NO: 4739 - protein, 18 aa, Homo sapiens
MHNAFFHLNIYKQKRPIF

SEQ ID NO: 4740 - protein, 53 aa, Homo sapiens
MHNDTRLIFIICVNSIQTGFHYVAQAGLKLLALSNPPNPGSQSAGTTGTSHCT

SEQ ID NO: 4741 - protein, 15 aa, Homo sapiens
MHNGTKRQSPLSPVS

SEQ ID NO: 4742 - protein, 32 aa, Homo sapiens
MHNLINLYGSPHCRPCPRVPPFLCTEVAAPEV

SEQ ID NO: 4743 - protein, 53 aa, Homo sapiens
MHPPLLPCSHPLCSPSAPILSITGPLHLLFLILEHFPVGCVSSHLLLLLQVSV

SEQ ID NO: 4744 - protein, 12 aa, Homo sapiens
MHPPWPPKVLGL

SEQ ID NO: 4745 - protein, 24 aa, Homo sapiens
MHPQGLHGLVSFQGHGLQHHLLLL

SEQ ID NO: 4746 - protein, 15 aa, Homo sapiens
MHPTPGYFFLYLNLF

SEQ ID NO: 4747 - protein, 27 aa, Homo sapiens
MHPTTQQSHSWMYFLFLCNKLLPDLVA

SEQ ID NO: 4748 - protein, 14 aa, Homo sapiens
MHQHSFFLKKKNPL

SEQ ID NO: 4749 - protein, 56 aa, Homo sapiens
MHRRLCFSSLQEALSLVTRVEMPIPQVLEQALHSVVWTRQLALIIVGSGPNVSSSR

SEQ ID NO: 4750 - protein, 29 aa, Homo sapiens
MHSITPGLFCPLRLHTAFQPNTQSLKEYS

SEQ ID NO: 4751 - protein, 14 aa, Homo sapiens
MHSIVFPLRSLSSF

SEQ ID NO: 4752 - protein, 73 aa, Homo sapiens
MHSLLLRARVDTAGLQSLWSLPVTHGPDRSRPLRARGALPQTSRPKQSAAEFFPLNTKTVPRCPTALEGPGHC

SEQ ID NO: 4753 - protein, 18 aa, Homo sapiens
MHSTFCFLDFRKNKLNTI

SEQ ID NO: 4754 - protein, 24 aa, Homo sapiens
MHTCHFEKNWHHDGQSLSCEKPVL

SEQ ID NO: 4755 - protein, 23 aa, Homo sapiens
MHTRVKTHRKIRSITMATYFQSS

SEQ ID NO: 4756 - protein, 14 aa, Homo sapiens
MHTYSTLVLSSTSK

SEQ ID NO: 4757 - protein, 41 aa, Homo sapiens
MHVGGQDIHHTPHSQGLTAWSHELLLLPVRGQALAQQRQAS

SEQ ID NO: 4758 - protein, 126 aa, Homo sapiens
MHVGGQDIHHTPHSQGLTAWSHELLLLPVRGQALAQQRQASLAEAFSTLLSLPYQAVGILHHSRKSGIPAPQHILQQVPSQAGLASVHQEQVVIELLDKALRHRDLFYLHLQWQLSPGAPHLDARH

SEQ ID NO: 4759 - protein, 11 aa, Homo sapiens
MHVVLHSSIHF

SEQ ID NO: 4760 - protein, 11 aa, Homo sapiens
MHYYVSGYVFI

SEQ ID NO: 4761 - protein, 35 aa, Homo sapiens
MIACWPWWYLLRCLCSELWLKKQWRRRKEIKRRKQ

SEQ ID NO: 4762 - protein, 114 aa, Homo sapiens
MIADKQSWEGGKGGEGGAGPGDCLPACCPSVSSPAFQEGAPPRSPEAWPEGEGTRAWGLGAQAPPSEAQGAGKKGDYKSQETTKLNTKVGTAGKGRGCGGERRGPVQADCPSGA

SEQ ID NO: 4763 - protein, 13 aa, Homo sapiens
MIALNECITTLLL

SEQ ID NO: 4764 - protein, 46 aa, Homo sapiens
MIASLASQSARITGVCHCTWLQHPKVSTLPKLIYTFNALLAVFPML

SEQ ID NO: 4765 - protein, 26 aa, Homo sapiens
MICKYFLPFCKLSFHFLDGVISNNSF

SEQ ID NO: 4766 - protein, 15 aa, Homo sapiens
MICLPQPPKVLGLKA

SEQ ID NO: 4767 - protein, 15 aa, Homo sapiens
MICLPRPPKVLGLQV

SEQ ID NO: 4768 - protein, 11 aa, Homo sapiens
MICPPQPPIML

SEQ ID NO: 4769 - protein, 15 aa, Homo sapiens
MICPPQPPNLLGLQA

SEQ ID NO: 4770 - protein, 91 aa, Homo sapiens
MICPPSPPKVLGLQVSATAPSLQLLLRFCQIWDVSSHYLNALSAPFFSPLLLAPQTYKCWFFCYCPTGPQGSVNFFCQPIFALSFRSGKFY

SEQ ID NO: 4771 - protein, 15 aa, Homo sapiens
MICPPWPPKVLGLQV

SEQ ID NO: 4772 - protein, 11 aa, Homo sapiens
MICSRARAQAS

SEQ ID NO: 4773 - protein, 14 aa, Homo sapiens
MICYSKTYIFQMDN

SEQ ID NO: 4774 - protein, 16 aa, Homo sapiens
MIEKNKTKNEPKSKCG

SEQ ID NO: 4775 - protein, 15 aa, Homo sapiens
MIFLFLTLFQKGHHF

SEQ ID NO: 4776 - protein, 18 aa, Homo sapiens
MIFNFKSNYNGLNSKSFK

SEQ ID NO: 4777 - protein, 57 aa, Homo sapiens
MIFSSLGIDHCHTIQISYITSFCSKVQQLRRHDFYTEKCCVKVGWIYFFKGPVQKNG

SEQ ID NO: 4778 - protein, 26 aa, Homo sapiens
MIGLPSWLGSPCDMSAQGSWHLSQTF

SEQ ID NO: 4779 - protein, 64 aa, Homo sapiens [sequence omitted]

SEQ ID NO: 4780 - protein, 49 aa, Homo sapiens
MIHDQFFGFVPRLNVFVGCNLLILHNKRSLWLLTVFKFWLPDCFFQFQI

SEQ ID NO: 4781 - protein, 32 aa, Homo sapiens
MIHGLHQMNKTSIFDTNNVPKPNLTKLMTASQ

SEQ ID NO: 4782 - protein, 15 aa, Homo sapiens
MIHLPRLPKVLGLQE

SEQ ID NO: 4783 - protein, 15 aa, Homo sapiens
MIHLPRSPKVLGLQA

SEQ ID NO: 4784 - protein, 13 aa, Homo sapiens
MIHLPWPPKVLGL

SEQ ID NO: 4785 - protein, 22 aa, Homo sapiens
MIHLPWPPKVVGLRAWATAPGL

SEQ ID NO: 4786 - protein, 36 aa, Homo sapiens
MIHNFWEALRVKSLPWSYQSNPADRRKTCTTAKEQG

SEQ ID NO: 4787 - protein, 43 aa, Homo sapiens
MIHPAQPPKCCDYRREPLDKSFLKRGSYAFQMYLLIEKCFWRR

SEQ ID NO: 4788 - protein, 15 aa, Homo sapiens
MIHPLQPPKVLGLQA

SEQ ID NO: 4789 - protein, 15 aa, Homo sapiens
MIHPPGPPKVLGLQA

SEQ ID NO: 4790 - protein, 44 aa, Homo sapiens
MIHPPHLPKCWDYRHEPPCPAWLWNFTGIYFVITMLARYFFRVL

SEQ ID NO: 4791 - protein, 46 aa, Homo sapiens
MIHPPHMIIPPSAGITGVSHHVRPYPQKRIYQNCVCVCVCVCVCMF

SEQ ID NO: 4792 - protein, 15 aa, Homo sapiens
MIHPPLPPKVLGLQA

SEQ ID NO: 4793 - protein, 49 aa, Homo sapiens
MIHPPQPPKCWDYRHEPRHPALSRLSNERNMGERAGVVVELSLQRLRLT

SEQ ID NO: 4794 - protein, 15 aa, Homo sapiens
MIHPPQPPRVLGLQA

SEQ ID NO: 4795 - protein, 15 aa, Homo sapiens
MIHPPRPPEVLRLQA

SEQ ID NO: 4796 - protein, 15 aa, Homo sapiens
MIHPPRRPKALGLQA

SEQ ID NO: 4797 - protein, 15 aa, Homo sapiens
MIHPPWPPKVLGLQV

SEQ ID NO: 4798 - protein, 15 aa, Homo sapiens
MIHRPQPPRVLGLQA

SEQ ID NO: 4799 - protein, 13 aa, Homo sapiens
MIHRPWSPKVLEL

SEQ ID NO: 4800 - protein, 15 aa, Homo sapiens
MIHSPWTPIVLGLQT

SEQ ID NO: 4801 - protein, 14 aa, Homo sapiens
MIIHSPSKLTAYSA

SEQ ID NO: 4802 - protein, 20 aa, Homo sapiens
MIIKYIFIFFSWRNVVTLAA

SEQ ID NO: 4803 - protein, 21 aa, Homo sapiens
MIILEKLKFINSIKIKDLPIH

SEQ ID NO: 4804 - protein, 13 aa, Homo sapiens
MIINNFIQGEQNC

SEQ ID NO: 4805 - protein, 30 aa, Homo sapiens
MIIYISLHPCQNLALLNFFVNTDEAEIVSH

SEQ ID NO: 4806 - protein, 44 aa, Homo sapiens
MIKGILELLTTEFCLLNPRHYSSGPKSAVISYFGLLIFHINSSS

SEQ ID NO: 4807 - protein, 20 aa, Homo sapiens
MIKSLLFRERASLPLTSDII

SEQ ID NO: 4808 - protein, 52 aa, Homo sapiens [sequence omitted]

SEQ ID NO: 4809 - protein, 85 aa, Homo sapiens
MILAHCNLCLPGSSDPPASTSRVAGITGAHYHAQLIFVFFSRGRVSPCWPGWPQLLTSSDLPTSASQSAAITGVSHCARPICYNF

SEQ ID NO: 4810 - protein, 78 aa, Homo sapiens
MILAHCNLHLPGSSNSPASGSRIAEFTGARHHTRLIFVFLVETGFHHVGHLVSNSSGDPPTSVSLSAGDYWHEPPGPA

SEQ ID NO: 4811 - protein, 21 aa, Homo sapiens
MILEIRIKIFLSQKKLPEIKI

SEQ ID NO: 4812 - protein, 23 aa, Homo sapiens
MILFSKYFIFQGKKFDSYVFLSF

SEQ ID NO: 4813 - protein, 12 aa, Homo sapiens
MILKSSSLRDAP

SEQ ID NO: 4814 - protein, 12 aa, Homo sapiens
MILLIRRMSPQH

SEQ ID NO: 4815 - protein, 28 aa, Homo sapiens
MILLPPPPLSSPRCESHCQGQKEPLIVP

SEQ ID NO: 4816 - protein, 34 aa, Homo sapiens
MILYTGQYLDASCLPILQLLSLILLFLYWTFLRC

SEQ ID NO: 4817 - protein, 119 aa, Homo sapiens
MIMITPLHSSLGRRGRPCQEGCGGGERERDKRGRRRSWRGKRRRREKRRGRGGERKGGEGRGREGRGEEGRGREGKGGEGRGRERKGEEGEGEGKGKGRREKEGKKKKGANTGLLCTAP

SEQ ID NO: 4818 - protein, 20 aa, Homo sapiens
MIMKIHSHTHIHVHTTSMGC

SEQ ID NO: 4819 - protein, 30 aa, Homo sapiens
MIMSLAILSNEGRLPLTKTIQRLVCMMVDQ

SEQ ID NO: 4820 - protein, 12 aa, Homo sapiens
MINFRKYHVKKS

SEQ ID NO: 4821 - protein, 24 aa, Homo sapiens
MINHPHAKKNSAFHNVHSAEVGKS

SEQ ID NO: 4822 - protein, 28 aa, Homo sapiens
MINILLKCMRNILQDRPSIRPHTNSQKH

SEQ ID NO: 4823 - protein, 15 aa, Homo sapiens
MIPCENIGHSYPGYR

SEQ ID NO: 4824 - protein, 62 aa, Homo sapiens
MIPHPPHVCFLNSTATINQWVNGTPHFVLCNLKLNGHGWFLFSFIFPQCACAFELAFENRAS

SEQ ID NO: 4825 - protein, 12 aa, Homo sapiens
MIPKSSSYPSRG

SEQ ID NO: 4826 - protein, 18 aa, Homo sapiens
MIPRSPLGNVRKHPQQML

SEQ ID NO: 4827 - protein, 43 aa, Homo sapiens
MIPTTKTFSTFFTLMSFFTCSTVLIEMALSHYCAHRVGSLSTS

SEQ ID NO: 4828 - protein, 23 aa, Homo sapiens
MIQAFHLEILCFGACYNRFSVFY

SEQ ID NO: 4829 - protein, 22 aa, Homo sapiens
MIQHLGLPKCWGYRHGPPLPTQ

SEQ ID NO: 4830 - protein, 34 aa, Homo sapiens
MIQIAQDEFQSQKSNAGEYHSKVLNKHFLYCQSW

SEQ ID NO: 4831 - protein, 13 aa, Homo sapiens
MIQNKKVVNSKNL

SEQ ID NO: 4832 - protein, 38 aa, Homo sapiens
MIQRFERPYTVNKNMSISFFKAYWTIKHSEGNEGWTGR

SEQ ID NO: 4833 - protein, 29 aa, Homo sapiens
MIQRTKWGWVERKLVISLFRFSLCRADTV

SEQ ID NO: 4834 - protein, 120 aa, Homo sapiens
MIRKQSQHHGPSLSMSSKPCQALQLLSTLPSGLPVCGGQKRKTTQGECLLPPAGKQLGHHLSESRCCSSWQQSHSERSCVHCLSGRPCQSPSLPPPYLCRKPGHHHFKALPSFLGRAQPQ

SEQ ID NO: 4835 - protein, 62 aa, Homo sapiens
MIRLWSALVSMFSSCSESMGSSFFSHSTSAAGTPSGGRQCSTIMPSMGTSLPCGSCSKFFRK

SEQ ID NO: 4836 - protein, 15 aa, Homo sapiens
MIRPPRPPKALGLQV

SEQ ID NO: 4837 - protein, 15 aa, Homo sapiens
MIRPPRPPKVLGLEA

SEQ ID NO: 4838 - protein, 15 aa, Homo sapiens
MIRPPRPPKVLGLQM

SEQ ID NO: 4839 - protein, 41 aa, Homo sapiens
MIRPPRPPKVLGLRAWATTPSQGMTNFKASNVYHQMASKRL

SEQ ID NO: 4840 - protein, 17 aa, Homo sapiens
MIRVACVRPTKGHLLPH

SEQ ID NO: 4841 - protein, 34 aa, Homo sapiens
MISDLTNFKCITMFQAMYLYSRSTMEYMPMSLLL

SEQ ID NO: 4842 - protein, 17 aa, Homo sapiens
MISHCQCDHICPPFVQV

SEQ ID NO: 4843 - protein, 14 aa, Homo sapiens
MISLHKLIPPFFFL

SEQ ID NO: 4844 - protein, 36 aa, Homo sapiens
MISSRKPFSQSLVFGLIFTALPFTFIPSTSRTLRAE

SEQ ID NO: 4845 - protein, 26 aa, Homo sapiens
MISVHTQVASVLSNLCQSTNSLCEAK

SEQ ID NO: 4846 - protein, 35 aa, Homo sapiens
MITAALYSYLLQSLFFYFLSNTSYIVFYVYLPQEI

SEQ ID NO: 4847 - protein, 117 aa, Homo sapiens
MITPLHSSLGRRGRPCQEGCGGGERERDKRGRRRSWRGKRRRREKRRGRGGERKGGEGRGREGRGEEGRGREGKGGEGRGRERKGEEGEGEGKGKGRREKEGKKKKGANTGLLCTAP

SEQ ID NO: 4848 - protein, 54 aa, Homo sapiens
MITQSPCIHFMAYPAFKKPRLFLVLILNYLKNPEVLEISKNCSISEQMHRLQSM

SEQ ID NO: 4849 - protein, 14 aa, Homo sapiens
MITSIMDIASDQEL

SEQ ID NO: 4850 - protein, 44 aa, Homo sapiens
MITSSAGAVLSLLYSSIVLITVRFVSVFSSDFRTGLPPVELVLV

SEQ ID NO: 4851 - protein, 52 aa, Homo sapiens
MIVCELSLGPSQFSLLGFFGHHGVGREVGLGSHWRDPGEDSDMPPVMYHTAM

SEQ ID NO: 4852 - protein, 52 aa, Homo sapiens
MIVCKLFLGPSQFSLLGFFGHHGVGRVVGLGSHWRDPGEDSDMPPVTYHTAM

SEQ ID NO: 4853 - protein, 15 aa, Homo sapiens
MIVKGIGKNTAIVVL

SEQ ID NO: 4854 - protein, 55 aa, Homo sapiens
MIWTVAALRPAGASDRSTHGVGCGWKEIGFHCRGISVDSGTSHSAGPPPPCWRIV

SEQ ID NO: 4855 - protein, 15 aa, Homo sapiens
MIYPPWPPKVLGLQA

SEQ ID NO: 4856 - protein, 32 aa, Homo sapiens
MIYVIIEPKHNLLRGLDENSQLLRERVGNRIL

SEQ ID NO: 4857 - protein, 54 aa, Homo sapiens
MKAATSGRLPTDKPKVVHVSDALRAKGYLLKIFLQCYFFGVRTDEVNFRLANCF

SEQ ID NO: 4858 - protein, 277 aa, Homo sapiens
MKAATSGRLPTDKPKVVHVSDALRAKGYLLKIFLQCYFFGVRTDEVNFRLANREEHSSIFLDICGLHNIVSANEVVLNVALLEGAEEAAASEAPILQLLPKGQRAQAGLGEGLAHGPAHRLLAPCGRGMGRVGAGALGPPAAADVIELLDALVDQGRRSLLVRHRHAAAEEHLELLGKRVVELGRAVQLLLPGDLPRLTDGADDLRHFCLIIGFEHIADTLPVDSVFLNQTSKVTWVMTVVNQFVNTLRLALKDAGIDQGIPLLTSPWLRFTSQSRG

SEQ ID NO: 4859 - protein, 215 aa, Homo sapiens
MKAATSGRLPTDKPKVVHVSDALRAKGYLLKIFLQCYFFGVRTDEVNFRLANREEHSSIFLDICGLHNIVSANEVVLNVALLEGAEEAAASEAPILQLLPKGQRAQAGLGEGLAHGPAHRLLAPCGRGMGRVGAGALGPPAAADVIELLDALVDQGRRSLLVRHRHAAAEEHLELLGKRVVELGRAVQLLLPGDLPRLTDGADDLRHLGHPAEQW

SEQ ID NO: 4860 - protein, 24 aa, Homo sapiens
MKAELLSAHFLLQLWVTAVDSDCG

SEQ ID NO: 4861 - protein, 32 aa, Homo sapiens
MKALVTNKRSVCGPLLTSWLLPYERDKHLALF

SEQ ID NO: 4862 - protein, 63 aa, Homo sapiens
MKAQDSTLEKLSLGPNVYTLASTTFFAFIMTSKCPTGAVIPVVPKRILERGAIPLHFLPVARF

SEQ ID NO: 4863 - protein, 56 aa, Homo sapiens
MKAQDSTLEKLSLGPNVYTLASTTVARRERPRPRPHSDPAAAAAVSPARVNRHLRP

SEQ ID NO: 4864 - protein, 66 aa, Homo sapiens
MKCCFIFLPHFLSKVYAFVMNSEMIPTTKTFSTFFTLMSFFTCSTVLIEMALSHYCAHRVGSLSTS

SEQ ID NO: 4865 - protein, 16 aa, Homo sapiens
MKEDCSMKSGQMTFSC

SEQ ID NO: 4866 - protein, 31 aa, Homo sapiens
MKESAQLLSEKIAFKTSDFSRGSPNAKPKVF

SEQ ID NO: 4867 - protein, 11 aa, Homo sapiens
MKEVEHFKCFF

SEQ ID NO: 4868 - protein, 22 aa, Homo sapiens
MKEYLLYKECEYSRDLCSKSPG

SEQ ID NO: 4869 - protein, 24 aa, Homo sapiens
MKFFPLSVCCLSVNCSTCHFTAQT

SEQ ID NO: 4870 - protein, 11 aa, Homo sapiens
MKFSGFLQCQT

SEQ ID NO: 4871 - protein, 93 aa, Homo sapiens
MKFTASSLFFPVSGTQVPLQRGRWDIQGLHNLLAHCTVLLCPPSSPLHDFILPRVPDGGFLLDVDLPVHRAVISVVPPGVFIWSGHKITLLAL

SEQ ID NO: 4872 - protein, 28 aa, Homo sapiens
MKFYFLIGHFIETRIYCQLFFYSHVLCT

SEQ ID NO: 4873 - protein, 19 aa, Homo sapiens
MKGASKCVAFCIFQILIRI

SEQ ID NO: 4874 - protein, 37 aa, Homo sapiens
MKGFSKGTTIVNKIAAGISLSPSSSKFGLTYMKKRDP

SEQ ID NO: 4875 - protein, 24 aa, Homo sapiens
MKGLDLIVSKVCSVELMALLNFFG

SEQ ID NO: 4876 - protein, 28 aa, Homo sapiens
MKGMWYQALRCSQSIQGDRYQANCDTVY

SEQ ID NO: 4877 - protein, 41 aa, Homo sapiens
MKGRKKETEEGMNERKKKKKKIAFAFVFLLTLQGFLFLTAT

SEQ ID NO: 4878 - protein, 20 aa, Homo sapiens
MKHHKCQLSRFNFPEIIFHK

SEQ ID NO: 4879 - protein, 13 aa, Homo sapiens
MKHHTWPFLFIFF

SEQ ID NO: 4880 - protein, 19 aa, Homo sapiens
MKHKPPSKARSNKNLWPIS

SEQ ID NO: 4881 - protein, 17 aa, Homo sapiens
MKHNGDSRRHRSEFGWL

SEQ ID NO: 4882 - protein, 21 aa, Homo sapiens
MKHRIHHPDASQCLVPLRNPS

SEQ ID NO: 4883 - protein, 14 aa, Homo sapiens
MKHVLIQREVVLPK

SEQ ID NO: 4884 - protein, 30 aa, Homo sapiens
MKIETIFYGQGTTDTISNKTYSSAFMEHFL

SEQ ID NO: 4885 - protein, 26 aa, Homo sapiens
MKIHEDSKIPTFNSKFLRCHGLLIPQ

SEQ ID NO: 4886 - protein, 12 aa, Homo sapiens
MKIHEDSKIPTL

SEQ ID NO: 4887 - protein, 13 aa, Homo sapiens
MKIHEDSKIPTLC

SEQ ID NO: 4888 - protein, 25 aa, Homo sapiens
MKIHEDSKIPTLIFFFDNILSCHDW

SEQ ID NO: 4889 - protein, 33 aa, Homo sapiens
MKIHEDSKIPTLKLLFISKWISVLFAQIQGSFI

SEQ ID NO: 4890 - protein, 18 aa, Homo sapiens
MKIHSHTHIHVHTTSMGC

SEQ ID NO: 4891 - protein, 22 aa, Homo sapiens
MKILSRMSPLSMQCSSKHKETG

SEQ ID NO: 4892 - protein, 30 aa, Homo sapiens
MKIPCVYLLSIHHLHGIPHTNTLMRILTGD

SEQ ID NO: 4893 - protein, 12 aa, Homo sapiens
MKITAPPKNLGN

SEQ ID NO: 4894 - protein, 12 aa, Homo sapiens
MKIWKKRVHVAL

SEQ ID NO: 4895 - protein, 23 aa, Homo sapiens
MKKGKFVQQMMLEQLNTHIQIYI

SEQ ID NO: 4896 - protein, 22 aa, Homo sapiens
MKKPSRAKRVKNTLEDTLLKYL

SEQ ID NO: 4897 - protein, 35 aa, Homo sapiens
MKKPSRAKRVKNTLEDTLPREAQLPSPASKLQAYV

SEQ ID NO: 4898 - protein, 19 aa, Homo sapiens
MKKRYIFDSRKMISVNHNV

SEQ ID NO: 4899 - protein, 23 aa, Homo sapiens
MKLMQKWRVNVWQCFTEQFKRSF

SEQ ID NO: 4900 - protein, 52 aa, Homo sapiens
MKLPGLSLRCFSVPEEDDRRRKIASPSEMKARVPLLRTYNNQLPKLLVCVSY

SEQ ID NO: 4901 - protein, 35 aa, Homo sapiens
MKMDLISLDKKVCLSVPKLNSISLLERLVVLVYRS

SEQ ID NO: 4902 - protein, 37 aa, Homo sapiens
MKMRSLFTTRKFSMVFPLAKTMSPVSFTASGKISFTS

SEQ ID NO: 4903 - protein, 35 aa, Homo sapiens
MKMSLSSPNPHPLVRTDRSSHTQWSQPLGRGTCSR

SEQ ID NO: 4904 - protein, 32 aa, Homo sapiens
MKNLGHLLKIWSLQKKKRKLISWGCCRIQSNL

SEQ ID NO: 4905 - protein, 21 aa, Homo sapiens
MKNLLKEAKINCFILREHIIE

SEQ ID NO: 4906 - protein, 28 aa, Homo sapiens
MKPGRKSAKMQWWLCRYSYYVSESVQPV

SEQ ID NO: 4907 - protein, 35 aa, Homo sapiens [sequence omitted]

SEQ ID NO: 4908 - protein, 11 aa, Homo sapiens
MKPTKVLGLQT

SEQ ID NO: 4909 - protein, 24 aa, Homo sapiens
MKQVIRRLSKAADHMHQLFSIHWH

SEQ ID NO: 4910 - protein, 36 aa, Homo sapiens
MKRDEVKLLLNFRTETSINSEVRTNISYARVFLVKS

SEQ ID NO: 4911 - protein, 15 aa, Homo sapiens
MKRDSPETDWEKKAQ

SEQ ID NO: 4912 - protein, 12 aa, Homo sapiens
MKRHERNLNAYY

SEQ ID NO: 4913 - protein, 17 aa, Homo sapiens
MKRLRVKKEPKMMKMTK

SEQ ID NO: 4914 - protein, 20 aa, Homo sapiens
MKRLVRPGKGVRVPEATLEG

SEQ ID NO: 4915 - protein, 20 aa, Homo sapiens
MKRYLGNIFKIHYCLKMETL

SEQ ID NO: 4916 - protein, 69 aa, Homo sapiens
MKSAEGPSSSLAWLRKCKMRSSPWPSSRLSRSSKSWGSVMPKAAYTRSRIHSTRRSSMAPRSAEGAGRR

SEQ ID NO: 4917 - protein, 168 aa, Homo sapiens
MKSAEGPSSSLAWLRKCKMRSSPWPSSRLSRSSKSWGSVMPKAAYTRSRIHSTRRSSMAPRSAEGAGRRAGVRGNGGPSNGRPGNGRSSPRRRRRRWGLQARQCPAPGPSIPNPRAAAHAPAPGSRRRAPGPRAAEVGWLLPGPGSAHAPGCGAGPSPPGAALGPLQP

SEQ ID NO: 4918 - protein, 169 aa, Homo sapiens
MKSAEGPSSSLAWLRKCKMRSSPWPSSRLSRSSKSWGSVMPKAAYTRSRIHSTRRSSMAPRSAEGAGRRAGVRGNGGPSNGRPGNGRSSPRRRRRRWGLQARQCPAPGPSIPNPRAAAHAPAPGSRRRAPGPRAAEVGWLLPGPGSAHAPGCGAGPSPPGAALGPLQPR

SEQ ID NO: 4919 - protein, 171 aa, Homo sapiens
MKSAEGPSSSLAWLRKCKMRSSPWPSSRLSRSSKSWGSVMPKAAYTRSRIHSTRRSSMAPRSAEGAGRRAGVRGNGGPSNGRPGNGRSSPRRRRRRWGLQARQCPAPGPSIPNPRAAAHAPAPGSRRRAPGPRAAEVGWLLPGPGSAHAPGCGAGPSPPGAALGPLQPRVR

SEQ ID NO: 4920 - protein, 84 aa, Homo sapiens
MKSFLDISGPFRSSPSITAIPPRRRPHPHHCPPPRRRPHHRHPHHCHPHHCPPHHRHPHPHPDLPFCHQMCCSQTPPPPEPGAS

SEQ ID NO: 4921 - protein, 81 aa, Homo sapiens
MKSFSFGFRGKVHAGKVKPLNWTVWIVTANHLPIGDLVAQAVRGFVWVHGHVQHIRGVHGQDGVSELRPSFVLLFLWCVFL

SEQ ID NO: 4922 - protein, 24 aa, Homo sapiens
MKSFYFLHWLEEPQPLHGSAPLSH

SEQ ID NO: 4923 - protein, 185 aa, Homo sapiens [sequence omitted]

SEQ ID NO: 4924 - protein, 54 aa, Homo sapiens
MKSHCAAQAGVRWHDLGSLQPLPPGLKRSSCFDLPSSWDYRGPLPCPANFCIFQ

SEQ ID NO: 4925 - protein, 57 aa, Homo sapiens [sequence omitted]

SEQ ID NO: 4926 - protein, 11 aa, Homo sapiens
MKSHIPLQLKF

SEQ ID NO: 4927 - protein, 33 aa, Homo sapiens
MKSKVLDISEGFPTFLTFIGFLSSVNPTMDSKL

SEQ ID NO: 4928 - protein, 63 aa, Homo sapiens
MKSSAICLQNHPKDGLHLQVFNLNLYCEDSYGFPFKSRHPLTLSPNSRGAIIHTDICYRFQKC

SEQ ID NO: 4929 - protein, 23 aa, Homo sapiens
MKSSDWALSNKVFCYNLVLFSSH

SEQ ID NO: 4930 - protein, 11 aa, Homo sapiens
MKSSLWPPKHE

SEQ ID NO: 4931 - protein, 19 aa, Homo sapiens
MKTEWAAWVKVPAVFSLEY

SEQ ID NO: 4932 - protein, 11 aa, Homo sapiens
MKTFIFCTSSR

SEQ ID NO: 4933 - protein, 15 aa, Homo sapiens
MKTVEVHRDDTNCSR

SEQ ID NO: 4934 - protein, 46 aa, Homo sapiens
MKWVALQERHPELRELELIESFIIGSKHAFPLFHRHYLHIAKLFPI

SEQ ID NO: 4935 - protein, 17 aa, Homo sapiens
MKYMITSIMDIASDQEL

SEQ ID NO: 4936 - protein, 20 aa, Homo sapiens
MKYQGLGCRTLCVPSCSEPK

SEQ ID NO: 4937 - protein, 37 aa, Homo sapiens
MKYQGLGCRTLCVPSCSEPQQYPSWFCFHEVHYILYT

SEQ ID NO: 4938 - protein, 56 aa, Homo sapiens
MKYQGLGCRTLCVPSCSEPSLKFWPGIFLELFDNVKKFFCSVFTVYLVFRCLQQKS

SEQ ID NO: 4939 - protein, 28 aa, Homo sapiens
MKYQGLGCRTLCVPSCSEPVGSFHPLCV

SEQ ID NO: 4940 - protein, 24 aa, Homo sapiens
MLAAPWGEVLQSQRLYGPTWPWTT

SEQ ID NO: 4941 - protein, 73 aa, Homo sapiens [sequence omitted]

SEQ ID NO: 4942 - protein, 12 aa, Homo sapiens
MLAKLVSNSNLR

SEQ ID NO: 4943 - protein, 12 aa, Homo sapiens
MLALFLLSHTCW

SEQ ID NO: 4944 - protein, 21 aa, Homo sapiens
MLAPSCWCPSSRGHEETTSRL

SEQ ID NO: 4945 - protein, 41 aa, Homo sapiens
MLARLDLEHLTPGDPPASASQSAGITGMSHHARPGGTFLKT

SEQ ID NO: 4946 - protein, 27 aa, Homo sapiens
MLARLFSNAQPQVIHPPRPPKMLGLQM

SEQ ID NO: 4947 - protein, 40 aa, Homo sapiens
MLARLFSNSWPQAICLLQPPKVLGLQVSHCAQPWAHISCG

SEQ ID NO: 4948 - protein, 42 aa, Homo sapiens
MLARLVLASRSAGIAGMSHRTQPRKIIFVPILEVRKIGPEIK

SEQ ID NO: 4949 - protein, 12 aa, Homo sapiens
MLARLVLNSDLK

SEQ ID NO: 4950 - protein, 27 aa, Homo sapiens
MLARLVLNSQPQVIRPPQPPKVLGLQT

SEQ ID NO: 4951 - protein, 27 aa, Homo sapiens
MLARLVLNSRPQAIHLPWPPKVLGLEA

SEQ ID NO: 4952 - protein, 27 aa, Homo sapiens
MLARLVLNSSPQVICPLRPPKVLKLQA

SEQ ID NO: 4953 - protein, 81 aa, Homo sapiens
MLARLVLNSSSQVIRPPRPPKVLVLQAWATAPGLFLKISSCPIFSISPKMFRLFTFSIFYQFLQSIFLNSHISSSLSNLLV

SEQ ID NO: 4954 - protein, 27 aa, Homo sapiens
MLARLVLNSWLQVICLPWRPKVLGLQE

SEQ ID NO: 4955 - protein, 27 aa, Homo sapiens
MLARLVLNSWPQVIHPPWPPKMLGLQV

SEQ ID NO: 4956 - protein, 12 aa, Homo sapiens
MLARLVSKLLTL

SEQ ID NO: 4957 - protein, 27 aa, Homo sapiens
MLARLVSNCLLQAIRQPRPPKVLGLQA

SEQ ID NO: 4958 - protein, 42 aa, Homo sapiens
MLARLVSNCWPQVIRLPRPPQSAGITGMSHHTPPSPLLLASL

SEQ ID NO: 4959 - protein, 27 aa, Homo sapiens
MLARLVSNSCPQMFHPPWPPKVLGLQA

SEQ ID NO: 4960 - protein, 27 aa, Homo sapiens
MLARLVSNSLPQVLCLPWPPKVLGRQA

SEQ ID NO: 4961 - protein, 27 aa, Homo sapiens
MLARLVSNSRPQVICPPRPPKVLGLQA

SEQ ID NO: 4962 - protein, 27 aa, Homo sapiens
MLARLVSNSSPQMIRPPQPPKVLGLQV

SEQ ID NO: 4963 - protein, 57 aa, Homo sapiens
MLARLVSNSWPHDPPALATQSGGITGMGHCTWPLEGCIIITINYILSFIVIKIMPLL

SEQ ID NO: 4964 - protein, 39 aa, Homo sapiens
MLARLVSNSWPKVVCPPWPPKVLGLQAWATAPGLQETFL

SEQ ID NO: 4965 - protein, 27 aa, Homo sapiens
MLARLVSNSWPQVIRLPQPSKVLGLQV

SEQ ID NO: 4966 - protein, 20 aa, Homo sapiens
MLARLVWNSRPQVIHSPWPR

SEQ ID NO: 4967 - protein, 47 aa, Homo sapiens
MLARLYINILSFIFGPGFPGSALYLSFARKPFLNFTIICYLERISIF

SEQ ID NO: 4968 - protein, 46 aa, Homo sapiens
MLARPVSNSWPQVICPPRHHKVLGLQCETSCLACIIFKKAIHCMYN

SEQ ID NO: 4969 - protein, 120 aa, Homo sapiens [sequence omitted]

SEQ ID NO: 4970 - protein, 20 aa, Homo sapiens
MLARVVLNSWAQVICLLQPM

SEQ ID NO: 4971 - protein, 37 aa, Homo sapiens
MLARVVSNSQLQVICLPWPPKVLLYRRELPRLALQGY

SEQ ID NO: 4972 - protein, 26 aa, Homo sapiens
MLARWSPSLDLLIHLPRPPKVLGLQA

SEQ ID NO: 4973 - protein, 27 aa, Homo sapiens
MLASMVSNSGPCMIRPPRPPKVLGLQM

SEQ ID NO: 4974 - protein, 108 aa, Homo sapiens
MLAVFFFFETESCSVTQAGVQWLGLSSLQSLPPRGSSDSPASASQVAETTGACHHAQLIFVFLVETGFHYVGQAGLKLPTSSDPPASASQSAGITGVSHCAWLLIYFS

SEQ ID NO: 4975 - protein, 34 aa, Homo sapiens
MLAVNFVQIWILEMLTKCKKRKREHMQTYLIKIW

SEQ ID NO: 4976 - protein, 26 aa, Homo sapiens
MLAWLGDSLYHFVSGRVVFLRNFLFH

SEQ ID NO: 4977 - protein, 64 aa, Homo sapiens
MLCACLLLQARVLLGASLFLHQLWLLWGLQGGLWLLWGLQGGLWLLWGFQGGLWFLWLLPVQLL

SEQ ID NO: 4978 - protein, 67 aa, Homo sapiens
MLCTYLVHSGLDQVKFNNKLNSILNRSSLGNFLLIRPSSLFEKTMAEEPRASPQPEVTRRRRRPLSW

SEQ ID NO: 4979 - protein, 66 aa, Homo sapiens
MLCTYLVHSGLDQVKFNNKLNSILNRSSLGNFLLIRPSSLFEKTPAPEVATAQIPFYLLQASNELL

SEQ ID NO: 4980 - protein, 25 aa, Homo sapiens
MLCYPLYLLWKKKQEEKPLFFFQSC

SEQ ID NO: 4981 - protein, 28 aa, Homo sapiens
MLDFSVLRATNLQSTISGTPLHFNNKDP

SEQ ID NO: 4982 - protein, 71 aa, Homo sapiens
MLDHVFHHFPVDSTGTLIRLDVHLVVVHVDLRDVHLKVIGQELDWFPHSANARPARCLEHLLQGGQVSARS

SEQ ID NO: 4983 - protein, 92 aa, Homo sapiens
MLDHVFHHFPVDSTGTLIRLDVHLVVVHVDLRDVHLKVIGQELDWFPHSANARPARCLEHLLQGGQVSARSCSRGSRFHPIYPCGGQAARRL

SEQ ID NO: 4984 - protein, 11 aa, Homo sapiens
MLDLMRPSLYL

SEQ ID NO: 4985 - protein, 15 aa, Homo sapiens
MLEFQLPGELILSLL

SEQ ID NO: 4986 - protein, 24 aa, Homo sapiens
MLEKLFLKKKYERQEIKLLHNTEN

SEQ ID NO: 4987 - protein, 14 aa, Homo sapiens
MLEVAHSDSECFSR

SEQ ID NO: 4988 - protein, 28 aa, Homo sapiens
MLEVPRSSGLREKVNSDSLSIGIFSSLN

SEQ ID NO: 4989 - protein, 15 aa, Homo sapiens
MLFFINVFSQIPDEL

SEQ ID NO: 4990 - protein, 74 aa, Homo sapiens
MLFGALGEVGVADELSQKRRYLWADVQLFLKQCQVPVIVVNSSGSLQGGKKRAALSVVAMSGAQGVPHPVDSQG

SEQ ID NO: 4991 - protein, 101 aa, Homo sapiens
MLFGALGEVGVADELSQKRRYLWADVQLFLKQCQVPVIVVNSSGSLQGGKKRAALSVVAMSQCAGCQGFGVLRDRPGSALQIDEAAHSTFGCHGPKVAGWL

SEQ ID NO: 4992 - protein, 127 aa, Homo sapiens
MLFGALGEVGVADELSQKRRYLWADVQLFLKQCQVPVIVVNSSGSLQGGKKRAALSVVAMSVRVIQLGALPVVHPTEPLEVVIVAAPRPVHWHHGEVRHRAGSAPPHPPSQPPAAVPAAVPAAPGRH

SEQ ID NO: 4993 - protein, 44 aa, Homo sapiens
MLFGALGEVGVADELSQKRRYLWADVQLFRPSHPARRAPRSPPN

SEQ ID NO: 4994 - protein, 31 aa, Homo sapiens
MLFGDIPSYVPLSNNAPLSSSALNCSTEMKL

SEQ ID NO: 4995 - protein, 11 aa, Homo sapiens
MLFHLFLACLF

SEQ ID NO: 4996 - protein, 24 aa, Homo sapiens
MLFICQLSFVRLSVLSITNMWTFP

SEQ ID NO: 4997 - protein, 17 aa, Homo sapiens
MLFLCMIPKSSSYPSRG

SEQ ID NO: 4998 - protein, 19 aa, Homo sapiens
MLFPLDSGIFRLLGAQPVR

SEQ ID NO: 4999 - protein, 35 aa, Homo sapiens
MLFWMPKRMWRNRNTFTLLLCWWEYKLVQPLWRTV

SEQ ID NO: 5000 - protein, 16 aa, Homo sapiens
MLFYENRNHILWSGYN

SEQ ID NO: 5001 - protein, 37 aa, Homo sapiens
MLGAQQQYEKAGYYLKLRTVQPGWEERELWSSVSSRN

SEQ ID NO: 5002 - protein, 18 aa, Homo sapiens
MLGCHILVRNRKAGGEYG

SEQ ID NO: 5003 - protein, 34 aa, Homo sapiens
MLGERCEILLFEAAQCILHLNDNSLREYYVPKLN

SEQ ID NO: 5004 - protein, 49 aa, Homo sapiens
MLGFFFFFFFFFFCRDRVSLCCPGWSQVTNSWAQTILMPWLPKVLGLQV

SEQ ID NO: 5005 - protein, 16 aa, Homo sapiens
MLGLLALEHKPHGNQT

SEQ ID NO: 5006 - protein, 23 aa, Homo sapiens
MLGRLAGQELLMVRPGGGRPWFP

SEQ ID NO: 5007 - protein, 20 aa, Homo sapiens
MLGSEDSEKGKEIRGYAPKT

SEQ ID NO: 5008 - protein, 31 aa, Homo sapiens [sequence omitted]

SEQ ID NO: 5009 - protein, 20 aa, Homo sapiens
MLHHSALKALSCMLYSQHPG

SEQ ID NO: 5010 - protein, 17 aa, Homo sapiens
MLHNEKRKFLWHLSQSY

SEQ ID NO: 5011 - protein, 36 aa, Homo sapiens [sequence omitted]

SEQ ID NO: 5012 - protein, 71 aa, Homo sapiens
MLHSALCPHSSSRSIREFTNKMPFCRFTSRRSPCVLDATRNRRCTSSASSSPRSCAMRPTKVPCLASSETE

SEQ ID NO: 5013 - protein, 12 aa, Homo sapiens
MLHVCQYCNFSP

SEQ ID NO: 5014 - protein, 26 aa, Homo sapiens
MLIAYGLVLPIPSLYWEIMPFLGFAT

SEQ ID NO: 5015 - protein, 68 aa, Homo sapiens [sequence omitted]

SEQ ID NO: 5016 - protein, 14 aa, Homo sapiens
MLILSMNYLLLLLS

SEQ ID NO: 5017 - protein, 31 aa, Homo sapiens
MLILYPATVRNLFISSNSFLVESLGFSKYKI

SEQ ID NO: 5018 - protein, 12 aa, Homo sapiens
MLIPGQQPECLG

SEQ ID NO: 5019 - protein, 20 aa, Homo sapiens
MLIPSNLILRDKTEALHKKS

SEQ ID NO: 5020 - protein, 12 aa, Homo sapiens
MLISCTGHCASC

SEQ ID NO: 5021 - protein, 22 aa, Homo sapiens
MLISCTGHCASFIFLTMKNTNK

SEQ ID NO: 5022 - protein, 17 aa, Homo sapiens
MLISNLQGQKHKYHPVP

SEQ ID NO: 5023 - protein, 11 aa, Homo sapiens
MLIWKCFKHSP

SEQ ID NO: 5024 - protein, 13 aa, Homo sapiens
MLKDNSKCSTCPY

SEQ ID NO: 5025 - protein, 26 aa, Homo sapiens
MLKIHRLTLQFVFIKIHKGKFITQAF

SEQ ID NO: 5026 - protein, 12 aa, Homo sapiens
MLKIYSQSLFLL

SEQ ID NO: 5027 - protein, 19 aa, Homo sapiens
MLKKAKQFLFFNCRSSHSL

SEQ ID NO: 5028 - protein, 17 aa, Homo sapiens
MLKKTLIDYTGQEATEI

SEQ ID NO: 5029 - protein, 46 aa, Homo sapiens
MLKMDLPEIQGHPVSRFVSSSLSKTLQVGPALSASGFSLARLRSAP

SEQ ID NO: 5030 - protein, 89 aa, Homo sapiens
MLKSFLLQNCWRGSSRICSKISSSLSVSQKGSGWDLAPFSLMLLPATCFWKEQVLEPSSSSSSSSSSSSSSWMSDRSELRPWSTREFTR

SEQ ID NO: 5031 - protein, 22 aa, Homo sapiens
MLKTILSFAEFHFWWHIIWRLY

SEQ ID NO: 5032 - protein, 241 aa, Homo sapiens
MLKTLNKLGIDGTYVKIIRAIYDKPTANIILNGQKLEAFPVKTGTRQGCPLSPLLFNIVLEVLARAIRQDKEIKGIQLGKEEVKLSLFADDMIVYLENPIVSAQNLLKLISNFSKVSGYKINVQKSQAFLYTNNRQTESQIMSELPFTIASKRIKYLGIQLTRDVKNLFKDNYKPLLKEIKEDTNKWKNIPCSWVGRINIMKMAILSKVIYRFNAIPIKLPMTFFTELGKNYLKVHMEPKK

SEQ ID NO: 5033 - protein, 24 aa, Homo sapiens
MLKTPPAMGIKFQHEICRGQTNHI

SEQ ID NO: 5034 - protein, 34 aa, Homo sapiens
MLKYWGLVPLIFLPKCGDYRHQPPCPASTIIFLI

SEQ ID NO: 5035 - protein, 68 aa, Homo sapiens
MLLDIKVTILSGNKKCEGGACMVKVFKGMQKMDKVINISCRFWCGYTFTLIYMPSCTAEHCATILNKK

SEQ ID NO: 5036 - protein, 16 aa, Homo sapiens
MLLFFVTTVLILRLVF

SEQ ID NO: 5037 - protein, 18 aa, Homo sapiens
MLLFLKFHCCQRSYSVIF

SEQ ID NO: 5038 - protein, 23 aa, Homo sapiens
MLLFLVETGFHHVGQAGLELLTL

SEQ ID NO: 5039 - protein, 23 aa, Homo sapiens
MLLFRFLRNFNCQLESCHFGLKQ

SEQ ID NO: 5040 - protein, 13 aa, Homo sapiens
MLLGKKIHQGQGL

SEQ ID NO: 5041 - protein, 14 aa, Homo sapiens
MLLGYYIKIHHVVV

SEQ ID NO: 5042 - protein, 29 aa, Homo sapiens
MLLIAISRQNGVLCGLVLPCPREYGTQSF

SEQ ID NO: 5043 - protein, 11 aa, Homo sapiens
MLLIGIILSKT

SEQ ID NO: 5044 - protein, 62 aa, Homo sapiens
MLLKKESFLVADEGGEPVNSLPPGKLSTLGDELMFLELSPLFNCTGMLSDFISLCCCCCCCK

SEQ ID NO: 5045 - protein, 52 aa, Homo sapiens
MLLKKESFLVADEGGEPVNSLPPGKLSTLGDELMFLELSPWRSVRVWTGTET

SEQ ID NO: 5046 - protein, 16 aa, Homo sapiens
MLLKKGKKQKTVATLL

SEQ ID NO: 5047 - protein, 71 aa, Homo sapiens [sequence omitted]

SEQ ID NO: 5048 - protein, 26 aa, Homo sapiens
MLLKSNIIPAMAIPVLMFCGSSYSGG

SEQ ID NO: 5049 - protein, 41 aa, Homo sapiens
MLLKSNIIPAMAIPVLMFCNPNTLGGRGRQITRPGDRDHPD

SEQ ID NO: 5050 - protein, 26 aa, Homo sapiens
MLLKSNIIPAMAIPVLMFCNPSYSGG

SEQ ID NO: 5051 - protein, 64 aa, Homo sapiens
MLLKSNIIPAMAIPVLMFRTRRRWSSAHCEIRATTLGSIPSLSADGEPVAAGCPAMFPASCERP

SEQ ID NO: 5052 - protein, 13 aa, Homo sapiens
MLLLTLFLLTRNS

SEQ ID NO: 5053 - protein, 25 aa, Homo sapiens
MLLLVIYPCQLYFHEFVDKILQIFA

SEQ ID NO: 5054 - protein, 12 aa, Homo sapiens
MLLNFTYIFVAL

SEQ ID NO: 5055 - protein, 23 aa, Homo sapiens
MLLPGPVGAPGQQLLLGHLADQH

SEQ ID NO: 5056 - protein, 118 aa, Homo sapiens
MLLPGPVGAPGQQLLLGHLADQHLSRLLTGSIFQEPGDEEVELRSQLREAFPLTRHVYGSLQGRRRDTPPPRGSGDGAAACPIAVSVCSRAELRLHHSSNGGGGGGGGGGNNNSQAAT

SEQ ID NO: 5057 - protein, 131 aa, Homo sapiens
MLLPGPVGAPGQQLLLGHLADQHLSRLLTGSIFQEPGDEEVELRSQLREAFPLTRHVYGSLQGRRRDTPPPRGSGDGAAACPIAVSVCSRAELRLHHSSNGGGGGGGGGGNNNSQAATTAVAASAADPSAA

SEQ ID NO: 5058 - protein, 34 aa, Homo sapiens
MLLPSSLPDLPTHPPRRNHPLEVCVYYYQINGRL

SEQ ID NO: 5059 - protein, 119 aa, Homo sapiens
MLLRSTASRSCRGGSWTRCCRPLMVSTSSWWNSWMTSSSRPASFSPRQKVNVSSPMAAVQSPGSSQVSMVMVAGDPFTSAAAGVRGMYSADVGLLRDTRAPERSIFVLRQVLEQTLSCW

SEQ ID NO: 5060 - protein, 75 aa, Homo sapiens
MLLSLILGWRSLMIPRKIQYVLFFLWLFLFYTFILAKHPIWLDYEHRELSFLLILSQGSFPFVLAVFLGSVKHEL

SEQ ID NO: 5061 - protein, 22 aa, Homo sapiens
MLLVELNPLKVQYKAGCSGSCL

SEQ ID NO: 5062 - protein, 31 aa, Homo sapiens
MLLWWWRKLHESLPAKVWWWWGCLGLLGQRL

SEQ ID NO: 5063 - protein, 23 aa, Homo sapiens
MLLWWWRKQFWRLANPRSKACIW

SEQ ID NO: 5064 - protein, 27 aa, Homo sapiens
MLLYLTDTSNCSHSHITVQNFHKSKAR

SEQ ID NO: 5065 - protein, 35 aa, Homo sapiens
MLMFKKLICSTHTFKIYCNSYSSLDIFLPLKKKSF

SEQ ID NO: 5066 - protein, 36 aa, Homo sapiens
MLMLSSMAEKGQETKKSCGRTDWQRHREGTATALHR

SEQ ID NO: 5067 - protein, 13 aa, Homo sapiens
MLNFFTSSFTSSM

SEQ ID NO: 5068 - protein, 13 aa, Homo sapiens
MLNGILSFYRETV

SEQ ID NO: 5069 - protein, 21 aa, Homo sapiens
MLNKYSFFCYSKKNPSFVINL

SEQ ID NO: 5070 - protein, 47 aa, Homo sapiens
MLNLRPSPHIKNFVGSQWASLVDSPISKDTALINVVFHKWVDSKGSS

SEQ ID NO: 5071 - protein, 22 aa, Homo sapiens
MLNPDRESSFAHSRIFFLLHLL

SEQ ID NO: 5072 - protein, 14 aa, Homo sapiens
MLPAHLRKHRYRYS

SEQ ID NO: 5073 - protein, 18 aa, Homo sapiens
MLPATLQAWQGSVLLTLW

SEQ ID NO: 5074 - protein, 38 aa, Homo sapiens
MLPEKHLCPWSGEPMHPQGLHGLVSFQGHGLQHHLLLL

SEQ ID NO: 5075 - protein, 82 aa, Homo sapiens
MLPGQEFLLLWCLDFLGVEEVGVFGAVHQDLGPVPVLGAPRAVPPGRLMATMPLQRGALTAGIAHDGGLPRQAAARTQGARR

SEQ ID NO: 5076 - protein, 85 aa, Homo sapiens [sequence omitted]

SEQ ID NO: 5077 - protein, 12 aa, Homo sapiens
MLPGWSRTPDLK

SEQ ID NO: 5078 - protein, 12 aa, Homo sapiens
MLPKLDSSNIPE

SEQ ID NO: 5079 - protein, 27 aa, Homo sapiens
MLPKLVSNSWAQVIFLTWPLKVLVLQM

SEQ ID NO: 5080 - protein, 11 aa, Homo sapiens
MLPKLVSNSWP

SEQ ID NO: 5081 - protein, 48 aa, Homo sapiens
MLPKRIPAKVNGPPPDESSSLSESDMMAAVTVAAALSSKSQPGRINRK

SEQ ID NO: 5082 - protein, 13 aa, Homo sapiens
MLPMGSRRSAICR

SEQ ID NO: 5083 - protein, 20 aa, Homo sapiens
MLPNTLISDFFQILAFRSTL

SEQ ID NO: 5084 - protein, 11 aa, Homo sapiens
MLPQLHNPTVH

SEQ ID NO: 5085 - protein, 25 aa, Homo sapiens
MLPRLILNSWAQVILLPWAPTMLGL

SEQ ID NO: 5086 - protein, 50 aa, Homo sapiens
MLPRLISSSRAQAILPPRLPRVLGLQALVTAPGQAQPFSKTEFAWVDRGL

SEQ ID NO: 5087 - protein, 27 aa, Homo sapiens
MLPRLLSNSWTQATHLSQPPKVLGLQA

SEQ ID NO: 5088 - protein, 27 aa, Homo sapiens
MLPRLVLNSWAQVIYPPQPPKVLGLQG

SEQ ID NO: 5089 - protein, 27 aa, Homo sapiens
MLPRLVLNSWTQAIHPFWPPKLLVLQV

SEQ ID NO: 5090 - protein, 88 aa, Homo sapiens
MLPRLVSNSWAQAILPPQPPKALGITGVSPSAQPAPCVSAGLGPRSHRLQGNICLPVFGVAISASIRHFPQQTRLPTLMLLELQARGW

SEQ ID NO: 5091 - protein, 47 aa, Homo sapiens
MLPRLVSRLLSSSDPPASASQSAGITGMHHCASLYLINFDYKSVFLN

SEQ ID NO: 5092 - protein, 20 aa, Homo sapiens
MLPRLVSTEVSILIRRNKKY

SEQ ID NO: 5093 - protein, 40 aa, Homo sapiens
MLPRMVTSYKLLGSNNPHALASQSVGITGVSHLSGPGSWF

SEQ ID NO: 5094 - protein, 69 aa, Homo sapiens
MLPVGPDQVWTMPGARPPPLIYTHARIRSSMGNRSKISVKSKSQEGSMWREVKFRPCPGNYDTQNIPLV

SEQ ID NO: 5095 - protein, 47 aa, Homo sapiens
MLPVGPDQVWTMPGARPPPLIYTHARIRSSMGNRSKISVKSKSRGWE

SEQ ID NO: 5096 - protein, 30 aa, Homo sapiens
MLPWLEVGVPWESPCTEPSSSEPEEVSGGV

SEQ ID NO: 5097 - protein, 16 aa, Homo sapiens
MLPYCFVGNLVLIFRI

SEQ ID NO: 5098 - protein, 16 aa, Homo sapiens
MLQLFGSSLVSLNNVL

SEQ ID NO: 5099 - protein, 61 aa, Homo sapiens
MLRAWTFLLKDFGRGMTMQTVRRMLGVLLEGVILCTHLGYQRNLFSSSLQLEYERVWDQQP

SEQ ID NO: 5100 - protein, 63 aa, Homo sapiens
MLRFDLGYLSTREIKYFFTQEFKNHHIILTETFAGPTCSNNITDKSWPMFGPFLFQYLNKDHI

SEQ ID NO: 5101 - protein, 64 aa, Homo sapiens
MLRFDLGYLSTREIKYFFTQEFKNHHIILTETFAGPTCSNNITDKSWPMFGPFLFQYLYTSWVR

SEQ ID NO: 5102 - protein, 37 aa, Homo sapiens
MLRHNSGGCFTVYHANSTSAAGNYATNIQDLKNSSFP

SEQ ID NO: 5103 - protein, 12 aa, Homo sapiens
MLRIATRVSGSF

SEQ ID NO: 5104 - protein, 14 aa, Homo sapiens
MLRPFIRVLQASGS

SEQ ID NO: 5105 - protein, 12 aa, Homo sapiens
MLRRRARKREHK

SEQ ID NO: 5106 - protein, 34 aa, Homo sapiens
MLRSATSFFSPVCSAISWSNTAPNSSWIFCISLM

SEQ ID NO: 5107 - protein, 83 aa, Homo sapiens
MLRSKSQGFQRSFNQCFLKVPTVLGSAGGGGGGSRSSCAELGLAGREVKGSGRLSTGTSHRIQPGNYSSGEVTAARCALQREA

SEQ ID NO: 5108 - protein, 80 aa, Homo sapiens
MLRSKSQGFQRSFNQCFLKVPTVLGSDGSAPSVWSETAGNLVLVLPSAGDLRQGHPSGLTQPGLVYLAAAAAAAGPPALS

SEQ ID NO: 5109 - protein, 82 aa, Homo sapiens
MLRSKSQGFQRSFNQCFLKVPTVLGSGGGGGGSRSSCAELGLAGREVKGSGRLSTGTSHRIQPGNYSSGEVTAARCALQREA

SEQ ID NO: 5110 - protein, 19 aa, Homo sapiens
MLSFIQVYISDVLKQFSLS

SEQ ID NO: 5111 - protein, 118 aa, Homo sapiens
MLSFISASDLLLCPSVFCDSFSFARSVYTFSSSAPAASSRRGDIPSPFFFTTVRNAVLPIFCLCLVKAASIFFFWASIARLFSSSFILRCTISEANSWVVSRPCGSPVSSGICAQATT

SEQ ID NO: 5112 - protein, 33 aa, Homo sapiens
MLSFKCLDLTWVICPLEKSNTSSLKSLRITILF

SEQ ID NO: 5113 - protein, 39 aa, Homo sapiens
MLSFLVFTCQNDNASLCIATVKIIISLMIIINLLHKFSS

SEQ ID NO: 5114 - protein, 146 aa, Homo sapiens
MLSGARRKAHLLSACRERSRNSKENQATHTVSSTNRLRHLGEHSPRSSSARMSGMVLRQRPTAVTATKDTDTQAKSLPASPECGLSTTSRRRRRPRCSRPRGPRARAGLPCAPRSVGPARASAASSSRRRRRRRQQRSRRASSMPQ

SEQ ID NO: 5115 - protein, 34 aa, Homo sapiens
MLSGGRTGPRRAHSGSMARRRRLLARLPAPPPPP

SEQ ID NO: 5116 - protein, 42 aa, Homo sapiens
MLSGGRTGPRRAHSGSMARRRRLLARLPAPPPPPSGAADQDD

SEQ ID NO: 5117 - protein, 46 aa, Homo sapiens [sequence omitted]

SEQ ID NO: 5118 - protein, 15 aa, Homo sapiens
MLSGLCLQRLAPLRY

SEQ ID NO: 5119 - protein, 25 aa, Homo sapiens
MLSHIFFLKSALFSLSFPSGMQIWS

SEQ ID NO: 5120 - protein, 32 aa, Homo sapiens
MLSKDTCSVLRSSRISSPFKQTETHSPHIEGP

SEQ ID NO: 5121 - protein, 16 aa, Homo sapiens
MLSNCPKYFYTRIISH

SEQ ID NO: 5122 - protein, 13 aa, Homo sapiens
MLSPYFSFLEFAF

SEQ ID NO: 5123 - protein, 42 aa, Homo sapiens
MLSRFRMISSRKPFSQSLVFGLIFTALPFTFIPSTSRTLRAE

SEQ ID NO: 5124 - protein, 27 aa, Homo sapiens
MLSRLVSNSWPRAIHMPQPPKVLGLQV

SEQ ID NO: 5125 - protein, 24 aa, Homo sapiens
MLSSICVAQTTGLPAKLQRPIIIF

SEQ ID NO: 5126 - protein, 12 aa, Homo sapiens
MLSSLSSSHYVR

SEQ ID NO: 5127 - protein, 34 aa, Homo sapiens
MLSSMAEKGQETKKSCGRTDWQRHREGTATALHR

SEQ ID NO: 5128 - protein, 154 aa, Homo sapiens
MLSTLKPWLWCGGGAEGAGGGGAESAPSRLSGRADGRLPGGLLPLDRLLLLLSGLSILGTAAALPLPRAAAGDRGWGGEGHVPFSVLMSWMRTGGGCGPGALPSACSGGAGGGWRPGGGGSLRCSLSFSSLSFTASFFLKRRRRRRKLPFSNML

SEQ ID NO: 5129 - protein, 34 aa, Homo sapiens
MLSTMPEANSSGIFPSVCPLTHWFMVFLASSEAC

SEQ ID NO: 5130 - protein, 15 aa, Homo sapiens
MLTCHTCGPFSSFLI

SEQ ID NO: 5131 - protein, 59 aa, Homo sapiens
MLTCPGWSPAPGLKRSSCLSLPKCWDYRHEPLSLAFLMSWTKKDLLFFLEVFGRRNSEK

SEQ ID NO: 5132 - protein, 138 aa, Homo sapiens
MLTFFFLMFLALNSYRIRRMAATISTLLLGLGTSRLPTYLASKQMPCWKASSLCKGIRRSCPSSTRLYLVLLGMVTRGGPAPSEAAAAGRGWRDPGEGRLELGAATRGGAWERWAGGALAARRPDPERCRGPSGSGLS

SEQ ID NO: 5133 - protein, 21 aa, Homo sapiens
MLTKCKKRKREHMQTYLIKIW

SEQ ID NO: 5134 - protein, 24 aa, Homo sapiens
MLTLIFLIISCIFQIHVASPSEKT

SEQ ID NO: 5135 - protein, 20 aa, Homo sapiens
MLTPGQNSVEGLVSRGPCAI

SEQ ID NO: 5136 - protein, 40 aa, Homo sapiens
MLTPLSTTGIQIVRIKALWFFQFVQYCSNIHYLFSKDGVS

SEQ ID NO: 5137 - protein, 88 aa, Homo sapiens
MLTRPVDTLFSLTAFFYLRLCQVFCFPFQFSPTYTFCSFVYPVRFSVTLCYPLLFPFTVSSVAFLLNRSLVIWASPSFLSWLLIHMGD

SEQ ID NO: 5138 - protein, 16 aa, Homo sapiens
MLTSFSVLVRVSVTGG

SEQ ID NO: 5139 - protein, 11 aa, Homo sapiens
MLTVHRTLQLT

SEQ ID NO: 5140 - protein, 12 aa, Homo sapiens
MLTVHRTLQLTM

SEQ ID NO: 5141 - protein, 14 aa, Homo sapiens
MLTVHRTLQLTMRM

SEQ ID NO: 5142 - protein, 14 aa, Homo sapiens
MLTVYPGRQIPGKL

SEQ ID NO: 5143 - protein, 31 aa, Homo sapiens
MLTWKFTSRYPQLLSLLQLNDDVWLGDIISC

SEQ ID NO: 5144 - protein, 27 aa, Homo sapiens
MLTYYFIFYGMLLSKDKKTNCCFIATY

SEQ ID NO: 5145 - protein, 12 aa, Homo sapiens
MLVEVTDADVGC

SEQ ID NO: 5146 - protein, 55 aa, Homo sapiens
MLVFLVERGFHHVGQAGLELLTSGALSALASQSARTTGMSHFSQPNSFQNRSQSS

SEQ ID NO: 5147 - protein, 48 aa, Homo sapiens
MLVKLVSNSQPQVIHLPRPPKVLGLQACATTPSLGCFSFSSSSTFILF

SEQ ID NO: 5148 - protein, 105 aa, Homo sapiens
MLVLELGEALRFLLLFCEVGGELSYSVFQQFLFLGQLAVLVLQDDLLLLQLFQLRLGGHLLQLQLLPGALLLLQLLLKLLDVLLHLLLLRLQVLAALLLLLHPGL

SEQ ID NO: 5149 - protein, 13 aa, Homo sapiens
MLVLGRQSYWDEI

SEQ ID NO: 5150 - protein, 66 aa, Homo sapiens [sequence omitted]

SEQ ID NO: 5151 - protein, 37 aa, Homo sapiens
MLVMADLKLLTSDDLPASASQSAGLTSVSHHTWLTPS

SEQ ID NO: 5152 - protein, 18 aa, Homo sapiens
MLVRLGRNRNAYTLFVRM

SEQ ID NO: 5153 - protein, 27 aa, Homo sapiens
MLVRLVANSQPQVIRLPWPPKVLGLQA

SEQ ID NO: 5154 - protein, 27 aa, Homo sapiens
MLVRLVANSRPQVILPPQPPKVLGLQA

SEQ ID NO: 5155 - protein, 27 aa, Homo sapiens
MLVRLVLNSQPQVICLPRPHKVLGLQV

SEQ ID NO: 5156 - protein, 23 aa, Homo sapiens
MLVRLVLNSQPQVIHPSRPPKVL

SEQ ID NO: 5157 - protein, 27 aa, Homo sapiens
MLVRLVLNSQPQVIYPPRPSKVLGLQT

SEQ ID NO: 5158 - protein, 27 aa, Homo sapiens
MLVRLVLNSRPQVIRPPRPPKVLGLQV

SEQ ID NO: 5159 - protein, 12 aa, Homo sapiens
MLVRLVLNSSLR

SEQ ID NO: 5160 - protein, 48 aa, Homo sapiens
MLVRLVSELLTSGDPPASASQSAGITGMSYRAWPKPYAFEVECRPCDN

SEQ ID NO: 5161 - protein, 27 aa, Homo sapiens
MLVRLVSNSRPQVICPPLPPKVLGLQA

SEQ ID NO: 5162 - protein, 27 aa, Homo sapiens
MLVRLVSNSRPQVICPPRPPKMLGLQA

SEQ ID NO: 5163 - protein, 27 aa, Homo sapiens
MLVRLVSNSRPQVICPPWLPKVLGLQA

SEQ ID NO: 5164 - protein, 27 aa, Homo sapiens
MLVRLVSNSRPQVILPPRPPKVLGLQA

SEQ ID NO: 5165 - protein, 11 aa, Homo sapiens
MLVRLWRKGNT

SEQ ID NO: 5166 - protein, 27 aa, Homo sapiens
MLVRMVSIALLGLPKCWDYRHESPRLA

SEQ ID NO: 5167 - protein, 27 aa, Homo sapiens
MLVRMVSNSQPQVIRLPRPLKALGLQG

SEQ ID NO: 5168 - protein, 18 aa, Homo sapiens
MLVRMWRKETPCTLLVGT

SEQ ID NO: 5169 - protein, 15 aa, Homo sapiens
MLVRTWRKGTLLVGM

SEQ ID NO: 5170 - protein, 21 aa, Homo sapiens
MLVSSLLSGLDPVLALSCDLA

SEQ ID NO: 5171 - protein, 19 aa, Homo sapiens
MLVWMRSKGNFYTAGGNAN

SEQ ID NO: 5172 - protein, 14 aa, Homo sapiens
MLVYLLDLWDLLLM

SEQ ID NO: 5173 - protein, 28 aa, Homo sapiens
MLWASSKTTTALRASSLDTRSAILGSRR

SEQ ID NO: 5174 - protein, 142 aa, Homo sapiens
MLWGFRQEAYEWPICNLCGNLLHGAGERLTGAAVLQGLHVAEEALGLLNFCQELIHVPAGVVLHLWAVAVVVAPNSFCKVLQDSRGHLIIASVGDEVDDEVSSHGGLLDVVRQDFRRLIWAASHDGHQGIQSLESEDLLQSL

SEQ ID NO: 5175 - protein, 34 aa, Homo sapiens [sequence omitted]

SEQ ID NO: 5176 - protein, 81 aa, Homo sapiens
MLWLTARSPKSQEALTSRSSRKELRRVSAEVFLASLCPVEQDVRAARRNMVPFITMTRTTGPAKLQMRGSWTEIQQKSGFP

SEQ ID NO: 5177 - protein, 20 aa, Homo sapiens
MLWNVFQYLIDGLCLHVFVC

SEQ ID NO: 5178 - protein, 73 aa, Homo sapiens
MLWPTCSVSGSCPVLQPLSSLMLLPKPQLVRRGQSLLGNSNHPTWVTADLEEHRPSPLRGWKIKVVWSKENGK

SEQ ID NO: 5179 - protein, 59 aa, Homo sapiens
MLYHLWCPPVSITSSCWQKSHGIFVMQIKICWELPEMRFPFSGMENSQEEINGILSIGI

SEQ ID NO: 5180 - protein, 16 aa, Homo sapiens
MLYIIKYLQENLKLQF

SEQ ID NO: 5181 - protein, 16 aa, Homo sapiens
MLYVNVQKVNLFNTYI

SEQ ID NO: 5182 - protein, 25 aa, Homo sapiens
MLYVPLLARYINSILHRQQTHSNFD

SEQ ID NO: 5183 - protein, 32 aa, Homo sapiens
MMCLSLKPLLKMKNLLKEAKINCFILREHIIE

SEQ ID NO: 5184 - protein, 16 aa, Homo sapiens
MMEERTKSQGIHGMQL

SEQ ID NO: 5185 - protein, 13 aa, Homo sapiens
MMFLKILLFFNCD

SEQ ID NO: 5186 - protein, 39 aa, Homo sapiens
MMIQRFERPYTVNKNMSISFFKAYWTIKHSEGNEGWTGR

SEQ ID NO: 5187 - protein, 25 aa, Homo sapiens
MMKGLDLIVSKVCSVELMALLNFFG

SEQ ID NO: 5188 - protein, 64 aa, Homo sapiens [sequence omitted]

SEQ ID NO: 5189 - protein, 36 aa, Homo sapiens
MMKMSLSSPNPHPLVRTDRSSHTQWSQPLGRGTCSR

SEQ ID NO: 5190 - protein, 14 aa, Homo sapiens
MMLEQLNTHIQIYI

SEQ ID NO: 5191 - protein, 29 aa, Homo sapiens
MMLEVPRSSGLREKVNSDSLSIGIFSSLN

SEQ ID NO: 5192 - protein, 17 aa, Homo sapiens
MMLGLLALEHKPHGNQT

SEQ ID NO: 5193 - protein, 147 aa, Homo sapiens
MMLSGARRKAHLLSACRERSRNSKENQATHTVSSTNRLRHLGEHSPRSSSARMSGMVLRQRPTAVTATKDTDTQAKSLPASPECGLSTTSRRRRRPRCSRPRGPRARAGLPCAPRSVGPARASAASSSRRRRRRRQQRSRRASSMPQ

SEQ ID NO: 5194 - protein, 14 aa, Homo sapiens
MMLSPYFSFLEFAF

SEQ ID NO: 5195 - protein, 155 aa, Homo sapiens
MMLSTLKPWLWCGGGAEGAGGGGAESAPSRLSGRADGRLPGGLLPLDRLLLLLSGLSILGTAAALPLPRAAAGDRGWGGEGHVPFSVLMSWMRTGGGCGPGALPSACSGGAGGGWRPGGGGSLRCSLSFSSLSFTASFFLKRRRRRRKLPFSNML

SEQ ID NO: 5196 - protein, 41 aa, Homo sapiens
MMLTPLSTTGIQIVRIKALWFFQFVQYCSNIHYLFSKDGVS

SEQ ID NO: 5197 - protein, 19 aa, Homo sapiens
MMLVRLGRNRNAYTLFVRM

SEQ ID NO: 5198 - protein, 33 aa, Homo sapiens
MMMCLSLKPLLKMKNLLKEAKINCFILREHIIE

SEQ ID NO: 5199 - protein, 65 aa, Homo sapiens [sequence omitted]

SEQ ID NO: 5200 - protein, 42 aa, Homo sapiens
MMMMMMTALCNMPRTCHTKAWREGKEELLLFILCLSAPFEKK

SEQ ID NO: 5201 - protein, 41 aa, Homo sapiens
MMMMMTALCNMPRTCHTKAWREGKEELLLFILCLSAPFEKK

SEQ ID NO: 5202 - protein, 40 aa, Homo sapiens
MMMMTALCNMPRTCHTKAWREGKEELLLFILCLSAPFEKK

SEQ ID NO: 5203 - protein, 23 aa, Homo sapiens
MMMRKSLEHGEHGRLWLMRSSVP

SEQ ID NO: 5204 - protein, 39 aa, Homo sapiens
MMMTALCNMPRTCHTKAWREGKEELLLFILCLSAPFEKK

SEQ ID NO: 5205 - protein, 17 aa, Homo sapiens
MMMVSPLYTEANQISPT

SEQ ID NO: 5206 - protein, 45 aa, Homo sapiens [sequence omitted]

SEQ ID NO: 5207 - protein, 47 aa, Homo sapiens
MMRFCRIGQAGLELLTSSDLPALASQSTGITGMSHRTQSKMEYDIRL

SEQ ID NO: 5208 - protein, 22 aa, Homo sapiens
MMRKSLEHGEHGRLWLMRSSVP

SEQ ID NO: 5209 - protein, 46 aa, Homo sapiens
MMSDFSCGHCLVLGIARELNDQGLVMLLGIGELRLYFPLVIISKHL

SEQ ID NO: 5210 - protein, 16 aa, Homo sapiens
MMSLGSRCWDDLHCAG

SEQ ID NO: 5211 - protein, 14 aa, Homo sapiens
MMSLRVRSPVKRSG

SEQ ID NO: 5212 - protein, 149 aa, Homo sapiens
MMSMSCKFSRLVSTSSCPSPEFSSSPLSSTPSSSGLRPLLDLFDVFLFPSEVISISSGLPPSSSIAFFSRSIKTLLLPLESTFRFLSSARRSITRRSLRRRVPVSDEAELRAAAPAAPESPRPDRVSAIPGTLAPPPTFHRTGPVLSGS

SEQ ID NO: 5213 - protein, 52 aa, Homo sapiens
MMSRLPSSVNRYISRNSRKSISWRWGKAEKPTRMNSDMEVWFSPSMTATPSW

SEQ ID NO: 5214 - protein, 18 aa, Homo sapiens
MMSSWIRVGPNPVWLSSL

SEQ ID NO: 5215 - protein, 38 aa, Homo sapiens
MMTALCNMPRTCHTKAWREGKEELLLFILCLSAPFEKK

SEQ ID NO: 5216 - protein, 68 aa, Homo sapiens
MMTFGLVISYLVNGKRRRTWASCSASESPKYKMLPPHKPRKLDGCSSPTSHPRMLSSHQGPVAATPPG

SEQ ID NO: 5217 - protein, 21 aa, Homo sapiens
MMTPMKRLRVKKEPKMMKMTK

SEQ ID NO: 5218 - protein, 28 aa, Homo sapiens
MMTSQWSLPHTTGLTPKYVFHMGCFICG

SEQ ID NO: 5219 - protein, 40 aa, Homo sapiens
MMTVSLVILSDNWSQKLIKHFHLHYPLKLKFLYLLFCHSG

SEQ ID NO: 5220 - protein, 22 aa, Homo sapiens
MMVAGFGLGLYMFCYCPGSLAE

SEQ ID NO: 5221 - protein, 303 aa, Homo sapiens
MMVEMVSRHLLSPALLSLGSGRILSWWIGCFCLFAILWFRVFWASASVIEVAAVPTLRWLLTLGLISLIFFIFFIAVLSRLSLARRAPAESWSISPIHILPHWSTLFSCTLVVSTLHHFSLHRRVGILWSTPIGSPHVVRWEPSPAVGPALLGLAFGSTLRSLVLFPTLTILVILLVIAWRTPTTWIASIMVTVCCIFTALNWNTTRTCNICCLRTLFSFNNIKLHSLSISYTAKVLPGVILLYGSLVYKYIFLGVIPAILFQIRPAWASGPSHAGRRGHLTALSLHRPGAGPRSRRRRRTRG

SEQ ID NO: 5222 - protein, 356 aa, Homo sapiens
MMVEMVSRHLLSPALLSLGSGRILSWWIGCFCLFAILWFRVFWASASVIEVAAVPTLRWLLTLGLISLIFFIFFIAVLSRLSLARRAPAESWSISPIHILPHWSTLFSCTLVVSTLHHFSLHRRVGILWSTPIGSPHVVRWEPSPAVGPALLGLAFGSTLRSLVLFPTLTILVILLVIAWRTPTTWIASIMVTVCCIFTALNWNTTRTCNICCLRTLFSFNNIKLHSLSISYTAKVLPGVILLYGSLVYKYIFLGVIPVDETISVPYIEPFYCSQNLRCDDLLVPAGRRRRCEAARATAPCAAARSAGLGVGGAEGGGGGGGGGRLLGLGLAAHGCGDGDWGRLRQLRLLPGCDGN

SEQ ID NO: 5223 - protein, 53 aa, Homo sapiens
MMVFWANTVRRKAQAPPPRTHLPPRKMLYSSGAARQLASLCTGSVKAHLNPRK

SEQ ID NO: 5224 - protein, 84 aa, Homo sapiens
MMVPDWRLVMVAGYSKLLGLWVVTPISMEPDHLSTSLSIRISNISLSRRGRLVMTTPLLNSSRGRRRSAVLLLLLSLMRVPHFS

SEQ ID NO: 5225 - protein, 16 aa, Homo sapiens
MMVSPLYTEANQISPT

SEQ ID NO: 5226 - protein, 15 aa, Homo sapiens
MMVVLRFFPIGKLIL

SEQ ID NO: 5227 - protein, 20 aa, Homo sapiens
MMYMKYMITSIMDIASDQEL

SEQ ID NO: 5228 - protein, 15 aa, Homo sapiens
MNCIKPLCNTLILSY

SEQ ID NO: 5229 - protein, 12 aa, Homo sapiens
MNCSPLPGMTLW

SEQ ID NO: 5230 - protein, 21 aa, Homo sapiens
MNETLLIIDLLYILWCLFISC

SEQ ID NO: 5231 - protein, 17 aa, Homo sapiens
MNFRARSQMQVSIIPKS

SEQ ID NO: 5232 - protein, 13 aa, Homo sapiens
MNFSFPRTLPQVA

SEQ ID NO: 5233 - protein, 11 aa, Homo sapiens
MNFSRSPTVFW

SEQ ID NO: 5234 - protein, 22 aa, Homo sapiens
MNFVRTKSIVRNSEKRQNACIQ

SEQ ID NO: 5235 - protein, 44 aa, Homo sapiens
MNGMSAPNFSTIVLDLFCCNYIFITSVLFFFFFFRDQVSLCCLG

SEQ ID NO: 5236 - protein, 16 aa, Homo sapiens
MNGNKIEDLSPEPHYP

SEQ ID NO: 5237 - protein, 28 aa, Homo sapiens
MNHHARLIFCVFSRDGVSPCWPGLISNT

SEQ ID NO: 5238 - protein, 22 aa, Homo sapiens
MNIHDIVDLVVVPSFKSPLIQI

SEQ ID NO: 5239 - protein, 14 aa, Homo sapiens
MNILNKEFSRWSVR

SEQ ID NO: 5240 - protein, 12 aa, Homo sapiens
MNIPVKGSAQVV

SEQ ID NO: 5241 - protein, 16 aa, Homo sapiens
MNKELGISSYKFCGMG

SEQ ID NO: 5242 - protein, 25 aa, Homo sapiens
MNKTSIFDTNNVPKPNLTKLMTASQ

SEQ ID NO: 5243 - protein, 17 aa, Homo sapiens
MNKYSLEFCQCHIRVCY

SEQ ID NO: 5244 - protein, 25 aa, Homo sapiens
MNLFWFLSVPSISLTLMARGGFHCR

SEQ ID NO: 5245 - protein, 52 aa, Homo sapiens [sequence omitted]

SEQ ID NO: 5246 - protein, 13 aa, Homo sapiens
MNLLTKYCRFLPK

SEQ ID NO: 5247 - protein, 40 aa, Homo sapiens
MNLMASSTLCTFTMGRMGPKISSCITGSVSCTSTSTVGAM

SEQ ID NO: 5248 - protein, 21 aa, Homo sapiens
MNLNFNSSQIVSQHHYMTENL

SEQ ID NO: 5249 - protein, 20 aa, Homo sapiens
MNLPVHFYLLGLISQSSRPL

SEQ ID NO: 5250 - protein, 11 aa, Homo sapiens
MNLYLLQMAFF

SEQ ID NO: 5251 - protein, 13 aa, Homo sapiens
MNNHCFKHLCVFT

SEQ ID NO: 5252 - protein, 21 aa, Homo sapiens
MNNQSIPSAVLSTRPSLKYFP

SEQ ID NO: 5253 - protein, 49 aa, Homo sapiens
MNPETLKLPFADFLFFYLFFLRRSLTLSPRLECNGTISAHYNFCLPGSK

SEQ ID NO: 5254 - protein, 37 aa, Homo sapiens
MNPGSQEARSGVPRLGRVRAPQRDPEPAAEAPFGISQ

SEQ ID NO: 5255 - protein, 11 aa, Homo sapiens
MNPNQSVVKLI

SEQ ID NO: 5256 - protein, 39 aa, Homo sapiens
MNPSTQSYGARWSSPLCPADKSCQAKNKVYKSKLSHFIT

SEQ ID NO: 5257 - protein, 45 aa, Homo sapiens
MNQRDTSSVHSTPRRSIRAPTAGSFARTSSPRTSWSVFRPSMAGL

SEQ ID NO: 5258 - protein, 68 aa, Homo sapiens
MNRALSFSISCQERIGIFNSSPTTMPGPWVGGPPVNSMILAPVFGKVPSSKPTAMDKATPVDRKGLFP

SEQ ID NO: 5259 - protein, 11 aa, Homo sapiens
MNRGPYGSICL

SEQ ID NO: 5260 - protein, 13 aa, Homo sapiens
MNSDPMTALMWSK

SEQ ID NO: 5261 - protein, 47 aa, Homo sapiens
MNSEMIPTTKTFSTFFTLMSFFTCSTVLIEMALSHYCAHRVGSLSTS

SEQ ID NO: 5262 - protein, 15 aa, Homo sapiens
MNSFLPPCLELVSSL

SEQ ID NO: 5263 - protein, 39 aa, Homo sapiens
MNSIKNCFLYQEIGNKLVQKHITIASCFPPFFPSSVESC

SEQ ID NO: 5264 - protein, 23 aa, Homo sapiens
MNSQNFLFVGYNEFFPFNTVLQT

SEQ ID NO: 5265 - protein, 14 aa, Homo sapiens
MNSSRTFGNFREIL

SEQ ID NO: 5266 - protein, 50 aa, Homo sapiens
MNTFKGCFSPVLGQSSTVCLLLMASGEQDRGLAPDHMVQKFSSTSRISST

SEQ ID NO: 5267 - protein, 50 aa, Homo sapiens
MNTFKGCFSPVLGQSSTVCLLLMASGEQDRSLAPDHMVQKFSSTSRISST

SEQ ID NO: 5268 - protein, 12 aa, Homo sapiens
MNTHQPGAGFLK

SEQ ID NO: 5269 - protein, 123 aa, Homo sapiens [sequence omitted]

SEQ ID NO: 5270 - protein, 23 aa, Homo sapiens
MNTPIKSQTIMAKHKTAMATKIR

SEQ ID NO: 5271 - protein, 20 aa, Homo sapiens
MNVCVCVCTTIPTYSGSDSQ

SEQ ID NO: 5272 - protein, 16 aa, Homo sapiens
MNVPKPPRKSLLLHNT

SEQ ID NO: 5273 - protein, 18 aa, Homo sapiens
MNVSKMDNEPGHERKVFV

SEQ ID NO: 5274 - protein, 70 aa, Homo sapiens
MNVSKMDNEPGHERKVFVPGLGLQENMALHILAGFTVCHTSFPHGILAVVPATWEADVGGSLEPRRWRLQ

SEQ ID NO: 5275 - protein, 90 aa, Homo sapiens
MNVSKMDNEPGHERKVFVPGLGLQENMALHILAGFTVCHTSFPHGILDLTDQLLPEGGAPPVGLLPGNVHACSPAPAARIPLGRHRRRLS

SEQ ID NO: 5276 - protein, 72 aa, Homo sapiens
MNVSKMDNEPGHERKVFVRAEAHPARQIQTLARPPLESASRKRAVSAQLGWPITGTKKQEGDREPPTATPLP

SEQ ID NO: 5277 - protein, 18 aa, Homo sapiens
MNVSTSTLRASGSGTESA

SEQ ID NO: 5278 - protein, 29 aa, Homo sapiens
MNVYYFYNQKKMCFVLRNGGRFRIVLPLL

SEQ ID NO: 5279 - protein, 46 aa, Homo sapiens
MNYYPGLSLIKHFINMQVCLGISCLFHRCCTLFLYRYHPVLITVAT

SEQ ID NO: 5280 - protein, 76 aa, Homo sapiens
MPADFLYLSRGGVSPSCPGWSQTPELRQLPVSASQSARIIGMSHHAQPHLLFLTGIYFFASEIKHPSIWLLLLFLL

SEQ ID NO: 5281 - protein, 53 aa, Homo sapiens
MPAHCRSRRPPPRTRWPWPTVKASPRPEQSPPAHRPTRSRGPEGCPAPMSSNS

SEQ ID NO: 5282 - protein, 76 aa, Homo sapiens
MPAKSRCYPMVLTSVLFFSGISSSCSRYCQTSNPSPDASLQGLFPTLLMDISRRISCQHFKHDRSAGVNRGHKTYT

SEQ ID NO: 5283 - protein, 17 aa, Homo sapiens
MPALRRTAKSPNSCGSS

SEQ ID NO: 5284 - protein, 38 aa, Homo sapiens
MPCHFTKNCRSGRPSKGFGEGVLGSASGGRGTGVGDGG

SEQ ID NO: 5285 - protein, 68 aa, Homo sapiens [sequence omitted]

SEQ ID NO: 5286 - protein, 38 aa, Homo sapiens
MPCLSRPNLKLFSPPETFPLLCPHSYSAGCLSMAFINS

SEQ ID NO: 5287 - protein, 12 aa, Homo sapiens
MPCSLFFALLPG

SEQ ID NO: 5288 - protein, 21 aa, Homo sapiens
MPDARVDTHPPTVLNSRESGS

SEQ ID NO: 5289 - protein, 12 aa, Homo sapiens
MPDDVSGKQMLG

SEQ ID NO: 5290 - protein, 21 aa, Homo sapiens
MPDSDSLFALSCLTGVSSFQW

SEQ ID NO: 5291 - protein, 30 aa, Homo sapiens
MPEANSSGIFPSVCPLTHWFMVFLASSEAC

SEQ ID NO: 5292 - protein, 48 aa, Homo sapiens
MPEFIYEHSLKKKKKIYIYIYIYIYFLVQNSLISTSSITIEMMIGKLQ

SEQ ID NO: 5293 - protein, 11 aa, Homo sapiens
MPELSEDNHSL

SEQ ID NO: 5294 - protein, 21 aa, Homo sapiens
MPFGEQLFAARRRGPPHKPGW

SEQ ID NO: 5295 - protein, 49 aa, Homo sapiens
MPFLPRSCHSMFVSLVITMNTEIPLIRDFAFHSCSQPRSSLLIASILAG

SEQ ID NO: 5296 - protein, 17 aa, Homo sapiens
MPFVTTEYYLAIIGIKN

SEQ ID NO: 5297 - protein, 39 aa, Homo sapiens
MPGACIFLQWNWTIFSCAVKEQSNSGHFVCSDMCLSYFS

SEQ ID NO: 5298 - protein, 58 aa, Homo sapiens
MPGARPPPLIYTHARIRSSMGNRSKISVKSKSQEGSMWREVKFRPCPGNYDTQNIPLV

SEQ ID NO: 5299 - protein, 36 aa, Homo sapiens
MPGARPPPLIYTHARIRSSMGNRSKISVKSKSRGWE

SEQ ID NO: 5300 - protein, 27 aa, Homo sapiens
MPGCFVFLVETEVSPCWPGWSRTPDLR

SEQ ID NO: 5301 - protein, 11 aa, Homo sapiens
MPGCILFFLET

SEQ ID NO: 5302 - protein, 104 aa, Homo sapiens [sequence omitted]

SEQ ID NO: 5303 - protein, 13 aa, Homo sapiens
MPGLIFFFFFFFF

SEQ ID NO: 5304 - protein, 39 aa, Homo sapiens
MPGPTHNTLIPFMIYPLVHQTSQQVQKASFASWDLVWLL

SEQ ID NO: 5305 - protein, 53 aa, Homo sapiens
MPGPTLFYFILIFSLLFLRWCLIQSPRMECSGMISAHCNLCLLGSSDSPASAS

SEQ ID NO: 5306 - protein, 12 aa, Homo sapiens
MPGSPKATHISL

SEQ ID NO: 5307 - protein, 49 aa, Homo sapiens
MPGTASPPKQMTAYWSLVTTWLLAYSLAFPNMCCFSSVLQSDHNILPRQ

SEQ ID NO: 5308 - protein, 40 aa, Homo sapiens
MPGTGLSAQSPLPAVPRGSPAHPPWEAALPQNFCTFCFLL

SEQ ID NO: 5309 - protein, 45 aa, Homo sapiens
MPGTSLPVERVQTFHSVLQAQHHPTAKCLKKSLQTETRQMFDTAL

SEQ ID NO: 5310 - protein, 17 aa, Homo sapiens
MPGYIFCIFSRDGVSPC

SEQ ID NO: 5311 - protein, 32 aa, Homo sapiens
MPHEARAFGRKMKHRIHHPDASQCLVPLRNPS

SEQ ID NO: 5312 - protein, 12 aa, Homo sapiens
MPHHTQLIFVFL

SEQ ID NO: 5313 - protein, 33 aa, Homo sapiens
MPHPSSRKHNMNPPCSFSLSTEKTSSLSAPASL

SEQ ID NO: 5314 - protein, 61 aa, Homo sapiens
MPIFTPPLPSLFFLYLLALNERRLPGRATQGLQPLAISMWNSLLNLMSSFCGIVEEKALKC

SEQ ID NO: 5315 - protein, 26 aa, Homo sapiens
MPIHPQRLWAQGGGIDPGRGGPLKSH

SEQ ID NO: 5316 - protein, 30 aa, Homo sapiens
MPIIFSHYLIKKRNQATKLIFRQKKRFFFQ

SEQ ID NO: 5317 - protein, 35 aa, Homo sapiens
MPIPQVLEQALHSVVWTRQLALIIVGSGPNVSSSR

SEQ ID NO: 5318 - protein, 22 aa, Homo sapiens
MPIYYLHESNTTIENNPETKII

SEQ ID NO: 5319 - protein, 35 aa, Homo sapiens
MPKDMRSSVCVSVREKEREKERERGTKHTIVPSIS

SEQ ID NO: 5320 - protein, 16 aa, Homo sapiens
MPKISNEGSPMNREDY

SEQ ID NO: 5321 - protein, 31 aa, Homo sapiens
MPKRMWRNRNTFTLLLCWWEYKLVQPLWRTV

SEQ ID NO: 5322 - protein, 27 aa, Homo sapiens
MPLCMTNFCIFSRDGDFVMLARLVSNS

SEQ ID NO: 5323 - protein, 16 aa, Homo sapiens
MPLDTRMPIIKKIIKC

SEQ ID NO: 5324 - protein, 42 aa, Homo sapiens
MPLGASPSRAPRGTEHQGVSPRSSWEIRAGLGNGNAREATAP

SEQ ID NO: 5325 - protein, 16 aa, Homo sapiens
MPLMSGLLLTAKCIPK

SEQ ID NO: 5326 - protein, 22 aa, Homo sapiens
MPLPDGEEERKEMHRPIVAGMI

SEQ ID NO: 5327 - protein, 45 aa, Homo sapiens
MPLSLGGFQRPCTSPSRCPVCGLSEAQDPPVRPLPCLGASCSLRY

SEQ ID NO: 5328 - protein, 16 aa, Homo sapiens
MPLSPVLIIRIWDSAQ

SEQ ID NO: 5329 - protein, 55 aa, Homo sapiens
MPLSYFQRMGPINFELVYLVTALVPSDTACLASSPGSSRRTAVWISRDVMVERLL

SEQ ID NO: 5330 - protein, 14 aa, Homo sapiens
MPLSYFQRMGPINI

SEQ ID NO: 5331 - protein, 29 aa, Homo sapiens
MPLVADFYIPGLQTYILTKGGFTNTCQNR

SEQ ID NO: 5332 - protein, 26 aa, Homo sapiens
MPNASFRGLRKPWLQSLHHKQNQYFS

SEQ ID NO: 5333 - protein, 35 aa, Homo sapiens
MPNIKLRNKNKILSSPTNSFWPRVTLKTEFSAMIG

SEQ ID NO: 5334 - protein, 31 aa, Homo sapiens
MPNKFNEKREVCSTNDAGTIEHTHTNIYLSM

SEQ ID NO: 5335 - protein, 20 aa, Homo sapiens
MPNLINSTLVINGMTGVTAR

SEQ ID NO: 5336 - protein, 11 aa, Homo sapiens
MPPCLAKFLYF

SEQ ID NO: 5337 - protein, 30 aa, Homo sapiens
MPPCPANFCIFSRDGVSPHWPVWSQTPDLK

SEQ ID NO: 5338 - protein, 50 aa, Homo sapiens
MPPCPANFCILVEIGFHCLAKLVLNSRPHDPPTSASQSAGITGVSHRAQT

SEQ ID NO: 5339 - protein, 30 aa, Homo sapiens
MPPCPVNFFIFCKGGASLCCPSWSQTPGLK

SEQ ID NO: 5340 - protein, 52 aa, Homo sapiens [sequence omitted]

SEQ ID NO: 5341 - protein, 13 aa, Homo sapiens
MPPHLANFIYLFF

SEQ ID NO: 5342 - protein, 14 aa, Homo sapiens
MPPHPAIFFFFLYL

SEQ ID NO: 5343 - protein, 85 aa, Homo sapiens
MPPHPANFCVFSRERVSPCWPGWSPSLDLLIHPPRSGITGMSHHTCGFFILLFYYFYFLNHLYFYFLNHLKQTAFSGEREDTAIK

SEQ ID NO: 5344 - protein, 23 aa, Homo sapiens
MPPLIRYLKKKSLNIFTNKYLRF

SEQ ID NO: 5345 - protein, 51 aa, Homo sapiens [sequence omitted]

SEQ ID NO: 5346 - protein, 22 aa, Homo sapiens
MPPNLANFYIFSREGISPCWPG

SEQ ID NO: 5347 - protein, 24 aa, Homo sapiens
MPPPVNIITLVFYISTSKFGGTHP

SEQ ID NO: 5348 - protein, 19 aa, Homo sapiens
MPPQVSFQFSSHSTSLLKA

SEQ ID NO: 5349 - protein, 44 aa, Homo sapiens
MPPRLAKFCIFSRDGVSPYWPGWSQTPNLVIHPPQPPRVLGLQA

SEQ ID NO: 5350 - protein, 30 aa, Homo sapiens
MPPRPANFCIFSRDGFLPRWPGWSQTPDLR

SEQ ID NO: 5351 - protein, 22 aa, Homo sapiens
MPPRPANFCIFSRDGISPCWSG

SEQ ID NO: 5352 - protein, 55 aa, Homo sapiens
MPPRPANFCIFSRDRVSPCWPGWSRTAYFRRSASLGLLKCWDYRREPPRPPINHF

SEQ ID NO: 5353 - protein, 30 aa, Homo sapiens
MPPRPANFYIFSRERVSPFWPGWSRTPDLK

SEQ ID NO: 5354 - protein, 97 aa, Homo sapiens
MPQASNSIFCQISMGTSTSSPGISSIKTELLTATIVPGTNIGPFLSYSVKYFNLLQVDSKAGSHGYRFCGIILVAPSDRPVCMCSVRPVDVSPKDCN

SEQ ID NO: 5355 - protein, 35 aa, Homo sapiens
MPQEHSLLEELIVTAQLHRQVFKTWCSARRGGSCL

SEQ ID NO: 5356 - protein, 27 aa, Homo sapiens
MPQLMTTLLGFRARRSTSSMEIWSILL

SEQ ID NO: 5357 - protein, 19 aa, Homo sapiens
MPQTQVTHIHVSEPVSLSK

SEQ ID NO: 5358 - protein, 65 aa, Homo sapiens
MPRAVILLPANLRFSICPQPTRASGQWGSRGQPSKSRWMGASLCSRMLVRVARSVQVSGKLWKGS

SEQ ID NO: 5359 - protein, 68 aa, Homo sapiens
MPRAVILLPANPSICSLPIVGKLLERASAKASPHFLLLKLGAGHQVQGSKKLLQAEVGESIACLLVPR

SEQ ID NO: 5360 - protein, 93 aa, Homo sapiens
MPRAVILLPANPSICSLPIVGKLLERASAKASPHFLLLKLRFSICPQPTRASGQWGSRGQPSKSRWMGASLCSRMLVRVARSVQVSGKLWKGS

SEQ ID NO: 5361 - protein, 109 aa, Homo sapiens
MPRAVILLPANQASPAEDPSQLQGLAHPSICSLPIVGKLLERASAKASPHFLLLKLRFSICPQPTRASGQWGSRGQPSKSRWMGASLCSRMLVRVARSVQVSGKLWKGS

SEQ ID NO: 5362 - protein, 13 aa, Homo sapiens
MPRAVILLPGIPS

SEQ ID NO: 5363 - protein, 70 aa, Homo sapiens
MPRAVILLPQHLQPPHCRQAPGEGFCKGIPTLPALKAEILYLPTAYQSLRAVGLQGTAIKIQVDGGLPVL

SEQ ID NO: 5364 - protein, 31 aa, Homo sapiens
MPRDPPRGTRIFSVLKPLVGTLWTNSLNLRR

SEQ ID NO: 5365 - protein, 15 aa, Homo sapiens
MPRKFRGYCYTSLWQ

SEQ ID NO: 5366 - protein, 69 aa, Homo sapiens [sequence omitted]

SEQ ID NO: 5367 - protein, 63 aa, Homo sapiens
MPRPHPTPTTPCEEEAQAGTALGTLKLCFLEVLKSASSRTSPNTKRSVSTSSSTKDFGGLEGE

SEQ ID NO: 5368 - protein, 16 aa, Homo sapiens
MPRPQNLAPPRDRHTF

SEQ ID NO: 5369 - protein, 31 aa, Homo sapiens
MPRTCHTKAWREGKEELLLFILCLSAPFEKK

SEQ ID NO: 5370 - protein, 31 aa, Homo sapiens
MPRTSPDGAAFLIPIKLESEQKEWPTRYSTA

SEQ ID NO: 5371 - protein, 72 aa, Homo sapiens [sequence omitted]

SEQ ID NO: 5372 - protein, 30 aa, Homo sapiens
MPRTSPDGAFLIPIKLESEQKEWPTRYSTA

SEQ ID NO: 5373 - protein, 18 aa, Homo sapiens
MPRWMVFRFTLWKHMVPL

SEQ ID NO: 5374 - protein, 52 aa, Homo sapiens
MPRYFFFFVFSVETGFHHVGQAGLELLTSTDPPTLASQSAGITGVSHRTQPI

SEQ ID NO: 5375 - protein, 18 aa, Homo sapiens
MPSAGYTGTRQARVTVRL

SEQ ID NO: 5376 - protein, 31 aa, Homo sapiens
MPSALRANFIYWIYTKVGSISSIARSLLYIL

SEQ ID NO: 5377 - protein, 55 aa, Homo sapiens
MPSCPANFFFFFFLVETRLRCVAQAGLKLLAPSDPPTSVSQSAITGMNHHAWPTF

SEQ ID NO: 5378 - protein, 40 aa, Homo sapiens
MPSFTLSEFCPGHLSSDNFFFIRAIFRKTAQNLRNDPIFQ

SEQ ID NO: 5379 - protein, 23 aa, Homo sapiens
MPSGRQKAALPPGEQDAVGREVT

SEQ ID NO: 5380 - protein, 19 aa, Homo sapiens
MPSHPTNFCIFSRDRVSPC

SEQ ID NO: 5381 - protein, 29 aa, Homo sapiens
MPSICSWATLTSSVGPSRVILSSPSVNSM

SEQ ID NO: 5382 - protein, 13 aa, Homo sapiens
MPSINCFIFCERN

SEQ ID NO: 5383 - protein, 34 aa, Homo sapiens
MPSLLALGSLCTKAKRSSSAPWASQKLGAVHLFA

SEQ ID NO: 5384 - protein, 22 aa, Homo sapiens
MPSLLNLINLIPLFSDFCFLVH

SEQ ID NO: 5385 - protein, 11 aa, Homo sapiens
MPSNTSLNGYY

SEQ ID NO: 5386 - protein, 27 aa, Homo sapiens
MPSNVPPAMASQSAGITGVSHHAQPKF

SEQ ID NO: 5387 - protein, 15 aa, Homo sapiens
MPSTKTHIIIHVPSS

SEQ ID NO: 5388 - protein, 72 aa, Homo sapiens
MPSYFCIFVQTGFQHVGQAGLQLLTSGEPPASASETAGITGVSHRARRHLSTLKIQLSLAIPGVLVSRPPRT

SEQ ID NO: 5389 - protein, 20 aa, Homo sapiens
MPTCFTGYEVKFVRGIISVF

SEQ ID NO: 5390 - protein, 116 aa, Homo sapiens
MPTCPDGWFSDSHFGNTWCLSEAIVYCFLTSMISLLRILFLPKVVSHSIGLSSHLRAGPGSQVSLFPNILVYFKTARENVHLCLLKGNGLQGLLPELELSSRAILPSLPTVEIKGK

SEQ ID NO: 5391 - protein, 52 aa, Homo sapiens
MPTGGLGRVGGPGDQRKLRAPLPSPMVQPCPLPGQSGRGRPQSTQPDSALAS

SEQ ID NO: 5392 - protein, 37 aa, Homo sapiens
MPTPNTTTSWPTSRANKTSLNTAKHACSYICTLLIQQ

SEQ ID NO: 5393 - protein, 12 aa, Homo sapiens
MPTQMCPYMGAG

SEQ ID NO: 5394 - protein, 42 aa, Homo sapiens
MPTQMCPYMGALEDTLGSKSKSNQRDGPESSPQHRARPGAPC

SEQ ID NO: 5395 - protein, 33 aa, Homo sapiens
MPTSSNEMVLGEQNRTEWEENPRHPDTPLLQFC

SEQ ID NO: 5396 - protein, 44 aa, Homo sapiens
MPTYAHTKYNDKLANFKGKQNQSEHCKTCLLLYLHLTNTAMKFG

SEQ ID NO: 5397 - protein, 19 aa, Homo sapiens
MPVAAPASMPSARSLSLSR

SEQ ID NO: 5398 - protein, 11 aa, Homo sapiens
MPVEFHAHMPF

SEQ ID NO: 5399 - protein, 45 aa, Homo sapiens
MPVGTLEGLSSPTNVILSLVGISNPALPGVPGERESINIPPGTHP

SEQ ID NO: 5400 - protein, 118 aa, Homo sapiens
MPVIGSNSVDCWFSKCGPQTSSVISPESLLKMQTLRPHRRSTYRISISEDEAQQSVLINHPVDSGAHWSLRTTVVKAPDLFLLALQGGLRLGVRWEAGLCVRVCWAEAWGEGKWRVGC

SEQ ID NO: 5401 - protein, 28 aa, Homo sapiens
MPVIPAFWEAEAGRSPEVWSSRPAWNNI

SEQ ID NO: 5402 - protein, 28 aa, Homo sapiens
MPVIPALWEAEAGGLLELKLLRPAWATW

SEQ ID NO: 5403 - protein, 33 aa, Homo sapiens
MPVNNFLMMSSLRNCCFLHIRNTWERKGSQICL

SEQ ID NO: 5404 - protein, 30 aa, Homo sapiens
MPVRPANFFVFLVDMGFHHVGQDGLHLLTS

SEQ ID NO: 5405 - protein, 14 aa, Homo sapiens
MPWGGRSPEGRSSW

SEQ ID NO: 5406 - protein, 13 aa, Homo sapiens
MPWLIDSTVTTDL

SEQ ID NO: 5407 - protein, 36 aa, Homo sapiens
MPWVKCHNKFPLLEPAKSSLVVAKTKAGKGPTKELV

SEQ ID NO: 5408 - protein, 20 aa, Homo sapiens
MPWVRAELGSQMHPERSQGL

SEQ ID NO: 5409 - protein, 27 aa, Homo sapiens
MPYINHAIKLNAKFAHYCMLDVIIHAR

SEQ ID NO: 5410 - protein, 24 aa, Homo sapiens
MPYLPLLRTPWAVPWIVFQILGAS

SEQ ID NO: 5411 - protein, 17 aa, Homo sapiens
MQAPQHPAKIAKKYTFL

SEQ ID NO: 5412 - protein, 11 aa, Homo sapiens
MQCSSKHKETG

SEQ ID NO: 5413 - protein, 18 aa, Homo sapiens
MQEDSPTTVPVLQVLSPS

SEQ ID NO: 5414 - protein, 32 aa, Homo sapiens
MQEKHGDAHPPPEALGPGWGHRPRQGRTSQVA

SEQ ID NO: 5415 - protein, 22 aa, Homo sapiens
MQELKFLLIIFHFLKHPITPAF

SEQ ID NO: 5416 - protein, 41 aa, Homo sapiens
MQENLLNQGGGGCNELGRRHCRPAWVTEQGPCKNSSLQAMK

SEQ ID NO: 5417 - protein, 12 aa, Homo sapiens
MQFHLTQRNGHL

SEQ ID NO: 5418 - protein, 75 aa, Homo sapiens
MQFQFHWLLKTAICILHIWRADTYCPQPRDRNAHHSHPPPRFQLLSECCLLSAGVFRHLPNSTQVHLSLIYVLDE

SEQ ID NO: 5419 - protein, 14 aa, Homo sapiens
MQGIFLNILDTISA

SEQ ID NO: 5420 - protein, 13 aa, Homo sapiens
MQGPANTMEDKNN

SEQ ID NO: 5421 - protein, 15 aa, Homo sapiens
MQGQPVTEGDITVET

SEQ ID NO: 5422 - protein, 24 aa, Homo sapiens
MQHANFLRLKLGSSTDVKDFCVCV

SEQ ID NO: 5423 - protein, 22 aa, Homo sapiens
MQHHRAPAHPGPGRRPSLPDPL

SEQ ID NO: 5424 - protein, 172 aa, Homo sapiens [sequence omitted]

SEQ ID NO: 5425 - protein, 15 aa, Homo sapiens
MQIFLVLIKNVIGLQ

SEQ ID NO: 5426 - protein, 165 aa, Homo sapiens [sequence omitted]

SEQ ID NO: 5427 - protein, 72 aa, Homo sapiens
MQINNCFISGNIHRAFKSAGDAIVLKNSFFISGRVSLNLLCPLAYIIEVLYADPAIVIMDAGHDIITTHFLV

SEQ ID NO: 5428 - protein, 11 aa, Homo sapiens
MQITYHIASAQ

SEQ ID NO: 5429 - protein, 31 aa, Homo sapiens
MQKFEKKKQHQGLVIAQSQYYFQTKMSVMGI

SEQ ID NO: 5430 - protein, 24 aa, Homo sapiens
MQKMPDSDSLFALSCLTGVSSFQW

SEQ ID NO: 5431 - protein, 78 aa, Homo sapiens [sequence omitted]

SEQ ID NO: 5432 - protein, 45 aa, Homo sapiens [sequence omitted]

SEQ ID NO: 5433 - protein, 19 aa, Homo sapiens
MQKSSFSVGTPVIASLMKW

SEQ ID NO: 5434 - protein, 20 aa, Homo sapiens
MQKWRVNVWQCFTEQFKRSF

SEQ ID NO: 5435 - protein, 32 aa, Homo sapiens
MQKYCTYFIRVIPRYLLLLMLFIWYILKKTKH

SEQ ID NO: 5436 - protein, 60 aa, Homo sapiens
MQLCPAPGPQQPIRGSGRYHQASEPRGKPRRARVGGGLQRKPQGQRRGGMRFDQSSTPGL

SEQ ID NO: 5437 - protein, 71 aa, Homo sapiens [sequence omitted]

SEQ ID NO: 5438 - protein, 29 aa, Homo sapiens
MQLGRGTRGAWWACRSSVSTGAHGPRRPF

SEQ ID NO: 5439 - protein, 38 aa, Homo sapiens
MQLIHFSYPGDTHPCCSNRTHTLPWSTLNVNTSLRERA

SEQ ID NO: 5440 - protein, 11 aa, Homo sapiens
MQLIVTSNAYV

SEQ ID NO: 5441 - protein, 13 aa, Homo sapiens
MQLKAKFQLLMQY

SEQ ID NO: 5442 - protein, 78 aa, Homo sapiens
MQLLLCQARMVVSRTGSSLSPQVPWPSTGHWGKDLISRLRVLSSIPYHPAPSHLLKQSFLFQVIQVIQPGIKSTWYLG

SEQ ID NO: 5443 - protein, 35 aa, Homo sapiens
MQLLLCQARMVVSRTGSSLSPQVPWPSTPTCVSPL

SEQ ID NO: 5444 - protein, 24 aa, Homo sapiens
MQLMLNKYSFFCYSKKNPSFVINL

SEQ ID NO: 5445 - protein, 12 aa, Homo sapiens
MQLSVDIFALPK

SEQ ID NO: 5446 - protein, 18 aa, Homo sapiens
MQLTPVKQWPLISTFLSL

SEQ ID NO: 5447 - protein, 65 aa, Homo sapiens
MQLVGDTRLKADRIRKYQVPGMWLQSPLDAIILGHQMPTQAVGRHRPWTLHNQFQLCPLLRDLGL

SEQ ID NO: 5448 - protein, 14 aa, Homo sapiens
MQLWRSRGSLTAHP

SEQ ID NO: 5449 - protein, 13 aa, Homo sapiens
MQMSRTFKEERRI

SEQ ID NO: 5450 - protein, 56 aa, Homo sapiens
MQNCSFQADYPSLQVHPPLHLCENGWWAIVEGGHMQSPFLALTQVPGAPAIVTADC

SEQ ID NO: 5451 - protein, 11 aa, Homo sapiens
MQNLHIIACLM

SEQ ID NO: 5452 - protein, 74 aa, Homo sapiens
MQNSATAFRKSGSSSKGYHSTQQFHSLYVPKRNKNTYSLKNLSQMFMAALFIEARKWKQFKCLSTNEWTNVVRP

SEQ ID NO: 5453 - protein, 124 aa, Homo sapiens
MQPHGDVLRDLDILLQTTDKLAVHLAGLGGTETAALGFAQPVLQDAAGLAGLVQLLSQLLQLIHVLLHIDVPHLQHLGPQLLNLVLLCRSSFYLLTGRELPDLCFPHLDPRADHTRLEITVLRS

SEQ ID NO: 5454 - protein, 36 aa, Homo sapiens
MQRHGKSIVCTKRNYPFNLCQFVVHDIGQSTCKLFL

SEQ ID NO: 5455 - protein, 22 aa, Homo sapiens
MQRNWKPHTAGGNVKRCSHVGK

SEQ ID NO: 5456 - protein, 34 aa, Homo sapiens
MQRRCVLGFSIFHITITICAGLVFSYMLFPKSNS

SEQ ID NO: 5457 - protein, 11 aa, Homo sapiens
MQRYYLHHFQS

SEQ ID NO: 5458 - protein, 26 aa, Homo sapiens
MQSAHLSLLKCWDYRCEPPRLARICL

SEQ ID NO: 5459 - protein, 26 aa, Homo sapiens
MQSVLRNCYIQYHCLCHMRQEHLDVK

SEQ ID NO: 5460 - protein, 33 aa, Homo sapiens
MQTLSMLWASSKTTTALRASSLDTRSAILGSRR

SEQ ID NO: 5461 - protein, 46 aa, Homo sapiens
MQTSSGAGQYNKLQRLSQDPVVGLMVLLITSFDVYLSQNVLFDSFR

SEQ ID NO: 5462 - protein, 31 aa, Homo sapiens
MQVCLGISCLFHRCCTLFLYRYHPVLITVAT

SEQ ID NO: 5463 - protein, 53 aa, Homo sapiens
MQVLRSRQMEEKNIYASVSESQVVVLALPFSKVYSQKQVAFLLRCRAHWNPRG

SEQ ID NO: 5464 - protein, 91 aa, Homo sapiens
MQWGPATLARHCQVAAVQTQDRKLRPAWGLCSRRPQGTALFSLVPPSRPDLPARLQPGASLACERTDWGRRAASLVKRPVYHSSRINHSPC

SEQ ID NO: 5465 - protein, 19 aa, Homo sapiens
MQWWLCRYSYYVSESVQPV

SEQ ID NO: 5466 - protein, 21 aa, Homo sapiens
MQYHARLIFVVLGERGFHHVG

SEQ ID NO: 5467 - protein, 81 aa, Homo sapiens
MQYKRINFLGFFHTQIRIMFLETRFWRFALDRQGRARSTGLSGGPSRGPGRRTGGLPGAPHAPLTHWPRRLRCHGDRARTY

SEQ ID NO: 5468 - protein, 65 aa, Homo sapiens
MQYTWLTPGRIVLLFSLVHPYICSKLSLFQLIPLLLSPVGVGVLETYSLGLSFLFHVLAGVVPTH

SEQ ID NO: 5469 - protein, 16 aa, Homo sapiens
MRAAILVSIHSRRKPW

SEQ ID NO: 5470 - protein, 24 aa, Homo sapiens
MRANRLAADQTDTAFLVKGTVRRN

SEQ ID NO: 5471 - protein, 23 aa, Homo sapiens
MRCGVTKGQKTRGRNKGPKNPKP

SEQ ID NO: 5472 - protein, 14 aa, Homo sapiens
MRCIHFIYLIKCLF

SEQ ID NO: 5473 - protein, 14 aa, Homo sapiens
MRCLWNLWSMLIST

SEQ ID NO: 5474 - protein, 19 aa, Homo sapiens
MRDPLHAQNTSSNGDQIST

SEQ ID NO: 5475 - protein, 56 aa, Homo sapiens
MREAALQHAVPGDLTQVAGAQLPHLSCNGIFFHKCFLRVVELHGVIGGKRNMQSLV

SEQ ID NO: 5476 - protein, 126 aa, Homo sapiens [sequence omitted]

SEQ ID NO: 5477 - protein, 54 aa, Homo sapiens
MREVQGGPRALLLPLKSYHINALYVYSFTTLIFFKYLRALDHFNNASGRQGRPC

SEQ ID NO: 5478 - protein, 46 aa, Homo sapiens
MRFCRIGQAGLELLTSSDLPALASQSTGITGMSHRTQSKMEYDIRL

SEQ ID NO: 5479 - protein, 24 aa, Homo sapiens
MRFHHAGQAGLELLTSSDPPTTAS

SEQ ID NO: 5480 - protein, 16 aa, Homo sapiens
MRFHHVGQAGLELLTS

SEQ ID NO: 5481 - protein, 16 aa, Homo sapiens
MRFHHVGQDGLDLLTS

SEQ ID NO: 5482 - protein, 75 aa, Homo sapiens
MRFHNVGQHGLELRTLHDPPASAPQSAGITDVSHCAQPAFLIFEKCESGNILLPFPTHIPGELCSRYMGKIFTVN

SEQ ID NO: 5483 - protein, 65 aa, Homo sapiens
MRFRHVGQTVLELLASSNLPASASQSVGITGEPLRPAMGTYFMWIKLRREKDMFFSTWKVFFKLV

SEQ ID NO: 5484 - protein, 33 aa, Homo sapiens
MRGGNTWSYMTICHRGQERGHQGTRADRKEMWI

SEQ ID NO: 5485 - protein, 29 aa, Homo sapiens
MRHDTQLIFFFFFCIFSRDGVLPCWPGWS

SEQ ID NO: 5486 - protein, 12 aa, Homo sapiens
MRHHAPLILYFK

SEQ ID NO: 5487 - protein, 30 aa, Homo sapiens
MRHHAQLFLYFCTDRVSACWPGWSPTPDLR

SEQ ID NO: 5488 - protein, 12 aa, Homo sapiens
MRHHAQLIFLYF

SEQ ID NO: 5489 - protein, 11 aa, Homo sapiens
MRHHAQLIFVF

SEQ ID NO: 5490 - protein, 30 aa, Homo sapiens [sequence omitted]

SEQ ID NO: 5491 - protein, 51 aa, Homo sapiens [sequence omitted]

SEQ ID NO: 5492 - protein, 35 aa, Homo sapiens
MRHHAQLIFVFLVETGFYHVGQAGLELLTSGDLPA

SEQ ID NO: 5493 - protein, 29 aa, Homo sapiens
MRHHARLIFVLLVETGFHQVIQAALELLI

SEQ ID NO: 5494 - protein, 81 aa, Homo sapiens [sequence omitted]

SEQ ID NO: 5495 - protein, 11 aa, Homo sapiens
MRHHARPILYF

SEQ ID NO: 5496 - protein, 79 aa, Homo sapiens [sequence omitted]

SEQ ID NO: 5497 - protein, 12 aa, Homo sapiens
MRHHAWLIFLYF

SEQ ID NO: 5498 - protein, 31 aa, Homo sapiens
MRHHAWLIFVFFSRDGVSPCWSGWSRTPDLR

SEQ ID NO: 5499 - protein, 62 aa, Homo sapiens
MRHHAWLIFVFLVEMGFHHVGQAGLELLTSTDLPTSASHSARITGMSQHAWPGSSFKASKPK

SEQ ID NO: 5500 - protein, 17 aa, Homo sapiens
MRHHDGTQGLFMKLSNQ

SEQ ID NO: 5501 - protein, 12 aa, Homo sapiens
MRHHPRLILYVW

SEQ ID NO: 5502 - protein, 24 aa, Homo sapiens
MRHHTRQIFVFLVEGVSPYWSGWS

SEQ ID NO: 5503 - protein, 58 aa, Homo sapiens
MRHQAHLISVILVETGFHHVGQAGLKLLTSGDPPASASQSAGIIGMSHHTQPKGLLKK

SEQ ID NO: 5504 - protein, 15 aa, Homo sapiens
MRHRFIFYFCWSVLF

SEQ ID NO: 5505 - protein, 15 aa, Homo sapiens
MRHRKDLTQNNKSHI

SEQ ID NO: 5506 - protein, 38 aa, Homo sapiens
MRHRWGRTPGIHSHSRQETGRGLNNMAPEFEIFHPKHH

SEQ ID NO: 5507 - protein, 27 aa, Homo sapiens
MRIFVSEFYYFPFLHYAVSFLLTLGLV

SEQ ID NO: 5508 - protein, 18 aa, Homo sapiens
MRIISCMPDDVSGKQMLG

SEQ ID NO: 5509 - protein, 11 aa, Homo sapiens
MRIRSTDKSGK

SEQ ID NO: 5510 - protein, 25 aa, Homo sapiens
MRKHWQAFLRGISTPRPSSLALKHR

SEQ ID NO: 5511 - protein, 16 aa, Homo sapiens
MRKIFQPDGHSKKLEL

SEQ ID NO: 5512 - protein, 28 aa, Homo sapiens
MRKKDSAVCAFMSCAEHISHAEEVRSRL

SEQ ID NO: 5513 - protein, 21 aa, Homo sapiens
MRKKKNPQNSSLQCKELLLER

SEQ ID NO: 5514 - protein, 25 aa, Homo sapiens
MRKLRLSTASWKPVQLTPVPSGELL

SEQ ID NO: 5515 - protein, 14 aa, Homo sapiens
MRKNFFLSISLLIL

SEQ ID NO: 5516 - protein, 21 aa, Homo sapiens
MRKSLEHGEHGRLWLMRSSVP

SEQ ID NO: 5517 - protein, 27 aa, Homo sapiens
MRLHSHFGLKIKQFSHTKWFDILFFGK

SEQ ID NO: 5518 - protein, 33 aa, Homo sapiens
MRLKLFHISCHFYLFLCESLAGFCGSFFLSTSL

SEQ ID NO: 5519 - protein, 24 aa, Homo sapiens
MRLLALEKLNFVQSLGEPAVYEHS

SEQ ID NO: 5520 - protein, 32 aa, Homo sapiens
MRLLALEKLNFVQSLGEPAVYEHSCKRKCTGG

SEQ ID NO: 5521 - protein, 15 aa, Homo sapiens
MRLLCDSCISSLQGH

SEQ ID NO: 5522 - protein, 89 aa, Homo sapiens
MRLRGSKEGPFPAEGSMLWPTCSVSGSCPVLQPLSSLMLLPKPQLVRRGQSLLGNSNHPTWVTADLEEHRPSPLRGWKIKVVWSKENGK

SEQ ID NO: 5523 - protein, 16 aa, Homo sapiens
MRLSLVPAFTPSRFWT

SEQ ID NO: 5524 - protein, 53 aa, Homo sapiens
MRMCSKLSSTKKTKSSVTIKKVVFRSIFNGSGVIDNSYIKSFFGKLFISFHFH

SEQ ID NO: 5525 - protein, 66 aa, Homo sapiens
MRMEGNWNPHIAWWECKIVQLLSVSLAVPQKVITAPNNSIPCMCPRETKTHIHSKTYHKCLWQHYS

SEQ ID NO: 5526 - protein, 12 aa, Homo sapiens
MRMLSTSSQEKR

SEQ ID NO: 5527 - protein, 24 aa, Homo sapiens
MRMQRNWKPHTAGGNVKRCSHVGK

SEQ ID NO: 5528 - protein, 30 aa, Homo sapiens
MRMRKKDSAVCAFMSCAEHISHAEEVRSRL

SEQ ID NO: 5529 - protein, 49 aa, Homo sapiens
MRNHGQLIFGFFLRRSLTLSPGWSAVVRSQLTATSTSRVQAILLPQPPK

SEQ ID NO: 5530 - protein, 20 aa, Homo sapiens
MRNILQDRPSIRPHTNSQKH

SEQ ID NO: 5531 - protein, 12 aa, Homo sapiens
MRNKEHILFFFF

SEQ ID NO: 5532 - protein, 17 aa, Homo sapiens
MRNPVSKDERILVIQGM

SEQ ID NO: 5533 - protein, 23 aa, Homo sapiens
MRPITPSRTFLISIRFWGWTNWS

SEQ ID NO: 5534 - protein, 11 aa, Homo sapiens
MRPSVQREFLA

SEQ ID NO: 5535 - protein, 92 aa, Homo sapiens
MRQAGVIIVTKARPVIVTRTGWGRDHTLNQVSTRCGPFIGATKRGQPAMWPRHLTPGTPTWRREMKELTFPQGLSQTSRPLSGESACVCTCV

SEQ ID NO: 5536 - protein, 20 aa, Homo sapiens
MRQSMRAAILVSIHSRRKPW

SEQ ID NO: 5537 - protein, 16 aa, Homo sapiens
MRQVICYNFTVEPKHI

SEQ ID NO: 5538 - protein, 30 aa, Homo sapiens
MRRARRLDSSSLVVLRLSSLRLEGEDGRLS

SEQ ID NO: 5539 - protein, 20 aa, Homo sapiens
MRRELQFFRLSKPTAGCTAD

SEQ ID NO: 5540 - protein, 21 aa, Homo sapiens
MRRGILSWILASESSVICFSQ

SEQ ID NO: 5541 - protein, 32 aa, Homo sapiens
MRRITKAFTGTFIPIIMFSWALRSCPTWHITI

SEQ ID NO: 5542 - protein, 47 aa, Homo sapiens
MRRSQDPGRVITVSGDQPALRPGEEVAPGYWLRAASPRLGLCCSCTS

SEQ ID NO: 5543 - protein, 46 aa, Homo sapiens
MRRVLTPVHKDLLHQIEVKGHLLILASNTLLSPKALGCIWNSCTQL

SEQ ID NO: 5544 - protein, 91 aa, Homo sapiens
MRRWAGYPGCTTCRAITSTSITAQPSCWNTWITELLPEAMPPVRPTRNIFQERELSARLRSQELQNHWRAGQVWPMGAVHQRSARRTCRET

SEQ ID NO: 5545 - protein, 126 aa, Homo sapiens
MRRWAGYPGCTTCRAITSTSITAQPSCWNTWITELLPEAMPPVRPTRNIFQERELSARLRSQELQNHWRAGQVWPMGAVHQRSARRTLKAVASGWVRWLTPVIPTLSEAEAGGSPEVRSSGPAWPT

SEQ ID NO: 5546 - protein, 105 aa, Homo sapiens
MRRWAGYPGCTTCRAITSTSITAQPSCWNTWITELLPEAMPPVRPTRNIFQERELSARLRSQELQNHWRAGQVWPMGAVHQRSARRTLRPFFPQSVAECLGFRVS

SEQ ID NO: 5547 - protein, 99 aa, Homo sapiens
MRRWAGYPGCTTCRAITSTSITAQPSCWNTWITELLPEAMPPVRPTRNIFQERELSARLRSQELQNHWRAGQVWPMGAVHQRSARRTLVLAAYDALNTS

SEQ ID NO: 5548 - protein, 98 aa, Homo sapiens
MRRWAGYPGCTTCRAITSTSITAQPSCWNTWITELLPEAMPPVRPTRNIFQERELSARLRSQELQNHWRAGQVWPMGAVHQRSARRTQRLRRGPGLRL

SEQ ID NO: 5549 - protein, 90 aa, Homo sapiens
MRRWAGYPGCTTCRAITSTSITAQPSCWNTWITELLPEAMPPVRPTRNIFQERELSARLRSQELQNHWRAGQVWPMGAVHQRSARRTRET

SEQ ID NO: 5550 - protein, 31 aa, Homo sapiens
MRSFLAVSASCSTSPTREERAAKRSFIWAIS

SEQ ID NO: 5551 - protein, 15 aa, Homo sapiens
MRSKGNFYTAGGNAN

SEQ ID NO: 5552 - protein, 38 aa, Homo sapiens
MRSKGVVSESRKDFGTYRFDKNPSLFLPDLYTLIWGRV

SEQ ID NO: 5553 - protein, 35 aa, Homo sapiens
MRSLFTTRKFSMVFPLAKTMSPVSFTASGKISFTS

SEQ ID NO: 5554 - protein, 59 aa, Homo sapiens
MRSLSLSRDVISAFSRSISISPSSICCRSCLATVFSVSTICSRCRYFCINASCSVARVL

SEQ ID NO: 5555 - protein, 11 aa, Homo sapiens
MRSLTVNSIIY

SEQ ID NO: 5556 - protein, 67 aa, Homo sapiens
MRSSLVTEKERWEYKTCQVQKPTSLSMSLLHKCFQISLLENFLHVRIYPNLKWKLKRKKDPLYRNYI

SEQ ID NO: 5557 - protein, 27 aa, Homo sapiens
MRSTCCIGFVYSVLERNFHEWMYSILM

SEQ ID NO: 5558 - protein, 13 aa, Homo sapiens
MRSVRSSFLVHLW

SEQ ID NO: 5559 - protein, 15 aa, Homo sapiens
MRTARSPPVTHTRRR

SEQ ID NO: 5560 - protein, 20 aa, Homo sapiens
MRTPANSRFTVVERWDKALI

SEQ ID NO: 5561 - protein, 12 aa, Homo sapiens
MRTWSFSKSLKK

SEQ ID NO: 5562 - protein, 79 aa, Homo sapiens
MRTWTGPAFFTGSSSSELHSYVFSENPPQLFLSLRFLAMVVQELVAVRRCHCARCLLRGRRLLAVGGSVPALGAVRSDS

SEQ ID NO: 5563 - protein, 131 aa, Homo sapiens
MRTWTGPAFFTGSSSSELHSYVFSENPPQLFLSLRFLAMVVQELVAVRRCHCARCLLRGRRLLAVGGSVPALGAVRSDSEDVAVAPLQAADKDTEMLPNMLFCPRAHTEEVVEPEPVCDPFVLLLRNSWSH

SEQ ID NO: 5564 - protein, 21 aa, Homo sapiens
MRVAQEQTQNANSDVSLHGRS

SEQ ID NO: 5565 - protein, 27 aa, Homo sapiens
MRVAQEQTQNANSDVSLHGRWVRGEGR

SEQ ID NO: 5566 - protein, 24 aa, Homo sapiens
MRVICIFFRPIFSQLSLFPYIPNI

SEQ ID NO: 5567 - protein, 11 aa, Homo sapiens
MRVKNRANGTW

SEQ ID NO: 5568 - protein, 12 aa, Homo sapiens
MRVQSHKYSVPS

SEQ ID NO: 5569 - protein, 18 aa, Homo sapiens
MRVRKPGFQSQLYYLLAV

SEQ ID NO: 5570 - protein, 34 aa, Homo sapiens
MRWLAGADCPSLKSLPSSWLGQRFTTSVTCSAFL

SEQ ID NO: 5571 - protein, 22 aa, Homo sapiens
MRWPGGELSQDRCFKPSLQGWY

SEQ ID NO: 5572 - protein, 21 aa, Homo sapiens
MRYHYKPIRMAKIQNTGNIKC

SEQ ID NO: 5573 - protein, 13 aa, Homo sapiens
MRYSYLTSVTFLI

SEQ ID NO: 5574 - protein, 29 aa, Homo sapiens
MSADRWPLGSPRTGALFYSSPCSQHCHNG

SEQ ID NO: 5575 - protein, 34 aa, Homo sapiens
MSADRWPLGSPRTGALFYSSPCSQHSITELFQSW

SEQ ID NO: 5576 - protein, 113 aa, Homo sapiens
MSAFAPNDKGFCGISGVTPAGQSCGGSVSRHHVEQCCSQPSLPDHRNTHTELLKQLSTSTPRVYPDPRTPGRHQNSNRIKTHKHTHWSIRCGLFFFFLKKDSSKALKSILSRL

SEQ ID NO: 5577 - protein, 31 aa, Homo sapiens [sequence omitted]

SEQ ID NO: 5578 - protein, 65 aa, Homo sapiens
MSAKSRGTMTASGCQPPPPPAWLAFPAPGQPETFMVPLTPRLPGLLQPSGSPRAGSSRGCGRCNS

SEQ ID NO: 5579 - protein, 41 aa, Homo sapiens
MSAPNFSTIVLDLFCCNYIFITSVLFFFFFFRDQVSLCCLG

SEQ ID NO: 5580 - protein, 27 aa, Homo sapiens
MSARLVSNSRPQVIHPPQPPKMLGLQA

SEQ ID NO: 5581 - protein, 13 aa, Homo sapiens
MSASGTYPSSPGL

SEQ ID NO: 5582 - protein, 27 aa, Homo sapiens
MSATSTDKLAVAHSEGEPPSRAVTTNS

SEQ ID NO: 5583 - protein, 36 aa, Homo sapiens
MSAWLFQGCQGRDSQELRLSGGCQTGLGGKTSQGEG

SEQ ID NO: 5584 - protein, 33 aa, Homo sapiens
MSAWSFCRLLLMFSISSWALFCRMSMLESREEK

SEQ ID NO: 5585 - protein, 17 aa, Homo sapiens
MSCAEHISHAEEVRSRL

SEQ ID NO: 5586 - protein, 96 aa, Homo sapiens
MSCGPEKVWPTGTGFGSRSCFSCHPLQTQRLNLCDISHHQVGVSTHIWPCAGGVSFGSSYILNRIHTYRDVPAVHILQDMENDTRYQAHSGQKQLF

SEQ ID NO: 5587 - protein, 29 aa, Homo sapiens
MSCIFSISYFLSTFMANIFPVFAPVTFRT

SEQ ID NO: 5588 - protein, 13 aa, Homo sapiens
MSCIFSISYYHCL

SEQ ID NO: 5589 - protein, 23 aa, Homo sapiens
MSCIFSISYYHCLSIAPFTKYPK

SEQ ID NO: 5590 - protein, 80 aa, Homo sapiens
MSCIFSISYYHCPLLQLILRARVLWLVQVYVKHSCHVLSFPVSEVRGWVKAVPPPSSPHGPGPAAATTAAAAITGCLGSV

SEQ ID NO: 5591 - protein, 11 aa, Homo sapiens
MSCILPYLRSL

SEQ ID NO: 5592 - protein, 146 aa, Homo sapiens
MSCKFSRLVSTSSCPSPEFSSSPLSSTPSSSGLRPLLDLFDVFLFPSEVISISSGLPPSSSIAFFSRSIKTLLLPLESTFRFLSSARRSITRRSLRRRVPVSDEAELRAAAPAAPESPRPDRVSAIPGTLAPPPTFHRTGPVLSGS

SEQ ID NO: 5593 - protein, 53 aa, Homo sapiens
MSCLHIWDLGFPNGHCLCSNCEPYSYLDTSSVLRLRIPSQMKKGELYLHQVFQ

SEQ ID NO: 5594 - protein, 14 aa, Homo sapiens
MSCLLQGKTLWRDW

SEQ ID NO: 5595 - protein, 30 aa, Homo sapiens
MSCSALHRSCNCCSFFAESCSNVALAVFSS

SEQ ID NO: 5596 - protein, 49 aa, Homo sapiens
MSCWKASSKNFCRSFSFICWVCSISRTFWACSASSSALKVSSSFLLFFL

SEQ ID NO: 5597 - protein, 45 aa, Homo sapiens
MSDFSCGHCLVLGIARELNDQGLVMLLGIGELRLYFPLVIISKHL

SEQ ID NO: 5598 - protein, 17 aa, Homo sapiens
MSEQCKWMKFIVPVLKI

SEQ ID NO: 5599 - protein, 131 aa, Homo sapiens
MSFFCSQYEVRHWPSRGRLPEVGQRGVTCLGQDTQHPSGDCMKCQDVLLSQCHGKEAGFQCRLEPGVTHFPGLPEDQCAGSNQHHTQHSRHLGSCEATHWGPCPAQTSLELSHGLSPFPSLLPVRAGGPFP

SEQ ID NO: 5600 - protein, 93 aa, Homo sapiens
MSFFCSQYEVRHWPSRGRLPWRKPSAHSSVCRTRLWAFCTTAGSRAYQLLSTSCSRFRARRVLPVYTKSRWSLSFWTKPSGTVTSSTSTFSGS

SEQ ID NO: 5601 - protein, 15 aa, Homo sapiens
MSFFNSSELSREITD

SEQ ID NO: 5602 - protein, 27 aa, Homo sapiens
MSFFSSQFPFFSPCNPNALGGQGERIA

SEQ ID NO: 5603 - protein, 36 aa, Homo sapiens
MSFPPNFFFCWLKLSMMTPMKRLRVKKEPKMMKMTK

SEQ ID NO: 5604 - protein, 59 aa, Homo sapiens
MSFPSFKNLHFLPIAESLLSDSDSLRDTEDSPGSGPISSCQPSPQPQPSMFPTHVLQPY

SEQ ID NO: 5605 - protein, 61 aa, Homo sapiens
MSFSLSILCCKRSFILTTSCCRKSSLSGSDSEGGGVIVGIQILLKGFPSRRYDPLNVTYSS

SEQ ID NO: 5606 - protein, 179 aa, Homo sapiens
MSFSNVLSHMALELQCVQIRYLHNLPVFLALLFHVLGLSLFSLCRSKSRPLSFPSLVFSSILSFTLYFSLYFFPRAISSGIGGGGLGVRGPFFLLWLVFEFLCWSNRGEDTADVFLSFLLAEDDFGLDFRFGDLLDFLREGDGDNFDLTTSGETSFLMIISSLFSMFSCSSFINSLCIF

SEQ ID NO: 5607 - protein, 93 aa, Homo sapiens
MSFTSTFTWKTCSGLSTITSRWMLHSALCPHSSSRSIREFTNKMPFCRFTSRRSPCVLDATRNRRCTSSASSSPRSCAMRPTKVPCLASSETE

SEQ ID NO: 5608 - protein, 76 aa, Homo sapiens
MSFTSTSTWKTCSGLSTITSRWILHSALRPHSFSRSIREFTNKMPFCRFTSRRSPCLLDATRNRRGTSSASSSPRS

SEQ ID NO: 5609 - protein, 28 aa, Homo sapiens
MSFYCPNLNPGSQPRLPSLLQYFCPMDH

SEQ ID NO: 5610 - protein, 50 aa, Homo sapiens
MSGDNFFGTILVGRRWGCCSIPCNTQGWGCGAHNKELSGNRAGAVNPALQ

SEQ ID NO: 5611 - protein, 46 aa, Homo sapiens
MSGLGAGGRLPTARSEPRRWAPFRPCRQTASRWPRAAPPCSRPPAS

SEQ ID NO: 5612 - protein, 13 aa, Homo sapiens
MSGLLLTAKCIPK

SEQ ID NO: 5613 - protein, 38 aa, Homo sapiens
MSGPFVISVEISSMVQVSASQGLLCCRACTWLRRLWAF

SEQ ID NO: 5614 - protein, 48 aa, Homo sapiens [sequence omitted]

SEQ ID NO: 5615 - protein, 11 aa, Homo sapiens
MSHHAQLILYF

SEQ ID NO: 5616 - protein, 31 aa, Homo sapiens
MSHHVAQADFKLLNSWAQVILPPQAPKVLPL

SEQ ID NO: 5617 - protein, 43 aa, Homo sapiens
MSHPHPSTGPFYYRPRRHRKCKEGLEPQKPGASGVRCPDSQEP

SEQ ID NO: 5618 - protein, 47 aa, Homo sapiens
MSIESPELAAAMHFAAYHPICLAWVHSLICCQTGLSCQDVVQMSPAA

SEQ ID NO: 5619 - protein, 60 aa, Homo sapiens
MSILKAGVLSQPHLYIQRLAPCLVNRYVICVCCKTHLCRTQTGDLILSSISRVCFIFPRQ

SEQ ID NO: 5620 - protein, 19 aa, Homo sapiens
MSINIECLLISTLNCFMST

SEQ ID NO: 5621 - protein, 21 aa, Homo sapiens
MSIRARSLVLASCIRSQCSFS

SEQ ID NO: 5622 - protein, 24 aa, Homo sapiens
MSISFFKAYWTIKHSEGNEGWTGR

SEQ ID NO: 5623 - protein, 21 aa, Homo sapiens
MSITIPVALLFILSGLALSLL

SEQ ID NO: 5624 - protein, 69 aa, Homo sapiens [sequence omitted]

SEQ ID NO: 5625 - protein, 16 aa, Homo sapiens
MSKCPEKKSALIESLE

SEQ ID NO: 5626 - protein, 15 aa, Homo sapiens
MSKRCCCPLFLDGEV

SEQ ID NO: 5627 - protein, 39 aa, Homo sapiens
MSKVCNENKSAIKIYAFFLFFFFSIFYTNSTNSIAHNNK

SEQ ID NO: 5628 - protein, 22 aa, Homo sapiens
MSLAHLDPLACLGHKPVRHQPP

SEQ ID NO: 5629 - protein, 28 aa, Homo sapiens
MSLAILSNEGRLPLTKTIQRLVCMMVDQ

SEQ ID NO: 5630 - protein, 41 aa, Homo sapiens
MSLATRERYSSELKPILQGRFRRLLGLLWNPPLGREPSVLS

SEQ ID NO: 5631 - protein, 58 aa, Homo sapiens
MSLATRERYSSERAGSHLECPLFITKGTGRLGVMRRWPEGTRPVRGSRGWAAVSLHYL

SEQ ID NO: 5632 - protein, 46 aa, Homo sapiens
MSLATRERYSSRALPGSWPSGKHGSPYPCWIYCVPHQLSSWHPRFD

SEQ ID NO: 5633 - protein, 73 aa, Homo sapiens
MSLATRERYSSRVLAFRKTWLSISLLDLLCATPAFLMASSLWSQLLGRLTWEDRLSPGGGGCSEPQSRHCTSA

SEQ ID NO: 5634 - protein, 37 aa, Homo sapiens
MSLFTKRTKFSSGHMGLGERLWWSWQKEVWNVTSTPL

SEQ ID NO: 5635 - protein, 65 aa, Homo sapiens
MSLGLVDCCRSLREPSTNARVTHLPTLNPRIHATKQDSFLHGMCRFQMTQHPMQKTLEFFLGTRL

SEQ ID NO: 5636 - protein, 53 aa, Homo sapiens
MSLGLVDCCRSLREPSTNARVTHLPTLNPRIHATKQDSFLHGMCRFQMTQHRM

SEQ ID NO: 5637 - protein, 15 aa, Homo sapiens
MSLGSRCWDDLHCAG

SEQ ID NO: 5638 - protein, 60 aa, Homo sapiens
MSLIRSQIGLLHRPIYNGWISSEVPPSTEERRSSPVTFFSFCIEVSPLSVFSFRELSFVP

SEQ ID NO: 5639 - protein, 26 aa, Homo sapiens
MSLKGQNLLEKNTHVCICIFISVVFF

SEQ ID NO: 5640 - protein, 55 aa, Homo sapiens
MSLKMNHQHLSLEVWLFICIPTAFPSIPLQQPIDIVTPNHVTKHGSQHFPLLKPN

SEQ ID NO: 5641 - protein, 24 aa, Homo sapiens
MSLQYLKKMVISHLHSYLTPSSSC

SEQ ID NO: 5642 - protein, 38 aa, Homo sapiens
MSLRLLWLAQGCLHSSTTTESALAGMKPRRKTLRQPQL

SEQ ID NO: 5643 - protein, 13 aa, Homo sapiens
MSLRVRSPVKRSG

SEQ ID NO: 5644 - protein, 28 aa, Homo sapiens
MSLSLTQAYRFSLHELIFVSYEDAFLWG

SEQ ID NO: 5645 - protein, 24 aa, Homo sapiens
MSLSLTQAYRFSLHELSKDEDRVV

SEQ ID NO: 5646 - protein, 33 aa, Homo sapiens
MSLSSPNPHPLVRTDRSSHTQWSQPLGRGTCSR

SEQ ID NO: 5647 - protein, 74 aa, Homo sapiens
MSLSSSLGATVWVDWMRSLSLSRDVISAFSRSISISPSSICCRSCLATVFSVSTICSRCRYFCINASCSVARVL

SEQ ID NO: 5648 - protein, 45 aa, Homo sapiens
MSMEIKLLRDQLELRSSTPGSRLPPTTPHWHRLKQRLVNYNQVDR

SEQ ID NO: 5649 - protein, 149 aa, Homo sapiens
MSMMLSGARRKAHLLSACRERSRNSKENQATHTVSSTNRLRHLGEHSPRSSSARMSGMVLRQRPTAVTATKDTDTQAKSLPASPECGLSTTSRRRRRPRCSRPRGPRARAGLPCAPRSVGPARASAASSSRRRRRRRQQRSRRASSMPQ

SEQ ID NO: 5650 - protein, 148 aa, Homo sapiens
MSMSCKFSRLVSTSSCPSPEFSSSPLSSTPSSSGLRPLLDLFDVFLFPSEVISISSGLPPSSSIAFFSRSIKTLLLPLESTFRFLSSARRSITRRSLRRRVPVSDEAELRAAAPAAPESPRPDRVSAIPGTLAPPPTFHRTGPVLSGS

SEQ ID NO: 5651 - protein, 13 aa, Homo sapiens
MSNADIFWCRPVQ

SEQ ID NO: 5652 - protein, 42 aa, Homo sapiens
MSNEISTTTCTCVIFTHSKRRFFRWYNDRICAVLFLSHSNTG

SEQ ID NO: 5653 - protein, 88 aa, Homo sapiens
MSNESQLRSLIRSSKKLSVHAWCMAAQSKHRSFGSFPVLTLVARREKKHKLLFLQLVLHTKMSTHIKTETTFEKIHRTLQTPLLFVEL

SEQ ID NO: 5654 - protein, 50 aa, Homo sapiens
MSNHTRLIFVFLVETGFHYVGQAGLELLTSSDPPAFASRSAGITGVSHCA

SEQ ID NO: 5655 - protein, 12 aa, Homo sapiens
MSNLILKILPTF

SEQ ID NO: 5656 - protein, 106 aa, Homo sapiens
MSPFSSKTSVPKTSTMRRWAGYPGCTTCRAITSTSITAQPSCWNTWITELLPEAMPPVRPTRNIFQERELSARLRSQELQNHWRAGQVWPMGAVHQRSARRTCRET

SEQ ID NO: 5657 - protein, 141 aa, Homo sapiens
MSPFSSKTSVPKTSTMRRWAGYPGCTTCRAITSTSITAQPSCWNTWITELLPEAMPPVRPTRNIFQERELSARLRSQELQNHWRAGQVWPMGAVHQRSARRTLKAVASGWVRWLTPVIPTLSEAEAGGSPEVRSSGPAWPT

SEQ ID NO: 5658 - protein, 120 aa, Homo sapiens
MSPFSSKTSVPKTSTMRRWAGYPGCTTCRAITSTSITAQPSCWNTWITELLPEAMPPVRPTRNIFQERELSARLRSQELQNHWRAGQVWPMGAVHQRSARRTLRPFFPQSVAECLGFRVS

SEQ ID NO: 5659 - protein, 114 aa, Homo sapiens
MSPFSSKTSVPKTSTMRRWAGYPGCTTCRAITSTSITAQPSCWNTWITELLPEAMPPVRPTRNIFQERELSARLRSQELQNHWRAGQVWPMGAVHQRSARRTLVLAAYDALNTS

SEQ ID NO: 5660 - protein, 113 aa, Homo sapiens
MSPFSSKTSVPKTSTMRRWAGYPGCTTCRAITSTSITAQPSCWNTWITELLPEAMPPVRPTRNIFQERELSARLRSQELQNHWRAGQVWPMGAVHQRSARRTQRLRRGPGLRL

SEQ ID NO: 5661 - protein, 105 aa, Homo sapiens
MSPFSSKTSVPKTSTMRRWAGYPGCTTCRAITSTSITAQPSCWNTWITELLPEAMPPVRPTRNIFQERELSARLRSQELQNHWRAGQVWPMGAVHQRSARRTRET

SEQ ID NO: 5662 - protein, 65 aa, Homo sapiens
MSPINFFFHKNQFLSRFCHVHKRLWHQLAFVLSPPPLFFFLVFFGNLFVGKISYFSNLHYPHTQL

SEQ ID NO: 5663 - protein, 55 aa, Homo sapiens
MSPIRPPEPEPPEPLPPPAPELFFTLPAMAWAGSEPRRVRRLGSTASEGEKQGVK

SEQ ID NO: 5664 - protein, 16 aa, Homo sapiens
MSPLSMQCSSKHKETG

SEQ ID NO: 5665 - protein, 53 aa, Homo sapiens
MSPLSSVFTDLTNMGAGSKGFGMNCAVASVNSSTALAGISTRVKIKACSSSPS

SEQ ID NO: 5666 - protein, 22 aa, Homo sapiens
MSPMVGITGLLDFTVVHSSGGS

SEQ ID NO: 5667 - protein, 16 aa, Homo sapiens
MSPNASGNFGRFVFSN

SEQ ID NO: 5668 - protein, 79 aa, Homo sapiens [sequence omitted]

SEQ ID NO: 5669 - protein, 67 aa, Homo sapiens
MSPSAVAGDSSSLWKRLGRPAGGSRHWKVTAVPASAFISLEKPSEEPSKQRPMAISLAKRGLWSVTV

SEQ ID NO: 5670 - protein, 65 aa, Homo sapiens
MSPVTSWALSVGCLGTAHGRNVSRKRRGLVFNPLLMHFITFGFSGSLMFLRDPLVQDPVISAHVW

SEQ ID NO: 5671 - protein, 68 aa, Homo sapiens
MSQGPGKGAPGDQGGQKRNVDLMVSNRGTADKRVIVHLLDGHFCGLFFFFFFFEIEICSCCPGWSVVP

SEQ ID NO: 5672 - protein, 57 aa, Homo sapiens
MSQHLQGVGSSGSIWAPWSLISMFCNASGISTLLCSVFSVLHSARHSLCLVFGSGSS

SEQ ID NO: 5673 - protein, 84 aa, Homo sapiens
MSQHLQGVGSSGSIWAPWSLISMFCNASGISTLLCSVFSVLHSARHSLCLVFGSGSSEAGGNCTLQLTRVTWLLLTRAAGQVLH

SEQ ID NO: 5674 - protein, 12 aa, Homo sapiens
MSQSRPFPQFLC

SEQ ID NO: 5675 - protein, 47 aa, Homo sapiens
MSRKWIMSLATRERYSSELKPILQGRFRRLLGLLWNPPLGREPSVLS

SEQ ID NO: 5676 - protein, 64 aa, Homo sapiens
MSRKWIMSLATRERYSSERAGSHLECPLFITKGTGRLGVMRRWPEGTRPVRGSRGWAAVSLHYL

SEQ ID NO: 5677 - protein, 52 aa, Homo sapiens
MSRKWIMSLATRERYSSRALPGSWPSGKHGSPYPCWIYCVPHQLSSWHPRFD

SEQ ID NO: 5678 - protein, 79 aa, Homo sapiens
MSRKWIMSLATRERYSSRVLAFRKTWLSISLLDLLCATPAFLMASSLWSQLLGRLTWEDRLSPGGGGCSEPQSRHCTSA

SEQ ID NO: 5679 - protein, 51 aa, Homo sapiens
MSRLPSSVNRYISRNSRKSISWRWGKAEKPTRMNSDMEVWFSPSMTATPSW

SEQ ID NO: 5680 - protein, 26 aa, Homo sapiens
MSRLVSSSRAQAILLPQPPQVLGLQA

SEQ ID NO: 5681 - protein, 91 aa, Homo sapiens
MSRRAWFSAFGRPFFFPSVLSLAGLPGSKQRGAWPGTVCPPRTTGIPIFGGSCSIGSRTSFRLPSFPGPLLLDPGSRRPPTQKGSVIFCNF

SEQ ID NO: 5682 - protein, 100 aa, Homo sapiens
MSRRAWFSAFGRPFFFPSVLSLAGLPGSKQRGAWPGTVCPPRTTGIPIFGGSCSIGSRTSFRLPSFPGPLLLDPGSRRPPTQKGSVISAAPSGAAAGPGR

SEQ ID NO: 5683 - protein, 101 aa, Homo sapiens
MSRRAWFSAFGRPFFFPSVLSLAGLPGSKQRGAWPGTVCPPRTTGIPIFGGSCSIGSRTSFRLPSFPGPLLLDPGSRRPPTQKGSVISVTWGRERARGAGL

SEQ ID NO: 5684 - protein, 11 aa, Homo sapiens
MSRTFKEERRI

SEQ ID NO: 5685 - protein, 78 aa, Homo sapiens
MSRTHLSTRWLVHTTGSMFCVSQRARRSWRASLLKFTWYSSSIPSRMLTWWNFLDTFRCFSRSRFIREFSIRPSTRWF

SEQ ID NO: 5686 - protein, 46 aa, Homo sapiens
MSSDPPTSASQSAGITGVSHRAWPVLTLKVGIQRQKRGGRLRGSWG

SEQ ID NO: 5687 - protein, 46 aa, Homo sapiens
MSSILFSLSVLPNIHLLQFCLSSPLFCNTLLPPSVPLHCFLCCFPP

SEQ ID NO: 5688 - protein, 51 aa, Homo sapiens
MSSSISLTASVSMSSSVEALEVPAESEGDVAGGDKESSGDSGSSGGRLPPL

SEQ ID NO: 5689 - protein, 13 aa, Homo sapiens
MSSSSSNSARFLS

SEQ ID NO: 5690 - protein, 90 aa, Homo sapiens
MSSSSVRVIQLGALPVVHPTEPLEVVIVAAPRPVHWHHGEVRHRAGSAPPHPPSQPPAAVPAAVPAAPGRHAPPARIPPRCAHFLRPPPG

SEQ ID NO: 5691 - protein, 39 aa, Homo sapiens
MSSSVEALEVPAESEGDVAGGDKESSGDSGSSGGRLPPL

SEQ ID NO: 5692 - protein, 16 aa, Homo sapiens
MSSTISTPPMTWMKKI

SEQ ID NO: 5693 - protein, 16 aa, Homo sapiens
MSSTISTPPTTWMKKI

SEQ ID NO: 5694 - protein, 17 aa, Homo sapiens
MSSTSSRSARWILCRSQ

SEQ ID NO: 5695 - protein, 15 aa, Homo sapiens
MSSVHEVGCITGEAP

SEQ ID NO: 5696 - protein, 17 aa, Homo sapiens
MSSWIRVGPNPVWLSSL

SEQ ID NO: 5697 - protein, 13 aa, Homo sapiens
MSSWSVYLSCCAY

SEQ ID NO: 5698 - protein, 24 aa, Homo sapiens
MSTCRCFNSFVSDPSDRLPLLCAI

SEQ ID NO: 5699 - protein, 35 aa, Homo sapiens
MSTLKQLRLSRCGLPIDPQMNGNKIEDLSPEPHYP

SEQ ID NO: 5700 - protein, 51 aa, Homo sapiens
MSTNRQMNQRDTSSVHSTPRRSIRAPTAGSFARTSSPRTSWSVFRPSMAGL

SEQ ID NO: 5701 - protein, 13 aa, Homo sapiens
MSTQFQSLKHSSG

SEQ ID NO: 5702 - protein, 52 aa, Homo sapiens
MSTRASSSPRLASLSSTSPWTAPSPSLLLAAFSWLWDMALLCVGCLRPPCSH

SEQ ID NO: 5703 - protein, 28 aa, Homo sapiens
MSTTQTWNRTPYMLLKKGKKQKTVATLL

SEQ ID NO: 5704 - protein, 19 aa, Homo sapiens
MSVECFSKVTLFQLWPFQC

SEQ ID NO: 5705 - protein, 49 aa, Homo sapiens
MSVISANISKNLCRTISHLQALSSRTLLSFKAISPLPKGFTVLKLELSF

SEQ ID NO: 5706 - protein, 42 aa, Homo sapiens
MSVLIVVWSNGQALRWSLFRHILQTVWPQPKLMGFRIVSSKV

SEQ ID NO: 5707 - protein, 21 aa, Homo sapiens
MSVMRIISCMPDDVSGKQMLG

SEQ ID NO: 5708 - protein, 12 aa, Homo sapiens
MSVPQVLYSILV

SEQ ID NO: 5709 - protein, 36 aa, Homo sapiens
MSVPVYCAHCWAWIICAIEHSSSTNAGVTRCSNHFS

SEQ ID NO: 5710 - protein, 17 aa, Homo sapiens
MSWEGALLLISQRKQGP

SEQ ID NO: 5711 - protein, 78 aa, Homo sapiens
MSYFIPNTGNLYLFSFLPSSYFSFYLQLLLIFFFFFFVERGVLYVPRLVSNSWPQAILLSLPAKCWNYQHEPPHWANL

SEQ ID NO: 5712 - protein, 21 aa, Homo sapiens
MSYLQEIKSLGISKGSEGLTP

SEQ ID NO: 5713 - protein, 37 aa, Homo sapiens
MTALCNMPRTCHTKAWREGKEELLLFILCLSAPFEKK

SEQ ID NO: 5714 - protein, 12 aa, Homo sapiens
MTALEHSGPRGT

SEQ ID NO: 5715 - protein, 57 aa, Homo sapiens
MTASGCQPPPPPAWLAFPAPGQPETFMVPLTPRLPGLLQPSGSPRAGSSRGCGRCNS

SEQ ID NO: 5716 - protein, 15 aa, Homo sapiens
MTAVVFLQLPVDMSE

SEQ ID NO: 5717 - protein, 60 aa, Homo sapiens
MTCCLWALAALQSAGSQWTGTAPCPAGRLPQKTSAAPSASFAGCAPFPGPSGRALHLVQL

SEQ ID NO: 5718 - protein, 21 aa, Homo sapiens
MTCDFAVTSFPNSLHFAPSPC

SEQ ID NO: 5719 - protein, 19 aa, Homo sapiens
MTCGHPGMLSSLSSSHYVR

SEQ ID NO: 5720 - protein, 39 aa, Homo sapiens
MTCTITTFFKLSFQLLSCYASLYMSCQIVLINPENSIHL

SEQ ID NO: 5721 - protein, 47 aa, Homo sapiens
MTCVLSSTSHTPRPLCPISLFLYVCIFAQSSAATHLLAINKEPFSSP

SEQ ID NO: 5722 - protein, 89 aa, Homo sapiens
MTDLRQNHSQYHTEWVNLEAFPLKAGTRQGCPLSPLLFKIVLKVLARAIRQEKEIKGIQIGKQEVKLSLFADDMNCIYREPHHLSPKSP

SEQ ID NO: 5723 - protein, 43 aa, Homo sapiens
MTDQKCPAFARCVCGRCPPFSASCFLSQLSSEASPCADSCFTL

SEQ ID NO: 5724 - protein, 70 aa, Homo sapiens
MTDQKCPAFARCVCGRCPPFSASCFLSQLSSEASPCADSCFTLGKEEGMVVVRANAMVSFTCWKASEMHL

SEQ ID NO: 5725 - protein, 62 aa, Homo sapiens
MTDQKCPAFARCVCGRCPPFSASCFLSQLSSEASPCADSCFTLNFWLQCNSLIDFKLKKRNK

SEQ ID NO: 5726 - protein, 136 aa, Homo sapiens
MTDQKCPAFARCVCGRCPPFSASCFLSQLSSEASPCADSCFTLSSRGCSRGVPATGRPAAKTAQQLSVLPNSRGCSAPVRGTDGRELLVAGPVLGACTQGPRSGTQPRPHAPGSPATPTRGGVLPTPPGGRWTVLL

SEQ ID NO: 5727 - protein, 96 aa, Homo sapiens
MTEDGYRSTDSSCQSSTESCTNCEPITEVVDAIPHDHHPGYISYSCFFQIGSRMTGAMGMMRMLVVPLVIMLPQHSFVLAVVVMCSSMEIMLMNGM

SEQ ID NO: 5728 - protein, 70 aa, Homo sapiens
MTFCKLSPCDSRQASKLFLFSFLFLFNNVVRSIFFLMECKKAISMLHFGYEGLSSSSQQSCIAESQIILN

SEQ ID NO: 5729 - protein, 72 aa, Homo sapiens
MTFCKLSPCDSRQASKLFLFSFLFLFNNVVRSIFFLMECKKAISMLHFGYEGLSSSSQQSCIAESQIILNLE

SEQ ID NO: 5730 - protein, 29 aa, Homo sapiens
MTFCKLSPCDSRQASKLFLFSFRERSGSA

SEQ ID NO: 5731 - protein, 11 aa, Homo sapiens
MTFCKLSPKYM

SEQ ID NO: 5732 - protein, 67 aa, Homo sapiens
MTFGLVISYLVNGKRRRTWASCSASESPKYKMLPPHKPRKLDGCSSPTSHPRMLSSHQGPVAATPPG

SEQ ID NO: 5733 - protein, 34 aa, Homo sapiens
MTFNCVQEGSSLNTPTLHPQSYKLRYFLTVTHPI

SEQ ID NO: 5734 - protein, 12 aa, Homo sapiens
MTGEGKLPPQVK

SEQ ID NO: 5735 - protein, 32 aa, Homo sapiens [sequence omitted]

SEQ ID NO: 5736 - protein, 23 aa, Homo sapiens
MTGMTILYGMKHVLIQREVVLPK

SEQ ID NO: 5737 - protein, 13 aa, Homo sapiens
MTGPLKLQIDVEF

SEQ ID NO: 5738 - protein, 33 aa, Homo sapiens
MTGSGSKTGAFSLMGVLDGQSPSSDKNRLWYAS

SEQ ID NO: 5739 - protein, 39 aa, Homo sapiens
MTGSGSKTGAFSLMGVLDGQSPYFSEMKILSASFFPNSL

SEQ ID NO: 5740 - protein, 15 aa, Homo sapiens
MTHTPRPPKVLGLQA

SEQ ID NO: 5741 - protein, 109 aa, Homo sapiens
MTHYPATQRSAPTSPAAGSQEWQGHWESGRQHRVSSFTKTEKRGSSRVGVGAQRTGRKGGRRRYDITPAPTVGTQTQASWESLGTVKNPHLSITLPRGGVGYVHIPIIP

SEQ ID NO: 5742 - protein, 24 aa, Homo sapiens
MTICHRGQERGHQGTRADRKEMWI

SEQ ID NO: 5743 - protein, 20 aa, Homo sapiens
MTILYGMKHVLIQREVVLPK

SEQ ID NO: 5744 - protein, 13 aa, Homo sapiens
MTITKKSKNNRCW

SEQ ID NO: 5745 - protein, 16 aa, Homo sapiens
MTKNPKANATKTKINR

SEQ ID NO: 5746 - protein, 43 aa, Homo sapiens
MTKPDDGRDGKPAFTQPRPAQPRERTNSQLVDRLLLSLCHLVV

SEQ ID NO: 5747 - protein, 25 aa, Homo sapiens
MTKTQKPMATKAQIEKWDLIKLKSF

SEQ ID NO: 5748 - protein, 22 aa, Homo sapiens
MTKVKTQRATTGPSALGSSPEL

SEQ ID NO: 5749 - protein, 33 aa, Homo sapiens
MTLFGNGLCRYNQINMMSSWIRVGPNPVWLSSL

SEQ ID NO: 5750 - protein, 28 aa, Homo sapiens
MTLKLNCLYVLPSSIGLTNMYAYMFPKS

SEQ ID NO: 5751 - protein, 28 aa, Homo sapiens
MTLKSISQSPLLGFIFKYLLGIFTYVTQ

SEQ ID NO: 5752 - protein, 33 aa, Homo sapiens
MTLKVIHISEGFPTFLTFIRFLSSVSPTMHSKV

SEQ ID NO: 5753 - protein, 11 aa, Homo sapiens
MTLLQLLGVFL

SEQ ID NO: 5754 - protein, 12 aa, Homo sapiens
MTLLSIAGIIFR

SEQ ID NO: 5755 - protein, 34 aa, Homo sapiens
MTLSKIYYLITHLRNKRRFSKCGVSNPNWRVKFI

SEQ ID NO: 5756 - protein, 22 aa, Homo sapiens
MTLSVIELKYLFYSSLNLTAKG

SEQ ID NO: 5757 - protein, 18 aa, Homo sapiens
MTMLSNCPKYFYTRIISH

SEQ ID NO: 5758 - protein, 11 aa, Homo sapiens
MTMTYFPENGP

SEQ ID NO: 5759 - protein, 23 aa, Homo sapiens
MTNFCIFSRDGDFVMLARLVSNS

SEQ ID NO: 5760 - protein, 35 aa, Homo sapiens
MTNYLELYRLHGSSIPVVNLYKSGHLHTSLIRTTA

SEQ ID NO: 5761 - protein, 49 aa, Homo sapiens
MTPANSRLTEIMGTDSGLVSGTILAELDPLDMYISVVISGILVGVIDSP

SEQ ID NO: 5762 - protein, 30 aa, Homo sapiens
MTPCVTGIQIRILGRVICPFFYQYSQTPTT

SEQ ID NO: 5763 - protein, 42 aa, Homo sapiens
MTPHFITLVNLAPVALPGCPVQITALSDTHFYSSQNCQAKFM

SEQ ID NO: 5764 - protein, 15 aa, Homo sapiens
MTPLILAIIQLHLDL

SEQ ID NO: 5765 - protein, 20 aa, Homo sapiens
MTPMKRLRVKKEPKMMKMTK

SEQ ID NO: 5766 - protein, 12 aa, Homo sapiens
MTQHPDVSARRN

SEQ ID NO: 5767 - protein, 45 aa, Homo sapiens
MTRGLSITPGDFVSLGMIQRTKWGWVERKLVISLFRFSLCRADTV

SEQ ID NO: 5768 - protein, 28 aa, Homo sapiens
MTRKKVTLWNTICGQLMPTLWIIHEAAG

SEQ ID NO: 5769 - protein, 33 aa, Homo sapiens
MTRTGQLGRREGGGRGSGRREGGGSAEGGGPGR

SEQ ID NO: 5770 - protein, 82 aa, Homo sapiens
MTRTGQLGRREGGGRGSGRREGGGSAEGGGPGRGRCGGRGPGPGPGPGQCREGLVGRPQSRRRAGRGGRSGREERGRAGADP

SEQ ID NO: 5771 - protein, 46 aa, Homo sapiens
MTSCTPFLDSSLLCLGSCPWNSFFFSCSFPDMSWTLVLIQQCCSRP

SEQ ID NO: 5772 - protein, 68 aa, Homo sapiens
MTSEPMKAQDSTLEKLSLGPNVYTLASTTFFAFIMTSKCPTGAVIPVVPKRILERGAIPLHFLPVARF

SEQ ID NO: 5773 - protein, 61 aa, Homo sapiens
MTSEPMKAQDSTLEKLSLGPNVYTLASTTVARRERPRPRPHSDPAAAAAVSPARVNRHLRP

SEQ ID NO: 5774 - protein, 52 aa, Homo sapiens
MTSLPGPSMPWSSAIPLPQSISAGEREEFNPRRAISSGLARTEVKIMGTGSC

SEQ ID NO: 5775 - protein, 35 aa, Homo sapiens
MTSPYIKERFSWRVYIRLHLSLMHSDMKSPTEFSQ

SEQ ID NO: 5776 - protein, 27 aa, Homo sapiens
MTSQWSLPHTTGLTPKYVFHMGCFICG

SEQ ID NO: 5777 - protein, 19 aa, Homo sapiens
MTSRDRTILNSCPVSKQDL

SEQ ID NO: 5778 - protein, 167 aa, Homo sapiens [sequence omitted]

SEQ ID NO: 5779 - protein, 23 aa, Homo sapiens
MTTLLGFRARRSTSSMEIWSILL

SEQ ID NO: 5780 - protein, 24 aa, Homo sapiens
MTTPTIDAFYLPVIFCEVICPEYN

SEQ ID NO: 5781 - protein, 12 aa, Homo sapiens
MTTQVCVLPQSR

SEQ ID NO: 5782 - protein, 14 aa, Homo sapiens
MTTSWPDWGSLTNW

SEQ ID NO: 5783 - protein, 37 aa, Homo sapiens
MTTVSYTQPSGTPFTLITDFKITKGSQAFKCSTLIFD

SEQ ID NO: 5784 - protein, 19 aa, Homo sapiens
MTVNFMCQFDWAKGCPNIW

SEQ ID NO: 5785 - protein, 38 aa, Homo sapiens
MTVNTKLKLILGSWSIHEATLNSDDSKQGSNICLFKKY

SEQ ID NO: 5786 - protein, 39 aa, Homo sapiens
MTVSLVILSDNWSQKLIKHFHLHYPLKLKFLYLLFCHSG

SEQ ID NO: 5787 - protein, 69 aa, Homo sapiens [sequence omitted]

SEQ ID NO: 5788 - protein, 84 aa, Homo sapiens [sequence omitted]

SEQ ID NO: 5789 - protein, 15 aa, Homo sapiens
MTYCIFPSEKLSCLL

SEQ ID NO: 5790 - protein, 12 aa, Homo sapiens
MTYSSLVLCKAH

SEQ ID NO: 5791 - protein, 21 aa, Homo sapiens
MVAAYMIYLFPSFYFQLAFII

SEQ ID NO: 5792 - protein, 16 aa, Homo sapiens
MVADACNPSILGGRGR

SEQ ID NO: 5793 - protein, 21 aa, Homo sapiens
MVAGFGLGLYMFCYCPGSLAE

SEQ ID NO: 5794 - protein, 22 aa, Homo sapiens
MVAGHSQDGAGCSQDGSKPFVL

SEQ ID NO: 5795 - protein, 26 aa, Homo sapiens
MVAGRALMGQLHSSRWHLRLLSLSSL

SEQ ID NO: 5796 - protein, 75 aa, Homo sapiens
MVAGYSKLLGLWVVTPISMEPDHLSTSLSIRISNISLSRRGRLVMTTPLLNSSRGRRRSAVLLLLLSLMRVPHFS

SEQ ID NO: 5797 - protein, 27 aa, Homo sapiens
MVAWLVSNSWPQVIRPPRPPKVLGLQA

SEQ ID NO: 5798 - protein, 36 aa, Homo sapiens
MVAWSPSPGCFSECWAALPGPLRMRTSSPAPGQALP

SEQ ID NO: 5799 - protein, 17 aa, Homo sapiens
MVCLLLSVLSLFHSLLL

SEQ ID NO: 5800 - protein, 17 aa, Homo sapiens
MVCLLLSVLSLFYSLLL

SEQ ID NO: 5801 - protein, 18 aa, Homo sapiens
MVCPPFSMHVVLHSSIHF

SEQ ID NO: 5802 - protein, 39 aa, Homo sapiens
MVDCCILGELLQDSQFYPTIYLILGDFNVPEDESPTSQP

SEQ ID NO: 5803 - protein, 54 aa, Homo sapiens
MVDILAGSMMSDFSCGHCLVLGIARELNDQGLVMLLGIGELRLYFPLVIISKHL

SEQ ID NO: 5804 - protein, 20 aa, Homo sapiens
MVDPTAQRFCTKRKMRTILT

SEQ ID NO: 5805 - protein, 101 aa, Homo sapiens
MVEGQLLAGRVARQGILLPLPQGEPPSRSQATGCRAPELHPAAVVAGTQEGWLWRAGLGRLGRARRWGTPSLPARPLVSTRSPSLLRCPCCSAGCGRGSSR

SEQ ID NO: 5806 - protein, 302 aa, Homo sapiens
MVEMVSRHLLSPALLSLGSGRILSWWIGCFCLFAILWFRVFWASASVIEVAAVPTLRWLLTLGLISLIFFIFFIAVLSRLSLARRAPAESWSISPIHILPHWSTLFSCTLVVSTLHHFSLHRRVGILWSTPIGSPHVVRWEPSPAVGPALLGLAFGSTLRSLVLFPTLTILVILLVIAWRTPTTWIASIMVTVCCIFTALNWNTTRTCNICCLRTLFSFNNIKLHSLSISYTAKVLPGVILLYGSLVYKYIFLGVIPAILFQIRPAWASGPSHAGRRGHLTALSLHRPGAGPRSRRRRRTRG

SEQ ID NO: 5807 - protein, 355 aa, Homo sapiens
MVEMVSRHLLSPALLSLGSGRILSWWIGCFCLFAILWFRVFWASASVIEVAAVPTLRWLLTLGLISLIFFIFFIAVLSRLSLARRAPAESWSISPIHILPHWSTLFSCTLVVSTLHHFSLHRRVGILWSTPIGSPHVVRWEPSPAVGPALLGLAFGSTLRSLVLFPTLTILVILLVIAWRTPTTWIASIMVTVCCIFTALNWNTTRTCNICCLRTLFSFNNIKLHSLSISYTAKVLPGVILLYGSLVYKYIFLGVIPVDETISVPYIEPFYCSQNLRCDDLLVPAGRRRRCEAARATAPCAAARSAGLGVGGAEGGGGGGGGGRLLGLGLAAHGCGDGDWGRLRQLRLLPGCDGN

SEQ ID NO: 5808 - protein, 45 aa, Homo sapiens
MVFLIHPAILGPYSKIRKASLGEVIACRKISKHCSLFDAKKVNRS

SEQ ID NO: 5809 - protein, 24 aa, Homo sapiens
MVFPLAKTMSPVSFTASGKISFTS

SEQ ID NO: 5810 - protein, 14 aa, Homo sapiens
MVFRFTLWKHMVPL

SEQ ID NO: 5811 - protein, 52 aa, Homo sapiens
MVFWANTVRRKAQAPPPRTHLPPRKMLYSSGAARQLASLCTGSVKAHLNPRK

SEQ ID NO: 5812 - protein, 20 aa, Homo sapiens
MVGAGGGPRSGSSARGAGAE

SEQ ID NO: 5813 - protein, 46 aa, Homo sapiens
MVGAGGGPRSGSSARGAGAEVGIRRGARVSLRCWGGRGRLPRTQAP

SEQ ID NO: 5814 - protein, 157 aa, Homo sapiens [sequence omitted]

SEQ ID NO: 5815 - protein, 20 aa, Homo sapiens
MVGAGLAEVTGRGLSSTATS

SEQ ID NO: 5816 - protein, 59 aa, Homo sapiens
MVGATVVCLQHESEAVNKSHHTEDGKKKNTVWIHNGILLLLTKPSNCHLSCCENKNNSP

SEQ ID NO: 5817 - protein, 14 aa, Homo sapiens
MVGGSLECRSYRLQ

SEQ ID NO: 5818 - protein, 19 aa, Homo sapiens
MVGITGLLDFTVVHRSGGS

SEQ ID NO: 5819 - protein, 19 aa, Homo sapiens
MVGITGLLDFTVVHSSGGS

SEQ ID NO: 5820 - protein, 21 aa, Homo sapiens
MVGSCGSGCGCGRDWLRFWVP

SEQ ID NO: 5821 - protein, 48 aa, Homo sapiens
MVHEPGMSNEISTTTCTCVIFTHSKRRFFRWYNDRICAVLFLSHSNTG

SEQ ID NO: 5822 - protein, 31 aa, Homo sapiens
MVHHTVALVQEFHHFSAQKWQHQKFSCDEKN

SEQ ID NO: 5823 - protein, 21 aa, Homo sapiens
MVIFDNEDLDWSCLFHWLLLF

SEQ ID NO: 5824 - protein, 16 aa, Homo sapiens
MVIHCLTRSPKVLKQN

SEQ ID NO: 5825 - protein, 46 aa, Homo sapiens
MVIIKKSGNNRMLFWMPKRMWRNRNTFTLLLCWWEYKLVQPLWRTV

SEQ ID NO: 5826 - protein, 97 aa, Homo sapiens
MVILSCWPGWSRTPDLKSSIRPGLPNCWNYRLTPLHEMCCSGSGFCIVLRGFFHWFVFVFVCFRRQKSCLDRFTKHISPSPCSQQLSVSMLSSFKDS

SEQ ID NO: 5827 - protein, 23 aa, Homo sapiens
MVKALFAPKGTTPSICANLLSMI

SEQ ID NO: 5828 - protein, 35 aa, Homo sapiens
MVKIYISKQKLVPFLMAKQGKHPHQNNLNNKDPHY

SEQ ID NO: 5829 - protein, 17 aa, Homo sapiens
MVKRKTQSGFTMAYYFC

SEQ ID NO: 5830 - protein, 19 aa, Homo sapiens
MVKSLFGMSQSRPFPQFLC

SEQ ID NO: 5831 - protein, 57 aa, Homo sapiens
MVKTVFVLLSSSFHLSSNKSIYGGFFYQFFCLIPTATTWLFSAISAYIVIFRNIALW

SEQ ID NO: 5832 - protein, 22 aa, Homo sapiens
MVLFGIFFRYQGIPTGFINRIF

SEQ ID NO: 5833 - protein, 26 aa, Homo sapiens
MVLGEQNRTEWEENPRHPDTPLLQFC

SEQ ID NO: 5834 - protein, 24 aa, Homo sapiens
MVLLPALVDVFDQLLGSLLQDVNA

SEQ ID NO: 5835 - protein, 84 aa, Homo sapiens [sequence omitted]

SEQ ID NO: 5836 - protein, 13 aa, Homo sapiens
MVLMKDSCSTCFP

SEQ ID NO: 5837 - protein, 67 aa, Homo sapiens
MVLTSVLFFSGISSSCSRYCQTSNPSPDASLQGLFPTLLMDISRRISCQHFKHDRSAGVNRGHKTYT

SEQ ID NO: 5838 - protein, 11 aa, Homo sapiens
MVMACLPSSSP

SEQ ID NO: 5839 - protein, 53 aa, Homo sapiens
MVNALSPLVSTSKYNFFLLAKVSWYFCDANKNLLGAPRDEVSLQWDGKLPGRD

SEQ ID NO: 5840 - protein, 18 aa, Homo sapiens
MVNDDIPVVTSTHHRFDP

SEQ ID NO: 5841 - protein, 83 aa, Homo sapiens
MVPDWRLVMVAGYSKLLGLWVVTPISMEPDHLSTSLSIRISNISLSRRGRLVMTTPLLNSSRGRRRSAVLLLLLSLMRVPHFS

SEQ ID NO: 5842 - protein, 15 aa, Homo sapiens
MVPHLEQHCSVFLHV

SEQ ID NO: 5843 - protein, 18 aa, Homo sapiens
MVPIISIRINNTCKSPTI

SEQ ID NO: 5844 - protein, 31 aa, Homo sapiens
MVPLGILCKHKTLCRSLCSLSLGKCMVKPME

SEQ ID NO: 5845 - protein, 11 aa, Homo sapiens
MVPRDRALSLP

SEQ ID NO: 5846 - protein, 21 aa, Homo sapiens
MVQGVAQGSVAVNREQDGDPD

SEQ ID NO: 5847 - protein, 20 aa, Homo sapiens
MVQKKEKPELQKSQIYLMKN

SEQ ID NO: 5848 - protein, 26 aa, Homo sapiens
MVQYFKDGFHQAGSLVQVIFCVGNLF

SEQ ID NO: 5849 - protein, 17 aa, Homo sapiens
MVREVNLKATYRDPVFS

SEQ ID NO: 5850 - protein, 53 aa, Homo sapiens
MVRGASCFGGLGKRLMSGPFVISVEISSMVQVSASQGLLCCRACTWLRRLWAF

SEQ ID NO: 5851 - protein, 74 aa, Homo sapiens
MVRLCGKKRVCVIVCMCVFLCVSVCVMVCLCGGEGMCVIVCLCVCLCMSVCVCVCNGVSLWQGGAVCVFLCMCV

SEQ ID NO: 5852 - protein, 12 aa, Homo sapiens
MVRMLTVHRTLQ

SEQ ID NO: 5853 - protein, 14 aa, Homo sapiens
MVRMLTVHRTLQLT

SEQ ID NO: 5854 - protein, 15 aa, Homo sapiens
MVRMLTVHRTLQLTM

SEQ ID NO: 5855 - protein, 17 aa, Homo sapiens
MVRMLTVHRTLQLTMRM

SEQ ID NO: 5856 - protein, 13 aa, Homo sapiens
MVRPPRPPKVLGL

SEQ ID NO: 5857 - protein, 15 aa, Homo sapiens
MVRSLRPPKVLGLQV

SEQ ID NO: 5858 - protein, 93 aa, Homo sapiens
MVRSPWTLLSLVRILTVPLIFSFSPTTKMKLYCANCAFRIFLFNVQPGSRSMSAMNLASWNCCRTFWAYSSQVGPTGTTITWRGDSQKGHLPP

SEQ ID NO: 5859 - protein, 35 aa, Homo sapiens
MVRVQLTRFPTKPTLLHLWSTFFESNHMEINLLFI

SEQ ID NO: 5860 - protein, 18 aa, Homo sapiens
MVSAHGSHIYRPGSRLWH

SEQ ID NO: 5861 - protein, 54 aa, Homo sapiens
MVSAITPGFFWICILLSMSISTFTVPVVMGITSGPRISGITALFGISAIISHLP

SEQ ID NO: 5862 - protein, 21 aa, Homo sapiens
MVSFHFVLTWWERLKSSFCLI

SEQ ID NO: 5863 - protein, 21 aa, Homo sapiens
MVSHFVVSFILLFFSCYSIYF

SEQ ID NO: 5864 - protein, 156 aa, Homo sapiens [sequence omitted]

SEQ ID NO: 5865 - protein, 23 aa, Homo sapiens
MVSIALLGLPKCWDYRHESPRLA

SEQ ID NO: 5866 - protein, 11 aa, Homo sapiens
MVSIVCWTQRS

SEQ ID NO: 5867 - protein, 72 aa, Homo sapiens
MVSLNNEPRSHNNIRTIGCKYSSHTGMGFASSTELCYPGSIASDGLLRNDLSTEANKLNWFLIETSCKLFLP

SEQ ID NO: 5868 - protein, 23 aa, Homo sapiens
MVSNSGPCMIRPPRPPKVLGLQM

SEQ ID NO: 5869 - protein, 23 aa, Homo sapiens
MVSNSQPQVIRLPRPLKALGLQG

SEQ ID NO: 5870 - protein, 24 aa, Homo sapiens
MVSPGNHGVLWPCRGSFLRPQPEV

SEQ ID NO: 5871 - protein, 57 aa, Homo sapiens
MVSPGVNVLVLFRVNGLFIFQPFHLGSRDSLWWAAVQYNHAFNGNFPSLWVLFKVFP

SEQ ID NO: 5872 - protein, 15 aa, Homo sapiens
MVSPLYTEANQISPT

SEQ ID NO: 5873 - protein, 299 aa, Homo sapiens
MVSRHLLSPALLSLGSGRILSWWIGCFCLFAILWFRVFWASASVIEVAAVPTLRWLLTLGLISLIFFIFFIAVLSRLSLARRAPAESWSISPIHILPHWSTLFSCTLVVSTLHHFSLHRRVGILWSTPIGSPHVVRWEPSPAVGPALLGLAFGSTLRSLVLFPTLTILVILLVIAWRTPTTWIASIMVTVCCIFTALNWNTTRTCNICCLRTLFSFNNIKLHSLSISYTAKVLPGVILLYGSLVYKYIFLGVIPAILFQIRPAWASGPSHAGRRGHLTALSLHRPGAGPRSRRRRRTRG

SEQ ID NO: 5874 - protein, 352 aa, Homo sapiens
MVSRHLLSPALLSLGSGRILSWWIGCFCLFAILWFRVFWASASVIEVAAVPTLRWLLTLGLISLIFFIFFIAVLSRLSLARRAPAESWSISPIHILPHWSTLFSCTLVVSTLHHFSLHRRVGILWSTPIGSPHVVRWEPSPAVGPALLGLAFGSTLRSLVLFPTLTILVILLVIAWRTPTTWIASIMVTVCCIFTALNWNTTRTCNICCLRTLFSFNNIKLHSLSISYTAKVLPGVILLYGSLVYKYIFLGVIPVDETISVPYIEPFYCSQNLRCDDLLVPAGRRRRCEAARATAPCAAARSAGLGVGGAEGGGGGGGGGRLLGLGLAAHGCGDGDWGRLRQLRLLPGCDGN

SEQ ID NO: 5875 - protein, 21 aa, Homo sapiens
MVSRSRVSFSRTTAFTVSVTE

SEQ ID NO: 5876 - protein, 56 aa, Homo sapiens
MVSSIATESLLGTAKLPSLSWDASDRVVLLREASSGMEPLVLITLGSSLSSLVPSS

SEQ ID NO: 5877 - protein, 32 aa, Homo sapiens
MVSSLRCQLTGGLSALPGQGPCFIHLRVPNTQ

SEQ ID NO: 5878 - protein, 56 aa, Homo sapiens
MVSSLRCQLTGGLSALPGQGPCFIHLRVPNTVTMDDTQQALTKCHSSVRKIFPFYS

SEQ ID NO: 5879 - protein, 273 aa, Homo sapiens
MVSTSPLQKGRSCSAVPWKLYLAIHSVPDGQAACIADIFSGALASPSHSKANLSLGTIRALLGHCGPGHLAAGGISGLRDGPCGQGGGEGRRGPQGVRYKEVWVQGEGRRDRQAEAGGRTHGPGRGGKKGGGRGREGVGGRKQCSRRGPGRVPLPSAATEVRFWNVALAAGGRPGRSIGAAGLLALHAPRAPAARGWLGREGRRAGLRPRRRRSRAVARLGPHPGRSPRARRGWGRSGRAAAGSAAAAANLGSPRAPLGGSSQAWREEARPGS

SEQ ID NO: 5880 - protein, 96 aa, Homo sapiens
MVSTSSWWNSWMTSSSRPASFSPRQKVNVSSPMAAVQSPGSSQVSMVMVAGDPFTSAAAGVRGMYSADVGLLRDTRAPERSIFVLRQVLEQTLSCW

SEQ ID NO: 5881 - protein, 13 aa, Homo sapiens
MVSYTMWPFVTAL

SEQ ID NO: 5882 - protein, 14 aa, Homo sapiens
MVSYTMWPFVTALF

SEQ ID NO: 5883 - protein, 28 aa, Homo sapiens
MVTAFVVTVNLIAILILPVYYDFGSPLK

SEQ ID NO: 5884 - protein, 36 aa, Homo sapiens
MVTSYKLLGSNNPHALASQSVGITGVSHLSGPGSWF

SEQ ID NO: 5885 - protein, 49 aa, Homo sapiens
MVVCENTLPYSVPSANPTSACVKPNLILLCLNCLANCSNSSEVGVSSSE

SEQ ID NO: 5886 - protein, 22 aa, Homo sapiens
MVVCISEGLVVISPLSFFIESI

SEQ ID NO: 5887 - protein, 72 aa, Homo sapiens [sequence omitted]

SEQ ID NO: 5888 - protein, 75 aa, Homo sapiens
MVVLFWMLPVGPDQVWTMPGARPPPLIYTHARIRSSMGNRSKISVKSKSQEGSMWREVKFRPCPGNYDTQNIPLV

SEQ ID NO: 5889 - protein, 53 aa, Homo sapiens
MVVLFWMLPVGPDQVWTMPGARPPPLIYTHARIRSSMGNRSKISVKSKSRGWE

SEQ ID NO: 5890 - protein, 14 aa, Homo sapiens
MVVLRFFPIGKLIL

SEQ ID NO: 5891 - protein, 19 aa, Homo sapiens
MVVQFCGWEVHMADWAVRE

SEQ ID NO: 5892 - protein, 69 aa, Homo sapiens
MVVSRTGSSLSPQVPWPSTGHWGKDLISRLRVLSSIPYHPAPSHLLKQSFLFQVIQVIQPGIKSTWYLG

SEQ ID NO: 5893 - protein, 26 aa, Homo sapiens
MVVSRTGSSLSPQVPWPSTPTCVSPL

SEQ ID NO: 5894 - protein, 161 aa, Homo sapiens
MVVVLQLVQHPLPQGLLHHHLCGGAVHRAAFLQLLVLVLQGLEGLLYYRVIANRARRVPATHRKALRSHSHKTHRGRGPWRSRHYAKALGPQSPTAEVIASGGCVHRVDGSAAAKWNIQAVPQPQGAGTAEMSRIPWTTPRDGVPRRRREAGGRPAAAAPQ

SEQ ID NO: 5895 - protein, 26 aa, Homo sapiens
MVVVVVALGGSVKTSGSSSTLSFSFS

SEQ ID NO: 5896 - protein, 13 aa, Homo sapiens
MVWFSQYPLFIGR

SEQ ID NO: 5897 - protein, 12 aa, Homo sapiens
MVYYGQMVEKCY

SEQ ID NO: 5898 - protein, 62 aa, Homo sapiens
MWANTCRNPTTASHRRLCARLCWFPVQGPWMYSVRLLNTCLATDMALEKFLLPCSSMTSLPE

SEQ ID NO: 5899 - protein, 126 aa, Homo sapiens
MWCGKGAGAPSRVCPSPTALPGGQSAPSLQPPRPALPWSPADSSTPGSCAQSSSAAPPVAGSEGSGCMFTSATPNAPQLWGAQVRGGRRYGPSPAREYPLSFFASRWRPSLYSPTLPRSPRQPLRT

SEQ ID NO: 5900 - protein, 40 aa, Homo sapiens
MWFHCVRQAGLKLLTSGDLPTSASQSAGITGVSHRARPKS

SEQ ID NO: 5901 - protein, 32 aa, Homo sapiens
MWFHHVGQTGLELLTSSDLPISGPPKVLGLQV

SEQ ID NO: 5902 - protein, 93 aa, Homo sapiens
MWGPLEAVLRDTPLGRVPPDHGLAQGPTSTAPEAPCSLPLGALSSSGDADPGTLPSTVVSSCTHWAQTRLLGPLGGPQGAGSAPRSGVQGRQQ

SEQ ID NO: 5903 - protein, 15 aa, Homo sapiens
MWIDCSLLRKMGCGS

SEQ ID NO: 5904 - protein, 12 aa, Homo sapiens
MWKMKLRSLPCM

SEQ ID NO: 5905 - protein, 32 aa, Homo sapiens
MWKRFSLLTSLKYGSLSCPSLISILIILTGIF

SEQ ID NO: 5906 - protein, 19 aa, Homo sapiens
MWKSHVDFLLVCLETRYSR

SEQ ID NO: 5907 - protein, 30 aa, Homo sapiens
MWKSKPRKRKIMASNWKQIPHKRQSESLGY

SEQ ID NO: 5908 - protein, 18 aa, Homo sapiens
MWLNLTHWKGLQKLLKRI

SEQ ID NO: 5909 - protein, 68 aa, Homo sapiens
MWLQMLCACLLLQARVLLGASLFLHQLWLLWGLQGGLWLLWGLQGGLWLLWGFQGGLWFLWLLPVQLL

SEQ ID NO: 5910 - protein, 27 aa, Homo sapiens
MWLSICFHFWSSPVRMTTQVCVLPQSR

SEQ ID NO: 5911 - protein, 26 aa, Homo sapiens
MWPGWSRTQPPVNHLPQPPKVLGLQA

SEQ ID NO: 5912 - protein, 14 aa, Homo sapiens
MWPKEAKRWDTLAS

SEQ ID NO: 5913 - protein, 100 aa, Homo sapiens [sequence omitted]

SEQ ID NO: 5914 - protein, 41 aa, Homo sapiens
MWRAGLHCSTDIAATPCLYYTYFGEVSYICVVEACCEVLLC

SEQ ID NO: 5915 - protein, 19 aa, Homo sapiens
MWRGWLPLTPLGEAALSWE

SEQ ID NO: 5916 - protein, 14 aa, Homo sapiens
MWRKETPCTLLVGT

SEQ ID NO: 5917 - protein, 27 aa, Homo sapiens
MWRNRNTFTLLLCWWEYKLVQPLWRTV

SEQ ID NO: 5918 - protein, 11 aa, Homo sapiens
MWSPDQQRHIT

SEQ ID NO: 5919 - protein, 190 aa, Homo sapiens
MWSPGWYCSPSWPPVSRRTRMVALVDLLLCRFSTERIVAWNIFRLCTWIRPGSNCRPSAWALSRYLWRFQLRLGLKMSRAAALASSPTQKVSQAAWKAAWAQPRKASSWPHSSSPWPSCSSRSPPSSSSRVSTARAKAQKWGYAREPSPNTQNLRVPRAPALSVLLDSFLFRRQEDTSGSEQEMLLKRIL

SEQ ID NO: 5920 - protein, 44 aa, Homo sapiens
MWSQHGQSREPWGPLAMQRLVPQAPARGLRGGMAVAPIPRPSSL

SEQ ID NO: 5921 - protein, 22 aa, Homo sapiens
MWTHPPAPEGTGQSRHNFHQSR

SEQ ID NO: 5922 - protein, 47 aa, Homo sapiens
MWTRRCVWALNLSSESLSLSLFSSLSDAVSMLDIDNFFNLFFPLLAL

SEQ ID NO: 5923 - protein, 89 aa, Homo sapiens [sequence omitted]

SEQ ID NO: 5924 - protein, 25 aa, Homo sapiens
MWYQALRCSQSIQGDRYQANCDTVY

SEQ ID NO: 5925 - protein, 13 aa, Homo sapiens
MYAHIWQKKTITI

SEQ ID NO: 5926 - protein, 22 aa, Homo sapiens
MYALTLFSPRSSHPPSKKKPSS

SEQ ID NO: 5927 - protein, 34 aa, Homo sapiens
MYCCWQNATSCRFLYSWTPDIHINQGWIYKYLPK

SEQ ID NO: 5928 - protein, 55 aa, Homo sapiens
MYCFIKMQFIPMRPTGKASVKNSCSILTASTMISLTLSSEGLFTKYWNIRQAKSQ

SEQ ID NO: 5929 - protein, 16 aa, Homo sapiens
MYDEGIGLDCLKGLFS

SEQ ID NO: 5930 - protein, 16 aa, Homo sapiens
MYFLFLCNKLLPDLVA

SEQ ID NO: 5931 - protein, 50 aa, Homo sapiens
MYFPPRFRNIFSSNPLNFIASSTPTSRMDLEGSFRPFLQFRKRIYSSRIR

SEQ ID NO: 5932 - protein, 16 aa, Homo sapiens
MYFRSHRTTPLSGLLE

SEQ ID NO: 5933 - protein, 37 aa, Homo sapiens
MYFSRDGGLIMLARLVLNSWPQVIHPPWPPKMLGLQV

SEQ ID NO: 5934 - protein, 13 aa, Homo sapiens
MYGNHIASVKKMF

SEQ ID NO: 5935 - protein, 29 aa, Homo sapiens [sequence omitted]

SEQ ID NO: 5936 - protein, 20 aa, Homo sapiens
MYGTIWYFFQIPRNTDRIHK

SEQ ID NO: 5937 - protein, 45 aa, Homo sapiens
MYHHAWLIFVFLVETGFHHVGQAGLELLTSSDPPALASQSAGLQA

SEQ ID NO: 5938 - protein, 96 aa, Homo sapiens
MYHPQAWGKPGLSAVKAPPTRAHSGRCTVMLARRGLLCPVHLAPSRCVQGRVSGMAMGGGHLTGATRQTCTSRDLTQIWEGVNSLRWLLNKHSGFS

SEQ ID NO: 5939 - protein, 31 aa, Homo sapiens
MYHPVCLIFCIFSRDGVSPCWPGWSRTPDLK

SEQ ID NO: 5940 - protein, 31 aa, Homo sapiens
MYICWLTGTEGGRGYIRASMVYYGQMVEKCY

SEQ ID NO: 5941 - protein, 50 aa, Homo sapiens
MYIHNIYTHIHTICIHISVCVYECVHIKYIYIYICRERERESYKKLLTQL

SEQ ID NO: 5942 - protein, 48 aa, Homo sapiens
MYILAPEGLKPSPLETQSSPRKGVMEFCRHFSSRGTFEISSIFLPYKS

SEQ ID NO: 5943 - protein, 51 aa, Homo sapiens
MYILAPEGLKPSPLETQSSPRKGVMEFCRHFSSRGTLIFLNGFKKGSPVET

SEQ ID NO: 5944 - protein, 14 aa, Homo sapiens
MYILSTFWIRPSKI

SEQ ID NO: 5945 - protein, 26 aa, Homo sapiens
MYIYFCGVFLITHRSLYFNTGLCKGN

SEQ ID NO: 5946 - protein, 27 aa, Homo sapiens
MYKPESTVNLANLVQMLISCTGHCASC

SEQ ID NO: 5947 - protein, 37 aa, Homo sapiens
MYKPESTVNLANLVQMLISCTGHCASFIFLTMKNTNK

SEQ ID NO: 5948 - protein, 29 aa, Homo sapiens
MYLGINSWVLSQRGNSILKHYVEWSSKKC

SEQ ID NO: 5949 - protein, 54 aa, Homo sapiens [sequence omitted]

SEQ ID NO: 5950 - protein, 39 aa, Homo sapiens
MYLIPTHSWADLYFINKLNITLFKIRCFSKSHSLFNHII

SEQ ID NO: 5951 - protein, 21 aa, Homo sapiens
MYLNFLFLYFNEVSPCWPGWF

SEQ ID NO: 5952 - protein, 13 aa, Homo sapiens
MYLPEEISCKIYL

SEQ ID NO: 5953 - protein, 18 aa, Homo sapiens
MYLYSRSTMEYMPMSLLL

SEQ ID NO: 5954 - protein, 12 aa, Homo sapiens
MYMFFLNWLARK

SEQ ID NO: 5955 - protein, 19 aa, Homo sapiens
MYMKYMITSIMDIASDQEL

SEQ ID NO: 5956 - protein, 28 aa, Homo sapiens
MYMYIYFCGVFLITHRSLYFNTGLCKGN

SEQ ID NO: 5957 - protein, 17 aa, Homo sapiens
MYNIVLEYVSCGIVKLS

SEQ ID NO: 5958 - protein, 15 aa, Homo sapiens
MYNYTSSLERLINQY

SEQ ID NO: 5959 - protein, 57 aa, Homo sapiens
MYPPFDEYLDLHGPCSHGHHEWTENLWDHGSLWYLCYNLSSPLSPACLWSLLVPFGP

SEQ ID NO: 5960 - protein, 30 aa, Homo sapiens
MYPPVISKERKFLRAHVSENIFFPFSHLMV

SEQ ID NO: 5961 - protein, 54 aa, Homo sapiens
MYSAGKCPQMPVGTLEGLSSPTNVILSLVGISNPALPGVPGERESINIPPGTHP

SEQ ID NO: 5962 - protein, 80 aa, Homo sapiens [sequence omitted]

SEQ ID NO: 5963 - protein, 16 aa, Homo sapiens
MYSHCILYIIFMFMLR

SEQ ID NO: 5964 - protein, 19 aa, Homo sapiens
MYSSNHQMILLIRRMSPQH

SEQ ID NO: 5965 - protein, 21 aa, Homo sapiens
MYSTTSRLTLRGHLSGLMSTS

SEQ ID NO: 5966 - protein, 58 aa, Homo sapiens
MYSYYSLHSTREVLYLHLLPLSGNTTGQGQVNQIFHFRSFGDHTGSINSGHFRGDRLR

SEQ ID NO: 5967 - protein, 24 aa, Homo sapiens
MYTDHLCVLTKPSAFLEYSQMYAN

SEQ ID NO: 5968 - protein, 14 aa, Homo sapiens
MYTFYIFNKMPILR

SEQ ID NO: 5969 - protein, 46 aa, Homo sapiens
MYTISWKTFCRARFCSSRVRRAPTSPVSRAHWRRTLSRWAATRRIS

SEQ ID NO: 5970 - protein, 39 aa, Homo sapiens
MYTNTQTHTRIHTHTHDHIFHARFSNYQFKTMTHDYSRR

SEQ ID NO: 5971 - protein, 53 aa, Homo sapiens
MYTSDFTFTHMSHPHPSTGPFYYRPRRHRKCKEGLEPQKPGASGVRCPDSQEP

SEQ ID NO: 5972 - protein, 13 aa, Homo sapiens
MYVASVSDVLFHS

SEQ ID NO: 5973 - protein, 46 aa, Homo sapiens
MYVNRIYVIIIVGSDGTTSIQGSHSTAPSLSVYTVLTLAGAGKSLI

SEQ ID NO: 5974 - protein, 21 aa, Homo sapiens
MYVYVYLFLWCFSNHSSEFIF

SEQ ID NO: 5975 - protein, 17 aa, Homo sapiens
MYWSLCFFYFFNHEKHK

SEQ ID NO: 5976 - protein, 20 aa, Homo sapiens
MYWSLCFLLILRELLHTSCL

SEQ ID NO: 5977 - protein, 46 aa, Homo sapiens
MAADVLSRSLLGSPLAPVEETPLAFPPRLPLRTPRGWPAGGWRPAT

SEQ ID NO: 5978 - protein, 25 aa, Homo sapiens
MAAGFILIIVVIKLIAGRMEEAPAW

SEQ ID NO: 5979 - protein, 41 aa, Homo sapiens
MAAPNITGKLILCFKTHIAGGHFGDSLSHREFQDNDDNRMC

SEQ ID NO: 5980 - protein, 40 aa, Homo sapiens
MAAPTRLPIKAPTMIPTSGCEEVRSISQELLPSLLMAVHW

SEQ ID NO: 5981 - protein, 32 aa, Homo sapiens
MACDKLFKGYMHIQCILMCRINTRNVVIAIGR

SEQ ID NO: 5982 - protein, 19 aa, Homo sapiens
MACSASSFDRSVSCCCSVV

SEQ ID NO: 5983 - protein, 18 aa, Homo sapiens
MADKTAQTLLAYESLIQE

SEQ ID NO: 5984 - protein, 43 aa, Homo sapiens
MAEWASRIFSRSQIQTGTIWVATCMTFCQHCIEHICQLIKETP

SEQ ID NO: 5985 - protein, 27 aa, Homo sapiens
MAFIWLFSSACSLMSSKVGRQTEGLPT

SEQ ID NO: 5986 - protein, 27 aa, Homo sapiens
MAFIWLFSSVCSLMSSKVGRQTEGLPT

SEQ ID NO: 5987 - protein, 12 aa, Homo sapiens
MAFLQCMFSHVI

SEQ ID NO: 5988 - protein, 12 aa, Homo sapiens
MAFLQCVFSHVI

SEQ ID NO: 5989 - protein, 21 aa, Homo sapiens
MAGEPQPRATGSRATPSSLCH

SEQ ID NO: 5990 - protein, 82 aa, Homo sapiens
MAGGRLAWSCLRAPLLTLFLGPGYSGGGLLGMRARAACSWALYSIFSRSMGIWGTDSGASSSSSSLSLLWISIVASEKVFLW

SEQ ID NO: 5991 - protein, 11 aa, Homo sapiens
MAGISLPATCL

SEQ ID NO: 5992 - protein, 51 aa, Homo sapiens
MAHLGLQSAGITGVSHRAWPFLAAYTHSPCRKHRDQAGAAVGSEERSPQRW

SEQ ID NO: 5993 - protein, 17 aa, Homo sapiens
MAHPYHFHFCFVLFFIP

SEQ ID NO: 5994 - protein, 15 aa, Homo sapiens
MAHRVIDFGKHSDVG

SEQ ID NO: 5995 - protein, 52 aa, Homo sapiens
MAIIKKQKTPKDKCWLGCGENWNPCAQLAEMQMMQLWKTVWRFLKKLKIELI

SEQ ID NO: 5996 - protein, 157 aa, Homo sapiens
MAIIKKSGNNRCWRGCGEIGTLLHCWWDCKLVQPLWKSVWRFLRNLELEIPFDPAIPLLGIYSKDYKSCCYKDTCTRMFIAALFTIAKTWNQPKCPTMIDWIKKMWHIYTMEYYAAIKKDEFMSFVGTWMKLEIIILSKLSQGQKTKHHMFSLIDGN

SEQ ID NO: 5997 - protein, 30 aa, Homo sapiens
MAIIKKSGNNRCWRGCGETGTLFTVGGIVN

SEQ ID NO: 5998 - protein, 40 aa, Homo sapiens
MAIIKKSGNNRCWRGYGELGTLLHCWWECKLVQPLWKTVW

SEQ ID NO: 5999 - protein, 24 aa, Homo sapiens
MAIIKKSKDNKCWQGCGKKRTFVH

SEQ ID NO: 6000 - protein, 22 aa, Homo sapiens
MAIIKKSKNNRHWRGCGEKEML

SEQ ID NO: 6001 - protein, 67 aa, Homo sapiens
MAIIKKSRNNRCWRGCGEIGTLLYCWWECKLVQPLWKTVWRVLKDLEMEISFDPAILLLGIYPKEYK

SEQ ID NO: 6002 - protein, 36 aa, Homo sapiens
MAIIKKWHGGHRCWKGQGEIGILLHCWWECKLVQPL

SEQ ID NO: 6003 - protein, 11 aa, Homo sapiens
MAIIKQMKDKC

SEQ ID NO: 6004 - protein, 28 aa, Homo sapiens
MAIIKSGNNRCWRECREIGSFYTLLVGV

SEQ ID NO: 6005 - protein, 27 aa, Homo sapiens
MAIIQKNEKMLARLWRNRNAFTLLIGV

SEQ ID NO: 6006 - protein, 27 aa, Homo sapiens
MAIIQKTEKMLARLWRNRNAFTPLIGV

SEQ ID NO: 6007 - protein, 11 aa, Homo sapiens
MAISNRLHTFP

SEQ ID NO: 6008 - protein, 13 aa, Homo sapiens
MAITKKSKNNRCL

SEQ ID NO: 6009 - protein, 14 aa, Homo sapiens
MAKACDHKCMGSPK

SEQ ID NO: 6010 - protein, 22 aa, Homo sapiens
MAKAEQYKSIVFLDVKCQSVLA

SEQ ID NO: 6011 - protein, 12 aa, Homo sapiens
MAKIQNTDNIKC

SEQ ID NO: 6012 - protein, 67 aa, Homo sapiens [sequence omitted]

SEQ ID NO: 6013 - protein, 12 aa, Homo sapiens
MAKSFLVFRFLP

SEQ ID NO: 6014 - protein, 96 aa, Homo sapiens
MALAGPCLSTLALAMAGGRLAWSCLRAPLLTLFLGPGYSGGGLLGMRARAACSWALYSIFSRSMGIWGTDSGASSSSSSLSLLWISIVASEKVFLW

SEQ ID NO: 6015 - protein, 19 aa, Homo sapiens
MALGLSRSRDSAPRRACRQ

SEQ ID NO: 6016 - protein, 21 aa, Homo sapiens
MALGLSRSRDSAPRRACRQSA

SEQ ID NO: 6017 - protein, 31 aa, Homo sapiens
MALGLSRSRDSAPRRACRQSAHPPEAAATGH

SEQ ID NO: 6018 - protein, 27 aa, Homo sapiens
MALITYPQEHRSTNFGISLLYTSLFFF

SEQ ID NO: 6019 - protein, 82 aa, Homo sapiens
MALLFSIEILAWCARISLLSLSWDSFSCWVCCSWALMSSFFSSSHCWLRCRSRISCSSALWVLIISDHSFVCCATISLTLDL

SEQ ID NO: 6020 - protein, 39 aa, Homo sapiens
MALPKLETVNHVSRINSPGLGGQRRLSSFSCGLQELTVA

SEQ ID NO: 6021 - protein, 35 aa, Homo sapiens
MALWQRTVPDSSLATAQVDTVLTKSPRRAVAGEGF

SEQ ID NO: 6022 - protein, 24 aa, Homo sapiens
MALYCSYHCSICKGAFFYRSTLPC

SEQ ID NO: 6023 - protein, 45 aa, Homo sapiens
MALYCSYLTAGGQSTAPSRRPGRRRGRFCAELPPSPASPASRASQ

SEQ ID NO: 6024 - protein, 50 aa, Homo sapiens
MALYCSYTLGLDFLDHFHLHVKKHKMKEHMERSSAETIIAAVPAEAHTSG

SEQ ID NO: 6025 - protein, 29 aa, Homo sapiens [sequence omitted]

SEQ ID NO: 6026 - protein, 16 aa, Homo sapiens
MANPVKPGYRARFLYR

SEQ ID NO: 6027 - protein, 30 aa, Homo sapiens
MAPLDLAFGFRWQYYAIPCNRDIMCKLYRT

SEQ ID NO: 6028 - protein, 29 aa, Homo sapiens
MAPSQFITLTRTNLRRFSLALNVHPVSTI

SEQ ID NO: 6029 - protein, 64 aa, Homo sapiens
MAPVIVIVVAHDLDGLLHVPITQGHQGHCEWLPHRVQCVLDHLSPVDQHPLAIVSWLIKLQKGV

SEQ ID NO: 6030 - protein, 18 aa, Homo sapiens
MAQIQGTDSSKCGEDVEQ

SEQ ID NO: 6031 - protein, 13 aa, Homo sapiens
MAQMQIIDNTKCW

SEQ ID NO: 6032 - protein, 18 aa, Homo sapiens
MARLGESTVFPSMLLALL

SEQ ID NO: 6033 - protein, 17 aa, Homo sapiens
MARLRARDSGVAPGRRW

SEQ ID NO: 6034 - protein, 26 aa, Homo sapiens
MARTLQKATCCINPQDLEKQEVSLLL

SEQ ID NO: 6035 - protein, 68 aa, Homo sapiens [sequence omitted]

SEQ ID NO: 6036 - protein, 28 aa, Homo sapiens
MASGEQDRGLAPDHMVQKFSSTSRNSST

SEQ ID NO: 6037 - protein, 95 aa, Homo sapiens
MASGRRLPSELELVDEGKTVLFSFAEVVCICPQARPQRASRNGRPSARSSPSPGFAMGWVAGWQRRGRGFSRSPLLPHLRPGAPATGHLARASLT

SEQ ID NO: 6038 - protein, 98 aa, Homo sapiens
MASGRRLPSELELVDEGKTVLFSFAEVVCICPQARPQRASRNGRPSARSSPSPGFAMGWVAGWQRRGRGFSRSPLLPHLRPGAPATGHLGERTSGLCT

SEQ ID NO: 6039 - protein, 36 aa, Homo sapiens
MASKDKAGSHLAGISDPEGTDFVGTRGSSVEAGGGP

SEQ ID NO: 6040 - protein, 29 aa, Homo sapiens
MASSNRLLPFQQSQVLSKKVAFTNESHRS

SEQ ID NO: 6041 - protein, 24 aa, Homo sapiens
MASTCPSGTLHFSKYLWLLITRLS

SEQ ID NO: 6042 - protein, 11 aa, Homo sapiens
MASTLRTTLKL

SEQ ID NO: 6043 - protein, 41 aa, Homo sapiens
MASTWKGHLRTGLLDVHRKASLCLSPKPLNFYCCFTRLVQK

SEQ ID NO: 6044 - protein, 67 aa, Homo sapiens
MASVTEPIWLTLSSRQLQAFSSTARSIRFGLVTVRSSPTIWIPTLAVNLDQAAQSSWSNGSSMETTG

SEQ ID NO: 6045 - protein, 21 aa, Homo sapiens
MASWTCNLCSCTRLCLEAPHT

SEQ ID NO: 6046 - protein, 17 aa, Homo sapiens
MATFGKHLIAWLINALS

SEQ ID NO: 6047 - protein, 13 aa, Homo sapiens
MATKAKIDKMRSN

SEQ ID NO: 6048 - protein, 24 aa, Homo sapiens
MATKAKIDKWDIIKLNSFCTAEDE

SEQ ID NO: 6049 - protein, 20 aa, Homo sapiens
MATPPSPRPGYPPRQPFLAR

SEQ ID NO: 6050 - protein, 16 aa, Homo sapiens
MAVDFQQTPQQSTINC

SEQ ID NO: 6051 - protein, 135 aa, Homo sapiens
MAVGWSPGSAPAGGGWTCRGTGVSPAASPPGYSPDSTCPPQGCIGAKRAAPPVLGTSVWPRTLSRPGPQAPRGGRPGSGPGQSHTASLCSWHPGAHWTASGPGAQRAPSGGTGWPAGAGRRWSARGRPAAGRPSG

SEQ ID NO: 6052 - protein, 36 aa, Homo sapiens
MAVLLLCVGVCVCVHVVCLYVCVWSRVYMHTCVVRK

SEQ ID NO: 6053 - protein, 47 aa, Homo sapiens [sequence omitted]

SEQ ID NO: 6054 - protein, 15 aa, Homo sapiens
MCAFHQLLSTCALEP

SEQ ID NO: 6055 - protein, 34 aa, Homo sapiens
MCEVSVKQTTVHWIYSEPPCEECCKIAVSCQYFT

SEQ ID NO: 6056 - protein, 41 aa, Homo sapiens
MCFKFIKDLISASIFISLEQVIFFQQQQKDPLRTTRNIWKF

SEQ ID NO: 6057 - protein, 47 aa, Homo sapiens
MCHGGLLHLWTHPLSSLPSTPNPLQAFMCVVPFSVSMCSQCSTSTYG

SEQ ID NO: 6058 - protein, 13 aa, Homo sapiens
MCHHAQLFFFLYF

SEQ ID NO: 6059 - protein, 30 aa, Homo sapiens
MCHHARIIFVFLVETGFHRVGQAGLELLTS

SEQ ID NO: 6060 - protein, 11 aa, Homo sapiens
MCHHARLIFCI

SEQ ID NO: 6061 - protein, 57 aa, Homo sapiens
MCHHARLIFVFLVEMGFHHVGQACLELLTSSDLPTSASQSAGITGMSHRSWPECFRV

SEQ ID NO: 6062 - protein, 35 aa, Homo sapiens
MCHHARLIFVILIETRFHHVGQASLKLLTSGDLPA

SEQ ID NO: 6063 - protein, 21 aa, Homo sapiens
MCHHARLMFVFLEEMGFHHVG

SEQ ID NO: 6064 - protein, 152 aa, Homo sapiens
MCHHAWLIFCIFSRDRVSPCWPSWSRTPDLKLSTHLSLPKCRGYRHKPLCSVQFYHFKCHLHLMTSNWYSKLDLSCELHVDHMSIETDIQVDLSKYPLDRSTWVSNRHLKLSMSCTKPLILPPLKLSLPEAFLLSGNDTSPLPVAQGKKKSL

SEQ ID NO: 6065 - protein, 26 aa, Homo sapiens
MCHHGWLSFVFLVEMGFHHVGWPGWS

SEQ ID NO: 6066 - protein, 60 aa, Homo sapiens [sequence omitted]

SEQ ID NO: 6067 - protein, 11 aa, Homo sapiens
MCHHTQLILYF

SEQ ID NO: 6068 - protein, 41 aa, Homo sapiens
MCHHTWLIFVFLVEMGFHPVDQAGLELLTSSDLPHLGLPKC

SEQ ID NO: 6069 - protein, 31 aa, Homo sapiens
MCHHVRLIFCIFSRDGVSPRWSGWSRTPDLR

SEQ ID NO: 6070 - protein, 20 aa, Homo sapiens
MCHIMRNLILIYRILLLTKN

SEQ ID NO: 6071 - protein, 114 aa, Homo sapiens
MCHRAQLTFVFLIEMGFCHVGQAGLELLTSSDPPASASQSAGITGMSHHTWPKQGILTTKNKWHLCLSHFAYISPSCLTFTRLLLASMHSFVYLLSASVLLNVAVQGEGDIWMT

SEQ ID NO: 6072 - protein, 12 aa, Homo sapiens
MCIWYTQLVVIN

SEQ ID NO: 6073 - protein, 18 aa, Homo sapiens
MCKGGGVSCPAHHSQELF

SEQ ID NO: 6074 - protein, 36 aa, Homo sapiens
MCKPFGIIVGVKSGTEFTGCTFCIKVIMESYFFLFK

SEQ ID NO: 6075 - protein, 13 aa, Homo sapiens
MCLAKRRHKDHTC

SEQ ID NO: 6076 - protein, 15 aa, Homo sapiens
MCLCLTPSIIRITLG

SEQ ID NO: 6077 - protein, 17 aa, Homo sapiens
MCLHPWIPYNRKILLNN

SEQ ID NO: 6078 - protein, 22 aa, Homo sapiens
MCLSFSSGITELKGYVSLISLV

SEQ ID NO: 6079 - protein, 35 aa, Homo sapiens
MCLVPESDKLVMYSGNVSTLGSLSRSSDSSDGELP

SEQ ID NO: 6080 - protein, 31 aa, Homo sapiens
MCLYNRMIYNPLGIYPVMGLLGQMVFLILDP

SEQ ID NO: 6081 - protein, 16 aa, Homo sapiens
MCMAKACDHKCMGSPK

SEQ ID NO: 6082 - protein, 20 aa, Homo sapiens
MCNLGSSFSVCIRLLSNTNQ

SEQ ID NO: 6083 - protein, 47 aa, Homo sapiens
MCNNVSASLDSLNSVGCRHETAFKKPSLQLGSTFQFLDGILENLKTP

SEQ ID NO: 6084 - protein, 34 aa, Homo sapiens
MCPGTVATAPGIPALWEAEVDGLLEPRRSASTTQ

SEQ ID NO: 6085 - protein, 12 aa, Homo sapiens
MCPQSLLSDDSP

SEQ ID NO: 6086 - protein, 21 aa, Homo sapiens
MCQACTKLFTYNYLKPSHGEG

SEQ ID NO: 6087 - protein, 109 aa, Homo sapiens
MCQFLFAFLDFNFSGACHLDGHSLHLCEEVQFHNIFLPFRQIGQAGSHFLLDGPGPGLKERSQVLLHLVGEHLDPQIHFVNIFCGQVGLVPVLGEETDEWLPTKGFLEL

SEQ ID NO: 6088 - protein, 18 aa, Homo sapiens
MCQFLFAFLDFNFSGASV

SEQ ID NO: 6089 - protein, 25 aa, Homo sapiens
MCRFLNIIKFSVFSCSLLTSLKQLL

SEQ ID NO: 6090 - protein, 15 aa, Homo sapiens
MCRINTRNVVIAIGR

SEQ ID NO: 6091 - protein, 85 aa, Homo sapiens [sequence omitted]

SEQ ID NO: 6092 - protein, 18 aa, Homo sapiens
MCSGKSLCSEQENKPASG

SEQ ID NO: 6093 - protein, 33 aa, Homo sapiens
MCSICSTLPWSIFTLDICHHFDPTFILFSSYIL

SEQ ID NO: 6094 - protein, 26 aa, Homo sapiens
MCSILFGGIVISLIPFPEDLAWDQTL

SEQ ID NO: 6095 - protein, 24 aa, Homo sapiens
MCSLGFCKRCSNIRNVIMLISSDM

SEQ ID NO: 6096 - protein, 12 aa, Homo sapiens
MCTCRLQRFTCF

SEQ ID NO: 6097 - protein, 26 aa, Homo sapiens
MCTGVVKKTAVIQIFHPKHKLLTSKT

SEQ ID NO: 6098 - protein, 21 aa, Homo sapiens
MCTHTGWLHGHATCAVAQDCA

SEQ ID NO: 6099 - protein, 73 aa, Homo sapiens
MCTSRHAENLESHLPVQVPCQPEPLWSLAGLQLPCARGLSRDAATLLPSLFCQPDASRTEYLRENCLDNYSVP

SEQ ID NO: 6100 - protein, 16 aa, Homo sapiens
MCVVSDRHIHPTYMYM

SEQ ID NO: 6101 - protein, 58 aa, Homo sapiens
MCWEPLRYSCSKAGRINWWRLKRLCSMRVSAGVGGSRHSGMNTMKDRGSGELSSSLSK

SEQ ID NO: 6102 - protein, 34 aa, Homo sapiens
MCWVQWLMPVIPALWEAKTGGSFEAKNLRPAWPT

SEQ ID NO: 6103 - protein, 27 aa, Homo sapiens
MCYHARLIFVFLVETGFTMLARLVLNS

SEQ ID NO: 6104 - protein, 70 aa, Homo sapiens
MCYHVWLIFCIFSRDGVLHVGQAGLELVTSDDPPASASQSVGITGVSHHTRQYVVFLSLASFNNLIIYKF

SEQ ID NO: 6105 - protein, 17 aa, Homo sapiens
MCYRGIRCFMTKRYTWL

SEQ ID NO: 6106 - protein, 24 aa, Homo sapiens
MDAKPPKQQAQFVEIHFTHFLPEH

SEQ ID NO: 6107 - protein, 47 aa, Homo sapiens
MDFLQPVTVNHDIMCEVSVKQTTVHWIYSEPPCEECCKIAVSCQYFT

SEQ ID NO: 6108 - protein, 15 aa, Homo sapiens
MDGFLKITKYSEKLK

SEQ ID NO: 6109 - protein, 20 aa, Homo sapiens
MDICATAIQHHKKVVTHHNI

SEQ ID NO: 6110 - protein, 11 aa, Homo sapiens
MDICLQTLPDH

SEQ ID NO: 6111 - protein, 13 aa, Homo sapiens
MDIISQCTPNSQQ

SEQ ID NO: 6112 - protein, 11 aa, Homo sapiens
MDIKLLLGCFR

SEQ ID NO: 6113 - protein, 58 aa, Homo sapiens
MDKWAVFFEEFSKPRRQLHVYLFSWFHNLQLSSDLVKTLDNAMCDLASSHICIQLTSC

SEQ ID NO: 6114 - protein, 15 aa, Homo sapiens
MDLIQIITFYLLWLH

SEQ ID NO: 6115 - protein, 12 aa, Homo sapiens
MDLMYNKMHVAR

SEQ ID NO: 6116 - protein, 37 aa, Homo sapiens
MDMQPVQLHKTVLRSTPHLIFERGPYSFILPLVPQIM

SEQ ID NO: 6117 - protein, 79 aa, Homo sapiens
MDMTDWAKLLLAGPSGEEIVDDRGVPVQDDWSIAPDDDKVRFSLSGVTPHSWGLWGDTTGHGASASHLCWRKGSGRRSG

SEQ ID NO: 6118 - protein, 42 aa, Homo sapiens
MDNPRARISIPTTTGSRPAGTPLFRLSRMAKSPTISIPVPRT

SEQ ID NO: 6119 - protein, 18 aa, Homo sapiens
MDPLILCISAFIREYLTY

SEQ ID NO: 6120 - protein, 56 aa, Homo sapiens
MDPPASASQSAGLTGMSHCARPDFLISKMFFPVHCEAQPKKVTCLLLLFHCTAERE

SEQ ID NO: 6121 - protein, 53 aa, Homo sapiens
MDPSFKFPSLNPQPPTGLHVCCSLLCVHVFSVFNFHLWVRTCGVWFSVPVLVC

SEQ ID NO: 6122 - protein, 17 aa, Homo sapiens
MDSNSWAQVIFPPHPPE

SEQ ID NO: 6123 - protein, 28 aa, Homo sapiens
MDTLLLQLVICWCFSSKIKNLHLFHNFL

SEQ ID NO: 6124 - protein, 21 aa, Homo sapiens
MDTQTEIHIKHVLLINENANI

SEQ ID NO: 6125 - protein, 29 aa, Homo sapiens
MDVFFHSVSYWLDACILFYAEVIHSSSLM

SEQ ID NO: 6126 - protein, 78 aa, Homo sapiens
MDVKEMLLSLILGWRSLMIPRKIQYVLFFLWLFLFYTFILAKHPIWLDYEHRELSFLLILSQGSFPFVLAVFLSPSGV

SEQ ID NO: 6127 - protein, 32 aa, Homo sapiens
MDVKEMLLSLILGWRSLMIPRKIQYVLSPSGV

SEQ ID NO: 6128 - protein, 12 aa, Homo sapiens
MDYHINSHNIPV

SEQ ID NO: 6129 - protein, 61 aa, Homo sapiens
MEAIRGFTAIRSRACFMRSVHADGAGSGGRCATSNLDNSFNPFLQYNLLLKLNTDFHSFHD

SEQ ID NO: 6130 - protein, 28 aa, Homo sapiens
MEALRGCFRKISVCPADSRWRSFASIMI

SEQ ID NO: 6131 - protein, 57 aa, Homo sapiens
MEAMFRTVISLKVAAIPHRHLYKGKPGLPMVARWRGGRAAARRPGVRLSVWLGEGGR

SEQ ID NO: 6132 - protein, 59 aa, Homo sapiens
MEAMFRTVISLKVAAIPHRHLYKGKPGLPMVARWRGGRAAARRPGVRLSVWLGEGGREE

SEQ ID NO: 6133 - protein, 27 aa, Homo sapiens
MEASLGGPEPNGVINEEAKAGATGKRR

SEQ ID NO: 6134 - protein, 20 aa, Homo sapiens
MECCCAHTTLWLGDHTTASS

SEQ ID NO: 6135 - protein, 24 aa, Homo sapiens
MEEAPKPKGPSHQRGHIQSTFDRE

SEQ ID NO: 6136 - protein, 11 aa, Homo sapiens
MEEISILWKQI

SEQ ID NO: 6137 - protein, 24 aa, Homo sapiens
MEEQVEANTITAQYRWEVVWHPFV

SEQ ID NO: 6138 - protein, 92 aa, Homo sapiens
MEETVSVLIWEDAMDMTDWAKLLLAGPSGEEIVDDRGVPVQDDWSIAPDDDKVRFSLSGVTPHSWGLWGDTTGHGASASHLCWRKGSGRRSG

SEQ ID NO: 6139 - protein, 59 aa, Homo sapiens
MEEWSCRWSKGKITPDKGGESVLISNAASPYCCVFSLLDRVGLHTLSQFRLAISKRAGV

SEQ ID NO: 6140 - protein, 59 aa, Homo sapiens
MEEWSCRWSKGKITPDKGGESVLISNSASPYCCVFSLLDRVGLHTLSQFRLAISKRAGV

SEQ ID NO: 6141 - protein, 44 aa, Homo sapiens
MEFHHIGQAGLGLLTSGDPPTSASQSAGITGMSHRTQPTKIFID

SEQ ID NO: 6142 - protein, 154 aa, Homo sapiens
MEFHHTVQAGLELLTLGSACLGLPKCWYYRHEPPRPASLFYFIHLFTPSLENTGLELMCLRHRCTHGAQKRVGQSPGLCSVTWPLGPTDPSLQLLSPFLQVPRKPSLAAFITLTSSLPPTYQHQMHQLCSSFPLPSVALHFGRLRQVDHPRSGV

SEQ ID NO: 6143 - protein, 32 aa, Homo sapiens
MEFHHVGQAGLELLTSGDPSPPWSPKVIGLQA

SEQ ID NO: 6144 - protein, 44 aa, Homo sapiens [sequence omitted]

SEQ ID NO: 6145 - protein, 76 aa, Homo sapiens [sequence omitted]

SEQ ID NO: 6146 - protein, 30 aa, Homo sapiens
MEFISFIPPKLLLIYFLKVFEVFIVLSILL

SEQ ID NO: 6147 - protein, 13 aa, Homo sapiens
MEFLLPSFPNPIS

SEQ ID NO: 6148 - protein, 20 aa, Homo sapiens
MEFQRPLNIRREPIRNRKYT

SEQ ID NO: 6149 - protein, 32 aa, Homo sapiens
MEFSLESANYRSLWRFDDHSLVSGTTKGFWGV

SEQ ID NO: 6150 - protein, 21 aa, Homo sapiens
MEGAPECQEEQQDREGGSFPS

SEQ ID NO: 6151 - protein, 30 aa, Homo sapiens
MEGHAVFRVLHAGLQHLQHQGLLIFPHLPH

SEQ ID NO: 6152 - protein, 25 aa, Homo sapiens
MEGLMIRMLELVHCAEAGFRGGSEG

SEQ ID NO: 6153 - protein, 35 aa, Homo sapiens
MEGVPRELRGLRRAGEIQSCWGFDGFVFSLLFPLQ

SEQ ID NO: 6154 - protein, 29 aa, Homo sapiens
MEIESSSNSEVLSSLSIDDWGLSGEPLEV

SEQ ID NO: 6155 - protein, 57 aa, Homo sapiens
MEIRTDNKSQHSYGSSQNWELFFKYIIASHPPCAGRGVHDREMRRDQAPAFLSGSFQ

SEQ ID NO: 6156 - protein, 15 aa, Homo sapiens
MEKQECFYTVDRSVN

SEQ ID NO: 6157 - protein, 79 aa, Homo sapiens [sequence omitted]

SEQ ID NO: 6158 - protein, 15 aa, Homo sapiens
MEKYGLDICPLQISC

SEQ ID NO: 6159 - protein, 37 aa, Homo sapiens
MELCPFQRQYILIVQHMKFHCGFVVSFLGLFSFLPFS

SEQ ID NO: 6160 - protein, 41 aa, Homo sapiens
MELCPFQRQYILIVQHMKFHCGFVVSFLGLFSFLPLDTLLT

SEQ ID NO: 6161 - protein, 17 aa, Homo sapiens
MELFGISFGPGALRREY

SEQ ID NO: 6162 - protein, 19 aa, Homo sapiens
MELHVHCSTIHYSKDIELT

SEQ ID NO: 6163 - protein, 26 aa, Homo sapiens
MELISMPVLLLLESNEVIYSKYLTII

SEQ ID NO: 6164 - protein, 15 aa, Homo sapiens
MELSNFTSVNSWNFP

SEQ ID NO: 6165 - protein, 27 aa, Homo sapiens
MELTFNQSYLPTSMVYILYRKISNYLF

SEQ ID NO: 6166 - protein, 24 aa, Homo sapiens
MENKNMSPNRIICILMIQGFMHVY

SEQ ID NO: 6167 - protein, 54 aa, Homo sapiens
MENLSIIPKFRSFLLYCAVWPHINYQFSFFLLESLLLPLSSFTLFLSWFNPSSV

SEQ ID NO: 6168 - protein, 50 aa, Homo sapiens
MENSHMILWEILEEYLPCTLLSVVFPQRVFCLIKVLQSKHGLQSESLLVH

SEQ ID NO: 6169 - protein, 21 aa, Homo sapiens
MENTQFKKSMVYMQYIQNIHI

SEQ ID NO: 6170 - protein, 13 aa, Homo sapiens
MEPFQGEKSYRDD

SEQ ID NO: 6171 - protein, 41 aa, Homo sapiens
MEQREPSFIASGMQNSTATLEGSLAVSCKTKYSFNISYLPK

SEQ ID NO: 6172 - protein, 18 aa, Homo sapiens
MEQRQDHTGQGRGKCSYF

SEQ ID NO: 6173 - protein, 18 aa, Homo sapiens
MEQRQDHTRQGRGKCSYF

SEQ ID NO: 6174 - protein, 23 aa, Homo sapiens
MEQSQFTATSASQVQVMLPASVP

SEQ ID NO: 6175 - protein, 31 aa, Homo sapiens
MEREGSQQLECTQHSLLPLQLLILAGEGHVW

SEQ ID NO: 6176 - protein, 104 aa, Homo sapiens
MERHAAAAAWMNSAFLLTDGRVLLSPRILSRWKANTSLMSKGCLRSPQGLGPQRSTAPGAPPSSTSKRAPLLEDTGRSPATALSAKSRILRMSSLLSQEGALSL

SEQ ID NO: 6177 - protein, 12 aa, Homo sapiens
MERIPDYTCFLR

SEQ ID NO: 6178 - protein, 12 aa, Homo sapiens
MERRQQEVLTFR

SEQ ID NO: 6179 - protein, 36 aa, Homo sapiens [sequence omitted]

SEQ ID NO: 6180 - protein, 86 aa, Homo sapiens
MESHPVAQATVEWRNLGSLQPPPPRFKQFSCLSFPSSWDYRHPSPHPANFCIFSRDGGSPCWPGWSRTPDLMICPSQPLKLLGLQA

SEQ ID NO: 6181 - protein, 30 aa, Homo sapiens
MESLVINRSILFSVNKGLGCMRVQEDELVT

SEQ ID NO: 6182 - protein, 44 aa, Homo sapiens
MESLVINRSILFSVNKGLGCMRVQEDELVTCGLLLTDLCAEMAV

SEQ ID NO: 6183 - protein, 32 aa, Homo sapiens
MESLVINRSILFSVNKGLGCMRVQEDELVTLV

SEQ ID NO: 6184 - protein, 17 aa, Homo sapiens
MESRPGGPVQVTPTSSL

SEQ ID NO: 6185 - protein, 12 aa, Homo sapiens
METGFLHVGQAG

SEQ ID NO: 6186 - protein, 99 aa, Homo sapiens
METGGWLGGPSVGCIPRNSRLLSFRRKASLIRLRDILMAFSTSVLGMISDTFLGAVTKKLKEILGFKLATRTSSSNSFCPASVEFEMSHLCRGPSCLAA

SEQ ID NO: 6187 - protein, 80 aa, Homo sapiens
METGGWLGGPSVGCIPRNSRLLSFRRKASLIRLRDILMAFSTSVLGMISDTFLGAVTKKLKEILGFKLATRTSSSPKRII

SEQ ID NO: 6188 - protein, 28 aa, Homo sapiens
METKMSTTISAFKRVQLIGKTRQEYIYI

SEQ ID NO: 6189 - protein, 11 aa, Homo sapiens
METSVSWLLLH

SEQ ID NO: 6190 - protein, 16 aa, Homo sapiens
MEVGMERRQQEVLTFR

SEQ ID NO: 6191 - protein, 24 aa, Homo sapiens
MEVHCVAQTGLKLLGSINPPTSAS

SEQ ID NO: 6192 - protein, 16 aa, Homo sapiens
MEVHTISDHKPSGLSA

SEQ ID NO: 6193 - protein, 15 aa, Homo sapiens
MFAFLFILSRISLFF

SEQ ID NO: 6194 - protein, 54 aa, Homo sapiens
MFAFLLRFLLHLHQSIIGTIGCLHAIFTISFSVSYIFFSLFLSSCFCIKHLFLV

SEQ ID NO: 6195 - protein, 20 aa, Homo sapiens
MFAFSLVSLSYTVAYFFFFF

SEQ ID NO: 6196 - protein, 21 aa, Homo sapiens
MFARLFPCAGNRSTDQEDWGR

SEQ ID NO: 6197 - protein, 34 aa, Homo sapiens
MFFHNFVQLIHWFLIDVLLPRGRFRLKSISLESL

SEQ ID NO: 6198 - protein, 11 aa, Homo sapiens
MFFKDIPNYKI

SEQ ID NO: 6199 - protein, 15 aa, Homo sapiens
MFFLGCPHSFPKMEG

SEQ ID NO: 6200 - protein, 16 aa, Homo sapiens
MFFLMFPFCFQERAIF

SEQ ID NO: 6201 - protein, 58 aa, Homo sapiens
MFFSSWQDWTGLLLGCCAVFMAPCLEVSSAGIGRLHASSILGSNLVLFCRLLCGRLHN

SEQ ID NO: 6202 - protein, 30 aa, Homo sapiens
MFHNSSQNTCQKSSEHMVAFFPCCKHNVSI

SEQ ID NO: 6203 - protein, 23 aa, Homo sapiens
MFIAALFTIAKMWNQPKCPSLDG

SEQ ID NO: 6204 - protein, 29 aa, Homo sapiens
MFIKCRTTGHPPGWCEEMTFSKRVAFRQL

SEQ ID NO: 6205 - protein, 14 aa, Homo sapiens
MFIKVPFFNNGILY

SEQ ID NO: 6206 - protein, 30 aa, Homo sapiens
MFILTAPGKISNNCHFDLSIYLSPLNLQML

SEQ ID NO: 6207 - protein, 15 aa, Homo sapiens
MFILYPPYRLLQNKH

SEQ ID NO: 6208 - protein, 30 aa, Homo sapiens
MFIRCGDCRQWKVWSLTVPFSSVSTKVWVV

SEQ ID NO: 6209 - protein, 57 aa, Homo sapiens
MFISRMNFCTVIIYPFNMYKVFLGMGVYSLTVPCFIQASTCKFVYIMAFNDPPFSFL

SEQ ID NO: 6210 - protein, 12 aa, Homo sapiens
MFITGCLPTFGE

SEQ ID NO: 6211 - protein, 13 aa, Homo sapiens
MFKFFLECCFFQS

SEQ ID NO: 6212 - protein, 37 aa, Homo sapiens
MFKHFGKQISLSYLSLTGEAVCHGGQHRVSGIDNPDF

SEQ ID NO: 6213 - protein, 19 aa, Homo sapiens
MFLFSLKKIFRLGTICWWL

SEQ ID NO: 6214 - protein, 37 aa, Homo sapiens
MFLGLRPLVLGLQCSCSTLMRNYAFMVLSPLLSSELL

SEQ ID NO: 6215 - protein, 77 aa, Homo sapiens
MFLGRLANFPAAIILNSCLFLLSPGQLGSDEAALFGEAIHNSHPCTFFLDVPRMQDPDHALLGPFLSVVFAASNLEG

SEQ ID NO: 6216 - protein, 104 aa, Homo sapiens
MFLGRLANFPAAIILNSEKLASSEPWASTRALWALASARPRPASAKRGRAGQGGVAGRAAPTGRGSGEASAREDAARVPPSKMPGRQSLSAPRRGPRLGESQRA

SEQ ID NO: 6217 - protein, 96 aa, Homo sapiens
MFLGRLANFPAAIILNSPGAALGARALRISGPPAGAQRRRAAGLAPPAPRLLPELGTLMVRGACPPRIPRASSRCAPQLRLRSRPRPPPGQQQAQL

SEQ ID NO: 6218 - protein, 48 aa, Homo sapiens
MFLGTSKDPVCPRLFVFSGLISFLVVSSHCFWSPFLIRRGPSPCSFLG

SEQ ID NO: 6219 - protein, 15 aa, Homo sapiens
MFLGVILFFFFSVCW

SEQ ID NO: 6220 - protein, 28 aa, Homo sapiens
MFLKIAGKTLGLIVSGTTPIFLPSILVI

SEQ ID NO: 6221 - protein, 12 aa, Homo sapiens
MFLLAFHPHHQN

SEQ ID NO: 6222 - protein, 13 aa, Homo sapiens
MFLNLKKKKEKEK

SEQ ID NO: 6223 - protein, 62 aa, Homo sapiens
MFLQAEASVSSPGMVFMSLLGHIYTELWQILNTRAFEDSLVDRSLNTCFSAFLRKISLGVAS

SEQ ID NO: 6224 - protein, 14 aa, Homo sapiens
MFLSFLASFNSKSN

SEQ ID NO: 6225 - protein, 16 aa, Homo sapiens
MFLSGHLKIYSCYEKF

SEQ ID NO: 6226 - protein, 13 aa, Homo sapiens
MFLSSGNNFLASR

SEQ ID NO: 6227 - protein, 22 aa, Homo sapiens
MFMNNLDSNISKSCNIHKSIIS

SEQ ID NO: 6228 - protein, 15 aa, Homo sapiens
MFMPSLTLKGIVTTP

SEQ ID NO: 6229 - protein, 53 aa, Homo sapiens
MFNFNSQLTEQIGIPFPEKQCFRLQMCLLETQAGLPTIPQSTADLLCVQGFFL

SEQ ID NO: 6230 - protein, 121 aa, Homo sapiens
MFNKLFLEMHCIEVQPPDVAWIIGHINLSFFFSVLACYSKVFVLIHHKPCKRQIHFCCHLCKICIPCNLLEFFPAFLIHWIPWSPWNLPVLYFFLFYGDQCHAEGQQSHTLIFYLPFDFLL

SEQ ID NO: 6231 - protein, 127 aa, Homo sapiens
MFNKLFLEMHCIEVQPPDVAWIIGHINLSFFFSVLACYSKVFVLIHHKPCKRQIHFCCHLCKICIPCNLLEFFPAFLIHWIPWSPWNLPVLYFFLFYGDQCHAEGQQSHTLIFYLPPSCSIAFSNTI

SEQ ID NO: 6232 - protein, 36 aa, Homo sapiens
MFNQETHLPGLNSHTQQTLLRNCLLSRCSFLRQSSY

SEQ ID NO: 6233 - protein, 12 aa, Homo sapiens
MFPFCFQERAIF

SEQ ID NO: 6234 - protein, 25 aa, Homo sapiens
MFPKQTITSSERLRSFCRALRPSRF

SEQ ID NO: 6235 - protein, 12 aa, Homo sapiens
MFPSIRRIVLYM

SEQ ID NO: 6236 - protein, 12 aa, Homo sapiens
MFPSLHFPFEIF

SEQ ID NO: 6237 - protein, 59 aa, Homo sapiens
MFPSVLLALLQMNKGMILDKRINVGIEHIKHSGSQDSFLKHVKENDQKKKPKRRVPGLN

SEQ ID NO: 6238 - protein, 33 aa, Homo sapiens
MFPTVVSFQDNGVGVTPQSSCPHSAGSLSHQLS

SEQ ID NO: 6239 - protein, 42 aa, Homo sapiens
MFQFCQFHSQFFFLFELEFFQSLVFFCLLNGLFHIQLKLFIL

SEQ ID NO: 6240 - protein, 43 aa, Homo sapiens
MFQSLLCHLASLNPLMLTINIFPILFLSYISFTFVLKNCISLF

SEQ ID NO: 6241 - protein, 20 aa, Homo sapiens
MFQSSSVYALVTNPWVTCKM

SEQ ID NO: 6242 - protein, 26 aa, Homo sapiens
MFRHVGQAGLELLSSSDLPTSASQSA

SEQ ID NO: 6243 - protein, 54 aa, Homo sapiens
MFRTVISLKVAAIPHRHLYKGKPGLPMVARWRGGRAAARRPGVRLSVWLGEGGR

SEQ ID NO: 6244 - protein, 56 aa, Homo sapiens
MFRTVISLKVAAIPHRHLYKGKPGLPMVARWRGGRAAARRPGVRLSVWLGEGGREE

SEQ ID NO: 6245 - protein, 22 aa, Homo sapiens
MFSCRHKGRSVKVRPLKAGLVI

SEQ ID NO: 6246 - protein, 22 aa, Homo sapiens
MFSCRHKGRSVKVRPLKAGRTT

SEQ ID NO: 6247 - protein, 17 aa, Homo sapiens
MFSEQNSVVLNSADLAI

SEQ ID NO: 6248 - protein, 35 aa, Homo sapiens
MFSFLTSMTSLVTASNTCPHCKTASPFCLLSSGET

SEQ ID NO: 6249 - protein, 19 aa, Homo sapiens
MFSIFEMSFSVNNSNLRCQ

SEQ ID NO: 6250 - protein, 15 aa, Homo sapiens
MFSIIELYYTILLLQ

SEQ ID NO: 6251 - protein, 21 aa, Homo sapiens
MFSKDGVLPCWPGWSGPLDLR

SEQ ID NO: 6252 - protein, 72 aa, Homo sapiens
MFSLETPRVQDKHYDLHNDGISITYFPVVLQSCRDVQNTLASPECRFTFHSILVSKTKWSSGLQKFRSWIPA

SEQ ID NO: 6253 - protein, 13 aa, Homo sapiens
MFSLVSTGIEKSL

SEQ ID NO: 6254 - protein, 21 aa, Homo sapiens
MFSNCIVRVSQNKQSPDVFDM

SEQ ID NO: 6255 - protein, 13 aa, Homo sapiens
MFSRDGVSPCWPG

SEQ ID NO: 6256 - protein, 35 aa, Homo sapiens
MFSRDGVSTLLAGWSPSPDLVICLPRPPKVLGLQA

SEQ ID NO: 6257 - protein, 21 aa, Homo sapiens
MFSRFIHVAACSRTSFLFKAK

SEQ ID NO: 6258 - protein, 14 aa, Homo sapiens
MFSRLIHTVACSMY

SEQ ID NO: 6259 - protein, 51 aa, Homo sapiens
MFSVKKGGTLPILLGWDYFPTPFPSPSLVSSRSDPHAEPGRPWAPHMLPAR

SEQ ID NO: 6260 - protein, 18 aa, Homo sapiens
MFTAALLGQKTENNSYVL

SEQ ID NO: 6261 - protein, 12 aa, Homo sapiens
MFTCFLGSITFS

SEQ ID NO: 6262 - protein, 16 aa, Homo sapiens
MFTGCSLARLPSSTRG

SEQ ID NO: 6263 - protein, 23 aa, Homo sapiens
MFTLKSQSNQYLLRTHCVQFTML

SEQ ID NO: 6264 - protein, 29 aa, Homo sapiens
MFTLPSGKLCAHQRALGKAAGLHCGQFRS

SEQ ID NO: 6265 - protein, 28 aa, Homo sapiens
MFTMLASVVSNSSHQVIHPPRWVLGLQA

SEQ ID NO: 6266 - protein, 21 aa, Homo sapiens
MFTRYHSTEPTLKLDNIYLLT

SEQ ID NO: 6267 - protein, 22 aa, Homo sapiens
MFTVIFVRFVFLVIFWSFFLLS

SEQ ID NO: 6268 - protein, 14 aa, Homo sapiens
MFVFLEEMGFHHVG

SEQ ID NO: 6269 - protein, 23 aa, Homo sapiens
MFVFLVEMGLHHVGHAGLEVLTS

SEQ ID NO: 6270 - protein, 12 aa, Homo sapiens
MFVHRNKTYIEC

SEQ ID NO: 6271 - protein, 24 aa, Homo sapiens
MFVILLFLRSLSQDHGGPQQALRP

SEQ ID NO: 6272 - protein, 23 aa, Homo sapiens
MFVLLVETGLHHIGQVGLELLAS

SEQ ID NO: 6273 - protein, 61 aa, Homo sapiens
MFVLTALSAVFLQTTYEYFLVQTSCLSPLLNPLFLHLLFPQRIYLIHLGVQVHKLHKVLGL

SEQ ID NO: 6274 - protein, 13 aa, Homo sapiens
MFWALNLSVKTAL

SEQ ID NO: 6275 - protein, 31 aa, Homo sapiens
MFWIFRLFFSGIRCVHKNYECQRKYFMKLCS

SEQ ID NO: 6276 - protein, 46 aa, Homo sapiens
MFYAPVLFQTLRRYCLSNHKHVIRPGVIKHIYDERDHLDCCSRIHL

SEQ ID NO: 6277 - protein, 12 aa, Homo sapiens
MFYDQEIYLVVK

SEQ ID NO: 6278 - protein, 39 aa, Homo sapiens
MFYGSSIPLPLLFCFVFYSIGRCVLPLAGADIWNESASK

SEQ ID NO: 6279 - protein, 23 aa, Homo sapiens
MGADRSPEGRQKPGGFLYMGCRL

SEQ ID NO: 6280 - protein, 32 aa, Homo sapiens
MGAHRPGLRSQSKLVQSPHTPAPPGPRFPRFK

SEQ ID NO: 6281 - protein, 14 aa, Homo sapiens
MGCLPGWSRTPDFR

SEQ ID NO: 6282 - protein, 15 aa, Homo sapiens
MGCPYTVIVRVFREV

SEQ ID NO: 6283 - protein, 38 aa, Homo sapiens
MGEMALWQRTVPDSSLATAQVDTVLTKSPRRAVAGEGF

SEQ ID NO: 6284 - protein, 25 aa, Homo sapiens
MGENILKHLSSDYNFSDHMVKCVQE

SEQ ID NO: 6285 - protein, 48 aa, Homo sapiens
MGFAMLPRLLLAYFDIDCYSFDLQLTLKQCGGLGTPTPRSSQKSTYNF

SEQ ID NO: 6286 - protein, 37 aa, Homo sapiens
MGFCHVAQAGLKLLNSSILPPWSPKVLGLQACTTTPG

SEQ ID NO: 6287 - protein, 42 aa, Homo sapiens
MGFCHVGQAGLELLTSGDPSSLASQSARIISMSHHAWPTIYF

SEQ ID NO: 6288 - protein, 100 aa, Homo sapiens
MGFCHVGQAGLELLTSSDPPASASQSAGITGMSHHTWPKQGILTTKNKWHLCLSHFAYISPSCLTFTRLLLASMHSFVYLLSASVLLNVAVQGEGDIWMT

SEQ ID NO: 6289 - protein, 58 aa, Homo sapiens
MGFCHVGQAGLELLTSSDPPTSASQSAQITGVSHCTQPKGNFIWNAFHDFISCSLSLQ

SEQ ID NO: 6290 - protein, 50 aa, Homo sapiens
MGFCHVGQAGLKLLTSGDPPALAPQSAEITGMRHHTQLNHTFHHLTIWHL

SEQ ID NO: 6291 - protein, 31 aa, Homo sapiens
MGFCHVGQGGLKLLTSGDPLPQPPKVLELQA

SEQ ID NO: 6292 - protein, 31 aa, Homo sapiens
MGFCNVGQAGLELLTSVIHLPRPPKVLRLEA

SEQ ID NO: 6293 - protein, 11 aa, Homo sapiens
MGFHCIGQAGL

SEQ ID NO: 6294 - protein, 16 aa, Homo sapiens
MGFHCVGQASLKLLTS

SEQ ID NO: 6295 - protein, 31 aa, Homo sapiens
MGFHCVIQDGPGSPDLMIRLPRPPKVLGLQS

SEQ ID NO: 6296 - protein, 16 aa, Homo sapiens
MGFHCVSQDGLDLLTL

SEQ ID NO: 6297 - protein, 16 aa, Homo sapiens
MGFHHAGQAGLELLTL

SEQ ID NO: 6298 - protein, 38 aa, Homo sapiens
MGFHHFGQARLKLLIPGDPPASASQSAGIIGMRHHARP

SEQ ID NO: 6299 - protein, 15 aa, Homo sapiens
MGFHHIGHVTLVLNS

SEQ ID NO: 6300 - protein, 81 aa, Homo sapiens
MGFHHIGQAGLEFLTSGDSPTSASQSAGITGVSHWACPLPFFFWRQSLTLSPRMECYSTFSAHCNLCLQGSSNFPALGLQA

SEQ ID NO: 6301 - protein, 15 aa, Homo sapiens
MGFHHIGQAGLELLG

SEQ ID NO: 6302 - protein, 16 aa, Homo sapiens [sequence omitted]

SEQ ID NO: 6303 - protein, 28 aa, Homo sapiens
MGFHHIGQAGLKLLTSGDLHPRLASQSV

SEQ ID NO: 6304 - protein, 38 aa, Homo sapiens
MGFHHIGQAVLKLLTLLSTRLGLPKCWNYRHEPPCPAS

SEQ ID NO: 6305 - protein, 16 aa, Homo sapiens
MGFHHLGQADLELLIS

SEQ ID NO: 6306 - protein, 58 aa, Homo sapiens
MGFHHLGQAGFEPLTSSDLPALASQSARITGMSHHPAFFFFNYLFTTFFSDCKKIWPQ

SEQ ID NO: 6307 - protein, 16 aa, Homo sapiens
MGFHHLGQAGLELLTL

SEQ ID NO: 6308 - protein, 38 aa, Homo sapiens
MGFHHLGQAGLELLTSGDTPALASQSAGITGMNHCAQP

SEQ ID NO: 6309 - protein, 16 aa, Homo sapiens
MGFHHMGQAGLELLTR

SEQ ID NO: 6310 - protein, 67 aa, Homo sapiens
MGFHHVAQAGLELLSSGNPPALASQSVRITPCPARLFSDNDLSDSKQKILRISVCTDPTQPYSLENL

SEQ ID NO: 6311 - protein, 17 aa, Homo sapiens
MGFHHVAQAGLELLSSK

SEQ ID NO: 6312 - protein, 21 aa, Homo sapiens
MGFHHVAQAGLELLSSSDPPT

SEQ ID NO: 6313 - protein, 39 aa, Homo sapiens
MGFHHVCQAGLKLLTSGDPPALASRSAGITGVSHYIQPR

SEQ ID NO: 6314 - protein, 16 aa, Homo sapiens
MGFHHVDQDGLDLLTL

SEQ ID NO: 6315 - protein, 51 aa, Homo sapiens
MGFHHVDQVGLELLTSGDPPASAFQSAGITGMSHRARPSSFFNEKNLTFLQ

SEQ ID NO: 6316 - protein, 41 aa, Homo sapiens
MGFHHVGHAGLKLLTSRDPPASASQSAGITGMRHCAWSQIC

SEQ ID NO: 6317 - protein, 16 aa, Homo sapiens
MGFHHVGHDGLHLLTS

SEQ ID NO: 6318 - protein, 43 aa, Homo sapiens
MGFHHVGQACLELLTSSDLPTSASQSAGITGMSHRSWPECFRV

SEQ ID NO: 6319 - protein, 41 aa, Homo sapiens
MGFHHVGQADFELLTSSDLPVSASQSAGITGVSHRARPLSS

SEQ ID NO: 6320 - protein, 20 aa, Homo sapiens
MGFHHVGQADLEFLTSNDPK

SEQ ID NO: 6321 - protein, 39 aa, Homo sapiens
MGFHHVGQAEGGRFLSQLIFLKIPKLNRLSLKSSEILYH

SEQ ID NO: 6322 - protein, 30 aa, Homo sapiens
MGFHHVGQAEPSEGVWLGPHLDFRLLVSWF

SEQ ID NO: 6323 - protein, 60 aa, Homo sapiens
MGFHHVGQAGHELLISSDPPALSLPNCWDYRHEPPCLACFNFLMPLCKRHLIMENRKKQN

SEQ ID NO: 6324 - protein, 39 aa, Homo sapiens
MGFHHVGQAGIELLASSDPPASASQSAGIRGVSHCARPY

SEQ ID NO: 6325 - protein, 46 aa, Homo sapiens
MGFHHVGQAGLELLTLSDPPASASQSAGITGVSHCARPPGVYFIQC

SEQ ID NO: 6326 - protein, 42 aa, Homo sapiens
MGFHHVGQAGLELLTSGDPLVSASQSAGITGVSHRARPKLIS

SEQ ID NO: 6327 - protein, 59 aa, Homo sapiens
MGFHHVGQAGLELLTSGDPPALASQSAGITGVSHCALPTIYSFLQSYTASFCFLFYCTG

SEQ ID NO: 6328 - protein, 107 aa, Homo sapiens
MGFHHVGQAGLELLTSGDPPISASQNVGITGVSHCAQLEGLLLLLLLLLLFIIIIFEMESCSVTQAGVQWCGLSSLPAPPPWFMPFSCLSLPSSWDPPPHPANFLYF

SEQ ID NO: 6329 - protein, 116 aa, Homo sapiens
MGFHHVGQAGLELLTSGEPPALASQSAGLTVLSCANPMCLPPPSSSWLLCPRPHSALPGLPEWSVSGAASELCDASESLMGNCPWERCQRGKHCSQEMWQDGAGRPVSSPGQASGL

SEQ ID NO: 6330 - protein, 42 aa, Homo sapiens
MGFHHVGQAGLELLTSNDPPTSASQSAGITGGSYCARPIGAS

SEQ ID NO: 6331 - protein, 79 aa, Homo sapiens
MGFHHVGQAGLELLTSSDLPTSASQSAGITGMSHCARPRKSVFLEGITALEKMMMGATPYRKTLYYTAHSHQAGTGVTP

SEQ ID NO: 6332 - protein, 39 aa, Homo sapiens
MGFHHVGQAGLELLTSSDPPLSASQSAGITGMSHCAQPI

SEQ ID NO: 6333 - protein, 56 aa, Homo sapiens
MGFHHVGQAGLELLTSSDPPTLASQSAGITGVSHCAWWRGYYFTLAEEIKLQFTCL

SEQ ID NO: 6334 - protein, 21 aa, Homo sapiens
MGFHHVGQAGLELLTSSEEIA

SEQ ID NO: 6335 - protein, 43 aa, Homo sapiens
MGFHHVGQAGLELLTYGPPALAYQSARITGVSHRSWPGFFFKS

SEQ ID NO: 6336 - protein, 39 aa, Homo sapiens
MGFHHVGQAGLEPLTSGDPPVSASQSAGIIGVSHHAQPE

SEQ ID NO: 6337 - protein, 92 aa, Homo sapiens
MGFHHVGQAGLEPLTSGYPPALASQSAGITGMSHLAWPLLLFFACHVFVLLETRDIGPIDLTLFWILLTASPWSLFVCLFVMKSCSVTQAGV

SEQ ID NO: 6338 - protein, 105 aa, Homo sapiens
MGFHHVGQAGLKFLTSGDPPASASQSAGITGVSHCAWPTTLILKMFCKDRVSPCCLGWSQTPSLKQSSRLSLPKCWDYRRKPWSPVLNFPFSTIQTLNLFFLFFF

SEQ ID NO: 6339 - protein, 16 aa, Homo sapiens
MGFHHVGQAGLKFVTS

SEQ ID NO: 6340 - protein, 52 aa, Homo sapiens [sequence omitted]

SEQ ID NO: 6341 - protein, 54 aa, Homo sapiens
MGFHHVGQAGLKLLASSDPPTSASQSAGITGVSRHAQPRCKLFYKCKCTSLSRF

SEQ ID NO: 6342 - protein, 43 aa, Homo sapiens
MGFHHVGQAGLKLLTSGDLPASASQSAGITGISHPIRPINNVL

SEQ ID NO: 6343 - protein, 113 aa, Homo sapiens
MGFHHVGQAGLKLLTSGDTPRLGLPKCWDYKREPPCPARLFFKEFMPPLHTDLSRAGPQSVHVERTPHCTASDSSVANRVYLGRIPKGASRYGTSDKAPEQHRRDPRHNFGKS

SEQ ID NO: 6344 - protein, 47 aa, Homo sapiens
MGFHHVGQAGLKLLTSGHLTSQSAGITGVSHHAQPINIFFLLNSQSL

SEQ ID NO: 6345 - protein, 80 aa, Homo sapiens
MGFHHVGQAGLKLPTSSDPPTLASQSAGITGVSHHTQKNLILFLPRYGQEAGCSIRTGDPWSFICLHRINNCKPHLTPAT

SEQ ID NO: 6346 - protein, 39 aa, Homo sapiens
MGFHHVGQAGLKLVASSDPPASVSQSAEMTGVSHHALPG

SEQ ID NO: 6347 - protein, 50 aa, Homo sapiens
MGFHHVGQAGTWVLNKIPLSVMATSKPLKVSCGHTTCGQHEMLLLTLRVT

SEQ ID NO: 6348 - protein, 46 aa, Homo sapiens
MGFHHVGQASLKLLTSSDPPASASENSGITGISHHPGHKYFLLILH

SEQ ID NO: 6349 - protein, 16 aa, Homo sapiens
MGFHHVGQDGLNLLTS

SEQ ID NO: 6350 - protein, 16 aa, Homo sapiens
MGFHHVGQSGLELLTS

SEQ ID NO: 6351 - protein, 50 aa, Homo sapiens
MGFHHVGQTGLELRTSSDLPALASQSAGIRGVSHRSRPSIIQFHHIIYAV

SEQ ID NO: 6352 - protein, 31 aa, Homo sapiens
MGFHHVGQTGLVLLTSSDPPTSASTVLGLQV

SEQ ID NO: 6353 - protein, 16 aa, Homo sapiens
MGFHHVGQVGLDLLTL

SEQ ID NO: 6354 - protein, 54 aa, Homo sapiens
MGFHHVGQVGLQLLTSGDLFTSASQSAGITDVSHRAQPYLPLYLLPQSDLMKHN

SEQ ID NO: 6355 - protein, 21 aa, Homo sapiens
MGFHHVGQVGQLTGQQTPDLR

SEQ ID NO: 6356 - protein, 12 aa, Homo sapiens
MGFHHVGWPGWS

SEQ ID NO: 6357 - protein, 13 aa, Homo sapiens
MGFHHVNQLVSNS

SEQ ID NO: 6358 - protein, 12 aa, Homo sapiens
MGFHHVRLVSNS

SEQ ID NO: 6359 - protein, 42 aa, Homo sapiens
MGFHHVSQAGLELLTSSDRPTSASQSAGITGMSPHAWPMPGF

SEQ ID NO: 6360 - protein, 52 aa, Homo sapiens
MGFHHVSQAGLELLTSSYPPTSASQKSGIAGVSHRIQPNVLMADLNRQKKNP

SEQ ID NO: 6361 - protein, 16 aa, Homo sapiens
MGFHHVSQDGFDLLTS

SEQ ID NO: 6362 - protein, 43 aa, Homo sapiens
MGFHHVTQAGLELLGSSSLPTSASQSGGITGVSCVPSQNIMYF

SEQ ID NO: 6363 - protein, 16 aa, Homo sapiens
MGFHLVSQNGLDLLTL

SEQ ID NO: 6364 - protein, 16 aa, Homo sapiens
MGFHNVGQAGLELLTS

SEQ ID NO: 6365 - protein, 27 aa, Homo sapiens
MGFHPVDQAGLELLTSSDLPHLGLPKC

SEQ ID NO: 6366 - protein, 13 aa, Homo sapiens
MGFHQLGQAGLEL

SEQ ID NO: 6367 - protein, 16 aa, Homo sapiens
MGFHRGSQDGLDLLTS

SEQ ID NO: 6368 - protein, 17 aa, Homo sapiens
MGFHRVGKGGLEPLTSK

SEQ ID NO: 6369 - protein, 79 aa, Homo sapiens
MGFHRVGQAGLKLLSSSDLSTSASQSARITSMSHHTWPHNSLSTVFYPILLVACLSVFPLQIAQTLIFWSVDLLLFNSS

SEQ ID NO: 6370 - protein, 16 aa, Homo sapiens
MGFHRVGQDGLDLLTS

SEQ ID NO: 6371 - protein, 16 aa, Homo sapiens
MGFHRVSEDGLDLLTS

SEQ ID NO: 6372 - protein, 16 aa, Homo sapiens
MGFHRVSQDGLDLLIS

SEQ ID NO: 6373 - protein, 15 aa, Homo sapiens
MGFHRVSQDGLDLTS

SEQ ID NO: 6374 - protein, 16 aa, Homo sapiens
MGFHRVSQEGLDLVTS

SEQ ID NO: 6375 - protein, 16 aa, Homo sapiens
MGFHRVSQGGLDLLTS

SEQ ID NO: 6376 - protein, 30 aa, Homo sapiens
MGFHYAGQNGLKLDLVIHPPRPRKVLGLQA

SEQ ID NO: 6377 - protein, 16 aa, Homo sapiens
MGFHYLGQAGLELLAL

SEQ ID NO: 6378 - protein, 62 aa, Homo sapiens
MGFHYVDQAGLELLNLSSAHLSLPKCWDYRREPPCPANPELLTTVQAALYWPGRSPCLTHLQ

SEQ ID NO: 6379 - protein, 40 aa, Homo sapiens
MGFHYVGQAGHKLLTSGDPPISASQSAGITGVSHHAWPQV

SEQ ID NO: 6380 - protein, 50 aa, Homo sapiens
MGFHYVGQAGLELPTSDDPPALASQSAEITGMSHRVQPKLNVYRNTNQLK

SEQ ID NO: 6381 - protein, 89 aa, Homo sapiens
MGFLCFDQGGLELPTSGDPPASASQSAGITGMSHRAWPACCFHLILISEYRRGAELVFTNKHRSFVTFTVSFLAKPEWYVCGVMRFSPL

SEQ ID NO: 6382 - protein, 115 aa, Homo sapiens
MGFLHVGPAGLKLLTSGDPQALASQGAGITGMSHCAWLRLCLCGSCPPVLLGSQCTLEVTEGTLAGCREDSGGGMLPGWAQVESQPTGLLCSATLAEVCTLLGVSSETLLSTKHT

SEQ ID NO: 6383 - protein, 37 aa, Homo sapiens
MGFLHVGQAGLELLTSGDPPTSASQSAGIKATTPGHL

SEQ ID NO: 6384 - protein, 78 aa, Homo sapiens
MGFLHVGQAGLELPPSGGSLASASQSAGITGMSHHAQIEAPCKSIHLVGELGLSSALLVTAPSSSSGSVIQKALSGLQ

SEQ ID NO: 6385 - protein, 31 aa, Homo sapiens
MGFLHVGQAGLELPTSGDPPALPPKVLGLQA

SEQ ID NO: 6386 - protein, 38 aa, Homo sapiens
MGFLHVGQAGRELPTSGDPPTSASQSAGITGVSHCTRP

SEQ ID NO: 6387 - protein, 77 aa, Homo sapiens [sequence omitted]

SEQ ID NO: 6388 - protein, 11 aa, Homo sapiens
MGFLPCWPGWS

SEQ ID NO: 6389 - protein, 13 aa, Homo sapiens
MGFMPKYTVNTGP

SEQ ID NO: 6390 - protein, 52 aa, Homo sapiens [sequence omitted]

SEQ ID NO: 6391 - protein, 44 aa, Homo sapiens
MGFRHIGQASLELLTSSDPPASTSQSAWITGMSHCAWSVISSIS

SEQ ID NO: 6392 - protein, 51 aa, Homo sapiens
MGFRHVAQAGLKLLGSSDPLTSAFQSAGITGVSHHAQPRLFLKIRTYSPGL

SEQ ID NO: 6393 - protein, 50 aa, Homo sapiens
MGFRHVGQAGLELLTSAYLPTSASQSAGITSMSHRARPLYFLSVFSQEVL

SEQ ID NO: 6394 - protein, 61 aa, Homo sapiens
MGFRHVGQAGLELLTSSDPPASVSQSAGITGVSHCARPITPLFNKMSGTEQSIVPASERQD

SEQ ID NO: 6395 - protein, 47 aa, Homo sapiens
MGFRHVGQAGLKHLTSSNRPASASQSAGITGMSHRAQPERQEWLLLK

SEQ ID NO: 6396 - protein, 36 aa, Homo sapiens
MGFRHVGQAGLKLLTLSDLPASVSPNAGIIVMSPQL

SEQ ID NO: 6397 - protein, 21 aa, Homo sapiens
MGFRLVEMGCLPGWSRTPDFR

SEQ ID NO: 6398 - protein, 13 aa, Homo sapiens
MGFRMLARVVSNS

SEQ ID NO: 6399 - protein, 55 aa, Homo sapiens
MGFRPVGQAGFELLTSGDPPASASQSAAITGVSHRASKRFNRKTICTGSKRVLRS

SEQ ID NO: 6400 - protein, 41 aa, Homo sapiens
MGFRYVETGLKLLTSGDPPVSVSQSAGITGVSHCAQPANLM

SEQ ID NO: 6401 - protein, 40 aa, Homo sapiens
MGFRYVGLAGLKLLTSGDPPASASQSARITGMSHRTRPIF

SEQ ID NO: 6402 - protein, 13 aa, Homo sapiens
MGFSMLVRLVWNS

SEQ ID NO: 6403 - protein, 28 aa, Homo sapiens
MGFTMFVILLFLRSLSQDHGGPQQALRP

SEQ ID NO: 6404 - protein, 13 aa, Homo sapiens
MGFTMLARLIWNS

SEQ ID NO: 6405 - protein, 31 aa, Homo sapiens
MGFTMLARLVLNSWVPVILPPQPPKVLGLEV

SEQ ID NO: 6406 - protein, 85 aa, Homo sapiens
MGFWCGCPFCLLVFLLTDRTLSCRSVGIPCRVRCQCAPAGGCLPVRLLGGQGSGTHLRRQSAHSQISSCVLGEPLLSSKLSDRDI

SEQ ID NO: 6407 - protein, 35 aa, Homo sapiens
MGFYHVDQAGLKLLTSGDLPASASQSPFSALFCKH

SEQ ID NO: 6408 - protein, 16 aa, Homo sapiens
MGFYHVGQAGLKLLTS

SEQ ID NO: 6409 - protein, 61 aa, Homo sapiens
MGFYHVGQDGLKLLTSNDPPALASQIAGITGVSHRTRPYYSIFNLFIHVKKHSLTAAQYDN

SEQ ID NO: 6410 - protein, 13 aa, Homo sapiens
MGFYHVGQLVSNS

SEQ ID NO: 6411 - protein, 26 aa, Homo sapiens
MGGCVLGVSATREDSPEAPWSQAAGS

SEQ ID NO: 6412 - protein, 80 aa, Homo sapiens
MGGECLGLTPRGNESPGQPFNYPSLKPSPPPLRVTGGTPPDSKGAAQRSSEPFWASTGPAPFCDPAVHQLGSSGRPSLLQ

SEQ ID NO: 6413 - protein, 43 aa, Homo sapiens
MGGEKGNPFLLGLDVSSLIWGASRLLPLLLDHTTSLCCSCQHC

SEQ ID NO: 6414 - protein, 32 aa, Homo sapiens
MGGFHQVGQAGLELPTSGDLPTLASQVLGLQA

SEQ ID NO: 6415 - protein, 13 aa, Homo sapiens
MGGHLYDILPALH

SEQ ID NO: 6416 - protein, 232 aa, Homo sapiens [sequence omitted]

SEQ ID NO: 6417 - protein, 267 aa, Homo sapiens
MGGIRDSVAGRRVTSAFMSLSNSSSWFRSSVVGPPPRGAAAALTLVQDGVGRLVPRQRLLGEVLVALGQALGLGEAGVEGHGGVRRLLRQVQVGRPPQLLLNHQRLLQELEPPGQELIFHLQKVPLIGFSFKWLVDNGKLSIILDVLPPCIAMEDNPSQKPIVMSSVPDLIEFPRGNSCPFLILPQCVKLCEATIGDIEHEPGLLCLFLSSPIGPWLISRPWSKLPVTFYIFCSLAQIPCFPLRPLPVFLSIQRLLLPPFSWRRLCG

SEQ ID NO: 6418 - protein, 266 aa, Homo sapiens
MGGIRDSVAGRRVTSAFMSLSNSSSWFRSSVVGPPPRGAAAALTLVQDGVGRLVPRQRLLGEVLVALGQALGLGEAGVEGHGGVRRLLRQVQVGRPPQLLLNHQRLLQELEPPGQELIFHLQKVPLIGFSFKWLVDNGKLSIILDVLPPCIAMEDNPSQKPIVMSSVPDLIEFPRGNSCPFLILPQCVKLCEATIGDIEHEPGLLCLFLSSPIGPWLISRPWSKLPVTFYIFSLAQIPCFPLRPLPVFLSIQRLLLPPFSWRRLCG

SEQ ID NO: 6419 - protein, 77 aa, Homo sapiens
MGGIRDSVAGRRVTSAFMSLSNSSSWFRTLCRTALAGLFPASDSLERCWWLSARHSASAKRAWRAMAGCAGSCDRFR

SEQ ID NO: 6420 - protein, 193 aa, Homo sapiens
MGGPGRIWDTPVSGGSGRRWDTPVSGGSGRRLDTGVLGGSGLRWDTPVSGGSGRRWDTGVSGGFRQNSPQGCLPGSVGTSVVFSWVSQQAQASSSSLSGSRCFSTCSRRSGGISSPRLGYMAKGCLAISWASTCSTNAFRASWAGESLENRAAFLSSFFCPLLGSAWGPLRDILGSKNSSRRQTRVSSGDGQP

SEQ ID NO: 6421 - protein, 17 aa, Homo sapiens
MGGPILDGNWGRRSLCD

SEQ ID NO: 6422 - protein, 30 aa, Homo sapiens
MGGVSPCWPGWFRTPDLIIYLPWPPKVLGL

SEQ ID NO: 6423 - protein, 69 aa, Homo sapiens
MGHFYFRLLSEEIQSKLQILQPLSVDGINFSELGGKCCFLFLHFGGRRLEPGSLAHVASPSILQVEKRP

SEQ ID NO: 6424 - protein, 102 aa, Homo sapiens
MGHGRPSWMNSAFLLTDGRVLLSPRILSRWKANTSLMSKGCLRSPQGLGPQRSTAPGAPPSSTSKRAPLLEDTGRSPATALSAKSRILRMSSLLSQEGALSL

SEQ ID NO: 6425 - protein, 23 aa, Homo sapiens
MGHSSLRRLRAETGHRSLGRLRA

SEQ ID NO: 6426 - protein, 35 aa, Homo sapiens
MGHSSLWRLRAEMGHSSLRRLRAETGHRSLGRLRA

SEQ ID NO: 6427 - protein, 12 aa, Homo sapiens
MGIFFLYYPGGL

SEQ ID NO: 6428 - protein, 16 aa, Homo sapiens
MGIHHVSQAGLELLTS

SEQ ID NO: 6429 - protein, 22 aa, Homo sapiens
MGIILSTVLLSIEISCRSGWQA

SEQ ID NO: 6430 - protein, 81 aa, Homo sapiens
MGILHKHFSDFIPSHFHSDVQLELVHSVRHLPIPGAVELAHPPLGLVHVPTENGLHEGAGGRSSLADAAPRHLAKASTPQP

SEQ ID NO: 6431 - protein, 68 aa, Homo sapiens
MGILQKRKELYWLLTGSLIASCYQSITGVFQRWRECLGSSGVCAGLEKYKAVGALTALSSHSFSLFSD

SEQ ID NO: 6432 - protein, 11 aa, Homo sapiens
MGISLCWPGWS

SEQ ID NO: 6433 - protein, 12 aa, Homo sapiens
MGIWVGSKSLLL

SEQ ID NO: 6434 - protein, 12 aa, Homo sapiens
MGIWVGSMSLLL

SEQ ID NO: 6435 - protein, 39 aa, Homo sapiens
MGKENKINRTDYCQKPFLWSIPAMHIELKLKTKKQPNCT

SEQ ID NO: 6436 - protein, 13 aa, Homo sapiens
MGKTKKIKCTFTV

SEQ ID NO: 6437 - protein, 52 aa, Homo sapiens
MGLHHVAQAGLKLVDSSGPPTSASQNAGITGVSHHAQLGSLLWRGETNIHHI

SEQ ID NO: 6438 - protein, 16 aa, Homo sapiens
MGLHHVGHAGLEVLTS

SEQ ID NO: 6439 - protein, 38 aa, Homo sapiens
MGLHHVGPAGLKLLTSGDPPTSASQSAGITGVSHHAWT

SEQ ID NO: 6440 - protein, 24 aa, Homo sapiens
MGLPSVRLDLMVTIMSIFPTTVPI

SEQ ID NO: 6441 - protein, 22 aa, Homo sapiens
MGLWKSLPLSISPWLHGVGMSS

SEQ ID NO: 6442 - protein, 30 aa, Homo sapiens
MGMLSQKVVKERRVCEKCISVLCTVSVCVM

SEQ ID NO: 6443 - protein, 27 aa, Homo sapiens
MGNAKQDLKEGKTSFGTDFSFIVLGRR

SEQ ID NO: 6444 - protein, 12 aa, Homo sapiens
MGNAMLASTVDP

SEQ ID NO: 6445 - protein, 13 aa, Homo sapiens
MGPAWGLGTRLGH

SEQ ID NO: 6446 - protein, 57 aa, Homo sapiens
MGPCLHLHFSVVIFKETDKTPFRVNQIMSNPCLKLSLPNKTTNTLEMQFKFFTLKSF

SEQ ID NO: 6447 - protein, 19 aa, Homo sapiens
MGPEASKHLSRCNNQALFL

SEQ ID NO: 6448 - protein, 58 aa, Homo sapiens
MGPVCPLLGFHLHCQNRTVLPLPLHYYWYHISFHFLQEREAGALAGPCCSSRCLSQLC

SEQ ID NO: 6449 - protein, 11 aa, Homo sapiens
MGQAGLELLTR

SEQ ID NO: 6450 - protein, 39 aa, Homo sapiens
MGQGSWSQNPRDSGGMEERDGFTGDTCITYYNDFSAITH

SEQ ID NO: 6451 - protein, 61 aa, Homo sapiens
MGQSPPVGAGKTPKHSRDGVPVGGGQGQHPLKSPLQTWSPTMVGGRTGRPGLLCDYSGKRT

SEQ ID NO: 6452 - protein, 15 aa, Homo sapiens
MGRLQRNLRRCPCLT

SEQ ID NO: 6453 - protein, 15 aa, Homo sapiens
MGRLSLGVYDLVESL

SEQ ID NO: 6454 - protein, 22 aa, Homo sapiens
MGRRKKLPLISIFYMLLFFFCP

SEQ ID NO: 6455 - protein, 14 aa, Homo sapiens
MGSDQLNPPNPLQL

SEQ ID NO: 6456 - protein, 18 aa, Homo sapiens
MGSHHIGQAGCELLTSGD

SEQ ID NO: 6457 - protein, 16 aa, Homo sapiens
MGSHHVRQDGLDLLTS

SEQ ID NO: 6458 - protein, 55 aa, Homo sapiens
MGSLCVAQASLELLGSRDPPTLASQSVGIIGMRHHAQQRILDQIQSSCLSRGGPA

SEQ ID NO: 6459 - protein, 69 aa, Homo sapiens
MGSLWEGGKVSIPSKAPCKPGAPPWLGAAQAGQGCCVTTVGRGHERLWLSTSRGGHSAWSQNWTQSPQG

SEQ ID NO: 6460 - protein, 12 aa, Homo sapiens
MGSQTIQSLPSC

SEQ ID NO: 6461 - protein, 13 aa, Homo sapiens
MGSTMLARMVSIS

SEQ ID NO: 6462 - protein, 22 aa, Homo sapiens
MGTSDSTWHHQNKVKRLKWEGR

SEQ ID NO: 6463 - protein, 21 aa, Homo sapiens
MGTSILFSWIFSTGLHCQVSM

SEQ ID NO: 6464 - protein, 39 aa, Homo sapiens
MGTVQKGITHRCYHGKTGSVYNVPQCTAGIVANEQGHDS

SEQ ID NO: 6465 - protein, 15 aa, Homo sapiens
MGTVQKGMPHKCHHG

SEQ ID NO: 6466 - protein, 33 aa, Homo sapiens
MGVCARHTHTVFLYMHAYLCMYREVSRHQFLIK

SEQ ID NO: 6467 - protein, 13 aa, Homo sapiens
MGVDIGTWLLALY

SEQ ID NO: 6468 - protein, 32 aa, Homo sapiens
MGVHHHARLIFVFLVETEFHHIGQAGLELLTS

SEQ ID NO: 6469 - protein, 42 aa, Homo sapiens
MGVHHVGQAGLKLLTSGDPPTLASQSAGFADGSHHAQPSLTL

SEQ ID NO: 6470 - protein, 13 aa, Homo sapiens
MGVKHAFKRKTLN

SEQ ID NO: 6471 - protein, 17 aa, Homo sapiens
MGVSPCGPGWSRTPNRG

SEQ ID NO: 6472 - protein, 44 aa, Homo sapiens
MGVSPCWPGWSRTPDLRYPLASASQSAMITGVSHRAWPRSQFFL

SEQ ID NO: 6473 - protein, 12 aa, Homo sapiens
MGYECRTCRFVP

SEQ ID NO: 6474 - protein, 23 aa, Homo sapiens
MGYEVHMSWFLQYECMYIYKVWL

SEQ ID NO: 6475 - protein, 46 aa, Homo sapiens
MGYGCQRDAAVPYSWMEKFDDTQKDPVCPLSLWCLTHWHSLRISFL

SEQ ID NO: 6476 - protein, 12 aa, Homo sapiens
MGYHCLALLFCC

SEQ ID NO: 6477 - protein, 36 aa, Homo sapiens
MGYHQIGQAGLEFLTSGDPPASASQSAGVTGMSHCT

SEQ ID NO: 6478 - protein, 56 aa, Homo sapiens [sequence omitted]

SEQ ID NO: 6479 - protein, 12 aa, Homo sapiens
MHCFGFTFQYTN

SEQ ID NO: 6480 - protein, 22 aa, Homo sapiens
MHCFYNHEKTQLKYNRLLIPCS

SEQ ID NO: 6481 - protein, 66 aa, Homo sapiens
MHCVCAPYTFVYVWAHTQNTLKFCDVSCSAARYFFQISHLIPRLFITREDLSARSPALWRKSPAAL

SEQ ID NO: 6482 - protein, 11 aa, Homo sapiens
MHDLLNLASFA

SEQ ID NO: 6483 - protein, 28 aa, Homo sapiens
MHEVVLVVYLGKGDVASSLNVIHKLLCR

SEQ ID NO: 6484 - protein, 50 aa, Homo sapiens
MHHCTQLIFVFLAEMGFRHVGQAGLKLLTLSDLPASVSPNAGIIVMSPQL

SEQ ID NO: 6485 - protein, 34 aa, Homo sapiens
MHHHAGLIFVLSLFFLVETGFHHVGQAGLELLTS

SEQ ID NO: 6486 - protein, 42 aa, Homo sapiens
MHHHAQLIFVFLVEMGFHHIGQAGLKLLTSGDLHPRLASQSV

SEQ ID NO: 6487 - protein, 54 aa, Homo sapiens
MHHHAQLIFVFLVETGFHHVGQAGLKLLTSGAPSASASQSARITGVNHHAWPGY

SEQ ID NO: 6488 - protein, 26 aa, Homo sapiens
MHHHARLILVFLVETGFHHVVQADLN

SEQ ID NO: 6489 - protein, 55 aa, Homo sapiens
MHHHAWLIFVFLVEAGFRHVGQAGLKLLTSSQPRQPALALLREVRDPEQRDLLKP

SEQ ID NO: 6490 - protein, 25 aa, Homo sapiens
MHHHAWLIFVFLVETGFSPCWLGWS

SEQ ID NO: 6491 - protein, 11 aa, Homo sapiens
MHHHAWLIFYF

SEQ ID NO: 6492 - protein, 25 aa, Homo sapiens
MHHHTRLIFYIFSRDGVSPCWSGWS

SEQ ID NO: 6493 - protein, 52 aa, Homo sapiens
MHHHTWLIFVFLVEMGFLHVGQAGRELPTSGDPPTSASQSAGITGVSHCTRP

SEQ ID NO: 6494 - protein, 17 aa, Homo sapiens
MHHLCPATFFFFFLYFY

SEQ ID NO: 6495 - protein, 17 aa, Homo sapiens
MHIKEGVRDSQNVLYTF

SEQ ID NO: 6496 - protein, 22 aa, Homo sapiens
MHIQCILMCRINTRNVVIAIGR

SEQ ID NO: 6497 - protein, 24 aa, Homo sapiens
MHIYHLCQSVLMLLIKSYPRLGNL

SEQ ID NO: 6498 - protein, 35 aa, Homo sapiens [sequence omitted]

SEQ ID NO: 6499 - protein, 17 aa, Homo sapiens
MHKGIIGIGVTLPYSQL

SEQ ID NO: 6500 - protein, 52 aa, Homo sapiens
MHKIHILDKMFQSLLCHLASLNPLMLTINIFPILFLSYISFTFVLKNCISLF

SEQ ID NO: 6501 - protein, 21 aa, Homo sapiens
MHLILDMLKSLHINKIKPLRF

SEQ ID NO: 6502 - protein, 42 aa, Homo sapiens
MHLLLPVLTAGWSSCSPRPSYSHYVRSGFFFFFLDEVSLSTI

SEQ ID NO: 6503 - protein, 46 aa, Homo sapiens
MHLPHTSVWKQSSYSGLFRCNDCSHRKNGSFSTFDSFSMSSHNHPH

SEQ ID NO: 6504 - protein, 11 aa, Homo sapiens
MHNHARLILYF

SEQ ID NO: 6505 - protein, 60 aa, Homo sapiens
MHNNARRIFCILIETVLPCWPGWSRTPELKRSTCLGLPKCWDYRRASLCLAAANHFLVKF

SEQ ID NO: 6506 - protein, 12 aa, Homo sapiens
MHNSEKLKYTEY

SEQ ID NO: 6507 - protein, 63 aa, Homo sapiens [sequence omitted]

SEQ ID NO: 6508 - protein, 14 aa, Homo sapiens
MHPPRPPKLLGLQG

SEQ ID NO: 6509 - protein, 18 aa, Homo sapiens
MHQHAQLILGYTLNSIQS

SEQ ID NO: 6510 - protein, 58 aa, Homo sapiens
MHRQHASPGGSLAAPFFMPGRTSGFLFNSTGLPHHPTSLCKPLLYCDLDPLGQAGAYV

SEQ ID NO: 6511 - protein, 11 aa, Homo sapiens
MHSEYPQEIDK

SEQ ID NO: 6512 - protein, 33 aa, Homo sapiens
MHSNSSGTLSRASHICDTEVWNSPMKSWPPSLS

SEQ ID NO: 6513 - protein, 37 aa, Homo sapiens
MHSQLTAMKGTGTQKYNRQGIHQTSSKLQGCLGQKRL

SEQ ID NO: 6514 - protein, 65 aa, Homo sapiens
MHTPACLANFCIFVETGFHHVGQAGLKLLISGNLPTLISQSAGITVVSHCAWLRFFLKYNLLQVI

SEQ ID NO: 6515 - protein, 18 aa, Homo sapiens
MHTSVHTHVQSADGSSSV

SEQ ID NO: 6516 - protein, 29 aa, Homo sapiens
MHVQPGDTSAGLKLPYPANIAEKLFIKQM

SEQ ID NO: 6517 - protein, 14 aa, Homo sapiens
MHWIIYCTEKVLYI

SEQ ID NO: 6518 - protein, 14 aa, Homo sapiens
MHWPRPPKVLGLQV

SEQ ID NO: 6519 - protein, 36 aa, Homo sapiens
MIAAVSPSSWLSHIGICFCCPSFPIHLPEERRSTWS

SEQ ID NO: 6520 - protein, 19 aa, Homo sapiens
MIALVYNENVFLLKLHFVQ

SEQ ID NO: 6521 - protein, 99 aa, Homo sapiens
MIAVMASGRRLPSELELVDEGKTVLFSFAEVVCICPQARPQRASRNGRPSARSSPSPGFAMGWVAGWQRRGRGFSRSPLLPHLRPGAPATGHLARASLT

SEQ ID NO: 6522 - protein, 102 aa, Homo sapiens
MIAVMASGRRLPSELELVDEGKTVLFSFAEVVCICPQARPQRASRNGRPSARSSPSPGFAMGWVAGWQRRGRGFSRSPLLPHLRPGAPATGHLGERTSGLCT

SEQ ID NO: 6523 - protein, 22 aa, Homo sapiens
MICCFCFFSKKTQQAGRSGSCL

SEQ ID NO: 6524 - protein, 13 aa, Homo sapiens
MICLPRHPKVLGL

SEQ ID NO: 6525 - protein, 13 aa, Homo sapiens
MICLPWPPKVLGL

SEQ ID NO: 6526 - protein, 15 aa, Homo sapiens
MICLPWPPKVLGLQA

SEQ ID NO: 6527 - protein, 15 aa, Homo sapiens
MICLPWPPKVLGLQV

SEQ ID NO: 6528 - protein, 15 aa, Homo sapiens
MICLPWPPKVLRLQA

SEQ ID NO: 6529 - protein, 37 aa, Homo sapiens
MICLPWPPKVMRLPGLRFLNRNFKVKILMAIFKSSTS

SEQ ID NO: 6530 - protein, 15 aa, Homo sapiens
MICPLWPPKMLGLQA

SEQ ID NO: 6531 - protein, 15 aa, Homo sapiens
MICPPQPPKVLALQA

SEQ ID NO: 6532 - protein, 39 aa, Homo sapiens
MICPPWPPQSAGITGVSHCAWPRSIIFKVTMLIWQFSIF

SEQ ID NO: 6533 - protein, 15 aa, Homo sapiens
MICPPWPPRVLGLQA

SEQ ID NO: 6534 - protein, 15 aa, Homo sapiens
MICPSQPLKLLGLQA

SEQ ID NO: 6535 - protein, 15 aa, Homo sapiens
MICPTSPTKVLGLQA

SEQ ID NO: 6536 - protein, 28 aa, Homo sapiens
MICSSCLLIILMCLHPWIPYNRKILLNN

SEQ ID NO: 6537 - protein, 18 aa, Homo sapiens
MIEGSLKKYQTGLGSSLT

SEQ ID NO: 6538 - protein, 50 aa, Homo sapiens
MIFGFLFFFYFIFRDGVSPCRSGYSGVAQSWLTATSASQVQAILLPQLPK

SEQ ID NO: 6539 - protein, 15 aa, Homo sapiens
MIFPCHLGPHISWLE

SEQ ID NO: 6540 - protein, 15 aa, Homo sapiens
MIHLPRPPKVLGLQV

SEQ ID NO: 6541 - protein, 15 aa, Homo sapiens
MIHLPWPHKVLRLQA

SEQ ID NO: 6542 - protein, 11 aa, Homo sapiens
MIHLPWPPKVL

SEQ ID NO: 6543 - protein, 13 aa, Homo sapiens
MIHLPWPTKVLGL

SEQ ID NO: 6544 - protein, 13 aa, Homo sapiens
MIHPARPPKVRGL

SEQ ID NO: 6545 - protein, 15 aa, Homo sapiens
MIHPHQTPKVLGLQA

SEQ ID NO: 6546 - protein, 15 aa, Homo sapiens
MIHPPLPPKVLGLQG

SEQ ID NO: 6547 - protein, 43 aa, Homo sapiens
MIHPPQLKTIQKISQAWWCMPVIPATWKAEARESLEPGRQRLQ

SEQ ID NO: 6548 - protein, 26 aa, Homo sapiens
MIHPPQPLKSAGIKGVSHHTQPRGFF

SEQ ID NO: 6549 - protein, 15 aa, Homo sapiens
MIHPPQPPKVLGLQT

SEQ ID NO: 6550 - protein, 15 aa, Homo sapiens
MIHPPRPPRVLGLQA

SEQ ID NO: 6551 - protein, 15 aa, Homo sapiens
MIHPPWPPKLLVLQA

SEQ ID NO: 6552 - protein, 12 aa, Homo sapiens
MIHPPWPPKVLG

SEQ ID NO: 6553 - protein, 15 aa, Homo sapiens
MIHPPWPSKLLGLQA

SEQ ID NO: 6554 - protein, 15 aa, Homo sapiens
MIHPSRPPKVLGLQV

SEQ ID NO: 6555 - protein, 64 aa, Homo sapiens
MIHRLQTFPITTFQLVLHQQTFERMLFHRLTILNSLLIKLVVVGNFLIESNSKHNEQMLASSNQ

SEQ ID NO: 6556 - protein, 15 aa, Homo sapiens
MIHSPQPLKVLGLQV

SEQ ID NO: 6557 - protein, 12 aa, Homo sapiens
MIINNFPTGSHF

SEQ ID NO: 6558 - protein, 24 aa, Homo sapiens
MIKLHEFHPQYVHEQLGLQHFEVL

SEQ ID NO: 6559 - protein, 21 aa, Homo sapiens
MILAHCNLRVPGSSDSPALAS

SEQ ID NO: 6560 - protein, 15 aa, Homo sapiens
MILDFHTYNHLTFKE

SEQ ID NO: 6561 - protein, 100 aa, Homo sapiens
MILETSCSGTIRSFVCAFKYFLFISLLRFASDLTLGSFCICCLSTAKGWGSCGTVFVKFCSPFTIVKVSLLDISLVFGDFSWNLGRQILFSLSRFVLGSV

SEQ ID NO: 6562 - protein, 38 aa, Homo sapiens
MILGKLFNLLGVSVFYFSIFLCFHFCLLLYLRWWFRCQ

SEQ ID NO: 6563 - protein, 46 aa, Homo sapiens
MILILALQYRLHAPPPPCAHCRMVFLQSKTQLQSLCPEWVFFFLFR

SEQ ID NO: 6564 - protein, 25 aa, Homo sapiens
MILITEAKTHSERCLNPSECSSVKC

SEQ ID NO: 6565 - protein, 25 aa, Homo sapiens
MILITVFLLSFNIIQLTLQEPVFLY

SEQ ID NO: 6566 - protein, 127 aa, Homo sapiens
MILLSFMFNKLFLEMHCIEVQPPDVAWIIGHINLSFFFSVLACYSKVFVLIHHKPCKRQIHFCCHLCKICIPCNLLEFFPAFLIHWIPWSPWNLPVLYFFLFYGDQCHAEGQQSHTLIFYLPFDFLL

SEQ ID NO: 6567 - protein, 133 aa, Homo sapiens
MILLSFMFNKLFLEMHCIEVQPPDVAWIIGHINLSFFFSVLACYSKVFVLIHHKPCKRQIHFCCHLCKICIPCNLLEFFPAFLIHWIPWSPWNLPVLYFFLFYGDQCHAEGQQSHTLIFYLPPSCSIAFSNTI

SEQ ID NO: 6568 - protein, 28 aa, Homo sapiens
MILLSFMFTVIFVRFVFLVIFWSFFLLS

SEQ ID NO: 6569 - protein, 46 aa, Homo sapiens
MILLTRWRPRTAPPVAPVSRISMGSSNSLSLSSMMEIFIKLKFCPC

SEQ ID NO: 6570 - protein, 24 aa, Homo sapiens
MILNLSGLEQKRLISYLCHVSFED

SEQ ID NO: 6571 - protein, 15 aa, Homo sapiens
MILPPRPPKVLGLQA

SEQ ID NO: 6572 - protein, 39 aa, Homo sapiens
MILRFFKICLTFGLLSKYTRLTFTLLSEPRHCRVAIVRF

SEQ ID NO: 6573 - protein, 45 aa, Homo sapiens
MILWEILEEYLPCTLLSVVFPQRVFCLIKVLQSKHGLQSESLLVH

SEQ ID NO: 6574 - protein, 23 aa, Homo sapiens
MIMFSRFIHVAACSRTSFLFKAK

SEQ ID NO: 6575 - protein, 24 aa, Homo sapiens
MINHLLHTPPSNPVIFESKASYSL

SEQ ID NO: 6576 - protein, 35 aa, Homo sapiens
MIPLKHSNFLCDSMSSPRLGLYLIYFGVFDMKHII

SEQ ID NO: 6577 - protein, 34 aa, Homo sapiens
MIPLVNFSCFLRRRKWRTAFCITDAALFRWLRHS

SEQ ID NO: 6578 - protein, 16 aa, Homo sapiens
MIPNRCFLKRALILFK

SEQ ID NO: 6579 - protein, 27 aa, Homo sapiens
MIPTSGCEEVRSISQELLPSLLMAVHW

SEQ ID NO: 6580 - protein, 11 aa, Homo sapiens
MIQNDEMSTPH

SEQ ID NO: 6581 - protein, 25 aa, Homo sapiens
MIQRKGYINNVMSSTTKSPQDSRTP

SEQ ID NO: 6582 - protein, 18 aa, Homo sapiens
MIRILPQQSMDYLLFKSH

SEQ ID NO: 6583 - protein, 17 aa, Homo sapiens
MIRKDMRYNFSQSFQIY

SEQ ID NO: 6584 - protein, 108 aa, Homo sapiens
MIRKSGFLMILETSCSGTIRSFVCAFKYFLFISLLRFASDLTLGSFCICCLSTAKGWGSCGTVFVKFCSPFTIVKVSLLDISLVFGDFSWNLGRQILFSLSRFVLGSV

SEQ ID NO: 6585 - protein, 15 aa, Homo sapiens
MIRLPQPLKVLGLQA

SEQ ID NO: 6586 - protein, 15 aa, Homo sapiens
MIRLPRPPKMLGLQV

SEQ ID NO: 6587 - protein, 15 aa, Homo sapiens
MIRLPRPPKVLGLQS

SEQ ID NO: 6588 - protein, 15 aa, Homo sapiens
MIRLPWPPKVLGLQA

SEQ ID NO: 6589 - protein, 21 aa, Homo sapiens
MIRMLELVHCAEAGFRGGSEG

SEQ ID NO: 6590 - protein, 15 aa, Homo sapiens
MIRPHWPPKVLGLQV

SEQ ID NO: 6591 - protein, 106 aa, Homo sapiens
MIRPPQPPKVLGLQVGATVPGPLVLLNNRVELQVPSYLLSLSPLQFHMDLLPLGRGEKPIPNVCGYFTHLVSFLPRQIQLNNRTYFSSKDQHTALLGADICSFPSH

SEQ ID NO: 6592 - protein, 15 aa, Homo sapiens
MIRPPRPPKLLGLQR

SEQ ID NO: 6593 - protein, 15 aa, Homo sapiens
MIRPPRPPKVLGLQV

SEQ ID NO: 6594 - protein, 15 aa, Homo sapiens
MIRPPWPPRVLGLQV

SEQ ID NO: 6595 - protein, 15 aa, Homo sapiens
MIRPPWPSKVLGLQA

SEQ ID NO: 6596 - protein, 15 aa, Homo sapiens
MIRPTWPPKVLGLQT

SEQ ID NO: 6597 - protein, 15 aa, Homo sapiens
MIRSPWPPKVLGLQV

SEQ ID NO: 6598 - protein, 74 aa, Homo sapiens [sequence omitted]

SEQ ID NO: 6599 - protein, 39 aa, Homo sapiens
MISCTCEKYDQNVSFGSSAHLLTSCLIISSNSVLVKDTG

SEQ ID NO: 6600 - protein, 53 aa, Homo sapiens
MISDTFLGAVTKKLKEILGFKLATRTSSSNSFCPASVEFEMSHLCRGPSCLAA

SEQ ID NO: 6601 - protein, 34 aa, Homo sapiens
MISDTFLGAVTKKLKEILGFKLATRTSSSPKRII

SEQ ID NO: 6602 - protein, 59 aa, Homo sapiens
MISFSVMNTCCSSPSICASHFHHVIYRHFFCSVNNVIFIIIIFNITLIQNHFNYFTIGQ

SEQ ID NO: 6603 - protein, 35 aa, Homo sapiens
MISIISVGSITTLLISKGPLNVSTRQISRTLGESF

SEQ ID NO: 6604 - protein, 59 aa, Homo sapiens
MISPQRSILKHDPPPAKRLALTKGPDNCWHFFNNKLFLKYIFFRHNAIAHLVCYSIVYK

SEQ ID NO: 6605 - protein, 35 aa, Homo sapiens
MISRLPPHCHTRNEISRFSPPHTSIIMSYFPSSSK

SEQ ID NO: 6606 - protein, 33 aa, Homo sapiens
MISTRPGLPKCWDYRRKPLCLVFFLLKYRHLYL

SEQ ID NO: 6607 - protein, 27 aa, Homo sapiens
MITETLSIVNKKNNNSSSLFKLCFLVT

SEQ ID NO: 6608 - protein, 29 aa, Homo sapiens
MITHWSAVLQKDSGEFDSVVSKGSSESSV

SEQ ID NO: 6609 - protein, 11 aa, Homo sapiens
MIVSLTTFSYF

SEQ ID NO: 6610 - protein, 22 aa, Homo sapiens
MIVYYTLCAFNSSTLVMFDNQE

SEQ ID NO: 6611 - protein, 14 aa, Homo sapiens
MIWLNLCNSEVGSS

SEQ ID NO: 6612 - protein, 19 aa, Homo sapiens
MIWRPCNEYPFISLGILRI

SEQ ID NO: 6613 - protein, 16 aa, Homo sapiens
MIYLLLDHCPEALPLL

SEQ ID NO: 6614 - protein, 25 aa, Homo sapiens
MIYNPLGIYPVMGLLGQMVFLILDP

SEQ ID NO: 6615 - protein, 87 aa, Homo sapiens
MKAKQCYSHLQKWSVFAPRLGPSGPAGTAGPAPEAAPARGSPWAGWRVGSAEEGASRARPSYRISGQGHLRRGTWESALPACAPEPR

SEQ ID NO: 6616 - protein, 79 aa, Homo sapiens
MKAKQCYSHLQKWSVFAPRLGPSGPAGTAGPAPEAAPARGSPWAGWRVGSAEEGASRARPSYRISGQGHLRRGTWPGRL

SEQ ID NO: 6617 - protein, 26 aa, Homo sapiens
MKARTIASLLEMYERRHAKLKIVLKN

SEQ ID NO: 6618 - protein, 11 aa, Homo sapiens
MKCQLHINLTL

SEQ ID NO: 6619 - protein, 31 aa, Homo sapiens
MKDVQHFIWRNSHFLDPFSRRSSLGPDVVKM

SEQ ID NO: 6620 - protein, 17 aa, Homo sapiens
MKDVQHLQYSAVEYIHS

SEQ ID NO: 6621 - protein, 17 aa, Homo sapiens
MKEAAAAVASDRVPQRR

SEQ ID NO: 6622 - protein, 34 aa, Homo sapiens
MKEAGANPLTERNQRVLAMDIGHLVRMLLWVFMR

SEQ ID NO: 6623 - protein, 17 aa, Homo sapiens
MKEFHNILFRQACNSAP

SEQ ID NO: 6624 - protein, 63 aa, Homo sapiens
MKFLSPSKKYVLLVQRSFYAFSTVSLSFQILPPASSHQPRHFILLSNRADNLIPAVWEAKAGS

SEQ ID NO: 6625 - protein, 37 aa, Homo sapiens
MKFQRYFILLSYTHTHTHTHTHTHTHHTLDRISPHFL

SEQ ID NO: 6626 - protein, 74 aa, Homo sapiens [sequence omitted]

SEQ ID NO: 6627 - protein, 12 aa, Homo sapiens
MKGIFTREKFLD

SEQ ID NO: 6628 - protein, 53 aa, Homo sapiens
MKGLADVFRTEFSGSQLCRFSHLKYRVQWHEVHSHCCTTITTIRLQNSFIFPD

SEQ ID NO: 6629 - protein, 46 aa, Homo sapiens
MKGRRSSEPKAKGWRTRASSEQSGSAETSSRMPPGRGVVEKHRATG

SEQ ID NO: 6630 - protein, 54 aa, Homo sapiens
MKGSFGLPTQLMGGEKGNPFLLGLDVSSLIWGASRLLPLLLDHTTSLCCSCQHC

SEQ ID NO: 6631 - protein, 30 aa, Homo sapiens
MKGTGTQKYNRQGIHQTSSKLQGCLGQKRL

SEQ ID NO: 6632 - protein, 22 aa, Homo sapiens
MKHHRTSFRMAQMQIIDNTKCW

SEQ ID NO: 6633 - protein, 20 aa, Homo sapiens
MKHHYGIHAKIHGEHRTIDF

SEQ ID NO: 6634 - protein, 16 aa, Homo sapiens
MKIAAFYLPLSHFEYI

SEQ ID NO: 6635 - protein, 12 aa, Homo sapiens
MKIENDLALFYV

SEQ ID NO: 6636 - protein, 77 aa, Homo sapiens
MKIENDLALFYVYCHLCKICIPCNLLEFFPAFLIHWIPWSPWNLPVLYFFLFYGDQCHAEGQQSHTLIFYLPFDFLL

SEQ ID NO: 6637 - protein, 36 aa, Homo sapiens
MKIENDLALFYVYFLRTSQSLQFPDLHHQDKTRNGP

SEQ ID NO: 6638 - protein, 12 aa, Homo sapiens
MKIIQENLSHDM

SEQ ID NO: 6639 - protein, 28 aa, Homo sapiens
MKISANRGPSWSMNGVLYNELNKFLKFH

SEQ ID NO: 6640 - protein, 28 aa, Homo sapiens
MKKFVYSFSFIFYFFFSLTEHNSELKAL

SEQ ID NO: 6641 - protein, 36 aa, Homo sapiens
MKKHQDFRNIFFFGQSYMTQINMTKKMKTFFPYLYF

SEQ ID NO: 6642 - protein, 28 aa, Homo sapiens
MKKTMINHLLHTPPSNPVIFESKASYSL

SEQ ID NO: 6643 - protein, 20 aa, Homo sapiens
MKKYEGGMLTSLVYLLYSKI

SEQ ID NO: 6644 - protein, 19 aa, Homo sapiens
MKKYLEESFQKLSPRKKKD

SEQ ID NO: 6645 - protein, 34 aa, Homo sapiens
MKLPLKSPHCSWAALFSSSMASWKISKLPEYHRS

SEQ ID NO: 6646 - protein, 30 aa, Homo sapiens
MKLTPFLTKNLQIHGRLTYVTTFIFIKSPT

SEQ ID NO: 6647 - protein, 20 aa, Homo sapiens
MKMCSGKSLCSEQENKPASG

SEQ ID NO: 6648 - protein, 11 aa, Homo sapiens
MKMYVHIKTCT

SEQ ID NO: 6649 - protein, 14 aa, Homo sapiens
MKNACSTRRHICRA

SEQ ID NO: 6650 - protein, 32 aa, Homo sapiens
MKNLFAQETVGKNKTNQSVFKKLDTVKTWLGF

SEQ ID NO: 6651 - protein, 39 aa, Homo sapiens
MKPENVLYLLLLPPCALPPSSLMKTSSPASRCRITLLLA

SEQ ID NO: 6652 - protein, 55 aa, Homo sapiens
MKPGWSPSPDLVIPPPWPPKVLGLQARATAPTSSKFRYMYLLLKKNMPNLKQIVL

SEQ ID NO: 6653 - protein, 15 aa, Homo sapiens
MKPHNMWSLCLVSFI

SEQ ID NO: 6654 - protein, 23 aa, Homo sapiens
MKPRTLALSVTVLKGGVSGVCSF

SEQ ID NO: 6655 - protein, 17 aa, Homo sapiens
MKRCWQDYGETGMLLHC

SEQ ID NO: 6656 - protein, 34 aa, Homo sapiens
MKRGPCRKFSRSSGSWPCCWWSRGTSLGSSPVMA

SEQ ID NO: 6657 - protein, 17 aa, Homo sapiens
MKRLLLCNALIIRYYPR

SEQ ID NO: 6658 - protein, 36 aa, Homo sapiens
MKSEVDKLTFKKYISLLSKLRQEDHLSPGVRGFNEL

SEQ ID NO: 6659 - protein, 17 aa, Homo sapiens
MKSPMLFLAELTHLCLA

SEQ ID NO: 6660 - protein, 37 aa, Homo sapiens
MKSYSMLSFVPGFFHFQHAFRVHHVCKAVSLCRKQKH

SEQ ID NO: 6661 - protein, 21 aa, Homo sapiens
MKTKKPYFRFKYLKFCLPNYL

SEQ ID NO: 6662 - protein, 33 aa, Homo sapiens
MKTLFQNSLTLLPVQETSFHILLLLQNLPFMIT

SEQ ID NO: 6663 - protein, 14 aa, Homo sapiens
MKTRIYKRNEEHQK

SEQ ID NO: 6664 - protein, 30 aa, Homo sapiens
MKTSKAIATKANIGKWDLIKLKRFCKRSYH

SEQ ID NO: 6665 - protein, 12 aa, Homo sapiens
MKVFPLFSKLCT

SEQ ID NO: 6666 - protein, 95 aa, Homo sapiens
MKVINCPTKANHLLYANRHHQELRGHSQQHPAHAPQEVPSPRSMHGSFHRASTSLHSQKPVRMKRKGTCPTNPPKAPEHQPPPHKTIKMLTDFSQ

SEQ ID NO: 6667 - protein, 11 aa, Homo sapiens
MKVKESVTVCT

SEQ ID NO: 6668 - protein, 34 aa, Homo sapiens
MKVKNNYFSKNGNQPPYLFLSSSTELSFNPDLSM

SEQ ID NO: 6669 - protein, 12 aa, Homo sapiens
MKVQASHSTTLL

SEQ ID NO: 6670 - protein, 37 aa, Homo sapiens
MKWASRWFWRLREAWRGRPCRVKAMNQPSCRAFWKAV

SEQ ID NO: 6671 - protein, 40 aa, Homo sapiens
MKYITWFPPSFNFFRCGFNSSLQYAHVSCYPVENIKTHSI

SEQ ID NO: 6672 - protein, 142 aa, Homo sapiens
MLAAATPPVRGSERGLLARPPPLLLRPPTARSALPFNSPRGDPSMRFLLPLFVRLLLRRHRPYYAHRSDLRSHFTHKHTFKWPDRPPVRASRKRRPRTARWALESLLRPPLVGRSSSRDEHAGSGRSQLFSAGLSNRASIVK

SEQ ID NO: 6673 - protein, 66 aa, Homo sapiens
MLAGNPLQCSEGSRPENDQVQSIGSKGPQKLGEKFTETIQRFQKNLVTAPIVSSTILFLLFCFQHP

SEQ ID NO: 6674 - protein, 32 aa, Homo sapiens
MLAIYFIFVMDTSPCLIYFYQHVPLKARASAE

SEQ ID NO: 6675 - protein, 11 aa, Homo sapiens
MLAKMVSNSTS

SEQ ID NO: 6676 - protein, 51 aa, Homo sapiens
MLALSDGYLFIYLFILRQSLALLPRLECNGAISAHCNLRLPGSRNSPASAS

SEQ ID NO: 6677 - protein, 47 aa, Homo sapiens
MLALTGDKSASFVTSSLDMSSASCFIPLLISVRSTVCPVCRNTSTAC

SEQ ID NO: 6678 - protein, 44 aa, Homo sapiens
MLARIVSISSPRDLPASASQSAGIIGVSHGARPLYYLCIFLIVF

SEQ ID NO: 6679 - protein, 27 aa, Homo sapiens
MLARLFSNSRPQTICLPRPPKVLGLQV

SEQ ID NO: 6680 - protein, 16 aa, Homo sapiens
MLARLKEADFCPSLSF

SEQ ID NO: 6681 - protein, 18 aa, Homo sapiens
MLARLQRNRNTFTLLVGK

SEQ ID NO: 6682 - protein, 36 aa, Homo sapiens
MLARLSLQRECGSDRTLISDFWSLGFDATSSSTVVG

SEQ ID NO: 6683 - protein, 26 aa, Homo sapiens
MLARLVFNSYLVIHPPRPPKVLGLQA

SEQ ID NO: 6684 - protein, 27 aa, Homo sapiens
MLARLVLNSWAQAICPPQPPRALGLQE

SEQ ID NO: 6685 - protein, 24 aa, Homo sapiens
MLARLVLNSWPHVICPPWPLKVLE

SEQ ID NO: 6686 - protein, 27 aa, Homo sapiens
MLARLVLNSWVPVILPPQPPKVLGLEV

SEQ ID NO: 6687 - protein, 25 aa, Homo sapiens
MLARLVSGPQVICTLRLPKLLELQS

SEQ ID NO: 6688 - protein, 27 aa, Homo sapiens
MLARLVSKSQPQVIHLPWPPKVLGLQA

SEQ ID NO: 6689 - protein, 27 aa, Homo sapiens
MLARLVSNSGLQVIHPPQPLKVLGLQV

SEQ ID NO: 6690 - protein, 27 aa, Homo sapiens
MLARLVSNSLPQVIHPTHPPKVLRLQA

SEQ ID NO: 6691 - protein, 27 aa, Homo sapiens
MLARLVSNSQPQVIHPPWPPKVLGLQV

SEQ ID NO: 6692 - protein, 27 aa, Homo sapiens
MLARLVSNSRPQMIHLPWPHKVLRLQA

SEQ ID NO: 6693 - protein, 27 aa, Homo sapiens
MLARLVSNSSPQVISPPRPPKVLRLQV

SEQ ID NO: 6694 - protein, 37 aa, Homo sapiens
MLARLVSNSWPCDPPAAASQSAAIRGVSHRTQSSISF

SEQ ID NO: 6695 - protein, 37 aa, Homo sapiens
MLARLVSNSWPCDPPSAASQSAGIRGLSYRSRSSISF

SEQ ID NO: 6696 - protein, 24 aa, Homo sapiens
MLARLVSNSWPQVGCLPRPPKVLG

SEQ ID NO: 6697 - protein, 27 aa, Homo sapiens
MLARLVSNSWPQVIHPLRPPKVLGLQA

SEQ ID NO: 6698 - protein, 52 aa, Homo sapiens
MLARLVSNSWPRVIRPPRLPKVPGLQIGMSYRTRPQCTLNKASQKKKQKQNK

SEQ ID NO: 6699 - protein, 27 aa, Homo sapiens
MLARLVSNSYPQVICPPRPPKVLGLQA

SEQ ID NO: 6700 - protein, 18 aa, Homo sapiens
MLARLWRNRNAFTLLIGV

SEQ ID NO: 6701 - protein, 18 aa, Homo sapiens
MLARLWRNRNAFTPLIGV

SEQ ID NO: 6702 - protein, 18 aa, Homo sapiens
MLARLWRNRNTFILLVGM

SEQ ID NO: 6703 - protein, 21 aa, Homo sapiens
MLARMVSISRISFLSLFSFAS

SEQ ID NO: 6704 - protein, 37 aa, Homo sapiens
MLARMVSISRPRDPPASASQSAGTTGMSHRARPCFCF

SEQ ID NO: 6705 - protein, 19 aa, Homo sapiens
MLARMVSIYRPQDLPISAS

SEQ ID NO: 6706 - protein, 11 aa, Homo sapiens
MLARMVSNTWP

SEQ ID NO: 6707 - protein, 26 aa, Homo sapiens
MLARMVSSPDLVIHPPQPPKVLGLQA

SEQ ID NO: 6708 - protein, 12 aa, Homo sapiens
MLASLLPSGGQH

SEQ ID NO: 6709 - protein, 24 aa, Homo sapiens
MLASNSRPQVIHPPQPPRVLGLQA

SEQ ID NO: 6710 - protein, 25 aa, Homo sapiens
MLASVVSNSSHQVIHPPRWVLGLQA

SEQ ID NO: 6711 - protein, 27 aa, Homo sapiens
MLATLVSNSWPQVIHPPWPAKVLRLQA

SEQ ID NO: 6712 - protein, 24 aa, Homo sapiens
MLAVSPKTFSSSAAAVRVNDASEL

SEQ ID NO: 6713 - protein, 54 aa, Homo sapiens
MLDLWPSLQIYKVDFYFAVRAKALQGSYSPVLNECCPFGFCVSFFLVGIIGCND

SEQ ID NO: 6714 - protein, 83 aa, Homo sapiens
MLDLWPSLQIYKVDFYFAVRAKALQGSYSPVLNECCPFGFCVSFLHLQFSDASHVFWEDPRQLFQSATAISEVFLVGIIGCND

SEQ ID NO: 6715 - protein, 51 aa, Homo sapiens
MLDQAGLELLASGHLPTSASQIAGITGVSHRARPPFPLCCAPLYTVGGRSW

SEQ ID NO: 6716 - protein, 27 aa, Homo sapiens
MLDVLVLDSWPEVIYLPQPPKVLGLQV

SEQ ID NO: 6717 - protein, 61 aa, Homo sapiens [sequence omitted]

SEQ ID NO: 6718 - protein, 20 aa, Homo sapiens
MLEEYCFSKFFISFLRDVPI

SEQ ID NO: 6719 - protein, 87 aa, Homo sapiens
MLEGMWRNRNTFHCWWDCKLVQPLWKTVWQFLKDLELEIPFNPAIPLLGIYPKDYKSFYYKDTCMFTAALLTIAKTWNQPKCPSVID

SEQ ID NO: 6720 - protein, 15 aa, Homo sapiens
MLEHVINTSFFFMAK

SEQ ID NO: 6721 - protein, 18 aa, Homo sapiens
MLELVHCAEAGFRGGSEG

SEQ ID NO: 6722 - protein, 24 aa, Homo sapiens
MLEPLLNLRAAAEAMEGSSGGWAS

SEQ ID NO: 6723 - protein, 26 aa, Homo sapiens
MLEQKANWIFDSSFKELRKITHNWFK

SEQ ID NO: 6724 - protein, 18 aa, Homo sapiens
MLERIWRTRNTFTLLVGV

SEQ ID NO: 6725 - protein, 18 aa, Homo sapiens
MLERTGRNRNTFTLLVGV

SEQ ID NO: 6726 - protein, 27 aa, Homo sapiens
MLFGRHGVSALQPKVEVADLTSHRDAH

SEQ ID NO: 6727 - protein, 14 aa, Homo sapiens
MLFKISTLSEGFPT

SEQ ID NO: 6728 - protein, 14 aa, Homo sapiens
MLFKISTLTEGFPT

SEQ ID NO: 6729 - protein, 14 aa, Homo sapiens
MLFKTSTLTEGFPT

SEQ ID NO: 6730 - protein, 21 aa, Homo sapiens
MLFKYFISSLSLTNSRFSLSS

SEQ ID NO: 6731 - protein, 13 aa, Homo sapiens
MLFLAELTHLCLA

SEQ ID NO: 6732 - protein, 60 aa, Homo sapiens
MLFLHVGEAGLELWISGDPPTLASQSVGITGMSHCARQRKSLLKLMSYPSGCLKLGPVQT

SEQ ID NO: 6733 - protein, 32 aa, Homo sapiens
MLFLVQLTIAVQRRSRCWETIFLLPLENWMQF

SEQ ID NO: 6734 - protein, 26 aa, Homo sapiens
MLFRLVSTADLMIHPSRPPKVLGLQV

SEQ ID NO: 6735 - protein, 39 aa, Homo sapiens
MLFSCCCQWRIVSIRYTHMLMFPTSTDLPTLWTSVHKDV

SEQ ID NO: 6736 - protein, 20 aa, Homo sapiens
MLFSCSTPSILDSNWLTTVS

SEQ ID NO: 6737 - protein, 45 aa, Homo sapiens
MLFSLTCCLIFSSFRLSCFSFANSIASFSSCLSWSSFNLLFSSAF

SEQ ID NO: 6738 - protein, 120 aa, Homo sapiens
MLFTHFLHYHPLIFQHRPDVGEGLPQHQLDLKGLEASDPRKSHPVAFLGQLQPPRHFVNHHLDLVFIRRAANSPVPSQDIVSNFLLLFFIHIWDSVFEKLVIVEAILIQKLNTGSLEGEF

SEQ ID NO: 6739 - protein, 82 aa, Homo sapiens
MLFTHFLHYHPLIFQHRPDVGEGLPQHQLDLKGLEASDPRKSHPVAFLGQLQPPRHFVNHHLDLVFIRRAKEDDFFSEALMQ

SEQ ID NO: 6740 - protein, 17 aa, Homo sapiens
MLGNGLIVSATKWHCPN

SEQ ID NO: 6741 - protein, 83 aa, Homo sapiens
MLGRACLSTSWTSKAWKPVIPGRVIQSPSLASSSHRVTSSITTLIWSLSGELRTLQFPVRISCLIFFSCSSFIYGIPFLRNLL

SEQ ID NO: 6742 - protein, 90 aa, Homo sapiens
MLGRACLSTSWTSKAWKPVIPGRVIQSPSLASSSHRVTSSITTLIWSLSGEQKKTISSLRLLCNRKPNNWKNSPQPSIGSRHIFNPLLLH

SEQ ID NO: 6743 - protein, 41 aa, Homo sapiens
MLGSTLQGQLLPHPHLLPKCLHNMQSCCPPKASFVGQKMSL

SEQ ID NO: 6744 - protein, 42 aa, Homo sapiens
MLHHNQLIFVFSVETGFHHVGQAGLELLTSSDPSTLASQSMC

SEQ ID NO: 6745 - protein, 13 aa, Homo sapiens
MLHWCGSYFSCFC

SEQ ID NO: 6746 - protein, 24 aa, Homo sapiens
MLIHCWGEHKLVQQLWKTVWQFLK

SEQ ID NO: 6747 - protein, 33 aa, Homo sapiens
MLIIIKSKNNRYLQGCRERKAHGVACSLQHYSL

SEQ ID NO: 6748 - protein, 26 aa, Homo sapiens
MLIMVNFVQFLCPLCTCSSKLFWFCY

SEQ ID NO: 6749 - protein, 26 aa, Homo sapiens
MLINVFLVETGFHHVGQAGHELLTSK

SEQ ID NO: 6750 - protein, 27 aa, Homo sapiens
MLIRLASNSQPQVICPPQPPKVLGLQA

SEQ ID NO: 6751 - protein, 27 aa, Homo sapiens
MLIRLVTNAQPQVIHPPWLPKVLRLQA

SEQ ID NO: 6752 - protein, 31 aa, Homo sapiens
MLIRYTLSIKSTFDFLGLLSIPNISNFISPL

SEQ ID NO: 6753 - protein, 33 aa, Homo sapiens
MLISCNSKSFNADFSALYGNYLEYCTSFNRNIM

SEQ ID NO: 6754 - protein, 29 aa, Homo sapiens
MLISVPYMGIILSTVLLSIEISCRSGWQA

SEQ ID NO: 6755 - protein, 40 aa, Homo sapiens [sequence omitted]

SEQ ID NO: 6756 - protein, 35 aa, Homo sapiens [sequence omitted]

SEQ ID NO: 6757 - protein, 32 aa, Homo sapiens
MLKKEASLSTSKKLPLYMMLFKYMDKITHFMM

SEQ ID NO: 6758 - protein, 16 aa, Homo sapiens
MLKRMKIENDLALFYV

SEQ ID NO: 6759 - protein, 81 aa, Homo sapiens
MLKRMKIENDLALFYVYCHLCKICIPCNLLEFFPAFLIHWIPWSPWNLPVLYFFLFYGDQCHAEGQQSHTLIFYLPFDFLL

SEQ ID NO: 6760 - protein, 40 aa, Homo sapiens
MLKRMKIENDLALFYVYFLRTSQSLQFPDLHHQDKTRNGP

SEQ ID NO: 6761 - protein, 143 aa, Homo sapiens
MLKTLNKLDIDGMYLKIIKAIYDKLTANIILNGQNLEAFPEKTVTRQGCPLSPLLFNIMLEVLARAIRQEKKIKGIQIEREEFKLSLFADDMILYLENPIVSAQNLLKLISNFSKVSGYKINVQKPQAFLYTNNKKNREPNHE

SEQ ID NO: 6762 - protein, 106 aa, Homo sapiens
MLKTLNKLGIDGVYFKIIRAIYDKPTANIILNGQKLEAFPLKTGTRQGCPLSPLVFNIVLEVLARAIRQEKEIKGIQLGKEEVKLSVCRRHDCISRKPHRLSPKSP

SEQ ID NO: 6763 - protein, 105 aa, Homo sapiens
MLKTLNKLGTDGTYFKTIGAFYDKPTANIILNGQKLEAFPLKTSTKQGCPLSPLLFNIVLEVLVRASRQEKEIKGIKIGREEVKLSLFADDMIFRKPHHLSPKTP

SEQ ID NO: 6764 - protein, 44 aa, Homo sapiens
MLLAPGGGSYWPCLCIKSARFRALAATFRRTSPSPGLGLATSFT

SEQ ID NO: 6765 - protein, 21 aa, Homo sapiens
MLLCKMLRISFLSCPGAFPGP

SEQ ID NO: 6766 - protein, 25 aa, Homo sapiens
MLLCLHMFLLHCLVPHLDFQHHQSA

SEQ ID NO: 6767 - protein, 35 aa, Homo sapiens
MLLDYPKLQETSSQSVTLSRVSYHPIVNDVDSSSQ

SEQ ID NO: 6768 - protein, 65 aa, Homo sapiens
MLLEETPKISPHKTGERRTEICIIFCISKKSRASTIYPFFFPFPPLPSLAVFLCKLDPLHFETAI

SEQ ID NO: 6769 - protein, 14 aa, Homo sapiens
MLLFHRLYYILKVF

SEQ ID NO: 6770 - protein, 37 aa, Homo sapiens
MLLFKSAILCSRHLHGSKIILFFMCSLQTACGTRMNR

SEQ ID NO: 6771 - protein, 56 aa, Homo sapiens [sequence omitted]

SEQ ID NO: 6772 - protein, 16 aa, Homo sapiens
MLLHRMIQNDEMSTPH

SEQ ID NO: 6773 - protein, 21 aa, Homo sapiens
MLLIKASMFLSFLASFNSKSN

SEQ ID NO: 6774 - protein, 13 aa, Homo sapiens
MLLIKSYPRLGNL

SEQ ID NO: 6775 - protein, 15 aa, Homo sapiens
MLLLSVIVEWTTIIL

SEQ ID NO: 6776 - protein, 45 aa, Homo sapiens
MLLLVCYRNYSACQFFNHPKREQIQALFALFNILRSPMPISKPLS

SEQ ID NO: 6777 - protein, 13 aa, Homo sapiens
MLLNIRHALEILP

SEQ ID NO: 6778 - protein, 39 aa, Homo sapiens
MLLPSQKCMSAQAQTKLQIQENKINHADQRQTSREMKCL

SEQ ID NO: 6779 - protein, 15 aa, Homo sapiens
MLLQDSCLNFCSLEL

SEQ ID NO: 6780 - protein, 122 aa, Homo sapiens [sequence omitted]

SEQ ID NO: 6781 - protein, 16 aa, Homo sapiens
MLLRATLKSSYTMFSL

SEQ ID NO: 6782 - protein, 47 aa, Homo sapiens
MLLRLVSNSSAQSDPPTSASQSAGITGVSHHTQPFRLFLTRCYSNDS

SEQ ID NO: 6783 - protein, 30 aa, Homo sapiens
MLLSAEGSQPSGTLLPVLYFACTPLAWLLH

SEQ ID NO: 6784 - protein, 73 aa, Homo sapiens
MLLSLILGWRSLMIPRKIQYVLFFLWLFLFYTFILAKHPIWLDYEHRELSFLLILSQGSFPFVLAVFLSPSGV

SEQ ID NO: 6785 - protein, 27 aa, Homo sapiens
MLLSLILGWRSLMIPRKIQYVLSPSGV

SEQ ID NO: 6786 - protein, 20 aa, Homo sapiens
MLLSRLATLWQCSVLVPVEN

SEQ ID NO: 6787 - protein, 62 aa, Homo sapiens [sequence omitted]

SEQ ID NO: 6788 - protein, 24 aa, Homo sapiens
MLLWKDTSKSWRLNLLLKMEIQEF

SEQ ID NO: 6789 - protein, 98 aa, Homo sapiens
MLMALAGPCLSTLALAMAGGRLAWSCLRAPLLTLFLGPGYSGGGLLGMRARAACSWALYSIFSRSMGIWGTDSGASSSSSSLSLLWISIVASEKVFLW

SEQ ID NO: 6790 - protein, 29 aa, Homo sapiens
MLMVQGVVEDVPPQIWIIPLIPSFNTTCS

SEQ ID NO: 6791 - protein, 38 aa, Homo sapiens
MLNEGLYLKISNTQFWFNKFQFQFYILIGYIEFWPTES

SEQ ID NO: 6792 - protein, 15 aa, Homo sapiens
MLNFCVSSRDGVSPC

SEQ ID NO: 6793 - protein, 18 aa, Homo sapiens
MLPAKESNSLSDAMSSGC

SEQ ID NO: 6794 - protein, 105 aa, Homo sapiens
MLPCVWLKHVTTNVWGHQSKVQLSTLQQSHFVHQRLYSASSLTKKKKKDFSKAFTEKVINYICSSPFPFSTSPPYIYCRNFLLLCFFLWNIIDRRATLKHIYFFT

SEQ ID NO: 6795 - protein, 39 aa, Homo sapiens
MLPGNKGHHTYEFDTVSDIFIALNKPHNNSHGLIKSRCT

SEQ ID NO: 6796 - protein, 13 aa, Homo sapiens
MLPGWSRTPDLRF

SEQ ID NO: 6797 - protein, 58 aa, Homo sapiens [sequence omitted]

SEQ ID NO: 6798 - protein, 31 aa, Homo sapiens
MLPKRKPAKENGPPPAESSSLSVSDMMAAAV

SEQ ID NO: 6799 - protein, 40 aa, Homo sapiens
MLPKRKPAKENGPPPAESSSLSVSDMMAAAVMVAAVRSSK

SEQ ID NO: 6800 - protein, 49 aa, Homo sapiens
MLPKRKPAKENGPPPAESSSLSVSDMMAAAVMVAAVRSSKSQPGPIDRK

SEQ ID NO: 6801 - protein, 25 aa, Homo sapiens
MLPPGFFFSASGYTLSLPSGNSTVI

SEQ ID NO: 6802 - protein, 14 aa, Homo sapiens
MLPPRPPKVLGLQA

SEQ ID NO: 6803 - protein, 27 aa, Homo sapiens
MLPQHEDSLTYSLVCPKQPLASSVCFQ

SEQ ID NO: 6804 - protein, 24 aa, Homo sapiens
MLPRLANFLYFSRHGISPCCPGWS

SEQ ID NO: 6805 - protein, 44 aa, Homo sapiens
MLPRLLLAYFDIDCYSFDLQLTLKQCGGLGTPTPRSSQKSTYNF

SEQ ID NO: 6806 - protein, 24 aa, Homo sapiens
MLPRLVFSSWAQAIHPHWPPKVLR

SEQ ID NO: 6807 - protein, 27 aa, Homo sapiens
MLPRLVLNSRAQMIRPPWPPRVLGLQV

SEQ ID NO: 6808 - protein, 11 aa, Homo sapiens
MLPRLVLNSWA

SEQ ID NO: 6809 - protein, 27 aa, Homo sapiens
MLPRLVLNSWTQAVHPPRPPKMLGLQE

SEQ ID NO: 6810 - protein, 17 aa, Homo sapiens
MLPRLVSNCWAQAILLP

SEQ ID NO: 6811 - protein, 27 aa, Homo sapiens
MLPRLVSNSWAQVIHSPRPSKALGLQA

SEQ ID NO: 6812 - protein, 27 aa, Homo sapiens
MLPRLVSNSWTQAIFLPWPPKVLGLQA

SEQ ID NO: 6813 - protein, 25 aa, Homo sapiens
MLPRLVSNSWTQVTLPPWHPKVLGL

SEQ ID NO: 6814 - protein, 21 aa, Homo sapiens
MLPRMDSNSWAQVIFPPHPPE

SEQ ID NO: 6815 - protein, 50 aa, Homo sapiens
MLPVSLLKHSKGHLYSSSHQVPHRHLRPPQPAFYCTYRYRHCGQSHLTSL

SEQ ID NO: 6816 - protein, 34 aa, Homo sapiens
MLQGRTIPWSKMGADRSPEGRQKPGGFLYMGCRL

SEQ ID NO: 6817 - protein, 41 aa, Homo sapiens
MLQHAAELHSFLRLNNIPLDGYTTFCLSIHPLLHISVVSTF

SEQ ID NO: 6818 - protein, 21 aa, Homo sapiens
MLQHCRSQCSVECAYTDGNAN

SEQ ID NO: 6819 - protein, 30 aa, Homo sapiens
MLQRPRSAGPWQESHSQEPQAAGRRHLRCV

SEQ ID NO: 6820 - protein, 13 aa, Homo sapiens
MLRFFSQPGLEFS

SEQ ID NO: 6821 - protein, 16 aa, Homo sapiens
MLRISFLSCPGAFPGP

SEQ ID NO: 6822 - protein, 31 aa, Homo sapiens
MLRMEALRGCFRKISVCPADSRWRSFASIMI

SEQ ID NO: 6823 - protein, 40 aa, Homo sapiens
MLRRPANFLYFSRDGVSPCCPGWSQTPELRQSSHLGLPKC

SEQ ID NO: 6824 - protein, 87 aa, Homo sapiens
MLRSKSQGFQRSFNQCFLKVPTVLGSAGGGGGGSRSSCAELGLAGREVKGSGRLSTGTSHRIQPGNYSSGEVTAARCALQREAGASC

SEQ ID NO: 6825 - protein, 25 aa, Homo sapiens
MLRSKSSSSPPDENLLARGTLGDPW

SEQ ID NO: 6826 - protein, 118 aa, Homo sapiens
MLRSSPLITKSLQFSLLRCVSSFLHFLTSISVGHLCEEVQFHNIFLPFRQIGQAGSHFLLDGPGPGLKERSQVLLHLVGEHLDPQIHFVNIFCGQVGLVPVLGEETDEWLPTKGFLEL

SEQ ID NO: 6827 - protein, 59 aa, Homo sapiens
MLRSSPLITKSLQFSLLRCVSSFLHFLTSISVGPATSMGTPYICVRRYNFIIFSFHSGR

SEQ ID NO: 6828 - protein, 18 aa, Homo sapiens
MLRTHPNHYTLLCSPYLK

SEQ ID NO: 6829 - protein, 28 aa, Homo sapiens
MLSARPSDISQCLLWRGPRTKKTVKSYR

SEQ ID NO: 6830 - protein, 34 aa, Homo sapiens
MLSCAIGCEHCRSLATLFTLVVFSSMNYLTYNQV

SEQ ID NO: 6831 - protein, 15 aa, Homo sapiens
MLSCMSQNSKKTAQF

SEQ ID NO: 6832 - protein, 33 aa, Homo sapiens
MLSDGLSLPCTFVLLLILEKVLECSNIIELISA

SEQ ID NO: 6833 - protein, 18 aa, Homo sapiens
MLSECRQPFPKVTPRKEI

SEQ ID NO: 6834 - protein, 32 aa, Homo sapiens
MLSFVPGFFHFQHAFRVHHVCKAVSLCRKQKH

SEQ ID NO: 6835 - protein, 27 aa, Homo sapiens
MLSGFTMFARLFPCAGNRSTDQEDWGR

SEQ ID NO: 6836 - protein, 27 aa, Homo sapiens
MLSHTAYIHKVFSQSGSFHVYEGNWDT

SEQ ID NO: 6837 - protein, 38 aa, Homo sapiens
MLSILPSFLWLNNIPLCYTHTQWNTIQSLKRRQSSQIW

SEQ ID NO: 6838 - protein, 48 aa, Homo sapiens
MLSNGPLPPPTFLCSHFQGNRQDTLSSKSDHVKPLLKTITSQQNYKHT

SEQ ID NO: 6839 - protein, 25 aa, Homo sapiens
MLSPFLSTPYFVNFLRFFWLEVSLH

SEQ ID NO: 6840 - protein, 14 aa, Homo sapiens
MLSPLENIISNCFI

SEQ ID NO: 6841 - protein, 28 aa, Homo sapiens
MLSQKVVKERRVCEKCISVLCTVSVCVM

SEQ ID NO: 6842 - protein, 27 aa, Homo sapiens
MLSRLVLNSWPQETHPPQAPTALGLQA

SEQ ID NO: 6843 - protein, 50 aa, Homo sapiens
MLSTSLARRCCRPEGLRRVFSATAFISWKSDVAWSVSPVRKQSSGIRWAS

SEQ ID NO: 6844 - protein, 14 aa, Homo sapiens
MLTADQACGPAILL

SEQ ID NO: 6845 - protein, 32 aa, Homo sapiens
MLTCLELLTSGNPPTSASQSAGITGVSHHTWP

SEQ ID NO: 6846 - protein, 17 aa, Homo sapiens
MLTDLILSPVDNVCLLS

SEQ ID NO: 6847 - protein, 16 aa, Homo sapiens
MLTEMQSSRNSHSLLV

SEQ ID NO: 6848 - protein, 45 aa, Homo sapiens
MLTRKLYDTSDRNYTNCLAILTNIVLKTQLNIMILKNKENTTCSW

SEQ ID NO: 6849 - protein, 11 aa, Homo sapiens
MLTRPLLLPPF

SEQ ID NO: 6850 - protein, 12 aa, Homo sapiens
MLTSWSRTPDLK

SEQ ID NO: 6851 - protein, 16 aa, Homo sapiens
MLVARELPVSIPAVLG

SEQ ID NO: 6852 - protein, 43 aa, Homo sapiens
MLVEMGFHHVCQAGLKLLTSGDPPALASRSAGITGVSHYIQPR

SEQ ID NO: 6853 - protein, 12 aa, Homo sapiens
MLVEQGWFISLS

SEQ ID NO: 6854 - protein, 15 aa, Homo sapiens
MLVFLVEDKKSSSFS

SEQ ID NO: 6855 - protein, 27 aa, Homo sapiens
MLVGLVSNSQPQVTHPPRPPRVLGLQA

SEQ ID NO: 6856 - protein, 27 aa, Homo sapiens
MLVGLVSNSRPQVIRPPWPPKVLGLQA

SEQ ID NO: 6857 - protein, 12 aa, Homo sapiens
MLVGQAGLELLT

SEQ ID NO: 6858 - protein, 19 aa, Homo sapiens
MLVIENLEDIKDNKEEIKS

SEQ ID NO: 6859 - protein, 101 aa, Homo sapiens
MLVKIWSNGNPHSSLVECKTVQPLWKAVWLCLARLNIALTYHIYPNELKTYVHTKTCIQIFIVALFITDQTWKQPRCPSVGEWINKQWYIQKMDECLVLKK

SEQ ID NO: 6860 - protein, 27 aa, Homo sapiens
MLVKLVSNSGPQVICPPWPPKVLGLEA

SEQ ID NO: 6861 - protein, 24 aa, Homo sapiens
MLVRLDNIFISPRKSLAPTWRTSF

SEQ ID NO: 6862 - protein, 16 aa, Homo sapiens
MLVRLGLGFLIKYHSL

SEQ ID NO: 6863 - protein, 18 aa, Homo sapiens
MLVRLQRKENAYTLLGGT

SEQ ID NO: 6864 - protein, 79 aa, Homo sapiens
MLVRLVANSRPQVIHPPRPPKVLGLQAGATVPGHRNGIFKVLGFVHFPLLVEEGELSLLKFVPDLAPAHRLRRLQDTVP

SEQ ID NO: 6865 - protein, 64 aa, Homo sapiens
MLVRLVANSRPQVIHPPRPPKVLGLQAGATVPGHRNGIFKVLGFVHFPLLVEEGEVSMCGSDIC

SEQ ID NO: 6866 - protein, 27 aa, Homo sapiens
MLVRLVLNLRPQVIRPPWSPQVLGLQV

SEQ ID NO: 6867 - protein, 27 aa, Homo sapiens
MLVRLVLNSHPQVVRSPQPPKVLGLQA

SEQ ID NO: 6868 - protein, 38 aa, Homo sapiens
MLVRLVLNSQPQVIRPPCLPKCWDYRREPPRPAAFVDF

SEQ ID NO: 6869 - protein, 27 aa, Homo sapiens
MLVRLVLNSQSQVICPPWPPKVMGLQA

SEQ ID NO: 6870 - protein, 27 aa, Homo sapiens
MLVRLVLNSRPQVIFPPQPPKVLVLQA

SEQ ID NO: 6871 - protein, 12 aa, Homo sapiens
MLVRLVLNSYLR

SEQ ID NO: 6872 - protein, 27 aa, Homo sapiens
MLVRLVSNSGSQVIHPPWPPKVLGLQA

SEQ ID NO: 6873 - protein, 25 aa, Homo sapiens
MLVRLVSNSQPQVIACLGLPTECGF

SEQ ID NO: 6874 - protein, 27 aa, Homo sapiens
MLVRLVSNSQPQVICPPWPPKVLGLQA

SEQ ID NO: 6875 - protein, 53 aa, Homo sapiens
MLVRLVSNSQPQVIHPPRPPKVLELQAWATAPGLNRFLKNCHLQNFQLSYLGT

SEQ ID NO: 6876 - protein, 17 aa, Homo sapiens
MLVRLVSNSQPQVTYLS

SEQ ID NO: 6877 - protein, 45 aa, Homo sapiens
MLVRLVSNSRLRDPPALAFQSAGITGMSHCAGPKQNFKSAIGIQY

SEQ ID NO: 6878 - protein, 27 aa, Homo sapiens
MLVRLVSNSRPQVIHLPQPPEVLGLQA

SEQ ID NO: 6879 - protein, 27 aa, Homo sapiens
MLVRLVSNSRPQVIHLPRSLKVLGLQV

SEQ ID NO: 6880 - protein, 27 aa, Homo sapiens
MLVRLVSNSRPQVIHLPWSLKVLGLQA

SEQ ID NO: 6881 - protein, 27 aa, Homo sapiens
MLVRLVSNSRPQVIHPPRPPKVLGLQA

SEQ ID NO: 6882 - protein, 29 aa, Homo sapiens
MLVRLVSNSRPQVIRLPRPPKPWILYSPL

SEQ ID NO: 6883 - protein, 46 aa, Homo sapiens
MLVRLVSNSRPQVIRPLRPPKVLSQHFYRDEPPRLAVLHFFFSLQL

SEQ ID NO: 6884 - protein, 27 aa, Homo sapiens
MLVRLVSNSRPQVIRPPRPPKVLGSQA

SEQ ID NO: 6885 - protein, 27 aa, Homo sapiens
MLVRLVSNSWPQVIHLPQPPKVLGLEV

SEQ ID NO: 6886 - protein, 27 aa, Homo sapiens
MLVRLVVNSRPQVIRPPRPPKVLGLQA

SEQ ID NO: 6887 - protein, 14 aa, Homo sapiens
MLVRLWEKRNASTL

SEQ ID NO: 6888 - protein, 71 aa, Homo sapiens
MLVRMAIIKKSRNNRCWRGCGEIGTLLYCWWECKLVQPLWKTVWRVLKDLEMEISFDPAILLLGIYPKEYK

SEQ ID NO: 6889 - protein, 52 aa, Homo sapiens
MLVRMWSKWNSQILLREVGNGASSLENSLMIFIKLSIYLCCDSEIPSLTIYL

SEQ ID NO: 6890 - protein, 20 aa, Homo sapiens
MLVSCKVFTCLRRSFRSCSF

SEQ ID NO: 6891 - protein, 32 aa, Homo sapiens
MLVSIAESTLPSSAVSTADLSDSPGSSGAQAP

SEQ ID NO: 6892 - protein, 22 aa, Homo sapiens
MLVSLVLNSRPQVIRPGTGSEF

SEQ ID NO: 6893 - protein, 48 aa, Homo sapiens
MLVYLMMSHKFISLCSLFIFYSFCFSETVFSIFFSSSSWLPLCVQIYS

SEQ ID NO: 6894 - protein, 51 aa, Homo sapiens
MLVYLMMSHRFISLCSLFIFYSFCFSEYFPFSSLQVHGFLCVCKYTLKSLW

SEQ ID NO: 6895 - protein, 20 aa, Homo sapiens
MLWAFPRGWPLRPLGGLGTP

SEQ ID NO: 6896 - protein, 12 aa, Homo sapiens
MLWNNPFFCLCL

SEQ ID NO: 6897 - protein, 57 aa, Homo sapiens
MLWSLIFPTDIGIGLSSCSSKIADPGIYCLNFACTYIRWKNTSFIHSCYCFLCNLTS

SEQ ID NO: 6898 - protein, 60 aa, Homo sapiens
MLWSLIFPTDIGIGLSSCSSKIADPGIYCLNFACTYIRWKNTSHLTFIHSCYCFLCNLTS

SEQ ID NO: 6899 - protein, 45 aa, Homo sapiens
MLWSLIFPTDIGIGLSSCSSKIADPGIYCLNFIHSCYCFLCNLTS

SEQ ID NO: 6900 - protein, 59 aa, Homo sapiens
MLYFLQLDRQAAWNISICLFSVILVSLKTHLYPTFTIFCNFHMHCVCYSVHVSTPITEA

SEQ ID NO: 6901 - protein, 15 aa, Homo sapiens
MLYNIYLYIYNYMYI

SEQ ID NO: 6902 - protein, 22 aa, Homo sapiens
MLYSSLCRMTGHQRRQNTPRGM

SEQ ID NO: 6903 - protein, 41 aa, Homo sapiens
MMAAPTRLPIKAPTMIPTSGCEEVRSISQELLPSLLMAVHW

SEQ ID NO: 6904 - protein, 21 aa, Homo sapiens
MMECCCAHTTLWLGDHTTASS

SEQ ID NO: 6905 - protein, 51 aa, Homo sapiens
MMENSHMILWEILEEYLPCTLLSVVFPQRVFCLIKVLQSKHGLQSESLLVH

SEQ ID NO: 6906 - protein, 13 aa, Homo sapiens
MMFPSLHFPFEIF

SEQ ID NO: 6907 - protein, 27 aa, Homo sapiens
MMFRHVGQAGLELLSSSDLPTSASQSA

SEQ ID NO: 6908 - protein, 23 aa, Homo sapiens
MMFSCRHKGRSVKVRPLKAGLVI

SEQ ID NO: 6909 - protein, 23 aa, Homo sapiens
MMFSCRHKGRSVKVRPLKAGRTT

SEQ ID NO: 6910 - protein, 32 aa, Homo sapiens
MMFWIFRLFFSGIRCVHKNYECQRKYFMKLCS

SEQ ID NO: 6911 - protein, 103 aa, Homo sapiens
MMGHGRPSWMNSAFLLTDGRVLLSPRILSRWKANTSLMSKGCLRSPQGLGPQRSTAPGAPPSSTSKRAPLLEDTGRSPATALSAKSRILRMSSLLSQEGALSL

SEQ ID NO: 6912 - protein, 14 aa, Homo sapiens
MMGKTKKIKCTFTV

SEQ ID NO: 6913 - protein, 67 aa, Homo sapiens [sequence omitted]

SEQ ID NO: 6914 - protein, 15 aa, Homo sapiens
MMHPPRPPKLLGLQG

SEQ ID NO: 6915 - protein, 23 aa, Homo sapiens
MMICCFCFFSKKTQQAGRSGSCL

SEQ ID NO: 6916 - protein, 12 aa, Homo sapiens
MMKCQLHINLTL

SEQ ID NO: 6917 - protein, 40 aa, Homo sapiens
MMKPENVLYLLLLPPCALPPSSLMKTSSPASRCRITLLLA

SEQ ID NO: 6918 - protein, 31 aa, Homo sapiens
MMKTSKAIATKANIGKWDLIKLKRFCKRSYH

SEQ ID NO: 6919 - protein, 38 aa, Homo sapiens
MMLLFKSAILCSRHLHGSKIILFFMCSLQTACGTRMNR

SEQ ID NO: 6920 - protein, 25 aa, Homo sapiens
MMLPRLVFSSWAQAIHPHWPPKVLR

SEQ ID NO: 6921 - protein, 42 aa, Homo sapiens
MMMAAPTRLPIKAPTMIPTSGCEEVRSISQELLPSLLMAVHW

SEQ ID NO: 6922 - protein, 15 aa, Homo sapiens
MMNRKKLEALATCLV

SEQ ID NO: 6923 - protein, 27 aa, Homo sapiens
MMNSWWDGGHWIMMSEFLSCFWHQIVG

SEQ ID NO: 6924 - protein, 29 aa, Homo sapiens
MMPQSSELEFWCILPPLDLGREEGFLPNC

SEQ ID NO: 6925 - protein, 120 aa, Homo sapiens [sequence omitted]

SEQ ID NO: 6926 - protein, 26 aa, Homo sapiens
MMRKKNTDDFAKLPIAGCDLFYSPSL

SEQ ID NO: 6927 - protein, 43 aa, Homo sapiens
MMSHKFISLCSLFIFYSFCFSETVFSIFFSSSSWLPLCVQIYS

SEQ ID NO: 6928 - protein, 46 aa, Homo sapiens
MMSHRFISLCSLFIFYSFCFSEYFPFSSLQVHGFLCVCKYTLKSLW

SEQ ID NO: 6929 - protein, 33 aa, Homo sapiens
MMSIRTVRFNSFFSYTLINWTYSLTLESSFSNF

SEQ ID NO: 6930 - protein, 92 aa, Homo sapiens
MMSSATRKKACSSSTHQPTVQARWRLSASCFLGSTSSRNATTTVKPRLYLPPMALYSRTCSQIRIPARSRLLAGTPKSRIRSAIGSVGRVVP

SEQ ID NO: 6931 - protein, 103 aa, Homo sapiens
MMSSATRKKACSSSTHQPTVQARWRLSASCFLGSTSSRNATTTVKPRLYLPPMALYSRTCSQIRIPARSRLLAGTPKSRIRSAIGSVGRVVPALPTLRAEIYN

SEQ ID NO: 6932 - protein, 87 aa, Homo sapiens
MMSSATRKKACSSSTHQPTVQARWRLSASCFLGSTSSRNATTTVKPRLYLPPMALYSRTSLSRAIASPISGCPISSSVSTLTIWEKC

SEQ ID NO: 6933 - protein, 22 aa, Homo sapiens
MMSSLNCMVSCWSMVKPPDSHL

SEQ ID NO: 6934 - protein, 53 aa, Homo sapiens
MMSSLNCMVSCWSMVKPPDSNRKLWNFLYLRSIRDSCDNHGLIFLLLFMMDDT

SEQ ID NO: 6935 - protein, 21 aa, Homo sapiens
MMTPMNKFKVKNDPKMIKTTK

SEQ ID NO: 6936 - protein, 28 aa, Homo sapiens
MMTSLRATSSYLRSASSAMCLASFSWIS

SEQ ID NO: 6937 - protein, 17 aa, Homo sapiens [sequence omitted]

SEQ ID NO: 6938 - protein, 16 aa, Homo sapiens
MMWKIHFSARRSGSHL

SEQ ID NO: 6939 - protein, 21 aa, Homo sapiens
MMWLKGERKRPTYRPVATFHH

SEQ ID NO: 6940 - protein, 18 aa, Homo sapiens
MNCFPDWVELSICFPISH

SEQ ID NO: 6941 - protein, 27 aa, Homo sapiens
MNDLTKLKATGNSFGARITIKFFRVSG

SEQ ID NO: 6942 - protein, 53 aa, Homo sapiens
MNERSRCKSPHREKPKGPGYGYWSPSEDAVVGLYEMMNRVALDALMMPTCSFC

SEQ ID NO: 6943 - protein, 52 aa, Homo sapiens
MNFCTVIIYPFNMYKVFLGMGVYSLTVPCFIQASTCKFVYIMAFNDPPFSFL

SEQ ID NO: 6944 - protein, 46 aa, Homo sapiens
MNFLIIRTAHFLLWIAFRARAPRQWASSLMAACLFFTYSLLPRQRL

SEQ ID NO: 6945 - protein, 25 aa, Homo sapiens
MNFLVTSNILILRQKATQSLKRANN

SEQ ID NO: 6946 - protein, 20 aa, Homo sapiens
MNFPWEELKIWVLQSEVGHR

SEQ ID NO: 6947 - protein, 17 aa, Homo sapiens
MNFYVHLLTTSQTQKQH

SEQ ID NO: 6948 - protein, 56 aa, Homo sapiens
MNGRCTIEERERSVCLHIFLQIAEAVEFLHSKGLMHRDLKVCICGASPLGFQSDVL

SEQ ID NO: 6949 - protein, 55 aa, Homo sapiens
MNGSEPSSGSGKDTKTQQGWGPCGRGARSASPQKPPANLEPHHGWGPHRQARAAV

SEQ ID NO: 6950 - protein, 16 aa, Homo sapiens
MNGVLYNELNKFLKFH

SEQ ID NO: 6951 - protein, 47 aa, Homo sapiens
MNHFDIHFSFVQFFKTLPVLLKVSASKFCFLQLLKSGVHLKKNSHKV

SEQ ID NO: 6952 - protein, 26 aa, Homo sapiens
MNHQSATHSTPGIVSATSSIRQSRMK

SEQ ID NO: 6953 - protein, 31 aa, Homo sapiens
MNHRAKPVSFWHLPLSLLLLFCAVSDEFCGC

SEQ ID NO: 6954 - protein, 18 aa, Homo sapiens
MNHRAKPVSILPRLVSIS

SEQ ID NO: 6955 - protein, 11 aa, Homo sapiens
MNHRAKPVSVQ

SEQ ID NO: 6956 - protein, 11 aa, Homo sapiens
MNHYASSFLYF

SEQ ID NO: 6957 - protein, 14 aa, Homo sapiens
MNIFLYRHHACLHC

SEQ ID NO: 6958 - protein, 22 aa, Homo sapiens
MNIGPRIRAPLPDAVNQPMYTP

SEQ ID NO: 6959 - protein, 25 aa, Homo sapiens
MNIGPRIRAPLPDAVNQPMYTPCWG

SEQ ID NO: 6960 - protein, 25 aa, Homo sapiens
MNIGPRIRAPLPDAVNQPMYTPWLT

SEQ ID NO: 6961 - protein, 12 aa, Homo sapiens
MNIIKKTDNNNC

SEQ ID NO: 6962 - protein, 12 aa, Homo sapiens
MNILWSTMKINA

SEQ ID NO: 6963 - protein, 29 aa, Homo sapiens
MNIRLFHIVPQIPKGLLIFFTFFSVIQTR

SEQ ID NO: 6964 - protein, 17 aa, Homo sapiens
MNKFKVKNDPKMIKTTK

SEQ ID NO: 6965 - protein, 48 aa, Homo sapiens
MNKGMILDKRINVGIEHIKHSGSQDSFLKHVKENDQKKKPKRRVPGLN

SEQ ID NO: 6966 - protein, 16 aa, Homo sapiens
MNLEFKLSELRRKKVS

SEQ ID NO: 6967 - protein, 64 aa, Homo sapiens
MNLLVLSEVRAMSKALPTLLTFIEHPSRAKCLFTKRQRVNYRGLIAPMLNVFLFSTSLLVFTDI

SEQ ID NO: 6968 - protein, 78 aa, Homo sapiens
MNMRLSATPLQIDVGRQRYTEPSRAVPMSWSSRARICAWADMVAGGGDGVGRDDFSQAGGGSGVDKRWSRRPRAHSAL

SEQ ID NO: 6969 - protein, 18 aa, Homo sapiens
MNNKIRAAVLVKEIEIDF

SEQ ID NO: 6970 - protein, 20 aa, Homo sapiens
MNNLDSNISKSCNIHKSIIS

SEQ ID NO: 6971 - protein, 50 aa, Homo sapiens
MNPLMNFLIIRTAHFLLWIAFRARAPRQWASSLMAACLFFTYSLLPRQRL

SEQ ID NO: 6972 - protein, 60 aa, Homo sapiens
MNRICILKEHIAKPFADACHFVSHNPHGHDTSTVQKVLLNGRFFNFIREIPHKNRSLVSR

SEQ ID NO: 6973 - protein, 59 aa, Homo sapiens
MNRICILKEHIAKPFADACHFVSHNPHGHDTSTVQKVLLNGRFFNIREIPHKNRSLVSR

SEQ ID NO: 6974 - protein, 14 aa, Homo sapiens
MNRKKLEALATCLV

SEQ ID NO: 6975 - protein, 17 aa, Homo sapiens
MNRLQGTMNPAIIENMV

SEQ ID NO: 6976 - protein, 40 aa, Homo sapiens
MNRQPTEWEKIFAIYLSDKGNLNKFTRKKQTTLSKSGQMT

SEQ ID NO: 6977 - protein, 25 aa, Homo sapiens
MNRQRKGSLMEVHTISDHKPSGLSA

SEQ ID NO: 6978 - protein, 22 aa, Homo sapiens
MNSDHLHTDDILDRTAVSKCFH

SEQ ID NO: 6979 - protein, 37 aa, Homo sapiens
MNSDHLHTDDILDRTAVSKCFWDSGRLCLGFSARAAH

SEQ ID NO: 6980 - protein, 28 aa, Homo sapiens
MNSILNMFMNNLDSNISKSCNIHKSIIS

SEQ ID NO: 6981 - protein, 28 aa, Homo sapiens
MNSKMSFVKRFGNQSTHCVLFLFTNKNL

SEQ ID NO: 6982 - protein, 49 aa, Homo sapiens
MNSPIFALEFIHSVTAHEHRNQRTCREPPFIGLGMPNQMAFKVSRLRSS

SEQ ID NO: 6983 - protein, 35 aa, Homo sapiens
MNSPIFALEFIHSVTAHEHRNQRTCREPPFIGSHN

SEQ ID NO: 6984 - protein, 26 aa, Homo sapiens
MNSWWDGGHWIMMSEFLSCFWHQIVG

SEQ ID NO: 6985 - protein, 53 aa, Homo sapiens
MNTCCSSPSICASHFHHVIYRHFFCSVNNVIFIIIIFNITLIQNHFNYFTIGQ

SEQ ID NO: 6986 - protein, 50 aa, Homo sapiens
MNTFKGCFSPVLGQSSTVCLLLMASGEQDRGLAPDHMVQKFSSTSRNSST

SEQ ID NO: 6987 - protein, 39 aa, Homo sapiens
MNTKNLHLQSYLSLQMTAKKSSWLLSQNQQQSKNLPIFR

SEQ ID NO: 6988 - protein, 18 aa, Homo sapiens
MNTRIQKLVDWFGKNFTT

SEQ ID NO: 6989 - protein, 38 aa, Homo sapiens
MNTSNKPSGLDPKTTVAVLQQKRLRWPWDLSRKYSSSI

SEQ ID NO: 6990 - protein, 26 aa, Homo sapiens
MNVCTYIKYGCKGVGDLQIKHIIHKI

SEQ ID NO: 6991 - protein, 13 aa, Homo sapiens
MNVGLFDDVPQIH

SEQ ID NO: 6992 - protein, 12 aa, Homo sapiens
MNVHSSFIRAKN

SEQ ID NO: 6993 - protein, 26 aa, Homo sapiens
MNVKNISSFSFPSTQNQKSSVQLSKK

SEQ ID NO: 6994 - protein, 11 aa, Homo sapiens
MNYHVNNWNVN

SEQ ID NO: 6995 - protein, 16 aa, Homo sapiens
MPAHFCIFNRDSVSLC

SEQ ID NO: 6996 - protein, 74 aa, Homo sapiens
MPALPLQPHHTPVSWGRRTSTCCLLKGSQVGWHNDQPDHAGRSWGGTSLYSCWGLWLFTESKLFRVSGNYVQEL

SEQ ID NO: 6997 - protein, 21 aa, Homo sapiens
MPANFCIFNRDRVSPYWPDWS

SEQ ID NO: 6998 - protein, 17 aa, Homo sapiens
MPARAPGPRGASPAPPG

SEQ ID NO: 6999 - protein, 11 aa, Homo sapiens
MPARFILQNKA

SEQ ID NO: 7000 - protein, 109 aa, Homo sapiens
MPCSLMVLIPSGPSRDTACFTRSVRPQFSIRKPRSCLNLASMATASSFRDAQKQSSALSWRGSQSTPGSSSRAAWRTSSLSMEKLRRWPACATATRIHSISGGSTRKGL

SEQ ID NO: 7001 - protein, 133 aa, Homo sapiens
MPCSLMVLIPSGPSRDTACFTRSVRPQFSIRKPRSCLNLASMATASSFRDAQKQSSALSWRGSQSTPGSSSRAAWRTSSLSMEKLRRWPACATATRIHSISGGSTRKGLSTWRLTLEGSTLGFSHSICGQCMK

SEQ ID NO: 7002 - protein, 18 aa, Homo sapiens
MPFLSFSLISSIVLKSSA

SEQ ID NO: 7003 - protein, 20 aa, Homo sapiens
MPFWPPPISSMLIVLPVFLA

SEQ ID NO: 7004 - protein, 22 aa, Homo sapiens
MPGLCFNSSMLLNIRHALEILP

SEQ ID NO: 7005 - protein, 20 aa, Homo sapiens
MPGLIASFLGGNYFGFKCKD

SEQ ID NO: 7006 - protein, 14 aa, Homo sapiens
MPGNRPSAASQPPA

SEQ ID NO: 7007 - protein, 52 aa, Homo sapiens
MPGQFWGFFVFLVETGFCHFDQANLEPLTSGDPPALASQSAGITGMSHHTQQ

SEQ ID NO: 7008 - protein, 25 aa, Homo sapiens
MPGRSRKLHGKRSARTHEPALWRPL

SEQ ID NO: 7009 - protein, 41 aa, Homo sapiens
MPGRTSGFLFNSTGLPHHPTSLCKPLLYCDLDPLGQAGAYV

SEQ ID NO: 7010 - protein, 11 aa, Homo sapiens
MPGTQLSINGF

SEQ ID NO: 7011 - protein, 31 aa, Homo sapiens
MPGYFFFFFFVFLLETGFHRVSQDGLDLLTS

SEQ ID NO: 7012 - protein, 12 aa, Homo sapiens
MPHGQKRSRINW

SEQ ID NO: 7013 - protein, 31 aa, Homo sapiens
MPHHGPANFCNFSRNGVSLRWPGWSQTPDLR

SEQ ID NO: 7014 - protein, 21 aa, Homo sapiens
MPHILRAEQTHVTSGYHTELR

SEQ ID NO: 7015 - protein, 54 aa, Homo sapiens
MPITRHSSLTGWPSGTPQFCSFSRITGAFFTSLATTESSRLKEFCPVLLVAMHL

SEQ ID NO: 7016 - protein, 22 aa, Homo sapiens
MPIVTHPSFNKYLLSVCYIPSS

SEQ ID NO: 7017 - protein, 12 aa, Homo sapiens
MPIVVPSEHTLG

SEQ ID NO: 7018 - protein, 15 aa, Homo sapiens
MPIYLTLTSVSFIPL

SEQ ID NO: 7019 - protein, 48 aa, Homo sapiens
MPKAIATKAKIDKWDLIKLKSFCTALRTYQQSKPTTYRMGENFCTLSI

SEQ ID NO: 7020 - protein, 36 aa, Homo sapiens [sequence omitted]

SEQ ID NO: 7021 - protein, 26 aa, Homo sapiens
MPKKGESRSLPWGRSQFSWGRQDRRS

SEQ ID NO: 7022 - protein, 14 aa, Homo sapiens
MPKSFMCSLQIALL

SEQ ID NO: 7023 - protein, 29 aa, Homo sapiens
MPLCPANFCIFSRDGVSPCWPGWSRTRDL

SEQ ID NO: 7024 - protein, 17 aa, Homo sapiens
MPLFLEGDGLKFFISIS

SEQ ID NO: 7025 - protein, 11 aa, Homo sapiens
MPLISWNSEMT

SEQ ID NO: 7026 - protein, 37 aa, Homo sapiens
MPLLLEESWQEGDIIWLLSPLTCHNALCGQDQGRRVK

SEQ ID NO: 7027 - protein, 42 aa, Homo sapiens
MPLRPAKFLYFSRDGVSPCCPGWSRTPEVRQSARLGLPKCWD

SEQ ID NO: 7028 - protein, 49 aa, Homo sapiens
MPLTHCLILLIFHPPAFLTKPQVSLSRAVLHCFLLQNLVLVYEQGRNRY

SEQ ID NO: 7029 - protein, 80 aa, Homo sapiens [sequence omitted]

SEQ ID NO: 7030 - protein, 41 aa, Homo sapiens
MPNFCSFSRDGGFAMRARLVSNSQPWVICPPRPPKVLGSQA

SEQ ID NO: 7031 - protein, 74 aa, Homo sapiens [sequence omitted]

SEQ ID NO: 7032 - protein, 57 aa, Homo sapiens
MPNRKVKLTTLRRFLNTSSLRVRLLLLPFLPQICTITTMNMAMFRKNMTPKYPAQVT

SEQ ID NO: 7033 - protein, 46 aa, Homo sapiens
MPPAQVCQAGTWEMQCWRQQWTLKYLWPEKLQEASLVSNIQHSFLL

SEQ ID NO: 7034 - protein, 31 aa, Homo sapiens
MPPCLANFFCIFSRDRVSSCWPGRSQTPDLK

SEQ ID NO: 7035 - protein, 74 aa, Homo sapiens [sequence omitted]

SEQ ID NO: 7036 - protein, 26 aa, Homo sapiens
MPPCPANFLFYYYYYFRDGVSLCCPG

SEQ ID NO: 7037 - protein, 11 aa, Homo sapiens
MPPCQANFLYF

SEQ ID NO: 7038 - protein, 75 aa, Homo sapiens
MPPGPANFCIFLVQMGFYHVGQDGLKLLTSNDPPALASQIAGITGVSHRTRPYYSIFNLFIHVKKHSLTAAQYDN

SEQ ID NO: 7039 - protein, 19 aa, Homo sapiens
MPPHLANFCIFSGDGVSPC

SEQ ID NO: 7040 - protein, 34 aa, Homo sapiens
MPPHLANFCSFSRMGFHHVGQVGQLTGQQTPDLR

SEQ ID NO: 7041 - protein, 24 aa, Homo sapiens
MPPHPANFCIFSRDGVSPCWSGWS

SEQ ID NO: 7042 - protein, 22 aa, Homo sapiens
MPPHPANFCIISRDGVSSCWPG

SEQ ID NO: 7043 - protein, 30 aa, Homo sapiens
MPPHPANFCVFSRDRVSPYWSGWSRTPDLR

SEQ ID NO: 7044 - protein, 11 aa, Homo sapiens
MPPHPDNFLYF

SEQ ID NO: 7045 - protein, 16 aa, Homo sapiens
MPPLFHNLLMLLLPSY

SEQ ID NO: 7046 - protein, 26 aa, Homo sapiens
MPPLTFPIILLYFTPLDLSLSNMLHN

SEQ ID NO: 7047 - protein, 15 aa, Homo sapiens
MPPQRGYHTVTQMGA

SEQ ID NO: 7048 - protein, 38 aa, Homo sapiens
MPPQSANFCSLLVETGFHQAGLKLLTSGDPSASARISL

SEQ ID NO: 7049 - protein, 43 aa, Homo sapiens
MPPRLANFVFLVKARFLHIGQAGLPFLIYSSIFSSKAIIYIYI

SEQ ID NO: 7050 - protein, 30 aa, Homo sapiens
MPPRPANFCIFSRDGVSPYWSGWSRIPDLR

SEQ ID NO: 7051 - protein, 120 aa, Homo sapiens
MPPRPANFCILVEMGFHHVGQAGLELLTSGDPPISASQNVGITGVSHCAQLEGLLLLLLLLLLFIIIIFEMESCSVTQAGVQWCGLSSLPAPPPWFMPFSCLSLPSSWDPPPHPANFLYF

SEQ ID NO: 7052 - protein, 44 aa, Homo sapiens [sequence omitted]

SEQ ID NO: 7053 - protein, 30 aa, Homo sapiens
MPPRPANFYIFSRDGLSPCWPGWSRTPDLK

SEQ ID NO: 7054 - protein, 14 aa, Homo sapiens
MPPRPATFPLFYFL

SEQ ID NO: 7055 - protein, 30 aa, Homo sapiens
MPPRPDNFCVFSGDGVSPCWTGWSRTSDLR

SEQ ID NO: 7056 - protein, 56 aa, Homo sapiens
MPPSPANLYIFSRDGVSPCWPGWSQTSDVRSPDLPKCWNYRCEPPCPAYKHFFFIK

SEQ ID NO: 7057 - protein, 51 aa, Homo sapiens
MPPVSLLKHNNNTYLCSSSQQLPHLHLRPLQPRPYCPYCCQACGQSHSTSL

SEQ ID NO: 7058 - protein, 30 aa, Homo sapiens
MPPWLANFCIFSRDGVSPCWPGWSRTPDLK

SEQ ID NO: 7059 - protein, 40 aa, Homo sapiens
MPPYFQSHHWTQSFHQWIFSETSDNEQTQQEGIPSRRTGR

SEQ ID NO: 7060 - protein, 79 aa, Homo sapiens
MPQHPGSGHGGRKAGLVLPQSPIAHTLPWTGVLRRGLVGDAGQGRLQLGTVLHLLPEHGDLGHRFWSLLLLLLTLAAVD

SEQ ID NO: 7061 - protein, 17 aa, Homo sapiens
MPQKAKPGMEALQKNTA

SEQ ID NO: 7062 - protein, 15 aa, Homo sapiens
MPQSRPTALHSKYHY

SEQ ID NO: 7063 - protein, 67 aa, Homo sapiens
MPQVPKCCWLLEVGHTGLVSALSPPGSGRWPPPSGGLHPPPGSAWPPPSRRGFPVLPACQSARLTYC

SEQ ID NO: 7064 - protein, 196 aa, Homo sapiens
MPQVPKCCWLLEVGHTGLVSALSPPGSGRWPPPSGGLHPPPGSAWPPPSRRGFPVLPACQSARLTYCLRTQGRAGQDRTGQGRAGQDRAGQDRTGQGPLYPRGAAQPQAGTAAPPAGQRLAALVCRGPGLRPELLPGKSSAASRPIPPGTQMGTAGSGMAVQGWMRQSRTTPKRIRQITLPLSWKPPARPGSPAPV

SEQ ID NO: 7065 - protein, 89 aa, Homo sapiens
MPQVPKCCWLLEVGHTGLVSALSPPGSGRWPPPSGGLHPPPGSAWPPPSRRGFPVLPACQSARLTYCSWPGSPPMHQAAPSGSGSCGSR

SEQ ID NO: 7066 - protein, 12 aa, Homo sapiens
MPRKDQEQPRNS

SEQ ID NO: 7067 - protein, 97 aa, Homo sapiens
MPRSIMSSSPLEATITANISMDGSSRGGPPSPARALPRGARLSARPRGSAPFGAASGVSGRGNMVLKGWGPARARPIRGRPGRRARAGGGRRVWDRG

SEQ ID NO: 7068 - protein, 14 aa, Homo sapiens
MPSAWKDTLLLLLG

SEQ ID NO: 7069 - protein, 13 aa, Homo sapiens
MPSLTLKGIVTTP

SEQ ID NO: 7070 - protein, 63 aa, Homo sapiens
MPSQFFVFLVETGFHHVGQAGLKLRTSGDTPTSAAQSVGITGVSHRSRPCNLTYRPPKISDSL

SEQ ID NO: 7071 - protein, 18 aa, Homo sapiens
MPSSASLSAGITGLSHCT

SEQ ID NO: 7072 - protein, 27 aa, Homo sapiens
MPSVGRTKAGESNDLGAGSSSMSQITL

SEQ ID NO: 7073 - protein, 39 aa, Homo sapiens
MPSVGRTKAGESNDLGAGSSSMSQITLDAWPTDLSQSLL

SEQ ID NO: 7074 - protein, 21 aa, Homo sapiens
MPSYFCIFSRDRVSPCWPGWS

SEQ ID NO: 7075 - protein, 42 aa, Homo sapiens
MPSYFFFCIFSRDGVSPCWPGWSRSPDLVICSPRLPKVLRLL

SEQ ID NO: 7076 - protein, 74 aa, Homo sapiens
MPTDDAPCQSATAANPQFRHGTLWPGARHHPAAASFVLFFPKHFASVDLKPLACSEGCLLLLLHLIQLDHFLLY

SEQ ID NO: 7077 - protein, 77 aa, Homo sapiens [sequence omitted]

SEQ ID NO: 7078 - protein, 22 aa, Homo sapiens
MPTLPANFCIFSRDGVSPHWPG

SEQ ID NO: 7079 - protein, 21 aa, Homo sapiens
MPTRKTLLQRTSSGRVKSKKQ

SEQ ID NO: 7080 - protein, 11 aa, Homo sapiens
MPTSHVILLKT

SEQ ID NO: 7081 - protein, 115 aa, Homo sapiens
MPTTITPITTPKTISHMETGGWLGGPSVGCIPRNSRLLSFRRKASLIRLRDILMAFSTSVLGMISDTFLGAVTKKLKEILGFKLATRTSSSNSFCPASVEFEMSHLCRGPSCLAA

SEQ ID NO: 7082 - protein, 96 aa, Homo sapiens
MPTTITPITTPKTISHMETGGWLGGPSVGCIPRNSRLLSFRRKASLIRLRDILMAFSTSVLGMISDTFLGAVTKKLKEILGFKLATRTSSSPKRII

SEQ ID NO: 7083 - protein, 16 aa, Homo sapiens
MPTVERSQNKEDCQII

SEQ ID NO: 7084 - protein, 33 aa, Homo sapiens
MPVILALWEAEAGGSRGQEIKTILANTVKPRLY

SEQ ID NO: 7085 - protein, 21 aa, Homo sapiens
MPVLLLLESNEVIYSKYLTII

SEQ ID NO: 7086 - protein, 51 aa, Homo sapiens
MPVLNYFFIRNHMMIQRFERPYTVNKNMSISFFKAYWTIKHSEGNEGWTGR

SEQ ID NO: 7087 - protein, 119 aa, Homo sapiens [sequence omitted]

SEQ ID NO: 7088 - protein, 15 aa, Homo sapiens
MPVMLVEQGWFISLS

SEQ ID NO: 7089 - protein, 13 aa, Homo sapiens
MPVMPALWEAEEG

SEQ ID NO: 7090 - protein, 40 aa, Homo sapiens
MPVRMAIIKKWHGGHRCWKGQGEIGILLHCWWECKLVQPL

SEQ ID NO: 7091 - protein, 22 aa, Homo sapiens
MPVSNFYIFSRDGVSPCWPGWS

SEQ ID NO: 7092 - protein, 44 aa, Homo sapiens
MPVTMVIIKKSKNDRCWQGCREIGTLLHCWWESKLVQTLWKTVW

SEQ ID NO: 7093 - protein, 24 aa, Homo sapiens
MPWLLILGSHVKCDLLPQRTLQFE

SEQ ID NO: 7094 - protein, 93 aa, Homo sapiens
MPYSNLSSPKALTSGGASRVQPGDPRAGGSSILQMEAMFRTVISLKVAAIPHRHLYKGKPGLPMVARWRGGRAAARRPGVRLSVWLGEGGREE

SEQ ID NO: 7095 - protein, 49 aa, Homo sapiens
MQAAEGGPEVLVLLSIEAGDLEVLPRVHSFSQPLGAQLQGGSWPSDPRG

SEQ ID NO: 7096 - protein, 29 aa, Homo sapiens
MQAKQAAFVWSSSEAFLSRSCILAQEQSL

SEQ ID NO: 7097 - protein, 22 aa, Homo sapiens
MQASFSVPVMLPNVKISLKTGK

SEQ ID NO: 7098 - protein, 18 aa, Homo sapiens
MQCFLNFLAHMLLCSCTT

SEQ ID NO: 7099 - protein, 35 aa, Homo sapiens
MQCIQLFLLIKSFFLFQSKEPHQVLSPSTGNIQQK

SEQ ID NO: 7100 - protein, 33 aa, Homo sapiens
MQCWRQQWTLKYLWPEKLQEASLVSNIQHSFLL

SEQ ID NO: 7101 - protein, 13 aa, Homo sapiens
MQDRSYSEECTGP

SEQ ID NO: 7102 - protein, 22 aa, Homo sapiens
MQHCHKRQRQKCKRNKGYIAFI

SEQ ID NO: 7103 - protein, 29 aa, Homo sapiens
MQHIWYLFIQFFIPCFLFSVTICGTPSMC

SEQ ID NO: 7104 - protein, 19 aa, Homo sapiens
MQHPIKMEFLLPSFPNPIS

SEQ ID NO: 7105 - protein, 67 aa, Homo sapiens
MQIFLLLYALGRFVLLVTFSPLVLSLSYPVLVSFYLRYPSVLFVFLHNVVSLVFGYPLQNQQGLIHP

SEQ ID NO: 7106 - protein, 15 aa, Homo sapiens
MQIIFKMHSIYISFE

SEQ ID NO: 7107 - protein, 12 aa, Homo sapiens
MQINFQPRSLHS

SEQ ID NO: 7108 - protein, 21 aa, Homo sapiens
MQIPCLVYALTPLCFSILDML

SEQ ID NO: 7109 - protein, 56 aa, Homo sapiens
MQKTSSLIFLFRSLASRSRSGAWLDSSSHVQEDSAGTLPPSCLPSSANQTLPGRSI

SEQ ID NO: 7110 - protein, 23 aa, Homo sapiens
MQKYKPKGHVYQMQNHRSPTRLV

SEQ ID NO: 7111 - protein, 68 aa, Homo sapiens
MQLCRKENLKDWMNGRCTIEERERSVCLHIFLQIAEAVEFLHSKGLMHRDLKVCICGASPLGFQSDVL

SEQ ID NO: 7112 - protein, 22 aa, Homo sapiens
MQLGSIELSGIQADGGSSAFDK

SEQ ID NO: 7113 - protein, 17 aa, Homo sapiens
MQLHESVDLSNGTCEEM

SEQ ID NO: 7114 - protein, 24 aa, Homo sapiens
MQLKDPGLGCSFAVGTAGNGKSGH

SEQ ID NO: 7115 - protein, 25 aa, Homo sapiens
MQLLSPIMPYKDICHIVSRCSQIFV

SEQ ID NO: 7116 - protein, 25 aa, Homo sapiens
MQLQGILKGSCTGGPHVPWQAAGIS

SEQ ID NO: 7117 - protein, 70 aa, Homo sapiens
MQLQGILKGSHVKQILFGAVLRLGGVQTLGVDIQVLLVVRGAPGVRLHVAVPRWSCTGGPHVPWQAAGIS

SEQ ID NO: 7118 - protein, 28 aa, Homo sapiens
MQNDRSSKAAKYSKRNVNGESRKVVSPT

SEQ ID NO: 7119 - protein, 32 aa, Homo sapiens
MQNDRSSKAAKYSKRNVNGESRKVVSPTSPIK

SEQ ID NO: 7120 - protein, 11 aa, Homo sapiens
MQNHRSPTRLV

SEQ ID NO: 7121 - protein, 28 aa, Homo sapiens
MQNLQLKPILQCIKNTDFSSKPTIYHVK

SEQ ID NO: 7122 - protein, 13 aa, Homo sapiens
MQNPMSCPTERSS

SEQ ID NO: 7123 - protein, 50 aa, Homo sapiens
MQPASVIYHDIEQNRNILAEHARPLSPPLIDTYRVSLENQSQSWWHMLHW

SEQ ID NO: 7124 - protein, 23 aa, Homo sapiens
MQPSPEKVCNLSYPRSQQALLYC

SEQ ID NO: 7125 - protein, 35 aa, Homo sapiens
MQPVQLHKTVLRSTPHLIFERGPYSFILPLVPQIM

SEQ ID NO: 7126 - protein, 18 aa, Homo sapiens
MQPYFAGSDILDLHAQSF

SEQ ID NO: 7127 - protein, 16 aa, Homo sapiens
MQRHRFVVYKVISKTH

SEQ ID NO: 7128 - protein, 18 aa, Homo sapiens
MQSCCPPKASFVGQKMSL

SEQ ID NO: 7129 - protein, 36 aa, Homo sapiens
MQSLLNSRLNLLRYISHIFFLNIESLDFSRLHLTSG

SEQ ID NO: 7130 - protein, 12 aa, Homo sapiens
MQSSRNSHSLLV

SEQ ID NO: 7131 - protein, 70 aa, Homo sapiens
MQVCSIGIHVPWWFAAPMDPSFKFPSLNPQPPTGLHVCCSLLCVHVFSVFNFHLWVRTCGVWFSVPVLVC

SEQ ID NO: 7132 - protein, 13 aa, Homo sapiens
MQVFHPVNTGTYN

SEQ ID NO: 7133 - protein, 35 aa, Homo sapiens
MQVGDYFWRLEVEPSYGWNKPPCYMPLISWNSEMT

SEQ ID NO: 7134 - protein, 16 aa, Homo sapiens
MQVISKTLQAETQKTI

SEQ ID NO: 7135 - protein, 120 aa, Homo sapiens
MQVPTAARKEEVFHGEIASWGQVHRISRLLSTDPSSWAPHFQVYGHRGFRYLDHWPWGCGGARVARMIGEAGPLARLGRMAAGGGGGWSAAWRGVLGVGGEVFGDATITAFGGPEWGAGQ

SEQ ID NO: 7136 - protein, 96 aa, Homo sapiens
MQWLFTFSCCSVNIGKSLLLVLVSRPFSSLPPTTKEVAPNFMSSDLNTISHCCSHTYIKVKLPLSNDFSSSLLFQSQSWFEPWLFFICPELKSQTS

SEQ ID NO: 7137 - protein, 104 aa, Homo sapiens
MQYCQRALIHPPTLSDRHHVDTPMHLMGKALGCGRKLQDLEKTHTDMGKTCQLHTVSLAQELNFFSHQCYNKMTLNKILFQDPLYLVDVVRIRIFPRWRQREVQ

SEQ ID NO: 7138 - protein, 19 aa, Homo sapiens
MQYIHGSPSWEQRLRLFGS

SEQ ID NO: 7139 - protein, 55 aa, Homo sapiens
MRAQVGPTLTTGPGQGRTPATSSAETLARGSLLAQTPSTSRRVCRATPHPRDDHV

SEQ ID NO: 7140 - protein, 27 aa, Homo sapiens
MRARLVSNSQPWVICPPRPPKVLGSQA

SEQ ID NO: 7141 - protein, 70 aa, Homo sapiens
MRCHHISRAIIGPKASINGFSLKPQIMNKPNKKASQVEGQEDEDTEKTGFHINRFFNGRDNGHFKVLFSL

SEQ ID NO: 7142 - protein, 40 aa, Homo sapiens
MRDDQNFTTTKYGLLAFQITLGSYFVSPHIISAQGQSYSV

SEQ ID NO: 7143 - protein, 15 aa, Homo sapiens
MRFHHVDLSRAPDLR

SEQ ID NO: 7144 - protein, 116 aa, Homo sapiens
MRFHHVGQAGLELLISGDPPALTSQSTGITGVSHCAWPASFGGSFLPPFCWEGEFVRGLSLAAGALLAIFGVPWLIAASARSLPSSSCVSVFKFLLFIRTRVVSDWGPPSSTVTSS

SEQ ID NO: 7145 - protein, 42 aa, Homo sapiens
MRFHHVGQAGLELLTSGDPPTLASQSAGITGMSHCAWLHCVL

SEQ ID NO: 7146 - protein, 24 aa, Homo sapiens
MRFHHVVQAGLKLLTSSDPPTSAS

SEQ ID NO: 7147 - protein, 16 aa, Homo sapiens
MRFHRVSQDDLSPLTS

SEQ ID NO: 7148 - protein, 41 aa, Homo sapiens
MRFRHVGQAGLELLTSGDLPASASQSAEITGVSHHAWPEIS

SEQ ID NO: 7149 - protein, 17 aa, Homo sapiens
MRGLQLKGQEHKTTRAF

SEQ ID NO: 7150 - protein, 24 aa, Homo sapiens
MRGPRRPSLLATVCGLGKCGWAPE

SEQ ID NO: 7151 - protein, 26 aa, Homo sapiens
MRGREERREGEEFNREREGGMMREQR

SEQ ID NO: 7152 - protein, 20 aa, Homo sapiens
MRGYTEPEARRDLGDLGRAG

SEQ ID NO: 7153 - protein, 15 aa, Homo sapiens
MRHCVQLMVLIKVGI

SEQ ID NO: 7154 - protein, 77 aa, Homo sapiens
MRHDAQLIFVFLVDGVSPRWPGWSGTPDLSLSAHLSLPKCWDYKHEPPGPASLFSFSVFPGSSLNIQGLHRWTSHKR

SEQ ID NO: 7155 - protein, 11 aa, Homo sapiens
MRHHAGLILYF

SEQ ID NO: 7156 - protein, 91 aa, Homo sapiens [sequence omitted]

SEQ ID NO: 7157 - protein, 30 aa, Homo sapiens
MRHHAQLIFVFLVETRFHRVGQDGLDLLTS

SEQ ID NO: 7158 - protein, 11 aa, Homo sapiens
MRHHAQLILYF

SEQ ID NO: 7159 - protein, 31 aa, Homo sapiens
MRHHARLIFCVFSRDEVSPCWSGWSRTPDIR

SEQ ID NO: 7160 - protein, 18 aa, Homo sapiens
MRHHARLIFVLARLVLNS

SEQ ID NO: 7161 - protein, 25 aa, Homo sapiens
MRHHARLIIIFFSRDRVSLCWPGWF

SEQ ID NO: 7162 - protein, 35 aa, Homo sapiens
MRHHARLILVFLVETGFHQAGLKLLTSGDPPTSAS

SEQ ID NO: 7163 - protein, 40 aa, Homo sapiens
MRHHTQLFFFFLRRCLTFVPQAGVRWHDLSSLQPPCPRFK

SEQ ID NO: 7164 - protein, 29 aa, Homo sapiens
MRHHTQLIFVLLVETGFHHVGQDGLNLLT

SEQ ID NO: 7165 - protein, 11 aa, Homo sapiens
MRHHTQLILHF

SEQ ID NO: 7166 - protein, 11 aa, Homo sapiens
MRHHTQLILYF

SEQ ID NO: 7167 - protein, 12 aa, Homo sapiens
MRHHTQLILYLW

SEQ ID NO: 7168 - protein, 11 aa, Homo sapiens
MRHHTRLILYF

SEQ ID NO: 7169 - protein, 30 aa, Homo sapiens
MRHHTWLFCIFSRDGVSPCWSGWSPTPDLR

SEQ ID NO: 7170 - protein, 30 aa, Homo sapiens
MRHHTWLFCIFSRDGVSPCWSGWSRTPDLR

SEQ ID NO: 7171 - protein, 75 aa, Homo sapiens [sequence omitted]

SEQ ID NO: 7172 - protein, 42 aa, Homo sapiens
MRHQARLIILVEMGGVSPCWPGWFRTPDLIIYLPWPPKVLGL

SEQ ID NO: 7173 - protein, 25 aa, Homo sapiens
MRKKNTDDFAKLPIAGCDLFYSPSL

SEQ ID NO: 7174 - protein, 18 aa, Homo sapiens
MRKLRFREGVPYSIFNTW

SEQ ID NO: 7175 - protein, 22 aa, Homo sapiens
MRLFSSPTVTCLARSTAWSTCC

SEQ ID NO: 7176 - protein, 16 aa, Homo sapiens
MRLIRDASWKRRIWGK

SEQ ID NO: 7177 - protein, 18 aa, Homo sapiens
MRLKPYPSWTWFQPSRFP

SEQ ID NO: 7178 - protein, 76 aa, Homo sapiens
MRLSATPLQIDVGRQRYTEPSRAVPMSWSSRARICAWADMVAGGGDGVGRDDFSQAGGGSGVDKRWSRRPRAHSAL

SEQ ID NO: 7179 - protein, 81 aa, Homo sapiens
MRLVFWVWRSWTRSLASRSSCSAIFLLLSVCSRVAHSSSISACSRLALRSTIASCSLRSSWPRRASSRWSWVSFRIPWVFL

SEQ ID NO: 7180 - protein, 21 aa, Homo sapiens
MRMIWRPCNEYPFISLGILRI

SEQ ID NO: 7181 - protein, 41 aa, Homo sapiens
MRMNTKNLHLQSYLSLQMTAKKSSWLLSQNQQQSKNLPIFR

SEQ ID NO: 7182 - protein, 16 aa, Homo sapiens
MRMWINWNSHTLLVGM

SEQ ID NO: 7183 - protein, 16 aa, Homo sapiens
MRMWRNWNSHTLLVGM

SEQ ID NO: 7184 - protein, 35 aa, Homo sapiens
MRNHAQLIFVILVEMGFRLVEMGCLPGWSRTPDFR

SEQ ID NO: 7185 - protein, 24 aa, Homo sapiens
MRNINSIKHVFKSPYLTSLTPPTF

SEQ ID NO: 7186 - protein, 16 aa, Homo sapiens
MRNLILIYRILLLTKN

SEQ ID NO: 7187 - protein, 16 aa, Homo sapiens
MRNLKQSRLAFRLPHV

SEQ ID NO: 7188 - protein, 36 aa, Homo sapiens [sequence omitted]

SEQ ID NO: 7189 - protein, 50 aa, Homo sapiens
MRNWMHLPHTSVWKQSSYSGLFRCNDCSHRKNGSFSTFDSFSMSSHNHPH

SEQ ID NO: 7190 - protein, 23 aa, Homo sapiens
MRPGGTGDSPACFWEGLQIFLQP

SEQ ID NO: 7191 - protein, 19 aa, Homo sapiens
MRSGRARWLTPIIPALCEA

SEQ ID NO: 7192 - protein, 29 aa, Homo sapiens
MRSKQILVFKVALSTTIWLLFCFFLENQQ

SEQ ID NO: 7193 - protein, 45 aa, Homo sapiens
MRSVHADGAGSGGRCATSNLDNSFNPFLQYNLLLKLNTDFHSFHD

SEQ ID NO: 7194 - protein, 95 aa, Homo sapiens [sequence omitted]

SEQ ID NO: 7195 - protein, 41 aa, Homo sapiens
MRTPAAMCLVPESDKLVMYSGNVSTLGSLSRSSDSSDGELP

SEQ ID NO: 7196 - protein, 51 aa, Homo sapiens
MRTTTLKSCRHGLTWGLARSLVVTVILTQGYGSSFPFIFRKQLHNYHISMN

SEQ ID NO: 7197 - protein, 32 aa, Homo sapiens
MRVCGIFHILPVPQPLCSDRSRSRKVLSLVAC

SEQ ID NO: 7198 - protein, 33 aa, Homo sapiens
MRVLPFWKERIPAGRGQAVPGGPGANGTRRVGQ

SEQ ID NO: 7199 - protein, 30 aa, Homo sapiens
MRYHAQLIFAFLVKTGFHHFGQADFELLTS

SEQ ID NO: 7200 - protein, 50 aa, Homo sapiens
MRYHARLIFVFLVEVGFRHVGQAGLKPLTSGDLPTSASQSARITGMSHHA

SEQ ID NO: 7201 - protein, 76 aa, Homo sapiens
MRYHLMLVRMAIIKKSRNNRCWRGCGEIGTLLYCWWECKLVQPLWKTVWRVLKDLEMEISFDPAILLLGIYPKEYK

SEQ ID NO: 7202 - protein, 40 aa, Homo sapiens
MRYNCTSTRLAKLKTKTVNTSTDQDMEKYGLDICPLQISC

SEQ ID NO: 7203 - protein, 12 aa, Homo sapiens
MRYNFSQSFQIY

SEQ ID NO: 7204 - protein, 13 aa, Homo sapiens
MRYSPSFIWSHKP

SEQ ID NO: 7205 - protein, 24 aa, Homo sapiens
MRYVMDICATAIQHHKKVVTHHNI

SEQ ID NO: 7206 - protein, 26 aa, Homo sapiens
MSAAAMSSQQARVIGHVCSPRHSNLQ

SEQ ID NO: 7207 - protein, 68 aa, Homo sapiens
MSAGGKKRLVLTALSAVFLQTTYEYFLVQTSCLSPLLNPLFLHLLFPQRIYLIHLGVQVHKLHKVLGL

SEQ ID NO: 7208 - protein, 31 aa, Homo sapiens
MSAQAQTKLQIQENKINHADQRQTSREMKCL

SEQ ID NO: 7209 - protein, 35 aa, Homo sapiens
MSARLVLNSRPCDLLALASQSSGITGMSHYASPRN

SEQ ID NO: 7210 - protein, 48 aa, Homo sapiens
MSCDPPTAASQSAGITGVSHCTQPLGYFLLIQEKKLQSLNNVTIQFYF

SEQ ID NO: 7211 - protein, 39 aa, Homo sapiens
MSCILFESNVLNCKFNPLKWFHANTPLKFLLYKILMHNV

SEQ ID NO: 7212 - protein, 24 aa, Homo sapiens
MSCSSMKTLISNRMAHCKKIQWKH

SEQ ID NO: 7213 - protein, 66 aa, Homo sapiens
MSCWKASSKNFCRSFSFICWVCSISRTFWACSASSSALHVLFPLLERPSHPHRPFISHKQLFTFQD

SEQ ID NO: 7214 - protein, 65 aa, Homo sapiens
MSCWKASSKNFCRSFSFICWVCSISRTFWACSASSSASKTSFSGRPSTNSSGVCCSIQMFPHPCV

SEQ ID NO: 7215 - protein, 47 aa, Homo sapiens
MSCWKASSKNFCRSFSFICWVCSISRTFWACSASSSASPCPSPLRQA

SEQ ID NO: 7216 - protein, 40 aa, Homo sapiens
MSCWKASSKNFCRSFSFICWVCSISRTFWACSASSSEGSL

SEQ ID NO: 7217 - protein, 23 aa, Homo sapiens
MSEAVIPLSSLMKGIFTREKFLD

SEQ ID NO: 7218 - protein, 38 aa, Homo sapiens
MSEERSSFSLCTLACRAWVDWFLLLASSEMPMVWATFL

SEQ ID NO: 7219 - protein, 11 aa, Homo sapiens
MSEKYLCFILS

SEQ ID NO: 7220 - protein, 58 aa, Homo sapiens
MSEVLPLQRVLALLLVEQRHFPGLQPRDGLRPVLLGVEMDLPDLLGGGTRTGLLPPIA

SEQ ID NO: 7221 - protein, 22 aa, Homo sapiens
MSFFCGCVILSVYFNGFISFSC

SEQ ID NO: 7222 - protein, 17 aa, Homo sapiens
MSFGSSMKVKESVTVCT

SEQ ID NO: 7223 - protein, 39 aa, Homo sapiens
MSFLFVSFPSNRQNPQLQVCWNTLPCEVSVCPCWGVPPS

SEQ ID NO: 7224 - protein, 13 aa, Homo sapiens
MSFSVNNSNLRCQ

SEQ ID NO: 7225 - protein, 24 aa, Homo sapiens
MSFVKRFGNQSTHCVLFLFTNKNL

SEQ ID NO: 7226 - protein, 20 aa, Homo sapiens
MSGKNHNVNSCFQFFLFNYA

SEQ ID NO: 7227 - protein, 11 aa, Homo sapiens
MSGWSQTPDLR

SEQ ID NO: 7228 - protein, 18 aa, Homo sapiens
MSHCAQELTLACKNTALK

SEQ ID NO: 7229 - protein, 13 aa, Homo sapiens
MSHFCPPGWSAMA

SEQ ID NO: 7230 - protein, 20 aa, Homo sapiens
MSHFRSAKRMLQNICSEKGE

SEQ ID NO: 7231 - protein, 37 aa, Homo sapiens
MSHGTLQYTMETKMSTTISAFKRVQLIGKTRQEYIYI

SEQ ID NO: 7232 - protein, 31 aa, Homo sapiens
MSHHARLIFVFFVETGVSPSWPDLSRTLDLR

SEQ ID NO: 7233 - protein, 20 aa, Homo sapiens
MSHHTQLIFCIFSRDGVSPC

SEQ ID NO: 7234 - protein, 42 aa, Homo sapiens
MSHKFISLCSLFIFYSFCFSETVFSIFFSSSSWLPLCVQIYS

SEQ ID NO: 7235 - protein, 93 aa, Homo sapiens
MSHLSQQRIYSGENPFACKVCGKVFSHKSNLTEHEHFHTREKPFECNECGKAFSQKQYVIKHQNTHTGEKLFECNECGKSFSQKENLLTHQKI

SEQ ID NO: 7236 - protein, 35 aa, Homo sapiens
MSHNLVGALHQWQSLFQLYRMLPTFPEQRMNSVQL

SEQ ID NO: 7237 - protein, 45 aa, Homo sapiens
MSHRFISLCSLFIFYSFCFSEYFPFSSLQVHGFLCVCKYTLKSLW

SEQ ID NO: 7238 - protein, 34 aa, Homo sapiens
MSHRGDSGMNHQSATHSTPGIVSATSSIRQSRMK

SEQ ID NO: 7239 - protein, 11 aa, Homo sapiens
MSHTLCPLTQV

SEQ ID NO: 7240 - protein, 31 aa, Homo sapiens
MSILFTIAHSAKSDSPETFSCSGCLLFLAAL

SEQ ID NO: 7241 - protein, 53 aa, Homo sapiens
MSILHKLDGIYNVLLQCLAHSFQLMASSNRLLPFQQSQVLSKKVAFTNESHRS

SEQ ID NO: 7242 - protein, 18 aa, Homo sapiens
MSIRCFLRIFQITKYEFL

SEQ ID NO: 7243 - protein, 32 aa, Homo sapiens
MSIRTVRFNSFFSYTLINWTYSLTLESSFSNF

SEQ ID NO: 7244 - protein, 26 aa, Homo sapiens
MSIRTYNPTKFCVVTWYHGQHTPICP

SEQ ID NO: 7245 - protein, 86 aa, Homo sapiens
MSISPSKPSSRAWASSPGSPALSAPGASWPGPSVEVGFLGRVGVHRANSVIWVAFHFGTTVTNSSSSSSSPLSFLFKNLPWYLWFR

SEQ ID NO: 7246 - protein, 110 aa, Homo sapiens
MSISPSKPSSRAWASSPGSPALSAPGASWPGPSVEVGFLGRVGVHRANSVIWVAFHFGTTVTNSSSSSSSPLSISVKRYSPCCSHPTSNTYFPGPTGFLFKNLPWYLWFR

SEQ ID NO: 7247 - protein, 20 aa, Homo sapiens
MSIYLSQTPSPPPSIPTQRR

SEQ ID NO: 7248 - protein, 53 aa, Homo sapiens
MSKALPTLLTFIEHPSRAKCLFTKRQRVNYRGLIAPMLNVFLFSTSLLVFTDI

SEQ ID NO: 7249 - protein, 25 aa, Homo sapiens
MSKLGLGKIFPNPILDASTSVAGKS

SEQ ID NO: 7250 - protein, 24 aa, Homo sapiens
MSLCLSHQICDHNVQLTYALKDVC

SEQ ID NO: 7251 - protein, 15 aa, Homo sapiens
MSLESIVQGWEVREG

SEQ ID NO: 7252 - protein, 20 aa, Homo sapiens
MSLFMFFLMFPFCFQERAIF

SEQ ID NO: 7253 - protein, 58 aa, Homo sapiens
MSLGPNPRSLVSHKGEIQTQGQTSMEGRWPHENRGRSETSTSQGTSKTHRKLSGAREK

SEQ ID NO: 7254 - protein, 26 aa, Homo sapiens
MSLIKCHLLSEAFPITLSKVATFIPY

SEQ ID NO: 7255 - protein, 38 aa, Homo sapiens
MSLKSFLFSNVGIYSYNFHSQPCFGILCFCFHSSQIIF

SEQ ID NO: 7256 - protein, 33 aa, Homo sapiens
MSLKTPAHFLSSVSLYWSLISNKRSKSRFTGKP

SEQ ID NO: 7257 - protein, 46 aa, Homo sapiens
MSLLGHIYTELWQILNTRAFEDSLVDRSLNTCFSAFLRKISLGVAS

SEQ ID NO: 7258 - protein, 20 aa, Homo sapiens
MSLLSLGASGFCLSSFFLPL

SEQ ID NO: 7259 - protein, 82 aa, Homo sapiens
MSLLSRCDFLYSKTRGLPRCLQVCPCCASSDVLGGNSFFFLLSLLVRIGGDSCIKEARPVWWLMLVIPALCQANVGHMRSGV

SEQ ID NO: 7260 - protein, 45 aa, Homo sapiens
MSLNVHMISCTCEKYDQNVSFGSSAHLLTSCLIISSNSVLVKDTG

SEQ ID NO: 7261 - protein, 17 aa, Homo sapiens
MSLSATRTTHRSGLCLS

SEQ ID NO: 7262 - protein, 32 aa, Homo sapiens
MSLVQWRKQERVSLLITFTPLVYLNQQEKSVV

SEQ ID NO: 7263 - protein, 75 aa, Homo sapiens
MSLWLPVPRGQLCFAASSSSQTGALSPPSLVSNVHPLELKALPAGSTAPSPGPPSACAPRSVPCPRLPPVPHGLC

SEQ ID NO: 7264 - protein, 75 aa, Homo sapiens
MSMCTSRHAENLESHLPVQVPCQPEPLWSLAGLQLPCARGLSRDAATLLPSLFCQPDASRTEYLRENCLDNYSVP

SEQ ID NO: 7265 - protein, 23 aa, Homo sapiens
MSNEISMTTFTCVNFTHSKRRFF

SEQ ID NO: 7266 - protein, 53 aa, Homo sapiens
MSNTAFPWNSHILPGWENKECQAHGKTRCCCCLDELCFPAHRRQGPVEPQDPV

SEQ ID NO: 7267 - protein, 53 aa, Homo sapiens
MSPIINRVHKSTGFELSSFCAMRVCGIFHILPVPQPLCSDRSRSRKVLSLVAC

SEQ ID NO: 7268 - protein, 19 aa, Homo sapiens
MSPNRIICILMIQGFMHVY

SEQ ID NO: 7269 - protein, 22 aa, Homo sapiens
MSPQPLCSDRSRSRKVLSLVAC

SEQ ID NO: 7270 - protein, 27 aa, Homo sapiens
MSPRLVSNSWAQVVFLPQPPKVVGLQV

SEQ ID NO: 7271 - protein, 32 aa, Homo sapiens
MSPWLDWESLQCSPACCWHCCKQVRARFLPRE

SEQ ID NO: 7272 - protein, 16 aa, Homo sapiens
MSPWSSYIMARVENGS

SEQ ID NO: 7273 - protein, 48 aa, Homo sapiens
MSQCPLWAGPRQESQMIWVLGPAVCHKLPCDLDPCIRITHPTFNCLQL

SEQ ID NO: 7274 - protein, 54 aa, Homo sapiens
MSQCPLWAGPRQESQMIWVLGPAVCHKLPWMLGPLICHNPFCRQDPGKTDSNIC

SEQ ID NO: 7275 - protein, 39 aa, Homo sapiens
MSQCSLLGQVIYHNAYCGEVPEQRRLSNHIGDGARDMSQ

SEQ ID NO: 7276 - protein, 34 aa, Homo sapiens [sequence omitted]

SEQ ID NO: 7277 - protein, 11 aa, Homo sapiens
MSQNSKKTAQF

SEQ ID NO: 7278 - protein, 13 aa, Homo sapiens
MSQRVRIARRIER

SEQ ID NO: 7279 - protein, 24 aa, Homo sapiens
MSQWNAPLQQVPLAAHHTAVMRGA

SEQ ID NO: 7280 - protein, 24 aa, Homo sapiens
MSRCLKSQNVAGSWRWVILALSLH

SEQ ID NO: 7281 - protein, 54 aa, Homo sapiens
MSRFTSLSVVISVLINVASTMIIFLIYRPAFQIMAITHFRVIVFAALVLLGTAM

SEQ ID NO: 7282 - protein, 33 aa, Homo sapiens
MSRHSCFLKRLLWTISFIDCTFCFWSFTGGMQV

SEQ ID NO: 7283 - protein, 126 aa, Homo sapiens
MSRRAWFSAFGRPFFFPSVLSLAGLPGSKQRGAWPGTVCPPRTTGIPIFGGSCSIGSRTSFRLPSFPGPLLLDPGSRRPPTQKGSVISAAPSGAAAGPGRAGAGGAGRGALGPGGAGCAPRCAHAR

SEQ ID NO: 7284 - protein, 35 aa, Homo sapiens
MSRVRSKYLNNPFSILHKQHPKSFRECANFKIKSR

SEQ ID NO: 7285 - protein, 25 aa, Homo sapiens
MSRYLTSGNWLQWPPPGKATSELAC

SEQ ID NO: 7286 - protein, 124 aa, Homo sapiens
MSSALCLRPLTISKPSIFPTTNTKLPGPTNPSNPDRMNGTSPTGEPAEFTGITSNVFFVTPASPKYIMPPVLELTQISPISSVLQSWGGPSGFTMHIIPPGITCPTSWTVSAEFLSSVLTRITP

SEQ ID NO: 7287 - protein, 91 aa, Homo sapiens
MSSATRKKACSSSTHQPTVQARWRLSASCFLGSTSSRNATTTVKPRLYLPPMALYSRTCSQIRIPARSRLLAGTPKSRIRSAIGSVGRVVP

SEQ ID NO: 7288 - protein, 102 aa, Homo sapiens
MSSATRKKACSSSTHQPTVQARWRLSASCFLGSTSSRNATTTVKPRLYLPPMALYSRTCSQIRIPARSRLLAGTPKSRIRSAIGSVGRVVPALPTLRAEIYN

SEQ ID NO: 7289 - protein, 86 aa, Homo sapiens
MSSATRKKACSSSTHQPTVQARWRLSASCFLGSTSSRNATTTVKPRLYLPPMALYSRTSLSRAIASPISGCPISSSVSTLTIWEKC

SEQ ID NO: 7290 - protein, 26 aa, Homo sapiens
MSSCKQMLLSRLATLWQCSVLVPVEN

SEQ ID NO: 7291 - protein, 30 aa, Homo sapiens
MSSEEEEHSYKCIITEDRPLWAKVQSGHNW

SEQ ID NO: 7292 - protein, 11 aa, Homo sapiens
MSSELFNFRAR

SEQ ID NO: 7293 - protein, 14 aa, Homo sapiens
MSSKVGRQTEGLPT

SEQ ID NO: 7294 - protein, 49 aa, Homo sapiens
MSSLLWAQGLGFRKPSGCLHDPRIGFQLPRREFGAWSLELGAWSLEFGA

SEQ ID NO: 7295 - protein, 21 aa, Homo sapiens
MSSLNCMVSCWSMVKPPDSHL

SEQ ID NO: 7296 - protein, 52 aa, Homo sapiens
MSSLNCMVSCWSMVKPPDSNRKLWNFLYLRSIRDSCDNHGLIFLLLFMMDDT

SEQ ID NO: 7297 - protein, 21 aa, Homo sapiens
MSSQQARVIGHVCSPRHSNLQ

SEQ ID NO: 7298 - protein, 29 aa, Homo sapiens
MSSRAPGQAGSPSGGSRCCVCRLCFMRRF

SEQ ID NO: 7299 - protein, 92 aa, Homo sapiens
MSSSPLEATITANISMDGSSRGGPPSPARALPRGARLSARPRGSAPFGAASGVSGRGNMVLKGWGPARARPIRGRPGRRARAGGGRRVWDRG

SEQ ID NO: 7300 - protein, 14 aa, Homo sapiens
MSSTTKSPQDSRTP

SEQ ID NO: 7301 - protein, 18 aa, Homo sapiens
MSSWLEACLCSLHRVSGN

SEQ ID NO: 7302 - protein, 15 aa, Homo sapiens
MSSYNSNVSTSLDTI

SEQ ID NO: 7303 - protein, 36 aa, Homo sapiens
MSSYSMWPFVSGFFYLPSRFIYLVACISTLFLFMTK

SEQ ID NO: 7304 - protein, 16 aa, Homo sapiens
MSTAFLIDSWSSQLNL

SEQ ID NO: 7305 - protein, 22 aa, Homo sapiens
MSTKAKIDKWDLIKLKSFCTAK

SEQ ID NO: 7306 - protein, 144 aa, Homo sapiens
MSTKGTGIRECFSTFLTLIRLLSRVTPFMSKIGSVTTECFITFATFTGLLPSVSSFMYLKGMTPTEGFATLFTFIWLSPSVGSFMCLKRTGTMECFPTLLTFIRLFSSVSSFMYSMGSRITKGFNTLFTFIRFLSSVSSFMDKI

SEQ ID NO: 7307 - protein, 15 aa, Homo sapiens
MSTPLPGTIWSPTLW

SEQ ID NO: 7308 - protein, 23 aa, Homo sapiens
MSTQHIQNYAYGKWPFVLVLLIY

SEQ ID NO: 7309 - protein, 24 aa, Homo sapiens
MSTTISAFKRVQLIGKTRQEYIYI

SEQ ID NO: 7310 - protein, 77 aa, Homo sapiens
MSVKQSTCLPRWLTAGDSHGLHSFPWQSLTHRSSSPQGQSWIKCTSSSVLCSPRSCWVPREPGGGGWRWGFLPSPNQ

SEQ ID NO: 7311 - protein, 52 aa, Homo sapiens
MSVNAQNGGAGRIWGHGRDMRVLPFWKERIPAGRGQAVPGGPGANGTRRVGQ

SEQ ID NO: 7312 - protein, 30 aa, Homo sapiens
MSVPGKFPGHLGNHSEGDGNLLTTSTAILK

SEQ ID NO: 7313 - protein, 13 aa, Homo sapiens
MSVQFSHGGKACL

SEQ ID NO: 7314 - protein, 40 aa, Homo sapiens
MSVQMAVLLLCVGVCVCVHVVCLYVCVWSRVYMHTCVVRK

SEQ ID NO: 7315 - protein, 33 aa, Homo sapiens
MSVSLPVLLPVSILVLHFFLCFFIFLRPPVAFP

SEQ ID NO: 7316 - protein, 17 aa, Homo sapiens
MSWAFTFTHHSLIDSCR

SEQ ID NO: 7317 - protein, 17 aa, Homo sapiens
MSWFLQYECMYIYKVWL

SEQ ID NO: 7318 - protein, 33 aa, Homo sapiens
MSWLLLSHILTFLEVLELAEEEKENVKETNPTS

SEQ ID NO: 7319 - protein, 30 aa, Homo sapiens
MSYCTEASVHDFMSSWLEACLCSLHRVSGN

SEQ ID NO: 7320 - protein, 27 aa, Homo sapiens
MSYLFTSIRIATIKKQKITVLMRMWSD

SEQ ID NO: 7321 - protein, 29 aa, Homo sapiens
MSYLSPIFCKEENNWEGKEKAPLYRKLQF

SEQ ID NO: 7322 - protein, 13 aa, Homo sapiens
MSYNEYTLEHNEN

SEQ ID NO: 7323 - protein, 45 aa, Homo sapiens
MSYSPTWRGKPKNWSVCFGYNTELENVPRSAWHLRREITHLILYR

SEQ ID NO: 7324 - protein, 12 aa, Homo sapiens
MSYYNAWHTAFN

SEQ ID NO: 7325 - protein, 24 aa, Homo sapiens
MTAKKSSWLLSQNQQQSKNLPIFR

SEQ ID NO: 7326 - protein, 29 aa, Homo sapiens
MTATNSFYEFNCHSICTINKTSSFNSIYI

SEQ ID NO: 7327 - protein, 89 aa, Homo sapiens
MTCCLWALAALQSAGSQWTGTAPCPAGRLPQKTSAAPSASFAGCAPFPGPSGRALHLVQLCMCCSLCWNDLPTRIAHSSVTNSCSPSKT

SEQ ID NO: 7328 - protein, 66 aa, Homo sapiens
MTCCLWALAALQSAGSQWTGTAPCPAGRLPQKTSAAPSASFAGCAPFPGPSGRALHLVQLPLALLP

SEQ ID NO: 7329 - protein, 114 aa, Homo sapiens
MTCCLWALAALQSAGSQWTGTAPCPAGRLPQKTSAAPSASFAGCAPFPGPSGRALHLVQLPRPASQVVLLLTPVESAAPSRCFHIPVFRLLQLTYKNCSAIAKDLESLQDCDHV

SEQ ID NO: 7330 - protein, 67 aa, Homo sapiens
MTCCLWALAALQSAGSQWTGTAPCPAGRLPQKTSAAPSASFAGCAPFPGPSGRALHLVQRDPSDYFR

SEQ ID NO: 7331 - protein, 77 aa, Homo sapiens
MTDWAKLLLAGPSGEEIVDDRGVPVQDDWSIAPDDDKVRFSLSGVTPHSWGLWGDTTGHGASASHLCWRKGSGRRSG

SEQ ID NO: 7332 - protein, 58 aa, Homo sapiens [sequence omitted]

SEQ ID NO: 7333 - protein, 25 aa, Homo sapiens
MTEPTDEKAAEAFCPAWDKVSDVFL

SEQ ID NO: 7334 - protein, 41 aa, Homo sapiens
MTESVRSWGGLRVKFSHWHAPGSHLGGKHGCWVHHRGSAHH

SEQ ID NO: 7335 - protein, 51 aa, Homo sapiens
MTESVRSWGGLRVKFSHWHAPGSHLGGKHGCWVHHRGSAHRGSFSTGMLAS

SEQ ID NO: 7336 - protein, 19 aa, Homo sapiens
MTFCQHCIEHICQLIKETP

SEQ ID NO: 7337 - protein, 16 aa, Homo sapiens
MTFHYVGQAGFELLTS

SEQ ID NO: 7338 - protein, 12 aa, Homo sapiens
MTFSKRVAFRQL

SEQ ID NO: 7339 - protein, 14 aa, Homo sapiens
MTFTLIIFKKTKLK

SEQ ID NO: 7340 - protein, 17 aa, Homo sapiens
MTGFHHVGQDGLDLLTS

SEQ ID NO: 7341 - protein, 14 aa, Homo sapiens
MTGHQRRQNTPRGM

SEQ ID NO: 7342 - protein, 14 aa, Homo sapiens
MTGIPERDGESVSN

SEQ ID NO: 7343 - protein, 40 aa, Homo sapiens
MTGNKEDFTLYFRCAVDRVQLRYGTCSTMKSKSKVREGTV

SEQ ID NO: 7344 - protein, 38 aa, Homo sapiens
MTGSRMSRHSCFLKRLLWTISFIDCTFCFWSFTGGMQV

SEQ ID NO: 7345 - protein, 122 aa, Homo sapiens
MTHHDPPAILLGQLARLDGFSDRADLVDLEQQTVAGLFFHCPLNTFWVGHCQVITHNLDPYIGCELGPGSPIILVKWVLNGDHRIVPDKVLVECPQLVPSDVSGRISGRLEVQVIFAITIKL

SEQ ID NO: 7346 - protein, 22 aa, Homo sapiens
MTHIPKHAAISLVSGSQKQQQN

SEQ ID NO: 7347 - protein, 13 aa, Homo sapiens
MTKHQKQCQQKLK

SEQ ID NO: 7348 - protein, 13 aa, Homo sapiens
MTKMCLLEVLPIS

SEQ ID NO: 7349 - protein, 51 aa, Homo sapiens
MTKMPKAIATKAKIDKWDLIKLKSFCTALRTYQQSKPTTYRMGENFCTLSI

SEQ ID NO: 7350 - protein, 18 aa, Homo sapiens
MTKTPKQWQQKPKLTNGI

SEQ ID NO: 7351 - protein, 100 aa, Homo sapiens
MTKTSKAMTTKAKIDKWDQIKLKSFCTGKEIISRVNRQPTEWEKIFVIYPSDKGLISRIYKEFKQIYKKKTNNPIKMWAKDVNRHFWDSPGSSDSPASAS

SEQ ID NO: 7352 - protein, 31 aa, Homo sapiens
MTLAKQNETQSCKICVKDHENLLTTSTYQFP

SEQ ID NO: 7353 - protein, 30 aa, Homo sapiens
MTLCVRSQLNRLQSTGSILNHLVRNAVKLQ

SEQ ID NO: 7354 - protein, 14 aa, Homo sapiens
MTLKMCGFFWNSSP

SEQ ID NO: 7355 - protein, 33 aa, Homo sapiens
MTLKVLHRSEGFPTFLTFIGLLSSVSPTMQLKV

SEQ ID NO: 7356 - protein, 20 aa, Homo sapiens
MTLLLKTVPHFPLFICVFTG

SEQ ID NO: 7357 - protein, 45 aa, Homo sapiens
MTLRVSQPLLQILNFAMEPFGLAQGTIQLLLPLFCFFQNILPALI

SEQ ID NO: 7358 - protein, 18 aa, Homo sapiens
MTLSFLPMSSELFNFRAR

SEQ ID NO: 7359 - protein, 14 aa, Homo sapiens
MTLSLCKTNKCFCG

SEQ ID NO: 7360 - protein, 24 aa, Homo sapiens
MTLSTPSIVFSALSLRLVLSHCIS

SEQ ID NO: 7361 - protein, 14 aa, Homo sapiens
MTLVTEIIQTAWLS

SEQ ID NO: 7362 - protein, 16 aa, Homo sapiens
MTMAPRCHSRILRRAR

SEQ ID NO: 7363 - protein, 16 aa, Homo sapiens
MTMGSDQLNPPNPLQL

SEQ ID NO: 7364 - protein, 117 aa, Homo sapiens
MTMPTTITPITTPKTISHMETGGWLGGPSVGCIPRNSRLLSFRRKASLIRLRDILMAFSTSVLGMISDTFLGAVTKKLKEILGFKLATRTSSSNSFCPASVEFEMSHLCRGPSCLAA

SEQ ID NO: 7365 - protein, 98 aa, Homo sapiens
MTMPTTITPITTPKTISHMETGGWLGGPSVGCIPRNSRLLSFRRKASLIRLRDILMAFSTSVLGMISDTFLGAVTKKLKEILGFKLATRTSSSPKRII

SEQ ID NO: 7366 - protein, 39 aa, Homo sapiens
MTNPVIIINSSLRNVFEKPLFHKIFTLFKLHDSNIFFLF

SEQ ID NO: 7367 - protein, 20 aa, Homo sapiens
MTPMNKFKVKNDPKMIKTTK

SEQ ID NO: 7368 - protein, 81 aa, Homo sapiens
MTPQPFSWASLHAWMASVTEPIWLTLSSRQLQAFSSTARSIRFGLVTVRSSPTIWIPTLAVNLDQAAQSSWSNGSSMETTG

SEQ ID NO: 7369 - protein, 19 aa, Homo sapiens
MTQINMTKKMKTFFPYLYF

SEQ ID NO: 7370 - protein, 28 aa, Homo sapiens
MTRLAVHKVGSRCSPGAGHGPGGRFSSA

SEQ ID NO: 7371 - protein, 23 aa, Homo sapiens
MTRMLFSCSTPSILDSNWLTTVS

SEQ ID NO: 7372 - protein, 48 aa, Homo sapiens
MTRRSTTLGSVTWAFFINISRTLSRPIFTVMSSWNWCTVFGTSRYQAR

SEQ ID NO: 7373 - protein, 22 aa, Homo sapiens
MTRSHCTAIKMAKIQNTDNIKC

SEQ ID NO: 7374 - protein, 27 aa, Homo sapiens
MTSLRATSSYLRSASSAMCLASFSWIS

SEQ ID NO: 7375 - protein, 28 aa, Homo sapiens
MTSLVTASNTCPHCKTASPFCLLSSGET

SEQ ID NO: 7376 - protein, 19 aa, Homo sapiens
MTSSTAEDFSTDVLIVHPL

SEQ ID NO: 7377 - protein, 17 aa, Homo sapiens
MTTFTCVNFTHSKRRFF

SEQ ID NO: 7378 - protein, 93 aa, Homo sapiens [sequence omitted]

SEQ ID NO: 7379 - protein, 40 aa, Homo sapiens [sequence omitted]

SEQ ID NO: 7380 - protein, 12 aa, Homo sapiens
MVATDAGKDREK

SEQ ID NO: 7381 - protein, 65 aa, Homo sapiens
MVAWPETGGTRGRGSEPLLGEEAGSSPERAGGLARKAWPVSARGRSGRATRGASLGSKTGSMRVG

SEQ ID NO: 7382 - protein, 25 aa, Homo sapiens
MVCGGGFGTELIYINRSNKHRSSQI

SEQ ID NO: 7383 - protein, 12 aa, Homo sapiens
MVCQNHLCVLSR

SEQ ID NO: 7384 - protein, 51 aa, Homo sapiens
MVELVFIQGFLRRPAGRLAGGLRSVQLAEGGGRLLRAEASPHLFELKPSDC

SEQ ID NO: 7385 - protein, 11 aa, Homo sapiens
MVEMQNGRATL

SEQ ID NO: 7386 - protein, 42 aa, Homo sapiens
MVFHHVGQAGLELLTSSDPPTLASQSAGITGVSHRAQPRPSL

SEQ ID NO: 7387 - protein, 16 aa, Homo sapiens
MVFIMSYYNAWHTAFN

SEQ ID NO: 7388 - protein, 134 aa, Homo sapiens
MVFLLLAWSFPAKRGVGGSVPGGCSQPRWGVMACKRMTSGSLPRAGRGGGGEAVADPPSPSLQECRGESALLFHKSTRQCTHLLPGTMTRNKELRCRAGSLEGNTEELGDTVISSSGSQSLSGPCPWGGGSGSN

SEQ ID NO: 7389 - protein, 24 aa, Homo sapiens
MVFLQSKTQLQSLCPEWVFFFLFR

SEQ ID NO: 7390 - protein, 49 aa, Homo sapiens
MVFMSLLGHIYTELWQILNTRAFEDSLVDRSLNTCFSAFLRKISLGVAS

SEQ ID NO: 7391 - protein, 11 aa, Homo sapiens
MVFSTMNLTNF

SEQ ID NO: 7392 - protein, 14 aa, Homo sapiens
MVHEAAPVWPLLNF

SEQ ID NO: 7393 - protein, 15 aa, Homo sapiens
MVHLLRTPEVLRCQA

SEQ ID NO: 7394 - protein, 15 aa, Homo sapiens
MVHPPWPTKVLGLQV

SEQ ID NO: 7395 - protein, 40 aa, Homo sapiens
MVIIKKSKNDRCWQGCREIGTLLHCWWESKLVQTLWKTVW

SEQ ID NO: 7396 - protein, 18 aa, Homo sapiens
MVILRIPLTTSLPMGKIK

SEQ ID NO: 7397 - protein, 12 aa, Homo sapiens
MVIYGKIKSRCV

SEQ ID NO: 7398 - protein, 20 aa, Homo sapiens
MVKAVKWSLLPDTCCIPLVF

SEQ ID NO: 7399 - protein, 24 aa, Homo sapiens
MVKAVKWSLLPDTCCIPLVFSPIK

SEQ ID NO: 7400 - protein, 30 aa, Homo sapiens
MVKAVKWSLLPDTCCIPLVFYKIKIAIPIL

SEQ ID NO: 7401 - protein, 13 aa, Homo sapiens
MVKAVKWSLLPHL

SEQ ID NO: 7402 - protein, 24 aa, Homo sapiens
MVKKKKERQCLTMNILWSTMKINA

SEQ ID NO: 7403 - protein, 28 aa, Homo sapiens
MVKNAEKGKDYCSLHDPVPHQCPLVFTR

SEQ ID NO: 7404 - protein, 88 aa, Homo sapiens
MVKSIKPVRKESEDGPIQLGSQNLPFQALASSLVTHSRRLLKFCTAVTIIWGIHIDPLCENWYPVFSHHQSSLNTISCFIQGPLSSQR

SEQ ID NO: 7405 - protein, 36 aa, Homo sapiens
MVLCNQVLNSRCFGHSQEGGHLGPWEGWAHHSTASW

SEQ ID NO: 7406 - protein, 110 aa, Homo sapiens [sequence omitted]

SEQ ID NO: 7407 - protein, 66 aa, Homo sapiens
MVLIPAFMVSLAMSRFTSLSVVISVLINVASTMIIFLIYRPAFQIMAITHFRVIVFAALVLLGTAM

SEQ ID NO: 7408 - protein, 104 aa, Homo sapiens
MVLIPSGPSRDTACFTRSVRPQFSIRKPRSCLNLASMATASSFRDAQKQSSALSWRGSQSTPGSSSRAAWRTSSLSMEKLRRWPACATATRIHSISGGSTRKGL

SEQ ID NO: 7409 - protein, 128 aa, Homo sapiens
MVLIPSGPSRDTACFTRSVRPQFSIRKPRSCLNLASMATASSFRDAQKQSSALSWRGSQSTPGSSSRAAWRTSSLSMEKLRRWPACATATRIHSISGGSTRKGLSTWRLTLEGSTLGFSHSICGQCMK

SEQ ID NO: 7410 - protein, 16 aa, Homo sapiens
MVLLCYPGWTRIPGLK

SEQ ID NO: 7411 - protein, 19 aa, Homo sapiens
MVLLNLRVKVKQVTIGSLF

SEQ ID NO: 7412 - protein, 14 aa, Homo sapiens
MVLQMIPNLFDRFS

SEQ ID NO: 7413 - protein, 14 aa, Homo sapiens
MVLSASAVSNRLSD

SEQ ID NO: 7414 - protein, 15 aa, Homo sapiens
MVLSIPFLQPLPGRE

SEQ ID NO: 7415 - protein, 35 aa, Homo sapiens
MVMFPTVVSFQDNGVGVTPQSSCPHSAGSLSHQLS

SEQ ID NO: 7416 - protein, 61 aa, Homo sapiens
MVMPIKGHGAMHQDVEENTQGPAVHLSYPGAKTGMLQKGSEMLSIAFPARDSHKHKSYSQV

SEQ ID NO: 7417 - protein, 149 aa, Homo sapiens
MVMPIKGHGAMHQDVEENTQGPAVHLWACVGLPIDNLWRGIEGAPTECLQELALMVEVGETEVSNLDIPIGIQEDVLQLEISVDNSVLMAIVHGRDDLPEEMPSFALTELLPLADVVIKVAPAGILHDDHDLAAVLKHFMDGNDVRVVE

SEQ ID NO: 7418 - protein, 16 aa, Homo sapiens
MVMYRWVFGVDVLSVC

SEQ ID NO: 7419 - protein, 29 aa, Homo sapiens
MVNEPGMSNEISMTTFTCVNFTHSKRRFF

SEQ ID NO: 7420 - protein, 23 aa, Homo sapiens
MVNFVQFLCPLCTCSSKLFWFCY

SEQ ID NO: 7421 - protein, 85 aa, Homo sapiens
MVNWNEHKQQTLRPGSQNNSRGSATEKAALALGPVSEILLIHLVSPRTTRPNPTGIYREASGHRLKAVKGRRRRSGPSHRPATDY

SEQ ID NO: 7422 - protein, 68 aa, Homo sapiens
MVPAFPFPLKKKKTIINKGQGIKVIDLEYCSQGMEQEVSWEEQYSKGRSRNTREGQTPRQRSTKTLGL

SEQ ID NO: 7423 - protein, 20 aa, Homo sapiens
MVPKSSSSSCVLFKLPVVPE

SEQ ID NO: 7424 - protein, 52 aa, Homo sapiens
MVPTSFSSSPFTVFVFLISDESQSQTRLCAVNLDRMPNWISFHVAAAPSLQC

SEQ ID NO: 7425 - protein, 67 aa, Homo sapiens
MVPTSFSSSPFTVFVFLISDESQSQTRLCAVNLDRMPNWISFHVAGEVCCPFTPMLGVTLVRSPPQL

SEQ ID NO: 7426 - protein, 82 aa, Homo sapiens
MVPTSFSSSPFTVFVFLISDESQSQTRLCAVNLDRMPNWISFHVAGEVSQSRWKARRNKSHLLPLHSNVRCHAGQESSPALK

SEQ ID NO: 7427 - protein, 46 aa, Homo sapiens
MVPTSFSSSPFTVFVFLISDESQSQTRLCAVNLDRMPNWISSEAET

SEQ ID NO: 7428 - protein, 41 aa, Homo sapiens
MVPTSFSSSPFTVFVFLISDESQSQTRLHFAQAGLHLLTSS

SEQ ID NO: 7429 - protein, 44 aa, Homo sapiens
MVPTSFSSSPFTVFVFLISDESQSQTRLLLASAIISSPALLCCV

SEQ ID NO: 7430 - protein, 27 aa, Homo sapiens
MVQGVVEDVPPQIWIIPLIPSFNTTCS

SEQ ID NO: 7431 - protein, 15 aa, Homo sapiens
MVQSNLALKISLSRH

SEQ ID NO: 7432 - protein, 15 aa, Homo sapiens
MVRGIKNFVVEYRKI

SEQ ID NO: 7433 - protein, 41 aa, Homo sapiens
MVRKHRQCLRQKEDTSKCIFSQILMATFGKHLIAWLINALS

SEQ ID NO: 7434 - protein, 38 aa, Homo sapiens
MVSFSMMSIRTVRFNSFFSYTLINWTYSLTLESSFSNF

SEQ ID NO: 7435 - protein, 89 aa, Homo sapiens
MVSISCPCDPPASASQSAGITGVSYHARPSCVFFTVTGSFLRKVISFVFGFPQLIKIYQKHYNLQGKRFFNGCRNQKEIAFLICINTNI

SEQ ID NO: 7436 - protein, 17 aa, Homo sapiens
MVSISRISFLSLFSFAS

SEQ ID NO: 7437 - protein, 45 aa, Homo sapiens
MVSISRPCEPPASASQSAGITGMSHHARPSYCNFSNALFVFASRW

SEQ ID NO: 7438 - protein, 54 aa, Homo sapiens
MVSISRPHDLPASASQSAGITGVSHRARPLFMLFKAFLTQALLPLPSDYHFHSL

SEQ ID NO: 7439 - protein, 32 aa, Homo sapiens
MVSISRPRDLPASTSQSAGITGMSHCARPGVG

SEQ ID NO: 7440 - protein, 33 aa, Homo sapiens
MVSISRPRDPPASASQSAGTTGMSHRARPCFCF

SEQ ID NO: 7441 - protein, 15 aa, Homo sapiens
MVSIYRPQDLPISAS

SEQ ID NO: 7442 - protein, 93 aa, Homo sapiens [sequence omitted]

SEQ ID NO: 7443 - protein, 59 aa, Homo sapiens
MVSLAMSRFTSLSVVISVLINVASTMIIFLIYRPAFQIMAITHFRVIVFAALVLLGTAM

SEQ ID NO: 7444 - protein, 16 aa, Homo sapiens
MVSLMVCQNHLCVLSR

SEQ ID NO: 7445 - protein, 83 aa, Homo sapiens
MVSNSRPRDPPTSASQSAGITGMSHCARPKNNSLKMYLRATCKASLLSNPRLGPPVFLSSYPSQPPLQASDALFSSSVSVQLL

SEQ ID NO: 7446 - protein, 16 aa, Homo sapiens
MVSPCWPGWSRTPHLR

SEQ ID NO: 7447 - protein, 115 aa, Homo sapiens
MVSRISSSWWRVDVPGNRGLPRSISPRIQPRLHMSTPRVYRCEESSTSGARYQRVATYSVTAWSSGPSGRSPRERARPKSHSFTVQLASRSTLDGFWSRCTTCPEWRNRVARRSW

SEQ ID NO: 7448 - protein, 19 aa, Homo sapiens
MVSSGFGIAPDLPCPKSAW

SEQ ID NO: 7449 - protein, 22 aa, Homo sapiens
MVSSPDLVIHPPQPPKVLGLQA

SEQ ID NO: 7450 - protein, 18 aa, Homo sapiens
MVSTIIPHTRLNAHRGPQ

SEQ ID NO: 7451 - protein, 90 aa, Homo sapiens
MVSVPEPQGPPVRSTGPLPTLWPEPWTHVAAAQGPRRACRGTLRAAPRLPAPSLPGCTRLSLPGMGDTAPLPIPTAGCSLAAPWPDARGL

SEQ ID NO: 7452 - protein, 61 aa, Homo sapiens
MVTCFESFRKMPVLNYFFIRNHMMIQRFERPYTVNKNMSISFFKAYWTIKHSEGNEGWTGR

SEQ ID NO: 7453 - protein, 24 aa, Homo sapiens
MVTEPPSCSFVDGFTEITVFLGDM

SEQ ID NO: 7454 - protein, 51 aa, Homo sapiens
MVTGSDSVGCWTVFGSSPAGESCLPSESSRASQMPFLSFSLISSIVLKSSA

SEQ ID NO: 7455 - protein, 29 aa, Homo sapiens
MVTNADTMPGLCFNSSMLLNIRHALEILP

SEQ ID NO: 7456 - protein, 40 aa, Homo sapiens
MVTTELIHLIYIYNLPLKNDALCVCTVHICLRVGTHTKHT

SEQ ID NO: 7457 - protein, 14 aa, Homo sapiens
MVTVLTLEFNNCMG

SEQ ID NO: 7458 - protein, 11 aa, Homo sapiens
MVVCCTYGPIL

SEQ ID NO: 7459 - protein, 63 aa, Homo sapiens
MVVKERDLAATSAARPAVKVKSGDSCSRASLCLMEGCNESLGVGGAVVRPLPSACGSSSLSHW

SEQ ID NO: 7460 - protein, 16 aa, Homo sapiens
MVVVALQRCARFRRTR

SEQ ID NO: 7461 - protein, 14 aa, Homo sapiens
MVWIFVPCKYHVEM

SEQ ID NO: 7462 - protein, 11 aa, Homo sapiens
MVYFIILKGFF

SEQ ID NO: 7463 - protein, 14 aa, Homo sapiens
MVYILYRKISNYLF

SEQ ID NO: 7464 - protein, 27 aa, Homo sapiens
MWARLVSNFWPQVTCPLQPPKMLGLQV

SEQ ID NO: 7465 - protein, 12 aa, Homo sapiens
MWASWSRTPDLK

SEQ ID NO: 7466 - protein, 49 aa, Homo sapiens
MWGKLEPLCTVGRNANDATMENSMEVPQKIKNRTNMIQQSHYWVYIQKK

SEQ ID NO: 7467 - protein, 19 aa, Homo sapiens
MWGLGDSLRRQSCFCGEQQ

SEQ ID NO: 7468 - protein, 57 aa, Homo sapiens
MWIFIFNKYYQHVKSPTMSRTGKSATCDGCGMAAHCSRCWGLSWGLGEALSYSKNVS

SEQ ID NO: 7469 - protein, 14 aa, Homo sapiens
MWINWNSHTLLVGM

SEQ ID NO: 7470 - protein, 15 aa, Homo sapiens
MWKIHFSARRSGSHL

SEQ ID NO: 7471 - protein, 15 aa, Homo sapiens
MWKKENLCTLMVGCK

SEQ ID NO: 7472 - protein, 12 aa, Homo sapiens
MWKSLQPQIKPH

SEQ ID NO: 7473 - protein, 17 aa, Homo sapiens
MWLIMFLSSGNNFLASR

SEQ ID NO: 7474 - protein, 20 aa, Homo sapiens
MWLKGERKRPTYRPVATFHH

SEQ ID NO: 7475 - protein, 40 aa, Homo sapiens
MWLSVCVPCWPHSSQVEGSTEIVVLMMNRKKLEALATCLV

SEQ ID NO: 7476 - protein, 12 aa, Homo sapiens
MWNQPKCPSLDG

SEQ ID NO: 7477 - protein, 31 aa, Homo sapiens
MWPFVSGFFYLPSRFIYLVACISTLFLFMTK

SEQ ID NO: 7478 - protein, 18 aa, Homo sapiens
MWPRTTLNVAQPKFVNFL

SEQ ID NO: 7479 - protein, 83 aa, Homo sapiens
MWRNRNTFHCWWDCKLVQPLWKTVWQFLKDLELEIPFNPAIPLLGIYPKDYKSFYYKDTCMFTAALLTIAKTWNQPKCPSVID

SEQ ID NO: 7480 - protein, 14 aa, Homo sapiens
MWRNWNSHTLLVGM

SEQ ID NO: 7481 - protein, 17 aa, Homo sapiens
MWSCFWKSLHLRLDLAS

SEQ ID NO: 7482 - protein, 19 aa, Homo sapiens
MWSCFWKSLHLRLDLASTQ

SEQ ID NO: 7483 - protein, 11 aa, Homo sapiens
MWSFEFYKWFL

SEQ ID NO: 7484 - protein, 26 aa, Homo sapiens
MWSIRTLLKEGLSCFWYHRFSCAFQI

SEQ ID NO: 7485 - protein, 48 aa, Homo sapiens
MWSKWNSQILLREVGNGASSLENSLMIFIKLSIYLCCDSEIPSLTIYL

SEQ ID NO: 7486 - protein, 38 aa, Homo sapiens
MWYEATVSFHNSGCSGPTTGLTNFGRGDEILFSPHFHG

SEQ ID NO: 7487 - protein, 22 aa, Homo sapiens
MYCSLISWKTGFFDPECGGDDE

SEQ ID NO: 7488 - protein, 24 aa, Homo sapiens
MYDYKFIIKYLEVNIACICERQIL

SEQ ID NO: 7489 - protein, 15 aa, Homo sapiens
MYERRHAKLKIVLKN

SEQ ID NO: 7490 - protein, 20 aa, Homo sapiens
MYFAYEKDINFGKQGHNVMV

SEQ ID NO: 7491 - protein, 19 aa, Homo sapiens
MYFGGVPAWVNKNMRVSKK

SEQ ID NO: 7492 - protein, 39 aa, Homo sapiens
MYFLTNINGNLWETSHCLAYKRFILSLIQTVKQLQKSQL

SEQ ID NO: 7493 - protein, 129 aa, Homo sapiens
MYFRDLTRVYTIWYLFLYISSLRVLYHHFLVAMAGTNHSFFFETESRSVAQADVQWRDLGSLQPLPPGFKRFSCLSLLSSWDYRRPPPCPANFCVFSRDGVSPYWPSWSRNPDLVICPPQPPKVLGLQA

SEQ ID NO: 7494 - protein, 37 aa, Homo sapiens
MYFYIVYPGSLFITNSQISLHCLEIFSEPTSSLPSSK

SEQ ID NO: 7495 - protein, 29 aa, Homo sapiens
MYGVTKVRSNCPLFSSPILCIKGFIQPQA

SEQ ID NO: 7496 - protein, 34 aa, Homo sapiens
MYHCTWLICGCVCVFSRGGVSPCWPHWSRTPGLK

SEQ ID NO: 7497 - protein, 27 aa, Homo sapiens
MYHFHSMMECCCAHTTLWLGDHTTASS

SEQ ID NO: 7498 - protein, 73 aa, Homo sapiens
MYHHAWLIFLFFVDTGFHHVGQAGLELLTSSDLPASACQSVGITSMSYRTCPQICFGFRDRISLSPPDCSAVV

SEQ ID NO: 7499 - protein, 12 aa, Homo sapiens
MYHHTWLIFVFM

SEQ ID NO: 7500 - protein, 11 aa, Homo sapiens
MYHHTWLILYF

SEQ ID NO: 7501 - protein, 27 aa, Homo sapiens
MYHRGEREERVSAHLPADRRGSGVSSQ

SEQ ID NO: 7502 - protein, 28 aa, Homo sapiens
MYIISENASMIALVYNENVFLLKLHFVQ

SEQ ID NO: 7503 - protein, 14 aa, Homo sapiens
MYIKTSHCILYTFL

SEQ ID NO: 7504 - protein, 16 aa, Homo sapiens
MYILYKGDNGELLFSF

SEQ ID NO: 7505 - protein, 21 aa, Homo sapiens
MYISLLHHKHKNNINIFTYMY

SEQ ID NO: 7506 - protein, 21 aa, Homo sapiens
MYIVLCRSNSFIFIDVGYAIL

SEQ ID NO: 7507 - protein, 35 aa, Homo sapiens
MYIYLCWTRCSFLLGRTGQAFYLAAVLCSWHPAWR

SEQ ID NO: 7508 - protein, 39 aa, Homo sapiens
MYKRNSVGYLLEKTLHVRTFSQQVMLKPAMLLNAQTKQN

SEQ ID NO: 7509 - protein, 40 aa, Homo sapiens
MYKVFLGMGVYSLTVPCFIQASTCKFVYIMAFNDPPFSFL

SEQ ID NO: 7510 - protein, 131 aa, Homo sapiens
MYLKIIKAIYDKLTANIILNGQNLEAFPEKTVTRQGCPLSPLLFNIMLEVLARAIRQEKKIKGIQIEREEFKLSLFADDMILYLENPIVSAQNLLKLISNFSKVSGYKINVQKPQAFLYTNNKKNREPNHE

SEQ ID NO: 7511 - protein, 30 aa, Homo sapiens
MYLKSHYSIKYLHCLNYMTATFSFYFSSTY

SEQ ID NO: 7512 - protein, 40 aa, Homo sapiens
MYLMKFQRYFILLSYTHTHTHTHTHTHTHHTLDRISPHFL

SEQ ID NO: 7513 - protein, 14 aa, Homo sapiens
MYLPVCLFNFAGNQ

SEQ ID NO: 7514 - protein, 11 aa, Homo sapiens
MYLSADVFEFL

SEQ ID NO: 7515 - protein, 17 aa, Homo sapiens
MYLTCDITKYHTEMETA

SEQ ID NO: 7516 - protein, 12 aa, Homo sapiens
MYQDQPGTCEER

SEQ ID NO: 7517 - protein, 42 aa, Homo sapiens
MYQYFIPFYDQIIFHCTDIPRFAYPFTQLIVDRLWVFILFGC

SEQ ID NO: 7518 - protein, 25 aa, Homo sapiens
MYRHARLIFVFLVETGFHHVGQTGL

SEQ ID NO: 7519 - protein, 21 aa, Homo sapiens
MYRLSFSHTNSLSTSTYIFPT

SEQ ID NO: 7520 - protein, 14 aa, Homo sapiens
MYRWVFGVDVLSVC

SEQ ID NO: 7521 - protein, 25 aa, Homo sapiens
MYSALKSTLVHSNVLGLHIHSPFTH

SEQ ID NO: 7522 - protein, 16 aa, Homo sapiens
MYSCYKISKKHTNRKH

SEQ ID NO: 7523 - protein, 160 aa, Homo sapiens
MYTFVCGVSSEGLLFNQGAPVKTWASVRKLTCPLAEMMLKYVFHTDFQSSPGRFSSQGPNCLDKSPFIGCSSSLANFLTILLVFLEIASCVPRVCYDEAGVRCGMVNCQYLDHIHVHKNWSHARATAGQEREDVVHGSQTRDAGRARWLTLVIPALWEAE

SEQ ID NO: 7524 - protein, 20 aa, Homo sapiens
MYVKIADKNKSLTCNTKFLT

SEQ ID NO: 7525 - protein, 26 aa, Homo sapiens
MYVKKGGFTKHKQKTTFIYDVIQIHG

SEQ ID NO: 7526 - protein, 15 aa, Homo sapiens
MYVSTSPDETSNPGK

SEQ ID NO: 7527 - protein, 56 aa, Homo sapiens
MYYIKYIFIHICAHTQDGFMDMQPVQLHKTVLRSTPHLIFERGPYSFILPLVPQIM

SEQ ID NO: 7528 - protein, 27 aa, Homo sapiens
MAFIWLFSSACSLMSSKVGGQTEGLPT

SEQ ID NO: 7529 - protein, 51 aa, Homo sapiens
MAFLHVGQAGLELPTSGDLPTFASQSAGITGVSHRARPCYHLLPTPLSKVD

SEQ ID NO: 7530 - protein, 26 aa, Homo sapiens
MAGWRCVVQVLHEAKRGSWDTAGRGD

SEQ ID NO: 7531 - protein, 18 aa, Homo sapiens
MAHTCNPSTLGGQDRRTA

SEQ ID NO: 7532 - protein, 12 aa, Homo sapiens
MAIKKTKDNKCW

SEQ ID NO: 7533 - protein, 26 aa, Homo sapiens
MAILKKTKDNKYGLGCREKGTLVHSW

SEQ ID NO: 7534 - protein, 42 aa, Homo sapiens
MAKIKNADNTKLCQEFLQITGGSIGICTSENMFTKRLVISCL

SEQ ID NO: 7535 - protein, 33 aa, Homo sapiens
MALLFQVLLYDEFYFVLLLLPFFFYFNLHWLEK

SEQ ID NO: 7536 - protein, 21 aa, Homo sapiens
MALLLKTWYSWHPEKRHCYVI

SEQ ID NO: 7537 - protein, 56 aa, Homo sapiens
MALVLEAGGLSREDDDRGPLKDALRLWRGMLELALVGKSTTTRLSLITPSASVVPS

SEQ ID NO: 7538 - protein, 94 aa, Homo sapiens [sequence omitted]

SEQ ID NO: 7539 - protein, 21 aa, Homo sapiens
MALYVYWRRGFTTLARLVSNS

SEQ ID NO: 7540 - protein, 20 aa, Homo sapiens
MANFCIFSTDRVSPSWPRWS

SEQ ID NO: 7541 - protein, 109 aa, Homo sapiens
MAPGQSGRERGRRGGLGRRSPGSGPQWTWHLALRGALGWGAREGRAGPPPGKGRRTCALRKAGGRGHAEPAGGGPGADGRLTEAARRVGGRRPGGAAAGAARWRPGVRG

SEQ ID NO: 7542 - protein, 133 aa, Homo sapiens
MAPHLRPQQAAECQTAPRLRPHQAAQCHAAPRLGPHQATRCQRRPKPQDSPSHTVPSHPTPWASPSRTVPVTSHALGLSKPHGANAAPRLRPQQVARCQAEVKHISAVLWHFQCPGLCPFLQALWPHGHLCPC

SEQ ID NO: 7543 - protein, 42 aa, Homo sapiens
MAPLIFVFFLVEMGFHHVGQAGLKLLTSGDLPSLASQSVKLF

SEQ ID NO: 7544 - protein, 70 aa, Homo sapiens
MAPQNYMLRTPPDKQTGFQAEGPLDLREGSGSAGPCRFARREPGGRPASHPHPTPAPWGLPILDTLVPER

SEQ ID NO: 7545 - protein, 24 aa, Homo sapiens
MAPSRLTATSASQIQVILLPQPSK

SEQ ID NO: 7546 - protein, 24 aa, Homo sapiens
MAPSWPTATSASWVQAILLPQPPE

SEQ ID NO: 7547 - protein, 528 aa, Homo sapiens
MARGHELLFLLVPPAAQSEALPDALGGPAGVLGAGGVAQAVVLRGQLRVGEVAGPRPGEWLQDGRLAPQALVRRRRRWPGGRRWLGRVGAGVRVPVLAVLATLLGLGPQHGGRGCHSEDGVGRGGALLDVLGLGGRGLVHPDGLGSEGAGAAHGAAGRGAGTRGPGGLHAVVPLQAVAEGVLVPGRQEAVLGGQRLGQQHQRRLRDGHGPRLDALEGGGLGLERVDAVVDDLVDLVHLLGDGGDLGHRTLAVGARPAQLTVPAFRRVPGSNLHVAALAGLGGVRALHQLVLLHLAGRRQVRDARHGLGAQQRALGQRGQAGRLQLWPVLELDDGLLEAASCGCRGGLLVLLLLAPPPAQAVVDGAQHQHHAEEAAQDGHDVVGGRGGAGHRTRRAGQPGQADGEAGVVVAQPGAGGHHAVGVVGEREQVGQTDLLLGLGQPGHGGGLAVVEMLQGVHPVERAGQLDGDGGRVLSELLDLDEGAGLGLRGQRGQGHQWRGAVPGEALIIGTGHVTGLRRRRGRRGAARL

SEQ ID NO: 7548 - protein, 12 aa, Homo sapiens
MASCRKLPDIHF

SEQ ID NO: 7549 - protein, 38 aa, Homo sapiens
MASYDVWPFVSGFFRLTMFSRCIMSKHGSVRHSFSGLK

SEQ ID NO: 7550 - protein, 274 aa, Homo sapiens
MATKDKIDKWDLIQLKSFCTAKETTIRVNRQLTKWQKIFATYSSDKGLISRIYNELKQIYKKKTNNPIKKWAKDMNRHFSKEDIYAAKKHMKKCSPSLTIREMQIKTTMRYHLTPVRMAIIKKSGNNRCWRGCGEIGTLLHCWWDCKLVQPLWKSVWRFLRNLELEIPFDPAIPLLGIYSKDYKSCCYKDTCTRMFIAALFTIAKTWNQPKCPTMIDWIKKMWHIYTMEYYAAIKKDEFMSFVGTWMKLEIIILSKLSQGQKTKHHMFSLIDGN

SEQ ID NO: 7551 - protein, 11 aa, Homo sapiens
MATYNQGPQSA

SEQ ID NO: 7552 - protein, 12 aa, Homo sapiens
MAWSWLTATSAS

SEQ ID NO: 7553 - protein, 26 aa, Homo sapiens
MAYFVLCLLGDEVRHIHRWLLLAKAM

SEQ ID NO: 7554 - protein, 11 aa, Homo sapiens
MCCEYKILTGF

SEQ ID NO: 7555 - protein, 12 aa, Homo sapiens
MCCLPPPPRTGK

SEQ ID NO: 7556 - protein, 73 aa, Homo sapiens
MCHHALLISYIIEMGFHHVGQAGLELLTSNDVPVSASQNSGITGMSHCVQPAFSKLLPHWFTLKVKAIARISY

SEQ ID NO: 7557 - protein, 20 aa, Homo sapiens
MCHHAQLIFCIFSRDGVSPC

SEQ ID NO: 7558 - protein, 25 aa, Homo sapiens
MCHHAQLIFLCVFFSRDGVSPCWPG

SEQ ID NO: 7559 - protein, 12 aa, Homo sapiens
MCHHAQLIFLYF

SEQ ID NO: 7560 - protein, 43 aa, Homo sapiens
MCHHAQLIFVFFSRDGVSPCWPGWSRSLDLVILLPRPPKVLGF

SEQ ID NO: 7561 - protein, 27 aa, Homo sapiens
MCHHAQLIFVFLVETEFTMLARLVSNS

SEQ ID NO: 7562 - protein, 38 aa, Homo sapiens
MCHHAQLIFVFLVETGFHHVGQAGLELLTSGDLPASAS

SEQ ID NO: 7563 - protein, 12 aa, Homo sapiens
MCHHAQVIFLYF

SEQ ID NO: 7564 - protein, 56 aa, Homo sapiens
MCHHARLIFVFLVETGFHHVGQTVLELLTSGNPPASASQSAGITGISHCAQPVTFL

SEQ ID NO: 7565 - protein, 43 aa, Homo sapiens
MCHHARLIFVFLVETGLHHVGQACLELRTSSDPPALASRSAGI

SEQ ID NO: 7566 - protein, 11 aa, Homo sapiens
MCHHARLIFYF

SEQ ID NO: 7567 - protein, 21 aa, Homo sapiens
MCHHARQIFVFLVETWSRHVG

SEQ ID NO: 7568 - protein, 20 aa, Homo sapiens
MCHHAWLIFCIFSTDRVSPC

SEQ ID NO: 7569 - protein, 44 aa, Homo sapiens
MCHHAWLIFFVFLVEMGFHHVGHAGLELLTSGDLPASGSQVLGL

SEQ ID NO: 7570 - protein, 45 aa, Homo sapiens
MCHHAWLIFVFFVETGFCHVGQAGFKFLTSSDPPPWPPKVLGLQA

SEQ ID NO: 7571 - protein, 27 aa, Homo sapiens
MCHHAWLLFVCLVETGFTMLPRLLCNF

SEQ ID NO: 7572 - protein, 50 aa, Homo sapiens
MCHHAWLVFVFLVKMQFHHIAQAGLILLASSDPPASASQSAGITGMSQRA

SEQ ID NO: 7573 - protein, 13 aa, Homo sapiens
MCHHTQINFLYFW

SEQ ID NO: 7574 - protein, 18 aa, Homo sapiens
MCHHTQLVFFFLLFFFFF

SEQ ID NO: 7575 - protein, 11 aa, Homo sapiens
MCHHTRLILYF

SEQ ID NO: 7576 - protein, 25 aa, Homo sapiens
MCHHTWLIFLYFSRDGVSPFWPAWS

SEQ ID NO: 7577 - protein, 51 aa, Homo sapiens
MCHHTWLIFVETGFCHVGQAGLELLGLPKCWDYRHGLPCLAQIHLFCFIFI

SEQ ID NO: 7578 - protein, 31 aa, Homo sapiens
MCHHTWLIFVFLVEMGFHYVGQAGLKTPDLR

SEQ ID NO: 7579 - protein, 89 aa, Homo sapiens
MCHHTWPLTFILTEKGRLICEIACFPGFWRWVESRHCPSRGCGPCLSEPAPGRCPGEHGELEAPPWGCLESTVLGLRLHVLPSVLSQLS

SEQ ID NO: 7580 - protein, 55 aa, Homo sapiens
MCHHVWLIFVFSVEKGFHHVGQADLDLLTSGDPPVWASQSAGITGVSHHAQPPYC

SEQ ID NO: 7581 - protein, 11 aa, Homo sapiens
MCHYDWLILYF

SEQ ID NO: 7582 - protein, 13 aa, Homo sapiens
MCLGLRAENFVLS

SEQ ID NO: 7583 - protein, 31 aa, Homo sapiens
MCLHAWLIFCIFSRGGVSPCWPGWSQTPDLR

SEQ ID NO: 7584 - protein, 15 aa, Homo sapiens
MCLSSSALISKEKKS

SEQ ID NO: 7585 - protein, 14 aa, Homo sapiens
MCPPRPPKVLGIQA

SEQ ID NO: 7586 - protein, 14 aa, Homo sapiens
MCPSRPPKILGLQA

SEQ ID NO: 7587 - protein, 12 aa, Homo sapiens
MCPSSAELLCQP

SEQ ID NO: 7588 - protein, 42 aa, Homo sapiens
MCRHAQLIFVFLVEIGISPGWPGWSRSDLMICPLWLPKVLGL

SEQ ID NO: 7589 - protein, 71 aa, Homo sapiens
MCRHAWLILYFLWRRDRPIFPRLVNLIFNCCFFFFSRCCPVQVWQEPGRSRCQAATDQRGGAAEEERGPAE

SEQ ID NO: 7590 - protein, 13 aa, Homo sapiens
MCRNSIHYKYLCE

SEQ ID NO: 7591 - protein, 25 aa, Homo sapiens
MCWQGRAKNGTLIHCWWECKLVQSL

SEQ ID NO: 7592 - protein, 25 aa, Homo sapiens
MCYHAWLILCSFSRDGVSACCPGWS

SEQ ID NO: 7593 - protein, 11 aa, Homo sapiens
MCYHAWLVLYF

SEQ ID NO: 7594 - protein, 31 aa, Homo sapiens
MDELRSNIIDPSRSETPSAPTGQSRFPRGEA

SEQ ID NO: 7595 - protein, 15 aa, Homo sapiens
MDFRHVSQAGLELLT

SEQ ID NO: 7596 - protein, 82 aa, Homo sapiens
MDGSFLRSANIFLGWSSQRRVQAAIFAVSQPSLVRHPGTGKFEVTRDWSRPLGYYSSPLDDLGSLIWAFLSSRTYQVSQGMY

SEQ ID NO: 7597 - protein, 14 aa, Homo sapiens
MDPGLFPRQFAETE

SEQ ID NO: 7598 - protein, 76 aa, Homo sapiens
MDQHARLIFVFLVETGFLHVGQAGLELPTSGDLPASASQSAGITGVSHRARPISILFSRDRVSPCWSGWSGNPDLR

SEQ ID NO: 7599 - protein, 21 aa, Homo sapiens
MDTQAEICIKHVLLINENANV

SEQ ID NO: 7600 - protein, 21 aa, Homo sapiens
MDTQTKICIKYVLLINENVSI

SEQ ID NO: 7601 - protein, 21 aa, Homo sapiens
MDTQTKICIKYVLLISENVNI

SEQ ID NO: 7602 - protein, 45 aa, Homo sapiens
MECHSVAQAGVQWCDLSSLQPLPPGFKRFLYLSLSSSWCYKHEPP

SEQ ID NO: 7603 - protein, 58 aa, Homo sapiens
MECITSSINSNKKLGTQIWLFRLKIFITGRFAFPRKTYHWKHLENANWVKPIPKSIIK

SEQ ID NO: 7604 - protein, 51 aa, Homo sapiens
MEFHHVGQAGLELLTSSDPPTLTSQSAGITGVIHHARPHRSIFHIPKPSIE

SEQ ID NO: 7605 - protein, 49 aa, Homo sapiens
MEFHHVGQAGLKLLTLSDLSLSNCWDYRREPPRPASIICLSFASLSPSF

SEQ ID NO: 7606 - protein, 16 aa, Homo sapiens
MEFHHVSQDGLNLLTS

SEQ ID NO: 7607 - protein, 16 aa, Homo sapiens
MEFHRVSQDGLHLLTS

SEQ ID NO: 7608 - protein, 56 aa, Homo sapiens
MEFLHVGQAGLQLPNSGDLPTSASQSAGITGVRHCARPTLNIFLKSRCTQGSGLCW

SEQ ID NO: 7609 - protein, 31 aa, Homo sapiens
MEFRHVGQAGLELLTSSDPPALASQSAGIQA

SEQ ID NO: 7610 - protein, 72 aa, Homo sapiens
MEFYHVGQAGLKLLTSGNPPTLASESAGITGMSHRAQPTFFFFFLIQTFFLDTVSLCHSVWSAMARSQLTLA

SEQ ID NO: 7611 - protein, 23 aa, Homo sapiens
MEKINYIQEYKTPKVFFNYQQVK

SEQ ID NO: 7612 - protein, 15 aa, Homo sapiens
MEKLESLHTTDGSAI

SEQ ID NO: 7613 - protein, 47 aa, Homo sapiens [sequence omitted]

SEQ ID NO: 7614 - protein, 22 aa, Homo sapiens
MELLLSKASPRLKSSPSSSRRR

SEQ ID NO: 7615 - protein, 65 aa, Homo sapiens
MELTMLPRLVLNSWSQAILPLQPSKVLGVQAQATVPSCQTLSFNYAPNSSPQILFTKAPGWSSPS

SEQ ID NO: 7616 - protein, 38 aa, Homo sapiens
MENHTWLVFVFLVEMKFHHVGLAGLKLLTSSDLPALVS

SEQ ID NO: 7617 - protein, 23 aa, Homo sapiens
MENLSLGIPVTPTFLIHIVFILV

SEQ ID NO: 7618 - protein, 127 aa, Homo sapiens
MEPLFILHMLIDVSCLPVPLVWGAHASSGPARPGLVPGSRPSAPPPAPVAPALSPAAWQQPDFLPCSDPESGPLTFGSGPFQCHHSGAASPGPAAPDHAPGSAPFPLPGTAVACTFQCPAGIGPPVP

SEQ ID NO: 7619 - protein, 12 aa, Homo sapiens
MEPLFTVGGSVN

SEQ ID NO: 7620 - protein, 11 aa, Homo sapiens
MEPMQGSQEGQ

SEQ ID NO: 7621 - protein, 24 aa, Homo sapiens
MEQSRLTATSASWVQAILLSQLPD

SEQ ID NO: 7622 - protein, 12 aa, Homo sapiens
MERIPDNTCFLR

SEQ ID NO: 7623 - protein, 14 aa, Homo sapiens
MESCSCCPGWSAMA

SEQ ID NO: 7624 - protein, 69 aa, Homo sapiens
MESCSITQVGVQRHDLGLLQPLPPGFKRLFCLSLPSSWDYRRPPPCPVNFLYFYQRWGFTMLSRLVSNS

SEQ ID NO: 7625 - protein, 72 aa, Homo sapiens
MESHSVAQAGVPWRNLSSLQTPPPGFTPFSCLSLQSSWDYRHLPQHPANFFVFLVETGFHCVSQDGLDLLTS

SEQ ID NO: 7626 - protein, 52 aa, Homo sapiens
MFAEIYLYQRQFIVHNLSGLCFTWGLRFRERVVSHKCLLNTNNLPHCTTEGK

SEQ ID NO: 7627 - protein, 68 aa, Homo sapiens [sequence omitted]

SEQ ID NO: 7628 - protein, 11 aa, Homo sapiens
MFAMAAEPSYG

SEQ ID NO: 7629 - protein, 38 aa, Homo sapiens [sequence omitted]

SEQ ID NO: 7630 - protein, 13 aa, Homo sapiens
MFFLQKTANNRCW

SEQ ID NO: 7631 - protein, 89 aa, Homo sapiens
MFFVFLVETRFCHVGQVGLKLLTSSDPPASAFQSAGVTGLSHCTWPPSFQAGKPSFPVVVCLWAVTMRQSLWKCQIVTALKANIQDNGE

SEQ ID NO: 7632 - protein, 47 aa, Homo sapiens [sequence omitted]

SEQ ID NO: 7633 - protein, 18 aa, Homo sapiens
MFICKFMREGLESYPLNF

SEQ ID NO: 7634 - protein, 38 aa, Homo sapiens
MFIFSSLCQSKREFLSTLHSEKLLRLLKVKIMSIGRIS

SEQ ID NO: 7635 - protein, 85 aa, Homo sapiens
MFIRLLSNSGPQVIRLPWPPEVLGLQMRATVPSSIHPFYKYLLNASYVPGTVLGTGDTAEKKWTATTACTTLTFHLRCPRLESRD

SEQ ID NO: 7636 - protein, 24 aa, Homo sapiens
MFLCAYKFQILLGKYLGCDCWVIC

SEQ ID NO: 7637 - protein, 13 aa, Homo sapiens
MFLENHPLIPSIR

SEQ ID NO: 7638 - protein, 18 aa, Homo sapiens
MFLVERGFTMLARLVSNS

SEQ ID NO: 7639 - protein, 45 aa, Homo sapiens
MFLVETGFHHVGQAGLKLLTSSDPPALASQSAGITDVSHCTQAPL

SEQ ID NO: 7640 - protein, 30 aa, Homo sapiens
MFPSPIMPATPIPLLAGPRWGQQQPSGLGM

SEQ ID NO: 7641 - protein, 29 aa, Homo sapiens
MFQAVSSAPPSGLKLSMEAFRLSCLCGKS

SEQ ID NO: 7642 - protein, 15 aa, Homo sapiens
MFQFEGGAASDPGGS

SEQ ID NO: 7643 - protein, 19 aa, Homo sapiens
MFQFEGPAAGDPWGSDVPV

SEQ ID NO: 7644 - protein, 15 aa, Homo sapiens
MFQFEVHAAGDLVGS

SEQ ID NO: 7645 - protein, 11 aa, Homo sapiens
MFRHVGQAGLE

SEQ ID NO: 7646 - protein, 15 aa, Homo sapiens
MFRRDGVSPCWSGWS

SEQ ID NO: 7647 - protein, 12 aa, Homo sapiens
MFRSTLRWHSAQ

SEQ ID NO: 7648 - protein, 12 aa, Homo sapiens
MFSGIFAEEVLK

SEQ ID NO: 7649 - protein, 32 aa, Homo sapiens
MFSICCRRISITLSFSVICSLRASHSVCTFLR

SEQ ID NO: 7650 - protein, 21 aa, Homo sapiens
MFSISRPQVIHLPQPPKVLGL

SEQ ID NO: 7651 - protein, 17 aa, Homo sapiens
MFSPQALQLHLLGCSGH

SEQ ID NO: 7652 - protein, 21 aa, Homo sapiens
MFSRCIMSKHGSVRHSFSGLK

SEQ ID NO: 7653 - protein, 15 aa, Homo sapiens
MFSRDGVSPCWPGWS

SEQ ID NO: 7654 - protein, 35 aa, Homo sapiens
MFSRDGVSPCWPGWSQSLDLVICPPRPPKVLGLKA

SEQ ID NO: 7655 - protein, 35 aa, Homo sapiens
MFSSDGVSPRWPRWSQSVDLMIRSPQPPKVLGLQV

SEQ ID NO: 7656 - protein, 32 aa, Homo sapiens
MFSWEKQKTPRRPPRMVVSKTTLLSATSSGPS

SEQ ID NO: 7657 - protein, 21 aa, Homo sapiens
MFTGDGVSPRWPGWFLTPDLK

SEQ ID NO: 7658 - protein, 13 aa, Homo sapiens
MFTNKVWNSCWPM

SEQ ID NO: 7659 - protein, 46 aa, Homo sapiens
MFTRSPFSFRFWVEGRQKFEEFGYFQGPTEFTIFNILISLNVIDIL

SEQ ID NO: 7660 - protein, 50 aa, Homo sapiens
MFVFLLETRFHRVGQAGLGLLTSGDLPASASQSAGITGVSYCARQLTSYF

SEQ ID NO: 7661 - protein, 16 aa, Homo sapiens
MFVKFYMSIILHSISS

SEQ ID NO: 7662 - protein, 22 aa, Homo sapiens
MFVVILFCLFREKLLLKQFCNK

SEQ ID NO: 7663 - protein, 74 aa, Homo sapiens [sequence omitted]

SEQ ID NO: 7664 - protein, 13 aa, Homo sapiens
MGFALLASGVSNS

SEQ ID NO: 7665 - protein, 162 aa, Homo sapiens
MGFCDVGQAGLKLLASSDLPASASQSAGIPGGSHPHLAQAGFFFFFEAKSCSCPQAGVQWRDLGSLQPLPPRFKPFSCLSLPSSWDYRCLPPCLANFLFLVEMGFHHVGQAGLKLLTSRDPPTSTSQSAGIPGMSHRTRPARAVFKRIYPGLLLCSFPKVSI

SEQ ID NO: 7666 - protein, 64 aa, Homo sapiens
MGFCHVGQAGLELLNSGDLPVSASQSVGITSVSHCTQTLLPYSKGQRATACMRVCTTAFCNSHR

SEQ ID NO: 7667 - protein, 78 aa, Homo sapiens
MGFCHVGQAGLELLTSGDLPTLASQSAGITGMSHHAWPILSTYKKFLCSWWINWLHNKIILVQWIDSCQIHPVANYLN

SEQ ID NO: 7668 - protein, 39 aa, Homo sapiens
MGFCHVGQAGLELLTSGDLPTSASQNAGITGVSHWARPT

SEQ ID NO: 7669 - protein, 13 aa, Homo sapiens
MGFCHVGQAGSSS

SEQ ID NO: 7670 - protein, 41 aa, Homo sapiens
MGFCHVGQASLELLTSSNPPTLASQSAGITGMSHHARLFSV

SEQ ID NO: 7671 - protein, 38 aa, Homo sapiens
MGFCYVAWAGLKLLASSDPPASASQSAGIIGMSCCARP

SEQ ID NO: 7672 - protein, 40 aa, Homo sapiens
MGFGHDGQAGKLKHNFTIIPFSTLNNKSRILSVFLSYTHE

SEQ ID NO: 7673 - protein, 16 aa, Homo sapiens
MGFHCVGQDGLDLLTS

SEQ ID NO: 7674 - protein, 16 aa, Homo sapiens
MGFHCVGRAGLELLTS

SEQ ID NO: 7675 - protein, 16 aa, Homo sapiens
MGFHCVSPDGLDLLTS

SEQ ID NO: 7676 - protein, 28 aa, Homo sapiens
MGFHCVSQDGLELLTCPPRPPKVLGLQA

SEQ ID NO: 7677 - protein, 16 aa, Homo sapiens
MGFHCVSQDGLNLLTS

SEQ ID NO: 7678 - protein, 16 aa, Homo sapiens
MGFHHAGQAELELLTS

SEQ ID NO: 7679 - protein, 16 aa, Homo sapiens
MGFHHFGQHGLDLLTS

SEQ ID NO: 7680 - protein, 43 aa, Homo sapiens
MGFHHFGRADLKLLTSSDPPTLWCWDYRREPPCPVSCWLVSFT

SEQ ID NO: 7681 - protein, 43 aa, Homo sapiens
MGFHHGGQAGLKLLTLSDLPTLASYSDGITGLSHHARPEVEFF

SEQ ID NO: 7682 - protein, 41 aa, Homo sapiens
MGFHHIGQAGFKLLTSGDSPASASQSAGITGVSHCAWPINV

SEQ ID NO: 7683 - protein, 16 aa, Homo sapiens
MGFHHIGQAGHELLTL

SEQ ID NO: 7684 - protein, 42 aa, Homo sapiens
MGFHHIGQAGLKLLTSSDPLASASQSAGITGVTHCARPANKF

SEQ ID NO: 7685 - protein, 16 aa, Homo sapiens
MGFHHIGQDDIDLLTL

SEQ ID NO: 7686 - protein, 16 aa, Homo sapiens
MGFHHIGQDGLDLLTP

SEQ ID NO: 7687 - protein, 16 aa, Homo sapiens
MGFHHNSQDGLYLLTS

SEQ ID NO: 7688 - protein, 60 aa, Homo sapiens
MGFHHVAQAGLELLSSGNPPTSASRKHWDYRRAPLRLALTAFSNTIPCSYQRNLFVSFIF

SEQ ID NO: 7689 - protein, 25 aa, Homo sapiens
MGFHHVAQAGLELWTGLDLRFRPDL

SEQ ID NO: 7690 - protein, 59 aa, Homo sapiens
MGFHHVCQAGLELLTSSDLPASASQSVGDYRHEPLHPAISTVLSSGQVSCRMYPTSGFV

SEQ ID NO: 7691 - protein, 61 aa, Homo sapiens
MGFHHVCQASLELLTSSDLPALASQSAGITGVSHRARQHQIFIEGVPPKGTELCLAILISS

SEQ ID NO: 7692 - protein, 29 aa, Homo sapiens
MGFHHVGHAGLELLTSGDLPASGSQVLGL

SEQ ID NO: 7693 - protein, 62 aa, Homo sapiens
MGFHHVGQADLEFLTSGAPPASASQSTGITGVSHRTRPIFCIFNRDRVSSCWPGWPRTSDLR

SEQ ID NO: 7694 - protein, 47 aa, Homo sapiens
MGFHHVGQADLELLTSGDPPTLASQSAGITGVSHHTRPWVGNLNMQQ

SEQ ID NO: 7695 - protein, 16 aa, Homo sapiens
MGFHHVGQADLEVLTL

SEQ ID NO: 7696 - protein, 15 aa, Homo sapiens
MGFHHVGQAGFELMT

SEQ ID NO: 7697 - protein, 70 aa, Homo sapiens
MGFHHVGQAGLDLLTSGDLSASASQSAEITGVSHHIWSDSFFHSRVPNNPVSYDHYYYYTHCTGEETGSQ

SEQ ID NO: 7698 - protein, 89 aa, Homo sapiens
MGFHHVGQAGLELLASSDPPTSASQSTGIIGVRHCARPRTICHKLTFLVLPMHGESEPKPGNCRPRQCRALVHTHPSPSKLRQPWKGEV

SEQ ID NO: 7699 - protein, 44 aa, Homo sapiens
MGFHHVGQAGLELLTPGDPPTTASQSAGITAVSHHAQPRRDFEI

SEQ ID NO: 7700 - protein, 64 aa, Homo sapiens
MGFHHVGQAGLELLTSDLPASASQSARIKGVSQRAQPTQDFFYFCCITFKGAKRKMRFHTHILS

SEQ ID NO: 7701 - protein, 53 aa, Homo sapiens
MGFHHVGQAGLELLTSGDPPASAGGQSAGITGMSHRTRPTCGTFKIDALHSGI

SEQ ID NO: 7702 - protein, 102 aa, Homo sapiens
MGFHHVGQAGLELLTSGDPPASASQSAGIIGMGHCARPQSPVSFLSFSFLFIFRQDLAVLPRLECSDAVIALFSLQLLGSSDPLCLNLLSSWDSQVHTTMPG

SEQ ID NO: 7703 - protein, 42 aa, Homo sapiens
MGFHHVGQAGLELLTSGDPPASASQSAGITDISHCTQPFYTL

SEQ ID NO: 7704 - protein, 42 aa, Homo sapiens
MGFHHVGQAGLELLTSGDPPTLDSQSAGITGVSHHAWPRVAF

SEQ ID NO: 7705 - protein, 31 aa, Homo sapiens
MGFHHVGQAGLELLTSGGPPASASQSAGITA

SEQ ID NO: 7706 - protein, 48 aa, Homo sapiens
MGFHHVGQAGLELLTSGNPPASAFQSLRITGLSHRAQPIPVFKKACDC

SEQ ID NO: 7707 - protein, 60 aa, Homo sapiens
MGFHHVGQAGLELLTSNDVPVSASQNSGITGMSHCVQPAFSKLLPHWFTLKVKAIARISY

SEQ ID NO: 7708 - protein, 87 aa, Homo sapiens
MGFHHVGQAGLELLTSSDPPASASQIAGITGMSHHARPGSQISESTRVGLRVLYPPTTCSHPTRCLSSGLSLIVLGVPVSCLSMAEP

SEQ ID NO: 7709 - protein, 59 aa, Homo sapiens
MGFHHVGQAGLELLTSSDPPTLASQSAGITGVSHHVQPGEGFCNCCCVVESGPFKERVG

SEQ ID NO: 7710 - protein, 15 aa, Homo sapiens
MGFHHVGQAGLELTS

SEQ ID NO: 7711 - protein, 29 aa, Homo sapiens
MGFHHVGQAGLKLLSSGVLLTLTSQKCWD

SEQ ID NO: 7712 - protein, 30 aa, Homo sapiens
MGFHHVGQAGLKLLTSGDLPSLASQSVKLF

SEQ ID NO: 7713 - protein, 60 aa, Homo sapiens
MGFHHVGQAGLKLLTSSDPLPSASQSAGITGVSHHTQQILSSFIREKCTFLCLCFLHFWN

SEQ ID NO: 7714 - protein, 61 aa, Homo sapiens
MGFHHVGQAGLKLLTSSDPPTSLSQSGGITGVSHHTQLYTSLVIKIYRLSFSSPSGMVFCH

SEQ ID NO: 7715 - protein, 39 aa, Homo sapiens
MGFHHVGQAGLKTPELKQSSCLSLPKCWDYRREPLHPAQ

SEQ ID NO: 7716 - protein, 23 aa, Homo sapiens
MGFHHVGQAGQGFFSLEKSLTIV

SEQ ID NO: 7717 - protein, 58 aa, Homo sapiens
MGFHHVGQAGVVELLTLGDPPASASQGARITGMRHRAQSAAYLLNKVNFKNRYFIFWA

SEQ ID NO: 7718 - protein, 92 aa, Homo sapiens
MGFHHVGQASLELLTSSDPPTLASQSASITGMSHHARPLFTEISVTCSPTHLHRREMGPAHGTMCFSCPGTHLEGGREGEKVSKNGPALVLE

SEQ ID NO: 7719 - protein, 38 aa, Homo sapiens
MGFHHVGQASLKLLTSGDPPTLASQSAGITSVSHHTQP

SEQ ID NO: 7720 - protein, 42 aa, Homo sapiens
MGFHHVGQDGLKLLTSGDPPVSASQSAWITGVSHRARPIFNI

SEQ ID NO: 7721 - protein, 16 aa, Homo sapiens
MGFHHVGQDGLNPLTL

SEQ ID NO: 7722 - protein, 16 aa, Homo sapiens
MGFHHVGQDGVDLLTL

SEQ ID NO: 7723 - protein, 67 aa, Homo sapiens
MGFHHVGQPGLELLTSGDPPVSVSQSAGIIGVSHRTQPLLSSCVGFGSDTIHWGGNSGQGLAPVPGI

SEQ ID NO: 7724 - protein, 42 aa, Homo sapiens
MGFHHVGQTGLELPTSGDPPTSASQSAGITGVSHHARPQKCS

SEQ ID NO: 7725 - protein, 48 aa, Homo sapiens
MGFHHVGQTGLKLVTLSDPPASASQSAGITGKSHYAWTFILCNRCFMM

SEQ ID NO: 7726 - protein, 72 aa, Homo sapiens
MGFHHVGQVGLELLTSGNLPISASQTADVSPHTRPHWTLSVPIPLPGAINSEVQYSFSALRMFIVWCGKQKM

SEQ ID NO: 7727 - protein, 32 aa, Homo sapiens
MGFHHVGQVGLELLTSSDLLALVSQSAGITKE

SEQ ID NO: 7728 - protein, 43 aa, Homo sapiens
MGFHHVHQAALELRTSSDPPALASRSAGITDASYRAQFHPSIL

SEQ ID NO: 7729 - protein, 16 aa, Homo sapiens
MGFHHVNQDGLDLLTS

SEQ ID NO: 7730 - protein, 41 aa, Homo sapiens
MGFHHVSQAGLELLTSSDPPASASQSAGITGVSHCAWPIYF

SEQ ID NO: 7731 - protein, 16 aa, Homo sapiens
MGFHHVSQDGLNILTS

SEQ ID NO: 7732 - protein, 16 aa, Homo sapiens
MGFHHVSRDGLDLLTL

SEQ ID NO: 7733 - protein, 16 aa, Homo sapiens
MGFHLPRSPKVLGLQA

SEQ ID NO: 7734 - protein, 43 aa, Homo sapiens
MGFHLVGQACLKFLTSGDPPTSASQSAGITGMSHHTWPKVLLK

SEQ ID NO: 7735 - protein, 86 aa, Homo sapiens [sequence omitted]

SEQ ID NO: 7736 - protein, 13 aa, Homo sapiens
MGFHMLVRLASNS

SEQ ID NO: 7737 - protein, 43 aa, Homo sapiens
MGFHNVGQAALEQLTSVDPQVLTSQSAGIIGMSHHTRPEADPF

SEQ ID NO: 7738 - protein, 16 aa, Homo sapiens
MGFHPVGQAGLELLTS

SEQ ID NO: 7739 - protein, 16 aa, Homo sapiens
MGFHPVSQDGLDLLTS

SEQ ID NO: 7740 - protein, 39 aa, Homo sapiens
MGFHQTAGHAGLELLTSGDMPALASQSAGITGMSHSTWP

SEQ ID NO: 7741 - protein, 58 aa, Homo sapiens
MGFHQVGQTGLELLTSSNPPILASQSAGIIGMSHHARPSILLKMILKHGSLFFKSTFV

SEQ ID NO: 7742 - protein, 32 aa, Homo sapiens
MGFHRISQDGLDLSPDLMIHPLWPPKVLGLHA

SEQ ID NO: 7743 - protein, 46 aa, Homo sapiens
MGFHRVGQAGLELLTSSDLPASASQSARITGLRHQARLSIFLITYK

SEQ ID NO: 7744 - protein, 31 aa, Homo sapiens
MGFHRVGQDGLKLLTSGDLPASPPKVLGLQV

SEQ ID NO: 7745 - protein, 53 aa, Homo sapiens
MGFHRVSQDGLDLLTSWSAHLGLPKCWDYRREPLCLALLYSFKKYLLYFPVMS

SEQ ID NO: 7746 - protein, 16 aa, Homo sapiens
MGFHRVSQDSLDLLTS

SEQ ID NO: 7747 - protein, 50 aa, Homo sapiens
MGFHYFAQASLKLLTSSDPPASASQSAGITGMSHRAQQFFATFCLFLFCF

SEQ ID NO: 7748 - protein, 41 aa, Homo sapiens
MGFHYVGQAGLDLPTSGDPPALASQRVGGLQARATVPGCYS

SEQ ID NO: 7749 - protein, 17 aa, Homo sapiens
MGFHYVGQAGLKTPDLR

SEQ ID NO: 7750 - protein, 31 aa, Homo sapiens
MGFISTDFFFFFFFETEFCSCRPGWSAMAQS

SEQ ID NO: 7751 - protein, 11 aa, Homo sapiens
MGFLHFGQAGL

SEQ ID NO: 7752 - protein, 72 aa, Homo sapiens [sequence omitted]

SEQ ID NO: 7753 - protein, 64 aa, Homo sapiens
MGFLHVGQAGLELLTSGDPCLGLQKCWDYKCEPPRPASWQTLESPRGSPVDLTASKRGGWDSLN

SEQ ID NO: 7754 - protein, 44 aa, Homo sapiens
MGFLHVGQAGLELLTSGHPPASASQSAGITGVSHRTRPAASILI

SEQ ID NO: 7755 - protein, 52 aa, Homo sapiens
MGFLHVGQAGLELPTSGDPPALASQSAGITGVSHCTSAALALSPTAPPPGPA

SEQ ID NO: 7756 - protein, 42 aa, Homo sapiens
MGFLHVGQAGLKFLTSGDPPASASQSAGITGVSHHTWPNMYY

SEQ ID NO: 7757 - protein, 38 aa, Homo sapiens
MGFLHVGQASLKLLTSGDPPASASQSVGITGMIHRAWP

SEQ ID NO: 7758 - protein, 43 aa, Homo sapiens
MGFLHVGRAGLELLTSGDSSASASQSAGITGMSHHAKLVDSLF

SEQ ID NO: 7759 - protein, 21 aa, Homo sapiens
MGFQHFGQAGFKLLTSGLPKC

SEQ ID NO: 7760 - protein, 16 aa, Homo sapiens
MGFQHTGQAGLELLTL

SEQ ID NO: 7761 - protein, 25 aa, Homo sapiens
MGFQHVGQAGLKLLSSSDLLALADL

SEQ ID NO: 7762 - protein, 105 aa, Homo sapiens [sequence omitted]

SEQ ID NO: 7763 - protein, 110 aa, Homo sapiens
MGFQRVSQDGLNLLTRLGLPKCWDYRREPLRLAFPCFQIISLTLRNLAPIFLNRFTSSLNQLSYLLNVAHCWLPPRPEGTGTTWLPLDLSPCPSTQPWSHKAGNSDTSMQ

SEQ ID NO: 7764 - protein, 31 aa, Homo sapiens
MGFRHIGQAGLELLTSGDPPTRPPKVLRLQE

SEQ ID NO: 7765 - protein, 69 aa, Homo sapiens
MGFRHIVQAGLKLLTSGDPPASASQSARTTGLSHCAGLLVSFYPKIVKFFFQEHSRGRAGELRHIAKSD

SEQ ID NO: 7766 - protein, 68 aa, Homo sapiens
MGFRHVASAGPELLSSDDLLALASQSARITGVSHRARLRILKLSFCWFHKFFFLQCAYIPFGIISNER

SEQ ID NO: 7767 - protein, 45 aa, Homo sapiens
MGFRHVGEAGLELLTSGDPPTSASQSARITGMSHRNRPKQALPRQ

SEQ ID NO: 7768 - protein, 51 aa, Homo sapiens
MGFRHVGQAGLELLASSDSPASASQSAGITRREPPCQATSVFFTLDIWKGL

SEQ ID NO: 7769 - protein, 21 aa, Homo sapiens
MGFRHVGQAGLELLTSGDLPA

SEQ ID NO: 7770 - protein, 37 aa, Homo sapiens
MGFRHVGQAGLEPLTSGDPPVSASQSAGITGVSHYTR

SEQ ID NO: 7771 - protein, 46 aa, Homo sapiens
MGFRHVGQAGLKCLTLGHPAALASQSAGITGMSHRAQPVNSTFYRI

SEQ ID NO: 7772 - protein, 43 aa, Homo sapiens
MGFRHVGQAGRELPTSGDPPASDHPKCWDYRHEPLCLARIMFL

SEQ ID NO: 7773 - protein, 50 aa, Homo sapiens
MGFRHVSQAGLELLTSGDPPTLASQSAGITGVSHCARPESLFLCCRPVCR

SEQ ID NO: 7774 - protein, 17 aa, Homo sapiens
MGFRHVWSGWSQTPDLR

SEQ ID NO: 7775 - protein, 47 aa, Homo sapiens
MGFRQGSSDSPASASRVAGTTGTHHHTQLIFCIFSRDGVLPCCPGWS

SEQ ID NO: 7776 - protein, 13 aa, Homo sapiens
MGFTMLARLVLNS

SEQ ID NO: 7777 - protein, 145 aa, Homo sapiens [sequence omitted]

SEQ ID NO: 7778 - protein, 43 aa, Homo sapiens
MGFYHVVQASLELLISSDPPASQRAGIDSMSHHARPCSTNFNT

SEQ ID NO: 7779 - protein, 17 aa, Homo sapiens
MGGEQALSLQGLWSVSF

SEQ ID NO: 7780 - protein, 25 aa, Homo sapiens
MGGFSPALTSSQVYTLASLTAPHSW

SEQ ID NO: 7781 - protein, 20 aa, Homo sapiens
MGKMYGNFHLIAQVQDNPAH

SEQ ID NO: 7782 - protein, 17 aa, Homo sapiens
MGLEALTCPRHRWVPGR

SEQ ID NO: 7783 - protein, 293 aa, Homo sapiens
MGLIVLWDGVIAAVTQVGPDDVLLGEAEDPQAATPHGCVQDHVAVGHQLRALIESHPDVAHLGPVLQEPTIGLLVLPTHVSRVLPQQPHLGLCVSCMPQSVPQLFPGACGRLHSLELDARLGHSTEGVRLPIRLLHLLPHDHVEAGAVLVAKDEARIVVIRDRVHMERALEVHAIEGSVTHSQAWVAVHCLHDLPSLVEHHPVGVNLRVTLRVQHDCLEGPEVGERDFSVLRTHVDLVYHLVCIKVVLAHVAHAVPVRVLLAGVRHQAAVVPTVRDSVIVVVVVAGITLAIVV

SEQ ID NO: 7784 - protein, 12 aa, Homo sapiens
MGNQGLLYMFGR

SEQ ID NO: 7785 - protein, 38 aa, Homo sapiens
MGPQAGLLQPGTAPPTPAQRRLLLAGDDSLRAPNTIPT

SEQ ID NO: 7786 - protein, 32 aa, Homo sapiens
MGRPLILMYQKYILKSKGRNNLIQFLNSLPLK

SEQ ID NO: 7787 - protein, 35 aa, Homo sapiens
MGSFQPLFQHFFSYWYNQSSQELPPQIVIGFKWKH

SEQ ID NO: 7788 - protein, 36 aa, Homo sapiens
MGSHHIAQAGLELPGPRDPTTTASQSAGITGLRHYV

SEQ ID NO: 7789 - protein, 24 aa, Homo sapiens
MGSLGCLLPLRWTLDSAATIIQQL

SEQ ID NO: 7790 - protein, 35 aa, Homo sapiens
MGSNSTQELLHSKRNYHQSEQATYKMAENFRNLLI

SEQ ID NO: 7791 - protein, 59 aa, Homo sapiens
MGSRHVAKASLELLSSSDLTTSASQSAGITGMNHGAWPLMKIMIQDYRISYSASAAWVS

SEQ ID NO: 7792 - protein, 35 aa, Homo sapiens
MGSSRQSRREGKKKHIKIAFMNLSQSVNIMAQELQ

SEQ ID NO: 7793 - protein, 17 aa, Homo sapiens
MGVLPCWPGWSRTPDLR

SEQ ID NO: 7794 - protein, 18 aa, Homo sapiens
MGVQYSIMLWTTVWRFLN

SEQ ID NO: 7795 - protein, 11 aa, Homo sapiens
MGVSPCWPGWS

SEQ ID NO: 7796 - protein, 15 aa, Homo sapiens
MHAHAHIYTYTHICM

SEQ ID NO: 7797 - protein, 18 aa, Homo sapiens
MHFQLRDFKSTIEINVSV

SEQ ID NO: 7798 - protein, 24 aa, Homo sapiens
MHHCAWLIFCIFFRRHGVSPCWPG

SEQ ID NO: 7799 - protein, 14 aa, Homo sapiens
MHHCTGKNFLNDIK

SEQ ID NO: 7800 - protein, 30 aa, Homo sapiens
MHHHAQIIFVFLVKKGFHHVGQDSLHLLTS

SEQ ID NO: 7801 - protein, 34 aa, Homo sapiens
MHHHAQLIFAFLVDTRFCHVGQDDCLFFIVCLSH

SEQ ID NO: 7802 - protein, 13 aa, Homo sapiens
MHHHAQLIFLYFY

SEQ ID NO: 7803 - protein, 12 aa, Homo sapiens
MHHHAQLILYIQ

SEQ ID NO: 7804 - protein, 11 aa, Homo sapiens
MHHHAQVILYF

SEQ ID NO: 7805 - protein, 30 aa, Homo sapiens
MHHHAWLGDIGFAYHSFPVMRYSFKKVDFS

SEQ ID NO: 7806 - protein, 30 aa, Homo sapiens
MHHHAWLIFVFLIEMGFQHTGQAGLELLTL

SEQ ID NO: 7807 - protein, 15 aa, Homo sapiens
MHHHAWLIFVFLVEM

SEQ ID NO: 7808 - protein, 63 aa, Homo sapiens
MHHHAWLIFVFLVEMEFHHVGQAGLKLLTLSDLSLSNCWDYRREPPRPASIICLSFASLSPSF

SEQ ID NO: 7809 - protein, 54 aa, Homo sapiens
MHHHPQLIFVFLVEGVSLCWPVWSRTPDLVICLPRPPKVLGLRCEPLCPVSFFT

SEQ ID NO: 7810 - protein, 24 aa, Homo sapiens
MHHHTQLIFCIFTTDHISSWLGWS

SEQ ID NO: 7811 - protein, 25 aa, Homo sapiens
MHHHTQLIFVFLVEKGFHHVDQAGL

SEQ ID NO: 7812 - protein, 30 aa, Homo sapiens
MHHHTQLIFVFLVETGFHHVGQDGLDLLTS

SEQ ID NO: 7813 - protein, 55 aa, Homo sapiens
MHHHTQLIFVFLVQMGFHYVGQAGLDLPTSGDPPALASQRVGGLQARATVPGCYS

SEQ ID NO: 7814 - protein, 11 aa, Homo sapiens
MHHHTQLILYF

SEQ ID NO: 7815 - protein, 12 aa, Homo sapiens
MHHHTRLIFLYF

SEQ ID NO: 7816 - protein, 23 aa, Homo sapiens
MHHHTRLIFLYFSRDGVSLCWPG

SEQ ID NO: 7817 - protein, 29 aa, Homo sapiens [sequence omitted]

SEQ ID NO: 7818 - protein, 75 aa, Homo sapiens
MHHHTWLIFVFLEKIGFYHVGQASLELLTSSDSPTSASQRAGITGMSLCTQHIIVIIILRQGLAVYPGWNALVWS

SEQ ID NO: 7819 - protein, 67 aa, Homo sapiens
MHHHVRLIFVFLVETRFHHVGQAGLELLTSGDPPASASQSAGITGVCHHAQPLSEFFLVKHQILFHR

SEQ ID NO: 7820 - protein, 56 aa, Homo sapiens
MHHHVRLIFVFLVETVFCHVGQAGLKLLTSGDVPASASQSAGNTGVSYCAQPLTFL

SEQ ID NO: 7821 - protein, 88 aa, Homo sapiens
MHHNARLIFCIFFFFFERESRSVARLECSGVISAHCNLHLLGSSDSPASASLVVGTTGMRHHAQLIFVFLIETGFHHVGQDGLDLLTL

SEQ ID NO: 7822 - protein, 31 aa, Homo sapiens
MHHNAWLLFCIFSRDGILPCWPGWSQTPDLR

SEQ ID NO: 7823 - protein, 53 aa, Homo sapiens
MHHNTQLIFVYLVETGFHHVGQAGPELLTSSDPSTQASQSAGITGMSHRTWPR

SEQ ID NO: 7824 - protein, 58 aa, Homo sapiens [sequence omitted]

SEQ ID NO: 7825 - protein, 23 aa, Homo sapiens
MHLLSFVAGFCNLAYCLQGSSTL

SEQ ID NO: 7826 - protein, 39 aa, Homo sapiens
MHMHTYIHTHIYACDNINNEKFYSGYLQRSEIRPIINLN

SEQ ID NO: 7827 - protein, 11 aa, Homo sapiens
MHMITYYKYVI

SEQ ID NO: 7828 - protein, 30 aa, Homo sapiens
MHNLTVQKNCVIFTWLAHGKNKLYTRIQNS

SEQ ID NO: 7829 - protein, 24 aa, Homo sapiens
MHPLCFILKDVSTPKMHYLVITCT

SEQ ID NO: 7830 - protein, 37 aa, Homo sapiens
MHTYIHTHIYACDNINNEKFYSGYLQRSEIRPIINLN

SEQ ID NO: 7831 - protein, 12 aa, Homo sapiens
MHYHAQLIFVFF

SEQ ID NO: 7832 - protein, 70 aa, Homo sapiens
MHYHAQLIFVFLVEKGFRHVGQAGLELLTSGDPPASASQSARVTGKKLCYFLNLPCSDIGYQGDFLGNLI

SEQ ID NO: 7833 - protein, 15 aa, Homo sapiens
MICLPQPPKVLGLLV

SEQ ID NO: 7834 - protein, 13 aa, Homo sapiens
MICPLWLPKVLGL

SEQ ID NO: 7835 - protein, 13 aa, Homo sapiens
MICPPQPLNMLGL

SEQ ID NO: 7836 - protein, 23 aa, Homo sapiens
MICPPQPPKMLGLQALATAPSHI

SEQ ID NO: 7837 - protein, 15 aa, Homo sapiens
MICPPRLPKVLGLQA

SEQ ID NO: 7838 - protein, 27 aa, Homo sapiens
MICPPRPPKVLGLQASATTPSYLSLFF

SEQ ID NO: 7839 - protein, 15 aa, Homo sapiens
MICPPWPPKVLELQV

SEQ ID NO: 7840 - protein, 15 aa, Homo sapiens
MICPSRPPKVLGLQA

SEQ ID NO: 7841 - protein, 15 aa, Homo sapiens
MICSPWPPKVLGLQA

SEQ ID NO: 7842 - protein, 12 aa, Homo sapiens
MIDFLTCRLLWG

SEQ ID NO: 7843 - protein, 15 aa, Homo sapiens
MIHLLRPPKVLGLQA

SEQ ID NO: 7844 - protein, 15 aa, Homo sapiens
MIHLPGPPKVLGLQV

SEQ ID NO: 7845 - protein, 15 aa, Homo sapiens
MIHLPQPPKVLGLQA

SEQ ID NO: 7846 - protein, 15 aa, Homo sapiens
MIHLPWPPKVLELQA

SEQ ID NO: 7847 - protein, 11 aa, Homo sapiens
MIHLTQPPKVL

SEQ ID NO: 7848 - protein, 15 aa, Homo sapiens
MIHPLWPPKVLGLHA

SEQ ID NO: 7849 - protein, 15 aa, Homo sapiens
MIHPPQPPEVLGLQA

SEQ ID NO: 7850 - protein, 15 aa, Homo sapiens
MIHPPQPPKVLGLQV

SEQ ID NO: 7851 - protein, 15 aa, Homo sapiens
MIHPPRPPKVLGLQV

SEQ ID NO: 7852 - protein, 15 aa, Homo sapiens
MIHPPWPPKVLGLQG

SEQ ID NO: 7853 - protein, 25 aa, Homo sapiens
MIHPPWPPKVLGSTAPGLFWLVLKR

SEQ ID NO: 7854 - protein, 15 aa, Homo sapiens
MIHPPWPPKVLRLQA

SEQ ID NO: 7855 - protein, 15 aa, Homo sapiens
MIHPSRPPKMLGLQV

SEQ ID NO: 7856 - protein, 12 aa, Homo sapiens
MIHPSRPPKVLG

SEQ ID NO: 7857 - protein, 15 aa, Homo sapiens
MIHQPRPPQVLGLQV

SEQ ID NO: 7858 - protein, 13 aa, Homo sapiens
MIKNHFGERVSNC

SEQ ID NO: 7859 - protein, 20 aa, Homo sapiens
MILIVPLQTAAMPPPSPVHF

SEQ ID NO: 7860 - protein, 15 aa, Homo sapiens
MILPPQNPKVLGLQA

SEQ ID NO: 7861 - protein, 14 aa, Homo sapiens
MIMRVPLRHTAGTD

SEQ ID NO: 7862 - protein, 12 aa, Homo sapiens
MINCIMRLLAHS

SEQ ID NO: 7863 - protein, 32 aa, Homo sapiens
MIRLPRSPKVLDYRREPPRPAPNLGFLSPGSL

SEQ ID NO: 7864 - protein, 13 aa, Homo sapiens
MIRPPRPPKVLGL

SEQ ID NO: 7865 - protein, 15 aa, Homo sapiens
MIRPPWPPKVLGLQE

SEQ ID NO: 7866 - protein, 15 aa, Homo sapiens
MIRPSRPPKVLGLQA

SEQ ID NO: 7867 - protein, 15 aa, Homo sapiens
MIRSPQPPKVLGLQV

SEQ ID NO: 7868 - protein, 96 aa, Homo sapiens
MISAHCNLCLLGSSDPPASASQVAEVIGAHHHAQLIFFFFFFETEPRSFAQARVQWRDLGSLQALPPRFTPFSCLSLPSSWYYRCPPPSPANFCIF

SEQ ID NO: 7869 - protein, 25 aa, Homo sapiens
MISKMQLYCSSHQFHSERIFCCLPF

SEQ ID NO: 7870 - protein, 16 aa, Homo sapiens
MITGSVPKPPSPSKKA

SEQ ID NO: 7871 - protein, 11 aa, Homo sapiens
MITMMIMMTVP

SEQ ID NO: 7872 - protein, 31 aa, Homo sapiens
MKCLKKCPYEMGTFGDRCTHRKNPREVRGRD

SEQ ID NO: 7873 - protein, 30 aa, Homo sapiens
MKEKLEILPISAIKTIKLVCLLFLTKCSYR

SEQ ID NO: 7874 - protein, 24 aa, Homo sapiens
MKFHHVGLAGLKLLTSSDLPALVS

SEQ ID NO: 7875 - protein, 83 aa, Homo sapiens
MKIENDLALFYVYCHLCKICIPCNLLEFFPAFLIHWIPWSPWNLPVLYFFLFYGDQCHAEGQQSHTLIFYLPPSCSIAFSNTI

SEQ ID NO: 7876 - protein, 25 aa, Homo sapiens
MKKDIRNYSVNLQVENYLFSHSHRN

SEQ ID NO: 7877 - protein, 16 aa, Homo sapiens
MKKIILPFFNVHSDHH

SEQ ID NO: 7878 - protein, 42 aa, Homo sapiens
MKKQTSSLNTGVFLSRKSLASSTITGSSVSSSKTCRVATAAW

SEQ ID NO: 7879 - protein, 43 aa, Homo sapiens
MKLAQNLISEIFMFHFSQRNKIHSDPIIIESQKKPLRAFALLN

SEQ ID NO: 7880 - protein, 70 aa, Homo sapiens [sequence omitted]

SEQ ID NO: 7881 - protein, 17 aa, Homo sapiens
MKNLAIASHVTDSQGQK

SEQ ID NO: 7882 - protein, 24 aa, Homo sapiens
MKRASAMAHTCNPSTLGGQDRRTA

SEQ ID NO: 7883 - protein, 13 aa, Homo sapiens
MKSFIQATCKGLR

SEQ ID NO: 7884 - protein, 25 aa, Homo sapiens
MKSIRQSSQIAPEKLNLNSTLQVSP

SEQ ID NO: 7885 - protein, 47 aa, Homo sapiens
MKWDLFNHCFSIFSLIGTIRVPKNYLPKLLLVLNGNTDEFNTQRTKE

SEQ ID NO: 7886 - protein, 40 aa, Homo sapiens
MLAERVQGLCESNGPRTFSTAIALCSGASRTHLFWSIPDP

SEQ ID NO: 7887 - protein, 20 aa, Homo sapiens
MLAGVRGQCAHSKFCSFEHC

SEQ ID NO: 7888 - protein, 87 aa, Homo sapiens
MLAHQLCHVLNLLSQNLDHLVLLCHLQFEGLTFCLHISEMIPFIFQVLQLLQFQVHPGAELCDLCIGSLDGSLFFLERSCQVRYCPL

SEQ ID NO: 7889 - protein, 66 aa, Homo sapiens
MLAKMVSNSWPRDLPVSASQSAGITGVNHHAQPRSQPFFGSGSNSRAMTLVVETGLCSNKCHHPGH

SEQ ID NO: 7890 - protein, 27 aa, Homo sapiens
MLAKQVSNYQPQGIRPPRPPKVLGLQA

SEQ ID NO: 7891 - protein, 12 aa, Homo sapiens
MLARLARAPDLR

SEQ ID NO: 7892 - protein, 48 aa, Homo sapiens [sequence omitted]

SEQ ID NO: 7893 - protein, 27 aa, Homo sapiens
MLARLILNSGPQAICPPRPPKVLGLQV

SEQ ID NO: 7894 - protein, 27 aa, Homo sapiens
MLARLISNSRPQVIRPPRPPKVLGLWA

SEQ ID NO: 7895 - protein, 27 aa, Homo sapiens
MLARLMQLLTEAWGASVLPSPPAKSTR

SEQ ID NO: 7896 - protein, 63 aa, Homo sapiens
MLARLVANSRPQVIRLPQITQSAGITGMSHCAWPGSCFFKPHMIPRRHHNRVGFIIFLILGYA

SEQ ID NO: 7897 - protein, 36 aa, Homo sapiens
MLARLVLNSCPCDLPASASQSAGITGVSHCTQSKIF

SEQ ID NO: 7898 - protein, 73 aa, Homo sapiens
MLARLVLNSCPLRPPKVLESQACATAPSQPLFFFFFFLDFLCGTIIECSRFISYFSIPGAIITLLLSMSSKLV

SEQ ID NO: 7899 - protein, 25 aa, Homo sapiens
MLARLVLNSRPQVILPPRPPKVLGL

SEQ ID NO: 7900 - protein, 64 aa, Homo sapiens
MLARLVLNSRPQVIRPPRPPKVLGLQASRGKGKFSSLIHLFKGWCTQAGLDQLAGPHHLLQCHF

SEQ ID NO: 7901 - protein, 40 aa, Homo sapiens
MLARLVLNSWPQVILLPQPPKVLGLLGVSRHARPLVFSLL

SEQ ID NO: 7902 - protein, 27 aa, Homo sapiens
MLARLVLNSWPWVIHLLWPPKVLGLQA

SEQ ID NO: 7903 - protein, 15 aa, Homo sapiens
MLARLVLRQKQKIMQ

SEQ ID NO: 7904 - protein, 27 aa, Homo sapiens
MLARLVSDSWPPAIRPLRPPQVLGLQA

SEQ ID NO: 7905 - protein, 42 aa, Homo sapiens
MLARLVSKLLTSGDPPALASKSAGITGLSHCTRPGIYNSFTG

SEQ ID NO: 7906 - protein, 27 aa, Homo sapiens
MLARLVSNFSPQVFCLPRPPKVLGLQA

SEQ ID NO: 7907 - protein, 27 aa, Homo sapiens
MLARLVSNFWPQVIHQPQPPKVLGLQV

SEQ ID NO: 7908 - protein, 50 aa, Homo sapiens [sequence omitted]

SEQ ID NO: 7909 - protein, 27 aa, Homo sapiens
MLARLVSNSLPQVICSSWPPKVLELQA

SEQ ID NO: 7910 - protein, 27 aa, Homo sapiens
MLARLVSNSRPQVIHPPQPPKVLGLQV

SEQ ID NO: 7911 - protein, 55 aa, Homo sapiens
MLARLVSNSSASQSAGITGMGYRAWPRYTYFVLFLFSRDRVSPCWPGWSQTPDLK

SEQ ID NO: 7912 - protein, 27 aa, Homo sapiens
MLARLVSNSSSQVIHPVLPPKVLGLQA

SEQ ID NO: 7913 - protein, 27 aa, Homo sapiens
MLARLVSNSWPQLIRPPQPPKVLGLQA

SEQ ID NO: 7914 - protein, 95 aa, Homo sapiens
MLARLVSNSWPQVICPPQPPKVLGFQAGATHTWLKLGFFFFLRRSLALVPRPECNGAISAHCNLCLPGSSHSPASASQVAGITGACHHAWLIFYF

SEQ ID NO: 7915 - protein, 17 aa, Homo sapiens
MLARLVSNSWPQVIHLP

SEQ ID NO: 7916 - protein, 25 aa, Homo sapiens
MLARLVSNSWPQVIHPPQPPKVQGL

SEQ ID NO: 7917 - protein, 17 aa, Homo sapiens
MLARLVSNSWPQVILPP

SEQ ID NO: 7918 - protein, 27 aa, Homo sapiens
MLARLVSNSWSQVIRPPRPPKVLGLQA

SEQ ID NO: 7919 - protein, 36 aa, Homo sapiens
MLARLVSNWPHDLTASASQSAGITGVSHHAWPCSFF

SEQ ID NO: 7920 - protein, 49 aa, Homo sapiens
MLARLVSRLLTSSDLLTLASQSAGITGVSHRAWLILQLFENLLCIDFVA

SEQ ID NO: 7921 - protein, 57 aa, Homo sapiens [sequence omitted]

SEQ ID NO: 7922 - protein, 100 aa, Homo sapiens [sequence omitted]

SEQ ID NO: 7923 - protein, 17 aa, Homo sapiens
MLARLVWNSGPQVIRLP

SEQ ID NO: 7924 - protein, 18 aa, Homo sapiens
MLARMTVYSLLSVFLIRV

SEQ ID NO: 7925 - protein, 27 aa, Homo sapiens
MLARMVLISWPQMIHPPWPPKVLRLQA

SEQ ID NO: 7926 - protein, 19 aa, Homo sapiens
MLARMVSISGQSLFCKYPW

SEQ ID NO: 7927 - protein, 165 aa, Homo sapiens [sequence omitted]

SEQ ID NO: 7928 - protein, 49 aa, Homo sapiens
MLARMVSISRPRDLPFSASQSAGITGVSHRARPSCPLNQTVLLPLENVH

SEQ ID NO: 7929 - protein, 11 aa, Homo sapiens
MLARMVSISTS

SEQ ID NO: 7930 - protein, 17 aa, Homo sapiens
MLARQVSNSWPQMICPP

SEQ ID NO: 7931 - protein, 67 aa, Homo sapiens
MLASGISGLVVIMVFEITVAVMQFRNLSKFILTSEANITVSRGIQLCASRMDSLSQHVIAKDDSVSS

SEQ ID NO: 7932 - protein, 12 aa, Homo sapiens
MLASWSRTPDLR

SEQ ID NO: 7933 - protein, 27 aa, Homo sapiens
MLAWLVSNSGHQVIHPPQPPKMLGLQA

SEQ ID NO: 7934 - protein, 21 aa, Homo sapiens
MLCKYITAVHHSTPIGAMPQH

SEQ ID NO: 7935 - protein, 27 aa, Homo sapiens
MLCRLVSNSWAPAIHPPQPPKVLGLQA

SEQ ID NO: 7936 - protein, 34 aa, Homo sapiens
MLCSFVVQMWVLEVSRKLLGHLGCRHFPAASPHA

SEQ ID NO: 7937 - protein, 62 aa, Homo sapiens
MLEFVLQLAQTLDAALAAPPLPLPESHVRLRVGAGAAVVPVGGRSSGRSLSLAGCSVGLMTA

SEQ ID NO: 7938 - protein, 25 aa, Homo sapiens
MLEVASVFKFACFFFQLFFSCPKYG

SEQ ID NO: 7939 - protein, 70 aa, Homo sapiens
MLEVGLELLTSGDPPTLASQSAGIIGLSYSARPTSAFYTLSALSCKMIHYLVFLVSTVKGKYLGPPKSLS

SEQ ID NO: 7940 - protein, 15 aa, Homo sapiens
MLFHAEVTDNTCFLR

SEQ ID NO: 7941 - protein, 12 aa, Homo sapiens
MLGRVYRPCWQV

SEQ ID NO: 7942 - protein, 13 aa, Homo sapiens
MLHIHQLTLFGLY

SEQ ID NO: 7943 - protein, 45 aa, Homo sapiens
MLHIHQLTLFGPLAAFTLNLNLLNASSVSKLHLTNSYKACSLSFM

SEQ ID NO: 7944 - protein, 119 aa, Homo sapiens
MLIDVSCLPVPLVWGAHASSGPARPGLVPGSRPSAPPPAPVAPALSPAAWQQPDFLPCSDPESGPLTFGSGPFQCHHSGAASPGPAAPDHAPGSAPFPLPGTAVACTFQCPAGIGPPVP

SEQ ID NO: 7945 - protein, 15 aa, Homo sapiens
MLIFCIFSRDGVSLC

SEQ ID NO: 7946 - protein, 17 aa, Homo sapiens
MLIHHSTDNISGFSIQL

SEQ ID NO: 7947 - protein, 24 aa, Homo sapiens
MLIIVISNDRIRSNFHFLYFFVRL

SEQ ID NO: 7948 - protein, 27 aa, Homo sapiens
MLIRLVSNSPPQVIRLPWPPKVVGLQA

SEQ ID NO: 7949 - protein, 27 aa, Homo sapiens
MLITLVSNSQPQVIHPPWPPKVLGLQA

SEQ ID NO: 7950 - protein, 20 aa, Homo sapiens
MLIYYCKIVSLAKSEGNRTF

SEQ ID NO: 7951 - protein, 87 aa, Homo sapiens
MLKRMKIENDLALFYVYCHLCKICIPCNLLEFFPAFLIHWIPWSPWNLPVLYFFLFYGDQCHAEGQQSHTLIFYLPPSCSIAFSNTI

SEQ ID NO: 7952 - protein, 663 aa, Homo sapiens
MLKTLNKSGIDGTYLKIIRAIYDKPTANIILNGQKLEAFPLKTGTRQGCPLSPLLFNIVLEVLARAIRQEKEVKSIQLGKEEVKLSLFADDMIVYLENPIVSAQNLLKLISNFSKVSGYKINVQKSQAFLYTNNRQTESQIMSELPFTIASKRTKYLGIQLTRDVKDLFKENYKPLLNEIKEDTNKWKNIPCSWIGRINIVKMAILPKVIYRFNAIPIKLPMTFFTELEKTTLKFIWNQKRARIAKSILSQKNKAGGIMLPDFKLYYKATITKTAWYWYQNRDIDQWNTKEPSEITPHVYSYLIFDKPEKNKQWGKDSLLNKWCWENWLAICRKLKLDPFLTPYTKIISRWIKDLHVRPKTIKTLEENLGITIQDIGMGKDFMSKTPKAMATKDKIDKWDLIQLKSFCTAKETTIRVNRQLTKWQKIFATYSSDKGLISRIYNELKQIYKKKTNNPIKKWAKDMNRHFSKEDIYAAKKHMKKCSPSLTIREMQIKTTMRYHLTPVRMAIIKKSGNNRCWRGCGEIGTLLHCWWDCKLVQPLWKSVWRFLRNLELEIPFDPAIPLLGIYSKDYKSCCYKDTCTRMFIAALFTIAKTWNQPKCPTMIDWIKKMWHIYTMEYYAAIKKDEFMSFVGTWMKLEIIILSKLSQGQKTKHHMFSLIDGN

SEQ ID NO: 7953 - protein, 55 aa, Homo sapiens
MLKTLTKLKYINIIYISARRMAKIHILFSRLFFPKISLLLTQKENHLLIFNLPPE

SEQ ID NO: 7954 - protein, 16 aa, Homo sapiens
MLLDYPKLQETSSQSG

SEQ ID NO: 7955 - protein, 51 aa, Homo sapiens
MLLQMTHSTHALIVFCFFFHLRSIAFHFIYQTVFTVDRHCSSHVPYGFVLS

SEQ ID NO: 7956 - protein, 51 aa, Homo sapiens
MLLQMTHSTHALIVFCFSFHLRSIAFHFIYQTVFTVDRHCSSHVPYGFVLS

SEQ ID NO: 7957 - protein, 34 aa, Homo sapiens
MLLRLVLNSCTQVICLPWPPKVLELQASCFFIFK

SEQ ID NO: 7958 - protein, 32 aa, Homo sapiens
MLLRLVSNSWAQAIHLPWLPKVLGLQAPAPDL

SEQ ID NO: 7959 - protein, 30 aa, Homo sapiens
MLLRPANLCIFIRDGVSPYWPGWSQTPDLK

SEQ ID NO: 7960 - protein, 51 aa, Homo sapiens
MLPCLANFCIFYFFGDGVLLHHPGWSAEARSWLTATSASWVQAIILPQPPK

SEQ ID NO: 7961 - protein, 30 aa, Homo sapiens
MLPCQANFYIFIRDGVLPCWPGRSRTPGLR

SEQ ID NO: 7962 - protein, 28 aa, Homo sapiens
MLPEKHLSMSCWDRATCALSFTSSSCSV

SEQ ID NO: 7963 - protein, 25 aa, Homo sapiens
MLPGLVSNSWPQVIRPPQPPKVLGL

SEQ ID NO: 7964 - protein, 27 aa, Homo sapiens
MLPKLVSNSWTQAISPSWLPKVLGLQV

SEQ ID NO: 7965 - protein, 18 aa, Homo sapiens
MLPPLLVNFCIFSRDGIL

SEQ ID NO: 7966 - protein, 27 aa, Homo sapiens
MLPRLFSNSWAQAMRPPQPPKVLGLQV

SEQ ID NO: 7967 - protein, 14 aa, Homo sapiens
MLPRLVLNSGLVWT

SEQ ID NO: 7968 - protein, 61 aa, Homo sapiens
MLPRLVLNSWSQAILPLQPSKVLGVQAQATVPSCQTLSFNYAPNSSPQILFTKAPGWSSPS

SEQ ID NO: 7969 - protein, 63 aa, Homo sapiens
MLPRPANFLYFIRDEVSLCCPGWFRTPELRQSARLSLPKCWDYRREPPCPTNCMQFLKDLTYI

SEQ ID NO: 7970 - protein, 43 aa, Homo sapiens
MLPRVDKNVEQLEFSYISGRNVKLYSHFGKHLVAFKAKYIPTI

SEQ ID NO: 7971 - protein, 74 aa, Homo sapiens
MLPSASNICRLYLLIVSCRNCSSSGKGEMLRIYRIWRGFGTSGNFLCTAAWKRCRRAVQSLPPLKPTQSWVRLY

SEQ ID NO: 7972 - protein, 27 aa, Homo sapiens
MLPSLVLNFWAHTILLPWPPKVLGLQA

SEQ ID NO: 7973 - protein, 69 aa, Homo sapiens
MLPTYLTQVVFFLQVCKVWMGFLKTSRGSARSNYCHNITKMLFAFPRHSLRSIWWGLPKATMTCGLSAD

SEQ ID NO: 7974 - protein, 84 aa, Homo sapiens
MLRSKSQGFQRSFNQCFLKVPTVLGSAGGGGGGSRSSCAELGLAGREVKGSGRLSTGTSHRIQPGNYSSGEVTAARCALQREAG

SEQ ID NO: 7975 - protein, 64 aa, Homo sapiens
MLRTPPDKQTGFQAEGPLDLREGSGSAGPCRFARREPGGRPASHPHPTPAPWGLPILDTLVPER

SEQ ID NO: 7976 - protein, 63 aa, Homo sapiens
MLSLVFLWKVLIQLDNLRLLLLIQEAETHSPERSILLHSRSSLLGLNLQNPFQQYWYQWCLLK

SEQ ID NO: 7977 - protein, 22 aa, Homo sapiens
MLSMQILTKLFEQTALQLLDML

SEQ ID NO: 7978 - protein, 27 aa, Homo sapiens
MLSRLVLNSSAQMICPPRLPKVLGLQA

SEQ ID NO: 7979 - protein, 15 aa, Homo sapiens
MLSSLRSWASGGSSS

SEQ ID NO: 7980 - protein, 11 aa, Homo sapiens
MLSSSRESRFL

SEQ ID NO: 7981 - protein, 25 aa, Homo sapiens
MLTRMFSISRPQVIHLPQPPKVLGL

SEQ ID NO: 7982 - protein, 14 aa, Homo sapiens
MLVGQAGLELLTSA

SEQ ID NO: 7983 - protein, 27 aa, Homo sapiens
MLVKLVSNSRPQVICPLRPPKVLGLQA

SEQ ID NO: 7984 - protein, 20 aa, Homo sapiens
MLVKMWKKGELLHTLGGNVN

SEQ ID NO: 7985 - protein, 54 aa, Homo sapiens
MLVRLDKAFFLWRNHSRSYEFASKTSKFNVLMQGLVRLKIHITSLIVKSLASYY

SEQ ID NO: 7986 - protein, 35 aa, Homo sapiens
MLVRLFLNSRPQMICPPQPPKMLGLQALATAPSHI

SEQ ID NO: 7987 - protein, 191 aa, Homo sapiens
MLVRLVLKLLNSNSPPASASQSVGITGVSHCTQPSDYMLKKVLGSHDMGLSIESAWQTGGARQMPAPSSPPQARLQCQLRDSGFATYAQSFWLAKLRLLETLAFELSRLLPRCSFLICLTTAVALNACLHLLLAKFFRIWALTDSWMFLLRAVSPAIHGCRAACSHVYLLFGSFSIRFRMKSFAESEMSSQ

SEQ ID NO: 7988 - protein, 27 aa, Homo sapiens
MLVRLVLNSGPQVIRPPWPPKMLGLQA

SEQ ID NO: 7989 - protein, 27 aa, Homo sapiens
MLVRLVLNSRPQVIHLPWPPKVLGLQA

SEQ ID NO: 7990 - protein, 27 aa, Homo sapiens
MLVRLVLNSRPQVIRLPRPPKVLGLQA

SEQ ID NO: 7991 - protein, 27 aa, Homo sapiens
MLVRLVLNSRPQVIYPPLPPKVLGLQA

SEQ ID NO: 7992 - protein, 27 aa, Homo sapiens
MLVRLVLNSWPQVIHPPRPPKVLGLQA

SEQ ID NO: 7993 - protein, 27 aa, Homo sapiens
MLVRLVSNPRPQVIHPPWPHRMLRLQA

SEQ ID NO: 7994 - protein, 27 aa, Homo sapiens
MLVRLVSNSQPQVIHPPRTPKVLGLQA

SEQ ID NO: 7995 - protein, 35 aa, Homo sapiens
MLVRLVSNSRPQVICPAHLGLPKCQDYRREPPHPA

SEQ ID NO: 7996 - protein, 25 aa, Homo sapiens
MLVRLVSNSRPQVICPPGPPKVLGL

SEQ ID NO: 7997 - protein, 27 aa, Homo sapiens
MLVRLVSNSRTQVICPPRPPKVLGLQA

SEQ ID NO: 7998 - protein, 30 aa, Homo sapiens
MLVRLVSNSYPQVICLRWQICNPKMLGLQM

SEQ ID NO: 7999 - protein, 27 aa, Homo sapiens
MLVRLVWNSRPQVICPPRPPKVLGLQA

SEQ ID NO: 8000 - protein, 35 aa, Homo sapiens
MLVRMWRKGKPLFTIGRNVNFHSHGREHYGGSSKN

SEQ ID NO: 8001 - protein, 11 aa, Homo sapiens
MLWTTVWRFLN

SEQ ID NO: 8002 - protein, 15 aa, Homo sapiens
MMCPSRPPKILGLQA

SEQ ID NO: 8003 - protein, 32 aa, Homo sapiens
MMDELRSNIIDPSRSETPSAPTGQSRFPRGEA

SEQ ID NO: 8004 - protein, 33 aa, Homo sapiens
MMFSWEKQKTPRRPPRMVVSKTTLLSATSSGPS

SEQ ID NO: 8005 - protein, 15 aa, Homo sapiens
MMIMRVPLRHTAGTD

SEQ ID NO: 8006 - protein, 12 aa, Homo sapiens
MMITMMIMMTVP

SEQ ID NO: 8007 - protein, 70 aa, Homo sapiens
MMLPTYLTQVVFFLQVCKVWMGFLKTSRGSARSNYCHNITKMLFAFPRHSLRSIWWGLPKATMTCGLSAD

SEQ ID NO: 8008 - protein, 36 aa, Homo sapiens
MMMQGVSEGEERKGSTVERNKEGFCPDRDDLLLLGL

SEQ ID NO: 8009 - protein, 58 aa, Homo sapiens
MMNSTLSYYYCHSSFILICIGLKNNWLSFYSFNYLELTPIFISVFPDFEVNSCSLQKS

SEQ ID NO: 8010 - protein, 35 aa, Homo sapiens
MMQGVSEGEERKGSTVERNKEGFCPDRDDLLLLGL

SEQ ID NO: 8011 - protein, 19 aa, Homo sapiens
MMRLYMWKSLNLESLDICL

SEQ ID NO: 8012 - protein, 84 aa, Homo sapiens
MNCKQHPSSKMPKIIVCGFFLSGGGSRAEPKQPAPQEAGADPGGAGPVRCVHPCPVSLCGKEGGLQLSASSGLRMLKTRKLLCN

SEQ ID NO: 8013 - protein, 93 aa, Homo sapiens
MNCKQHPSSKMPKIIVCGFFLSGGGSRAEPKQPAPQEAGADPGGAGPVRCVHPCPVSLCGKEGGLQLSASSGLRMLKTRKLLKTRRLHVIRVT

SEQ ID NO: 8014 - protein, 46 aa, Homo sapiens
MNCSLYQVDSRYYFQKYKSAAALGHPRPRTARRSPLLLEDLTPKLP

SEQ ID NO: 8015 - protein, 49 aa, Homo sapiens
MNCSLYQVDSRYYFQKYKSAAALGHPRPRTARRSPLLLEDLTPKLVCML

SEQ ID NO: 8016 - protein, 22 aa, Homo sapiens
MNFAASVFLNFEIKCSDKYSTF

SEQ ID NO: 8017 - protein, 19 aa, Homo sapiens
MNFSLTPFLSIPLTDMPKR

SEQ ID NO: 8018 - protein, 24 aa, Homo sapiens
MNHFGFRELSFFKKETLKKKSLYE

SEQ ID NO: 8019 - protein, 45 aa, Homo sapiens
MNHFKITNLIEPCPQTSLKWYILFGHHKFFSKSQFSDLYITPSFE

SEQ ID NO: 8020 - protein, 12 aa, Homo sapiens
MNITDEFFSSKK

SEQ ID NO: 8021 - protein, 16 aa, Homo sapiens
MNKAATNIYIHVFMCI

SEQ ID NO: 8022 - protein, 19 aa, Homo sapiens
MNKDRPGGQGSGNFPHHCH

SEQ ID NO: 8023 - protein, 11 aa, Homo sapiens
MNLIFHNKLHS

SEQ ID NO: 8024 - protein, 15 aa, Homo sapiens
MNLSQSVNIMAQELQ

SEQ ID NO: 8025 - protein, 45 aa, Homo sapiens
MNLVVRKKTTKLFKTQISRFTSVFPSWVFLAPKSHLFLLMSGSQP

SEQ ID NO: 8026 - protein, 47 aa, Homo sapiens
MNMNLVVRKKTTKLFKTQISRFTSVFPSWVFLAPKSHLFLLMSGSQP

SEQ ID NO: 8027 - protein, 15 aa, Homo sapiens
MNNFSNFLFFFFFLF

SEQ ID NO: 8028 - protein, 27 aa, Homo sapiens
MNRIMHLLSFVAGFCNLAYCLQGSSTL

SEQ ID NO: 8029 - protein, 22 aa, Homo sapiens
MNRIVILHLERFLPNISIFACH

SEQ ID NO: 8030 - protein, 37 aa, Homo sapiens
MNSHDRTSLFQSLLVLFIKQVFTVCKKMLKMTQNKHR

SEQ ID NO: 8031 - protein, 36 aa, Homo sapiens
MNSIIKRHKCDCTCIENLLEQKASKLKWLKEDRDDL

SEQ ID NO: 8032 - protein, 105 aa, Homo sapiens
MNSIIKRHKCDCTCIENLSRITRNLVEVVISSLSDGPIRNWLSALGVPCFFQRLLITWWSELEVRTREKNLYGPMKSGRLILRQKARLLGSLSGHSQLVVLCQLF

SEQ ID NO: 8033 - protein, 27 aa, Homo sapiens
MNSIIKRHKCDCTCIENQVQYYRSKQI

SEQ ID NO: 8034 - protein, 35 aa, Homo sapiens
MNSPIFTLEFIHSVTAHECRNQRTRREPPFIGSHN

SEQ ID NO: 8035 - protein, 32 aa, Homo sapiens
MNSSSSLCRRRLSLKRSQMLWEARQVYSGLEE

SEQ ID NO: 8036 - protein, 57 aa, Homo sapiens
MNSTLSYYYCHSSFILICIGLKNNWLSFYSFNYLELTPIFISVFPDFEVNSCSLQKS

SEQ ID NO: 8037 - protein, 24 aa, Homo sapiens
MNVFKLEVKLLKFLPNRRNPYQIG

SEQ ID NO: 8038 - protein, 14 aa, Homo sapiens
MNVGIKGHVGNLLS

SEQ ID NO: 8039 - protein, 35 aa, Homo sapiens
MNYILSSQNSHYKMNFAASVFLNFEIKCSDKYSTF

SEQ ID NO: 8040 - protein, 28 aa, Homo sapiens
MPASPPKLGVSGIWPENLQLLNILYRKL

SEQ ID NO: 8041 - protein, 22 aa, Homo sapiens
MPCNGFVCLLETGFHHVGQAGF

SEQ ID NO: 8042 - protein, 32 aa, Homo sapiens
MPCSSRLESRPWLMSSYPYPYISIKSLVSINR

SEQ ID NO: 8043 - protein, 27 aa, Homo sapiens
MPDLGASSCLGLPKCWDYRHEPPCPAC

SEQ ID NO: 8044 - protein, 33 aa, Homo sapiens
MPEWMVSSLVVLFLLLFLDNERQPFLTGDKDHL

SEQ ID NO: 8045 - protein, 112 aa, Homo sapiens [sequence omitted]

SEQ ID NO: 8046 - protein, 112 aa, Homo sapiens
MPGICKKGLERRSRGRACYFLSRPHCKRIWLCSCVSLLEAGTRWWAGLVWLRPLRGGIRSGRGGCEERGSGGCSDTGLGPCARDRLLLGMRLVSQEPVYFHHCLRGQLAQHQ

SEQ ID NO: 8047 - protein, 27 aa, Homo sapiens
MPGNFFVFLIEMGFHPVGQAGLELLTS

SEQ ID NO: 8048 - protein, 47 aa, Homo sapiens
MPGQAPDSALGNALNIIAQYLAMALGTAFPKAFSGLAPNRHDKQVRT

SEQ ID NO: 8049 - protein, 17 aa, Homo sapiens
MPGYFFCIFNRDRVSPC

SEQ ID NO: 8050 - protein, 28 aa, Homo sapiens
MPGYFFCIFSRDGVSSCWPGWSRTPDLR

SEQ ID NO: 8051 - protein, 17 aa, Homo sapiens
MPGYFFCIFTRDGVSPH

SEQ ID NO: 8052 - protein, 67 aa, Homo sapiens
MPHHAQIIFVFLVETRFLHIGQTGLELLASNDLPTSASQHAGIIGLSYHARPKGHIFAFRRKYATIS

SEQ ID NO: 8053 - protein, 28 aa, Homo sapiens
MPHHAWLIFVYLVEMRFHHVGQAGPDFN

SEQ ID NO: 8054 - protein, 39 aa, Homo sapiens
MPIRMTTIKNTEDKMCWQGRAKNGTLIHCWWECKLVQSL

SEQ ID NO: 8055 - protein, 27 aa, Homo sapiens
MPKMLIIVISNDRIRSNFHFLYFFVRL

SEQ ID NO: 8056 - protein, 13 aa, Homo sapiens
MPLRQANFFFFFF

SEQ ID NO: 8057 - protein, 59 aa, Homo sapiens
MPLWGFPDRAGLLGSPGSSGPGKRRPILAGQPYKLLELQARFLGPGHKSLVWTGDMATG

SEQ ID NO: 8058 - protein, 23 aa, Homo sapiens
MPNFCIFSTDGVSPCLVRLVSNS

SEQ ID NO: 8059 - protein, 29 aa, Homo sapiens
MPPCLAEFLYRWGFTMLPRLVLNSGLVWT

SEQ ID NO: 8060 - protein, 58 aa, Homo sapiens
MPPCLANFCILVETVSHHVGQAGLELLTSSDLPTSASQSAGITGVSHHIQPIYLFYVI

SEQ ID NO: 8061 - protein, 30 aa, Homo sapiens
MPPCLANFFVFLVETGFHSVSQYGLHLLTS

SEQ ID NO: 8062 - protein, 55 aa, Homo sapiens [sequence omitted]

SEQ ID NO: 8063 - protein, 21 aa, Homo sapiens
MPPCPANFCIFLVESGFLLTG

SEQ ID NO: 8064 - protein, 13 aa, Homo sapiens
MPPCPANFCIFSK

SEQ ID NO: 8065 - protein, 55 aa, Homo sapiens
MPPCPANFCIFSRDRFSPCCPGWLQTPELKQSARLGLPKCWDYRHEPLCPASCEF

SEQ ID NO: 8066 - protein, 24 aa, Homo sapiens
MPPCPANFCIFSRDRVSPCWPGWS

SEQ ID NO: 8067 - protein, 60 aa, Homo sapiens [sequence omitted]

SEQ ID NO: 8068 - protein, 11 aa, Homo sapiens
MPPCPANFLSF

SEQ ID NO: 8069 - protein, 30 aa, Homo sapiens
MPPCPTNFFVFLVETGYHHVGQDGLDLLTS

SEQ ID NO: 8070 - protein, 11 aa, Homo sapiens
MPPGPANFLYF

SEQ ID NO: 8071 - protein, 94 aa, Homo sapiens
MPPHLANFFCILVETGFHHVAQAGLKLLSSGNLPASASQTARITGVSHRTRPPLGYLRPYFHLDLSCPTHSLQSGFSFFEYKVDTGWLAYSFSV

SEQ ID NO: 8072 - protein, 26 aa, Homo sapiens
MPPHLANFLFLYFSRGGISPCCPGWS

SEQ ID NO: 8073 - protein, 16 aa, Homo sapiens
MPPHPANFCILRRDWV

SEQ ID NO: 8074 - protein, 56 aa, Homo sapiens
MPPHPANFFIFSRDKGFHHVRQAGLQLLTSGNPPASVFQSAGITGVSRCPRLKMYF

SEQ ID NO: 8075 - protein, 11 aa, Homo sapiens
MPPHPANFLYF

SEQ ID NO: 8076 - protein, 14 aa, Homo sapiens
MPPLIPEVSFPAQI

SEQ ID NO: 8077 - protein, 30 aa, Homo sapiens
MPPRLANFCIFSRDRVSPCWPGWFQTGLMI

SEQ ID NO: 8078 - protein, 11 aa, Homo sapiens
MPPRLANFSFF

SEQ ID NO: 8079 - protein, 22 aa, Homo sapiens
MPPRLANFYIFSRDGVSLFCPG

SEQ ID NO: 8080 - protein, 22 aa, Homo sapiens
MPPRPANFCIFSRHGVSPCWPG

SEQ ID NO: 8081 - protein, 30 aa, Homo sapiens
MPPRPANFCILIRDGVSTCWSGWSQTPILK

SEQ ID NO: 8082 - protein, 54 aa, Homo sapiens
MPPRPANFFVFLVEIGFYHVGQAGLEILTPGDQPTSVSQSAGITGVSHCAWQVK

SEQ ID NO: 8083 - protein, 30 aa, Homo sapiens
MPPWPANFCIFSGDGISPYCPGRSQTPDLR

SEQ ID NO: 8084 - protein, 73 aa, Homo sapiens
MPPYRASFCIFSRDGVSPCWSGWSQTPDLVICLGGLLTATNSTKTGPGCAFLSFGTSRNVPHLKEIVVFHRWL

SEQ ID NO: 8085 - protein, 26 aa, Homo sapiens
MPRRPANFCIFSRWGFTMLAKMVSIS

SEQ ID NO: 8086 - protein, 30 aa, Homo sapiens
MPSCPAHLFFCIDGITLCYPVGITGMSHCT

SEQ ID NO: 8087 - protein, 56 aa, Homo sapiens
MPSCPANLNIVFRDGAHYVAQAGLEFLVSSNPPTAAFQSAGRTSASHCAQLSDAEF

SEQ ID NO: 8088 - protein, 24 aa, Homo sapiens
MPSHLANFYIFSRDRVSPCWQGWS

SEQ ID NO: 8089 - protein, 18 aa, Homo sapiens
MPSQLANFCIFSRDGVWP

SEQ ID NO: 8090 - protein, 12 aa, Homo sapiens
MPSSFHSYLRLC

SEQ ID NO: 8091 - protein, 30 aa, Homo sapiens
MPSVLANFCIFSRDGVSPCWPGWSRSPDLS

SEQ ID NO: 8092 - protein, 13 aa, Homo sapiens
MPTNGSFIPSVAL

SEQ ID NO: 8093 - protein, 28 aa, Homo sapiens
MPTSASQNVGITGVSHGAQPHITFLLGK

SEQ ID NO: 8094 - protein, 26 aa, Homo sapiens
MPTSASQSAGITGMSHHAQPHVYFLK

SEQ ID NO: 8095 - protein, 36 aa, Homo sapiens
MQFHHIAQAGLILLASSDPPASASQSAGITGMSQRA

SEQ ID NO: 8096 - protein, 17 aa, Homo sapiens
MQFQGILIHLLTMILQE

SEQ ID NO: 8097 - protein, 34 aa, Homo sapiens
MQGVSEGEERKGSTVERNKEGFCPDRDDLLLLGL

SEQ ID NO: 8098 - protein, 11 aa, Homo sapiens
MQHHTWLILYF

SEQ ID NO: 8099 - protein, 22 aa, Homo sapiens
MQIHHCSAPQHTYWSYATALRY

SEQ ID NO: 8100 - protein, 19 aa, Homo sapiens
MQILTKLFEQTALQLLDML

SEQ ID NO: 8101 - protein, 31 aa, Homo sapiens
MQIWRNWNLCTPPMGVQYSIMLWTTVWRFLN

SEQ ID NO: 8102 - protein, 26 aa, Homo sapiens
MQKRYLPGPIVPTDPSQQLEVIVSSS

SEQ ID NO: 8103 - protein, 13 aa, Homo sapiens
MQLEIWWGADVPV

SEQ ID NO: 8104 - protein, 26 aa, Homo sapiens
MQLIFVFLVETGFHHVGQDGLDLLTS

SEQ ID NO: 8105 - protein, 22 aa, Homo sapiens
MQLLTEAWGASVLPSPPAKSTR

SEQ ID NO: 8106 - protein, 21 aa, Homo sapiens
MQLYCSSHQFHSERIFCCLPF

SEQ ID NO: 8107 - protein, 33 aa, Homo sapiens
MQMTCLLYFLMSLVDPGNRTFKTKSPYVAGCGG

SEQ ID NO: 8108 - protein, 12 aa, Homo sapiens
MQNVSKLFSSHI

SEQ ID NO: 8109 - protein, 40 aa, Homo sapiens
MQPSIQTQGQTHTPVRATGFPWQKETFSIVSIHKERPVLG

SEQ ID NO: 8110 - protein, 103 aa, Homo sapiens
MQRPLGPGRRRRLRRPSLQRRPRPGPASWARAALSRERPWRKAAAAQAGRAATTGGPAPAAVARCTWPRSPTPPSVAPSPCPGPSSAWCAGSGTRPSPGSRRG

SEQ ID NO: 8111 - protein, 12 aa, Homo sapiens
MQTHLQISHHLF

SEQ ID NO: 8112 - protein, 32 aa, Homo sapiens [sequence omitted]

SEQ ID NO: 8113 - protein, 13 aa, Homo sapiens
MRAPQLFTCLSGW

SEQ ID NO: 8114 - protein, 27 aa, Homo sapiens
MRDRLRPLAALRASRLAPTGAATTTTS

SEQ ID NO: 8115 - protein, 12 aa, Homo sapiens
MREGLESYPLNF

SEQ ID NO: 8116 - protein, 14 aa, Homo sapiens
MRFHHVGQAGPDFN

SEQ ID NO: 8117 - protein, 59 aa, Homo sapiens
MRFHHVGQASLELLTSSNLPTSVSQSWDYRREPPRSSLKTILEYLQEHPGMSSVTGLKC

SEQ ID NO: 8118 - protein, 31 aa, Homo sapiens
MRFHHVGQASLELLTSVIDPPWPPKVLGLQA

SEQ ID NO: 8119 - protein, 31 aa, Homo sapiens
MRFHHVGQAVLKLLTSGDPPASASQSLGLQA

SEQ ID NO: 8120 - protein, 40 aa, Homo sapiens
MRFHRVGQVGVKLLASNDPPALASQSVGITGMSHHAQLVK

SEQ ID NO: 8121 - protein, 16 aa, Homo sapiens
MRFHYVGRDGLYLLTS

SEQ ID NO: 8122 - protein, 63 aa, Homo sapiens
MRFLHVGQAGLELPTSGDLPTWASQSAGIIGMSHCAQPSILFFLHVLQLGPTIAATAIKLYNK

SEQ ID NO: 8123 - protein, 56 aa, Homo sapiens
MRHHAQLIFAFLVEMGFHHVGQTGLELPTSGDPPTSASQSAGITGVSHHARPQKCS

SEQ ID NO: 8124 - protein, 30 aa, Homo sapiens
MRHHAQLIFVFLVETGSCHVGQAGLELLTS

SEQ ID NO: 8125 - protein, 19 aa, Homo sapiens
MRHHARLRDGVSLCWPGWS

SEQ ID NO: 8126 - protein, 56 aa, Homo sapiens [sequence omitted]

SEQ ID NO: 8127 - protein, 54 aa, Homo sapiens
MRHHAWLISMFLVETGFHHVGQAGLKLLTSSDPPALASQSAGITDVSHCTQAPL

SEQ ID NO: 8128 - protein, 12 aa, Homo sapiens
MRHHTQLIFLYF

SEQ ID NO: 8129 - protein, 31 aa, Homo sapiens
MRHHTQPICCIFSGDEVSPCWPGWCQTPGLK

SEQ ID NO: 8130 - protein, 56 aa, Homo sapiens
MRHHTWLFVFLVETGFLHVGQAGLKLPTSGDPPTSDSQSARVTGVSHCTQPGNLHF

SEQ ID NO: 8131 - protein, 25 aa, Homo sapiens
MRHHTWLILYFLVETGFLHVGQAGL

SEQ ID NO: 8132 - protein, 51 aa, Homo sapiens
MRHHTWLILYFLVETGFLHVGQAGLELLTSGDPPTLASHSAGITGHRAQPI

SEQ ID NO: 8133 - protein, 11 aa, Homo sapiens
MRHHTWLTLYF

SEQ ID NO: 8134 - protein, 86 aa, Homo sapiens
MRHYSRLIFVFLVEMEFYHVGQAGLKLLTSGNPPTLASESAGITGMSHRAQPTFFFFFLIQTFFLDTVSLCHSVWSAMARSQLTLA

SEQ ID NO: 8135 - protein, 80 aa, Homo sapiens
MRKGWRGPGRQDDHTKWILDYFPGNSLKQNRPAWAPLCFRPPPAARGCGCPNTRAEKGPPEGGAVFTVGIDQADCFLVVE

SEQ ID NO: 8136 - protein, 33 aa, Homo sapiens
MRKYNLRIYTEEDTYHILITKLGLYQKSQQNIF

SEQ ID NO: 8137 - protein, 25 aa, Homo sapiens
MRLLDQKLLNKQQSLSWLYGCSEGF

SEQ ID NO: 8138 - protein, 19 aa, Homo sapiens
MRLTPPCRAKRRIVHLVMP

SEQ ID NO: 8139 - protein, 18 aa, Homo sapiens
MRLYMWKSLNLESLDICL

SEQ ID NO: 8140 - protein, 50 aa, Homo sapiens
MRMTAQKGRSEFPVKGSFLLGEYPSTRTLLLSRVKFCSWVPFRVIRRNSS

SEQ ID NO: 8141 - protein, 23 aa, Homo sapiens
MRPKMRLTPPCRAKRRIVHLVMP

SEQ ID NO: 8142 - protein, 14 aa, Homo sapiens
MRPPQPPKVLGLQV

SEQ ID NO: 8143 - protein, 11 aa, Homo sapiens
MRQHARLILYF

SEQ ID NO: 8144 - protein, 69 aa, Homo sapiens
MRSTYRKGWEKSEKASWRRWKLQHLRMGRICISRAAGKDTSGKGYCARKRAGSSQLLKSSQCLKLHFFP

SEQ ID NO: 8145 - protein, 12 aa, Homo sapiens
MRVPLRHTAGTD

SEQ ID NO: 8146 - protein, 93 aa, Homo sapiens
MRVSQHLPSTEAMSGKSQKRIHFMMLPTYLTQVVFFLQVCKVWMGFLKTSRGSARSNYCHNITKMLFAFPRHSLRSIWWGLPKATMTCGLSAD

SEQ ID NO: 8147 - protein, 30 aa, Homo sapiens [sequence omitted]

SEQ ID NO: 8148 - protein, 11 aa, Homo sapiens
MRYSFKKVDFS

SEQ ID NO: 8149 - protein, 14 aa, Homo sapiens
MSAKTYYLVLFCVC

SEQ ID NO: 8150 - protein, 24 aa, Homo sapiens
MSCSSMKMLVSNRMTQCKKIQRKR

SEQ ID NO: 8151 - protein, 42 aa, Homo sapiens
MSCSSTKMLMSNRMAHCKKIQRKRQHRTLGTLRKMTLNFSLL

SEQ ID NO: 8152 - protein, 42 aa, Homo sapiens
MSCSSTKTLMSNRMAHCKKIQRKRQHRTLGTLRKMTLNFSLL

SEQ ID NO: 8153 - protein, 24 aa, Homo sapiens
MSCSSVKMLISNRMTHFKKIQWKR

SEQ ID NO: 8154 - protein, 20 aa, Homo sapiens
MSCWDRATCALSFTSSSCSV

SEQ ID NO: 8155 - protein, 34 aa, Homo sapiens
MSFCCSGWSAMVRSQLTAASASWVQAILVPQPLK

SEQ ID NO: 8156 - protein, 111 aa, Homo sapiens
MSFFCSQYEVRHWPSRGRLPEVGQRGVTCLGQDTQHPSWRKPSAHSSVCRTRLWAFCTTAGSRAYQLLSTSCSRFRARRVLPVYTKSRWSLSFWTKPSGTVTSSTSTFSGS

SEQ ID NO: 8157 - protein, 19 aa, Homo sapiens
MSFSTRCQSTLMYPEWFAS

SEQ ID NO: 8158 - protein, 29 aa, Homo sapiens
MSGDPSALASQSAGITGVSHRTQPEKSII

SEQ ID NO: 8159 - protein, 81 aa, Homo sapiens
MSGKSQKRIHFMMLPTYLTQVVFFLQVCKVWMGFLKTSRGSARSNYCHNITKMLFAFPRHSLRSIWWGLPKATMTCGLSAD

SEQ ID NO: 8160 - protein, 36 aa, Homo sapiens
MSHCTWPSLTLFVYRPNITLSHSSSLLCELRLGGII

SEQ ID NO: 8161 - protein, 31 aa, Homo sapiens
MSHHARLIFCIFSRDRVSPCWSGWSQIPDLR

SEQ ID NO: 8162 - protein, 122 aa, Homo sapiens
MSHHARLIFVVLVERGFCHFGQAGLELLTSVDPPASASQSVGIMGMSHHAQPTTALTVFFFFFFFFLRLSLAVLPRLEYCGVISAHCNLRLLGLSKSPASASQIAGITGTCHHARLINNIIF

SEQ ID NO: 8163 - protein, 15 aa, Homo sapiens
MSKHGSVRHSFSGLK

SEQ ID NO: 8164 - protein, 92 aa, Homo sapiens
MSKRRRRRSRAGGGPARASARLEVTIALPQGLCRLLPGSLQEGQLLGFLLLVSRLILQPVGDDPLDDEVCGEVAATVNLTEDAPSLGLLEVT

SEQ ID NO: 8165 - protein, 114 aa, Homo sapiens
MSKRRRRRSRAGGGPARASARLEVTIALPQGLCRLLPGSLQEGQLLGFLLLVSRLILQPVGDDPLDDEVCGEVAATVNLTEDAPSLGLLVWVGAIPVRDNFCLAVTHQVHLEVT

SEQ ID NO: 8166 - protein, 281 aa, Homo sapiens
MSKTPKAMATKDKIDKWDLIQLKSFCTAKETTIRVNRQLTKWQKIFATYSSDKGLISRIYNELKQIYKKKTNNPIKKWAKDMNRHFSKEDIYAAKKHMKKCSPSLTIREMQIKTTMRYHLTPVRMAIIKKSGNNRCWRGCGEIGTLLHCWWDCKLVQPLWKSVWRFLRNLELEIPFDPAIPLLGIYSKDYKSCCYKDTCTRMFIAALFTIAKTWNQPKCPTMIDWIKKMWHIYTMEYYAAIKKDEFMSFVGTWMKLEIIILSKLSQGQKTKHHMFSLIDGN

SEQ ID NO: 8167 - protein, 42 aa, Homo sapiens
MSLRARCIPNLEHDLSRQMRPSVFSLFENKMWGGHDGNSTWG

SEQ ID NO: 8168 - protein, 18 aa, Homo sapiens
MSLSSVLSNHFPMALNCL

SEQ ID NO: 8169 - protein, 63 aa, Homo sapiens
MSLVPGWSAVEAFYYHLPICIRRLVSLNAVQFCGADVGIRGLQKAAGTPGMQALSCCITTCLI

SEQ ID NO: 8170 - protein, 15 aa, Homo sapiens
MSLVSSAAPHPNDDA

SEQ ID NO: 8171 - protein, 40 aa, Homo sapiens
MSMGPQAGLLQPGTAPPTPAQRRLLLAGDDSLRAPNTIPT

SEQ ID NO: 8172 - protein, 12 aa, Homo sapiens
MSMPFLHPLGLR

SEQ ID NO: 8173 - protein, 28 aa, Homo sapiens
MSNCWYFLRKYIVQLWLPRTAGKALLFM

SEQ ID NO: 8174 - protein, 35 aa, Homo sapiens
MSNQDGLSFVIYCNCACHMQFQGILIHLLTMILQE

SEQ ID NO: 8175 - protein, 33 aa, Homo sapiens
MSNSRKRSIPTRDVNSVLEQLLTEESLDESDFS

SEQ ID NO: 8176 - protein, 30 aa, Homo sapiens
MSPCLVNFCISSRDGVLPCWPGWSQTLDIR

SEQ ID NO: 8177 - protein, 14 aa, Homo sapiens
MSPGLFFGFHPEFL

SEQ ID NO: 8178 - protein, 79 aa, Homo sapiens
MSPGLFFGFHPEFLNLFHQEFLCSVTLFLGLGNLQLGIGFHVAILQVGFCLHLLQLVLEVSNILILTLDFKLPFLFDIN

SEQ ID NO: 8179 - protein, 15 aa, Homo sapiens
MSQVLRQWLEKINIL

SEQ ID NO: 8180 - protein, 14 aa, Homo sapiens
MSSISLLCILSVLF

SEQ ID NO: 8181 - protein, 14 aa, Homo sapiens
MSSKVGGQTEGLPT

SEQ ID NO: 8182 - protein, 31 aa, Homo sapiens [sequence omitted]

SEQ ID NO: 8183 - protein, 14 aa, Homo sapiens
MSTCSIVDLLLGTN

SEQ ID NO: 8184 - protein, 50 aa, Homo sapiens
MSVAMNCSLYQVDSRYYFQKYKSAAALGHPRPRTARRSPLLLEDLTPKLP

SEQ ID NO: 8185 - protein, 53 aa, Homo sapiens
MSVAMNCSLYQVDSRYYFQKYKSAAALGHPRPRTARRSPLLLEDLTPKLVCML

SEQ ID NO: 8186 - protein, 11 aa, Homo sapiens
MSVFNILLCKT

SEQ ID NO: 8187 - protein, 27 aa, Homo sapiens
MSVRLVSISRPQMIHLLRPPKVLGLQA

SEQ ID NO: 8188 - protein, 48 aa, Homo sapiens
MTAQKGRSEFPVKGSFLLGEYPSTRTLLLSRVKFCSWVPFRVIRRNSS

SEQ ID NO: 8189 - protein, 12 aa, Homo sapiens
MTCGLLCLASSA

SEQ ID NO: 8190 - protein, 31 aa, Homo sapiens
MTCLLYFLMSLVDPGNRTFKTKSPYVAGCGG

SEQ ID NO: 8191 - protein, 18 aa, Homo sapiens
MTGSHNLKEYTCNETSLP

SEQ ID NO: 8192 - protein, 24 aa, Homo sapiens
MTHLHFCLLRTILICCIIRIIISV

SEQ ID NO: 8193 - protein, 47 aa, Homo sapiens
MTHSTHALIVFCFFFHLRSIAFHFIYQTVFTVDRHCSSHVPYGFVLS

SEQ ID NO: 8194 - protein, 47 aa, Homo sapiens
MTHSTHALIVFCFSFHLRSIAFHFIYQTVFTVDRHCSSHVPYGFVLS

SEQ ID NO: 8195 - protein, 17 aa, Homo sapiens
MTKNAYLDSQPIRKVGH

SEQ ID NO: 8196 - protein, 13 aa, Homo sapiens
MTKTRLKYNMSKI

SEQ ID NO: 8197 - protein, 11 aa, Homo sapiens
MTLGNLLFKID

SEQ ID NO: 8198 - protein, 13 aa, Homo sapiens
MTLNKQVVLYTVN

SEQ ID NO: 8199 - protein, 33 aa, Homo sapiens
MTPDAPDELTDTWNNRVHKHGVPHGEVTKAEEG

SEQ ID NO: 8200 - protein, 41 aa, Homo sapiens
MTPFKCTYGISPIRRAGSVISNIFSAYCVPGTTLSLYMLLF

SEQ ID NO: 8201 - protein, 30 aa, Homo sapiens
MTPHNTRYYEVSETEDNLTEDACREGTGSV

SEQ ID NO: 8202 - protein, 15 aa, Homo sapiens
MTPLTGKQAGVHRDL

SEQ ID NO: 8203 - protein, 59 aa, Homo sapiens
MTPRSPAKPMRMTAQKGRSEFPVKGSFLLGEYPSTRTLLLSRVKFCSWVPFRVIRRNSS

SEQ ID NO: 8204 - protein, 22 aa, Homo sapiens
MTRISGRPRELSSLMSSGTRVL

SEQ ID NO: 8205 - protein, 25 aa, Homo sapiens
MTRKPPPHLELSRLCRWNHCSSYIC

SEQ ID NO: 8206 - protein, 28 aa, Homo sapiens
MTSSHVPSSACVYWKLLTQHSTKELTAG

SEQ ID NO: 8207 - protein, 23 aa, Homo sapiens
MTSSYPLASASQNAGITGLSHHA

SEQ ID NO: 8208 - protein, 35 aa, Homo sapiens
MTTIKNTEDKMCWQGRAKNGTLIHCWWECKLVQSL

SEQ ID NO: 8209 - protein, 15 aa, Homo sapiens
MTTRNGSWIISQAIR

SEQ ID NO: 8210 - protein, 14 aa, Homo sapiens
MTVYSLLSVFLIRV

SEQ ID NO: 8211 - protein, 25 aa, Homo sapiens
MVCMELLLSKASPRLKSSPSSSRRR

SEQ ID NO: 8212 - protein, 19 aa, Homo sapiens
MVDDDHDDDNDDSTIIDHD

SEQ ID NO: 8213 - protein, 26 aa, Homo sapiens
MVFCGTSWFPQSLESIHPSHWFSEEL

SEQ ID NO: 8214 - protein, 55 aa, Homo sapiens
MVFEITVAVMQFRNLSKFILTSEANITVSRGIQLCASRMDSLSQHVIAKDDSVSS

SEQ ID NO: 8215 - protein, 43 aa, Homo sapiens [sequence omitted]

SEQ ID NO: 8216 - protein, 15 aa, Homo sapiens
MVFHHVSQDGHLLTS

SEQ ID NO: 8217 - protein, 11 aa, Homo sapiens
MVFPLLEERDL

SEQ ID NO: 8218 - protein, 239 aa, Homo sapiens
MVHHLLQALAEGAPPDAHEALLRLREGDGPDARCHPKLLHHGVGDAGDLPQVVLCPRSDLVEGQCFRGPSSQGHAHPLKQLLLGEEVLVSGEHLSKAQGGVCPRGYGDLHHGLRVLQHPAHQGVARLMKRNHFLFFLGQDLALFGSPCEDALHGVLEVESVHGSVSLPRRVQRSLIADVGDVSPTESWCQLCQTLGVKGAGLGQLQALQVLLKNLPPLLGDGGCSEPRSRRCTPAWGIE

SEQ ID NO: 8219 - protein, 493 aa, Homo sapiens
MVHHLLQALAEGAPPDAHEALLRLREGDGPDARCHPKLLHHGVGDAGDLPQVVLCPRSDLVEGQCFRGPSSQGHAHPLKQLLLGEEVLVSGEHLSKAQGGVCPRGYGDLHHGLRVLQHPAHQGVARLMKRNHFLFFLGQDLALFGSPCEDALHGVLEVESVHGSVSLPRRVQRSLIADVGDVSPTESWCQLCQTLGVKGAGLGQLQALQVLLKNLPPLLQRGEINEDVPVQSAWPHQSTVQNVSSVRGRQDDDMVCGTHSIHFYQKLVERLLLLRVGEAGHGGGALLAHRVDLIDVDDAGGPGSGFLKEAPHTGSAEASNDLHELWAGHRQEGHLSLRGHRLGQQRLPTAGGAEQQCALWDLGAKLEEAFWALQIIHKLADFQFGFVHSCHVFEADSFPHLPIHNGETSHFKLIKSTESTFPSSHPGQTENIPQDGQAHCRHPHRVQGISKESCSLVGNWDPVLGLDIQLIFSCSKLLFKLVNICNLHSVHQG

SEQ ID NO: 8220 - protein, 200 aa, Homo sapiens
MVHHLLQALAEGAPPDAHEALLRLREGDGPDARCHPKLLHHGVGDAGDLPQVVLCPRSDLVEGQCFRGPSSQGHAHPLKQLLLGEEVLVSGEHLSKAQGGVCPRGYGDLHHGLRVLQHPAHQGVARLMKRNHFLFFLGQDLALFGSPPSEAFCLRDKAFFLSVTGSHSVAQAGGQWCDHGSLLLQPPRFKQSSCCSLLSS

SEQ ID NO: 8221 - protein, 54 aa, Homo sapiens
MVHSIVENSLNWGPEDPALLLSSCVTLGKAVAFSLLICETKIHLPAQDILNKDC

SEQ ID NO: 8222 - protein, 37 aa, Homo sapiens
MVKFTAGATHQHPEPTFNQVSLFVLCLLHILFHKKGE

SEQ ID NO: 8223 - protein, 23 aa, Homo sapiens
MVLISWPQMIHPPWPPKVLRLQA

SEQ ID NO: 8224 - protein, 21 aa, Homo sapiens
MVLKFPFLPLGLNSEFTWSNF

SEQ ID NO: 8225 - protein, 34 aa, Homo sapiens
MVNRELWAYFKCLFSPLSAKAKGNFSLLCTVRSC

SEQ ID NO: 8226 - protein, 90 aa, Homo sapiens
MVPSRLTATSASQIQVILLPQPSKWMGLQACAITPGYFVFLVETGFLHVGQAGLQLPTSGDPPTLVSQSAGITGVSHRARSVLLAVMGFH

SEQ ID NO: 8227 - protein, 14 aa, Homo sapiens
MVRGPAPCVICQLD

SEQ ID NO: 8228 - protein, 24 aa, Homo sapiens
MVRSQLTAASASWVQAILVPQPLK

SEQ ID NO: 8229 - protein, 16 aa, Homo sapiens
MVSFNKRLNWYMIIFK

SEQ ID NO: 8230 - protein, 15 aa, Homo sapiens
MVSHTYKSQHFGRPR

SEQ ID NO: 8231 - protein, 15 aa, Homo sapiens
MVSISGQSLFCKYPW

SEQ ID NO: 8232 - protein, 40 aa, Homo sapiens
MVSISQPCDPPTSASQSAGITGVSHCAWTKTMLSKAHSAA

SEQ ID NO: 8233 - protein, 161 aa, Homo sapiens
MVSISRPHDPPALASQSAGITGVSHSAWPDLFSKIGQFPQKIILQSPARREGLGVLLFIHSFTFNPPVSCMLAAPSTSSCVSKCKPPCEPPQRGSMQFLAGTGERQPSCCRRGSAILFPYRLLVHSSVFSPSVPLSPPSRRIQCFYILKLSRGLWYKTGCF

SEQ ID NO: 8234 - protein, 45 aa, Homo sapiens
MVSISRPRDLPFSASQSAGITGVSHRARPSCPLNQTVLLPLENVH

SEQ ID NO: 8235 - protein, 22 aa, Homo sapiens
MVSISRPRDPPASASRSAGITG

SEQ ID NO: 8236 - protein, 62 aa, Homo sapiens
MVSNSWPRDLPVSASQSAGITGVNHHAQPRSQPFFGSGSNSRAMTLVVETGLCSNKCHHPGH

SEQ ID NO: 8237 - protein, 16 aa, Homo sapiens
MVSPCWLGWSRTPDLK

SEQ ID NO: 8238 - protein, 13 aa, Homo sapiens
MVSSCPIKMGFHL

SEQ ID NO: 8239 - protein, 29 aa, Homo sapiens
MVSSLVVLFLLLFLDNERQPFLTGDKDHL

SEQ ID NO: 8240 - protein, 37 aa, Homo sapiens
MVSTRALWEAQVHLWTQLWRRQVSLMRTDIQAAACAA

SEQ ID NO: 8241 - protein, 13 aa, Homo sapiens
MVWIRSAMGSKKS

SEQ ID NO: 8242 - protein, 61 aa, Homo sapiens [sequence omitted]

SEQ ID NO: 8243 - protein, 16 aa, Homo sapiens
MWFHHVGQDGLDLLTS

SEQ ID NO: 8244 - protein, 16 aa, Homo sapiens
MWFYHVGQAGLELLTS

SEQ ID NO: 8245 - protein, 16 aa, Homo sapiens
MWKKGELLHTLGGNVN

SEQ ID NO: 8246 - protein, 14 aa, Homo sapiens
MWKSLNLESLDICL

SEQ ID NO: 8247 - protein, 16 aa, Homo sapiens
MWLPVRRRPGLNCFLV

SEQ ID NO: 8248 - protein, 31 aa, Homo sapiens
MWRKGKPLFTIGRNVNFHSHGREHYGGSSKN

SEQ ID NO: 8249 - protein, 12 aa, Homo sapiens
MWRTENSCTLLV

SEQ ID NO: 8250 - protein, 24 aa, Homo sapiens
MWSNWNSLTFQVGMLNCTVTLEST

SEQ ID NO: 8251 - protein, 14 aa, Homo sapiens
MWYCCQYYLQELGF

SEQ ID NO: 8252 - protein, 26 aa, Homo sapiens
MYAGKSLPTLLASLIPVGPHHLFRRK

SEQ ID NO: 8253 - protein, 86 aa, Homo sapiens
MYFIFLVKMGFCHVGQAGLELLTSGDLPTLASQSAGITGMSHHAWPILSTYKKFLCSWWINWLHNKIILVQWIDSCQIHPVANYLN

SEQ ID NO: 8254 - protein, 17 aa, Homo sapiens
MYGNFHLIAQVQDNPAH

SEQ ID NO: 8255 - protein, 11 aa, Homo sapiens
MYHHTRLVLYF

SEQ ID NO: 8256 - protein, 50 aa, Homo sapiens
MYHKRQLQMKCFAKGIHNFHFVNVAMEKFRGKLFIKCGPLIICNSAILTN

SEQ ID NO: 8257 - protein, 24 aa, Homo sapiens
MYHLAVCIHQACKHISKYLITCSR

SEQ ID NO: 8258 - protein, 20 aa, Homo sapiens
MYKKIGITQCCAVLWCRCGY

SEQ ID NO: 8259 - protein, 11 aa, Homo sapiens
MYLSDFWNEYM

SEQ ID NO: 8260 - RNA, 2059 nt, Homo sapiens
  source 1..2059: mol_type = other RNA
aaaaaccacaattacttttccaccaacctaataattttctctttttagaatgttaagtatgacattttaaactctattatttctagtaatatttaacaagtattatattttaaactctattatttctagtaatatttaacaaaattacagcattcatatggactaggatggaattatttttaatgaccacctacaaagtcgtatgaagacaagaggcaaaatgacccagttttgtgttttcttttcatctttctcagagattttcataaatattatgaaaatatccatctaagcttttatagtgaactgttgggttatttcctggtctattatacagcaaaactcaacagacactcaactcaccaagttgtataaagatgggagacaaaatgacccagtattatgttttcttataaatcatctttctcagagattttcaaaaatattatgaaaatactcatctatgctcttattttttggatttgtagattttttgtttattccctggtctataatacaacaaaattcaacagatcttgggatagaatgtctcatgatatattctaaatttgcattaacaaacaagtcaatagtttaaaatgctgagagagatttttccagtacatttattcagttaacatatatgggcaaatgatccaaaacttctcaatgttcacgatgatctactcaaaaaatacacttgacatcttaaatgaaaaaatattttttcccaaattccgcaatcttggatatatacaacacatctgatgagtagtgagaattggaaagtagcagcattgtttaatactagagcttggttagaagtctgcatcttgaactgccatttaattttatttcagtgatcaaattagcagtcattttttttaaataaagcaactcatttctactaaagttaaataaaataaacaacaaacatgtatagcattgtaaacaaaaaccacaataatcgtatttggtgcaacaaaaatttcactgtccgggaactacagtgtctgccacggtggttgaatgggtgtattaacaccatcttgtcaactaatctaatagcagggaaaagctgtcaaaaagctcatttccttatctctgtgaaaaatagagaaattgattgaatggattaagctccattacttaagcatactaataaaataaccaccatttatcaagtacctatcatttatattgttctataaataaatatgtttgttagcctttacaacaactttgtaaggttggtttttgagaagaacccatggtggagccaagctaagcagttgaatccaggactcacgtgaatgcatctcatggacaggacttccctcctgtgtggctcagatgcttgtccaccagatgcctctggctagtttttactctaatggtgtcactcaaaaaacatggcctttccatttaccgtttcagtatgctgccatttttttcctttgtttcctttctttctctttcttaacttccttacttgattctcctggaagcatttgaatatgaatccacatcttgttggtttctgggaaccccaatcaaatactcccctgatttagccattcggtattaactcattatcttctatagagcatgcctataatcttgacattttctcagggatgaagtgctggtctctggaaaacagcttcatctttttttcttcatcttgctcagaggcagaaggaaaagtggagagaccattagaatagcaagttttgttctactgaaacaaataagatccacccttggaagccttgttagaaaattttggatttcatgcttccatgacctcagtttacgtaaggccacattaggaaaaaagaataggcaggacattccaaggagcattggccaccaccctcacaaagaccaatattaggacaaaattcatgtaagagtgtcacccaacaatccctttttagaattacatttttaaaatgatgtatcattgtatattggttatattggggtggaaaacttgtcttttcattcaaagtcccattgaacaggagttggcaaacattttctgcaaaggaccata

SEQ ID NO: 8261 - RNA, 255 nt, Homo sapiens
  source 1..255: mol_type = other RNA
aaaaaccacaattacttttccaccaaccttacacaagtaaggtaaatgcaaagagattcacactgagatacgttgtattcaaattgtcaaaagtcacaaagagaatcttgaaagcaagaagagaagaggctcatcacttacaagagattcttaataagattagcagctggtttttcttcagatactgtggatgccaaaaagacagtaggataaatatttaaggtgctgaaagagaccaaaaaaaaaaaaaaccta

SEQ ID NO: 8262 - RNA, 4338 nt, Homo sapiens
  source 1..4338: mol_type = other RNA
aaaaaccacaattacttttctatcaatgtaatagtagaaacggggtttcactgtgttggccaggctgttcttgaactcctgacctcaagtgatccgcctgcctcagcctcccaaagagctgggattagaagtgtgagtcactgatcctggctgaaataaaaaaaattaaaaaatatattttattgttttgaattttatttaaaactctttgcaagaaatgatgctggaagactacctgtttagaattgtaatccatatatccacaagctctggcagctttaaagagaggcaatagaagaatgaatgcccaaatgtagcagattggcttttactcattttcatagtctcctcaccctagcactggtataatatgattctgagaatgttaggcagctaaagctgtttcttttaattcttgtccactttggtgacatgaggaatcaaactcaccattttatatatttagatactgaatattctggtagctcagcaccagactctgtgaagtcattccttttgcttatctatgacttggattacattccaagtatgaattaacatacagccagactagatgaacagctttagaagaatatgacttgcttttttttttttgacaagctcatttagaaggtgatacattcttttccatgttcatttccaaatgcttatataaagaatgctgagtgaactcttgcctagtgatcttaaacattaacttacacaaagtaccttccttccttgtctcagcatgttaatacatcctgtctctcccatagatatctagggcaatgaagttgatgctagcccagttcttataacctgctgccaagtattttgatggctttatctgaagagtaggtaagatctttgctgacccagctacccagcatgcagctggatgtgtggagagtagaaatatgctggccttgtgcagatggatttcaagtacaatggccaacatttttactgtccctgctatattaaaccaaccaatttaatgccttctttctagttaagctccagttccttgaaaaatatattgtttataatatagttataatagatgtcatttattaaacacaataaatactggctgtcttttaatattttacatctattttctcagtgaatgctcaaaactataagatagacactattattgtaaacattttagagttgacagaggtgagccttagagagatcaagtaactatccccaggtaactttggtagaaagttgaaaatctgggatttgaactaaagcctatgttttaagccactatatgacattgctcccactgtaccataggttttagtagaaatgtgggtgtaggggaacttaatgatttagatgtggctattcaagaacacttcttgttcttgtagtgcattaaatttggaatatattgaatattatcactaatctctagctagcaaccaaagaaaacaagatactcagaatagcaacagctttacataaaatactttttcaaaaatattatacattctccaataccttctgtggctctgataatttgctctcataatcagttcaatccagcttgttccttaaatgcttgagaagtacctcattttactcaacatattaccacatataaagcatgtgaaaataccagattgtgttccacttttaccccaaatagtaacaaagctcctgcaattttttaagatattattaaactgtgtacaaatgctcagattaaaaaaaagtgcttacttccattgaaattggacactaccactacctattcaaattcaagttgtcattgccttgaatccatgtgtaaagtttttggtaggatagtctatttctagttgtttttcaagactcataatttggaacattctagatataagattgcattgacactttatattctttttactttataaaatggtcatccatggtttatgttacaaacgaaagcaaaaatctgggggaaagttaaagaagtagagccagataacagaattttcttttctaatatctaataaagtgaaacaaaaggatgaaaataaaatcatgataggaaggaaaaaattaccagaaactatcaaagagagagaaaacagatctcatgccattaacttaaaatgtcacctaagaaaagaaacaatagattttgtctaggagaatgaaagccttctaaacttgtctctagaaacctgttttaaccataaactagaaaatggacatattaagttgacaaaaatcttaaaaattttctcctcatttggagaaaagtagactaaatatatattctttcattttcctcttatgaaaggagggaagttgcaatggttacatttgaaatatagatgaaaaaatggaggagaagaaaaattattcactcctcgatggaaacatagtctccagggctccatgctgaagaacaatgctgatactacattctcctcaaaacaattctgaaaatttcttgactcatgaaacccagctaactcagtagttgtaattacttacttttatgatctggtttcctttttcactctaaattcttatcctcctactcttctaaataaacaatctgttttgcttcttaaatttcaaataatttatggaaaacagaactaattctttccaactgttccttttcagatccccattcactcttctctaataacaattaaaatattattttgttttttgtaaatttattacataaatttaccatttatatatctttccttgattctagactatagttttcttgaaattaagacatatacttttcctattttaatcttcaagggccaatttagcacttgaaatatagacattcaatgcatatttgttaagtgaaaatgtattttgaagtgtaatctccttttttaaagtttcacaatctttttgactgagtccttgaaagcttgtttcacttgctgatttcttaaagtatatatgaagggattcagtaagggagtaaccgaagtaatgagtacagctattcctttgttgaaagcacctccttcttttgcagaaggattaatgtacataaacatgcagctgccataagagagggagatgacaatcatgtgggaggaacaagtggaaaaggcctttgtcctttgctgggcagaagggatcctcagaatagtcctgataatgtatgtgtaagaaagtgtcaccagcaccagagtaaccatgagagtcacaacggccaagaggatgaccatcagttctaagaggcttgtgtctgagcaggcaagctccacgagaggcccatagtcacagtaatagtgattcagaatgttggagacacagaaatctacctgggtcatcaggatgattggtggtaagattgctaggaatccccccaaccaggagcagaacactagttgtatgcagactctgctgctcataatagtcaggtaatgcaagggtttgcagatggccacataacgatcataagacatggaggccaggaggtaaaactcggtagctccaagaaatatagcaaaaaaatactgagtcaagcagccagcaaagctgataactttatttcctgttgtcatgctggtcagaaatctgggaataaaaatggatgtgaaggaaatttctaagaaggagaaattccggaggaagaaatacatgggggtctggaggtgggggtctagtaaggtgagggtgataatagtcagatttcctaggatacttagcatgtaggtgaggaacagaaagatgaatatcatcacttggagttcaggttgatttgtaaggcccagtagaataaactcaccaaacatggttctgtttttcattgttgaccttcggaaaacctgtggtctttggcaagtactgcattttcttccagattttcacagttgattcatttcatgatccacatttatagaatgataaaatcagtgactttaaaaacatatgttgctcatacctttgacaacctgaatgactatagtatactgtttaccttgttgttcctaagaggtaaatcaaagatgagatgtgccacgtgaatctttgagtagtatatactttaacatgttttctattggcttccatccacattttacctttctcttaatagaagtatccaaacttatggaacttaaccagaaaaaagagcatattattttccattctaagaatccaatccagaatcaaatcatagttcctgagagacagagaacttcacataggtaataaaaaataaaaacaaagcccatagcagttattgaattggaagaaaatactttgagagacagaaaatttctgaaaatttatgttctaagagagattatgttgaagttcttagatggcagaggatgggcatct

SEQ ID NO: 8263 - RNA, 4186 nt, Homo sapiens
  source 1..4186: mol_type = other RNA
aaaaaccacaattacttttctatcaatgtaatagtagaaacggggtttcactgtgttggccaggctgttcttgaactcctgacctcaagtgatccgcctgcctcagcctcccaaagagctgggattagaagtgtgagtcactgatcctggctgaaataaaaaaaattaaaaaatatattttattgttttgaattttatttaaaactctttgcaagaaatgatgctggaagactacctgtttagaattgtaatccatatatccacaagctctggcagctttaaagagaggcaatagaagaatgaatgcccaaatgtagcagattggcttttactcattttcatagtctcctcaccctagcactggtataatatgattctgagaatgttaggcagctaaagctgtttcttttaattcttgtccactttggtgacatgaggaatcaaactcaccattttatatatttagatactgaatattctggtagctcagcaccagactctgtgaagtcattccttttgcttatctatgacttggattacattccaagtatgaattaacatacagccagactagatgaacagctttagaagaatatgacttgcttttttttttttgacaagctcatttagaaggtgatacattcttttccatgttcatttccaaatgcttatataaagaatgctgagtgaactcttgcctagtgatcttaaacattaacttacacaaagtaccttccttccttgtctcagcatgttaatacatcctgtctctcccatagatatctagggcaatgaagttgatgctagcccagttcttataacctgctgccaagtattttgatggctttatctgaagagtaggtaagatctttgctgacccagctacccagcatgcagctggatgtgtggagagtagaaatatgctggccttgtgcagatggatttcaagtacaatggccaacatttttactgtccctgctatattaaaccaaccaatttaatgccttctttctagttaagctccagttccttgaaaaatatattgtttataatatagttataatagatgtcatttattaaacacaataaatactggctgtcttttaatattttacatctattttctcagtgaatgctcaaaactataagatagacactattattgtaaacattttagagttgacagaggtgagccttagagagatcaagtaactatccccaggtaactttggtagaaagttgaaaatctgggatttgaactaaagcctatgttttaagccactatatgacattgctcccactgtaccataggttttagtagaaatgtgggtgtaggggaacttaatgatttagatgtggctattcaagaacacttcttgttcttgtagtgcattaaatttggaatatattgaatattatcactaatctctagctagcaaccaaagaaaacaagatactcagaatagcaacagctttacataaaatactttttcaaaaatattatacattctccaataccttctgtggctctgataatttgctctcataatcagttcaatccagcttgttccttaaatgcttgagaagtacctcattttactcaacatattaccacatataaagcatgtgaaaataccagattgtgttccacttttaccccaaatagtaacaaagctcctgcaattttttaagatattattaaactgtgtacaaatgctcagattaaaaaaaagtgcttacttccattgaaattggacactaccactacctattcaaattcaagttgtcattgccttgaatccatgtgtaaagtttttggtaggatagtctatttctagttgtttttcaagactcataatttggaacattctagatataagattgcattgacactttatattctttttactttataaaatggtcatccatggtttatgttacaaacgaaagcaaaaatctgggggaaagttaaagaagtagagccagataacagaattttcttttctaatatctaataaagtgaaacaaaaggatgaaaataaaatcatgataggaaggaaaaaattaccagaaactatcaaagagagagaaaacagatctcatgccattaacttaaaatgtcacctaagaaaagaaacaatagattttgtctaggagaatgaaagccttctaaacttgtctctagaaacctgttttaaccataaactagaaaatggacatattaagttgacaaaaatcttaaaaattttctcctcatttggagaaaagtagactaaatatatattctttcattttcctcttatgaaaggagggaagttgcaatggttacatttgaaatatagatgaaaaaatggaggagaagaaaaattattcactcctcgatggaaacatagtctccagggctccatgctgaagaacaatgctgatactacattctcctcaaaacaattctgaaaatttcttgactcatgaaacccagctaactcagtagttgtaattacttacttttatgatctggtttcctttttcactctaaattcttatcctcctactcttctaaataaacaatctgttttgcttcttaaatttcaaataatttatggaaaacagaactaattctttccaactgttccttttcagatccccattcactcttctctaataacaattaaaatattattttgttttttgtaaatttattacataaatttaccatttatatatctttccttgattctagactatagttttcttgaaattaagacatatacttttcctattttaatcttcaagggccaatttagcacttgaaatatagacattcaatgcatatttgttaagtgaaaatgtattttgaagtgtaatctccttttttaaagtttcacaatctttttgactgagtccttgaaagcttgtttcacttgctgatttcttaaagtatatatgaagggattcagtaagggagtaaccgaagtaatgagtacagctattcctttgttgaaagcacctccttcttttgcagaaggattaatgtacataaacatgcagctgccataagagagggagatgacaatcatgtgggaggaacaagtggaaaaggcctttgtcctttgctgggcagaagggatcctcagaatagtcctgataatgtatgtgtaagaaagtgtcaccagcaccagagtaaccatgagagtcacaacggccaagaggatgaccatcagttctaagaggcttgtgtctgagcaggcaagctccacgagaggcccatagtcacagtaatagtgattcagaatgttggagacacagaaatctacctgggtcatcaggatgattggtggtaagattgctaggaatccccccaaccaggagcagaacactagttgtatgcagactctgctgctcataatagtcaggtaatgcaagggtttgcagatggccacataacgatcataagacatggaggccaggaggtaaaactcggtagctccaagaaatatagcaaaaaaatactgagtcaagcagccagcaaagctgataactttatttcctgttgtcatgctggtcagaaatctgggaataaaaatggatgtgaaggaaatttctaagaaggagaaattccggaggaagaaatacatgggggtctggaggtgggggtctagtaaggtgagggtgataatagtcagatttcctaggatacttagcatgtaggtgaggaacagaaagatgaatatcatcacttggagttcaggttgatttgtaaggcccagtagaataaactcaccaaacatggttctgtttttcattgttgaccttcggaaaaccttgttgttcctaagaggtaaatcaaagatgagatgtgccacgtgaatctttgagtagtatatactttaacatgttttctattggcttccatccacattttacctttctcttaatagaagtatccaaacttatggaacttaaccagaaaaaagagcatattattttccattctaagaatccaatccagaatcaaatcatagttcctgagagacagagaacttcacataggtaataaaaaataaaaacaaagcccatagcagttattgaattggaagaaaatactttgagagacagaaaatttctgaaaatttatgttctaagagagattatgttgaagttcttagatggcagaggatgggcatct

SEQ ID NO: 8264 - RNA, 24 nt, Homo sapiens
  source 1..24: mol_type = other RNA
aaaaaccacaattacttttgcaca

SEQ ID NO: 8265 - RNA, 25 nt, Homo sapiens
  source 1..25: mol_type = other RNA
aaaaaccacaattacttttgcacca

SEQ ID NO: 8266 - RNA, 42 nt, Homo sapiens
  source 1..42: mol_type = other RNA
aaaaaccacaattacttttgcaccaaaccaacagcatcaatc

SEQ ID NO: 8267 - RNA, 1129 nt, Homo sapiens
  source 1..1129: mol_type = other RNA
aaaaaccacaattacttttgcaccaaactaagacaggaactttgagatctctaatcttattacacttttccgtattattctcttacaatgtttaaaatcaaaacatatttggtcatttgacctagagaaagagaattcatcatgtcttcttgcgaataactccctgagaggacacagcccataccttgtctcctgcagcgccgcatagtgcctggagcatgttaggagcttgttgggtgtgttcaatgagtggagcagacctacatctaggccttccaggtcctatctttcattacccattcatttctctttggagttctcttacctacaactctcaccttacaatttttcaatgtcaagacctatgaaatgttcattattataggcatttgcataatttatctcttattttagcatcttattcagttctttgttcatatttctaaaagtaaaatctgccgtctcattttaaagtctcttctgagcacctacctgaaagtgtttgcctcggccaggtcatcacagtcacagtgagagaaagaatagatgcctgacttcattgttcttgggagcctccatcgaatggccatgtccaactcactagacttagcaccaaatttcagttctggaggacagaaagtccaagatcaaggagctgcaggttcagctgtcttttaagagcttctcactgcttgcaagttggcactttgatgctgcatcctctgggggagttgaatgctgtgccttaaccaactgggtcatctggtcattggcgaatttattcccttgctagagcagctgtgatgtactcatttgccaaacctgggtcttgagcttagccctggagtaggagagcagtcagtgtatctaaatcactgagaattgtagttggaaaagtagtggttcctgaaagcaaactgaagtacaactaacagaataaaggggataggatcttggacttctgaaaacaactgtcctctacagattcctgcacttcctccccagcacaccagcagcatcctcactctctggcctgcctgctggaaatgtaataaagctgcttaagaacaagagggccgggcgcggtggctcacacctgtaatcccagcactttgggaggctgaggcaa

SEQ ID NO: 8268 - RNA, 3008 nt, Homo sapiens
  source 1..3008: mol_type = other RNA
aaaaaccacaattacttttgcaccaaactaagacaggaactttgagatctctaatcttattacacttttccgtattattctcttacaatgtttaaaatcaaaacatatttggtcatttgacctagagaaagagaattcatcatgtcttcttgcgaataactccctgagaggacacagcccataccttgtctcctgcagcgccgcatagtgcctggagcatgttaggagcttgttgggtgtgttcaatgagtggagcagacctacatctaggccttccaggtcctatctttcattacccattcatttctctttggagttctcttacctacaactctcaccttacaatttttcaatgtcaagacctatgaaatgttcattattataggcatttgcataatttatctcttattttagcatcttattcagttctttgttcatatttctaaaagtaaaatctgccgtctcattttaaagtctcttctgagcacctacctgaaagtgtttgcctcggccaggtcatcacagtcacagtgagagaaagaatagatgcctgacttcattgttcttgggagcctccatcgaatggccatgtccaactcactagacttagcaccaaatttcagttctggaggacagaaagtccaagatcaaggagctgcaggttcagctgtcttttaagagcttctcactgcttgcaagttggcactttgatgctgcatcctctgggggagttgaatgctgtgccttaaccaactgggtcatctggtcattggcgaatttattcccttgctagagcagctgtgatgtactcatttgccaaacctgggtcttgagcttagccctgtttagtatgaagaatattagaaaggatacaggtgaagagatgcatagggagaggtatgaaggaaggggtgcaaaggtcccatgccatccctgggtgcaccaccctccaggaacctccatgtgtttagctattttggaagctctctaaaccctgtctttttgggtttttatggagcctttattacataggcatgattgacaaccatgtagaaatgtgactggacaaaaagggtatgatgtcacactgagtggggaaaactagcaagacctgtctcttcagattcttcttgaacctgaagaaggaccctctctagaatgaggttctttgtacccacaatcagtttgtagtctcaccttgaacaggtaaaaggaggccaggagatcagagagagagagagattgtttcctggggcctgttcctgaggcctaaagcaccccaacattataacaaaagactgtaacaaaggctaagggaattacgaggcaggaactgtggatgaaaatcaatatatatattaagtcataatatcacatacggctaataagaatttttagtcccttctataattttcttcaagatactatttttgagtttggacagtaaattgcccctctttgcttgttgatgggtgggatatcacctctgggtctctggtttccggaagcctttggtacccaaggagaagaaggcaggatatggattctggctgaatccaaatttcctttccagtaccaaaatccagtcactgaaatgtattagctttgcttaggtgtgtcttttgtcctcaagcaaaactcttactgatgtgtcatgtatctctgttctatttggcttctcaaaagcatattcactagtctaacattaaagttaagtactatttcaaaaaataaagattcttcacttttcattctaaccctgtgtccagctataaatcatctatttagtctttggcctctgaagtctggagacatatttcctctacagctgatgccatccttctttttattagggacagtgacagactcattttttttttccttttgatcattttgcaaagcttcagtggttaacatacttcaagcccttcctggttcagatatataggtgttcacttcaattgtttcccttttccaaggatcaaaaccttgtgttgccagtttctcaatgtctgaaaccatttttttcataaatttagttgaggaggtaggagaacaagtctgacaccagttaccacctcacagcaagatacattactaagattttcaagtgtcttattcggatatcagagtaatgcaaaatactcaatttatgaaaaaaatagatttttaaaacttatggtctaaaagcagttttaatagaaacagaacgactagtttctttgggagttgaaaattatcatgtgaaatcctctggtccttttcttagtcatagtttttccctaatattctcatagtttttatttttacaagtttattagacttcttaactcaaaattcttcttgtatcaattttggtgatttgtgtttccttggaagtagtatccatttcacctggatttaatttgttagttcacaaagacttactattttaatttactctttaattatgatttcttcccctttcttagtcataattacttgacttttttttcctctgccatttcctcttctctattagactgtttatttacctattttattatagtcaaaccaatccccaacaggggaaaaaaatcatgtgatgtatttttttaaatttagagttccaggatacatgtgcaggatgttcaggtttgttgcataggtaaacatgcgccatggtgctttgctgcatctatcagcccacatgtgatgtagttttaaaattaattctactgtttctttgctttccatttttcccaattttttgtttgtatatttcttaattcattctttctgatgtttttctctaacttcttggttgattctttttctttttaattgaggtacaatttacaatgaagtgcacacaatttaaatgtacagttcaatgaatttgtacagtcttagttcttggtggctaagttctggcttcaatcattttgaggcttagctgtaagtcaaggctttgtgctctataatagtgcttctcaagttttttttttgtttttttttgtttttttttg

SEQ ID NO: 8269 - RNA, 57 nt, Homo sapiens
  source 1..57: mol_type = other RNA
aaaaaccacaattacttttgcaccaaactaataggatgcaaacttcggagccatcta

SEQ ID NO: 8270 - RNA, 4572 nt, Homo sapiens
  source 1..4572: mol_type = other RNA
aaaaaccacaattacttttgcaccaaactatagtattaatgaatgtgatttttaacactgtattgaaattggtcaagttggaaaagttatataactcagggaaccaatattgtctaaatgattaatgtacactattatgaaatcattgcatgggttaaaatttattcaaagtgaaaaatagataaatggatcttaataaaatcatataaaatgttatgtgattatgcagtacactttaagaaactactacttattgagttttgatgagatatcaatgaagaatactcacaattatttgaagggctgttaaaatactccacccttttccaaccgcatatttggatgaggccagtttttcttcatacccttcagtcaaaacaacttggtgcaacagattgaatgcagaagcagatatgagatccaggtgtcttatgaagccttgtgaagccctttcccacagtcattcaggacattgcagaaacaagcacacatatccaaatggaccaatttcagccaaggtccttgaagctgccagtttgactcatggttggcaaaatggtgctattagctgagagttcacttagactgtgggtcctggttcttcttaacgtgggcctctttatgggctgcttgggcttccttacaacttggacatagggttccaagcatgagcattctgcaagagcaaagtagaagcgcatagcatatttgttacctaattcagaagtcacactgcttacttccaccacataggttgaggatcccttatccaaaatgcttggggccagaagtgttttggattttggatattttgggattagcgatacacaacaacctgtactatatttgtcaagacaatcattaaagcctgcccaggattgaagggagagaacacagagggaacactccttaatggaacattgtcaaggttacaggagagtatgtggggtgggaaacattatgaccatctttggaaaacacaacctgctaccacaaataactttcctgttgagaattcacccgtaatatgagagatagtacagttttaaaatgagaatgtagaggatcttcttccagagtccaaaacttccttccctaagagatgcagattaactcagtttataatttatagtctcttcttttcataatttattgtgttgtcttttgaggagattcattgtcaaagagaccatgcctagaataactatcaatggccaaaacaaaacaaggcaaggttcagaaggaatacatgatccatctttagctagagaacaaatattcactaaaaatatgagttgccatgaaaatgtattaaaagtgaaagacaaaactaggctccctttcagtagagtcgcttgtagaatatgtaaacagtgggaagtatgagagttagggacagagaggggctatgaacacattctttgaagtcaggcaagcctgagtttaaatcctggctctgccatttactacctgtgtgatctcaacttactgttgtataactagatattatgaaacccacatgacagagctgttgttataattaaagatctatttcatgccaagtagttacagactttcctgtgcctggcatttagtaagtgctccataagcaattgttattatgtttagggaatgtagtgagtttctatgacacctactgtgtgctagcactgatagaatgctgataagaggatagatgcttgcctttaaatggttttccacttagttgaaaagctaaaacttacacaagttaaactataggaagaatattcacgtgtgagtacataccagacatcactcaagtatgttagtaatgaccaagcgtgatgctcttcataaatcaatcacatattcattgaacactaatgtgtaccttaagctgcagcagtcacaaaaggttaagtcttgacttcagtggtttggaatataacacattgctagaggaaataactaatgaataatatcaaaggtgatataattaagcattataaatgggtgtttctatctcaaaaaaaaaaaaagaaaatcagagatctcattaaaacggcaacataagattttctgtctcatggaaatagaggtatagaaaaggttaggaaagaggaaaaaaaggagagaaaattgccagtgatgacagagaaaggggaagtggtggttggaggaaaaaggataggttcattttgaagaccagattatatgatacccactaccgtgggatgcagcctgttatcgttcaccccttactgctctttgcaatggtgtctccactgaggaaaagctctttgcaattgttcagctgcttaattctttgactattgtgtgatgtaatcagattagttaatcatactggaaaccagaaattacttgggggcaacagtggccaaaataatatcgccctaaataatcatagcatgcatcttgggagagggctttatcaagtatttgacacatatgtctgtttcctagtatcccagtgatatgagtgttgttctcattgatgaggaaaactgagattcagaaatgttatataactttctcagagtcacattactcatatgtgataaggtgatctctccaactgttgtcttaggtggcttattctggcacggaagttagttcctgtcgtggggaaaccagcaaagagtattttgggtgggagggttagtcatggatagggttataacaaggggtgtgtagggaaggagcatgcagagaaggtttgacaagcaatgttcaatagtgcttggtgactgattacaaatgatgaaagagagagaaaattcaaggatgactgactctaaggatttgcacctagaaggctggaagaatgatggcaattctaagaagcgtgatagctggtaacggaacctagattggcagagaaaataattctactttagacatgtgagtttggaaaagagtagtcaacttgtagagagacgtcagtaagtcaggatgcatgtgtgagatcaggcctggatatgtagctcctcatagggcaggaactggggctcatgatgagcaagagaaagaatgtcctggaaagaagggcagcaggtgctgagcagagcaaagcttggccttgcctgttagatgtggctgtattttcaaagcctctagttctgggattctatctattgcttggcagtacacatacaaagactttgtccagcaggcactaaacttataggaagatttccccttccttccatcatagagtttttcttattaggaatctaaataatgaatctcaaaagcttctctaatacatagacatgtagctctgtttcatctctctacctttaccttgtctgaattttgctgatttttataaactttgcataatcatactgattattttagaaagaatttaagaggtggccaagtcatggcccgtaagccaaggtggcatgagagagaaactcagtggcacttggactgccagccaccaacacatttctctgcaattgtggcaagtgaggttgtaccatgtcaccaagtttcccagcccctagtcagcacagggactcaccctcctccctcctgagaatgggaaacagcccatgggcaccctcactccctcctccagtcatagaggaattgggacattgtcacaaacctgtctccagccacttgggaaaagacgagacagaactttggcatctaatttaagcaatggccaaacctcagtcagtttcaaaggcctgaatgagaatttaacgttaaccatgtgctaaaaggtttttcatttaattggctgaaagtttgtttcatggaataggtagaaaaccctgaccaatgcacttgttggtgacttttggtcctggcctcctttctgcacacaaaggagaggacagtttcaatactggcagaggagtgagcatgtgatgggtcaaccctctgcttgtcttttcagagaaatgctggttccattggtctgttctcactgcaccatggtgggacctcccaccctgtgtgggtaagatttgacagactctctgtccccagacaagcccagttggtccatgtgcctggtgacagcattgacgtcagcccttgtggtagaggaaatagttgaagcccaaagggaaaaagaggccaaaaaaagaaaaattcaatccaacaagaccaaagctatttctttttattttgtggttctcagcagctgttaagctttgctggctttcgatagtaagaaagtgtccaagaatagaacagtgcaatgtcagagttaatgggatcacagcaataaaatgtctctactactgagcaatctgatggtattaagttgatgtggaagttgctttgcaccctgcacacagagtggactccctgcttgccctcccattctgagtgttcccccaacacacctattctgagaggaaagcaaccacttctaaagtggtaaatgcattgcaaaagaagtgtcttcaggccgggcacggtggctcacgcctgtaatctcagcactttgggaggctgaggcaggtggattacctgaggtcaggagttcaagaccagtctggccaatatggtgaaaccccgtctctactaaaaatacaaaaaattagc

SEQ ID NO: 8271 - RNA, 801 nt, Homo sapiens
  source 1..801: mol_type = other RNA
aaaaaccacaattacttttgcaccaaatgaatatcatttctcagtcccaagccaatgcttctattttttgcaatgtttagttggacatctataacggccttccatgaggcagcctactgtctcccagagcatgataaggaagttccttgggttagatatctttctagcctgaaacataacaatttgcatttcagcccattgaattagacatttttctcttcagataatttctttggaaatgaaaatgttcctcaaagtgtagctacctattgggtcactgaagctttaatattagcaggtttgctggttcgctgtcttcaagaatagtggatattttgccacaaagggagaataggaagccagagtggaaagaggggaacaaaaacagggatagatacaagggaagaagatagacggtattagcatttactaccccatcattatatgtaccttgatttgttcctggagttgctgaaggatggctcagtttcccctttcttgtataattctttgattcagttgtagtctgacttttgaaagctgactgggtattggtgatggaaagcatatcctgaaattggagatagcaagactcttggtgaactgttgagtagactgggttgaattcagtgaaggatcaggcagcaggacacagcaaggccagccacggcacagcctcctcctccaccatctcaccaggctccctgccagggccggcgcagggcagcgcctgagctactagggagtctggtccggctgctgctccgccgccgccgccgccttctcacagccacaacaaca

SEQ ID NO: 8272 - RNA, 1650 nt, Homo sapiens
  source 1..1650: mol_type = other RNA
aaaaaccacaattacttttgcaccaaatgaatatcatttctcagtcccaagccaatgcttctattttttgcaatgtttagttggacatctataacggccttccatgaggcagcctactgtctcccagagcatgataaggaagttccttgggttagatatctttctagcctgaaacataacaatttgcatttcagcccattgaattagacatttttctcttcagataatttctttggaaatgaaaatgttcctcaaagtgtagctacctattgggtcactgaagctttaatattagcaggtttgctggttcgctgtcttcaagaatagtggatattttgccacaaagggagaataggaagccagagtggaaagaggggaacaaaaacagggatagatacaagggaagaagatagacggtattagcatttactaccccatcattatatgtaccttgatttgttcctggagttgctgaaggatggctcagtttcccctttcttgtataattctttgattcagttgtagtctgacttttgaaagctgactgtagaaagaggaatatttagaaaaataggcaaagtgatgttatggtttaaaatcatcaagtgggaaatccaaaaccacggttctcaaccttagctactcatggaaaccacctgggaaatttttaaaaatactgatggatgggttccatgcccatagatttttaaaaaattcttccaaaggattctgacatcctaatcagggttgaaagctactgctccaaagagcttgacataatcaaatgaacatttatcaggtgttcacaaggtttaggaaggcccagcacaaagcaaaaccatagagacgttgagtactcttttgcttcagcattcagcatccaattccaactccatgcttttccttacttccaacttccatctttgccccgagcaacctgtgcagaaaaccatcagtttccctgctccactggacatctaaggactatggtggtgataaaaaatgagagtcatcaaaaaggtccaagtttagtgaagatgtgcaaagggaagcagcccttcccaaagaattcagtgaatgagccaagattctccagaaaccgctcagctttgcagtgataattttctgggtattggtgatggaaagcatatcctgaaattggagatagcaagactcttggtgaactgttgagtagactgggttgaattcagtgaaggatctaattattaccaggtcaggaagatgtcctgctgcacgctcaggcggtcactcctcctttccacaaggcccatgtccgcaccgttcgccccggggctcccatggcccccgacctccagtctccggcaacgatggaccctcacagacacggcagggagcgaagggcgcacactcacctcccaggcagcaggacacagcaaggccagccacggcacagcctcctcctccaccatctcaccaggctccctgccagggccggcgcagggcagcgcctgagctactagggagtctggtccggctgctgctccgccgccgccgccgccttctcacagccacaacaacactgcagcagcgaccacacagagcgcgctcccgacgccgagccgggcgacgagcggggacgcgctcgcacgctcgggcgctgaacccggt

SEQ ID NO: 8273 - RNA, 1745 nt, Homo sapiens
  source 1..1745: mol_type = other RNA
aaaaaccacaattacttttgcaccaaatgaatatcatttctcagtcccaagccaatgcttctattttttgcaatgtttagttggacatctataacggccttccatgaggcagcctactgtctcccagagcatgataaggaagttccttgggttagatatctttctagcctgaaacataacaatttgcatttcagcccattgaattagacatttttctcttcagataatttctttggaaatgaaaatgttcctcaaagtgtagctacctattgggtcactgaagctttaatattagcaggtttgctggttcgctgtcttcaagaatagtggatattttgccacaaagggagaataggaagccagagtggaaagaggggaacaaaaacagggatagatacaagggaagaagatagacggtattagcatttactaccccatcattatatgtaccttgatttgttcctggagttgctgaaggatggctcagtttcccctttcttgtataattctttgattcagttgtagtctgacttttgaaagctgactgtagaaagaggaatatttagaaaaataggcaaagtgatgttatggtttaaaatcatcaagtgggaaatccaaaaccacggttctcaaccttagctactcatggaaaccacctgggaaatttttaaaaatactgatggatgggttccatgcccatagatttttaaaaaattcttccaaaggattctgacatcctaatcagggttgaaagctactgctccaaagagcttgacataatcaaatgaacatttatcaggtgttcacaaggtttaggaaggcccagcacaaagcaaaaccatagagacgttgagtactcttttgcttcagcattcagcatccaattccaactccatgcttttccttacttccaacttccatctttgccccgagcaacctgtgcagaaaaccatcagtttccctgctccactggacatctaaggactatggtggtgataaaaaatgagagtcatcaaaaaggtccaagtttagtgaagatgtgcaaagggaagcagcccttcccaaagaattcagtgaatgagccaagattctccagaaaccgctcagctttgcagtgataattttctgggtattggtgatggaaagcatatcctgaaattggagatagcaagactcttggtgaactgttgagtagactgggttgaattcagtgaaggatctgtaatcccagctacttgggaggctgaggggagaatcgattgaactcgggcagcagtggttgcagtagccgagattgcaccattgcactccagcctaattattaccaggtcaggaagatgtcctgctgcacgctcaggcggtcactcctcctttccacaaggcccatgtccgcaccgttcgccccggggctcccatggcccccgacctccagtctccggcaacgatggaccctcacagacacggcagggagcgaagggcgcacactcacctcccaggcagcaggacacagcaaggccagccacggcacagcctcctcctccaccatctcaccaggctccctgccagggccggcgcagggcagcgcctgagctactagggagtctggtccggctgctgctccgccgccgccgccgccttctcacagccacaacaacactgcagcagcgaccacacagagcgcgctcccgacgccgagccgggcgacgagcggggacgcgctcgcacgctcgggcgctgaacccggt

SEQ ID NO: 8274 - RNA, 4375 nt, Homo sapiens
  source 1..4375: mol_type = other RNA
aaaaaccacaattacttttgcaccaaattcatacttcatgtataaaccagataattacaatttcttatgtgcaatcatttcctttaggggttgctacaaggaagagtaaatactgttttactagaggaatggcgctaaattgctcttacgacaaatcaatgtgttatctgcataatttgtaatatgttacagctcatggttaaagtagagcattcccattgttgggaatgacagttggtggttcagctgtgagtggaaggggagtgttaagattggaggtttctcactcactgtctgctgagaaatccccatgccgggagccttggccacatagctacctacagaccatactacagagtgttgtctttcctttcctctctgttcgagtgaatgatgcttttctctaaaggaccacttcttccttttttgttggtaggtgggggttgtggcatagagggaaggtgggagcctggtcaacttttcccaaataataatgttggagtagattgaaaatttagcactatgatctggatcatctttcagaaaggttgatgtatttgacttgcagtttaattgacatcgttaacagaaaatattgaatgtcttgattcaaaatataaactgcaattattttgcacaaacctagtaaaaaaaatacgtggcaagttgttctgtgatgccatcagttttctgatagtgtggctttgaatgtggcaatgctgttaaagttttactttttaagaatacttagaagtcatggtaaaattaaaagaatgaattccaatttttattatataaattgttgaaaataaaaaaatgcacaattttgactcaccgtaatttactggataatttctaaatactttgtcgatagaatcatgtatgataatttgtttgaaagaattttaggatcaaatatcagatttggttttaaaaactctgggcgtatttattgtctaaggagataaagacatttatttcatcaacatgactcactatatgtaataaatacttcactaggtggcactgaaaaacccaaaccaaaccaaaaaaaaaaaaaaaaaagaccaagtgtgatgaaaaatggtcatgaaaatgcagggttcataccctgctgtcatgttttcccatcacatatcccgtgggcttcaccaacgtggcctcactcagctgtcctgtttcagccacaagcatcacctactatctgtgcagaaatcaactcttgaatactagtgtatattttctgctattgtttgaaaacagaggaatacatcttctttctattgcgtttttcttgcttttaacagtagaatagtacctttttactagcaggttgttaacacatatttgtccactagatgggtatttcattttttttttttgagtgttgtcttcattctttatacacttcaatgtttaatatataaatatattttaatttccccctagcttcccccactgctttctttatacatacaaatatgatgcataggtctggatttcctttttaattcaatgcctggggagttttttcttgggactattccagagtctagttgttcgttcattctaaaaaacacagggaggatttaccacatcagaaactacatttaatgttggagatccaaaacctaacatagggacccatttgaggagagcgtaggaactgctggctggggaaacacctggactttcacagagcattgaggagcagagctgattagaaatagcatcatgattggctttgtaaagaccaaagaaggagaaaggagttggaggtcaagatggcacagttaagaaacagtatggttgacatggtttaatggtaatgtggtatttgtatacattgctctgcatacaattatgttattttaatatgcattattttatttatttcctacaagaactccatgaggtgtgaacaggaggtgtcagcagatcatttcataagcagacctttagtagacctggattagagttgccttcaggccccggactggaaccttggttttctgacttgcattatttcttctaccacactaatattctgttatttgaggcaaccacaattgcatattctgtctgcatgtgtgtgagtgtgtgtgtgtgagagagaaggaaaactagcaacagccatcctacactcctcttatcataacatatgtgtttcaatatttactttattatgagttttacaccttctgaaccagtgtacttaatacaaaagtaggaaaattcatctggaatgaaaaaaacaacagctacaacaaaaagtcactttgatgaagcagcagcccaggctgagtctattatgtatacagtttcagaactgcaaaagagataacgtaaaaaccaggtatggcaaatgatttgagggtcaatctatgtttgtttttatatcccttgctcccacagaagactgtgaacatgtcaagtattaaggacctattttgaattactaaatagacgagatcattaccattagcaaaaattagcaccaaaggatgtataatgagaattattttggcccactaccacccaccaaaaggttggagtttctatatctgtgaattttgcagctctgcagagcttatgaaaacctgctcattttgtcattaacacaagccctactccttagtacttgggggactttgaacatgttcttaacttttccatttccaggttcttccctagtagagcaaggataacagcaatgtccttatttgtaggatccttaggattatggaagtaagctcctggagaacacgtagccagggcatggttccctgaaaaggatctattagtgtgtgctattcttactgttcttatttctgcagtccttgccacatcactgctaccaggactccttcatgaaggatggagtccaactcccaggcacgtgtggatagggtaggggttggcctgctttggtaaagtgagatgataacagatcacacagcaagacgggctgcggacagagaagaaaatccgaacctatagtcagaaagggtctggttccacttgctaaattctgtctcttatcaaaagacaggttttgaaaattattgcaacagaattatcagttatgtgagctttgagagttcttcatttaaaaagatacctcagatattcttaattaatccattttgtgtcttgccattttgttctgtaatttccttgctcatctgattgtgggtgagatttgtaatgaactttctgatacataactatattataccgttttaacgctgctgataaaggcataccggagacttggcaattaacaaaagcaagaggcttgattagactcacagttccacatggctggggaggcctcacaattatggcagaaggcaaggaggagcaagtcacgtcttatgtggatggcagcaggcaaagagagagaatttgtgcagagaacctcccatttttataaatcatcagctctcacgagactcattcactatcacgagaacagcccaggaaagacttgcctccatagttcaatcacctccccccaggctcctcccacaacacatgggaatcatgggagctacaattctagatgagatttgggtggggacacagccaaaccgtatcaatgactccagaggtttttcacagttcacttgattttcaaaatttaataaaaactaggatacaaaaaggcaggctatctgggaactttcataatgatcccttaaaatgtacacatcttctcatggtgtgcctgccatggcgtgcaatttgacctgacagttttcccaggagctaaagcgctgagttttctcctacatggagcttgagtaaccatacagtaggccacccaggtgcttggttttcctttcacacttaagtatccagtgaagagctttctctaatctatgccttctgttcttatgagctatgtctattgaaatgtttggcttataccagaggagggcaataaaataggcaacttttcttcgcaataggacctgagggccacctttttctaccataaagttaccttgcaattctgttatttttgtctctttatttttgtatccatcaatgaaataaaaagcattactctatcatatcatgtatcactgctatagtagacaagaaggaaacattcattcattaaatcttcgaagtagaattttcttatataaatgcatattcttcaagaacaacataaaatgcagcaggtatatgattctttaaaaatacaaataatacaggctattatcgatgttttgttttgttttttctttttctattttagccctgcttaaaggttcttaaggcttcccagctcatcttcccatttcctatctttactcatttatctggaaggaaaattcattcttccttcacagctatgtcttga

SEQ ID NO: 8275 - RNA, 29 nt, Homo sapiens
  source 1..29: mol_type = other RNA
aaaaaccacaattacttttgcaccaacat

SEQ ID NO: 8276 - RNA, 2807 nt, Homo sapiens
  source 1..2807: mol_type = other RNA
aaaaaccacaattacttttgcaccaaccaatataaattgtaacagatttgagacaaaatataaaatttttcaaattgagcagaatttatcaacccagaatctataatgtatgaaataaattaatagagaacccaacagatcatgttatgttgtaaatataacatctatctttaggttaaagtaacatagcaaaaatatatatttatgggtgcaagacacatacataatttgtaccaatctcacagaactaattcaattcaaaacaacaaaaaacttactctattatctaatggatgcaataaaaattaaccatttgaagataagttctcttgcacttcccctacttacgtttttcctggcacctgctatactgtgtatgtatttcttcaccgctttactgcctgactcccctactagatcataagttccaagagggcaagccctctgaaacactgctatgtctccagcacctagaacttggcatgtagtaggcatccaatacataagtgttaaatgagtgaatttaaaacacgtacatgccaggaatggtggctcaggcctgtaatcccagcactttgggaggccgaggcgggggatggcctgaggtcaggagttccagaccagcctggctaatatggtgaaaccccgactctactaaaaatacaaaaattagctcttcctttctctgccattgtggtgtgtgcttgactctgcttcttgccatgtcttctcataagacttccaggattaagtgattcctgaccgagaaattaaaacaaaatcgccccactccccagtggattcagatgaaaactggtaataaaatcaggtacaactccaaaaggagacattgaagaagaaccaagctagccctataaggaattgcacatgagagggcacacatatttatgctgtctgaaggtcacagtcatgttaccacatcaagctgaaaatgtcaccgctctctggagaattgtacatgttttattgggaatatattttttctttctgaatctgttatgaatgcattggttggctgggttcagtaataaatatgtgagacctttcattaaaaaaaaatacaaaaattagctgggcatggtggcgcacacctgtagtaccagctactctggaggctgaggcgggagaattgcttcaacccagaaggcggaggttgcagtgagctgagatcgcgccactgcactccagcctgtgtgacagagtgagactttgtctcaaaaaacaaacaaaacatgcacacatttaatcaatataaaatattatttctgcgaagtcacttcaagctgatactgcatactccatatatgctaaacttcacaaggtctttacctcatacctgactctctttcctgaccccctgcggggtaagtcaatgccctggggttgcttagccacttggtactaccagctttgggcaccaggtctgtttcagctcattggtgtatgccccggctggcttttcccatagggcagagttgcacaagttgtgggtgtgaagctgagaggtgagcagaggaggaagggaggtagacagtcctcatcccagtgtccctctgaactgccgcgtgtgttgctccagcttctcagcctccgcctggaggtgccccagcgcggcagggctggggtacgtgagcacggcattcttagtggccagcgctacgtccttgagcaggctgcagaggtgactgctgccacggaggatctcgttgcgcacgtccctctcctgggtctccatgcacagcgtgtccaccagcttctgtcccaccatgatgaccagcttgctctgagtgatgatctccgcgggctggctgctgctgaggctgccgtgaaatgcgctgatggctttgaagagcgccccaaagtagagccggcagtgttcagataagcggggtttcctctcaggagtctgttgactcgaaggctgaggtataagagggccaggattacttgcttggctgtctgggggatggagtcctgccttcttggggctggctggtatgtcatataactgctgcttctctggctccttcaggaccacggggccccggtgctgggtaggcacgtcatacacctgggaaggcagagtcggcagtgaggcccggacaggtctgggaagcgtgaggatggcctgttttggaaagctgagagtcttttcacagatgattctggcactggtgggagggtcggggaattcatagacttgggcagtagggggctggggcccctccgcccaactcctcatctgctcataaacggggcctggagtgggagggcggggtagagtgggcacctgataggtctcctctgagctggcaggagcttcttccaggcctctcaggaatggggggcacggcctgtctgcagcgacctccgtgaggatttggaggcggttggcaggggccaggccttgcctcccatggagcaaacacttccaccaaccctcgctttctggcacgtgttgctccagaatggtcaggatgtcccctctgctgaaagccagctcgtcagagcagtcagggcagttgtcataaagtgccctggccaggagtgccttgggcgcacagtccatgatgcctgttcccttcatgtcggtgatgtggagcagctcccctgagctctgcagctagtatctccagcttcagaggcagattgtgcaatgtcactgcatgcttctggctggttctcagaaactgaattctatggagctatctgacaacacatgggaaacgatcaaaaagactctcccagcaggcaaactttctggaaagcacgataagagtaaaatg

SEQ ID NO: 8277 - RNA, 3956 nt, Homo sapiens
  source 1..3956: mol_type = other RNA
aaaaaccacaattacttttgcaccaaccaatataaattgtaacagatttgagacaaaatataaaatttttcaaattgagcagaatttatcaacccagaatctataatgtatgaaataaattaatagagaacccaacagatcatgttatgttgtaaatataacatctatctttaggttaaagtaacatagcaaaaatatatatttatgggtgcaagacacatacataatttgtaccaatctcacagaactaattcaattcaaaacaacaaaaaacttactctattatctaatggatgcaataaaaattaaccatttgaagataagttctcttgcacttcccctacttacgtttttcctggcacctgctatactgtgtatgtatttcttcaccgctttactgcctgactcccctactagatcataagttccaagagggcaagccctctgaaacactgctatgtctccagcacctagaacttggcatgtagtaggcatccaatacataagtgttaaatgagtgaatttaaaacacgtacatgccaggaatggtggctcaggcctgtaatcccagcactttgggaggccgaggcgggggatggcctgaggtcaggagttccagaccagcctggctaatatggtgaaaccccgactctactaaaaatacaaaaattagctcttcctttctctgccattgtggtgtgtgcttgactctgcttcttgccatgtcttctcataagacttccaggattaagtgattcctgaccgagaaattaaaacaaaatcgccccactccccagtggattcagatgaaaactggtaataaaatcaggtacaactccaaaaggagacattgaagaagaaccaagctagccctataaggaattgcacatgagagggcacacatatttatgctgtctgaaggtcacagtcatgttaccacatcaagctgaaaatgtcaccgctctctggagaattgtacatgttttattgggaatatattttttctttctgaatctgttatgaatgcattggttggctgggttcagtaataaatatgtgagacctttcattaaaaaaaaatacaaaaattagctgggcatggtggcgcacacctgtagtaccagctactctggaggctgaggcgggagaattgcttcaacccagaaggcggaggttgcagtgagctgagatcgcgccactgcactccagcctgtgtgacagagtgagactttgtctcaaaaaacaaacaaaacatgcacacatttaatcaatataaaatattatttctgcgaagtcacttcaagctgatactgcatactccatatatgctaaacttcacaaggtctttacctcatacctgactctctttcctgaccccctgcggggtaagtcaatgccctggggttgcttagccacttggtactaccagctttgggcaccaggtctgtttcagctcattggtgtatgccccggctggcttttcccatagggcagagttgcacaagttgtgggtgtgaagctgagaggtgagcagaggaggaagggaggtagacagtcctcatcccagtgtccctctgaactgccgcgtgtgttgctccagcttctcagcctccgcctggaggtgccccagcgcggcagggctggggtacgtgagcacggcattcttagtggccagcgctacgtccttgagcaggctgcagaggtgactgctgccacggaggatctcgttgcgcacgtccctctcctgggtctccatgcacagcgtgtccaccagcttctgtcccaccatgatgaccagcttgctctgagtgatgatctccgcgggctggctgctgctgaggctgccgtgaaatgcgctgatggctttgaagagcgccccaaagtagagccggcagtgttcagataagcggggtttcctctcaggagtctgttgactcgaaggctgaggtataagagggccaggattctgtccacagatatttgccctatttttctttaatagttcagaagagtgttcatcttccctttgcttagtggaaggggtactcttttggtgtgattcagtttctctttggggaggctggatgtatttttcacacttaaattctgcatttggggtcaactgcacagtctcttccttttcacagttccgcttaaaaaggagccttccattggcaatgacaatggaggcaaacctcttgatgtcttctggaagcatccgtgccaccatgacaaacctctcaaggtcatctgggctgttctggacactgtcagtcacaagaacttccagaggccaattgcgattatccaagctttcctttgtttcaagcaggatgcggtaggagttggagatggtctgcatctggtcccgaattctgttctgaaggttactgtcagtgaggttacaggcagtcccatggactcctcgggcaaaatccagaaattctcttacagattcttctatgtgatcagtggacctgtggattgcatcaatgttggcctccagatagtctcggaatctccacttcctgctgacaaagagcatcaggccagcgacagagctgaccaccttgtgctgcagagccatcactgtctccttggccacatccaggtccaaggagagctcctttgctgactcctccgaggaagagctggaggagtcgtcggtggatgtggtggagcacgaggaaacgatgctagctctgctgtcagaactggaacctgataatctgtccggttcaggagatggggaagttgtccgtctggagaaccatgaggaattatggcccgcggaattctctgacacctccttggctttctccagctccttcccagcctgagaaacactcgacgttgctttagggatgtcataaatattgggcttggtgttctgctgttccactcggggaatcagaaagcttgaaggaaccttgtagctgacatcttcatccaaaggaaatgtgcctctgggtacaagaaagccataagaaggaatttctggaaggctgagttttttctgcatgggcacattgttattcagttgtggagtgagggacctggatctgccacttggaggattgtagaaagtggagctggaactggggagagcgtggggccttgattcttccgcaaagctggtgagaggcgtgtttctgacgctggcctttcctggagacactggagtgtcataaatccattccgatttctgaggatttggtaatgtgctgtaaccgcctcttcttaaggtagtcactgatatcaggggaacaccctgcccacttgcttggctgtctgggggatggagtcctgccttcttggggctggctggtatgtcatataactgctgcttctctggctccttcaggaccacggggccccggtgctgggtaggcacgtcatacacctgggaaggcagagtcggcagtgaggcccggacaggtctgggaagcgtgaggatggcctgataggtctcctctgagctggcaggagcttcttccaggcctctcaggaatggggggcacggcctgtctgcagcgacctccgtgaggatttggaggcggttggcaggggccaggccttgcctcccatggagcaaacacttccaccaaccctcgctttctggcacgtgttgctccagaatggtcaggatgtcccctctgctgaaagccagctcgtcagagcagtcagggcagttgtcataaagtgccctggccaggagtgccttgggcgcacagtccatgatgcctgttcccttcatgtcggtgatgtggagcagctcccctgagctctgcagctagtatctccagcttcagaggcagattgtgcaatgtcactgcatgcttctggctggttctcagaaactgaattctatggagctatctgacaacacatgggaaacgatcaaaaagactctcccagcaggcaaactttctggaaagcacgataagagtaaaatg

SEQ ID NO: 8278 - RNA, 4118 nt, Homo sapiens
  source 1..4118: mol_type = other RNA
aaaaaccacaattacttttgcaccaaccaatataaattgtaacagatttgagacaaaatataaaatttttcaaattgagcagaatttatcaacccagaatctataatgtatgaaataaattaatagagaacccaacagatcatgttatgttgtaaatataacatctatctttaggttaaagtaacatagcaaaaatatatatttatgggtgcaagacacatacataatttgtaccaatctcacagaactaattcaattcaaaacaacaaaaaacttactctattatctaatggatgcaataaaaattaaccatttgaagataagttctcttgcacttcccctacttacgtttttcctggcacctgctatactgtgtatgtatttcttcaccgctttactgcctgactcccctactagatcataagttccaagagggcaagccctctgaaacactgctatgtctccagcacctagaacttggcatgtagtaggcatccaatacataagtgttaaatgagtgaatttaaaacacgtacatgccaggaatggtggctcaggcctgtaatcccagcactttgggaggccgaggcgggggatggcctgaggtcaggagttccagaccagcctggctaatatggtgaaaccccgactctactaaaaatacaaaaattagctcttcctttctctgccattgtggtgtgtgcttgactctgcttcttgccatgtcttctcataagacttccaggattaagtgattcctgaccgagaaattaaaacaaaatcgccccactccccagtggattcagatgaaaactggtaataaaatcaggtacaactccaaaaggagacattgaagaagaaccaagctagccctataaggaattgcacatgagagggcacacatatttatgctgtctgaaggtcacagtcatgttaccacatcaagctgaaaatgtcaccgctctctggagaattgtacatgttttattgggaatatattttttctttctgaatctgttatgaatgcattggttggctgggttcagtaataaatatgtgagacctttcattaaaaaaaaatacaaaaattagctgggcatggtggcgcacacctgtagtaccagctactctggaggctgaggcgggagaattgcttcaacccagaaggcggaggttgcagtgagctgagatcgcgccactgcactccagcctgtgtgacagagtgagactttgtctcaaaaaacaaacaaaacatgcacacatttaatcaatataaaatattatttctgcgaagtcacttcaagctgatactgcatactccatatatgctaaacttcacaaggtctttacctcatacctgactctctttcctgaccccctgcggggtaagtcaatgccctggggttgcttagccacttggtactaccagctttgggcaccaggtctgtttcagctcattggtgtatgccccggctggcttttcccatagggcagagttgcacaagttgtgggtgtgaagctgagaggtgagcagaggaggaagggaggtagacagtcctcatcccagtgtccctctgaactgccgcgtgtgttgctccagcttctcagcctccgcctggaggtgccccagcgcggcagggctggggtacgtgagcacggcattcttagtggccagcgctacgtccttgagcaggctgcagaggtgactgctgccacggaggatctcgttgcgcacgtccctctcctgggtctccatgcacagcgtgtccaccagcttctgtcccaccatgatgaccagcttgctctgagtgatgatctccgcgggctggctgctgctgaggctgccgtgaaatgcgctgatggctttgaagagcgccccaaagtagagccggcagtgttcagataagcggggtttcctctcaggagtctgttgactcgaaggctgaggtataagagggccaggattctgtccacagatatttgccctatttttctttaatagttcagaagagtgttcatcttccctttgcttagtggaaggggtactcttttggtgtgattcagtttctctttggggaggctggatgtatttttcacacttaaattctgcatttggggtcaactgcacagtctcttccttttcacagttccgcttaaaaaggagccttccattggcaatgacaatggaggcaaacctcttgatgtcttctggaagcatccgtgccaccatgacaaacctctcaaggtcatctgggctgttctggacactgtcagtcacaagaacttccagaggccaattgcgattatccaagctttcctttgtttcaagcaggatgcggtaggagttggagatggtctgcatctggtcccgaattctgttctgaaggttactgtcagtgaggttacaggcagtcccatggactcctcgggcaaaatccagaaattctcttacagattcttctatgtgatcagtggacctgtggattgcatcaatgttggcctccagatagtctcggaatctccacttcctgctgacaaagagcatcaggccagcgacagagctgaccaccttgtgctgcagagccatcactgtctccttggccacatccaggtccaaggagagctcctttgctgactcctccgaggaagagctggaggagtcgtcggtggatgtggtggagcacgaggaaacgatgctagctctgctgtcagaactggaacctgataatctgtccggttcaggagatggggaagttgtccgtctggagaaccatgaggaattatggcccgcggaattctctgacacctccttggctttctccagctccttcccagcctgagaaacactcgacgttgctttagggatgtcataaatattgggcttggtgttctgctgttccactcggggaatcagaaagcttgaaggaaccttgtagctgacatcttcatccaaaggaaatgtgcctctgggtacaagaaagccataagaaggaatttctggaaggctgagttttttctgcatgggcacattgttattcagttgtggagtgagggacctggatctgccacttggaggattgtagaaagtggagctggaactggggagagcgtggggccttgattcttccgcaaagctggtgagaggcgtgtttctgacgctggcctttcctggagacactggagtgtcataaatccattccgatttctgaggatttggtaatgtgctgtaaccgcctcttcttaaggtagtcactgatatcaggggaacaccctgcccacttgcttggctgtctgggggatggagtcctgccttcttggggctggctggtatgtcatataactgctgcttctctggctccttcaggaccacggggccccggtgctgggtaggcacgtcatacacctgggaaggcagagtcggcagtgaggcccggacaggtctgggaagcgtgaggatggcctgttttggaaagctgagagtcttttcacagatgattctggcactggtgggagggtcggggaattcatagacttgggcagtagggggctggggcccctccgcccaactcctcatctgctcataaacggggcctggagtgggagggcggggtagagtgggcacctgataggtctcctctgagctggcaggagcttcttccaggcctctcaggaatggggggcacggcctgtctgcagcgacctccgtgaggatttggaggcggttggcaggggccaggccttgcctcccatggagcaaacacttccaccaaccctcgctttctggcacgtgttgctccagaatggtcaggatgtcccctctgctgaaagccagctcgtcagagcagtcagggcagttgtcataaagtgccctggccaggagtgccttgggcgcacagtccatgatgcctgttcccttcatgtcggtgatgtggagcagctcccctgagctctgcagctagtatctccagcttcagaggcagattgtgcaatgtcactgcatgcttctggctggttctcagaaactgaattctatggagctatctgacaacacatgggaaacgatcaaaaagactctcccagcaggcaaactttctggaaagcacgataagagtaaaatg

SEQ ID NO: 8279 - RNA, 4220 nt, Homo sapiens
  source 1..4220: mol_type = other RNA
aaaaaccacaattacttttgcaccaaccaatataaattgtaacagatttgagacaaaatataaaatttttcaaattgagcagaatttatcaacccagaatctataatgtatgaaataaattaatagagaacccaacagatcatgttatgttgtaaatataacatctatctttaggttaaagtaacatagcaaaaatatatatttatgggtgcaagacacatacataatttgtaccaatctcacagaactaattcaattcaaaacaacaaaaaacttactctattatctaatggatgcaataaaaattaaccatttgaagataagttctcttgcacttcccctacttacgtttttcctggcacctgctatactgtgtatgtatttcttcaccgctttactgcctgactcccctactagatcataagttccaagagggcaagccctctgaaacactgctatgtctccagcacctagaacttggcatgtagtaggcatccaatacataagtgttaaatgagtgaatttaaaacacgtacatgccaggaatggtggctcaggcctgtaatcccagcactttgggaggccgaggcgggggatggcctgaggtcaggagttccagaccagcctggctaatatggtgaaaccccgactctactaaaaatacaaaaattagctcttcctttctctgccattgtggtgtgtgcttgactctgcttcttgccatgtcttctcataagacttccaggattaagtgattcctgaccgagaaattaaaacaaaatcgccccactccccagtggattcagatgaaaactggtaataaaatcaggtacaactccaaaaggagacattgaagaagaaccaagctagccctataaggaattgcacatgagagggcacacatatttatgctgtctgaaggtcacagtcatgttaccacatcaagctgaaaatgtcaccgctctctggagaattgtacatgttttattgggaatatattttttctttctgaatctgttatgaatgcattggttggctgggttcagtaataaatatgtgagacctttcattaaaaaaaaatacaaaaattagctgggcatggtggcgcacacctgtagtaccagctactctggaggctgaggcgggagaattgcttcaacccagaaggcggaggttgcagtgagctgagatcgcgccactgcactccagcctgtgtgacagagtgagactttgtctcaaaaaacaaacaaaacatgcacacatttaatcaatataaaatattatttctgcgaagtcacttcaagctgatactgcatactccatatatgctaaacttcacaaggtctttacctcatacctgactctctttcctgaccccctgcggggtaagtcaatgccctggggttgcttagccacttggtactaccagctttgggcaccaggtctgtttcagctcattggtgtatgccccggctggcttttcccatagggcagagttgcacaagttgtgggtgtgaagctgagaggtgagcagaggaggaagggaggtagacagtcctcatcccagtgtccctctgaactgccgcgtgtgttgctccagcttctcagcctccgcctggaggtgccccagcgcggcagggctggggtacgtgagcacggcattcttagtggccagcgctacgtccttgagcaggctgcagaggtgactgctgccacggaggatctcgttgcgcacgtccctctcctgggtctccatgcacagcgtgtccaccagcttctgtcccaccatgatgaccagcttgctctgagtgatgatctccgcgggctggctgctgctgaggctgccgtgaaatgcgctgatggctttgaagagcgccccaaagtagagccggcagtgttcagataagcggggtttcctctcaggagtctgttgactcgaaggctgaggtataagagggccaggattctgtccacagatatttgccctatttttctttaatagttcagaagagtgttcatcttccctttgcttagtggaaggggtactcttttggtgtgattcagtttctctttggggaggctggatgtatttttcacacttaaattctgcatttggggtcaactgcacagtctcttccttttcacagttccgcttaaaaaggagccttccattggcaatgacaatggaggcaaacctcttgatgtcttctggaagcatccgtgccaccatgacaaacctctcaaggtcatctgggctgttctggacactgtcagtcacaagaacttccagaggccaattgcgattatccaagctttcctttgtttcaagcaggatgcggtaggagttggagatggtctgcatctggtcccgaattctgttctgaaggttactgtcagtgaggttacaggcagtcccatggactcctcgggcaaaatccagaaattctcttacagattcttctatgtgatcagtggacctgtggattgcatcaatgttggcctccagatagtctcggaatctccacttcctgctgacaaagagcatcaggccagcgacagagctgaccaccttgtgctgcagagccatcactgtctccttggccacatccaggtccaaggagagctcctttgctgactcctccgaggaagagctggaggagtcgtcggtggatgtggtggagcacgaggaaacgatgctagctctgctgtcagaactggaacctgataatctgtccggttcaggagatggggaagttgtccgtctggagaaccatgaggaattatggcccgcggaattctctgacacctccttggctttctccagctccttcccagcctgagaaacactcgacgttgctttagggatgtcataaatattgggcttggtgttctgctgttccactcggggaatcagaaagcttgaaggaaccttgtagctgacatcttcatccaaaggaaatgtgcctctgggtacaagaaagccataagaaggaatttctggaaggctgagttttttctgcatgggcacattgttattcagttgtggagtgagggacctggatctgccacttggaggattgtagaaagtggagctggaactggggagagcgtggggccttgattcttccgcaaagctggtgagaggcgtgtttctgacgctggcctttcctggagacactggagtgtcataaatccattccgatttctgaggatttggtaatgtgctgtaaccgcctcttcttaaggtagtcactgatatcaggggaacaccctgcccacttgcttggctgtctgggggatggagtcctgccttcttggggctggctggtatgtcatataactgctgcttctctggctccttcaggaccacggggccccggtgctgggtaggcacgtcatacacctgggaaggcagagtcggcagtgaggcccggacaggtctgggaagcgtgaggatggcctgttttggaaagctgagagtcttttcacagatgattctggcactggtgggagggtcggggaattcatagacttgggcagtagggggctggggcccctccgcccaactcctcatctgctcataaacggggcctggagtgggagggcggggtagagtgggcacctgataggtctcctctgagctggcaggagcttcttccaggcctctcaggaatggggggcacggcctgtctgcagcgacctccgtgaggatttggaggcggttggcaggggccaggccttgcctcccatggagcaaacacttccaccaaccctcgctttctggcacgtgttgctccagaatggtcaggatgtcccctctgctgaaagccagctcgtcagagcagtcagggcagttgtcataaagtgccctggccaggagtgccttgggcgcacagtccatgatgcctgttcccttcatgtcggtgatgtggagcagctcccctgagctctgcagctagtatctccagcttcagaggcagattgtgcaatgtcactgcatgcttctggctggttctcagaaactgaattctatggagctatgtctcaatgcctgacgtctcactttgtctgtaagtagagactgtcactcatttgctatgtgaaaccacaaaagaagaagaagaagaaaaaaacaccactcttctgctttatagggcgaagttcctacttcgaagagctcagtgtatgaacacacagcattcttgtcctttgaactctgt

SEQ ID NO: 8280 - RNA, 31328 nt, Homo sapiens
  source 1..31328: mol_type = other RNA
aaaaaccacaattacttttgcaccaacccactacatcagaacctacctttaagggttgatttgtgggttaaataagtgaagatatgtaaagactttaagtaatgctctcagaagatgttaactattagctggtaccaggcattttgggagtagataggggatctgctgaatgttggcagaatgacccatccctagagcagacattgtctatcaatacccattctctgcttcttccttgctaacatcaattatttctgtagatatctgaccttcatggaagatgacctcatctctgggggaaaatactattgaaagccaatcacaatgccattctcagtgtcagtggattggcatgaggtgggtggttctagccaatgagtcataagaggttttttgttttttttttttttatttggggtctcactctgtcacttaaggctagaatgcagtggtgtgatcgtagctcactgcagcctcaaattcctgggctcaagtgatcctcctgcctcagcctccctagtaggtggaaccacaggcgagagccaccatgccccgctcattttttatattttttgtagagacagggtcttgctatgttccaggctggtcttaaactcctggactcaaacaatcccccaaccttggcctcccaaagtgttgagattataggtgtgagccgctgtgcccggcctagaagaggattcttgaaggacttctgggaaatggttccttcattccttagaagaaaacacagaagagatgctcctgttcttttatgaatgttatctctgggtgtgatgcctgaaactgcagcagcaggaaggcaggcagtctgagagcacagctgacctaattagaatggcaaggaagaaagatggaaagaattcaggccccttaagaggtctcagagttgctgaatcaccaaactcctgggcttacctactcacgtactaatgttatgaaataaaataaattttcctcataatttaattcttgtccagagcatcctgattcatatagccagggaccatagttacacatatttttacttcctccaggacctaacaactggtgttgtgtgctatgagcaaaggaagagcagtagctggaaatgaataacctgggtaggacacaggaagactcaaaaatgttctaggctatgcaaatcaaaaccatgagatagtaatatcacctaataccttttaagatgccattatgaaaaaacaaaacattacaagtgttggagaggatgtggagaaactggaacccttgtacattgttggtgggaatgtaaaatggtctagtcactatggaaaacagtatgaaggtcttcaaagaattaaaaacagaacaatatatgatccagcaatcctacttctgggtatttatctaaaataattaaaagcagggcctcgaagaaacagtcacactcccatgttcactgcagcattgttttcaacaatcaaggcgcggagccaacctaaatgtccctcaatgaatgaacaaagaaaatgtggcatagccatacaatggaatgttttcagccttaaaaagaaaattctgtcacatgctgtaacgtggatgaacctggaggacattatgctaagtgaaataagccagtcaaaggacaaacactgcatgattccacttatatgaggcgttcaaagtagtcaaactcacagaagcagaaagtagaacagtgattgccagaggctggtgggaggggaaacgaggagtggctgttcaatgggtataaacttttggttatgcaagatgaaaaacttgtagcagtctgctacaaagcactgtgctgcttctagttaataatgtaccgtctcaaaataaataaataatgtactgtacacttaagagggtagatctcacattatgtgtttctttacaacaataagaaaatcaccttgtaaactggaaatttccaaaatggaaattggagtagcttgtattgattttaaaatttatacatgctctcactcataggtgggaattgaacaatgagaacacttggacacaggaaggtgaacatcacacactggggcctgttgtgaggtcgggggagggggaagggatagcatcaggagatatacctaatgtaaatgacgagttaacgggtgcagcacaccaacacggcacatgtatacatatgcaacaaacctgcatgttgtgcacatgttccctagaacttaatgtataataataataaaaataaaatttatacatgctcctaggctcagatttaggaatttattttccatttaggttttattaagtctaatccaacaatgcaaaaatgaaactgtgagttatatgtgatgaaaaagtatagctttcttgaattcaaataagcaatggcaaagatcacatttagaatttgacagaaagaacacagcatccctgcctcgtcttttttatagatagtaagaaaagggaaagtagtcttatttcaaatatcaaaattctgacttaaatgaataaaatttagtcacgagtaaatacaaaaaacaagcaaacaataaaaccttcctggatcagcacaggcccaattcttccctgccttttatcaccctgtcagctgggagtatcttttctacctgtggctctctaccaattgttactctcttgttgtctgaacctgctagccaaacttggcaggtcgttttcaaagccagatgagttctgattgttcccttggcaatatccattatttccctcctgggtagaaggaggatctgaggacagcttatctttttggggtacgtggagtagaggtggggactcttatataatacgaaataaaaataagttctttgggctggaagtgtcaaaagattccttagaatttatagccacagggatttcatggtgtgtctgatgtactgattttgtgccacatttgagccagaactggcagcagattcaaagcaacacaggtggctaagtacacatgaggggaaggtaggtatggggagagaaaagtggcataaaacaaggctgtccccctatgctcatcgagaataggatcttagccctcactgaaggagcttaatgatcagctctaatacattggctggactcctgcaggtactcacggaaagtagagatgctgagctaccttttcttgtcaaagtctagggctggagatgcttcaagaactttggagccataaagtcactgtaatggtcaacttttaaggctagaagaggccatgagacatctcattcatctccttgcctttgggcaagaattgcacacctaagcctcccgaatacatcagacacaatttagggttaaaagcctccagaggggcaaaaaagtaaaaagattttacaactttcttccacaaaccactttaattgtgtgctcatcaccgacttcagaatctaagagaactttgacacttgtttttgacaccccattgccttctcatcagtctaactccaagaccttcctccgagtggtaggctctggtaattcagcgaaagcaaggcgctaacaggcgagtgtgaagccaaagggctcccagtgacatccttgacatctttttgccagctattcacatgcatttaatatacagcacttccctgtgactgtctgcagccttttctaccagcaattcctcctgatttatccttctccagcaattcccagttgccttgcctttctaatagatgttgcagtctgacaaaacacctttgccttcatgctggtgttgttaaaggactgattataaccgtaaggaatgggaaataagaagctattccttgtaagtttgctaatcttatctgttcagaataataaaagttctctgtcaaagacttaggaagggagatttcatcccccagccttgctagtcctactctttgtgcattcttaagacaggaggcaagtgctttccattctccttggaaaaactgaggctgaatatgcagcttgtcatgcagttttgctgaagacagagagagggtcaaaaattcaaaaactcaattgctctagggcagggggttgggagcaaagccaataaataaaatgggtggtataaatgcctttcaggaaagggtgtgaagggtggggtggatttaccagaagctttggcagtcagctttgaagtcttctggaaaggaaagtgtagcctcccaggcaagcagcctcatgacatcttccataaggctgatgtgttgggaaacagcaacacatgagcaagaagttccttgaaaaattttcttccctccttcttcttctggaactgttgggaaactagattagacccaggagtctggtttttgagaatggccctgaatgaatttttagtttccgggtaggaacagagagctgagaaggttgttttctcctccaaggaaatctggccacagtttttttcctgttctatctagagcttgtgtgctggtggattaagcacatgtgtgcacagggccaggattctggcaaacaatctcagggaggatggcaaaaggagaagcaaaaggggttcattcctctacctcacagcttcttttcccaaaggaaacaggatctactcaccagcaacaatcccaacatcacaaaaggaacagggaaataaacgtgcatacaactgggacacacagacccctgtcacctgctacaaatggagcagaagtgggagagaagtgagccaccgagaacctaggccttcttagctgtagcctacttgaagagggcacgggcttcctgactggtctctggtggccgagtaactctacttccctgacctgggaagaaggcgtgaataaccagctaagaggagacacccatcctcttagagttgcctggggtatctgaggcagaggtggtagcagcagactcctcaacagaggcactgagatccaagaattccaggatgatgtccccaaggcagtaaatcaaatgcctgaaacgaatggacaaaaaacttagggtctggctcaatcaggaaacacaagatcctgtttatgacatttattttctcctcccccatcaccgacaccctaaacttcaatagcttgatgaaacctctgccatgaaattaatgttttttgaactaataaagcctctgaccctaataaaggcaagaacagtttttatataagactagttttatataagactaagttttataaaattccatttctctttacatagttacattagcactgctctgaagaactgtgataacaaatccttgagatgtcaggttactagacactttcagagctcctgactactgctgtttctcataattaattaccttaaatttataggctgccttacaggcagtgaggtaaagccaggatccttgaggaagttaacgaacacagtctactttggggtagggtttgagtgcaaggttactcaatacttccagaagagtaacagcccaagggatggaatctacctcttctggattattctaggactcttcacccagcatttctggtccctttatgaaattccaaccttactatcttgtctacctgatatgaagcaaagacaactcctggtcttgacatgaatcacagctttgctataaggccagggctcatggtgaacatctttacatggtctgtgatacacaggccagggtacgctcttggagcattcacaggggctggcagatgttggaaagagcactgagcaagtatgctgaacaagcctggaggataagaggtcattttcagcagctcatgtgggggcctgcatagagttcttccaaacacaaatggtgggtggtccaagagtgatttcctagcacatgacgacctgctcagaagcctgatggtgtggattttacttagagtgtgtggatctggacgtcaaactctgtagtcagtgcccagagcaagtaaagactacaatcctattctttggaatgtgggcttttcactcagaaaccttggatacctctgagaccagaggtggctgtaactatgctgatgttggaataacattttcccacttacctgttgatgaggggttgttgtagtgactccaggactagaccccagctcagccggcatttgttcaccccaagaatttctactacgagatctgaggaggaaaaaacagatggaatttgcgtgttatcactgaagttttagattctaaggacagtctctccccaggatctctgccgtttttacataggttaggtatttcaggcctacctctaaaccatacagccaaactaaaatcctcacaaaacaggaaaaacctgagaaaaatatgtttctcaagttaggtgtctacataagaatgggcttcaaaaattattttgtaacctgtcactcaaatgcaggtactccttccaatgtaacagtttaggttggcaaacagagttataataataagggtaaataaaactgattgtccagagctaagttcacaattgtttcctggttatcacagccataggcaacaaactgccttcctggccctctaaaaacacaatgcaaggaaaaacaaccttctcagattttgttttaacttattgctaaaggccatgtaccatactcaatggctgcaatttattaagttggagcttctgtgagacatgtgattttcttccttggtcccaaaatgctatgaattggtagagaatctgaagtcttcatctcctggaaatggctctgagacctgtccctgcaggcagagcttccccagacctgccagcaggtagagagaaagttattaacctaaatatctgcaggattgtcacctagtatttagggtgcagctgtagagttcctttccattcccttggcatcagctgagcaatggataaaagaattgcagccctgttcattttcctattagcctgggaaatgatgggtcaacagagttttgaatctagccacattcagggcccttttacaaacaggaaaaggtgcaggggtaatggtggcaaagcagaatggaagagaaatgtgattggtataattgatctcattggtccaattacctgggaggactcccatcaggctctgcaaagcctgtttctcagcagccagtttctgctcttgggtccttacgggccgtggaaacttaggcaaaactccaccaggccagatggactcctgaagaagcaggaggtactgcacccagcgctgtggacttgttaaattagctacctgcacctctagccacctgtggtagaagagagacgaaagcttagataaagctgaaggaaaggaaataacaaggcagcggactgactgtttatgttcccctgcagattcgtgtgtcaaaatcctaaccctcaaggtgatggcagtaggaggtggggcctttggggaggtgattaggtcatgggggcaaaggtaaatgcccttataaaagaaacctgagagagacttctcaccccttttgccatatgaggacacagggagaagacagctgtctatgaacaaggaaaagggcccttgccagacaccagttctgctggtaccttgatcttgaacctcccggcctttagaaactgtgagaaataaatttctgttgtttataagccattcagtttatggtattttgttatagcagcccaaacagactaagataccatgaattacatgagcaatcagaacaggacaaagtcagcactgactcttgcaaaggaaaccaagacaattcaacagcctgggataacagaatttgaagatgagtaacaataagaatcgtgttatttatggagcgttcactatgtgccatctaccgtacaagaagttttacagaacagaacactaaaagggcctccgtctctgggtgagcctgcacctataccttcccaactctcctctggcaaggctgcacctattatctttctagctctcctctgatgggaagcattataaccttcttggtaacatgtacacacagacttcacagctacggacttagcgatctttaaacaaattcctctctctacctccccagccatatcttctggtcctcatgactgtcttagggatttcctacatctgccctttgttcataatagttctctcactaacaagggcctcttctcgccttgcctgaagagcaagtctcaagtctgcccttctggcaagacctgtttcaaccctacttcctccatgaaatccttgaccatcacagctggaagtgctctccttctccatagacctcctttggcaggtagctctggaacaattactttggaatatgcatctttttaaaggtgtttatagctttacttcttcaactaaattataagctgtaagagttctgtgtcttgtactttaaaaaaactccccgccgtgcttggtgctcaagaaatggttgactgactgataactgttcttatttcaatgaaaaattttccctttgtcttactttcgaaaatgagtcaaaattttccctttatcttactttcaaaaatgagtcaaaaatgagggggaagatataccaaatctggagttcagctggaaacctagaaagtggttcaacgttattcttgatctgttcctgaatttttttcaaagtgatatggtcagaagtgaggttcaaggctgttgaggcctccccttcacccacctcatttaagactgacatagctgtgtgggtcatggatggacaatcaaccacttctattcatgcacggaagactcgtttgatcctgcaccacatggcagctcatgccatcactcctcgctcctatactcgagtcacttgtcactcatccaagagcagagggggctgccaaggcaaactttatttaacctccactctgccagacagtctgcattccactcaagctgggcattccagccatgagggctgcaatcccccaagcccaaggctcacaactgattctaagaataggaagtgtgtaaggtaatagcagggcaagaatggcagccatcgatggagatcaagagtggcacaaagctgttcttgtccaaaatagccaacacgatcgtatttgttattattagggccgcatctcctttttatagggcttttcattcagtgagcctaagatgcctgatgaaaggaatccagtagcaagaattcctgttcctgtttatgtaagagggtcactagagggaggtggctgcaatgacctgatcggcttctctgcaggggattaagtgacccaaggtctcctttcttcacctcaagccatgtatacttctgcaatttttgctgaggagaatgatgtgtcttagggtctcatctaactgtcttgagggagaggggcaaagtcttgcaaactaaaatctttagccacatgatccttcctagactgaacatgttgtaacatgccagcaagcctaggtacctcagccatcttctggcatgtcttacaaagcaagagttacattcttttgaatgaacattaatttatctgatggggacaggacctcacatggcattaggacaaggatatcctccttgttctcttgcatggtgattaagtgtctcatgtacatgtgtgggatgcaaaatgaattttatcatgtggcaaaatataaatttataaacttatacaaatctataagacagcttttcagactctaaatggaaatgttggggagagacataaaagtaggaaaagtaaaaataagcacctgatgatgaagatgagtctatgagtcaaataaatttgtggaagctaataagcacaactcaccgaagaaaaggagtgccatctctgagtaagtatcagctgctgatgagacaaagacactgtcaagcactgtacatacaaggcacagaactggccaacaggaggccctggaaaaagtcaggcccaggaatataagaaacaggactttcacaaactggcagaaataaactccctccaggcctacaaagagggacagagtttggaaagtgacttctagtccctgggagctgcagagtgccagctttccttattcttctccacactctgaagataaaagacacaaaccacacacttgcaccacgcatggtttaaacatttgctctctttcctggattctcctcttgcctacgttctgcccacccttccccctgtcagcaaacagaggctttatcctaggcctttgggctcagcatggtcttatttcctagtcccaggcagcctgtgtagaagaccaagtgcaacaaatctttcttgttcacagaacttctgagcgatggtgtctcgttaaaaatgatgagcacgccaatctggaaggaaaacatgataaagagcaaaccaaaaaaatcaccaccacaactgccactgccctcacacaatacaatctctaaattttttaagctgtaattcaatttctaagacacactttattatcactcactatgcctttcttaagttgtaaatggctgtatattcagggatttggtatactttgccttgcccaacacctggatggaaccaactgccactggttcttgagagcaatgaagaaggtggagatttcttcatccaaatatctttcctctccctttcatccctaccttcccttcctttggttctatcatccttctctaaggtaaagctccatacacaccaccatttcattatctaactttattaactcccctaatcatgcttgatttatttggaaactggctagagcacggaagacaaagacattaggtgtaggattgttaaaaggggcagaagtctcaactcctctccattaactctcttcatctcgcgatttctacactgcatctttctattcttatcataggagtgggaaggttaaaaagagattcgtaaccctatagagctctctttaagtggaagggatggaatttatgtgtctgaactctaatacatcataggaggttttccagcatcagtttctggactttgctggtaccatttactattaggctgacagaaatctaaagcttcaaggtcaacacacacacacgtttctcttactattcattagaaattacttataataggccgggcatagtggctcacacctgtaatcccagcactttggaaggctgaggcgggcagatcacctgaggtcaagagtttagaccagcctggccaacatggtgaagcctcgtctctactaaaaatacaaaaaaaattagctgggcacggtggcgcacgcctgtagtctccagctactcggggaggctgaggcaggagactcgcttgaacccaggaggcagaggctgcagtgagccaagatcacgccactgtactccagcctgggtgacagagggagactccatctcaaaaaaaaaaaaaaaaaaaaaattacttataataaatcatttactaaatacaaatgctcttgttcatgtaatacaagatgcatgaagtaaatatgctaaaataaatatggtagagaatagcctcagatagcactggttttattttccactactattccaggtctgatatttgatttagagatatctctttctattatcctgccttcatcccaaagaagagaagaaaaaagaacccaaaccaggtctcttgtgtcaagccatctctgaatgattcagagccttaatagggggcctagaaatagccagtaaaatggccaaaaaaccccactccacaaccacattttgaccccaagacattcaagagcttcccttatgccagacaggggagaagaaaggatgtggagatcagggcttgtcagtagctgggactgcacatccactccatgttcaagggaacctggtctgaaatagccgcagataggggaatgaagcaatgactaaaaaggagacagtttaatactagggcttaagatggcacttcaaggttagtagaaggtcatttcccatcaaaacagcagaatcaaatctcatgagtaaggagaaggctttagagaccatgtctaatccaattagccaaatccccttcatttcttttctaagacagcagctatggctgagtgagaaagggtcttgaatcagtatggcttaatgaagaggagaaagggaagaagatactaaaatcataaaacagaaaatattcataagatccacaacaatattctaaacaaaaatgcctggtgcagtctaaatataaggaaaataacaggtccattccttccagcctatttatctattggctgtacctctatagacaatccaagggcaattatgctccaaccttaagataccaaatacagttcaaaggaaaagagaaagaaaaggaagatcaagttaaagcttctatcatcctaagtacaccttcagtaaattagaagtattgacttattttattaccctgagagcagggttttcaacgttggtactactgatattttggactgcgaaatctttgtcataggggctttcctgtgcattataaaacattccacaacatccttgcccctcctcccctcaaactagatgctagttttgccaaccaaacatgtctccaaacattgcggcatgtcccctgaggacaaaattgctccagttgagaattactgccttagacccagggacttttggatataattgtatcaggctactttcacagtcattttaaacctcatggttgtagcgcaatgtttttcgacctgtgggctggacatcattagaggtcatatcatctgttttgttgtttgtgataacataaaaaggcatctcatgtttggagacacttgtttcgtatgtatgtacatatatatgtatatatcagatctgcgtgcatgcatatgtgtgtatgcgcctgtgcctatgtgcatgctcacagtgggctgcaacgtacaatgcattttttactgtaggttgaagttttaaaaaaagtttgaaaaacactcatgcagtgtcaagaattaggagttccgagagaaagtaggagaagcccaagccacatttttagcttcctggaaatgctccccatctccacccacccaagcaccctgtaaaatgtttgcaggggcctcaaccatgaacactgtgttctgtactgccagtcctagcacataagtatgagtattggctcatccaatcagtagcagcaatctatagggtgggagagaaaggaggtcttggaggtgatggtgtagattcaggacattatccattaaacaaaatgtttttgcccatttcacacctgataaaagttatacttcttttctctctgatgccgttcccaggcctctgtcttcctgccatggccccttcttgtgtttatagacagtttcccctgtcagctctcagctctaggcttctgtcctgtaactatccagacccaagttactcagctgtgtctgagaaagttcaacactgctgccctctgactgtgtatctaggtcaccatcctttcctgcccagtgctggggaagaatgaggaggaaatgaaccccgagggcaagaaactaccacttctttctcccaatactactgtgaaatctaaaatggctcagagttggcacaatttcttctctgatttttgctttcatgttttaaatcatggatccacatctttgaatcatgtacttcaagggaagacttgacattctcctaaataccacaatataagaatctgagttccatacatttatatctagccacaaacagtttttgtttttgattagtaatgtacacatcacagatataaaattaatatgtattaaaaaatggaaggattcttaaggaaggaacttcaaaaaatcatctgttcaaccttagtggtttttccaatctcaccaactctacatatgaaagcattgggcaccaaaaggaaatattttacatcaagtggcttataagaacatacaacttgagagttggaaggaaacttagaggttattttatccagtctcctcccaaagcagaaacctcctctgtaatataacggcatagacaagggttgggtcctgtgaatccagaaacttgggcttttatcttagttctgctacccaattagcaatgtgacctcaggcaagtggcttaattccttaaaagcataatctaaattcattgaagatgcttcttaaaccttgccaacccaaatcggcctccttgtgttaatgaattctagtcattggtcctagttctactctctggagttaccagatattaggttaaatctcttccaaaagacaacattttgcatttttaaattcagctattatttctcccctatgtctcttctacatcccatacatccgtgattttgccaacctcaaagacactcaataaatgtctgatgaaagaaggagagaaatgaaccactcctcaacctggctccatcctctgggtgtgctgcttagcttttcttttaaaatgatgtgcccagaaccaaacagctctgagatgtgacctgaccagcaaagaacataggggattgagccttcctttagatttagatactatacttctcatacagccgaagattgtgttagctttttggcacacacgtcaaaagcactgactcatattgagttttcagccagctaaaatcctaagtccacacaggtacattacaaaaaaaaaaaaaatcgtgtgcccctctgttaagtatagtcttgcccttctgtatttgtgcaattaaaaaaaaatctaaattatagttcatcttgttggctttagattatcattctaagttttctaaatgtttttgaatcttaattttcatcatctagagttttaactactcctctaagattagaattacttgcaaattttctgatgaaaaaattgatcaggataagatgaagagcagtgctctattactagaaatttccctctaggatggcatcagtttatgatattatttaatacccttgggctaaagacactcgactagccacaaattacttaaatgtactataatgcaggcaacatattccattctgtccatatggatattatggcaaaaacttgttggaatccatacacaatgtaactacaactgcatgctaatcaggcagggcacactcctactgaacccataatggtttctagggttccccattgcccttcccaaatgttcacaaacatctatttcgtcatctgcttcagaaatttccagaaataaatgttggggtcaagaacctttaaccattttttaaaaaggcaagatatctgtgcatctctaacccatatggacaaatggcaatgtttcttaatgaccttaggtctttaatgttaaatataaatttgttaagtttcatgggatataattcatctaggccatgtacaggtttaaatgtacaaactttaaaataggttacgtgctctattattattttcatttctattttggtcgccaattctactttaatcatgtctgttcaattcttcttgctaggccattttccttgacaaagaaaatagaaaacagcctagcaaataatagacccattcattcactgctgaatgaatgaataaatgctttcaccatgtaatcagttgatactacagcatctgtcccaaacaattacctacatatattttttcttgttagtaacatgtgacacgtgtatgtgtttttcacctaagtcttttcccttaatatttatctacaacctcagctccttctgagttgaagcttactggaccctgttcttactagttctattactactatttttgcattgttcagtatgtgtcccctctttctgtttttaaaatatgttcacctagaatctgatcgcagttaactaccctggtttcatttgatgctgactctttttcttcctcattggaaatgggtgtttaatttgttcattcatttactcaaagcattggttgagcttcttgtaaatgccccccgaccccccagaaaaagactcttaaggttttgaaggcagaaatcttatgtaattcattttgacatctcctttagcatttaatagtgtcattcacaaataaacaatcaaatatttactgaatgaatcgatcctgttgcaaaactttgagtgataccttcaggcgtgaattttaagttaatctgttcttacagcatgtaaaacagtttttatctcattctgttacgctcctgtgaattccagtactctcatctatctctgctttcctttctgtgtcagctgtttttctcaatatccagttttaactttatctgaatttttttgtcaatgtcttactcttcactgggttgatggtctgctgacaaacacattctttctactatttttgagttgtattctgtctgtggtcagaagttcaccatgtgaataatcatacgtcatggcacagaaaatttaaaaaccttgccttggtaccagctacaaggttagctattcattctctgttttcatttttcttctaaagaaacttacagatagaaaaaaagttgaaaatataatctgggccttaagttttctactaaaaagaatctcaaaattattagagatacagtacaggcttctctgggtgcatcattgatttttatataaatcagagtagatactaatctattactttagtaagcaacaggattttaaccacaaccccaatatgctgttcagaaagatattaccccatctttttagttatgcttctcaatctgcaaggtggaaaactgtgtgagtcattcttgatttgtctttttctcaaccctaatccaacaccacataatcatttaaatagtcactaaatataggtgatcctacctcctcaatatctcatgaatctattacccctttaccatctctatagcaatgatctcagctgaatgcctcatcaccttttctatcaatgaaactcctccctaatttgtcttcctgtttctaactttggccccttcaattaattaatcctccacagcactatttaaatgatttttctcaattgcaaatttgctcatgtcatcatctgtttatgttttgtaaaattgtttcctatcaaatgagtgacaaatgttttgttcttggaatgactcacaggagtctgaatgagcagactccctttaaactcttcactgttatcatcagccattattcttgcatatcatatattcctaatcaatcatactaacttctttgagtaccacaaatacactatattgttttactgctctgccttgaatgttctctctctctctcactgtccgctggcaacgccccacattctttaaatctcatctctgatgtcatctactataagccttccctgcacctctcataattgataaatcccttctctgaatcacatatagagttcttttcaaagcactgattttatactacaactcctatttataagtttgcacctccaattggatatcacacttcctatggtagggatttgggtcttttttttttttttgtattttgatcacttaacgaagtgcctaccacagagaaagcaatcaataaatattggttactaagtgaattcatgctgtatatgggacaaacactggtcttaaagcatggcacacagttcaaaataggttctgcagaaagcatacatcccaatacttacaacagcaaaaacattgagctcttaattattcatgcttacagaggaagacaattatagattttaaaaaatcatggacaatataaaaatcctttatatttggcattccatatatgtttatatacacgtctgacagatttactttcctaataatcttttgtttaggctaataataaaatgaaactgtgggctaatacaccagcgatagagctgatgttgtaacgggtatgctaggtaataagtcaggtggtctagaactaagaataatccatgaaatgggcattcacacctggctatgcattcctctggaagggaagagagctggaaggcaagggagtgggtcagccatgctccttatctcacactataaatcctggaggagagagacagctgccagtagcttatgtttggtcaattttcctgggaaataggcccagaggatagaagagattgaaagtcaaacaaaaagcaaaggggggttatgaggactatgagtcacacttgtattttgggaagtgcctctgacggatggagcagcattgaattgattccaacccattatttgaaactagtaagaagaaaagaagagaggaaggtagcagaatgggggaggaaagaccaaaagcaaaggtcaggttacctttctaacaaatgtagaaagagaaaaagacacttggggtctgtgtatttttaggataaataagactgattgtaaagggaaagctctaacaatttctatatttgagtattgtgacatgtttaagatttcattctgaaagttttttcttttttttttttttgagacagtctcattctgtcgcccaggctggagtgcagtggtgcaatctcggctcactgaaacctccacctcctgggttcaagtgattctcttgcctcagcctcccgagtacctgggactaagggcatgcgccacgatgcccggcaaattttttttgtattttcagtaaagacggggtttcaccatgttgatcaggctggtctgaaactcctgacctcaaatgatccacccaccttggcctcccaaagtgctgggattacaggcatgagccactgcgcccggccaatctgaaagttttctatgcacaaatctagtgtgcctctgaagtctttcaagtcaacctttttttggccccatactatgttgctaccgacatactataatccagttctgagaaaatcaggactgacagactttaaaaatgacactgaaaagcgacagacaggtttgaacctggcttaaccacataaaagttgaacaaactctctgagctctggcttccttcattataaaatgggcaaattcttgccttgcctttttcacaaagttatcatcaagatgaaataagaaaaataaaaagtatttctaaaagtgcttgtgtgtttgcacatgtaaaagagaaaaagactacttcagaccttctgtaaaaattcaaccaggttcagcgaactaatgatggcaggatctggagtaagctttgcatttcatgcctcagttttctcacttgtaaagcttactcttcctggcaggctcagggaagtaaatactgaaaccagtaaagcatttggtactgagcagttaagaaaattgggacgaggcctcagggggttttggataatatgaaaactctatttccgaatccttcctaaaaccagacctccatgtaccaaccaataaaactttcactgcagagactataggatccaaatgtctctgtctcttctttccttgtccccgtgtgaacagcaagcctggctcattctcagtccccaggtagttatcctgagcctgcctttctcagcagcaagggcaagggcagagaggtggggtggggaagggggaaggtaattaaaatggccacccattcagaagaaaattgagtccgtggaggggaaagggcagggagagggagcaaaacccttagtgctgaagcaccaggaagaaaggcaagacacaaaagagggaagaaggcagtaatttagtggttgtcttgacgaccagagtccctattgttcatgggggctttacctcacagggagatctccctgttctgctctgcacatagaactcccaccacaggaaaggaggatgggaagggaagggttgcaggaggcagaagtgataagtaattatgtgctcgcagaaggggctgacctccaaatttctgcaaatattacggataacagatttagagtgtgctcagccatgatttggaagaaaattattagggatttatttaaatcagcagacatgggaggacttcaaattatgctgtgaaaatggctacaggaggctggaaaagaccagccttgaggagaataaagaatacatatatgagaagcagatgcccaagataaacaaagagaaaaaacactgagaggggtgtagaggagaaggaaaagtgactatcattaacaccatcaccttggtgtagaagagctacccaaaagtatttccagttccctgtctacaggctgaaatgtaaaacctttccaagtagaaggccatctatcccgttatgaaggacgtagggacaccgaagtggcaactccagaatctccacagaataggaactttgggagcactgactatgggtagaaaacacagaggagtaataaataaaactggaaaaacaacaaaaaggaaacctgggggagagaggaggcaggtgttgaggaacttaccttgatgctgcatttgcacaccagcctccctcccaggaaggctgaatcctctccgagaaatctttcggggccagcattatattagagctaaagtatatttcccaccaatttacccaactccctccctgctccagtaccaaatagctctacttctccaaagggcacttggagaagcctgcaaggacagaggtaaagatcaaaagtaagcaataacatatggttgcttctccaaaaccaagttaatgggggagagccaaacggtctccatccatggccgaaagcaatagggaatgtccttgattatgtaacaggttgataagattcctaacatcggggctattcagcactgacaatctccatcttagtgaatacataatgtataagattttaggatcacaggagaccctgaatataggtccaagtagtttatacagaatattaacaaaattcttgcaattcagatgtctagctggtctcatcaccacagactctgttctgctcactctgttctgaatgaatcagctccagcactgaatttttaacgggtgggatccactcaaaggggcaacttctggtcatccacaccactcagagaagcaagcatatgctgaagacgcattagagcagaaggaagaagggtgaaagatcaaagaaacagggcttatctaaaagtcactggcactaaggagtaggcagataagtggcctctaaaccgtagagcaagccagggaatggcttcaatatactgtatcaacatcacggcaggggacctataactgcaaaacaaacaggtcttcctcaaaggacagtgaatggtattgtttaacctgcagcgccacctggtgcccatagagagaattcctgtgcccacgccatgcagcagcagtttggtaggctttttgtcacctatttgaaacaataaaagcaacacacattcagaaagaagctggctaaaaatattccaggttgctttttatttgaaagtagaatgcccctcctcctgttttaaaaatgtcttagtgtctagaatattatttagcctaaaccagtctaaatgacacctatctcacaagatctagctgttataccttcctctataaagcctctctaacatttacctctaaattatctcttatccccccaaagaacttcatgcactaggctatgatttctatttcgacagtaacagacaaaggaagttaagtggtttgttctaagtcacatagcctcaaagcaagatctgatttcagatctgacttcaaagtccaagttcttgctttccatgtggaaggaaagaggtggagaaagtacaacagcaggagatgcttccagagagggcaggctcggtggggcttcatactgggaggcccaggttgtggaggggcgctgcactctttggaaaggagagagccattagaatgggagatggcctgaagggcccccaaacctctttgcttaggccgtaccatggctctgggaatcagaattccccaattaactgaagatctgggtatgccctgtgtggagggaatgaaagactcagtttccattttgcttctggtcccccagcactgttgaggaaaccctaagattcttaatagtgataagcagagggactgcctccagtagaatgacgtgtgatcttctgtgttcatttatttgacacaaatttactaggtgccttctatgcatggggctgggtgttgaagatataatggtaaataagacgcagtccctgccctcaggatgctgacatacattctaaagctgtcatcaaaatgtcaaaatcttaggttcctgtttgcagtcacagatgggcaagagatgccaagaacctgacttggaaaaaaaggctctgaggtttaaatacctcatgatattctgttttttgttaacttttacaatgagcaattttgtacctctatttgagtatatgagacttcaagagcacacacacacagaaatgcaaatgcaatgctcaggcacacggctgtcagctgccatccacctgctacaatctcaaagatatattccagtagagactgtcactatgtgacaggaaagccatgatgtcttcatcctaagatgggtgtagaataagtgatacccaagaaatatgacaggcagaccactcatatgacaggggaaactgctagggcccatcctggcccagtctatagaagtcaagagcttccctttggcatggcctaatggaagaggcctgggacaagcagtactccttcccagggagccacagtacaatctgagcaaagccatcaatgagaaaaattaatttcagcacctctaaaaacagcccaagccaatgactggagagccagaaaataagcgagaattctgaagactgagcttgagttaattttgtatgtgggggtcttgcaaaagtatgcgtatttctagaaaagctgtgcataggaagagatggggtataagacatagccaggcatcagagctgaactggaagaaaaagttacacagcaaaggaaaaaactgtaatctatgcttcctgagaaactctgagtcttaacgttgataatcttttcctgattgtgaatagcatataaatagagatagctaagagacaatctctggctcagaagtgctttaaaaataaaatcagaatatgcagacaaaaataatttatatgctaccatcagatgcgtgtgtccctgagaccagctggatggaaagcaagagaggctagatgggaatacggcaagggaactttcaggtgaacccagttctagtggccactgctttgtgggaaagcttgcatggaggggaagcatggcagagcagtgggaaacacatgagctctgaggccaggatgacttaagtggaatcttaaggtgtggttgttacgacttttatgattttgggaacgttattttatctgaatgtaattttcttcacttatgaaatgtagaactacatgtctatctcatagaattgaacattaatataaacagtacatagctgctttcctggtattaatattgtaataagcgtcagttcctttcccattgcaattactcgtgcacttttggtggcagacctggaggttctcttaagaaataaccaatgtcacaaagaactgttatccacctgctagttagacatgcccaccaagaaagaggcccttgaagtagagttccacagaaagcgccttgattctggagcgttctaagagaacagtggaagcaagagggttcatggtcaacctttcccaactgtccttaggggaggtggacgttgcgccttgcagcacagcactctccagtgctcccagactctgccgcagctctcctgacctttcctaggagatggtttagagagagacatcttctctaagaaagtgattccaaggtctggtgtaaggtctagagcttgccatcaagtttctcctgggtgccctgcttgttggactccttaaacctgcacaccctttcttttcttcttcctctctggatacttcctaactttacacacttcacgctcccctctgccagaacctttccccctggctttctgccaagccattccattcccacatgcccccaacactcacacacacacactctgtctctatcttacacacacacacacagacacacacacacacactccctttttaactgagaaatcctgacgcagatgccaggaatgtgtctgctgcccttttgacacaggtctgatgccatcgttggggccatggggagggcagcgccgcggacgtggcattcacgcattctgctgctggcatggttcctatttttatcgtggcattgctctgggtgtccaggcagggcgccggtccagcttctcattccttcactttccatcaggactccacaccaatcctaccccttaccttggctggatcttcctgccccaaaccccctaccatcaatgcagcacagtgtatctctcctctttccctccaacccagtctaactctgagtacttgcccagtttgctaaatctgattctgatgtttgcagagatattttcaagtttcttctgttttcgggcatgagcagagtttgcacaagccggatttgctccttggctcagagtgctacccgctctccccttcccctccctttgtctctcattccaaataaggagtgcttcttgttacataattggatgttcccagcacagaagctgacacatgaggttaggcgcacatgcatgcaagacttccctttgacttaacaatgccttttttgggcatctaacttctcttcagctcccctcccacttctctccacatcatcaacaatcaacggagatttataagcctggctcagatcagagctcttccaactttggcttagaaggaggggttatgaggtcgaacttactctgttttttttttttcctttgcaggatagagagtgtgcttataatttgacagaagtctatggcgtccaaggcagtaatgtacacaggtcttttaaagttgcaagatgggtatacaaagttggaagcagaggaataaacttgcctgcttggggataataatactggaggttggaacatgaggacattttaaggaggagatgcactcaaatctggtgactacagcatccctgatggtcaaactgcagtgagttctaaataactagagaagtggcagtaccacgtgtggcaccaacaccaactatcctgctcttttaagcacggaacttaaaggaagagaacccaagtaccctgcaaaagcatatggctcagctacccgtggtttcagggaggacaaacatgtagcctcctaggcagcagtcatggggatgggaggcaacgggacctcatatcatgcctcttgtgggagatgcagggggtacagtggagaggtgctgcagctctggagatgtcaagtttccagcatattggcttaccaaagcaaataaagctgaagcatgcagcaatgcatacaccactttttaaaattaaaacctgcaactgtcccagggatagtaacatgggctgtctttagactgcagcactgcccttaggttagctgcaagtgtgtagatacggagatgcagtttggattctacaaactgcctgataatctccagtacttggagacagagatttttgggttggcttttatcctgctgaattgcagggcaaagatctgatcctgaaatttagacaatcatcacagctataaatcagaaaaacctgggttcaaattctgcttgtgatatttattaaccctgtgattttgactagataacccacattctttgtaaaccttagtttccttgtctttaaaatgagggtcatagtaccgctttcgcaggacttggaggaattaaatggtattaagttggtgcaaaagtaactgtggcttttgaacagcatgtgcatacagtgttcagtacagtatttgcactaagtcaactctcgataaacatttgctggacagcaaatgtgctgatgctgacgagattatcaacgtttacactctgaatgctaaaatgtgttagctccatgtctataatgcacagggtgcttccaggtatgagaccatgggccaccagtgccagatctttggaagctctagtggaagaaccggttctttctttagatatcatgacttctagcttcctatcttaaggaggcttcaggaaaactgtgaaaccagctataaggtacttcagaagagggccaaaaatgtcattaaaaagatgggaaaaatgatttgtagggatacatgaatggcctcaaacagagaagtatgagattcttcatttaattctagtctgtggaagcttgggtgaggagactgctaaccagatgtggtcctattttcattgcagctaatacaaaaccaaatgggctaaggataaagttgtattcttagatataagaacttgttgacaggaagggatatgaggtaactgaacatgtataaaacatcttcacctggaaatatgtacaatgaaccaaagataacaggccatagttacaacaagtttttcaaaagtaactagccgcaaaatgctgttcttgcccaatattcacagtggcttcattcaaattcaccaaatatattcagagttttcccacttttcccatcacaatagtgatgcttttccataaaacagaataagacaaaaccaaaaaacaaaaagtcagaatgtgaaaagaggagaaagtctagggaaattcagctgtaagccctctccctcatttcctttatggcatgagctacatttgggttttgctagtctgcattcaccagactttacccagctcactggagttgtggttgtagttggggagtgtcagggacaggaatggaaaggtgaggaacttgcctgggcaacatagtgagaccccatctcaaccaaaaaatttaaaaaattagccaagcacggtggtgtgtgcctgtagtcctagctacctgggaggctgaggtgggaggatggcttgagcccaggaggttacagtgagctatgattgcagtgccactgcactccagcctgggcgacagaatgaaatcccatctcactgatatttcatatattgacattttatcctcaatatatgaaaaatgaaaaagaaagaagtctcacagcctctgctctgaactctaaaatgagccctgtcttttccatgtctgccacgcagctggagcttgcttcgctcgtatttaacttttctgccttagatctcccagggccccggccacatgaaaaagtacttctgtgatcattctctaactcccagaatataggtatttctcctttatctggactagcccaaacccttgagcactctgagttattcaaacttcaggtcaactttttcctaccccttttatataaggatctcaatcttttttgaatttctcctaactcatctatacttttatcctcatactgaataatttctcgtgttctgaaaccaatctgtcatgtaaatgacctcaaggagaaggggtcatattagatcacacactagctagttttgggatcttctcattttgtttttttaaaccacttagaagattagcaaagggaagtccaaaaaaagaagaagagaaatgaaggcctaattagtgacatccagaggtgacagaataaaactaaagagactatactttcaagtgtaaaggtactgggaagggaaatgtttatttctttattcaatatttaatgagtacctactatgtccaggccctgtataagctgctggggagacaaagctagttccggtccttaaagaactaatagtctacacagcatttctcaagcttggtaacactgatattttgggcaggataattcacgttgtttggcatggtggactgtcctgtgtagctgcaggatgtttagcagcatccttggcctacatccactagatgccagtaggcatcccacatctccttcccagttgtgacaacaaaaaatatctccagataatggcaagtgtcccctgggggacaaaagtgtaccccagttgacaaccactagtgtaggaaaagcagatcatttatataaacacactgtgacaagtattattatcaaaactttgcaagttagagaagaggactccttaattctcggggaaagagagcagatgctacagaaggtttcacagaataaatgacattttatgcttaatatatgaaaaatgttttgcagtaggccaagcagacaagaagaggaaaagttaggaacacatggaaggaacagggaaataacaggtagagaaagaccattcgaaggcagatacaggaagatgagcaaaggcctgggggtaaaagaccacagaatattcaggcaatgatggacgtttacacggtggaaaatgaaaaataagactgaaaccagatcatgccaagtaagaaaggaggtggaattttaatataaagaaataaatgcatattttaaacagagtggagccccttttcaaacaaagcgttacctagagccccagtatattaaactgatcaaagtgtaacttctgtggttgggtcatggtccactcagttttccctgagcttctaagttggcttcagaagcacttctgcagaaccctagaactctttgaactagggtcccaaagataagacgaagaaacttttgcatgttttcggtacatagccatttccactgttctgttagtagcaagaggagcagatccagggctgtgtcagctaactctgtctctgttcctggatcgctgttgctggggtcttgggctggcacggctgcatctgacacgcaactgtccacacgtcctttgggaggttgttcaggatctttttctggggcttttgttggctgcatttccagtaactttgtctgtttttcaataaaagattccatcgcagacatggatagagtctcagactccacattgccttcctggagacaataaagaatcttgtcttgtgcttcagtcacacttagtgctggagaaattttactggatgagaacctcagcctagacttgctagccttcttgccttctgtctggggcttgctttcggtctcggcctcactcagctcctctgtggggctctggggttcagagcgaggaaacgctgtcttcaaggtgtccacaatggcactcaccaccatcttgtctattctagagaccataaatggtttcttgacaaaggcaatacgagcatctgtgttcagagcaaggaactcctgcacctcctcactgttagcgatctccggaatggcacagagttgctttaggaatgattctaggaggctcttacgggcttctactctgtcactgtccatgtttcccaatggaagatctggaaagagctttttaggacccttcacatttttgatgaactttcgtagatctggtttctcctccagacgggtctgcagattcaagaactcccgatagcgacgattcacagtgtggtaggccagctgctgcaggccgctgctgttttcaccgtcaagggctgtctcgtacttcacagtatagagtgtgtatgggtggaatccagtgccactgtgctctcgggctgtaatggtgccagtgatacgaaggttctggatgataactggaccatcgggactgcttaggggctcaaagctgaaggtggctgagctgagaggaccaggtggagaggaggaaagcagaactggtggcagagtaggatcaagggagctcacatcattggtgagatccttctctaagcatgacggccgtgaggggcaggtcttttctggcccctccagcaaagctgtaacagaggcggtaacatctccttgttctatctccttgtctgctgtgtcaatatggatctctgggcaggaattcagtgtggagaccggcaggcctgtctctgtttctgtccctggaccctcctcagcctctgctccttcagatgcctcaccatctttgggttccagagcctgggaactctctagggcacacagggcatcctgaatcctgtcagagagaaagctgcctggagtcatgagcatgatggtttctttgcccagttcagacagcggagactccagctctgagtcttcacataagaacaggggacctcgaacatttggctgtaggaaatgagatgagttgtttcctacttttctttcttcacacatcccacccaaatctccctctacagcttcgtggccttcttcaacctctggagaggggcctgcagaaccctctggctcactgtaacttaggaatactggggctgctactggagaagctctcccttctggaagctgctctacctcagcaatcagtggcagagatgtcggcactgagggctgttcgggggcactggctgggcagggtgctggatctctggccttggaaaagatacccacgagtacaaggtggatccagtcaggatctgacagcctgctgatcagtggtaagattacattgcatgtgatgagttcgaccactacatggcgtccggtacgagtctccaagtggggcttgggcaccagcccttgaagcaacaaattcacaacgccacgcgtataggtgacttcagcactggggctgtgcacagcaggatgtggggcagtcgcccggcagtaagcctcccagaggtgggaaggctcaactggaccattcttccctgcagtggcctcctttgcctgaatgtagctctgcaggtgacaaccgcagagagtcagaacactctgggcaacagcatgactgtccatcacgctcatccttctccgaagctcctggaccaaccctttcatggctgcctccatttcttcctcaaaggctggctcctggctcacggaacggtaccaagataacacaaaatctcgaataatcatctggatggtgcggttgatctcccgttccagctgcctttctgcctcagggcatggaggacaggtggccaacgggatgaagcgttccagatgcagtcgacctgaagccactccagcgaggctggagcccagccatcctcccagcaccactagcaatgccgacagaaggcacagcagccacacgttgaccagaaggtgtatgaccaggagccagccaagcaagacccccacagccatcagcttccggctactcaacaggttattgaggtgacagctcgatccagctggagtttcctggaacggtggcactgtttctgtcttcatggctgaacggacaaggtggcttccccagatgacagccctcaagattttacttcagagttagggaaggggggcatgaactgtgtctcagatatggggcgatctgggtgctgttcagggaaccggggctccaggccctcaaagtcctacaggcactgcaaagcgacagctgcagctccgcgtctccccatggctaccactaacagagccctccaactcgccccttccagctgaggtgtggctttggaggaaaactctgtggccttcacactgccccaggcggaaggcctcttcggggcctcggggcgggcgctgcaaggccctggggcccacggacacttacacacgcagcgggcagcggccggcgaagactgggtcacacgccgccgggaaccgcgcgcccacactcagccccgacctgaagtggactcatcgcggtcctctccgggagcctcggccctctgccgccgtaaacctgggcgactgcgctccgcagccgggcctgtgtgaaggctgaccgccggccggccgccggcgacagct

SEQ ID NO: 8281 - RNA, 8841 nt, Homo sapiens
  source 1..8841: mol_type = other RNA
aaaaaccacaattacttttgcaccaacccactacatcagaacctacctttaagggttgatttgtgggttaaataagtgaagatatgtaaagactttaagtaatgctctcagaagatgttaactattagctggtaccaggcattttgggagtagataggggatctgctgaatgttggcagaatgacccatccctagagcagacattgtctatcaatacccattctctgcttcttccttgctaacatcaattatttctgtagatatctgaccttcatggaagatgacctcatctctgggggaaaatactattgaaagccaatcacaatgccattctcagtgtcagtggattggcatgaggtgggtggttctagccaatgagtcataagaggttttttgttttttttttttttatttggggtctcactctgtcacttaaggctagaatgcagtggtgtgatcgtagctcactgcagcctcaaattcctgggctcaagtgatcctcctgcctcagcctccctagtaggtggaaccacaggcgagagccaccatgccccgctcattttttatattttttgtagagacagggtcttgctatgttccaggctggtcttaaactcctggactcaaacaatcccccaaccttggcctcccaaagtgttgagattataggtgtgagccgctgtgcccggcctagaagaggattcttgaaggacttctgggaaatggttccttcattccttagaagaaaacacagaagagatgctcctgttcttttatgaatgttatctctgggtgtgatgcctgaaactgcagcagcaggaaggcaggcagtctgagagcacagctgacctaattagaatggcaaggaagaaagatggaaagaattcaggccccttaagaggtctcagagttgctgaatcaccaaactcctgggcttacctactcacgtactaatgttatgaaataaaataaattttcctcataatttaattcttgtccagagcatcctgattcatatagccagggaccatagttacacatatttttacttcctccaggacctaacaactggtgttgtgtgctatgagcaaaggaagagcagtagctggaaatgaataacctgggtaggacacaggaagactcaaaaatgttctaggctatgcaaatcaaaaccatgagatagtaatatcacctaataccttttaagatgccattatgaaaaaacaaaacattacaagtgttggagaggatgtggagaaactggaacccttgtacattgttggtgggaatgtaaaatggtctagtcactatggaaaacagtatgaaggtcttcaaagaattaaaaacagaacaatatatgatccagcaatcctacttctgggtatttatctaaaataattaaaagcagggcctcgaagaaacagtcacactcccatgttcactgcagcattgttttcaacaatcaaggcgcggagccaacctaaatgtccctcaatgaatgaacaaagaaaatgtggcatagccatacaatggaatgttttcagccttaaaaagaaaattctgtcacatgctgtaacgtggatgaacctggaggacattatgctaagtgaaataagccagtcaaaggacaaacactgcatgattccacttatatgaggcgttcaaagtagtcaaactcacagaagcagaaagtagaacagtgattgccagaggctggtgggaggggaaacgaggagtggctgttcaatgggtataaacttttggttatgcaagatgaaaaacttgtagcagtctgctacaaagcactgtgctgcttctagttaataatgtaccgtctcaaaataaataaataatgtactgtacacttaagagggtagatctcacattatgtgtttctttacaacaataagaaaatcaccttgtaaactggaaatttccaaaatggaaattggagtagcttgtattgattttaaaatttatacatgctctcactcataggtgggaattgaacaatgagaacacttggacacaggaaggtgaacatcacacactggggcctgttgtgaggtcgggggagggggaagggatagcatcaggagatatacctaatgtaaatgacgagttaacgggtgcagcacaccaacacggcacatgtatacatatgcaacaaacctgcatgttgtgcacatgttccctagaacttaatgtataataataataaaaataaaatttatacatgctcctaggctcagatttaggaatttattttccatttaggttttattaagtctaatccaacaatgcaaaaatgaaactgtgagttatatgtgatgaaaaagtatagctttcttgaattcaaataagcaatggcaaagatcacatttagaatttgacagaaagaacacagcatccctgcctcgtcttttttatagatagtaagaaaagggaaagtagtcttatttcaaatatcaaaattctgacttaaatgaataaaatttagtcacgagtaaatacaaaaaacaagcaaacaataaaaccttcctggatcagcacaggcccaattcttccctgccttttatcaccctgtcagctgggagtatcttttctacctgtggctctctaccaattgttactctcttgttgtctgaacctgctagccaaacttggcaggtcgttttcaaagccagatgagttctgattgttcccttggcaatatccattatttccctcctgggtagaaggaggatctgaggacagcttatctttttggggtacgtggagtagaggtggggactcttatataatacgaaataaaaataagttctttgggctggaagtgtcaaaagattccttagaatttatagccacagggatttcatggtgtgtctgatgtactgattttgtgccacatttgagccagaactggcagcagattcaaagcaacacaggtggctaagtacacatgaggggaaggtaggtatggggagagaaaagtggcataaaacaaggctgtccccctatgctcatcgagaataggatcttagccctcactgaaggagcttaatgatcagctctaatacattggctggactcctgcaggtactcacggaaagtagagatgctgagctaccttttcttgtcaaagtctagggctggagatgcttcaagaactttggagccataaagtcactgtaatggtcaacttttaaggctagaagaggccatgagacatctcattcatctccttgcctttgggcaagaattgcacacctaagcctcccgaatacatcagacacaatttagggttaaaagcctccagaggggcaaaaaagtaaaaagattttacaactttcttccacaaaccactttaattgtgtgctcatcaccgacttcagaatctaagagaactttgacacttgtttttgacaccccattgccttctcatcagtctaactccaagaccttcctccgagtggtaggctctggtaattcagcgaaagcaaggcgctaacaggcgagtgtgaagccaaagggctcccagtgacatccttgacatctttttgccagctattcacatgcatttaatatacagcacttccctgtgactgtctgcagccttttctaccagcaattcctcctgatttatccttctccagcaattcccagttgccttgcctttctaatagatgttgcagtctgacaaaacacctttgccttcatgctggtgttgttaaaggactgattataaccgtaaggaatgggaaataagaagctattccttgtaagtttgctaatcttatctgttcagaataataaaagttctctgtcaaagacttaggaagggagatttcatcccccagccttgctagtcctactctttgtgcattcttaagacaggaggcaagtgctttccattctccttggaaaaactgaggctgaatatgcagcttgtcatgcagttttgctgaagacagagagagggtcaaaaattcaaaaactcaattgctctagggcagggggttgggagcaaagccaataaataaaatgggtggtataaatgcctttcaggaaagggtgtgaagggtggggtggatttaccagaagctttggcagtcagctttgaagtcttctggaaaggaaagtgtagcctcccaggcaagcagcctcatgacatcttccataaggctgatgtgttgggaaacagcaacacatgagcaagaagttccttgaaaaattttcttccctccttcttcttctggaactgttgggaaactagattagacccaggagtctggtttttgagaatggccctgaatgaatttttagtttccgggtaggaacagagagctgagaaggttgttttctcctccaaggaaatctggccacagtttttttcctgttctatctagagcttgtgtgctggtggattaagcacatgtgtgcacagggccaggattctggcaaacaatctcagggaggatggcaaaaggagaagcaaaaggggttcattcctctacctcacagcttcttttcccaaaggaaacaggatctactcaccagcaacaatcccaacatcacaaaaggaacagggaaataaacgtgcatacaactgggacacacagacccctgtcacctgctacaaatggagcagaagtgggagagaagtgagccaccgagaacctaggccttcttagctgtagcctacttgaagagggcacgggcttcctgactggtctctggtggccgagtaactctacttccctgacctgggaagaaggcgtgaataaccagctaagaggagacacccatcctcttagagttgcctggggtatctgaggcagaggtggtagcagcagactcctcaacagaggcactgagatccaagaattccaggatgatgtccccaaggcagtaaatcaaatgcctgttgatgaggggttgttgtagtgactccaggactagaccccagctcagccggcatttgttcaccccaagaatttctactacgagatctgggaggactcccatcaggctctgcaaagcctgtttctcagcagccagtttctgctcttgggtccttacgggccgtggaaacttaggcaaaactccaccaggccagatggactcctgaagaagcaggaggtactgcacccagcgctgtggacttgttaaattagctacctgcacctctagccaccgaagaaaaggagtgccatctctgagtaagtatcagctgctgatgagacaaagacactgtcaagcactgtacatacaaggcacagaactggccaacaggaggccctggaaaaagtcaggcccaggaatataagaaacaggactttcacaaactggcagaaataaactccctccaggcctacaaagagggacagagtttggaaagtgacttctagtccctgggagctgcagagtgccagctttccttattcttctccacactctgaagataaaagacacaaaccacacacttgcaccacgcatggtttaaacatttgctctctttcctggattctcctcttgcctacgttctgcccacccttccccctgtcagcaaacagaggctttatcctaggcctttgggctcagcatggtcttatttcctagtcccaggcagcctgtgtagaagaccaagtgcaacaaatctttcttgttcacagaacttctgagcgatggtgtctcgttaaaaatgatgagcacgccaatctttgaactagggtcccaaagataagacgaagaaacttttgcatgttttcggtacatagccatttccactgttctgttagtagcaagaggagcagatccagggctgtgtcagctaactctgtctctgttcctggatcgctgttgctggggtcttgggctggcacggctgcatctgacacgcaactgtccacacgtcctttgggaggttgttcaggatctttttctggggcttttgttggctgcatttccagtaactttgtctgtttttcaataaaagattccatcgcagacatggatagagtctcagactccacattgccttcctggagacaataaagaatcttgtcttgtgcttcagtcacacttagtgctggagaaattttactggatgagaacctcagcctagacttgctagccttcttgccttctgtctggggcttgctttcggtctcggcctcactcagctcctctgtggggctctggggttcagagcgaggaaacgctgtcttcaaggtgtccacaatggcactcaccaccatcttgtctattctagagaccataaatggtttcttgacaaaggcaatacgagcatctgtgttcagagcaaggaactcctgcacctcctcactgttagcgatctccggaatggcacagagttgctttaggaatgattctaggaggctcttacgggcttctactctgtcactgtccatgtttcccaatggaagatctggaaagagctttttaggacccttcacatttttgatgaactttcgtagatctggtttctcctccagacgggtctgcagattcaagaactcccgatagcgacgattcacagtgtggtaggccagctgctgcaggccgctgctgttttcaccgtcaagggctgtctcgtacttcacagtatagagtgtgtatgggtggaatccagtgccactgtgctctcgggctgtaatggtgccagtgatacgaaggttctggatgataactggaccatcgggactgcttaggggctcaaagctgaaggtggctgagctgagaggaccaggtggagaggaggaaagcagaactggtggcagagtaggatcaagggagctcacatcattggtgagatccttctctaagcatgacggccgtgaggggcaggtcttttctggcccctccagcaaagctgtaacagaggcggtaacatctccttgttctatctccttgtctgctgtgtcaatatggatctctgggcaggaattcagtgtggagaccggcaggcctgtctctgtttctgtccctggaccctcctcagcctctgctccttcagatgcctcaccatctttgggttccagagcctgggaactctctagggcacacagggcatcctgaatcctgtcagagagaaagctgcctggagtcatgagcatgatggtttctttgcccagttcagacagcggagactccagctctgagtcttcacataagaacaggggacctcgaacatttggctgtaggaaatgagatgagttgtttcctacttttctttcttcacacatcccacccaaatctccctctacagcttcgtggccttcttcaacctctggagaggggcctgcagaaccctctggctcactgtaacttaggaatactggggctgctactggagaagctctcccttctggaagctgctctacctcagcaatcagtggcagagatgtcggcactgagggctgttcgggggcactggctgggcagggtgctggatctctggccttggaaaagatacccacgagtacaaggtggatccagtcaggatctgacagcctgctgatcagtggtaagattacattgcatgtgatgagttcgaccactacatggcgtccggtacgagtctccaagtggggcttgggcaccagcccttgaagcaacaaattcacaacgccacgcgtataggtgacttcagcactggggctgtgcacagcaggatgtggggcagtcgcccggcagtaagcctcccagaggtgggaaggctcaactggaccattcttccctgcagtggcctcctttgcctgaatgtagctctgcaggtgacaaccgcagagagtcagaacactctgggcaacagcatgactgtccatcacgctcatccttctccgaagctcctggaccaaccctttcatggctgcctccatttcttcctcaaaggctggctcctggctcacggaacggtaccaagataacacaaaatctcgaataatcatctggatggtgcggttgatctcccgttccagctgcctttctgcctcagggcatggaggacaggtggccaacgggatgaagcgttccagatgcagtcgacctgaagccactccagcgaggctggagcccagccatcctcccagcaccactagcaatgccgacagaaggcacagcagccacacgttgaccagaaggtgtatgaccaggagccagccaagcaagacccccacagccatcagcttccggctactcaacaggttattgaggtgacagctcgatccagctggagtttcctggaacggtggcactgtttctgtcttcatggctgaacggacaaggtggcttccccagatgacagccctcaagattttacttcagagttagggaaggggggcatgaactgtgtctcagatatggggcgatctgggtgctgttcagggaaccggggctccaggccctcaaagtcctacaggcactgcaaagcgacagctgcagctccgcgtctccccatggctaccactaacagagccctccaactcgccccttccagctgaggtgtggctttggaggaaaactctgtggccttcacactgccccaggcggaaggcctcttcggggcctcggggcgggcgctgcaaggccctggggcccacggacacttacacacgcagcgggcagcggccggcgaagactgggtcacacgccgccgggaaccgcgcgcccacactcagccccgacctgaagtggactcatcgcggtcctctccgggagcctcggccctctgccgccgtaaacctgggcgactgcgctccgcagccgggcctgtgtgaaggctgaccgccggccggccgccggcgacagcttccgggt

SEQ ID NO: 8282 - RNA, 6730 nt, Homo sapiens
  source 1..6730: mol_type = other RNA
aaaaaccacaattacttttgcaccaacccactacatcagaacctacctttaagggttgatttgtgggttaaataagtgaagatatgtaaagactttaagtaatgctctcagaagatgttaactattagctggtaccaggcattttgggagtagataggggatctgctgaatgttggcagaatgacccatccctagagcagacattgtctatcaatacccattctctgcttcttccttgctaacatcaattatttctgtagatatctgaccttcatggaagatgacctcatctctgggggaaaatactattgaaagccaatcacaatgccattctcagtgtcagtggattggcatgaggtgggtggttctagccaatgagtcataagaggttttttgttttttttttttttatttggggtctcactctgtcacttaaggctagaatgcagtggtgtgatcgtagctcactgcagcctcaaattcctgggctcaagtgatcctcctgcctcagcctccctagtaggtggaaccacaggcgagagccaccatgccccgctcattttttatattttttgtagagacagggtcttgctatgttccaggctggtcttaaactcctggactcaaacaatcccccaaccttggcctcccaaagtgttgagattataggtgtgagccgctgtgcccggcctagaagaggattcttgaaggacttctgggaaatggttccttcattccttagaagaaaacacagaagagatgctcctgttcttttatgaatgttatctctgggtgtgatgcctgaaactgcagcagcaggaaggcaggcagtctgagagcacagctgacctaattagaatggcaaggaagaaagatggaaagaattcaggccccttaagaggtctcagagttgctgaatcaccaaactcctgggcttacctactcacgtactaatgttatgaaataaaataaattttcctcataatttaattcttgtccagagcatcctgattcatatagccagggaccatagttacacatatttttacttcctccaggacctaacaactggtgttgtgtgctatgagcaaaggaagagcagtagctggaaatgaataacctgggtaggacacaggaagactcaaaaatgttctaggctatgcaaatcaaaaccatgagatagtaatatcacctaataccttttaagatgccattatgaaaaaacaaaacattacaagtgttggagaggatgtggagaaactggaacccttgtacattgttggtgggaatgtaaaatggtctagtcactatggaaaacagtatgaaggtcttcaaagaattaaaaacagaacaatatatgatccagcaatcctacttctgggtatttatctaaaataattaaaagcagggcctcgaagaaacagtcacactcccatgttcactgcagcattgttttcaacaatcaaggcgcggagccaacctaaatgtccctcaatgaatgaacaaagaaaatgtggcatagccatacaatggaatgttttcagccttaaaaagaaaattctgtcacatgctgtaacgtggatgaacctggaggacattatgctaagtgaaataagccagtcaaaggacaaacactgcatgattccacttatatgaggcgttcaaagtagtcaaactcacagaagcagaaagtagaacagtgattgccagaggctggtgggaggggaaacgaggagtggctgttcaatgggtataaacttttggttatgcaagatgaaaaacttgtagcagtctgctacaaagcactgtgctgcttctagttaataatgtaccgtctcaaaataaataaataatgtactgtacacttaagagggtagatctcacattatgtgtttctttacaacaataagaaaatcaccttgtaaactggaaatttccaaaatggaaattggagtagcttgtattgattttaaaatttatacatgctctcactcataggtgggaattgaacaatgagaacacttggacacaggaaggtgaacatcacacactggggcctgttgtgaggtcgggggagggggaagggatagcatcaggagatatacctaatgtaaatgacgagttaacgggtgcagcacaccaacacggcacatgtatacatatgcaacaaacctgcatgttgtgcacatgttccctagaacttaatgtataataataataaaaataaaatttatacatgctcctaggctcagatttaggaatttattttccatttaggttttattaagtctaatccaacaatgcaaaaatgaaactgtgagttatatgtgatgaaaaagtatagctttcttgaattcaaataagcaatggcaaagatcacatttagaatttgacagaaagaacacagcatccctgcctcgtcttttttatagatagtaagaaaagggaaagtagtcttatttcaaatatcaaaattctgacttaaatgaataaaatttagtcacgagtaaatacaaaaaacaagcaaacaataaaaccttcctggatcagcacaggcccaattcttccctgccttttatcaccctgtcagctgggagtatcttttctacctgtggctctctaccaattgttactctcttgttgtctgaacctgctagccaaacttggcaggtcgttttcaaagccagatgagttctgattgttcccttggcaatatccattatttccctcctgggtagaaggaggatctgaggacagcttatctttttggggtacgtggagtagaggtggggactcttatataatacgaaataaaaataagttctttgggctggaagtgtcaaaagattccttagaatttatagccacagggatttcatggtgtgtctgatgtactgattttgtgccacatttgagccagaactggcagcagattcaaagcaacacaggtggctaagtacacatgaggggaaggtaggtatggggagagaaaagtggcataaaacaaggctgtccccctatgctcatcgagaataggatcttagccctcactgaaggagcttaatgatcagctctaatacattggctggactcctgcaggtactcacggaaagtagagatgctgagctaccttttcttgtcaaagtctagggctggagatgcttcaagaactttggagccataaagtcactgtaatggtcaacttttaaggctagaagaggccatgagacatctcattcatctccttgcctttgggcaagaattgcacacctaagcctcccgaatacatcagacacaatttagggttaaaagcctccagaggggcaaaaaagtaaaaagattttacaactttcttccacaaaccactttaattgtgtgctcatcaccgacttcagaatctaagagaactttgacacttgtttttgacaccccattgccttctcatcagtctaactccaagaccttcctccgagtggtaggctctggtaattcagcgaaagcaaggcgctaacaggcgagtgtgaagccaaagggctcccagtgacatccttgacatctttttgccagctattcacatgcatttaatatacagcacttccctgtgactgtctgcagccttttctaccagcaattcctcctgatttatccttctccagcaattcccagttgccttgcctttctaatagatgttgcagtctgacaaaacacctttgccttcatgctggtgttgttaaaggactgattataaccgtaaggaatgggaaataagaagctattccttgtaagtttgctaatcttatctgttcagaataataaaagttctctgtcaaagacttaggaagggagatttcatcccccagccttgctagtcctactctttgtgcattcttaagacaggaggcaagtgctttccattctccttggaaaaactgaggctgaatatgcagcttgtcatgcagttttgctgaagacagagagagggtcaaaaattcaaaaactcaattgctctagggcagggggttgggagcaaagccaataaataaaatgggtggtataaatgcctttcaggaaagggtgtgaagggtggggtggatttaccagaagctttggcagtcagctttgaagtcttctggaaaggaaagtgtagcctcccaggcaagcagcctcatgacatcttccataaggctgatgtgttgggaaacagcaacacatgagcaagaagttccttgaaaaattttcttccctccttcttcttctggaactgttgggaaactagattagacccaggagtctggtttttgagaatggccctgaatgaatttttagtttccgggtaggaacagagagctgagaaggttgttttctcctccaaggaaatctggccacagtttttttcctgttctatctagagcttgtgtgctggtggattaagcacatgtgtgcacagggccaggattctggcaaacaatctcagggaggatggcaaaaggagaagcaaaaggggttcattcctctacctcacagcttcttttcccaaaggaaacaggatctactcaccagcaacaatcccaacatcacaaaaggaacagggaaataaacgtgcatacaactgggacacacagacccctgtcacctgctacaaatggagcagaagtgggagagaagtgagccaccgagaacctaggccttcttagctgtagcctacttgaagagggcacgggcttcctgactggtctctggtggccgagtaactctacttccctgacctgggaagaaggcgtgaataaccagctaagaggagacacccatcctcttagagttgcctggggtatctgaggcagaggtggtagcagcagactcctcaacagaggcactgagatccaagaattccaggatgatgtccccaaggcagtaaatcaaatgcctgttgatgaggggttgttgtagtgactccaggactagaccccagctcagccggcatttgttcaccccaagaatttctactacgagatctgggaggactcccatcaggctctgcaaagcctgtttctcagcagccagtttctgctcttgggtccttacgggccgtggaaacttaggcaaaactccaccaggccagatggactcctgaagaagcaggaggtactgcacccagcgctgtggacttgttaaattagctacctgcacctctagccacctgcagcgccacctggtgcccatagagagaattcctgtgcccacgccatgcagcagcagtttggtaggctttttgtcaccctcaaagcaagatctgatttcagatctgacttcaaagtccaagttcttgctttccatgtggaaggaaagaggtggagaaagtacaacagcaggagatgcttccagagagggcaggctcggtggggcttcatactgggaggcccaggttgtggaggggcgctgcactctttgaactagggtcccaaagataagacgaagaaacttttgcatgttttcggtacatagccatttccactgttctgttagtagcaagaggagcagatccagggctgtgtcagctaactctgtctctgttcctggatcgctgttgctggggtcttgggctggcacggctgcatctgacacgcaactgtccacacgtcctttgggaggttgttcaggatctttttctggggcttttgttggctgcatttccagtaactttgtctgtttttcaataaaagattccatcgcagacatggatagagtctcagactccacattgccttcctggagacaataaagaatcttgtcttgtgcttcagtcacacttagtgctggagaaattttactggatgagaacctcagcctagacttgctagccttcttgccttctgtctggggcttgctttcggtctcggcctcactcagctcctctgtggggctctggggttcagagcgaggaaacgctgtcttcaaggtgtccacaatggcactcaccaccatcttgtctattctagagaccataaatggtttcttgacaaaggcaatacgagcatctgtgttcagagcaaggaactcctgcacctcctcactgttagcgatctccggaatggcacagagttgctttaggaatgattctaggaggctcttacgggcttctactctgtcactgtccatgtttcccaatggaagatctggaaagagctttttaggacccttcacatctctgaaagaatgtgattgctgctgtccagcactaaacttcaaaactcctgaagcaaatccagggagcagagaaccttgaaacggcattctcctccccgatccctcccataaaccaacaggccaatcagcgtggctcgacgtgggaagcaagcgggcagtaggggttggggaaactcctgacttttgatgaactttcgtagatctggtttctcctccagacgggtctgcagattcaagaactcccgatagcgacgattcacagtgtggtaggccagctgctgcaggccgctgctgttttcaccgtcaagggctgtctcgtaacacgcagcgggcagcggccggcgaagactgggtcacacgccgccgggaaccgcgcgcccacactcagccccgacctgaagtggactcatcgcggtcctctccgggagcctcggccctctgccgccgtaaacctgggcgactgcgctccgcagccgggcctgtgtgaaggctgaccgccggccggccgccggcgacagcttccggg

SEQ ID NO: 8283 - RNA, 6547 nt, Homo sapiens
  source 1..6547: mol_type = other RNA
aaaaaccacaattacttttgcaccaacccactacatcagaacctacctttaagggttgatttgtgggttaaataagtgaagatatgtaaagactttaagtaatgctctcagaagatgttaactattagctggtaccaggcattttgggagtagataggggatctgctgaatgttggcagaatgacccatccctagagcagacattgtctatcaatacccattctctgcttcttccttgctaacatcaattatttctgtagatatctgaccttcatggaagatgacctcatctctgggggaaaatactattgaaagccaatcacaatgccattctcagtgtcagtggattggcatgaggtgggtggttctagccaatgagtcataagaggttttttgttttttttttttttatttggggtctcactctgtcacttaaggctagaatgcagtggtgtgatcgtagctcactgcagcctcaaattcctgggctcaagtgatcctcctgcctcagcctccctagtaggtggaaccacaggcgagagccaccatgccccgctcattttttatattttttgtagagacagggtcttgctatgttccaggctggtcttaaactcctggactcaaacaatcccccaaccttggcctcccaaagtgttgagattataggtgtgagccgctgtgcccggcctagaagaggattcttgaaggacttctgggaaatggttccttcattccttagaagaaaacacagaagagatgctcctgttcttttatgaatgttatctctgggtgtgatgcctgaaactgcagcagcaggaaggcaggcagtctgagagcacagctgacctaattagaatggcaaggaagaaagatggaaagaattcaggccccttaagaggtctcagagttgctgaatcaccaaactcctgggcttacctactcacgtactaatgttatgaaataaaataaattttcctcataatttaattcttgtccagagcatcctgattcatatagccagggaccatagttacacatatttttacttcctccaggacctaacaactggtgttgtgtgctatgagcaaaggaagagcagtagctggaaatgaataacctgggtaggacacaggaagactcaaaaatgttctaggctatgcaaatcaaaaccatgagatagtaatatcacctaataccttttaagatgccattatgaaaaaacaaaacattacaagtgttggagaggatgtggagaaactggaacccttgtacattgttggtgggaatgtaaaatggtctagtcactatggaaaacagtatgaaggtcttcaaagaattaaaaacagaacaatatatgatccagcaatcctacttctgggtatttatctaaaataattaaaagcagggcctcgaagaaacagtcacactcccatgttcactgcagcattgttttcaacaatcaaggcgcggagccaacctaaatgtccctcaatgaatgaacaaagaaaatgtggcatagccatacaatggaatgttttcagccttaaaaagaaaattctgtcacatgctgtaacgtggatgaacctggaggacattatgctaagtgaaataagccagtcaaaggacaaacactgcatgattccacttatatgaggcgttcaaagtagtcaaactcacagaagcagaaagtagaacagtgattgccagaggctggtgggaggggaaacgaggagtggctgttcaatgggtataaacttttggttatgcaagatgaaaaacttgtagcagtctgctacaaagcactgtgctgcttctagttaataatgtaccgtctcaaaataaataaataatgtactgtacacttaagagggtagatctcacattatgtgtttctttacaacaataagaaaatcaccttgtaaactggaaatttccaaaatggaaattggagtagcttgtattgattttaaaatttatacatgctctcactcataggtgggaattgaacaatgagaacacttggacacaggaaggtgaacatcacacactggggcctgttgtgaggtcgggggagggggaagggatagcatcaggagatatacctaatgtaaatgacgagttaacgggtgcagcacaccaacacggcacatgtatacatatgcaacaaacctgcatgttgtgcacatgttccctagaacttaatgtataataataataaaaataaaatttatacatgctcctaggctcagatttaggaatttattttccatttaggttttattaagtctaatccaacaatgcaaaaatgaaactgtgagttatatgtgatgaaaaagtatagctttcttgaattcaaataagcaatggcaaagatcacatttagaatttgacagaaagaacacagcatccctgcctcgtcttttttatagatagtaagaaaagggaaagtagtcttatttcaaatatcaaaattctgacttaaatgaataaaatttagtcacgagtaaatacaaaaaacaagcaaacaataaaaccttcctggatcagcacaggcccaattcttccctgccttttatcaccctgtcagctgggagtatcttttctacctgtggctctctaccaattgttactctcttgttgtctgaacctgctagccaaacttggcaggtcgttttcaaagccagatgagttctgattgttcccttggcaatatccattatttccctcctgggtagaaggaggatctgaggacagcttatctttttggggtacgtggagtagaggtggggactcttatataatacgaaataaaaataagttctttgggctggaagtgtcaaaagattccttagaatttatagccacagggatttcatggtgtgtctgatgtactgattttgtgccacatttgagccagaactggcagcagattcaaagcaacacaggtggctaagtacacatgaggggaaggtaggtatggggagagaaaagtggcataaaacaaggctgtccccctatgctcatcgagaataggatcttagccctcactgaaggagcttaatgatcagctctaatacattggctggactcctgcaggtactcacggaaagtagagatgctgagctaccttttcttgtcaaagtctagggctggagatgcttcaagaactttggagccataaagtcactgtaatggtcaacttttaaggctagaagaggccatgagacatctcattcatctccttgcctttgggcaagaattgcacacctaagcctcccgaatacatcagacacaatttagggttaaaagcctccagaggggcaaaaaagtaaaaagattttacaactttcttccacaaaccactttaattgtgtgctcatcaccgacttcagaatctaagagaactttgacacttgtttttgacaccccattgccttctcatcagtctaactccaagaccttcctccgagtggtaggctctggtaattcagcgaaagcaaggcgctaacaggcgagtgtgaagccaaagggctcccagtgacatccttgacatctttttgccagctattcacatgcatttaatatacagcacttccctgtgactgtctgcagccttttctaccagcaattcctcctgatttatccttctccagcaattcccagttgccttgcctttctaatagatgttgcagtctgacaaaacacctttgccttcatgctggtgttgttaaaggactgattataaccgtaaggaatgggaaataagaagctattccttgtaagtttgctaatcttatctgttcagaataataaaagttctctgtcaaagacttaggaagggagatttcatcccccagccttgctagtcctactctttgtgcattcttaagacaggaggcaagtgctttccattctccttggaaaaactgaggctgaatatgcagcttgtcatgcagttttgctgaagacagagagagggtcaaaaattcaaaaactcaattgctctagggcagggggttgggagcaaagccaataaataaaatgggtggtataaatgcctttcaggaaagggtgtgaagggtggggtggatttaccagaagctttggcagtcagctttgaagtcttctggaaaggaaagtgtagcctcccaggcaagcagcctcatgacatcttccataaggctgatgtgttgggaaacagcaacacatgagcaagaagttccttgaaaaattttcttccctccttcttcttctggaactgttgggaaactagattagacccaggagtctggtttttgagaatggccctgaatgaatttttagtttccgggtaggaacagagagctgagaaggttgttttctcctccaaggaaatctggccacagtttttttcctgttctatctagagcttgtgtgctggtggattaagcacatgtgtgcacagggccaggattctggcaaacaatctcagggaggatggcaaaaggagaagcaaaaggggttcattcctctacctcacagcttcttttcccaaaggaaacaggatctactcaccagcaacaatcccaacatcacaaaaggaacagggaaataaacgtgcatacaactgggacacacagacccctgtcacctgctacaaatggagcagaagtgggagagaagtgagccaccgagaacctaggccttcttagctgtagcctacttgaagagggcacgggcttcctgactggtctctggtggccgagtaactctacttccctgacctgggaagaaggcgtgaataaccagctaagaggagacacccatcctcttagagttgcctggggtatctgaggcagaggtggtagcagcagactcctcaacagaggcactgagatccaagaattccaggatgatgtccccaaggcagtaaatcaaatgcctgttgatgaggggttgttgtagtgactccaggactagaccccagctcagccggcatttgttcaccccaagaatttctactacgagatctgggaggactcccatcaggctctgcaaagcctgtttctcagcagccagtttctgctcttgggtccttacgggccgtggaaacttaggcaaaactccaccaggccagatggactcctgaagaagcaggaggtactgcacccagcgctgtggacttgttaaattagctacctgcacctctagccacctgcagcgccacctggtgcccatagagagaattcctgtgcccacgccatgcagcagcagtttggtaggctttttgtcaccctcaaagcaagatctgatttcagatctgacttcaaagtccaagttcttgctttccatgtggaaggaaagaggtggagaaagtacaacagcaggagatgcttccagagagggcaggctcggtggggcttcatactgggaggcccaggttgtggaggggcgctgcactctttgaactagggtcccaaagataagacgaagaaacttttgcatgttttcggtacatagccatttccactgttctgttagtagcaagaggagcagatccagggctgtgtcagctaactctgtctctgttcctggatcgctgttgctggggtcttgggctggcacggctgcatctgacacgcaactgtccacacgtcctttgggaggttgttcaggatctttttctggggcttttgttggctgcatttccagtaactttgtctgtttttcaataaaagattccatcgcagacatggatagagtctcagactccacattgccttcctggagacaataaagaatcttgtcttgtgcttcagtcacacttagtgctggagaaattttactggatgagaacctcagcctagacttgctagccttcttgccttctgtctggggcttgctttcggtctcggcctcactcagctcctctgtggggctctggggttcagagcgaggaaacgctgtcttcaaggtgtccacaatggcactcaccaccatcttgtctattctagagaccataaatggtttcttgacaaaggcaatacgagcatctgtgttcagagcaaggaactcctgcacctcctcactgttagcgatctccggaatggcacagagttgctttaggaatgattctaggaggctcttacgggcttctactctgtcactgtccatgtttcccaatggaagatctggaaagagctttttaggacccttcacatttttgatgaactttcgtagatctggtttctcctccagacgggtctgcagattcaagaactcccgatagcgacgattcacagtgtggtaggccagctgctgcaggccgctgctgttttcaccgtcaagggctgtctcgtaacacgcagcgggcagcggccggcgaagactgggtcacacgccgccgggaaccgcgcgcccacactcagccccgacctgaagtggactcatcgcggtcctctccgggagcctcggccctctgccgccgtaaacctgggcgactgcgctccgcagccgggcctgtgtgaaggctgaccgccggccggccgccggcgacagcttccgg

SEQ ID NO: 8284 - RNA, 8563 nt, Homo sapiens
  source 1..8563: mol_type = other RNA
aaaaaccacaattacttttgcaccaacccactacatcagaacctacctttaagggttgatttgtgggttaaataagtgaagatatgtaaagactttaagtaatgctctcagaagatgttaactattagctggtaccaggcattttgggagtagataggggatctgctgaatgttggcagaatgacccatccctagagcagacattgtctatcaatacccattctctgcttcttccttgctaacatcaattatttctgtagatatctgaccttcatggaagatgacctcatctctgggggaaaatactattgaaagccaatcacaatgccattctcagtgtcagtggattggcatgaggtgggtggttctagccaatgagtcataagaggttttttgttttttttttttttatttggggtctcactctgtcacttaaggctagaatgcagtggtgtgatcgtagctcactgcagcctcaaattcctgggctcaagtgatcctcctgcctcagcctccctagtaggtggaaccacaggcgagagccaccatgccccgctcattttttatattttttgtagagacagggtcttgctatgttccaggctggtcttaaactcctggactcaaacaatcccccaaccttggcctcccaaagtgttgagattataggtgtgagccgctgtgcccggcctagaagaggattcttgaaggacttctgggaaatggttccttcattccttagaagaaaacacagaagagatgctcctgttcttttatgaatgttatctctgggtgtgatgcctgaaactgcagcagcaggaaggcaggcagtctgagagcacagctgacctaattagaatggcaaggaagaaagatggaaagaattcaggccccttaagaggtctcagagttgctgaatcaccaaactcctgggcttacctactcacgtactaatgttatgaaataaaataaattttcctcataatttaattcttgtccagagcatcctgattcatatagccagggaccatagttacacatatttttacttcctccaggacctaacaactggtgttgtgtgctatgagcaaaggaagagcagtagctggaaatgaataacctgggtaggacacaggaagactcaaaaatgttctaggctatgcaaatcaaaaccatgagatagtaatatcacctaataccttttaagatgccattatgaaaaaacaaaacattacaagtgttggagaggatgtggagaaactggaacccttgtacattgttggtgggaatgtaaaatggtctagtcactatggaaaacagtatgaaggtcttcaaagaattaaaaacagaacaatatatgatccagcaatcctacttctgggtatttatctaaaataattaaaagcagggcctcgaagaaacagtcacactcccatgttcactgcagcattgttttcaacaatcaaggcgcggagccaacctaaatgtccctcaatgaatgaacaaagaaaatgtggcatagccatacaatggaatgttttcagccttaaaaagaaaattctgtcacatgctgtaacgtggatgaacctggaggacattatgctaagtgaaataagccagtcaaaggacaaacactgcatgattccacttatatgaggcgttcaaagtagtcaaactcacagaagcagaaagtagaacagtgattgccagaggctggtgggaggggaaacgaggagtggctgttcaatgggtataaacttttggttatgcaagatgaaaaacttgtagcagtctgctacaaagcactgtgctgcttctagttaataatgtaccgtctcaaaataaataaataatgtactgtacacttaagagggtagatctcacattatgtgtttctttacaacaataagaaaatcaccttgtaaactggaaatttccaaaatggaaattggagtagcttgtattgattttaaaatttatacatgctctcactcataggtgggaattgaacaatgagaacacttggacacaggaaggtgaacatcacacactggggcctgttgtgaggtcgggggagggggaagggatagcatcaggagatatacctaatgtaaatgacgagttaacgggtgcagcacaccaacacggcacatgtatacatatgcaacaaacctgcatgttgtgcacatgttccctagaacttaatgtataataataataaaaataaaatttatacatgctcctaggctcagatttaggaatttattttccatttaggttttattaagtctaatccaacaatgcaaaaatgaaactgtgagttatatgtgatgaaaaagtatagctttcttgaattcaaataagcaatggcaaagatcacatttagaatttgacagaaagaacacagcatccctgcctcgtcttttttatagatagtaagaaaagggaaagtagtcttatttcaaatatcaaaattctgacttaaatgaataaaatttagtcacgagtaaatacaaaaaacaagcaaacaataaaaccttcctggatcagcacaggcccaattcttccctgccttttatcaccctgtcagctgggagtatcttttctacctgtggctctctaccaattgttactctcttgttgtctgaacctgctagccaaacttggcaggtcgttttcaaagccagatgagttctgattgttcccttggcaatatccattatttccctcctgggtagaaggaggatctgaggacagcttatctttttggggtacgtggagtagaggtggggactcttatataatacgaaataaaaataagttctttgggctggaagtgtcaaaagattccttagaatttatagccacagggatttcatggtgtgtctgatgtactgattttgtgccacatttgagccagaactggcagcagattcaaagcaacacaggtggctaagtacacatgaggggaaggtaggtatggggagagaaaagtggcataaaacaaggctgtccccctatgctcatcgagaataggatcttagccctcactgaaggagcttaatgatcagctctaatacattggctggactcctgcaggtactcacggaaagtagagatgctgagctaccttttcttgtcaaagtctagggctggagatgcttcaagaactttggagccataaagtcactgtaatggtcaacttttaaggctagaagaggccatgagacatctcattcatctccttgcctttgggcaagaattgcacacctaagcctcccgaatacatcagacacaatttagggttaaaagcctccagaggggcaaaaaagtaaaaagattttacaactttcttccacaaaccactttaattgtgtgctcatcaccgacttcagaatctaagagaactttgacacttgtttttgacaccccattgccttctcatcagtctaactccaagaccttcctccgagtggtaggctctggtaattcagcgaaagcaaggcgctaacaggcgagtgtgaagccaaagggctcccagtgacatccttgacatctttttgccagctattcacatgcatttaatatacagcacttccctgtgactgtctgcagccttttctaccagcaattcctcctgatttatccttctccagcaattcccagttgccttgcctttctaatagatgttgcagtctgacaaaacacctttgccttcatgctggtgttgttaaaggactgattataaccgtaaggaatgggaaataagaagctattccttgtaagtttgctaatcttatctgttcagaataataaaagttctctgtcaaagacttaggaagggagatttcatcccccagccttgctagtcctactctttgtgcattcttaagacaggaggcaagtgctttccattctccttggaaaaactgaggctgaatatgcagcttgtcatgcagttttgctgaagacagagagagggtcaaaaattcaaaaactcaattgctctagggcagggggttgggagcaaagccaataaataaaatgggtggtataaatgcctttcaggaaagggtgtgaagggtggggtggatttaccagaagctttggcagtcagctttgaagtcttctggaaaggaaagtgtagcctcccaggcaagcagcctcatgacatcttccataaggctgatgtgttgggaaacagcaacacatgagcaagaagttccttgaaaaattttcttccctccttcttcttctggaactgttgggaaactagattagacccaggagtctggtttttgagaatggccctgaatgaatttttagtttccgggtaggaacagagagctgagaaggttgttttctcctccaaggaaatctggccacagtttttttcctgttctatctagagcttgtgtgctggtggattaagcacatgtgtgcacagggccaggattctggcaaacaatctcagggaggatggcaaaaggagaagcaaaaggggttcattcctctacctcacagcttcttttcccaaaggaaacaggatctactcaccagcaacaatcccaacatcacaaaaggaacagggaaataaacgtgcatacaactgggacacacagacccctgtcacctgctacaaatggagcagaagtgggagagaagtgagccaccgagaacctaggccttcttagctgtagcctacttgaagagggcacgggcttcctgactggtctctggtggccgagtaactctacttccctgacctgggaagaaggcgtgaataaccagctaagaggagacacccatcctcttagagttgcctggggtatctgaggcagaggtggtagcagcagactcctcaacagaggcactgagatccaagaattccaggatgatgtccccaaggcagtaaatcaaatgcctgttgatgaggggttgttgtagtgactccaggactagaccccagctcagccggcatttgttcaccccaagaatttctactacgagatctgggaggactcccatcaggctctgcaaagcctgtttctcagcagccagtttctgctcttgggtccttacgggccgtggaaacttaggcaaaactccaccaggccagatggactcctgaagaagcaggaggtactgcacccagcgctgtggacttgttaaattagctacctgcacctctagccacctgcagcgccacctggtgcccatagagagaattcctgtgcccacgccatgcagcagcagtttggtaggctttttgtcaccctcaaagcaagatctgatttcagatctgacttcaaagtccaagttcttgctttccatgtggaaggaaagaggtggagaaagtacaacagcaggagatgcttccagagagggcaggctcggtggggcttcatactgggaggcccaggttgtggaggggcgctgcactctttgaactagggtcccaaagataagacgaagaaacttttgcatgttttcggtacatagccatttccactgttctgttagtagcaagaggagcagatccagggctgtgtcagctaactctgtctctgttcctggatcgctgttgctggggtcttgggctggcacggctgcatctgacacgcaactgtccacacgtcctttgggaggttgttcaggatctttttctggggcttttgttggctgcatttccagtaactttgtctgtttttcaataaaagattccatcgcagacatggatagagtctcagactccacattgccttcctggagacaataaagaatcttgtcttgtgcttcagtcacacttagtgctggagaaattttactggatgagaacctcagcctagacttgctagccttcttgccttctgtctggggcttgctttcggtctcggcctcactcagctcctctgtggggctctggggttcagagcgaggaaacgctgtcttcaaggtgtccacaatggcactcaccaccatcttgtctattctagagaccataaatggtttcttgacaaaggcaatacgagcatctgtgttcagagcaaggaactcctgcacctcctcactgttagcgatctccggaatggcacagagttgctttaggaatgattctaggaggctcttacgggcttctactctgtcactgtccatgtttcccaatggaagatctggaaagagctttttaggacccttcacatttttgatgaactttcgtagatctggtttctcctccagacgggtctgcagattcaagaactcccgatagcgacgattcacagtgtggtaggccagctgctgcaggccgctgctgttttcaccgtcaagggctgtctcgtacttcacagtatagagtgtgtatgggtggaatccagtgccactgtgctctcgggctgtaatggtgccagtgatacgaaggttctggatgataactggaccatcgggactgcttaggggctcaaagctgaaggtggctgagctgagaggaccaggtggagaggaggaaagcagaactggtggcagagtaggatcaagggagctcacatcattggtgagatccttctctaagcatgacggccgtgaggggcaggtcttttctggcccctccagcaaagctgtaacagaggcggtaacatctccttgttctatctccttgtctgctgtgtcaatatggatctctgggcaggaattcagtgtggagaccggcaggcctgtctctgtttctgtccctggaccctcctcagcctctgctccttcagatgcctcaccatctttgggttccagagcctgggaactctctagggcacacagggcatcctgaatcctgtcagagagaaagctgcctggagtcatgagcatgatggtttctttgcccagttcagacagcggagactccagctctgagtcttcacataagaacaggggacctcgaacatttggctgtaggaaatgagatgagttgtttcctacttttctttcttcacacatcccacccaaatctccctctacagcttcgtggccttcttcaacctctggagaggggcctgcagaaccctctggctcactgtaacttaggaatactggggctgctactggagaagctctcccttctggaagctgctctacctcagcaatcagtggcagagatgtcggcactgagggctgttcgggggcactggctgggcagggtgctggatctctggccttggaaaagatacccacgagtacaaggtggatccagtcaggatctgacagcctgctgatcagtggtaagattacattgcatgtgatgagttcgaccactacatggcgtccggtacgagtctccaagtggggcttgggcaccagcccttgaagcaacaaattcacaacgccacgcgtataggtgacttcagcactggggctgtgcacagcaggatgtggggcagtcgcccggcagtaagcctcccagaggtgggaaggctcaactggaccattcttccctgcagtggcctcctttgcctgaatgtagctctgcaggtgacaaccgcagagagtcagaacactctgggcaacagcatgactgtccatcacgctcatccttctccgaagctcctggaccaaccctttcatggctgcctccatttcttcctcaaaggctggctcctggctcacggaacggtaccaagataacacaaaatctcgaataatcatctggatggtgcggttgatctcccgttccagctgcctttctgcctcagggcatggaggacaggtggccaacgggatgaagcgttccagatgcagtcgacctgaagccactccagcgaggctggagcccagccatcctcccagcaccactagcaatgccgacagaaggcacagcagccacacgttgaccagaaggtgtatgaccaggagccagccaagcaagacccccacagccatcagcttccggctactcaacaggttattgaggtgacagctcgatccagctggagtttcctggaacggtggcactgtttctgtcttcatggctgaacggacaaggtggcttccccagatgacagccctcaagattttacttcagagttagggaaggggggcatgaactgtgtctcagatatggggcgatctgggtgctgttcagggaaccggggctccaggccctcaaagtcctacaggcactgcaaagcgacagctgcagctccgcgtctccccatggctaccactaacagagccctccaactcgccccttccagctgaggtgtggctttggaggaaaactctgtggccttcacactgccccaggcggaaggcctcttcggggcctcggggcgggcgctgcaaggccctggggcccacggacacttacacacgcagcgggcagcggccggcgaagactgggtcacacgccgccgggaaccgcgcgcccacactcagccccgacctgaagtggactcatcgcggtcctctccgggagcctcggccctctgccgccgtaaacctgggcgactgcgctccgcagccgggcctgtgtgaaggctgaccgccggccggccgccggcgacagcttccgggt

SEQ ID NO: 8285 - RNA, 7468 nt, Homo sapiens
  source 1..7468: mol_type = other RNA
aaaaaccacaattacttttgcaccaacccactacatcagaacctacctttaagggttgatttgtgggttaaataagtgaagatatgtaaagactttaagtaatgctctcagaagatgttaactattagctggtaccaggcattttgggagtagataggggatctgctgaatgttggcagaatgacccatccctagagcagacattgtctatcaatacccattctctgcttcttccttgctaacatcaattatttctgtagatatctgaccttcatggaagatgacctcatctctgggggaaaatactattgaaagccaatcacaatgccattctcagtgtcagtggattggcatgaggtgggtggttctagccaatgagtcataagaggttttttgttttttttttttttatttggggtctcactctgtcacttaaggctagaatgcagtggtgtgatcgtagctcactgcagcctcaaattcctgggctcaagtgatcctcctgcctcagcctccctagtaggtggaaccacaggcgagagccaccatgccccgctcattttttatattttttgtagagacagggtcttgctatgttccaggctggtcttaaactcctggactcaaacaatcccccaaccttggcctcccaaagtgttgagattataggtgtgagccgctgtgcccggcctagaagaggattcttgaaggacttctgggaaatggttccttcattccttagaagaaaacacagaagagatgctcctgttcttttatgaatgttatctctgggtgtgatgcctgaaactgcagcagcaggaaggcaggcagtctgagagcacagctgacctaattagaatggcaaggaagaaagatggaaagaattcaggccccttaagaggtctcagagttgctgaatcaccaaactcctgggcttacctactcacgtactaatgttatgaaataaaataaattttcctcataatttaattcttgtccagagcatcctgattcatatagccagggaccatagttacacatatttttacttcctccaggacctaacaactggtgttgtgtgctatgagcaaaggaagagcagtagctggaaatgaataacctgggtaggacacaggaagactcaaaaatgttctaggctatgcaaatcaaaaccatgagatagtaatatcacctaataccttttaagatgccattatgaaaaaacaaaacattacaagtgttggagaggatgtggagaaactggaacccttgtacattgttggtgggaatgtaaaatggtctagtcactatggaaaacagtatgaaggtcttcaaagaattaaaaacagaacaatatatgatccagcaatcctacttctgggtatttatctaaaataattaaaagcagggcctcgaagaaacagtcacactcccatgttcactgcagcattgttttcaacaatcaaggcgcggagccaacctaaatgtccctcaatgaatgaacaaagaaaatgtggcatagccatacaatggaatgttttcagccttaaaaagaaaattctgtcacatgctgtaacgtggatgaacctggaggacattatgctaagtgaaataagccagtcaaaggacaaacactgcatgattccacttatatgaggcgttcaaagtagtcaaactcacagaagcagaaagtagaacagtgattgccagaggctggtgggaggggaaacgaggagtggctgttcaatgggtataaacttttggttatgcaagatgaaaaacttgtagcagtctgctacaaagcactgtgctgcttctagttaataatgtaccgtctcaaaataaataaataatgtactgtacacttaagagggtagatctcacattatgtgtttctttacaacaataagaaaatcaccttgtaaactggaaatttccaaaatggaaattggagtagcttgtattgattttaaaatttatacatgctctcactcataggtgggaattgaacaatgagaacacttggacacaggaaggtgaacatcacacactggggcctgttgtgaggtcgggggagggggaagggatagcatcaggagatatacctaatgtaaatgacgagttaacgggtgcagcacaccaacacggcacatgtatacatatgcaacaaacctgcatgttgtgcacatgttccctagaacttaatgtataataataataaaaataaaatttatacatgctcctaggctcagatttaggaatttattttccatttaggttttattaagtctaatccaacaatgcaaaaatgaaactgtgagttatatgtgatgaaaaagtatagctttcttgaattcaaataagcaatggcaaagatcacatttagaatttgacagaaagaacacagcatccctgcctcgtcttttttatagatagtaagaaaagggaaagtagtcttatttcaaatatcaaaattctgacttaaatgaataaaatttagtcacgagtaaatacaaaaaacaagcaaacaataaaaccttcctggatcagcacaggcccaattcttccctgccttttatcaccctgtcagctgggagtatcttttctacctgtggctctctaccaattgttactctcttgttgtctgaacctgctagccaaacttggcaggtcgttttcaaagccagatgagttctgattgttcccttggcaatatccattatttccctcctgggtagaaggaggatctgaggacagcttatctttttggggtacgtggagtagaggtggggactcttatataatacgaaataaaaataagttctttgggctggaagtgtcaaaagattccttagaatttatagccacagggatttcatggtgtgtctgatgtactgattttgtgccacatttgagccagaactggcagcagattcaaagcaacacaggtggctaagtacacatgaggggaaggtaggtatggggagagaaaagtggcataaaacaaggctgtccccctatgctcatcgagaataggatcttagccctcactgaaggagcttaatgatcagctctaatacattggctggactcctgcaggtactcacggaaagtagagatgctgagctaccttttcttgtcaaagtctagggctggagatgcttcaagaactttggagccataaagtcactgtaatggtcaacttttaaggctagaagaggccatgagacatctcattcatctccttgcctttgggcaagaattgcacacctaagcctcccgaatacatcagacacaatttagggttaaaagcctccagaggggcaaaaaagtaaaaagattttacaactttcttccacaaaccactttaattgtgtgctcatcaccgacttcagaatctaagagaactttgacacttgtttttgacaccccattgccttctcatcagtctaactccaagaccttcctccgagtggtaggctctggtaattcagcgaaagcaaggcgctaacaggcgagtgtgaagccaaagggctcccagtgacatccttgacatctttttgccagctattcacatgcatttaatatacagcacttccctgtgactgtctgcagccttttctaccagcaattcctcctgatttatccttctccagcaattcccagttgccttgcctttctaatagatgttgcagtctgacaaaacacctttgccttcatgctggtgttgttaaaggactgattataaccgtaaggaatgggaaataagaagctattccttgtaagtttgctaatcttatctgttcagaataataaaagttctctgtcaaagacttaggaagggagatttcatcccccagccttgctagtcctactctttgtgcattcttaagacaggaggcaagtgctttccattctccttggaaaaactgaggctgaatatgcagcttgtcatgcagttttgctgaagacagagagagggtcaaaaattcaaaaactcaattgctctagggcagggggttgggagcaaagccaataaataaaatgggtggtataaatgcctttcaggaaagggtgtgaagggtggggtggatttaccagaagctttggcagtcagctttgaagtcttctggaaaggaaagtgtagcctcccaggcaagcagcctcatgacatcttccataaggctgatgtgttgggaaacagcaacacatgagcaagaagttccttgaaaaattttcttccctccttcttcttctggaactgttgggaaactagattagacccaggagtctggtttttgagaatggccctgaatgaatttttagtttccgggtaggaacagagagctgagaaggttgttttctcctccaaggaaatctggccacagtttttttcctgttctatctagagcttgtgtgctggtggattaagcacatgtgtgcacagggccaggattctggcaaacaatctcagggaggatggcaaaaggagaagcaaaaggggttcattcctctacctcacagcttcttttcccaaaggaaacaggatctactcaccagcaacaatcccaacatcacaaaaggaacagggaaataaacgtgcatacaactgggacacacagacccctgtcacctgctacaaatggagcagaagtgggagagaagtgagccaccgagaacctaggccttcttagctgtagcctacttgaagagggcacgggcttcctgactggtctctggtggccgagtaactctacttccctgacctgggaagaaggcgtgaataaccagctaagaggagacacccatcctcttagagttgcctggggtatctgaggcagaggtggtagcagcagactcctcaacagaggcactgagatccaagaattccaggatgatgtccccaaggcagtaaatcaaatgcctgttgatgaggggttgttgtagtgactccaggactagaccccagctcagccggcatttgttcaccccaagaatttctactacgagatctgggaggactcccatcaggctctgcaaagcctgtttctcagcagccagtttctgctcttgggtccttacgggccgtggaaacttaggcaaaactccaccaggccagatggactcctgaagaagcaggaggtactgcacccagcgctgtggacttgttaaattagctacctgcacctctagccacctgcagcgccacctggtgcccatagagagaattcctgtgcccacgccatgcagcagcagtttggtaggctttttgtcaccctcaaagcaagatctgatttcagatctgacttcaaagtccaagttcttgctttccatgtggaaggaaagaggtggagaaagtacaacagcaggagatgcttccagagagggcaggctcggtggggcttcatactgggaggcccaggttgtggaggggcgctgcactctttgaactagggtcccaaagataagacgaagaaacttttgcatgttttcggtacatagccatttccactgttctgttagtagcaagaggagcagatccagggctgtgtcagctaactctgtctctgttcctggatcgctgttgctggggtcttgggctggcacggctgcatctgacacgcaactgtccacacgtcctttgggaggttgttcaggatctttttctggggcttttgttggctgcatttccagtaactttgtctgtttttcaataaaagattccatcgcagacatggatagagtctcagactccacattgccttcctggagacaataaagaatcttgtcttgtgcttcagtcacacttagtgctggagaaattttactggatgagaacctcagcctagacttgctagccttcttgccttctgtctggggcttgctttcggtctcggcctcactcagctcctctgtggggctctggggttcagagcgaggaaacgctgtcttcaaggtgtccacaatggcactcaccaccatcttgtctattctagagaccataaatggtttcttgacaaaggcaatacgagcatctgtgttcagagcaaggaactcctgcacctcctcactgttagcgatctccggaatggcacagagttgctttaggaatgattctaggaggctcttacgggcttctactctgtcactgtccatgtttcccaatggaagatctggaaagagctttttaggacccttcacatttttgatgaactttcgtagatctggtttctcctccagacgggtctgcagattcaagaactcccgatagcgacgattcacagtgtggtaggccagctgctgcaggccgctgctgttttcaccgtcaagggctgtctcgtagagtacaaggtggatccagtcaggatctgacagcctgctgatcagtggtaagattacattgcatgtgatgagttcgaccactacatggcgtccggtacgagtctccaagtggggcttgggcaccagcccttgaagcaacaaattcacaacgccacgcgtataggtgacttcagcactggggctgtgcacagcaggatgtggggcagtcgcccggcagtaagcctcccagaggtgggaaggctcaactggaccattcttccctgcagtggcctcctttgcctgaatgtagctctgcaggtgacaaccgcagagagtcagaacactctgggcaacagcatgactgtccatcacgctcatccttctccgaagctcctggaccaaccctttcatggctgcctccatttcttcctcaaaggctggctcctggctcacggaacggtaccaagataacacaaaatctcgaataatcatctggatggtgcggttgatctcccgttccagctgcctttctgcctcagggcatggaggacaggtggccaacgggatgaagcgttccagatgcagtcgacctgaagccactccagcgaggctggagcccagccatcctcccagcaccactagcaatgccgacagaaggcacagcagccacacgttgaccagaaggtgtatgaccaggagccagccaagcaagacccccacagccatcagcttccggctactcaacaggttattgaggtgacagctcgatccagctggagtttcctggaacggtggcactgtttctgtcttcatggctgaacggacaaggtggcttccccagatgacagccctcaagattttacttcagagttagggaaggggggcatgaactgtgtctcagatatggggcgatctgggtgctgttcagggaaccggggctccaggccctcaaagtcctacaggcactgcaaagcgacagctgcagctccgcgtctccccatggctaccactaacagagccctccaactcgccccttccagctgaggtgtggctttggaggaaaactctgtggccttcacactgccccaggcggaaggcctcttcggggcctcggggcgggcgctgcaaggccctggggcccacggac

SEQ ID NO: 8286 - RNA, 8443 nt, Homo sapiens
  source 1..8443: mol_type = other RNA
aaaaaccacaattacttttgcaccaacccactacatcagaacctacctttaagggttgatttgtgggttaaataagtgaagatatgtaaagactttaagtaatgctctcagaagatgttaactattagctggtaccaggcattttgggagtagataggggatctgctgaatgttggcagaatgacccatccctagagcagacattgtctatcaatacccattctctgcttcttccttgctaacatcaattatttctgtagatatctgaccttcatggaagatgacctcatctctgggggaaaatactattgaaagccaatcacaatgccattctcagtgtcagtggattggcatgaggtgggtggttctagccaatgagtcataagaggttttttgttttttttttttttatttggggtctcactctgtcacttaaggctagaatgcagtggtgtgatcgtagctcactgcagcctcaaattcctgggctcaagtgatcctcctgcctcagcctccctagtaggtggaaccacaggcgagagccaccatgccccgctcattttttatattttttgtagagacagggtcttgctatgttccaggctggtcttaaactcctggactcaaacaatcccccaaccttggcctcccaaagtgttgagattataggtgtgagccgctgtgcccggcctagaagaggattcttgaaggacttctgggaaatggttccttcattccttagaagaaaacacagaagagatgctcctgttcttttatgaatgttatctctgggtgtgatgcctgaaactgcagcagcaggaaggcaggcagtctgagagcacagctgacctaattagaatggcaaggaagaaagatggaaagaattcaggccccttaagaggtctcagagttgctgaatcaccaaactcctgggcttacctactcacgtactaatgttatgaaataaaataaattttcctcataatttaattcttgtccagagcatcctgattcatatagccagggaccatagttacacatatttttacttcctccaggacctaacaactggtgttgtgtgctatgagcaaaggaagagcagtagctggaaatgaataacctgggtaggacacaggaagactcaaaaatgttctaggctatgcaaatcaaaaccatgagatagtaatatcacctaataccttttaagatgccattatgaaaaaacaaaacattacaagtgttggagaggatgtggagaaactggaacccttgtacattgttggtgggaatgtaaaatggtctagtcactatggaaaacagtatgaaggtcttcaaagaattaaaaacagaacaatatatgatccagcaatcctacttctgggtatttatctaaaataattaaaagcagggcctcgaagaaacagtcacactcccatgttcactgcagcattgttttcaacaatcaaggcgcggagccaacctaaatgtccctcaatgaatgaacaaagaaaatgtggcatagccatacaatggaatgttttcagccttaaaaagaaaattctgtcacatgctgtaacgtggatgaacctggaggacattatgctaagtgaaataagccagtcaaaggacaaacactgcatgattccacttatatgaggcgttcaaagtagtcaaactcacagaagcagaaagtagaacagtgattgccagaggctggtgggaggggaaacgaggagtggctgttcaatgggtataaacttttggttatgcaagatgaaaaacttgtagcagtctgctacaaagcactgtgctgcttctagttaataatgtaccgtctcaaaataaataaataatgtactgtacacttaagagggtagatctcacattatgtgtttctttacaacaataagaaaatcaccttgtaaactggaaatttccaaaatggaaattggagtagcttgtattgattttaaaatttatacatgctctcactcataggtgggaattgaacaatgagaacacttggacacaggaaggtgaacatcacacactggggcctgttgtgaggtcgggggagggggaagggatagcatcaggagatatacctaatgtaaatgacgagttaacgggtgcagcacaccaacacggcacatgtatacatatgcaacaaacctgcatgttgtgcacatgttccctagaacttaatgtataataataataaaaataaaatttatacatgctcctaggctcagatttaggaatttattttccatttaggttttattaagtctaatccaacaatgcaaaaatgaaactgtgagttatatgtgatgaaaaagtatagctttcttgaattcaaataagcaatggcaaagatcacatttagaatttgacagaaagaacacagcatccctgcctcgtcttttttatagatagtaagaaaagggaaagtagtcttatttcaaatatcaaaattctgacttaaatgaataaaatttagtcacgagtaaatacaaaaaacaagcaaacaataaaaccttcctggatcagcacaggcccaattcttccctgccttttatcaccctgtcagctgggagtatcttttctacctgtggctctctaccaattgttactctcttgttgtctgaacctgctagccaaacttggcaggtcgttttcaaagccagatgagttctgattgttcccttggcaatatccattatttccctcctgggtagaaggaggatctgaggacagcttatctttttggggtacgtggagtagaggtggggactcttatataatacgaaataaaaataagttctttgggctggaagtgtcaaaagattccttagaatttatagccacagggatttcatggtgtgtctgatgtactgattttgtgccacatttgagccagaactggcagcagattcaaagcaacacaggtggctaagtacacatgaggggaaggtaggtatggggagagaaaagtggcataaaacaaggctgtccccctatgctcatcgagaataggatcttagccctcactgaaggagcttaatgatcagctctaatacattggctggactcctgcaggtactcacggaaagtagagatgctgagctaccttttcttgtcaaagtctagggctggagatgcttcaagaactttggagccataaagtcactgtaatggtcaacttttaaggctagaagaggccatgagacatctcattcatctccttgcctttgggcaagaattgcacacctaagcctcccgaatacatcagacacaatttagggttaaaagcctccagaggggcaaaaaagtaaaaagattttacaactttcttccacaaaccactttaattgtgtgctcatcaccgacttcagaatctaagagaactttgacacttgtttttgacaccccattgccttctcatcagtctaactccaagaccttcctccgagtggtaggctctggtaattcagcgaaagcaaggcgctaacaggcgagtgtgaagccaaagggctcccagtgacatccttgacatctttttgccagctattcacatgcatttaatatacagcacttccctgtgactgtctgcagccttttctaccagcaattcctcctgatttatccttctccagcaattcccagttgccttgcctttctaatagatgttgcagtctgacaaaacacctttgccttcatgctggtgttgttaaaggactgattataaccgtaaggaatgggaaataagaagctattccttgtaagtttgctaatcttatctgttcagaataataaaagttctctgtcaaagacttaggaagggagatttcatcccccagccttgctagtcctactctttgtgcattcttaagacaggaggcaagtgctttccattctccttggaaaaactgaggctgaatatgcagcttgtcatgcagttttgctgaagacagagagagggtcaaaaattcaaaaactcaattgctctagggcagggggttgggagcaaagccaataaataaaatgggtggtataaatgcctttcaggaaagggtgtgaagggtggggtggatttaccagaagctttggcagtcagctttgaagtcttctggaaaggaaagtgtagcctcccaggcaagcagcctcatgacatcttccataaggctgatgtgttgggaaacagcaacacatgagcaagaagttccttgaaaaattttcttccctccttcttcttctggaactgttgggaaactagattagacccaggagtctggtttttgagaatggccctgaatgaatttttagtttccgggtaggaacagagagctgagaaggttgttttctcctccaaggaaatctggccacagtttttttcctgttctatctagagcttgtgtgctggtggattaagcacatgtgtgcacagggccaggattctggcaaacaatctcagggaggatggcaaaaggagaagcaaaaggggttcattcctctacctcacagcttcttttcccaaaggaaacaggatctactcaccagcaacaatcccaacatcacaaaaggaacagggaaataaacgtgcatacaactgggacacacagacccctgtcacctgctacaaatggagcagaagtgggagagaagtgagccaccgagaacctaggccttcttagctgtagcctacttgaagagggcacgggcttcctgactggtctctggtggccgagtaactctacttccctgacctgggaagaaggcgtgaataaccagctaagaggagacacccatcctcttagagttgcctggggtatctgaggcagaggtggtagcagcagactcctcaacagaggcactgagatccaagaattccaggatgatgtccccaaggcagtaaatcaaatgcctgttgatgaggggttgttgtagtgactccaggactagaccccagctcagccggcatttgttcaccccaagaatttctactacgagatctgggaggactcccatcaggctctgcaaagcctgtttctcagcagccagtttctgctcttgggtccttacgggccgtggaaacttaggcaaaactccaccaggccagatggactcctgaagaagcaggaggtactgcacccagcgctgtggacttgttaaattagctacctgcacctctagccacctgcagcgccacctggtgcccatagagagaattcctgtgcccacgccatgcagcagcagtttggtaggctttttgtcaccctcaaagcaagatctgatttcagatctgacttcaaagtccaagttcttgctttccatgtggaaggaaagaggtggagaaagtacaacagcaggagatgcttccagagagggcaggctcggtggggcttcatactgggaggcccaggttgtggaggggcgctgcactctttgaactagggtcccaaagataagacgaagaaacttttgcatgttttcggtacatagccatttccactgttctgttagtagcaagaggagcagatccagggctgtgtcagctaactctgtctctgttcctggatcgctgttgctggggtcttgggctggcacggctgcatctgacacgcaactgtccacacgtcctttgggaggttgttcaggatctttttctggggcttttgttggctgcatttccagtaactttgtctgtttttcaataaaagattccatcgcagacatggatagagtctcagactccacattgccttcctggagacaataaagaatcttgtcttgtgcttcagtcacacttagtgctggagaaattttactggatgagaacctcagcctagacttgctagccttcttgccttctgtctggggcttgctttcggtctcggcctcactcagctcctctgtggggctctggggttcagagcgaggaaacgctgtcttcaaggtgtccacaatggcactcaccaccatctttaggaatgattctaggaggctcttacgggcttctactctgtcactgtccatgtttcccaatggaagatctggaaagagctttttaggacccttcacatttttgatgaactttcgtagatctggtttctcctccagacgggtctgcagattcaagaactcccgatagcgacgattcacagtgtggtaggccagctgctgcaggccgctgctgttttcaccgtcaagggctgtctcgtacttcacagtatagagtgtgtatgggtggaatccagtgccactgtgctctcgggctgtaatggtgccagtgatacgaaggttctggatgataactggaccatcgggactgcttaggggctcaaagctgaaggtggctgagctgagaggaccaggtggagaggaggaaagcagaactggtggcagagtaggatcaagggagctcacatcattggtgagatccttctctaagcatgacggccgtgaggggcaggtcttttctggcccctccagcaaagctgtaacagaggcggtaacatctccttgttctatctccttgtctgctgtgtcaatatggatctctgggcaggaattcagtgtggagaccggcaggcctgtctctgtttctgtccctggaccctcctcagcctctgctccttcagatgcctcaccatctttgggttccagagcctgggaactctctagggcacacagggcatcctgaatcctgtcagagagaaagctgcctggagtcatgagcatgatggtttctttgcccagttcagacagcggagactccagctctgagtcttcacataagaacaggggacctcgaacatttggctgtaggaaatgagatgagttgtttcctacttttctttcttcacacatcccacccaaatctccctctacagcttcgtggccttcttcaacctctggagaggggcctgcagaaccctctggctcactgtaacttaggaatactggggctgctactggagaagctctcccttctggaagctgctctacctcagcaatcagtggcagagatgtcggcactgagggctgttcgggggcactggctgggcagggtgctggatctctggccttggaaaagatacccacgagtacaaggtggatccagtcaggatctgacagcctgctgatcagtggtaagattacattgcatgtgatgagttcgaccactacatggcgtccggtacgagtctccaagtggggcttgggcaccagcccttgaagcaacaaattcacaacgccacgcgtataggtgacttcagcactggggctgtgcacagcaggatgtggggcagtcgcccggcagtaagcctcccagaggtgggaaggctcaactggaccattcttccctgcagtggcctcctttgcctgaatgtagctctgcaggtgacaaccgcagagagtcagaacactctgggcaacagcatgactgtccatcacgctcatccttctccgaagctcctggaccaaccctttcatggctgcctccatttcttcctcaaaggctggctcctggctcacggaacggtaccaagataacacaaaatctcgaataatcatctggatggtgcggttgatctcccgttccagctgcctttctgcctcagggcatggaggacaggtggccaacgggatgaagcgttccagatgcagtcgacctgaagccactccagcgaggctggagcccagccatcctcccagcaccactagcaatgccgacagaaggcacagcagccacacgttgaccagaaggtgtatgaccaggagccagccaagcaagacccccacagccatcagcttccggctactcaacaggttattgaggtgacagctcgatccagctggagtttcctggaacggtggcactgtttctgtcttcatggctgaacggacaaggtggcttccccagatgacagccctcaagattttacttcagagttagggaaggggggcatgaactgtgtctcagatatggggcgatctgggtgctgttcagggaaccggggctccaggccctcaaagtcctacaggcactgcaaagcgacagctgcagctccgcgtctccccatggctaccactaacagagccctccaactcgccccttccagctgaggtgtggctttggaggaaaactctgtggccttcacactgccccaggcggaaggcctcttcggggcctcggggcgggcgctgcaaggccctggggcccacggacacttacacacgcagcgggcagcggccggcgaagactgggtcacacgccgccgggaaccgcgcgcccacactcagccccgacctgaagtggactcatcgcggtcctctccgggagcctcggccctctgccgccgtaaacctgggcgactgcgctccgcagccgggcctgtgtgaaggctgaccgccggccggccgccggcgacagcttccgggt

SEQ ID NO: 8287 - RNA, 8551 nt, Homo sapiens
  source 1..8551: mol_type = other RNA
aaaaaccacaattacttttgcaccaacccactacatcagaacctacctttaagggttgatttgtgggttaaataagtgaagatatgtaaagactttaagtaatgctctcagaagatgttaactattagctggtaccaggcattttgggagtagataggggatctgctgaatgttggcagaatgacccatccctagagcagacattgtctatcaatacccattctctgcttcttccttgctaacatcaattatttctgtagatatctgaccttcatggaagatgacctcatctctgggggaaaatactattgaaagccaatcacaatgccattctcagtgtcagtggattggcatgaggtgggtggttctagccaatgagtcataagaggttttttgttttttttttttttatttggggtctcactctgtcacttaaggctagaatgcagtggtgtgatcgtagctcactgcagcctcaaattcctgggctcaagtgatcctcctgcctcagcctccctagtaggtggaaccacaggcgagagccaccatgccccgctcattttttatattttttgtagagacagggtcttgctatgttccaggctggtcttaaactcctggactcaaacaatcccccaaccttggcctcccaaagtgttgagattataggtgtgagccgctgtgcccggcctagaagaggattcttgaaggacttctgggaaatggttccttcattccttagaagaaaacacagaagagatgctcctgttcttttatgaatgttatctctgggtgtgatgcctgaaactgcagcagcaggaaggcaggcagtctgagagcacagctgacctaattagaatggcaaggaagaaagatggaaagaattcaggccccttaagaggtctcagagttgctgaatcaccaaactcctgggcttacctactcacgtactaatgttatgaaataaaataaattttcctcataatttaattcttgtccagagcatcctgattcatatagccagggaccatagttacacatatttttacttcctccaggacctaacaactggtgttgtgtgctatgagcaaaggaagagcagtagctggaaatgaataacctgggtaggacacaggaagactcaaaaatgttctaggctatgcaaatcaaaaccatgagatagtaatatcacctaataccttttaagatgccattatgaaaaaacaaaacattacaagtgttggagaggatgtggagaaactggaacccttgtacattgttggtgggaatgtaaaatggtctagtcactatggaaaacagtatgaaggtcttcaaagaattaaaaacagaacaatatatgatccagcaatcctacttctgggtatttatctaaaataattaaaagcagggcctcgaagaaacagtcacactcccatgttcactgcagcattgttttcaacaatcaaggcgcggagccaacctaaatgtccctcaatgaatgaacaaagaaaatgtggcatagccatacaatggaatgttttcagccttaaaaagaaaattctgtcacatgctgtaacgtggatgaacctggaggacattatgctaagtgaaataagccagtcaaaggacaaacactgcatgattccacttatatgaggcgttcaaagtagtcaaactcacagaagcagaaagtagaacagtgattgccagaggctggtgggaggggaaacgaggagtggctgttcaatgggtataaacttttggttatgcaagatgaaaaacttgtagcagtctgctacaaagcactgtgctgcttctagttaataatgtaccgtctcaaaataaataaataatgtactgtacacttaagagggtagatctcacattatgtgtttctttacaacaataagaaaatcaccttgtaaactggaaatttccaaaatggaaattggagtagcttgtattgattttaaaatttatacatgctctcactcataggtgggaattgaacaatgagaacacttggacacaggaaggtgaacatcacacactggggcctgttgtgaggtcgggggagggggaagggatagcatcaggagatatacctaatgtaaatgacgagttaacgggtgcagcacaccaacacggcacatgtatacatatgcaacaaacctgcatgttgtgcacatgttccctagaacttaatgtataataataataaaaataaaatttatacatgctcctaggctcagatttaggaatttattttccatttaggttttattaagtctaatccaacaatgcaaaaatgaaactgtgagttatatgtgatgaaaaagtatagctttcttgaattcaaataagcaatggcaaagatcacatttagaatttgacagaaagaacacagcatccctgcctcgtcttttttatagatagtaagaaaagggaaagtagtcttatttcaaatatcaaaattctgacttaaatgaataaaatttagtcacgagtaaatacaaaaaacaagcaaacaataaaaccttcctggatcagcacaggcccaattcttccctgccttttatcaccctgtcagctgggagtatcttttctacctgtggctctctaccaattgttactctcttgttgtctgaacctgctagccaaacttggcaggtcgttttcaaagccagatgagttctgattgttcccttggcaatatccattatttccctcctgggtagaaggaggatctgaggacagcttatctttttggggtacgtggagtagaggtggggactcttatataatacgaaataaaaataagttctttgggctggaagtgtcaaaagattccttagaatttatagccacagggatttcatggtgtgtctgatgtactgattttgtgccacatttgagccagaactggcagcagattcaaagcaacacaggtggctaagtacacatgaggggaaggtaggtatggggagagaaaagtggcataaaacaaggctgtccccctatgctcatcgagaataggatcttagccctcactgaaggagcttaatgatcagctctaatacattggctggactcctgcaggtactcacggaaagtagagatgctgagctaccttttcttgtcaaagtctagggctggagatgcttcaagaactttggagccataaagtcactgtaatggtcaacttttaaggctagaagaggccatgagacatctcattcatctccttgcctttgggcaagaattgcacacctaagcctcccgaatacatcagacacaatttagggttaaaagcctccagaggggcaaaaaagtaaaaagattttacaactttcttccacaaaccactttaattgtgtgctcatcaccgacttcagaatctaagagaactttgacacttgtttttgacaccccattgccttctcatcagtctaactccaagaccttcctccgagtggtaggctctggtaattcagcgaaagcaaggcgctaacaggcgagtgtgaagccaaagggctcccagtgacatccttgacatctttttgccagctattcacatgcatttaatatacagcacttccctgtgactgtctgcagccttttctaccagcaattcctcctgatttatccttctccagcaattcccagttgccttgcctttctaatagatgttgcagtctgacaaaacacctttgccttcatgctggtgttgttaaaggactgattataaccgtaaggaatgggaaataagaagctattccttgtaagtttgctaatcttatctgttcagaataataaaagttctctgtcaaagacttaggaagggagatttcatcccccagccttgctagtcctactctttgtgcattcttaagacaggaggcaagtgctttccattctccttggaaaaactgaggctgaatatgcagcttgtcatgcagttttgctgaagacagagagagggtcaaaaattcaaaaactcaattgctctagggcagggggttgggagcaaagccaataaataaaatgggtggtataaatgcctttcaggaaagggtgtgaagggtggggtggatttaccagaagctttggcagtcagctttgaagtcttctggaaaggaaagtgtagcctcccaggcaagcagcctcatgacatcttccataaggctgatgtgttgggaaacagcaacacatgagcaagaagttccttgaaaaattttcttccctccttcttcttctggaactgttgggaaactagattagacccaggagtctggtttttgagaatggccctgaatgaatttttagtttccgggtaggaacagagagctgagaaggttgttttctcctccaaggaaatctggccacagtttttttcctgttctatctagagcttgtgtgctggtggattaagcacatgtgtgcacagggccaggattctggcaaacaatctcagggaggatggcaaaaggagaagcaaaaggggttcattcctctacctcacagcttcttttcccaaaggaaacaggatctactcaccagcaacaatcccaacatcacaaaaggaacagggaaataaacgtgcatacaactgggacacacagacccctgtcacctgctacaaatggagcagaagtgggagagaagtgagccaccgagaacctaggccttcttagctgtagcctacttgaagagggcacgggcttcctgactggtctctggtggccgagtaactctacttccctgacctgggaagaaggcgtgaataaccagctaagaggagacacccatcctcttagagttgcctggggtatctgaggcagaggtggtagcagcagactcctcaacagaggcactgagatccaagaattccaggatgatgtccccaaggcagtaaatcaaatgcctgttgatgaggggttgttgtagtgactccaggactagaccccagctcagccggcatttgttcaccccaagaatttctactacgagatctgggaggactcccatcaggctctgcaaagcctgtttctcagcagccagtttctgctcttgggtccttacgggccgtggaaacttaggcaaaactccaccaggccagatggactcctgaagaagcaggaggtactgcacccagcgctgtggacttgttaaattagctacctgcacctctagccacctggtgcccatagagagaattcctgtgcccacgccatgcagcagcagtttggtaggctttttgtcaccctcaaagcaagatctgatttcagatctgacttcaaagtccaagttcttgctttccatgtggaaggaaagaggtggagaaagtacaacagcaggagatgcttccagagagggcaggctcggtggggcttcatactgggaggcccaggttgtggaggggcgctgcactctttgaactagggtcccaaagataagacgaagaaacttttgcatgttttcggtacatagccatttccactgttctgttagtagcaagaggagcagatccagggctgtgtcagctaactctgtctctgttcctggatcgctgttgctggggtcttgggctggcacggctgcatctgacacgcaactgtccacacgtcctttgggaggttgttcaggatctttttctggggcttttgttggctgcatttccagtaactttgtctgtttttcaataaaagattccatcgcagacatggatagagtctcagactccacattgccttcctggagacaataaagaatcttgtcttgtgcttcagtcacacttagtgctggagaaattttactggatgagaacctcagcctagacttgctagccttcttgccttctgtctggggcttgctttcggtctcggcctcactcagctcctctgtggggctctggggttcagagcgaggaaacgctgtcttcaaggtgtccacaatggcactcaccaccatcttgtctattctagagaccataaatggtttcttgacaaaggcaatacgagcatctgtgttcagagcaaggaactcctgcacctcctcactgttagcgatctccggaatggcacagagttgctttaggaatgattctaggaggctcttacgggcttctactctgtcactgtccatgtttcccaatggaagatctggaaagagctttttaggacccttcacatttttgatgaactttcgtagatctggtttctcctccagacgggtctgcagattcaagaactcccgatagcgacgattcacagtgtggtaggccagctgctgcaggccgctgctgttttcaccgtcaagggctgtctcgtacttcacagtatagagtgtgtatgggtggaatccagtgccactgtgctctcgggctgtaatggtgccagtgatacgaaggttctggatgataactggaccatcgggactgcttaggggctcaaagctgaaggtggctgagctgagaggaccaggtggagaggaggaaagcagaactggtggcagagtaggatcaagggagctcacatcattggtgagatccttctctaagcatgacggccgtgaggggcaggtcttttctggcccctccagcaaagctgtaacagaggcggtaacatctccttgttctatctccttgtctgctgtgtcaatatggatctctgggcaggaattcagtgtggagaccggcaggcctgtctctgtttctgtccctggaccctcctcagcctctgctccttcagatgcctcaccatctttgggttccagagcctgggaactctctagggcacacagggcatcctgaatcctgtcagagagaaagctgcctggagtcatgagcatgatggtttctttgcccagttcagacagcggagactccagctctgagtcttcacataagaacaggggacctcgaacatttggctgtaggaaatgagatgagttgtttcctacttttctttcttcacacatcccacccaaatctccctctacagcttcgtggccttcttcaacctctggagaggggcctgcagaaccctctggctcactgtaacttaggaatactggggctgctactggagaagctctcccttctggaagctgctctacctcagcaatcagtggcagagatgtcggcactgagggctgttcgggggcactggctgggcagggtgctggatctctggccttggaaaagatacccacgagtacaaggtggatccagtcaggatctgacagcctgctgatcagtggtaagattacattgcatgtgatgagttcgaccactacatggcgtccggtacgagtctccaagtggggcttgggcaccagcccttgaagcaacaaattcacaacgccacgcgtataggtgacttcagcactggggctgtgcacagcaggatgtggggcagtcgcccggcagtaagcctcccagaggtgggaaggctcaactggaccattcttccctgcagtggcctcctttgcctgaatgtagctctgcaggtgacaaccgcagagagtcagaacactctgggcaacagcatgactgtccatcacgctcatccttctccgaagctcctggaccaaccctttcatggctgcctccatttcttcctcaaaggctggctcctggctcacggaacggtaccaagataacacaaaatctcgaataatcatctggatggtgcggttgatctcccgttccagctgcctttctgcctcagggcatggaggacaggtggccaacgggatgaagcgttccagatgcagtcgacctgaagccactccagcgaggctggagcccagccatcctcccagcaccactagcaatgccgacagaaggcacagcagccacacgttgaccagaaggtgtatgaccaggagccagccaagcaagacccccacagccatcagcttccggctactcaacaggttattgaggtgacagctcgatccagctggagtttcctggaacggtggcactgtttctgtcttcatggctgaacggacaaggtggcttccccagatgacagccctcaagattttacttcagagttagggaaggggggcatgaactgtgtctcagatatggggcgatctgggtgctgttcagggaaccggggctccaggccctcaaagtcctacaggcactgcaaagcgacagctgcagctccgcgtctccccatggctaccactaacagagccctccaactcgccccttccagctgaggtgtggctttggaggaaaactctgtggccttcacactgccccaggcggaaggcctcttcggggcctcggggcgggcgctgcaaggccctggggcccacggacacttacacacgcagcgggcagcggccggcgaagactgggtcacacgccgccgggaaccgcgcgcccacactcagccccgacctgaagtggactcatcgcggtcctctccgggagcctcggccctctgccgccgtaaacctgggcgactgcgctccgcagccgggcctgtgtgaaggctgaccgccggccggccgccggcgacagcttccgggt

SEQ ID NO: 8288 - RNA, 6026 nt, Homo sapiens
  source 1..6026: mol_type = other RNA
aaaaaccacaattacttttgcaccaacccactacatcagaacctacctttaagggttgatttgtgggttaaataagtgaagatatgtaaagactttaagtaatgctctcagaagatgttaactattagctggtaccaggcattttgggagtagataggggatctgctgaatgttggcagaatgacccatccctagagcagacattgtctatcaatacccattctctgcttcttccttgctaacatcaattatttctgtagatatctgaccttcatggaagatgacctcatctctgggggaaaatactattgaaagccaatcacaatgccattctcagtgtcagtggattggcatgaggtgggtggttctagccaatgagtcataagaggttttttgttttttttttttttatttggggtctcactctgtcacttaaggctagaatgcagtggtgtgatcgtagctcactgcagcctcaaattcctgggctcaagtgatcctcctgcctcagcctccctagtaggtggaaccacaggcgagagccaccatgccccgctcattttttatattttttgtagagacagggtcttgctatgttccaggctggtcttaaactcctggactcaaacaatcccccaaccttggcctcccaaagtgttgagattataggtgtgagccgctgtgcccggcctagaagaggattcttgaaggacttctgggaaatggttccttcattccttagaagaaaacacagaagagatgctcctgttcttttatgaatgttatctctgggtgtgatgcctgaaactgcagcagcaggaaggcaggcagtctgagagcacagctgacctaattagaatggcaaggaagaaagatggaaagaattcaggccccttaagaggtctcagagttgctgaatcaccaaactcctgggcttacctactcacgtactaatgttatgaaataaaataaattttcctcataatttaattcttgtccagagcatcctgattcatatagccagggaccatagttacacatatttttacttcctccaggacctaacaactggtgttgtgtgctatgagcaaaggaagagcagtagctggaaatgaataacctgggtaggacacaggaagactcaaaaatgttctaggctatgcaaatcaaaaccatgagatagtaatatcacctaataccttttaagatgccattatgaaaaaacaaaacattacaagtgttggagaggatgtggagaaactggaacccttgtacattgttggtgggaatgtaaaatggtctagtcactatggaaaacagtatgaaggtcttcaaagaattaaaaacagaacaatatatgatccagcaatcctacttctgggtatttatctaaaataattaaaagcagggcctcgaagaaacagtcacactcccatgttcactgcagcattgttttcaacaatcaaggcgcggagccaacctaaatgtccctcaatgaatgaacaaagaaaatgtggcatagccatacaatggaatgttttcagccttaaaaagaaaattctgtcacatgctgtaacgtggatgaacctggaggacattatgctaagtgaaataagccagtcaaaggacaaacactgcatgattccacttatatgaggcgttcaaagtagtcaaactcacagaagcagaaagtagaacagtgattgccagaggctggtgggaggggaaacgaggagtggctgttcaatgggtataaacttttggttatgcaagatgaaaaacttgtagcagtctgctacaaagcactgtgctgcttctagttaataatgtaccgtctcaaaataaataaataatgtactgtacacttaagagggtagatctcacattatgtgtttctttacaacaataagaaaatcaccttgtaaactggaaatttccaaaatggaaattggagtagcttgtattgattttaaaatttatacatgctctcactcataggtgggaattgaacaatgagaacacttggacacaggaaggtgaacatcacacactggggcctgttgtgaggtcgggggagggggaagggatagcatcaggagatatacctaatgtaaatgacgagttaacgggtgcagcacaccaacacggcacatgtatacatatgcaacaaacctgcatgttgtgcacatgttccctagaacttaatgtataataataataaaaataaaatttatacatgctcctaggctcagatttaggaatttattttccatttaggttttattaagtctaatccaacaatgcaaaaatgaaactgtgagttatatgtgatgaaaaagtatagctttcttgaattcaaataagcaatggcaaagatcacatttagaatttgacagaaagaacacagcatccctgcctcgtcttttttatagatagtaagaaaagggaaagtagtcttatttcaaatatcaaaattctgacttaaatgaataaaatttagtcacgagtaaatacaaaaaacaagcaaacaataaaaccttcctggatcagcacaggcccaattcttccctgccttttatcaccctgtcagctgggagtatcttttctacctgtggctctctaccaattgttactctcttgttgtctgaacctgctagccaaacttggcaggtcgttttcaaagccagatgagttctgattgttcccttggcaatatccattatttccctcctgggtagaaggaggatctgaggacagcttatctttttggggtacgtggagtagaggtggggactcttatataatacgaaataaaaataagttctttgggctggaagtgtcaaaagattccttagaatttatagccacagggatttcatggtgtgtctgatgtactgattttgtgccacatttgagccagaactggcagcagattcaaagcaacacaggtggctaagtacacatgaggggaaggtaggtatggggagagaaaagtggcataaaacaaggctgtccccctatgctcatcgagaataggatcttagccctcactgaaggagcttaatgatcagctctaatacattggctggactcctgcaggtactcacggaaagtagagatgctgagctaccttttcttgtcaaagtctagggctggagatgcttcaagaactttggagccataaagtcactgtaatggtcaacttttaaggctagaagaggccatgagacatctcattcatctccttgcctttgggcaagaattgcacacctaagcctcccgaatacatcagacacaatttagggttaaaagcctccagaggggcaaaaaagtaaaaagattttacaactttcttccacaaaccactttaattgtgtgctcatcaccgacttcagaatctaagagaactttgacacttgtttttgacaccccattgccttctcatcagtctaactccaagaccttcctccgagtggtaggctctggtaattcagcgaaagcaaggcgctaacaggcgagtgtgaagccaaagggctcccagtgacatccttgacatctttttgccagctattcacatgcatttaatatacagcacttccctgtgactgtctgcagccttttctaccagcaattcctcctgatttatccttctccagcaattcccagttgccttgcctttctaatagatgttgcagtctgacaaaacacctttgccttcatgctggtgttgttaaaggactgattataaccgtaaggaatgggaaataagaagctattccttgtaagtttgctaatcttatctgttcagaataataaaagttctctgtcaaagacttaggaagggagatttcatcccccagccttgctagtcctactctttgtgcattcttaagacaggaggcaagtgctttccattctccttggaaaaactgaggctgaatatgcagcttgtcatgcagttttgctgaagacagagagagggtcaaaaattcaaaaactcaattgctctagggcagggggttgggagcaaagccaataaataaaatgggtggtataaatgcctttcaggaaagggtgtgaagggtggggtggatttaccagaagctttggcagtcagctttgaagtcttctggaaaggaaagtgtagcctcccaggcaagcagcctcatgacatcttccataaggctgatgtgttgggaaacagcaacacatgagcaagaagttccttgaaaaattttcttccctccttcttcttctggaactgttgggaaactagattagacccaggagtctggtttttgagaatggccctgaatgaatttttagtttccgggtaggaacagagagctgagaaggttgttttctcctccaaggaaatctggccacagtttttttcctgttctatctagagcttgtgtgctggtggattaagcacatgtgtgcacagggccaggattctggcaaacaatctcagggaggatggcaaaaggagaagcaaaaggggttcattcctctacctcacagcttcttttcccaaaggaaacaggatctactcaccagcaacaatcccaacatcacaaaaggaacagggaaataaacgtgcatacaactgggacacacagacccctgtcacctgctacaaatggagcagaagtgggagagaagtgagccaccgagaacctaggccttcttagctgtagcctacttgaagagggcacgggcttcctgactggtctctggtggccgagtaactctacttccctgacctgggaagaaggcgtgaataaccagctaagaggagacacccatcctcttagagttgcctggggtatctgaggcagaggtggtagcagcagactcctcaacagaggcactgagatccaagaattccaggatgatgtccccaaggcagtaaatcaaatgcctgttgatgaggggttgttgtagtgactccaggactagaccccagctcagccggcatttgttcaccccaagaatttctactacgagatctgggaggactcccatcaggctctgcaaagcctgtttctcagcagccagtttctgctcttgggtccttacgggccgtggaaacttaggcaaaactccaccaggccagatggactcctgaagaagcaggaggtactgcacccagcgctgtggacttgttaaattagctacctgcacctctagccacctttgaactagggtcccaaagataagacgaagaaacttttgcatgttttcggtacatagccatttccactgttctgttagtagcaagaggagcagatccagggctgtgtcagctaactctgtctctgttcctggatcgctgttgctggggtcttgggctggcacggctgcatctgacacgcaactgtccacacgtcctttgggaggttgttcaggatctttttctggggcttttgttggctgcatttccagtaactttgtctgtttttcaataaaagattccatcgcagacatggatagagtctcagactccacattgccttcctggagacaataaagaatcttgtcttgtgcttcagtcacacttagtgctggagaaattttactggatgagaacctcagcctagaccttgtctattctagagaccataaatggtttcttgacaaaggcaatacgagcatctgtgttcagagcaaggaactcctgcacctcctcactgttagcgatctccggaatggcacagagttgctttaggaatgattctaggaggctcttacgggcttctactctgtcactgtccatgtttcccaatggaagatctggaaagagctttttaggacccttcacatacacgcagcgggcagcggccggcgaagactgggtcacacgccgccgggaaccgcgcgcccacactcagccccgacctgaagtggactcatcgcggtcctctccgggagcctcggccctctgccgccgtaaacctgggcgactgcgctccgcagccgggcctgtgtgaaggctgaccgccggccggccgccggcgacagct

SEQ ID NO: 8289 - RNA, 8187 nt, Homo sapiens
  source 1..8187: mol_type = other RNA
aaaaaccacaattacttttgcaccaacccactacatcagaacctacctttaagggttgatttgtgggttaaataagtgaagatatgtaaagactttaagtaatgctctcagaagatgttaactattagctggtaccaggcattttgggagtagataggggatctgctgaatgttggcagaatgacccatccctagagcagacattgtctatcaatacccattctctgcttcttccttgctaacatcaattatttctgtagatatctgaccttcatggaagatgacctcatctctgggggaaaatactattgaaagccaatcacaatgccattctcagtgtcagtggattggcatgaggtgggtggttctagccaatgagtcataagaggttttttgttttttttttttttatttggggtctcactctgtcacttaaggctagaatgcagtggtgtgatcgtagctcactgcagcctcaaattcctgggctcaagtgatcctcctgcctcagcctccctagtaggtggaaccacaggcgagagccaccatgccccgctcattttttatattttttgtagagacagggtcttgctatgttccaggctggtcttaaactcctggactcaaacaatcccccaaccttggcctcccaaagtgttgagattataggtgtgagccgctgtgcccggcctagaagaggattcttgaaggacttctgggaaatggttccttcattccttagaagaaaacacagaagagatgctcctgttcttttatgaatgttatctctgggtgtgatgcctgaaactgcagcagcaggaaggcaggcagtctgagagcacagctgacctaattagaatggcaaggaagaaagatggaaagaattcaggccccttaagaggtctcagagttgctgaatcaccaaactcctgggcttacctactcacgtactaatgttatgaaataaaataaattttcctcataatttaattcttgtccagagcatcctgattcatatagccagggaccatagttacacatatttttacttcctccaggacctaacaactggtgttgtgtgctatgagcaaaggaagagcagtagctggaaatgaataacctgggtaggacacaggaagactcaaaaatgttctaggctatgcaaatcaaaaccatgagatagtaatatcacctaataccttttaagatgccattatgaaaaaacaaaacattacaagtgttggagaggatgtggagaaactggaacccttgtacattgttggtgggaatgtaaaatggtctagtcactatggaaaacagtatgaaggtcttcaaagaattaaaaacagaacaatatatgatccagcaatcctacttctgggtatttatctaaaataattaaaagcagggcctcgaagaaacagtcacactcccatgttcactgcagcattgttttcaacaatcaaggcgcggagccaacctaaatgtccctcaatgaatgaacaaagaaaatgtggcatagccatacaatggaatgttttcagccttaaaaagaaaattctgtcacatgctgtaacgtggatgaacctggaggacattatgctaagtgaaataagccagtcaaaggacaaacactgcatgattccacttatatgaggcgttcaaagtagtcaaactcacagaagcagaaagtagaacagtgattgccagaggctggtgggaggggaaacgaggagtggctgttcaatgggtataaacttttggttatgcaagatgaaaaacttgtagcagtctgctacaaagcactgtgctgcttctagttaataatgtaccgtctcaaaataaataaataatgtactgtacacttaagagggtagatctcacattatgtgtttctttacaacaataagaaaatcaccttgtaaactggaaatttccaaaatggaaattggagtagcttgtattgattttaaaatttatacatgctctcactcataggtgggaattgaacaatgagaacacttggacacaggaaggtgaacatcacacactggggcctgttgtgaggtcgggggagggggaagggatagcatcaggagatatacctaatgtaaatgacgagttaacgggtgcagcacaccaacacggcacatgtatacatatgcaacaaacctgcatgttgtgcacatgttccctagaacttaatgtataataataataaaaataaaatttatacatgctcctaggctcagatttaggaatttattttccatttaggttttattaagtctaatccaacaatgcaaaaatgaaactgtgagttatatgtgatgaaaaagtatagctttcttgaattcaaataagcaatggcaaagatcacatttagaatttgacagaaagaacacagcatccctgcctcgtcttttttatagatagtaagaaaagggaaagtagtcttatttcaaatatcaaaattctgacttaaatgaataaaatttagtcacgagtaaatacaaaaaacaagcaaacaataaaaccttcctggatcagcacaggcccaattcttccctgccttttatcaccctgtcagctgggagtatcttttctacctgtggctctctaccaattgttactctcttgttgtctgaacctgctagccaaacttggcaggtcgttttcaaagccagatgagttctgattgttcccttggcaatatccattatttccctcctgggtagaaggaggatctgaggacagcttatctttttggggtacgtggagtagaggtggggactcttatataatacgaaataaaaataagttctttgggctggaagtgtcaaaagattccttagaatttatagccacagggatttcatggtgtgtctgatgtactgattttgtgccacatttgagccagaactggcagcagattcaaagcaacacaggtggctaagtacacatgaggggaaggtaggtatggggagagaaaagtggcataaaacaaggctgtccccctatgctcatcgagaataggatcttagccctcactgaaggagcttaatgatcagctctaatacattggctggactcctgcaggtactcacggaaagtagagatgctgagctaccttttcttgtcaaagtctagggctggagatgcttcaagaactttggagccataaagtcactgtaatggtcaacttttaaggctagaagaggccatgagacatctcattcatctccttgcctttgggcaagaattgcacacctaagcctcccgaatacatcagacacaatttagggttaaaagcctccagaggggcaaaaaagtaaaaagattttacaactttcttccacaaaccactttaattgtgtgctcatcaccgacttcagaatctaagagaactttgacacttgtttttgacaccccattgccttctcatcagtctaactccaagaccttcctccgagtggtaggctctggtaattcagcgaaagcaaggcgctaacaggcgagtgtgaagccaaagggctcccagtgacatccttgacatctttttgccagctattcacatgcatttaatatacagcacttccctgtgactgtctgcagccttttctaccagcaattcctcctgatttatccttctccagcaattcccagttgccttgcctttctaatagatgttgcagtctgacaaaacacctttgccttcatgctggtgttgttaaaggactgattataaccgtaaggaatgggaaataagaagctattccttgtaagtttgctaatcttatctgttcagaataataaaagttctctgtcaaagacttaggaagggagatttcatcccccagccttgctagtcctactctttgtgcattcttaagacaggaggcaagtgctttccattctccttggaaaaactgaggctgaatatgcagcttgtcatgcagttttgctgaagacagagagagggtcaaaaattcaaaaactcaattgctctagggcagggggttgggagcaaagccaataaataaaatgggtggtataaatgcctttcaggaaagggtgtgaagggtggggtggatttaccagaagctttggcagtcagctttgaagtcttctggaaaggaaagtgtagcctcccaggcaagcagcctcatgacatcttccataaggctgatgtgttgggaaacagcaacacatgagcaagaagttccttgaaaaattttcttccctccttcttcttctggaactgttgggaaactagattagacccaggagtctggtttttgagaatggccctgaatgaatttttagtttccgggtaggaacagagagctgagaaggttgttttctcctccaaggaaatctggccacagtttttttcctgttctatctagagcttgtgtgctggtggattaagcacatgtgtgcacagggccaggattctggcaaacaatctcagggaggatggcaaaaggagaagcaaaaggggttcattcctctacctcacagcttcttttcccaaaggaaacaggatctactcaccagcaacaatcccaacatcacaaaaggaacagggaaataaacgtgcatacaactgggacacacagacccctgtcacctgctacaaatggagcagaagtgggagagaagtgagccaccgagaacctaggccttcttagctgtagcctacttgaagagggcacgggcttcctgactggtctctggtggccgagtaactctacttccctgacctgggaagaaggcgtgaataaccagctaagaggagacacccatcctcttagagttgcctggggtatctgaggcagaggtggtagcagcagactcctcaacagaggcactgagatccaagaattccaggatgatgtccccaaggcagtaaatcaaatgcctgttgatgaggggttgttgtagtgactccaggactagaccccagctcagccggcatttgttcaccccaagaatttctactacgagatctgggaggactcccatcaggctctgcaaagcctgtttctcagcagccagtttctgctcttgggtccttacgggccgtggaaacttaggcaaaactccaccaggccagatggactcctgaagaagcaggaggtactgcacccagcgctgtggacttgttaaattagctacctgcacctctagccacctttgaactagggtcccaaagataagacgaagaaacttttgcatgttttcggtacatagccatttccactgttctgttagtagcaagaggagcagatccagggctgtgtcagctaactctgtctctgttcctggatcgctgttgctggggtcttgggctggcacggctgcatctgacacgcaactgtccacacgtcctttgggaggttgttcaggatctttttctggggcttttgttggctgcatttccagtaactttgtctgtttttcaataaaagattccatcgcagacatggatagagtctcagactccacattgccttcctggagacaataaagaatcttgtcttgtgcttcagtcacacttagtgctggagaaattttactggatgagaacctcagcctagaccttgtctattctagagaccataaatggtttcttgacaaaggcaatacgagcatctgtgttcagagcaaggaactcctgcacctcctcactgttagcgatctccggaatggcacagagttgctttaggaatgattctaggaggctcttacgggcttctactctgtcactgtccatgtttcccaatggaagatctggaaagagctttttaggacccttcacatttttgatgaactttcgtagatctggtttctcctccagacgggtctgcagattcaagaactcccgatagcgacgattcacagtgtggtaggccagctgctgcaggccgctgctgttttcaccgtcaagggctgtctcgtacttcacagtatagagtgtgtatgggtggaatccagtgccactgtgctctcgggctgtaatggtgccagtgatacgaaggttctggatgataactggaccatcgggactgcttaggggctcaaagctgaaggtggctgagctgagaggaccaggtggagaggaggaaagcagaactggtggcagagtaggatcaagggagctcacatcattggtgagatccttctctaagcatgacggccgtgaggggcaggtcttttctggcccctccagcaaagctgtaacagaggcggtaacatctccttgttctatctccttgtctgctgtgtcaatatggatctctgggcaggaattcagtgtggagaccggcaggcctgtctctgtttctgtccctggaccctcctcagcctctgctccttcagatgcctcaccatctttgggttccagagcctgggaactctctagggcacacagggcatcctgaatcctgtcagagagaaagctgcctggagtcatgagcatgatggtttctttgcccagttcagacagcggagactccagctctgagtcttcacataagaacaggggacctcgaacatttggctgtaggaaatgagatgagttgtttcctacttttctttcttcacacatcccacccaaatctccctctacagcttcgtggccttcttcaacctctggagaggggcctgcagaaccctctggctcactgtaacttaggaatactggggctgctactggagaagctctcccttctggaagctgctctacctcagcaatcagtggcagagatgtcggcactgagggctgttcgggggcactggctgggcagggtgctggatctctggccttggaaaagatacccacgagtacaaggtggatccagtcaggatctgacagcctgctgatcagtggtaagattacattgcatgtgatgagttcgaccactacatggcgtccggtacgagtctccaagtggggcttgggcaccagcccttgaagcaacaaattcacaacgccacgcgtataggtgacttcagcactggggctgtgcacagcaggatgtggggcagtcgcccggcagtaagcctcccagaggtgggaaggctcaactggaccattcttccctgcagtggcctcctttgcctgaatgtagctctgcaggtgacaaccgcagagagtcagaacactctgggcaacagcatgactgtccatcacgctcatccttctccgaagctcctggaccaaccctttcatggctgcctccatttcttcctcaaaggctggctcctggctcacggaacggtaccaagataacacaaaatctcgaataatcatctggatggtgcggttgatctcccgttccagctgcctttctgcctcagggcatggaggacaggtggccaacgggatgaagcgttccagatgcagtcgacctgaagccactccagcgaggctggagcccagccatcctcccagcaccactagcaatgccgacagaaggcacagcagccacacgttgaccagaaggtgtatgaccaggagccagccaagcaagacccccacagccatcagcttccggctactcaacaggttattgaggtgacagctcgatccagctggagtttcctggaacggtggcactgtttctgtcttcatggctgaacggacaaggtggcttccccagatgacagccctcaagattttacttcagagttagggaaggggggcatgaactgtgtctcagatatggggcgatctgggtgctgttcagggaaccggggctccaggccctcaaagtcctacaggcactgcaaagcgacagctgcagctccgcgtctccccatggctaccactaacagagccctccaactcgccccttccagctgaggtgtggctttggaggaaaactctgtggccttcacactgccccaggcggaaggcctcttcggggcctcggggcgggcgctgcaaggccctggggcccacggacacttacacacgcagcgggcagcggccggcgaagactgggtcacacgccgccgggaaccgcgcgcccacactcagccccgacctgaagtggactcatcgcggtcctctccgggagcctcggccctctgccgccgtaaacctgggcgactgcgctccgcagccgggcctgtgtgaaggctgaccgccggccggccgccggcgacagcttccgggtc

SEQ ID NO: 8290 - RNA, 6563 nt, Homo sapiens
  source 1..6563: mol_type = other RNA
aaaaaccacaattacttttgcaccaacccactacatcagaacctacctttaagggttgatttgtgggttaaataagtgaagatatgtaaagactttaagtaatgctctcagaagatgttaactattagctggtaccaggcattttgggagtagataggggatctgctgaatgttggcagaatgacccatccctagagcagacattgtctatcaatacccattctctgcttcttccttgctaacatcaattatttctgtagatatctgaccttcatggaagatgacctcatctctgggggaaaatactattgaaagccaatcacaatgccattctcagtgtcagtggattggcatgaggtgggtggttctagccaatgagtcataagaggttttttgttttttttttttttatttggggtctcactctgtcacttaaggctagaatgcagtggtgtgatcgtagctcactgcagcctcaaattcctgggctcaagtgatcctcctgcctcagcctccctagtaggtggaaccacaggcgagagccaccatgccccgctcattttttatattttttgtagagacagggtcttgctatgttccaggctggtcttaaactcctggactcaaacaatcccccaaccttggcctcccaaagtgttgagattataggtgtgagccgctgtgcccggcctagaagaggattcttgaaggacttctgggaaatggttccttcattccttagaagaaaacacagaagagatgctcctgttcttttatgaatgttatctctgggtgtgatgcctgaaactgcagcagcaggaaggcaggcagtctgagagcacagctgacctaattagaatggcaaggaagaaagatggaaagaattcaggccccttaagaggtctcagagttgctgaatcaccaaactcctgggcttacctactcacgtactaatgttatgaaataaaataaattttcctcataatttaattcttgtccagagcatcctgattcatatagccagggaccatagttacacatatttttacttcctccaggacctaacaactggtgttgtgtgctatgagcaaaggaagagcagtagctggaaatgaataacctgggtaggacacaggaagactcaaaaatgttctaggctatgcaaatcaaaaccatgagatagtaatatcacctaataccttttaagatgccattatgaaaaaacaaaacattacaagtgttggagaggatgtggagaaactggaacccttgtacattgttggtgggaatgtaaaatggtctagtcactatggaaaacagtatgaaggtcttcaaagaattaaaaacagaacaatatatgatccagcaatcctacttctgggtatttatctaaaataattaaaagcagggcctcgaagaaacagtcacactcccatgttcactgcagcattgttttcaacaatcaaggcgcggagccaacctaaatgtccctcaatgaatgaacaaagaaaatgtggcatagccatacaatggaatgttttcagccttaaaaagaaaattctgtcacatgctgtaacgtggatgaacctggaggacattatgctaagtgaaataagccagtcaaaggacaaacactgcatgattccacttatatgaggcgttcaaagtagtcaaactcacagaagcagaaagtagaacagtgattgccagaggctggtgggaggggaaacgaggagtggctgttcaatgggtataaacttttggttatgcaagatgaaaaacttgtagcagtctgctacaaagcactgtgctgcttctagttaataatgtaccgtctcaaaataaataaataatgtactgtacacttaagagggtagatctcacattatgtgtttctttacaacaataagaaaatcaccttgtaaactggaaatttccaaaatggaaattggagtagcttgtattgattttaaaatttatacatgctctcactcataggtgggaattgaacaatgagaacacttggacacaggaaggtgaacatcacacactggggcctgttgtgaggtcgggggagggggaagggatagcatcaggagatatacctaatgtaaatgacgagttaacgggtgcagcacaccaacacggcacatgtatacatatgcaacaaacctgcatgttgtgcacatgttccctagaacttaatgtataataataataaaaataaaatttatacatgctcctaggctcagatttaggaatttattttccatttaggttttattaagtctaatccaacaatgcaaaaatgaaactgtgagttatatgtgatgaaaaagtatagctttcttgaattcaaataagcaatggcaaagatcacatttagaatttgacagaaagaacacagcatccctgcctcgtcttttttatagatagtaagaaaagggaaagtagtcttatttcaaatatcaaaattctgacttaaatgaataaaatttagtcacgagtaaatacaaaaaacaagcaaacaataaaaccttcctggatcagcacaggcccaattcttccctgccttttatcaccctgtcagctgggagtatcttttctacctgtggctctctaccaattgttactctcttgttgtctgaacctgctagccaaacttggcaggtcgttttcaaagccagatgagttctgattgttcccttggcaatatccattatttccctcctgggtagaaggaggatctgaggacagcttatctttttggggtacgtggagtagaggtggggactcttatataatacgaaataaaaataagttctttgggctggaagtgtcaaaagattccttagaatttatagccacagggatttcatggtgtgtctgatgtactgattttgtgccacatttgagccagaactggcagcagattcaaagcaacacaggtggctaagtacacatgaggggaaggtaggtatggggagagaaaagtggcataaaacaaggctgtccccctatgctcatcgagaataggatcttagccctcactgaaggagcttaatgatcagctctaatacattggctggactcctgcaggtactcacggaaagtagagatgctgagctaccttttcttgtcaaagtctagggctggagatgcttcaagaactttggagccataaagtcactgtaatggtcaacttttaaggctagaagaggccatgagacatctcattcatctccttgcctttgggcaagaattgcacacctaagcctcccgaatacatcagacacaatttagggttaaaagcctccagaggggcaaaaaagtaaaaagattttacaactttcttccacaaaccactttaattgtgtgctcatcaccgacttcagaatctaagagaactttgacacttgtttttgacaccccattgccttctcatcagtctaactccaagaccttcctccgagtggtaggctctggtaattcagcgaaagcaaggcgctaacaggcgagtgtgaagccaaagggctcccagtgacatccttgacatctttttgccagctattcacatgcatttaatatacagcacttccctgtgactgtctgcagccttttctaccagcaattcctcctgatttatccttctccagcaattcccagttgccttgcctttctaatagatgttgcagtctgacaaaacacctttgccttcatgctggtgttgttaaaggactgattataaccgtaaggaatgggaaataagaagctattccttgtaagtttgctaatcttatctgttcagaataataaaagttctctgtcaaagacttaggaagggagatttcatcccccagccttgctagtcctactctttgtgcattcttaagacaggaggcaagtgctttccattctccttggaaaaactgaggctgaatatgcagcttgtcatgcagttttgctgaagacagagagagggtcaaaaattcaaaaactcaattgctctagggcagggggttgggagcaaagccaataaataaaatgggtggtataaatgcctttcaggaaagggtgtgaagggtggggtggatttaccagaagctttggcagtcagctttgaagtcttctggaaaggaaagtgtagcctcccaggcaagcagcctcatgacatcttccataaggctgatgtgttgggaaacagcaacacatgagcaagaagttccttgaaaaattttcttccctccttcttcttctggaactgttgggaaactagattagacccaggagtctggtttttgagaatggccctgaatgaatttttagtttccgggtaggaacagagagctgagaaggttgttttctcctccaaggaaatctggccacagtttttttcctgttctatctagagcttgtgtgctggtggattaagcacatgtgtgcacagggccaggattctggcaaacaatctcagggaggatggcaaaaggagaagcaaaaggggttcattcctctacctcacagcttcttttcccaaaggaaacaggatctactcaccagcaacaatcccaacatcacaaaaggaacagggaaataaacgtgcatacaactgggacacacagacccctgtcacctgctacaaatggagcagaagtgggagagaagtgagccaccgagaacctaggccttcttagctgtagcctacttgaagagggcacgggcttcctgactggtctctggtggccgagtaactctacttccctgacctgggaagaaggcgtgaataaccagctaagaggagacacccatcctcttagagttgcctggggtatctgaggcagaggtggtagcagcagactcctcaacagaggcactgagatccaagaattccaggatgatgtccccaaggcagtaaatcaaatgcctgttgatgaggggttgttgtagtgactccaggactagaccccagctcagccggcatttgttcaccccaagaatttctactacgagatctgggaggactcccatcaggctctgcaaagcctgtttctcagcagccagtttctgctcttgggtccttacgggccgtggaaacttaggcaaaactccaccaggccagatggactcctgaagaagcaggaggtactgcacccagcgctgtggacttgttaaattagctacctgcacctctagccacctttgaactagggtcccaaagataagacgaagaaacttttgcatgttttcggtacatagccatttccactgttctgttagtagcaagaggagcagatccagggctgtgtcagctaactctgtctctgttcctggatcgctgttgctggggtcttgggctggcacggctgcatctgacacgcaactgtccacacgtcctttgggaggttgttcaggatctttttctggggcttttgttggctgcatttccagtaactttgtctgtttttcaataaaagattccatcgcagacatggatagagtctcagactccacattgccttcctggagacaataaagaatcttgtcttgtgcttcagtcacacttagtgctggagaaattttactggatgagaacctcagcctagacttgctagccttcttgccttctgtctggggcttgctttcggtctcggcctcactcagctcctctgtggggctctggggttcagagcgaggaaacgctgtcttcaaggtgtccacaatggcactcaccaccatctgagttctgcgggctggtgatgtatttttcaatttctttctttttaagtaaaaaggtgatttctagtttccaaatcggtaacaccttgtctattctagagaccataaatggtttcttgacaaaggcaatacgagcatctgtgttcagagcaaggaactcctgcacctcctcactgttagcgatctccggaatggcacagagttgctttaggaatgattctaggaggctcttacgggcttctactctgtcactgtccatgtttcccaatggaagatctggaaagagctttttaggacccttcacatctctgaaagaatgtgattgctgctgtccagcactaaacttcaaaactcctgaagcaaatccagggagcagagaaccttgaaacggcattctcctccccgatccctcccataaaccaacaggccaatcagcgtggctcgacgtgggaagcaagcgggcagtaggggttggggaaactcctgacttttgatgaactttcgtagatctggtttctcctccagacgggtctgcagattcaagaactcccgatagcgacgattcacagtgtggtaggccagctgctgcaggccgctgctgttttcaccgtcaagggctgtctcgtaacacgcagcgggcagcggccggcgaagactgggtcacacgccgccgggaaccgcgcgcccacactcagccccgacctgaagtggactcatcgcggtcctctccgggagcctcggccctctgccgccgtaaacctgggcgactgcgctccgcagccgggcctgtgtgaaggctgaccgccggccggccgccggcgacagct

SEQ ID NO: 8291 - RNA, 8395 nt, Homo sapiens
  source 1..8395: mol_type = other RNA
aaaaaccacaattacttttgcaccaacccactacatcagaacctacctttaagggttgatttgtgggttaaataagtgaagatatgtaaagactttaagtaatgctctcagaagatgttaactattagctggtaccaggcattttgggagtagataggggatctgctgaatgttggcagaatgacccatccctagagcagacattgtctatcaatacccattctctgcttcttccttgctaacatcaattatttctgtagatatctgaccttcatggaagatgacctcatctctgggggaaaatactattgaaagccaatcacaatgccattctcagtgtcagtggattggcatgaggtgggtggttctagccaatgagtcataagaggttttttgttttttttttttttatttggggtctcactctgtcacttaaggctagaatgcagtggtgtgatcgtagctcactgcagcctcaaattcctgggctcaagtgatcctcctgcctcagcctccctagtaggtggaaccacaggcgagagccaccatgccccgctcattttttatattttttgtagagacagggtcttgctatgttccaggctggtcttaaactcctggactcaaacaatcccccaaccttggcctcccaaagtgttgagattataggtgtgagccgctgtgcccggcctagaagaggattcttgaaggacttctgggaaatggttccttcattccttagaagaaaacacagaagagatgctcctgttcttttatgaatgttatctctgggtgtgatgcctgaaactgcagcagcaggaaggcaggcagtctgagagcacagctgacctaattagaatggcaaggaagaaagatggaaagaattcaggccccttaagaggtctcagagttgctgaatcaccaaactcctgggcttacctactcacgtactaatgttatgaaataaaataaattttcctcataatttaattcttgtccagagcatcctgattcatatagccagggaccatagttacacatatttttacttcctccaggacctaacaactggtgttgtgtgctatgagcaaaggaagagcagtagctggaaatgaataacctgggtaggacacaggaagactcaaaaatgttctaggctatgcaaatcaaaaccatgagatagtaatatcacctaataccttttaagatgccattatgaaaaaacaaaacattacaagtgttggagaggatgtggagaaactggaacccttgtacattgttggtgggaatgtaaaatggtctagtcactatggaaaacagtatgaaggtcttcaaagaattaaaaacagaacaatatatgatccagcaatcctacttctgggtatttatctaaaataattaaaagcagggcctcgaagaaacagtcacactcccatgttcactgcagcattgttttcaacaatcaaggcgcggagccaacctaaatgtccctcaatgaatgaacaaagaaaatgtggcatagccatacaatggaatgttttcagccttaaaaagaaaattctgtcacatgctgtaacgtggatgaacctggaggacattatgctaagtgaaataagccagtcaaaggacaaacactgcatgattccacttatatgaggcgttcaaagtagtcaaactcacagaagcagaaagtagaacagtgattgccagaggctggtgggaggggaaacgaggagtggctgttcaatgggtataaacttttggttatgcaagatgaaaaacttgtagcagtctgctacaaagcactgtgctgcttctagttaataatgtaccgtctcaaaataaataaataatgtactgtacacttaagagggtagatctcacattatgtgtttctttacaacaataagaaaatcaccttgtaaactggaaatttccaaaatggaaattggagtagcttgtattgattttaaaatttatacatgctctcactcataggtgggaattgaacaatgagaacacttggacacaggaaggtgaacatcacacactggggcctgttgtgaggtcgggggagggggaagggatagcatcaggagatatacctaatgtaaatgacgagttaacgggtgcagcacaccaacacggcacatgtatacatatgcaacaaacctgcatgttgtgcacatgttccctagaacttaatgtataataataataaaaataaaatttatacatgctcctaggctcagatttaggaatttattttccatttaggttttattaagtctaatccaacaatgcaaaaatgaaactgtgagttatatgtgatgaaaaagtatagctttcttgaattcaaataagcaatggcaaagatcacatttagaatttgacagaaagaacacagcatccctgcctcgtcttttttatagatagtaagaaaagggaaagtagtcttatttcaaatatcaaaattctgacttaaatgaataaaatttagtcacgagtaaatacaaaaaacaagcaaacaataaaaccttcctggatcagcacaggcccaattcttccctgccttttatcaccctgtcagctgggagtatcttttctacctgtggctctctaccaattgttactctcttgttgtctgaacctgctagccaaacttggcaggtcgttttcaaagccagatgagttctgattgttcccttggcaatatccattatttccctcctgggtagaaggaggatctgaggacagcttatctttttggggtacgtggagtagaggtggggactcttatataatacgaaataaaaataagttctttgggctggaagtgtcaaaagattccttagaatttatagccacagggatttcatggtgtgtctgatgtactgattttgtgccacatttgagccagaactggcagcagattcaaagcaacacaggtggctaagtacacatgaggggaaggtaggtatggggagagaaaagtggcataaaacaaggctgtccccctatgctcatcgagaataggatcttagccctcactgaaggagcttaatgatcagctctaatacattggctggactcctgcaggtactcacggaaagtagagatgctgagctaccttttcttgtcaaagtctagggctggagatgcttcaagaactttggagccataaagtcactgtaatggtcaacttttaaggctagaagaggccatgagacatctcattcatctccttgcctttgggcaagaattgcacacctaagcctcccgaatacatcagacacaatttagggttaaaagcctccagaggggcaaaaaagtaaaaagattttacaactttcttccacaaaccactttaattgtgtgctcatcaccgacttcagaatctaagagaactttgacacttgtttttgacaccccattgccttctcatcagtctaactccaagaccttcctccgagtggtaggctctggtaattcagcgaaagcaaggcgctaacaggcgagtgtgaagccaaagggctcccagtgacatccttgacatctttttgccagctattcacatgcatttaatatacagcacttccctgtgactgtctgcagccttttctaccagcaattcctcctgatttatccttctccagcaattcccagttgccttgcctttctaatagatgttgcagtctgacaaaacacctttgccttcatgctggtgttgttaaaggactgattataaccgtaaggaatgggaaataagaagctattccttgtaagtttgctaatcttatctgttcagaataataaaagttctctgtcaaagacttaggaagggagatttcatcccccagccttgctagtcctactctttgtgcattcttaagacaggaggcaagtgctttccattctccttggaaaaactgaggctgaatatgcagcttgtcatgcagttttgctgaagacagagagagggtcaaaaattcaaaaactcaattgctctagggcagggggttgggagcaaagccaataaataaaatgggtggtataaatgcctttcaggaaagggtgtgaagggtggggtggatttaccagaagctttggcagtcagctttgaagtcttctggaaaggaaagtgtagcctcccaggcaagcagcctcatgacatcttccataaggctgatgtgttgggaaacagcaacacatgagcaagaagttccttgaaaaattttcttccctccttcttcttctggaactgttgggaaactagattagacccaggagtctggtttttgagaatggccctgaatgaatttttagtttccgggtaggaacagagagctgagaaggttgttttctcctccaaggaaatctggccacagtttttttcctgttctatctagagcttgtgtgctggtggattaagcacatgtgtgcacagggccaggattctggcaaacaatctcagggaggatggcaaaaggagaagcaaaaggggttcattcctctacctcacagcttcttttcccaaaggaaacaggatctactcaccagcaacaatcccaacatcacaaaaggaacagggaaataaacgtgcatacaactgggacacacagacccctgtcacctgctacaaatggagcagaagtgggagagaagtgagccaccgagaacctaggccttcttagctgtagcctacttgaagagggcacgggcttcctgactggtctctggtggccgagtaactctacttccctgacctgggaagaaggcgtgaataaccagctaagaggagacacccatcctcttagagttgcctggggtatctgaggcagaggtggtagcagcagactcctcaacagaggcactgagatccaagaattccaggatgatgtccccaaggcagtaaatcaaatgcctgttgatgaggggttgttgtagtgactccaggactagaccccagctcagccggcatttgttcaccccaagaatttctactacgagatctgggaggactcccatcaggctctgcaaagcctgtttctcagcagccagtttctgctcttgggtccttacgggccgtggaaacttaggcaaaactccaccaggccagatggactcctgaagaagcaggaggtactgcacccagcgctgtggacttgttaaattagctacctgcacctctagccacctttgaactagggtcccaaagataagacgaagaaacttttgcatgttttcggtacatagccatttccactgttctgttagtagcaagaggagcagatccagggctgtgtcagctaactctgtctctgttcctggatcgctgttgctggggtcttgggctggcacggctgcatctgacacgcaactgtccacacgtcctttgggaggttgttcaggatctttttctggggcttttgttggctgcatttccagtaactttgtctgtttttcaataaaagattccatcgcagacatggatagagtctcagactccacattgccttcctggagacaataaagaatcttgtcttgtgcttcagtcacacttagtgctggagaaattttactggatgagaacctcagcctagacttgctagccttcttgccttctgtctggggcttgctttcggtctcggcctcactcagctcctctgtggggctctggggttcagagcgaggaaacgctgtcttcaaggtgtccacaatggcactcaccaccatctgagttctgcgggctggtgatgtatttttcaatttctttctttttaagtaaaaaggtgatttctagtttccaaatcggtaacaccttgtctattctagagaccataaatggtttcttgacaaaggcaatacgagcatctgtgttcagagcaaggaactcctgcacctcctcactgttagcgatctccggaatggcacagagttgctttaggaatgattctaggaggctcttacgggcttctactctgtcactgtccatgtttcccaatggaagatctggaaagagctttttaggacccttcacatttttgatgaactttcgtagatctggtttctcctccagacgggtctgcagattcaagaactcccgatagcgacgattcacagtgtggtaggccagctgctgcaggccgctgctgttttcaccgtcaagggctgtctcgtacttcacagtatagagtgtgtatgggtggaatccagtgccactgtgctctcgggctgtaatggtgccagtgatacgaaggttctggatgataactggaccatcgggactgcttaggggctcaaagctgaaggtggctgagctgagaggaccaggtggagaggaggaaagcagaactggtggcagagtaggatcaagggagctcacatcattggtgagatccttctctaagcatgacggccgtgaggggcaggtcttttctggcccctccagcaaagctgtaacagaggcggtaacatctccttgttctatctccttgtctgctgtgtcaatatggatctctgggcaggaattcagtgtggagaccggcaggcctgtctctgtttctgtccctggaccctcctcagcctctgctccttcagatgcctcaccatctttgggttccagagcctgggaactctctagggcacacagggcatcctgaatcctgtcagagagaaagctgcctggagtcatgagcatgatggtttctttgcccagttcagacagcggagactccagctctgagtcttcacataagaacaggggacctcgaacatttggctgtaggaaatgagatgagttgtttcctacttttctttcttcacacatcccacccaaatctccctctacagcttcgtggccttcttcaacctctggagaggggcctgcagaaccctctggctcactgtaacttaggaatactggggctgctactggagaagctctcccttctggaagctgctctacctcagcaatcagtggcagagatgtcggcactgagggctgttcgggggcactggctgggcagggtgctggatctctggccttggaaaagatacccacgagtacaaggtggatccagtcaggatctgacagcctgctgatcagtggtaagattacattgcatgtgatgagttcgaccactacatggcgtccggtacgagtctccaagtggggcttgggcaccagcccttgaagcaacaaattcacaacgccacgcgtataggtgacttcagcactggggctgtgcacagcaggatgtggggcagtcgcccggcagtaagcctcccagaggtgggaaggctcaactggaccattcttccctgcagtggcctcctttgcctgaatgtagctctgcaggtgacaaccgcagagagtcagaacactctgggcaacagcatgactgtccatcacgctcatccttctccgaagctcctggaccaaccctttcatggctgcctccatttcttcctcaaaggctggctcctggctcacggaacggtaccaagataacacaaaatctcgaataatcatctggatggtgcggttgatctcccgttccagctgcctttctgcctcagggcatggaggacaggtggccaacgggatgaagcgttccagatgcagtcgacctgaagccactccagcgaggctggagcccagccatcctcccagcaccactagcaatgccgacagaaggcacagcagccacacgttgaccagaaggtgtatgaccaggagccagccaagcaagacccccacagccatcagcttccggctactcaacaggttattgaggtgacagctcgatccagctggagtttcctggaacggtggcactgtttctgtcttcatggctgaacggacaaggtggcttccccagatgacagccctcaagattttacttcagagttagggaaggggggcatgaactgtgtctcagatatggggcgatctgggtgctgttcagggaaccggggctccaggccctcaaagtcctacaggcactgcaaagcgacagctgcagctccgcgtctccccatggctaccactaacagagccctccaactcgccccttccagctgaggtgtggctttggaggaaaactctgtggccttcacactgccccaggcggaaggcctcttcggggcctcggggcgggcgctgcaaggccctggggcccacggacacttacacacgcagcgggcagcggccggcgaagactgggtcacacgccgccgggaaccgcgcgcccacactcagccccgacctgaagtggactcatcgcggtcctctccgggagcctcggccctctgccgccgtaaacctgggcgactgcgctccgcagccgggcctgtgtgaaggctgaccgccggccggccgccggcgacagct

SEQ ID NO: 8292 - RNA, 6478 nt, Homo sapiens
  source 1..6478: mol_type = other RNA
aaaaaccacaattacttttgcaccaacccactacatcagaacctacctttaagggttgatttgtgggttaaataagtgaagatatgtaaagactttaagtaatgctctcagaagatgttaactattagctggtaccaggcattttgggagtagataggggatctgctgaatgttggcagaatgacccatccctagagcagacattgtctatcaatacccattctctgcttcttccttgctaacatcaattatttctgtagatatctgaccttcatggaagatgacctcatctctgggggaaaatactattgaaagccaatcacaatgccattctcagtgtcagtggattggcatgaggtgggtggttctagccaatgagtcataagaggttttttgttttttttttttttatttggggtctcactctgtcacttaaggctagaatgcagtggtgtgatcgtagctcactgcagcctcaaattcctgggctcaagtgatcctcctgcctcagcctccctagtaggtggaaccacaggcgagagccaccatgccccgctcattttttatattttttgtagagacagggtcttgctatgttccaggctggtcttaaactcctggactcaaacaatcccccaaccttggcctcccaaagtgttgagattataggtgtgagccgctgtgcccggcctagaagaggattcttgaaggacttctgggaaatggttccttcattccttagaagaaaacacagaagagatgctcctgttcttttatgaatgttatctctgggtgtgatgcctgaaactgcagcagcaggaaggcaggcagtctgagagcacagctgacctaattagaatggcaaggaagaaagatggaaagaattcaggccccttaagaggtctcagagttgctgaatcaccaaactcctgggcttacctactcacgtactaatgttatgaaataaaataaattttcctcataatttaattcttgtccagagcatcctgattcatatagccagggaccatagttacacatatttttacttcctccaggacctaacaactggtgttgtgtgctatgagcaaaggaagagcagtagctggaaatgaataacctgggtaggacacaggaagactcaaaaatgttctaggctatgcaaatcaaaaccatgagatagtaatatcacctaataccttttaagatgccattatgaaaaaacaaaacattacaagtgttggagaggatgtggagaaactggaacccttgtacattgttggtgggaatgtaaaatggtctagtcactatggaaaacagtatgaaggtcttcaaagaattaaaaacagaacaatatatgatccagcaatcctacttctgggtatttatctaaaataattaaaagcagggcctcgaagaaacagtcacactcccatgttcactgcagcattgttttcaacaatcaaggcgcggagccaacctaaatgtccctcaatgaatgaacaaagaaaatgtggcatagccatacaatggaatgttttcagccttaaaaagaaaattctgtcacatgctgtaacgtggatgaacctggaggacattatgctaagtgaaataagccagtcaaaggacaaacactgcatgattccacttatatgaggcgttcaaagtagtcaaactcacagaagcagaaagtagaacagtgattgccagaggctggtgggaggggaaacgaggagtggctgttcaatgggtataaacttttggttatgcaagatgaaaaacttgtagcagtctgctacaaagcactgtgctgcttctagttaataatgtaccgtctcaaaataaataaataatgtactgtacacttaagagggtagatctcacattatgtgtttctttacaacaataagaaaatcaccttgtaaactggaaatttccaaaatggaaattggagtagcttgtattgattttaaaatttatacatgctctcactcataggtgggaattgaacaatgagaacacttggacacaggaaggtgaacatcacacactggggcctgttgtgaggtcgggggagggggaagggatagcatcaggagatatacctaatgtaaatgacgagttaacgggtgcagcacaccaacacggcacatgtatacatatgcaacaaacctgcatgttgtgcacatgttccctagaacttaatgtataataataataaaaataaaatttatacatgctcctaggctcagatttaggaatttattttccatttaggttttattaagtctaatccaacaatgcaaaaatgaaactgtgagttatatgtgatgaaaaagtatagctttcttgaattcaaataagcaatggcaaagatcacatttagaatttgacagaaagaacacagcatccctgcctcgtcttttttatagatagtaagaaaagggaaagtagtcttatttcaaatatcaaaattctgacttaaatgaataaaatttagtcacgagtaaatacaaaaaacaagcaaacaataaaaccttcctggatcagcacaggcccaattcttccctgccttttatcaccctgtcagctgggagtatcttttctacctgtggctctctaccaattgttactctcttgttgtctgaacctgctagccaaacttggcaggtcgttttcaaagccagatgagttctgattgttcccttggcaatatccattatttccctcctgggtagaaggaggatctgaggacagcttatctttttggggtacgtggagtagaggtggggactcttatataatacgaaataaaaataagttctttgggctggaagtgtcaaaagattccttagaatttatagccacagggatttcatggtgtgtctgatgtactgattttgtgccacatttgagccagaactggcagcagattcaaagcaacacaggtggctaagtacacatgaggggaaggtaggtatggggagagaaaagtggcataaaacaaggctgtccccctatgctcatcgagaataggatcttagccctcactgaaggagcttaatgatcagctctaatacattggctggactcctgcaggtactcacggaaagtagagatgctgagctaccttttcttgtcaaagtctagggctggagatgcttcaagaactttggagccataaagtcactgtaatggtcaacttttaaggctagaagaggccatgagacatctcattcatctccttgcctttgggcaagaattgcacacctaagcctcccgaatacatcagacacaatttagggttaaaagcctccagaggggcaaaaaagtaaaaagattttacaactttcttccacaaaccactttaattgtgtgctcatcaccgacttcagaatctaagagaactttgacacttgtttttgacaccccattgccttctcatcagtctaactccaagaccttcctccgagtggtaggctctggtaattcagcgaaagcaaggcgctaacaggcgagtgtgaagccaaagggctcccagtgacatccttgacatctttttgccagctattcacatgcatttaatatacagcacttccctgtgactgtctgcagccttttctaccagcaattcctcctgatttatccttctccagcaattcccagttgccttgcctttctaatagatgttgcagtctgacaaaacacctttgccttcatgctggtgttgttaaaggactgattataaccgtaaggaatgggaaataagaagctattccttgtaagtttgctaatcttatctgttcagaataataaaagttctctgtcaaagacttaggaagggagatttcatcccccagccttgctagtcctactctttgtgcattcttaagacaggaggcaagtgctttccattctccttggaaaaactgaggctgaatatgcagcttgtcatgcagttttgctgaagacagagagagggtcaaaaattcaaaaactcaattgctctagggcagggggttgggagcaaagccaataaataaaatgggtggtataaatgcctttcaggaaagggtgtgaagggtggggtggatttaccagaagctttggcagtcagctttgaagtcttctggaaaggaaagtgtagcctcccaggcaagcagcctcatgacatcttccataaggctgatgtgttgggaaacagcaacacatgagcaagaagttccttgaaaaattttcttccctccttcttcttctggaactgttgggaaactagattagacccaggagtctggtttttgagaatggccctgaatgaatttttagtttccgggtaggaacagagagctgagaaggttgttttctcctccaaggaaatctggccacagtttttttcctgttctatctagagcttgtgtgctggtggattaagcacatgtgtgcacagggccaggattctggcaaacaatctcagggaggatggcaaaaggagaagcaaaaggggttcattcctctacctcacagcttcttttcccaaaggaaacaggatctactcaccagcaacaatcccaacatcacaaaaggaacagggaaataaacgtgcatacaactgggacacacagacccctgtcacctgctacaaatggagcagaagtgggagagaagtgagccaccgagaacctaggccttcttagctgtagcctacttgaagagggcacgggcttcctgactggtctctggtggccgagtaactctacttccctgacctgggaagaaggcgtgaataaccagctaagaggagacacccatcctcttagagttgcctggggtatctgaggcagaggtggtagcagcagactcctcaacagaggcactgagatccaagaattccaggatgatgtccccaaggcagtaaatcaaatgcctgttgatgaggggttgttgtagtgactccaggactagaccccagctcagccggcatttgttcaccccaagaatttctactacgagatctgggaggactcccatcaggctctgcaaagcctgtttctcagcagccagtttctgctcttgggtccttacgggccgtggaaacttaggcaaaactccaccaggccagatggactcctgaagaagcaggaggtactgcacccagcgctgtggacttgttaaattagctacctgcacctctagccacctttgaactagggtcccaaagataagacgaagaaacttttgcatgttttcggtacatagccatttccactgttctgttagtagcaagaggagcagatccagggctgtgtcagctaactctgtctctgttcctggatcgctgttgctggggtcttgggctggcacggctgcatctgacacgcaactgtccacacgtcctttgggaggttgttcaggatctttttctggggcttttgttggctgcatttccagtaactttgtctgtttttcaataaaagattccatcgcagacatggatagagtctcagactccacattgccttcctggagacaataaagaatcttgtcttgtgcttcagtcacacttagtgctggagaaattttactggatgagaacctcagcctagacttgctagccttcttgccttctgtctggggcttgctttcggtctcggcctcactcagctcctctgtggggctctggggttcagagcgaggaaacgctgtcttcaaggtgtccacaatggcactcaccaccatcttgtctattctagagaccataaatggtttcttgacaaaggcaatacgagcatctgtgttcagagcaaggaactcctgcacctcctcactgttagcgatctccggaatggcacagagttgctttaggaatgattctaggaggctcttacgggcttctactctgtcactgtccatgtttcccaatggaagatctggaaagagctttttaggacccttcacatctctgaaagaatgtgattgctgctgtccagcactaaacttcaaaactcctgaagcaaatccagggagcagagaaccttgaaacggcattctcctccccgatccctcccataaaccaacaggccaatcagcgtggctcgacgtgggaagcaagcgggcagtaggggttggggaaactcctgacttttgatgaactttcgtagatctggtttctcctccagacgggtctgcagattcaagaactcccgatagcgacgattcacagtgtggtaggccagctgctgcaggccgctgctgttttcaccgtcaagggctgtctcgtaacacgcagcgggcagcggccggcgaagactgggtcacacgccgccgggaaccgcgcgcccacactcagccccgacctgaagtggactcatcgcggtcctctccgggagcctcggccctctgccgccgtaaacctgggcgactgcgctccgcagccgggcctgtgtgaaggctgaccgccggccggccgccggcgacagct

SEQ ID NO: 8293 - RNA, 8501 nt, Homo sapiens
  source 1..8501: mol_type = other RNA
aaaaaccacaattacttttgcaccaacccactacatcagaacctacctttaagggttgatttgtgggttaaataagtgaagatatgtaaagactttaagtaatgctctcagaagatgttaactattagctggtaccaggcattttgggagtagataggggatctgctgaatgttggcagaatgacccatccctagagcagacattgtctatcaatacccattctctgcttcttccttgctaacatcaattatttctgtagatatctgaccttcatggaagatgacctcatctctgggggaaaatactattgaaagccaatcacaatgccattctcagtgtcagtggattggcatgaggtgggtggttctagccaatgagtcataagaggttttttgttttttttttttttatttggggtctcactctgtcacttaaggctagaatgcagtggtgtgatcgtagctcactgcagcctcaaattcctgggctcaagtgatcctcctgcctcagcctccctagtaggtggaaccacaggcgagagccaccatgccccgctcattttttatattttttgtagagacagggtcttgctatgttccaggctggtcttaaactcctggactcaaacaatcccccaaccttggcctcccaaagtgttgagattataggtgtgagccgctgtgcccggcctagaagaggattcttgaaggacttctgggaaatggttccttcattccttagaagaaaacacagaagagatgctcctgttcttttatgaatgttatctctgggtgtgatgcctgaaactgcagcagcaggaaggcaggcagtctgagagcacagctgacctaattagaatggcaaggaagaaagatggaaagaattcaggccccttaagaggtctcagagttgctgaatcaccaaactcctgggcttacctactcacgtactaatgttatgaaataaaataaattttcctcataatttaattcttgtccagagcatcctgattcatatagccagggaccatagttacacatatttttacttcctccaggacctaacaactggtgttgtgtgctatgagcaaaggaagagcagtagctggaaatgaataacctgggtaggacacaggaagactcaaaaatgttctaggctatgcaaatcaaaaccatgagatagtaatatcacctaataccttttaagatgccattatgaaaaaacaaaacattacaagtgttggagaggatgtggagaaactggaacccttgtacattgttggtgggaatgtaaaatggtctagtcactatggaaaacagtatgaaggtcttcaaagaattaaaaacagaacaatatatgatccagcaatcctacttctgggtatttatctaaaataattaaaagcagggcctcgaagaaacagtcacactcccatgttcactgcagcattgttttcaacaatcaaggcgcggagccaacctaaatgtccctcaatgaatgaacaaagaaaatgtggcatagccatacaatggaatgttttcagccttaaaaagaaaattctgtcacatgctgtaacgtggatgaacctggaggacattatgctaagtgaaataagccagtcaaaggacaaacactgcatgattccacttatatgaggcgttcaaagtagtcaaactcacagaagcagaaagtagaacagtgattgccagaggctggtgggaggggaaacgaggagtggctgttcaatgggtataaacttttggttatgcaagatgaaaaacttgtagcagtctgctacaaagcactgtgctgcttctagttaataatgtaccgtctcaaaataaataaataatgtactgtacacttaagagggtagatctcacattatgtgtttctttacaacaataagaaaatcaccttgtaaactggaaatttccaaaatggaaattggagtagcttgtattgattttaaaatttatacatgctctcactcataggtgggaattgaacaatgagaacacttggacacaggaaggtgaacatcacacactggggcctgttgtgaggtcgggggagggggaagggatagcatcaggagatatacctaatgtaaatgacgagttaacgggtgcagcacaccaacacggcacatgtatacatatgcaacaaacctgcatgttgtgcacatgttccctagaacttaatgtataataataataaaaataaaatttatacatgctcctaggctcagatttaggaatttattttccatttaggttttattaagtctaatccaacaatgcaaaaatgaaactgtgagttatatgtgatgaaaaagtatagctttcttgaattcaaataagcaatggcaaagatcacatttagaatttgacagaaagaacacagcatccctgcctcgtcttttttatagatagtaagaaaagggaaagtagtcttatttcaaatatcaaaattctgacttaaatgaataaaatttagtcacgagtaaatacaaaaaacaagcaaacaataaaaccttcctggatcagcacaggcccaattcttccctgccttttatcaccctgtcagctgggagtatcttttctacctgtggctctctaccaattgttactctcttgttgtctgaacctgctagccaaacttggcaggtcgttttcaaagccagatgagttctgattgttcccttggcaatatccattatttccctcctgggtagaaggaggatctgaggacagcttatctttttggggtacgtggagtagaggtggggactcttatataatacgaaataaaaataagttctttgggctggaagtgtcaaaagattccttagaatttatagccacagggatttcatggtgtgtctgatgtactgattttgtgccacatttgagccagaactggcagcagattcaaagcaacacaggtggctaagtacacatgaggggaaggtaggtatggggagagaaaagtggcataaaacaaggctgtccccctatgctcatcgagaataggatcttagccctcactgaaggagcttaatgatcagctctaatacattggctggactcctgcaggtactcacggaaagtagagatgctgagctaccttttcttgtcaaagtctagggctggagatgcttcaagaactttggagccataaagtcactgtaatggtcaacttttaaggctagaagaggccatgagacatctcattcatctccttgcctttgggcaagaattgcacacctaagcctcccgaatacatcagacacaatttagggttaaaagcctccagaggggcaaaaaagtaaaaagattttacaactttcttccacaaaccactttaattgtgtgctcatcaccgacttcagaatctaagagaactttgacacttgtttttgacaccccattgccttctcatcagtctaactccaagaccttcctccgagtggtaggctctggtaattcagcgaaagcaaggcgctaacaggcgagtgtgaagccaaagggctcccagtgacatccttgacatctttttgccagctattcacatgcatttaatatacagcacttccctgtgactgtctgcagccttttctaccagcaattcctcctgatttatccttctccagcaattcccagttgccttgcctttctaatagatgttgcagtctgacaaaacacctttgccttcatgctggtgttgttaaaggactgattataaccgtaaggaatgggaaataagaagctattccttgtaagtttgctaatcttatctgttcagaataataaaagttctctgtcaaagacttaggaagggagatttcatcccccagccttgctagtcctactctttgtgcattcttaagacaggaggcaagtgctttccattctccttggaaaaactgaggctgaatatgcagcttgtcatgcagttttgctgaagacagagagagggtcaaaaattcaaaaactcaattgctctagggcagggggttgggagcaaagccaataaataaaatgggtggtataaatgcctttcaggaaagggtgtgaagggtggggtggatttaccagaagctttggcagtcagctttgaagtcttctggaaaggaaagtgtagcctcccaggcaagcagcctcatgacatcttccataaggctgatgtgttgggaaacagcaacacatgagcaagaagttccttgaaaaattttcttccctccttcttcttctggaactgttgggaaactagattagacccaggagtctggtttttgagaatggccctgaatgaatttttagtttccgggtaggaacagagagctgagaaggttgttttctcctccaaggaaatctggccacagtttttttcctgttctatctagagcttgtgtgctggtggattaagcacatgtgtgcacagggccaggattctggcaaacaatctcagggaggatggcaaaaggagaagcaaaaggggttcattcctctacctcacagcttcttttcccaaaggaaacaggatctactcaccagcaacaatcccaacatcacaaaaggaacagggaaataaacgtgcatacaactgggacacacagacccctgtcacctgctacaaatggagcagaagtgggagagaagtgagccaccgagaacctaggccttcttagctgtagcctacttgaagagggcacgggcttcctgactggtctctggtggccgagtaactctacttccctgacctgggaagaaggcgtgaataaccagctaagaggagacacccatcctcttagagttgcctggggtatctgaggcagaggtggtagcagcagactcctcaacagaggcactgagatccaagaattccaggatgatgtccccaaggcagtaaatcaaatgcctgttgatgaggggttgttgtagtgactccaggactagaccccagctcagccggcatttgttcaccccaagaatttctactacgagatctgggaggactcccatcaggctctgcaaagcctgtttctcagcagccagtttctgctcttgggtccttacgggccgtggaaacttaggcaaaactccaccaggccagatggactcctgaagaagcaggaggtactgcacccagcgctgtggacttgttaaattagctacctgcacctctagccacctttgaactagggtcccaaagataagacgaagaaacttttgcatgttttcggtacatagccatttccactgttctgttagtagcaagaggagcagatccagggctgtgtcagctaactctgtctctgttcctggatcgctgttgctggggtcttgggctggcacggctgcatctgacacgcaactgtccacacgtcctttgggaggttgttcaggatctttttctggggcttttgttggctgcatttccagtaactttgtctgtttttcaataaaagattccatcgcagacatggatagagtctcagactccacattgccttcctggagacaataaagaatcttgtcttgtgcttcagtcacacttagtgctggagaaattttactggatgagaacctcagcctagacttgctagccttcttgccttctgtctggggcttgctttcggtctcggcctcactcagctcctctgtggggctctggggttcagagcgaggaaacgctgtcttcaaggtgtccacaatggcactcaccaccatcttgtctattctagagaccataaatggtttcttgacaaaggcaatacgagcatctgtgttcagagcaaggaactcctgcacctcctcactgttagcgatctccggaatggcacagagttgctttaggaatgattctaggaggctcttacgggcttctactctgtcactgtccatgtttcccaatggaagatctggaaagagctttttaggacccttcacatctctgaaagaatgtgattgctgctgtccagcactaaacttcaaaactcctgaagcaaatccagggagcagagaaccttgaaacggcattctcctccccgatccctcccataaaccaacaggccaatcagcgtggctcgacgtgggaagcaagcgggcagtaggggttggggaaactcctgacttttgatgaactttcgtagatctggtttctcctccagacgggtctgcagattcaagaactcccgatagcgacgattcacagtgtggtaggccagctgctgcaggccgctgctgttttcaccgtcaagggctgtctcgtacttcacagtatagagtgtgtatgggtggaatccagtgccactgtgctctcgggctgtaatggtgccagtgatacgaaggttctggatgataactggaccatcgggactgcttaggggctcaaagctgaaggtggctgagctgagaggaccaggtggagaggaggaaagcagaactggtggcagagtaggatcaagggagctcacatcattggtgagatccttctctaagcatgacggccgtgaggggcaggtcttttctggcccctccagcaaagctgtaacagaggcggtaacatctccttgttctatctccttgtctgctgtgtcaatatggatctctgggcaggaattcagtgtggagaccggcaggcctgtctctgtttctgtccctggaccctcctcagcctctgctccttcagatgcctcaccatctttgggttccagagcctgggaactctctagggcacacagggcatcctgaatcctgtcagagagaaagctgcctggagtcatgagcatgatggtttctttgcccagttcagacagcggagactccagctctgagtcttcacataagaacaggggacctcgaacatttggctgtaggaaatgagatgagttgtttcctacttttctttcttcacacatcccacccaaatctccctctacagcttcgtggccttcttcaacctctggagaggggcctgcagaaccctctggctcactgtaacttaggaatactggggctgctactggagaagctctcccttctggaagctgctctacctcagcaatcagtggcagagatgtcggcactgagggctgttcgggggcactggctgggcagggtgctggatctctggccttggaaaagatacccacgagtacaaggtggatccagtcaggatctgacagcctgctgatcagtggtaagattacattgcatgtgatgagttcgaccactacatggcgtccggtacgagtctccaagtggggcttgggcaccagcccttgaagcaacaaattcacaacgccacgcgtataggtgacttcagcactggggctgtgcacagcaggatgtggggcagtcgcccggcagtaagcctcccagaggtgggaaggctcaactggaccattcttccctgcagtggcctcctttgcctgaatgtagctctgcaggtgacaaccgcagagagtcagaacactctgggcaacagcatgactgtccatcacgctcatccttctccgaagctcctggaccaaccctttcatggctgcctccatttcttcctcaaaggctggctcctggctcacggaacggtaccaagataacacaaaatctcgaataatcatctggatggtgcggttgatctcccgttccagctgcctttctgcctcagggcatggaggacaggtggccaacgggatgaagcgttccagatgcagtcgacctgaagccactccagcgaggctggagcccagccatcctcccagcaccactagcaatgccgacagaaggcacagcagccacacgttgaccagaaggtgtatgaccaggagccagccaagcaagacccccacagccatcagcttccggctactcaacaggttattgaggtgacagctcgatccagctggagtttcctggaacggtggcactgtttctgtcttcatggctgaacggacaaggtggcttccccagatgacagccctcaagattttacttcagagttagggaaggggggcatgaactgtgtctcagatatggggcgatctgggtgctgttcagggaaccggggctccaggccctcaaagtcctacaggcactgcaaagcgacagctgcagctccgcgtctccccatggctaccactaacagagccctccaactcgccccttccagctgaggtgtggctttggaggaaaactctgtggccttcacactgccccaggcggaaggcctcttcggggcctcggggcgggcgctgcaaggccctggggcccacggacacttacacacgcagcgggcagcggccggcgaagactgggtcacacgccgccgggaaccgcgcgcccacactcagccccgacctgaagtggactcatcgcggtcctctccgggagcctcggccctctgccgccgtaaacctgggcgactgcgctccgcagccgggcctgtgtgaaggctgaccgccggccggccgccggcgacagcttccgggtcg

SEQ ID NO: 8294 - RNA, 6296 nt, Homo sapiens
  source 1..6296: mol_type = other RNA
aaaaaccacaattacttttgcaccaacccactacatcagaacctacctttaagggttgatttgtgggttaaataagtgaagatatgtaaagactttaagtaatgctctcagaagatgttaactattagctggtaccaggcattttgggagtagataggggatctgctgaatgttggcagaatgacccatccctagagcagacattgtctatcaatacccattctctgcttcttccttgctaacatcaattatttctgtagatatctgaccttcatggaagatgacctcatctctgggggaaaatactattgaaagccaatcacaatgccattctcagtgtcagtggattggcatgaggtgggtggttctagccaatgagtcataagaggttttttgttttttttttttttatttggggtctcactctgtcacttaaggctagaatgcagtggtgtgatcgtagctcactgcagcctcaaattcctgggctcaagtgatcctcctgcctcagcctccctagtaggtggaaccacaggcgagagccaccatgccccgctcattttttatattttttgtagagacagggtcttgctatgttccaggctggtcttaaactcctggactcaaacaatcccccaaccttggcctcccaaagtgttgagattataggtgtgagccgctgtgcccggcctagaagaggattcttgaaggacttctgggaaatggttccttcattccttagaagaaaacacagaagagatgctcctgttcttttatgaatgttatctctgggtgtgatgcctgaaactgcagcagcaggaaggcaggcagtctgagagcacagctgacctaattagaatggcaaggaagaaagatggaaagaattcaggccccttaagaggtctcagagttgctgaatcaccaaactcctgggcttacctactcacgtactaatgttatgaaataaaataaattttcctcataatttaattcttgtccagagcatcctgattcatatagccagggaccatagttacacatatttttacttcctccaggacctaacaactggtgttgtgtgctatgagcaaaggaagagcagtagctggaaatgaataacctgggtaggacacaggaagactcaaaaatgttctaggctatgcaaatcaaaaccatgagatagtaatatcacctaataccttttaagatgccattatgaaaaaacaaaacattacaagtgttggagaggatgtggagaaactggaacccttgtacattgttggtgggaatgtaaaatggtctagtcactatggaaaacagtatgaaggtcttcaaagaattaaaaacagaacaatatatgatccagcaatcctacttctgggtatttatctaaaataattaaaagcagggcctcgaagaaacagtcacactcccatgttcactgcagcattgttttcaacaatcaaggcgcggagccaacctaaatgtccctcaatgaatgaacaaagaaaatgtggcatagccatacaatggaatgttttcagccttaaaaagaaaattctgtcacatgctgtaacgtggatgaacctggaggacattatgctaagtgaaataagccagtcaaaggacaaacactgcatgattccacttatatgaggcgttcaaagtagtcaaactcacagaagcagaaagtagaacagtgattgccagaggctggtgggaggggaaacgaggagtggctgttcaatgggtataaacttttggttatgcaagatgaaaaacttgtagcagtctgctacaaagcactgtgctgcttctagttaataatgtaccgtctcaaaataaataaataatgtactgtacacttaagagggtagatctcacattatgtgtttctttacaacaataagaaaatcaccttgtaaactggaaatttccaaaatggaaattggagtagcttgtattgattttaaaatttatacatgctctcactcataggtgggaattgaacaatgagaacacttggacacaggaaggtgaacatcacacactggggcctgttgtgaggtcgggggagggggaagggatagcatcaggagatatacctaatgtaaatgacgagttaacgggtgcagcacaccaacacggcacatgtatacatatgcaacaaacctgcatgttgtgcacatgttccctagaacttaatgtataataataataaaaataaaatttatacatgctcctaggctcagatttaggaatttattttccatttaggttttattaagtctaatccaacaatgcaaaaatgaaactgtgagttatatgtgatgaaaaagtatagctttcttgaattcaaataagcaatggcaaagatcacatttagaatttgacagaaagaacacagcatccctgcctcgtcttttttatagatagtaagaaaagggaaagtagtcttatttcaaatatcaaaattctgacttaaatgaataaaatttagtcacgagtaaatacaaaaaacaagcaaacaataaaaccttcctggatcagcacaggcccaattcttccctgccttttatcaccctgtcagctgggagtatcttttctacctgtggctctctaccaattgttactctcttgttgtctgaacctgctagccaaacttggcaggtcgttttcaaagccagatgagttctgattgttcccttggcaatatccattatttccctcctgggtagaaggaggatctgaggacagcttatctttttggggtacgtggagtagaggtggggactcttatataatacgaaataaaaataagttctttgggctggaagtgtcaaaagattccttagaatttatagccacagggatttcatggtgtgtctgatgtactgattttgtgccacatttgagccagaactggcagcagattcaaagcaacacaggtggctaagtacacatgaggggaaggtaggtatggggagagaaaagtggcataaaacaaggctgtccccctatgctcatcgagaataggatcttagccctcactgaaggagcttaatgatcagctctaatacattggctggactcctgcaggtactcacggaaagtagagatgctgagctaccttttcttgtcaaagtctagggctggagatgcttcaagaactttggagccataaagtcactgtaatggtcaacttttaaggctagaagaggccatgagacatctcattcatctccttgcctttgggcaagaattgcacacctaagcctcccgaatacatcagacacaatttagggttaaaagcctccagaggggcaaaaaagtaaaaagattttacaactttcttccacaaaccactttaattgtgtgctcatcaccgacttcagaatctaagagaactttgacacttgtttttgacaccccattgccttctcatcagtctaactccaagaccttcctccgagtggtaggctctggtaattcagcgaaagcaaggcgctaacaggcgagtgtgaagccaaagggctcccagtgacatccttgacatctttttgccagctattcacatgcatttaatatacagcacttccctgtgactgtctgcagccttttctaccagcaattcctcctgatttatccttctccagcaattcccagttgccttgcctttctaatagatgttgcagtctgacaaaacacctttgccttcatgctggtgttgttaaaggactgattataaccgtaaggaatgggaaataagaagctattccttgtaagtttgctaatcttatctgttcagaataataaaagttctctgtcaaagacttaggaagggagatttcatcccccagccttgctagtcctactctttgtgcattcttaagacaggaggcaagtgctttccattctccttggaaaaactgaggctgaatatgcagcttgtcatgcagttttgctgaagacagagagagggtcaaaaattcaaaaactcaattgctctagggcagggggttgggagcaaagccaataaataaaatgggtggtataaatgcctttcaggaaagggtgtgaagggtggggtggatttaccagaagctttggcagtcagctttgaagtcttctggaaaggaaagtgtagcctcccaggcaagcagcctcatgacatcttccataaggctgatgtgttgggaaacagcaacacatgagcaagaagttccttgaaaaattttcttccctccttcttcttctggaactgttgggaaactagattagacccaggagtctggtttttgagaatggccctgaatgaatttttagtttccgggtaggaacagagagctgagaaggttgttttctcctccaaggaaatctggccacagtttttttcctgttctatctagagcttgtgtgctggtggattaagcacatgtgtgcacagggccaggattctggcaaacaatctcagggaggatggcaaaaggagaagcaaaaggggttcattcctctacctcacagcttcttttcccaaaggaaacaggatctactcaccagcaacaatcccaacatcacaaaaggaacagggaaataaacgtgcatacaactgggacacacagacccctgtcacctgctacaaatggagcagaagtgggagagaagtgagccaccgagaacctaggccttcttagctgtagcctacttgaagagggcacgggcttcctgactggtctctggtggccgagtaactctacttccctgacctgggaagaaggcgtgaataaccagctaagaggagacacccatcctcttagagttgcctggggtatctgaggcagaggtggtagcagcagactcctcaacagaggcactgagatccaagaattccaggatgatgtccccaaggcagtaaatcaaatgcctgttgatgaggggttgttgtagtgactccaggactagaccccagctcagccggcatttgttcaccccaagaatttctactacgagatctgggaggactcccatcaggctctgcaaagcctgtttctcagcagccagtttctgctcttgggtccttacgggccgtggaaacttaggcaaaactccaccaggccagatggactcctgaagaagcaggaggtactgcacccagcgctgtggacttgttaaattagctacctgcacctctagccacctttgaactagggtcccaaagataagacgaagaaacttttgcatgttttcggtacatagccatttccactgttctgttagtagcaagaggagcagatccagggctgtgtcagctaactctgtctctgttcctggatcgctgttgctggggtcttgggctggcacggctgcatctgacacgcaactgtccacacgtcctttgggaggttgttcaggatctttttctggggcttttgttggctgcatttccagtaactttgtctgtttttcaataaaagattccatcgcagacatggatagagtctcagactccacattgccttcctggagacaataaagaatcttgtcttgtgcttcagtcacacttagtgctggagaaattttactggatgagaacctcagcctagacttgctagccttcttgccttctgtctggggcttgctttcggtctcggcctcactcagctcctctgtggggctctggggttcagagcgaggaaacgctgtcttcaaggtgtccacaatggcactcaccaccatcttgtctattctagagaccataaatggtttcttgacaaaggcaatacgagcatctgtgttcagagcaaggaactcctgcacctcctcactgttagcgatctccggaatggcacagagttgctttaggaatgattctaggaggctcttacgggcttctactctgtcactgtccatgtttcccaatggaagatctggaaagagctttttaggacccttcacatttttgatgaactttcgtagatctggtttctcctccagacgggtctgcagattcaagaactcccgatagcgacgattcacagtgtggtaggccagctgctgcaggccgctgctgttttcaccgtcaagggctgtctcgtaacacgcagcgggcagcggccggcgaagactgggtcacacgccgccgggaaccgcgcgcccacactcagccccgacctgaagtggactcatcgcggtcctctccgggagcctcggccctctgccgccgtaaacctgggcgactgcgctccgcagccgggcctgtgtgaaggctgaccgccggccggccgccggcgacagct

SEQ ID NO: 8295 - RNA, 6352 nt, Homo sapiens
  source 1..6352: mol_type = other RNA
aaaaaccacaattacttttgcaccaacccactacatcagaacctacctttaagggttgatttgtgggttaaataagtgaagatatgtaaagactttaagtaatgctctcagaagatgttaactattagctggtaccaggcattttgggagtagataggggatctgctgaatgttggcagaatgacccatccctagagcagacattgtctatcaatacccattctctgcttcttccttgctaacatcaattatttctgtagatatctgaccttcatggaagatgacctcatctctgggggaaaatactattgaaagccaatcacaatgccattctcagtgtcagtggattggcatgaggtgggtggttctagccaatgagtcataagaggttttttgttttttttttttttatttggggtctcactctgtcacttaaggctagaatgcagtggtgtgatcgtagctcactgcagcctcaaattcctgggctcaagtgatcctcctgcctcagcctccctagtaggtggaaccacaggcgagagccaccatgccccgctcattttttatattttttgtagagacagggtcttgctatgttccaggctggtcttaaactcctggactcaaacaatcccccaaccttggcctcccaaagtgttgagattataggtgtgagccgctgtgcccggcctagaagaggattcttgaaggacttctgggaaatggttccttcattccttagaagaaaacacagaagagatgctcctgttcttttatgaatgttatctctgggtgtgatgcctgaaactgcagcagcaggaaggcaggcagtctgagagcacagctgacctaattagaatggcaaggaagaaagatggaaagaattcaggccccttaagaggtctcagagttgctgaatcaccaaactcctgggcttacctactcacgtactaatgttatgaaataaaataaattttcctcataatttaattcttgtccagagcatcctgattcatatagccagggaccatagttacacatatttttacttcctccaggacctaacaactggtgttgtgtgctatgagcaaaggaagagcagtagctggaaatgaataacctgggtaggacacaggaagactcaaaaatgttctaggctatgcaaatcaaaaccatgagatagtaatatcacctaataccttttaagatgccattatgaaaaaacaaaacattacaagtgttggagaggatgtggagaaactggaacccttgtacattgttggtgggaatgtaaaatggtctagtcactatggaaaacagtatgaaggtcttcaaagaattaaaaacagaacaatatatgatccagcaatcctacttctgggtatttatctaaaataattaaaagcagggcctcgaagaaacagtcacactcccatgttcactgcagcattgttttcaacaatcaaggcgcggagccaacctaaatgtccctcaatgaatgaacaaagaaaatgtggcatagccatacaatggaatgttttcagccttaaaaagaaaattctgtcacatgctgtaacgtggatgaacctggaggacattatgctaagtgaaataagccagtcaaaggacaaacactgcatgattccacttatatgaggcgttcaaagtagtcaaactcacagaagcagaaagtagaacagtgattgccagaggctggtgggaggggaaacgaggagtggctgttcaatgggtataaacttttggttatgcaagatgaaaaacttgtagcagtctgctacaaagcactgtgctgcttctagttaataatgtaccgtctcaaaataaataaataatgtactgtacacttaagagggtagatctcacattatgtgtttctttacaacaataagaaaatcaccttgtaaactggaaatttccaaaatggaaattggagtagcttgtattgattttaaaatttatacatgctctcactcataggtgggaattgaacaatgagaacacttggacacaggaaggtgaacatcacacactggggcctgttgtgaggtcgggggagggggaagggatagcatcaggagatatacctaatgtaaatgacgagttaacgggtgcagcacaccaacacggcacatgtatacatatgcaacaaacctgcatgttgtgcacatgttccctagaacttaatgtataataataataaaaataaaatttatacatgctcctaggctcagatttaggaatttattttccatttaggttttattaagtctaatccaacaatgcaaaaatgaaactgtgagttatatgtgatgaaaaagtatagctttcttgaattcaaataagcaatggcaaagatcacatttagaatttgacagaaagaacacagcatccctgcctcgtcttttttatagatagtaagaaaagggaaagtagtcttatttcaaatatcaaaattctgacttaaatgaataaaatttagtcacgagtaaatacaaaaaacaagcaaacaataaaaccttcctggatcagcacaggcccaattcttccctgccttttatcaccctgtcagctgggagtatcttttctacctgtggctctctaccaattgttactctcttgttgtctgaacctgctagccaaacttggcaggtcgttttcaaagccagatgagttctgattgttcccttggcaatatccattatttccctcctgggtagaaggaggatctgaggacagcttatctttttggggtacgtggagtagaggtggggactcttatataatacgaaataaaaataagttctttgggctggaagtgtcaaaagattccttagaatttatagccacagggatttcatggtgtgtctgatgtactgattttgtgccacatttgagccagaactggcagcagattcaaagcaacacaggtggctaagtacacatgaggggaaggtaggtatggggagagaaaagtggcataaaacaaggctgtccccctatgctcatcgagaataggatcttagccctcactgaaggagcttaatgatcagctctaatacattggctggactcctgcaggtactcacggaaagtagagatgctgagctaccttttcttgtcaaagtctagggctggagatgcttcaagaactttggagccataaagtcactgtaatggtcaacttttaaggctagaagaggccatgagacatctcattcatctccttgcctttgggcaagaattgcacacctaagcctcccgaatacatcagacacaatttagggttaaaagcctccagaggggcaaaaaagtaaaaagattttacaactttcttccacaaaccactttaattgtgtgctcatcaccgacttcagaatctaagagaactttgacacttgtttttgacaccccattgccttctcatcagtctaactccaagaccttcctccgagtggtaggctctggtaattcagcgaaagcaaggcgctaacaggcgagtgtgaagccaaagggctcccagtgacatccttgacatctttttgccagctattcacatgcatttaatatacagcacttccctgtgactgtctgcagccttttctaccagcaattcctcctgatttatccttctccagcaattcccagttgccttgcctttctaatagatgttgcagtctgacaaaacacctttgccttcatgctggtgttgttaaaggactgattataaccgtaaggaatgggaaataagaagctattccttgtaagtttgctaatcttatctgttcagaataataaaagttctctgtcaaagacttaggaagggagatttcatcccccagccttgctagtcctactctttgtgcattcttaagacaggaggcaagtgctttccattctccttggaaaaactgaggctgaatatgcagcttgtcatgcagttttgctgaagacagagagagggtcaaaaattcaaaaactcaattgctctagggcagggggttgggagcaaagccaataaataaaatgggtggtataaatgcctttcaggaaagggtgtgaagggtggggtggatttaccagaagctttggcagtcagctttgaagtcttctggaaaggaaagtgtagcctcccaggcaagcagcctcatgacatcttccataaggctgatgtgttgggaaacagcaacacatgagcaagaagttccttgaaaaattttcttccctccttcttcttctggaactgttgggaaactagattagacccaggagtctggtttttgagaatggccctgaatgaatttttagtttccgggtaggaacagagagctgagaaggttgttttctcctccaaggaaatctggccacagtttttttcctgttctatctagagcttgtgtgctggtggattaagcacatgtgtgcacagggccaggattctggcaaacaatctcagggaggatggcaaaaggagaagcaaaaggggttcattcctctacctcacagcttcttttcccaaaggaaacaggatctactcaccagcaacaatcccaacatcacaaaaggaacagggaaataaacgtgcatacaactgggacacacagacccctgtcacctgctacaaatggagcagaagtgggagagaagtgagccaccgagaacctaggccttcttagctgtagcctacttgaagagggcacgggcttcctgactggtctctggtggccgagtaactctacttccctgacctgggaagaaggcgtgaataaccagctaagaggagacacccatcctcttagagttgcctggggtatctgaggcagaggtggtagcagcagactcctcaacagaggcactgagatccaagaattccaggatgatgtccccaaggcagtaaatcaaatgcctgttgatgaggggttgttgtagtgactccaggactagaccccagctcagccggcatttgttcaccccaagaatttctactacgagatctgggaggactcccatcaggctctgcaaagcctgtttctcagcagccagtttctgctcttgggtccttacgggccgtggaaacttaggcaaaactccaccaggccagatggactcctgaagaagcaggaggtactgcacccagcgctgtggacttgttaaattagctacctgcacctctagccacctttgaactagggtcccaaagataagacgaagaaacttttgcatgttttcggtacatagccatttccactgttctgttagtagcaagaggagcagatccagggctgtgtcagctaactctgtctctgttcctggatcgctgttgctggggtcttgggctggcacggctgcatctgacacgcaactgtccacacgtcctttgggaggttgttcaggatctttttctggggcttttgttggctgcatttccagtaactttgtctgtttttcaataaaagattccatcgcagacatggatagagtctcagactccacattgccttcctggagacaataaagaatcttgtcttgtgcttcagtcacacttagtgctggagaaattttactggatgagaacctcagcctagacttgctagccttcttgccttctgtctggggcttgctttcggtctcggcctcactcagctcctctgtggggctctggggttcagagcgaggaaacgctgtcttcaaggtgtccacaatggcactcaccaccatcttgtctattctagagaccataaatggtttcttgacaaaggcaatacgagcatctgtgttcagagcaaggaactcctgcacctcctcactgttagcgatctccggaatggcacagagttgctttaggaatgattctaggaggctcttacgggcttctactctgtcactgtccatgtttcccaatggaagatctggaaagagctttttaggacccttcacatttttgatgaactttcgtagatctggtttctcctccagacgggtctgcagattcaagaactcccgatagcgacgattcacagtgtggtaggccagctgctgcaggccgctgctgttttcaccgtcaagggctgtctcgtacatctttgggttccagagcctgggaactctctagggcacacagggcatcctgaatcacacgcagcgggcagcggccggcgaagactgggtcacacgccgccgggaaccgcgcgcccacactcagccccgacctgaagtggactcatcgcggtcctctccgggagcctcggccctctgccgccgtaaacctgggcgactgcgctccgcagccgggcctgtgtgaaggctgaccgccggccggccgccggcgacagct

SEQ ID NO: 8296 - RNA, 8310 nt, Homo sapiens
  source 1..8310: mol_type = other RNA
aaaaaccacaattacttttgcaccaacccactacatcagaacctacctttaagggttgatttgtgggttaaataagtgaagatatgtaaagactttaagtaatgctctcagaagatgttaactattagctggtaccaggcattttgggagtagataggggatctgctgaatgttggcagaatgacccatccctagagcagacattgtctatcaatacccattctctgcttcttccttgctaacatcaattatttctgtagatatctgaccttcatggaagatgacctcatctctgggggaaaatactattgaaagccaatcacaatgccattctcagtgtcagtggattggcatgaggtgggtggttctagccaatgagtcataagaggttttttgttttttttttttttatttggggtctcactctgtcacttaaggctagaatgcagtggtgtgatcgtagctcactgcagcctcaaattcctgggctcaagtgatcctcctgcctcagcctccctagtaggtggaaccacaggcgagagccaccatgccccgctcattttttatattttttgtagagacagggtcttgctatgttccaggctggtcttaaactcctggactcaaacaatcccccaaccttggcctcccaaagtgttgagattataggtgtgagccgctgtgcccggcctagaagaggattcttgaaggacttctgggaaatggttccttcattccttagaagaaaacacagaagagatgctcctgttcttttatgaatgttatctctgggtgtgatgcctgaaactgcagcagcaggaaggcaggcagtctgagagcacagctgacctaattagaatggcaaggaagaaagatggaaagaattcaggccccttaagaggtctcagagttgctgaatcaccaaactcctgggcttacctactcacgtactaatgttatgaaataaaataaattttcctcataatttaattcttgtccagagcatcctgattcatatagccagggaccatagttacacatatttttacttcctccaggacctaacaactggtgttgtgtgctatgagcaaaggaagagcagtagctggaaatgaataacctgggtaggacacaggaagactcaaaaatgttctaggctatgcaaatcaaaaccatgagatagtaatatcacctaataccttttaagatgccattatgaaaaaacaaaacattacaagtgttggagaggatgtggagaaactggaacccttgtacattgttggtgggaatgtaaaatggtctagtcactatggaaaacagtatgaaggtcttcaaagaattaaaaacagaacaatatatgatccagcaatcctacttctgggtatttatctaaaataattaaaagcagggcctcgaagaaacagtcacactcccatgttcactgcagcattgttttcaacaatcaaggcgcggagccaacctaaatgtccctcaatgaatgaacaaagaaaatgtggcatagccatacaatggaatgttttcagccttaaaaagaaaattctgtcacatgctgtaacgtggatgaacctggaggacattatgctaagtgaaataagccagtcaaaggacaaacactgcatgattccacttatatgaggcgttcaaagtagtcaaactcacagaagcagaaagtagaacagtgattgccagaggctggtgggaggggaaacgaggagtggctgttcaatgggtataaacttttggttatgcaagatgaaaaacttgtagcagtctgctacaaagcactgtgctgcttctagttaataatgtaccgtctcaaaataaataaataatgtactgtacacttaagagggtagatctcacattatgtgtttctttacaacaataagaaaatcaccttgtaaactggaaatttccaaaatggaaattggagtagcttgtattgattttaaaatttatacatgctctcactcataggtgggaattgaacaatgagaacacttggacacaggaaggtgaacatcacacactggggcctgttgtgaggtcgggggagggggaagggatagcatcaggagatatacctaatgtaaatgacgagttaacgggtgcagcacaccaacacggcacatgtatacatatgcaacaaacctgcatgttgtgcacatgttccctagaacttaatgtataataataataaaaataaaatttatacatgctcctaggctcagatttaggaatttattttccatttaggttttattaagtctaatccaacaatgcaaaaatgaaactgtgagttatatgtgatgaaaaagtatagctttcttgaattcaaataagcaatggcaaagatcacatttagaatttgacagaaagaacacagcatccctgcctcgtcttttttatagatagtaagaaaagggaaagtagtcttatttcaaatatcaaaattctgacttaaatgaataaaatttagtcacgagtaaatacaaaaaacaagcaaacaataaaaccttcctggatcagcacaggcccaattcttccctgccttttatcaccctgtcagctgggagtatcttttctacctgtggctctctaccaattgttactctcttgttgtctgaacctgctagccaaacttggcaggtcgttttcaaagccagatgagttctgattgttcccttggcaatatccattatttccctcctgggtagaaggaggatctgaggacagcttatctttttggggtacgtggagtagaggtggggactcttatataatacgaaataaaaataagttctttgggctggaagtgtcaaaagattccttagaatttatagccacagggatttcatggtgtgtctgatgtactgattttgtgccacatttgagccagaactggcagcagattcaaagcaacacaggtggctaagtacacatgaggggaaggtaggtatggggagagaaaagtggcataaaacaaggctgtccccctatgctcatcgagaataggatcttagccctcactgaaggagcttaatgatcagctctaatacattggctggactcctgcaggtactcacggaaagtagagatgctgagctaccttttcttgtcaaagtctagggctggagatgcttcaagaactttggagccataaagtcactgtaatggtcaacttttaaggctagaagaggccatgagacatctcattcatctccttgcctttgggcaagaattgcacacctaagcctcccgaatacatcagacacaatttagggttaaaagcctccagaggggcaaaaaagtaaaaagattttacaactttcttccacaaaccactttaattgtgtgctcatcaccgacttcagaatctaagagaactttgacacttgtttttgacaccccattgccttctcatcagtctaactccaagaccttcctccgagtggtaggctctggtaattcagcgaaagcaaggcgctaacaggcgagtgtgaagccaaagggctcccagtgacatccttgacatctttttgccagctattcacatgcatttaatatacagcacttccctgtgactgtctgcagccttttctaccagcaattcctcctgatttatccttctccagcaattcccagttgccttgcctttctaatagatgttgcagtctgacaaaacacctttgccttcatgctggtgttgttaaaggactgattataaccgtaaggaatgggaaataagaagctattccttgtaagtttgctaatcttatctgttcagaataataaaagttctctgtcaaagacttaggaagggagatttcatcccccagccttgctagtcctactctttgtgcattcttaagacaggaggcaagtgctttccattctccttggaaaaactgaggctgaatatgcagcttgtcatgcagttttgctgaagacagagagagggtcaaaaattcaaaaactcaattgctctagggcagggggttgggagcaaagccaataaataaaatgggtggtataaatgcctttcaggaaagggtgtgaagggtggggtggatttaccagaagctttggcagtcagctttgaagtcttctggaaaggaaagtgtagcctcccaggcaagcagcctcatgacatcttccataaggctgatgtgttgggaaacagcaacacatgagcaagaagttccttgaaaaattttcttccctccttcttcttctggaactgttgggaaactagattagacccaggagtctggtttttgagaatggccctgaatgaatttttagtttccgggtaggaacagagagctgagaaggttgttttctcctccaaggaaatctggccacagtttttttcctgttctatctagagcttgtgtgctggtggattaagcacatgtgtgcacagggccaggattctggcaaacaatctcagggaggatggcaaaaggagaagcaaaaggggttcattcctctacctcacagcttcttttcccaaaggaaacaggatctactcaccagcaacaatcccaacatcacaaaaggaacagggaaataaacgtgcatacaactgggacacacagacccctgtcacctgctacaaatggagcagaagtgggagagaagtgagccaccgagaacctaggccttcttagctgtagcctacttgaagagggcacgggcttcctgactggtctctggtggccgagtaactctacttccctgacctgggaagaaggcgtgaataaccagctaagaggagacacccatcctcttagagttgcctggggtatctgaggcagaggtggtagcagcagactcctcaacagaggcactgagatccaagaattccaggatgatgtccccaaggcagtaaatcaaatgcctgttgatgaggggttgttgtagtgactccaggactagaccccagctcagccggcatttgttcaccccaagaatttctactacgagatctgggaggactcccatcaggctctgcaaagcctgtttctcagcagccagtttctgctcttgggtccttacgggccgtggaaacttaggcaaaactccaccaggccagatggactcctgaagaagcaggaggtactgcacccagcgctgtggacttgttaaattagctacctgcacctctagccacctttgaactagggtcccaaagataagacgaagaaacttttgcatgttttcggtacatagccatttccactgttctgttagtagcaagaggagcagatccagggctgtgtcagctaactctgtctctgttcctggatcgctgttgctggggtcttgggctggcacggctgcatctgacacgcaactgtccacacgtcctttgggaggttgttcaggatctttttctggggcttttgttggctgcatttccagtaactttgtctgtttttcaataaaagattccatcgcagacatggatagagtctcagactccacattgccttcctggagacaataaagaatcttgtcttgtgcttcagtcacacttagtgctggagaaattttactggatgagaacctcagcctagacttgctagccttcttgccttctgtctggggcttgctttcggtctcggcctcactcagctcctctgtggggctctggggttcagagcgaggaaacgctgtcttcaaggtgtccacaatggcactcaccaccatcttgtctattctagagaccataaatggtttcttgacaaaggcaatacgagcatctgtgttcagagcaaggaactcctgcacctcctcactgttagcgatctccggaatggcacagagttgctttaggaatgattctaggaggctcttacgggcttctactctgtcactgtccatgtttcccaatggaagatctggaaagagctttttaggacccttcacatttttgatgaactttcgtagatctggtttctcctccagacgggtctgcagattcaagaactcccgatagcgacgattcacagtgtggtaggccagctgctgcaggccgctgctgttttcaccgtcaagggctgtctcgtacttcacagtatagagtgtgtatgggtggaatccagtgccactgtgctctcgggctgtaatggtgccagtgatacgaaggttctggatgataactggaccatcgggactgcttaggggctcaaagctgaaggtggctgagctgagaggaccaggtggagaggaggaaagcagaactggtggcagagtaggatcaagggagctcacatcattggtgagatccttctctaagcatgacggccgtgaggggcaggtcttttctggcccctccagcaaagctgtaacagaggcggtaacatctccttgttctatctccttgtctgctgtgtcaatatggatctctgggcaggaattcagtgtggagaccggcaggcctgtctctgtttctgtccctggaccctcctcagcctctgctccttcagatgcctcaccatctttgggttccagagcctgggaactctctagggcacacagggcatcctgaatcctgtcagagagaaagctgcctggagtcatgagcatgatggtttctttgcccagttcagacagcggagactccagctctgagtcttcacataagaacaggggacctcgaacatttggctgtaggaaatgagatgagttgtttcctacttttctttcttcacacatcccacccaaatctccctctacagcttcgtggccttcttcaacctctggagaggggcctgcagaaccctctggctcactgtaacttaggaatactggggctgctactggagaagctctcccttctggaagctgctctacctcagcaatcagtggcagagatgtcggcactgagggctgttcgggggcactggctgggcagggtgctggatctctggccttggaaaagatacccacgagtacaaggtggatccagtcaggatctgacagcctgctgatcagtggtaagattacattgcatgtgatgagttcgaccactacatggcgtccggtacgagtctccaagtggggcttgggcaccagcccttgaagcaacaaattcacaacgccacgcgtataggtgacttcagcactggggctgtgcacagcaggatgtggggcagtcgcccggcagtaagcctcccagaggtgggaaggctcaactggaccattcttccctgcagtggcctcctttgcctgaatgtagctctgcaggtgacaaccgcagagagtcagaacactctgggcaacagcatgactgtccatcacgctcatccttctccgaagctcctggaccaaccctttcatggctgcctccatttcttcctcaaaggctggctcctggctcacggaacggtaccaagataacacaaaatctcgaataatcatctggatggtgcggttgatctcccgttccagctgcctttctgcctcagggcatggaggacaggtggccaacgggatgaagcgttccagatgcagtcgacctgaagccactccagcgaggctggagcccagccatcctcccagcaccactagcaatgccgacagaaggcacagcagccacacgttgaccagaaggtgtatgaccaggagccagccaagcaagacccccacagccatcagcttccggctactcaacaggttattgaggtgacagctcgatccagctggagtttcctggaacggtggcactgtttctgtcttcatggctgaacggacaaggtggcttccccagatgacagccctcaagattttacttcagagttagggaaggggggcatgaactgtgtctcagatatggggcgatctgggtgctgttcagggaaccggggctccaggccctcaaagtcctacaggcactgcaaagcgacagctgcagctccgcgtctccccatggctaccactaacagagccctccaactcgccccttccagctgaggtgtggctttggaggaaaactctgtggccttcacactgccccaggcggaaggcctcttcggggcctcggggcgggcgctgcaaggccctggggcccacggacacttacacacgcagcgggcagcggccggcgaagactgggtcacacgccgccgggaaccgcgcgcccacactcagccccgacctgaagtggactcatcgcggtcctctccgggagcctcggccctctgccgccgtaaacctgggcgactgcgctccgcagccgggcctgtgtgaaggctgaccgccggccggccgccggcgacagct

SEQ ID NO: 8297 - RNA, 6037 nt, Homo sapiens
  source 1..6037: mol_type = other RNA
aaaaaccacaattacttttgcaccaacccactacatcagaacctacctttaagggttgatttgtgggttaaataagtgaagatatgtaaagactttaagtaatgctctcagaagatgttaactattagctggtaccaggcattttgggagtagataggggatctgctgaatgttggcagaatgacccatccctagagcagacattgtctatcaatacccattctctgcttcttccttgctaacatcaattatttctgtagatatctgaccttcatggaagatgacctcatctctgggggaaaatactattgaaagccaatcacaatgccattctcagtgtcagtggattggcatgaggtgggtggttctagccaatgagtcataagaggttttttgttttttttttttttatttggggtctcactctgtcacttaaggctagaatgcagtggtgtgatcgtagctcactgcagcctcaaattcctgggctcaagtgatcctcctgcctcagcctccctagtaggtggaaccacaggcgagagccaccatgccccgctcattttttatattttttgtagagacagggtcttgctatgttccaggctggtcttaaactcctggactcaaacaatcccccaaccttggcctcccaaagtgttgagattataggtgtgagccgctgtgcccggcctagaagaggattcttgaaggacttctgggaaatggttccttcattccttagaagaaaacacagaagagatgctcctgttcttttatgaatgttatctctgggtgtgatgcctgaaactgcagcagcaggaaggcaggcagtctgagagcacagctgacctaattagaatggcaaggaagaaagatggaaagaattcaggccccttaagaggtctcagagttgctgaatcaccaaactcctgggcttacctactcacgtactaatgttatgaaataaaataaattttcctcataatttaattcttgtccagagcatcctgattcatatagccagggaccatagttacacatatttttacttcctccaggacctaacaactggtgttgtgtgctatgagcaaaggaagagcagtagctggaaatgaataacctgggtaggacacaggaagactcaaaaatgttctaggctatgcaaatcaaaaccatgagatagtaatatcacctaataccttttaagatgccattatgaaaaaacaaaacattacaagtgttggagaggatgtggagaaactggaacccttgtacattgttggtgggaatgtaaaatggtctagtcactatggaaaacagtatgaaggtcttcaaagaattaaaaacagaacaatatatgatccagcaatcctacttctgggtatttatctaaaataattaaaagcagggcctcgaagaaacagtcacactcccatgttcactgcagcattgttttcaacaatcaaggcgcggagccaacctaaatgtccctcaatgaatgaacaaagaaaatgtggcatagccatacaatggaatgttttcagccttaaaaagaaaattctgtcacatgctgtaacgtggatgaacctggaggacattatgctaagtgaaataagccagtcaaaggacaaacactgcatgattccacttatatgaggcgttcaaagtagtcaaactcacagaagcagaaagtagaacagtgattgccagaggctggtgggaggggaaacgaggagtggctgttcaatgggtataaacttttggttatgcaagatgaaaaacttgtagcagtctgctacaaagcactgtgctgcttctagttaataatgtaccgtctcaaaataaataaataatgtactgtacacttaagagggtagatctcacattatgtgtttctttacaacaataagaaaatcaccttgtaaactggaaatttccaaaatggaaattggagtagcttgtattgattttaaaatttatacatgctctcactcataggtgggaattgaacaatgagaacacttggacacaggaaggtgaacatcacacactggggcctgttgtgaggtcgggggagggggaagggatagcatcaggagatatacctaatgtaaatgacgagttaacgggtgcagcacaccaacacggcacatgtatacatatgcaacaaacctgcatgttgtgcacatgttccctagaacttaatgtataataataataaaaataaaatttatacatgctcctaggctcagatttaggaatttattttccatttaggttttattaagtctaatccaacaatgcaaaaatgaaactgtgagttatatgtgatgaaaaagtatagctttcttgaattcaaataagcaatggcaaagatcacatttagaatttgacagaaagaacacagcatccctgcctcgtcttttttatagatagtaagaaaagggaaagtagtcttatttcaaatatcaaaattctgacttaaatgaataaaatttagtcacgagtaaatacaaaaaacaagcaaacaataaaaccttcctggatcagcacaggcccaattcttccctgccttttatcaccctgtcagctgggagtatcttttctacctgtggctctctaccaattgttactctcttgttgtctgaacctgctagccaaacttggcaggtcgttttcaaagccagatgagttctgattgttcccttggcaatatccattatttccctcctgggtagaaggaggatctgaggacagcttatctttttggggtacgtggagtagaggtggggactcttatataatacgaaataaaaataagttctttgggctggaagtgtcaaaagattccttagaatttatagccacagggatttcatggtgtgtctgatgtactgattttgtgccacatttgagccagaactggcagcagattcaaagcaacacaggtggctaagtacacatgaggggaaggtaggtatggggagagaaaagtggcataaaacaaggctgtccccctatgctcatcgagaataggatcttagccctcactgaaggagcttaatgatcagctctaatacattggctggactcctgcaggtactcacggaaagtagagatgctgagctaccttttcttgtcaaagtctagggctggagatgcttcaagaactttggagccataaagtcactgtaatggtcaacttttaaggctagaagaggccatgagacatctcattcatctccttgcctttgggcaagaattgcacacctaagcctcccgaatacatcagacacaatttagggttaaaagcctccagaggggcaaaaaagtaaaaagattttacaactttcttccacaaaccactttaattgtgtgctcatcaccgacttcagaatctaagagaactttgacacttgtttttgacaccccattgccttctcatcagtctaactccaagaccttcctccgagtggtaggctctggtaattcagcgaaagcaaggcgctaacaggcgagtgtgaagccaaagggctcccagtgacatccttgacatctttttgccagctattcacatgcatttaatatacagcacttccctgtgactgtctgcagccttttctaccagcaattcctcctgatttatccttctccagcaattcccagttgccttgcctttctaatagatgttgcagtctgacaaaacacctttgccttcatgctggtgttgttaaaggactgattataaccgtaaggaatgggaaataagaagctattccttgtaagtttgctaatcttatctgttcagaataataaaagttctctgtcaaagacttaggaagggagatttcatcccccagccttgctagtcctactctttgtgcattcttaagacaggaggcaagtgctttccattctccttggaaaaactgaggctgaatatgcagcttgtcatgcagttttgctgaagacagagagagggtcaaaaattcaaaaactcaattgctctagggcagggggttgggagcaaagccaataaataaaatgggtggtataaatgcctttcaggaaagggtgtgaagggtggggtggatttaccagaagctttggcagtcagctttgaagtcttctggaaaggaaagtgtagcctcccaggcaagcagcctcatgacatcttccataaggctgatgtgttgggaaacagcaacacatgagcaagaagttccttgaaaaattttcttccctccttcttcttctggaactgttgggaaactagattagacccaggagtctggtttttgagaatggccctgaatgaatttttagtttccgggtaggaacagagagctgagaaggttgttttctcctccaaggaaatctggccacagtttttttcctgttctatctagagcttgtgtgctggtggattaagcacatgtgtgcacagggccaggattctggcaaacaatctcagggaggatggcaaaaggagaagcaaaaggggttcattcctctacctcacagcttcttttcccaaaggaaacaggatctactcaccagcaacaatcccaacatcacaaaaggaacagggaaataaacgtgcatacaactgggacacacagacccctgtcacctgctacaaatggagcagaagtgggagagaagtgagccaccgagaacctaggccttcttagctgtagcctacttgaagagggcacgggcttcctgactggtctctggtggccgagtaactctacttccctgacctgggaagaaggcgtgaataaccagctaagaggagacacccatcctcttagagttgcctggggtatctgaggcagaggtggtagcagcagactcctcaacagaggcactgagatccaagaattccaggatgatgtccccaaggcagtaaatcaaatgcctgttgatgaggggttgttgtagtgactccaggactagaccccagctcagccggcatttgttcaccccaagaatttctactacgagatctgggaggactcccatcaggctctgcaaagcctgtttctcagcagccagtttctgctcttgggtccttacgggccgtggaaacttaggcaaaactccaccaggccagatggactcctgaagaagcaggaggtactgcacccagcgctgtggacttgttaaattagctacctgcacctctagccacctttgaactagggtcccaaagataagacgaagaaacttttgcatgttttcggtacatagccatttccactgttctgttagtagcaagaggagcagatccagggctgtgtcagctaactctgtctctgttcctggatcgctgttgctggggtcttgggctggcacggctgcatctgacacgcaactgtccacacgtcctttgggaggttgttcaggatctttttctggggcttttgttggctgcatttccagtaactttgtctgtttttcaataaaagattccatcgcagacatggatagagtctcagactccacattgccttcctggagacaataaagaatcttgtcttgtgcttcagtcacacttagtgctggagaaattttactggatgagaacctcagcctagacttgctagccttcttgccttctgtctggggcttgctttcggtctcggcctcactcagctcctctgtggggctctggggttcagagcgaggaaacgctgtcttcaaggtgtccacaatggcactcaccaccatctttaggaatgattctaggaggctcttacgggcttctactctgtcactgtccatgtttcccaatggaagatctggaaagagctttttaggacccttcacatacacgcagcgggcagcggccggcgaagactgggtcacacgccgccgggaaccgcgcgcccacactcagccccgacctgaagtggactcatcgcggtcctctccgggagcctcggccctctgccgccgtaaacctgggcgactgcgctccgcagccgggcctgtgtgaaggctgaccgccggccggccgccggcgacagct

SEQ ID NO: 8298 - RNA, 8190 nt, Homo sapiens
  source 1..8190: mol_type = other RNA
aaaaaccacaattacttttgcaccaacccactacatcagaacctacctttaagggttgatttgtgggttaaataagtgaagatatgtaaagactttaagtaatgctctcagaagatgttaactattagctggtaccaggcattttgggagtagataggggatctgctgaatgttggcagaatgacccatccctagagcagacattgtctatcaatacccattctctgcttcttccttgctaacatcaattatttctgtagatatctgaccttcatggaagatgacctcatctctgggggaaaatactattgaaagccaatcacaatgccattctcagtgtcagtggattggcatgaggtgggtggttctagccaatgagtcataagaggttttttgttttttttttttttatttggggtctcactctgtcacttaaggctagaatgcagtggtgtgatcgtagctcactgcagcctcaaattcctgggctcaagtgatcctcctgcctcagcctccctagtaggtggaaccacaggcgagagccaccatgccccgctcattttttatattttttgtagagacagggtcttgctatgttccaggctggtcttaaactcctggactcaaacaatcccccaaccttggcctcccaaagtgttgagattataggtgtgagccgctgtgcccggcctagaagaggattcttgaaggacttctgggaaatggttccttcattccttagaagaaaacacagaagagatgctcctgttcttttatgaatgttatctctgggtgtgatgcctgaaactgcagcagcaggaaggcaggcagtctgagagcacagctgacctaattagaatggcaaggaagaaagatggaaagaattcaggccccttaagaggtctcagagttgctgaatcaccaaactcctgggcttacctactcacgtactaatgttatgaaataaaataaattttcctcataatttaattcttgtccagagcatcctgattcatatagccagggaccatagttacacatatttttacttcctccaggacctaacaactggtgttgtgtgctatgagcaaaggaagagcagtagctggaaatgaataacctgggtaggacacaggaagactcaaaaatgttctaggctatgcaaatcaaaaccatgagatagtaatatcacctaataccttttaagatgccattatgaaaaaacaaaacattacaagtgttggagaggatgtggagaaactggaacccttgtacattgttggtgggaatgtaaaatggtctagtcactatggaaaacagtatgaaggtcttcaaagaattaaaaacagaacaatatatgatccagcaatcctacttctgggtatttatctaaaataattaaaagcagggcctcgaagaaacagtcacactcccatgttcactgcagcattgttttcaacaatcaaggcgcggagccaacctaaatgtccctcaatgaatgaacaaagaaaatgtggcatagccatacaatggaatgttttcagccttaaaaagaaaattctgtcacatgctgtaacgtggatgaacctggaggacattatgctaagtgaaataagccagtcaaaggacaaacactgcatgattccacttatatgaggcgttcaaagtagtcaaactcacagaagcagaaagtagaacagtgattgccagaggctggtgggaggggaaacgaggagtggctgttcaatgggtataaacttttggttatgcaagatgaaaaacttgtagcagtctgctacaaagcactgtgctgcttctagttaataatgtaccgtctcaaaataaataaataatgtactgtacacttaagagggtagatctcacattatgtgtttctttacaacaataagaaaatcaccttgtaaactggaaatttccaaaatggaaattggagtagcttgtattgattttaaaatttatacatgctctcactcataggtgggaattgaacaatgagaacacttggacacaggaaggtgaacatcacacactggggcctgttgtgaggtcgggggagggggaagggatagcatcaggagatatacctaatgtaaatgacgagttaacgggtgcagcacaccaacacggcacatgtatacatatgcaacaaacctgcatgttgtgcacatgttccctagaacttaatgtataataataataaaaataaaatttatacatgctcctaggctcagatttaggaatttattttccatttaggttttattaagtctaatccaacaatgcaaaaatgaaactgtgagttatatgtgatgaaaaagtatagctttcttgaattcaaataagcaatggcaaagatcacatttagaatttgacagaaagaacacagcatccctgcctcgtcttttttatagatagtaagaaaagggaaagtagtcttatttcaaatatcaaaattctgacttaaatgaataaaatttagtcacgagtaaatacaaaaaacaagcaaacaataaaaccttcctggatcagcacaggcccaattcttccctgccttttatcaccctgtcagctgggagtatcttttctacctgtggctctctaccaattgttactctcttgttgtctgaacctgctagccaaacttggcaggtcgttttcaaagccagatgagttctgattgttcccttggcaatatccattatttccctcctgggtagaaggaggatctgaggacagcttatctttttggggtacgtggagtagaggtggggactcttatataatacgaaataaaaataagttctttgggctggaagtgtcaaaagattccttagaatttatagccacagggatttcatggtgtgtctgatgtactgattttgtgccacatttgagccagaactggcagcagattcaaagcaacacaggtggctaagtacacatgaggggaaggtaggtatggggagagaaaagtggcataaaacaaggctgtccccctatgctcatcgagaataggatcttagccctcactgaaggagcttaatgatcagctctaatacattggctggactcctgcaggtactcacggaaagtagagatgctgagctaccttttcttgtcaaagtctagggctggagatgcttcaagaactttggagccataaagtcactgtaatggtcaacttttaaggctagaagaggccatgagacatctcattcatctccttgcctttgggcaagaattgcacacctaagcctcccgaatacatcagacacaatttagggttaaaagcctccagaggggcaaaaaagtaaaaagattttacaactttcttccacaaaccactttaattgtgtgctcatcaccgacttcagaatctaagagaactttgacacttgtttttgacaccccattgccttctcatcagtctaactccaagaccttcctccgagtggtaggctctggtaattcagcgaaagcaaggcgctaacaggcgagtgtgaagccaaagggctcccagtgacatccttgacatctttttgccagctattcacatgcatttaatatacagcacttccctgtgactgtctgcagccttttctaccagcaattcctcctgatttatccttctccagcaattcccagttgccttgcctttctaatagatgttgcagtctgacaaaacacctttgccttcatgctggtgttgttaaaggactgattataaccgtaaggaatgggaaataagaagctattccttgtaagtttgctaatcttatctgttcagaataataaaagttctctgtcaaagacttaggaagggagatttcatcccccagccttgctagtcctactctttgtgcattcttaagacaggaggcaagtgctttccattctccttggaaaaactgaggctgaatatgcagcttgtcatgcagttttgctgaagacagagagagggtcaaaaattcaaaaactcaattgctctagggcagggggttgggagcaaagccaataaataaaatgggtggtataaatgcctttcaggaaagggtgtgaagggtggggtggatttaccagaagctttggcagtcagctttgaagtcttctggaaaggaaagtgtagcctcccaggcaagcagcctcatgacatcttccataaggctgatgtgttgggaaacagcaacacatgagcaagaagttccttgaaaaattttcttccctccttcttcttctggaactgttgggaaactagattagacccaggagtctggtttttgagaatggccctgaatgaatttttagtttccgggtaggaacagagagctgagaaggttgttttctcctccaaggaaatctggccacagtttttttcctgttctatctagagcttgtgtgctggtggattaagcacatgtgtgcacagggccaggattctggcaaacaatctcagggaggatggcaaaaggagaagcaaaaggggttcattcctctacctcacagcttcttttcccaaaggaaacaggatctactcaccagcaacaatcccaacatcacaaaaggaacagggaaataaacgtgcatacaactgggacacacagacccctgtcacctgctacaaatggagcagaagtgggagagaagtgagccaccgagaacctaggccttcttagctgtagcctacttgaagagggcacgggcttcctgactggtctctggtggccgagtaactctacttccctgacctgggaagaaggcgtgaataaccagctaagaggagacacccatcctcttagagttgcctggggtatctgaggcagaggtggtagcagcagactcctcaacagaggcactgagatccaagaattccaggatgatgtccccaaggcagtaaatcaaatgcctgttgatgaggggttgttgtagtgactccaggactagaccccagctcagccggcatttgttcaccccaagaatttctactacgagatctgggaggactcccatcaggctctgcaaagcctgtttctcagcagccagtttctgctcttgggtccttacgggccgtggaaacttaggcaaaactccaccaggccagatggactcctgaagaagcaggaggtactgcacccagcgctgtggacttgttaaattagctacctgcacctctagccacctttgaactagggtcccaaagataagacgaagaaacttttgcatgttttcggtacatagccatttccactgttctgttagtagcaagaggagcagatccagggctgtgtcagctaactctgtctctgttcctggatcgctgttgctggggtcttgggctggcacggctgcatctgacacgcaactgtccacacgtcctttgggaggttgttcaggatctttttctggggcttttgttggctgcatttccagtaactttgtctgtttttcaataaaagattccatcgcagacatggatagagtctcagactccacattgccttcctggagacaataaagaatcttgtcttgtgcttcagtcacacttagtgctggagaaattttactggatgagaacctcagcctagacttgctagccttcttgccttctgtctggggcttgctttcggtctcggcctcactcagctcctctgtggggctctggggttcagagcgaggaaacgctgtcttcaaggtgtccacaatggcactcaccaccatctttaggaatgattctaggaggctcttacgggcttctactctgtcactgtccatgtttcccaatggaagatctggaaagagctttttaggacccttcacatttttgatgaactttcgtagatctggtttctcctccagacgggtctgcagattcaagaactcccgatagcgacgattcacagtgtggtaggccagctgctgcaggccgctgctgttttcaccgtcaagggctgtctcgtacttcacagtatagagtgtgtatgggtggaatccagtgccactgtgctctcgggctgtaatggtgccagtgatacgaaggttctggatgataactggaccatcgggactgcttaggggctcaaagctgaaggtggctgagctgagaggaccaggtggagaggaggaaagcagaactggtggcagagtaggatcaagggagctcacatcattggtgagatccttctctaagcatgacggccgtgaggggcaggtcttttctggcccctccagcaaagctgtaacagaggcggtaacatctccttgttctatctccttgtctgctgtgtcaatatggatctctgggcaggaattcagtgtggagaccggcaggcctgtctctgtttctgtccctggaccctcctcagcctctgctccttcagatgcctcaccatctttgggttccagagcctgggaactctctagggcacacagggcatcctgaatcctgtcagagagaaagctgcctggagtcatgagcatgatggtttctttgcccagttcagacagcggagactccagctctgagtcttcacataagaacaggggacctcgaacatttggctgtaggaaatgagatgagttgtttcctacttttctttcttcacacatcccacccaaatctccctctacagcttcgtggccttcttcaacctctggagaggggcctgcagaaccctctggctcactgtaacttaggaatactggggctgctactggagaagctctcccttctggaagctgctctacctcagcaatcagtggcagagatgtcggcactgagggctgttcgggggcactggctgggcagggtgctggatctctggccttggaaaagatacccacgagtacaaggtggatccagtcaggatctgacagcctgctgatcagtggtaagattacattgcatgtgatgagttcgaccactacatggcgtccggtacgagtctccaagtggggcttgggcaccagcccttgaagcaacaaattcacaacgccacgcgtataggtgacttcagcactggggctgtgcacagcaggatgtggggcagtcgcccggcagtaagcctcccagaggtgggaaggctcaactggaccattcttccctgcagtggcctcctttgcctgaatgtagctctgcaggtgacaaccgcagagagtcagaacactctgggcaacagcatgactgtccatcacgctcatccttctccgaagctcctggaccaaccctttcatggctgcctccatttcttcctcaaaggctggctcctggctcacggaacggtaccaagataacacaaaatctcgaataatcatctggatggtgcggttgatctcccgttccagctgcctttctgcctcagggcatggaggacaggtggccaacgggatgaagcgttccagatgcagtcgacctgaagccactccagcgaggctggagcccagccatcctcccagcaccactagcaatgccgacagaaggcacagcagccacacgttgaccagaaggtgtatgaccaggagccagccaagcaagacccccacagccatcagcttccggctactcaacaggttattgaggtgacagctcgatccagctggagtttcctggaacggtggcactgtttctgtcttcatggctgaacggacaaggtggcttccccagatgacagccctcaagattttacttcagagttagggaaggggggcatgaactgtgtctcagatatggggcgatctgggtgctgttcagggaaccggggctccaggccctcaaagtcctacaggcactgcaaagcgacagctgcagctccgcgtctccccatggctaccactaacagagccctccaactcgccccttccagctgaggtgtggctttggaggaaaactctgtggccttcacactgccccaggcggaaggcctcttcggggcctcggggcgggcgctgcaaggccctggggcccacggacacttacacacgcagcgggcagcggccggcgaagactgggtcacacgccgccgggaaccgcgcgcccacactcagccccgacctgaagtggactcatcgcggtcctctccgggagcctcggccctctgccgccgtaaacctgggcgactgcgctccgcagccgggcctgtgtgaaggctgaccgccggccggccgccggcgacagct

SEQ ID NO: 8299 - RNA, 6111 nt, Homo sapiens
  source 1..6111: mol_type = other RNA
aaaaaccacaattacttttgcaccaacccactacatcagaacctacctttaagggttgatttgtgggttaaataagtgaagatatgtaaagactttaagtaatgctctcagaagatgttaactattagctggtaccaggcattttgggagtagataggggatctgctgaatgttggcagaatgacccatccctagagcagacattgtctatcaatacccattctctgcttcttccttgctaacatcaattatttctgtagatatctgaccttcatggaagatgacctcatctctgggggaaaatactattgaaagccaatcacaatgccattctcagtgtcagtggattggcatgaggtgggtggttctagccaatgagtcataagaggttttttgttttttttttttttatttggggtctcactctgtcacttaaggctagaatgcagtggtgtgatcgtagctcactgcagcctcaaattcctgggctcaagtgatcctcctgcctcagcctccctagtaggtggaaccacaggcgagagccaccatgccccgctcattttttatattttttgtagagacagggtcttgctatgttccaggctggtcttaaactcctggactcaaacaatcccccaaccttggcctcccaaagtgttgagattataggtgtgagccgctgtgcccggcctagaagaggattcttgaaggacttctgggaaatggttccttcattccttagaagaaaacacagaagagatgctcctgttcttttatgaatgttatctctgggtgtgatgcctgaaactgcagcagcaggaaggcaggcagtctgagagcacagctgacctaattagaatggcaaggaagaaagatggaaagaattcaggccccttaagaggtctcagagttgctgaatcaccaaactcctgggcttacctactcacgtactaatgttatgaaataaaataaattttcctcataatttaattcttgtccagagcatcctgattcatatagccagggaccatagttacacatatttttacttcctccaggacctaacaactggtgttgtgtgctatgagcaaaggaagagcagtagctggaaatgaataacctgggtaggacacaggaagactcaaaaatgttctaggctatgcaaatcaaaaccatgagatagtaatatcacctaataccttttaagatgccattatgaaaaaacaaaacattacaagtgttggagaggatgtggagaaactggaacccttgtacattgttggtgggaatgtaaaatggtctagtcactatggaaaacagtatgaaggtcttcaaagaattaaaaacagaacaatatatgatccagcaatcctacttctgggtatttatctaaaataattaaaagcagggcctcgaagaaacagtcacactcccatgttcactgcagcattgttttcaacaatcaaggcgcggagccaacctaaatgtccctcaatgaatgaacaaagaaaatgtggcatagccatacaatggaatgttttcagccttaaaaagaaaattctgtcacatgctgtaacgtggatgaacctggaggacattatgctaagtgaaataagccagtcaaaggacaaacactgcatgattccacttatatgaggcgttcaaagtagtcaaactcacagaagcagaaagtagaacagtgattgccagaggctggtgggaggggaaacgaggagtggctgttcaatgggtataaacttttggttatgcaagatgaaaaacttgtagcagtctgctacaaagcactgtgctgcttctagttaataatgtaccgtctcaaaataaataaataatgtactgtacacttaagagggtagatctcacattatgtgtttctttacaacaataagaaaatcaccttgtaaactggaaatttccaaaatggaaattggagtagcttgtattgattttaaaatttatacatgctctcactcataggtgggaattgaacaatgagaacacttggacacaggaaggtgaacatcacacactggggcctgttgtgaggtcgggggagggggaagggatagcatcaggagatatacctaatgtaaatgacgagttaacgggtgcagcacaccaacacggcacatgtatacatatgcaacaaacctgcatgttgtgcacatgttccctagaacttaatgtataataataataaaaataaaatttatacatgctcctaggctcagatttaggaatttattttccatttaggttttattaagtctaatccaacaatgcaaaaatgaaactgtgagttatatgtgatgaaaaagtatagctttcttgaattcaaataagcaatggcaaagatcacatttagaatttgacagaaagaacacagcatccctgcctcgtcttttttatagatagtaagaaaagggaaagtagtcttatttcaaatatcaaaattctgacttaaatgaataaaatttagtcacgagtaaatacaaaaaacaagcaaacaataaaaccttcctggatcagcacaggcccaattcttccctgccttttatcaccctgtcagctgggagtatcttttctacctgtggctctctaccaattgttactctcttgttgtctgaacctgctagccaaacttggcaggtcgttttcaaagccagatgagttctgattgttcccttggcaatatccattatttccctcctgggtagaaggaggatctgaggacagcttatctttttggggtacgtggagtagaggtggggactcttatataatacgaaataaaaataagttctttgggctggaagtgtcaaaagattccttagaatttatagccacagggatttcatggtgtgtctgatgtactgattttgtgccacatttgagccagaactggcagcagattcaaagcaacacaggtggctaagtacacatgaggggaaggtaggtatggggagagaaaagtggcataaaacaaggctgtccccctatgctcatcgagaataggatcttagccctcactgaaggagcttaatgatcagctctaatacattggctggactcctgcaggtactcacggaaagtagagatgctgagctaccttttcttgtcaaagtctagggctggagatgcttcaagaactttggagccataaagtcactgtaatggtcaacttttaaggctagaagaggccatgagacatctcattcatctccttgcctttgggcaagaattgcacacctaagcctcccgaatacatcagacacaatttagggttaaaagcctccagaggggcaaaaaagtaaaaagattttacaactttcttccacaaaccactttaattgtgtgctcatcaccgacttcagaatctaagagaactttgacacttgtttttgacaccccattgccttctcatcagtctaactccaagaccttcctccgagtggtaggctctggtaattcagcgaaagcaaggcgctaacaggcgagtgtgaagccaaagggctcccagtgacatccttgacatctttttgccagctattcacatgcatttaatatacagcacttccctgtgactgtctgcagccttttctaccagcaattcctcctgatttatccttctccagcaattcccagttgccttgcctttctaatagatgttgcagtctgacaaaacacctttgccttcatgctggtgttgttaaaggactgattataaccgtaaggaatgggaaataagaagctattccttgtaagtttgctaatcttatctgttcagaataataaaagttctctgtcaaagacttaggaagggagatttcatcccccagccttgctagtcctactctttgtgcattcttaagacaggaggcaagtgctttccattctccttggaaaaactgaggctgaatatgcagcttgtcatgcagttttgctgaagacagagagagggtcaaaaattcaaaaactcaattgctctagggcagggggttgggagcaaagccaataaataaaatgggtggtataaatgcctttcaggaaagggtgtgaagggtggggtggatttaccagaagctttggcagtcagctttgaagtcttctggaaaggaaagtgtagcctcccaggcaagcagcctcatgacatcttccataaggctgatgtgttgggaaacagcaacacatgagcaagaagttccttgaaaaattttcttccctccttcttcttctggaactgttgggaaactagattagacccaggagtctggtttttgagaatggccctgaatgaatttttagtttccgggtaggaacagagagctgagaaggttgttttctcctccaaggaaatctggccacagtttttttcctgttctatctagagcttgtgtgctggtggattaagcacatgtgtgcacagggccaggattctggcaaacaatctcagggaggatggcaaaaggagaagcaaaaggggttcattcctctacctcacagcttcttttcccaaaggaaacaggatctactcaccagcaacaatcccaacatcacaaaaggaacagggaaataaacgtgcatacaactgggacacacagacccctgtcacctgctacaaatggagcagaagtgggagagaagtgagccaccgagaacctaggccttcttagctgtagcctacttgaagagggcacgggcttcctgactggtctctggtggccgagtaactctacttccctgacctgggaagaaggcgtgaataaccagctaagaggagacacccatcctcttagagttgcctggggtatctgaggcagaggtggtagcagcagactcctcaacagaggcactgagatccaagaattccaggatgatgtccccaaggcagtaaatcaaatgcctgttgatgaggggttgttgtagtgactccaggactagaccccagctcagccggcatttgttcaccccaagaatttctactacgagatctttgaactagggtcccaaagataagacgaagaaacttttgcatgttttcggtacatagccatttccactgttctgttagtagcaagaggagcagatccagggctgtgtcagctaactctgtctctgttcctggatcgctgttgctggggtcttgggctggcacggctgcatctgacacgcaactgtccacacgtcctttgggaggttgttcaggatctttttctggggcttttgttggctgcatttccagtaactttgtctgtttttcaataaaagattccatcgcagacatggatagagtctcagactccacattgccttcctggagacaataaagaatcttgtcttgtgcttcagtcacacttagtgctggagaaattttactggatgagaacctcagcctagacttgctagccttcttgccttctgtctggggcttgctttcggtctcggcctcactcagctcctctgtggggctctggggttcagagcgaggaaacgctgtcttcaaggtgtccacaatggcactcaccaccatcttgtctattctagagaccataaatggtttcttgacaaaggcaatacgagcatctgtgttcagagcaaggaactcctgcacctcctcactgttagcgatctccggaatggcacagagttgctttaggaatgattctaggaggctcttacgggcttctactctgtcactgtccatgtttcccaatggaagatctggaaagagctttttaggacccttcacatttttgatgaactttcgtagatctggtttctcctccagacgggtctgcagattcaagaactcccgatagcgacgattcacagtgtggtaggccagctgctgcaggccgctgctgttttcaccgtcaagggctgtctcgtaacacgcagcgggcagcggccggcgaagactgggtcacacgccgccgggaaccgcgcgcccacactcagccccgacctgaagtggactcatcgcggtcctctccgggagcctcggccctctgccgccgtaaacctgggcgactgcgctccgcagccgggcctgtgtgaaggctgaccgccggccggccgccggcgacagct

SEQ ID NO: 8300 - RNA, 8125 nt, Homo sapiens
  source 1..8125: mol_type = other RNA
aaaaaccacaattacttttgcaccaacccactacatcagaacctacctttaagggttgatttgtgggttaaataagtgaagatatgtaaagactttaagtaatgctctcagaagatgttaactattagctggtaccaggcattttgggagtagataggggatctgctgaatgttggcagaatgacccatccctagagcagacattgtctatcaatacccattctctgcttcttccttgctaacatcaattatttctgtagatatctgaccttcatggaagatgacctcatctctgggggaaaatactattgaaagccaatcacaatgccattctcagtgtcagtggattggcatgaggtgggtggttctagccaatgagtcataagaggttttttgttttttttttttttatttggggtctcactctgtcacttaaggctagaatgcagtggtgtgatcgtagctcactgcagcctcaaattcctgggctcaagtgatcctcctgcctcagcctccctagtaggtggaaccacaggcgagagccaccatgccccgctcattttttatattttttgtagagacagggtcttgctatgttccaggctggtcttaaactcctggactcaaacaatcccccaaccttggcctcccaaagtgttgagattataggtgtgagccgctgtgcccggcctagaagaggattcttgaaggacttctgggaaatggttccttcattccttagaagaaaacacagaagagatgctcctgttcttttatgaatgttatctctgggtgtgatgcctgaaactgcagcagcaggaaggcaggcagtctgagagcacagctgacctaattagaatggcaaggaagaaagatggaaagaattcaggccccttaagaggtctcagagttgctgaatcaccaaactcctgggcttacctactcacgtactaatgttatgaaataaaataaattttcctcataatttaattcttgtccagagcatcctgattcatatagccagggaccatagttacacatatttttacttcctccaggacctaacaactggtgttgtgtgctatgagcaaaggaagagcagtagctggaaatgaataacctgggtaggacacaggaagactcaaaaatgttctaggctatgcaaatcaaaaccatgagatagtaatatcacctaataccttttaagatgccattatgaaaaaacaaaacattacaagtgttggagaggatgtggagaaactggaacccttgtacattgttggtgggaatgtaaaatggtctagtcactatggaaaacagtatgaaggtcttcaaagaattaaaaacagaacaatatatgatccagcaatcctacttctgggtatttatctaaaataattaaaagcagggcctcgaagaaacagtcacactcccatgttcactgcagcattgttttcaacaatcaaggcgcggagccaacctaaatgtccctcaatgaatgaacaaagaaaatgtggcatagccatacaatggaatgttttcagccttaaaaagaaaattctgtcacatgctgtaacgtggatgaacctggaggacattatgctaagtgaaataagccagtcaaaggacaaacactgcatgattccacttatatgaggcgttcaaagtagtcaaactcacagaagcagaaagtagaacagtgattgccagaggctggtgggaggggaaacgaggagtggctgttcaatgggtataaacttttggttatgcaagatgaaaaacttgtagcagtctgctacaaagcactgtgctgcttctagttaataatgtaccgtctcaaaataaataaataatgtactgtacacttaagagggtagatctcacattatgtgtttctttacaacaataagaaaatcaccttgtaaactggaaatttccaaaatggaaattggagtagcttgtattgattttaaaatttatacatgctctcactcataggtgggaattgaacaatgagaacacttggacacaggaaggtgaacatcacacactggggcctgttgtgaggtcgggggagggggaagggatagcatcaggagatatacctaatgtaaatgacgagttaacgggtgcagcacaccaacacggcacatgtatacatatgcaacaaacctgcatgttgtgcacatgttccctagaacttaatgtataataataataaaaataaaatttatacatgctcctaggctcagatttaggaatttattttccatttaggttttattaagtctaatccaacaatgcaaaaatgaaactgtgagttatatgtgatgaaaaagtatagctttcttgaattcaaataagcaatggcaaagatcacatttagaatttgacagaaagaacacagcatccctgcctcgtcttttttatagatagtaagaaaagggaaagtagtcttatttcaaatatcaaaattctgacttaaatgaataaaatttagtcacgagtaaatacaaaaaacaagcaaacaataaaaccttcctggatcagcacaggcccaattcttccctgccttttatcaccctgtcagctgggagtatcttttctacctgtggctctctaccaattgttactctcttgttgtctgaacctgctagccaaacttggcaggtcgttttcaaagccagatgagttctgattgttcccttggcaatatccattatttccctcctgggtagaaggaggatctgaggacagcttatctttttggggtacgtggagtagaggtggggactcttatataatacgaaataaaaataagttctttgggctggaagtgtcaaaagattccttagaatttatagccacagggatttcatggtgtgtctgatgtactgattttgtgccacatttgagccagaactggcagcagattcaaagcaacacaggtggctaagtacacatgaggggaaggtaggtatggggagagaaaagtggcataaaacaaggctgtccccctatgctcatcgagaataggatcttagccctcactgaaggagcttaatgatcagctctaatacattggctggactcctgcaggtactcacggaaagtagagatgctgagctaccttttcttgtcaaagtctagggctggagatgcttcaagaactttggagccataaagtcactgtaatggtcaacttttaaggctagaagaggccatgagacatctcattcatctccttgcctttgggcaagaattgcacacctaagcctcccgaatacatcagacacaatttagggttaaaagcctccagaggggcaaaaaagtaaaaagattttacaactttcttccacaaaccactttaattgtgtgctcatcaccgacttcagaatctaagagaactttgacacttgtttttgacaccccattgccttctcatcagtctaactccaagaccttcctccgagtggtaggctctggtaattcagcgaaagcaaggcgctaacaggcgagtgtgaagccaaagggctcccagtgacatccttgacatctttttgccagctattcacatgcatttaatatacagcacttccctgtgactgtctgcagccttttctaccagcaattcctcctgatttatccttctccagcaattcccagttgccttgcctttctaatagatgttgcagtctgacaaaacacctttgccttcatgctggtgttgttaaaggactgattataaccgtaaggaatgggaaataagaagctattccttgtaagtttgctaatcttatctgttcagaataataaaagttctctgtcaaagacttaggaagggagatttcatcccccagccttgctagtcctactctttgtgcattcttaagacaggaggcaagtgctttccattctccttggaaaaactgaggctgaatatgcagcttgtcatgcagttttgctgaagacagagagagggtcaaaaattcaaaaactcaattgctctagggcagggggttgggagcaaagccaataaataaaatgggtggtataaatgcctttcaggaaagggtgtgaagggtggggtggatttaccagaagctttggcagtcagctttgaagtcttctggaaaggaaagtgtagcctcccaggcaagcagcctcatgacatcttccataaggctgatgtgttgggaaacagcaacacatgagcaagaagttccttgaaaaattttcttccctccttcttcttctggaactgttgggaaactagattagacccaggagtctggtttttgagaatggccctgaatgaatttttagtttccgggtaggaacagagagctgagaaggttgttttctcctccaaggaaatctggccacagtttttttcctgttctatctagagcttgtgtgctggtggattaagcacatgtgtgcacagggccaggattctggcaaacaatctcagggaggatggcaaaaggagaagcaaaaggggttcattcctctacctcacagcttcttttcccaaaggaaacaggatctactcaccagcaacaatcccaacatcacaaaaggaacagggaaataaacgtgcatacaactgggacacacagacccctgtcacctgctacaaatggagcagaagtgggagagaagtgagccaccgagaacctaggccttcttagctgtagcctacttgaagagggcacgggcttcctgactggtctctggtggccgagtaactctacttccctgacctgggaagaaggcgtgaataaccagctaagaggagacacccatcctcttagagttgcctggggtatctgaggcagaggtggtagcagcagactcctcaacagaggcactgagatccaagaattccaggatgatgtccccaaggcagtaaatcaaatgcctgttgatgaggggttgttgtagtgactccaggactagaccccagctcagccggcatttgttcaccccaagaatttctactacgagatctttgaactagggtcccaaagataagacgaagaaacttttgcatgttttcggtacatagccatttccactgttctgttagtagcaagaggagcagatccagggctgtgtcagctaactctgtctctgttcctggatcgctgttgctggggtcttgggctggcacggctgcatctgacacgcaactgtccacacgtcctttgggaggttgttcaggatctttttctggggcttttgttggctgcatttccagtaactttgtctgtttttcaataaaagattccatcgcagacatggatagagtctcagactccacattgccttcctggagacaataaagaatcttgtcttgtgcttcagtcacacttagtgctggagaaattttactggatgagaacctcagcctagacttgctagccttcttgccttctgtctggggcttgctttcggtctcggcctcactcagctcctctgtggggctctggggttcagagcgaggaaacgctgtcttcaaggtgtccacaatggcactcaccaccatcttgtctattctagagaccataaatggtttcttgacaaaggcaatacgagcatctgtgttcagagcaaggaactcctgcacctcctcactgttagcgatctccggaatggcacagagttgctttaggaatgattctaggaggctcttacgggcttctactctgtcactgtccatgtttcccaatggaagatctggaaagagctttttaggacccttcacatttttgatgaactttcgtagatctggtttctcctccagacgggtctgcagattcaagaactcccgatagcgacgattcacagtgtggtaggccagctgctgcaggccgctgctgttttcaccgtcaagggctgtctcgtacttcacagtatagagtgtgtatgggtggaatccagtgccactgtgctctcgggctgtaatggtgccagtgatacgaaggttctggatgataactggaccatcgggactgcttaggggctcaaagctgaaggtggctgagctgagaggaccaggtggagaggaggaaagcagaactggtggcagagtaggatcaagggagctcacatcattggtgagatccttctctaagcatgacggccgtgaggggcaggtcttttctggcccctccagcaaagctgtaacagaggcggtaacatctccttgttctatctccttgtctgctgtgtcaatatggatctctgggcaggaattcagtgtggagaccggcaggcctgtctctgtttctgtccctggaccctcctcagcctctgctccttcagatgcctcaccatctttgggttccagagcctgggaactctctagggcacacagggcatcctgaatcctgtcagagagaaagctgcctggagtcatgagcatgatggtttctttgcccagttcagacagcggagactccagctctgagtcttcacataagaacaggggacctcgaacatttggctgtaggaaatgagatgagttgtttcctacttttctttcttcacacatcccacccaaatctccctctacagcttcgtggccttcttcaacctctggagaggggcctgcagaaccctctggctcactgtaacttaggaatactggggctgctactggagaagctctcccttctggaagctgctctacctcagcaatcagtggcagagatgtcggcactgagggctgttcgggggcactggctgggcagggtgctggatctctggccttggaaaagatacccacgagtacaaggtggatccagtcaggatctgacagcctgctgatcagtggtaagattacattgcatgtgatgagttcgaccactacatggcgtccggtacgagtctccaagtggggcttgggcaccagcccttgaagcaacaaattcacaacgccacgcgtataggtgacttcagcactggggctgtgcacagcaggatgtggggcagtcgcccggcagtaagcctcccagaggtgggaaggctcaactggaccattcttccctgcagtggcctcctttgcctgaatgtagctctgcaggtgacaaccgcagagagtcagaacactctgggcaacagcatgactgtccatcacgctcatccttctccgaagctcctggaccaaccctttcatggctgcctccatttcttcctcaaaggctggctcctggctcacggaacggtaccaagataacacaaaatctcgaataatcatctggatggtgcggttgatctcccgttccagctgcctttctgcctcagggcatggaggacaggtggccaacgggatgaagcgttccagatgcagtcgacctgaagccactccagcgaggctggagcccagccatcctcccagcaccactagcaatgccgacagaaggcacagcagccacacgttgaccagaaggtgtatgaccaggagccagccaagcaagacccccacagccatcagcttccggctactcaacaggttattgaggtgacagctcgatccagctggagtttcctggaacggtggcactgtttctgtcttcatggctgaacggacaaggtggcttccccagatgacagccctcaagattttacttcagagttagggaaggggggcatgaactgtgtctcagatatggggcgatctgggtgctgttcagggaaccggggctccaggccctcaaagtcctacaggcactgcaaagcgacagctgcagctccgcgtctccccatggctaccactaacagagccctccaactcgccccttccagctgaggtgtggctttggaggaaaactctgtggccttcacactgccccaggcggaaggcctcttcggggcctcggggcgggcgctgcaaggccctggggcccacggacacttacacacgcagcgggcagcggccggcgaagactgggtcacacgccgccgggaaccgcgcgcccacactcagccccgacctgaagtggactcatcgcggtcctctccgggagcctcggccctctgccgccgtaaacctgggcgactgcgctccgcagccgggcctgtgtgaaggctgaccgccggccggccgccggcgacagct

SEQ ID NO: 8301 - RNA, 3385 nt, Homo sapiens
  source 1..3385: mol_type = other RNA
aaaaaccacaattacttttgcaccaacccattacaaacaagttttaacaatcacaagactaatgttttagtgacggctcctaaaacttcagggaaaaaaaaagtgcatttctgactggcaatagtttgcaaaataatcgtaatgaaactacttatttctttattttaaaagttaataaaaggaaacctctcaatttttaggaagaattcaattacaataaaatcatgatgtcttatgatctggcatcttataatctgtgtctcagaaagaagggcaatttacagcatcagatgaatactggagtttaggtcagacttaagttatctgaaaagaacataaggcatttacagtttttagcagggaaaaataatcaaatctctttttttaaaaaaaaccttcttagtatcttggttaaatgtccaaaaagctgtattatttttagttttaaaccagtaggcactattcgaaactgagaattcaggatgttatcaaatacaaatttttaaaagcttgaccattaaagcataaattgcctaatgagacacatgtaatcataaaaactaacgccaggatcatttacttgtgattggatatatgccatttatttttctggcttctttctaatgtgtaattcctgctgaattgagtgagcatgtcagatttctatctttatcttagtgtgtgtaaaagttctcaacctagacaaggacaaattttagaattttccaatgaacatcattcactatgtatgatgctgttttgttaaactagctgtttggaaaacaataaagatttcatttgttttgcgttagccacagagagtggacttgtttagaatgtaaaagtatttatctcaaatactaaaatcaaactcaagaaaaatcaaacaatgctggagctgagaaaaataatggctatatatctggttgaacatgttgaaagaaaagtgaaaacacagccaggcatggtggtgcgcacctgtaatcccagctacttgggaggctgagacaggagaattgcttgaatctaggaggcagaggttgcagtgagccaagatcaaccactgcactacacagcctgggtgacacagactccttcacgcacacacaaaaaagtgaaaacaaacttggaagtctagaatgaagaattacatctaatgcagtaatattcttcccacctttccatattaaatgtaagaagcaccagcaaaaaatactaaagacagagaaatgacctggcaaaatgattcaaataccacagagcgtgagaatattcctcagtaaagctcaagatattatgaagtagctagcagaagaaatggcaggggtagcggaagtaaaaattctaaccatatgacagactctaacagtaagtcataaattctaaaggtttaattagtaaattcattatttcctccaaaatatactgtcattcttctcttaacaatgaatgtttgacacaaatccaattttgatgttaaaagtcaacatacatagataggtccctcatgttgacagagcacagaattggaaaaaaaaactgcaaatgagaaataggggtatttctaaatcttctgtattcctaaaatatcacactgcgcccttgcttcagcctccctgatagactggtttgggtgtgcaatattaatgcaggaatacgtggaataccagcacaaagccggggagggagactagcaaactctcgccatcaattatttctcaactacatttagtattcttcgcagttttagatttttttttcctttaagcgaaaaccactccactgaaaaaaattccaaacttgttttttaaaaattgcaggaatttcttcgtattttatcaacaaaaataccagaaattaaagagctgacagaaattcaagcagatccaaattcaaccatccatttttcatacttctccaagtctgcagcagagacagacttagcaattttctttagggccaattcaaagtctcctttggtaacaggcatctgaagttcctctttagaaagtgcacggatttcttctggacttaagccattgatacgccgtctcattgccattaaagaggcatccctgcaaacattagtgatgtcagcaccagaatagccctcaatcttctcggctatatcttccagttgaatatcaggatctaattcgacctcacgaaggttgatcttcagaagctcagctcttccttttgctgttgggagaggtatatatatccttttttctaaccttcttcgcaaagcttcatcaatgtcccacgggaaattagtagcagccaataccataaccattttggaaggatcatcattttctaaagctcctccaactccatccatctgaatgagcagttcagacttgaccctgcgacttgcctcatgttcatcagaggttcctcttcgactgcagatagaatctatctcatcaatgaagatcgtggtaggggcataaaatctagccatctcaaacaacagacgaactaacttctcagattcacctctgtatttagatgtcagtgtagaagacgaaacgttgaagaatgttgtaccacattcagtggcaacagctttagctagcatagttttaccagtgcctgggggtccaaccatcagtacacccttccatggccttctaatccctttgaaaaagtcaggcatccacattggaagaacaacagcttcccttagcaacttcttagcttcttccagatctgctatgtcatcccaatgaatgctaggattcctggatacaatgtctctttcaagggcttccaccagatccttatcataaccagcaccatcaaattttggcatttcaccatcacttgcaccatcttgcatattcttccttccctgtgttctgcaggaacagggggtggccaaacagcaggatctctaaatggttcatcttgacaggacacagggaaatctggaggcttgtcaattttaaaactttctaaagtgctgacaatacttttaacttgttcatattcctccaataattcctgccgaacctgttgccatttgcctttgatagctggatctctgactgactggcaatgtctctgaatctgctgcatcaccccctggtaatataccattgatgagtcgtaatttccaagaagggcatattctcttcctttctttgcattatcacaaatctcagccaaattcatcttctttcagagacccagaaataaacgtatccaggaaaggagaaaaacctgttaaaacacggtttctcaggtctcacatccaatgtgtgacatacatacggttctgcaccgaaaggcagcaacctgcgagggtcagaggcgccgaagacccgaggccctgcagcttgggcggctgctcatccctgagactgtgcagggcggtggc

SEQ ID NO: 8302 - RNA, 3365 nt, Homo sapiens
  source 1..3365: mol_type = other RNA
aaaaaccacaattacttttgcaccaacccattacaaacaagttttaacaatcacaagactaatgttttagtgacggctcctaaaacttcagggaaaaaaaaagtgcatttctgactggcaatagtttgcaaaataatcgtaatgaaactacttatttctttattttaaaagttaataaaaggaaacctctcaatttttaggaagaattcaattacaataaaatcatgatgtcttatgatctggcatcttataatctgtgtctcagaaagaagggcaatttacagcatcagatgaatactggagtttaggtcagacttaagttatctgaaaagaacataaggcatttacagtttttagcagggaaaaataatcaaatctctttttttaaaaaaaaccttcttagtatcttggttaaatgtccaaaaagctgtattatttttagttttaaaccagtaggcactattcgaaactgagaattcaggatgttatcaaatacaaatttttaaaagcttgaccattaaagcataaattgcctaatgagacacatgtaatcataaaaactaacgccaggatcatttacttgtgattggatatatgccatttatttttctggcttctttctaatgtgtaattcctgctgaattgagtgagcatgtcagatttctatctttatcttagtgtgtgtaaaagttctcaacctagacaaggacaaattttagaattttccaatgaacatcattcactatgtatgatgctgttttgttaaactagctgtttggaaaacaataaagatttcatttgttttgcgttagccacagagagtggacttgtttagaatgtaaaagtatttatctcaaatactaaaatcaaactcaagaaaaatcaaacaatgctggagctgagaaaaataatggctatatatctggttgaacatgttgaaagaaaagtgaaaacacagccaggcatggtggtgcgcacctgtaatcccagctacttgggaggctgagacaggagaattgcttgaatctaggaggcagaggttgcagtgagccaagatcaaccactgcactacacagcctgggtgacacagactccttcacgcacacacaaaaaagtgaaaacaaacttggaagtctagaatgaagaattacatctaatgcagtaatattcttcccacctttccatattaaatgtaagaagcaccagcaaaaaatactaaagacagagaaatgacctggcaaaatgattcaaataccacagagcgtgagaatattcctcagtaaagctcaagatattatgaagtagctagcagaagaaatggcaggggtagcggaagtaaaaattctaaccatatgacagactctaacagtaagtcataaattctaaaggtttaattagtaaattcattatttcctccaaaatatactgtcattcttctcttaacaatgaatgtttgacacaaatccaattttgatgttaaaagtcaacatacatagataggtccctcatgttgacagagcacagaattggaaaaaaaaactgcaaatgagaaataggggtatttctaaatcttctgtattcctaaaatatcacactgcgcccttgcttcagcctccctgatagactggtttgggtgtgcaatattaatgcaggaatacgtggaataccagcacaaagccggggagggagactagcaaactctcgccatcaattatttctcaactacatttagtattcttcgcagttttagatttttttttcctttaagcgaaaaccactccactgaaaaaaattccaaacttgttttttaaaaattgcaggaatttcttcgtattttatcaacaaaaataccagaaattaaagagctgacagaaattcaagcagatccaaattcaaccatccatttttcatacttctccaagtctgcagcagagacagacttagcaattttctttagggccaattcaaagtctcctttggtaacaggcatctgaagttcctctttagaaagtgcacggatttcttctggacttaagccattgatacgccgtctcattgccattaaagaggcatccctgcaaacattagtgatgtcagcaccagaatagccctcaatcttctcggctatatcttccagttgaatatcaggatctaattcgacctcacgaaggttgatcttcagaagctcagctcttccttttgctgttgggagaggtatatatatccttttttctaaccttcttcgcaaagcttcatcaatgtcccacgggaaattagtagcagccaataccataaccattttggaaggatcatcattttctaaagctcctccaactccatccatctgaatgagcagttcagacttgaccctgcgacttgcctcatgttcatcagaggttcctcttcgactgcagatagaatctatctcatcaatgaagatcgtggtaggggcataaaatctagccatctcaaacaacagacgaactaacttctcagattcacctctgtatttagatgtcagtgtagaagacgaaacgttgaagaatgttgtaccacattcagtggcaacagctttagctagcatagttttaccagtgcctgggggtccaaccatcagtacacccttccatggccttctaatccctttgaaaaagtcaggcatccacattggaagaacaacagcttcccttagcaacttcttagcttcttccagatctgctatgtcatcccaatgaatgctaggattcctggatacaatgtctctttcaagggcttccaccagatccttatcataaccagcaccatcaaattttggcatttcaccatcacttgcaccatcttgcatattcttccttccctgtgttctgcaggaacagggggtggccaaacagcaggatctctaaatggttcatcttgacaggacacagggaaatctggaggcttgtcaattttaaaactttctaaagtgctgacaatacttttaacttgttcatattcctccaataattcctgccgaacctgttgccatttgcctttgatagctggatctctgactgactggcaatgtctctgaatctgctgcatcaccccctggtaatataccattgatgagtcgtaatttccaagaagggcatattctcttcctttctttgcattatcacaaatctcagccaaattcatcttctttcagagacccagaaggcgcaggtccgggcacattcagcgatgcggtccagatggggtgcgggtggggcgcaggccgccgccgccgccgccgccgagtccgttagctcgcgacgtgcgtgaaaaggcggcggcggcgtagtgttgccatggcagccgcggccgcgcggtgggcgcagcgc

SEQ ID NO: 8303 - RNA, 3493 nt, Homo sapiens
  source 1..3493: mol_type = other RNA
aaaaaccacaattacttttgcaccaacccattacaaacaagttttaacaatcacaagactaatgttttagtgacggctcctaaaacttcagggaaaaaaaaagtgcatttctgactggcaatagtttgcaaaataatcgtaatgaaactacttatttctttattttaaaagttaataaaaggaaacctctcaatttttaggaagaattcaattacaataaaatcatgatgtcttatgatctggcatcttataatctgtgtctcagaaagaagggcaatttacagcatcagatgaatactggagtttaggtcagacttaagttatctgaaaagaacataaggcatttacagtttttagcagggaaaaataatcaaatctctttttttaaaaaaaaccttcttagtatcttggttaaatgtccaaaaagctgtattatttttagttttaaaccagtaggcactattcgaaactgagaattcaggatgttatcaaatacaaatttttaaaagcttgaccattaaagcataaattgcctaatgagacacatgtaatcataaaaactaacgccaggatcatttacttgtgattggatatatgccatttatttttctggcttctttctaatgtgtaattcctgctgaattgagtgagcatgtcagatttctatctttatcttagtgtgtgtaaaagttctcaacctagacaaggacaaattttagaattttccaatgaacatcattcactatgtatgatgctgttttgttaaactagctgtttggaaaacaataaagatttcatttgttttgcgttagccacagagagtggacttgtttagaatgtaaaagtatttatctcaaatactaaaatcaaactcaagaaaaatcaaacaatgctggagctgagaaaaataatggctatatatctggttgaacatgttgaaagaaaagtgaaaacacagccaggcatggtggtgcgcacctgtaatcccagctacttgggaggctgagacaggagaattgcttgaatctaggaggcagaggttgcagtgagccaagatcaaccactgcactacacagcctgggtgacacagactccttcacgcacacacaaaaaagtgaaaacaaacttggaagtctagaatgaagaattacatctaatgcagtaatattcttcccacctttccatattaaatgtaagaagcaccagcaaaaaatactaaagacagagaaatgacctggcaaaatgattcaaataccacagagcgtgagaatattcctcagtaaagctcaagatattatgaagtagctagcagaagaaatggcaggggtagcggaagtaaaaattctaaccatatgacagactctaacagtaagtcataaattctaaaggtttaattagtaaattcattatttcctccaaaatatactgtcattcttctcttaacaatgaatgtttgacacaaatccaattttgatgttaaaagtcaacatacatagataggtccctcatgttgacagagcacagaattggaaaaaaaaactgcaaatgagaaataggggtatttctaaatcttctgtattcctaaaatatcacactgcgcccttgcttcagcctccctgatagactggtttgggtgtgcaatattaatgcaggaatacgtggaataccagcacaaagccggggagggagactagcaaactctcgccatcaattatttctcaactacatttagtattcttcgcagttttagatttttttttcctttaagcgaaaaccactccactgaaaaaaattccaaacttgttttttaaaaattgcaggaatttcttcgtattttatcaacaaaaataccagaaattaaagagctgacagaaattcaagcagatccaaattcaaccatccatttttcatacttctccaagtctgcagcagagacagacttagcaattttctttagggccaattcaaagtctcctttggtaacaggcatctgaagttcctctttagaaagtgcacggatttcttctggacttaagccattgatacgccgtctcattgccattaaagaggcatccctgcaaacattagtgatgtcagcaccagaatagccctcaatcttctcggctatatcttccagttgaatatcaggatctaattcgacctcacgaaggttgatcttcagaagctcagctcttccttttgctgttgggagaggtatatatatccttttttctaaccttcttcgcaaagcttcatcaatgtcccacgggaaattagtagcagccaataccataaccattttggaaggatcatcattttctaaagctcctccaactccatccatctgaatgagcagttcagacttgaccctgcgacttgcctcatgttcatcagaggttcctcttcgactgcagatagaatctatctcatcaatgaagatcgtggtaggggcataaaatctagccatctcaaacaacagacgaactaacttctcagattcacctctgtatttagatgtcagtgtagaagacgaaacgttgaagaatgttgtaccacattcagtggcaacagctttagctagcatagttttaccagtgcctgggggtccaaccatcagtacacccttccatggccttctaatccctttgaaaaagtcaggcatccacattggaagaacaacagcttcccttagcaacttcttagcttcttccagatctgctatgtcatcccaatgaatgctaggattcctggatacaatgtctctttcaagggcttccaccagatccttatcataaccagcaccatcaaattttggcatttcaccatcacttgcaccatcttgcatattcttccttccctgtgttctgcaggaacagggggtggccaaacagcaggatctctaaatggttcatcttgacaggacacagggaaatctggaggcttgtcaattttaaaactttctaaagtgctgacaatacttttaacttgttcatattcctccaataattcctgccgaacctgttgccatttgcctttgatagctggatctctgactgactggcaatgtctctgaatctgctgcatcaccccctggtaatataccattgatgagtcgtaatttccaagaagggcatattctcttcctttctttgcattatcacaaatctcagccaaattcatcttctttcagagacctgttaaaacacggtttctcaggtctcacatccaatgtgtgacatacatacggttctgcaccgaaaggcagcaacctgcgagggtcagaggcgccgaagacccgaggccctgcagcttgggcggctgctcatccctgagactgtgcagggcggtggcccagccggggtggggctgagcgctgcaactggggcgggcccagctacagggcgggaagcccgaggctcacctccacttccctttcccaacgcacagagcccaggtccgcgaccactcaacagccccctcaagacaaagagag

SEQ ID NO: 8304 - RNA, 3475 nt, Homo sapiens
  source 1..3475: mol_type = other RNA
aaaaaccacaattacttttgcaccaacccattacaaacaagttttaacaatcacaagactaatgttttagtgacggctcctaaaacttcagggaaaaaaaaagtgcatttctgactggcaatagtttgcaaaataatcgtaatgaaactacttatttctttattttaaaagttaataaaaggaaacctctcaatttttaggaagaattcaattacaataaaatcatgatgtcttatgatctggcatcttataatctgtgtctcagaaagaagggcaatttacagcatcagatgaatactggagtttaggtcagacttaagttatctgaaaagaacataaggcatttacagtttttagcagggaaaaataatcaaatctctttttttaaaaaaaaccttcttagtatcttggttaaatgtccaaaaagctgtattatttttagttttaaaccagtaggcactattcgaaactgagaattcaggatgttatcaaatacaaatttttaaaagcttgaccattaaagcataaattgcctaatgagacacatgtaatcataaaaactaacgccaggatcatttacttgtgattggatatatgccatttatttttctggcttctttctaatgtgtaattcctgctgaattgagtgagcatgtcagatttctatctttatcttagtgtgtgtaaaagttctcaacctagacaaggacaaattttagaattttccaatgaacatcattcactatgtatgatgctgttttgttaaactagctgtttggaaaacaataaagatttcatttgttttgcgttagccacagagagtggacttgtttagaatgtaaaagtatttatctcaaatactaaaatcaaactcaagaaaaatcaaacaatgctggagctgagaaaaataatggctatatatctggttgaacatgttgaaagaaaagtgaaaacacagccaggcatggtggtgcgcacctgtaatcccagctacttgggaggctgagacaggagaattgcttgaatctaggaggcagaggttgcagtgagccaagatcaaccactgcactacacagcctgggtgacacagactccttcacgcacacacaaaaaagtgaaaacaaacttggaagtctagaatgaagaattacatctaatgcagtaatattcttcccacctttccatattaaatgtaagaagcaccagcaaaaaatactaaagacagagaaatgacctggcaaaatgattcaaataccacagagcgtgagaatattcctcagtaaagctcaagatattatgaagtagctagcagaagaaatggcaggggtagcggaagtaaaaattctaaccatatgacagactctaacagtaagtcataaattctaaaggtttaattagtaaattcattatttcctccaaaatatactgtcattcttctcttaacaatgaatgtttgacacaaatccaattttgatgttaaaagtcaacatacatagataggtccctcatgttgacagagcacagaattggaaaaaaaaactgcaaatgagaaataggggtatttctaaatcttctgtattcctaaaatatcacactgcgcccttgcttcagcctccctgatagactggtttgggtgtgcaatattaatgcaggaatacgtggaataccagcacaaagccggggagggagactagcaaactctcgccatcaattatttctcaactacatttagtattcttcgcagttttagatttttttttcctttaagcgaaaaccactccactgaaaaaaattccaaacttgttttttaaaaattgcaggaatttcttcgtattttatcaacaaaaataccagaaattaaagagctgacagaaattcaagcagatccaaattcaaccatccatttttcatacttctccaagtctgcagcagagacagacttagcaattttctttagggccaattcaaagtctcctttggtaacaggcatctgaagttcctctttagaaagtgcacggatttcttctggacttaagccattgatacgccgtctcattgccattaaagaggcatccctgcaaacattagtgatgtcagcaccagaatagccctcaatcttctcggctatatcttccagttgaatatcaggatctaattcgacctcacgaaggttgatcttcagaagctcagctcttccttttgctgttgggagaggtatatatatccttttttctaaccttcttcgcaaagcttcatcaatgtcccacgggaaattagtagcagccaataccataaccattttggaaggatcatcattttctaaagctcctccaactccatccatctgaatgagcagttcagacttgaccctgcgacttgcctcatgttcatcagaggttcctcttcgactgcagatagaatctatctcatcaatgaagatcgtggtaggggcataaaatctagccatctcaaacaacagacgaactaacttctcagattcacctctgtatttagatgtcagtgtagaagacgaaacgttgaagaatgttgtaccacattcagtggcaacagctttagctagcatagttttaccagtgcctgggggtccaaccatcagtacacccttccatggccttctaatccctttgaaaaagtcaggcatccacattggaagaacaacagcttcccttagcaacttcttagcttcttccagatctgctatgtcatcccaatgaatgctaggattcctggatacaatgtctctttcaagggcttccaccagatccttatcataaccagcaccatcaaattttggcatttcaccatcacttgcaccatcttgcatattcttccttcccttgtcatctctccctcttgctctatagtccttgtccctacttgtagaaggcttttcactctttgatataggatgtgctcggcctacaggtccccgggctcctactcctgccatttctttcctcagaggtcttacttctcgattgggacgcctgatctgaggtggagctctgtgttctgcaggaacagggggtggccaaacagcaggatctctaaatggttcatcttgacaggacacagggaaatctggaggcttgtcaattttaaaactttctaaagtgctgacaatacttttaacttgttcatattcctccaataattcctgccgaacctgttgccatttgcctttgatagctggatctctgactgactggcaatgtctctgaatctgctgcatcaccccctggtaatataccattgatgagtcgtaatttccaagaagggcatattctcttcctttctttgcattatcacaaatctcagccaaattcatcttctttcagagacatacggttctgcaccgaaaggcagcaacctgcgagggtcagaggcgccgaagacccgaggccctgcagcttgggcggctgctcatccctgagactgtgcagggcggtggccc

SEQ ID NO: 8305 - RNA, 3556 nt, Homo sapiens
  source 1..3556: mol_type = other RNA
aaaaaccacaattacttttgcaccaacccattacaaacaagttttaacaatcacaagactaatgttttagtgacggctcctaaaacttcagggaaaaaaaaagtgcatttctgactggcaatagtttgcaaaataatcgtaatgaaactacttatttctttattttaaaagttaataaaaggaaacctctcaatttttaggaagaattcaattacaataaaatcatgatgtcttatgatctggcatcttataatctgtgtctcagaaagaagggcaatttacagcatcagatgaatactggagtttaggtcagacttaagttatctgaaaagaacataaggcatttacagtttttagcagggaaaaataatcaaatctctttttttaaaaaaaaccttcttagtatcttggttaaatgtccaaaaagctgtattatttttagttttaaaccagtaggcactattcgaaactgagaattcaggatgttatcaaatacaaatttttaaaagcttgaccattaaagcataaattgcctaatgagacacatgtaatcataaaaactaacgccaggatcatttacttgtgattggatatatgccatttatttttctggcttctttctaatgtgtaattcctgctgaattgagtgagcatgtcagatttctatctttatcttagtgtgtgtaaaagttctcaacctagacaaggacaaattttagaattttccaatgaacatcattcactatgtatgatgctgttttgttaaactagctgtttggaaaacaataaagatttcatttgttttgcgttagccacagagagtggacttgtttagaatgtaaaagtatttatctcaaatactaaaatcaaactcaagaaaaatcaaacaatgctggagctgagaaaaataatggctatatatctggttgaacatgttgaaagaaaagtgaaaacacagccaggcatggtggtgcgcacctgtaatcccagctacttgggaggctgagacaggagaattgcttgaatctaggaggcagaggttgcagtgagccaagatcaaccactgcactacacagcctgggtgacacagactccttcacgcacacacaaaaaagtgaaaacaaacttggaagtctagaatgaagaattacatctaatgcagtaatattcttcccacctttccatattaaatgtaagaagcaccagcaaaaaatactaaagacagagaaatgacctggcaaaatgattcaaataccacagagcgtgagaatattcctcagtaaagctcaagatattatgaagtagctagcagaagaaatggcaggggtagcggaagtaaaaattctaaccatatgacagactctaacagtaagtcataaattctaaaggtttaattagtaaattcattatttcctccaaaatatactgtcattcttctcttaacaatgaatgtttgacacaaatccaattttgatgttaaaagtcaacatacatagataggtccctcatgttgacagagcacagaattggaaaaaaaaactgcaaatgagaaataggggtatttctaaatcttctgtattcctaaaatatcacactgcgcccttgcttcagcctccctgatagactggtttgggtgtgcaatattaatgcaggaatacgtggaataccagcacaaagccggggagggagactagcaaactctcgccatcaattatttctcaactacatttagtattcttcgcagttttagatttttttttcctttaagcgaaaaccactccactgaaaaaaattccaaacttgttttttaaaaattgcaggaatttcttcgtattttatcaacaaaaataccagaaattaaagagctgacagaaattcaagcagatccaaattcaaccatccatttttcatacttctccaagtctgcagcagagacagacttagcaattttctttagggccaattcaaagtctcctttggtaacaggcatctgaagttcctctttagaaagtgcacggatttcttctggacttaagccattgatacgccgtctcattgccattaaagaggcatccctgcaaacattagtgatgtcagcaccagaatagccctcaatcttctcggctatatcttccagttgaatatcaggatctaattcgacctcacgaaggttgatcttcagaagctcagctcttccttttgctgttgggagaggtatatatatccttttttctaaccttcttcgcaaagcttcatcaatgtcccacgggaaattagtagcagccaataccataaccattttggaaggatcatcattttctaaagctcctccaactccatccatctgaatgagcagttcagacttgaccctgcgacttgcctcatgttcatcagaggttcctcttcgactgcagatagaatctatctcatcaatgaagatcgtggtaggggcataaaatctagccatctcaaacaacagacgaactaacttctcagattcacctctgtatttagatgtcagtgtagaagacgaaacgttgaagaatgttgtaccacattcagtggcaacagctttagctagcatagttttaccagtgcctgggggtccaaccatcagtacacccttccatggccttctaatccctttgaaaaagtcaggcatccacattggaagaacaacagcttcccttagcaacttcttagcttcttccagatctgctatgtcatcccaatgaatgctaggattcctggatacaatgtctctttcaagggcttccaccagatccttatcataaccagcaccatcaaattttggcatttcaccatcacttgcaccatcttgcatattcttccttcccttgtcatctctccctcttgctctatagtccttgtccctacttgtagaaggcttttcactctttgatataggatgtgctcggcctacaggtccccgggctcctactcctgccatttctttcctcagaggtcttacttctcgattgggacgcctgatctgaggtggagctctgtgttctgcaggaacagggggtggccaaacagcaggatctctaaatggttcatcttgacaggacacagggaaatctggaggcttgtcaattttaaaactttctaaagtgctgacaatacttttaacttgttcatattcctccaataattcctgccgaacctgttgccatttgcctttgatagctggatctctgactgactggcaatgtctctgaatctgctgcatcaccccctggtaatataccattgatgagtcgtaatttccaagaagggcatattctcttcctttctttgcattatcacaaatctcagccaaattcatcttctttcagagacccagaaataaacgtatccaggaaaggagaaaaacctgttaaaacacggtttctcaggtctcacatccaatgtgtgacatacatacggttctgcaccgaaaggcagcaacctgcgagggtcagaggcgccgaagacccgaggccctgcagcttgggcggctgctcatccctgagactgtgcagggcggtggccc

SEQ ID NO: 8306 - RNA, 3584 nt, Homo sapiens
  source 1..3584: mol_type = other RNA
aaaaaccacaattacttttgcaccaacccattacaaacaagttttaacaatcacaagactaatgttttagtgacggctcctaaaacttcagggaaaaaaaaagtgcatttctgactggcaatagtttgcaaaataatcgtaatgaaactacttatttctttattttaaaagttaataaaaggaaacctctcaatttttaggaagaattcaattacaataaaatcatgatgtcttatgatctggcatcttataatctgtgtctcagaaagaagggcaatttacagcatcagatgaatactggagtttaggtcagacttaagttatctgaaaagaacataaggcatttacagtttttagcagggaaaaataatcaaatctctttttttaaaaaaaaccttcttagtatcttggttaaatgtccaaaaagctgtattatttttagttttaaaccagtaggcactattcgaaactgagaattcaggatgttatcaaatacaaatttttaaaagcttgaccattaaagcataaattgcctaatgagacacatgtaatcataaaaactaacgccaggatcatttacttgtgattggatatatgccatttatttttctggcttctttctaatgtgtaattcctgctgaattgagtgagcatgtcagatttctatctttatcttagtgtgtgtaaaagttctcaacctagacaaggacaaattttagaattttccaatgaacatcattcactatgtatgatgctgttttgttaaactagctgtttggaaaacaataaagatttcatttgttttgcgttagccacagagagtggacttgtttagaatgtaaaagtatttatctcaaatactaaaatcaaactcaagaaaaatcaaacaatgctggagctgagaaaaataatggctatatatctggttgaacatgttgaaagaaaagtgaaaacacagccaggcatggtggtgcgcacctgtaatcccagctacttgggaggctgagacaggagaattgcttgaatctaggaggcagaggttgcagtgagccaagatcaaccactgcactacacagcctgggtgacacagactccttcacgcacacacaaaaaagtgaaaacaaacttggaagtctagaatgaagaattacatctaatgcagtaatattcttcccacctttccatattaaatgtaagaagcaccagcaaaaaatactaaagacagagaaatgacctggcaaaatgattcaaataccacagagcgtgagaatattcctcagtaaagctcaagatattatgaagtagctagcagaagaaatggcaggggtagcggaagtaaaaattctaaccatatgacagactctaacagtaagtcataaattctaaaggtttaattagtaaattcattatttcctccaaaatatactgtcattcttctcttaacaatgaatgtttgacacaaatccaattttgatgttaaaagtcaacatacatagataggtccctcatgttgacagagcacagaattggaaaaaaaaactgcaaatgagaaataggggtatttctaaatcttctgtattcctaaaatatcacactgcgcccttgcttcagcctccctgatagactggtttgggtgtgcaatattaatgcaggaatacgtggaataccagcacaaagccggggagggagactagcaaactctcgccatcaattatttctcaactacatttagtattcttcgcagttttagatttttttttcctttaagcgaaaaccactccactgaaaaaaattccaaacttgttttttaaaaattgcaggaatttcttcgtattttatcaacaaaaataccagaaattaaagagctgacagaaattcaagcagatccaaattcaaccatccatttttcatacttctccaagtctgcagcagagacagacttagcaattttctttagggccaattcaaagtctcctttggtaacaggcatctgaagttcctctttagaaagtgcacggatttcttctggacttaagccattgatacgccgtctcattgccattaaagaggcatccctgcaaacattagtgatgtcagcaccagaatagccctcaatcttctcggctatatcttccagttgaatatcaggatctaattcgacctcacgaaggttgatcttcagaagctcagctcttccttttgctgttgggagaggtatatatatccttttttctaaccttcttcgcaaagcttcatcaatgtcccacgggaaattagtagcagccaataccataaccattttggaaggatcatcattttctaaagctcctccaactccatccatctgaatgagcagttcagacttgaccctgcgacttgcctcatgttcatcagaggttcctcttcgactgcagatagaatctatctcatcaatgaagatcgtggtaggggcataaaatctagccatctcaaacaacagacgaactaacttctcagattcacctctgtatttagatgtcagtgtagaagacgaaacgttgaagaatgttgtaccacattcagtggcaacagctttagctagcatagttttaccagtgcctgggggtccaaccatcagtacacccttccatggccttctaatccctttgaaaaagtcaggcatccacattggaagaacaacagcttcccttagcaacttcttagcttcttccagatctgctatgtcatcccaatgaatgctaggattcctggatacaatgtctctttcaagggcttccaccagatccttatcataaccagcaccatcaaattttggcatttcaccatcacttgcaccatcttgcatattcttccttcccttgtcatctctccctcttgctctatagtccttgtccctacttgtagaaggcttttcactctttgatataggatgtgctcggcctacaggtccccgggctcctactcctgccatttctttcctcagaggtcttacttctcgattgggacgcctgatctgaggtggagctctgtgttctgcaggaacagggggtggccaaacagcaggatctctaaatggttcatcttgacaggacacagggaaatctggaggcttgtcaattttaaaactttctaaagtgctgacaatacttttaacttgttcatattcctccaataattcctgccgaacctgttgccatttgcctttgatagctggatctctgactgactggcaatgtctctgaatctgctgcatcaccccctggtaatataccattgatgagtcgtaatttccaagaagggcatattctcttcctttctttgcattatcacaaatctcagccaaattcatcttctttcagagacccagaaggcgcaggtccgggcacattcagcgatgcggtccagatggggtgcgggtggggcgcaggccgccgccgccgccgccgccgagtccgttagctcgcgacgtgcgtgaaaaggcggcggcggcgtagtgttgccatggcagccgcggccgcgcggtgggcgcagcgcgggagggagcgcgggggctgtgagtccgctctggggcggagcttgggact

SEQ ID NO: 8307 - RNA, 3435 nt, Homo sapiens
  source 1..3435: mol_type = other RNA
aaaaaccacaattacttttgcaccaacccattacaaacaagttttaacaatcacaagactaatgttttagtgacggctcctaaaacttcagggaaaaaaaaagtgcatttctgactggcaatagtttgcaaaataatcgtaatgaaactacttatttctttattttaaaagttaataaaaggaaacctctcaatttttaggaagaattcaattacaataaaatcatgatgtcttatgatctggcatcttataatctgtgtctcagaaagaagggcaatttacagcatcagatgaatactggagtttaggtcagacttaagttatctgaaaagaacataaggcatttacagtttttagcagggaaaaataatcaaatctctttttttaaaaaaaaccttcttagtatcttggttaaatgtccaaaaagctgtattatttttagttttaaaccagtaggcactattcgaaactgagaattcaggatgttatcaaatacaaatttttaaaagcttgaccattaaagcataaattgcctaatgagacacatgtaatcataaaaactaacgccaggatcatttacttgtgattggatatatgccatttatttttctggcttctttctaatgtgtaattcctgctgaattgagtgagcatgtcagatttctatctttatcttagtgtgtgtaaaagttctcaacctagacaaggacaaattttagaattttccaatgaacatcattcactatgtatgatgctgttttgttaaactagctgtttggaaaacaataaagatttcatttgttttgcgttagccacagagagtggacttgtttagaatgtaaaagtatttatctcaaatactaaaatcaaactcaagaaaaatcaaacaatgctggagctgagaaaaataatggctatatatctggttgaacatgttgaaagaaaagtgaaaacacagccaggcatggtggtgcgcacctgtaatcccagctacttgggaggctgagacaggagaattgcttgaatctaggaggcagaggttgcagtgagccaagatcaaccactgcactacacagcctgggtgacacagactccttcacgcacacacaaaaaagtgaaaacaaacttggaagtctagaatgaagaattacatctaatgcagtaatattcttcccacctttccatattaaatgtaagaagcaccagcaaaaaatactaaagacagagaaatgacctggcaaaatgattcaaataccacagagcgtgagaatattcctcagtaaagctcaagatattatgaagtagctagcagaagaaatggcaggggtagcggaagtaaaaattctaaccatatgacagactctaacagtaagtcataaattctaaaggtttaattagtaaattcattatttcctccaaaatatactgtcattcttctcttaacaatgaatgtttgacacaaatccaattttgatgttaaaagtcaacatacatagataggtccctcatgttgacagagcacagaattggaaaaaaaaactgcaaatgagaaataggggtatttctaaatcttctgtattcctaaaatatcacactgcgcccttgcttcagcctccctgatagactggtttgggtgtgcaatattaatgcaggaatacgtggaataccagcacaaagccggggagggagactagcaaactctcgccatcaattatttctcaactacatttagtattcttcgcagttttagatttttttttcctttaagcgaaaaccactccactgaaaaaaattccaaacttgttttttaaaaattgcaggaatttcttcgtattttatcaacaaaaataccagaaattaaagagctgacagaaattcaagcagatccaaattcaaccatccatttttcatacttctccaagtctgcagcagagacagacttagcaattttctttagggccaattcaaagtctcctttggtaacaggcatctgaagttcctctttagaaagtgcacggatttcttctggacttaagccattgatacgccgtctcattgccattaaagaggcatccctgcaaacattagtgatgtcagcaccagaatagccctcaatcttctcggctatatcttccagttgaatatcaggatctaattcgacctcacgaaggttgatcttcagaagctcagctcttccttttgctgttgggagaggtatatatatccttttttctaaccttcttcgcaaagcttcatcaatgtcccacgggaaattagtagcagccaataccataaccattttggaaggatcatcattttctaaagctcctccaactccatccatctgaatgagcagttcagacttgaccctgcgacttgcctcatgttcatcagaggttcctcttcgactgcagatagaatctatctcatcaatgaagatcgtggtaggggcataaaatctagccatctcaaacaacagacgaactaacttctcagattcacctctgtatttagatgtcagtgtagaagacgaaacgttgaagaatgttgtaccacattcagtggcaacagctttagctagcatagttttaccagtgcctgggggtccaaccatcagtacacccttccatggccttctaatccctttgaaaaagtcaggcatccacattggaagaacaacagcttcccttagcaacttcttagcttcttccagatctgctatgtcatcccaatgaatgctaggattcctggatacaatgtctctttcaagggcttccaccagatccttatcataaccagcaccatcaaattttggcatttcaccatcacttgcaccatcttgcatattcttccttcccttgtcatctctccctcttgctctatagtccttgtccctacttgtagaaggcttttcactctttgatataggatgtgctcggcctacaggtccccgggctcctactcctgccatttctttcctcagaggtcttacttctcgattgggacgcctgatctgaggtggagctctgtgttctgcaggaacagggggtggccaaacagcaggatctctaaatggttcatcttgacaggacacagggaaatctggaggcttgtcaattttaaaactttctaaagtgctgacaatacttttaacttgttcatattcctccaataattcctgccgaacctgttgccatttgcctttgatagctggatctctgactgactggcaatgtctctgaatctgctgcatcaccccctggtaatataccattgatgagtcgtaatttccaagaagggcatattctcttcctttctttgcattatcacaaatctcagccaaattcatcttctttcagagacctccacttccctttcccaacgcacagagcccaggtccgcgaccactcaacagccccctcaagacaaagagag

SEQ ID NO: 8308 - RNA, 3662 nt, Homo sapiens
  source 1..3662: mol_type = other RNA
aaaaaccacaattacttttgcaccaacccattacaaacaagttttaacaatcacaagactaatgttttagtgacggctcctaaaacttcagggaaaaaaaaagtgcatttctgactggcaatagtttgcaaaataatcgtaatgaaactacttatttctttattttaaaagttaataaaaggaaacctctcaatttttaggaagaattcaattacaataaaatcatgatgtcttatgatctggcatcttataatctgtgtctcagaaagaagggcaatttacagcatcagatgaatactggagtttaggtcagacttaagttatctgaaaagaacataaggcatttacagtttttagcagggaaaaataatcaaatctctttttttaaaaaaaaccttcttagtatcttggttaaatgtccaaaaagctgtattatttttagttttaaaccagtaggcactattcgaaactgagaattcaggatgttatcaaatacaaatttttaaaagcttgaccattaaagcataaattgcctaatgagacacatgtaatcataaaaactaacgccaggatcatttacttgtgattggatatatgccatttatttttctggcttctttctaatgtgtaattcctgctgaattgagtgagcatgtcagatttctatctttatcttagtgtgtgtaaaagttctcaacctagacaaggacaaattttagaattttccaatgaacatcattcactatgtatgatgctgttttgttaaactagctgtttggaaaacaataaagatttcatttgttttgcgttagccacagagagtggacttgtttagaatgtaaaagtatttatctcaaatactaaaatcaaactcaagaaaaatcaaacaatgctggagctgagaaaaataatggctatatatctggttgaacatgttgaaagaaaagtgaaaacacagccaggcatggtggtgcgcacctgtaatcccagctacttgggaggctgagacaggagaattgcttgaatctaggaggcagaggttgcagtgagccaagatcaaccactgcactacacagcctgggtgacacagactccttcacgcacacacaaaaaagtgaaaacaaacttggaagtctagaatgaagaattacatctaatgcagtaatattcttcccacctttccatattaaatgtaagaagcaccagcaaaaaatactaaagacagagaaatgacctggcaaaatgattcaaataccacagagcgtgagaatattcctcagtaaagctcaagatattatgaagtagctagcagaagaaatggcaggggtagcggaagtaaaaattctaaccatatgacagactctaacagtaagtcataaattctaaaggtttaattagtaaattcattatttcctccaaaatatactgtcattcttctcttaacaatgaatgtttgacacaaatccaattttgatgttaaaagtcaacatacatagataggtccctcatgttgacagagcacagaattggaaaaaaaaactgcaaatgagaaataggggtatttctaaatcttctgtattcctaaaatatcacactgcgcccttgcttcagcctccctgatagactggtttgggtgtgcaatattaatgcaggaatacgtggaataccagcacaaagccggggagggagactagcaaactctcgccatcaattatttctcaactacatttagtattcttcgcagttttagatttttttttcctttaagcgaaaaccactccactgaaaaaaattccaaacttgttttttaaaaattgcaggaatttcttcgtattttatcaacaaaaataccagaaattaaagagctgacagaaattcaagcagatccaaattcaaccatccatttttcatacttctccaagtctgcagcagagacagacttagcaattttctttagggccaattcaaagtctcctttggtaacaggcatctgaagttcctctttagaaagtgcacggatttcttctggacttaagccattgatacgccgtctcattgccattaaagaggcatccctgcaaacattagtgatgtcagcaccagaatagccctcaatcttctcggctatatcttccagttgaatatcaggatctaattcgacctcacgaaggttgatcttcagaagctcagctcttccttttgctgttgggagaggtatatatatccttttttctaaccttcttcgcaaagcttcatcaatgtcccacgggaaattagtagcagccaataccataaccattttggaaggatcatcattttctaaagctcctccaactccatccatctgaatgagcagttcagacttgaccctgcgacttgcctcatgttcatcagaggttcctcttcgactgcagatagaatctatctcatcaatgaagatcgtggtaggggcataaaatctagccatctcaaacaacagacgaactaacttctcagattcacctctgtatttagatgtcagtgtagaagacgaaacgttgaagaatgttgtaccacattcagtggcaacagctttagctagcatagttttaccagtgcctgggggtccaaccatcagtacacccttccatggccttctaatccctttgaaaaagtcaggcatccacattggaagaacaacagcttcccttagcaacttcttagcttcttccagatctgctatgtcatcccaatgaatgctaggattcctggatacaatgtctctttcaagggcttccaccagatccttatcataaccagcaccatcaaattttggcatttcaccatcacttgcaccatcttgcatattcttccttcccttgtcatctctccctcttgctctatagtccttgtccctacttgtagaaggcttttcactctttgatataggatgtgctcggcctacaggtccccgggctcctactcctgccatttctttcctcagaggtcttacttctcgattgggacgcctgatctgaggtggagctctgtgttctgcaggaacagggggtggccaaacagcaggatctctaaatggttcatcttgacaggacacagggaaatctggaggcttgtcaattttaaaactttctaaagtgctgacaatacttttaacttgttcatattcctccaataattcctgccgaacctgttgccatttgcctttgatagctggatctctgactgactggcaatgtctctgaatctgctgcatcaccccctggtaatataccattgatgagtcgtaatttccaagaagggcatattctcttcctttctttgcattatcacaaatctcagccaaattcatcttctttcagagacctgttaaaacacggtttctcaggtctcacatccaatgtgtgacatacatacggttctgcaccgaaaggcagcaacctgcgagggtcagaggcgccgaagacccgaggccctgcagcttgggcggctgctcatccctgagactgtgcagggcggtggcccagccggggtggggctgagcgctgcaactggggcgggcccagctacagggcgggaagcccgaggctcacctccacttccctttcccaacgcacagagcccaggtccgcgaccactcaacagccccctcaagacaaagagag

SEQ ID NO: 8309 - RNA, 3694 nt, Homo sapiens
  source 1..3694: mol_type = other RNA
aaaaaccacaattacttttgcaccaacccattacaaacaagttttaacaatcacaagactaatgttttagtgacggctcctaaaacttcagggaaaaaaaaagtgcatttctgactggcaatagtttgcaaaataatcgtaatgaaactacttatttctttattttaaaagttaataaaaggaaacctctcaatttttaggaagaattcaattacaataaaatcatgatgtcttatgatctggcatcttataatctgtgtctcagaaagaagggcaatttacagcatcagatgaatactggagtttaggtcagacttaagttatctgaaaagaacataaggcatttacagtttttagcagggaaaaataatcaaatctctttttttaaaaaaaaccttcttagtatcttggttaaatgtccaaaaagctgtattatttttagttttaaaccagtaggcactattcgaaactgagaattcaggatgttatcaaatacaaatttttaaaagcttgaccattaaagcataaattgcctaatgagacacatgtaatcataaaaactaacgccaggatcatttacttgtgattggatatatgccatttatttttctggcttctttctaatgtgtaattcctgctgaattgagtgagcatgtcagatttctatctttatcttagtgtgtgtaaaagttctcaacctagacaaggacaaattttagaattttccaatgaacatcattcactatgtatgatgctgttttgttaaactagctgtttggaaaacaataaagatttcatttgttttgcgttagccacagagagtggacttgtttagaatgtaaaagtatttatctcaaatactaaaatcaaactcaagaaaaatcaaacaatgctggagctgagaaaaataatggctatatatctggttgaacatgttgaaagaaaagtgaaaacacagccaggcatggtggtgcgcacctgtaatcccagctacttgggaggctgagacaggagaattgcttgaatctaggaggcagaggttgcagtgagccaagatcaaccactgcactacacagcctgggtgacacagactccttcacgcacacacaaaaaagtgaaaacaaacttggaagtctagaatgaagaattacatctaatgcagtaatattcttcccacctttccatattaaatgtaagaagcaccagcaaaaaatactaaagacagagaaatgacctggcaaaatgattcaaataccacagagcgtgagaatattcctcagtaaagctcaagatattatgaagtagctagcagaagaaatggcaggggtagcggaagtaaaaattctaaccatatgacagactctaacagtaagtcataaattctaaaggtttaattagtaaattcattatttcctccaaaatatactgtcattcttctcttaacaatgaatgtttgacacaaatccaattttgatgttaaaagtcaacatacatagataggtccctcatgttgacagagcacagaattggaaaaaaaaactgcaaatgagaaataggggtatttctaaatcttctgtattcctaaaatatcacactgcgcccttgcttcagcctccctgatagactggtttgggtgtgcaatattaatgcaggaatacgtggaataccagcacaaagccggggagggagactagcaaactctcgccatcaattatttctcaactacatttagtattcttcgcagttttagatttttttttcctttaagcgaaaaccactccactgaaaaaaattccaaacttgttttttaaaaattgcaggaatttcttcgtattttatcaacaaaaataccagaaattaaagagctgacagaaattcaagcagatccaaattcaaccatccatttttcatacttctccaagtctgcagcagagacagacttagcaattttctttagggccaattcaaagtctcctttggtaacaggcatctgaagttcctctttagaaagtgcacggatttcttctggacttaagccattgatacgccgtctcattgccattaaagaggcatccctgcaaacattagtgatgtcagcaccagaatagccctcaatcttctcggctatatcttccagttgaatatcaggatctaattcgacctcacgaaggttgatcttcagaagctcagctcttccttttgctgttgggagaggtatatatatccttttttctaaccttcttcgcaaagcttcatcaatgtcccacgggaaattagtagcagccaataccataaccattttggaaggatcatcattttctaaagctcctccaactccatccatctgaatgagcagttcagacttgaccctgcgacttgcctcatgttcatcagaggttcctcttcgactgcagatagaatctatctcatcaatgaagatcgtggtaggggcataaaatctagccatctcaaacaacagacgaactaacttctcagattcacctctgtatttagatgtcagtgtagaagacgaaacgttgaagaatgttgtaccacattcagtggcaacagctttagctagcatagttttaccagtgcctgggggtccaaccatcagtacacccttccatggccttctaatccctttgaaaaagtcaggcatccacattggaagaacaacagcttcccttagcaacttcttagcttcttccagatctgctatgtcatcccaatgaatgctaggattcctggatacaatgtctctttcaagggcttccaccagatccttatcataaccagcaccatcaaattttggcatttcaccatcacttgcaccatcttgcatattcttccttcctgaaaaacagcattttaagcttggatctaacctgaagcctgtcagtaattttaaaaaagaaaaagaaaaaagacataatcagtctcagaaaataaactcgtattattataagaagacagtaagcattttcaaataagagtctgtatagcataatgattaaaaaactcaggtattacacatagacaaggttcaaatcctagttcaccatctatttgcagttaagacttcagtgtctcaatttctctacacataaaacaggaaaaataatgctgagctcacaggattatgcagggatcaaataaaccaataaatgtaaaaagcttcaaagcgggctttttttgtagaaagcttcaaaaaggataagtgcgctcaaggaagactaacatttgctactactgctattattagttgttccatcatacagttcccaacaccaaattaaaaatccaaaaatataccagggaccttaagcaagatatgtctaacttctcttatcctcaattttttttacatctataaagttaagtacatagttagagtgctgcagcagctttcaaaattctgacccaggcacaaagtaataaatgcattctggatcatgagctggtgtacataaacatatgaataaatttgtatatatttttatcaaaataatactgtacttatgggcaataaactgagttttctgttctactctgcttcaattttaaagctggcagcaatacacaaaactgatcttaagaaaaacaaatacaataaacactggggactcccatatctctgagggtacttccaaacaacactaattttcctttcttttttttttttttgagacca

SEQ ID NO: 8310 - RNA, 29 nt, Homo sapiens
  source 1..29: mol_type = other RNA
aaaaaccacaattacttttgcaccaacct

SEQ ID NO: 8311 - RNA, 217 nt, Homo sapiens
  source 1..217: mol_type = other RNA
aaaaaccacaattacttttgcaccaacctaaaatataataaaaaagtgtcttctctttataacttttctgttgttttgcttaagttatcattgctattcctctgcaacctaaaaagaaatcattgaatatacatttaattttagaataatcactacacaaatgccctaaaagtgtatgtataacatccctgatgtctgcatttgtcctttgactggt

SEQ ID NO: 8312 - RNA, 43 nt, Homo sapiens
  source 1..43: mol_type = other RNA
aaaaaccacaattacttttgcaccaacctaaatcttccctctc

SEQ ID NO: 8313 - RNA, 34 nt, Homo sapiens
  source 1..34: mol_type = other RNA
aaaaaccacaattacttttgcaccaacctaacag

SEQ ID NO: 8314 - RNA, 32 nt, Homo sapiens
  source 1..32: mol_type = other RNA
aaaaaccacaattacttttgcaccaacctaat

SEQ ID NO: 8315 - RNA, 4502 nt, Homo sapiens
  source 1..4502: mol_type = other RNA
aaaaaccacaattacttttgcaccaacctaataaaactagtgctaaattttacaacctagaagcaaaggttttccacagagagcccttgagtagaacgtgagaggaaagtgttacctggcaagccctgtagaaaaatctgtctattaatggccaatcctttaaagcaatgtgccccttgaactattaatttgatgatcaatataattttggatacagtttacaatgtttgaactgtccttcatctttatttttaaaaaatgtggcatgttgataattgtttgtgatttttaccaggcagtagtttttctgccacttacttccatgctacttcagccatggcagaactgccttggcttactatggaggaagggtcaaagtatcagaaaagtgagaatatgagagtggttttgttgctttaggccagagaagccagtgcatgggagggcctagaggatatggcctttactagggtgctaaggtgcactggtgggaggggcactgatagcactgagccacctccatggtggtttcctctgtattccggggccgacagtaggagatgctgctatggaactgagctgcctcctttcaacaggaaagttgggttccagaatggcaggcactacatggggcacttggatagatggaaggtagacacgattactctactggatagtaaggctagacaggcccttcaggtgtcttaccctgcagggatctgtggtgataatgagctgtgttctgagagataagatagagagccagtgggaatactacttggcttgtacaacatcaagaaaatgtccaagactgatgagtgaaactgaaacagttttccacttagggtggaaaatcatagtcctctaccaagtttcccgatctgagttggttcgcagacccagaacccgtttgttttaagagagaccacatcccttgtttaagagtcttgtactgccaccagaagtaaatattccccccgaagggagctactggcatttgacatggtcctgcacacaaagaagaaaacaaaaattttacccaaatcttaccttccggaaacgactgctgttaatcttaggtgagcattattccagaaatttcatgttgagaagttcggactgggtccgcttggccagtgatctccagtttgtggtttatactgtctgtgctgccatctgcaatgcctctaccattcctccactttaatattccacttgttacacttattatcccacttagtaattatttagagcagtgttctcccaagtggggttcaaaaactaaaatgaagttgttggaagccttggctccttctggaggttccaggggaaaaaagtatgtttccttgactttccagcctctacaggcccacagcattcctgcttgcagccctatgtcatgtcacctgtcctcttggtgctgtcattgtcacaatgccttctttctgaccctgtcattcctggcctcgctgtgatatggaccctcatgattacgattaccttgggcctacaacataattcaggggaatttcccatctcaaaatcattgatttaatcatatttgctgagtcccttttcacatataaggtaacattttgggaaagggatgcattattcagtttacgcagatgggatagtgatttgttgtgtaaatggagtttcttttctgtccctcctcccaatatatctctccctgagtgggaatttagagtgagttctggttttgggggaatagatgtgttagaattcaggccccttaagggctggaatgaagagaggctttattctggggttgtagaagccatactagaagctgtgggttttcccagattgttcattccattttttttttttttagggaagagccttctgtttttcacctggactgcctacaatctgtaggttggggtgggtccaacccctctgtatgcaggcttttgggggctcgtccttattttcacttctcactgttttctccatctttatagtaccagagcccagagcctcttgagaatgtgtgatagctaaatgggctcctagatctgctgaagcctccccactagttccggctttcacagcatgttccattcctcaacacctcgatattgtcctattttctctcctccaaaagtggtggaaagctgttcttaactgatgagtgtcccccaaacacgcctgtcccattttttgtctttatggttggctttgttttgtacatatatcattttgttttactcaaggtcgcttagcagttcactaaattggttaaaggtcactaaaagcagacttttaaaaaatgtgtatatttgcttcatcattttttcagcttcattgggggtataattgacaaatagctttatatgtttaagatgcataatttgatgttttagcatacatatacattgtggaataatcaccacaatcaagctaattgacacatccgacatctcacagtttcccttcttccctccctcccttccttccttccttctttttttgcaatgagaacaggtaagatctaccctcataacaaatttcaagtatacaaaacagtattgttaattatagtcacattggtatatattagatctccagaacttattcatcttgtgtaattgaaacagtatcatttgaccaacacttcccaatgctccctggaatgaggagttgcctattctgttctctgtttctatcagttttactattttagagtccacatataagtggcatcatatagtatttgtctgtctgtgtctggcttttttcacttggcgtaatatcctccaggttcatccatttttgtcacaaatatgaagaaatttaagggtgaataatattccattgtgtatatgtgtacatctcatatcacatcacataatttcatgcctactaatttttaaactaatggccatagaaatcgactggaatgaaggataactagatatattcatagaaatcagcctaccattttcctttgcagttttacatagtgtttttttacatagtgttcttacatagggtttttacatagtgttacatagtgttacaaagaaccttattaagagcttcagtttgcatggtattgtcttagttttgggttattctagaaatagagtccctgagaccatttatggcaaattgtaggagtctgaagtgagggaatgaggagagtgagacagaaaagggagaacaacaaataaagggtgcctccttgagcaagctactactttaagagtaagggagactccattccactgaggacccctgggtaatcttttagaatgtacacagagttgtcccaccaaagaaagggagtctacagcacttaaccctggacttccagctctttgtgtttgagggtgctcccaaagggcatctgcccctgcatttcctggccacacttgttcttcctgcatggccctgcacttcctgcctcttcctgtacttcctggtcacacctgcacttgggcttagcaggcttccctgggtttggagaaagcccaaggtgggaaaactggattagatttgaattgcagctggactgcaatcagacagagggctgggccgcaatcaggcagtaaaccccttaccaagccgactctagccacacacacgtgcagagcttctcatctgcattttactgccttgaataggaacagataatcgcagattatctgaagtttaaggctggcctgagaggcatgagaaagactaaacaaacagatgatcacagagaaaaaacaagaacctcaggatacaaaaaagaagatttaaggaaagcaaaactgaaatatcgaaaatgatataatattcataaaagaagaacaggctgctctgaaaatgtaacaatcaaaataagaaggggctcttagaaattaaatttttttaaaggccagccaaaattgatatcaagaatatttttcacaaaacagaacaacaagcagagacaaaaatagagtgtaaaaatatatttcaaaaatctaagacattgatgattaatccaagatgttcaagaaacagaaaatgtagtggaggaattagctacataataatgatagtgaagtcaatgaagttacagggccgaagggtataggtctataggttgaaaaggttaataagtaccagcatcacaaaagaaaaggtccatgtctccacatatcattgctacatttcagaacagaaggaataaaagagagatcccaaaaactcccagaggaaaatcaggtcctctatgtaggaacaagatagattggcatcagatttcaaataataaatggtaaaagagaaaaatgcctttattagaactatgaaaaggaaaaattacaagtcagacttctatacataagccaatattcaatattgtatagaaatctcaggttggataagacgttacaagcatgcaaggatttggaaagtttattttctgcatttctttggaggttgtatggatgttcttaaataaaatggaggaataaatatgaaagagaaatacagaagattcg

SEQ ID NO: 8316 - RNA, 2490 nt, Homo sapiens
  source 1..2490: mol_type = other RNA
aaaaaccacaattacttttgcaccaacctaataaaatatgtcttgttactagatatgagagtgcatatttcaatttaagataagttttgagtaaggatagaaactgcttcttttctaaataatacaaagaatcaaattaatgttgatctttctgtgaggacaaaatgcatcaacaactgaaacttttaatttaacaataatacaattgaaagaacatgagatcttaagttctatgatctgaacttgagtatcagattctagtatttactagtctgttatcttaggctagttacctaacctttacaaagcttgatttattcatgttatgtggaggtgatgactaatatatctctcataaatacattcagacatatatcagatatatctctcagatatattcatgtcctttaatactcagaagcaaatattttctacactgcgaactactacgagatactactgctcctactattactaacaataatacacaagattataaatactgtcaaattattttaacactgtcattcatcattctcttgtaatggaaacaaatgaaggctaggaaagctttgtagggtcttaattttttctcttgcaggtgaaaaaaactgagtcaaataggcatggcaggcaattttgtggcagaaaatctgtctcctaggagtacaaaaggtttagggggagttggggaggaaaacctgtccctgaggttctccctccctactgctgatatgaaacatcaaaatgtcttttagtcctaataactctgtttctcttaaagaaaaaaataaccaaggctagtcactgaaatgtcctataacttattctctcagtcttttatagccttcgaaagagacatagataaatatcatatttgatgaacactgggtatgaaatttaagaaacatttaaattgaaaaagaaccctttcttcaaagctctagaagctcaggactctctgcatttgacatgcctccatgatcccctggaacacagtttgaaaaccactagtctcagagagccttgcagggcattaggtatttcagattaaggctgaaattatgatctattaaagaacagaaccaatatagagatatcagtgggacctgcagatgagggagagtaatacatcaccaatgtcatacttttcctagtaattttcacaaatctctgcttcaaaatagaggcttttatcacctgtaaaacgaaacgtatagctgtattttccagggctaacagccatgcacacctgtcatcactttttagaagtgtcaagggagtcttataaagtgctgggtttcttttaaattatcaaaatgatttcaagtcttagtgacacacatttggttggcatctagaagtgatttcccaggtaactaaatactactccttttctcaaacaaaaacatcacctgataaatttcctagagagatatccatagctgcacacacacacacacacacacacacacacacacacacacacacaccccactggctgccaggaagctcaaagctaaaatttgtgttcaaatgcaccaatttccttagcccagttttctgtcacaattattttctttcgttacataaatcctattaacttttctttcttcaaaatcttattacatacagtttttaaattttaaagtcacatgcttttaaatgtttttccccagtgatttatctttattttaataattgccatgtatgcatttgtttttcagaagtggcaagatgcccaggtacaatggctcatgcttgtgggggttgaggcaggtggactgcttgagcccaggagttcaagaccatcctgggcaacatcatgaagccccatctctactaaaaatacaaaaattagccaggcataatggcacagcacttgtagtcccagctactcaggaggatgaggtaggaggatcgatgcccaggaggtcgaggctgcagcgatccgacatcatgccactctgtactcttgcctgggcgaccgaaaccccatctacagttgggaggagggtccaatgtgatttctgcaagttccttctgaattcttttagcactagttgacaatttagcagcggttttgctggatatttttccctcctttttcttgggctgaacttgttctctttctggttcttgctgaacactttcacgttgatctccatcggaacttcctccactagtgcttggactgtcatcaactctttgtgcctcagtggacattttagatccctcagcgccgccgctgccgccgcccccggccgttccagctccggctcctgaggctgctgcccgcggctgtcgctgtggctgcccctgagtcctggaaagtgaagccaccacctccgggagccgccgccgcccggccgtccgcgcgcgcacccgcgagtgcgcgtgcctgcgcgcccgcccgggagagaccgcgagagcgcgagccccacgtcggccatgcggcgccgcgcgcctccctcctccccccgcccctcc

SEQ ID NO: 8317 - RNA, 1408 nt, Homo sapiens
  source 1..1408: mol_type = other RNA
aaaaaccacaattacttttgcaccaacctaataataacaggagttatttgtagaattgacggattttagaagggtaaaaggaaaaaggaaagctaagaaatgtgaaataaagaaaaaagcagacaacttagttacacgccaagtccttaactgagcgagaagagaaataaattctggaatctgtctattaataattcttcctcacccacaagataaaaacagtagcttccaatctgagacacactcatgcaacttcctctgtgacagagtgctctgaacactatgtgagtgggaccatagtgttctcagtattgcactttctacggtaaatttggctaagaaacacttttgttcttttcctgtaagtcaaaagaaagtcctcctaaactaactaaaatctaaaatttgtctgactctaggagattttttttctccagacaaattcaaattaaatgataacatctcttaaggatttctcaccagtatcagataaaaatacattgaatccaagctatttgaatggacaatactcagttgcacatacacaccatcaactgcagggggcgccaatgccttttccctcaggcccttcagaaaaggcggtgcagctggaattttaatttcttcctgtctgttaagtgtgattattgatgaagtactgcgctcatcccagtacccaaattgaagcttctcgaacatatacgaaatggaactgggccttacaacaaaggcaaatctagttcccatgtttaaaatagtctccggggtccatttggagtgaggagtaaggaagggaagggacttatgcaggtctttccatgcggccttgatttagtccacggagtccaaagcccattctgaggcagggtctctaggttcttggtttacacctatatacaggcgagcgcgcccccgggccgcggaccgcgcgcacagcccgcactgccccacgccgcgggctagggacacccggcccgccaccatgacttccagcaagatagagatgcccggcgaggtgaaggccgaccccgccgccctcatggcgtcgctgcacctcctgccgtcgcccacgcccaatctcgaaattaagtacaccaaggtaagcggccgcccagcgcccgtcgtccacggagactttctagaaccttcttcggtttccccgatctcttcagcgggtgagggctgcgggacggggccggggtcgtcggggccagcctgtcatcccggcgcagcagagggaccccctgcctgtcttcgggactggggcgtttgaagccccgccgtggtctgaggacgccttggggacttaacccaacccgaagcgcagcgttgaggggcagccgtcaacggctcctgccccggactctgaggctggtttctgtccgattctcccggtcccgactgccgc

SEQ ID NO: 8318 - RNA, 4732 nt, Homo sapiens
  source 1..4732: mol_type = other RNA
aaaaaccacaattacttttgcaccaacctaataattttaataatatatataacatttaattacagtgtagaactatcaatgttttcgcagtgtaatttgctgtaatatctattaaatcccatagacttgcagtctataaacatgtatacactctaagtaaaatattaaatgaaattaaattagctactcaattttcctcctacacataatcttctgtacatgccttcattatttgtatagtgttgtgacttccgaaaatatcaggcacattcatattaaaatattagatacaaaatgcattctaaactcaagtaatacttttgagtttatctgagcactgttgctaagttctaatatggagataaatatatacttacacaaaatattttcatatttaggaatatcataaatgaatcccttgatgacaggcttttcttaataataaaaagatacccatggcagaattcgaaagtaattacttgtattataattttttttttgagactcttgtcacccaggctggtgtgcaatggcgcaatctcagctcattgcaacctctgcctcccaggttcaagtgattctcctgcctcagcctcccaagtagctgagactacaggcgcgtgccaccacacccagctaatttttgtatttttagtacagacggtgtttcaccatgttggccaggctagtctcgaactcttggcctcaagtgatccgcctgccaaggcctccgaaactgttggcacttgaggcactgcgctgagccttgtattataatttttttaagttataagtcttgtaagcacctgcagcgttgattgatgaagagagagatgcattgttaaacaagatgccctcaggctttcctttaaggaataaagattaataggacactcagaaaagtaaacacataatgtaagtgtgaataaagtggtgtaattcagattctatgggaactcagaggacagacactcaaatgtctgatgaatgaaggcttgtgtccattttaatttatatattcagcagatcgatcacttttgaatacaatactcctcgatgaaaaagtatagtctgaagtaaccttaagattgtatgtattatttttcacaaatgcaaagttgaaatgattattcccagagggtgagcagggccacagaaaagaataaaacaggaaatttctaaaactgcattgagatacttgtttcttggagacttggtacccgttccaatgcttagcatttatcaagttattatggtttgccagaaaatgtgctcaaaggactctttaccctttaaccctcctaaccctattaatgtagtactagtattatgttcatcttttacatgtggaaacggggacccacagaggttatagaacctacctcaaattagaaagctggaaggcaagcttttaacaactgtgagtaaatcttcttttacagtgtgagaaaaatcctaaaacagagggaaagggagacagggtggcaaggggagaggtatttggtggagcgtagaataacacaacgtcaaattctcttttattttttttagatgggtgtcactctgttgcccagtctggagtgcagtggcatgatcatagctcactgtagccttgacctcctgggctcaagcaatcttcctgccccagcctcctaagtagctgggactatagttgcagatcaccatgcccagctaatttttgtattttttgtagaggtagaatctctccatgttgcccaggctggtctcagactcctggactccagtgatctacctgcctcaacctcccaaagtgctgggattacacgtgtgagccaccacagccggccatatgtcaaattcttaagcttcattcttaagccatatgtctcattcttaatgatttgttatcacagatcattgaagaaactggctacataaatcattactcttgcattatcagcctctcacaaatctctctagcatctgaaaattactatcaaatgaacagtgctgactgttcagagtgtcccaacagggtgaaagcaagttgcatgactctgtatctaattattttataacatcaatatatccatgatatagtatcacataagacactgatacattggctattatatttgtaagccgaacttttaattttaaacagggcttgtactttgattatttatcaaagtatcaaattccacaaataaaatattcttttactttgaaatctctgtcttcactttatggctttttattatgaaactttatcttggtattactgatgtaccttgacttcattatactaaacaacactcatattagtacttcagtactggcaatacagctaagccttaaactgagccaaatatctgttaaagtgaattgctttttatgctgaaatcaatttattgaataaaagtcccttgccacaatggaataaagaatataattccacctttgaaggaacccctaaaactacaattttcaaatttttaaaaagtataatccagccgggcgtggtggctcacacctgtaatcccagcactttggaaggccgaggtgggcagatcacctgaggtcaggagtttgagaccagcctggccaacatggtgaaacctcgtctctactaaaaatacaaaaattagccagcgtggtggcaggtgcctgtattcccagctacttgggaggctgaggcaggagaatcgcttgaacccgggagatacaggttgcagtgagctgagaacgcgccatcgcactccagcctaggggacaagagcgagacatcgtctcaaaaaaaaaaaaaaaagtataacctaaaaattattcaataatttcaagtgtgttttttaaaactaaatttaatcaatcaattcatataatgctatctatataaaagataaaaatcttattcttgggctaacttgatggaaaaggttcttagttttttaaagggctccgttgaagagtattcttagaaaaagcgtggtatacatcagtggtccccaacctttttggcaccagggactagttttgtggaagacaatttttccacagccagggttgggggtggggttgggttctgggatgaaactgtcccacctcagatcatcaggtattagattttcttaaagagcgaaagctagatcccttgcatacgcagttcacaatagggtttgggctcctatgaggatctaatgctgctgctgatctgacaggaggcggaatgcaggcgggaacgctcagtttgaggttcaccacgtgctgtgcggtctgcttgctaacagatcacggaccagtactgggaccatggtccaggggttggggacctcagtatacataactaactaaaattagctgctaacattttctagaaatacctgagagccaacttataagaatattactttacttaaatttagcaccatttgtatatgtaaaaaaaaaaactgatatgctagagttagtaaaaatggcttattctctacaatctagtcatttcctttatagtgcaaacacctacgccccaagaaaaaaagaaggattacaaatgtgcacacaggtatcacaaagaggccttactagatcccatttcctttttaaaatggagacatttcaaaggcagaaaaaatcctgattctggttaggtaattgaagtaaatgtaagagagagtcacgaggatatttttacacaggcccagtacgggtgtgatagtccccagggcaatgattaaaccaagtctaacaaaaacgaatggtaaatcttgcagcaggacgctcagggaattgagaagagggttttggggagtgaatgtaattcgaaggagagaaataaaactgaatatgtagactgggtatagccagcttgacttgtacacgttggggtgaccagccacacgcaccatttctatcgtgtcagaccacaggagaaagctccataagaataactctgcccggacatctcgccgggacatcattctcaggattccggagtcacaggagggctcctggggtcccatgaacacagactcctggctccgtgtcatggctcctgatggctgcgacacctgggtgctgttggttgcctggggagatgcagcgttttctggactttgcctcacttgctccgtcacagtttttatgtgttgcaaagaggttgaatggatgtgtccattttcactactcttttgactccctctaagaggatatatcctgagtttttcaataatatcaaccatgatcagggataacagaaccagagatacgggcaggtcaggtaacatatcaggtaagacatcagcggacccattaatgctcttttgaacctcagtcactgctatggaaaaggtgaggcagggcagtgtggtgaggaccacacacatcatcagaacaggtctccatcctttaatttttctgtaaatataacgtttcttgtgcaggataacttttacaggaacccagatcagtagagtcactaacgcaacataggcaatagaacaggagatgatcagccagtagtgtgtgttgtcagatctagcccttgttccttggtaggcggtggcaaactgttctgtgatcacgagtgtggggatggagaaagcggcaaactctaggagctcaaaaaccacgaacttaatgagccttccagaagccatcctgaggaaaagcaagctgccaagaacctgggactccctctttgactgtgggcagcatatggacccacagacactgaactgggatcaagttcctt

SEQ ID NO: 8319 - RNA, 34 nt, Homo sapiens
  source 1..34: mol_type = other RNA
aaaaaccacaattacttttgcaccaacctaatac

SEQ ID NO: 8320 - RNA, 1453 nt, Homo sapiens
  source 1..1453: mol_type = other RNA
aaaaaccacaattacttttgcaccaacctaatacataaacttatttttctatttctctaagaggaaaagtaaatatatgcatacaaagaaaagagatctagagacaccaaggtttaacagttaacagatctgattcataggattacaaaatctgttggtgaaggtctttttaaatggggacgatttagggggcataactccatgtatgttctaatttttcttagcatattgaatctgtaataagttggggggtgggggtgttgttttaatttcaaacctaagagtcacatgcaaaagaaggccagggaatcacagtttgacagcacaatccttgagactggagcagtggttctcaaaggcattcctagcaacagaactcttgcaaagaaactgaaaccaggtcccccgaaatctgggggtacagtctgcagcaaactcaaaatttcttaggagtctcccaattgatcttaaaaattaaagcaaatactgcattctactaaataatctgtctttgtcctatcataaaaatgtattatattatttaccagttaaattatttaacattttccccaaagcctttgtgttgattttgcagacaaagaagatgctctatgtgttccccacccactacaactactcgtttgagaagcacagcgccagggtgcttagatgtttcaagaatacatactggcttaatccaccaccaagttcttactgaaaaccttaacttgtgtgtcccgaatttatgaaagattactgtgaaaacaccagtgaaataaagtcacctgttttgtaaacatatatgcatataaaatatatgtaaataaaatgatcttagtaagttcctcaaagtcatgctgtaactctccccactcaaagatagttttaaataacgattaagcaaataaatcctgtttggtactagttattttttttaagtaccaaatgcttttccctaatctgaaaccctaattcagtaacgaatggatatgcctctatctttggctaaaacatttaacagggcttagttagttcaattctacaaatacttcttaatcatatactctgcacaaggtaatgtgtaagtgctttaagacatttcatcctttatttaattggaatatgaaggctattttattacaaacatgttttcacacttttaaaacgtcaaagcttatttcttgctgttttgttttttcacaattaaaatggatctcatagagtccctcatttcagtttacaaggctaaggctctaacaaggcaactaaagaaacttaaggtcccaagctagaagcaaagacagtctctgagacgcccatctccttaatgtcctgtcagagctctctgtaccatgtcttacatgagaccatacatcttatcagtgtaccttttaacactattggaaacacatttctatttatccataaaataaaccaactgcacttttttttt

SEQ ID NO: 8321 - RNA, 4940 nt, Homo sapiens
  source 1..4940: mol_type = other RNA
aaaaaccacaattacttttgcaccaacctaatacatataaaatatgttacaatcgaacagtatccacgcatctcactctgcagatgaggtaactagggccagggaatacaaactagttgtaattacactaggttgcctgagtcctgttccagctcccattcactcattcagcaaataattatgaactcccattttctgtctactattttcaaagttaaaattattgacgattctgtaatgggtaattgctggtcatgggttgatagtctggattgacctttcaaatttaaagaaaacactgtacagaactacattcagtatcatattcagcatgctgagtaattttgtttgggttgattaggtttaatattttagaataaaagagatttctaatgaagcttacattaagtaaaccctccctaggtcaaattttattaagtttatgttaattatgacctttattggaataccaccttattcttaaaataattattttttaaaagcatgagaaaacggtttccagcaactttttaatatgaaaagtctccattaatgaaacttatctctttctagatctttttgagaaaatatgtttcttagaacaaagattaacttaagtagtgacaattaataaactagatgttaaaagtggtggccagaggccttagaaatgtaaagaaaacagtagaaaagcttgtataccaaagaaattaggaagctgcattgctcacagaggcaacagctggataggaatccaaagggaaagaggcttggtcctattattggctactattgatctaatgacttaatatttgcttggaaatcgatgtctgggactgaccattgatcttttcacttcacagtgtattcttgagagtaatatatggttcttaatcatctgagtattcataatatctggctctgcattaataaatacacaatttaatgaatgaataaatgaatggatggacaataatatgaaaatgcatagttttttttcttataggagcagttaaattttgagtcagcttccattatgtacatactcaacctgaatagtagtttcagtaacacgttaaaagtaaatgttggccagacgcagtggctcatgcctgtaatcccagcactttgggaggccaaagtgattattgtatcacttatttgtgattattgtatcacagccttacaaatattcaattatttgtgtagatcaaaatgagaatcaaaggggtaacagccttatttgtaacattttagatttttatcaggaggaaatattactgtattccttatgcaattaacatcaatttgaatgctttaaaatgagaatcattagcagaatggaaaattataacaaaccttcgatgtacaagaggaaaagagataggttttaggtaaattctttattttttcgtaatgagagcaaaattaattgttttaacaatgattatatcaggatacagatgaatagcactaaattctaaatagaattggggtgagactaacaatgttattcttgggaacggacctagaggtaggccggagatttcagtttctgttactctgttactgttaattgtcatttgaatgccccttcctccccaaataggcacatacttatgtattcaattgtgaaactattagtagtttttacataatcttaatgaaatacatactcctagaggtggccaaagagttttgaattatatgtcttaactaataaacgaaatgaaaacatttgacacggcaaaatcctttcgtaacatgcaagtcatccatgtttgggcaaatctcagaaaactggcatccagctacttccaccttgttttcatgaaaccaatctccgtttccaaggaaacaagaacaaaaaggcagttggcagctagcatctgggacttagaagaactctcacatgtcaatttcaactgctggctgccggctcaaacgtaaagatgtggggtattaaaatcaccttcagacttgtaacgtacaaaagaatattaaggttttttccttagtgtttaaataatcaagtttaatagcaaaccatttaaaatatcctttgaaatactataacaaatattataattgttaaaaattatctaatacaaaaacttgttttatttaaaaacagtaggcacatatattgcagatattttctcagttttacaccataaatttttgccacttttccccttttacttaatcatttcactttctcctttttaaataatgattcatatggtcccaactacttactcctttctcttttcttttttttttttttttttttttgattcatgcaaaatatccagatagtgtctgttttatccgtaaagctttgtggccatgtttagtgttttaataaagtgttttaatgatgaaacatgaaaatgcacattgtcatttttctcttaaaaatataatttcatgattctaggcttggacacctacattaacacaacctgcttcttccgaatagcacttgttcgtttcacatgggtaggcacttcagagttcactgcagtcctcatcattccatgcagtctccaggccttctgtgtcatggcttttagatacgtttgagtttttagactcctgttgtgtgtttgtcaccatactccaacttacagcaaaagccgtaaacagtcaacgagtagttaaagttgtagcaggtatcaactaagtgttgagtttcagtaacagaatcttttcagcctctgattcttaccaatgggcggtacaatcgtatcagagaacatggtgagcccctgcctccatttgcaactgagattgcatacttttcttcctctctatgtttcctcccatttaggagaaataaaaccacagagcttgttgtacctcactgcccttgtttagtgccttcttgcatctttaaaatgtaaacttcctaatccagaaaagggattgtcttttctagcatcccaagtttagctcaatagctggcacattgcgggcactcagccaatgtctgtgaatgtctttaatccataaacgggaaaactgaggcccagagataagtaaagtggcttgtctgaagccactcagcttatttgctggcagaactgtgagtcctcactcttgtaagtctaataatctttccacagaaccacaccacataaagcaatgcagttagcctatgtacattccggttatttcaattatgcttttgtcctctatctgctttataacaatattctgaacagacttgctccttgaactcctgaaaaccaaaacttgcactcatccatgaatatatcacctttgcccctactctatgctctgcttgttttgcacattttggaatcttgcctgtgctttcagagctaagaaatctccccattgtaattgcctgagtgtctgcctgatggtcattagccacataatcccaaagcagccagaaagcaaaatttcacttatcacgtattttatctttattgatacacagtgtgattatacctctgaagagttaatgctccagaaatattaggtatgttcatatgagatccatgagccatttcagatgataaaaaagtaccactttatggaattcaaaccagtccattaactttgcattgcctaaaactatcaggttaggatttttacttgaatgggcttgaactttcttagtggctatttcttcctttctatattaaaatctcacccttattgctgctgagtatataaacaagcatatacatatacaaacactccacttaattaaaaccagaaagctcattcacttaattagttagtgtgaataaagcaccctttggaaaagatgctacttttcccactttagaaaagcaatttaacaaatattagtgactctctttggctcggtgtaaattgtgttcagaaatgtgccaatatttacatgcacacacacttcagatgcctcaacaagacattaaacaaattcatagcatatataatcagaaacattttatcatttgtagaaaaattaaactagtgaagaacttcttgatttttctttttaatttttctctacagtttaataagcaaacctgttggctgttaaacataagtattcttctaaaatgctccacatgagctatcttctgacaatgctaacaaaaacattataagagagtgtaactattgcctccacatatagatgagggaactgaggcacatgtaggttaaataatttgccaatggtggagcttgaatttgaatccaggaaatcttgattccaaagttggtgcatttaatcattggcctgtacaaccgtgttaggcaaaacaagtgtaaactttgtattttatttgaaaacatatttgcctaactattcgcaggtatctatgaatactgcaggtatctttcactgttcaaatgtaaacctttctgtgatttaaattctgctggacattgcacaacacatctaaaataattatttagtctctcatgcattgatttaccatgctcctctgtaataagggaaacttttccctaaaatgacttaaatcatctctctgattgctcattactttgattttaatgactcaaatattatttttgatttcctcaatattttaatactacctcagtttgggaacctcccctaaattattagaaaattcatggactaggtatctgaaatactttacagctttagtatgagctaaagctacataatacacttgttggaaccacgtttaggaatttataaactactgtatcactcaaagcttaagctgaatagtgttctgattttcaagcccatccggaattagaaactgaaatccacaagaaatggacgagtaaagtggaagcgaccacttggtactaaagaaggaagcttggacacacaaaaattcacacagatttgtgttattacaatgtttaatgataaatattcaaaataagaacacacattatcaataaagagcaaaatg

SEQ ID NO: 8322 - RNA, 47 nt, Homo sapiens
  source 1..47: mol_type = other RNA
aaaaaccacaattacttttgcaccaacctaatacatgcagaatcaga

SEQ ID NO: 8323 - RNA, 7250 nt, Homo sapiens
  source 1..7250: mol_type = other RNA
aaaaaccacaattacttttgcaccaacctaatacattctaaatcactaaaccattgtaaaaggtcctataaggttggtgttattcctgttttgcagatgcagacactgaggctcacgagtgtgaagcagtttgctcaaggttaagtggcagagatgttggcagggctgcctggccccattctaagtggttctttcctccgtgctatccttgaagagcactctgtatgtggatgaaagcaggtgtttagcatcacagtgtatgatgtccccagggcatctgtgactgtgttctatgtcagtctggggatctttccagggcaaaaaaagaagagacaccacatagcaagaagagacgccacccatcacacagcatattttgtgttaagatgttactctcattgtctgtcactgagagcattattattcctgatcatttacagaatccactggcaagcagtcatggcagcaccactgcaagcactgggatgaaaagatgtcatcaaagaataaaaaggggcaccgggtgcagtggctcacgcctgtaatcctagcactttgggaggatcacaaggtcaggagattgagatcatcctggctaacacggtgaaaccccgtctctaccaaaaatacaaaaaaattagtcgggtgtggtggcgggcacctgtagtcccagctactcaggagattgaggcaggagaatggggtgaacccgggaggtggagcttgcagtgagccgagatcgcaccactgcactccagccttggtgacagagtgagactctgtctcaaaaaaaaaaaaaaaaaaaaaaagaataaaaaggggcatgtttcttcacggcagtacttttcagagcctttaatatgctattttaaatttggatctgtaagaggataatttagaatctattaatcacatctgtattgtattgtattttcacaaagctggaccagttctgtgaaattccctttgagaaacactggtgtgaggccatctcttcttttcctctgccttcacacaaacaaaaactgcttctagatttctagttcttcatttcctctactcccagacagcagcaatggtgcaaattacattaaagtatttatcctaattgacactgaactcctttggcctgggatggttatagccaggggctatcaaagccattttctaatatattaacagttcttcttgaccaaagcaggtacacatgtccccaagcacgtgacgtgctgagaagagataggacatgcccatcaaagttctaaaggcataaacacaaacacacgtgcaagggaaaaaatactccccaaagaagcacacatctttaaaattcatggtaaattttacactgaaattggcattttactttttaaaacttaggaaaatggttttgctttgttgttgttactgttgttgttttgcttttatttgttttgaagtggggacagacagaaagatccaagcactgtgtcaggcttccctcgaaatgctactgtagctggatgtttcgtgtgtgtgccagagtgccagagtttggaatcactaaatgctgaagacttggggaacatgccagtttagattaactacctgccaggcattctctgaaatttccacctggggttgcacggtggatgaaccaacctttggaaagttcggttttgacaggtgggagtggaattttgaagcccggtgtcatcaacgcagtgctctgcacacctcttggaaataactcttccacatatggagagctgggacagatgaaattaaagctcttctttagaagatgtttcagttgtaagaaacagaaagcagctctagttgggggaaaaaatgcttgcattggcaggctctgggtggctcacagtactgaaagaagagctgagcaaccatttcaggcaggcaggaaatggggcactctggggcatctggaagtaggggcttatgtttttcttctctaagaggctgccattaaggtggctcagctctgttctagctcctaggagtgagatgagattggctcacctaggctgggggtctcccttttgagtggggagggggaagggaagtttgccagtcatcatttctggaaccctagtcctgtgtgtgaggattttttctaaggaaagaagaaccttcccaagtggggtcaactccagatgtgaagaggaagcagataactatgaatgtgacccccatttgttctgaaccggaaagaatgggacatatcttaagtgataagtcatgggaggtgagaaaacggtgagtttaaggaaaagaacagtatcttcaaaatggtaaagctgaggggaacgtgccagaagcttcaggaagatggagtatgcccagacaacaaggaccatggctttagctagaaaagctctttaggagaagggcaattcaatagggctaaatagattgactaaagagctggctcttctgctcaaattctaacccactaagaagacatgtgagccctaaaggagactgcaaacagcctgctctacatttttatgtgactgatgtgccatttttgtgttttaattaaacaagtttggtgctgtcacagatgctgttcattgtcaacccaatggccattgtttaacccttttcccaagcaggtagaatctttctcctgcaaagagactgaaaatgctggatattcactcttccaagcccccatgacttctgggggtggccatccaacatcattctagccaatgcaagtaaaggggatatttctcaggggtgctgggaaacattttcttccctgataaacagaccgacaagtagagttatcttgtcacatgactgggctcctttctttcttcgtttgagcatgatgggatgaggatgtgattcttggagatgctgcagccaccttgtgatcatgagggagaatcactggcatactgaagatggtggagcaagagcatgggaaagcctgggggctttgagaccaccaacctctcaatttcttattatttttaatcttaataaacccctactgattaagcttctttcactggggtgtattgttggttgcattctaatgtatctcaatggaaacagttgcccaaggtaaaatcaaacaatctcatataaaatgaagattcttgacttctcttgggggaatatgtgtttgggctgggcgctgtggctcacacctgtaatccaggcactttgggaggccgaggcaggcggatcatgaggtcaggagatcaagaccatcctggctaacacagtgaaaccctgtctctactaaaaaatacaaaaaattagccgggcatggcagtgggtgcctgtagtcccagctactcaggaggctgaggcaggagaatggcgtgaacccaggaggccgagcttgcagtgagcagggatcgcgccactgcactccagcaccacttccctggggtgtgtgcttttagtcttccacagtctccactattccttaatgaccccacttgcctcattcactgtattctcttcctagtacctcaaggtatctgagcttgtggctgccgatctctaacatggactctgagtaagtttactcaaagaggaagaaattccgacatcccacagctcccagggtgggctcggactcttcacactgtgtgtaacctgcttttccaaagagactgaattaggaaccccacatccaaaaaaaaatcaggggttgaggaataaacgttctcattatggccatttaattggtacactgtgatgttatatttacttcacgtgaatagagcatgaaattgaaacataaggatctgtaaaaatgcctgccttttgtgaactggcttacactgttcattatggctcctgaggatcctaccaccagcttcatgttattacatcatctgtaatttgaattatattttaatcaaagcttttacatggccagtattaggattttccatgtaattatcagcattagtaatactctgttgttactttgcagagtacttcctggccatttatctttaaataaaattatttatattaaatttacacttgatggtccagaattttaagtctttattaactgaagtacaacccttttcctttcctcttgctcagataaaactagaatcaaataagaatgtgggccacatcaggatggggtttttttttttaacagtagcaaaggatctttttcctacatttctattttgggctttatttttgaaaattatagagtttttagttaaattagagtattgtttaattttctaattttaaatgaattttagctcagaatttaaaattatgtcttttcaattgctatgatttatctcttaaaatatctcacattcatcttcaaagttgcttgccaatgtaactgctataatttttaaaaaatcaatggcttgactttggatgaaagtcaattcaagcctccccctctcccactccatccaggggacaatcacatgaccgtgccaaagccagtttggaaggaccagggctggagagggctgcactggggctcatggagcatagtcagtggtacatgcactccaagcttaagcccatggagcttaacagaaatggctgatcaaagatattctgatgcttctaacttgcacacgcagcccagggctgataagctgaccatttaggcagccacctgagtctctcaaaatgcagtctgttatgctaactgcccaaaagcaacactcttggccaggtgcagtggctcacgcttataatcccagcactttgggaggccgaggtgggcagatcacttgaggctaggagtccgagaccagcctggccaacgtggtgaaaccccgtgtctactaaaaatacaaaaattagccaggtgtggtggcgggcacctgtagtcctagctacttgggaggctgaggcacgagaatagcttgaacccagaggcaaaggttgcagtgagccaagatcacgccactgcactccagtgcagtctcgacacagcgagactccatctcaaaaaaaaaaaaaaaaaagtgacactctggatagcaaagatgcatcacctcgtagcacccaggcccaggaatctgaacaaccacatggtacatccaatcagaattggatgaaggggatgctccttgccttgaaaaaactagctggccaaggagcagcgtgctctatactcagactgaaaaaggttcatattgactggctgtattcaacaatgcaaagagctgagcgagagacacagcacattcctgattctgttcttgtaccttctaccagagtcctatcatgctgaaatattgccagctagataggaacaggaacacaccaccacttggagaatccttagagcagagctctgcaaaactcagatcctaaaggggaaaaattctcagcctgaagttgcttcttatccccaatggccactcagccactcccttgagatgagccccaggcatgcggtttctgatctgtgagatcggtcacatcacttcttgcagaagagccaagtaaagcccccgtgccccaaaaattcactgtatgaggcagagctacagaagtggctccataaacttagactggaagatgggaaggatattgtgcccatgaaccctcaggcaactgctgtgacctcatcccccacacatgcactcatgcatcttcatgctcattgtgtttggtggaagtctgtgcatgaagttattaattttatttgcttccagattcaatgattcaaaagccctggaaatgctcaagctgtcactccaagtttcaaatctattttagagacgtgggctatgagaagctgatggctcagaaaggttctgagcctttgcttccaagctcagcacctggaatgacctacagacagagctggctttgggtctctgagaaacctgctgcatctccaaatgacttgttgcgctgggtggccaacaccaagtcttccacgtgggaggttttattatgttttacaaccatgaaaacataggaaggtggctgttacagcaaacatttcagatagacgaatcggccaagctccccaaaccccaccttcacagcctcttccacacgtctctcagagattgttgtccttcacttgcaaattcaaggatgttggaagtagacatttaaagtagcaggaacaccatcagtgaaacagaagcagaagtacgatgactttgagaaacaactgatgaaaaatacactacagaaaaccatttctattgtgttatgatgtcagggtggcagatgtgcccagggcttagtgtccatcctcccaggacactggtcataccgggccttcggtgatcccctccagaggcaagctgggtgcgctgtcagctgtgggcctctcctctttcttcagtgaggctgggactcgcagactaacgtagggtttatggcaagctgtgttggccagaggaggatagtgctgtctgtagcaaatgtatgcaaaaatgaggccgatgactccacccacaaaggaataggaggaatggatgctggggaagcttttgcggccctcggacaccagatcggggtcacctgtgcaatgcatttccgagttcatcactccatctggaaagcagcggtaaaagaaatcggggcgaggtcttcccactattaatttaatagtgtttgtgcagactccattcaaagcaagagccaaggacaccgctaagaaggcttccttaatttcagtcttgtctgttcgccggataattttcaccacacaaataacagccaggggtgtgaggaaagaaattgcaaacatgaggcgggtaggtatgttatctgattgcaccaaaggatttttatagagccagatctcttctggctggatgactctctggaacggatccaaaaactctgtaaaaacgaagactccgaagagcagggctcgcaccccgatctcaatggccagctcccgcatggtgcggccggagcagctcccgcggcgtcagctggtgctctccgcggctcccgcagctcggccggcgccggctcgccagaccctgggaggcgagggaggcgcgctccaggccgcgggcgggggcggaggcgggcgccgggcgggggcaggcgccggggagggctcagcctaaacctcgcgcctcgggctccggggctccgggaagccgcgccggccgctggcgatactgcggaccccgcctcctagtgcggagccggggccgcctcagggactcccggatccctctccccaggagccgcctccgcctcctgggcccgcgccgggcacccgcggaccggggaggggaagcccg

SEQ ID NO: 8324 - RNA, 7041 nt, Homo sapiens
  source 1..7041: mol_type = other RNA
aaaaaccacaattacttttgcaccaacctaatacattctaaatcactaaaccattgtaaaaggtcctataaggttggtgttattcctgttttgcagatgcagacactgaggctcacgagtgtgaagcagtttgctcaaggttaagtggcagagatgttggcagggctgcctggccccattctaagtggttctttcctccgtgctatccttgaagagcactctgtatgtggatgaaagcaggtgtttagcatcacagtgtatgatgtccccagggcatctgtgactgtgttctatgtcagtctggggatctttccagggcaaaaaaagaagagacaccacatagcaagaagagacgccacccatcacacagcatattttgtgttaagatgttactctcattgtctgtcactgagagcattattattcctgatcatttacagaatccactggcaagcagtcatggcagcaccactgcaagcactgggatgaaaagatgtcatcaaagaataaaaaggggcaccgggtgcagtggctcacgcctgtaatcctagcactttgggaggatcacaaggtcaggagattgagatcatcctggctaacacggtgaaaccccgtctctaccaaaaatacaaaaaaattagtcgggtgtggtggcgggcacctgtagtcccagctactcaggagattgaggcaggagaatggggtgaacccgggaggtggagcttgcagtgagccgagatcgcaccactgcactccagccttggtgacagagtgagactctgtctcaaaaaaaaaaaaaaaaaaaaaaagaataaaaaggggcatgtttcttcacggcagtacttttcagagcctttaatatgctattttaaatttggatctgtaagaggataatttagaatctattaatcacatctgtattgtattgtattttcacaaagctggaccagttctgtgaaattccctttgagaaacactggtgtgaggccatctcttcttttcctctgccttcacacaaacaaaaactgcttctagatttctagttcttcatttcctctactcccagacagcagcaatggtgcaaattacattaaagtatttatcctaattgacactgaactcctttggcctgggatggttatagccaggggctatcaaagccattttctaatatattaacagttcttcttgaccaaagcaggtacacatgtccccaagcacgtgacgtgctgagaagagataggacatgcccatcaaagttctaaaggcataaacacaaacacacgtgcaagggaaaaaatactccccaaagaagcacacatctttaaaattcatggtaaattttacactgaaattggcattttactttttaaaacttaggaaaatggttttgctttgttgttgttactgttgttgttttgcttttatttgttttgaagtggggacagacagaaagatccaagcactgtgtcaggcttccctcgaaatgctactgtagctggatgtttcgtgtgtgtgccagagtgccagagtttggaatcactaaatgctgaagacttggggaacatgccagtttagattaactacctgccaggcattctctgaaatttccacctggggttgcacggtggatgaaccaacctttggaaagttcggttttgacaggtgggagtggaattttgaagcccggtgtcatcaacgcagtgctctgcacacctcttggaaataactcttccacatatggagagctgggacagatgaaattaaagctcttctttagaagatgtttcagttgtaagaaacagaaagcagctctagttgggggaaaaaatgcttgcattggcaggctctgggtggctcacagtactgaaagaagagctgagcaaccatttcaggcaggcaggaaatggggcactctggggcatctggaagtaggggcttatgtttttcttctctaagaggctgccattaaggtggctcagctctgttctagctcctaggagtgagatgagattggctcacctaggctgggggtctcccttttgagtggggagggggaagggaagtttgccagtcatcatttctggaaccctagtcctgtgtgtgaggattttttctaaggaaagaagaaccttcccaagtggggtcaactccagatgtgaagaggaagcagataactatgaatgtgacccccatttgttctgaaccggaaagaatgggacatatcttaagtgataagtcatgggaggtgagaaaacggtgagtttaaggaaaagaacagtatcttcaaaatggtaaagctgaggggaacgtgccagaagcttcaggaagatggagtatgcccagacaacaaggaccatggctttagctagaaaagctctttaggagaagggcaattcaatagggctaaatagattgactaaagagctggctcttctgctcaaattctaacccactaagaagacatgtgagccctaaaggagactgcaaacagcctgctctacatttttatgtgactgatgtgccatttttgtgttttaattaaacaagtttggtgctgtcacagatgctgttcattgtcaacccaatggccattgtttaacccttttcccaagcaggtagaatctttctcctgcaaagagactgaaaatgctggatattcactcttccaagcccccatgacttctgggggtggccatccaacatcattctagccaatgcaagtaaaggggatatttctcaggggtgctgggaaacattttcttccctgataaacagaccgacaagtagagttatcttgtcacatgactgggctcctttctttcttcgtttgagcatgatgggatgaggatgtgattcttggagatgctgcagccaccttgtgatcatgagggagaatcactggcatactgaagatggtggagcaagagcatgggaaagcctgggggctttgagaccaccaacctctcaatttcttattatttttaatcttaataaacccctactgattaagcttctttcactggggtgtattgttggttgcattctaatgtatctcaatggaaacagttgcccaaggtaaaatcaaacaatctcatataaaatgaagattcttgacttctcttgggggaatatgtgtttgggctgggcgctgtggctcacacctgtaatccaggcactttgggaggccgaggcaggcggatcatgaggtcaggagatcaagaccatcctggctaacacagtgaaaccctgtctctactaaaaaatacaaaaaattagccgggcatggcagtgggtgcctgtagtcccagctactcaggaggctgaggcaggagaatggcgtgaacccaggaggccgagcttgcagtgagcagggatcgcgccactgcactccagcaccacttccctggggtgtgtgcttttagtcttccacagtctccactattccttaatgaccccacttgcctcattcactgtattctcttcctagtacctcaaggtatctgagcttgtggctgccgatctctaacatggactctgagtaagtttactcaaagaggaagaaattccgacatcccacagctcccagggtgggctcggactcttcacactgtgtgtaacctgcttttccaaagagactgaattaggaaccccacatccaaaaaaaaatcaggggttgaggaataaacgttctcattatggccatttaattggtacactgtgatgttatatttacttcacgtgaatagagcatgaaattgaaacataaggatctgtaaaaatgcctgccttttgtgaactggcttacactgttcattatggctcctgaggatcctaccaccagcttcatgttattacatcatctgtaatttgaattatattttaatcaaagcttttacatggccagtattaggattttccatgtaattatcagcattagtaatactctgttgttactttgcagagtacttcctggccatttatctttaaataaaattatttatattaaatttacacttgatggtccagaattttaagtctttattaactgaagtacaacccttttcctttcctcttgctcagataaaactagaatcaaataagaatgtgggccacatcaggatggggtttttttttttaacagtagcaaaggatctttttcctacatttctattttgggctttatttttgaaaattatagagtttttagttaaattagagtattgtttaattttctaattttaaatgaattttagctcagaatttaaaattatgtcttttcaattgctatgatttatctcttaaaatatctcacattcatcttcaaagttgcttgccaatgtaactgctataatttttaaaaaatcaatggcttgactttggatgaaagtcaattcaagcctccccctctcccactccatccaggggacaatcacatgaccgtgccaaagccagtttggaaggaccagggctggagagggctgcactggggctcatggagcatagtcagtggtacatgcactccaagcttaagcccatggagcttaacagaaatggctgatcaaagatattctgatgcttctaacttgcacacgcagcccagggctgataagctgaccatttaggcagccacctgagtctctcaaaatgcagtctgttatgctaactgcccaaaagcaacactcttggccaggtgcagtggctcacgcttataatcccagcactttgggaggccgaggtgggcagatcacttgaggctaggagtccgagaccagcctggccaacgtggtgaaaccccgtgtctactaaaaatacaaaaattagccaggtgtggtggcgggcacctgtagtcctagctacttgggaggctgaggcacgagaatagcttgaacccagaggcaaaggttgcagtgagccaagatcacgccactgcactccagtgcagtctcgacacagcgagactccatctcaaaaaaaaaaaaaaaaaagtgacactctggatagcaaagatgcatcacctcgtagcacccaggcccaggaatctgaacaaccacatggtacatccaatcagaattggatgaaggggatgctccttgccttgaaaaaactagctggccaaggagcagcgtgctctatactcagactgaaaaaggttcatattgactggctgtattcaacaatgcaaagagctgagcgagagacacagcacattcctgattctgttcttgtaccttctaccagagtcctatcatgctgaaatattgccagctagataggaacaggaacacaccaccacttggagaatccttagagcagagctctgcaaaactcagatcctaaaggggaaaaattctcagcctgaagttgcttcttatccccaatggccactcagccactcccttgagatgagccccaggcatgcggtttctgatctgtgagatcggtcacatcacttcttgcagaagagccaagtaaagcccccgtgccccaaaaattcactgtatgaggcagagctacagaagtggctccataaacttagactggaagatgggaaggatattgtgcccatgaaccctcaggcaactgctgtgacctcatcccccacacatgcactcatgcatcttcatgctcattgtgtttggtggaagtctgtgcatgaagttattaattttatttgcttccagattcaatgattcaaaagccctggaaatgctcaagctgtcactccaagtttcaaatctattttagagacgtgggctatgagaagctgatggctcagaaaggttctgagcctttgcttccaagctcagcacctggaatgacctacagacagagctggctttgggtctctgagaaacctgctgcatctccaaatgacttgttgcgctgggtggccaacaccaagtcttccacgtgggaggttttattatgttttacaaccatgaaaacataggaaggtggctgttacagcaaacatttcagatagacgaatcggccaagctccccaaaccccaccttcacagcctcttccacacgtctctcagagattgttgtccttcacttgcaaattcaaggatgttggaagtagacatttaaagtagcaggaacaccatcagtgaaacagaagcagaagtacgatgactttgagaaacaactgatgaaaaatacactacagaaaaccatttctattgtgttatgatgtcagggtggcagatgtgcccagggcttagtgtccatcctcccaggacactggtcataccgggccttcggtgatcccctccagaggcaagctgggtgcgctgtcagctgtgggcctctcctctttcttcagtgaggctgggactcgcagactaacgtagggtttatggcaagctgtgttggccagaggaggatagtgctgtctgtagcaaatgtatgcaaaaatgaggccgatgactccacccacaaaggaatcttgccagtgatgcttgtagtcgcacatgcgggacagggcaatcatcatggcgcagtacaagggcaggatggcagcacagagccgccagctctttccccgcccactctcggtgaagcagtgcagcttgcccgccaagtagaacgtcgtgaagccaaggcccgaaaaggcaaaggaggaatggatgctggggaagcttttgcggccctcggacaccagatcggggtcacctgtgcaatgcatttccgagttcatcactccatctggaaagcagcggtaaaagaaatcggggcgaggtcttcccactattaatttaatagtgtttgtgcagactccattcaaagcaagagccaaggacaccgaaacatgaggcgggtaggtatgttatctgattgcaccaaaggatttttatagagccagatctcttctggctggatgactctctggaacggatccaaaaactctgtaaaaacgaagactccgaagagcagggctcgcaccccgatctcaatggccagctcccgcatggtgcggccggagcagctcccgcggcgtcagctggtgctctccgcggctcccgcagctcggcc

SEQ ID NO: 8325 - RNA, 7259 nt, Homo sapiens
  source 1..7259: mol_type = other RNA
aaaaaccacaattacttttgcaccaacctaatacattctaaatcactaaaccattgtaaaaggtcctataaggttggtgttattcctgttttgcagatgcagacactgaggctcacgagtgtgaagcagtttgctcaaggttaagtggcagagatgttggcagggctgcctggccccattctaagtggttctttcctccgtgctatccttgaagagcactctgtatgtggatgaaagcaggtgtttagcatcacagtgtatgatgtccccagggcatctgtgactgtgttctatgtcagtctggggatctttccagggcaaaaaaagaagagacaccacatagcaagaagagacgccacccatcacacagcatattttgtgttaagatgttactctcattgtctgtcactgagagcattattattcctgatcatttacagaatccactggcaagcagtcatggcagcaccactgcaagcactgggatgaaaagatgtcatcaaagaataaaaaggggcaccgggtgcagtggctcacgcctgtaatcctagcactttgggaggatcacaaggtcaggagattgagatcatcctggctaacacggtgaaaccccgtctctaccaaaaatacaaaaaaattagtcgggtgtggtggcgggcacctgtagtcccagctactcaggagattgaggcaggagaatggggtgaacccgggaggtggagcttgcagtgagccgagatcgcaccactgcactccagccttggtgacagagtgagactctgtctcaaaaaaaaaaaaaaaaaaaaaaagaataaaaaggggcatgtttcttcacggcagtacttttcagagcctttaatatgctattttaaatttggatctgtaagaggataatttagaatctattaatcacatctgtattgtattgtattttcacaaagctggaccagttctgtgaaattccctttgagaaacactggtgtgaggccatctcttcttttcctctgccttcacacaaacaaaaactgcttctagatttctagttcttcatttcctctactcccagacagcagcaatggtgcaaattacattaaagtatttatcctaattgacactgaactcctttggcctgggatggttatagccaggggctatcaaagccattttctaatatattaacagttcttcttgaccaaagcaggtacacatgtccccaagcacgtgacgtgctgagaagagataggacatgcccatcaaagttctaaaggcataaacacaaacacacgtgcaagggaaaaaatactccccaaagaagcacacatctttaaaattcatggtaaattttacactgaaattggcattttactttttaaaacttaggaaaatggttttgctttgttgttgttactgttgttgttttgcttttatttgttttgaagtggggacagacagaaagatccaagcactgtgtcaggcttccctcgaaatgctactgtagctggatgtttcgtgtgtgtgccagagtgccagagtttggaatcactaaatgctgaagacttggggaacatgccagtttagattaactacctgccaggcattctctgaaatttccacctggggttgcacggtggatgaaccaacctttggaaagttcggttttgacaggtgggagtggaattttgaagcccggtgtcatcaacgcagtgctctgcacacctcttggaaataactcttccacatatggagagctgggacagatgaaattaaagctcttctttagaagatgtttcagttgtaagaaacagaaagcagctctagttgggggaaaaaatgcttgcattggcaggctctgggtggctcacagtactgaaagaagagctgagcaaccatttcaggcaggcaggaaatggggcactctggggcatctggaagtaggggcttatgtttttcttctctaagaggctgccattaaggtggctcagctctgttctagctcctaggagtgagatgagattggctcacctaggctgggggtctcccttttgagtggggagggggaagggaagtttgccagtcatcatttctggaaccctagtcctgtgtgtgaggattttttctaaggaaagaagaaccttcccaagtggggtcaactccagatgtgaagaggaagcagataactatgaatgtgacccccatttgttctgaaccggaaagaatgggacatatcttaagtgataagtcatgggaggtgagaaaacggtgagtttaaggaaaagaacagtatcttcaaaatggtaaagctgaggggaacgtgccagaagcttcaggaagatggagtatgcccagacaacaaggaccatggctttagctagaaaagctctttaggagaagggcaattcaatagggctaaatagattgactaaagagctggctcttctgctcaaattctaacccactaagaagacatgtgagccctaaaggagactgcaaacagcctgctctacatttttatgtgactgatgtgccatttttgtgttttaattaaacaagtttggtgctgtcacagatgctgttcattgtcaacccaatggccattgtttaacccttttcccaagcaggtagaatctttctcctgcaaagagactgaaaatgctggatattcactcttccaagcccccatgacttctgggggtggccatccaacatcattctagccaatgcaagtaaaggggatatttctcaggggtgctgggaaacattttcttccctgataaacagaccgacaagtagagttatcttgtcacatgactgggctcctttctttcttcgtttgagcatgatgggatgaggatgtgattcttggagatgctgcagccaccttgtgatcatgagggagaatcactggcatactgaagatggtggagcaagagcatgggaaagcctgggggctttgagaccaccaacctctcaatttcttattatttttaatcttaataaacccctactgattaagcttctttcactggggtgtattgttggttgcattctaatgtatctcaatggaaacagttgcccaaggtaaaatcaaacaatctcatataaaatgaagattcttgacttctcttgggggaatatgtgtttgggctgggcgctgtggctcacacctgtaatccaggcactttgggaggccgaggcaggcggatcatgaggtcaggagatcaagaccatcctggctaacacagtgaaaccctgtctctactaaaaaatacaaaaaattagccgggcatggcagtgggtgcctgtagtcccagctactcaggaggctgaggcaggagaatggcgtgaacccaggaggccgagcttgcagtgagcagggatcgcgccactgcactccagcaccacttccctggggtgtgtgcttttagtcttccacagtctccactattccttaatgaccccacttgcctcattcactgtattctcttcctagtacctcaaggtatctgagcttgtggctgccgatctctaacatggactctgagtaagtttactcaaagaggaagaaattccgacatcccacagctcccagggtgggctcggactcttcacactgtgtgtaacctgcttttccaaagagactgaattaggaaccccacatccaaaaaaaaatcaggggttgaggaataaacgttctcattatggccatttaattggtacactgtgatgttatatttacttcacgtgaatagagcatgaaattgaaacataaggatctgtaaaaatgcctgccttttgtgaactggcttacactgttcattatggctcctgaggatcctaccaccagcttcatgttattacatcatctgtaatttgaattatattttaatcaaagcttttacatggccagtattaggattttccatgtaattatcagcattagtaatactctgttgttactttgcagagtacttcctggccatttatctttaaataaaattatttatattaaatttacacttgatggtccagaattttaagtctttattaactgaagtacaacccttttcctttcctcttgctcagataaaactagaatcaaataagaatgtgggccacatcaggatggggtttttttttttaacagtagcaaaggatctttttcctacatttctattttgggctttatttttgaaaattatagagtttttagttaaattagagtattgtttaattttctaattttaaatgaattttagctcagaatttaaaattatgtcttttcaattgctatgatttatctcttaaaatatctcacattcatcttcaaagttgcttgccaatgtaactgctataatttttaaaaaatcaatggcttgactttggatgaaagtcaattcaagcctccccctctcccactccatccaggggacaatcacatgaccgtgccaaagccagtttggaaggaccagggctggagagggctgcactggggctcatggagcatagtcagtggtacatgcactccaagcttaagcccatggagcttaacagaaatggctgatcaaagatattctgatgcttctaacttgcacacgcagcccagggctgataagctgaccatttaggcagccacctgagtctctcaaaatgcagtctgttatgctaactgcccaaaagcaacactcttggccaggtgcagtggctcacgcttataatcccagcactttgggaggccgaggtgggcagatcacttgaggctaggagtccgagaccagcctggccaacgtggtgaaaccccgtgtctactaaaaatacaaaaattagccaggtgtggtggcgggcacctgtagtcctagctacttgggaggctgaggcacgagaatagcttgaacccagaggcaaaggttgcagtgagccaagatcacgccactgcactccagtgcagtctcgacacagcgagactccatctcaaaaaaaaaaaaaaaaaagtgacactctggatagcaaagatgcatcacctcgtagcacccaggcccaggaatctgaacaaccacatggtacatccaatcagaattggatgaaggggatgctccttgccttgaaaaaactagctggccaaggagcagcgtgctctatactcagactgaaaaaggttcatattgactggctgtattcaacaatgcaaagagctgagcgagagacacagcacattcctgattctgttcttgtaccttctaccagagtcctatcatgctgaaatattgccagctagataggaacaggaacacaccaccacttggagaatccttagagcagagctctgcaaaactcagatcctaaaggggaaaaattctcagcctgaagttgcttcttatccccaatggccactcagccactcccttgagatgagccccaggcatgcggtttctgatctgtgagatcggtcacatcacttcttgcagaagagccaagtaaagcccccgtgccccaaaaattcactgtatgaggcagagctacagaagtggctccataaacttagactggaagatgggaaggatattgtgcccatgaaccctcaggcaactgctgtgacctcatcccccacacatgcactcatgcatcttcatgctcattgtgtttggtggaagtctgtgcatgaagttattaattttatttgcttccagattcaatgattcaaaagccctggaaatgctcaagctgtcactccaagtttcaaatctattttagagacgtgggctatgagaagctgatggctcagaaaggttctgagcctttgcttccaagctcagcacctggaatgacctacagacagagctggctttgggtctctgagaaacctgctgcatctccaaatgacttgttgcgctgggtggccaacaccaagtcttccacgtgggaggttttattatgttttacaaccatgaaaacataggaaggtggctgttacagcaaacatttcagatagacgaatcggccaagctccccaaaccccaccttcacagcctcttccacacgtctctcagagattgttgtccttcacttgcaaattcaaggatgttggaagtagacatttaaagtagcaggaacaccatcagtgaaacagaagcagaagtacgatgactttgagaaacaactgatgaaaaatacactacagaaaaccatttctattgtgttatgatgtcagggtggcagatgtgcccagggcttagtgtccatcctcccaggacactggtcataccgggccttcggtgatcccctccagaggcaagctgggtgcgctgtcagctgtgggcctctcctctttcttcagtgaggctgggactcgcagactaacgtagggtttatggcaagctgtgttggccagaggaggatagtgctgtctgtagcaaatgtatgcaaaaatgaggccgatgactccacccacaaaggaatcttgccagtgatgcttgtagtcgcacatgcgggacagggcaatcatcatggcgcagtacaagggcaggatggcagcacagagccgccagctctttccccgcccactctcggtgaagcagtgcagcttgcccgccaagtagaacgtcgtgaagccaaggcccgaaaaggcaaaggaggaatggatgctggggaagcttttgcggccctcggacaccagatcggggtcacctgtgcaatgcatttccgagttcatcactccatctggaaagcagcggtaaaagaaatcggggcgaggtcttcccactattaatttaatagtgtttgtgcagactccattcaaagcaagagccaaggacaccgctaagaaggcttccttaatttcagtcttgtctgttcgccggataattttcaccacacaaataacagccaggggtgtgaggaaagaaattgcaaacatgaggcgggtaggtatgttatctgattgcaccaaaggatttttatagagccagatctcttctggctggatgactctctggaacggatccaaaaactctgtaaaacttgcgttcttcatcatctatcccaactgatggagctatatcagccctgctgcactcactgagaattggatttgatatatgacagctgcctgaaccgctccttattcatgcagtaaatgagacgtcatcttcagaggcacacgaagactccgaagagcagggctcgcaccccgatctcaatggccagctcccgcatggtgcggccggagcagctcccgcggcgtcagctggtgctctccgcggctc

SEQ ID NO: 8326 - RNA, 7149 nt, Homo sapiens
  source 1..7149: mol_type = other RNA
aaaaaccacaattacttttgcaccaacctaatacattctaaatcactaaaccattgtaaaaggtcctataaggttggtgttattcctgttttgcagatgcagacactgaggctcacgagtgtgaagcagtttgctcaaggttaagtggcagagatgttggcagggctgcctggccccattctaagtggttctttcctccgtgctatccttgaagagcactctgtatgtggatgaaagcaggtgtttagcatcacagtgtatgatgtccccagggcatctgtgactgtgttctatgtcagtctggggatctttccagggcaaaaaaagaagagacaccacatagcaagaagagacgccacccatcacacagcatattttgtgttaagatgttactctcattgtctgtcactgagagcattattattcctgatcatttacagaatccactggcaagcagtcatggcagcaccactgcaagcactgggatgaaaagatgtcatcaaagaataaaaaggggcaccgggtgcagtggctcacgcctgtaatcctagcactttgggaggatcacaaggtcaggagattgagatcatcctggctaacacggtgaaaccccgtctctaccaaaaatacaaaaaaattagtcgggtgtggtggcgggcacctgtagtcccagctactcaggagattgaggcaggagaatggggtgaacccgggaggtggagcttgcagtgagccgagatcgcaccactgcactccagccttggtgacagagtgagactctgtctcaaaaaaaaaaaaaaaaaaaaaaagaataaaaaggggcatgtttcttcacggcagtacttttcagagcctttaatatgctattttaaatttggatctgtaagaggataatttagaatctattaatcacatctgtattgtattgtattttcacaaagctggaccagttctgtgaaattccctttgagaaacactggtgtgaggccatctcttcttttcctctgccttcacacaaacaaaaactgcttctagatttctagttcttcatttcctctactcccagacagcagcaatggtgcaaattacattaaagtatttatcctaattgacactgaactcctttggcctgggatggttatagccaggggctatcaaagccattttctaatatattaacagttcttcttgaccaaagcaggtacacatgtccccaagcacgtgacgtgctgagaagagataggacatgcccatcaaagttctaaaggcataaacacaaacacacgtgcaagggaaaaaatactccccaaagaagcacacatctttaaaattcatggtaaattttacactgaaattggcattttactttttaaaacttaggaaaatggttttgctttgttgttgttactgttgttgttttgcttttatttgttttgaagtggggacagacagaaagatccaagcactgtgtcaggcttccctcgaaatgctactgtagctggatgtttcgtgtgtgtgccagagtgccagagtttggaatcactaaatgctgaagacttggggaacatgccagtttagattaactacctgccaggcattctctgaaatttccacctggggttgcacggtggatgaaccaacctttggaaagttcggttttgacaggtgggagtggaattttgaagcccggtgtcatcaacgcagtgctctgcacacctcttggaaataactcttccacatatggagagctgggacagatgaaattaaagctcttctttagaagatgtttcagttgtaagaaacagaaagcagctctagttgggggaaaaaatgcttgcattggcaggctctgggtggctcacagtactgaaagaagagctgagcaaccatttcaggcaggcaggaaatggggcactctggggcatctggaagtaggggcttatgtttttcttctctaagaggctgccattaaggtggctcagctctgttctagctcctaggagtgagatgagattggctcacctaggctgggggtctcccttttgagtggggagggggaagggaagtttgccagtcatcatttctggaaccctagtcctgtgtgtgaggattttttctaaggaaagaagaaccttcccaagtggggtcaactccagatgtgaagaggaagcagataactatgaatgtgacccccatttgttctgaaccggaaagaatgggacatatcttaagtgataagtcatgggaggtgagaaaacggtgagtttaaggaaaagaacagtatcttcaaaatggtaaagctgaggggaacgtgccagaagcttcaggaagatggagtatgcccagacaacaaggaccatggctttagctagaaaagctctttaggagaagggcaattcaatagggctaaatagattgactaaagagctggctcttctgctcaaattctaacccactaagaagacatgtgagccctaaaggagactgcaaacagcctgctctacatttttatgtgactgatgtgccatttttgtgttttaattaaacaagtttggtgctgtcacagatgctgttcattgtcaacccaatggccattgtttaacccttttcccaagcaggtagaatctttctcctgcaaagagactgaaaatgctggatattcactcttccaagcccccatgacttctgggggtggccatccaacatcattctagccaatgcaagtaaaggggatatttctcaggggtgctgggaaacattttcttccctgataaacagaccgacaagtagagttatcttgtcacatgactgggctcctttctttcttcgtttgagcatgatgggatgaggatgtgattcttggagatgctgcagccaccttgtgatcatgagggagaatcactggcatactgaagatggtggagcaagagcatgggaaagcctgggggctttgagaccaccaacctctcaatttcttattatttttaatcttaataaacccctactgattaagcttctttcactggggtgtattgttggttgcattctaatgtatctcaatggaaacagttgcccaaggtaaaatcaaacaatctcatataaaatgaagattcttgacttctcttgggggaatatgtgtttgggctgggcgctgtggctcacacctgtaatccaggcactttgggaggccgaggcaggcggatcatgaggtcaggagatcaagaccatcctggctaacacagtgaaaccctgtctctactaaaaaatacaaaaaattagccgggcatggcagtgggtgcctgtagtcccagctactcaggaggctgaggcaggagaatggcgtgaacccaggaggccgagcttgcagtgagcagggatcgcgccactgcactccagcaccacttccctggggtgtgtgcttttagtcttccacagtctccactattccttaatgaccccacttgcctcattcactgtattctcttcctagtacctcaaggtatctgagcttgtggctgccgatctctaacatggactctgagtaagtttactcaaagaggaagaaattccgacatcccacagctcccagggtgggctcggactcttcacactgtgtgtaacctgcttttccaaagagactgaattaggaaccccacatccaaaaaaaaatcaggggttgaggaataaacgttctcattatggccatttaattggtacactgtgatgttatatttacttcacgtgaatagagcatgaaattgaaacataaggatctgtaaaaatgcctgccttttgtgaactggcttacactgttcattatggctcctgaggatcctaccaccagcttcatgttattacatcatctgtaatttgaattatattttaatcaaagcttttacatggccagtattaggattttccatgtaattatcagcattagtaatactctgttgttactttgcagagtacttcctggccatttatctttaaataaaattatttatattaaatttacacttgatggtccagaattttaagtctttattaactgaagtacaacccttttcctttcctcttgctcagataaaactagaatcaaataagaatgtgggccacatcaggatggggtttttttttttaacagtagcaaaggatctttttcctacatttctattttgggctttatttttgaaaattatagagtttttagttaaattagagtattgtttaattttctaattttaaatgaattttagctcagaatttaaaattatgtcttttcaattgctatgatttatctcttaaaatatctcacattcatcttcaaagttgcttgccaatgtaactgctataatttttaaaaaatcaatggcttgactttggatgaaagtcaattcaagcctccccctctcccactccatccaggggacaatcacatgaccgtgccaaagccagtttggaaggaccagggctggagagggctgcactggggctcatggagcatagtcagtggtacatgcactccaagcttaagcccatggagcttaacagaaatggctgatcaaagatattctgatgcttctaacttgcacacgcagcccagggctgataagctgaccatttaggcagccacctgagtctctcaaaatgcagtctgttatgctaactgcccaaaagcaacactcttggccaggtgcagtggctcacgcttataatcccagcactttgggaggccgaggtgggcagatcacttgaggctaggagtccgagaccagcctggccaacgtggtgaaaccccgtgtctactaaaaatacaaaaattagccaggtgtggtggcgggcacctgtagtcctagctacttgggaggctgaggcacgagaatagcttgaacccagaggcaaaggttgcagtgagccaagatcacgccactgcactccagtgcagtctcgacacagcgagactccatctcaaaaaaaaaaaaaaaaaagtgacactctggatagcaaagatgcatcacctcgtagcacccaggcccaggaatctgaacaaccacatggtacatccaatcagaattggatgaaggggatgctccttgccttgaaaaaactagctggccaaggagcagcgtgctctatactcagactgaaaaaggttcatattgactggctgtattcaacaatgcaaagagctgagcgagagacacagcacattcctgattctgttcttgtaccttctaccagagtcctatcatgctgaaatattgccagctagataggaacaggaacacaccaccacttggagaatccttagagcagagctctgcaaaactcagatcctaaaggggaaaaattctcagcctgaagttgcttcttatccccaatggccactcagccactcccttgagatgagccccaggcatgcggtttctgatctgtgagatcggtcacatcacttcttgcagaagagccaagtaaagcccccgtgccccaaaaattcactgtatgaggcagagctacagaagtggctccataaacttagactggaagatgggaaggatattgtgcccatgaaccctcaggcaactgctgtgacctcatcccccacacatgcactcatgcatcttcatgctcattgtgtttggtggaagtctgtgcatgaagttattaattttatttgcttccagattcaatgattcaaaagccctggaaatgctcaagctgtcactccaagtttcaaatctattttagagacgtgggctatgagaagctgatggctcagaaaggttctgagcctttgcttccaagctcagcacctggaatgacctacagacagagctggctttgggtctctgagaaacctgctgcatctccaaatgacttgttgcgctgggtggccaacaccaagtcttccacgtgggaggttttattatgttttacaaccatgaaaacataggaaggtggctgttacagcaaacatttcagatagacgaatcggccaagctccccaaaccccaccttcacagcctcttccacacgtctctcagagattgttgtccttcacttgcaaattcaaggatgttggaagtagacatttaaagtagcaggaacaccatcagtgaaacagaagcagaagtacgatgactttgagaaacaactgatgaaaaatacactacagaaaaccatttctattgtgttatgatgtcagggtggcagatgtgcccagggcttagtgtccatcctcccaggacactggtcataccgggccttcggtgatcccctccagaggcaagctgggtgcgctgtcagctgtgggcctctcctctttcttcagtgaggctgggactcgcagactaacgtagggtttatggcaagctgtgttggccagaggaggatagtgctgtctgtagcaaatgtatgcaaaaatgaggccgatgactccacccacaaaggaatcttgccagtgatgcttgtagtcgcacatgcgggacagggcaatcatcatggcgcagtacaagggcaggatggcagcacagagccgccagctctttccccgcccactctcggtgaagcagtgcagcttgcccgccaagtagaacgtcgtgaagccaaggcccgaaaaggcaaaggaggaatggatgctggggaagcttttgcggccctcggacaccagatcggggtcacctgtgcaatgcatttccgagttcatcactccatctggaaagcagcggtaaaagaaatcggggcgaggtcttcccactattaatttaatagtgtttgtgcagactccattcaaagcaagagccaaggacaccgctaagaaggcttccttaatttcagtcttgtctgttcgccggataattttcaccacacaaataacagccaggggtgtgaggaaagaaattgcaaacatgaggcgggtaggtatgttatctgattgcaccaaaggatttttatagagccagatctcttctggctggatgactctctggaacggatccaaaaactctgtaaaatgagaattggatttgatatatgacagctgcctgaaccgctccttattcatgcagtaaatgagacgtcatcttcagaggcacacgaagactccgaagagcagggctcgcaccccgatctcaatggccagctcccgca

SEQ ID NO: 8327 - RNA, 6832 nt, Homo sapiens
  source 1..6832: mol_type = other RNA
aaaaaccacaattacttttgcaccaacctaatacattctaaatcactaaaccattgtaaaaggtcctataaggttggtgttattcctgttttgcagatgcagacactgaggctcacgagtgtgaagcagtttgctcaaggttaagtggcagagatgttggcagggctgcctggccccattctaagtggttctttcctccgtgctatccttgaagagcactctgtatgtggatgaaagcaggtgtttagcatcacagtgtatgatgtccccagggcatctgtgactgtgttctatgtcagtctggggatctttccagggcaaaaaaagaagagacaccacatagcaagaagagacgccacccatcacacagcatattttgtgttaagatgttactctcattgtctgtcactgagagcattattattcctgatcatttacagaatccactggcaagcagtcatggcagcaccactgcaagcactgggatgaaaagatgtcatcaaagaataaaaaggggcaccgggtgcagtggctcacgcctgtaatcctagcactttgggaggatcacaaggtcaggagattgagatcatcctggctaacacggtgaaaccccgtctctaccaaaaatacaaaaaaattagtcgggtgtggtggcgggcacctgtagtcccagctactcaggagattgaggcaggagaatggggtgaacccgggaggtggagcttgcagtgagccgagatcgcaccactgcactccagccttggtgacagagtgagactctgtctcaaaaaaaaaaaaaaaaaaaaaaagaataaaaaggggcatgtttcttcacggcagtacttttcagagcctttaatatgctattttaaatttggatctgtaagaggataatttagaatctattaatcacatctgtattgtattgtattttcacaaagctggaccagttctgtgaaattccctttgagaaacactggtgtgaggccatctcttcttttcctctgccttcacacaaacaaaaactgcttctagatttctagttcttcatttcctctactcccagacagcagcaatggtgcaaattacattaaagtatttatcctaattgacactgaactcctttggcctgggatggttatagccaggggctatcaaagccattttctaatatattaacagttcttcttgaccaaagcaggtacacatgtccccaagcacgtgacgtgctgagaagagataggacatgcccatcaaagttctaaaggcataaacacaaacacacgtgcaagggaaaaaatactccccaaagaagcacacatctttaaaattcatggtaaattttacactgaaattggcattttactttttaaaacttaggaaaatggttttgctttgttgttgttactgttgttgttttgcttttatttgttttgaagtggggacagacagaaagatccaagcactgtgtcaggcttccctcgaaatgctactgtagctggatgtttcgtgtgtgtgccagagtgccagagtttggaatcactaaatgctgaagacttggggaacatgccagtttagattaactacctgccaggcattctctgaaatttccacctggggttgcacggtggatgaaccaacctttggaaagttcggttttgacaggtgggagtggaattttgaagcccggtgtcatcaacgcagtgctctgcacacctcttggaaataactcttccacatatggagagctgggacagatgaaattaaagctcttctttagaagatgtttcagttgtaagaaacagaaagcagctctagttgggggaaaaaatgcttgcattggcaggctctgggtggctcacagtactgaaagaagagctgagcaaccatttcaggcaggcaggaaatggggcactctggggcatctggaagtaggggcttatgtttttcttctctaagaggctgccattaaggtggctcagctctgttctagctcctaggagtgagatgagattggctcacctaggctgggggtctcccttttgagtggggagggggaagggaagtttgccagtcatcatttctggaaccctagtcctgtgtgtgaggattttttctaaggaaagaagaaccttcccaagtggggtcaactccagatgtgaagaggaagcagataactatgaatgtgacccccatttgttctgaaccggaaagaatgggacatatcttaagtgataagtcatgggaggtgagaaaacggtgagtttaaggaaaagaacagtatcttcaaaatggtaaagctgaggggaacgtgccagaagcttcaggaagatggagtatgcccagacaacaaggaccatggctttagctagaaaagctctttaggagaagggcaattcaatagggctaaatagattgactaaagagctggctcttctgctcaaattctaacccactaagaagacatgtgagccctaaaggagactgcaaacagcctgctctacatttttatgtgactgatgtgccatttttgtgttttaattaaacaagtttggtgctgtcacagatgctgttcattgtcaacccaatggccattgtttaacccttttcccaagcaggtagaatctttctcctgcaaagagactgaaaatgctggatattcactcttccaagcccccatgacttctgggggtggccatccaacatcattctagccaatgcaagtaaaggggatatttctcaggggtgctgggaaacattttcttccctgataaacagaccgacaagtagagttatcttgtcacatgactgggctcctttctttcttcgtttgagcatgatgggatgaggatgtgattcttggagatgctgcagccaccttgtgatcatgagggagaatcactggcatactgaagatggtggagcaagagcatgggaaagcctgggggctttgagaccaccaacctctcaatttcttattatttttaatcttaataaacccctactgattaagcttctttcactggggtgtattgttggttgcattctaatgtatctcaatggaaacagttgcccaaggtaaaatcaaacaatctcatataaaatgaagattcttgacttctcttgggggaatatgtgtttgggctgggcgctgtggctcacacctgtaatccaggcactttgggaggccgaggcaggcggatcatgaggtcaggagatcaagaccatcctggctaacacagtgaaaccctgtctctactaaaaaatacaaaaaattagccgggcatggcagtgggtgcctgtagtcccagctactcaggaggctgaggcaggagaatggcgtgaacccaggaggccgagcttgcagtgagcagggatcgcgccactgcactccagcaccacttccctggggtgtgtgcttttagtcttccacagtctccactattccttaatgaccccacttgcctcattcactgtattctcttcctagtacctcaaggtatctgagcttgtggctgccgatctctaacatggactctgagtaagtttactcaaagaggaagaaattccgacatcccacagctcccagggtgggctcggactcttcacactgtgtgtaacctgcttttccaaagagactgaattaggaaccccacatccaaaaaaaaatcaggggttgaggaataaacgttctcattatggccatttaattggtacactgtgatgttatatttacttcacgtgaatagagcatgaaattgaaacataaggatctgtaaaaatgcctgccttttgtgaactggcttacactgttcattatggctcctgaggatcctaccaccagcttcatgttattacatcatctgtaatttgaattatattttaatcaaagcttttacatggccagtattaggattttccatgtaattatcagcattagtaatactctgttgttactttgcagagtacttcctggccatttatctttaaataaaattatttatattaaatttacacttgatggtccagaattttaagtctttattaactgaagtacaacccttttcctttcctcttgctcagataaaactagaatcaaataagaatgtgggccacatcaggatggggtttttttttttaacagtagcaaaggatctttttcctacatttctattttgggctttatttttgaaaattatagagtttttagttaaattagagtattgtttaattttctaattttaaatgaattttagctcagaatttaaaattatgtcttttcaattgctatgatttatctcttaaaatatctcacattcatcttcaaagttgcttgccaatgtaactgctataatttttaaaaaatcaatggcttgactttggatgaaagtcaattcaagcctccccctctcccactccatccaggggacaatcacatgaccgtgccaaagccagtttggaaggaccagggctggagagggctgcactggggctcatggagcatagtcagtggtacatgcactccaagcttaagcccatggagcttaacagaaatggctgatcaaagatattctgatgcttctaacttgcacacgcagcccagggctgataagctgaccatttaggcagccacctgagtctctcaaaatgcagtctgttatgctaactgcccaaaagcaacactcttggccaggtgcagtggctcacgcttataatcccagcactttgggaggccgaggtgggcagatcacttgaggctaggagtccgagaccagcctggccaacgtggtgaaaccccgtgtctactaaaaatacaaaaattagccaggtgtggtggcgggcacctgtagtcctagctacttgggaggctgaggcacgagaatagcttgaacccagaggcaaaggttgcagtgagccaagatcacgccactgcactccagtgcagtctcgacacagcgagactccatctcaaaaaaaaaaaaaaaaaagtgacactctggatagcaaagatgcatcacctcgtagcacccaggcccaggaatctgaacaaccacatggtacatccaatcagaattggatgaaggggatgctccttgccttgaaaaaactagctggccaaggagcagcgtgctctatactcagactgaaaaaggttcatattgactggctgtattcaacaatgcaaagagctgagcgagagacacagcacattcctgattctgttcttgtaccttctaccagagtcctatcatgctgaaatattgccagctagataggaacaggaacacaccaccacttggagaatccttagagcagagctctgcaaaactcagatcctaaaggggaaaaattctcagcctgaagttgcttcttatccccaatggccactcagccactcccttgagatgagccccaggcatgcggtttctgatctgtgagatcggtcacatcacttcttgcagaagagccaagtaaagcccccgtgccccaaaaattcactgtatgaggcagagctacagaagtggctccataaacttagactggaagatgggaaggatattgtgcccatgaaccctcaggcaactgctgtgacctcatcccccacacatgcactcatgcatcttcatgctcattgtgtttggtggaagtctgtgcatgaagttattaattttatttgcttccagattcaatgattcaaaagccctggaaatgctcaagctgtcactccaagtttcaaatctattttagagacgtgggctatgagaagctgatggctcagaaaggttctgagcctttgcttccaagctcagcacctggaatgacctacagacagagctggctttgggtctctgagaaacctgctgcatctccaaatgacttgttgcgctgggtggccaacaccaagtcttccacgtgggaggttttattatgttttacaaccatgaaaacataggaaggtggctgttacagcaaacatttcagatagacgaatcggccaagctccccaaaccccaccttcacagcctcttccacacgtctctcagagattgttgtccttcacttgcaaattcaaggatgttggaagtagacatttaaagtagcaggaacaccatcagtgaaacagaagcagaagtacgatgactttgagaaacaactgatgaaaaatacactacagaaaaccatttctattgtgttatgatgtcagggtggcagatgtgcccagggcttagtgtccatcctcccaggacactggtcataccgggccttcggtgatcccctccagaggcaagctgggtgcgctgtcagctgtgggcctctcctctttcttcagtgaggctgggactcgcagactaacgtagggtttatggcaagctgtgttggccagaggaggatagtgctgtctgtagcaaatgtatgcaaaaatgaggccgatgactccacccacaaaggaatcttgccagtgatgcttgtagtcgcacatgcgggacagggcaatcatcatggcgcagtacaagggcaggatggcagcacagagccgccagctctttccccgcccactctcggtgaagcagtgcagcttgcccgccaagtagaacgtcgtgaagccaaggcccgaaaaggcaaaggaggaatggatgctggggaagcttttgcggccctcggacaccagatcggggtcacctgtgcaatgcatttccgagttcatcactccatctggaaagcagcggtaaaagaaatcggggcgaggttttatgaccttgggaaggtcagttggtctcccccagcttcagtttccacatctgtagaagggggaaatcaatactgacccaaa

SEQ ID NO: 8328 - RNA, 7026 nt, Homo sapiens
  source 1..7026: mol_type = other RNA
aaaaaccacaattacttttgcaccaacctaatacattctaaatcactaaaccattgtaaaaggtcctataaggttggtgttattcctgttttgcagatgcagacactgaggctcacgagtgtgaagcagtttgctcaaggttaagtggcagagatgttggcagggctgcctggccccattctaagtggttctttcctccgtgctatccttgaagagcactctgtatgtggatgaaagcaggtgtttagcatcacagtgtatgatgtccccagggcatctgtgactgtgttctatgtcagtctggggatctttccagggcaaaaaaagaagagacaccacatagcaagaagagacgccacccatcacacagcatattttgtgttaagatgttactctcattgtctgtcactgagagcattattattcctgatcatttacagaatccactggcaagcagtcatggcagcaccactgcaagcactgggatgaaaagatgtcatcaaagaataaaaaggggcaccgggtgcagtggctcacgcctgtaatcctagcactttgggaggatcacaaggtcaggagattgagatcatcctggctaacacggtgaaaccccgtctctaccaaaaatacaaaaaaattagtcgggtgtggtggcgggcacctgtagtcccagctactcaggagattgaggcaggagaatggggtgaacccgggaggtggagcttgcagtgagccgagatcgcaccactgcactccagccttggtgacagagtgagactctgtctcaaaaaaaaaaaaaaaaaaaaaaagaataaaaaggggcatgtttcttcacggcagtacttttcagagcctttaatatgctattttaaatttggatctgtaagaggataatttagaatctattaatcacatctgtattgtattgtattttcacaaagctggaccagttctgtgaaattccctttgagaaacactggtgtgaggccatctcttcttttcctctgccttcacacaaacaaaaactgcttctagatttctagttcttcatttcctctactcccagacagcagcaatggtgcaaattacattaaagtatttatcctaattgacactgaactcctttggcctgggatggttatagccaggggctatcaaagccattttctaatatattaacagttcttcttgaccaaagcaggtacacatgtccccaagcacgtgacgtgctgagaagagataggacatgcccatcaaagttctaaaggcataaacacaaacacacgtgcaagggaaaaaatactccccaaagaagcacacatctttaaaattcatggtaaattttacactgaaattggcattttactttttaaaacttaggaaaatggttttgctttgttgttgttactgttgttgttttgcttttatttgttttgaagtggggacagacagaaagatccaagcactgtgtcaggcttccctcgaaatgctactgtagctggatgtttcgtgtgtgtgccagagtgccagagtttggaatcactaaatgctgaagacttggggaacatgccagtttagattaactacctgccaggcattctctgaaatttccacctggggttgcacggtggatgaaccaacctttggaaagttcggttttgacaggtgggagtggaattttgaagcccggtgtcatcaacgcagtgctctgcacacctcttggaaataactcttccacatatggagagctgggacagatgaaattaaagctcttctttagaagatgtttcagttgtaagaaacagaaagcagctctagttgggggaaaaaatgcttgcattggcaggctctgggtggctcacagtactgaaagaagagctgagcaaccatttcaggcaggcaggaaatggggcactctggggcatctggaagtaggggcttatgtttttcttctctaagaggctgccattaaggtggctcagctctgttctagctcctaggagtgagatgagattggctcacctaggctgggggtctcccttttgagtggggagggggaagggaagtttgccagtcatcatttctggaaccctagtcctgtgtgtgaggattttttctaaggaaagaagaaccttcccaagtggggtcaactccagatgtgaagaggaagcagataactatgaatgtgacccccatttgttctgaaccggaaagaatgggacatatcttaagtgataagtcatgggaggtgagaaaacggtgagtttaaggaaaagaacagtatcttcaaaatggtaaagctgaggggaacgtgccagaagcttcaggaagatggagtatgcccagacaacaaggaccatggctttagctagaaaagctctttaggagaagggcaattcaatagggctaaatagattgactaaagagctggctcttctgctcaaattctaacccactaagaagacatgtgagccctaaaggagactgcaaacagcctgctctacatttttatgtgactgatgtgccatttttgtgttttaattaaacaagtttggtgctgtcacagatgctgttcattgtcaacccaatggccattgtttaacccttttcccaagcaggtagaatctttctcctgcaaagagactgaaaatgctggatattcactcttccaagcccccatgacttctgggggtggccatccaacatcattctagccaatgcaagtaaaggggatatttctcaggggtgctgggaaacattttcttccctgataaacagaccgacaagtagagttatcttgtcacatgactgggctcctttctttcttcgtttgagcatgatgggatgaggatgtgattcttggagatgctgcagccaccttgtgatcatgagggagaatcactggcatactgaagatggtggagcaagagcatgggaaagcctgggggctttgagaccaccaacctctcaatttcttattatttttaatcttaataaacccctactgattaagcttctttcactggggtgtattgttggttgcattctaatgtatctcaatggaaacagttgcccaaggtaaaatcaaacaatctcatataaaatgaagattcttgacttctcttgggggaatatgtgtttgggctgggcgctgtggctcacacctgtaatccaggcactttgggaggccgaggcaggcggatcatgaggtcaggagatcaagaccatcctggctaacacagtgaaaccctgtctctactaaaaaatacaaaaaattagccgggcatggcagtgggtgcctgtagtcccagctactcaggaggctgaggcaggagaatggcgtgaacccaggaggccgagcttgcagtgagcagggatcgcgccactgcactccagcaccacttccctggggtgtgtgcttttagtcttccacagtctccactattccttaatgaccccacttgcctcattcactgtattctcttcctagtacctcaaggtatctgagcttgtggctgccgatctctaacatggactctgagtaagtttactcaaagaggaagaaattccgacatcccacagctcccagggtgggctcggactcttcacactgtgtgtaacctgcttttccaaagagactgaattaggaaccccacatccaaaaaaaaatcaggggttgaggaataaacgttctcattatggccatttaattggtacactgtgatgttatatttacttcacgtgaatagagcatgaaattgaaacataaggatctgtaaaaatgcctgccttttgtgaactggcttacactgttcattatggctcctgaggatcctaccaccagcttcatgttattacatcatctgtaatttgaattatattttaatcaaagcttttacatggccagtattaggattttccatgtaattatcagcattagtaatactctgttgttactttgcagagtacttcctggccatttatctttaaataaaattatttatattaaatttacacttgatggtccagaattttaagtctttattaactgaagtacaacccttttcctttcctcttgctcagataaaactagaatcaaataagaatgtgggccacatcaggatggggtttttttttttaacagtagcaaaggatctttttcctacatttctattttgggctttatttttgaaaattatagagtttttagttaaattagagtattgtttaattttctaattttaaatgaattttagctcagaatttaaaattatgtcttttcaattgctatgatttatctcttaaaatatctcacattcatcttcaaagttgcttgccaatgtaactgctataatttttaaaaaatcaatggcttgactttggatgaaagtcaattcaagcctccccctctcccactccatccaggggacaatcacatgaccgtgccaaagccagtttggaaggaccagggctggagagggctgcactggggctcatggagcatagtcagtggtacatgcactccaagcttaagcccatggagcttaacagaaatggctgatcaaagatattctgatgcttctaacttgcacacgcagcccagggctgataagctgaccatttaggcagccacctgagtctctcaaaatgcagtctgttatgctaactgcccaaaagcaacactcttggccaggtgcagtggctcacgcttataatcccagcactttgggaggccgaggtgggcagatcacttgaggctaggagtccgagaccagcctggccaacgtggtgaaaccccgtgtctactaaaaatacaaaaattagccaggtgtggtggcgggcacctgtagtcctagctacttgggaggctgaggcacgagaatagcttgaacccagaggcaaaggttgcagtgagccaagatcacgccactgcactccagtgcagtctcgacacagcgagactccatctcaaaaaaaaaaaaaaaaaagtgacactctggatagcaaagatgcatcacctcgtagcacccaggcccaggaatctgaacaaccacatggtacatccaatcagaattggatgaaggggatgctccttgccttgaaaaaactagctggccaaggagcagcgtgctctatactcagactgaaaaaggttcatattgactggctgtattcaacaatgcaaagagctgagcgagagacacagcacattcctgattctgttcttgtaccttctaccagagtcctatcatgctgaaatattgccagctagataggaacaggaacacaccaccacttggagaatccttagagcagagctctgcaaaactcagatcctaaaggggaaaaattctcagcctgaagttgcttcttatccccaatggccactcagccactcccttgagatgagccccaggcatgcggtttctgatctgtgagatcggtcacatcacttcttgcagaagagccaagtaaagcccccgtgccccaaaaattcactgtatgaggcagagctacagaagtggctccataaacttagactggaagatgggaaggatattgtgcccatgaaccctcaggcaactgctgtgacctcatcccccacacatgcactcatgcatcttcatgctcattgtgtttggtggaagtctgtgcatgaagttattaattttatttgcttccagattcaatgattcaaaagccctggaaatgctcaagctgtcactccaagtttcaaatctattttagagacgtgggctatgagaagctgatggctcagaaaggttctgagcctttgcttccaagctcagcacctggaatgacctacagacagagctggctttgggtctctgagaaacctgctgcatctccaaatgacttgttgcgctgggtggccaacaccaagtcttccacgtgggaggttttattatgttttacaaccatgaaaacataggaaggtggctgttacagcaaacatttcagatagacgaatcggccaagctccccaaaccccaccttcacagcctcttccacacgtctctcagagattgttgtccttcacttgcaaattcaaggatgttggaagtagacatttaaagtagcaggaacaccatcagtgaaacagaagcagaagtacgatgactttgagaaacaactgatgaaaaatacactacagaaaaccatttctattgtgttatgatgtcagggtggcagatgtgcccagggcttagtgtccatcctcccaggacactggtcataccgggccttcggtgatcccctccagaggcaagctgggtgcgctgtcagctgtgggcctctcctctttcttcagtgaggctgggactcgcagactaacgtagggtttatggcaagctgtgttggccagaggaggatagtgctgtctgtagcaaatgtatgcaaaaatgaggccgatgactccacccacaaaggaatcttgccagtgatgcttgtagtcgcacatgcgggacagggcaatcatcatggcgcagtacaagggcaggatggcagcacagagccgccagctctttccccgcccactctcggtgaagcagtgcagcttgcccgccaagtagaacgtcgtgaagccaaggcccgaaaaggcaaaggaggaatggatgctggggaagcttttgcggccctcggacaccagatcggggtcacctgtgcaatgcatttccgagttcatcactccatcttcccactattaatttaatagtgtttgtgcagactccattcaaagcaagagccaaggacaccgaaacatgaggcgggtaggtatgttatctgattgcaccaaaggatttttatagagccagatctcttctggctggatgactctctggaacggatccaaaaactctgtaaaaacgaagactccgaagagcagggctcgcaccccgatctcaatggccagctcccgcatggtgcggccggagcagctcccgcggcgtcagctggtgctctccgcggctcccgcagctcggccggcgccggctcgccagaccc

SEQ ID NO: 8329 - RNA, 6978 nt, Homo sapiens
  source 1..6978: mol_type = other RNA
aaaaaccacaattacttttgcaccaacctaatacattctaaatcactaaaccattgtaaaaggtcctataaggttggtgttattcctgttttgcagatgcagacactgaggctcacgagtgtgaagcagtttgctcaaggttaagtggcagagatgttggcagggctgcctggccccattctaagtggttctttcctccgtgctatccttgaagagcactctgtatgtggatgaaagcaggtgtttagcatcacagtgtatgatgtccccagggcatctgtgactgtgttctatgtcagtctggggatctttccagggcaaaaaaagaagagacaccacatagcaagaagagacgccacccatcacacagcatattttgtgttaagatgttactctcattgtctgtcactgagagcattattattcctgatcatttacagaatccactggcaagcagtcatggcagcaccactgcaagcactgggatgaaaagatgtcatcaaagaataaaaaggggcaccgggtgcagtggctcacgcctgtaatcctagcactttgggaggatcacaaggtcaggagattgagatcatcctggctaacacggtgaaaccccgtctctaccaaaaatacaaaaaaattagtcgggtgtggtggcgggcacctgtagtcccagctactcaggagattgaggcaggagaatggggtgaacccgggaggtggagcttgcagtgagccgagatcgcaccactgcactccagccttggtgacagagtgagactctgtctcaaaaaaaaaaaaaaaaaaaaaaagaataaaaaggggcatgtttcttcacggcagtacttttcagagcctttaatatgctattttaaatttggatctgtaagaggataatttagaatctattaatcacatctgtattgtattgtattttcacaaagctggaccagttctgtgaaattccctttgagaaacactggtgtgaggccatctcttcttttcctctgccttcacacaaacaaaaactgcttctagatttctagttcttcatttcctctactcccagacagcagcaatggtgcaaattacattaaagtatttatcctaattgacactgaactcctttggcctgggatggttatagccaggggctatcaaagccattttctaatatattaacagttcttcttgaccaaagcaggtacacatgtccccaagcacgtgacgtgctgagaagagataggacatgcccatcaaagttctaaaggcataaacacaaacacacgtgcaagggaaaaaatactccccaaagaagcacacatctttaaaattcatggtaaattttacactgaaattggcattttactttttaaaacttaggaaaatggttttgctttgttgttgttactgttgttgttttgcttttatttgttttgaagtggggacagacagaaagatccaagcactgtgtcaggcttccctcgaaatgctactgtagctggatgtttcgtgtgtgtgccagagtgccagagtttggaatcactaaatgctgaagacttggggaacatgccagtttagattaactacctgccaggcattctctgaaatttccacctggggttgcacggtggatgaaccaacctttggaaagttcggttttgacaggtgggagtggaattttgaagcccggtgtcatcaacgcagtgctctgcacacctcttggaaataactcttccacatatggagagctgggacagatgaaattaaagctcttctttagaagatgtttcagttgtaagaaacagaaagcagctctagttgggggaaaaaatgcttgcattggcaggctctgggtggctcacagtactgaaagaagagctgagcaaccatttcaggcaggcaggaaatggggcactctggggcatctggaagtaggggcttatgtttttcttctctaagaggctgccattaaggtggctcagctctgttctagctcctaggagtgagatgagattggctcacctaggctgggggtctcccttttgagtggggagggggaagggaagtttgccagtcatcatttctggaaccctagtcctgtgtgtgaggattttttctaaggaaagaagaaccttcccaagtggggtcaactccagatgtgaagaggaagcagataactatgaatgtgacccccatttgttctgaaccggaaagaatgggacatatcttaagtgataagtcatgggaggtgagaaaacggtgagtttaaggaaaagaacagtatcttcaaaatggtaaagctgaggggaacgtgccagaagcttcaggaagatggagtatgcccagacaacaaggaccatggctttagctagaaaagctctttaggagaagggcaattcaatagggctaaatagattgactaaagagctggctcttctgctcaaattctaacccactaagaagacatgtgagccctaaaggagactgcaaacagcctgctctacatttttatgtgactgatgtgccatttttgtgttttaattaaacaagtttggtgctgtcacagatgctgttcattgtcaacccaatggccattgtttaacccttttcccaagcaggtagaatctttctcctgcaaagagactgaaaatgctggatattcactcttccaagcccccatgacttctgggggtggccatccaacatcattctagccaatgcaagtaaaggggatatttctcaggggtgctgggaaacattttcttccctgataaacagaccgacaagtagagttatcttgtcacatgactgggctcctttctttcttcgtttgagcatgatgggatgaggatgtgattcttggagatgctgcagccaccttgtgatcatgagggagaatcactggcatactgaagatggtggagcaagagcatgggaaagcctgggggctttgagaccaccaacctctcaatttcttattatttttaatcttaataaacccctactgattaagcttctttcactggggtgtattgttggttgcattctaatgtatctcaatggaaacagttgcccaaggtaaaatcaaacaatctcatataaaatgaagattcttgacttctcttgggggaatatgtgtttgggctgggcgctgtggctcacacctgtaatccaggcactttgggaggccgaggcaggcggatcatgaggtcaggagatcaagaccatcctggctaacacagtgaaaccctgtctctactaaaaaatacaaaaaattagccgggcatggcagtgggtgcctgtagtcccagctactcaggaggctgaggcaggagaatggcgtgaacccaggaggccgagcttgcagtgagcagggatcgcgccactgcactccagcaccacttccctggggtgtgtgcttttagtcttccacagtctccactattccttaatgaccccacttgcctcattcactgtattctcttcctagtacctcaaggtatctgagcttgtggctgccgatctctaacatggactctgagtaagtttactcaaagaggaagaaattccgacatcccacagctcccagggtgggctcggactcttcacactgtgtgtaacctgcttttccaaagagactgaattaggaaccccacatccaaaaaaaaatcaggggttgaggaataaacgttctcattatggccatttaattggtacactgtgatgttatatttacttcacgtgaatagagcatgaaattgaaacataaggatctgtaaaaatgcctgccttttgtgaactggcttacactgttcattatggctcctgaggatcctaccaccagcttcatgttattacatcatctgtaatttgaattatattttaatcaaagcttttacatggccagtattaggattttccatgtaattatcagcattagtaatactctgttgttactttgcagagtacttcctggccatttatctttaaataaaattatttatattaaatttacacttgatggtccagaattttaagtctttattaactgaagtacaacccttttcctttcctcttgctcagataaaactagaatcaaataagaatgtgggccacatcaggatggggtttttttttttaacagtagcaaaggatctttttcctacatttctattttgggctttatttttgaaaattatagagtttttagttaaattagagtattgtttaattttctaattttaaatgaattttagctcagaatttaaaattatgtcttttcaattgctatgatttatctcttaaaatatctcacattcatcttcaaagttgcttgccaatgtaactgctataatttttaaaaaatcaatggcttgactttggatgaaagtcaattcaagcctccccctctcccactccatccaggggacaatcacatgaccgtgccaaagccagtttggaaggaccagggctggagagggctgcactggggctcatggagcatagtcagtggtacatgcactccaagcttaagcccatggagcttaacagaaatggctgatcaaagatattctgatgcttctaacttgcacacgcagcccagggctgataagctgaccatttaggcagccacctgagtctctcaaaatgcagtctgttatgctaactgcccaaaagcaacactcttggccaggtgcagtggctcacgcttataatcccagcactttgggaggccgaggtgggcagatcacttgaggctaggagtccgagaccagcctggccaacgtggtgaaaccccgtgtctactaaaaatacaaaaattagccaggtgtggtggcgggcacctgtagtcctagctacttgggaggctgaggcacgagaatagcttgaacccagaggcaaaggttgcagtgagccaagatcacgccactgcactccagtgcagtctcgacacagcgagactccatctcaaaaaaaaaaaaaaaaaagtgacactctggatagcaaagatgcatcacctcgtagcacccaggcccaggaatctgaacaaccacatggtacatccaatcagaattggatgaaggggatgctccttgccttgaaaaaactagctggccaaggagcagcgtgctctatactcagactgaaaaaggttcatattgactggctgtattcaacaatgcaaagagctgagcgagagacacagcacattcctgattctgttcttgtaccttctaccagagtcctatcatgctgaaatattgccagctagataggaacaggaacacaccaccacttggagaatccttagagcagagctctgcaaaactcagatcctaaaggggaaaaattctcagcctgaagttgcttcttatccccaatggccactcagccactcccttgagatgagccccaggcatgcggtttctgatctgtgagatcggtcacatcacttcttgcagaagagccaagtaaagcccccgtgccccaaaaattcactgtatgaggcagagctacagaagtggctccataaacttagactggaagatgggaaggatattgtgcccatgaaccctcaggcaactgctgtgacctcatcccccacacatgcactcatgcatcttcatgctcattgtgtttggtggaagtctgtgcatgaagttattaattttatttgcttccagattcaatgattcaaaagccctggaaatgctcaagctgtcactccaagtttcaaatctattttagagacgtgggctatgagaagctgatggctcagaaaggttctgagcctttgcttccaagctcagcacctggaatgacctacagacagagctggctttgggtctctgagaaacctgctgcatctccaaatgacttgttgcgctgggtggccaacaccaagtcttccacgtgggaggttttattatgttttacaaccatgaaaacataggaaggtggctgttacagcaaacatttcagatagacgaatcggccaagctccccaaaccccaccttcacagcctcttccacacgtctctcagagattgttgtccttcacttgcaaattcaaggatgttggaagtagacatttaaagtagcaggaacaccatcagtgaaacagaagcagaagtacgatgactttgagaaacaactgatgaaaaatacactacagaaaaccatttctattgtgttatgatgtcagggtggcagatgtgcccagggcttagtgtccatcctcccaggacactggtcataccgggccttcggtgatcccctccagaggcaagctgggtgcgctgtcagctgtgggcctctcctctttcttcagtgaggctgggactcgcagactaacgtagggtttatggcaagctgtgttggccagaggaggatagtgctgtctgtagcaaatgtatgcaaaaatgaggccgatgactccacccacaaaggaatcttgccagtgatgcttgtagtcgcacatgcgggacagggcaatcatcatggcgcagtacaagggcaggatggcagcacagagccgccagctctttccccgcccactctcggtgaagcagtgcagcttgcccgccaagtagaacgtcgtgaagccaaggcccgaaaaggcaaaggaggaatggatgctggggaagcttttgcggccctcggacaccagatcggggtcacctgtgcaatgcatttccgagttcatcactccatcttcccactattaatttaatagtgtttgtgcagactccattcaaagcaagagccaaggacaccgctaagaaggcttccttaatttcagtcttgtctgttcgccggataattttcaccacacaaataacagccaggggtgtgaggaaagaaattgcaaacatgaggcgggtaggtatgttatctgattgcaccaaaggatttttatagagccagatctcttctggctggatgactctctggaacggatccaaaaactctgtaaaa

SEQ ID NO: 8330 - RNA, 6798 nt, Homo sapiens
  source 1..6798: mol_type = other RNA
aaaaaccacaattacttttgcaccaacctaatacattctaaatcactaaaccattgtaaaaggtcctataaggttggtgttattcctgttttgcagatgcagacactgaggctcacgagtgtgaagcagtttgctcaaggttaagtggcagagatgttggcagggctgcctggccccattctaagtggttctttcctccgtgctatccttgaagagcactctgtatgtggatgaaagcaggtgtttagcatcacagtgtatgatgtccccagggcatctgtgactgtgttctatgtcagtctggggatctttccagggcaaaaaaagaagagacaccacatagcaagaagagacgccacccatcacacagcatattttgtgttaagatgttactctcattgtctgtcactgagagcattattattcctgatcatttacagaatccactggcaagcagtcatggcagcaccactgcaagcactgggatgaaaagatgtcatcaaagaataaaaaggggcaccgggtgcagtggctcacgcctgtaatcctagcactttgggaggatcacaaggtcaggagattgagatcatcctggctaacacggtgaaaccccgtctctaccaaaaatacaaaaaaattagtcgggtgtggtggcgggcacctgtagtcccagctactcaggagattgaggcaggagaatggggtgaacccgggaggtggagcttgcagtgagccgagatcgcaccactgcactccagccttggtgacagagtgagactctgtctcaaaaaaaaaaaaaaaaaaaaaaagaataaaaaggggcatgtttcttcacggcagtacttttcagagcctttaatatgctattttaaatttggatctgtaagaggataatttagaatctattaatcacatctgtattgtattgtattttcacaaagctggaccagttctgtgaaattccctttgagaaacactggtgtgaggccatctcttcttttcctctgccttcacacaaacaaaaactgcttctagatttctagttcttcatttcctctactcccagacagcagcaatggtgcaaattacattaaagtatttatcctaattgacactgaactcctttggcctgggatggttatagccaggggctatcaaagccattttctaatatattaacagttcttcttgaccaaagcaggtacacatgtccccaagcacgtgacgtgctgagaagagataggacatgcccatcaaagttctaaaggcataaacacaaacacacgtgcaagggaaaaaatactccccaaagaagcacacatctttaaaattcatggtaaattttacactgaaattggcattttactttttaaaacttaggaaaatggttttgctttgttgttgttactgttgttgttttgcttttatttgttttgaagtggggacagacagaaagatccaagcactgtgtcaggcttccctcgaaatgctactgtagctggatgtttcgtgtgtgtgccagagtgccagagtttggaatcactaaatgctgaagacttggggaacatgccagtttagattaactacctgccaggcattctctgaaatttccacctggggttgcacggtggatgaaccaacctttggaaagttcggttttgacaggtgggagtggaattttgaagcccggtgtcatcaacgcagtgctctgcacacctcttggaaataactcttccacatatggagagctgggacagatgaaattaaagctcttctttagaagatgtttcagttgtaagaaacagaaagcagctctagttgggggaaaaaatgcttgcattggcaggctctgggtggctcacagtactgaaagaagagctgagcaaccatttcaggcaggcaggaaatggggcactctggggcatctggaagtaggggcttatgtttttcttctctaagaggctgccattaaggtggctcagctctgttctagctcctaggagtgagatgagattggctcacctaggctgggggtctcccttttgagtggggagggggaagggaagtttgccagtcatcatttctggaaccctagtcctgtgtgtgaggattttttctaaggaaagaagaaccttcccaagtggggtcaactccagatgtgaagaggaagcagataactatgaatgtgacccccatttgttctgaaccggaaagaatgggacatatcttaagtgataagtcatgggaggtgagaaaacggtgagtttaaggaaaagaacagtatcttcaaaatggtaaagctgaggggaacgtgccagaagcttcaggaagatggagtatgcccagacaacaaggaccatggctttagctagaaaagctctttaggagaagggcaattcaatagggctaaatagattgactaaagagctggctcttctgctcaaattctaacccactaagaagacatgtgagccctaaaggagactgcaaacagcctgctctacatttttatgtgactgatgtgccatttttgtgttttaattaaacaagtttggtgctgtcacagatgctgttcattgtcaacccaatggccattgtttaacccttttcccaagcaggtagaatctttctcctgcaaagagactgaaaatgctggatattcactcttccaagcccccatgacttctgggggtggccatccaacatcattctagccaatgcaagtaaaggggatatttctcaggggtgctgggaaacattttcttccctgataaacagaccgacaagtagagttatcttgtcacatgactgggctcctttctttcttcgtttgagcatgatgggatgaggatgtgattcttggagatgctgcagccaccttgtgatcatgagggagaatcactggcatactgaagatggtggagcaagagcatgggaaagcctgggggctttgagaccaccaacctctcaatttcttattatttttaatcttaataaacccctactgattaagcttctttcactggggtgtattgttggttgcattctaatgtatctcaatggaaacagttgcccaaggtaaaatcaaacaatctcatataaaatgaagattcttgacttctcttgggggaatatgtgtttgggctgggcgctgtggctcacacctgtaatccaggcactttgggaggccgaggcaggcggatcatgaggtcaggagatcaagaccatcctggctaacacagtgaaaccctgtctctactaaaaaatacaaaaaattagccgggcatggcagtgggtgcctgtagtcccagctactcaggaggctgaggcaggagaatggcgtgaacccaggaggccgagcttgcagtgagcagggatcgcgccactgcactccagcaccacttccctggggtgtgtgcttttagtcttccacagtctccactattccttaatgaccccacttgcctcattcactgtattctcttcctagtacctcaaggtatctgagcttgtggctgccgatctctaacatggactctgagtaagtttactcaaagaggaagaaattccgacatcccacagctcccagggtgggctcggactcttcacactgtgtgtaacctgcttttccaaagagactgaattaggaaccccacatccaaaaaaaaatcaggggttgaggaataaacgttctcattatggccatttaattggtacactgtgatgttatatttacttcacgtgaatagagcatgaaattgaaacataaggatctgtaaaaatgcctgccttttgtgaactggcttacactgttcattatggctcctgaggatcctaccaccagcttcatgttattacatcatctgtaatttgaattatattttaatcaaagcttttacatggccagtattaggattttccatgtaattatcagcattagtaatactctgttgttactttgcagagtacttcctggccatttatctttaaataaaattatttatattaaatttacacttgatggtccagaattttaagtctttattaactgaagtacaacccttttcctttcctcttgctcagataaaactagaatcaaataagaatgtgggccacatcaggatggggtttttttttttaacagtagcaaaggatctttttcctacatttctattttgggctttatttttgaaaattatagagtttttagttaaattagagtattgtttaattttctaattttaaatgaattttagctcagaatttaaaattatgtcttttcaattgctatgatttatctcttaaaatatctcacattcatcttcaaagttgcttgccaatgtaactgctataatttttaaaaaatcaatggcttgactttggatgaaagtcaattcaagcctccccctctcccactccatccaggggacaatcacatgaccgtgccaaagccagtttggaaggaccagggctggagagggctgcactggggctcatggagcatagtcagtggtacatgcactccaagcttaagcccatggagcttaacagaaatggctgatcaaagatattctgatgcttctaacttgcacacgcagcccagggctgataagctgaccatttaggcagccacctgagtctctcaaaatgcagtctgttatgctaactgcccaaaagcaacactcttggccaggtgcagtggctcacgcttataatcccagcactttgggaggccgaggtgggcagatcacttgaggctaggagtccgagaccagcctggccaacgtggtgaaaccccgtgtctactaaaaatacaaaaattagccaggtgtggtggcgggcacctgtagtcctagctacttgggaggctgaggcacgagaatagcttgaacccagaggcaaaggttgcagtgagccaagatcacgccactgcactccagtgcagtctcgacacagcgagactccatctcaaaaaaaaaaaaaaaaaagtgacactctggatagcaaagatgcatcacctcgtagcacccaggcccaggaatctgaacaaccacatggtacatccaatcagaattggatgaaggggatgctccttgccttgaaaaaactagctggccaaggagcagcgtgctctatactcagactgaaaaaggttcatattgactggctgtattcaacaatgcaaagagctgagcgagagacacagcacattcctgattctgttcttgtaccttctaccagagtcctatcatgctgaaatattgccagctagataggaacaggaacacaccaccacttggagaatccttagagcagagctctgcaaaactcagatcctaaaggggaaaaattctcagcctgaagttgcttcttatccccaatggccactcagccactcccttgagatgagccccaggcatgcggtttctgatctgtgagatcggtcacatcacttcttgcagaagagccaagtaaagcccccgtgccccaaaaattcactgtatgaggcagagctacagaagtggctccataaacttagactggaagatgggaaggatattgtgcccatgaaccctcaggcaactgctgtgacctcatcccccacacatgcactcatgcatcttcatgctcattgtgtttggtggaagtctgtgcatgaagttattaattttatttgcttccagattcaatgattcaaaagccctggaaatgctcaagctgtcactccaagtttcaaatctattttagagacgtgggctatgagaagctgatggctcagaaaggttctgagcctttgcttccaagctcagcacctggaatgacctacagacagagctggctttgggtctctgagaaacctgctgcatctccaaatgacttgttgcgctgggtggccaacaccaagtcttccacgtgggaggttttattatgttttacaaccatgaaaacataggaaggtggctgttacagcaaacatttcagatagacgaatcggccaagctccccaaaccccaccttcacagcctcttccacacgtctctcagagattgttgtccttcacttgcaaattcaaggatgttggaagtagacatttaaagtagcaggaacaccatcagtgaaacagaagcagaagtacgatgactttgagaaacaactgatgaaaaatacactacagaaaaccatttctattgtgttatgatgtcagggtggcagatgtgcccagggcttagtgtccatcctcccaggacactggtcataccgggccttcggtgatcccctccagaggcaagctgggtgcgctgtcagctgtgggcctctcctctttcttcagtgaggctgggactcgcagactaacgtagggtttatggcaagctgtgttggccagaggaggatagtgctgtctgtagcaaatgtatgcaaaaatgaggccgatgactccacccacaaaggaatcttgccagtgatgcttgtagtcgcacatgcgggacagggcaatcatcatggcgcagtacaagggcaggatggcagcacagagccgccagctctttccccgcccactctcggtgaagcagtgcagcttgcccgccaagtagaacgtcgtgaagccaaggcccgaaaaggcaaaggaggaatggatgctggggaagcttttgcggccctcggacaccagatcggggtcacctgtgcaatgcatttccgagttcatcactccattttatgaccttgggaaggtcagttggtctcccccagcttcagtttccacatctgtagaagggggaaatcaatactgacccaaag

SEQ ID NO: 8331 - RNA, 37 nt, Homo sapiens
  source 1..37: mol_type = other RNA
aaaaaccacaattacttttgcaccaacctaatacctt

SEQ ID NO: 8332 - RNA, 44 nt, Homo sapiens
  source 1..44: mol_type = other RNA
aaaaaccacaattacttttgcaccaacctaatacgttagaactc

SEQ ID NO: 8333 - RNA, 5471 nt, Homo sapiens
  source 1..5471: mol_type = other RNA
aaaaaccacaattacttttgcaccaacctaatagaaagcatctctcaaactaacagacgtgtgcttccaaaagctaaatgctctgaaaagcttgtggggtagaaattatctcctttaagtcaacccttgagaggatcattgtctgcagtccagtcttgtgtttagggcttgtgcctcaggcaggctgacccaggaatgactgcattttgccttgaatagattccagcccgatggaaatgggtaaatgtgttactaggtgtaattttctaaagctggtagaggattcagggaaactagaaaaggataccaaatattttccactaaggcagggaccctctctggggccgttttatatgccacacaattgcattacaccttttaaaatcctcccaataatatcttgaggtttatcatattcttttaataaaatagataaccaaagcccaacaagtgtgaggacacaagtttggtcttctagaaagacacagaggcagcatttgaaaacagagcttctgacacctgaaaagagggcatctgacacctgaacttccttaagagctacacagctacctacgtgttctggggagtcatttaaaggcagccataaagttgtgatgaccaacatgtggctatctgaatttactgttctttgcaacatgccctcattgttttccaagttcacccatgtatatgagagcgataacaatccacataagtctcattttctcctcattttcaaatattcaagtgcctcatcttcttcccattttcaaatattcaaatgcagtcagtgtgatggttaagagcactgactccaaggacggatttcctgaatccaaaccatgtttctgccactagtaaaatgtatgactttggacaaattatttaaattgcctgtgtttaactttctccaactttgaaaaataggtacaatagtagtacttgccttcatggtcaacatgaggattaaatgagataatatatgtaaatacttagtaaaatgactggcaatacacgttcaataaatggtagttgttattttatgtaggagttatgttttatatcactgtaataatacacattttatatcactataaaatcattattttatggcagttaaattaaaaatagccttatacattgaacctactttgaggttcaatggaaagaaagtaaagatctggattctcaccatagctctggccaaatttgtgacttacgggccacgtggtcccaggtgaagcatctgacaactctatttcacttacttcatgtgtaaaaaggaagtctgcagttggtcctgatactacttccagatctttccaaatatatgcaatttaacatgtctatgagttatagaatgaatggaataattctagagaattttagaatctactcattacgtagcaagtgttatacttcgtattcatttgctcacttacatgtcacaaaaacattcccattttatagatgacactagtgaggtttagagaaattaagcaacttgtccaaaatccaaaattcatcctaaacacctaacttaaaacaaagcagtgcttgaaatgaaaagcagcagtagtggaagtgatggaagatgtgtgcaaatgtggctgattctgtgtgctggccctaacccgtgactctccctccatctgttcagctagggacccattaataaattcagtaacaatggtctttgttttaaccatccaagttaactaaaagttcattataaacagaaaatactaaatcaatttcctattagcaacaatggctattttcactgctaaaaagattagtaagtgtgagaagctaaatttaaatctacaattggcgagagattaaactaattcgggtctattttggaaggaagcttttaaaagaccagaactcaacttttcaagttaacaggattcaagctttcaatgctttcctttcttcttccctttaaccaaattcaactttgtagttttcatcttgtttttggaatctttccaggtcacctctgttaagaaacacaaggcccttggcactgaacttttgggaatgtgcccacatctgcctctgaatgtctgcctgcctacctttgatgccgcattcaacacctaacttaaaacaaagcagtgcttgaaacaaaaatctccttagagcacaatggtggacccattgctcaccagtcagtagcctcagtgataaatggcatgagcaaaaaggcctgaaaaccccaaatagttcaatattctaggacatgcccaactgattttcatttgggagaggaaaaggagcagtgcttcattatagggaaagaaaggaataaatgatgatgacagctgtgctgattcattgtttttttaaataattctgaaacattctaactatgttggtgtcacatagatccctcccagagctgaagaggttttgctcctatgtgtatatgtacttttatttataataaggttttcattttgacatgatactccaatttaaaaatgcagaattcttcttcacttcagttccttagaattgaatatgtcattcatcatcttggtggtcccagtaaaatgccctggaattctcatcccagttttcaatagttacgtattaatccatatggtaacaatattaccacaaccaaattcctgctaccagagacatcagattgttcagcttcagccccaggaatatttttttgtctctaagaagtaaatttcaatctgtaaattattggaagaggataaatataagctaaagcaatatcatttattgccctacaagtggggtgaccattcacataaggaggaaaagaagagattaaggcacatttctctttcaaacaagatgagcctctgcaaagcttggaggaattgagtcaaaaaaccactgtgactgaaaagcaggcagctgtagcagagctctgtgtatttgtctcttaacaatagctttattaatctcggaatctgaagatgtctgaggcaaagagttgcttctactggaaaatgaatggaaggaggagaatgtgctggggccttccattgtctgacagatcatctcctgttttgggatctgcccatgtgagattgagcctttcgagttcagaagaggcagggtgtggtggtagttaaaaacactgtaaggaatcaggtggcctcagttcttcctctgttttcttgttaattagcgggtgacttcaaaaacgtctaaagatttctggacttcagtttcctcattcaaaaaggaaagaatccaactagccaaaatcgaaggccacttttacttctaaagtttcaactgtgtgcaatgtagtcaagcaggactttctatactcctgggggagtaacagtagctatcatttcctaaacgcttttctgttccaggcacagtgctagggttttcttcatatggatgttcaacctcctggatgactctccaaggtagatttgattcctactttacagatgagaaaacccttacttgcttagagtcactcagctagtatgtgggaaacctgaagtgcaaacccagactgcccagctccaaaagctcgagctcttttgctaccatacagtgggtaccatccaaccctgctctgagaaaggcactgataagactgataatagtgacgctgaactagctggatgcccaagaggctggctatatgcagtgtctaggaacattaataggcaaaagtgatgacaaattcctacaaagtgggggtaacactaggattacctcatcgtctcatcattgtagggattcatgtttgtaaagtactaagatcaatgtgtttgttaaatttaaacaaataaataaaaacctgaggaaacagaaggctaatggatgtgtagcatacagggtcagggataaggtacagattggagatgattagaagtgggttgatccaggaacagagcaggaccagagagtcacaaaaggagcaacatgagagggccaggaccactgctacagagtgggctgcagtccctgacttgtttgtttacagggcctgcagtccttgagtggatctccatgttcaattcctcatcattgatttggggtatcacctgtcacatggtcttctggatgctaaggggccaattctgcagctcagggttctgtgttgtgccaatggcatgtgagctatggaaccccatggtggctgctacagaagcagctcctctcacctctgagatgcatgttcattccctttcccatctgccctgaggatattctccagtggtgcttgccgctgcagtgtttaccctaagataactttgccacaaaatatcttaattttattattatttttgcatcactctagtgtatcgactttggaacaaaagacatcatactctttatagcattctgtttttagtagtggtatctccgtttataaaatatagtaattctcgatcactgaaaatgtcaaatcctagaaaacatagcattcctacacgtgatgttaacatcattctcgaagagttattggccaaagattcatttgataaattcaattttttctgaaatagaggattctgatgattcggatgtttctgatgttagttcttcttagaaacaactctaagaacagtttttagattttattttcacattgaaaatgagttagatttgcttcagcctcaaatactgtgtttatgtacaattaaatgagcattggcagtgagctgcacttttttttttctaaacaggaaaagggttaacttgtatattcctttatttaggccgtggccaatatgttgtctgacttatggatatgcttgacagacacttagatcctgtagggaactggaagtcagagtgaaagtgaatgtgaggaaagtataacactgtctctggatgatcagaccaaatctccagggacaggagaaggaggtcagagtcacctggccactctcatgtttgtcggaagccaggaccatgcctttgagcttagtggagggatatccacagggctgtcaaaagagggcctcccgaggggagctctgcttaaatagctccactgggatgaggaaagagcttccaaggtcccctgctgggcttccttcagaaccccatgggttctgaactcaaatcaagtcttgaatgttagttttcaagcatgtggtgtgtttagacttggcgcctgttgctactgatgtttccacctccaccccacagttgttcattttcccagccctgtagctccacttctgtctgccccaggattttgctttgctgctcctgtatcaatgttaatggccaaagggaacactaggattcaacaaccgccaattcattgtcactgtacacacttgggattggacttctccatacggaatgctaaaatttattctatcattaccatcaacaagagcctatttgtgaatctcacatgtgtattgtgcacttaaaggtttccaaatttaaaagatacatatagatatggtgcagaatatgtcattaaaaataattaa

SEQ ID NO: 8334 - RNA, 43 nt, Homo sapiens
  source 1..43: mol_type = other RNA
aaaaaccacaattacttttgcaccaacctaatagatgccaatg

SEQ ID NO: 8335 - RNA, 35 nt, Homo sapiens
  source 1..35: mol_type = other RNA
aaaaaccacaattacttttgcaccaacctaatagc

SEQ ID NO: 8336 - RNA, 2944 nt, Homo sapiens
  source 1..2944: mol_type = other RNA
aaaaaccacaattacttttgcaccaacctaatagctatctatctagggctagggctatctatctagggctagggctatcgatctagggctgttaaaagtgtattcaacccaaggtatctaatacacatagtttataatggcatgtgagaaataaactccttccttaaaagattaaatattacttctttttccaaaacctaaattgtttcatcaatttccactagaaatgtatcttcaataagcaggctgggcacagtagctcatgcctataatcccagcactttcgacggccaagttgggaggactgcctgagctcaagagttcgagaccagctggggcaatatagtgagactctgtctctatttaataaataaaaaggataattaaaaaaataataagcataatggtgtagacctggtaaatcttttgacagcaacgtttataacccacatgccatgtatttcactacattcataaaggggcttggggatttatccagaatgacataccattcatttcaaaataacatacatcttttctctagacagctaagaatatttatagttgttaaagcaaaaagaaattcttggtaacaagttcttggtgtatggattgctttggctttgatggaaatatctactttctccaaagattggtccctgggcctcaaagcatttaccccaagaaataactgctatgacttaggtcttcaaggcagcttccagtgctcgagctttctctgtgatgttcttctgaaaaggcatcataaaatcgtcgaagtccacctcatgtgtaaacctctctcgccgtagttccctcttcctgatcagctctgctgttgtggcttcaggactccaaatcctccgtggaataaatgtgatatccactttcttagtataaccactggtaatcaatgaattcagatgaaccacattacccttctgtactttctttccctctgatgtggttggtacaccataaattgatgacagcagttcctcttctttcttaatttcagggccttcagtcttcagtataggaggtgtcttgccttttagtttttgattttctgctggtttcggcaagttatctagcttttctttaatcagatcaattattctataatcagcatatgcctttgcaacgtccatggcactatgcccttttctattttccagctggaatttagcaccaatatcaagtaggtattttactgtatccagtctgcagctttcaatggctctatttaaaggagttgagttgttgattgaagctgcatctattaaagctccagattcaacaagaagctcaacaatgtcttgttggcctgcatggcatgcaaaatgaagtggagtccacagaaagttatctgttgcattaacgttagctcctttttcaagaagaaacttgaccacatctatgtttccacttgcacacgccgtcattagcggagttttgtaataattatccttcatatccacaggtattcctgattcaaaggcctttttcagagaagccagatcccctgctttggtgataatattaatgtttgaaaataccttctctgaatcatcaatgtaccaaacagagtcatcctgaatgggatgttctgggggatgatctctattaaaccggctgctatcagtgacattcttgtaggtctcaatcatgtaatacggtggcccaccatcctgccggcgtggaaacgcgtactcaggaatgacacagattggaaggggtaagacaaatttccctttctttccttttttgcccatccctttttcctttttcttaggtccatacgatcctaagacaaaagacttgtttaaatatctggttcctttaaagaattcattaatattgacccctcctccccgggttttctcatgaaggtgagcgatggcagccagctgttctgagcttgcataatcctgcctttcctccaacaccatcacgaagtcgttcttgctgatgcttccatcacccctgtctaaaaccgcaaaggcttcccggaggaaagcctcacgttctacggaccaatcgtgcagtctaagggcccacagtggatttggatttttggctcctggcctggctagtttattagcgattctctctgctcggcgtatttctttgcttgctgctttgaagccgccttccttagccacagccctgggcgttttatgatctaaattcttccatttcaggtcacatcctcgctgagctatatatttacagcagtctgcaaaaccacccatggcagcataatgaagtggtgtgttcccatttatcgaaatcagccccacgtctccattgtaggcaaaaagaagcttcaatatatcgaaaaagcctcctttagcagcaaaatgagcagcgtgatgcctgtcgttgtcaaatgcattcacttcacctcctctttccaatatgcctcgaactatttccactaccccttctcttgacgcttccattaaagctgtgcggcctgtggatgagttgattgcattaggattggctcctttttccaaaaatgtcaggcacacatctttaacatcatgtgcatcttcacaagctctaaggaatattggctttccttcataggtagaattgttgacatctgcaccatgttcaagggcgatcagagcacagcgataatgccgcttagtcggtaaaatgcagtaaaacaaaacacctcttagtcttccgggcgatcagaagccagggatctctgggcacctatgtgcctgggcctgctggggcgaccggggaggcccctgctctcgtcctctgacgctcagcgctggcccagccgcgaccttgggctcccggagcccggcggaggcgcccaggcgtgaatgatgtcccttgggtagggctggtgagctggcgcgcgggacagcagggctgggtgtatgtgtccatgggccccgggtccccggaaggcgagcgc

SEQ ID NO: 8337 - RNA, 3469 nt, Homo sapiens
  source 1..3469: mol_type = other RNA
aaaaaccacaattacttttgcaccaacctaatagctatctatctagggctagggctatctatctagggctagggctatcgatctagggctgttaaaagtgtattcaacccaaggtatctaatacacatagtttataatggcatgtgagaaataaactccttccttaaaagattaaatattacttctttttccaaaacctaaattgtttcatcaatttccactagaaatgtatcttcaataagcaggctgggcacagtagctcatgcctataatcccagcactttcgacggccaagttgggaggactgcctgagctcaagagttcgagaccagctggggcaatatagtgagactctgtctctatttaataaataaaaaggataattaaaaaaataataagcataatggtgtagacctggtaaatcttttgacagcaacgtttataacccacatgccatgtatttcactacattcataaaggggcttggggatttatccagaatgacataccattcatttcaaaataacatacatcttttctctagacagctaagaatatttatagttgttaaagcaaaaagaaattcttggtaacaagttcttggtgtatggattgctttggctttgatggaaatatctactttctccaaagattggtccctgggcctcaaagcatttaccccaagaaataactgctatgacttaggtcttcaaggcagcttccagtgctcgagctttctctgtgatgttcttctgaaaaggcatcataaaatcgtcgaagtccacctcatgtgtaaacctctctcgccgtagttccctcttcctgatcagctctgctgttgtggcttcaggactccaaatcctccgtggaataaatgtgatatccactttcttagtataaccactggtaatcaatgaattcagatgaaccacattacccttctgtactttctttccctctgatgtggttggtacaccataaattgatgacagcagttcctcttctttcttaatttcagggccttcagtcttcagtataggaggtgtcttgccttttagtttttgattttctgctggtttcggcaagttatctagcttttctttaatcagatcaattattctataatcagcatatgcctttgcaacgtccatggcactatgcccttttctattttccagctggaatttagcaccaatatcaagtaggtattttactgtatccagtctgcagctttcaatggctctatttaaaggagttgagttgttgattgaagctgcatctattaaagctccagattcaacaagaagctcaacaatgtcttgttggcctgcatggcatgcaaaatgaagtggagtccacagaaagttatctgttgcattaacgttagctcctttttcaagaagaaacttgaccacatctatgtttccacttgcacacgccgtcattagcggagttttgtaataattatccttcatatccacaggtattcctgattcaaaggcctttttcagagaagccagatcccctgctttggtgataatattaatgtttgaaaataccttctctgaatcatcaatgtaccaaacagagtcatcctgaatgggatgttctgggggatgatctctattaaaccggctgctatcagtgacattcttgtaggtctcaatcatgtaatacggtggcccaccatcctgccggcgtggaaacgcgtactcaggaatgacacagattggaaggggtaagacaaatttccctttctttccttttttgcccatccctttttcctttttcttaggtccatacgatcctaagacaaaagacttgtttaaatatctggttcctttaaagaattcattaatattgacccctcctccccgggttttctcatgaaggtgagcgatggcagccagctgttctgagcttgcataatcctgcctttcctccaacaccatcacgaagtcgttcttgctgatgcttccatcacccctgtctaaaaccgcaaaggcttcccggaggaaagcctcacgttctacggaccaatcgtgcagtctaagggcccacagtggatttggatttttggctcctggcctggctagtttattagcgattctctctgctcggcgtatttctttgcttgctgctttgaagccgccttccttagccacagccctgggcgttttatgatctaaattcttccatttcaggtcacatcctcgctgagctatatatttacagcagtctgcaaaaccacccatggcagcataatgaagtggtgtgttcccatttatcgaaatcagccccacgtctccattgtaggcaaaaagaagcttcaatatatcgaaaaagcctcctttagcagcaaaatgagcagcgtgatgcctgtcgttgtcaaatgcattcacttcacctcctctttccaatatgcctcgaactatttccactaccccttctcttgacgcttccattaaagctgtgcggcctgtggatgagttgattgcattaggattggctcctttttccaaaaatgtcaggcacacatctttaacatcatgtgcatcttcacaagctctaaggaatattggctttccttcataggtagaattgttgacatctgcaccatgttcaagggcgatcagagcacagcgataatgccgcttagtcggtaaaatgcagtaaaacaaaacaccttatcatagaactggcatacggcattgaggactgagtacacatgccttttccttcattatcaactatagtcatatcagcctttgcctttgctaatatttccattgacaattcatggcccagttctgcagccctcattgtgggagtacagcccattcggtcttgcacatcagggtgagcaccaaggtcaaggagaaagctgaccatatcaatatcattggaaactgaggctaagtgcaaagcactaagtccattaatgggttctgtataattgattagttcagggtatccaagcttggtcagcttctctatctgcttcttgtctttgttccgcacacattgaagaactttgtagatctgtaagttctcaagtctcttatctgctaaagccatgcttgaccagctccttgaaaatgctttctggaccaaaactaaagctcttagtcttccgggcgatcagaagccagggatctctgggcacctatgtgcctgggcctgctggggcgaccggggaggcccctgctctcgtcctctgacgctcagcgctggcccagccgcgaccttgggctcccggagcccggcggaggcgcccaggcgtgaatgatgtcccttgggtagggctggtgagctggcgcgcgggacagcagggctgggtgtatgtgtccatgggccccgggtccccggaaggcgagcgcgcgggcaggtgagcgcagggggcggggtggaagccggagggaccgggctgattgtgagcttccgccacgcagggcgcggctgccggggc

SEQ ID NO: 8338 - RNA, 3487 nt, Homo sapiens
  source 1..3487: mol_type = other RNA
aaaaaccacaattacttttgcaccaacctaatagctatctatctagggctagggctatctatctagggctagggctatcgatctagggctgttaaaagtgtattcaacccaaggtatctaatacacatagtttataatggcatgtgagaaataaactccttccttaaaagattaaatattacttctttttccaaaacctaaattgtttcatcaatttccactagaaatgtatcttcaataagcaggctgggcacagtagctcatgcctataatcccagcactttcgacggccaagttgggaggactgcctgagctcaagagttcgagaccagctggggcaatatagtgagactctgtctctatttaataaataaaaaggataattaaaaaaataataagcataatggtgtagacctggtaaatcttttgacagcaacgtttataacccacatgccatgtatttcactacattcataaaggggcttggggatttatccagaatgacataccattcatttcaaaataacatacatcttttctctagacagctaagaatatttatagttgttaaagcaaaaagaaattcttggtaacaagttcttggtgtatggattgctttggctttgatggaaatatctactttctccaaagattggtccctgggcctcaaagcatttaccccaagaaataactgctatgacttaggtcttcaaggcagcttccagtgctcgagctttctctgtgatgttcttctgaaaaggcatcataaaatcgtcgaagtccacctcatgtgtaaacctctctcgccgtagttccctcttcctgatcagctctgctgttgtggcttcaggactccaaatcctccgtggaataaatgtgatatccactttcttagtataaccactggtaatcaatgaattcagatgaaccacattacccttctgtactttctttccctctgatgtggttggtacaccataaattgatgacagcagttcctcttctttcttaatttcagggccttcagtcttcagtataggaggtgtcttgccttttagtttttgattttctgctggtttcggcaagttatctagcttttctttaatcagatcaattattctataatcagcatatgcctttgcaacgtccatggcactatgcccttttctattttccagctggaatttagcaccaatatcaagtaggtattttactgtatccagtctgcagctttcaatggctctatttaaaggagttgagttgttgattgaagctgcatctattaaagctccagattcaacaagaagctcaacaatgtcttgttggcctgcatggcatgcaaaatgaagtggagtccacagaaagttatctgttgcattaacgttagctcctttttcaagaagaaacttgaccacatctatgtttccacttgcacacgccgtcattagcggagttttgtaataattatccttcatatccacaggtattcctgattcaaaggcctttttcagagaagccagatcccctgctttggtgataatattaatgtttgaaaataccttctctgaatcatcaatgtaccaaacagagtcatcctgaatgggatgttctgggggatgatctctattaaaccggctgctatcagtgacattcttgtaggtctcaatcatgtaatacggtggcccaccatcctgccggcgtggaaacgcgtactcaggaatgacacagattggaaggggtaagacaaatttccctttctttccttttttgcccatccctttttcctttttcttaggtccatacgatcctaagacaaaagacttgtttaaatatctggttcctttaaagaattcattaatattgacccctcctccccgggttttctcatgaaggtgagcgatggcagccagctgttctgagcttgcataatcctgcctttcctccaacaccatcacgaagtcgttcttgctgatgcttccatcacccctgtctaaaaccgcaaaggcttcccggaggaaagcctcacgttctacggaccaatcgtgcagtctaagggcccacagtggatttggatttttggctcctggcctggctagtttattagcgattctctctgctcggcgtatttctttgcttgctgctttgaagccgccttccttagccacagccctgggcgttttatgatctaaattcttccatttcaggtcacatcctcgctgagctatatatttacagcagtctgcaaaaccacccatggcagcataatgaagtggtgtgttcccatttatcgaaatcagccccacgtctccattgtaggcaaaaagaagcttcaatatatcgaaaaagcctcctttagcagcaaaatgagcagcgtgatgcctgtcgttgtcaaatgcattcacttcacctcctctttccaatatgcctcgaactatttccactaccccttctcttgacgcttccattaaagctgtgcggcctgtggatgagttgattgcattaggattggctcctttttccaaaaatgtcaggcacacatctttaacatcatgtgcatcttcacaagctctaaggaatattggctttccttcataggtagaattgttgacatctgcaccatgttcaagggcgatcagagcacagcgataatgccgcttagtcggtaaaatgcagtaaaacaaaacaccttttccttcattatcaactatagtcatatcagcctttgcctttgctaatatttccattgacaattcatggcccagttctgcagccctcattgtgggagtacagcccattcggtcttgcacatcagggtgagcaccaaggtcaaggagaaagctgaccatatcaatatcattggaaactgaggctaagtgcaaagcactaagtccattaatgggttctgtataattgattagttcagggtatccaagcttggtcagcttctctatctgcttcttgtctttgttccgcacacattgaagaactttgtagatctgtaagttctcaagtctcttatctgctaaagccatgcttgaccagctccttgaaaatgctttctggaccaaaactaaagctagtttttacctcagtttctgcatctgtgaactggcaatagcaatggtgcccacttcatgggactcttagtcttccgggcgatcagaagccagggatctctgggcacctatgtgcctgggcctgctggggcgaccggggaggcccctgctctcgtcctctgacgctcagcgctggcccagccgcgaccttgggctcccggagcccggcggaggcgcccaggcgtgaatgatgtcccttgggtagggctggtgagctggcgcgcgggacagcagggctgggtgtatgtgtccatgggccccgggtccccggaaggcgagcgcgcgggcaggtgagcgcagggggcggggtggaagccggagggaccgggctgattgtgagcttccgccacgcagggcgcggctgccggggc

SEQ ID NO: 8339 - RNA, 3423 nt, Homo sapiens
  source 1..3423: mol_type = other RNA
aaaaaccacaattacttttgcaccaacctaatagctatctatctagggctagggctatctatctagggctagggctatcgatctagggctgttaaaagtgtattcaacccaaggtatctaatacacatagtttataatggcatgtgagaaataaactccttccttaaaagattaaatattacttctttttccaaaacctaaattgtttcatcaatttccactagaaatgtatcttcaataagcaggctgggcacagtagctcatgcctataatcccagcactttcgacggccaagttgggaggactgcctgagctcaagagttcgagaccagctggggcaatatagtgagactctgtctctatttaataaataaaaaggataattaaaaaaataataagcataatggtgtagacctggtaaatcttttgacagcaacgtttataacccacatgccatgtatttcactacattcataaaggggcttggggatttatccagaatgacataccattcatttcaaaataacatacatcttttctctagacagctaagaatatttatagttgttaaagcaaaaagaaattcttggtaacaagttcttggtgtatggattgctttggctttgatggaaatatctactttctccaaagattggtccctgggcctcaaagcatttaccccaagaaataactgctatgacttaggtcttcaaggcagcttccagtgctcgagctttctctgtgatgttcttctgaaaaggcatcataaaatcgtcgaagtccacctcatgtgtaaacctctctcgccgtagttccctcttcctgatcagctctgctgttgtggcttcaggactccaaatcctccgtggaataaatgtgatatccactttcttagtataaccactggtaatcaatgaattcagatgaaccacattacccttctgtactttctttccctctgatgtggttggtacaccataaattgatgacagcagttcctcttctttcttaatttcagggccttcagtcttcagtataggaggtgtcttgccttttagtttttgattttctgctggtttcggcaagttatctagcttttctttaatcagatcaattattctataatcagcatatgcctttgcaacgtccatggcactatgcccttttctattttccagctggaatttagcaccaatatcaagtaggtattttactgtatccagtctgcagctttcaatggctctatttaaaggagttgagttgttgattgaagctgcatctattaaagctccagattcaacaagaagctcaacaatgtcttgttggcctgcatggcatgcaaaatgaagtggagtccacagaaagttatctgttgcattaacgttagctcctttttcaagaagaaacttgaccacatctatgtttccacttgcacacgccgtcattagcggagttttgtaataattatccttcatatccacaggtattcctgattcaaaggcctttttcagagaagccagatcccctgctttggtgataatattaatgtttgaaaataccttctctgaatcatcaatgtaccaaacagagtcatcctgaatgggatgttctgggggatgatctctattaaaccggctgctatcagtgacattcttgtaggtctcaatcatgtaatacggtggcccaccatcctgccggcgtggaaacgcgtactcaggaatgacacagattggaaggggtaagacaaatttccctttctttccttttttgcccatccctttttcctttttcttaggtccatacgatcctaagacaaaagacttgtttaaatatctggttcctttaaagaattcattaatattgacccctcctccccgggttttctcatgaaggtgagcgatggcagccagctgttctgagcttgcataatcctgcctttcctccaacaccatcacgaagtcgttcttgctgatgcttccatcacccctgtctaaaaccgcaaaggcttcccggaggaaagcctcacgttctacggaccaatcgtgcagtctaagggcccacagtggatttggatttttggctcctggcctggctagtttattagcgattctctctgctcggcgtatttctttgcttgctgctttgaagccgccttccttagccacagccctgggcgttttatgatctaaattcttccatttcaggtcacatcctcgctgagctatatatttacagcagtctgcaaaaccacccatggcagcataatgaagtggtgtgttcccatttatcgaaatcagccccacgtctccattgtaggcaaaaagaagcttcaatatatcgaaaaagcctcctttagcagcaaaatgagcagcgtgatgcctgtcgttgtcaaatgcattcacttcacctcctctttccaatatgcctcgaactatttccactaccccttctcttgacgcttccattaaagctgtgcggcctgtggatgagttgattgcattaggattggctcctttttccaaaaatgtcaggcacacatctttaacatcatgtgcatcttcacaagctctaaggaatattggctttccttcataggtagaattgttgacatctgcaccatgttcaagggcgatcagagcacagcgataatgccgcttagtcggtaaaatgcagtaaaacaaaacaccttttccttcattatcaactatagtcatatcagcctttgcctttgctaatatttccattgacaattcatggcccagttctgcagccctcattgtgggagtacagcccattcggtcttgcacatcagggtgagcaccaaggtcaaggagaaagctgaccatatcaatatcattggaaactgaggctaagtgcaaagcactaagtccattaatgggttctgtataattgattagttcagggtatccaagcttggtcagcttctctatctgcttcttgtctttgttccgcacacattgaagaactttgtagatctgtaagttctcaagtctcttatctgctaaagccatgcttgaccagctccttgaaaatgctttctggaccaaaactaaagctcttagtcttccgggcgatcagaagccagggatctctgggcacctatgtgcctgggcctgctggggcgaccggggaggcccctgctctcgtcctctgacgctcagcgctggcccagccgcgaccttgggctcccggagcccggcggaggcgcccaggcgtgaatgatgtcccttgggtagggctggtgagctggcgcgcgggacagcagggctgggtgtatgtgtccatgggccccgggtccccggaaggcgagcgcgcgggcaggtgagcgcagggggcggggtggaagccggagggaccgggctgattgtgagcttccgccacgcagggcgcggctgccggggc

SEQ ID NO: 8340 - RNA, 57 nt, Homo sapiens
  source 1..57: mol_type = other RNA
aaaaaccacaattacttttgcaccaacctaatagggtgcaaacttcagagccatctg

SEQ ID NO: 8341 - RNA, 41 nt, Homo sapiens
  source 1..41: mol_type = other RNA
aaaaaccacaattacttttgcaccaacctaatagtttaggc

SEQ ID NO: 8342 - RNA, 1305 nt, Homo sapiens
  source 1..1305: mol_type = other RNA
aaaaaccacaattacttttgcaccaacctaatagtttattcccactaacatcccaattcctaaaatatttctggtcctttgggactgaaaattagttaatctgatgccaccaccttttcactgtcccgcactcacctcgcgtccttaccctgtgtagattctacagtccatcagtataaattcccttgcatacactttcaactctcttgcccttctctcctttcattgtattttcttgaaaaggacccagtcctggcttaattcaattccccacacatgatgtttgcacatgcctgcagcttaatatggcaggagaaaatacacatccaaaccaggcggtcctgatttaaactcgttatcactcacctccggtgagacttttgtgctattcagcaatcccactacatcttcctagtctatttactgccccattctccttgtttagttcctctcccaccctcctaaatgactattttgtatcttttcctacaatatctccttttccaccctcatttcaagttcatgcccttacctccaaattcactaagaaaattaaagcaacctgaaaatgcccctcctcattcccatcaccacattcacttgcatctgttagtgcaccctgcgtgctacagtacacacatgttccatcccctgagctaagacaatccctctacttatagtcttagtttcttccccttccttgaaagttttagtaattgtactttgtcccttctttccctgtcttttatcagttttttcctcctctcttggatcattctcaccagcaagtaaatgtgctatattatcttccattggaaaaatgaaaatcttttccttatatcatatctcgactccccttcaggacaaaatttaaaggactgactgcattcactgtctctaagaccactcctccacttccctttgaactcacttcagtcatgttttcactctcacaggttgagctagtcaaaaatcactgatgacctccatgttgctaagtctcagtccttatcttacttaatcagtcagcagttgatcattcccttctacttgagacagtctcttggcttgctttctacctccctgactactccttctcaatctcctttgtggattcttcctctgttccttaatctttaatatatgggcatgcctctgatctcaatcctcagacctcttttttttctatgttcactaattcctctgccacctcacttgttttgtcaatatttataggctgatgacttcaaagcttatatatctagccaacacccctcctcttagccccagactcccatatccagc

SEQ ID NO: 8343 - RNA, 43 nt, Homo sapiens
  source 1..43: mol_type = other RNA
aaaaaccacaattacttttgcaccaacctaatataacttgttt

SEQ ID NO: 8344 - RNA, 1548 nt, Homo sapiens
  source 1..1548: mol_type = other RNA
aaaaaccacaattacttttgcaccaacctaatattaatccctcgtgagattaagatctaaataaaaggaatacatatttattaatcctagactatattttggtatattaacataatagcaagagaacttttttatattaattcttaacatatttgaaaatttctgagaatagaattctataaaatgtctcaaactttatgttctcgcaacactttatactattaaaaattattgagtactccagacagcacttatttatctgagttatacctatcaagaattatatattggatattaaattttaaaatattcatttatttactttaaaataactatagcaaaacttctacacagataacatagacagaatttttttaataaaaactaactacattttccaaaacagaaaaagaactaatgagaagagtgacactgttacaaatttttacaaatctttttagtatttagaggaacagctagatccccatatttttttctgcatttgacctgttgtgatatgttgtctcagttgagctacatgaggagaatcctccagcaggtgtgtagttggaaaatgaaagacaacataaattccctaaaaggggtcttggggaccccaaaagatctcccacaatactttgagaactattgatacatatggtaaagaacattctcgcttgggtcagtcatcaattagtcttctccaaaaatagttaattattccaaagaaattccataaattctacttaaattctcaggaggaagaggaagaaaaggaggaggagggaagggagaagaaagaggaggaaaaggggtagcaggaggaggaaaagcatcagggaattgaacaattatatgacttgggtgtcttgctactgtcatatttaaagatcaaaattctacatttataaaaattagaagtcattacgtaattacagcagtataaaagacctctgagattgtaccttgaaaattaacagaataaactatcaataaccaaagaggctgaagaattatccaaaaaaatggcaaaaatacacttataaaaaggctcagaatttagaaggggagacccagcttcaatgtaagtagacctttcttttcatatatttacatacaaatatccctaagtaatacatacagacacacagacacaatctaacgaacatatatataatcctacctttacttgtattcatacctgtaaaatacttaaatttcaagaaactactgatagtataatcaaactacataactgttatagattaataacatttcctatcttctcaatatttttcaagaataactttaaatataatgaaaattatttaattcagaattcagatcattgaacccactaagaaaacggatagtatcaaatacacaatttaaaatttataaagcaaaccatgcaatcaattctcaaatatttaatctatactacccacatttaaaggaaatcataagaacttggcccagtgtggtggctcacacctgtaatcccagcactttgggaggctgaggcaggtggatcacgaggtcaggaga

SEQ ID NO: 8345 - RNA, 1139 nt, Homo sapiens
  source 1..1139: mol_type = other RNA
aaaaaccacaattacttttgcaccaacctaatattattgcaaaaggacccataaaaatgctctaccattagtccaacatcttatgcatattatctcattaatcttgagaaaacctgcagcagtcagggtaggctaggttacgtttcaataacagacaacctcagagtctcaggtgcttcaaaacacccaaagatttatttcttggtctatttacatatctgtcacacgttggcttgaggctccactctgccatctttactctaggactcaggtttaaagagctggtactatctggaacatttccagtctattaaaaggaagaagtgggagaaggggagggaaaagagacaaaccaggcatacggcaaagggagaagagtagcaaattacacacagacttttaaaacatatacctggaaattacaggttacttctgcttccattccactggctaaagcaagtcccaaggtcatatcttcacaaagatcatgtagattctcttttcatctgtaaggtgatagatcccccatttcttggatccaatgtcttcctctttcttgttttcttccccttattttcttagattatatcctgcagtagcttcaggtgctcggagaattcagcctccaaatccgcaggtcacaggtcagccaagttttaagaaacactccgggttagcgactcttcctctctgcaactcccacccctgcgccgagggcagcgggacacggccgggcggtccccaggggaagatgaggccctggacgccccgcgtgcgctggaggcccggaggccaaggccgaggccgaggccgaggccgggagcatgccagcggggtcgcgccaccgaaagctcctccggcctgggcccgccgtgccccgaggccgcgggcggaggctggagcaacgagcccaactctccctccgccccggggaggcggggtctccgcctttcccgcgttcgggcctcaccgccccctccgccttctctgagcccccgcgccacttccgctcctcgcagcggagccggtcccctagggctcgggtcgcacggagctgacccctaacgaaatggggccgcgccaagggcggtggtggctgctgctctggctgccgcccctggccacactgcccgtgcgcg

SEQ ID NO: 8346 - RNA, 1034 nt, Homo sapiens
  source 1..1034: mol_type = other RNA
aaaaaccacaattacttttgcaccaacctaatattattgcaaaaggacccataaaaatgctctaccattagtccaacatcttatgcatattatctcattaatcttgagaaaacctgcagcagtcagggtaggctaggttacgtttcaataacagacaacctcagagtctcaggtgcttcaaaacacccaaagatttatttcttggtctatttacatatctgtcacacgttggcttgaggctccactctgccatctttactctaggactcaggtttaaagagctggtactatctggaacatttccagtctggaaattacaggttacttctgcttccattccactggctaaagcaagtcccaaggtcatatcttcacaaagatcatgtagattctcttttcatctgtaaggtgatagatcccccatttcttggatccaatgtcttcctctttcttgttttcttccccttattttcttagattatatcctgcagtagcttcaggtgctcggagaattcagcctccaaatccgcaggtcacaggtcagccaagttttaagaaacactccgggttagcgactcttcctctctgcaactcccacccctgcgccgagggcagcgggacacggccgggcggtccccaggggaagatgaggccctggacgccccgcgtgcgctggaggcccggaggccaaggccgaggccgaggccgaggccgggagcatgccagcggggtcgcgccaccgaaagctcctccggcctgggcccgccgtgccccgaggccgcgggcggaggctggagcaacgagcccaactctccctccgccccggggaggcggggtctccgcctttcccgcgttcgggcctcaccgccccctccgccttctctgagcccccgcgccacttccgctcctcgcagcggagccggtcccctagggctcgggtcgcacggagctgacccctaacgaaatggggccgcgccaagggcggtggtggctgctgctctggctgccgcccctggccacactgcccgtgcgcg

SEQ ID NO: 8347 - RNA, 2676 nt, Homo sapiens
  source 1..2676: mol_type = other RNA
aaaaaccacaattacttttgcaccaacctaatcaaaccaccaggacttggttggctgagggtgggagatgtggggtctaggctgactccttgagttcctagctggagtgtctggcttgctggtactgccaatggaaagaagacatgttatatctgagatgtctatggggcatctaggaaatatcatctgaaagtcaggggacaggtctgggctgacgatacaaactggaatgtcatcagcatgtaaatgatgcttgaaaacatgagagtagatgaaatcatccaaggcaaccatatacaatcaaatagacccggattttgaatcttagatctgtcattcactatctgcgtgaccttgagtaagttactatacctttctgagcctcacttttctcatgtttaactgggtattttctttttgtaaaatggttaccacagtgctgggcccagggtaaacgctcgattattattattctagctccaatagttactagcagtaggaaattgaaggtgatgtttctgttcagtgagcctcaggctcccatttgtaactactgctcagtatacacctaccccacagaatggatgctcaggaaatggttgctaaataaacgaataaatctaaaaaatgaaaacaacaatacctacttaatacaatgggtgagagaagtaagcaatatttttacaaaactatataaagatccaggtaaaggttaataaactgtcttaggaaaagtgcctagtatttagaaggtaggcaataatgttagtcccgtcccttctccccttgcttttcaactcatcttccttttttttggattttaaatctctccccttctaccagctctttcctttcagattacaaacgtgctccagtctcccctaatctaatccccacttccttgagtcttctacattcctcaaatccttgttccatcatttttaaatttcaccaactgtaccccttctcaactcaaaacacttttcagtgaacgaactccaccttttgttttagaaaaaaaagttcccagcttactattacttttaaaaaaacaagtattatttacgtaattgttaaaacaggcctgtgtagagatatttcattttaacatatatatgtatgtacttttttctactgcagtaattcatttcaagagaaatttcattatgtatcttctacagagccctaaactgagagcgccagcgtattcaaataaaccctgaggtgtgggaggcttcgggccagttcctcattagtagcctcagcatgggggctctggagaccaacgcagaaggtcttccagggagagctgaaacgttcagataagtgagctctgggaagaaggggtagttggctggctctcgcaggctcacccctgggatagagcaaagagaacagacaggggagttctgagaggcaccagagctatctaaactcagggggatggaaccgagtgagcggcagcggtaattgagtttcagttacctgcagggtggtgaaatatagtagtaacttcatctgactgacatgggggaagtttagaggtgtccttggcatattcacagtgaaatccatcaccctttcaccatgttgggtgatagcaaccgtatggcgcttcctagtgacagccagtgtgcgttctgttaggcagcaccagcgcactgcagctaatgaagcacattcctgcaggcctgtctcctagggctctccgaatcctctgtctgcaaaggaacggcaccatgggaaaatctagcacagccagcatcagccatcacccaaactcaaaagcgtctttgaacggcagagacaggcccattttcctctctgcctggcccagggctggaaccgtcctcaggtcactttttgtgggtctgtacaaacgtgccgactggcagcgagccgctcttcacctgagcccggatttcagctcggtgctttaatgtgaagaccagggctctcaccgtccgccggtacggcccattaatgaggcgggagcagagatgaaacgtttcccgttcaatattttcaaccagtaggtgatccatctttaattccaaggcttctgagagtaatttctgagcatttttcctcaacgactcggttttgggatcacttctaacttcaatagaaggtctatttgaatgtttttcagtgaaagttttccactcagtgtaaacttctctggcaagagaagccacttctgaatctgagtgtttacgcatcttgttcacagtgtgacctatccttgttgattttaacacttccctggagggtattttcttctttaattcttgtaaggcttcaacaagattctctttggtttgatcaggaagctccagcatagttttccatctttttatgtcttctacaaccacaactctcttcagagattcaatcgtggcctgcttgtaaacctttcctccagaatctttcttctgagggctattctggattctaggcgttcgaatgacgaatttatccattgttaggggactccgactaccttgacgtgcttgcagcgtgttcaggaaaagcagccctggtagctgctgttggcgccctccagactgcaacctcgtaggctcccaagcccagtcgtctgtgttgaaactaaacagacgcttcctcccagggcggtagttcctctgaagaaactccgccggccctcgcgcctct

SEQ ID NO: 8348 - RNA, 39 nt, Homo sapiens
  source 1..39: mol_type = other RNA
aaaaaccacaattacttttgcaccaacctaggaattggt

SEQ ID NO: 8349 - RNA, 46 nt, Homo sapiens
  source 1..46: mol_type = other RNA
aaaaaccacaattacttttgcaccaacctagtagtaagcatcttct

SEQ ID NO: 8350 - RNA, 856 nt, Homo sapiens
  source 1..856: mol_type = other RNA
aaaaaccacaattacttttgcaccaacctataattgctccaaccacaccgaactctttgcagatcagtttgttcaaaaccatcttaatcaccgtctccaccctccccttccagcctcatctcctactatattccagcccaccccttgttcatctctttgatgacctaaaaattcagtcttcattcttttctctccaaacttttgctcaagtttcccccaaatatttagaatagctttaagttcatcttttctggaacattttccttaataaatccacctcattgcacacagctgcctagatgtagcctcagccccattcctctctctctttctcaatcccacttttgtgattattgtatgtatctgcatctgttttctgtttagcttccaatatgagtcctagagaacatctcatctccatcatatgtccaggaaaagcttgttgattgactgaatactccaggtgccacaaaggaaagttctttagggatcatagttgttgctgggttttttgttttttgttttaattaaaaaaaaaaaaaaactcttgagtaaaggaaggaatacgatccatctgatctttctgagacttccaggctctgtcaacaactatttggaaataaattcttaggcaattagatcatggtatcttctttcagacagcatagggaaatgaatataaactctggggaaagccaaccaccatgtctgtgatgaggccactcaagcagcctatggcaagcagtccacatggcaaggaacagaagccccttgccaacagccagaatgaacttcctaggcttgtgtgggagttgccttgagaggaggttctccagccccagtcaagtcttcagat

SEQ ID NO: 8351 - RNA, 4257 nt, Homo sapiens
  source 1..4257: mol_type = other RNA
aaaaaccacaattacttttgcaccaacctatatatgcctatttaggcatgcttatttatgcatatttagccactcagcctatggctgagtggactatgtcagagaactgaacccaagttctagagagatctgtcccaagtcagcggacagccaatatacaaggaacctcgcagacagacatacagatgcagagataccccatcacatacatgttaaccagtttggacaatttgaatgaagcctgtggtcaccagggatatgggagcaattctaatcaggattgttagattatctctagaaggttgcttctgatagcttggacaagatgatggcggtgggggagaagcagggaattccttggcagtagggaggttgaatactttcctcattgtgctctagtaaactgaggaacttctagcagcaggagaaacatctgtcctttaaaagccatgtatcctgttcagaaaggcttggcattaatggagaccaaattgtcccactagaaaggacattgatgtcaagggggcatttggtgtcttttctggttctagtcctatgcaaaaaagcatatatcttaaaatatattaactacattttggcaaacaatagttcctgggaggttattatagtattatggtatgcccctatgggaaacttttctattttgtcaggattatagtttctaaaagttcctctccaagtatttaggttgctggcctggcttgtagagaacaacttgagttcaccatccttggtcatcacagaaggagagagcagggcacagttctgcttcggatgtcacagggccagggatttgtcccagatgttgtaagaaagattcaggggacacaggttcaagtacttcaggtctagcaaagtttctgaagactcttttggttgactagctcagggaagcacgagtgagggatgccttcctggaagatgacttattagcctccttcattcctttcaggctttccaggaggatgggctgatagaataccgctggagcttggggcaagggaggtgtggaaagcccctgttttaattctcctcctggccagacttatcagcatgttggactgtgccttgatgttcttctcctaaactgcagaggttctcacctatagctttcttgctctcttagtatctcttgcaacacacgcagcagggcttgagcaggagtggttaacacagcttcctttcttgattcccaaagatcttacttttcacatgactgccaccatggccaccattgctgatgttttatctacacattgtaaagcaggagtctcctattcaggtgttacctgtgtagtctctgtttcagagcctgcaatttgccctaccgtgagcatagttcaatctgtacagcagatgggtttggctgccttctatttagcttatccactagcacattcatggatgctgaattccagggccccactacccagccttctgaggcattctcttccccaagcacttgagaaagcactggaaagagaactgtgttagggttgagccccaaccttgccacatagcaagtcatatccaaccttgagacttttttccccatctgtaaaacaggattactgatgtttgatttacctcctgcacagggatgtgaaaagtcaaggagaatgatgcaaaaatactcatgaactatccggtgctgaacaaatagagggaagataatgatgctgctgacgaaactgatgaagaagaccacgatgatgataattgtgctttgctcgtaaagttacttgatttttgactgactgattagatgcagtttccctgaatggagctgcctaccgccttccttctagggcttatccagacaaccttgggtaagtcactcaactctctacgattaattcatctgtcaaatggggataataaaaaccaccaggcagtgttgctgtgagaattgaaagaagtgagtcaatagatataaaagtgcccagaggagtgcctggaccttatgaggaactttgtcagctctagttgaatttgaatttatataactctagagggaatggtgatgttccccaacttggatggggcagtagaaagagcacagactttatcttgctcatagtggcatgtgactttaacctctctgagccttagttgcctcatccgtaaaatgggaacaacagcgttcacctcaaaagatttgtgtgtgtgtgtgtcaaagggaatggtttgtgcagagagcttttcaaagtacctgacactggcaagggcttagtatttaatagctctctcaccctcatgcttaacgtgggtaagttgcttagaagaaaatgcaaagcctcatatggtcataactgtgctgcctttgtccccttttagctctgggtgctgccaggctgtgggtctgtggcccacagtgcactttcctggtgagaccctgtggcatgagcactgtggcaagaacagtcacatgattaggatcccaaggtgccaggactcttgctgccccagttgctgggcctcctgcctctctcttctgaagcaaaacttgagtgagaggcaggagcaagggcattgaaagtgtccatcctcagcctgctgcctgggacctcaccaactggtgacatttggtcatatgggggcagtcactgggaggtggtctcacctggtagctgctggtggaaggaggccaggggctgtcatagaggtgttcttactccctgtaggcagtggctggcattgctgagagctgacagttttggtgtcaggaggtgaggggtaggtttgagttctgtgccacaccccctctatacaagtaagtgaccaggaactgttcactcttctcaacacagcacactatgcatattctggcctctgccatgtgcagacacccttctttgcctacctgacaaagtagatatttcctgatgacccagttcacaaatcactctaatcttataattctcatggacattgctagatacagatgatggctcctcctctgggcctccataatgacgtgctcagagtcctgacatatagtcttaaagggaatagtttttggatctctctccttgaccagagggaagtgccttgagggcagggactgagtcagttcatctgatgttcccaattcctagcgtgccgcctggcccaaagcagatgctcatacaaaatgagtgtccccaccttgcttgaaccatgactgaggcagccaggtcaccatggaaccagagtgagcagtcagggagggcgtctggtggccagcagctgtggcggtcagcagcatggagggatgagaggcaggcatgtcagatctcttcctcttcactggccttgctccagcggtggcagcagttggcagtgatgcccaggaggaagttggtggccacagaagcaatggagaccacgaagcccacgaacgcaatgaataggtaatcatccagggtcagggtcaggtggcaggccttgaagctctcctcagtgagtgagaagagcggggcgccctcgacttcaggagggccccggcactcagccagctgagaatctgctgtacagcgctggatccggtttcgcagccacttcagcaggggttccatggtgcagccacacacccagggattgccaccgatctgcagggtcaccagccccggtaggccctcaagagcctccaggctgaggaaggccaggcccccataactgaggtccaggtctcggagctgcatgaggccctgaaaggcctggggatgcaccctccgcagccaggggttgtggctcaggtcgatgtggactagcccatgggcctcctggaacatgtcggctggcacatggctgaaattgttgtagctcaggtccaagtgtgccaagcgcttggcatggaggaagaggccccggggcagctccattaaggagttgttgtgcaaatccagcacctggagctccatgtagcatgtgaggtagccaggcggcactgctgtgatgcggttgtgggccaggctgaggtttcgggtgtccattggcaggtctgggggcacggagaatagccgctggctgctacaatccaccacctggttacggcatgtgcaaaggacggggcagctggtgccggcatccgagtgcatcaacccggctgccaagaggagggagatcagcagcattgctgggtggggtggcccgggccagggaagctgggcccaagtgtcacccatcttaggcagcaggcaacagcagtgctggagggagcccatgaggactgtgtccatggaatcgagagtctgt

SEQ ID NO: 8352 - RNA, 5384 nt, Homo sapiens
  source 1..5384: mol_type = other RNA
aaaaaccacaattacttttgcaccaacctcatagcttttcttggttttctttttatctttcttcctttcccactttcattcctttcctccctttattcatttttattttgttacaatcaaatgtttagttttctgttgtttaaaaaccagatataccctcctgatctcttagatggaacaagaacctgtgtctcatggttttagccactaccttttatgttataaacacggaatgaaggacaagagggaagggatgccataccaatattgacctcagtgtaccatgttggtacaaaataataaataataatagctgcgagtcatggatttgtagaaaggatggaaggaaaaactttctgataagatagtacatgtatcactaatgtgtcattttcttttattataacttcctttggtctgtactcttgatggttttaaatgttatgaattcatgtaaactccaaatcatgtgaaggggcattccaaaattttgtttataaattactgacttgggactttatataattaaaacatccttaccaatgttgtttggggtcctaggataccctaaaaaatatcattcaacacacaaaaatgaatctaagatatatatttaatacttttagtacttgttactggcatttatacaattttctcagaaaaaaatattgagttttatctcagtatgccaaggagatttggctgtgattctgttagggactgagttggacggggttgtaggagtgagtcacctaaaaatcagaggcatgttaacactatttatgcatatggaaagttaccttttccatttacataaaaatatgcaagctggtaatttggcttactctctagcagctacattgattcctatattcatggggagggacaagtataaatgctttgaatttagaccctcaattgtctggttgtatgtatgaaccaatctcacatcctaaattatgtcatgtgttgcttacatgagattttacatggtcaggaaatcacaagtcattaaaaactgtagatccagaaagaatatattgaaaatgaaataaccctctacatccttggaaggtaaactatatgaaattctttctaaaataatgattttcaacaaagtagtggtggtaagttgcatgcttgccttgtcagaatcataaacaatgtgagagactgctttagttcttaatatctccttccaacccccaagacacactcagctgagaatcttctgtggtaagtcactgatactgatggaagcgtgccatattgctcaggagtactgggtagtgaaaattctctaatgatgggtttattaagagaagggtaatcaaatgacagaaatctatgttggaaaaccttgagatgtttcagaatttgtgctataaaactttatgtaacttgctgattttttaaaataataaaacaggaatagatacctgaaaacaagtcatgagtctcaaaagaaataatttttcttgacctgtagccagcgtgttcttggatgattaaaattcctatattagttgtgcttggagaaaaaaagatgagtaaggaaggatgggtgcttgaggctgatagcttaataaaaagcaaagactgaaaggaagacaaaaaagtcaacatatattgaatacctattgctaggtcagagacttccacatatatcatctgttttaaatttcacaattctccgtactgaagcttacagcatgttgttttctccagatgagtatgttgaggttcagcttaaataattttctcaaggcatggctaacatggtgtaatagtaaaatctggcctcatgattttgagacctgtgcagttacacaaggccacgttcttagatgggccccaaacttagatgggctctgctgtcactgtcttgaaattcttaaaaatttttgaacaaggagcccacattttcatttcatactgagttttacacattatatagccaatcctgctggtaggctgtgccactctttccatagataatctctaaagacacactgtgaaaactcttccctgtaaagcagatgtagagatagagagccccagggcagacacagccagaactttgtgttctggaatcaagatttaggcttgggggatgtggctccctcagaagaagaatcattgcctcgtatgattgtgtaagtagtttctgggtgctaatgtggcttgatgcattatatcagttttctatggttgtgtaacaaatttagtgacttgaaacaacacatgtttattacctcacagtttctgtgggtcaggaggttgggcgtggcctacctggatcagaggctcagggtgtcagtaggctgcaatcaaggtgttggctgggctgcatttttttctggagcttaggacctcttccaagatcatgtgattattggcagaactcagttccttggtattgcaggactcaggccctcagctactagaggccacccacagtttcctgacatgggctcctctctccataggcagtttacacatgattgcttctttaaggccagcaggagattctctgattctctctctatctctctccagtcttctgcctttggagaggattgcagcactaccttttaatgatcttcagacatatgctaaagaaatgtcatagtgaagaacagttgtacaagaataagcccgaaggtgtcttcatctcaggtgcgttagccaacacctccatgattgcactggttcagacagctccaggcaggcctcagaaacaagttatttacttatgacatccagatggcaagtttttctctgatcattttggaattacacagtctggatagaaagggagaaataattgttgagcactgtttggaaaggattaaagaaaagcctctgacattttatttatgtacatgcactcttcttttctcttaagaaaactaacaaaaagttaaaggcaacaaaattaagacataaaacccaccatggttttaatattggatgttatcatctcagttttaaatactatctggtaaaatgatgcttgaggccaattccagtgaataggaataacttttggaaggcagcgctactgttatccatgggaacagatggctcttactctccaaaaatctagatcaatttcattctcttcttgggctattgtaatagaataccatctgatcctttctgtatccagtatagttttctacaaatcgatcctccatacttctagcaagttccaaaaaacaaatcctttccttgttccctgttgcctgtagaattaatcccaaactaaggcaaatgtagctctttatcctttatgaccacatcttgacctcttcatggtacagctttattttctgacagtcagccatggaattcaatgtcttgacctttttgatcccctggctgttctctaaaagcttcatgttctttcttgtttctgtgacttgcttctgtatatgttgctctcagtacttgaaatgcacatctcttgctatgtgccagctttgctttaaccacttgacatgaattactttattaaattcctacaacaatgctctgaggtagataatacagtcaatgccttcactgccttgtgtcattgtgacttaactctgatttcagtcatctccatggccattcctgaggccactcctatgtgactgctaagattgtgttcagatagcacatcctctgggaaatctttctgactgctatgacctctgggcagagtgtgttgctatctactttgtgtagcaattacacccaatatatacgtttatcttgatgtctagtgctttgactgacaaatgcttctttgctgcctgtagtacactgtgaagagactgagagcagtctttagtatttatttattcacttaatttattgttattatttttgtatcacatggtataaagcacttagtgtctggtaggcactcagtaaatgttaaaaagaagaatcacagctaacataattgatcccttgctatatgccaggttcgttctaaccactttacatgaattactttattaagtccctacaacaatgcttttgaggtagacaacacagccaatgcttccagtgccctgtgtcactgtgacataactcatatttcagccatcactatggcagagagttttgtgtgagctcagacttgtgctgagtgtctcaccccatgcacaagtatcagtctgcctgttcaggccttctctaaagtgcaggaagtcactagatctttctaatgtcctggcacagaagtgaagtggatttaacattctcagggcaaccctcaaccacagatgcacaggagctggtgggtaaattctctagcttcccaccctttgaatggacaattctaagaggcattctgtacactcttggaagtctcagctgagtcaaacttccattgcttatagaagcaacttctgtaatttactcctattgtagctctgtctcactcttgtcattcgtaactccttccagagaattctcccaagccaaatacctgcatccaagatcttgtcatgttctattttggagaaacccaaatgaagataagtactactattatccccagtgtatttgaaacagaggcacagagaggctaagctaagttacttgcctaagactttacacctggaaagtgaaagagactagatttgaactcggataatctggctgcagagccagcccattcctgactatcactctatgctcaatgaggtttataacagatataggggtctcaaacagtctaatattacctacctgcccttataatgtttaaaacttgtcttggctggaaggttaagttttcatatctcttacctaggtttggaagcaagggcatactgcttctttagattttcaccctctttcaaatgaattcccacttttaagctccaaagtgttttcccctcccccaccggaagaagaacaatctaaaagagtgacagagcaaacattaaagtattgtaacttcccactttcaaaagctccatttttaaaatctcacattggagggctttgaatagaggcagtgtgaaaagtggaatgagcgtttagattatcattgaggaaaccagtgtcatctgaatcactaactaggttcatcaccttgggtggctttattccccaatctgggcctcagtttttcctattgtgtaagataaagagtttgagttaaagtggctgctcttactgtttttagagtcattaagaatcttctgaactctatgtatatcatctctattatttctcctcccactctaaatacacatccacatgtacatgtattcttccttgagtaatttcagatgctggtgtcatctctggatcctctggggttaaaaatccatggacacaatctctaaatcctattccagttccagcctcctatggtc

SEQ ID NO: 8353 - RNA, 1692 nt, Homo sapiens
  source 1..1692: mol_type = other RNA
aaaaaccacaattacttttgcaccaacgcaataaattatgtgactttatgcaactcactaatcctggaagtttgcaaacataaaaggagtaaactgttacaaccgttttagaataattactcttcagttttccaagtcaatgttctctttctaaaattgatctgcctgagaaaacactacaattaggatgtaattcaatttctcttttccaacttttttcatgcatttatcctgtgggacaatccatattcaaaactatgtattaagcttttctgaaaataaaaagtcaaatatgtttgggttcatcttgtgtaacaagttgcattaaaatcctcgcctctttctctcccactgaatccttgtcactgttcaatatccagaacaaataacagctcctctgtgaggtcgacccagattccacgagacaaagctatcacttcctctacattatcaaactgttgggtatgcacctccacaatagcacctaatgtagatgatgggttgataggttcagcaaccaccatggcacatgtatacctatgtaataaaacctgcatgtcctgcacgtgtatcccagacccatcaagctatataggttgtcacaaaatgtactgaggcattccgttccattaaggtgagataggacgaagggcagaaagacggagtctgagtcctaaaatccttgctgcctcagggtaatagtaacttatttcaccatatttataggtcactaatggtaactgatccagaagaaatggtggcatcaaattgtccttggcctggttctgcaggctgtgtaagaatggcaccagcattactcagcttctggggaggcctcagggagctgttactcatggttgaaggcaaagaggaaccttcctctccctttttctcttctcactgcttcaattagtttatctttttcatttccaagtggaggggtaatggccagccaagatataaggatcacagcagtggtgcattctgtgttatcaattctacattaacactatcttcccttctgaggactctgatgtgaagttcatgaatgtttcatggattcttgagtgacagaagctttcaggaacagtgtttctctgatttccattgccaagagcatcagcatcctcttggatgctctgttgctcaggctggagtacagtgcagtggcacaatctcagctcactgcaacctctgcctcctgggttcaagcaattcttgtgcctcaacctcccaagtagctggtgagcactgccacgcctggctaagttttgtatttttagtagagatggggtttcgtcatgttggccgggtttaggccctcaagtcctctgcccgcctgggcctcccaaagtgctgggattacagtcgtgagccaatgtgaccggccttcatccttttcttaaaaacagatgccaaataccatcagggaagcttaggacctctctttggcctgaatttgttacatgctcatttctgaatctgtagctatagcaatgaagacaggatttttctgctccaggatagacggtttgatataaagggtatcttggccctgcgctcccgttgacgtcgcatcctgtcagtatttcgccaaacctccaggcgccatcagtgtgtgaaccgttacgcagctggtccaccgcgggcggagaacaagcgactatgcccagggatcctgcacgcatgcgt

SEQ ID NO: 8354 - RNA, 1004 nt, Homo sapiens
  source 1..1004: mol_type = other RNA
aaaaaccacaattacttttgcaccaacgcaataaattatgtgactttatgcaactcactaatcctggaagtttgcaaacataaaaggagtaaactgttacaaccgttttagaataattactcttcagttttccaagtcaatgttctctttctaaaattgatctgcctgagaaaacactacaattaggatgtaattcaatttctcttttccaacttttttcatgcatttatcctgtgggacaatccatattcaaaactatgtattaagcttttctgaaaataaaaagtcaaatatgtttgggttcatcttgtgtaacaagttgcattaaaatcctcgcctctttctctcccactgaatccttgtcactgttcaatatccagaacaaataacagctcctctgtgaggtcgacccagattccacgagacaaagctatcacttcctctacattatcaaactgttgggtatgcacctccacaatagcacctgtgtagaaatacctgtggtaggtttcaaaacaattctataaagggactatattctttaggcacaattttttttcacaactggaatcaggagatcaaagtagaaccttctaaagaagtggaatgttcttttttctcttgtattggacatataggcaaaccttaaacccatattttctgggcttggcttctgatgtgaagttcatgaatgtttcatggattcttgagtgacagaagctttcaggaacagtgtttctctgatttccattgcctctctttggcctgaatttgttacatgctcatttctgaatctgtagctatagcaatgaagacaggatttttctgctccaggatagacggtttgatataaagggtatcttggccctgcgctcccgttgacgtcgcatcctgtcagtatttcgccaaacctccaggcgccatcagtgtgtgaaccgttacgcagctggtccaccgcgggcggagaacaagcgactatgcccagggatcctgcacgcatgcgt

SEQ ID NO: 8355 - RNA, 28 nt, Homo sapiens
  source 1..28: mol_type = other RNA
aaaaaccacaattacttttgcaccaact

SEQ ID NO: 8356 - RNA, 1505 nt, Homo sapiens
  source 1..1505: mol_type = other RNA
aaaaaccacaattacttttgcaccaacttaaatatataacctctctgagctcccattttctcatctaaaaaatgaaataataccaacctcacagcactgttggaagggttggggtaaagcaccaagtacgtgggtagcttatatcctacagaataattttcaccaacatgacccatgaccatgaagtttatggtttgactatctgtaggaagggtacaaaaatacatcatgcaacaaggtcattcatttggaaatgtaatgctttctgaaaaacttgagcattcacttttcttcacttgcctgttctaataagagaggtttggtgtggtgatttttcaatagaaaggatgttaccaatatataaataacataaaaggatcacatgagaattaaagtgaagtaacttaacatacaattttcattctaatcttatacaataatttttcttgactattgatagatcacaataaaggtatgctgatgatataagttattttaagactttggggaaaaaggcttccgtctctggcattgaccttattgtggaggaccctccaaaatcttcagctctgcaccagcaggtatgctgagtcatgtatgatgacataaaccacaaggagtcaaggagctaaaacaaccacagcgactggctcagatctcagatgtgcaagatgaatcctcaggatttttcacacactgaagaaacttgtcaggtctgtagatattcttgcaggaaaattgaatattccttttgcttataatcgattccagctcttttatggtgggatcctggcataagtctctggaatcttctcttccaccatgtatcacccaggcctctagtgtctgaaccttctctggttgcaaattatggacttccacactcccaaaagtgctgtttttgtcaaagattttactgcgggatccattgagcatcacatggaccacatcacaggcagcttctgcaaacctgcgggaaaccgttttccagaatactgaaacagggttgttgctgcagtcctttctccagtctgggcaagattgatagtttatttcttgttgcaaggtacggtctgagttcccaacttcattagtggctgatagtcttcttcagtaatgttgcaaggatgttttgaaataaatgcacccttgaaagcatcccatacactttggcagtctacatgtctcatctcaggatgaatttcagtgtacttgacgcatcgcgccaggacggtctcgggaaagcgcttggtggtgcccggaccgctccactgctggcgccacctcgggacgaccaccgcgagcaccacgacgaggatcaggaccaggatactgacgccaagacagagttgggctctcctagagagccggcagcagggtttgtccccggacaccgggctgaactcgcagttggccatagggctccaggcggggttggctgggcgaagatgaggccggcaggaggctaggcagcaagagagaggctggctgggttctgaaactgc

SEQ ID NO: 8357 - RNA, 1641 nt, Homo sapiens
  source 1..1641: mol_type = other RNA
aaaaaccacaattacttttgcaccaacttaaatatataacctctctgagctcccattttctcatctaaaaaatgaaataataccaacctcacagcactgttggaagggttggggtaaagcaccaagtacgtgggtagcttatatcctacagaataattttcaccaacatgacccatgaccatgaagtttatggtttgactatctgtaggaagggtacaaaaatacatcatgcaacaaggtcattcatttggaaatgtaatgctttctgaaaaacttgagcattcacttttcttcacttgcctgttctaataagagaggtttggtgtggtgatttttcaatagaaaggatgttaccaatatataaataacataaaaggatcacatgagaattaaagtgaagtaacttaacatacaattttcattctaatcttatacaataatttttcttgactattgatagatcacaataaaggtatgctgatgatataagttattttaagactttggggaaaaaggcttccgtctctggcattgaccttattgtggaggaccctccaaaatcttcagctctgcaccagcaggtatgctgagtcatgtatgatgacataaaccacaaggagtcaaggagctaaaacaaccacagcgactggctcagatctcagatgtgcaagatgaatcctcaggatttttcacacactgaagaaacttgtcaggtctgtagatattcttgcaggaaaattgaatattccttttgcttataatcgattccagctcttttatggtgggatcctggcataagtctctggaatcttctcttccaccatgtatcacccaggcctctagtgtctgaaccttctctggttgcaaattatggacttccacactcccaaaagtgctgtttttgtcaaagattttactgcgggatccattgagcatcacatggaccacatcacaggcagcttctgcaaacctgcgggaaaccgttttccagaatactgaaacagggttgttgctgcagtcctttctccagtctgggcaagattgatagtttattttggaagtgttgaattcaccacaccatgtgaggtcatcagcaaggtagcctagcagcgtgtcctccagggtgaacatgtcccgctggacctgtgtgaactgatgggccagatcttttattctgctccaaagaagaatcttgttgcaaggtacggtctgagttcccaacttcattagtggctgatagtcttcttcagtaatgttgcaaggatgttttgaaataaatgcacccttgaaagcatcccatacactttggcagtctacatgtctcatctcaggatgaatttcagtgtacttgacgcatcgcgccaggacggtctcgggaaagcgcttggtggtgcccggaccgctccactgctggcgccacctcgggacgaccaccgcgagcaccacgacgaggatcaggaccaggatactgacgccaagacagagttgggctctcctagagagccggcagcagggtttgtccccggacaccgggctgaactcgcagttggccatagggctccaggcggggttggctgggcgaagatgaggccggcaggaggctaggcagcaagagagaggctggctgggttctgaaactgc

SEQ ID NO: 8358 - RNA, 43 nt, Homo sapiens
  source 1..43: mol_type = other RNA
aaaaaccacaattacttttgcaccaacttaatacctccctgca

SEQ ID NO: 8359 - RNA, 36 nt, Homo sapiens
  source 1..36: mol_type = other RNA
aaaaaccacaattacttttgcaccaacttaatactt

SEQ ID NO: 8360 - RNA, 2384 nt, Homo sapiens
  source 1..2384: mol_type = other RNA
aaaaaccacaattacttttgcaccaatttaatattttagagtgtacttctacttatttaaaaaaagttaactgtaaaacagcctcaggcagatcctacagaaggtattccagaagaaggcattgttatcataggagatgacagctccatgcatattactgctcctggaaggctttccagtcagctaagatgtgaagctgtaaaacagtgatattgataatcctgactgccccgctgtctacacctggtttcaaaccatatggtgtcagtactaggctggactgcaccagcagtccaggcagcagtggcaccccaactagacatagctgtgtaccatgtcctattaggaatggaagaacaccctttctaacagtgaaggctcggggtctaggggtgccccaggccccatggccttatcttgcattaggactacaggttccaagacctcttgcaactctgctgctaagggacttatacttagcgtactccactgctctaagtaggtgccccacttcgctaaagtggatgtctgtgctgtcccagtctgggggggtcattgctcatgaacgcacccatcccactatggggtaagccatccacacgactgtaacccatccagccacgctcttatgaacctgaagggcagcatatatggttactaactgcttctttattaatgaacactggggctcagctcccttccatagctgggactaaaagctgactggcgcttccaagcactccatatactgccataggccctagccaactctattggtggttacatgcacatctagtttaaatgggcaccctggttaaccacccagagggcttatgtcatcagaagggctgtttcagcctcatcatcccaatcccaggcaagaggggtgttgtggcctccaaaccagcaaaagaactagaggttaacataacatcattaataagaaaatgatatataatggggctatacatatagccctgcagcaacactatgaaagtccattgtcgccctcccatgaaggcaaactgttcctggctctctggagcaatgctgattgagaagaatgcattggtcaagtccaccacacagtggcaccatcccagttctgttgtcaaacggtccatcaagtccatgacaggtggcacagctgccaagtcttgcaaaacatccacccccaagaatgtcctcaggcatgcaagagacatacacagtgcataagtggagagccaagcagctgatgcccaggtgcaaagacacaggtttcactttcactgaccagctttcatagctgtctatgcagccttccctggaaacttatccgggtccagggaccagtggattgccaagtccatatatggcctttggttgtctggtatcccctaccaagccgggcaccttggccagttctcttatcaaacagaaaatgctttatacttccaccaactgcagcaggtactctttgaactggaacactctggcaggaccaggttgcgcagcaacatccttctcccaaatgacttgcaccaagtctcatcccattctcattgccagttgttaggtttagggttcgggtccagcccatgctgaggtacaagggagtgggtcccttacagaagatgtcatcaacaaaccagaggcggagatgtcactacaagatttgcagctccattacttcaaaatgcacgattatgatggcaattatttgcttgatggtttagaaatctccacagccatcactcatatacagggaccaggattttactccagttctgccgactccagtactggatctcttaagctggatcctagcagatctgcacaggtacctactggaatgcttggctccatgatccatggctctgtcccttgctctaactgggaaatcacatcaggtttagaaacttggagtcctatagagaccaggtgtgtataattttccaatgtcacatccctgaacaaatctctctggccagggtccagctgtttccattcttcctgggtaaagtccactatcacatccttgaaagtcaccgcttcctgaaaactggctgatgagagtagattatgtcccccttggagaagggtggagtctggagaggacagatcttccatctcaggagctcatcccgttcctctggaacttgaacaccagggttcgccaggcagcgttccttcagctggtatctcggtctaggactcagatgtctaactccccttgcagggaatctgcaacacgctgaggttgtctaccctgagctcccctccccctatagcgatccacacactctgatcccgggtccggaagcgcattgaccgccaccagacctaacgcagggagccgaagcaactggacttccagcgcgccaacctctttccacgcctac

SEQ ID NO: 8361 - RNA, 2599 nt, Homo sapiens
  source 1..2599: mol_type = other RNA
aaaaaccacaattacttttgcaccaatttaatattttagagtgtacttctacttatttaaaaaaagttaactgtaaaacagcctcaggcagatcctacagaaggtattccagaagaaggcattgttatcataggagatgacagctccatgcatattactgctcctggaaggctttccagtcagctaagatgtgaagctgtaaaacagtgatattgataatcctgactgccccgctgtctacacctggtttcaaaccatatggtgtcagtactaggctggactgcaccagcagtccaggcagcagtggcaccccaactagacatagctgtgtaccatgtcctattaggaatggaagaacaccctttctaacagtgaaggctcggggtctaggggtgccccaggccccatggccttatcttgcattaggactacaggttccaagacctcttgcaactctgctgctaagggacttatacttagcgtactccactgctctaagtaggtgccccacttcgctaaagtggatgtctgtgctgtcccagtctgggggggtcattgctcatgaacgcacccatcccactatggggtaagccatccacacgactgtaacccatccagccacgctcttatgaacctgaagggcagcatatatggttactaactgcttctttattaatgaacactggggctcagctcccttccatagctgggactaaaagctgactggcgcttccaagcactccatatactgccataggccctagccaactctattggtggttacatgcacatctagtttaaatgggcaccctggttaaccacccagagggcttatgtcatcagaagggctgtttcagcctcatcatcccaatcccaggcaagaggggtgttgtggcctccaaaccagcaaaagaactagaggttaacataacatcattaataagaaaatgatatataatggggctatacatatagccctgcagcaacactatgaaagtccattgtcgccctcccatgaaggcaaactgttcctggctctctggagcaatgctgattgagaagaatgcattggtcaagtccaccacacagtggcaccatcccagttctgttgtcaaacggtccatcaagtccatgacaggtggcacagctgccaagtcttgcaaaacatccacccccaagaatgtcctcaggcatgcaagagacatacacagtgcataagtggagagccaagcagctgatgcccaggtgcaaagacacaggtttcactttcactgaccagctttcatagctgtctatgcagccttccctggaaacttatccgggtccagggaccagtggattgccaagtccatatatggcctttggttgtctggtatcccctaccaagccgggcaccttggccagttctcttatcaaacagaaaatgctttatacttccaccaactgcagcaggtactctttgaactggaacactctggcaggaccaggttgcgcagcaacatccttctcccaaatgacttgcaccaagtctgtacaagagtgccaacattacttgcttaactcctacaacttagcaggggcacagacaacataggaagtgtgctccaccacagtagggggtctctggcccacccttggggcccaacagctgctcatgctctattttctggcagaccattgggtgaacctgtaacggaggttcttcctccctgtgtgcatccctcagggactgggcaggcacttcctcatcccattctcattgccagttgttaggtttagggttcgggtccagcccatgctgaggtacaagggagtgggtcccttacagaagatgtcatcaacaaaccagaggcggagatgtcactacaagatttgcagctccattacttcaaaatgcacgattatgatggcaattatttgcttgatggtttagaaatctccacagccatcactcatatacagggaccaggattttactccagttctgccgactccagtactggatctcttaagctggatcctagcagatctgcacaggtacctactggaatgcttggctccatgatccatggctctgtcccttgctctaactgggaaatcacatcaggtttagaaacttggagtcctatagagaccaggtgtgtataattttccaatgtcacatccctgaacaaatctctctggccagggtccagctgtttccattcttcctgggtaaagtccactatcacatccttgaaagtcaccgcttcctgaaaactggctgatgagagtagattatgtcccccttggagaagggtggagtctggagaggacagatcttccatctcaggagctcatcccgttcctctggaacttgaacaccagggttcgccaggcagcgttccttcagctggtatctcggtctaggactcagatgtctaactccccttgcagggaatctgcaacacgctgaggttgtctaccctgagctcccctccccctatagcgatccacacactctgatcccgggtccggaagcgcattgaccgccaccagacctaacgcagggagccgaagcaactggacttccagcgcgccaacctctttccacgcctac

SEQ ID NO: 8362 - RNA, 34 nt, Homo sapiens
  source 1..34: mol_type = other RNA
aaaaaccacaattacttttgcaccagcctaatat

SEQ ID NO: 8363 - RNA, 867 nt, Homo sapiens
  source 1..867: mol_type = other RNA
aaaaaccacaattacttttgcaccagcctaatattttctcaggccccaccccaggccaacagaatctatatctcaatggtgaagctcaagaatggacagctctgacaagtgcatcaggtgtttctgatgcccagtcgggtaggaaaatgacaaggttacatggatttggtctctttaaactataaacagttatgtttaatgagttgccaaggaactaaatacatagacatctgtaaccaggaataactttgtctcagataagccatctacgaataatcaggcaggcctgcaccttggcccaaaactccagacgttacctggtttccgacctagatgttagctgccaggctttgggtctgcctgctcacctgcccacctcccagattcctgatgcctgtcccctggtctggtatgattaccactgctcaagcctctctaaattcccggaagagattttctgaaaacaaaacatggtgtagaaaaatagtacaaaagaaacatgttctagaaatgaaaggtctatgttctaggagaagatttatgttccagaaacagaaattcctcctcctctgtatagatgtgcatcttgaaaaggtacttaaccagctactgttttgcactttcattatagtgctaagcactctgtgtttgctacatcatttaatcctttcttatattttgagatagggccattattattttatttacagatgagaacacaaaggctcagagagattgaataacttgtctaaggccagacagtgaacgaaaggcagaactgggattctaatttagtcttgactcttcacatctatgatggtgtttccccagtgtcctcatctgtaaaacaggaataatattggccag

SEQ ID NO: 8364 - RNA, 47 nt, Homo sapiens
  source 1..47: mol_type = other RNA
aaaaaccacaattacttttgcaccagctaactattcactggctgccc

SEQ ID NO: 8365 - RNA, 32 nt, Homo sapiens
  source 1..32: mol_type = other RNA
aaaaaccacaattacttttgcaccatcctaat

SEQ ID NO: 8366 - RNA, 2268 nt, Homo sapiens
  source 1..2268: mol_type = other RNA
aaaaaccacaattacttttgcaccatcctactacaagtttggtctccagaatatattgtatatcggatgaaacacaggctgaacatcccttttccggcacccttggcctattgatcatgatcttctttcctggcatgcttggactcaacttcagaatgtttcttgatactgtgtttcaggcaactgccaccaatcaattggtgttggcacaatccagaggaccgctaccggtctccagtagatttcacctggtgtagagagatctgaggcgtattatcgctggcaaaacgcgatggggagttcccggctgggcaccagggtgcctgagtgtagcatctcaacaggctcattgtctgtggcctggatgtcgtatttgcggacaatccaacaaagagccaaatgcagttgaagctctgctaatcggcgaccaatgcacattctttttccaacgccaaatggaagatgcgcaaaaggattaattttttccttctcctgaagccaacgttcaggtctaaactgacttgaatcttcaaaattgtcttcactggatcccaacacctgggtatttagcatgagcactgttcctttgggtaaagcatattcacccagaactgttgccttgtcaagagtccgagttgtaaatggtacactcggcgtaagcctcatagattctttcagacaggcttttaaatacggcatattcctcaaatcttctgcccgtggcacctgattctcaggtaatacactttgaatttccttaagaagcttttgttgcacttggggattacgggataaattgtagagaatccacattagactgtttgctgtcgtttccaccgcagccagctggagctctgtgacagcagcatacaattctttctttgaaagccgattctggtgataaatgtcacaaaggaaatctgcactaggctgctgagaatacttctctaaccggttgtcgatacaagctttgactgatttgaaaatggtgtcccaggccagagtgtggtcctgccagaccttggtgttgaggctcttgtgcagctcgactggagtgaccatcatcctcccaaacgtgctcatcattgttttgatggccatgatgaagttcacagcttcatcccctgcattcttctggagaagcccaaatctcttctcatacaacacgaggcagatactttcaaacgaccatttgttcagttcgctgtacaagtcttcaacgtggcctctttcatcacagagctcatctattctgcccataaaatcggccaagacctcattgattttgttgtccagcttcatcacttcccctggtttcattagtttcttttgaaaggcactccggacccgctgccagtcttccccttccaggatcagcagcccgtagccttctttgcggtagtcgcgataggccttccacggtttgatctccagccgctgcgggtacgcgctctcggtgcggtacagcgcttccagcaggcatggcgagcccaggtgcaccgactcaaaggaacccaacttcatgcggaaaatcttgccatacttcttgtggtactccaccagggtgtcgtgctgtttcttgagaccccctttccagagaatctgcagcaggctgcccagcagtggccagctggtggggcccggcagggcggccgcgttctgagtctcgccaccagctgtcagcgggcagactggcacctctcgcggctgaggggacgtgtacgccgtagatgtcaccagtctcgggggctgcctcggactgcgcagctgctgcaggaaggcggcaagcgagcggctcttgctgatgggggagctcatggcagcgggggacaccggagcgcgggaaggcaggaggatggggtggggcgaggttggtacgaggtgctagtgggagtcggggcttaacgattctgggaaaaggaagcaaagagggccagctggtgtgatggagcggggtgaggcgggacaggcagcagaaaggacctcggcgaggatgctcgacgctgcaccacgcgacagcctcagagcattggtgcctccttgcactggccgcaggggctggaagagggtggccggtgtctggggacctcttgaaaagggaaagctgggagtcctcctgttggtccgcaaggctgacctctagggtctggctggagccacggggaggtgtcaaggagggtagatgagatgctgctggcgctgcgtttcctcctgtccctctccatgttcctatgcccagggaccatgcatttatggagacagagcatg

SEQ ID NO: 8367 - RNA, 1736 nt, Homo sapiens
  source 1..1736: mol_type = other RNA
aaaaaccacaattacttttgcactaacctaatagttctctctgaagagaataaattagttctagtaatatgaagcatacccagttttaataaacttatacatacaaaacattcccaagctttgtgaggggccaacattacgagagcgatatgagatatctgaaaacaattttattttcccattattcaggcttttgaagcaggtcttaagctttcccagttctttgccacttaatttcttacatatgtttaaaatatatattaaaaaaactaatgtaatttgaggaccaccactgcacctaaaagaaattccatgttttccacctattcagttgttctttgtagaaatggtctaattattaagtccatttttacagttcaaaatatcactgatattaccacataaacctttgaatgtcctgactatttggccactgaaaagtcttgttcagaaagatgtaaaaagttatgaaattaacaattgcatagcaactcagttcacaaacaagtctggatgtgggaggcagagttatgttaagcctataaatgacataaggtaaaatgaagtaacgaaattccagcagtttctgaggaactataacaatgaacaagcatatgaaaaacattaaattccaaaaaattggctttgatttcaatgagtcagctatactccaaccagcaaatatataggctggaactaacaaatatttcagaattgcatatctttgaaaaactcttttccacacatagaaagtataatgtctattgtctgctagcaagtatttatgagcataagtgaatttccaaactaaaaacacagagactaaggtaaccaccaaaaacagaattccatgtttccaaactaaggaaagaaaagtcttaattttgctaggagacaggagatgaggaaaagaaaaaaagagagtaaatgaaaaaaagtagaatagttgaggaaaatgaagacaggcttcatgactactccgatcgccaataacaattccaccattaactactacaaaagcacaaaacagaaatcccagaaggatgtagggccaagtcaaacagaaaagcatactcaagtttttaaaggacatggaataagccaaaagaaactgaagaatttttctgaattctgcaaatggtcctttaataggtggaagtctgtcttccttcttttgtagctcagttttccaagcctcagttaacttttgtgcaatgacattccctgcacagaagacagcccagatgatatttgtttgccgaaacatgaagccacaaaatccaaggaaggctgaagttttatgatttccataaagacacatcaaatatgcaaaaagagtaaaaaacatagatcctgcttctgtataataaaggaagttaaaaaaataaagtgttggaaatactgctagtgttaatgttgacaagactctctggatacttgaggcagccttgtttctgggttgtaccttgtggaaaagcaaatatagtaaatagaagttgccaacactgaagagaagattaacaaatctgagcatcccaatggagcagacaacatgttcagaccatgcaaagatccaaatggcaggtttgaccactccaactgacaccaggtacaagccaggtaatgtagtaatcatgggatcccacggaaggcaaaggatgctgggagagcgcggatccggaaaacagcgggtcgctgtttcctggagtgacgggtttagataacggaccggatga

SEQ ID NO: 8368 - RNA, 1936 nt, Homo sapiens
  source 1..1936: mol_type = other RNA
aaaaaccacaattacttttgcactaacctaatagttctctctgaagagaataaattagttctagtaatatgaagcatacccagttttaataaacttatacatacaaaacattcccaagctttgtgaggggccaacattacgagagcgatatgagatatctgaaaacaattttattttcccattattcaggcttttgaagcaggtcttaagctttcccagttctttgccacttaatttcttacatatgtttaaaatatatattaaaaaaactaatgtaatttgaggaccaccactgcacctaaaagaaattccatgttttccacctattcagttgttctttgtagaaatggtctaattattaagtccatttttacagttcaaaatatcactgatattaccacataaacctttgaatgtcctgactatttggccactgaaaagtcttgttcagaaagatgtaaaaagttatgaaattaacaattgcatagcaactcagttcacaaacaagtctggatgtgggaggcagagttatgttaagcctataaatgacataaggtaaaatgaagtaacgaaattccagcagtttctgaggaactataacaatgaacaagcatatgaaaaacattaaattccaaaaaattggctttgatttcaatgagtcagctatactccaaccagcaaatatataggctggaactaacaaatatttcagaattgcatatctttgaaaaactcttttccacacatagaaagtataatgtctattgtctgctagcaagtatttatgagcataagtgaatttccaaactaaaaacacagagactaaggtaaccaccaaaaacagaattccatgtttccaaactaaggaaagaaaagtcttaattttgctaggagacaggagatgaggaaaagaaaaaaagagagtaaatgaaaaaaagtagaatagttgaggaaaatgaagacaggcttcatgactactccgatcgccaataacaattccaccattaactactacaaaagcacaaaacagaaatcccagaaggatgtagggccaagtcaaacagaaaagcatactcaagtttttaaaggacatggaataagccaaaagaaactgaagaatttttctgaattctgcaaatggtcctttaataggtggaagtctgtcttccttcttttgtagctcagttttccaagcctcagttaacttttgtgcaatgacattccctgcacagaagacagcccagatgatatttgtttgccgaaacatgaagccacaaaatccaaggaaggctgaagttttatgatttccataaagacacatcaaatatgcaaaaagagtaaaaaacatagatcctgcttctgtataataaaggaagttaaaaaaataaagtgttggaaatactgctagtgttaatgttgacaagactctctggatacttgaggcagccttgtttctgggttgtaccttgtggaaaagcaaatatagtaaatagaagttgccaacactgaagagaagattaacaaatctgagcatcccaatggagcagacaacatgttcagaccatgcaaagatccaaatggcaggtttgaccactccaactgacaccaggtacaagccaggtaatgtagtaatcatgggatcccactgggaaagggagaaatggccctcacagtagcgctgcgcctgaggcaggtggaagatctcgtccatgtagggctctcgcagcgcccggctgaaggcggagaagaggaggcaggacactaaaaaggtacagctcaaggcggccgagaaacagtaaccctctagctgcgccattcctgctcccacagccactgcccaagaacccactcctggaaaattctgagcccggaaacccgagctggaaacttgggctcgaaatgggcgcgctagacaggactagccagacggggccac

SEQ ID NO: 8369 - RNA, 1767 nt, Homo sapiens
  source 1..1767: mol_type = other RNA
aaaaaccacaattacttttgcactaacctaatatttctctctgaagagaataaattcattccagtaatatgaagcatacccagttttaataaacttgtacatacaaaacattcccaagctttttaaggggccaacattatgagagtgatatgagatatctgaaaacaattttatttttccatttttcaggcttttgaagcaggtcttaagctttctcagttctttgccacttaatttcttacatatgtttaaaatatatataaaaaaaactaatgtaatttgaagaccaccactgcacctaaaagaaattccatgttttccacctattcagttgttctttgtagaaatggtctaattattaagtccattttcacagttcgaaatatcactgatattaccacataaacctttgaatgtcctgactatttggccactgaaaagtcttgttcagaaagatgaaaaaagttatgaaattaacaactgcatagcagctcagttcacaaatgagtctggatgtgggaggcagaggtatgttaagcctataaatgacataaggtaaaatgaagtaacgaaattccagcagtttctgaggaactataacagtgaacaagcatatgaaaaacattaaattccaaaaaattgactttgatttcaatgagtcagctatactccaaccagcaaatatataggctggaactaacaaatattttacagtttcatatctttgaaaaactcttttccacacatagaaagtataatgtctattgtctgctagcaagtatttatgagcataagtgaatttccaaactaaaaacacagagactaaggtaaccacaaaaaacagaattctacgtttccaaactaaggaaagaaaagtcttaattttgctaggagacaggagatgaggaaaggaaaaaaagagagtaaatgaaaaaaagtagaatagttgaggaaaatgaagacaggcttcatgactactccgatcgccaataacaattccaccattaactactacaaaagcacaaaacagaaatcccagaaggatgtagggccaagtcagaagcaaaagcatactcaagtttttaaaggacatggaataagccaaaagaaactgaagaatttttctgaattctgcaaatggtcctttaataggtggaagtctgtcttccttcttttgtagctcagttttccaagcctccgttaacttttgtgcaatgacatttcctgcacagaagacagcccagatgatatttgtttgccgaaacatgaagccacaaaatccaaggaaggctgaagttttatgatttccataaagacacatcaaatacgcaaaaagagtaaaaaacatagatcctgcttctgtataataaaggaagttaaaaaaataaagtgttggaaatactgctagtgttaatgttgacaagactctctggatacttgaggcagccttgtttctgggttgtaccttgcagaaaagcaaatatagtaaatagaagttgccaacactgaagagaagattaacaaatctgagcatcccaatggagcagacaacatgttcagaccatccaaagatccaaatggcaggtttgatcactccaattgacaccaggtacaagccaggtaatgtagtaatcatgggatcccaccagtttctttcatgttctgaggcttgagggggtggaacaggacgagtgaagtctaaggatgggaggacgtggggacgctgggacctctcaggcctctcctggggtggggacaggttgggga

SEQ ID NO: 8370 - RNA, 1806 nt, Homo sapiens
  source 1..1806: mol_type = other RNA
aaaaaccacaattacttttgcactaacctaatatttctctctgaagagaataaattcattccagtaatatgaagcatacccagttttaataaacttgtacatacaaaacattcccaagctttttaaggggccaacattatgagagtgatatgagatatctgaaaacaattttatttttccatttttcaggcttttgaagcaggtcttaagctttctcagttctttgccacttaatttcttacatatgtttaaaatatatataaaaaaaactaatgtaatttgaagaccaccactgcacctaaaagaaattccatgttttccacctattcagttgttctttgtagaaatggtctaattattaagtccattttcacagttcgaaatatcactgatattaccacataaacctttgaatgtcctgactatttggccactgaaaagtcttgttcagaaagatgaaaaaagttatgaaattaacaactgcatagcagctcagttcacaaatgagtctggatgtgggaggcagaggtatgttaagcctataaatgacataaggtaaaatgaagtaacgaaattccagcagtttctgaggaactataacagtgaacaagcatatgaaaaacattaaattccaaaaaattgactttgatttcaatgagtcagctatactccaaccagcaaatatataggctggaactaacaaatattttacagtttcatatctttgaaaaactcttttccacacatagaaagtataatgtctattgtctgctagcaagtatttatgagcataagtgaatttccaaactaaaaacacagagactaaggtaaccacaaaaaacagaattctacgtttccaaactaaggaaagaaaagtcttaattttgctaggagacaggagatgaggaaaggaaaaaaagagagtaaatgaaaaaaagtagaatagttgaggaaaatgaagacaggcttcatgactactccgatcgccaataacaattccaccattaactactacaaaagcacaaaacagaaatcccagaaggatgtagggccaagtcagaagcaaaagcatactcaagtttttaaaggacatggaataagccaaaagaaactgaagaatttttctgaattctgcaaatggtcctttaataggtggaagtctgtcttccttcttttgtagctcagttttccaagcctccgttaacttttgtgcaatgacatttcctgcacagaagacagcccagatgatatttgtttgccgaaacatgaagccacaaaatccaaggaaggctgaagttttatgatttccataaagacacatcaaatacgcaaaaagagtaaaaaacatagatcctgcttctgtataataaaggaagttaaaaaaataaagtgttggaaatactgctagtgttaatgttgacaagactctctggatacttgaggcagccttgtttctgggttgtaccttgcagaaaagcaaatatagtaaatagaagttgccaacactgaagagaagattaacaaatctgagcatcccaatggagcagacaacatgttcagaccatccaaagatccaaatggcaggtttgatcactccaattgacaccaggtacaagccaggtaatgtagtaatcatgggatcccacggaaggcaaaggatgctgggagagcgcggatccggaaagatcgggtcgctgtttcccggagtgacgggtttagataacggaccggatgattaccctctcaatcgcattgcccggggcgcacaaagtgtcaaaacttccggaaggggcgggtctcggattt

SEQ ID NO: 8371 - RNA, 1920 nt, Homo sapiens
  source 1..1920: mol_type = other RNA
aaaaaccacaattacttttgcactaacctaatatttctctctgaagagaataaattcattccagtaatatgaagcatacccagttttaataaacttgtacatacaaaacattcccaagctttttaaggggccaacattatgagagtgatatgagatatctgaaaacaattttatttttccatttttcaggcttttgaagcaggtcttaagctttctcagttctttgccacttaatttcttacatatgtttaaaatatatataaaaaaaactaatgtaatttgaagaccaccactgcacctaaaagaaattccatgttttccacctattcagttgttctttgtagaaatggtctaattattaagtccattttcacagttcgaaatatcactgatattaccacataaacctttgaatgtcctgactatttggccactgaaaagtcttgttcagaaagatgaaaaaagttatgaaattaacaactgcatagcagctcagttcacaaatgagtctggatgtgggaggcagaggtatgttaagcctataaatgacataaggtaaaatgaagtaacgaaattccagcagtttctgaggaactataacagtgaacaagcatatgaaaaacattaaattccaaaaaattgactttgatttcaatgagtcagctatactccaaccagcaaatatataggctggaactaacaaatattttacagtttcatatctttgaaaaactcttttccacacatagaaagtataatgtctattgtctgctagcaagtatttatgagcataagtgaatttccaaactaaaaacacagagactaaggtaaccacaaaaaacagaattctacgtttccaaactaaggaaagaaaagtcttaattttgctaggagacaggagatgaggaaaggaaaaaaagagagtaaatgaaaaaaagtagaatagttgaggaaaatgaagacaggcttcatgactactccgatcgccaataacaattccaccattaactactacaaaagcacaaaacagaaatcccagaaggatgtagggccaagtcagaagcaaaagcatactcaagtttttaaaggacatggaataagccaaaagaaactgaagaatttttctgaattctgcaaatggtcctttaataggtggaagtctgtcttccttcttttgtagctcagttttccaagcctccgttaacttttgtgcaatgacatttcctgcacagaagacagcccagatgatatttgtttgccgaaacatgaagccacaaaatccaaggaaggctgaagttttatgatttccataaagacacatcaaatacgcaaaaagagtaaaaaacatagatcctgcttctgtataataaaggaagttaaaaaaataaagtgttggaaatactgctagtgttaatgttgacaagactctctggatacttgaggcagccttgtttctgggttgtaccttgcagaaaagcaaatatagtaaatagaagttgccaacactgaagagaagattaacaaatctgagcatcccaatggagcagacaacatgttcagaccatccaaagatccaaatggcaggtttgatcactccaattgacaccaggtacaagccaggtaatgtagtaatcatgggatcccactgggaaagggagaaatggccctcacagtagcgctgcgcctgaggcaggtggaagatctcgtccatgtagggctctcgcaacgcccggctgaaggcggagaagaggaggcaggatactaaaaaggtacagctcaaggcggccgagaaatagtaaccttccagctgcgccattccagctcccacagccactgcccaagaacctactcctggaaaattctgagcctggaaacccgagctggaaacttgggctcgaaatgggcgcgctaggcgggact

SEQ ID NO: 8372 - RNA, 2136 nt, Homo sapiens
  source 1..2136: mol_type = other RNA
aaaaaccacaattacttttgcatcaacctaatactttctcttcttgccctttctcaggttttagtttcctcttctcttttattccttcctcccacatttgatgcaagtaaaagccaggggaatgtaagcatcacatccctacctctttctaggaatagaaagatgggattgttttcacctgtcttccaagcctgggtggacagacagtagatgaagaacatcggtttcttgttcaggaaagggaagaagtggtttctgtgggacatgggtgagcttctttagctctcattcttgtagaactaaggtttctagatacacacagaacattcttcctcaaggagttcatttgagaatcacacagagagactatttaacctgaagagagctttcggcattttaaaaatggcaagtcttacagactccataaccactaccactgctaccaccacaaccacagagagagccagatctgaaaatacaggaactgatctgaaaatataggaactgaaaattcagtcagtcaaatttggagttgatttgggcagaggataggagatgaacaggctgaggatgtttctccagccaagacaagagtgcagcattttttttagttgaaattaaaaagaaaatgcagagtgtactttgtcccactcatttaccctaacgatcttcagcgtgtctctgtttctaaggaagtggagggcccaagtctctgattcatttccggaatgccacatagcacccttggatgaaagctcctctatccaagacgactttggaaacgccttttaaagtgttctttccctttacatcttggagttccattttgatggcagaaagtatattttaatcaatagagtcaaatgcagttaacatctgagtacacagattttgaatatgtctggcaagaaacaccttaataaagatgacaacttgacaacctcctacaatttattacataattaattgtggctattttttaaatatctagaacccaggaaccaggaaactccagcttttaaaatcaaattatctttgcatttagttctccccctttctcccttctccacatcaaaaaaatctaatttattccaaaacacagaattcagcaatacactaccatcaccctaaggtttaacattcttcctactaagaataagttaaaacagcacattatcctcaaatttggaggttaggaagagaaatatatgggaagatataacagctatccttaaattgcaatttgagggccaccgtcatttgcattctgcttgccctgaggcggcacatcgatgtgcagagtcatggtggcggcagcctggcctgggtgacagaaaccattaaagggaagcagaggggcaggccgtgctccgtgggtttcattagcttacttcttgtgtaggaggcaaaaggtatctgcagggctctgggcttgctaaccaaaccgttaatcgcttagaaacagcaagaagttcactagtgagatgtttatcacatacctggaacacgagttgactttctgtgagacatcattctggaatgaaagccaaaatctctctgctattcagttgaggctgaaaaaacaatcacatcagaattagtaaggcaaaagacaaagagagagaaatgaaaacaagccagtattcaatggggctagggggaaaattacctgggcttcaggaattacaggagagttggggttttgagaaggtaaaaaagtgggccaggtgcggtggctcaagcttgtaatcccagcactttggaacgccaaggcaggtggatcacgagctcaagagattgagaccagcctggccaacatggtgaaaccctgtctctactaaaaacacaaaaattagccgggcgtggtggcgggcgcctgtagtcccagctactccagaggctgaggcaggagaatcgcttgaacccgggagggggaggttgcagtgagccgagattgtgtctcagtgctccagcctggcaacagagcgagactctggctcaaaaaaaagaaaaaaaaaaaaaaagtggtagcactgcttctctcagaaagacaaatgtctggaatacacaagtggcactgaatgtctcaggtcactgagagaggctggacagaggactgtgggaaagtgcaagtac

SEQ ID NO: 8373 - RNA, 43 nt, Homo sapiens
  source 1..43: mol_type = other RNA
aaaaaccacaattacttttgcgccaacctaaatatatagtctg

SEQ ID NO: 8374 - RNA, 29 nt, Homo sapiens
  source 1..29: mol_type = other RNA
aaaaactgcaatcacttttgcaccaacct

SEQ ID NO: 8375 - RNA, 867 nt, Homo sapiens
  source 1..867: mol_type = other RNA
aaaaactgtaattacttttgcaccagcctaatattttctcaggccccaccccaggccaacagaatctatatctcaatggtgaagctcaagaatggacagctctgacaagtgcatcaggtgtttctgatgcccagtcgggtaggaaaatgacaaggttacatggatttggtctctttaaactataaacagttatgtttaatgagttgccaaggaactaaatacatagacatctgtaaccaggaataactttgtctcagataagccatctacgaataatcaggcaggcctgcaccttggcccaaaactccagacgttacctggtttccgacctagatgttagctgccaggctttgggtctgcctgctcacctgcccacctcccagattcctgatgcctgtcccctggtctggtatgattaccactgctcaagcctctctaaattcccggaagagattttctgaaaacaaaacatggtgtagaaaaatagtacaaaagaaacatgttctagaaatgaaaggtctatgttctaggagaagatttatgttccagaaacagaaattcctcctcctctgtatagatgtgcatcttgaaaaggtacttaaccagctactgttttgcactttcattatagtgctaagcactctgtgtttgctacatcatttaatcctttcttatattttgagatagggccattattattttatttacagatgagaacacaaaggctcagagagattgaataacttgtctaaggccagacagtgaacgaaaggcagaactgggattctaatttagtcttgactcttcacatctatgatggtgtttccccagtgtcctcatctgtaaaacaggaataatattggccag

SEQ ID NO: 8376 - RNA, 32 nt, Homo sapiens
  source 1..32: mol_type = other RNA
aaaaactgtgattacttttgcaccaacctaat

SEQ ID NO: 8377 - RNA, 3200 nt, Homo sapiens
  source 1..3200: mol_type = other RNA
aaaacggtgagattttgttttaaatgtagccatatttcaaaaggtaaaaagttggcttctatatttaatggcaagtgggacatcttctattttaaaattaacattcaaaaagtagtaaaatatacactatcatgaacacgatgtgttttatagaatggattcatgtccgaatactaatctgaatgtggaagaaatgtattatctgttaaaaaccacactggaaaaatgttcttttttataaaaagtagcttgaagtaaaaaggaacttgctaataaagccagtaaactttcacacgtgggatttttaaaaaatctccacccatcccacctctgaaaaaaaaagaaggagaagaataaaagaaagaaaaagaaaaaacccatatggtcaatctgagtagagccattcattacatgactgctcattctgtacaatgtggaagcctggttatttaggaaatatttcgtttcctaaagtgcatcttttgaagatttgcctagtaaaactgcaatatcatatacaaaacacttaacacaagacatgcaataacaaagctaaatcattccagtgtaaagttgttaaaactacttttaaaacttttgtttcaccaagaaataaagatgtaaaatacagtagcattcttgttctccaacagtatgcattgtatgcttttgttatttggcaaatcttttagagtcgaacaaaaataatagtctaaacaacatttcttctgtcattataatacgaatcccgggcagaacagtaagatgtagaggaagagttagatttttggaagctttggtgcattaaccacaggatttgcctcgtgcaagtatctcctccctgcactcttgtaatcataggtacagccatgagtttctgcataacgatgagatgcacagaagttgtttccacatctgcattcgtagctactagccagtcctgttttctttccacaaagaaaacaatgatttgttgttttcttctttgtctgaagaggggctttcacaggtgggaggtgatgagtagtacattctccaaaaaaactcctgtatgttctaactggggagaacttttcctaaagttttcttcctgaaaatgctggaggtttgtagacagcccagttccagagttctgaagcctgcctgccccacgtgtgctctgtaatctatttctgcttgtgctcccggccagtgaggcaagaaaactgatattatttacacaaccaacaggctctttggaagccttgttagtcatttctgtgatatcccgagcctcaactttggaaataacatcagatcttttcccaagtgaatcaactttaacaccttgaaagcaagtagtcctagagaaagaagaatcagttatgttttgaacatccagtgactgagaagaagaaggctgtagcttcccaaactcaaaacatttggactgtctctctggtttcaccagagaattatgtagcgacattggtgcagaacagcgaagaggtgacaagagtctattcttgtgaggacttaattcccggtagttaagaactgaagtctctactgattccccattcagcactcctgcaacatgcttgagatgctgctctggagctttcaaccctttgtcagcattagtgagtagcaactccagattcactttgcacgcaccttctaagccgctgctctgttcatcagcatttccttctgcaaatgaagccagtgagcccactttaggtagaagtgattgttcggttacacattcttctgaaggtaagacaatgttcccattactagatggcaagtttcctaaaaaatgttttgtttgcctaggcagggatgatccaagatggagaacagagtcagcaagctcctggtcatttcccaactccaaatggggtatctgaggaggtagtttgacgttgctactgaagtgagacagtgtgttattctcccagctattatcttccttaagaaattcaccagtgatagaagatatgtatctctcagcagagagttgagttgccaaacttgaaattccattcctggagatttcgggcggatatgcattcccaaaagcaggtgaacaagattgaccaatgttggggaggacccttaacaatcggtggcgagatggtgcagtggaaccactagaaggtcgaggagctacaggtgggtgaggttttatcttgacagctttcttaggctttttgctgagattcatgttcttcatcttagccttcagcagcttcatcttattcatagttattgaattttcaattatctgttgcccagaagaagaaggctcagtttcttcatcctcatctgtatctgaattatacatagaaccaccactcatacgatgttctccttttctccgtaggacatgcaaatgaaaatctattttctttgaagagtcagataacggtgttaaagtgccatctcccctatctactgcaggaaagaaattcaattgatctccttcttggtataccaaaaatgtaacttgtttgctgcaggaggtcttctcccagacctcaactcgactggaatccaagtactctgccatcttcctaagtggatcgtctgtaggaactcttctagtatttataggtccgccacgcatagccaaaactagcttcaaggtacacccttctgaaatgcttccaatcttcgaatttttgctttcacagaaataacagtttcaaaaggtgaaactctcagctcaaaacatgttccagttaatgtttcaatgaagagctccatggtatcacagaaatgaagtctgtagtaaaatggtcccatgttatcatcattgaagaatggaggctcttttctgttatccattactttgacttttctagttcttctaaaatatgtcgcaggcaactgtattccagttctaggcaaaccaggtttgaagattggtaatatatattgttgttcatgttttgagttttgtacacacttgaggccaccgagtcacctgcgcagccgttgctcctccaagaccaatccgggctccccagacccaccggcctgaatctggaggacagcagtccgcgtgacaacagcgactcggagatcagcacccgtcgggaaagccgcgtacccgttgaagctggcgtcacgcccaaaggaacaaacgccagagcgtgtgtcctgggcaaaggcggcccgccgctccggtccccgggcagcagcggccggcgtca

SEQ ID NO: 8378 - RNA, 3095 nt, Homo sapiens
  source 1..3095: mol_type = other RNA
aaaacggtgagattttgttttaaatgtagccatatttcaaaaggtaaaaagttggcttctatatttaatggcaagtgggacatcttctattttaaaattaacattcaaaaagtagtaaaatatacactatcatgaacacgatgtgttttatagaatggattcatgtccgaatactaatctgaatgtggaagaaatgtattatctgttaaaaaccacactggaaaaatgttcttttttataaaaagtagcttgaagtaaaaaggaacttgctaataaagccagtaaactttcacacgtgggatttttaaaaaatctccacccatcccacctctgaaaaaaaaagaaggagaagaataaaagaaagaaaaagaaaaaacccatatggtcaatctgagtagagccattcattacatgactgctcattctgtacaatgtggaagcctggttatttaggaaatatttcgtttcctaaagtgcatcttttgaagatttgcctagtaaaactgcaatatcatatacaaaacacttaacacaagacatgcaataacaaagctaaatcattccagtgtaaagttgttaaaactacttttaaaacttttgtttcaccaagaaataaagatgtaaaatacagtagcattcttgttctccaacagtatgcattgtatgcttttgttatttggcaaatcttttagagtcgaacaaaaataatagtctaaacaacatttcttctgtcattataatacgaatcccgggcagaacagtaagatgtagaggaagagttagatttttggaagctttggtgcattaaccacaggatttgcctcgtgcaagtatctcctccctgcactcttgtaatcataggtacagccatgagtttctgcataacgatgagatgcacagaagttgtttccacatctgcattcgtagctactagccagtcctgttttctttccacaaagaaaacaatgatttgttgttttcttctttgtctgaagaggggctttcacaggtgggaggtgatgagtagtacattctccaaaaaaactcctgtatgttctaactggggagaacttttcctaaagttttcttcctgaaaatgctggaggtttgtagacagcccagttccagagttctgaagcctgcctgccccacgtgtgctctgtaatctatttctgcttgtgctcccggccagtgaggcaagaaaactgatattatttacacaaccaacaggctctttggaagccttgttagtcatttctgtgatatcccgagcctcaactttggaaataacatcagatcttttcccaagtgaatcaactttaacaccttgaaagcaagtagtcctagagaaagaagaatcagttatgttttgaacatccagtgactgagaagaagaaggctgtagcttcccaaactcaaaacatttggactgtctctctggtttcaccagagaattatgtagcgacattggtgcagaacagcgaagaggtgacaagagtctattcttgtgaggacttaattcccggtagttaagaactgaagtctctactgattccccattcagcactcctgcaacatgcttgagatgctgctctggagctttcaaccctttgtcagcattagtgagtagcaactccagattcactttgcacgcaccttctaagccgctgctctgttcatcagcatttccttctgcaaatgaagccagtgagcccactttaggtagaagtgattgttcggttacacattcttctgaaggtaagacaatgttcccattactagatggcaagtttcctaaaaaatgttttgtttgcctaggcagggatgatccaagatggagaacagagtcagcaagctcctggtcatttcccaactccaaatggggtatctgaggaggtagtttgacgttgctactgaagtgagacagtgtgttattctcccagctattatcttccttaagaaattcaccagtgatagaagatatgtatctctcagcagagagttgagttgccaaacttgaaattccattcctggagatttcgggcggatatgcattcccaaaagcaggtgaacaagattgaccaatgttggggaggacccttaacaatcggtggcgagatggtgcagtggaaccactagaaggtcgaggagctacaggtgggtgaggttttatcttgacagctttcttaggctttttgctgagattcatgttcttcatcttagccttcagcagcttcatcttattcatagttattgaattttcaattatctgttgcccagaagaagaaggctcagtttcttcatcctcatctgtatctgaattatacatagaaccaccactcatacgatgttctccttttctccgtaggacatgcaaatgaaaatctattttctttgaagagtcagataacggtgttaaagtgccatctcccctatctactgcaggaaagaaattcaattgatctccttcttggtataccaaaaatgtaacttgtttgctgcaggaggtcttctcccagacctcaactcgactggaatccaagtactctgccatcttcctaagtggatcgtctgtaggaactcttctagtatttataggtccgccacgcatagccaaaactagcttcaaggtacacccttctgaaatgcttccaatcttcgaatttttgctttcacagaaataacagtttcaaaaggtgaaactctcagctcaaaacatgttccagttaatgtttcaatgaagagctccatggtatcacagaaatgaagtctgtagtaaaatggtcccatgttatcatcattgaagaatggaggctcttttctgttatccattactttgacttttctagttcttctaaaatatgtcgcaggcaactgtattccagttctaggcaaaccaggtttgaagattggtaatatatattgttgttcatgttttgagttttgtaccaatcgctggacggcgctttcgctgccctccaatcagcgcgggcgggggcaggcctggcccccggacgtgggcggttgccggggcgccagggccctggggccttcttggcattcgctggaggttgtgagttacgaggcccggatgt

SEQ ID NO: 8379 - RNA, 3476 nt, Homo sapiens
  source 1..3476: mol_type = other RNA
aaaacggtgagattttgttttaaatgtagccatatttcaaaaggtaaaaagttggcttctatatttaatggcaagtgggacatcttctattttaaaattaacattcaaaaagtagtaaaatatacactatcatgaacacgatgtgttttatagaatggattcatgtccgaatactaatctgaatgtggaagaaatgtattatctgttaaaaaccacactggaaaaatgttcttttttataaaaagtagcttgaagtaaaaaggaacttgctaataaagccagtaaactttcacacgtgggatttttaaaaaatctccacccatcccacctctgaaaaaaaaagaaggagaagaataaaagaaagaaaaagaaaaaacccatatggtcaatctgagtagagccattcattacatgactgctcattctgtacaatgtggaagcctggttatttaggaaatatttcgtttcctaaagtgcatcttttgaagatttgcctagtaaaactgcaatatcatatacaaaacacttaacacaagacatgcaataacaaagctaaatcattccagtgtaaagttgttaaaactacttttaaaacttttgtttcaccaagaaataaagatgtaaaatacagtagcattcttgttctccaacagtatgcattgtatgcttttgttatttggcaaatcttttagagtcgaacaaaaataatagtctaaacaacatttcttctgtcattataatacgaatcccgggcagaacagtaagatgtagaggaagagttagatttttggaagctttggtgcattaaccacaggatttgcctcgtgcaagtatctcctccctgcactcttgtaatcataggtacagccatgagtttctgcataacgatgagatgcacagaagttgtttccacatctgcattcgtagctactagccagtcctgttttctttccacaaagaaaacaatgatttgttgttttcttctttgtctgaagaggggctttcacaggtgggaggtgatgagtagtacattctccaaaaaaactcctgtatgttctaactggggagaacttttcctaaagttttcttcctgaaaatgctggaggtttgtagacagcccagttccagagttctgaagcctgcctgccccacgtgtgctctgtaatctatttctgcttgtgctcccggccagtgaggcaagaaaactgatattatttacacaaccaacaggctctttggaagccttgttagtcatttctgtgatatcccgagcctcaactttggaaataacatcagatcttttcccaagtgaatcaactttaacaccttgaaagcaagtagtcctagagaaagaagaatcagttatgttttgaacatccagtgactgagaagaagaaggctgtagcttcccaaactcaaaacatttggactgtctctctggtttcaccagagaattatgtagcgacattggtgcagaacagcgaagaggtgacaagagtctattcttgtgaggacttaattcccggtagttaagaactgaagtctctactgattccccattcagcactcctgcaacatgcttgagatgctgctctggagctttcaaccctttgtcagcattagtgagtagcaactccagattcactttgcacgcaccttctaagccgctgctctgttcatcagcatttccttctgcaaatgaagccagtgagcccactttaggtagaagtgattgttcggttacacattcttctgaaggtaagacaatgttcccattactagatggcaagtttcctaaaaaatgttttgtttgcctaggcagggatgatccaagatggagaacagagtcagcaagctcctggtcatttcccaactccaaatggggtatctgaggaggtagtttgacgttgctactgaagtgagacagtgtgttattctcccagctattatcttccttaagaaattcaccagtgatagaagatatgtatctctcagcagagagttgagttgccaaacttgaaattccattcctggagatttcgggcggatatgcattcccaaaagcaggtgaacaagattgaccaatgttggggaggacccttaacaatcggtggcgagatggtgcagtggaaccactagaaggtcgaggagctacaggtgggtgaggttttatcttgacagctttcttaggctttttgctgagattcatgttcttcatcttagccttcagcagcttcatcttattcatagttattgaattttcaattatctgttgcccagaagaagaaggctcagtttcttcatcctcatctgtatctgaattatacatagaaccaccactcatacgatgttctccttttctccgtaggacatgcaaatgaaaatctattttctttgaagagtcagataacggtgttaaagtgccatctcccctatctactgcaggaaagaaattcaattgatctccttcttggtataccaaaaatgtaacttgtttgctgcaggaggtcttctcccagacctcaactcgactggaatccaagtactctgccatcttcctaagtggatcgtctgtaggaactcttctagtatttataggtccgccacgcatagccaaaactagcttcaaggtacacccttctgaaatgcttccaatcttcgaatttttgctttcacagaaataacagtttcaaaaggtgaaactctcagctcaaaacatgttccagttaatgtttcaatgaagagctccatggtatcacagaaatgaagtctgtagtaaaatggtcccatgttatcatcattgaagaatggaggctcttttctgttatccattactttgacttttctagttcttctaaaatatgtcgcaggcaactgtattccagttctaggcaaaccaggtttgaagattggtaatatatattgttgttcatgttttgagttttgtacctgcgcagccgttgctcctccaagaccaatccgggctccccagacccaccggcctgaatctggaggacagcagtccgcgtgacaacagcgactcggagatcagcacccgtcgggaaagccgcgtacccgttgaagctggcgtcacgcccaaaggaacaaacgccagagcgtgtgtcctgggcaaaggcggcccgccgctccggtccccgggcagcagcggccggcgtcaggccgcaaggcgaggggcggggacaggactctacccggcagcccagcgccgagcgcccgcgccactccggccttgcgccattccggccccacgacggccggcggcggcagcgcggctgggctcagcggctcgcagcccgggcgccccccctgccggccgctcgctagctcagcctcacccgcagtcttgtccgctggctcgctcgcccgcctacaggtcgacagggcccaacgacccggcgagcaacttcacggaaggcactggccgacaacgctccgctgccgccgcgccccgcccc

SEQ ID NO: 8380 - RNA, 3122 nt, Homo sapiens
  source 1..3122: mol_type = other RNA
aaaacggtgagattttgttttaaatgtagccatatttcaaaaggtaaaaagttggcttctatatttaatggcaagtgggacatcttctattttaaaattaacattcaaaaagtagtaaaatatacactatcatgaacacgatgtgttttatagaatggattcatgtccgaatactaatctgaatgtggaagaaatgtattatctgttaaaaaccacactggaaaaatgttcttttttataaaaagtagcttgaagtaaaaaggaacttgctaataaagccagtaaactttcacacgtgggatttttaaaaaatctccacccatcccacctctgaaaaaaaaagaaggagaagaataaaagaaagaaaaagaaaaaacccatatggtcaatctgagtagagccattcattacatgactgctcattctgtacaatgtggaagcctggttatttaggaaatatttcgtttcctaaagtgcatcttttgaagatttgcctagtaaaactgcaatatcatatacaaaacacttaacacaagacatgcaataacaaagctaaatcattccagtgtaaagttgttaaaactacttttaaaacttttgtttcaccaagaaataaagatgtaaaatacagtagcattcttgttctccaacagtatgcattgtatgcttttgttatttggcaaatcttttagagtcgaacaaaaataatagtctaaacaacatttcttctgtcattataatacgaatcccgggcagaacagtaagatgtagaggaagagttagatttttggaagctttggtgcattaaccacaggatttgcctcgtgcaagtatctcctccctgcactcttgtaatcataggtacagccatgagtttctgcataacgatgagatgcacagaagttgtttccacatctgcattcgtagctactagccagtcctgttttctttccacaaagaaaacaatgatttgttgttttcttctttgtctgaagaggggctttcacaggtgggaggtgatgagtagtacattctccaaaaaaactcctgtatgttctaactggggagaacttttcctaaagttttcttcctgaaaatgctggaggtttgtagacagcccagttccagagttctgaagcctgcctgccccacgtgtgctctgtaatctatttctgcttgtgctcccggccagtgaggcaagaaaactgatattatttacacaaccaacaggctctttggaagccttgttagtcatttctgtgatatcccgagcctcaactttggaaataacatcagatcttttcccaagtgaatcaactttaacaccttgaaagcaagtagtcctagagaaagaagaatcagttatgttttgaacatccagtgactgagaagaagaaggctgtagcttcccaaactcaaaacatttggactgtctctctggtttcaccagagaattatgtagcgacattggtgcagaacagcgaagaggtgacaagagtctattcttgtgaggacttaattcccggtagttaagaactgaagtctctactgattccccattcagcactcctgcaacatgcttgagatgctgctctggagctttcaaccctttgtcagcattagtgagtagcaactccagattcactttgcacgcaccttctaagccgctgctctgttcatcagcatttccttctgcaaatgaagccagtgagcccactttaggtagaagtgattgttcggttacacattcttctgaaggtaagacaatgttcccattactagatggcaagtttcctaaaaaatgttttgtttgcctaggcagggatgatccaagatggagaacagagtcagcaagctcctggtcatttcccaactccaaatggggtatctgaggaggtagtttgacgttgctactgaagtgagacagtgtgttattctcccagctattatcttccttaagaaattcaccagtgatagaagatatgtatctctcagcagagagttgagttgccaaacttgaaattccattcctggagatttcgggcggatatgcattcccaaaagcaggtgaacaagattgaccaatgttggggaggacccttaacaatcggtggcgagatggtgcagtggaaccactagaaggtcgaggagctacaggtgggtgaggttttatcttgacagctttcttaggctttttgctgagattcatgttcttcatcttagccttcagcagcttcatcttattcatagttattgaattttcaattatctgttgcccagaagaagaaggctcagtttcttcatcctcatctgtatctgaattatacatagaaccaccactcatacgatgttctccttttctccgtaggacatgcaaatgaaaatctattttctttgaagagtcagataacggtgttaaagtgccatctcccctatctactgcaggaaagaaattcaattgatctccttcttggtataccaaaaatgtaacttgtttgctgcaggaggtcttctcccagacctcaactcgactggaatccaagtactctgccatcttcctaagtggatcgtctgtaggaactcttctagtatttataggtccgccacgcatagccaaaactagcttcaaggtacacccttctgaaatgttgtaatcattcaagcaataatcattttcaagttccatgttattccaaattaagtgttgtcgacagatgggaataccttccaatcttcgaatttttgctttcacagaaataacagtttcaaaaggtgaaactctcagctcaaaacatgttccagttaatgtttcaatgaagagctccatggtatcacagaaatgaagtctgtagtaaaatggtcccatgttatcatcattgaagaatggaggctcttttctgttatccattactttgacttttctagttcttctaaaatatgtcgcaggcaactgtattccagttctaggcaaaccaggtttgaagattggtaatatatattgttgttcatgttttgagttttgtacccgcagtcttgtccgctggctcgctcgcccgcctacaggtcgacagggcccaacgacccggcgagcaacttcacggaaggcactggccgacaacgct

SEQ ID NO: 8381 - RNA, 3408 nt, Homo sapiens
  source 1..3408: mol_type = other RNA
aaaacggtgagattttgttttaaatgtagccatatttcaaaaggtaaaaagttggcttctatatttaatggcaagtgggacatcttctattttaaaattaacattcaaaaagtagtaaaatatacactatcatgaacacgatgtgttttatagaatggattcatgtccgaatactaatctgaatgtggaagaaatgtattatctgttaaaaaccacactggaaaaatgttcttttttataaaaagtagcttgaagtaaaaaggaacttgctaataaagccagtaaactttcacacgtgggatttttaaaaaatctccacccatcccacctctgaaaaaaaaagaaggagaagaataaaagaaagaaaaagaaaaaacccatatggtcaatctgagtagagccattcattacatgactgctcattctgtacaatgtggaagcctggttatttaggaaatatttcgtttcctaaagtgcatcttttgaagatttgcctagtaaaactgcaatatcatatacaaaacacttaacacaagacatgcaataacaaagctaaatcattccagtgtaaagttgttaaaactacttttaaaacttttgtttcaccaagaaataaagatgtaaaatacagtagcattcttgttctccaacagtatgcattgtatgcttttgttatttggcaaatcttttagagtcgaacaaaaataatagtctaaacaacatttcttctgtcattataatacgaatcccgggcagaacagtaagatgtagaggaagagttagatttttggaagctttggtgcattaaccacaggatttgcctcgtgcaagtatctcctccctgcactcttgtaatcataggtacagccatgagtttctgcataacgatgagatgcacagaagttgtttccacatctgcattcgtagctactagccagtcctgttttctttccacaaagaaaacaatgatttgttgttttcttctttgtctgaagaggggctttcacaggtgggaggtgatgagtagtacattctccaaaaaaactcctgtatgttctaactggggagaacttttcctaaagttttcttcctgaaaatgctggaggtttgtagacagcccagttccagagttctgaagcctgcctgccccacgtgtgctctgtaatctatttctgcttgtgctcccggccagtgaggcaagaaaactgatattatttacacaaccaacaggctctttggaagccttgttagtcatttctgtgatatcccgagcctcaactttggaaataacatcagatcttttcccaagtgaatcaactttaacaccttgaaagcaagtagtcctagagaaagaagaatcagttatgttttgaacatccagtgactgagaagaagaaggctgtagcttcccaaactcaaaacatttggactgtctctctggtttcaccagagaattatgtagcgacattggtgcagaacagcgaagaggtgacaagagtctattcttgtgaggacttaattcccggtagttaagaactgaagtctctactgattccccattcagcactcctgcaacatgcttgagatgctgctctggagctttcaaccctttgtcagcattagtgagtagcaactccagattcactttgcacgcaccttctaagccgctgctctgttcatcagcatttccttctgcaaatgaagccagtgagcccactttaggtagaagtgattgttcggttacacattcttctgaaggtaagacaatgttcccattactagatggcaagtttcctaaaaaatgttttgtttgcctaggcagggatgatccaagatggagaacagagtcagcaagctcctggtcatttcccaactccaaatggggtatctgaggaggtagtttgacgttgctactgaagtgagacagtgtgttattctcccagctattatcttccttaagaaattcaccagtgatagaagatatgtatctctcagcagagagttgagttgccaaacttgaaattccattcctggagatttcgggcggatatgcattcccaaaagcaggtgaacaagattgaccaatgttggggaggacccttaacaatcggtggcgagatggtgcagtggaaccactagaaggtcgaggagctacaggtgggtgaggttttatcttgacagctttcttaggctttttgctgagattcatgttcttcatcttagccttcagcagcttcatcttattcatagttattgaattttcaattatctgttgcccagaagaagaaggctcagtttcttcatcctcatctgtatctgaattatacatagaaccaccactcatacgatgttctccttttctccgtaggacatgcaaatgaaaatctattttctttgaagagtcagataacggtgttaaagtgccatctcccctatctactgcaggaaagaaattcaattgatctccttcttggtataccaaaaatgtaacttgtttgctgcaggaggtcttctcccagacctcaactcgactggaatccaagtactctgccatcttcctaagtggatcgtctgtaggaacttccaatcttcgaatttttgctttcacagaaataacagtttcaaaaggtgaaactctcagctcaaaacatgttccagttaatgtttcaatgaagagctccatggtatcacagaaatgaagtctgtagtaaaatggtcccatgttatcatcattgaagaatggaggctcttttctgttatccattactttgacttttctagttcttctaaaatatgtcgcaggcaactgtattccagttctaggcaaaccaggtttgaagattggtaatatatattgttgttcatgttttgagttttgtacctgcgcagccgttgctcctccaagaccaatccgggctccccagacccaccggcctgaatctggaggacagcagtccgcgtgacaacagcgactcggagatcagcacccgtcgggaaagccgcgtacccgttgaagctggcgtcacgcccaaaggaacaaacgccagagcgtgtgtcctgggcaaaggcggcccgccgctccggtccccgggcagcagcggccggcgtcaggccgcaaggcgaggggcggggacaggactctacccggcagcccagcgccgagcgcccgcgccactccggccttgcgccattccggccccacgacggccggcggcggcagcgcggctgggctcagcggctcgcagcccgggcgccccccctgccggccgctcgctagctcagcctcacccgcagtcttgtccgctggctcgctcgcccgcctacaggtcgacagggcccaacgacccggcgagcaacttcacggaaggcactggccgacaacgctccgctgccgccgcgccccgcccc

SEQ ID NO: 8382 - RNA, 2940 nt, Homo sapiens
  source 1..2940: mol_type = other RNA
aaaacggtgagattttgttttaaatgtagccatatttcaaaaggtaaaaagttggcttctatatttaatggcaagtgggacatcttctattttaaaattaacattcaaaaagtagtaaaatatacactatcatgaacacgatgtgttttatagaatggattcatgtccgaatactaatctgaatgtggaagaaatgtattatctgttaaaaaccacactggaaaaatgttcttttttataaaaagtagcttgaagtaaaaaggaacttgctaataaagccagtaaactttcacacgtgggatttttaaaaaatctccacccatcccacctctgaaaaaaaaagaaggagaagaataaaagaaagaaaaagaaaaaacccatatggtcaatctgagtagagccattcattacatgactgctcattctgtacaatgtggaagcctggttatttaggaaatatttcgtttcctaaagtgcatcttttgaagatttgcctagtaaaactgcaatatcatatacaaaacacttaacacaagacatgcaataacaaagctaaatcattccagtgtaaagttgttaaaactacttttaaaacttttgtttcaccaagaaataaagatgtaaaatacagtagcattcttgttctccaacagtatgcattgtatgcttttgttatttggcaaatcttttagagtcgaacaaaaataatagtctaaacaacatttcttctgtcattataatacgaatcccgggcagaacagtaagatgtagaggaagagttagatttttggaagctttggtgcattaaccacaggatttgcctcgtgcaagtatctcctccctgcactcttgtaatcataggtacagccatgagtttctgcataacgatgagatgcacagaagttgtttccacatctgcattcgtagctactagccagtcctgttttctttccacaaagaaaacaatgatttgttgttttcttctttgtctgaagaggggctttcacaggtgggaggtgatgagtagtacattctccaaaaaaactcctgtatgttctaactggggagaacttttcctaaagttttcttcctgaaaatgctggaggtttgtagacagcccagttccagagttctgaagcctgcctgccccacgtgtgctctgtaatctatttctgcttgtgctcccggccagtgaggcaagaaaactgatattatttacacaaccaacaggctctttggaagccttgttagtcatttctgtgatatcccgagcctcaactttggaaataacatcagatcttttcccaagtgaatcaactttaacaccttgaaagcaagtagtcctagagaaagaagaatcagttatgttttgaacatccagtgactgagaagaagaaggctgtagcttcccaaactcaaaacatttggactgtctctctggtttcaccagagaattatgtagcgacattggtgcagaacagcgaagaggtgacaagagtctattcttgtgaggacttaattcccggtagttaagaactgaagtctctactgattccccattcagcactcctgcaacatgcttgagatgctgctctggagctttcaaccctttgtcagcattagtgagtagcaactccagattcactttgcacgcaccttctaagccgctgctctgttcatcagcatttccttctgcaaatgaagccagtgagcccactttaggtagaagtgattgttcggttacacattcttctgaaggtaagacaatgttcccattactagatggcaagtttcctaaaaaatgttttgtttgcctaggcagggatgatccaagatggagaacagagtcagcaagctcctggtcatttcccaactccaaatggggtatctgaggaggtagtttgacgttgctactgaagtgagacagtgtgttattctcccagctattatcttccttaagaaattcaccagtgatagaagatatgtatctctcagcagagagttgagttgccaaacttgaaattccattcctggagatttcgggcggatatgcattcccaaaagcaggtgaacaagattgaccaatgttggggaggacccttaacaatcggtggcgagatggtgcagtggaaccactagaaggtcgaggagctacaggtgggtgaggttttatcttgacagctttcttaggctttttgctgagattcatgttcttcatcttagccttcagcagcttcatcttattcatagttattgaattttcaattatctgttgcccagaagaagaaggctcagtttcttcatcctcatctgtatctgaattatacatagaaccaccactgcaaagaaaacaataactcatacgatgttctccttttctccgtaggacatgcaaatgaaaatctattttctttgaagagtcagataacggtgttaaagtgccatctcccctatctactgcaggaaagaaattcaattgatctccttcttggtataccaaaaatgtaacttgtttgctgcaggaggtcttctcccagacctcaactcgactggaatccaagtactctgccatcttcctaagtggatcgtctgtaggaactcttctagtatttataggtccgccacgcatagccaaaactagcttcaaggtacacccttctgaaatgttgtaatcattcaagcaataatcattttcaagttccatgttattccaaattaagtgttgtcgacagatgggaataccttccaatcttcgaatttttgctttcacagaaataacagtttcaaaaggtgaaactctcagctcaaaacatgttccagttaatgtttcaatgaagagctccatggtatcacagaaatgaagtctgtagtaaaatggtcccatgttatcatcattgaagaatggaggctcttttctgttatccattactttgacttttc

SEQ ID NO: 8383 - RNA, 2604 nt, Homo sapiens
  source 1..2604: mol_type = other RNA
aaaacggtgagattttgttttaaatgtagccatatttcaaaaggtaaaaagttggcttctatatttaatggcaagtgggacatcttctattttaaaattaacattcaaaaagtagtaaaatatacactatcatgaacacgatgtgttttatagaatggattcatgtccgaatactaatctgaatgtggaagaaatgtattatctgttaaaaaccacactggaaaaatgttcttttttataaaaagtagcttgaagtaaaaaggaacttgctaataaagccagtaaactttcacacgtgggatttttaaaaaatctccacccatcccacctctgaaaaaaaaagaaggagaagaataaaagaaagaaaaagaaaaaacccatatggtcaatctgagtagagccattcattacatgactgctcattctgtacaatgtggaagcctggttatttaggaaatatttcgtttcctaaagtgcatcttttgaagatttgcctagtaaaactgcaatatcatatacaaaacacttaacacaagacatgcaataacaaagctaaatcattccagtgtaaagttgttaaaactacttttaaaacttttgtttcaccaagaaataaagatgtaaaatacagtagcattcttgttctccaacagtatgcattgtatgcttttgttatttggcaaatcttttagagtcgaacaaaaataatagtctaaacaacatttcttctgtcattataatacgaatcccgggcagaacagtaagatgtagaggaagagttagatttttggaagctttggtgcattaaccacaggatttgcctcgtgcaagtatctcctccctgcactcttgtaatcataggtacagccatgagtttctgcataacgatgagatgcacagaagttgtttccacatctgcattcgtagctactagccagtcctgttttctttccacaaagaaaacaatgatttgttgttttcttctttgtctgaagaggggctttcacaggtgggaggtgatgagtagtacattctcctacgcttttccctgctgctgcattatttccattcattccaacaccatgggtagacaaaaaaactcctgtatgttctaactggggagaacttttcctaaagttttcttcctgaaaatgctggaggtttgtagacagcccagttccagagttctgaagcctgcctgccccacgtgtgctctgtaatctatttctgcttgtgctcccggccagtgaggcaagaaaactgatattatttacacaaccaacaggctctttggaagccttgttagtcatttctgtgatatcccgagcctcaactttggaaataacatcagatcttttcccaagtgaatcaactttaacaccttgaaagcaagtagtcctagagaaagaagaatcagttatgttttgaacatccagtgactgagaagaagaaggctgtagcttcccaaactcaaaacatttggactgtctctctggtttcaccagagaattatgtagcgacattggtgcagaacagcgaagaggtgacaagagtctattcttgtgaggacttaattcccggtagttaagaactgaagtctctactgattccccattcagcactcctgcaacatgcttgagatgctgctctggagctttcaaccctttgtcagcattagtgagtagcaactccagattcactttgcacgcaccttctaagccgctgctctgttcatcagcatttccttctgcaaatgaagccagtgagcccactttaggtagaagtgattgttcggttacacattcttctgaaggtaagacaatgttcccattactagatggcaagtttcctaaaaaatgttttgtttgcctaggcagggatgatccaagatggagaacagagtcagcaagctcctggtcatttcccaactccaaatggggtatctgaggaggtagtttgacgttgctactgaagtgagacagtgtgttattctcccagctattatcttccttaagaaattcaccagtgatagaagatatgtatctctcagcagagagttgagttgccaaacttgaaattccattcctggagatttcgggcggatatgcattcccaaaagcaggtgaacaagattgaccaatgttggggaggacccttaacaatcggtggcgagatggtgcagtggaaccactagaaggtcgaggagctacaggtgggtgaggttttatcttgacagctttcttaggctttttgctgagattcatgttcttcatcttagccttcagcagcttcatcttattcatagttattgaattttcaattatctgttgcccagaagaagaaggctcagtttcttcatcctcatctgtatctgaattatacatagaaccaccaatgtttgttttgccccttattctcccacatgtaagcaagttgaaagcagacattagactttatcttctgagtctgcaccaggcacagcgcttggcacatagccaataaatgtttgatgaactcatacgatgttctccttttctccgtaggacatgcaaatgaaaatctattttctttgaagagtcagataacggtgttaaagtgccatct

SEQ ID NO: 8384 - RNA, 3255 nt, Homo sapiens
  source 1..3255: mol_type = other RNA
aaaacggtgagattttgttttaaatgtagccatatttcaaaaggtaaaaagttggcttctatatttaatggcaagtgggacatcttctattttaaaattaacattcaaaaagtagtaaaatatacactatcatgaacacgatgtgttttatagaatggattcatgtccgaatactaatctgaatgtggaagaaatgtattatctgttaaaaaccacactggaaaaatgttcttttttataaaaagtagcttgaagtaaaaaggaacttgctaataaagccagtaaactttcacacgtgggatttttaaaaaatctccacccatcccacctctgaaaaaaaaagaaggagaagaataaaagaaagaaaaagaaaaaacccatatggtcaatctgagtagagccattcattacatgactgctcattctgtacaatgtggaagcctggttatttaggaaatatttcgtttcctaaagtgcatcttttgaagatttgcctagtaaaactgcaatatcatatacaaaacacttaacacaagacatgcaataacaaagctaaatcattccagtgtaaagttgttaaaactacttttaaaacttttgtttcaccaagaaataaagatgtaaaatacagtagcattcttgttctccaacagtatgcattgtatgcttttgttatttggcaaatcttttagagtcgaacaaaaataatagtctaaacaacatttcttctgtcattataatacgaatcccgggcagaacagtaagatgtagaggaagagttagatttttggaagctttggtgcattaaccacaggatttgcctcgtgcaagtatctcctccctgcactcttgtaatcataggtacagccatgagtttctgcataacgatgagatgcacagaagttgtttccacatctgcattcgtagctactagccagtcctgttttctttccacaaagaaaacaatgatttgttgttttcttctttgtctgaagaggggctttcacaggtgggaggtgatgagtagtacattctcctacgcttttccctgctgctgcattatttccattcattccaacaccatgggtagacaaaaaaactcctgtatgttctaactggggagaacttttcctaaagttttcttcctgaaaatgctggaggtttgtagacagcccagttccagagttctgaagcctgcctgccccacgtgtgctctgtaatctatttctgcttgtgctcccggccagtgaggcaagaaaactgatattatttacacaaccaacaggctctttggaagccttgttagtcatttctgtgatatcccgagcctcaactttggaaataacatcagatcttttcccaagtgaatcaactttaacaccttgaaagcaagtagtcctagagaaagaagaatcagttatgttttgaacatccagtgactgagaagaagaaggctgtagcttcccaaactcaaaacatttggactgtctctctggtttcaccagagaattatgtagcgacattggtgcagaacagcgaagaggtgacaagagtctattcttgtgaggacttaattcccggtagttaagaactgaagtctctactgattccccattcagcactcctgcaacatgcttgagatgctgctctggagctttcaaccctttgtcagcattagtgagtagcaactccagattcactttgcacgcaccttctaagccgctgctctgttcatcagcatttccttctgcaaatgaagccagtgagcccactttaggtagaagtgattgttcggttacacattcttctgaaggtaagacaatgttcccattactagatggcaagtttcctaaaaaatgttttgtttgcctaggcagggatgatccaagatggagaacagagtcagcaagctcctggtcatttcccaactccaaatggggtatctgaggaggtagtttgacgttgctactgaagtgagacagtgtgttattctcccagctattatcttccttaagaaattcaccagtgatagaagatatgtatctctcagcagagagttgagttgccaaacttgaaattccattcctggagatttcgggcggatatgcattcccaaaagcaggtgaacaagattgaccaatgttggggaggacccttaacaatcggtggcgagatggtgcagtggaaccactagaaggtcgaggagctacaggtgggtgaggttttatcttgacagctttcttaggctttttgctgagattcatgttcttcatcttagccttcagcagcttcatcttattcatagttattgaattttcaattatctgttgcccagaagaagaaggctcagtttcttcatcctcatctgtatctgaattatacatagaaccaccactcatacgatgttctccttttctccgtaggacatgcaaatgaaaatctattttctttgaagagtcagataacggtgttaaagtgccatctcccctatctactgcaggaaagaaattcaattgatctccttcttggtataccaaaaatgtaacttgtttgctgcaggaggtcttctcccagacctcaactcgactggaatccaagtactctgccatcttcctaagtggatcgtctgtaggaactcttctagtatttataggtccgccacgcatagccaaaactagcttcaaggtacacccttctgaaatgcttccaatcttcgaatttttgctttcacagaaataacagtttcaaaaggtgaaactctcagctcaaaacatgttccagttaatgtttcaatgaagagctccatggtatcacagaaatgaagtctgtagtaaaatggtcccatgttatcatcattgaagaatggaggctcttttctgttatccattactttgacttttctagttcttctaaaatatgtcgcaggcaactgtattccagttctaggcaaaccaggtttgaagattggtaatatatattgttgttcatgttttgagttttgtacacacttgaggccaccgagtcacctgcgcagccgttgctcctccaagaccaatccgggctccccagacccaccggcctgaatctggaggacagcagtccgcgtgacaacagcgactcggagatcagcacccgtcgggaaagccgcgtacccgttgaagctggcgtcacgcccaaaggaacaaacgccagagcgtgtgtcctgggcaaaggcggcccgccgctccggtccccgggcagcagcggccggcgtca

SEQ ID NO: 8385 - RNA, 3088 nt, Homo sapiens
  source 1..3088: mol_type = other RNA
aaaacggtgagattttgttttaaatgtagccatatttcaaaaggtaaaaagttggcttctatatttaatggcaagtgggacatcttctattttaaaattaacattcaaaaagtagtaaaatatacactatcatgaacacgatgtgttttatagaatggattcatgtccgaatactaatctgaatgtggaagaaatgtattatctgttaaaaaccacactggaaaaatgttcttttttataaaaagtagcttgaagtaaaaaggaacttgctaataaagccagtaaactttcacacgtgggatttttaaaaaatctccacccatcccacctctgaaaaaaaaagaaggagaagaataaaagaaagaaaaagaaaaaacccatatggtcaatctgagtagagccattcattacatgactgctcattctgtacaatgtggaagcctggttatttaggaaatatttcgtttcctaaagtgcatcttttgaagatttgcctagtaaaactgcaatatcatatacaaaacacttaacacaagacatgcaataacaaagctaaatcattccagtgtaaagttgttaaaactacttttaaaacttttgtttcaccaagaaataaagatgtaaaatacagtagcattcttgttctccaacagtatgcattgtatgcttttgttatttggcaaatcttttagagtcgaacaaaaataatagtctaaacaacatttcttctgtcattataatacgaatcccgggcagaacagtaagatgtagaggaagagttagatttttggaagctttggtgcattaaccacaggatttgcctcgtgcaagtatctcctccctgcactcttgtaatcataggtacagccatgagtttctgcataacgatgagatgcacagaagttgtttccacatctgcattcgtagctactagccagtcctgttttctttccacaaagaaaacaatgatttgttgttttcttctttgtctgaagaggggctttcacaggtgggaggtgatgagtagtacattctcctacgcttttccctgctgctgcattatttccattcattccaacaccatgggtagacaaaaaaactcctgtatgttctaactggggagaacttttcctaaagttttcttcctgaaaatgctggaggtttgtagacagcccagttccagagttctgaagcctgcctgccccacgtgtgctctgtaatctatttctgcttgtgctcccggccagtgaggcaagaaaactgatattatttacacaaccaacaggctctttggaagccttgttagtcatttctgtgatatcccgagcctcaactttggaaataacatcagatcttttcccaagtgaatcaactttaacaccttgaaagcaagtagtcctagagaaagaagaatcagttatgttttgaacatccagtgactgagaagaagaaggctgtagcttcccaaactcaaaacatttggactgtctctctggtttcaccagagaattatgtagcgacattggtgcagaacagcgaagaggtgacaagagtctattcttgtgaggacttaattcccggtagttaagaactgaagtctctactgattccccattcagcactcctgcaacatgcttgagatgctgctctggagctttcaaccctttgtcagcattagtgagtagcaactccagattcactttgcacgcaccttctaagccgctgctctgttcatcagcatttccttctgcaaatgaagccagtgagcccactttaggtagaagtgattgttcggttacacattcttctgaaggtaagacaatgttcccattactagatggcaagtttcctaaaaaatgttttgtttgcctaggcagggatgatccaagatggagaacagagtcagcaagctcctggtcatttcccaactccaaatggggtatctgaggaggtagtttgacgttgctactgaagtgagacagtgtgttattctcccagctattatcttccttaagaaattcaccagtgatagaagatatgtatctctcagcagagagttgagttgccaaacttgaaattccattcctggagatttcgggcggatatgcattcccaaaagcaggtgaacaagattgaccaatgttggggaggacccttaacaatcggtggcgagatggtgcagtggaaccactagaaggtcgaggagctacaggtgggtgaggttttatcttgacagctttcttaggctttttgctgagattcatgttcttcatcttagccttcagcagcttcatcttattcatagttattgaattttcaattatctgttgcccagaagaagaaggctcagtttcttcatcctcatctgtatctgaattatacatagaaccaccactcatacgatgttctccttttctccgtaggacatgcaaatgaaaatctattttctttgaagagtcagataacggtgttaaagtgccatctcccctatctactgcaggaaagaaattcaattgatctccttcttggtataccaaaaatgtaacttgtttgctgcaggaggtcttctcccagacctcaactcgactggaatccaagtactctgccatcttcctaagtggatcgtctgtaggaactcttctagtatttataggtccgccacgcatagccaaaactagcttcaaggtacacccttctgaaatgcttccaatcttcgaatttttgctttcacagaaataacagtttcaaaaggtgaaactctcagctcaaaacatgttccagttaatgtttcaatgaagagctccatggtatcacagaaatgaagtctgtagtaaaatggtcccatgttatcatcattgaagaatggaggctcttttctgttatccattactttgacttttctagttcttctaaaatatgtcgcaggcaactgtattccagttctaggcaaaccaggtttgaagattggtaatatatattgttgttcatgttttgagttttgtacccgcagtcttgtccgctggctcgctcgcccgcctacaggtcgacagggcccaacgacccggcgagcaacttcacggaaggcact

SEQ ID NO: 8386 - RNA, 3665 nt, Homo sapiens
  source 1..3665: mol_type = other RNA
aaaacggtgagattttgttttaaatgtagccatatttcaaaaggtaaaaagttggcttctatatttaatggcaagtgggacatcttctattttaaaattaacattcaaaaagtagtaaaatatacactatcatgaacacgatgtgttttatagaatggattcatgtccgaatactaatctgaatgtggaagaaatgtattatctgttaaaaaccacactggaaaaatgttcttttttataaaaagtagcttgaagtaaaaaggaacttgctaataaagccagtaaactttcacacgtgggatttttaaaaaatctccacccatcccacctctgaaaaaaaaagaaggagaagaataaaagaaagaaaaagaaaaaacccatatggtcaatctgagtagagccattcattacatgactgctcattctgtacaatgtggaagcctggttatttaggaaatatttcgtttcctaaagtgcatcttttgaagatttgcctagtaaaactgcaatatcatatacaaaacacttaacacaagacatgcaataacaaagctaaatcattccagtgtaaagttgttaaaactacttttaaaacttttgtttcaccaagaaataaagatgtaaaatacagtagcattcttgttctccaacagtatgcattgtatgcttttgttatttggcaaatcttttagagtcgaacaaaaataatagtctaaacaacatttcttctgtcattataatacgaatcccgggcagaacagtaagatgtagaggaagagttagatttttggaagctttggtgcattaaccacaggatttgcctcgtgcaagtatctcctccctgcactcttgtaatcataggtacagccatgagtttctgcataacgatgagatgcacagaagttgtttccacatctgcattcgtagctactagccagtcctgttttctttccacaaagaaaacaatgatttgttgttttcttctttgtctgaagaggggctttcacaggtgggaggtgatgagtagtacattctcctacgcttttccctgctgctgcattatttccattcattccaacaccatgggtagacaaaaaaactcctgtatgttctaactggggagaacttttcctaaagttttcttcctgaaaatgctggaggtttgtagacagcccagttccagagttctgaagcctgcctgccccacgtgtgctctgtaatctatttctgcttgtgctcccggccagtgaggcaagaaaactgatattatttacacaaccaacaggctctttggaagccttgttagtcatttctgtgatatcccgagcctcaactttggaaataacatcagatcttttcccaagtgaatcaactttaacaccttgaaagcaagtagtcctagagaaagaagaatcagttatgttttgaacatccagtgactgagaagaagaaggctgtagcttcccaaactcaaaacatttggactgtctctctggtttcaccagagaattatgtagcgacattggtgcagaacagcgaagaggtgacaagagtctattcttgtgaggacttaattcccggtagttaagaactgaagtctctactgattccccattcagcactcctgcaacatgcttgagatgctgctctggagctttcaaccctttgtcagcattagtgagtagcaactccagattcactttgcacgcaccttctaagccgctgctctgttcatcagcatttccttctgcaaatgaagccagtgagcccactttaggtagaagtgattgttcggttacacattcttctgaaggtaagacaatgttcccattactagatggcaagtttcctaaaaaatgttttgtttgcctaggcagggatgatccaagatggagaacagagtcagcaagctcctggtcatttcccaactccaaatggggtatctgaggaggtagtttgacgttgctactgaagtgagacagtgtgttattctcccagctattatcttccttaagaaattcaccagtgatagaagatatgtatctctcagcagagagttgagttgccaaacttgaaattccattcctggagatttcgggcggatatgcattcccaaaagcaggtgaacaagattgaccaatgttggggaggacccttaacaatcggtggcgagatggtgcagtggaaccactagaaggtcgaggagctacaggtgggtgaggttttatcttgacagctttcttaggctttttgctgagattcatgttcttcatcttagccttcagcagcttcatcttattcatagttattgaattttcaattatctgttgcccagaagaagaaggctcagtttcttcatcctcatctgtatctgaattatacatagaaccaccactcatacgatgttctccttttctccgtaggacatgcaaatgaaaatctattttctttgaagagtcagataacggtgttaaagtgccatctcccctatctactgcaggaaagaaattcaattgatctccttcttggtataccaaaaatgtaacttgtttgctgcaggaggtcttctcccagacctcaactcgactggaatccaagtactctgccatcttcctaagtggatcgtctgtaggaactcttctagtatttataggtccgccacgcatagccaaaactagcttcaaggtacacccttctgaaatgttgtaatcattcaagcaataatcattttcaagttccatgttattccaaattaagtgttgtcgacagatgggaataccaaatcatttagggcagacaaaagcttcaagagtcattactgaatgtgctgatgtggtcactggactcggccagccactcacttcagtaggatctcctgggtcttccaatcttcgaatttttgctttcacagaaataacagtttcaaaaggtgaaactctcagctcaaaacatgttccagttaatgtttcaatgaagagctccatggtatcacagaaatgaagtctgtagtaaaatggtcccatgttatcatcattgaagaatggaggctcttttctgttatccattactttgacttttctagttcttctaaaatatgtcgcaggcaactgtattccagttctaggcaaaccaggtttgaagattggtaatatatattgttgttcatgttttgagttttgtacacacttgaggccaccgagtcacctgcgcagccgttgctcctccaagaccaatccgggctccccagacccaccggcctgaatctggaggacagcagtccgcgtgacaacagcgactcggagatcagcacccgtcgggaaagccgcgtacccgttgaagctggcgtcacgcccaaaggaacaaacgccagagcgtgtgtcctgggcaaaggcggcccgccgctccggtccccgggcagcagcggccggcgtcaggccgcaaggcgaggggcggggacaggactctacccggcagcccagcgccgagcgcccgcgccactccggccttgcgccattccggccccacgacggccggcggcggcagcgcggctgggctcagcggctcgcagcccgggcgccccccctgccggccgctcgctagctcagcctcacccgcagtcttgtccgctggctcgctcgcccgcctacaggtcgacagggcccaac

SEQ ID NO: 8387 - RNA, 3317 nt, Homo sapiens
  source 1..3317: mol_type = other RNA
aaaacggtgagattttgttttaaatgtagccatatttcaaaaggtaaaaagttggcttctatatttaatggcaagtgggacatcttctattttaaaattaacattcaaaaagtagtaaaatatacactatcatgaacacgatgtgttttatagaatggattcatgtccgaatactaatctgaatgtggaagaaatgtattatctgttaaaaaccacactggaaaaatgttcttttttataaaaagtagcttgaagtaaaaaggaacttgctaataaagccagtaaactttcacacgtgggatttttaaaaaatctccacccatcccacctctgaaaaaaaaagaaggagaagaataaaagaaagaaaaagaaaaaacccatatggtcaatctgagtagagccattcattacatgactgctcattctgtacaatgtggaagcctggttatttaggaaatatttcgtttcctaaagtgcatcttttgaagatttgcctagtaaaactgcaatatcatatacaaaacacttaacacaagacatgcaataacaaagctaaatcattccagtgtaaagttgttaaaactacttttaaaacttttgtttcaccaagaaataaagatgtaaaatacagtagcattcttgttctccaacagtatgcattgtatgcttttgttatttggcaaatcttttagagtcgaacaaaaataatagtctaaacaacatttcttctgtcattataatacgaatcccgggcagaacagtaagatgtagaggaagagttagatttttggaagctttggtgcattaaccacaggatttgcctcgtgcaagtatctcctccctgcactcttgtaatcataggtacagccatgagtttctgcataacgatgagatgcacagaagttgtttccacatctgcattcgtagctactagccagtcctgttttctttccacaaagaaaacaatgatttgttgttttcttctttgtctgaagaggggctttcacaggtgggaggtgatgagtagtacattctcctacgcttttccctgctgctgcattatttccattcattccaacaccatgggtagacaaaaaaactcctgtatgttctaactggggagaacttttcctaaagttttcttcctgaaaatgctggaggtttgtagacagcccagttccagagttctgaagcctgcctgccccacgtgtgctctgtaatctatttctgcttgtgctcccggccagtgaggcaagaaaactgatattatttacacaaccaacaggctctttggaagccttgttagtcatttctgtgatatcccgagcctcaactttggaaataacatcagatcttttcccaagtgaatcaactttaacaccttgaaagcaagtagtcctagagaaagaagaatcagttatgttttgaacatccagtgactgagaagaagaaggctgtagcttcccaaactcaaaacatttggactgtctctctggtttcaccagagaattatgtagcgacattggtgcagaacagcgaagaggtgacaagagtctattcttgtgaggacttaattcccggtagttaagaactgaagtctctactgattccccattcagcactcctgcaacatgcttgagatgctgctctggagctttcaaccctttgtcagcattagtgagtagcaactccagattcactttgcacgcaccttctaagccgctgctctgttcatcagcatttccttctgcaaatgaagccagtgagcccactttaggtagaagtgattgttcggttacacattcttctgaaggtaagacaatgttcccattactagatggcaagtttcctaaaaaatgttttgtttgcctaggcagggatgatccaagatggagaacagagtcagcaagctcctggtcatttcccaactccaaatggggtatctgaggaggtagtttgacgttgctactgaagtgagacagtgtgttattctcccagctattatcttccttaagaaattcaccagtgatagaagatatgtatctctcagcagagagttgagttgccaaacttgaaattccattcctggagatttcgggcggatatgcattcccaaaagcaggtgaacaagattgaccaatgttggggaggacccttaacaatcggtggcgagatggtgcagtggaaccactagaaggtcgaggagctacaggtgggtgaggttttatcttgacagctttcttaggctttttgctgagattcatgttcttcatcttagccttcagcagcttcatcttattcatagttattgaattttcaattatctgttgcccagaagaagaaggctcagtttcttcatcctcatctgtatctgaattatacatagaaccaccactcatacgatgttctccttttctccgtaggacatgcaaatgaaaatctattttctttgaagagtcagataacggtgttaaagtgccatctcccctatctactgcaggaaagaaattcaattgatctccttcttggtataccaaaaatgtaacttgtttgctgcaggaggtcttctcccagacctcaactcgactggaatccaagtactctgccatcttcctaagtggatcgtctgtaggaactcttctagtatttataggtccgccacgcatagccaaaactagcttcaaggtacacccttctgaaatgttgtaatcattcaagcaataatcattttcaagttccatgttattccaaattaagtgttgtcgacagatgggaataccaaatcatttagggcagacaaaagcttcaagagtcattactgaatgtgctgatgtggtcactggactcggccagccactcacttcagtaggatctcctgggtcttccaatcttcgaatttttgctttcacagaaataacagtttcaaaaggtgaaactctcagctcaaaacatgttccagttaatgtttcaatgaagagctccatggtatcacagaaatgaagtctgtagtaaaatggtcccatgttatcatcattgaagaatggaggctcttttctgttatccattactttgacttttctagttcttctaaaatatgtcgcaggcaactgtattccagttctaggcaaaccaggtttgaagattggtaatatatattgttgttcatgttttgagttttgtacccgcagtcttgtccgctggctcgctcgcccgcctacaggtcgacagggcccaacgacccggcgagcaacttcacggaaggcactggccgacaacgctccgctgccgccgcgccccgcccctttgtgacaccacct

SEQ ID NO: 8388 - RNA, 3603 nt, Homo sapiens
  source 1..3603: mol_type = other RNA
aaaacggtgagattttgttttaaatgtagccatatttcaaaaggtaaaaagttggcttctatatttaatggcaagtgggacatcttctattttaaaattaacattcaaaaagtagtaaaatatacactatcatgaacacgatgtgttttatagaatggattcatgtccgaatactaatctgaatgtggaagaaatgtattatctgttaaaaaccacactggaaaaatgttcttttttataaaaagtagcttgaagtaaaaaggaacttgctaataaagccagtaaactttcacacgtgggatttttaaaaaatctccacccatcccacctctgaaaaaaaaagaaggagaagaataaaagaaagaaaaagaaaaaacccatatggtcaatctgagtagagccattcattacatgactgctcattctgtacaatgtggaagcctggttatttaggaaatatttcgtttcctaaagtgcatcttttgaagatttgcctagtaaaactgcaatatcatatacaaaacacttaacacaagacatgcaataacaaagctaaatcattccagtgtaaagttgttaaaactacttttaaaacttttgtttcaccaagaaataaagatgtaaaatacagtagcattcttgttctccaacagtatgcattgtatgcttttgttatttggcaaatcttttagagtcgaacaaaaataatagtctaaacaacatttcttctgtcattataatacgaatcccgggcagaacagtaagatgtagaggaagagttagatttttggaagctttggtgcattaaccacaggatttgcctcgtgcaagtatctcctccctgcactcttgtaatcataggtacagccatgagtttctgcataacgatgagatgcacagaagttgtttccacatctgcattcgtagctactagccagtcctgttttctttccacaaagaaaacaatgatttgttgttttcttctttgtctgaagaggggctttcacaggtgggaggtgatgagtagtacattctcctacgcttttccctgctgctgcattatttccattcattccaacaccatgggtagacaaaaaaactcctgtatgttctaactggggagaacttttcctaaagttttcttcctgaaaatgctggaggtttgtagacagcccagttccagagttctgaagcctgcctgccccacgtgtgctctgtaatctatttctgcttgtgctcccggccagtgaggcaagaaaactgatattatttacacaaccaacaggctctttggaagccttgttagtcatttctgtgatatcccgagcctcaactttggaaataacatcagatcttttcccaagtgaatcaactttaacaccttgaaagcaagtagtcctagagaaagaagaatcagttatgttttgaacatccagtgactgagaagaagaaggctgtagcttcccaaactcaaaacatttggactgtctctctggtttcaccagagaattatgtagcgacattggtgcagaacagcgaagaggtgacaagagtctattcttgtgaggacttaattcccggtagttaagaactgaagtctctactgattccccattcagcactcctgcaacatgcttgagatgctgctctggagctttcaaccctttgtcagcattagtgagtagcaactccagattcactttgcacgcaccttctaagccgctgctctgttcatcagcatttccttctgcaaatgaagccagtgagcccactttaggtagaagtgattgttcggttacacattcttctgaaggtaagacaatgttcccattactagatggcaagtttcctaaaaaatgttttgtttgcctaggcagggatgatccaagatggagaacagagtcagcaagctcctggtcatttcccaactccaaatggggtatctgaggaggtagtttgacgttgctactgaagtgagacagtgtgttattctcccagctattatcttccttaagaaattcaccagtgatagaagatatgtatctctcagcagagagttgagttgccaaacttgaaattccattcctggagatttcgggcggatatgcattcccaaaagcaggtgaacaagattgaccaatgttggggaggacccttaacaatcggtggcgagatggtgcagtggaaccactagaaggtcgaggagctacaggtgggtgaggttttatcttgacagctttcttaggctttttgctgagattcatgttcttcatcttagccttcagcagcttcatcttattcatagttattgaattttcaattatctgttgcccagaagaagaaggctcagtttcttcatcctcatctgtatctgaattatacatagaaccaccactcatacgatgttctccttttctccgtaggacatgcaaatgaaaatctattttctttgaagagtcagataacggtgttaaagtgccatctcccctatctactgcaggaaagaaattcaattgatctccttcttggtataccaaaaatgtaacttgtttgctgcaggaggtcttctcccagacctcaactcgactggaatccaagtactctgccatcttcctaagtggatcgtctgtaggaactcttctagtatttataggtccgccacgcatagccaaaactagcttcaaggtacacccttctgaaatgttgtaatcattcaagcaataatcattttcaagttccatgttattccaaattaagtgttgtcgacagatgggaataccttccaatcttcgaatttttgctttcacagaaataacagtttcaaaaggtgaaactctcagctcaaaacatgttccagttaatgtttcaatgaagagctccatggtatcacagaaatgaagtctgtagtaaaatggtcccatgttatcatcattgaagaatggaggctcttttctgttatccattactttgacttttctagttcttctaaaatatgtcgcaggcaactgtattccagttctaggcaaaccaggtttgaagattggtaatatatattgttgttcatgttttgagttttgtacacacttgaggccaccgagtcacctgcgcagccgttgctcctccaagaccaatccgggctccccagacccaccggcctgaatctggaggacagcagtccgcgtgacaacagcgactcggagatcagcacccgtcgggaaagccgcgtacccgttgaagctggcgtcacgcccaaaggaacaaacgccagagcgtgtgtcctgggcaaaggcggcccgccgctccggtccccgggcagcagcggccggcgtcaggccgcaaggcgaggggcggggacaggactctacccggcagcccagcgccgagcgcccgcgccactccggccttgcgccattccggccccacgacggccggcggcggcagcgcggctgggctcagcggctcgcagcccgggcgccccccctgccggccgctcgctagctcagcctcacccgcagtcttgtccgctggctcgctcgcccgcctacaggtcgacagggcccaacgacccggcgagcaacttcacggaaggcactggccgacaac

SEQ ID NO: 8389 - RNA, 3215 nt, Homo sapiens
  source 1..3215: mol_type = other RNA
aaaacggtgagattttgttttaaatgtagccatatttcaaaaggtaaaaagttggcttctatatttaatggcaagtgggacatcttctattttaaaattaacattcaaaaagtagtaaaatatacactatcatgaacacgatgtgttttatagaatggattcatgtccgaatactaatctgaatgtggaagaaatgtattatctgttaaaaaccacactggaaaaatgttcttttttataaaaagtagcttgaagtaaaaaggaacttgctaataaagccagtaaactttcacacgtgggatttttaaaaaatctccacccatcccacctctgaaaaaaaaagaaggagaagaataaaagaaagaaaaagaaaaaacccatatggtcaatctgagtagagccattcattacatgactgctcattctgtacaatgtggaagcctggttatttaggaaatatttcgtttcctaaagtgcatcttttgaagatttgcctagtaaaactgcaatatcatatacaaaacacttaacacaagacatgcaataacaaagctaaatcattccagtgtaaagttgttaaaactacttttaaaacttttgtttcaccaagaaataaagatgtaaaatacagtagcattcttgttctccaacagtatgcattgtatgcttttgttatttggcaaatcttttagagtcgaacaaaaataatagtctaaacaacatttcttctgtcattataatacgaatcccgggcagaacagtaagatgtagaggaagagttagatttttggaagctttggtgcattaaccacaggatttgcctcgtgcaagtatctcctccctgcactcttgtaatcataggtacagccatgagtttctgcataacgatgagatgcacagaagttgtttccacatctgcattcgtagctactagccagtcctgttttctttccacaaagaaaacaatgatttgttgttttcttctttgtctgaagaggggctttcacaggtgggaggtgatgagtagtacattctcctacgcttttccctgctgctgcattatttccattcattccaacaccatgggtagacaaaaaaactcctgtatgttctaactggggagaacttttcctaaagttttcttcctgaaaatgctggaggtttgtagacagcccagttccagagttctgaagcctgcctgccccacgtgtgctctgtaatctatttctgcttgtgctcccggccagtgaggcaagaaaactgatattatttacacaaccaacaggctctttggaagccttgttagtcatttctgtgatatcccgagcctcaactttggaaataacatcagatcttttcccaagtgaatcaactttaacaccttgaaagcaagtagtcctagagaaagaagaatcagttatgttttgaacatccagtgactgagaagaagaaggctgtagcttcccaaactcaaaacatttggactgtctctctggtttcaccagagaattatgtagcgacattggtgcagaacagcgaagaggtgacaagagtctattcttgtgaggacttaattcccggtagttaagaactgaagtctctactgattccccattcagcactcctgcaacatgcttgagatgctgctctggagctttcaaccctttgtcagcattagtgagtagcaactccagattcactttgcacgcaccttctaagccgctgctctgttcatcagcatttccttctgcaaatgaagccagtgagcccactttaggtagaagtgattgttcggttacacattcttctgaaggtaagacaatgttcccattactagatggcaagtttcctaaaaaatgttttgtttgcctaggcagggatgatccaagatggagaacagagtcagcaagctcctggtcatttcccaactccaaatggggtatctgaggaggtagtttgacgttgctactgaagtgagacagtgtgttattctcccagctattatcttccttaagaaattcaccagtgatagaagatatgtatctctcagcagagagttgagttgccaaacttgaaattccattcctggagatttcgggcggatatgcattcccaaaagcaggtgaacaagattgaccaatgttggggaggacccttaacaatcggtggcgagatggtgcagtggaaccactagaaggtcgaggagctacaggtgggtgaggttttatcttgacagctttcttaggctttttgctgagattcatgttcttcatcttagccttcagcagcttcatcttattcatagttattgaattttcaattatctgttgcccagaagaagaaggctcagtttcttcatcctcatctgtatctgaattatacatagaaccaccactcatacgatgttctccttttctccgtaggacatgcaaatgaaaatctattttctttgaagagtcagataacggtgttaaagtgccatctcccctatctactgcaggaaagaaattcaattgatctccttcttggtataccaaaaatgtaacttgtttgctgcaggaggtcttctcccagacctcaactcgactggaatccaagtactctgccatcttcctaagtggatcgtctgtaggaactcttctagtatttataggtccgccacgcatagccaaaactagcttcaaggtacacccttctgaaatgttgtaatcattcaagcaataatcattttcaagttccatgttattccaaattaagtgttgtcgacagatgggaataccttccaatcttcgaatttttgctttcacagaaataacagtttcaaaaggtgaaactctcagctcaaaacatgttccagttaatgtttcaatgaagagctccatggtatcacagaaatgaagtctgtagtaaaatggtcccatgttatcatcattgaagaatggaggctcttttctgttatccattactttgacttttctagttcttctaaaatatgtcgcaggcaactgtattccagttctaggcaaaccaggtttgaagattggtaatatatattgttgttcatgttttgagttttgtacccgcagtcttgtccgctggctcgctcgcccgcctacaggtcgacagggcccaacgacccggcgagcaacttcacggaaggcactggccgacaacgctccgctgccgccgcgccccgcccctttgtgacaccacct

SEQ ID NO: 8390 - RNA, 3476 nt, Homo sapiens
  source 1..3476: mol_type = other RNA
aaaacggtgagattttgttttaaatgtagccatatttcaaaaggtaaaaagttggcttctatatttaatggcaagtgggacatcttctattttaaaattaacattcaaaaagtagtaaaatatacactatcatgaacacgatgtgttttatagaatggattcatgtccgaatactaatctgaatgtggaagaaatgtattatctgttaaaaaccacactggaaaaatgttcttttttataaaaagtagcttgaagtaaaaaggaacttgctaataaagccagtaaactttcacacgtgggatttttaaaaaatctccacccatcccacctctgaaaaaaaaagaaggagaagaataaaagaaagaaaaagaaaaaacccatatggtcaatctgagtagagccattcattacatgactgctcattctgtacaatgtggaagcctggttatttaggaaatatttcgtttcctaaagtgcatcttttgaagatttgcctagtaaaactgcaatatcatatacaaaacacttaacacaagacatgcaataacaaagctaaatcattccagtgtaaagttgttaaaactacttttaaaacttttgtttcaccaagaaataaagatgtaaaatacagtagcattcttgttctccaacagtatgcattgtatgcttttgttatttggcaaatcttttagagtcgaacaaaaataatagtctaaacaacatttcttctgtcattataatacgaatcccgggcagaacagtaagatgtagaggaagagttagatttttggaagctttggtgcattaaccacaggatttgcctcgtgcaagtatctcctccctgcactcttgtaatcataggtacagccatgagtttctgcataacgatgagatgcacagaagttgtttccacatctgcattcgtagctactagccagtcctgttttctttccacaaagaaaacaatgatttgttgttttcttctttgtctgaagaggggctttcacaggtgggaggtgatgagtagtacattctcctacgcttttccctgctgctgcattatttccattcattccaacaccatgggtagacaaaaaaactcctgtatgttctaactggggagaacttttcctaaagttttcttcctgaaaatgctggaggtttgtagacagcccagttccagagttctgaagcctgcctgccccacgtgtgctctgtaatctatttctgcttgtgctcccggccagtgaggcaagaaaactgatattatttacacaaccaacaggctctttggaagccttgttagtcatttctgtgatatcccgagcctcaactttggaaataacatcagatcttttcccaagtgaatcaactttaacaccttgaaagcaagtagtcctagagaaagaagaatcagttatgttttgaacatccagtgactgagaagaagaaggctgtagcttcccaaactcaaaacatttggactgtctctctggtttcaccagagaattatgtagcgacattggtgcagaacagcgaagaggtgacaagagtctattcttgtgaggacttaattcccggtagttaagaactgaagtctctactgattccccattcagcactcctgcaacatgcttgagatgctgctctggagctttcaaccctttgtcagcattagtgagtagcaactccagattcactttgcacgcaccttctaagccgctgctctgttcatcagcatttccttctgcaaatgaagccagtgagcccactttaggtagaagtgattgttcggttacacattcttctgaaggtaagacaatgttcccattactagatggcaagtttcctaaaaaatgttttgtttgcctaggcagggatgatccaagatggagaacagagtcagcaagctcctggtcatttcccaactccaaatggggtatctgaggaggtagtttgacgttgctactgaagtgagacagtgtgttattctcccagctattatcttccttaagaaattcaccagtgatagaagatatgtatctctcagcagagagttgagttgccaaacttgaaattccattcctggagatttcgggcggatatgcattcccaaaagcaggtgaacaagattgaccaatgttggggaggacccttaacaatcggtggcgagatggtgcagtggaaccactagaaggtcgaggagctacaggtgggtgaggttttatcttgacagctttcttaggctttttgctgagattcatgttcttcatcttagccttcagcagcttcatcttattcatagttattgaattttcaattatctgttgcccagaagaagaaggctcagtttcttcatcctcatctgtatctgaattatacatagaaccaccactcatacgatgttctccttttctccgtaggacatgcaaatgaaaatctattttctttgaagagtcagataacggtgttaaagtgccatctcccctatctactgcaggaaagaaattcaattgatctccttcttggtataccaaaaatgtaacttgtttgctgcaggaggtcttctcccagacctcaactcgactggaatccaagtactctgccatcttcctaagtggatcgtctgtaggaacttccaatcttcgaatttttgctttcacagaaataacagtttcaaaaggtgaaactctcagctcaaaacatgttccagttaatgtttcaatgaagagctccatggtatcacagaaatgaagtctgtagtaaaatggtcccatgttatcatcattgaagaatggaggctcttttctgttatccattactttgacttttctagttcttctaaaatatgtcgcaggcaactgtattccagttctaggcaaaccaggtttgaagattggtaatatatattgttgttcatgttttgagttttgtacacacttgaggccaccgagtcacctgcgcagccgttgctcctccaagaccaatccgggctccccagacccaccggcctgaatctggaggacagcagtccgcgtgacaacagcgactcggagatcagcacccgtcgggaaagccgcgtacccgttgaagctggcgtcacgcccaaaggaacaaacgccagagcgtgtgtcctgggcaaaggcggcccgccgctccggtccccgggcagcagcggccggcgtcaggccgcaaggcgaggggcggggacaggactctacccggcagcccagcgccgagcgcccgcgccactccggccttgcgccattccggccccacgacggccggcggcggcagcgcggctgggctcagcggctcgcagcccgggcgccccccctgccggccgctcgctagctcagcctcacccgcagtcttgtccgctggctcgctcgcccgcctacaggtcgacagggcccaacgacccggcgagcaacttcacggaaggcactggccgacaacgctccgctgccgccgcg

SEQ ID NO: 8391 - RNA, 3047 nt, Homo sapiens
  source 1..3047: mol_type = other RNA
aaaacggtgagattttgttttaaatgtagccatatttcaaaaggtaaaaagttggcttctatatttaatggcaagtgggacatcttctattttaaaattaacattcaaaaagtagtaaaatatacactatcatgaacacgatgtgttttatagaatggattcatgtccgaatactaatctgaatgtggaagaaatgtattatctgttaaaaaccacactggaaaaatgttcttttttataaaaagtagcttgaagtaaaaaggaacttgctaataaagccagtaaactttcacacgtgggatttttaaaaaatctccacccatcccacctctgaaaaaaaaagaaggagaagaataaaagaaagaaaaagaaaaaacccatatggtcaatctgagtagagccattcattacatgactgctcattctgtacaatgtggaagcctggttatttaggaaatatttcgtttcctaaagtgcatcttttgaagatttgcctagtaaaactgcaatatcatatacaaaacacttaacacaagacatgcaataacaaagctaaatcattccagtgtaaagttgttaaaactacttttaaaacttttgtttcaccaagaaataaagatgtaaaatacagtagcattcttgttctccaacagtatgcattgtatgcttttgttatttggcaaatcttttagagtcgaacaaaaataatagtctaaacaacatttcttctgtcattataatacgaatcccgggcagaacagtaagatgtagaggaagagttagatttttggaagctttggtgcattaaccacaggatttgcctcgtgcaagtatctcctccctgcactcttgtaatcataggtacagccatgagtttctgcataacgatgagatgcacagaagttgtttccacatctgcattcgtagctactagccagtcctgttttctttccacaaagaaaacaatgatttgttgttttcttctttgtctgaagaggggctttcacaggtgggaggtgatgagtagtacattctcctacgcttttccctgctgctgcattatttccattcattccaacaccatgggtagacaaaaaaactcctgtatgttctaactggggagaacttttcctaaagttttcttcctgaaaatgctggaggtttgtagacagcccagttccagagttctgaagcctgcctgccccacgtgtgctctgtaatctatttctgcttgtgctcccggccagtgaggcaagaaaactgatattatttacacaaccaacaggctctttggaagccttgttagtcatttctgtgatatcccgagcctcaactttggaaataacatcagatcttttcccaagtgaatcaactttaacaccttgaaagcaagtagtcctagagaaagaagaatcagttatgttttgaacatccagtgactgagaagaagaaggctgtagcttcccaaactcaaaacatttggactgtctctctggtttcaccagagaattatgtagcgacattggtgcagaacagcgaagaggtgacaagagtctattcttgtgaggacttaattcccggtagttaagaactgaagtctctactgattccccattcagcactcctgcaacatgcttgagatgctgctctggagctttcaaccctttgtcagcattagtgagtagcaactccagattcactttgcacgcaccttctaagccgctgctctgttcatcagcatttccttctgcaaatgaagccagtgagcccactttaggtagaagtgattgttcggttacacattcttctgaaggtaagacaatgttcccattactagatggcaagtttcctaaaaaatgttttgtttgcctaggcagggatgatccaagatggagaacagagtcagcaagctcctggtcatttcccaactccaaatggggtatctgaggaggtagtttgacgttgctactgaagtgagacagtgtgttattctcccagctattatcttccttaagaaattcaccagtgatagaagatatgtatctctcagcagagagttgagttgccaaacttgaaattccattcctggagatttcgggcggatatgcattcccaaaagcaggtgaacaagattgaccaatgttggggaggacccttaacaatcggtggcgagatggtgcagtggaaccactagaaggtcgaggagctacaggtgggtgaggttttatcttgacagctttcttaggctttttgctgagattcatgttcttcatcttagccttcagcagcttcatcttattcatagttattgaattttcaattatctgttgcccagaagaagaaggctcagtttcttcatcctcatctgtatctgaattatacatagaaccaccactcatacgatgttctccttttctccgtaggacatgcaaatgaaaatctattttctttgaagagtcagataacggtgttaaagtgccatctcccctatctactgcaggaaagaaattcaattgatctccttcttggtataccaaaaatgtaacttgtttgctgcaggaggtcttctcccagacctcaactcgactggaatccaagtactctgccatcttcctaagtggatcgtctgtaggaacttccaatcttcgaatttttgctttcacagaaataacagtttcaaaaggtgaaactctcagctcaaaacatgttccagttaatgtttcaatgaagagctccatggtatcacagaaatgaagtctgtagtaaaatggtcccatgttatcatcattgaagaatggaggctcttttctgttatccattactttgacttttctagttcttctaaaatatgtcgcaggcaactgtattccagttctaggcaaaccaggtttgaagattggtaatatatattgttgttcatgttttgagttttgtacccgcagtcttgtccgctggctcgctcgcccgcctacaggtcgacagggcccaacgacccggcgagcaacttcacggaaggcactggccgacaacgctccgctgccgccgcg

SEQ ID NO: 8392 - RNA, 3159 nt, Homo sapiens
  source 1..3159: mol_type = other RNA
aaaacggtgagattttgttttaaatgtagccatatttcaaaaggtaaaaagttggcttctatatttaatggcaagtgggacatcttctattttaaaattaacattcaaaaagtagtaaaatatacactatcatgaacacgatgtgttttatagaatggattcatgtccgaatactaatctgaatgtggaagaaatgtattatctgttaaaaaccacactggaaaaatgttcttttttataaaaagtagcttgaagtaaaaaggaacttgctaataaagccagtaaactttcacacgtgggatttttaaaaaatctccacccatcccacctctgaaaaaaaaagaaggagaagaataaaagaaagaaaaagaaaaaacccatatggtcaatctgagtagagccattcattacatgactgctcattctgtacaatgtggaagcctggttatttaggaaatatttcgtttcctaaagtgcatcttttgaagatttgcctagtaaaactgcaatatcatatacaaaacacttaacacaagacatgcaataacaaagctaaatcattccagtgtaaagttgttaaaactacttttaaaacttttgtttcaccaagaaataaagatgtaaaatacagtagcattcttgttctccaacagtatgcattgtatgcttttgttatttggcaaatcttttagagtcgaacaaaaataatagtctaaacaacatttcttctgtcattataatacgaatcccgggcagaacagtaagatgtagaggaagagttagatttttggaagctttggtgcattaaccacaggatttgcctcgtgcaagtatctcctccctgcactcttgtaatcataggtacagccatgagtttctgcataacgatgagatgcacagaagttgtttccacatctgcattcgtagctactagccagtcctgttttctttccacaaagaaaacaatgatttgttgttttcttctttgtctgaagaggggctttcacaggtgggaggtgatgagtagtacattctcctacgcttttccctgctgctgcattatttccattcattccaacaccatgggtagacaaaaaaactcctgtatgttctaactggggagaacttttcctaaagttttcttcctgaaaatgctggaggtttgtagacagcccagttccagagttctgaagcctgcctgccccacgtgtgctctgtaatctatttctgcttgtgctcccggccagtgaggcaagaaaactgatattatttacacaaccaacaggctctttggaagccttgttagtcatttctgtgatatcccgagcctcaactttggaaataacatcagatcttttcccaagtgaatcaactttaacaccttgaaagcaagtagtcctagagaaagaagaatcagttatgttttgaacatccagtgactgagaagaagaaggctgtagcttcccaaactcaaaacatttggactgtctctctggtttcaccagagaattatgtagcgacattggtgcagaacagcgaagaggtgacaagagtctattcttgtgaggacttaattcccggtagttaagaactgaagtctctactgattccccattcagcactcctgcaacatgcttgagatgctgctctggagctttcaaccctttgtcagcattagtgagtagcaactccagattcactttgcacgcaccttctaagccgctgctctgttcatcagcatttccttctgcaaatgaagccagtgagcccactttaggtagaagtgattgttcggttacacattcttctgaaggtaagacaatgttcccattactagatggcaagtttcctaaaaaatgttttgtttgcctaggcagggatgatccaagatggagaacagagtcagcaagctcctggtcatttcccaactccaaatggggtatctgaggaggtagtttgacgttgctactgaagtgagacagtgtgttattctcccagctattatcttccttaagaaattcaccagtgatagaagatatgtatctctcagcagagagttgagttgccaaacttgaaattccattcctggagatttcgggcggatatgcattcccaaaagcaggtgaacaagattgaccaatgttggggaggacccttaacaatcggtggcgagatggtgcagtggaaccactagaaggtcgaggagctacaggtgggtgaggttttatcttgacagctttcttaggctttttgctgagattcatgttcttcatcttagccttcagcagcttcatcttattcatagttattgaattttcaattatctgttgcccagaagaagaaggctcagtttcttcatcctcatctgtatctgaattatacatagaaccaccactcatacgatgttctccttttctccgtaggacatgcaaatgaaaatctattttctttgaagagtcagataacggtgttaaagtgccatctcccctatctactgcaggaaagaaattcaattgatctccttcttggtataccaaaaatgtaacttgtttgctgcaggaggtcttctcccagacctcaactcgactggaatccaagtactctgccatcttcctaagtggatcgtctgtaggaacttccaatcttcgaatttttgctttcacagaaataacagtttcaaaaggtgaaactctcagctcaaaacatgttccagttaatgtttcaatgaagagctccatggtatcacagaaatgaagtctgtagtaaaatggtcccatgttatcatcattgaagaatggaggctcttttctgttatccattactttgacttttctagttcttctaaaatatgtcgcaggcaactgtattccagttctaggcaaaccaggtttgaagattggtaatatatattgttgttcatgttttgagttttgtacctttgaaacattttccccaacataaagatatccggaatgtgaagctgccattaaaactgtgacacagatctacatttactgatacatcaaaacatccctaaagttcgaaatacgagctacagaatcacatcaaccgcctaacttgtctgtagcctaaactctagtccggagttcatctgcaagcggaattgggaagtatttcagagccagcatctcctcgcgc

SEQ ID NO: 8393 - RNA, 3444 nt, Homo sapiens
  source 1..3444: mol_type = other RNA
aaaacggtgagattttgttttaaatgtagccatatttcaaaaggtaaaaagttggcttctatatttaatggcaagtgggacatcttctattttaaaattaacattcaaaaagtagtaaaatatacactatcatgaacacgatgtgttttatagaatggattcatgtccgaatactaatctgaatgtggaagaaatgtattatctgttaaaaaccacactggaaaaatgttcttttttataaaaagtagcttgaagtaaaaaggaacttgctaataaagccagtaaactttcacacgtgggatttttaaaaaatctccacccatcccacctctgaaaaaaaaagaaggagaagaataaaagaaagaaaaagaaaaaacccatatggtcaatctgagtagagccattcattacatgactgctcattctgtacaatgtggaagcctggttatttaggaaatatttcgtttcctaaagtgcatcttttgaagatttgcctagtaaaactgcaatatcatatacaaaacacttaacacaagacatgcaataacaaagctaaatcattccagtgtaaagttgttaaaactacttttaaaacttttgtttcaccaagaaataaagatgtaaaatacagtagcattcttgttctccaacagtatgcattgtatgcttttgttatttggcaaatcttttagagtcgaacaaaaataatagtctaaacaacatttcttctgtcattataatacgaatcccgggcagaacagtaagatgtagaggaagagttagatttttggaagctttggtgcattaaccacaggatttgcctcgtgcaagtatctcctccctgcactcttgtaatcataggtacagccatgagtttctgcataacgatgagatgcacagaagttgtttccacatctgcattcgtagctactagccagtcctgttttctttccacaaagaaaacaatgatttgttgttttcttctttgtctgaagaggggctttcacaggtgggaggtgatgagtagtacattctcctacgcttttccctgctgctgcattatttccattcattccaacaccatgggtagacaaaaaaactcctgtatgttctaactggggagaacttttcctaaagttttcttcctgaaaatgctggaggtttgtagacagcccagttccagagttctgaagcctgcctgccccacgtgtgctctgtaatctatttctgcttgtgctcccggccagtgaggcaagaaaactgatattatttacacaaccaacaggctctttggaagccttgttagtcatttctgtgatatcccgagcctcaactttggaaataacatcagatcttttcccaagtgaatcaactttaacaccttgaaagcaagtagtcctagagaaagaagaatcagttatgttttgaacatccagtgactgagaagaagaaggctgtagcttcccaaactcaaaacatttggactgtctctctggtttcaccagagaattatgtagcgacattggtgcagaacagcgaagaggtgacaagagtctattcttgtgaggacttaattcccggtagttaagaactgaagtctctactgattccccattcagcactcctgcaacatgcttgagatgctgctctggagctttcaaccctttgtcagcattagtgagtagcaactccagattcactttgcacgcaccttctaagccgctgctctgttcatcagcatttccttctgcaaatgaagccagtgagcccactttaggtagaagtgattgttcggttacacattcttctgaaggtaagacaatgttcccattactagatggcaagtttcctaaaaaatgttttgtttgcctaggcagggatgatccaagatggagaacagagtcagcaagctcctggtcatttcccaactccaaatggggtatctgaggaggtagtttgacgttgctactgaagtgagacagtgtgttattctcccagctattatcttccttaagaaattcaccagtgatagaagatatgtatctctcagcagagagttgagttgccaaacttgaaattccattcctggagatttcgggcggatatgcattcccaaaagcaggtgaacaagattgaccaatgttggggaggacccttaacaatcggtggcgagatggtgcagtggaaccactagaaggtcgaggagctacaggtgggtgaggttttatcttgacagctttcttaggctttttgctgagattcatgttcttcatcttagccttcagcagcttcatcttattcatagttattgaattttcaattatctgttgcccagaagaagaaggctcagtttcttcatcctcatctgtatctgaattatacatagaaccaccactcatacgatgttctccttttctccgtaggacatgcaaatgaaaatctattttctttgaagagtcagataacggtgttaaagtgccatctcccctatctactgcaggaaagaaattcaattgatctccttcttggtataccaaaaatgtaacttgtttgctgcaggaggtcttctcccagacctcaactcgactggaatccaagtactctgccatcttcctaagtggatcgtctgtaggaagttagattaaaagtacacagacacggccgggtgcggtggctcatgcctgtaatcccagcactttgggaggccgaggcgggcagatcatgaagtcaagagatcaagaccatcctggccaacatggtgaaaccccgtctctactcttctagtatttataggtccgccacgcatagccaaaactagcttcaaggtacacccttctgaaatgttgtaatcattcaagcaataatcattttcaagttccatgttattccaaattaagtgttgtcgacagatgggaataccttccaatcttcgaatttttgctttcacagaaataacagtttcaaaaggtgaaactctcagctcaaaacatgttccagttaatgtttcaatgaagagctccatggtatcacagaaatgaagtctgtagtaaaatggtcccatgttatcatcattgaagaatggaggctcttttctgttatccattactttgacttttctagttcttctaaaatatgtcgcaggcaactgtattccagttctaggcaaaccaggtttgaagattggtaatatatattgttgttcatgttttgagttttgtacccgttgaagctggcgtcacgcccaaaggaacaaacgccagagcgtgtgtcctgggcaaaggcggcccgccgctccggtccccgggcagcagcggccggcgtcaggccgcaaggcgaggggcggggacaggactctacccggcagcccagcgccgagcgcccgcgccactccggccttgcgccattccggccccacgacggccggcggcggcagcgcggctgggc

SEQ ID NO: 8394 - RNA, 3273 nt, Homo sapiens
  source 1..3273: mol_type = other RNA
aaaacggtgagattttgttttaaatgtagccatatttcaaaaggtaaaaagttggcttctatatttaatggcaagtgggacatcttctattttaaaattaacattcaaaaagtagtaaaatatacactatcatgaacacgatgtgttttatagaatggattcatgtccgaatactaatctgaatgtggaagaaatgtattatctgttaaaaaccacactggaaaaatgttcttttttataaaaagtagcttgaagtaaaaaggaacttgctaataaagccagtaaactttcacacgtgggatttttaaaaaatctccacccatcccacctctgaaaaaaaaagaaggagaagaataaaagaaagaaaaagaaaaaacccatatggtcaatctgagtagagccattcattacatgactgctcattctgtacaatgtggaagcctggttatttaggaaatatttcgtttcctaaagtgcatcttttgaagatttgcctagtaaaactgcaatatcatatacaaaacacttaacacaagacatgcaataacaaagctaaatcattccagtgtaaagttgttaaaactacttttaaaacttttgtttcaccaagaaataaagatgtaaaatacagtagcattcttgttctccaacagtatgcattgtatgcttttgttatttggcaaatcttttagagtcgaacaaaaataatagtctaaacaacatttcttctgtcattataatacgaatcccgggcagaacagtaagatgtagaggaagagttagatttttggaagctttggtgcattaaccacaggatttgcctcgtgcaagtatctcctccctgcactcttgtaatcataggtacagccatgagtttctgcataacgatgagatgcacagaagttgtttccacatctgcattcgtagctactagccagtcctgttttctttccacaaagaaaacaatgatttgttgttttcttctttgtctgaagaggggctttcacaggtgggaggtgatgagtagtacattctcctacgcttttccctgctgctgcattatttccattcattccaacaccatgggtagacaaaaaaactcctgtatgttctaactggggagaacttttcctaaagttttcttcctgaaaatgctggaggtttgtagacagcccagttccagagttctgaagcctgcctgccccacgtgtgctctgtaatctatttctgcttgtgctcccggccagtgaggcaagaaaactgatattatttacacaaccaacaggctctttggaagccttgttagtcatttctgtgatatcccgagcctcaactttggaaataacatcagatcttttcccaagtgaatcaactttaacaccttgaaagcaagtagtcctagagaaagaagaatcagttatgttttgaacatccagtgactgagaagaagaaggctgtagcttcccaaactcaaaacatttggactgtctctctggtttcaccagagaattatgtagcgacattggtgcagaacagcgaagaggtgacaagagtctattcttgtgaggacttaattcccggtagttaagaactgaagtctctactgattccccattcagcactcctgcaacatgcttgagatgctgctctggagctttcaaccctttgtcagcattagtgagtagcaactccagattcactttgcacgcaccttctaagccgctgctctgttcatcagcatttccttctgcaaatgaagccagtgagcccactttaggtagaagtgattgttcggttacacattcttctgaaggtaagacaatgttcccattactagatggcaagtttcctaaaaaatgttttgtttgcctaggcagggatgatccaagatggagaacagagtcagcaagctcctggtcatttcccaactccaaatggggtatctgaggaggtagtttgacgttgctactgaagtgagacagtgtgttattctcccagctattatcttccttaagaaattcaccagtgatagaagatatgtatctctcagcagagagttgagttgccaaacttgaaattccattcctggagatttcgggcggatatgcattcccaaaagcaggtgaacaagattgaccaatgttggggaggacccttaacaatcggtggcgagatggtgcagtggaaccactagaaggtcgaggagctacaggtgggtgaggttttatcttgacagctttcttaggctttttgctgagattcatgttcttcatcttagccttcagcagcttcatcttattcatagttattgaattttcaattatctgttgcccagaagaagaaggctcagtttcttcatcctcatctgtatctgaattatacatagaaccaccactgcaaagaaaacaataactcatacgatgttctccttttctccgtaggacatgcaaatgaaaatctattttctttgaagagtcagataacggtgttaaagtgccatctcccctatctactgcaggaaagaaattcaattgatctccttcttggtataccaaaaatgtaacttgtttgctgcaggaggtcttctcccagacctcaactcgactggaatccaagtactctgccatcttcctaagtggatcgtctgtaggaactcttctagtatttataggtccgccacgcatagccaaaactagcttcaaggtacacccttctgaaatgcttccaatcttcgaatttttgctttcacagaaataacagtttcaaaaggtgaaactctcagctcaaaacatgttccagttaatgtttcaatgaagagctccatggtatcacagaaatgaagtctgtagtaaaatggtcccatgttatcatcattgaagaatggaggctcttttctgttatccattactttgacttttctagttcttctaaaatatgtcgcaggcaactgtattccagttctaggcaaaccaggtttgaagattggtaatatatattgttgttcatgttttgagttttgtacacacttgaggccaccgagtcacctgcgcagccgttgctcctccaagaccaatccgggctccccagacccaccggcctgaatctggaggacagcagtccgcgtgacaacagcgactcggagatcagcacccgtcgggaaagccgcgtacccgttgaagctggcgtcacgcccaaaggaacaaacgccagagcgtgtgtcctgggcaaaggcggcccgccgctccggtccccgggcagcagcggccggcgtca

SEQ ID NO: 8395 - RNA, 3106 nt, Homo sapiens
  source 1..3106: mol_type = other RNA
aaaacggtgagattttgttttaaatgtagccatatttcaaaaggtaaaaagttggcttctatatttaatggcaagtgggacatcttctattttaaaattaacattcaaaaagtagtaaaatatacactatcatgaacacgatgtgttttatagaatggattcatgtccgaatactaatctgaatgtggaagaaatgtattatctgttaaaaaccacactggaaaaatgttcttttttataaaaagtagcttgaagtaaaaaggaacttgctaataaagccagtaaactttcacacgtgggatttttaaaaaatctccacccatcccacctctgaaaaaaaaagaaggagaagaataaaagaaagaaaaagaaaaaacccatatggtcaatctgagtagagccattcattacatgactgctcattctgtacaatgtggaagcctggttatttaggaaatatttcgtttcctaaagtgcatcttttgaagatttgcctagtaaaactgcaatatcatatacaaaacacttaacacaagacatgcaataacaaagctaaatcattccagtgtaaagttgttaaaactacttttaaaacttttgtttcaccaagaaataaagatgtaaaatacagtagcattcttgttctccaacagtatgcattgtatgcttttgttatttggcaaatcttttagagtcgaacaaaaataatagtctaaacaacatttcttctgtcattataatacgaatcccgggcagaacagtaagatgtagaggaagagttagatttttggaagctttggtgcattaaccacaggatttgcctcgtgcaagtatctcctccctgcactcttgtaatcataggtacagccatgagtttctgcataacgatgagatgcacagaagttgtttccacatctgcattcgtagctactagccagtcctgttttctttccacaaagaaaacaatgatttgttgttttcttctttgtctgaagaggggctttcacaggtgggaggtgatgagtagtacattctcctacgcttttccctgctgctgcattatttccattcattccaacaccatgggtagacaaaaaaactcctgtatgttctaactggggagaacttttcctaaagttttcttcctgaaaatgctggaggtttgtagacagcccagttccagagttctgaagcctgcctgccccacgtgtgctctgtaatctatttctgcttgtgctcccggccagtgaggcaagaaaactgatattatttacacaaccaacaggctctttggaagccttgttagtcatttctgtgatatcccgagcctcaactttggaaataacatcagatcttttcccaagtgaatcaactttaacaccttgaaagcaagtagtcctagagaaagaagaatcagttatgttttgaacatccagtgactgagaagaagaaggctgtagcttcccaaactcaaaacatttggactgtctctctggtttcaccagagaattatgtagcgacattggtgcagaacagcgaagaggtgacaagagtctattcttgtgaggacttaattcccggtagttaagaactgaagtctctactgattccccattcagcactcctgcaacatgcttgagatgctgctctggagctttcaaccctttgtcagcattagtgagtagcaactccagattcactttgcacgcaccttctaagccgctgctctgttcatcagcatttccttctgcaaatgaagccagtgagcccactttaggtagaagtgattgttcggttacacattcttctgaaggtaagacaatgttcccattactagatggcaagtttcctaaaaaatgttttgtttgcctaggcagggatgatccaagatggagaacagagtcagcaagctcctggtcatttcccaactccaaatggggtatctgaggaggtagtttgacgttgctactgaagtgagacagtgtgttattctcccagctattatcttccttaagaaattcaccagtgatagaagatatgtatctctcagcagagagttgagttgccaaacttgaaattccattcctggagatttcgggcggatatgcattcccaaaagcaggtgaacaagattgaccaatgttggggaggacccttaacaatcggtggcgagatggtgcagtggaaccactagaaggtcgaggagctacaggtgggtgaggttttatcttgacagctttcttaggctttttgctgagattcatgttcttcatcttagccttcagcagcttcatcttattcatagttattgaattttcaattatctgttgcccagaagaagaaggctcagtttcttcatcctcatctgtatctgaattatacatagaaccaccactgcaaagaaaacaataactcatacgatgttctccttttctccgtaggacatgcaaatgaaaatctattttctttgaagagtcagataacggtgttaaagtgccatctcccctatctactgcaggaaagaaattcaattgatctccttcttggtataccaaaaatgtaacttgtttgctgcaggaggtcttctcccagacctcaactcgactggaatccaagtactctgccatcttcctaagtggatcgtctgtaggaactcttctagtatttataggtccgccacgcatagccaaaactagcttcaaggtacacccttctgaaatgcttccaatcttcgaatttttgctttcacagaaataacagtttcaaaaggtgaaactctcagctcaaaacatgttccagttaatgtttcaatgaagagctccatggtatcacagaaatgaagtctgtagtaaaatggtcccatgttatcatcattgaagaatggaggctcttttctgttatccattactttgacttttctagttcttctaaaatatgtcgcaggcaactgtattccagttctaggcaaaccaggtttgaagattggtaatatatattgttgttcatgttttgagttttgtacccgcagtcttgtccgctggctcgctcgcccgcctacaggtcgacagggcccaacgacccggcgagcaacttcacggaaggcact

SEQ ID NO: 8396 - RNA, 3549 nt, Homo sapiens
  source 1..3549: mol_type = other RNA
aaaacggtgagattttgttttaaatgtagccatatttcaaaaggtaaaaagttggcttctatatttaatggcaagtgggacatcttctattttaaaattaacattcaaaaagtagtaaaatatacactatcatgaacacgatgtgttttatagaatggattcatgtccgaatactaatctgaatgtggaagaaatgtattatctgttaaaaaccacactggaaaaatgttcttttttataaaaagtagcttgaagtaaaaaggaacttgctaataaagccagtaaactttcacacgtgggatttttaaaaaatctccacccatcccacctctgaaaaaaaaagaaggagaagaataaaagaaagaaaaagaaaaaacccatatggtcaatctgagtagagccattcattacatgactgctcattctgtacaatgtggaagcctggttatttaggaaatatttcgtttcctaaagtgcatcttttgaagatttgcctagtaaaactgcaatatcatatacaaaacacttaacacaagacatgcaataacaaagctaaatcattccagtgtaaagttgttaaaactacttttaaaacttttgtttcaccaagaaataaagatgtaaaatacagtagcattcttgttctccaacagtatgcattgtatgcttttgttatttggcaaatcttttagagtcgaacaaaaataatagtctaaacaacatttcttctgtcattataatacgaatcccgggcagaacagtaagatgtagaggaagagttagatttttggaagctttggtgcattaaccacaggatttgcctcgtgcaagtatctcctccctgcactcttgtaatcataggtacagccatgagtttctgcataacgatgagatgcacagaagttgtttccacatctgcattcgtagctactagccagtcctgttttctttccacaaagaaaacaatgatttgttgttttcttctttgtctgaagaggggctttcacaggtgggaggtgatgagtagtacattctcctacgcttttccctgctgctgcattatttccattcattccaacaccatgggtagacaaaaaaactcctgtatgttctaactggggagaacttttcctaaagttttcttcctgaaaatgctggaggtttgtagacagcccagttccagagttctgaagcctgcctgccccacgtgtgctctgtaatctatttctgcttgtgctcccggccagtgaggcaagaaaactgatattatttacacaaccaacaggctctttggaagccttgttagtcatttctgtgatatcccgagcctcaactttggaaataacatcagatcttttcccaagtgaatcaactttaacaccttgaaagcaagtagtcctagagaaagaagaatcagttatgttttgaacatccagtgactgagaagaagaaggctgtagcttcccaaactcaaaacatttggactgtctctctggtttcaccagagaattatgtagcgacattggtgcagaacagcgaagaggtgacaagagtctattcttgtgaggacttaattcccggtagttaagaactgaagtctctactgattccccattcagcactcctgcaacatgcttgagatgctgctctggagctttcaaccctttgtcagcattagtgagtagcaactccagattcactttgcacgcaccttctaagccgctgctctgttcatcagcatttccttctgcaaatgaagccagtgagcccactttaggtagaagtgattgttcggttacacattcttctgaaggtaagacaatgttcccattactagatggcaagtttcctaaaaaatgttttgtttgcctaggcagggatgatccaagatggagaacagagtcagcaagctcctggtcatttcccaactccaaatggggtatctgaggaggtagtttgacgttgctactgaagtgagacagtgtgttattctcccagctattatcttccttaagaaattcaccagtgatagaagatatgtatctctcagcagagagttgagttgccaaacttgaaattccattcctggagatttcgggcggatatgcattcccaaaagcaggtgaacaagattgaccaatgttggggaggacccttaacaatcggtggcgagatggtgcagtggaaccactagaaggtcgaggagctacaggtgggtgaggttttatcttgacagctttcttaggctttttgctgagattcatgttcttcatcttagccttcagcagcttcatcttattcatagttattgaattttcaattatctgttgcccagaagaagaaggctcagtttcttcatcctcatctgtatctgaattatacatagaaccaccactgcaaagaaaacaataactcatacgatgttctccttttctccgtaggacatgcaaatgaaaatctattttctttgaagagtcagataacggtgttaaagtgccatctcccctatctactgcaggaaagaaattcaattgatctccttcttggtataccaaaaatgtaacttgtttgctgcaggaggtcttctcccagacctcaactcgactggaatccaagtactctgccatcttcctaagtggatcgtctgtaggaactcttctagtatttataggtccgccacgcatagccaaaactagcttcaaggtacacccttctgaaatgcttccaatcttcgaatttttgctttcacagaaataacagtttcaaaaggtgaaactctcagctcaaaacatgttccagttaatgtttcaatgaagagctccatggtatcacagaaatgaagtctgtagtaaaatggtcccatgttatcatcattgaagaatggaggctcttttctgttatccattactttgacttttctagttcttctaaaatatgtcgcaggcaactgtattccagttctaggcaaaccaggtttgaagattggtaatatatattgttgttcatgttttgagttttgtacctgcgcagccgttgctcctccaagaccaatccgggctccccagacccaccggcctgaatctggaggacagcagtccgcgtgacaacagcgactcggagatcagcacccgtcgggaaagccgcgtacccgttgaagctggcgtcacgcccaaaggaacaaacgccagagcgtgtgtcctgggcaaaggcggcccgccgctccggtccccgggcagcagcggccggcgtcaggccgcaaggcgaggggcggggacaggactctacccggcagcccagcgccgagcgcccgcgccactccggccttgcgccattccggccccacgacggccggcggcggcagcgcggctgggctcagcggctcgcagcccgggcgccccccctgccggccgctcgctagctcagcctcacccgcagtcttgtccgctggctcgctcgcccgcctacaggtcgacagggcccaacgacccggcgagcaacttcacggaaggcactggccgacaacgctccgctgccgccgcgccccgcccc

SEQ ID NO: 8397 - RNA, 3740 nt, Homo sapiens
  source 1..3740: mol_type = other RNA
aaaacggtgagattttgttttaaatgtagccatatttcaaaaggtaaaaagttggcttctatatttaatggcaagtgggacatcttctattttaaaattaacattcaaaaagtagtaaaatatacactatcatgaacacgatgtgttttatagaatggattcatgtccgaatactaatctgaatgtggaagaaatgtattatctgttaaaaaccacactggaaaaatgttcttttttataaaaagtagcttgaagtaaaaaggaacttgctaataaagccagtaaactttcacacgtgggatttttaaaaaatctccacccatcccacctctgaaaaaaaaagaaggagaagaataaaagaaagaaaaagaaaaaacccatatggtcaatctgagtagagccattcattacatgactgctcattctgtacaatgtggaagcctggttatttaggaaatatttcgtttcctaaagtgcatcttttgaagatttgcctagtaaaactgcaatatcatatacaaaacacttaacacaagacatgcaataacaaagctaaatcattccagtgtaaagttgttaaaactacttttaaaacttttgtttcaccaagaaataaagatgtaaaatacagtagcattcttgttctccaacagtatgcattgtatgcttttgttatttggcaaatcttttagagtcgaacaaaaataatagtctaaacaacatttcttctgtcattataatacgaatcccgggcagaacagtaagatgtagaggaagagttagatttttggaagctttggtgcattaaccacaggatttgcctcgtgcaagtatctcctccctgcactcttgtaatcataggtacagccatgagtttctgcataacgatgagatgcacagaagttgtttccacatctgcattcgtagctactagccagtcctgttttctttccacaaagaaaacaatgatttgttgttttcttctttgtctgaagaggggctttcacaggtgggaggtgatgagtagtacattctcctacgcttttccctgctgctgcattatttccattcattccaacaccatgggtagacaaaaaaactcctgtatgttctaactggggagaacttttcctaaagttttcttcctgaaaatgctggaggtttgtagacagcccagttccagagttctgaagcctgcctgccccacgtgtgctctgtaatctatttctgcttgtgctcccggccagtgaggcaagaaaactgatattatttacacaaccaacaggctctttggaagccttgttagtcatttctgtgatatcccgagcctcaactttggaaataacatcagatcttttcccaagtgaatcaactttaacaccttgaaagcaagtagtcctagagaaagaagaatcagttatgttttgaacatccagtgactgagaagaagaaggctgtagcttcccaaactcaaaacatttggactgtctctctggtttcaccagagaattatgtagcgacattggtgcagaacagcgaagaggtgacaagagtctattcttgtgaggacttaattcccggtagttaagaactgaagtctctactgattccccattcagcactcctgcaacatgcttgagatgctgctctggagctttcaaccctttgtcagcattagtgagtagcaactccagattcactttgcacgcaccttctaagccgctgctctgttcatcagcatttccttctgcaaatgaagccagtgagcccactttaggtagaagtgattgttcggttacacattcttctgaaggtaagacaatgttcccattactagatggcaagtttcctaaaaaatgttttgtttgcctaggcagggatgatccaagatggagaacagagtcagcaagctcctggtcatttcccaactccaaatggggtatctgaggaggtagtttgacgttgctactgaagtgagacagtgtgttattctcccagctattatcttccttaagaaattcaccagtgatagaagatatgtatctctcagcagagagttgagttgccaaacttgaaattccattcctggagatttcgggcggatatgcattcccaaaagcaggtgaacaagattgaccaatgttggggaggacccttaacaatcggtggcgagatggtgcagtggaaccactagaaggtcgaggagctacaggtgggtgaggttttatcttgacagctttcttaggctttttgctgagattcatgttcttcatcttagccttcagcagcttcatcttattcatagttattgaattttcaattatctgttgcccagaagaagaaggctcagtttcttcatcctcatctgtatctgaattatacatagaaccaccactgcaaagaaaacaataactcatacgatgttctccttttctccgtaggacatgcaaatgaaaatctattttctttgaagagtcagataacggtgttaaagtgccatctcccctatctactgcaggaaagaaattcaattgatctccttcttggtataccaaaaatgtaacttgtttgctgcaggaggtcttctcccagacctcaactcgactggaatccaagtactctgccatcttcctaagtggatcgtctgtaggaactcttctagtatttataggtccgccacgcatagccaaaactagcttcaaggtacacccttctgaaatgttgtaatcattcaagcaataatcattttcaagttccatgttattccaaattaagtgttgtcgacagatgggaataccaaatcatttagggcagacaaaagcttcaagagtcattactgaatgtgctgatgtggtcactggactcggccagccactcacttcagtaggatctcctgggtcttccaatcttcgaatttttgctttcacagaaataacagtttcaaaaggtgaaactctcagctcaaaacatgttccagttaatgtttcaatgaagagctccatggtatcacagaaatgaagtctgtagtaaaatggtcccatgttatcatcattgaagaatggaggctcttttctgttatccattactttgacttttctagttcttctaaaatatgtcgcaggcaactgtattccagttctaggcaaaccaggtttgaagattggtaatatatattgttgttcatgttttgagttttgtacacacttgaggccaccgagtcacctgcgcagccgttgctcctccaagaccaatccgggctccccagacccaccggcctgaatctggaggacagcagtccgcgtgacaacagcgactcggagatcagcacccgtcgggaaagccgcgtacccgttgaagctggcgtcacgcccaaaggaacaaacgccagagcgtgtgtcctgggcaaaggcggcccgccgctccggtccccgggcagcagcggccggcgtcaggccgcaaggcgaggggcggggacaggactctacccggcagcccagcgccgagcgcccgcgccactccggccttgcgccattccggccccacgacggccggcggcggcagcgcggctgggctcagcggctcgcagcccgggcgccccccctgccggccgctcgctagctcagcctcacccgcagtcttgtccgctggctcgctcgcccgcctacaggtcgacagggcccaacgacccggcgagcaacttcacggaaggcactggccgacaacgctccgctgccgccgcg

SEQ ID NO: 8398 - RNA, 3284 nt, Homo sapiens
  source 1..3284: mol_type = other RNA
aaaacggtgagattttgttttaaatgtagccatatttcaaaaggtaaaaagttggcttctatatttaatggcaagtgggacatcttctattttaaaattaacattcaaaaagtagtaaaatatacactatcatgaacacgatgtgttttatagaatggattcatgtccgaatactaatctgaatgtggaagaaatgtattatctgttaaaaaccacactggaaaaatgttcttttttataaaaagtagcttgaagtaaaaaggaacttgctaataaagccagtaaactttcacacgtgggatttttaaaaaatctccacccatcccacctctgaaaaaaaaagaaggagaagaataaaagaaagaaaaagaaaaaacccatatggtcaatctgagtagagccattcattacatgactgctcattctgtacaatgtggaagcctggttatttaggaaatatttcgtttcctaaagtgcatcttttgaagatttgcctagtaaaactgcaatatcatatacaaaacacttaacacaagacatgcaataacaaagctaaatcattccagtgtaaagttgttaaaactacttttaaaacttttgtttcaccaagaaataaagatgtaaaatacagtagcattcttgttctccaacagtatgcattgtatgcttttgttatttggcaaatcttttagagtcgaacaaaaataatagtctaaacaacatttcttctgtcattataatacgaatcccgggcagaacagtaagatgtagaggaagagttagatttttggaagctttggtgcattaaccacaggatttgcctcgtgcaagtatctcctccctgcactcttgtaatcataggtacagccatgagtttctgcataacgatgagatgcacagaagttgtttccacatctgcattcgtagctactagccagtcctgttttctttccacaaagaaaacaatgatttgttgttttcttctttgtctgaagaggggctttcacaggtgggaggtgatgagtagtacattctcctacgcttttccctgctgctgcattatttccattcattccaacaccatgggtagacaaaaaaactcctgtatgttctaactggggagaacttttcctaaagttttcttcctgaaaatgctggaggtttgtagacagcccagttccagagttctgaagcctgcctgccccacgtgtgctctgtaatctatttctgcttgtgctcccggccagtgaggcaagaaaactgatattatttacacaaccaacaggctctttggaagccttgttagtcatttctgtgatatcccgagcctcaactttggaaataacatcagatcttttcccaagtgaatcaactttaacaccttgaaagcaagtagtcctagagaaagaagaatcagttatgttttgaacatccagtgactgagaagaagaaggctgtagcttcccaaactcaaaacatttggactgtctctctggtttcaccagagaattatgtagcgacattggtgcagaacagcgaagaggtgacaagagtctattcttgtgaggacttaattcccggtagttaagaactgaagtctctactgattccccattcagcactcctgcaacatgcttgagatgctgctctggagctttcaaccctttgtcagcattagtgagtagcaactccagattcactttgcacgcaccttctaagccgctgctctgttcatcagcatttccttctgcaaatgaagccagtgagcccactttaggtagaagtgattgttcggttacacattcttctgaaggtaagacaatgttcccattactagatggcaagtttcctaaaaaatgttttgtttgcctaggcagggatgatccaagatggagaacagagtcagcaagctcctggtcatttcccaactccaaatggggtatctgaggaggtagtttgacgttgctactgaagtgagacagtgtgttattctcccagctattatcttccttaagaaattcaccagtgatagaagatatgtatctctcagcagagagttgagttgccaaacttgaaattccattcctggagatttcgggcggatatgcattcccaaaagcaggtgaacaagattgaccaatgttggggaggacccttaacaatcggtggcgagatggtgcagtggaaccactagaaggtcgaggagctacaggtgggtgaggttttatcttgacagctttcttaggctttttgctgagattcatgttcttcatcttagccttcagcagcttcatcttattcatagttattgaattttcaattatctgttgcccagaagaagaaggctcagtttcttcatcctcatctgtatctgaattatacatagaaccaccactgcaaagaaaacaataactcatacgatgttctccttttctccgtaggacatgcaaatgaaaatctattttctttgaagagtcagataacggtgttaaagtgccatctcccctatctactgcaggaaagaaattcaattgatctccttcttggtataccaaaaatgtaacttgtttgctgcaggaggtcttctcccagacctcaactcgactggaatccaagtactctgccatcttcctaagtggatcgtctgtaggaactcttctagtatttataggtccgccacgcatagccaaaactagcttcaaggtacacccttctgaaatgttgtaatcattcaagcaataatcattttcaagttccatgttattccaaattaagtgttgtcgacagatgggaataccaaatcatttagggcagacaaaagcttcaagagtcattactgaatgtgctgatgtggtcactggactcggccagccactcacttcagtaggatctcctgggtcttccaatcttcgaatttttgctttcacagaaataacagtttcaaaaggtgaaactctcagctcaaaacatgttccagttaatgtttcaatgaagagctccatggtatcacagaaatgaagtctgtagtaaaatggtcccatgttatcatcattgaagaatggaggctcttttctgttatccattactttgacttttctagttcttctaaaatatgtcgcaggcaactgtattccagttctaggcaaaccaggtttgaagattggtaatatatattgttgttcatgttttgagttttgtacccgcagtcttgtccgctggctcgctcgcccgcctacaggtcgacagggcccaacgacccggcgagcaacttcacggaaggcact

SEQ ID NO: 8399 - RNA, 3325 nt, Homo sapiens
  source 1..3325: mol_type = other RNA
aaaacggtgagattttgttttaaatgtagccatatttcaaaaggtaaaaagttggcttctatatttaatggcaagtgggacatcttctattttaaaattaacattcaaaaagtagtaaaatatacactatcatgaacacgatgtgttttatagaatggattcatgtccgaatactaatctgaatgtggaagaaatgtattatctgttaaaaaccacactggaaaaatgttcttttttataaaaagtagcttgaagtaaaaaggaacttgctaataaagccagtaaactttcacacgtgggatttttaaaaaatctccacccatcccacctctgaaaaaaaaagaaggagaagaataaaagaaagaaaaagaaaaaacccatatggtcaatctgagtagagccattcattacatgactgctcattctgtacaatgtggaagcctggttatttaggaaatatttcgtttcctaaagtgcatcttttgaagatttgcctagtaaaactgcaatatcatatacaaaacacttaacacaagacatgcaataacaaagctaaatcattccagtgtaaagttgttaaaactacttttaaaacttttgtttcaccaagaaataaagatgtaaaatacagtagcattcttgttctccaacagtatgcattgtatgcttttgttatttggcaaatcttttagagtcgaacaaaaataatagtctaaacaacatttcttctgtcattataatacgaatcccgggcagaacagtaagatgtagaggaagagttagatttttggaagctttggtgcattaaccacaggatttgcctcgtgcaagtatctcctccctgcactcttgtaatcataggtacagccatgagtttctgcataacgatgagatgcacagaagttgtttccacatctgcattcgtagctactagccagtcctgttttctttccacaaagaaaacaatgatttgttgttttcttctttgtctgaagaggggctttcacaggtgggaggtgatgagtagtacattctcctacgcttttccctgctgctgcattatttccattcattccaacaccatgggtagacaaaaaaactcctgtatgttctaactggggagaacttttcctaaagttttcttcctgaaaatgctggaggtttgtagacagcccagttccagagttctgaagcctgcctgccccacgtgtgctctgtaatctatttctgcttgtgctcccggccagtgaggcaagaaaactgatattatttacacaaccaacaggctctttggaagccttgttagtcatttctgtgatatcccgagcctcaactttggaaataacatcagatcttttcccaagtgaatcaactttaacaccttgaaagcaagtagtcctagagaaagaagaatcagttatgttttgaacatccagtgactgagaagaagaaggctgtagcttcccaaactcaaaacatttggactgtctctctggtttcaccagagaattatgtagcgacattggtgcagaacagcgaagaggtgacaagagtctattcttgtgaggacttaattcccggtagttaagaactgaagtctctactgattccccattcagcactcctgcaacatgcttgagatgctgctctggagctttcaaccctttgtcagcattagtgagtagcaactccagattcactttgcacgcaccttctaagccgctgctctgttcatcagcatttccttctgcaaatgaagccagtgagcccactttaggtagaagtgattgttcggttacacattcttctgaaggtaagacaatgttcccattactagatggcaagtttcctaaaaaatgttttgtttgcctaggcagggatgatccaagatggagaacagagtcagcaagctcctggtcatttcccaactccaaatggggtatctgaggaggtagtttgacgttgctactgaagtgagacagtgtgttattctcccagctattatcttccttaagaaattcaccagtgatagaagatatgtatctctcagcagagagttgagttgccaaacttgaaattccattcctggagatttcgggcggatatgcattcccaaaagcaggtgaacaagattgaccaatgttggggaggacccttaacaatcggtggcgagatggtgcagtggaaccactagaaggtcgaggagctacaggtgggtgaggttttatcttgacagctttcttaggctttttgctgagattcatgttcttcatcttagccttcagcagcttcatcttattcatagttattgaattttcaattatctgttgcccagaagaagaaggctcagtttcttcatcctcatctgtatctgaattatacatagaaccaccactgcaaagaaaacaataactcatacgatgttctccttttctccgtaggacatgcaaatgaaaatctattttctttgaagagtcagataacggtgttaaagtgccatctcccctatctactgcaggaaagaaattcaattgatctccttcttggtataccaaaaatgtaacttgtttgctgcaggaggtcttctcccagacctcaactcgactggaatccaagtactctgccatcttcctaagtggatcgtctgtaggaactcttctagtatttataggtccgccacgcatagccaaaactagcttcaaggtacacccttctgaaatgttgtaatcattcaagcaataatcattttcaagttccatgttattccaaattaagtgttgtcgacagatgggaataccttccaatcttcgaatttttgctttcacagaaataacagtttcaaaaggtgaaactctcagctcaaaacatgttccagttaatgtttcaatgaagagctccatggtatcacagaaatgaagtctgtagtaaaatggtcccatgttatcatcattgaagaatggaggctcttttctgttatccattactttgacttttctagttcttctaaaatatgtcgcaggcaactgtattccagttctaggcaaaccaggtttgaagattggtaatatatattgttgttcatgttttgagttttgtacacacttgaggccaccgagtcacctgcgcagccgttgctcctccaagaccaatccgggctccccagacccaccggcctgaatctggaggacagcagtccgcgtgacaacagcgactcggagatcagcacccgtcgggaaagccgcgtacccgttgaagctggcgtcacgcccaaaggaacaaacgccagagcgtgtgtcctgggcaaaggcggcccgccgctccggtc

SEQ ID NO: 8400 - RNA, 3245 nt, Homo sapiens
  source 1..3245: mol_type = other RNA
aaaacggtgagattttgttttaaatgtagccatatttcaaaaggtaaaaagttggcttctatatttaatggcaagtgggacatcttctattttaaaattaacattcaaaaagtagtaaaatatacactatcatgaacacgatgtgttttatagaatggattcatgtccgaatactaatctgaatgtggaagaaatgtattatctgttaaaaaccacactggaaaaatgttcttttttataaaaagtagcttgaagtaaaaaggaacttgctaataaagccagtaaactttcacacgtgggatttttaaaaaatctccacccatcccacctctgaaaaaaaaagaaggagaagaataaaagaaagaaaaagaaaaaacccatatggtcaatctgagtagagccattcattacatgactgctcattctgtacaatgtggaagcctggttatttaggaaatatttcgtttcctaaagtgcatcttttgaagatttgcctagtaaaactgcaatatcatatacaaaacacttaacacaagacatgcaataacaaagctaaatcattccagtgtaaagttgttaaaactacttttaaaacttttgtttcaccaagaaataaagatgtaaaatacagtagcattcttgttctccaacagtatgcattgtatgcttttgttatttggcaaatcttttagagtcgaacaaaaataatagtctaaacaacatttcttctgtcattataatacgaatcccgggcagaacagtaagatgtagaggaagagttagatttttggaagctttggtgcattaaccacaggatttgcctcgtgcaagtatctcctccctgcactcttgtaatcataggtacagccatgagtttctgcataacgatgagatgcacagaagttgtttccacatctgcattcgtagctactagccagtcctgttttctttccacaaagaaaacaatgatttgttgttttcttctttgtctgaagaggggctttcacaggtgggaggtgatgagtagtacattctcctacgcttttccctgctgctgcattatttccattcattccaacaccatgggtagacaaaaaaactcctgtatgttctaactggggagaacttttcctaaagttttcttcctgaaaatgctggaggtttgtagacagcccagttccagagttctgaagcctgcctgccccacgtgtgctctgtaatctatttctgcttgtgctcccggccagtgaggcaagaaaactgatattatttacacaaccaacaggctctttggaagccttgttagtcatttctgtgatatcccgagcctcaactttggaaataacatcagatcttttcccaagtgaatcaactttaacaccttgaaagcaagtagtcctagagaaagaagaatcagttatgttttgaacatccagtgactgagaagaagaaggctgtagcttcccaaactcaaaacatttggactgtctctctggtttcaccagagaattatgtagcgacattggtgcagaacagcgaagaggtgacaagagtctattcttgtgaggacttaattcccggtagttaagaactgaagtctctactgattccccattcagcactcctgcaacatgcttgagatgctgctctggagctttcaaccctttgtcagcattagtgagtagcaactccagattcactttgcacgcaccttctaagccgctgctctgttcatcagcatttccttctgcaaatgaagccagtgagcccactttaggtagaagtgattgttcggttacacattcttctgaaggtaagacaatgttcccattactagatggcaagtttcctaaaaaatgttttgtttgcctaggcagggatgatccaagatggagaacagagtcagcaagctcctggtcatttcccaactccaaatggggtatctgaggaggtagtttgacgttgctactgaagtgagacagtgtgttattctcccagctattatcttccttaagaaattcaccagtgatagaagatatgtatctctcagcagagagttgagttgccaaacttgaaattccattcctggagatttcgggcggatatgcattcccaaaagcaggtgaacaagattgaccaatgttggggaggacccttaacaatcggtggcgagatggtgcagtggaaccactagaaggtcgaggagctacaggtgggtgaggttttatcttgacagctttcttaggctttttgctgagattcatgttcttcatcttagccttcagcagcttcatcttattcatagttattgaattttcaattatctgttgcccagaagaagaaggctcagtttcttcatcctcatctgtatctgaattatacatagaaccaccactgcaaagaaaacaataactcatacgatgttctccttttctccgtaggacatgcaaatgaaaatctattttctttgaagagtcagataacggtgttaaagtgccatctcccctatctactgcaggaaagaaattcaattgatctccttcttggtataccaaaaatgtaacttgtttgctgcaggaggtcttctcccagacctcaactcgactggaatccaagtactctgccatcttcctaagtggatcgtctgtaggaactcttctagtatttataggtccgccacgcatagccaaaactagcttcaaggtacacccttctgaaatgttgtaatcattcaagcaataatcattttcaagttccatgttattccaaattaagtgttgtcgacagatgggaataccttccaatcttcgaatttttgctttcacagaaataacagtttcaaaaggtgaaactctcagctcaaaacatgttccagttaatgtttcaatgaagagctccatggtatcacagaaatgaagtctgtagtaaaatggtcccatgttatcatcattgaagaatggaggctcttttctgttatccattactttgacttttctagttcttctaaaatatgtcgcaggcaactgtattccagttctaggcaaaccaggtttgaagattggtaatatatattgttgttcatgttttgagttttgtaccaatcgctggacggcgctttcgctgccctccaatcagcgcgggcgggggcaggcctggcccccggacgtgggcggttgccggggcgccagggccctggggccttcttggcattcgctggaggttgtgagttacgaggcccggatgtt

SEQ ID NO: 8401 - RNA, 3195 nt, Homo sapiens
  source 1..3195: mol_type = other RNA
aaaacggtgagattttgttttaaatgtagccatatttcaaaaggtaaaaagttggcttctatatttaatggcaagtgggacatcttctattttaaaattaacattcaaaaagtagtaaaatatacactatcatgaacacgatgtgttttatagaatggattcatgtccgaatactaatctgaatgtggaagaaatgtattatctgttaaaaaccacactggaaaaatgttcttttttataaaaagtagcttgaagtaaaaaggaacttgctaataaagccagtaaactttcacacgtgggatttttaaaaaatctccacccatcccacctctgaaaaaaaaagaaggagaagaataaaagaaagaaaaagaaaaaacccatatggtcaatctgagtagagccattcattacatgactgctcattctgtacaatgtggaagcctggttatttaggaaatatttcgtttcctaaagtgcatcttttgaagatttgcctagtaaaactgcaatatcatatacaaaacacttaacacaagacatgcaataacaaagctaaatcattccagtgtaaagttgttaaaactacttttaaaacttttgtttcaccaagaaataaagatgtaaaatacagtagcattcttgttctccaacagtatgcattgtatgcttttgttatttggcaaatcttttagagtcgaacaaaaataatagtctaaacaacatttcttctgtcattataatacgaatcccgggcagaacagtaagatgtagaggaagagttagatttttggaagctttggtgcattaaccacaggatttgcctcgtgcaagtatctcctccctgcactcttgtaatcataggtacagccatgagtttctgcataacgatgagatgcacagaagttgtttccacatctgcattcgtagctactagccagtcctgttttctttccacaaagaaaacaatgatttgttgttttcttctttgtctgaagaggggctttcacaggtgggaggtgatgagtagtacattctcctacgcttttccctgctgctgcattatttccattcattccaacaccatgggtagacaaaaaaactcctgtatgttctaactggggagaacttttcctaaagttttcttcctgaaaatgctggaggtttgtagacagcccagttccagagttctgaagcctgcctgccccacgtgtgctctgtaatctatttctgcttgtgctcccggccagtgaggcaagaaaactgatattatttacacaaccaacaggctctttggaagccttgttagtcatttctgtgatatcccgagcctcaactttggaaataacatcagatcttttcccaagtgaatcaactttaacaccttgaaagcaagtagtcctagagaaagaagaatcagttatgttttgaacatccagtgactgagaagaagaaggctgtagcttcccaaactcaaaacatttggactgtctctctggtttcaccagagaattatgtagcgacattggtgcagaacagcgaagaggtgacaagagtctattcttgtgaggacttaattcccggtagttaagaactgaagtctctactgattccccattcagcactcctgcaacatgcttgagatgctgctctggagctttcaaccctttgtcagcattagtgagtagcaactccagattcactttgcacgcaccttctaagccgctgctctgttcatcagcatttccttctgcaaatgaagccagtgagcccactttaggtagaagtgattgttcggttacacattcttctgaaggtaagacaatgttcccattactagatggcaagtttcctaaaaaatgttttgtttgcctaggcagggatgatccaagatggagaacagagtcagcaagctcctggtcatttcccaactccaaatggggtatctgaggaggtagtttgacgttgctactgaagtgagacagtgtgttattctcccagctattatcttccttaagaaattcaccagtgatagaagatatgtatctctcagcagagagttgagttgccaaacttgaaattccattcctggagatttcgggcggatatgcattcccaaaagcaggtgaacaagattgaccaatgttggggaggacccttaacaatcggtggcgagatggtgcagtggaaccactagaaggtcgaggagctacaggtgggtgaggttttatcttgacagctttcttaggctttttgctgagattcatgttcttcatcttagccttcagcagcttcatcttattcatagttattgaattttcaattatctgttgcccagaagaagaaggctcagtttcttcatcctcatctgtatctgaattatacatagaaccaccactgcaaagaaaacaataactcatacgatgttctccttttctccgtaggacatgcaaatgaaaatctattttctttgaagagtcagataacggtgttaaagtgccatctcccctatctactgcaggaaagaaattcaattgatctccttcttggtataccaaaaatgtaacttgtttgctgcaggaggtcttctcccagacctcaactcgactggaatccaagtactctgccatcttcctaagtggatcgtctgtaggaactcttctagtatttataggtccgccacgcatagccaaaactagcttcaaggtacacccttctgaaatgttgtaatcattcaagcaataatcattttcaagttccatgttattccaaattaagtgttgtcgacagatgggaataccttccaatcttcgaatttttgctttcacagaaataacagtttcaaaaggtgaaactctcagctcaaaacatgttccagttaatgtttcaatgaagagctccatggtatcacagaaatgaagtctgtagtaaaatggtcccatgttatcatcattgaagaatggaggctcttttctgttatccattactttgacttttctagttcttctaaaatatgtcgcaggcaactgtattccagttctaggcaaaccaggtttgaagattggtaatatatattgttgttcatgttttgagttttgtacccgcagtcttgtccgctggctcgctcgcccgcctacaggtcgacagggcccaacgacccggcgagcaacttcacggaaggcactggccgacaacgct

SEQ ID NO: 8402 - RNA, 3182 nt, Homo sapiens
  source 1..3182: mol_type = other RNA
aaaacggtgagattttgttttaaatgtagccatatttcaaaaggtaaaaagttggcttctatatttaatggcaagtgggacatcttctattttaaaattaacattcaaaaagtagtaaaatatacactatcatgaacacgatgtgttttatagaatggattcatgtccgaatactaatctgaatgtggaagaaatgtattatctgttaaaaaccacactggaaaaatgttcttttttataaaaagtagcttgaagtaaaaaggaacttgctaataaagccagtaaactttcacacgtgggatttttaaaaaatctccacccatcccacctctgaaaaaaaaagaaggagaagaataaaagaaagaaaaagaaaaaacccatatggtcaatctgagtagagccattcattacatgactgctcattctgtacaatgtggaagcctggttatttaggaaatatttcgtttcctaaagtgcatcttttgaagatttgcctagtaaaactgcaatatcatatacaaaacacttaacacaagacatgcaataacaaagctaaatcattccagtgtaaagttgttaaaactacttttaaaacttttgtttcaccaagaaataaagatgtaaaatacagtagcattcttgttctccaacagtatgcattgtatgcttttgttatttggcaaatcttttagagtcgaacaaaaataatagtctaaacaacatttcttctgtcattataatacgaatcccgggcagaacagtaagatgtagaggaagagttagatttttggaagctttggtgcattaaccacaggatttgcctcgtgcaagtatctcctccctgcactcttgtaatcataggtacagccatgagtttctgcataacgatgagatgcacagaagttgtttccacatctgcattcgtagctactagccagtcctgttttctttccacaaagaaaacaatgatttgttgttttcttctttgtctgaagaggggctttcacaggtgggaggtgatgagtagtacattctcctacgcttttccctgctgctgcattatttccattcattccaacaccatgggtagacaaaaaaactcctgtatgttctaactggggagaacttttcctaaagttttcttcctgaaaatgctggaggtttgtagacagcccagttccagagttctgaagcctgcctgccccacgtgtgctctgtaatctatttctgcttgtgctcccggccagtgaggcaagaaaactgatattatttacacaaccaacaggctctttggaagccttgttagtcatttctgtgatatcccgagcctcaactttggaaataacatcagatcttttcccaagtgaatcaactttaacaccttgaaagcaagtagtcctagagaaagaagaatcagttatgttttgaacatccagtgactgagaagaagaaggctgtagcttcccaaactcaaaacatttggactgtctctctggtttcaccagagaattatgtagcgacattggtgcagaacagcgaagaggtgacaagagtctattcttgtgaggacttaattcccggtagttaagaactgaagtctctactgattccccattcagcactcctgcaacatgcttgagatgctgctctggagctttcaaccctttgtcagcattagtgagtagcaactccagattcactttgcacgcaccttctaagccgctgctctgttcatcagcatttccttctgcaaatgaagccagtgagcccactttaggtagaagtgattgttcggttacacattcttctgaaggtaagacaatgttcccattactagatggcaagtttcctaaaaaatgttttgtttgcctaggcagggatgatccaagatggagaacagagtcagcaagctcctggtcatttcccaactccaaatggggtatctgaggaggtagtttgacgttgctactgaagtgagacagtgtgttattctcccagctattatcttccttaagaaattcaccagtgatagaagatatgtatctctcagcagagagttgagttgccaaacttgaaattccattcctggagatttcgggcggatatgcattcccaaaagcaggtgaacaagattgaccaatgttggggaggacccttaacaatcggtggcgagatggtgcagtggaaccactagaaggtcgaggagctacaggtgggtgaggttttatcttgacagctttcttaggctttttgctgagattcatgttcttcatcttagccttcagcagcttcatcttattcatagttattgaattttcaattatctgttgcccagaagaagaaggctcagtttcttcatcctcatctgtatctgaattatacatagaaccaccactgcaaagaaaacaataactcatacgatgttctccttttctccgtaggacatgcaaatgaaaatctattttctttgaagagtcagataacggtgttaaagtgccatctcccctatctactgcaggaaagaaattcaattgatctccttcttggtataccaaaaatgtaacttgtttgctgcaggaggtcttctcccagacctcaactcgactggaatccaagtactctgccatcttcctaagtggatcgtctgtaggaacttccaatcttcgaatttttgctttcacagaaataacagtttcaaaaggtgaaactctcagctcaaaacatgttccagttaatgtttcaatgaagagctccatggtatcacagaaatgaagtctgtagtaaaatggtcccatgttatcatcattgaagaatggaggctcttttctgttatccattactttgacttttctagttcttctaaaatatgtcgcaggcaactgtattccagttctaggcaaaccaggtttgaagattggtaatatatattgttgttcatgttttgagttttgtacccgttgaagctggcgtcacgcccaaaggaacaaacgccagagcgtgtgtcctgggcaaaggcggcccgccgctccggtccccgggcagcagcggccggcgtcaggccgcaaggcgaggggcggggacaggactctacccggcagcccagcgccgagcgcccgcgccactccggccttgcgccattccggccccacgacggccggcggcggcagcgcggctgggctcag

SEQ ID NO: 8403 - RNA, 3334 nt, Homo sapiens
  source 1..3334: mol_type = other RNA
aaaacggtgagattttgttttaaatgtagccatatttcaaaaggtaaaaagttggcttctatatttaatggcaagtgggacatcttctattttaaaattaacattcaaaaagtagtaaaatatacactatcatgaacacgatgtgttttatagaatggattcatgtccgaatactaatctgaatgtggaagaaatgtattatctgttaaaaaccacactggaaaaatgttcttttttataaaaagtagcttgaagtaaaaaggaacttgctaataaagccagtaaactttcacacgtgggatttttaaaaaatctccacccatcccacctctgaaaaaaaaagaaggagaagaataaaagaaagaaaaagaaaaaacccatatggtcaatctgagtagagccattcattacatgactgctcattctgtacaatgtggaagcctggttatttaggaaatatttcgtttcctaaagtgcatcttttgaagatttgcctagtaaaactgcaatatcatatacaaaacacttaacacaagacatgcaataacaaagctaaatcattccagtgtaaagttgttaaaactacttttaaaacttttgtttcaccaagaaataaagatgtaaaatacagtagcattcttgttctccaacagtatgcattgtatgcttttgttatttggcaaatcttttagagtcgaacaaaaataatagtctaaacaacatttcttctgtcattataatacgaatcccgggcagaacagtaagatgtagaggaagagttagatttttggaagctttggtgcattaaccacaggatttgcctcgtgcaagtatctcctccctgcactcttgtaatcataggtacagccatgagtttctgcataacgatgagatgcacagaagttgtttccacatctgcattcgtagctactagccagtcctgttttctttccacaaagaaaacaatgatttgttgttttcttctttgtctgaagaggggctttcacaggtgggaggtgatgagtagtacattctcctacgcttttccctgctgctgcattatttccattcattccaacaccatgggtagacaaaaaaactcctgtatgttctaactggggagaacttttcctaaagttttcttcctgaaaatgctggaggtttgtagacagcccagttccagagttctgaagcctgcctgccccacgtgtgctctgtaatctatttctgcttgtgctcccggccagtgaggcaagaaaactgatattatttacacaaccaacaggctctttggaagccttgttagtcatttctgtgatatcccgagcctcaactttggaaataacatcagatcttttcccaagtgaatcaactttaacaccttgaaagcaagtagtcctagagaaagaagaatcagttatgttttgaacatccagtgactgagaagaagaaggctgtagcttcccaaactcaaaacatttggactgtctctctggtttcaccagagaattatgtagcgacattggtgcagaacagcgaagaggtgacaagagtctattcttgtgaggacttaattcccggtagttaagaactgaagtctctactgattccccattcagcactcctgcaacatgcttgagatgctgctctggagctttcaaccctttgtcagcattagtgagtagcaactccagattcactttgcacgcaccttctaagccgctgctctgttcatcagcatttccttctgcaaatgaagccagtgagcccactttaggtagaagtgattgttcggttacacattcttctgaaggtaagacaatgttcccattactagatggcaagtttcctaaaaaatgttttgtttgcctaggcagggatgatccaagatggagaacagagtcagcaagctcctggtcatttcccaactccaaatggggtatctgaggaggtagtttgacgttgctactgaagtgagacagtgtgttattctcccagctattatcttccttaagaaattcaccagtgatagaagatatgtatctctcagcagagagttgagttgccaaacttgaaattccattcctggagatttcgggcggatatgcattcccaaaagcaggtgaacaagattgaccaatgttggggaggacccttaacaatcggtggcgagatggtgcagtggaaccactagaaggtcgaggagctacaggtgggtgaggttttatcttgacagctttcttaggctttttgctgagattcatgttcttcatcttagccttcagcagcttcatcttattcatagttattgaattttcaattatctgttgcccagaagaagaaggctcagtttcttcatcctcatctgtatctgaattatacatagaaccaccactgcaaagaaaacaataactcatacgatgttctccttttctccgtaggacatgcaaatgaaaatctattttctttgaagagtcagataacggtgttaaagtgccatctcccctatctactgcaggaaagaaattcaattgatctccttcttggtataccaaaaatgtaacttgtttgctgcaggaggtcttctcccagacctcaactcgactggaatccaagtactctgccatcttcctaagtggatcgtctgtaggaacttccaatcttcgaatttttgctttcacagaaataacagtttcaaaaggtgaaactctcagctcaaaacatgttccagttaatgtttcaatgaagagctccatggtatcacagaaatgaagtctgtagtaaaatggtcccatgttatcatcattgaagaatggaggctcttttctgttatccattactttgacttttctagttcttctaaaatatgtcgcaggcaactgtattccagttctaggcaaaccaggtttgaagattggtaatatatattgttgttcatgttttgagttttgtacctacacacttgaggccaccgagtcacctgcgcagccgttgctcctccaagaccaatccgggctccccagacccaccggcctgaatctggaggacagcagtccgcgtgacaacagcgactcggagatcagcacccgtcgggaaagccgcgtacccgttgaagctggcgtcacgcccaaaggaacaaacgccagagcgtgtgtcctgggcaaaggcggcccgccgctccggtccccgggcagcagcggccggcgtcaggccgcaaggcgaggggcggggacaggactctacccggcagcccagcgccgagcgcccgcgccactccggccttgcgccattccggccccacgacggccggcggcggcagcgcggctgggctcag

SEQ ID NO: 8404 - RNA, 3179 nt, Homo sapiens
  source 1..3179: mol_type = other RNA
aaaacggtgagattttgttttaaatgtagccatatttcaaaaggtaaaaagttggcttctatatttaatggcaagtgggacatcttctattttaaaattaacattcaaaaagtagtaaaatatacactatcatgaacacgatgtgttttatagaatggattcatgtccgaatactaatctgaatgtggaagaaatgtattatctgttaaaaaccacactggaaaaatgttcttttttataaaaagtagcttgaagtaaaaaggaacttgctaataaagccagtaaactttcacacgtgggatttttaaaaaatctccacccatcccacctctgaaaaaaaaagaaggagaagaataaaagaaagaaaaagaaaaaacccatatggtcaatctgagtagagccattcattacatgactgctcattctgtacaatgtggaagcctggttatttaggaaatatttcgtttcctaaagtgcatcttttgaagatttgcctagtaaaactgcaatatcatatacaaaacacttaacacaagacatgcaataacaaagctaaatcattccagtgtaaagttgttaaaactacttttaaaacttttgtttcaccaagaaataaagatgtaaaatacagtagcattcttgttctccaacagtatgcattgtatgcttttgttatttggcaaatcttttagagtcgaacaaaaataatagtctaaacaacatttcttctgtcattataatacgaatcccgggcagaacagtaagatgtagaggaagagttagatttttggaagctttggtgcattaaccacaggatttgcctcgtgcaagtatctcctccctgcactcttgtaatcataggtacagccatgagtttctgcataacgatgagatgcacagaagttgtttccacatctgcattcgtagctactagccagtcctgttttctttccacaaagaaaacaatgatttgttgttttcttctttgtctgaagaggggctttcacaggtgggaggtgatgagtagtacattctcctacgcttttccctgctgctgcattatttccattcattccaacaccatgggtagacaaaaaaactcctgtatgttctaactggggagaacttttcctaaagttttcttcctgaaaatgctggaggtttgtagacagcccagttccagagttctgaagcctgcctgccccacgtgtgctctgtaatctatttctgcttgtgctcccggccagtgaggcaagaaaactgatattatttacacaaccaacaggctctttggaagccttgttagtcatttctgtgatatcccgagcctcaactttggaaataacatcagatcttttcccaagtgaatcaactttaacaccttgaaagcaagtagtcctagagaaagaagaatcagttatgttttgaacatccagtgactgagaagaagaaggctgtagcttcccaaactcaaaacatttggactgtctctctggtttcaccagagaattatgtagcgacattggtgcagaacagcgaagaggtgacaagagtctattcttgtgaggacttaattcccggtagttaagaactgaagtctctactgattccccattcagcactcctgcaacatgcttgagatgctgctctggagctttcaaccctttgtcagcattagtgagtagcaactccagattcactttgcacgcaccttctaagccgctgctctgttcatcagcatttccttctgcaaatgaagccagtgagcccactttaggtagaagtgattgttcggttacacattcttctgaaggtaagacaatgttcccattactagatggcaagtttcctaaaaaatgttttgtttgcctaggcagggatgatccaagatggagaacagagtcagcaagctcctggtcatttcccaactccaaatggggtatctgaggaggtagtttgacgttgctactgaagtgagacagtgtgttattctcccagctattatcttccttaagaaattcaccagtgatagaagatatgtatctctcagcagagagttgagttgccaaacttgaaattccattcctggagatttcgggcggatatgcattcccaaaagcaggtgaacaagattgaccaatgttggggaggacccttaacaatcggtggcgagatggtgcagtggaaccactagaaggtcgaggagctacaggtgggtgaggttttatcttgacagctttcttaggctttttgctgagattcatgttcttcatcttagccttcagcagcttcatcttattcatagttattgaattttcaattatctgttgcccagaagaagaaggctcagtttcttcatcctcatctgtatctgaattatacatagaaccaccactgcaaagaaaacaataactcatacgatgttctccttttctccgtaggacatgcaaatgaaaatctattttctttgaagagtcagataacggtgttaaagtgccatctcccctatctactgcaggaaagaaattcaattgatctccttcttggtataccaaaaatgtaacttgtttgctgcaggaggtcttctcccagacctcaactcgactggaatccaagtactctgccatcttcctaagtggatcgtctgtaggaacttccaatcttcgaatttttgctttcacagaaataacagtttcaaaaggtgaaactctcagctcaaaacatgttccagttaatgtttcaatgaagagctccatggtatcacagaaatgaagtctgtagtaaaatggtcccatgttatcatcattgaagaatggaggctcttttctgttatccattactttgacttttctagttcttctaaaatatgtcgcaggcaactgtattccagttctaggcaaaccaggtttgaagattggtaatatatattgttgttcatgttttgagttttgtacctttgaaacattttccccaacataaagatatccggaatgtgaagctgccattaaaactgtgacacagatctacatttactgatacatcaaaacatccctaaagttcgaaatacgagctacagaatcacatcaaccgcctaacttgtctgtagcctaaactctagtccggagttcatctgcaagcggaattgggaagtatttcagagccagcatctcctcgcgcca

SEQ ID NO: 8405 - RNA, 3413 nt, Homo sapiens
  source 1..3413: mol_type = other RNA
aaaacggtgagattttgttttaaatgtagccatatttcaaaaggtaaaaagttggcttctatatttaatggcaagtgggacatcttctattttaaaattaacattcaaaaagtagtaaaatatacactatcatgaacacgatgtgttttatagaatggattcatgtccgaatactaatctgaatgtggaagaaatgtattatctgttaaaaaccacactggaaaaatgttcttttttataaaaagtagcttgaagtaaaaaggaacttgctaataaagccagtaaactttcacacgtgggatttttaaaaaatctccacccatcccacctctgaaaaaaaaagaaggagaagaataaaagaaagaaaaagaaaaaacccatatggtcaatctgagtagagccattcattacatgactgctcattctgtacaatgtggaagcctggttatttaggaaatatttcgtttcctaaagtgcatcttttgaagatttgcctagtaaaactgcaatatcatatacaaaacacttaacacaagacatgcaataacaaagctaaatcattccagtgtaaagttgttaaaactacttttaaaacttttgtttcaccaagaaataaagatgtaaaatacagtagcattcttgttctccaacagtatgcattgtatgcttttgttatttggcaaatcttttagagtcgaacaaaaataatagtctaaacaacatttcttctgtcattataatacgaatcccgggcagaacagtaagatgtagaggaagagttagatttttggaagctttggtgcattaaccacaggatttgcctcgtgcaagtatctcctccctgcactcttgtaatcataggtacagccatgagtttctgcataacgatgagatgcacagaagttgtttccacatctgcattcgtagctactagccagtcctgttttctttccacaaagaaaacaatgatttgttgttttcttctttgtctgaagaggggctttcacaggtgggaggtgatgagtagtacattctcctacgcttttccctgctgctgcattatttccattcattccaacaccatgggtagacaaaaaaactcctgtatgttctaactggggagaacttttcctaaagttttcttcctgaaaatgctggaggtttgtagacagcccagttccagagttctgaagcctgcctgccccacgtgtgctctgtaatctatttctgcttgtgctcccggccagtgaggcaagaaaactgatattatttacacaaccaacaggctctttggaagccttgttagtcatttctgtgatatcccgagcctcaactttggaaataacatcagatcttttcccaagtgaatcaactttaacaccttgaaagcaagtagtcctagagaaagaagaatcagttatgttttgaacatccagtgactgagaagaagaaggctgtagcttcccaaactcaaaacatttggactgtctctctggtttcaccagagaattatgtagcgacattggtgcagaacagcgaagaggtgacaagagtctattcttgtgaggacttaattcccggtagttaagaactgaagtctctactgattccccattcagcactcctgcaacatgcttgagatgctgctctggagctttcaaccctttgtcagcattagtgagtagcaactccagattcactttgcacgcaccttctaagccgctgctctgttcatcagcatttccttctgcaaatgaagccagtgagcccactttaggtagaagtgattgttcggttacacattcttctgaaggtaagacaatgttcccattactagatggcaagtttcctaaaaaatgttttgtttgcctaggcagggatgatccaagatggagaacagagtcagcaagctcctggtcatttcccaactccaaatggggtatctgaggaggtagtttgacgttgctactgaagtgagacagtgtgttattctcccagctattatcttccttaagaaattcaccagtgatagaagatatgtatctctcagcagagagttgagttgccaaacttgaaattccattcctggagatttcgggcggatatgcattcccaaaagcaggtgaacaagattgaccaatgttggggaggacccttaacaatcggtggcgagatggtgcagtggaaccactagaaggtcgaggagctacaggtgggtgaggttttatcttgacagctttcttaggctttttgctgagattcatgttcttcatcttagccttcagcagcttcatcttattcatagttattgaattttcaattatctgttgcccagaagaagaaggctcagtttcttcatcctcatctgtatctgaattatacatagaaccaccactgcaaagaaaacaataactcatacgatgttctccttttctccgtaggacatgcaaatgaaaatctattttctttgaagagtcagataacggtgttaaagtgccatctcccctatctactgcaggaaagaaattcaattgatctccttcttggtataccaaaaatgtaacttgtttgctgcaggaggtcttctcccagacctcaactcgactggaatccaagtactctgccatcttcctaagtggatcgtctgtaggaagttagattaaaagtacacagacacggccgggtgcggtggctcatgcctgtaatcccagcactttgggaggccgaggcgggcagatcatgaagtcaagagatcaagaccatcctggccaacatggtgaaaccccgtctctactcttctagtatttataggtccgccacgcatagccaaaactagcttcaaggtacacccttctgaaatgcttccaatcttcgaatttttgctttcacagaaataacagtttcaaaaggtgaaactctcagctcaaaacatgttccagttaatgtttcaatgaagagctccatggtatcacagaaatgaagtctgtagtaaaatggtcccatgttatcatcattgaagaatggaggctcttttctgttatccattactttgacttttctagttcttctaaaatatgtcgcaggcaactgtattccagttctaggcaaaccaggtttgaagattggtaatatatattgttgttcatgttttgagttttgtacacacttgaggccaccgagtcacctgcgcagccgttgctcctccaagaccaatccgggctccccagacccaccggcctgaatctggaggacagcagtccgcgtgacaacagcgactcggagatcagcacccgtcgggaaagccgcgtacccgttgaagctggcgtcacgcccaaaggaacaaacgccagagcgtgtgtcctgggcaaaggcggcccgccgctccggtccccgggcagcagcggccggcgtca

SEQ ID NO: 8406 - RNA, 3466 nt, Homo sapiens
  source 1..3466: mol_type = other RNA
aaaacggtgagattttgttttaaatgtagccatatttcaaaaggtaaaaagttggcttctatatttaatggcaagtgggacatcttctattttaaaattaacattcaaaaagtagtaaaatatacactatcatgaacacgatgtgttttatagaatggattcatgtccgaatactaatctgaatgtggaagaaatgtattatctgttaaaaaccacactggaaaaatgttcttttttataaaaagtagcttgaagtaaaaaggaacttgctaataaagccagtaaactttcacacgtgggatttttaaaaaatctccacccatcccacctctgaaaaaaaaagaaggagaagaataaaagaaagaaaaagaaaaaacccatatggtcaatctgagtagagccattcattacatgactgctcattctgtacaatgtggaagcctggttatttaggaaatatttcgtttcctaaagtgcatcttttgaagatttgcctagtaaaactgcaatatcatatacaaaacacttaacacaagacatgcaataacaaagctaaatcattccagtgtaaagttgttaaaactacttttaaaacttttgtttcaccaagaaataaagatgtaaaatacagtagcattcttgttctccaacagtatgcattgtatgcttttgttatttggcaaatcttttagagtcgaacaaaaataatagtctaaacaacatttcttctgtcattataatacgaatcccgggcagaacagtaagatgtagaggaagagttagatttttggaagctttggtgcattaaccacaggatttgcctcgtgcaagtatctcctccctgcactcttgtaatcataggtacagccatgagtttctgcataacgatgagatgcacagaagttgtttccacatctgcattcgtagctactagccagtcctgttttctttccacaaagaaaacaatgatttgttgttttcttctttgtctgaagaggggctttcacaggtgggaggtgatgagtagtacattctcctacgcttttccctgctgctgcattatttccattcattccaacaccatgggtagacaaaaaaactcctgtatgttctaactggggagaacttttcctaaagttttcttcctgaaaatgctggaggtttgtagacagcccagttccagagttctgaagcctgcctgccccacgtgtgctctgtaatctatttctgcttgtgctcccggccagtgaggcaagaaaactgatattatttacacaaccaacaggctctttggaagccttgttagtcatttctgtgatatcccgagcctcaactttggaaataacatcagatcttttcccaagtgaatcaactttaacaccttgaaagcaagtagtcctagagaaagaagaatcagttatgttttgaacatccagtgactgagaagaagaaggctgtagcttcccaaactcaaaacatttggactgtctctctggtttcaccagagaattatgtagcgacattggtgcagaacagcgaagaggtgacaagagtctattcttgtgaggacttaattcccggtagttaagaactgaagtctctactgattccccattcagcactcctgcaacatgcttgagatgctgctctggagctttcaaccctttgtcagcattagtgagtagcaactccagattcactttgcacgcaccttctaagccgctgctctgttcatcagcatttccttctgcaaatgaagccagtgagcccactttaggtagaagtgattgttcggttacacattcttctgaaggtaagacaatgttcccattactagatggcaagtttcctaaaaaatgttttgtttgcctaggcagggatgatccaagatggagaacagagtcagcaagctcctggtcatttcccaactccaaatggggtatctgaggaggtagtttgacgttgctactgaagtgagacagtgtgttattctcccagctattatcttccttaagaaattcaccagtgatagaagatatgtatctctcagcagagagttgagttgccaaacttgaaattccattcctggagatttcgggcggatatgcattcccaaaagcaggtgaacaagattgaccaatgttggggaggacccttaacaatcggtggcgagatggtgcagtggaaccactagaaggtcgaggagctacaggtgggtgaggttttatcttgacagctttcttaggctttttgctgagattcatgttcttcatcttagccttcagcagcttcatcttattcatagttattgaattttcaattatctgttgcccagaagaagaaggctcagtttcttcatcctcatctgtatctgaattatacatagaaccaccactgcaaagaaaacaataactcatacgatgttctccttttctccgtaggacatgcaaatgaaaatctattttctttgaagagtcagataacggtgttaaagtgccatctcccctatctactgcaggaaagaaattcaattgatctccttcttggtataccaaaaatgtaacttgtttgctgcaggaggtcttctcccagacctcaactcgactggaatccaagtactctgccatcttcctaagtggatcgtctgtaggaagttagattaaaagtacacagacacggccgggtgcggtggctcatgcctgtaatcccagcactttgggaggccgaggcgggcagatcatgaagtcaagagatcaagaccatcctggccaacatggtgaaaccccgtctctactcttctagtatttataggtccgccacgcatagccaaaactagcttcaaggtacacccttctgaaatgttgtaatcattcaagcaataatcattttcaagttccatgttattccaaattaagtgttgtcgacagatgggaataccttccaatcttcgaatttttgctttcacagaaataacagtttcaaaaggtgaaactctcagctcaaaacatgttccagttaatgtttcaatgaagagctccatggtatcacagaaatgaagtctgtagtaaaatggtcccatgttatcatcattgaagaatggaggctcttttctgttatccattactttgacttttctagttcttctaaaatatgtcgcaggcaactgtattccagttctaggcaaaccaggtttgaagattggtaatatatattgttgttcatgttttgagttttgtacccgttgaagctggcgtcacgcccaaaggaacaaacgccagagcgtgtgtcctgggcaaaggcggcccgccgctccggtccccgggcagcagcggccggcgtcaggccgcaaggcgaggggcggggacaggactctacccggcagcccagcgccgagcgcccgcgccactccggccttgcgccattccggccccacgacggccggcggcggcagcgcggctgggctcag

SEQ ID NO: 8407 - RNA, 3362 nt, Homo sapiens
  source 1..3362: mol_type = other RNA
aaaacggtgagattttgttttaaatgtagccatatttcaaaaggtaaaaagttggcttctatatttaatggcaagtgggacatcttctattttaaaattaacattcaaaaagtagtaaaatatacactatcatgaacacgatgtgttttatagaatggattcatgtccgaatactaatctgaatgtggaagaaatgtattatctgttaaaaaccacactggaaaaatgttcttttttataaaaagtagcttgaagtaaaaaggaacttgctaataaagccagtaaactttcacacgtgggatttttaaaaaatctccacccatcccacctctgaaaaaaaaagaaggagaagaataaaagaaagaaaaagaaaaaacccatatggtcaatctgagtagagccattcattacatgactgctcattctgtacaatgtggaagcctggttatttaggaaatatttcgtttcctaaagtgcatcttttgaagatttgcctagtaaaactgcaatatcatatacaaaacacttaacacaagacatgcaataacaaagctaaatcattccagtgtaaagttgttaaaactacttttaaaacttttgtttcaccaagaaataaagatgtaaaatacagtagcattcttgttctccaacagtatgcattgtatgcttttgttatttggcaaatcttttagagtcgaacaaaaataatagtctaaacaacatttcttctgtcattataatacgaatcccgggcagaacagtaagatgtagaggaagagttagatttttggaagctttggtgcattaaccacaggatttgcctcgtgcaagtatctcctccctgcactcttgtaatcataggtacagccatgagtttctgcataacgatgagatgcacagaagttgtttccacatctgcattcgtagctactagccagtcctgttttctttccacaaagaaaacaatgatttgttgttttcttctttgtctgaagaggggctttcacaggtgggaggtgatgagtagtacattctcctacgcttttccctgctgctgcattatttccattcattccaacaccatgggtagacaaaaaaactcctgtatgttctaactggggagaacttttcctaaagttttcttcctgaaaatgctggaggtttgtagacagcccagttccagagttctgaagcctgcctgccccacgtgtgctctgtaatctatttctgcttgtgctcccggccagtgaggcaagaaaactgatattatttacacaaccaacaggctctttggaagccttgttagtcatttctgtgatatcccgagcctcaactttggaaataacatcagatcttttcccaagtgaatcaactttaacaccttgaaagcaagtagtcctagagaaagaagaatcagttatgttttgaacatccagtgactgagaagaagaaggctgtagcttcccaaactcaaaacatttggactgtctctctggtttcaccagagaattatgtagcgacattggtgcagaacagcgaagaggtgacaagagtctattcttgtgaggacttaattcccggtagttaagaactgaagtctctactgattccccattcagcactcctgcaacatgcttgagatgctgctctggagctttcaaccctttgtcagcattagtgagtagcaactccagattcactttgcacgcaccttctaagccgctgctctgttcatcagcatttccttctgcaaatgaagccagtgagcccactttaggtagaagtgattgttcggttacacattcttctgaaggtaagacaatgttcccattactagatggcaagtttcctaaaaaatgttttgtttgcctaggcagggatgatccaagatggagaacagagtcagcaagctcctggtcatttcccaactccaaatggggtatctgaggaggtagtttgacgttgctactgaagtgagacagtgtgttattctcccagctattatcttccttaagaaattcaccagtgatagaagatatgtatctctcagcagagagttgagttgccaaacttgaaattccattcctggagatttcgggcggatatgcattcccaaaagcaggtgaacaagattgaccaatgttggggaggacccttaacaatcggtggcgagatggtgcagtggaaccactagaaggtcgaggagctacaggtgggtgaggttttatcttgacagctttcttaggctttttgctgagattcatgttcttcatcttagccttcagcagcttcatcttattcatagttattgaattttcaattatctgttgcccagaagaagaaggctcagtttcttcatcctcatctgtatctgaattatacatagaaccaccactgccatatcattcccaaagaggcaaaatccatttccatgagaatgtctgatttcattttatcagccaaggctgataattgtgcaacccagacaacaggctgatgagatttccatgaatcagaatttttttaaatttggcacgggagagaagtacagatttttagtcatcctgaggagattctcactcatacgatgttctccttttctccgtaggacatgcaaatgaaaatctattttctttgaagagtcagataacggtgttaaagtgccatctcccctatctactgcaggaaagaaattcaattgatctccttcttggtataccaaaaatgtaacttgtttgctgcaggaggtcttctcccagacctcaactcgactggaatccaagtactctgccatcttcctaagtggatcgtctgtaggaactcttctagtatttataggtccgccacgcatagccaaaactagcttcaaggtacacccttctgaaatgttgtaatcattcaagcaataatcattttcaagttccatgttattccaaattaagtgttgtcgacagatgggaataccttccaatcttcgaatttttgctttcacagaaataacagtttcaaaaggtgaaactctcagctcaaaacatgttccagttaatgtttcaatgaagagctccatggtatcacagaaatgaagtctgtagtaaaatggtcccatgttatcatcattgaagaatggaggctcttttctgttatccattactttgacttttctagttcttctaaaatatgtcgcaggcaactgtattccagttctaggcaaaccaggtttgaagattggtaatatatattgttgttcatgttttgagttttgtacccgcagtcttgtccgctggctcgctcgcccgcctacaggtcgacagggcccaacgacccggcgagcaacttcacggaaggcactggccgacaacgct

SEQ ID NO: 8408 - RNA, 384 nt, Homo sapiens
  source 1..384: mol_type = other RNA
aaaacggtgagattttgttttctattacattgccaggccgcacattttctgaacttttatgctctgcttcccttgtaaaactgaatgcctataacagcacccatgtcacatcttgaatgctttgctgcttagaaatttcttctgccagataccctaaattatatctctcaatttcaaagttccacagatctctagggcaggggcaaaatgcctccagtctctttgctaaaacataacaagagtcacctttgctccagttcccaacaagttcttcatttccatctgagactacctcatcttggactttgttgtccatattgctaccagcattttgggaaaagtcattcaacaagtctccaggaagttccaaaccttcccacattt

SEQ ID NO: 8409 - RNA, 5863 nt, Homo sapiens
  source 1..5863: mol_type = other RNA
aaaacggtgagattttgtttttctaacaacttctccagtaatattgatgttgttggtctagggttagcatgttgagaacgaatgctttacacattttaaacctgtaaaatgttggaatgatgttttagcatagggtacccgagtgtattttctgagcactgggtctctagtaacaatcaggattttagggatgataaaagacattttggcacatagaattccctatttctgccttccacttttggtctttgtatttctttttcttctcctttatatatgtattttaaattcttcactcttattcaccttttcctcctgctccaagcctgacttagaagggtcttatgatccagacgattgtaacatgtaataggaatagtgtgagaaagaagccccaaggtaaaaggaatctgcttatctgctgtactcagggaaaaatctcgttgatgttaaactagtgtggtctctccttcctctagcatagttattcaggaatcaatcaatcaaaattatccaaatatcctgcaaacatttggcttaaaacttttatcagtattttcaacaactgtcaaatactcttgtacagaggaatgtggcaaagacggggagtgaatgagaagaagctgatagtaagtagctctacttttagtttcttattgtctacaatggctcttcattttgaagctggagctttgctttatggttggttcctggcttgctaataagaagcagatgtttcccacaaagatatttctgattctttttttctatacccctactttcaacttggagttggaaatcagtaagttcaagggaatttattacctttatcctcttagcacatgaaattggaagatgatagggttttaactagttgtcagattgttaggtgaaaggatatttctggctaaagaatggggctttcattgccgttattttcttttcaattctttctgcagttcctagaaagaaatcaaactagttacattgctaaggtgaagaagtacatgctctggtatttttgcagtgaagttcttcaggccctgatacctctcaagcccagatgtcaatcatttccagcaagtgcagcctttttttgccaccactgtgtaggacgtggttaccactcagaaattatggcaagttaatctgcaggccttattcaataattcttagaaacacatgaacacagttggtgcgctcgagcatttggaaaattaaattattctttagaattagcctactgagctggaagaaaataaagaacacttaccaaaggggaaaaaatgacaaaaaattctaatgactaatggtttttcattataattgcataatagtctcttgatacaagtgctactcattgttctgataattcactgatccattaggcccctccatacatatgcaagcacagatttgaagagagacatcagggtaggcttcccatccagaaggcagagagccagacaaacgacacttttgaagatatcggtgccactgctgaggatggctggattcatacctactagactgtaaactccttaaaggcacctggaggattccactttgcaaatgtatccaccttaaacctgtgaggtgtttgtttcctggggccagggcttgctggggcgttcagcagcctgcacaccagctgctgctctgctccccagtgtacatcttgtaacaacgcagctcctttgctggttgttgaataggtagaggggcagctgtgaagggcagaagaaagccgattatttcactttctttcttttcggaattctgctttgtgatcttgttccctcttagaatgtttcccgagaagcccgttctatttagctcttctcttgctagggagcattttctgacagttttccaaaatgtgtatattccaggcagttagttggaggtttcgcacatattctagttaggaaagctcagcctggcttttgtggcccagaagcccagaatttcagcaactcacaaagaactcaaatatccttatgtgtgatatttgaaggatagggctttgcaagtcagcctagaaaacgaggataatatctcttggctgtagaacaaactgaaaactcattccattctggcttggagaacaaggatttctctctcagaacaagttttcagggatgatagttaatgacctgtcatgtttttcttatgatttcaaaaaactaaattaaaattgctacttatttttataaattatatgtgaaatgtatttaataatttaaacttacttcttaaattgcttttcttcagagaccttttgtctcctctcacttgtttgacctcagtcttcagaagcaaaccaaaataccatttcaggtagatcagttagcaattgctaataaagtgtgagttgcagattttgagtgtatagagtaagtgtagctagctatgagcactgtgtacatgagaagtatctatcactgtgtctttctccattccacagctcttgcaaaccacagaactcaacatccatgcaactccttaactgatgtgcctgtttggatattcaaatactttctaaaaaaccaaaaattatgcattagcttgcagcacctacactctagaaaaatcaaccctcagggtcttttggtaccatggtctggagttgcttttattttcctagcttttgtcagcatactgctaactcggttgataagtgttctttctgtttaatgatttatgcttcagagggatttgtataggcaaaatagataaagccatatatttccttataggacatattttagatgacattactttgaattcagaacctgtgctctcactgtgggtatcaatgacttcctcaaaacaattcaataatttcaagggcactgtctcatttgtgaaggtcttttacagttaatatgactacctcagataattacaatactgcttctggtatgctacagtatataatagaatccagtgttattaactgaaatgaaatagtcgaatttttggtaaatgtaacaatttgataattagccacacatgctattatccattccatattcacataattggtaaatgttatgcagttttatcttcagtgaaaacatttaagtatcttgttgacttttgtttcagagaaaacatttttaaaattctatgaatgtcttagggcactagaattgaagtgaaatacatcttttgagcatacagagctgacatcattgtaggggtatgttgaatatatgttatgtattttatgtattttagtagaaaggtgctgtatgaatgtgaaagctcctaattagcttttgtaaatcctctagctatgaattgctttttaaacaaggatgaaatgatagcagaacacacacacacaaacacacacacacacacacacacatgcgctaatataatactgactcatcaggcagttgacatgatgtggtcattcaatatctagcctctacttttaaaaaattattgttggaatagtagataggaatatagatttagcaaagtgctttgagatttaggaagcatctctacagaatgccaagaaagtgttaaagaatttaaatgagacctaaaggagttttctactggtgaggcagtaattatattagaagccaaaccatcacatattaaggactgttttgtgctcaccatttgtaggtgaaaaggcaatcttttggaagacaaaaagaacaaacagcccatcatcatgtagaaatgtagaaacattgtgctgttcacaatcttgttaccaataattagctaattattcttttttactaaaagcgaaaggatacatgagcactgcacatcatgggaaaggagaggtgtcatcagaacaggctgcagacacacatccagggtaaagttagctggattattgtgggtcctggttggtcaaaccatggttgccaggaaaaccaggaagatttaagttatcaatctagttctagtagacctatgactgagggtatttatctgtctagaaggaagaatttttagtcaatggaggcaataattttaggcaaatatggtttccatcagaaaagtccaaaggaaaagtgttgctttgggaaatatgcgaagaatgacaaagggacaagactttagcccaaagattggtgcaacctaacctgagttgactcataagtccatgattcaatggaggacagtagttcatttttagtaggctagtcaaatatctaaaatggaaaaatgcaaatagatacacgtgtaagataagagacaattaggaaaaaaggctccttacaaagttagctcaagaaaattcaaaagaagcaggagaagccagactatttctagacacagaaaatataatgactagctcagcctcaacaaaaggtctgaaagtaaaattggactggaaaaatagaaggttctcagaccatacaaatgagaagttgggtgtttaagtgagacaagtgtaacatttactgcacttagttacacattaagggctctgcacacatcttgatgtatctgtgtattattcatccatgctgctgcttggcttattgtggatgaattcctatttctaaggatccgagttcaagcagtcaattcaagtgatgttaaagtaggaaaacggaagtatgggtggaataaaataaccacataatcacaacctgtgtctactccaggtacggagacaactctgaattgaacgcctagttatacaaacagtagttatgcaacaaacagcagctgtctgacttggatctatcatcttaccagggcgcactaagttgctctagcaccatctcttgccatttctagacttaaactttatactccagtaagactaaattgcttactatttcagaacttttcacactatttaccttgccttgatcttttcctgctcgttttcctgttgggctgctattcattcttcaactcttcagctaatcttctgtctcctttaaaaaaaaagtcttctgagagctcctcaacagtcttaattactcgttcctttgcactgccttgtctcttataggcttttttattcttgctgtttcacactgcattttaatttgtttgttatgtagttattttatccgcagcgcttgagctctttggaagaaacagtgtcttgttcatctttgtggcttcatagctggcatacagccagaattgccatggaagggactcaatgaactaccaataaattagcgaatgaatgaattagaacccaggaactcaaatatggatcacaaatgtggttgcctttagttctagcaaattttcatgcagtatctgtaagacacaacctcttaaaacacctatttggaggcagatactatgttaggcgtcagctactctactagtcctttacctgaagtaactcatatacagtgtcaccaaaaccctgtgagaagggatgttctccctttagataaggaagctgaggcataaagaggttaagtaattttcccaggattacacagtgaatagtaactgaactaagatgaaacagtggtagtgagtttcagagctgagctctcaaccaccataccactttttaataagattttatgaaagttggctcttcttagataattctgaaaaatgagtccggaatttcattttctggaatgataagaggcattttagctgaagcaacccaacatttgtaatggatttaatttgagaccatgccaggacagttatcatggttcatttaagtatccattaagtggatggggaaaagaaaaccactatgagaccagaaggggcctctaatgagaaaaaagaagaggatgtgggaaactaagtatctgaagtattgggaacatatattatacaacattatagagacgtgcacctgctcatattcataaattttaaaaaagcc

SEQ ID NO: 8410 - RNA, 5022 nt, Homo sapiens
  source 1..5022: mol_type = other RNA
aaaacggtgagattttgtttttctaacaacttctccagtaatattgatgttgttggtctagggttagcatgttgagaacgaatgctttacacattttaaacctgtaaaatgttggaatgatgttttagcatagggtacccgagtgtattttctgagcactgggtctctagtaacaatcaggattttagggatgataaaagacattttggcacatagaattccctatttctgccttccacttttggtctttgtatttctttttcttctcctttatatatgtattttaaattcttcactcttattcaccttttcctcctgctccaagcctgacttagaagggtcttatgatccagacgattgtaacatgtaataggaatagtgtgagaaagaagccccaaggtaaaaggaatctgcttatctgctgtactcagggaaaaatctcgttgatgttaaactagtgtggtctctccttcctctagcatagttattcaggaatcaatcaatcaaaattatccaaatatcctgcaaacatttggcttaaaacttttatcagtattttcaacaactgtcaaatactcttgtacagaggaatgtggcaaagacggggagtgaatgagaagaagctgatagtaagtagctctacttttagtttcttattgtctacaatggctcttcattttgaagctggagctttgctttatggttggttcctggcttgctaataagaagcagatgtttcccacaaagatatttctgattctttttttctatacccctactttcaacttggagttggaaatcagtaagttcaagggaatttattacctttatcctcttagcacatgaaattggaagatgatagggttttaactagttgtcagattgttaggtgaaaggatatttctggctaaagaatggggctttcattgccgttattttcttttcaattctttctgcagttcctagaaagaaatcaaactagttacattgctaaggtgaagaagtacatgctctggtatttttgcagtgaagttcttcaggccctgatacctctcaagcccagatgtcaatcatttccagcaagtgcagcctttttttgccaccactgtgtaggacgtggttaccactcagaaattatggcaagttaatctgcaggccttattcaataattcttagaaacacatgaacacagttggtgcgctcgagcatttggaaaattaaattattctttagaattagcctactgagctggaagaaaataaagaacacttaccaaaggggaaaaaatgacaaaaaattctaatgactaatggtttttcattataattgcataatagtctcttgatacaagtgctactcattgttctgataattcactgatccattaggcccctccatacatatgcaagcacagatttgaagagagacatcagggtaggcttcccatccagaaggcagagagccagacaaacgacacttttgaagatatcggtgccactgctgaggatggctggattcatacctgtgtagattacagggggttaaatatggtctacacatgtagtgccaaagtagtaatttaaaaatgcaaatctcatcaagctgctcttctcctcaaattccttcagtggctttccatttcacagaggatgaagaccaaggaggctgcatgatcatttgggtctccaatgcttcatcctcatccagtctcctgttgcctttacttactgtgttctagctactgaggccttcctttgcttctctacaactgtttgcttttacctaaaactcctgtttatgtttcaggattcatcctaaataatacttctcccaggaacttctgtttattctggtaagtttaaatccctttgttaagtgtactcatgccctttttgttgctaagattttattactcgggtaatttttgatgtttacatacctactagactgtaaactccttaaaggcacctggaggattccactttgcaaatgtatccacctggtttactcttttgaaaaatccaacccttgccgtctcccacacaaagctcttggccactgggtgaaatccaagctgggtagttgatcatgataattcccgcatgtcatgggcagcagcatctctcagagtcccacaagccaactgcttgaaacgaaccttgaaagctgcattctgtttttctcacttcaccagtttgaattgttgggctcttcatgctggtagtggccactttcggtgctctgctctgagcttcttctcataaccctatttccaggctcagagcaccacaacctggaaaggtatttatctgcttatttgtcactctttctcttaaattatgacctccttgagggcagggactggtgtcttgttttttccgatatctctagtgtctgcacctgacctttacacagtgaggatgaagcactgcacacagatctgtggtgtaccaatatgcacttaatgagcactccagctctctgcttttcaatttgtactcgctgaacttctattttttaaactcatgtgattaaaaatccactggacactttagaagtgcaggcagctcatgatacagctttctgatggcactcatcaattccacaacatgaagcaatttcaacatggatgctccaacttcatttgggatacttcacatataaggatcctatatcttgaaaccatctccagtggatttccttgaggcgctgttaattctccttcgtgtccttaaaatcccaagccaaggatgcgacgcacacaagtccaggggcttttcctggacttccccctcctcagctctgaaggctcctcctttccaagggatcaggaggggatggcggttcaaaagccctcaccatagaggcgcctccaagccttcgtaccagtggaaatggagaccgggaccaccttcccggcacccggaagcctcccagcccctcctgggccaacttggctgcctattcagttttcttccgtaaccccacagacacgtcagtcaattccctggcatcaggcaggatattctcagttgcggccgctcctcttgctttctctcgataatgcccctcccccctttctccccttaatttggaaaaatttctactccctgcccgaattaggtggggatgaggcggaaaggtgtaagaagagccactccaaggcacagcttcggaacaccgtctccctgggctgctgcagcgcgaaggtgtctacgctggggaaactttcaggggaggcagcgccggtgcggggctgggcgggcggcgggcggcggcgccaggtgaggaggctttgaggaggcggctgcaaggcgggacgcaggatagccggctggggcttggcagccgggctcagagctcgggctgcgcacacacacaggcgcgcacacccgcgcgcgcgcagctacacacgcacgcccagccctgcgcccgcggcccccggccagtggcgagcgaaaagtcgggagtcctgaggaggggtaggggttccaaggatgctgatgacagaaagagtcaatcaatcctcactagttagcggattgccggcaggcagttcctcgccgcacgccgttaagtccgttgggccacctctccgttctctgccctgtctggcatttcaactccctagctcttttcttgaagccagttacaccccctcgacacccagcgagaggccaccagactaaagatgagccccgttcccatcgccaccctccaggggccacctccgccccttctgtagtggagaattgaagtggctgcagcagctctcctgggagctgaggggctccccgaggtccttcgaatagaggagcctacacatcgcttcgtgaacataatcccctcgcatcccgtctttacctgcccactcccttcgtaacatttcccccaaggagctcccgaaagtcgcttagatgttttgaaaatgaatttcttagggaattgtagtgcctagcttttggaactgggttaatttaggtgctacgcttatattgtaaactggacggtagcaggtgaacggctcagctggagaaaggggagggattaggagtctggagacccaacccctttagcagccatttccaaggttttgcaccaggagtagctgtccgggtctctggctagctcctgtcccaacttctttttcttccctcgacggtcgggagggatcactgggtgctacaccgctggggcgtcccaggcaggagagacttcgctctcagaagcgcccccgtgtcatccacaactcccacgaaaggagcttcccaagaggagtttgttttacccggaatgggctgcaggaattaattgcttacagagagtaaacttttgcccgttgtttttttgttttttgtgctttttttaaccaaagcttgcatttgtgctccgcgtagtttctattgcaacagagcgctactctgccttttcaactgtgagacagaggattgctgaggatttctgccctctggggcttcgcgaatatctatggcttcggacctgctagcggaaaacgcaaagttgcccagcttggagatggcaccaggttcctttgctctggcgctggatgctccgctccgccacccaccgccgccgtctccatcgagaatctcctcaaaatcaagggagttcttgactgtccctctccaaattggaaggcggttgactttgccgggaaccgagttcctgagcggcaaacgtggagtcgcagagcgcagaagtgaagatttaatacaaaagatgaaacttgtaggatgacctctagcagcgctactcacagctctgaaatcgatccagagcattccacagtgagcgttgcggctcccaggggctccggaccggtaacttcaggcgcaagtctgaatttcagggatgaacctgctttggattctgtttgagccgactcagtgcagaggcagtgacaggggctgtgggtttaggggtgatggatccatgaaggctgccacttggagcgagcagacagttggcgataccctcccactaacttgctccgctgctccg

SEQ ID NO: 8411 - RNA, 6280 nt, Homo sapiens
  source 1..6280: mol_type = other RNA
aaaacggtgagattttgtttttctaacaacttctccagtaatattgatgttgttggtctagggttagcatgttgagaacgaatgctttacacattttaaacctgtaaaatgttggaatgatgttttagcatagggtacccgagtgtattttctgagcactgggtctctagtaacaatcaggattttagggatgataaaagacattttggcacatagaattccctatttctgccttccacttttggtctttgtatttctttttcttctcctttatatatgtattttaaattcttcactcttattcaccttttcctcctgctccaagcctgacttagaagggtcttatgatccagacgattgtaacatgtaataggaatagtgtgagaaagaagccccaaggtaaaaggaatctgcttatctgctgtactcagggaaaaatctcgttgatgttaaactagtgtggtctctccttcctctagcatagttattcaggaatcaatcaatcaaaattatccaaatatcctgcaaacatttggcttaaaacttttatcagtattttcaacaactgtcaaatactcttgtacagaggaatgtggcaaagacggggagtgaatgagaagaagctgatagtaagtagctctacttttagtttcttattgtctacaatggctcttcattttgaagctggagctttgctttatggttggttcctggcttgctaataagaagcagatgtttcccacaaagatatttctgattctttttttctatacccctactttcaacttggagttggaaatcagtaagttcaagggaatttattacctttatcctcttagcacatgaaattggaagatgatagggttttaactagttgtcagattgttaggtgaaaggatatttctggctaaagaatggggctttcattgccgttattttcttttcaattctttctgcagttcctagaaagaaatcaaactagttacattgctaaggtgaagaagtacatgctctggtatttttgcagtgaagttcttcaggccctgatacctctcaagcccagatgtcaatcatttccagcaagtgcagcctttttttgccaccactgtgtaggacgtggttaccactcagaaattatggcaagttaatctgcaggccttattcaataattcttagaaacacatgaacacagttggtgcgctcgagcatttggaaaattaaattattctttagaattagcctactgagctggaagaaaataaagaacacttaccaaaggggaaaaaatgacaaaaaattctaatgactaatggtttttcattataattgcataatagtctcttgatacaagtgctactcattgttctgataattcactgatccattaggcccctccatacatatgcaagcacagatttgaagagagacatcagggtaggcttcccatccagaaggcagagagccagacaaacgacacttttgaagatatcggtgccactgctgaggatggctggattcatacctgtgtagattacagggggttaaatatggtctacacatgtagtgccaaagtagtaatttaaaaatgcaaatctcatcaagctgctcttctcctcaaattccttcagtggctttccatttcacagaggatgaagaccaaggaggctgcatgatcatttgggtctccaatgcttcatcctcatccagtctcctgttgcctttacttactgtgttctagctactgaggccttcctttgcttctctacaactgtttgcttttacctaaaactcctgtttatgtttcaggattcatcctaaataatacttctcccaggaacttctgtttattctggtaagtttaaatccctttgttaagtgtactcatgccctttttgttgctaagattttattactcgggtaatttttgatgtttacatacctactagactgtaaactccttaaaggcacctggaggattccactttgcaaatgtatccaccttaaacctgtgaggtgtttgtttcctggggccagggcttgctggggcgttcagcagcctgcacaccagctgctgctctgctccccagtgtacatcttgtaacaacgcagctcctttgctggttgttgaataggtagaggggcagctgtgaagggcagaagaaagccgattatttcactttctttcttttcggaattctgctttgtgatcttgttccctcttagaatgtttcccgagaagcccgttctatttagctcttctcttgctagggagcattttctgacagttttccaaaatgtgtatattccaggcagttagttggaggtttcgcacatattctagttaggaaagctcagcctggcttttgtggcccagaagcccagaatttcagcaactcacaaagaactcaaatatccttatgtgtgatatttgaaggatagggctttgcaagtcagcctagaaaacgaggataatatctcttggctgtagaacaaactgaaaactcattccattctggcttggagaacaaggatttctctctcagaacaagttttcagggatgatagttaatgacctgtcatgtttttcttatgatttcaaaaaactaaattaaaattgctacttatttttataaattatatgtgaaatgtatttaataatttaaacttacttcttaaattgcttttcttcagagaccttttgtctcctctcacttgtttgacctcagtcttcagaagcaaaccaaaataccatttcaggtagatcagttagcaattgctaataaagtgtgagttgcagattttgagtgtatagagtaagtgtagctagctatgagcactgtgtacatgagaagtatctatcactgtgtctttctccattccacagctcttgcaaaccacagaactcaacatccatgcaactccttaactgatgtgcctgtttggatattcaaatactttctaaaaaaccaaaaattatgcattagcttgcagcacctacactctagaaaaatcaaccctcagggtcttttggtaccatggtctggagttgcttttattttcctagcttttgtcagcatactgctaactcggttgataagtgttctttctgtttaatgatttatgcttcagagggatttgtataggcaaaatagataaagccatatatttccttataggacatattttagatgacattactttgaattcagaacctgtgctctcactgtgggtatcaatgacttcctcaaaacaattcaataatttcaagggcactgtctcatttgtgaaggtcttttacagttaatatgactacctcagataattacaatactgcttctggtatgctacagtatataatagaatccagtgttattaactgaaatgaaatagtcgaatttttggtaaatgtaacaatttgataattagccacacatgctattatccattccatattcacataattggtaaatgttatgcagttttatcttcagtgaaaacatttaagtatcttgttgacttttgtttcagagaaaacatttttaaaattctatgaatgtcttagggcactagaattgaagtgaaatacatcttttgagcatacagagctgacatcattgtaggggtatgttgaatatatgttatgtattttatgtattttagtagaaaggtgctgtatgaatgtgaaagctcctaattagcttttgtaaatcctctagctatgaattgctttttaaacaaggatgaaatgatagcagaacacacacacacaaacacacacacacacacacacacatgcgctaatataatactgactcatcaggcagttgacatgatgtggtcattcaatatctagcctctacttttaaaaaattattgttggaatagtagataggaatatagatttagcaaagtgctttgagatttaggaagcatctctacagaatgccaagaaagtgttaaagaatttaaatgagacctaaaggagttttctactggtgaggcagtaattatattagaagccaaaccatcacatattaaggactgttttgtgctcaccatttgtaggtgaaaaggcaatcttttggaagacaaaaagaacaaacagcccatcatcatgtagaaatgtagaaacattgtgctgttcacaatcttgttaccaataattagctaattattcttttttactaaaagcgaaaggatacatgagcactgcacatcatgggaaaggagaggtgtcatcagaacaggctgcagacacacatccagggtaaagttagctggattattgtgggtcctggttggtcaaaccatggttgccaggaaaaccaggaagatttaagttatcaatctagttctagtagacctatgactgagggtatttatctgtctagaaggaagaatttttagtcaatggaggcaataattttaggcaaatatggtttccatcagaaaagtccaaaggaaaagtgttgctttgggaaatatgcgaagaatgacaaagggacaagactttagcccaaagattggtgcaacctaacctgagttgactcataagtccatgattcaatggaggacagtagttcatttttagtaggctagtcaaatatctaaaatggaaaaatgcaaatagatacacgtgtaagataagagacaattaggaaaaaaggctccttacaaagttagctcaagaaaattcaaaagaagcaggagaagccagactatttctagacacagaaaatataatgactagctcagcctcaacaaaaggtctgaaagtaaaattggactggaaaaatagaaggttctcagaccatacaaatgagaagttgggtgtttaagtgagacaagtgtaacatttactgcacttagttacacattaagggctctgcacacatcttgatgtatctgtgtattattcatccatgctgctgcttggcttattgtggatgaattcctatttctaaggatccgagttcaagcagtcaattcaagtgatgttaaagtaggaaaacggaagtatgggtggaataaaataaccacataatcacaacctgtgtctactccaggtacggagacaactctgaattgaacgcctagttatacaaacagtagttatgcaacaaacagcagctgtctgacttggatctatcatcttaccagggcgcactaagttgctctagcaccatctcttgccatttctagacttaaactttatactccagtaagactaaattgcttactatttcagaacttttcacactatttaccttgccttgatcttttcctgctcgttttcctgttgggctgctattcattcttcaactcttcagctaatcttctgtctcctttaaaaaaaaagtcttctgagagctcctcaacagtcttaattactcgttcctttgcactgccttgtctcttataggcttttttattcttgctgtttcacactgcattttaatttgtttgttatgtagttattttatccgcagcgcttgagctctttggaagaaacagtgtcttgttcatctttgtggcttcatagctggcatacagccagaattgccatggaagggactcaatgaactaccaataaattagcgaatgaatgaattagaacccaggaactcaaatatggatcacaaatgtggttgcctttagttctagcaaattttcatgcagtatctgtaagacacaacctcttaaaacacctatttggaggcagatactatgttaggcgtcagctactctactagtcctttacctgaagtaactcatatacagtgtcaccaaaaccctgtgagaagggatgttctccctttagataaggaagctgaggcataaagaggttaagtaattttcccaggattacacagtgaatagtaactgaactaagatgaaacagtggtagtgagtttcagagctgagctctcaaccaccataccactttttaataagattttatgaaagttggctcttcttagataattctgaaaaatgagtccggaatttcattttctggaatgataagaggcattttagctgaagcaacccaacatttgtaatggatttaatttgagaccatgccaggacagttatcatggttcatttaagtatccattaagtggatggggaaaagaaaaccactatgagaccagaaggggcctctaatgagaaaaaagaagaggatgtgggaaactaagtatctgaagtattgggaacatatattatacaacattatagagacgtgcacctgctcatattcataaattttaaaaaagcc

SEQ ID NO: 8412 - RNA, 3130 nt, Homo sapiens
  source 1..3130: mol_type = other RNA
aaaacggtgagattttgtttttctaacaacttctccagtaatattgatgttgttggtctagggttagcatgttgagaacgaatgctttacacattttaaacctgtaaaatgttggaatgatgttttagcatagggtacccgagtgtattttctgagcactgggtctctagtaacaatcaggattttagggatgataaaagacattttggcacatagaattccctatttctgccttccacttttggtctttgtatttctttttcttctcctttatatatgtattttaaattcttcactcttattcaccttttcctcctgctccaagcctgacttagaagggtcttatgatccagacgattgtaacatgtaataggaatagtgtgagaaagaagccccaaggtaaaaggaatctgcttatctgctgtactcagggaaaaatctcgttgatgttaaactagtgtggtctctccttcctctagcatagttattcaggaatcaatcaatcaaaattatccaaatatcctgcaaacatttggcttaaaacttttatcagtattttcaacaactgtcaaatactcttgtacagaggaatgtggcaaagacggggagtgaatgagaagaagctgatagtaagtagctctacttttagtttcttattgtctacaatggctcttcattttgaagctggagctttgctttatggttggttcctggcttgctaataagaagcagatgtttcccacaaagatatttctgattctttttttctatacccctactttcaacttggagttggaaatcagtaagttcaagggaatttattacctttatcctcttagcacatgaaattggaagatgatagggttttaactagttgtcagattgttaggtgaaaggatatttctggctaaagaatggggctttcattgccgttattttcttttcaattctttctgcagttcctagaaagaaatcaaactagttacattgctaaggtgaagaagtacatgctctggtatttttgcagtgaagttcttcaggccctgatacctctcaagcccagatgtcaatcatttccagcaagtgcagcctttttttgccaccactgtgtaggacgtggttaccactcagaaattatggcaagttaatctgcaggccttattcaataattcttagaaacacatgaacacagttggtgcgctcgagcatttggaaaattaaattattctttagaattagcctactgagctggaagaaaataaagaacacttaccaaaggggaaaaaatgacaaaaaattctaatgactaatggtttttcattataattgcataatagtctcttgatacaagtgctactcattgttctgataattcactgatccattaggcccctccatacatatgcaagcacctctagtgcttcaaaaactaaagtttgtacaaaaaatgtggtgataaaaaacaaaatagttcctgaagtgaataatttttagtgggtagagttatatatcacatatagcaaagttgtgtctcaaattgaatgtcaagagaactggaaattctttgatccaaaaggcaaccaaatcgtccacgctactcagtccttattcaagatcctttaacaaaatggaaatatattagtgggaagtaattcttggataggagctgggataacaagttcctcttattaaacctactgatttcattctcctattctcccaaggtttagcaaaagcaggccttacattacaaatttcttgtagtattgagaaaaggttccacttctgtacatggagcttacaaattttttatcccatggagaattgttaaagattataaaaatgcatagaacacacacagggcaataatgtattgaggagttttaaattgtaatttttactgtcaagcccgtaagtaaatcatcaatgcaagaattctgaggttcaacgtttaaataagaaaattagtactcttccttctatgtttaaattccgtgtttgacattgtctggaaaaatgtcaataaatattacttgtgatattttcaattttcaaagcaattattacattaggaacacaggttttggaaagaatcacaactaatgtccctgaaagggtaatgatgccaaggatagttgtttttaataaaaagttagaatgtacatcgtgacaaactaacaatcacaattagagctatctttgtcccttttctaccctcaaaacaacctgagactcaggtgataatcccagtttaccttaatgttaataatttttagttattaatttgttcattttacaaatatatattggatataactatgcaccctgaactgtgctgaatgtttcagatgcaatggagagcaaagcacttgaactctgatttacaagaggagaccaaataatcacacaaatatttaatgagaaactgtgctaactaaccgttatgaaggaaaagtaaaagggacaaaaaaaaaaaaaaaagatacctcagggatatattaaggaaatgtacctattctgaagtttaatggaggcttccttggagaagtggcatttgatcctgattttgtgaccaatgacctgcatttcctgattccaatttcttttccctcctcattccagctaatatccaagaataatctcagggtaattgctttaggttccaaatgggacctaaaattacattaaaagctggcagtagatacaatggcagtggcctatgtgggactctgagcataggcttggcattatgtccagggtttccgttgcagatcccaccacttccaaatacttaggtcaggctatctgaggtacaacatgagctacaaacccttttatcttctaggatatttttatcccctgaaagtctgacttctgaaatgaatttaatattatcaagaaataggaaggagaactgtatctgacaaatatgacatttcaaatcagagtcggaagttcttatagtaaaagacaaatttcccacagaaataataaaaacccctaagagactactatgaacacctctatgcacacaagctagaaaatctagaagaaatggataaatctctggaaatatacaacctcccaagactgaaccaggaagacactgaatctccaaacatatcaatga

SEQ ID NO: 8413 - RNA, 819 nt, Homo sapiens
  source 1..819: mol_type = other RNA
aaaacggtgagattttgttttttatctctctatagcctactattgcactttgcacacactggataaacatctgctgaatgagtggacaataaaacagaagcaaatttgtactaatttttcaattatgttttcttccttgtatgcattattgttgacaccagcttgttgggaataagagtaagaatttatcctttacagtttcatagatctcatttatcaccccatgagtaggccaattggtcagtggaggagtgacaggtgagcagtcagtgaggtgctggaggagggtggatgtggggggtgtgaaggtttaggagtagaaaaaactcacactcggggctctgggttgctgggtgctttctttgcagccctggtttgtgaagtgatttatgggccatacatcaccttcctggttggctttgttgacaccttgtcacattcttgcttgggcttgaggaattcattgttcttgtttgaactcagcagctcctcctccttgtctctgagggtctccagagtttgagagtttggtgtcatgttggcccaagagactgttgtccttttgacagctcggctgtttgtatctccagaatgaaacataatcagatttttttcagatgtagcatctgccttccctccaacatccttgggttaatcacgtgcttgctggccaggatatgtaaataagacttggctaaaaaaaacccttaaaggattatgaagcaatcttgcttaatagtagcagaacaaaacaaaacaaaaaaccactccaacaaatcctcctgtgtgctaccaagtaatggaaagatccagttatga

SEQ ID NO: 8414 - RNA, 24147 nt, Homo sapiens
  source 1..24147: mol_type = other RNA
aaaactgcagttacttttgccaacactgtttttcacttcaaagctatataatcctttgtcactcatttcggcacaggggattttaagggaagccactttattgatgaatgtaatgtgatgtttgctgtctgcagacaattctcttccatctttgaaccacttggctgagagttctggtgttccagtcactacacactctaatgcaaaaggatttccagtagtgacagtcatgggttcgggcttctctatgattcttgctggttctagtacagtcaagactgcagagcattctctcattccagcatcgtttttgatttggcatatatattttccagaattagatgcttctggactccccagctggagggttgcaatgttatcaatgaatgaaatcctggtattttcactctctctgatgacttcacctctatctttcagccagacaacagaaattggctggaagccctccactatggcccgtaactcaacagcatccccaataagggttgaggtgtcacttagctttttcacgaatcgtggaggttctttgaacttgacagagcaagaacacgtgtcacttcccacctcattagtagctttgcagtgatattccccgacatcggaggcttcaagattaaggatatgaagacttgtatcaaaatgttttgaagtgattttaaatttcttgctgtttctaacctgctttcgatctttaacccatactacttcaaatgggggagttcccgaaatttcacattggagaatcacatcagaacctttaagagctcctactggagaaggcttctgggtgaaaacaggaggtgctttcactgtcaacgctgtgctgcagctggcgtcaccaacaccattatgagcctcacaaatgtagtccccgctgtcttcagcactagcttcattgatcgtaagcaatgccacagaattaatgaatgacatgttgtatttccaactttcatgaagttcgctgtcatttcggaaccatgaaactttgatttctggggagccacttattttacattccagttgaatggattctccctgctttgcaacttttgaagcttctaatttcttaacaaactttggaggttcttttacactgagctgagctgagcacatgtctttgccaacatcattggttgcttggcaagtatattgaccagagtctcctttgcctactttaagaattctcaaatgaggagtgtttcccacacatgtgattgtatagtttcctccaggacggatctccttgttatcttttgaccaagtgattcgcatcggttgagcaccagtaacatgacactcaaaatcagcactttctccagcaataacatctatagatacaggcttgatgtcaaagaagggagatttcttgggttctcttgctgtgagtctagcactagaagatgctgttccaagtgggttggaagctgagcaagagtactggccagagtgactcaagtcagtttgcaaaatttttaaagttgccacattatctacaaatgaagtctgtagattttcatcgtctcttaaaagtactccatctctataccagcacacttggatgggtgcagagccatttaatcgacaagtgagtgtaacaggtaaccccacagtttgttcaatgtcctttaattgtcttgcaaaagaaggtgggagttggcgctcttgaattctgaacacagtcttagaagaagcagttcctatactattttctgctttgcatgtgtactctccactgtcattgatgttcactttattaaaaacaagtgtggccacattgtttgtaaagtaggtcctgtattcaggagttggccgtaatttggtatctcctttgtaccaagacactgtaatttctggtgtcccagcaacttggcattgtaaagaaaccgaatctccaactgctgcctccagaggttccagttccgtaacaaaataaggcggttctaatgtagataccagagctccacaaacatcccttcctgcctcattttcaatctcgcaggaatactgccctgcatctctttttgtgctattcagaatttccaggatacaagttttctctgttgtgactatgttacatttttcagaggtagttatgttaaaaccatcctttttccaagtgacagaaattggaagtgttccagtgtaggtgctctccagaattatggacttccctggttctacagaatgatcacttaatctcttcaaaaatgcagctggttctttcacaaagagacgggtagtgcaagatgcttggccagcgttgttagaaaccacacaggtgtattccccactctgagatatgtcaatattaaataattccagttctgccacagtgtcttcaaaatagatgttgcaccggtctcctttcactagttctctggcacctctgaaccagttgactttgaatggaggggttcctctaataacgcttgtgaaggttacatttttgcctggtagtacttccaaaggttcaggttctttcacaaaagagggtggttcttgtacagttagcactgcacgacattcatcagacccagcgacattagcagccacgcatgtgtaattgcccatatctgaggaatccagagaattcaactgcaatgtgcagacattatctgaaaatgtggtttggtactttgctccactgacaatcttggttttctcatgaaaccaggcaactgaaataggtgatgatccagctactttgcattccaagatgcaagaagcacctaacaccccaccagtatttttcagtcttcgtgtgaaagagggaggaactgctcggtctgaaacatcaaccacagctgtgcagctgcttttcccaacattattttgaacctggaaagtgtatgtgcctgcatcttgcctttcaactgagagaatccttaaggaagagattttgttgtagaagctaaatttgtgtttttggctgctggtcaacagctttccatccttgtaccattcaacagagagttccggagtgccagccaccttacactccagagtgcacgtttctcctacagtcaccgtcatcggtcctgccttctcaacaatgactgcgggctctaagaccatcagtgtggccatgttctccctcattccaccatcattcttgatttggcagatatactttccagcattagctggctctgcttttgcaaactgtagagttgcaacattttccacaaatgtaatcctgatgttttcactttctctaatcacttcttccttctctttaagccactggacaaaaataggctgggcgccttctatggatgcttgtaattcagcaggctctccggctacaacagtgaggctgttcagtttggagacaaatcttggtggttctttcaattttacagtacaaacacaagtatcacttcccacttcattctgtgctttgcagtggtattcaccgatgtctgaagtgtccacattgagaatgtgaatacttgtgtggaagtttttggatgcaatcttgtatttcttgctgcttctgagttgccgcttgtctttgtaccataccacctcaaacggtggtgttcccgaaagttcacattcaagactgacttcagcatttttaagggtttctactataggagggaagctgctaaaaacaggtggctcttttactataaccttggtactgcagcttgtgctgccagcgggattctgagcctcacaaatgaaatctccactgtcctcagtactgagattgttcatctgtatgacggccactgagtcaatgaaagtcattctgtacttatcactggctggaagttcatgttcatttcggaaccacacaactctgatttctggggatccagctatcttgcattcaagtcgtgaagagtcacctgctttcacaattttggaggcttctaatttctttacaaactttggtggttctgtcacaagcaacatcgtagtacaagagtcgctaccaacatcattggtaacatggcaagtatactgtccagtcttagaagcatccactgagtagagatttaagaagctagtcgacccttccaagccaatgaaacatttaggacctgagacaagttccacatcatccttaaaccattttattttaaatggtggtgttccttttagtattgccttaaattccactgtagaatcaggtatggcttgctgtcgcccaggtttcactaggaagcttggtggttctttcacagttaagatgccactgcatgcatcatctcctgctacatttgacactttgcatgtgtaatttgcagtatcttctaattccagattattaacttccagagacacagatctctcatggcacacaagtctgtattttgcacttgtagatatttcttttccatccttaaaccactgagcactaatgggaagtgaaccagacaccttgcactccatatgaatagaagagcccagaactttatccattttggttaattttttggtgaatgatggaggaatattttgatctagcactcttaagtaggcatcacagctactgcttccgaagtcattttccaccttgaaagtgtactgaccgctgtcctgcttcattactgactgaattctaaaactggccacgttattttcaaaactcattgaaaagtatctactgggaactatttgtttcccgtctttaagccatttcactttgagttctggtgttccagccacaacacattccaaggtcatgggatctttctccgtaacatcaactgatttagctttctctacgatttgagctggttcttgtactaaaaggaaagcataacacctctcaactcctgactcattcttggcttgacaggtatatctcccactgtgtccattatccacacttctgatttgaagtgtggccacactgtccacaaatgaaatatagacattatcatcttcatcaagaatctgatcatcctttagccaggttatagaaataggaggagaacctgccacggtactctgaaaggtggcagaacttttcaaaacagtagtggtattttctatcttcttaatgaatgatggtggttctttcagggcaactctagtactgcatgagcagctgccgccttcattggatacaatgcactggtattccccagtgtctgaagggtcacacttggttatatggaggttaaacacagacactctgtcggtcaatgtgtattttttgctgcttcgaatttccctgttattcttcagccaagtgacttcaaacggaggtgttcccgtaacttcacactccagctccacgtcactatattttactacctccacaggcttcagctctctgataaaggtggggggttctttcactttgagttcaatgctgcagctcgccgtgcctgcgtcatttcgagcttcacacacataagtcccactattttctaccctggcaccagaaatctggaaagtggctaaaccatcaatgaaggaaatgccatgtttctgaatggctgttatttcattcccgtctagataccaagacactcggattttaggagtgcctgttatttggcattcaaatgttgttgactgtccattcctcagcactaagactggactgggcttcttaatgaattgaggaggttcttttacaaagagagtggctttgctggttgctgtgccaacatcattgcttagttggcaaatgtaggttccagaatcggtagctttggctgcaaagagctctagactggtagaggtgtcatccttccaaactgagcgggctgctcctgagtgtaactctttgttatctttaaaccactttattgtcatgggtgcagtgccacccacaagagcctttaactgtacccttgtgttgggattgacatcttgtgactgtggcttttccacaaagtaagggggttctttgactgtcagatgcccactgcattggttgtgccctgccttatttgtggcagaacaagtgtatgtcccactgtctgtaccttccagctggctgatttccaagaaggcagtattgtcatgaaaagagaatttgtacttttcactagctgatatttcttggtcatctttgaaccactggatgcttatgggatgtgacccagccactatacattctaaatcaatgaaagaacctttaatgctgtccattttcttcagctttttggtgaatgaaggaggtatgataagatctaatacattaattctagccttgcagctgctcctcccaacatcattttggacctcgaaagtatattctccactatctttcttttctgtagaaataatcttcagtattgagactgtatcagtgacactgattttatattttgagcccagggtcagttcttggccatctttaaaccatttggctgtaatctccttagtccctgaaaatttaacctgcaaagtggctgggtctccttgggtgacatctatagacacagcttcctcggtgattgttgcaggttcttttactgagagtaatgcagaacatctttgtattcctgcatcatttttggcctgacagacatatttcccatcatgcttgacttcaatgccactgaggtacaaactggccacattgttctcaaaggtcattcttatattatcgtcttcagtgatttcatcgctgtcttttagccaagtcaccgtaattggcaaggagcccttcagagtggcctggaaggcagctgtgcctccccggagggagctggtactctcgatcttctttatgaaggatgggggttctcttaaagtcaccctggcactgcagatgctgctgcccacctcattggtcacccgacactggtattcgccagcatctgcagctacaaacttgaggatctgcaggctaaccagatgatcctgaatgaaagtcttatactttctaccacttcgcaggattgtgttatctttgaaccaagtgatctcaaagggaggagtgcctgccacctcagccagcaacatgacatcgtactcctttaagacttcaattggcttaaattccttggtaaaataaggtgactctttgactattacaatgctactgcagtggtcactgccagcctcattttgggcctcacacatatattcaccactgtcttcgatgccaacatctgtcagtcttagaactgcagtagactccacaaaagacattctgtgtttgctgctctccttaatttctctatcatttgcaaaccatgttattttaattggaggggtaccagttactttgcaggctagctgggtggcatctcccttctttaacagctgtgatggctctaacttttcaacaaatgtggcaggttcttttacaaacaagtttgcactgcattccacccctccagcgacattgctgactttacatgtgtacgtgcccgaatcagaggtttttactaaatagagttccagggaactctctaaagcttctttggtaatatagcagcttccaccagaaaccagctctttgttgcccttaaaccatctgattgtgagaggagtagatccttggaaagtgctcttcaggcagactgctgagccaggcagaacatcctttgagccgggtttagttacaaaactgggtggttcttgcacaatcagggctccactgctgtctttgcttcccacggaatttgtggctcgacaagtgaaattccctgcatcattcatgtctactctgatgatctccaaagaggctgtgccttccacaaatgctatcctgtatctgtcagaagcagctatttctttgccatccttaaaccaggacaccctcatggggagggagcctgcaattttgcagtccagtctgcaggtaccattaacaacactatccacgttgcgcaagggtttggtaaaaaatggagcaatgtctcgatctaatacagtgaatgtagtctcacaggagctgctgcccacttcattggaaatctcaaatgtgtattggccactgtcgtgcagctcagctgaataaaatttgagctgggcaacattgtttttaaaacttattcggtattttttactggcgaccaagggtctcccatctttgtaccatttgggcttcagttctggcgtgcctgccactgtgtactccagtgtggcgggatctcctgctgtcacctggatcagttctgctcgctcaatgattttggcaggttctttaactattaattccccaacagatgtttggcttccagcttcattttcagccaggcacgtgtatttgcctccaaaactaatctgaacatcagggattatcaagactgcaacaccattggaaaagctcattttgatttttccgtcttctctgatgacctcttgacctttcatccatgtgacagaaatgggctctgaccctctcacagcagcttgcagggtaacggtttgtcctcctagtgcaatcaaatcatctactttctttacaaaggttggaggttctttgagtaagtgggttgccatgcagccacacttgccgacttcattagcaacaacacattcatattcaccaacatctgcactattaaacgaaaagatctccagacacacaagagacttctgagaaaacaatctgtattttttactacttcgaatttgtttcttgtctttgaaccagctaatttcaaatggtccagtgcctgagacttcacactgaagtagagcatttgttcctctcactatgtctgcaggctcaagagttttgatgaaagaaggaggttctttgataactatttcagtactgcagctatcactgccgacgtcattcactgcttcacatgagtaactcccactgtcttcaacttttacatccgtaatatcaagtatagcctcagaattgacaaaatacattcggactgtgttactttcactgagttctttgttatttttaaaccaagtaacctggatcacaggtgagcctttcagcttgcaatggaggcgtgctgattcacctgggagcattaaataagagggatccaccttcttcacgaaggatggtggctctctgacagtgactgtggctgagcaggagctgcttccagcctcatttgaagctgtacagacataggttcctgaatctttcagtttggccaaaggaatctcaagtgttgctattttatcttcaaaacagatcttataatctttccctggggggagtttttgcccatctttgctccacgtaactgtgacttttctgtcttcatctacttggcactcaaggtggaccttcttattgatagcggactgcacaggctctaattctttaatgaaatgtggcttatcaatgatgatcaactctgcttggcagatgtctgctccaaacttgttggaagccttacaagaataaactcctctatcttgaatggtaaggtttgagagttctaaaatgtgtttgttttctgcgtcggaaatcctccagttaggtgaaggtgagagtgcagcaccatctttctgccaaatggtttctatcacaggagtccctgtcactgtgcagatgaacttggctgccttacccacaaaagttgtaagggacttaggtctggagagaaaggttggtggatatgcctctgtcacagttagtgtggctgtacagctgacactgccatactcattggaagctttgcatgtatactcgccgcagtcaaccacctgggttctcaggatttcaaggctggagatatactttgaagatcgaatagaacacttgtcactctcataaatttctcggccagctttaaaccactggaaccggacattgggagcactttggatctcacaggtgaatttggctaggtggcccagtgctacttccaggggttcgattttcctcttgatcactggggcagctctttttactacagtgagtttggctgaagttgctgtttttccgctgtcattcaaggcctcacagacatactctccttgatggtcttcggtatttactttgtcgatgactagcgtatatgtattttgatcttgtaaacacttgaacttttcatctgaaggcaccagtttattctcaaaataccaattcacctctttagcatttgttatggatgttgtgaggtgtacaatatcaccttcctcagaaacagtgtccactaaaggtgtatgtatcatggggccatcctctttgattaagccaccctcagcttcctgtatctttactgtagcaacctcctcagtaccactttcagaggaagactcctctttttcctctgatggtttcagactctcatcttgtttttcgtcagagacaacagctgaagcaacccctttagtgacaggtgtggcatccaaatatttaaccctactttgcacgttaaaataactgacctcttcagttgagatcagatatttagattcaacttctggttcagtaatgggttcaaccttctgtgaacctgaaaaagaatccatttcttcttgcaaacttgttttggctccttgctgaattctaggaccctcagctgttaggatgtctatttcctcatatataatagcacacaaagcatccctaagttccattttcaggttagccatttgaggatcaacatcttcaataatgatggttacttcttctgttacagactttgccgaagtaacaaggtacatgcacatgatgtgtctgggctcttgggtgatgtttacagcctcgacctccaccttttcaatatttcttagccactcagagaaaagacctggctgctcgctggccacggctgcttgcaaagcccggcagatttgaattttcaggtttaatctctgctcttctggaataccagaaagcaagctttccttagaaagaaggtcccttccctgtacctcctgcactttctttattgccacgggctctcttttagactcaatgatttggtctgggggcatcaccacgttgtcagaatgctcttctttgagcagtacctgcttttcttcaagtgctagtggaaatcttaaggacttgccttcctcaattctgaccgcagaatcttgccctgcattttccagtggatttgcactttctatcaaaattttacctccttctgtgcatgagtgttctgaagggactaggggctcatagtttacctgagagatcatgacatcaggactctggagactctccacgtgtccctcagctaagctctgactcaagatgagcgcactttgtgcctcttgcttttgaagagtcactctttgctctctgttggtgtcagatactgtcttttcttttggtgaaagtacttcctcagccacagaggttagataagaatgcattggaggttctattgaagactgtggataattcccttcaggttcagctaataaagttttcagaggctcaactgttaatgaattaatttgttctatggacatggcacttgggaagattttctcggtatctgatagaactgcctgtgtctcaggctcttcaggcattagaataccttctttggagaaggttttctgggactgtacaatctgcagctgtaggttgggagatggttccttgagaggctgaaagtgaatactgccattgatgcaaagaaattccctggtgctttcaggagtgagcttgtcttgctccaaaatggattgcaattcctgagctcccaaaggaagctgactgctcaattcattggctttagcaatatgctcataagatagttgctggttttcttctgtaattaaagcagctttcaaaatggtgtcttttacaaacgttgcaatttcctgctctgagtcaagtgcttcaactgcgggaccctttaagggtgtctgtggaaaatcctcaggagcctctggtgtggactttgctttgcagggggtatcagtcatgtctgtgtcttccagaagcacaagcagctctgctgcacaggtggactcacccaacatattctctgctttacagatatagaggccactgtcttccctctgagggtcattgacaatgaaagttccagagccattagggttatgaatgatagtgtaataaacactggtgcaaagctgcttgttttctttgaaccatgtaacagtaggggcaggctctccaaccactgtgtactcaaagatggcaggaagcccttgagcacagcgaattggttttaactccttaaggaagtgaggaggacaaggacctcccagcttttccagagattttgccactgctgattctgtttcagtgtctttgtgaccctctcctttggaattaatttttagataggcactacatattgtctttccatagtcattactggccatacatgtatactctccctcatcctccaatttggtgaacagaatgatcaggctatgatcatcaccgtcaaaaacaaatttgtagtcagcagaaggggttaatagcactccattaaagaaccactgaattttaggtttggggatgccaatgacagttacagacagtgtagccacatcccccatgcttatatcagcatttgacacttctttgatgaaaattgggccagtgccttccttttcggaatcaaatttagttgggtaaactggagattcagacaaaagttcaagtgtttcatttattttagataattgaagttcggcgctatgaagtccttcttcctcggcagacagaaaagaactagaaaactctttcatttccatctcaatctcttgttcaatcctctcatgcaaaattgattcaggagcaccttctacacttagtactgctgacgttgtcctctctccacagtcattgtgtacaatgcagctgtatagtccttggtctaccagctgaacattacatatggtaagaaactgaatatttccattttgtgattgtttcagtctctcggattcctctatctttgcaccttcgtgagtccaggttacatcaatgaaagaatcatcttttaaaacacagaggaattgagccgtgtcaccgcactttacagtgacgtcctgaagatgcaggaaaatcttgggcgcctcacccgtggactctttagcacattccttagatagctcagtgctttctgcaatttgtgaaagggatgcagtatggcacaactgtgtatcttgaacagatgcagctgtgtggatggaactttgagatacactttcaaaaacctgcacttcatattcatatgatgatccttgaaatgacttaatttccttttgagatattttgctctcctcctttgtgaaagaggaatctgccactgcctgggacttggtggactctcttacatctttcccagaactttgcctatctagggcttgcacttttggagtcactgtgagtgtagctgcacaagtggcttccccagcactattggctgctttgcaagagtactgcccagcatgctctgagtaagcatcaactataagcattaaagccatgcctgtggactcctcaaaatggaaaactacatcttttgttggtagaattagctgctggttatgaaaccattggatttctggcttgggaatgccagaaaccctcgcatgaaatctgactgtctccccgttgtgcaccctgaggcttgacagaggctggatgaagctgggcttttggccaaggggctccttcttaaatgaaactgataaagagacatgccattgggagtttgatgtattttcttcaaatttgctaaatccttccagactcaggttggctgtgcttgatacttggcctacagcattactagcaacaaacgtgtaagttccttcatcttctggataagcttcggcaatttccagttgataagtgtcttcaaattgagtcattctaaagaaccgagatggcttgattttcttgtctttgctgtaccacgacacttttagatctgttccagaaacccggcattgaaaacgggctggctgcccttcagaagtgacagtgtcctgaagcggggtgatgatggcaggtggataaacaggcatttcctgatcaggagacacaacttctggaacttccactgagagtgaagctgatgttgtggcaacaccatagtcattcttggcttcacaggtatagactgccgcatcctctgggaaggcttcaattagcaaaagcgtgtattcttgcccatcatgaagaaatttgcacttgaagccagtggaaagcagctgctcttccttgtaccaggaaattttgggctgtggtcttccggatatcacggcacagaagcgggcaggcttgccagactgcacagtgacaggctggagctcctgcagaacttggggcggttcaggagcattgacatagagagtgacagaactcctgttccttcctgccacaaaggtgtattctcctgcatcgctctgtctggtctcagagataaacattcggtggattcttctttccactacatatttgtgtcgttcttgaacttggaaattgatttcaatgccatctttataccagtgggcatcaacatcgtcttcattgacctcaaattcaacaacagcacgctgtttctcaatgacctgaacctcctttttaatacttcggatgcgaacatctctgccttctacaaagagttttgcagttgacacgttgcctcctgccaccactgtgtacttcccagcatcagacatccgggtggatgggatcagaaggcggtggacatatttctccttctgaatctttattctgtctgtgatctgcagttcctggtcatctttcatccactgtacagtgatgtcaggttcagaaacttcacattcaaacatggctcgcttcttctccagtaccttaatgtccttaatgtgtttcctaaattctatatgacgagcttccacataaagtgtggctgttgatgttgcttttccagccacaaaggtgtagtcagcagcatccccaaagtgaacattcctgatgttcagtgagtgtgtgagctttttggttctcatctggcacttgtcagttgatttgatttccacaccattctttaaccatttgtaagagatgccttcatagttcactgtcacctcaaaagtaatagtgtctttttcttcagcgttgatgtctttcagcatggaagtaatcatgattggggtgactgtcagggtggcactgacttggtcattgccacagacaaatgtgtattctgccgagtcctctgtgctggtgttcatgatgatcagctgatggagttttccctgcacaactatcttgaacttttcactcatctcaatttccacaccattcttcagccacatggaagggacattgaagtgggacacctcacactcaaaagaggcagttttggtctcaggcacctcgatatttttcatggtttttgtaatatgtaatgtctccacaaacagttttgctttgcattccaattgcccgaccacagctgtgtattccccagcatctgagggggagatgttctgcagcatcagcttgtggactttcctttctgagaccagtctgtgtttgtcacttggcttaatttccacactcttatggaaccattttactggaacagtgtcatgggaaacactaacttcaaaggcaacagtggcattttccaaggctgtcacatcctttggctttttaatgatcttgacagtctccacgtgcagtctggcactggctccaagccttccaagcctgaagccataaacagactcatccacgatggcacagtttttaatcctcagagagtaaattgttcctttgacagagatagcatacttttcattggattccagcacaactccatttttgatccactggacacctttgacattagggtgtgtaagctcgacagtgaaaacagcatcctgtgtttctgtcactgtgaggttcttcagagtcttcttaattttgacagcttcaactttgagtttggcagatgttttggaggtggccaccttgtaggtatattctccaatgtcatctaatttggtggcagcaatgataagtctccttttgtggccatcagactcacttctgatgttgttagtcagtggtaggtgtttgccatccctcaaccattcgcctttggaatctgggttggcaacttcacattcaaacacagcttcctgggattcagctacggtctgatctgtgagtggcttggagatggccccacctgccacagtaagttttccagatgtcatattttctcccgcgtaaaatgtgtattttccttcatcatctttcatcatatttagaactgtcaatttatatatttttccatgtgcttcaattttatatttagaactgggcttgatttccttgtccttaaaattccacaggacatcaattccagagtgggacagctcaacctcaaacaccacattttgagtttctgtacaggtaaggtcacgaagacctctgataattttaattttttctacagagagattacagttggtttcaactctgccaactatcagcttgtaaggtccttcgtctgaagcatgagttcggttaatgactagtcgctgtttagtacctttcacaatggcctgtacacggtcatcaggcttgatttgttcatcatttaagtaccacttaacagaagtcacatcagggactgacaccttacattcaagcacagccttggtgccttcaatcacattaacatcttttagaggtgttatcacgtccacactatagacagagacacgcccactggtggagaggccaagggctggaatggtgaaagagtaatttccagcatcttccttagtcatgtcttcaatgagcagcatatgagattgtttgtctatcacaatgtgaaccctgtcactgggctgcacttcttggccgtctttcatccagacgccttccacactttccaaggagactttaacttcaagctgaacaatgtcaccctcacagactttttggtcactaagtccttgtaggatagcaatggggcggggtttcatctttaatttacaggttgtctttttcccgtcgatgacaaagctgtattctccctggtcctccttggttacatccttgaccgtgaggttctgacgtccacgacgagatgtaattgtatatttgccattggatttaagctccacatcattatgataccattttccttctatattttctggggatacaatgcactctaattctcctgaatatgattctggaacttctatgtcctgaagttctttcacaaactcaacaactgcaccttcaacaataagtttagcagtcgttttgacattttcatcttccacaagtacacagctgtaatcttcagcatcagacgtatcaatggtcagtatggagaggaagtgaacctttctgtcagagtgcatcctgtatttatctccctcatgaacctccataccatctttataccatttcactttgacaaatggttctgaagtttcacattcaaaggttgccatagtgtctttttccttagcaacaacatcttgtaattcctgtgtgaaagtgatcaattgcttggcttggacaagtaagaatgcgtgactggaggtttctccagctatgttgatggcttttaccatgatgctggcagagtcctcagcagtcacatctcttatgaccaattcacaaacattgtcttcgggccagtaccagtagatccggtcagaccgttcaattttgacaccatttttgtaccattcacattcggggtctggtttccccacgactctgacccggaagtgtgcatcagatccttggcccactgtttggctctggattctttcgaagatttttggagcctccatactaggacttagttcaatcttgtcaggtttaaaagttggaatcgtgattttgccttcttcggcaagagctttcttttcctcttcagttaactctttggtccagtggagaagttcatcttttgtcttcctgaggagttcctcataggattcatccttctttcgagacttgagctccacagcggtaatggcttcataatagccctcttctgttctgcgcttgaatttactgcgcagctcttccgactcttcaggcactttttcatgggtaattctttcagcccttttcaacttcacaacttctttggtttcagtggtgtcaacaggtctatccactttttgtacttcaaactgaagctttcctggttcatgtacgtgaaactcaggccttggttcaggagctctcctaaggacagacctaaaatcttccctctgttgaatctcaagcttcactttatgctctatcacaccttcaggattttccgcggtgaccttcacttcacctgtgtcatatgatttgcagtccacgatgtccaggtaatggataccatcatagcgaactctgaaccttttgcttttgcggatgagctgtccattgaggtaccagttgactttgggctgagggtagcctgttaccctgcagcggaaccttgcagtctccccttcaagtactctaactggctctgggtacaagacaatgtctggcttttgcttttctttctgatctgttgttacacctgtaagtgcaccttcatgagccattctctctaattcttcaattctctgtaagcctttcctcccctcaggcaattgggattcttccacaagacttttctcatctttaacaataagggtagcagatgtgtgatctgttccatatttgttagtggctctgcaagtaatgataccactgtctctagaatatgcaacgccataatcaaggctgcagtacccaaattcattgatcatacggagcctgttggctgcttcaagtggctttccatcatggagccactccaccaccatcgttgggtcaccaatgggtgttagcctgcattcaaagtgggcaggcccaaagcgcttaagtcttaaggaagtgagttttttcttgaaaaatggtttctgttgtttctctttgtcatagagatcaccttcttcccattgctcttggccatatcgcaaatggaggggctccagttctggggctgcaatctcctttgctctatatgtcccccgtgggatgattaactttctctctggctcaggctctgcaaactcaacttcaacatttactttgcatcttgtagtgtctctgccagctttattaatagcagtcgcagtataccaggcagaatcttggctgacagtggaatcgattttaagggcagcttctcccttggttccttcaattctgattttgggatatttatgaggcacaatgatgtcactgtttttcaaccatacaatgtcagggttggggttacccgtagctctgactttcatttcaagtcgggaaccttcctttatattgacatttttcagtttttctacaaacatcggttttacctgatgttccacagcttccacagttaaaatcactgaaattgaagatctgcctgccctgttttgggcaaccacagtccattccccagaatcactgggtgtggcagggacaataattagtgattgagtaccatcttctttaatgactactttatgggtatagtcattgacaatttgctggccatcatgaaaccagaacgtctctggcataggtctaccaacaacctttaagtcaaatctggcagtttgcccttctaaacatttgaaagaaacaggttttaacacaaagactggtttatatagtctctcaagttgtgactcatctgtctcctccagcctacgtccaggggacattcttgcaggggacatccgtgcaggagacatccttgcaggtgacatccgtgcaggagacatgcgtataggagacctgctcactgaacgtggagagagagatctgattctgctcactggctctagtgtgggaatgtaagtcggagctccaagtggtgcagcaggctccacatacaatttccctgagcaaattgcatttcctttaatattgctggcaaatgcagtgtagattccttcatcttctggaagaacaacaggtatacgcagactagctctgccatcttgtagaaagtccatttggtatctttctccatgtttgatgcgcttgccatctttgtaccaagcaatctttggtaatggatatccagacatcttgcaatgaaaagtgacacccatcccctcaagaattctataattcttgattcttgaatcaaatcctgattcaacagcttcagattcagaaatgtcaactgccatcttttcttctccatcttcttcaagaagttcttctaatgtagtctttattattctatattcaatttctttaataagtctctcttcaaaggaagaaatatggaattcctgatcttctacataagttctgaccactacagtatctttggccattttcttcctaattaaggcttgttctttttcatactctttttcatactcagagtatacaaatccaggtgctgtttctccaactttaggttcttgaacaaatgcagtcacttgtgtctgataaagcatttcttgctgggacttcatcagtaactcataatcagcttcttcaagcaaggaagcagatgcagaagtttctccatgcttattgcgaacaacaatagtgtattctccagcatcatcagcaaaagtcatagaaatcaccagcttgcattcaccggtttgtttgttgtaactcactttgtatctgtatccagtggttagaggaacaccagattttttccagtatacatggggctttgggttgccgccaacttggcatccaaacaccacgctcccaccttccaccagtttctggaccactggttttgtaataaagtaaggcgcggcaggttctccaggccctgcttgttcctctgtgaggctagtatcagtcataaccacatctcttgactcaacaaagcgtttctcttctgtagtaaatttctcagtcacggctgtggtttccttttcaaattcttctgacacctgcacagccagatagcaggatgtgctgacggttccagcctcatttacagcactgcaagtaaatcgcccgctgtcttccgcaaatgcttcgcgaatcataagacgagcaattccactctggaaggttatctggaagtcaatggaactttcgatttggtagtcttccctgtaccatgtcactgtcggggatgggtatccagagatgtggcactccaaggtgacagattcaccttctatgacagtcacattttttaagcccgagaccaaagttggtggagtaacaggaatttcaacaggtgctggtactcttgctgtttctgttaccttggcttcgcgtccgtgcagtacttcaaagcgctcttcacggacggtggtgccagtgatgctcacccctacttcctttttcacctcaacgccagcttcactcttgtaagtatctggtgtgtcagcgaaggggaactgtggcaagggtgtgggctctgcccttactctagtctcactgggcttcacagtaggagccttcaccgatttggtgatcttctgagcagaagatgtggctgacaactctttttgtaatgtggcaatagcactaccggctattgatgcctcatatccatgttctgtcttaggaacagaaatttttgaaacagtaaagtgagggctagctgtgcgggggcgtttatccacatggactaatctttccgttgttagatctgtagttttcttgatctgtgatgatatgtgcattcccttttgatcagtagttttgatatgagtctcagaaggagcctggattactctaggcttgactgctttagggacaacgtggggttctgaggctggacgttggggaggctcagctacctttgcggcggaaatgcgttccttatatccgtactccaaagtggtctgctgagcataggattcttcaagatgcccaggctctctgggctctctgactcgggcctggtctactgcagcaacaactgttgctacagcttcagccttttttccaacgtccacctttccatgggtaacttggatttgttcttgtctagtagccatagtttctctagttctcagtattgtttcttgttctttggctttagcagtagcaactgctattgtagacaaggcagttttctcggcttcctttctcatcttctcctgagttatttgcacttgttctcttttggtagtaatgccttctctacctcttgatactaaatcttgttctttgactttgggtgtggcaactatgactttaggtacaactgttttcctagtttccttcattatcttttcataacttaggtgcatttgatcttgttgtgtggtagtttcttcttgagctcccgggactgtttctagttttgtggactttgcagtggcaactaccaccatggatgcagcagttatctcagtttcctgtcttattgcttcttgagttacttgtttctgtttcttagtaatttcttcagaaattctagtttcttgttctttggctttagctgcggaaattactacctttggtacaaatgttttttcagtttcttttcttatctgctcatgagttacgtgcatctgctcttgctttgtggtaattacttctttggttcttgattttaattcttgttccttggctttatcggcggccactactaccttagttacagcagtcttctccgcttcctttcttacctgttcttgagcaggttggatgtgcacagcagtcgtggttgtcctctgagcagtctgctctacagcgctgatcactggttctctcactctggccatatcaacggcagcaacaacagtcgcaacagctgcacttttgtcagcatcttgtttcacctctttagcaccagtggcaacagcctctgctgcgtagctagcactggccgacacactggcggcagcacccgcagcaccactgatggtcacttgctcctggacaccgtatctcccttcccatctctcttctgtcctgatctgagtagaggttgtcagcgttgtctctctcatctcagcctcagatgaggaggccacgtagccctcttgcttccaagggggaggcacttcaggacctgtggccacggtggatgcctgagtcttacgcatgagcaatggagacctaacagacctgatgggggatgtggagattcttgctgctggagacacggacctgaccggagatggggtcggtgcccgcacgtgtctgaccggggaaggggagtgtcttatgggcgatggggactgctgccgagccagctgtgctttggcagcaatagacggtggtgttggggatcttgactttggcttcggaggaatcctgggaggtgttttatgtggcagctgttgcccagcggcaccatctatgaccatctcaactgttgcaattgatctggcatcaaagtgggcttcaatcttcttttcaattcgggtttgtcttgattctgagatctgagcagtcgaaacaattgtctttgtctttttagcaggtacttcttcttcaccttgaaccagtaattcagcagtcgaagtagctcttccaacgctattggtggcatttactgaataggtccctgagtcctcagggtatgcttctgcaatcagtaagctgtagaggtcgccttcttgtgaaatttggaaatcaagggagctctggatttcggctccatcccggtagaacttcaccacaggtgtagggattccagtcactctcacttggagtctcacttggcttccttgtctcacggtcatgctctgcagtcgttgaacgaagttgggtggtgctgtctcagctttcacgagaagctcagcagtactagtcgcttgtccagatccattggtggctttcagggaatatcgtccactgttggctttagtcacggcggggatcgtcagtttagcgcggccatcgctaaaggagatctgcacgccgggcagagtggaagtggaaatcacctggccatccctaaaccagctcacctcaggaactggaaaaccactaatgtgagcctcaaaggttgcggtactaccctccagtaccacaacgctttgtaacggctgcgtaaacgtcggtgcttgagttgtcatctttctaggcactctgatttctcaagagtgcctaaaaagggtgggactaagcccaaggttgcttctgaaacgacgtcctatggagagttggtttttctgaccatctccgacatgaatcggtgagcctctaatcctaaaaacaaaactacacagtcaagactgtgtagttttgcttttctatgcaatccctacacccgaggcgaggctgggaatgcacgactgctc

SEQ ID NO: 8415 - RNA, 23199 nt, Homo sapiens
  source 1..23199: mol_type = other RNA
aaaactgcagttacttttgccaacactgtttttcacttcaaagctatataatcctttgtcactcatttcggcacaggggattttaagggaagccactttattgatgaatgtaatgtgatgtttgctgtctgcagacaattctcttccatctttgaaccacttggctgagagttctggtgttccagtcactacacactctaatgcaaaaggatttccagtagtgacagtcatgggttcgggcttctctatgattcttgctggttctagtacagtcaagactgcagagcattctctcattccagcatcgtttttgatttggcatatatattttccagaattagatgcttctggactccccagctggagggttgcaatgttatcaatgaatgaaatcctggtattttcactctctctgatgacttcacctctatctttcagccagacaacagaaattggctggaagccctccactatggcccgtaactcaacagcatccccaataagggttgaggtgtcacttagctttttcacgaatcgtggaggttctttgaacttgacagagcaagaacacgtgtcacttcccacctcattagtagctttgcagtgatattccccgacatcggaggcttcaagattaaggatatgaagacttgtatcaaaatgttttgaagtgattttaaatttcttgctgtttctaacctgctttcgatctttaacccatactacttcaaatgggggagttcccgaaatttcacattggagaatcacatcagaacctttaagagctcctactggagaaggcttctgggtgaaaacaggaggtgctttcactgtcaacgctgtgctgcagctggcgtcaccaacaccattatgagcctcacaaatgtagtccccgctgtcttcagcactagcttcattgatcgtaagcaatgccacagaattaatgaatgacatgttgtatttccaactttcatgaagttcgctgtcatttcggaaccatgaaactttgatttctggggagccacttattttacattccagttgaatggattctccctgctttgcaacttttgaagcttctaatttcttaacaaactttggaggttcttttacactgagctgagctgagcacatgtctttgccaacatcattggttgcttggcaagtatattgaccagagtctcctttgcctactttaagaattctcaaatgaggagtgtttcccacacatgtgattgtatagtttcctccaggacggatctccttgttatcttttgaccaagtgattcgcatcggttgagcaccagtaacatgacactcaaaatcagcactttctccagcaataacatctatagatacaggcttgatgtcaaagaagggagatttcttgggttctcttgctgtgagtctagcactagaagatgctgttccaagtgggttggaagctgagcaagagtactggccagagtgactcaagtcagtttgcaaaatttttaaagttgccacattatctacaaatgaagtctgtagattttcatcgtctcttaaaagtactccatctctataccagcacacttggatgggtgcagagccatttaatcgacaagtgagtgtaacaggtaaccccacagtttgttcaatgtcctttaattgtcttgcaaaagaaggtgggagttggcgctcttgaattctgaacacagtcttagaagaagcagttcctatactattttctgctttgcatgtgtactctccactgtcattgatgttcactttattaaaaacaagtgtggccacattgtttgtaaagtaggtcctgtattcaggagttggccgtaatttggtatctcctttgtaccaagacactgtaatttctggtgtcccagcaacttggcattgtaaagaaaccgaatctccaactgctgcctccagaggttccagttccgtaacaaaataaggcggttctaatgtagataccagagctccacaaacatcccttcctgcctcattttcaatctcgcaggaatactgccctgcatctctttttgtgctattcagaatttccaggatacaagttttctctgttgtgactatgttacatttttcagaggtagttatgttaaaaccatcctttttccaagtgacagaaattggaagtgttccagtgtaggtgctctccagaattatggacttccctggttctacagaatgatcacttaatctcttcaaaaatgcagctggttctttcacaaagagacgggtagtgcaagatgcttggccagcgttgttagaaaccacacaggtgtattccccactctgagatatgtcaatattaaataattccagttctgccacagtgtcttcaaaatagatgttgcaccggtctcctttcactagttctctggcacctctgaaccagttgactttgaatggaggggttcctctaataacgcttgtgaaggttacatttttgcctggtagtacttccaaaggttcaggttctttcacaaaagagggtggttcttgtacagttagcactgcacgacattcatcagacccagcgacattagcagccacgcatgtgtaattgcccatatctgaggaatccagagaattcaactgcaatgtgcagacattatctgaaaatgtggtttggtactttgctccactgacaatcttggttttctcatgaaaccaggcaactgaaataggtgatgatccagctactttgcattccaagatgcaagaagcacctaacaccccaccagtatttttcagtcttcgtgtgaaagagggaggaactgctcggtctgaaacatcaaccacagctgtgcagctgcttttcccaacattattttgaacctggaaagtgtatgtgcctgcatcttgcctttcaactgagagaatccttaaggaagagattttgttgtagaagctaaatttgtgtttttggctgctggtcaacagctttccatccttgtaccattcaacagagagttccggagtgccagccaccttacactccagagtgcacgtttctcctacagtcaccgtcatcggtcctgccttctcaacaatgactgcgggctctaagaccatcagtgtggccatgttctccctcattccaccatcattcttgatttggcagatatactttccagcattagctggctctgcttttgcaaactgtagagttgcaacattttccacaaatgtaatcctgatgttttcactttctctaatcacttcttccttctctttaagccactggacaaaaataggctgggcgccttctatggatgcttgtaattcagcaggctctccggctacaacagtgaggctgttcagtttggagacaaatcttggtggttctttcaattttacagtacaaacacaagtatcacttcccacttcattctgtgctttgcagtggtattcaccgatgtctgaagtgtccacattgagaatgtgaatacttgtgtggaagtttttggatgcaatcttgtatttcttgctgcttctgagttgccgcttgtctttgtaccataccacctcaaacggtggtgttcccgaaagttcacattcaagactgacttcagcatttttaagggtttctactataggagggaagctgctaaaaacaggtggctcttttactataaccttggtactgcagcttgtgctgccagcgggattctgagcctcacaaatgaaatctccactgtcctcagtactgagattgttcatctgtatgacggccactgagtcaatgaaagtcattctgtacttatcactggctggaagttcatgttcatttcggaaccacacaactctgatttctggggatccagctatcttgcattcaagtcgtgaagagtcacctgctttcacaattttggaggcttctaatttctttacaaactttggtggttctgtcacaagcaacatcgtagtacaagagtcgctaccaacatcattggtaacatggcaagtatactgtccagtcttagaagcatccactgagtagagatttaagaagctagtcgacccttccaagccaatgaaacatttaggacctgagacaagttccacatcatccttaaaccattttattttaaatggtggtgttccttttagtattgccttaaattccactgtagaatcaggtatggcttgctgtcgcccaggtttcactaggaagcttggtggttctttcacagttaagatgccactgcatgcatcatctcctgctacatttgacactttgcatgtgtaatttgcagtatcttctaattccagattattaacttccagagacacagatctctcatggcacacaagtctgtattttgcacttgtagatatttcttttccatccttaaaccactgagcactaatgggaagtgaaccagacaccttgcactccatatgaatagaagagcccagaactttatccattttggttaattttttggtgaatgatggaggaatattttgatctagcactcttaagtaggcatcacagctactgcttccgaagtcattttccaccttgaaagtgtactgaccgctgtcctgcttcattactgactgaattctaaaactggccacgttattttcaaaactcattgaaaagtatctactgggaactatttgtttcccgtctttaagccatttcactttgagttctggtgttccagccacaacacattccaaggtcatgggatctttctccgtaacatcaactgatttagctttctctacgatttgagctggttcttgtactaaaaggaaagcataacacctctcaactcctgactcattcttggcttgacaggtatatctcccactgtgtccattatccacacttctgatttgaagtgtggccacactgtccacaaatgaaatatagacattatcatcttcatcaagaatctgatcatcctttagccaggttatagaaataggaggagaacctgccacggtactctgaaaggtggcagaacttttcaaaacagtagtggtattttctatcttcttaatgaatgatggtggttctttcagggcaactctagtactgcatgagcagctgccgccttcattggatacaatgcactggtattccccagtgtctgaagggtcacacttggttatatggaggttaaacacagacactctgtcggtcaatgtgtattttttgctgcttcgaatttccctgttattcttcagccaagtgacttcaaacggaggtgttcccgtaacttcacactccagctccacgtcactatattttactacctccacaggcttcagctctctgataaaggtggggggttctttcactttgagttcaatgctgcagctcgccgtgcctgcgtcatttcgagcttcacacacataagtcccactattttctaccctggcaccagaaatctggaaagtggctaaaccatcaatgaaggaaatgccatgtttctgaatggctgttatttcattcccgtctagataccaagacactcggattttaggagtgcctgttatttggcattcaaatgttgttgactgtccattcctcagcactaagactggactgggcttcttaatgaattgaggaggttcttttacaaagagagtggctttgctggttgctgtgccaacatcattgcttagttggcaaatgtaggttccagaatcggtagctttggctgcaaagagctctagactggtagaggtgtcatccttccaaactgagcgggctgctcctgagtgtaactctttgttatctttaaaccactttattgtcatgggtgcagtgccacccacaagagcctttaactgtacccttgtgttgggattgacatcttgtgactgtggcttttccacaaagtaagggggttctttgactgtcagatgcccactgcattggttgtgccctgccttatttgtggcagaacaagtgtatgtcccactgtctgtaccttccagctggctgatttccaagaaggcagtattgtcatgaaaagagaatttgtacttttcactagctgatatttcttggtcatctttgaaccactggatgcttatgggatgtgacccagccactatacattctaaatcaatgaaagaacctttaatgctgtccattttcttcagctttttggtgaatgaaggaggtatgataagatctaatacattaattctagccttgcagctgctcctcccaacatcattttggacctcgaaagtatattctccactatctttcttttctgtagaaataatcttcagtattgagactgtatcagtgacactgattttatattttgagcccagggtcagttcttggccatctttaaaccatttggctgtaatctccttagtccctgaaaatttaacctgcaaagtggctgggtctccttgggtgacatctatagacacagcttcctcggtgattgttgcaggttcttttactgagagtaatgcagaacatctttgtattcctgcatcatttttggcctgacagacatatttcccatcatgcttgacttcaatgccactgaggtacaaactggccacattgttctcaaaggtcattcttatattatcgtcttcagtgatttcatcgctgtcttttagccaagtcaccgtaattggcaaggagcccttcagagtggcctggaaggcagctgtgcctccccggagggagctggtactctcgatcttctttatgaaggatgggggttctcttaaagtcaccctggcactgcagatgctgctgcccacctcattggtcacccgacactggtattcgccagcatctgcagctacaaacttgaggatctgcaggctaaccagatgatcctgaatgaaagtcttatactttctaccacttcgcaggattgtgttatctttgaaccaagtgatctcaaagggaggagtgcctgccacctcagccagcaacatgacatcgtactcctttaagacttcaattggcttaaattccttggtaaaataaggtgactctttgactattacaatgctactgcagtggtcactgccagcctcattttgggcctcacacatatattcaccactgtcttcgatgccaacatctgtcagtcttagaactgcagtagactccacaaaagacattctgtgtttgctgctctccttaatttctctatcatttgcaaaccatgttattttaattggaggggtaccagttactttgcaggctagctgggtggcatctcccttctttaacagctgtgatggctctaacttttcaacaaatgtggcaggttcttttacaaacaagtttgcactgcattccacccctccagcgacattgctgactttacatgtgtacgtgcccgaatcagaggtttttactaaatagagttccagggaactctctaaagcttctttggtaatatagcagcttccaccagaaaccagctctttgttgcccttaaaccatctgattgtgagaggagtagatccttggaaagtgctcttcaggcagactgctgagccaggcagaacatcctttgagccgggtttagttacaaaactgggtggttcttgcacaatcagggctccactgctgtctttgcttcccacggaatttgtggctcgacaagtgaaattccctgcatcattcatgtctactctgatgatctccaaagaggctgtgccttccacaaatgctatcctgtatctgtcagaagcagctatttctttgccatccttaaaccaggacaccctcatggggagggagcctgcaattttgcagtccagtctgcaggtaccattaacaacactatccacgttgcgcaagggtttggtaaaaaatggagcaatgtctcgatctaatacagtgaatgtagtctcacaggagctgctgcccacttcattggaaatctcaaatgtgtattggccactgtcgtgcagctcagctgaataaaatttgagctgggcaacattgtttttaaaacttattcggtattttttactggcgaccaagggtctcccatctttgtaccatttgggcttcagttctggcgtgcctgccactgtgtactccagtgtggcgggatctcctgctgtcacctggatcagttctgctcgctcaatgattttggcaggttctttaactattaattccccaacagatgtttggcttccagcttcattttcagccaggcacgtgtatttgcctccaaaactaatctgaacatcagggattatcaagactgcaacaccattggaaaagctcattttgatttttccgtcttctctgatgacctcttgacctttcatccatgtgacagaaatgggctctgaccctctcacagcagcttgcagggtaacggtttgtcctcctagtgcaatcaaatcatctactttctttacaaaggttggaggttctttgagtaagtgggttgccatgcagccacacttgccgacttcattagcaacaacacattcatattcaccaacatctgcactattaaacgaaaagatctccagacacacaagagacttctgagaaaacaatctgtattttttactacttcgaatttgtttcttgtctttgaaccagctaatttcaaatggtccagtgcctgagacttcacactgaagtagagcatttgttcctctcactatgtctgcaggctcaagagttttgatgaaagaaggaggttctttgataactatttcagtactgcagctatcactgccgacgtcattcactgcttcacatgagtaactcccactgtcttcaacttttacatccgtaatatcaagtatagcctcagaattgacaaaatacattcggactgtgttactttcactgagttctttgttatttttaaaccaagtaacctggatcacaggtgagcctttcagcttgcaatggaggcgtgctgattcacctgggagcattaaataagagggatccaccttcttcacgaaggatggtggctctctgacagtgactgtggctgagcaggagctgcttccagcctcatttgaagctgtacagacataggttcctgaatctttcagtttggccaaaggaatctcaagtgttgctattttatcttcaaaacagatcttataatctttccctggggggagtttttgcccatctttgctccacgtaactgtgacttttctgtcttcatctacttggcactcaaggtggaccttcttattgatagcggactgcacaggctctaattctttaatgaaatgtggcttatcaatgatgatcaactctgcttggcagatgtctgctccaaacttgttggaagccttacaagaataaactcctctatcttgaatggtaaggtttgagagttctaaaatgtgtttgttttctgcgtcggaaatcctccagttaggtgaaggtgagagtgcagcaccatctttctgccaaatggtttctatcacaggagtccctgtcactgtgcagatgaacttggctgccttacccacaaaagttgtaagggacttaggtctggagagaaaggttggtggatatgcctctgtcacagttagtgtggctgtacagctgacactgccatactcattggaagctttgcatgtatactcgccgcagtcaaccacctgggttctcaggatttcaaggctggagatatactttgaagatcgaatagaacacttgtcactctcataaatttctcggccagctttaaaccactggaaccggacattgggagcactttggatctcacaggtgaatttggctaggtggcccagtgctacttccaggggttcgattttcctcttgatcactggggcagctctttttactacagtgagtttggctgaagttgctgtttttccgctgtcattcaaggcctcacagacatactctccttgatggtcttcggtatttactttgtcgatgactagcgtatatgtattttgatcttgtaaacacttgaacttttcatctgaaggcaccagtttattctcaaaataccaattcacctctttagcatttgttatggatgttgtgaggtgtacaatatcaccttcctcagaaacagtgtccactaaaggtgtatgtatcatggggccatcctctttgattaagccaccctcagcttcctgtatctttactgtagcaacctcctcagtaccactttcagaggaagactcctctttttcctctgatggtttcagactctcatcttgtttttcgtcagagacaacagctgaagcaacccctttagtgacaggtgtggcatccaaatatttaaccctactttgcacgttaaaataactgacctcttcagttgagatcagatatttagattcaacttctggttcagtaatgggttcaaccttctgtgaacctgaaaaagaatccatttcttcttgcaaacttgttttggctccttgctgaattctaggaccctcagctgttaggatgtctatttcctcatatataatagcacacaaagcatccctaagttccattttcaggttagccatttgaggatcaacatcttcaataatgatggttacttcttctgttacagactttgccgaagtaacaaggtacatgcacatgatgtgtctgggctcttgggtgatgtttacagcctcgacctccaccttttcaatatttcttagccactcagagaaaagacctggctgctcgctggccacggctgcttgcaaagcccggcagatttgaattttcaggtttaatctctgctcttctggaataccagaaagcaagctttccttagaaagaaggtcccttccctgtacctcctgcactttctttattgccacgggctctcttttagactcaatgatttggtctgggggcatcaccacgttgtcagaatgctcttctttgagcagtacctgcttttcttcaagtgctagtggaaatcttaaggacttgccttcctcaattctgaccgcagaatcttgccctgcattttccagtggatttgcactttctatcaaaattttacctccttctgtgcatgagtgttctgaagggactaggggctcatagtttacctgagagatcatgacatcaggactctggagactctccacgtgtccctcagctaagctctgactcaagatgagcgcactttgtgcctcttgcttttgaagagtcactctttgctctctgttggtgtcagatactgtcttttcttttggtgaaagtacttcctcagccacagaggttagataagaatgcattggaggttctattgaagactgtggataattcccttcaggttcagctaataaagttttcagaggctcaactgttaatgaattaatttgttctatggacatggcacttgggaagattttctcggtatctgatagaactgcctgtgtctcaggctcttcaggcattagaataccttctttggagaaggttttctgggactgtacaatctgcagctgtaggttgggagatggttccttgagaggctgaaagtgaatactgccattgatgcaaagaaattccctggtgctttcaggagtgagcttgtcttgctccaaaatggattgcaattcctgagctcccaaaggaagctgactgctcaattcattggctttagcaatatgctcataagatagttgctggttttcttctgtaattaaagcagctttcaaaatggtgtcttttacaaacgttgcaatttcctgctctgagtcaagtgcttcaactgcgggaccctttaagggtgtctgtggaaaatcctcaggagcctctggtgtggactttgctttgcagggggtatcagtcatgtctgtgtcttccagaagcacaagcagctctgctgcacaggtggactcacccaacatattctctgctttacagatatagaggccactgtcttccctctgagggtcattgacaatgaaagttccagagccattagggttatgaatgatagtgtaataaacactggtgcaaagctgcttgttttctttgaaccatgtaacagtaggggcaggctctccaaccactgtgtactcaaagatggcaggaagcccttgagcacagcgaattggttttaactccttaaggaagtgaggaggacaaggacctcccagcttttccagagattttgccactgctgattctgtttcagtgtctttgtgaccctctcctttggaattaatttttagataggcactacatattgtctttccatagtcattactggccatacatgtatactctccctcatcctccaatttggtgaacagaatgatcaggctatgatcatcaccgtcaaaaacaaatttgtagtcagcagaaggggttaatagcactccattaaagaaccactgaattttaggtttggggatgccaatgacagttacagacagtgtagccacatcccccatgcttatatcagcatttgacacttctttgatgaaaattgggccagtgccttccttttcggaatcaaatttagttgggtaaactggagattcagacaaaagttcaagtgtttcatttattttagataattgaagttcggcgctatgaagtccttcttcctcggcagacagaaaagaactagaaaactctttcatttccatctcaatctcttgttcaatcctctcatgcaaaattgattcaggagcttccagactcaggttggctgtgcttgatacttggcctacagcattactagcaacaaacgtgtaagttccttcatcttctggataagcttcggcaatttccagttgataagtgtcttcaaattgagtcattctaaagaaccgagatggcttgattttcttgtctttgctgtaccacgacacttttagatctgttccagaaacccggcattgaaaacgggctggctgcccttcagaagtgacagtgtcctgaagcggggtgatgatggcaggtggataaacaggcatttcctgatcaggagacacaacttctggaacttccactgagagtgaagctgatgttgtggcaacaccatagtcattcttggcttcacaggtatagactgccgcatcctctgggaaggcttcaattagcaaaagcgtgtattcttgcccatcatgaagaaatttgcacttgaagccagtggaaagcagctgctcttccttgtaccaggaaattttgggctgtggtcttccggatatcacggcacagaagcgggcaggcttgccagactgcacagtgacaggctggagctcctgcagaacttggggcggttcaggagcattgacatagagagtgacagaactcctgttccttcctgccacaaaggtgtattctcctgcatcgctctgtctggtctcagagataaacattcggtggattcttctttccactacatatttgtgtcgttcttgaacttggaaattgatttcaatgccatctttataccagtgggcatcaacatcgtcttcattgacctcaaattcaacaacagcacgctgtttctcaatgacctgaacctcctttttaatacttcggatgcgaacatctctgccttctacaaagagttttgcagttgacacgttgcctcctgccaccactgtgtacttcccagcatcagacatccgggtggatgggatcagaaggcggtggacatatttctccttctgaatctttattctgtctgtgatctgcagttcctggtcatctttcatccactgtacagtgatgtcaggttcagaaacttcacattcaaacatggctcgcttcttctccagtaccttaatgtccttaatgtgtttcctaaattctatatgacgagcttccacataaagtgtggctgttgatgttgcttttccagccacaaaggtgtagtcagcagcatccccaaagtgaacattcctgatgttcagtgagtgtgtgagctttttggttctcatctggcacttgtcagttgatttgatttccacaccattctttaaccatttgtaagagatgccttcatagttcactgtcacctcaaaagtaatagtgtctttttcttcagcgttgatgtctttcagcatggaagtaatcatgattggggtgactgtcagggtggcactgacttggtcattgccacagacaaatgtgtattctgccgagtcctctgtgctggtgttcatgatgatcagctgatggagttttccctgcacaactatcttgaacttttcactcatctcaatttccacaccattcttcagccacatggaagggacattgaagtgggacacctcacactcaaaagaggcagttttggtctcaggcacctcgatatttttcatggtttttgtaatatgtaatgtctccacaaacagttttgctttgcattccaattgcccgaccacagctgtgtattccccagcatctgagggggagatgttctgcagcatcagcttgtggactttcctttctgagaccagtctgtgtttgtcacttggcttaatttccacactcttatggaaccattttactggaacagtgtcatgggaaacactaacttcaaaggcaacagtggcattttccaaggctgtcacatcctttggctttttaatgatcttgacagtctccacgtgcagtctggcactggctccaagccttccaagcctgaagccataaacagactcatccacgatggcacagtttttaatcctcagagagtaaattgttcctttgacagagatagcatacttttcattggattccagcacaactccatttttgatccactggacacctttgacattagggtgtgtaagctcgacagtgaaaacagcatcctgtgtttctgtcactgtgaggttcttcagagtcttcttaattttgacagcttcaactttgagtttggcagatgttttggaggtggccaccttgtaggtatattctccaatgtcatctaatttggtggcagcaatgataagtctccttttgtggccatcagactcacttctgatgttgttagtcagtggtaggtgtttgccatccctcaaccattcgcctttggaatctgggttggcaacttcacattcaaacacagcttcctgggattcagctacggtctgatctgtgagtggcttggagatggccccacctgccacagtaagttttccagatgtcatattttctcccgcgtaaaatgtgtattttccttcatcatctttcatcatatttagaactgtcaatttatatatttttccatgtgcttcaattttatatttagaactgggcttgatttccttgtccttaaaattccacaggacatcaattccagagtgggacagctcaacctcaaacaccacattttgagtttctgtacaggtaaggtcacgaagacctctgataattttaattttttctacagagagattacagttggtttcaactctgccaactatcagcttgtaaggtccttcgtctgaagcatgagttcggttaatgactagtcgctgtttagtacctttcacaatggcctgtacacggtcatcaggcttgatttgttcatcatttaagtaccacttaacagaagtcacatcagggactgacaccttacattcaagcacagccttggtgccttcaatcacattaacatcttttagaggtgttatcacgtccacactatagacagagacacgcccactggtggagaggccaagggctggaatggtgaaagagtaatttccagcatcttccttagtcatgtcttcaatgagcagcatatgagattgtttgtctatcacaatgtgaaccctgtcactgggctgcacttcttggccgtctttcatccagacgccttccacactttccaaggagactttaacttcaagctgaacaatgtcaccctcacagactttttggtcactaagtccttgtaggatagcaatggggcggggtttcatctttaatttacaggttgtctttttcccgtcgatgacaaagctgtattctccctggtcctccttggttacatccttgaccgtgaggttctgacgtccacgacgagatgtaattgtatatttgccattggatttaagctccacatcattatgataccattttccttctatattttctggggatacaatgcactctaattctcctgaatatgattctggaacttctatgtcctgaagttctttcacaaactcaacaactgcaccttcaacaataagtttagcagtcgttttgacattttcatcttccacaagtacacagctgtaatcttcagcatcagacgtatcaatggtcagtatggagaggaagtgaacctttctgtcagagtgcatcctgtatttatctccctcatgaacctccataccatctttataccatttcactttgacaaatggttctgaagtttcacattcaaaggttgccatagtgtctttttccttagcaacaacatcttgtaattcctgtgtgaaagtgatcaattgcttggcttggacaagtaagaatgcgtgactggaggtttctccagctatgttgatggcttttaccatgatgctggcagagtcctcagcagtcacatctcttatgaccaattcacaaacattgtcttcgggccagtaccagtagatccggtcagaccgttcaattttgacaccatttttgtaccattcacattcggggtctggtttccccacgactctgacccggaagtgtgcatcagatccttggcccactgtttggctctggattctttcgaagatttttggagcctccatactaggacttagttcaatcttgtcaggtttaaaagttggaatcgtgattttgccttcttcggcaagagctttcttttcctcttcagttaactctttggtccagtggagaagttcatcttttgtcttcctgaggagttcctcataggattcatccttctttcgagacttgagctccacagcggtaatggcttcataatagccctcttctgttctgcgcttgaatttactgcgcagctcttccgactcttcaggcactttttcatgggtaattctttcagcccttttcaacttcacaacttctttggtttcagtggtgtcaacaggtctatccactttttgtacttcaaactgaagctttcctggttcatgtacgtgaaactcaggccttggttcaggagctctcctaaggacagacctaaaatcttccctctgttgaatctcaagcttcactttatgctctatcacaccttcaggattttccgcggtgaccttcacttcacctgtgtcatatgatttgcagtccacgatgtccaggtaatggataccatcatagcgaactctgaaccttttgcttttgcggatgagctgtccattgaggtaccagttgactttgggctgagggtagcctgttaccctgcagcggaaccttgcagtctccccttcaagtactctaactggctctgggtacaagacaatgtctggcttttgcttttctttctgatctgttgttacacctgtaagtgcaccttcatgagccattctctctaattcttcaattctctgtaagcctttcctcccctcaggcaattgggattcttccacaagacttttctcatctttaacaataagggtagcagatgtgtgatctgttccatatttgttagtggctctgcaagtaatgataccactgtctctagaatatgcaacgccataatcaaggctgcagtacccaaattcattgatcatacggagcctgttggctgcttcaagtggctttccatcatggagccactccaccaccatcgttgggtcaccaatgggtgttagcctgcattcaaagtgggcaggcccaaagcgcttaagtcttaaggaagtgagttttttcttgaaaaatggtttctgttgtttctctttgtcatagagatcaccttcttcccattgctcttggccatatcgcaaatggaggggctccagttctggggctgcaatctcctttgctctatatgtcccccgtgggatgattaactttctctctggctcaggctctgcaaactcaacttcaacatttactttgcatcttgtagtgtctctgccagctttattaatagcagtcgcagtataccaggcagaatcttggctgacagtggaatcgattttaagggcagcttctcccttggttccttcaattctgattttgggatatttatgaggcacaatgatgtcactgtttttcaaccatacaatgtcagggttggggttacccgtagctctgactttcatttcaagtcgggaaccttcctttatattgacatttttcagtttttctacaaacatcggttttacctgatgttccacagcttccacagttaaaatcactgaaattgaagatctgcctgccctgttttgggcaaccacagtccattccccagaatcactgggtgtggcagggacaataattagtgattgagtaccatcttctttaatgactactttatgggtatagtcattgacaatttgctggccatcatgaaaccagaacgtctctggcataggtctaccaacaacctttaagtcaaatctggcagtttgcccttctaaacatttgaaagaaacaggttttaacacaaagactggtttatatagtctctcaagttgtgactcatctgtctcctccagcctacgtccaggggacattcttgcaggggacatccgtgcaggagacatccttgcaggtgacatccgtgcaggagacatgcgtataggagacctgctcactgaacgtggagagagagatctgattctgctcactggctctagtgtgggaatgtaagtcggagctccaagtggtgcagcaggctccacatacaatttccctgagcaaattgcatttcctttaatattgctggcaaatgcagtgtagattccttcatcttctggaagaacaacaggtatacgcagactagctctgccatcttgtagaaagtccatttggtatctttctccatgtttgatgcgcttgccatctttgtaccaagcaatctttggtaatggatatccagacatcttgcaatgaaaagtgacacccatcccctcaagaattctataattcttgattcttgaatcaaatcctgattcaacagcttcagattcagaaatgtcaactgccatcttttcttctccatcttcttcaagaagttcttctaatgtagtctttattattctatattcaatttctttaataagtctctcttcaaaggaagaaatatggaattcctgatcttctacataagttctgaccactacagtatctttggccattttcttcctaattaaggcttgttctttttcatactctttttcatactcagagtatacaaatccaggtgctgtttctccaactttaggttcttgaacaaatgcagtcacttgtgtctgataaagcatttcttgctgggacttcatcagtaactcataatcagcttcttcaagcaaggaagcagatgcagaagtttctccatgcttattgcgaacaacaatagtgtattctccagcatcatcagcaaaagtcatagaaatcaccagcttgcattcaccggtttgtttgttgtaactcactttgtatctgtatccagtggttagaggaacaccagattttttccagtatacatggggctttgggttgccgccaacttggcatccaaacaccacgctcccaccttccaccagtttctggaccactggttttgtaataaagtaaggcgcggcaggttctccaggccctgcttgttcctctgtgaggctagtatcagtcataaccacatctcttgactcaacaaagcgtttctcttctgtagtaaatttctcagtcacggctgtggtttccttttcaaattcttctgacacctgcacagccagatagcaggatgtgctgacggttccagcctcatttacagcactgcaagtaaatcgcccgctgtcttccgcaaatgcttcgcgaatcataagacgagcaattccactctggaaggttatctggaagtcaatggaactttcgatttggtagtcttccctgtaccatgtcactgtcggggatgggtatccagagatgtggcactccaaggtgacagattcaccttctatgacagtcacattttttaagcccgagaccaaagttggtggagtaacaggaatttcaacaggtgctggtactcttgctgtttctgttaccttggcttcgcgtccgtgcagtacttcaaagcgctcttcacggacggtggtgccagtgatgctcacccctacttcctttttcacctcaacgccagcttcactcttgtaagtatctggtgtgtcagcgaaggggaactgtggcaagggtgtgggctctgcccttactctagtctcactgggcttcacagtaggagccttcaccgatttggtgatcttctgagcagaagatgtggctgacaactctttttgtaatgtggcaatagcactaccggctattgatgcctcatatccatgttctgtcttaggaacagaaatttttgaaacagtaaagtgagggctagctgtgcgggggcgtttatccacatggactaatctttccgttgttagatctgtagttttcttgatctgtgatgatatgtgcattcccttttgatcagtagttttgatatgagtctcagaaggagcctggattactctaggcttgactgctttagggacaacgtggggttctgaggctggacgttggggaggctcagctacctttgcggcggaaatgcgttccttatatccgtactccaaagtggtctgctgagcataggattcttcaagatgcccaggctctctgggctctctgactcgggcctggtctactgcagcaacaactgttgctacagcttcagccttttttccaacgtccacctttccatgggtaacttggatttgttcttgtctagtagccatagtttctctagttctcagtattgtttcttgttctttggctttagcagtagcaactgctattgtagacaaggcagttttctcggcttcctttctcatcttctcctgagttatttgcacttgttctcttttggtagtaatgccttctctacctcttgatactaaatcttgttctttgactttgggtgtggcaactatgactttaggtacaactgttttcctagtttccttcattatcttttcataacttaggtgcatttgatcttgttgtgtggtagtttcttcttgagctcccgggactgtttctagttttgtggactttgcagtggcaactaccaccatggatgcagcagttatctcagtttcctgtcttattgcttcttgagttacttgtttctgtttcttagtaatttcttcagaaattctagtttcttgttctttggctttagctgcggaaattactacctttggtacaaatgttttttcagtttcttttcttatctgctcatgagttacgtgcatctgctcttgctttgtggtaattacttctttggttcttgattttaattcttgttccttggctttatcggcggccactactaccttagttacagcagtcttctccgcttcctttcttacctgctgttcttgagcaggttggatgtgcacagcagtcgtggttgtcctctgagcagtctgctctacagcgctgatcactggttctctcactctggccatatcaacggcagcaacaacagtcgcaacagctgcacttttgtcagcatcttgtttcacctctttagcaccagtggcaacagcctctgctgcgtagctagcactggccgacacactggcggcagcacccgcagcaccactgatggtcacttgctcctggacaccgtatctcccttcccatctctcttctgtcctgatctgagtagaggttgtcagcgttgtctctctcatctcagcctcagatgaggaggccacgtagccctcttgcttccaagggggaggcacttcaggacctgtggccacggtggatgcctgagtcttacgcatgagcaatggagacctaacagacctgatgggggatgtggagattcttgctgctggagacacggacctgaccggagatggggtcggtgcccgcacgtgtctgaccggggaaggggagtgtcttatgggcgatggggactgctgccgagccagctgtgctttggcagcaatagacggtggtgttggggatcttgactttggcttcggaggaatcctgggaggtgttttatgtggcagctgttgcccagcggcaccatctatgaccatctcaactgttgcaattgatctggcatcaaagtgggcttcaatcttcttttcaattcgggtttgtcttgattctgagatctgagcagtcgaaacaattgtctttgtctttttagcaggtacttcttcttcaccttgaaccagtaattcagcagtcgaagtagctcttccaacgctattggtggcatttactgaataggtccctgagtcctcagggtatgcttctgcaatcagtaagctgtagaggtcgccttcttgtgaaatttggaaatcaagggagctctggatttcggctccatcccggtagaacttcaccacaggtgtagggattccagtcactctcacttggagtctcacttggcttccttgtctcacggtcatgctctgcagtcgttgaacgaagttgggtggtgctgtctcagctttcacgagaagctcagcagtactagtcgcttgtccagatccattggtggctttcagggaatatcgtccactgttggctttagtcacggcggggatcgtcagtttagcgcggccatcgctaaaggagatctgcacgccgggcagagtggaagtggaaatcacctggccatccctaaaccagctcacctcaggaactggaaaaccactaatgtgagcctcaaaggttgcggtactaccctccagtaccacaacgctttgtaacggctgcgtaaacgtcggtgcttgagttgtcatctttctaggcactctgatttctcaagagtgcctaaaaagggtgggactaagcccaaggttgcttctgaaacgacgtcctatggagagttggtttttctgaccatctccgacatgaatcggtgagcctctaatcctaaaaacaaaactacacagtcaagactgtgtagttttgcttttctatgcaatccctacacccgaggcgaggctgggaatgcacgactgctc

SEQ ID NO: 8416 - RNA, 23196 nt, Homo sapiens
  source 1..23196: mol_type = other RNA
aaaactgcagttacttttgccaacactgtttttcacttcaaagctatataatcctttgtcactcatttcggcacaggggattttaagggaagccactttattgatgaatgtaatgtgatgtttgctgtctgcagacaattctcttccatctttgaaccacttggctgagagttctggtgttccagtcactacacactctaatgcaaaaggatttccagtagtgacagtcatgggttcgggcttctctatgattcttgctggttctagtacagtcaagactgcagagcattctctcattccagcatcgtttttgatttggcatatatattttccagaattagatgcttctggactccccagctggagggttgcaatgttatcaatgaatgaaatcctggtattttcactctctctgatgacttcacctctatctttcagccagacaacagaaattggctggaagccctccactatggcccgtaactcaacagcatccccaataagggttgaggtgtcacttagctttttcacgaatcgtggaggttctttgaacttgacagagcaagaacacgtgtcacttcccacctcattagtagctttgcagtgatattccccgacatcggaggcttcaagattaaggatatgaagacttgtatcaaaatgttttgaagtgattttaaatttcttgctgtttctaacctgctttcgatctttaacccatactacttcaaatgggggagttcccgaaatttcacattggagaatcacatcagaacctttaagagctcctactggagaaggcttctgggtgaaaacaggaggtgctttcactgtcaacgctgtgctgcagctggcgtcaccaacaccattatgagcctcacaaatgtagtccccgctgtcttcagcactagcttcattgatcgtaagcaatgccacagaattaatgaatgacatgttgtatttccaactttcatgaagttcgctgtcatttcggaaccatgaaactttgatttctggggagccacttattttacattccagttgaatggattctccctgctttgcaacttttgaagcttctaatttcttaacaaactttggaggttcttttacactgagctgagctgagcacatgtctttgccaacatcattggttgcttggcaagtatattgaccagagtctcctttgcctactttaagaattctcaaatgaggagtgtttcccacacatgtgattgtatagtttcctccaggacggatctccttgttatcttttgaccaagtgattcgcatcggttgagcaccagtaacatgacactcaaaatcagcactttctccagcaataacatctatagatacaggcttgatgtcaaagaagggagatttcttgggttctcttgctgtgagtctagcactagaagatgctgttccaagtgggttggaagctgagcaagagtactggccagagtgactcaagtcagtttgcaaaatttttaaagttgccacattatctacaaatgaagtctgtagattttcatcgtctcttaaaagtactccatctctataccagcacacttggatgggtgcagagccatttaatcgacaagtgagtgtaacaggtaaccccacagtttgttcaatgtcctttaattgtcttgcaaaagaaggtgggagttggcgctcttgaattctgaacacagtcttagaagaagcagttcctatactattttctgctttgcatgtgtactctccactgtcattgatgttcactttattaaaaacaagtgtggccacattgtttgtaaagtaggtcctgtattcaggagttggccgtaatttggtatctcctttgtaccaagacactgtaatttctggtgtcccagcaacttggcattgtaaagaaaccgaatctccaactgctgcctccagaggttccagttccgtaacaaaataaggcggttctaatgtagataccagagctccacaaacatcccttcctgcctcattttcaatctcgcaggaatactgccctgcatctctttttgtgctattcagaatttccaggatacaagttttctctgttgtgactatgttacatttttcagaggtagttatgttaaaaccatcctttttccaagtgacagaaattggaagtgttccagtgtaggtgctctccagaattatggacttccctggttctacagaatgatcacttaatctcttcaaaaatgcagctggttctttcacaaagagacgggtagtgcaagatgcttggccagcgttgttagaaaccacacaggtgtattccccactctgagatatgtcaatattaaataattccagttctgccacagtgtcttcaaaatagatgttgcaccggtctcctttcactagttctctggcacctctgaaccagttgactttgaatggaggggttcctctaataacgcttgtgaaggttacatttttgcctggtagtacttccaaaggttcaggttctttcacaaaagagggtggttcttgtacagttagcactgcacgacattcatcagacccagcgacattagcagccacgcatgtgtaattgcccatatctgaggaatccagagaattcaactgcaatgtgcagacattatctgaaaatgtggtttggtactttgctccactgacaatcttggttttctcatgaaaccaggcaactgaaataggtgatgatccagctactttgcattccaagatgcaagaagcacctaacaccccaccagtatttttcagtcttcgtgtgaaagagggaggaactgctcggtctgaaacatcaaccacagctgtgcagctgcttttcccaacattattttgaacctggaaagtgtatgtgcctgcatcttgcctttcaactgagagaatccttaaggaagagattttgttgtagaagctaaatttgtgtttttggctgctggtcaacagctttccatccttgtaccattcaacagagagttccggagtgccagccaccttacactccagagtgcacgtttctcctacagtcaccgtcatcggtcctgccttctcaacaatgactgcgggctctaagaccatcagtgtggccatgttctccctcattccaccatcattcttgatttggcagatatactttccagcattagctggctctgcttttgcaaactgtagagttgcaacattttccacaaatgtaatcctgatgttttcactttctctaatcacttcttccttctctttaagccactggacaaaaataggctgggcgccttctatggatgcttgtaattcagcaggctctccggctacaacagtgaggctgttcagtttggagacaaatcttggtggttctttcaattttacagtacaaacacaagtatcacttcccacttcattctgtgctttgcagtggtattcaccgatgtctgaagtgtccacattgagaatgtgaatacttgtgtggaagtttttggatgcaatcttgtatttcttgctgcttctgagttgccgcttgtctttgtaccataccacctcaaacggtggtgttcccgaaagttcacattcaagactgacttcagcatttttaagggtttctactataggagggaagctgctaaaaacaggtggctcttttactataaccttggtactgcagcttgtgctgccagcgggattctgagcctcacaaatgaaatctccactgtcctcagtactgagattgttcatctgtatgacggccactgagtcaatgaaagtcattctgtacttatcactggctggaagttcatgttcatttcggaaccacacaactctgatttctggggatccagctatcttgcattcaagtcgtgaagagtcacctgctttcacaattttggaggcttctaatttctttacaaactttggtggttctgtcacaagcaacatcgtagtacaagagtcgctaccaacatcattggtaacatggcaagtatactgtccagtcttagaagcatccactgagtagagatttaagaagctagtcgacccttccaagccaatgaaacatttaggacctgagacaagttccacatcatccttaaaccattttattttaaatggtggtgttccttttagtattgccttaaattccactgtagaatcaggtatggcttgctgtcgcccaggtttcactaggaagcttggtggttctttcacagttaagatgccactgcatgcatcatctcctgctacatttgacactttgcatgtgtaatttgcagtatcttctaattccagattattaacttccagagacacagatctctcatggcacacaagtctgtattttgcacttgtagatatttcttttccatccttaaaccactgagcactaatgggaagtgaaccagacaccttgcactccatatgaatagaagagcccagaactttatccattttggttaattttttggtgaatgatggaggaatattttgatctagcactcttaagtaggcatcacagctactgcttccgaagtcattttccaccttgaaagtgtactgaccgctgtcctgcttcattactgactgaattctaaaactggccacgttattttcaaaactcattgaaaagtatctactgggaactatttgtttcccgtctttaagccatttcactttgagttctggtgttccagccacaacacattccaaggtcatgggatctttctccgtaacatcaactgatttagctttctctacgatttgagctggttcttgtactaaaaggaaagcataacacctctcaactcctgactcattcttggcttgacaggtatatctcccactgtgtccattatccacacttctgatttgaagtgtggccacactgtccacaaatgaaatatagacattatcatcttcatcaagaatctgatcatcctttagccaggttatagaaataggaggagaacctgccacggtactctgaaaggtggcagaacttttcaaaacagtagtggtattttctatcttcttaatgaatgatggtggttctttcagggcaactctagtactgcatgagcagctgccgccttcattggatacaatgcactggtattccccagtgtctgaagggtcacacttggttatatggaggttaaacacagacactctgtcggtcaatgtgtattttttgctgcttcgaatttccctgttattcttcagccaagtgacttcaaacggaggtgttcccgtaacttcacactccagctccacgtcactatattttactacctccacaggcttcagctctctgataaaggtggggggttctttcactttgagttcaatgctgcagctcgccgtgcctgcgtcatttcgagcttcacacacataagtcccactattttctaccctggcaccagaaatctggaaagtggctaaaccatcaatgaaggaaatgccatgtttctgaatggctgttatttcattcccgtctagataccaagacactcggattttaggagtgcctgttatttggcattcaaatgttgttgactgtccattcctcagcactaagactggactgggcttcttaatgaattgaggaggttcttttacaaagagagtggctttgctggttgctgtgccaacatcattgcttagttggcaaatgtaggttccagaatcggtagctttggctgcaaagagctctagactggtagaggtgtcatccttccaaactgagcgggctgctcctgagtgtaactctttgttatctttaaaccactttattgtcatgggtgcagtgccacccacaagagcctttaactgtacccttgtgttgggattgacatcttgtgactgtggcttttccacaaagtaagggggttctttgactgtcagatgcccactgcattggttgtgccctgccttatttgtggcagaacaagtgtatgtcccactgtctgtaccttccagctggctgatttccaagaaggcagtattgtcatgaaaagagaatttgtacttttcactagctgatatttcttggtcatctttgaaccactggatgcttatgggatgtgacccagccactatacattctaaatcaatgaaagaacctttaatgctgtccattttcttcagctttttggtgaatgaaggaggtatgataagatctaatacattaattctagccttgcagctgctcctcccaacatcattttggacctcgaaagtatattctccactatctttcttttctgtagaaataatcttcagtattgagactgtatcagtgacactgattttatattttgagcccagggtcagttcttggccatctttaaaccatttggctgtaatctccttagtccctgaaaatttaacctgcaaagtggctgggtctccttgggtgacatctatagacacagcttcctcggtgattgttgcaggttcttttactgagagtaatgcagaacatctttgtattcctgcatcatttttggcctgacagacatatttcccatcatgcttgacttcaatgccactgaggtacaaactggccacattgttctcaaaggtcattcttatattatcgtcttcagtgatttcatcgctgtcttttagccaagtcaccgtaattggcaaggagcccttcagagtggcctggaaggcagctgtgcctccccggagggagctggtactctcgatcttctttatgaaggatgggggttctcttaaagtcaccctggcactgcagatgctgctgcccacctcattggtcacccgacactggtattcgccagcatctgcagctacaaacttgaggatctgcaggctaaccagatgatcctgaatgaaagtcttatactttctaccacttcgcaggattgtgttatctttgaaccaagtgatctcaaagggaggagtgcctgccacctcagccagcaacatgacatcgtactcctttaagacttcaattggcttaaattccttggtaaaataaggtgactctttgactattacaatgctactgcagtggtcactgccagcctcattttgggcctcacacatatattcaccactgtcttcgatgccaacatctgtcagtcttagaactgcagtagactccacaaaagacattctgtgtttgctgctctccttaatttctctatcatttgcaaaccatgttattttaattggaggggtaccagttactttgcaggctagctgggtggcatctcccttctttaacagctgtgatggctctaacttttcaacaaatgtggcaggttcttttacaaacaagtttgcactgcattccacccctccagcgacattgctgactttacatgtgtacgtgcccgaatcagaggtttttactaaatagagttccagggaactctctaaagcttctttggtaatatagcagcttccaccagaaaccagctctttgttgcccttaaaccatctgattgtgagaggagtagatccttggaaagtgctcttcaggcagactgctgagccaggcagaacatcctttgagccgggtttagttacaaaactgggtggttcttgcacaatcagggctccactgctgtctttgcttcccacggaatttgtggctcgacaagtgaaattccctgcatcattcatgtctactctgatgatctccaaagaggctgtgccttccacaaatgctatcctgtatctgtcagaagcagctatttctttgccatccttaaaccaggacaccctcatggggagggagcctgcaattttgcagtccagtctgcaggtaccattaacaacactatccacgttgcgcaagggtttggtaaaaaatggagcaatgtctcgatctaatacagtgaatgtagtctcacaggagctgctgcccacttcattggaaatctcaaatgtgtattggccactgtcgtgcagctcagctgaataaaatttgagctgggcaacattgtttttaaaacttattcggtattttttactggcgaccaagggtctcccatctttgtaccatttgggcttcagttctggcgtgcctgccactgtgtactccagtgtggcgggatctcctgctgtcacctggatcagttctgctcgctcaatgattttggcaggttctttaactattaattccccaacagatgtttggcttccagcttcattttcagccaggcacgtgtatttgcctccaaaactaatctgaacatcagggattatcaagactgcaacaccattggaaaagctcattttgatttttccgtcttctctgatgacctcttgacctttcatccatgtgacagaaatgggctctgaccctctcacagcagcttgcagggtaacggtttgtcctcctagtgcaatcaaatcatctactttctttacaaaggttggaggttctttgagtaagtgggttgccatgcagccacacttgccgacttcattagcaacaacacattcatattcaccaacatctgcactattaaacgaaaagatctccagacacacaagagacttctgagaaaacaatctgtattttttactacttcgaatttgtttcttgtctttgaaccagctaatttcaaatggtccagtgcctgagacttcacactgaagtagagcatttgttcctctcactatgtctgcaggctcaagagttttgatgaaagaaggaggttctttgataactatttcagtactgcagctatcactgccgacgtcattcactgcttcacatgagtaactcccactgtcttcaacttttacatccgtaatatcaagtatagcctcagaattgacaaaatacattcggactgtgttactttcactgagttctttgttatttttaaaccaagtaacctggatcacaggtgagcctttcagcttgcaatggaggcgtgctgattcacctgggagcattaaataagagggatccaccttcttcacgaaggatggtggctctctgacagtgactgtggctgagcaggagctgcttccagcctcatttgaagctgtacagacataggttcctgaatctttcagtttggccaaaggaatctcaagtgttgctattttatcttcaaaacagatcttataatctttccctggggggagtttttgcccatctttgctccacgtaactgtgacttttctgtcttcatctacttggcactcaaggtggaccttcttattgatagcggactgcacaggctctaattctttaatgaaatgtggcttatcaatgatgatcaactctgcttggcagatgtctgctccaaacttgttggaagccttacaagaataaactcctctatcttgaatggtaaggtttgagagttctaaaatgtgtttgttttctgcgtcggaaatcctccagttaggtgaaggtgagagtgcagcaccatctttctgccaaatggtttctatcacaggagtccctgtcactgtgcagatgaacttggctgccttacccacaaaagttgtaagggacttaggtctggagagaaaggttggtggatatgcctctgtcacagttagtgtggctgtacagctgacactgccatactcattggaagctttgcatgtatactcgccgcagtcaaccacctgggttctcaggatttcaaggctggagatatactttgaagatcgaatagaacacttgtcactctcataaatttctcggccagctttaaaccactggaaccggacattgggagcactttggatctcacaggtgaatttggctaggtggcccagtgctacttccaggggttcgattttcctcttgatcactggggcagctctttttactacagtgagtttggctgaagttgctgtttttccgctgtcattcaaggcctcacagacatactctccttgatggtcttcggtatttactttgtcgatgactagcgtatatgtattttgatcttgtaaacacttgaacttttcatctgaaggcaccagtttattctcaaaataccaattcacctctttagcatttgttatggatgttgtgaggtgtacaatatcaccttcctcagaaacagtgtccactaaaggtgtatgtatcatggggccatcctctttgattaagccaccctcagcttcctgtatctttactgtagcaacctcctcagtaccactttcagaggaagactcctctttttcctctgatggtttcagactctcatcttgtttttcgtcagagacaacagctgaagcaacccctttagtgacaggtgtggcatccaaatatttaaccctactttgcacgttaaaataactgacctcttcagttgagatcagatatttagattcaacttctggttcagtaatgggttcaaccttctgtgaacctgaaaaagaatccatttcttcttgcaaacttgttttggctccttgctgaattctaggaccctcagctgttaggatgtctatttcctcatatataatagcacacaaagcatccctaagttccattttcaggttagccatttgaggatcaacatcttcaataatgatggttacttcttctgttacagactttgccgaagtaacaaggtacatgcacatgatgtgtctgggctcttgggtgatgtttacagcctcgacctccaccttttcaatatttcttagccactcagagaaaagacctggctgctcgctggccacggctgcttgcaaagcccggcagatttgaattttcaggtttaatctctgctcttctggaataccagaaagcaagctttccttagaaagaaggtcccttccctgtacctcctgcactttctttattgccacgggctctcttttagactcaatgatttggtctgggggcatcaccacgttgtcagaatgctcttctttgagcagtacctgcttttcttcaagtgctagtggaaatcttaaggacttgccttcctcaattctgaccgcagaatcttgccctgcattttccagtggatttgcactttctatcaaaattttacctccttctgtgcatgagtgttctgaagggactaggggctcatagtttacctgagagatcatgacatcaggactctggagactctccacgtgtccctcagctaagctctgactcaagatgagcgcactttgtgcctcttgcttttgaagagtcactctttgctctctgttggtgtcagatactgtcttttcttttggtgaaagtacttcctcagccacagaggttagataagaatgcattggaggttctattgaagactgtggataattcccttcaggttcagctaataaagttttcagaggctcaactgttaatgaattaatttgttctatggacatggcacttgggaagattttctcggtatctgatagaactgcctgtgtctcaggctcttcaggcattagaataccttctttggagaaggttttctgggactgtacaatctgcagctgtaggttgggagatggttccttgagaggctgaaagtgaatactgccattgatgcaaagaaattccctggtgctttcaggagtgagcttgtcttgctccaaaatggattgcaattcctgagctcccaaaggaagctgactgctcaattcattggctttagcaatatgctcataagatagttgctggttttcttctgtaattaaagcagctttcaaaatggtgtcttttacaaacgttgcaatttcctgctctgagtcaagtgcttcaactgcgggaccctttaagggtgtctgtggaaaatcctcaggagcctctggtgtggactttgctttgcagggggtatcagtcatgtctgtgtcttccagaagcacaagcagctctgctgcacaggtggactcacccaacatattctctgctttacagatatagaggccactgtcttccctctgagggtcattgacaatgaaagttccagagccattagggttatgaatgatagtgtaataaacactggtgcaaagctgcttgttttctttgaaccatgtaacagtaggggcaggctctccaaccactgtgtactcaaagatggcaggaagcccttgagcacagcgaattggttttaactccttaaggaagtgaggaggacaaggacctcccagcttttccagagattttgccactgctgattctgtttcagtgtctttgtgaccctctcctttggaattaatttttagataggcactacatattgtctttccatagtcattactggccatacatgtatactctccctcatcctccaatttggtgaacagaatgatcaggctatgatcatcaccgtcaaaaacaaatttgtagtcagcagaaggggttaatagcactccattaaagaaccactgaattttaggtttggggatgccaatgacagttacagacagtgtagccacatcccccatgcttatatcagcatttgacacttctttgatgaaaattgggccagtgccttccttttcggaatcaaatttagttgggtaaactggagattcagacaaaagttcaagtgtttcatttattttagataattgaagttcggcgctatgaagtccttcttcctcggcagacagaaaagaactagaaaactctttcatttccatctcaatctcttgttcaatcctctcatgcaaaattgattcaggagcttccagactcaggttggctgtgcttgatacttggcctacagcattactagcaacaaacgtgtaagttccttcatcttctggataagcttcggcaatttccagttgataagtgtcttcaaattgagtcattctaaagaaccgagatggcttgattttcttgtctttgctgtaccacgacacttttagatctgttccagaaacccggcattgaaaacgggctggctgcccttcagaagtgacagtgtcctgaagcggggtgatgatggcaggtggataaacaggcatttcctgatcaggagacacaacttctggaacttccactgagagtgaagctgatgttgtggcaacaccatagtcattcttggcttcacaggtatagactgccgcatcctctgggaaggcttcaattagcaaaagcgtgtattcttgcccatcatgaagaaatttgcacttgaagccagtggaaagcagctgctcttccttgtaccaggaaattttgggctgtggtcttccggatatcacggcacagaagcgggcaggcttgccagactgcacagtgacaggctggagctcctgcagaacttggggcggttcaggagcattgacatagagagtgacagaactcctgttccttcctgccacaaaggtgtattctcctgcatcgctctgtctggtctcagagataaacattcggtggattcttctttccactacatatttgtgtcgttcttgaacttggaaattgatttcaatgccatctttataccagtgggcatcaacatcgtcttcattgacctcaaattcaacaacagcacgctgtttctcaatgacctgaacctcctttttaatacttcggatgcgaacatctctgccttctacaaagagttttgcagttgacacgttgcctcctgccaccactgtgtacttcccagcatcagacatccgggtggatgggatcagaaggcggtggacatatttctccttctgaatctttattctgtctgtgatctgcagttcctggtcatctttcatccactgtacagtgatgtcaggttcagaaacttcacattcaaacatggctcgcttcttctccagtaccttaatgtccttaatgtgtttcctaaattctatatgacgagcttccacataaagtgtggctgttgatgttgcttttccagccacaaaggtgtagtcagcagcatccccaaagtgaacattcctgatgttcagtgagtgtgtgagctttttggttctcatctggcacttgtcagttgatttgatttccacaccattctttaaccatttgtaagagatgccttcatagttcactgtcacctcaaaagtaatagtgtctttttcttcagcgttgatgtctttcagcatggaagtaatcatgattggggtgactgtcagggtggcactgacttggtcattgccacagacaaatgtgtattctgccgagtcctctgtgctggtgttcatgatgatcagctgatggagttttccctgcacaactatcttgaacttttcactcatctcaatttccacaccattcttcagccacatggaagggacattgaagtgggacacctcacactcaaaagaggcagttttggtctcaggcacctcgatatttttcatggtttttgtaatatgtaatgtctccacaaacagttttgctttgcattccaattgcccgaccacagctgtgtattccccagcatctgagggggagatgttctgcagcatcagcttgtggactttcctttctgagaccagtctgtgtttgtcacttggcttaatttccacactcttatggaaccattttactggaacagtgtcatgggaaacactaacttcaaaggcaacagtggcattttccaaggctgtcacatcctttggctttttaatgatcttgacagtctccacgtgcagtctggcactggctccaagccttccaagcctgaagccataaacagactcatccacgatggcacagtttttaatcctcagagagtaaattgttcctttgacagagatagcatacttttcattggattccagcacaactccatttttgatccactggacacctttgacattagggtgtgtaagctcgacagtgaaaacagcatcctgtgtttctgtcactgtgaggttcttcagagtcttcttaattttgacagcttcaactttgagtttggcagatgttttggaggtggccaccttgtaggtatattctccaatgtcatctaatttggtggcagcaatgataagtctccttttgtggccatcagactcacttctgatgttgttagtcagtggtaggtgtttgccatccctcaaccattcgcctttggaatctgggttggcaacttcacattcaaacacagcttcctgggattcagctacggtctgatctgtgagtggcttggagatggccccacctgccacagtaagttttccagatgtcatattttctcccgcgtaaaatgtgtattttccttcatcatctttcatcatatttagaactgtcaatttatatatttttccatgtgcttcaattttatatttagaactgggcttgatttccttgtccttaaaattccacaggacatcaattccagagtgggacagctcaacctcaaacaccacattttgagtttctgtacaggtaaggtcacgaagacctctgataattttaattttttctacagagagattacagttggtttcaactctgccaactatcagcttgtaaggtccttcgtctgaagcatgagttcggttaatgactagtcgctgtttagtacctttcacaatggcctgtacacggtcatcaggcttgatttgttcatcatttaagtaccacttaacagaagtcacatcagggactgacaccttacattcaagcacagccttggtgccttcaatcacattaacatcttttagaggtgttatcacgtccacactatagacagagacacgcccactggtggagaggccaagggctggaatggtgaaagagtaatttccagcatcttccttagtcatgtcttcaatgagcagcatatgagattgtttgtctatcacaatgtgaaccctgtcactgggctgcacttcttggccgtctttcatccagacgccttccacactttccaaggagactttaacttcaagctgaacaatgtcaccctcacagactttttggtcactaagtccttgtaggatagcaatggggcggggtttcatctttaatttacaggttgtctttttcccgtcgatgacaaagctgtattctccctggtcctccttggttacatccttgaccgtgaggttctgacgtccacgacgagatgtaattgtatatttgccattggatttaagctccacatcattatgataccattttccttctatattttctggggatacaatgcactctaattctcctgaatatgattctggaacttctatgtcctgaagttctttcacaaactcaacaactgcaccttcaacaataagtttagcagtcgttttgacattttcatcttccacaagtacacagctgtaatcttcagcatcagacgtatcaatggtcagtatggagaggaagtgaacctttctgtcagagtgcatcctgtatttatctccctcatgaacctccataccatctttataccatttcactttgacaaatggttctgaagtttcacattcaaaggttgccatagtgtctttttccttagcaacaacatcttgtaattcctgtgtgaaagtgatcaattgcttggcttggacaagtaagaatgcgtgactggaggtttctccagctatgttgatggcttttaccatgatgctggcagagtcctcagcagtcacatctcttatgaccaattcacaaacattgtcttcgggccagtaccagtagatccggtcagaccgttcaattttgacaccatttttgtaccattcacattcggggtctggtttccccacgactctgacccggaagtgtgcatcagatccttggcccactgtttggctctggattctttcgaagatttttggagcctccatactaggacttagttcaatcttgtcaggtttaaaagttggaatcgtgattttgccttcttcggcaagagctttcttttcctcttcagttaactctttggtccagtggagaagttcatcttttgtcttcctgaggagttcctcataggattcatccttctttcgagacttgagctccacagcggtaatggcttcataatagccctcttctgttctgcgcttgaatttactgcgcagctcttccgactcttcaggcactttttcatgggtaattctttcagcccttttcaacttcacaacttctttggtttcagtggtgtcaacaggtctatccactttttgtacttcaaactgaagctttcctggttcatgtacgtgaaactcaggccttggttcaggagctctcctaaggacagacctaaaatcttccctctgttgaatctcaagcttcactttatgctctatcacaccttcaggattttccgcggtgaccttcacttcacctgtgtcatatgatttgcagtccacgatgtccaggtaatggataccatcatagcgaactctgaaccttttgcttttgcggatgagctgtccattgaggtaccagttgactttgggctgagggtagcctgttaccctgcagcggaaccttgcagtctccccttcaagtactctaactggctctgggtacaagacaatgtctggcttttgcttttctttctgatctgttgttacacctgtaagtgcaccttcatgagccattctctctaattcttcaattctctgtaagcctttcctcccctcaggcaattgggattcttccacaagacttttctcatctttaacaataagggtagcagatgtgtgatctgttccatatttgttagtggctctgcaagtaatgataccactgtctctagaatatgcaacgccataatcaaggctgcagtacccaaattcattgatcatacggagcctgttggctgcttcaagtggctttccatcatggagccactccaccaccatcgttgggtcaccaatgggtgttagcctgcattcaaagtgggcaggcccaaagcgcttaagtcttaaggaagtgagttttttcttgaaaaatggtttctgttgtttctctttgtcatagagatcaccttcttcccattgctcttggccatatcgcaaatggaggggctccagttctggggctgcaatctcctttgctctatatgtcccccgtgggatgattaactttctctctggctcaggctctgcaaactcaacttcaacatttactttgcatcttgtagtgtctctgccagctttattaatagcagtcgcagtataccaggcagaatcttggctgacagtggaatcgattttaagggcagcttctcccttggttccttcaattctgattttgggatatttatgaggcacaatgatgtcactgtttttcaaccatacaatgtcagggttggggttacccgtagctctgactttcatttcaagtcgggaaccttcctttatattgacatttttcagtttttctacaaacatcggttttacctgatgttccacagcttccacagttaaaatcactgaaattgaagatctgcctgccctgttttgggcaaccacagtccattccccagaatcactgggtgtggcagggacaataattagtgattgagtaccatcttctttaatgactactttatgggtatagtcattgacaatttgctggccatcatgaaaccagaacgtctctggcataggtctaccaacaacctttaagtcaaatctggcagtttgcccttctaaacatttgaaagaaacaggttttaacacaaagactggtttatatagtctctcaagttgtgactcatctgtctcctccagcctacgtccaggggacattcttgcaggggacatccgtgcaggagacatccttgcaggtgacatccgtgcaggagacatgcgtataggagacctgctcactgaacgtggagagagagatctgattctgctcactggctctagtgtgggaatgtaagtcggagctccaagtggtgcagcaggctccacatacaatttccctgagcaaattgcatttcctttaatattgctggcaaatgcagtgtagattccttcatcttctggaagaacaacaggtatacgcagactagctctgccatcttgtagaaagtccatttggtatctttctccatgtttgatgcgcttgccatctttgtaccaagcaatctttggtaatggatatccagacatcttgcaatgaaaagtgacacccatcccctcaagaattctataattcttgattcttgaatcaaatcctgattcaacagcttcagattcagaaatgtcaactgccatcttttcttctccatcttcttcaagaagttcttctaatgtagtctttattattctatattcaatttctttaataagtctctcttcaaaggaagaaatatggaattcctgatcttctacataagttctgaccactacagtatctttggccattttcttcctaattaaggcttgttctttttcatactctttttcatactcagagtatacaaatccaggtgctgtttctccaactttaggttcttgaacaaatgcagtcacttgtgtctgataaagcatttcttgctgggacttcatcagtaactcataatcagcttcttcaagcaaggaagcagatgcagaagtttctccatgcttattgcgaacaacaatagtgtattctccagcatcatcagcaaaagtcatagaaatcaccagcttgcattcaccggtttgtttgttgtaactcactttgtatctgtatccagtggttagaggaacaccagattttttccagtatacatggggctttgggttgccgccaacttggcatccaaacaccacgctcccaccttccaccagtttctggaccactggttttgtaataaagtaaggcgcggcaggttctccaggccctgcttgttcctctgtgaggctagtatcagtcataaccacatctcttgactcaacaaagcgtttctcttctgtagtaaatttctcagtcacggctgtggtttccttttcaaattcttctgacacctgcacagccagatagcaggatgtgctgacggttccagcctcatttacagcactgcaagtaaatcgcccgctgtcttccgcaaatgcttcgcgaatcataagacgagcaattccactctggaaggttatctggaagtcaatggaactttcgatttggtagtcttccctgtaccatgtcactgtcggggatgggtatccagagatgtggcactccaaggtgacagattcaccttctatgacagtcacattttttaagcccgagaccaaagttggtggagtaacaggaatttcaacaggtgctggtactcttgctgtttctgttaccttggcttcgcgtccgtgcagtacttcaaagcgctcttcacggacggtggtgccagtgatgctcacccctacttcctttttcacctcaacgccagcttcactcttgtaagtatctggtgtgtcagcgaaggggaactgtggcaagggtgtgggctctgcccttactctagtctcactgggcttcacagtaggagccttcaccgatttggtgatcttctgagcagaagatgtggctgacaactctttttgtaatgtggcaatagcactaccggctattgatgcctcatatccatgttctgtcttaggaacagaaatttttgaaacagtaaagtgagggctagctgtgcgggggcgtttatccacatggactaatctttccgttgttagatctgtagttttcttgatctgtgatgatatgtgcattcccttttgatcagtagttttgatatgagtctcagaaggagcctggattactctaggcttgactgctttagggacaacgtggggttctgaggctggacgttggggaggctcagctacctttgcggcggaaatgcgttccttatatccgtactccaaagtggtctgctgagcataggattcttcaagatgcccaggctctctgggctctctgactcgggcctggtctactgcagcaacaactgttgctacagcttcagccttttttccaacgtccacctttccatgggtaacttggatttgttcttgtctagtagccatagtttctctagttctcagtattgtttcttgttctttggctttagcagtagcaactgctattgtagacaaggcagttttctcggcttcctttctcatcttctcctgagttatttgcacttgttctcttttggtagtaatgccttctctacctcttgatactaaatcttgttctttgactttgggtgtggcaactatgactttaggtacaactgttttcctagtttccttcattatcttttcataacttaggtgcatttgatcttgttgtgtggtagtttcttcttgagctcccgggactgtttctagttttgtggactttgcagtggcaactaccaccatggatgcagcagttatctcagtttcctgtcttattgcttcttgagttacttgtttctgtttcttagtaatttcttcagaaattctagtttcttgttctttggctttagctgcggaaattactacctttggtacaaatgttttttcagtttcttttcttatctgctcatgagttacgtgcatctgctcttgctttgtggtaattacttctttggttcttgattttaattcttgttccttggctttatcggcggccactactaccttagttacagcagtcttctccgcttcctttcttacctgttcttgagcaggttggatgtgcacagcagtcgtggttgtcctctgagcagtctgctctacagcgctgatcactggttctctcactctggccatatcaacggcagcaacaacagtcgcaacagctgcacttttgtcagcatcttgtttcacctctttagcaccagtggcaacagcctctgctgcgtagctagcactggccgacacactggcggcagcacccgcagcaccactgatggtcacttgctcctggacaccgtatctcccttcccatctctcttctgtcctgatctgagtagaggttgtcagcgttgtctctctcatctcagcctcagatgaggaggccacgtagccctcttgcttccaagggggaggcacttcaggacctgtggccacggtggatgcctgagtcttacgcatgagcaatggagacctaacagacctgatgggggatgtggagattcttgctgctggagacacggacctgaccggagatggggtcggtgcccgcacgtgtctgaccggggaaggggagtgtcttatgggcgatggggactgctgccgagccagctgtgctttggcagcaatagacggtggtgttggggatcttgactttggcttcggaggaatcctgggaggtgttttatgtggcagctgttgcccagcggcaccatctatgaccatctcaactgttgcaattgatctggcatcaaagtgggcttcaatcttcttttcaattcgggtttgtcttgattctgagatctgagcagtcgaaacaattgtctttgtctttttagcaggtacttcttcttcaccttgaaccagtaattcagcagtcgaagtagctcttccaacgctattggtggcatttactgaataggtccctgagtcctcagggtatgcttctgcaatcagtaagctgtagaggtcgccttcttgtgaaatttggaaatcaagggagctctggatttcggctccatcccggtagaacttcaccacaggtgtagggattccagtcactctcacttggagtctcacttggcttccttgtctcacggtcatgctctgcagtcgttgaacgaagttgggtggtgctgtctcagctttcacgagaagctcagcagtactagtcgcttgtccagatccattggtggctttcagggaatatcgtccactgttggctttagtcacggcggggatcgtcagtttagcgcggccatcgctaaaggagatctgcacgccgggcagagtggaagtggaaatcacctggccatccctaaaccagctcacctcaggaactggaaaaccactaatgtgagcctcaaaggttgcggtactaccctccagtaccacaacgctttgtaacggctgcgtaaacgtcggtgcttgagttgtcatctttctaggcactctgatttctcaagagtgcctaaaaagggtgggactaagcccaaggttgcttctgaaacgacgtcctatggagagttggtttttctgaccatctccgacatgaatcggtgagcctctaatcctaaaaacaaaactacacagtcaagactgtgtagttttgcttttctatgcaatccctacacccgaggcgaggctgggaatgcacgactgctc

SEQ ID NO: 8417 - RNA, 20418 nt, Homo sapiens
  source 1..20418: mol_type = other RNA
aaaactgcagttacttttgccaacactgtttttcacttcaaagctatataatcctttgtcactcatttcggcacaggggattttaagggaagccactttattgatgaatgtaatgtgatgtttgctgtctgcagacaattctcttccatctttgaaccacttggctgagagttctggtgttccagtcactacacactctaatgcaaaaggatttccagtagtgacagtcatgggttcgggcttctctatgattcttgctggttctagtacagtcaagactgcagagcattctctcattccagcatcgtttttgatttggcatatatattttccagaattagatgcttctggactccccagctggagggttgcaatgttatcaatgaatgaaatcctggtattttcactctctctgatgacttcacctctatctttcagccagacaacagaaattggctggaagccctccactatggcccgtaactcaacagcatccccaataagggttgaggtgtcacttagctttttcacgaatcgtggaggttctttgaacttgacagagcaagaacacgtgtcacttcccacctcattagtagctttgcagtgatattccccgacatcggaggcttcaagattaaggatatgaagacttgtatcaaaatgttttgaagtgattttaaatttcttgctgtttctaacctgctttcgatctttaacccatactacttcaaatgggggagttcccgaaatttcacattggagaatcacatcagaacctttaagagctcctactggagaaggcttctgggtgaaaacaggaggtgctttcactgtcaacgctgtgctgcagctggcgtcaccaacaccattatgagcctcacaaatgtagtccccgctgtcttcagcactagcttcattgatcgtaagcaatgccacagaattaatgaatgacatgttgtatttccaactttcatgaagttcgctgtcatttcggaaccatgaaactttgatttctggggagccacttattttacattccagttgaatggattctccctgctttgcaacttttgaagcttctaatttcttaacaaactttggaggttcttttacactgagctgagctgagcacatgtctttgccaacatcattggttgcttggcaagtatattgaccagagtctcctttgcctactttaagaattctcaaatgaggagtgtttcccacacatgtgattgtatagtttcctccaggacggatctccttgttatcttttgaccaagtgattcgcatcggttgagcaccagtaacatgacactcaaaatcagcactttctccagcaataacatctatagatacaggcttgatgtcaaagaagggagatttcttgggttctcttgctgtgagtctagcactagaagatgctgttccaagtgggttggaagctgagcaagagtactggccagagtgactcaagtcagtttgcaaaatttttaaagttgccacattatctacaaatgaagtctgtagattttcatcgtctcttaaaagtactccatctctataccagcacacttggatgggtgcagagccatttaatcgacaagtgagtgtaacaggtaaccccacagtttgttcaatgtcctttaattgtcttgcaaaagaaggtgggagttggcgctcttgaattctgaacacagtcttagaagaagcagttcctatactattttctgctttgcatgtgtactctccactgtcattgatgttcactttattaaaaacaagtgtggccacattgtttgtaaagtaggtcctgtattcaggagttggccgtaatttggtatctcctttgtaccaagacactgtaatttctggtgtcccagcaacttggcattgtaaagaaaccgaatctccaactgctgcctccagaggttccagttccgtaacaaaataaggcggttctaatgtagataccagagctccacaaacatcccttcctgcctcattttcaatctcgcaggaatactgccctgcatctctttttgtgctattcagaatttccaggatacaagttttctctgttgtgactatgttacatttttcagaggtagttatgttaaaaccatcctttttccaagtgacagaaattggaagtgttccagtgtaggtgctctccagaattatggacttccctggttctacagaatgatcacttaatctcttcaaaaatgcagctggttctttcacaaagagacgggtagtgcaagatgcttggccagcgttgttagaaaccacacaggtgtattccccactctgagatatgtcaatattaaataattccagttctgccacagtgtcttcaaaatagatgttgcaccggtctcctttcactagttctctggcacctctgaaccagttgactttgaatggaggggttcctctaataacgcttgtgaaggttacatttttgcctggtagtacttccaaaggttcaggttctttcacaaaagagggtggttcttgtacagttagcactgcacgacattcatcagacccagcgacattagcagccacgcatgtgtaattgcccatatctgaggaatccagagaattcaactgcaatgtgcagacattatctgaaaatgtggtttggtactttgctccactgacaatcttggttttctcatgaaaccaggcaactgaaataggtgatgatccagctactttgcattccaagatgcaagaagcacctaacaccccaccagtatttttcagtcttcgtgtgaaagagggaggaactgctcggtctgaaacatcaaccacagctgtgcagctgcttttcccaacattattttgaacctggaaagtgtatgtgcctgcatcttgcctttcaactgagagaatccttaaggaagagattttgttgtagaagctaaatttgtgtttttggctgctggtcaacagctttccatccttgtaccattcaacagagagttccggagtgccagccaccttacactccagagtgcacgtttctcctacagtcaccgtcatcggtcctgccttctcaacaatgactgcgggctctaagaccatcagtgtggccatgttctccctcattccaccatcattcttgatttggcagatatactttccagcattagctggctctgcttttgcaaactgtagagttgcaacattttccacaaatgtaatcctgatgttttcactttctctaatcacttcttccttctctttaagccactggacaaaaataggctgggcgccttctatggatgcttgtaattcagcaggctctccggctacaacagtgaggctgttcagtttggagacaaatcttggtggttctttcaattttacagtacaaacacaagtatcacttcccacttcattctgtgctttgcagtggtattcaccgatgtctgaagtgtccacattgagaatgtgaatacttgtgtggaagtttttggatgcaatcttgtatttcttgctgcttctgagttgccgcttgtctttgtaccataccacctcaaacggtggtgttcccgaaagttcacattcaagactgacttcagcatttttaagggtttctactataggagggaagctgctaaaaacaggtggctcttttactataaccttggtactgcagcttgtgctgccagcgggattctgagcctcacaaatgaaatctccactgtcctcagtactgagattgttcatctgtatgacggccactgagtcaatgaaagtcattctgtacttatcactggctggaagttcatgttcatttcggaaccacacaactctgatttctggggatccagctatcttgcattcaagtcgtgaagagtcacctgctttcacaattttggaggcttctaatttctttacaaactttggtggttctgtcacaagcaacatcgtagtacaagagtcgctaccaacatcattggtaacatggcaagtatactgtccagtcttagaagcatccactgagtagagatttaagaagctagtcgacccttccaagccaatgaaacatttaggacctgagacaagttccacatcatccttaaaccattttattttaaatggtggtgttccttttagtattgccttaaattccactgtagaatcaggtatggcttgctgtcgcccaggtttcactaggaagcttggtggttctttcacagttaagatgccactgcatgcatcatctcctgctacatttgacactttgcatgtgtaatttgcagtatcttctaattccagattattaacttccagagacacagatctctcatggcacacaagtctgtattttgcacttgtagatatttcttttccatccttaaaccactgagcactaatgggaagtgaaccagacaccttgcactccatatgaatagaagagcccagaactttatccattttggttaattttttggtgaatgatggaggaatattttgatctagcactcttaagtaggcatcacagctactgcttccgaagtcattttccaccttgaaagtgtactgaccgctgtcctgcttcattactgactgaattctaaaactggccacgttattttcaaaactcattgaaaagtatctactgggaactatttgtttcccgtctttaagccatttcactttgagttctggtgttccagccacaacacattccaaggtcatgggatctttctccgtaacatcaactgatttagctttctctacgatttgagctggttcttgtactaaaaggaaagcataacacctctcaactcctgactcattcttggcttgacaggtatatctcccactgtgtccattatccacacttctgatttgaagtgtggccacactgtccacaaatgaaatatagacattatcatcttcatcaagaatctgatcatcctttagccaggttatagaaataggaggagaacctgccacggtactctgaaaggtggcagaacttttcaaaacagtagtggtattttctatcttcttaatgaatgatggtggttctttcagggcaactctagtactgcatgagcagctgccgccttcattggatacaatgcactggtattccccagtgtctgaagggtcacacttggttatatggaggttaaacacagacactctgtcggtcaatgtgtattttttgctgcttcgaatttccctgttattcttcagccaagtgacttcaaacggaggtgttcccgtaacttcacactccagctccacgtcactatattttactacctccacaggcttcagctctctgataaaggtggggggttctttcactttgagttcaatgctgcagctcgccgtgcctgcgtcatttcgagcttcacacacataagtcccactattttctaccctggcaccagaaatctggaaagtggctaaaccatcaatgaaggaaatgccatgtttctgaatggctgttatttcattcccgtctagataccaagacactcggattttaggagtgcctgttatttggcattcaaatgttgttgactgtccattcctcagcactaagactggactgggcttcttaatgaattgaggaggttcttttacaaagagagtggctttgctggttgctgtgccaacatcattgcttagttggcaaatgtaggttccagaatcggtagctttggctgcaaagagctctagactggtagaggtgtcatccttccaaactgagcgggctgctcctgagtgtaactctttgttatctttaaaccactttattgtcatgggtgcagtgccacccacaagagcctttaactgtacccttgtgttgggattgacatcttgtgactgtggcttttccacaaagtaagggggttctttgactgtcagatgcccactgcattggttgtgccctgccttatttgtggcagaacaagtgtatgtcccactgtctgtaccttccagctggctgatttccaagaaggcagtattgtcatgaaaagagaatttgtacttttcactagctgatatttcttggtcatctttgaaccactggatgcttatgggatgtgacccagccactatacattctaaatcaatgaaagaacctttaatgctgtccattttcttcagctttttggtgaatgaaggaggtatgataagatctaatacattaattctagccttgcagctgctcctcccaacatcattttggacctcgaaagtatattctccactatctttcttttctgtagaaataatcttcagtattgagactgtatcagtgacactgattttatattttgagcccagggtcagttcttggccatctttaaaccatttggctgtaatctccttagtccctgaaaatttaacctgcaaagtggctgggtctccttgggtgacatctatagacacagcttcctcggtgattgttgcaggttcttttactgagagtaatgcagaacatctttgtattcctgcatcatttttggcctgacagacatatttcccatcatgcttgacttcaatgccactgaggtacaaactggccacattgttctcaaaggtcattcttatattatcgtcttcagtgatttcatcgctgtcttttagccaagtcaccgtaattggcaaggagcccttcagagtggcctggaaggcagctgtgcctccccggagggagctggtactctcgatcttctttatgaaggatgggggttctcttaaagtcaccctggcactgcagatgctgctgcccacctcattggtcacccgacactggtattcgccagcatctgcagctacaaacttgaggatctgcaggctaaccagatgatcctgaatgaaagtcttatactttctaccacttcgcaggattgtgttatctttgaaccaagtgatctcaaagggaggagtgcctgccacctcagccagcaacatgacatcgtactcctttaagacttcaattggcttaaattccttggtaaaataaggtgactctttgactattacaatgctactgcagtggtcactgccagcctcattttgggcctcacacatatattcaccactgtcttcgatgccaacatctgtcagtcttagaactgcagtagactccacaaaagacattctgtgtttgctgctctccttaatttctctatcatttgcaaaccatgttattttaattggaggggtaccagttactttgcaggctagctgggtggcatctcccttctttaacagctgtgatggctctaacttttcaacaaatgtggcaggttcttttacaaacaagtttgcactgcattccacccctccagcgacattgctgactttacatgtgtacgtgcccgaatcagaggtttttactaaatagagttccagggaactctctaaagcttctttggtaatatagcagcttccaccagaaaccagctctttgttgcccttaaaccatctgattgtgagaggagtagatccttggaaagtgctcttcaggcagactgctgagccaggcagaacatcctttgagccgggtttagttacaaaactgggtggttcttgcacaatcagggctccactgctgtctttgcttcccacggaatttgtggctcgacaagtgaaattccctgcatcattcatgtctactctgatgatctccaaagaggctgtgccttccacaaatgctatcctgtatctgtcagaagcagctatttctttgccatccttaaaccaggacaccctcatggggagggagcctgcaattttgcagtccagtctgcaggtaccattaacaacactatccacgttgcgcaagggtttggtaaaaaatggagcaatgtctcgatctaatacagtgaatgtagtctcacaggagctgctgcccacttcattggaaatctcaaatgtgtattggccactgtcgtgcagctcagctgaataaaatttgagctgggcaacattgtttttaaaacttattcggtattttttactggcgaccaagggtctcccatctttgtaccatttgggcttcagttctggcgtgcctgccactgtgtactccagtgtggcgggatctcctgctgtcacctggatcagttctgctcgctcaatgattttggcaggttctttaactattaattccccaacagatgtttggcttccagcttcattttcagccaggcacgtgtatttgcctccaaaactaatctgaacatcagggattatcaagactgcaacaccattggaaaagctcattttgatttttccgtcttctctgatgacctcttgacctttcatccatgtgacagaaatgggctctgaccctctcacagcagcttgcagggtaacggtttgtcctcctagtgcaatcaaatcatctactttctttacaaaggttggaggttctttgagtaagtgggttgccatgcagccacacttgccgacttcattagcaacaacacattcatattcaccaacatctgcactattaaacgaaaagatctccagacacacaagagacttctgagaaaacaatctgtattttttactacttcgaatttgtttcttgtctttgaaccagctaatttcaaatggtccagtgcctgagacttcacactgaagtagagcatttgttcctctcactatgtctgcaggctcaagagttttgatgaaagaaggaggttctttgataactatttcagtactgcagctatcactgccgacgtcattcactgcttcacatgagtaactcccactgtcttcaacttttacatccgtaatatcaagtatagcctcagaattgacaaaatacattcggactgtgttactttcactgagttctttgttatttttaaaccaagtaacctggatcacaggtgagcctttcagcttgcaatggaggcgtgctgattcacctgggagcattaaataagagggatccaccttcttcacgaaggatggtggctctctgacagtgactgtggctgagcaggagctgcttccagcctcatttgaagctgtacagacataggttcctgaatctttcagtttggccaaaggaatctcaagtgttgctattttatcttcaaaacagatcttataatctttccctggggggagtttttgcccatctttgctccacgtaactgtgacttttctgtcttcatctacttggcactcaaggtggaccttcttattgatagcggactgcacaggctctaattctttaatgaaatgtggcttatcaatgatgatcaactctgcttggcagatgtctgctccaaacttgttggaagccttacaagaataaactcctctatcttgaatggtaaggtttgagagttctaaaatgtgtttgttttctgcgtcggaaatcctccagttaggtgaaggtgagagtgcagcaccatctttctgccaaatggtttctatcacaggagtccctgtcactgtgcagatgaacttggctgccttacccacaaaagttgtaagggacttaggtctggagagaaaggttggtggatatgcctctgtcacagttagtgtggctgtacagctgacactgccatactcattggaagctttgcatgtatactcgccgcagtcaaccacctgggttctcaggatttcaaggctggagatatactttgaagatcgaatagaacacttgtcactctcataaatttctcggccagctttaaaccactggaaccggacattgggagcactttggatctcacaggtgaatttggctaggtggcccagtgctacttccaggggttcgattttcctcttgatcactggggcagctttcatttccatctcaatctcttgttcaatcctctcatgcaaaattgattcaggagcttccagactcaggttggctgtgcttgatacttggcctacagcattactagcaacaaacgtgtaagttccttcatcttctggataagcttcggcaatttccagttgataagtgtcttcaaattgagtcattctaaagaaccgagatggcttgattttcttgtctttgctgtaccacgacacttttagatctgttccagaaacccggcattgaaaacgggctggctgcccttcagaagtgacagtgtcctgaagcggggtgatgatggcaggtggataaacaggcatttcctgatcaggagacacaacttctggaacttccactgagagtgaagctgatgttgtggcaacaccatagtcattcttggcttcacaggtatagactgccgcatcctctgggaaggcttcaattagcaaaagcgtgtattcttgcccatcatgaagaaatttgcacttgaagccagtggaaagcagctgctcttccttgtaccaggaaattttgggctgtggtcttccggatatcacggcacagaagcgggcaggcttgccagactgcacagtgacaggctggagctcctgcagaacttggggcggttcaggagcattgacatagagagtgacagaactcctgttccttcctgccacaaaggtgtattctcctgcatcgctctgtctggtctcagagataaacattcggtggattcttctttccactacatatttgtgtcgttcttgaacttggaaattgatttcaatgccatctttataccagtgggcatcaacatcgtcttcattgacctcaaattcaacaacagcacgctgtttctcaatgacctgaacctcctttttaatacttcggatgcgaacatctctgccttctacaaagagttttgcagttgacacgttgcctcctgccaccactgtgtacttcccagcatcagacatccgggtggatgggatcagaaggcggtggacatatttctccttctgaatctttattctgtctgtgatctgcagttcctggtcatctttcatccactgtacagtgatgtcaggttcagaaacttcacattcaaacatggctcgcttcttctccagtaccttaatgtccttaatgtgtttcctaaattctatatgacgagcttccacataaagtgtggctgttgatgttgcttttccagccacaaaggtgtagtcagcagcatccccaaagtgaacattcctgatgttcagtgagtgtgtgagctttttggttctcatctggcacttgtcagttgatttgatttccacaccattctttaaccatttgtaagagatgccttcatagttcactgtcacctcaaaagtaatagtgtctttttcttcagcgttgatgtctttcagcatggaagtaatcatgattggggtgactgtcagggtggcactgacttggtcattgccacagacaaatgtgtattctgccgagtcctctgtgctggtgttcatgatgatcagctgatggagttttccctgcacaactatcttgaacttttcactcatctcaatttccacaccattcttcagccacatggaagggacattgaagtgggacacctcacactcaaaagaggcagttttggtctcaggcacctcgatatttttcatggtttttgtaatatgtaatgtctccacaaacagttttgctttgcattccaattgcccgaccacagctgtgtattccccagcatctgagggggagatgttctgcagcatcagcttgtggactttcctttctgagaccagtctgtgtttgtcacttggcttaatttccacactcttatggaaccattttactggaacagtgtcatgggaaacactaacttcaaaggcaacagtggcattttccaaggctgtcacatcctttggctttttaatgatcttgacagtctccacgtgcagtctggcactggctccaagccttccaagcctgaagccataaacagactcatccacgatggcacagtttttaatcctcagagagtaaattgttcctttgacagagatagcatacttttcattggattccagcacaactccatttttgatccactggacacctttgacattagggtgtgtaagctcgacagtgaaaacagcatcctgtgtttctgtcactgtgaggttcttcagagtcttcttaattttgacagcttcaactttgagtttggcagatgttttggaggtggccaccttgtaggtatattctccaatgtcatctaatttggtggcagcaatgataagtctccttttgtggccatcagactcacttctgatgttgttagtcagtggtaggtgtttgccatccctcaaccattcgcctttggaatctgggttggcaacttcacattcaaacacagcttcctgggattcagctacggtctgatctgtgagtggcttggagatggccccacctgccacagtaagttttccagatgtcatattttctcccgcgtaaaatgtgtattttccttcatcatctttcatcatatttagaactgtcaatttatatatttttccatgtgcttcaattttatatttagaactgggcttgatttccttgtccttaaaattccacaggacatcaattccagagtgggacagctcaacctcaaacaccacattttgagtttctgtacaggtaaggtcacgaagacctctgataattttaattttttctacagagagattacagttggtttcaactctgccaactatcagcttgtaaggtccttcgtctgaagcatgagttcggttaatgactagtcgctgtttagtacctttcacaatggcctgtacacggtcatcaggcttgatttgttcatcatttaagtaccacttaacagaagtcacatcagggactgacaccttacattcaagcacagccttggtgccttcaatcacattaacatcttttagaggtgttatcacgtccacactatagacagagacacgcccactggtggagaggccaagggctggaatggtgaaagagtaatttccagcatcttccttagtcatgtcttcaatgagcagcatatgagattgtttgtctatcacaatgtgaaccctgtcactgggctgcacttcttggccgtctttcatccagacgccttccacactttccaaggagactttaacttcaagctgaacaatgtcaccctcacagactttttggtcactaagtccttgtaggatagcaatggggcggggtttcatctttaatttacaggttgtctttttcccgtcgatgacaaagctgtattctccctggtcctccttggttacatccttgaccgtgaggttctgacgtccacgacgagatgtaattgtatatttgccattggatttaagctccacatcattatgataccattttccttctatattttctggggatacaatgcactctaattctcctgaatatgattctggaacttctatgtcctgaagttctttcacaaactcaacaactgcaccttcaacaataagtttagcagtcgttttgacattttcatcttccacaagtacacagctgtaatcttcagcatcagacgtatcaatggtcagtatggagaggaagtgaacctttctgtcagagtgcatcctgtatttatctccctcatgaacctccataccatctttataccatttcactttgacaaatggttctgaagtttcacattcaaaggttgccatagtgtctttttccttagcaacaacatcttgtaattcctgtgtgaaagtgatcaattgcttggcttggacaagtaagaatgcgtgactggaggtttctccagctatgttgatggcttttaccatgatgctggcagagtcctcagcagtcacatctcttatgaccaattcacaaacattgtcttcgggccagtaccagtagatccggtcagaccgttcaattttgacaccatttttgtaccattcacattcggggtctggtttccccacgactctgacccggaagtgtgcatcagatccttggcccactgtttggctctggattctttcgaagatttttggagcctccatactaggacttagttcaatcttgtcaggtttaaaagttggaatcgtgattttgccttcttcggcaagagctttcttttcctcttcagttaactctttggtccagtggagaagttcatcttttgtcttcctgaggagttcctcataggattcatccttctttcgagacttgagctccacagcggtaatggcttcataatagccctcttctgttctgcgcttgaatttactgcgcagctcttccgactcttcaggcactttttcatgggtaattctttcagcccttttcaacttcacaacttctttggtttcagtggtgtcaacaggtctatccactttttgtacttcaaactgaagctttcctggttcatgtacgtgaaactcaggccttggttcaggagctctcctaaggacagacctaaaatcttccctctgttgaatctcaagcttcactttatgctctatcacaccttcaggattttccgcggtgaccttcacttcacctgtgtcatatgatttgcagtccacgatgtccaggtaatggataccatcatagcgaactctgaaccttttgcttttgcggatgagctgtccattgaggtaccagttgactttgggctgagggtagcctgttaccctgcagcggaaccttgcagtctccccttcaagtactctaactggctctgggtacaagacaatgtctggcttttgcttttctttctgatctgttgttacacctgtaagtgcaccttcatgagccattctctctaattcttcaattctctgtaagcctttcctcccctcaggcaattgggattcttccacaagacttttctcatctttaacaataagggtagcagatgtgtgatctgttccatatttgttagtggctctgcaagtaatgataccactgtctctagaatatgcaacgccataatcaaggctgcagtacccaaattcattgatcatacggagcctgttggctgcttcaagtggctttccatcatggagccactccaccaccatcgttgggtcaccaatgggtgttagcctgcattcaaagtgggcaggcccaaagcgcttaagtcttaaggaagtgagttttttcttgaaaaatggtttctgttgtttctctttgtcatagagatcaccttcttcccattgctcttggccatatcgcaaatggaggggctccagttctggggctgcaatctcctttgctctatatgtcccccgtgggatgattaactttctctctggctcaggctctgcaaactcaacttcaacatttactttgcatcttgtagtgtctctgccagctttattaatagcagtcgcagtataccaggcagaatcttggctgacagtggaatcgattttaagggcagcttctcccttggttccttcaattctgattttgggatatttatgaggcacaatgatgtcactgtttttcaaccatacaatgtcagggttggggttacccgtagctctgactttcatttcaagtcgggaaccttcctttatattgacatttttcagtttttctacaaacatcggttttacctgatgttccacagcttccacagttaaaatcactgaaattgaagatctgcctgccctgttttgggcaaccacagtccattccccagaatcactgggtgtggcagggacaataattagtgattgagtaccatcttctttaatgactactttatgggtatagtcattgacaatttgctggccatcatgaaaccagaacgtctctggcataggtctaccaacaacctttaagtcaaatctggcagtttgcccttctaaacatttgaaagaaacaggttttaacacaaagactggtttatatagtctctcaagttgtgactcatctgtctcctccagcctacgtccaggggacattcttgcaggggacatccgtgcaggagacatccttgcaggtgacatccgtgcaggagacatgcgtataggagacctgctcactgaacgtggagagagagatctgattctgctcactggctctagtgtgggaatgtaagtcggagctccaagtggtgcagcaggctccacatacaatttccctgagcaaattgcatttcctttaatattgctggcaaatgcagtgtagattccttcatcttctggaagaacaacaggtatacgcagactagctctgccatcttgtagaaagtccatttggtatctttctccatgtttgatgcgcttgccatctttgtaccaagcaatctttggtaatggatatccagacatcttgcaatgaaaagtgacacccatcccctcaagaattctataattcttgattcttgaatcaaatcctgattcaacagcttcagattcagaaatgtcaactgccatcttttcttctccatcttcttcaagaagttcttctaatgtagtctttattattctatattcaatttctttaataagtctctcttcaaaggaagaaatatggaattcctgatcttctacataagttctgaccactacagtatctttggccattttcttcctaattaaggcttgttctttttcatactctttttcatactcagagtatacaaatccaggtgctgtttctccaactttaggttcttgaacaaatgcagtcacttgtgtctgataaagcatttcttgctgggacttcatcagtaactcataatcagcttcttcaagcaaggaagcagatgcagaagtttctccatgcttattgcgaacaacaatagtgtattctccagcatcatcagcaaaagtcatagaaatcaccagcttgcattcaccggtttgtttgttgtaactcactttgtatctgtatccagtggttagaggaacaccagattttttccagtatacatggggctttgggttgccgccaacttggcatccaaacaccacgctcccaccttccaccagtttctggaccactggttttgtaataaagtaaggcgcggcaggttctccaggccctgcttgttcctctgtgaggctagtatcagtcataaccacatctcttgactcaacaaagcgtttctcttctgtagtaaatttctcagtcacggctgtggtttccttttcaaattcttctgacacctgcacagccagatagcaggatgtgctgacggttccagcctcatttacagcactgcaagtaaatcgcccgctgtcttccgcaaatgcttcgcgaatcataagacgagcaattccactctggaaggttatctggaagtcaatggaactttcgatttggtagtcttccctgtaccatgtcactgtcggggatgggtatccagagatgtggcactccaaggtgacagattcaccttctatgacagtcacattttttaagcccgagaccaaagttggtggagtaacaggaatttcaacaggtgctggtactcttgctgtttctgttaccttggcttcgcgtccgtgcagtacttcaaagcgctcttcacggacggtggtgccagtgatgctcacccctacttcctttttcacctcaacgccagcttcactcttgtaagtatctggtgtgtcagcgaaggggaactgtggcaagggtgtgggctctgcccttactctagtctcactgggcttcacagtaggagccttcaccgatttggtgatcttctgagcagaagatgtggctgacaactctttttgtaatgtggcaatagcactaccggctattgatgcctcatatccatgttctgtcttaggaacagaaatttttgaaacagtaaagtgagggctagctgtgcgggggcgtttatccacatggactaatctttccgttgttagatctgtagttttcttgatctgtgatgatatgtgcattcccttttgatcagtagttttgatatgagtctcagaaggagcctggattactctaggcttgactgctttagggacaacgtggggttctgaggctggacgttggggaggctcagctacctttgcggcggaaatgcgttccttatatccgtactccaaagtggtctgctgagcataggattcttcaagatgcccaggctctctgggctctctgactcgggcctggtctactgcagcaacaactgttgctacagcttcagccttttttccaacgtccacctttccatgggtaacttggatttgttcttgtctagtagccatagtttctctagttctcagtattgtttcttgttctttggctttagcagtagcaactgctattgtagacaaggcagttttctcggcttcctttctcatcttctcctgagttatttgcacttgttctcttttggtagtaatgccttctctacctcttgatactaaatcttgttctttgactttgggtgtggcaactatgactttaggtacaactgttttcctagtttccttcattatcttttcataacttaggtgcatttgatcttgttgtgtggtagtttcttcttgagctcccgggactgtttctagttttgtggactttgcagtggcaactaccaccatggatgcagcagttatctcagtttcctgtcttattgcttcttgagttacttgtttctgtttcttagtaatttcttcagaaattctagtttcttgttctttggctttagctgcggaaattactacctttggtacaaatgttttttcagtttcttttcttatctgctcatgagttacgtgcatctgctcttgctttgtggtaattacttctttggttcttgattttaattcttgttccttggctttatcggcggccactactaccttagttacagcagtcttctccgcttcctttcttacctgctgttcttgagcaggttggatgtgcacagcagtcgtggttgtcctctgagcagtctgctctacagcgctgatcactggttctctcactctggccatatcaacggcagcaacaacagtcgcaacagctgcacttttgtcagcatcttgtttcacctctttagcaccagtggcaacagcctctgctgcgtagctagcactggccgacacactggcggcagcacccgcagcaccactgatggtcacttgctcctggacaccgtatctcccttcccatctctcttctgtcctgatctgagtagaggttgtcagcgttgtctctctcatctcagcctcagatgaggaggccacgtagccctcttgcttccaagggggaggcacttcaggacctgtggccacggtggatgcctgagtcttacgcatgagcaatggagacctaacagacctgatgggggatgtggagattcttgctgctggagacacggacctgaccggagatggggtcggtgcccgcacgtgtctgaccggggaaggggagtgtcttatgggcgatggggactgctgccgagccagctgtgctttggcagcaatagacggtggtgttggggatcttgactttggcttcggaggaatcctgggaggtgttttatgtggcagctgttgcccagcggcaccatctatgaccatctcaactgttgcaattgatctggcatcaaagtgggcttcaatcttcttttcaattcgggtttgtcttgattctgagatctgagcagtcgaaacaattgtctttgtctttttagcaggtacttcttcttcaccttgaaccagtaattcagcagtcgaagtagctcttccaacgctattggtggcatttactgaataggtccctgagtcctcagggtatgcttctgcaatcagtaagctgtagaggtcgccttcttgtgaaatttggaaatcaagggagctctggatttcggctccatcccggtagaacttcaccacaggtgtagggattccagtcactctcacttggagtctcacttggcttccttgtctcacggtcatgctctgcagtcgttgaacgaagttgggtggtgctgtctcagctttcacgagaagctcagcagtactagtcgcttgtccagatccattggtggctttcagggaatatcgtccactgttggctttagtcacggcggggatcgtcagtttagcgcggccatcgctaaaggagatctgcacgccgggcagagtggaagtggaaatcacctggccatccctaaaccagctcacctcaggaactggaaaaccactaatgtgagcctcaaaggttgcggtactaccctccagtaccacaacgctttgtaacggctgcgtaaacgtcggtgcttgagttgtcatctttctaggcactctgatttctcaagagtgcctaaaaagggtgggactaagcccaaggttgcttctgaaacgacgtcctatggagagttggtttttctgaccatctccgacatgaatcggtgagcctctaatcctaaaaacaaaactacacagtcaagactgtgtagttttgcttttctatgcaatccctacacccgaggcgaggctgggaatgcacgactgctc

SEQ ID NO: 8418 - RNA, 20415 nt, Homo sapiens
  source 1..20415: mol_type = other RNA
aaaactgcagttacttttgccaacactgtttttcacttcaaagctatataatcctttgtcactcatttcggcacaggggattttaagggaagccactttattgatgaatgtaatgtgatgtttgctgtctgcagacaattctcttccatctttgaaccacttggctgagagttctggtgttccagtcactacacactctaatgcaaaaggatttccagtagtgacagtcatgggttcgggcttctctatgattcttgctggttctagtacagtcaagactgcagagcattctctcattccagcatcgtttttgatttggcatatatattttccagaattagatgcttctggactccccagctggagggttgcaatgttatcaatgaatgaaatcctggtattttcactctctctgatgacttcacctctatctttcagccagacaacagaaattggctggaagccctccactatggcccgtaactcaacagcatccccaataagggttgaggtgtcacttagctttttcacgaatcgtggaggttctttgaacttgacagagcaagaacacgtgtcacttcccacctcattagtagctttgcagtgatattccccgacatcggaggcttcaagattaaggatatgaagacttgtatcaaaatgttttgaagtgattttaaatttcttgctgtttctaacctgctttcgatctttaacccatactacttcaaatgggggagttcccgaaatttcacattggagaatcacatcagaacctttaagagctcctactggagaaggcttctgggtgaaaacaggaggtgctttcactgtcaacgctgtgctgcagctggcgtcaccaacaccattatgagcctcacaaatgtagtccccgctgtcttcagcactagcttcattgatcgtaagcaatgccacagaattaatgaatgacatgttgtatttccaactttcatgaagttcgctgtcatttcggaaccatgaaactttgatttctggggagccacttattttacattccagttgaatggattctccctgctttgcaacttttgaagcttctaatttcttaacaaactttggaggttcttttacactgagctgagctgagcacatgtctttgccaacatcattggttgcttggcaagtatattgaccagagtctcctttgcctactttaagaattctcaaatgaggagtgtttcccacacatgtgattgtatagtttcctccaggacggatctccttgttatcttttgaccaagtgattcgcatcggttgagcaccagtaacatgacactcaaaatcagcactttctccagcaataacatctatagatacaggcttgatgtcaaagaagggagatttcttgggttctcttgctgtgagtctagcactagaagatgctgttccaagtgggttggaagctgagcaagagtactggccagagtgactcaagtcagtttgcaaaatttttaaagttgccacattatctacaaatgaagtctgtagattttcatcgtctcttaaaagtactccatctctataccagcacacttggatgggtgcagagccatttaatcgacaagtgagtgtaacaggtaaccccacagtttgttcaatgtcctttaattgtcttgcaaaagaaggtgggagttggcgctcttgaattctgaacacagtcttagaagaagcagttcctatactattttctgctttgcatgtgtactctccactgtcattgatgttcactttattaaaaacaagtgtggccacattgtttgtaaagtaggtcctgtattcaggagttggccgtaatttggtatctcctttgtaccaagacactgtaatttctggtgtcccagcaacttggcattgtaaagaaaccgaatctccaactgctgcctccagaggttccagttccgtaacaaaataaggcggttctaatgtagataccagagctccacaaacatcccttcctgcctcattttcaatctcgcaggaatactgccctgcatctctttttgtgctattcagaatttccaggatacaagttttctctgttgtgactatgttacatttttcagaggtagttatgttaaaaccatcctttttccaagtgacagaaattggaagtgttccagtgtaggtgctctccagaattatggacttccctggttctacagaatgatcacttaatctcttcaaaaatgcagctggttctttcacaaagagacgggtagtgcaagatgcttggccagcgttgttagaaaccacacaggtgtattccccactctgagatatgtcaatattaaataattccagttctgccacagtgtcttcaaaatagatgttgcaccggtctcctttcactagttctctggcacctctgaaccagttgactttgaatggaggggttcctctaataacgcttgtgaaggttacatttttgcctggtagtacttccaaaggttcaggttctttcacaaaagagggtggttcttgtacagttagcactgcacgacattcatcagacccagcgacattagcagccacgcatgtgtaattgcccatatctgaggaatccagagaattcaactgcaatgtgcagacattatctgaaaatgtggtttggtactttgctccactgacaatcttggttttctcatgaaaccaggcaactgaaataggtgatgatccagctactttgcattccaagatgcaagaagcacctaacaccccaccagtatttttcagtcttcgtgtgaaagagggaggaactgctcggtctgaaacatcaaccacagctgtgcagctgcttttcccaacattattttgaacctggaaagtgtatgtgcctgcatcttgcctttcaactgagagaatccttaaggaagagattttgttgtagaagctaaatttgtgtttttggctgctggtcaacagctttccatccttgtaccattcaacagagagttccggagtgccagccaccttacactccagagtgcacgtttctcctacagtcaccgtcatcggtcctgccttctcaacaatgactgcgggctctaagaccatcagtgtggccatgttctccctcattccaccatcattcttgatttggcagatatactttccagcattagctggctctgcttttgcaaactgtagagttgcaacattttccacaaatgtaatcctgatgttttcactttctctaatcacttcttccttctctttaagccactggacaaaaataggctgggcgccttctatggatgcttgtaattcagcaggctctccggctacaacagtgaggctgttcagtttggagacaaatcttggtggttctttcaattttacagtacaaacacaagtatcacttcccacttcattctgtgctttgcagtggtattcaccgatgtctgaagtgtccacattgagaatgtgaatacttgtgtggaagtttttggatgcaatcttgtatttcttgctgcttctgagttgccgcttgtctttgtaccataccacctcaaacggtggtgttcccgaaagttcacattcaagactgacttcagcatttttaagggtttctactataggagggaagctgctaaaaacaggtggctcttttactataaccttggtactgcagcttgtgctgccagcgggattctgagcctcacaaatgaaatctccactgtcctcagtactgagattgttcatctgtatgacggccactgagtcaatgaaagtcattctgtacttatcactggctggaagttcatgttcatttcggaaccacacaactctgatttctggggatccagctatcttgcattcaagtcgtgaagagtcacctgctttcacaattttggaggcttctaatttctttacaaactttggtggttctgtcacaagcaacatcgtagtacaagagtcgctaccaacatcattggtaacatggcaagtatactgtccagtcttagaagcatccactgagtagagatttaagaagctagtcgacccttccaagccaatgaaacatttaggacctgagacaagttccacatcatccttaaaccattttattttaaatggtggtgttccttttagtattgccttaaattccactgtagaatcaggtatggcttgctgtcgcccaggtttcactaggaagcttggtggttctttcacagttaagatgccactgcatgcatcatctcctgctacatttgacactttgcatgtgtaatttgcagtatcttctaattccagattattaacttccagagacacagatctctcatggcacacaagtctgtattttgcacttgtagatatttcttttccatccttaaaccactgagcactaatgggaagtgaaccagacaccttgcactccatatgaatagaagagcccagaactttatccattttggttaattttttggtgaatgatggaggaatattttgatctagcactcttaagtaggcatcacagctactgcttccgaagtcattttccaccttgaaagtgtactgaccgctgtcctgcttcattactgactgaattctaaaactggccacgttattttcaaaactcattgaaaagtatctactgggaactatttgtttcccgtctttaagccatttcactttgagttctggtgttccagccacaacacattccaaggtcatgggatctttctccgtaacatcaactgatttagctttctctacgatttgagctggttcttgtactaaaaggaaagcataacacctctcaactcctgactcattcttggcttgacaggtatatctcccactgtgtccattatccacacttctgatttgaagtgtggccacactgtccacaaatgaaatatagacattatcatcttcatcaagaatctgatcatcctttagccaggttatagaaataggaggagaacctgccacggtactctgaaaggtggcagaacttttcaaaacagtagtggtattttctatcttcttaatgaatgatggtggttctttcagggcaactctagtactgcatgagcagctgccgccttcattggatacaatgcactggtattccccagtgtctgaagggtcacacttggttatatggaggttaaacacagacactctgtcggtcaatgtgtattttttgctgcttcgaatttccctgttattcttcagccaagtgacttcaaacggaggtgttcccgtaacttcacactccagctccacgtcactatattttactacctccacaggcttcagctctctgataaaggtggggggttctttcactttgagttcaatgctgcagctcgccgtgcctgcgtcatttcgagcttcacacacataagtcccactattttctaccctggcaccagaaatctggaaagtggctaaaccatcaatgaaggaaatgccatgtttctgaatggctgttatttcattcccgtctagataccaagacactcggattttaggagtgcctgttatttggcattcaaatgttgttgactgtccattcctcagcactaagactggactgggcttcttaatgaattgaggaggttcttttacaaagagagtggctttgctggttgctgtgccaacatcattgcttagttggcaaatgtaggttccagaatcggtagctttggctgcaaagagctctagactggtagaggtgtcatccttccaaactgagcgggctgctcctgagtgtaactctttgttatctttaaaccactttattgtcatgggtgcagtgccacccacaagagcctttaactgtacccttgtgttgggattgacatcttgtgactgtggcttttccacaaagtaagggggttctttgactgtcagatgcccactgcattggttgtgccctgccttatttgtggcagaacaagtgtatgtcccactgtctgtaccttccagctggctgatttccaagaaggcagtattgtcatgaaaagagaatttgtacttttcactagctgatatttcttggtcatctttgaaccactggatgcttatgggatgtgacccagccactatacattctaaatcaatgaaagaacctttaatgctgtccattttcttcagctttttggtgaatgaaggaggtatgataagatctaatacattaattctagccttgcagctgctcctcccaacatcattttggacctcgaaagtatattctccactatctttcttttctgtagaaataatcttcagtattgagactgtatcagtgacactgattttatattttgagcccagggtcagttcttggccatctttaaaccatttggctgtaatctccttagtccctgaaaatttaacctgcaaagtggctgggtctccttgggtgacatctatagacacagcttcctcggtgattgttgcaggttcttttactgagagtaatgcagaacatctttgtattcctgcatcatttttggcctgacagacatatttcccatcatgcttgacttcaatgccactgaggtacaaactggccacattgttctcaaaggtcattcttatattatcgtcttcagtgatttcatcgctgtcttttagccaagtcaccgtaattggcaaggagcccttcagagtggcctggaaggcagctgtgcctccccggagggagctggtactctcgatcttctttatgaaggatgggggttctcttaaagtcaccctggcactgcagatgctgctgcccacctcattggtcacccgacactggtattcgccagcatctgcagctacaaacttgaggatctgcaggctaaccagatgatcctgaatgaaagtcttatactttctaccacttcgcaggattgtgttatctttgaaccaagtgatctcaaagggaggagtgcctgccacctcagccagcaacatgacatcgtactcctttaagacttcaattggcttaaattccttggtaaaataaggtgactctttgactattacaatgctactgcagtggtcactgccagcctcattttgggcctcacacatatattcaccactgtcttcgatgccaacatctgtcagtcttagaactgcagtagactccacaaaagacattctgtgtttgctgctctccttaatttctctatcatttgcaaaccatgttattttaattggaggggtaccagttactttgcaggctagctgggtggcatctcccttctttaacagctgtgatggctctaacttttcaacaaatgtggcaggttcttttacaaacaagtttgcactgcattccacccctccagcgacattgctgactttacatgtgtacgtgcccgaatcagaggtttttactaaatagagttccagggaactctctaaagcttctttggtaatatagcagcttccaccagaaaccagctctttgttgcccttaaaccatctgattgtgagaggagtagatccttggaaagtgctcttcaggcagactgctgagccaggcagaacatcctttgagccgggtttagttacaaaactgggtggttcttgcacaatcagggctccactgctgtctttgcttcccacggaatttgtggctcgacaagtgaaattccctgcatcattcatgtctactctgatgatctccaaagaggctgtgccttccacaaatgctatcctgtatctgtcagaagcagctatttctttgccatccttaaaccaggacaccctcatggggagggagcctgcaattttgcagtccagtctgcaggtaccattaacaacactatccacgttgcgcaagggtttggtaaaaaatggagcaatgtctcgatctaatacagtgaatgtagtctcacaggagctgctgcccacttcattggaaatctcaaatgtgtattggccactgtcgtgcagctcagctgaataaaatttgagctgggcaacattgtttttaaaacttattcggtattttttactggcgaccaagggtctcccatctttgtaccatttgggcttcagttctggcgtgcctgccactgtgtactccagtgtggcgggatctcctgctgtcacctggatcagttctgctcgctcaatgattttggcaggttctttaactattaattccccaacagatgtttggcttccagcttcattttcagccaggcacgtgtatttgcctccaaaactaatctgaacatcagggattatcaagactgcaacaccattggaaaagctcattttgatttttccgtcttctctgatgacctcttgacctttcatccatgtgacagaaatgggctctgaccctctcacagcagcttgcagggtaacggtttgtcctcctagtgcaatcaaatcatctactttctttacaaaggttggaggttctttgagtaagtgggttgccatgcagccacacttgccgacttcattagcaacaacacattcatattcaccaacatctgcactattaaacgaaaagatctccagacacacaagagacttctgagaaaacaatctgtattttttactacttcgaatttgtttcttgtctttgaaccagctaatttcaaatggtccagtgcctgagacttcacactgaagtagagcatttgttcctctcactatgtctgcaggctcaagagttttgatgaaagaaggaggttctttgataactatttcagtactgcagctatcactgccgacgtcattcactgcttcacatgagtaactcccactgtcttcaacttttacatccgtaatatcaagtatagcctcagaattgacaaaatacattcggactgtgttactttcactgagttctttgttatttttaaaccaagtaacctggatcacaggtgagcctttcagcttgcaatggaggcgtgctgattcacctgggagcattaaataagagggatccaccttcttcacgaaggatggtggctctctgacagtgactgtggctgagcaggagctgcttccagcctcatttgaagctgtacagacataggttcctgaatctttcagtttggccaaaggaatctcaagtgttgctattttatcttcaaaacagatcttataatctttccctggggggagtttttgcccatctttgctccacgtaactgtgacttttctgtcttcatctacttggcactcaaggtggaccttcttattgatagcggactgcacaggctctaattctttaatgaaatgtggcttatcaatgatgatcaactctgcttggcagatgtctgctccaaacttgttggaagccttacaagaataaactcctctatcttgaatggtaaggtttgagagttctaaaatgtgtttgttttctgcgtcggaaatcctccagttaggtgaaggtgagagtgcagcaccatctttctgccaaatggtttctatcacaggagtccctgtcactgtgcagatgaacttggctgccttacccacaaaagttgtaagggacttaggtctggagagaaaggttggtggatatgcctctgtcacagttagtgtggctgtacagctgacactgccatactcattggaagctttgcatgtatactcgccgcagtcaaccacctgggttctcaggatttcaaggctggagatatactttgaagatcgaatagaacacttgtcactctcataaatttctcggccagctttaaaccactggaaccggacattgggagcactttggatctcacaggtgaatttggctaggtggcccagtgctacttccaggggttcgattttcctcttgatcactggggcagctttcatttccatctcaatctcttgttcaatcctctcatgcaaaattgattcaggagcttccagactcaggttggctgtgcttgatacttggcctacagcattactagcaacaaacgtgtaagttccttcatcttctggataagcttcggcaatttccagttgataagtgtcttcaaattgagtcattctaaagaaccgagatggcttgattttcttgtctttgctgtaccacgacacttttagatctgttccagaaacccggcattgaaaacgggctggctgcccttcagaagtgacagtgtcctgaagcggggtgatgatggcaggtggataaacaggcatttcctgatcaggagacacaacttctggaacttccactgagagtgaagctgatgttgtggcaacaccatagtcattcttggcttcacaggtatagactgccgcatcctctgggaaggcttcaattagcaaaagcgtgtattcttgcccatcatgaagaaatttgcacttgaagccagtggaaagcagctgctcttccttgtaccaggaaattttgggctgtggtcttccggatatcacggcacagaagcgggcaggcttgccagactgcacagtgacaggctggagctcctgcagaacttggggcggttcaggagcattgacatagagagtgacagaactcctgttccttcctgccacaaaggtgtattctcctgcatcgctctgtctggtctcagagataaacattcggtggattcttctttccactacatatttgtgtcgttcttgaacttggaaattgatttcaatgccatctttataccagtgggcatcaacatcgtcttcattgacctcaaattcaacaacagcacgctgtttctcaatgacctgaacctcctttttaatacttcggatgcgaacatctctgccttctacaaagagttttgcagttgacacgttgcctcctgccaccactgtgtacttcccagcatcagacatccgggtggatgggatcagaaggcggtggacatatttctccttctgaatctttattctgtctgtgatctgcagttcctggtcatctttcatccactgtacagtgatgtcaggttcagaaacttcacattcaaacatggctcgcttcttctccagtaccttaatgtccttaatgtgtttcctaaattctatatgacgagcttccacataaagtgtggctgttgatgttgcttttccagccacaaaggtgtagtcagcagcatccccaaagtgaacattcctgatgttcagtgagtgtgtgagctttttggttctcatctggcacttgtcagttgatttgatttccacaccattctttaaccatttgtaagagatgccttcatagttcactgtcacctcaaaagtaatagtgtctttttcttcagcgttgatgtctttcagcatggaagtaatcatgattggggtgactgtcagggtggcactgacttggtcattgccacagacaaatgtgtattctgccgagtcctctgtgctggtgttcatgatgatcagctgatggagttttccctgcacaactatcttgaacttttcactcatctcaatttccacaccattcttcagccacatggaagggacattgaagtgggacacctcacactcaaaagaggcagttttggtctcaggcacctcgatatttttcatggtttttgtaatatgtaatgtctccacaaacagttttgctttgcattccaattgcccgaccacagctgtgtattccccagcatctgagggggagatgttctgcagcatcagcttgtggactttcctttctgagaccagtctgtgtttgtcacttggcttaatttccacactcttatggaaccattttactggaacagtgtcatgggaaacactaacttcaaaggcaacagtggcattttccaaggctgtcacatcctttggctttttaatgatcttgacagtctccacgtgcagtctggcactggctccaagccttccaagcctgaagccataaacagactcatccacgatggcacagtttttaatcctcagagagtaaattgttcctttgacagagatagcatacttttcattggattccagcacaactccatttttgatccactggacacctttgacattagggtgtgtaagctcgacagtgaaaacagcatcctgtgtttctgtcactgtgaggttcttcagagtcttcttaattttgacagcttcaactttgagtttggcagatgttttggaggtggccaccttgtaggtatattctccaatgtcatctaatttggtggcagcaatgataagtctccttttgtggccatcagactcacttctgatgttgttagtcagtggtaggtgtttgccatccctcaaccattcgcctttggaatctgggttggcaacttcacattcaaacacagcttcctgggattcagctacggtctgatctgtgagtggcttggagatggccccacctgccacagtaagttttccagatgtcatattttctcccgcgtaaaatgtgtattttccttcatcatctttcatcatatttagaactgtcaatttatatatttttccatgtgcttcaattttatatttagaactgggcttgatttccttgtccttaaaattccacaggacatcaattccagagtgggacagctcaacctcaaacaccacattttgagtttctgtacaggtaaggtcacgaagacctctgataattttaattttttctacagagagattacagttggtttcaactctgccaactatcagcttgtaaggtccttcgtctgaagcatgagttcggttaatgactagtcgctgtttagtacctttcacaatggcctgtacacggtcatcaggcttgatttgttcatcatttaagtaccacttaacagaagtcacatcagggactgacaccttacattcaagcacagccttggtgccttcaatcacattaacatcttttagaggtgttatcacgtccacactatagacagagacacgcccactggtggagaggccaagggctggaatggtgaaagagtaatttccagcatcttccttagtcatgtcttcaatgagcagcatatgagattgtttgtctatcacaatgtgaaccctgtcactgggctgcacttcttggccgtctttcatccagacgccttccacactttccaaggagactttaacttcaagctgaacaatgtcaccctcacagactttttggtcactaagtccttgtaggatagcaatggggcggggtttcatctttaatttacaggttgtctttttcccgtcgatgacaaagctgtattctccctggtcctccttggttacatccttgaccgtgaggttctgacgtccacgacgagatgtaattgtatatttgccattggatttaagctccacatcattatgataccattttccttctatattttctggggatacaatgcactctaattctcctgaatatgattctggaacttctatgtcctgaagttctttcacaaactcaacaactgcaccttcaacaataagtttagcagtcgttttgacattttcatcttccacaagtacacagctgtaatcttcagcatcagacgtatcaatggtcagtatggagaggaagtgaacctttctgtcagagtgcatcctgtatttatctccctcatgaacctccataccatctttataccatttcactttgacaaatggttctgaagtttcacattcaaaggttgccatagtgtctttttccttagcaacaacatcttgtaattcctgtgtgaaagtgatcaattgcttggcttggacaagtaagaatgcgtgactggaggtttctccagctatgttgatggcttttaccatgatgctggcagagtcctcagcagtcacatctcttatgaccaattcacaaacattgtcttcgggccagtaccagtagatccggtcagaccgttcaattttgacaccatttttgtaccattcacattcggggtctggtttccccacgactctgacccggaagtgtgcatcagatccttggcccactgtttggctctggattctttcgaagatttttggagcctccatactaggacttagttcaatcttgtcaggtttaaaagttggaatcgtgattttgccttcttcggcaagagctttcttttcctcttcagttaactctttggtccagtggagaagttcatcttttgtcttcctgaggagttcctcataggattcatccttctttcgagacttgagctccacagcggtaatggcttcataatagccctcttctgttctgcgcttgaatttactgcgcagctcttccgactcttcaggcactttttcatgggtaattctttcagcccttttcaacttcacaacttctttggtttcagtggtgtcaacaggtctatccactttttgtacttcaaactgaagctttcctggttcatgtacgtgaaactcaggccttggttcaggagctctcctaaggacagacctaaaatcttccctctgttgaatctcaagcttcactttatgctctatcacaccttcaggattttccgcggtgaccttcacttcacctgtgtcatatgatttgcagtccacgatgtccaggtaatggataccatcatagcgaactctgaaccttttgcttttgcggatgagctgtccattgaggtaccagttgactttgggctgagggtagcctgttaccctgcagcggaaccttgcagtctccccttcaagtactctaactggctctgggtacaagacaatgtctggcttttgcttttctttctgatctgttgttacacctgtaagtgcaccttcatgagccattctctctaattcttcaattctctgtaagcctttcctcccctcaggcaattgggattcttccacaagacttttctcatctttaacaataagggtagcagatgtgtgatctgttccatatttgttagtggctctgcaagtaatgataccactgtctctagaatatgcaacgccataatcaaggctgcagtacccaaattcattgatcatacggagcctgttggctgcttcaagtggctttccatcatggagccactccaccaccatcgttgggtcaccaatgggtgttagcctgcattcaaagtgggcaggcccaaagcgcttaagtcttaaggaagtgagttttttcttgaaaaatggtttctgttgtttctctttgtcatagagatcaccttcttcccattgctcttggccatatcgcaaatggaggggctccagttctggggctgcaatctcctttgctctatatgtcccccgtgggatgattaactttctctctggctcaggctctgcaaactcaacttcaacatttactttgcatcttgtagtgtctctgccagctttattaatagcagtcgcagtataccaggcagaatcttggctgacagtggaatcgattttaagggcagcttctcccttggttccttcaattctgattttgggatatttatgaggcacaatgatgtcactgtttttcaaccatacaatgtcagggttggggttacccgtagctctgactttcatttcaagtcgggaaccttcctttatattgacatttttcagtttttctacaaacatcggttttacctgatgttccacagcttccacagttaaaatcactgaaattgaagatctgcctgccctgttttgggcaaccacagtccattccccagaatcactgggtgtggcagggacaataattagtgattgagtaccatcttctttaatgactactttatgggtatagtcattgacaatttgctggccatcatgaaaccagaacgtctctggcataggtctaccaacaacctttaagtcaaatctggcagtttgcccttctaaacatttgaaagaaacaggttttaacacaaagactggtttatatagtctctcaagttgtgactcatctgtctcctccagcctacgtccaggggacattcttgcaggggacatccgtgcaggagacatccttgcaggtgacatccgtgcaggagacatgcgtataggagacctgctcactgaacgtggagagagagatctgattctgctcactggctctagtgtgggaatgtaagtcggagctccaagtggtgcagcaggctccacatacaatttccctgagcaaattgcatttcctttaatattgctggcaaatgcagtgtagattccttcatcttctggaagaacaacaggtatacgcagactagctctgccatcttgtagaaagtccatttggtatctttctccatgtttgatgcgcttgccatctttgtaccaagcaatctttggtaatggatatccagacatcttgcaatgaaaagtgacacccatcccctcaagaattctataattcttgattcttgaatcaaatcctgattcaacagcttcagattcagaaatgtcaactgccatcttttcttctccatcttcttcaagaagttcttctaatgtagtctttattattctatattcaatttctttaataagtctctcttcaaaggaagaaatatggaattcctgatcttctacataagttctgaccactacagtatctttggccattttcttcctaattaaggcttgttctttttcatactctttttcatactcagagtatacaaatccaggtgctgtttctccaactttaggttcttgaacaaatgcagtcacttgtgtctgataaagcatttcttgctgggacttcatcagtaactcataatcagcttcttcaagcaaggaagcagatgcagaagtttctccatgcttattgcgaacaacaatagtgtattctccagcatcatcagcaaaagtcatagaaatcaccagcttgcattcaccggtttgtttgttgtaactcactttgtatctgtatccagtggttagaggaacaccagattttttccagtatacatggggctttgggttgccgccaacttggcatccaaacaccacgctcccaccttccaccagtttctggaccactggttttgtaataaagtaaggcgcggcaggttctccaggccctgcttgttcctctgtgaggctagtatcagtcataaccacatctcttgactcaacaaagcgtttctcttctgtagtaaatttctcagtcacggctgtggtttccttttcaaattcttctgacacctgcacagccagatagcaggatgtgctgacggttccagcctcatttacagcactgcaagtaaatcgcccgctgtcttccgcaaatgcttcgcgaatcataagacgagcaattccactctggaaggttatctggaagtcaatggaactttcgatttggtagtcttccctgtaccatgtcactgtcggggatgggtatccagagatgtggcactccaaggtgacagattcaccttctatgacagtcacattttttaagcccgagaccaaagttggtggagtaacaggaatttcaacaggtgctggtactcttgctgtttctgttaccttggcttcgcgtccgtgcagtacttcaaagcgctcttcacggacggtggtgccagtgatgctcacccctacttcctttttcacctcaacgccagcttcactcttgtaagtatctggtgtgtcagcgaaggggaactgtggcaagggtgtgggctctgcccttactctagtctcactgggcttcacagtaggagccttcaccgatttggtgatcttctgagcagaagatgtggctgacaactctttttgtaatgtggcaatagcactaccggctattgatgcctcatatccatgttctgtcttaggaacagaaatttttgaaacagtaaagtgagggctagctgtgcgggggcgtttatccacatggactaatctttccgttgttagatctgtagttttcttgatctgtgatgatatgtgcattcccttttgatcagtagttttgatatgagtctcagaaggagcctggattactctaggcttgactgctttagggacaacgtggggttctgaggctggacgttggggaggctcagctacctttgcggcggaaatgcgttccttatatccgtactccaaagtggtctgctgagcataggattcttcaagatgcccaggctctctgggctctctgactcgggcctggtctactgcagcaacaactgttgctacagcttcagccttttttccaacgtccacctttccatgggtaacttggatttgttcttgtctagtagccatagtttctctagttctcagtattgtttcttgttctttggctttagcagtagcaactgctattgtagacaaggcagttttctcggcttcctttctcatcttctcctgagttatttgcacttgttctcttttggtagtaatgccttctctacctcttgatactaaatcttgttctttgactttgggtgtggcaactatgactttaggtacaactgttttcctagtttccttcattatcttttcataacttaggtgcatttgatcttgttgtgtggtagtttcttcttgagctcccgggactgtttctagttttgtggactttgcagtggcaactaccaccatggatgcagcagttatctcagtttcctgtcttattgcttcttgagttacttgtttctgtttcttagtaatttcttcagaaattctagtttcttgttctttggctttagctgcggaaattactacctttggtacaaatgttttttcagtttcttttcttatctgctcatgagttacgtgcatctgctcttgctttgtggtaattacttctttggttcttgattttaattcttgttccttggctttatcggcggccactactaccttagttacagcagtcttctccgcttcctttcttacctgttcttgagcaggttggatgtgcacagcagtcgtggttgtcctctgagcagtctgctctacagcgctgatcactggttctctcactctggccatatcaacggcagcaacaacagtcgcaacagctgcacttttgtcagcatcttgtttcacctctttagcaccagtggcaacagcctctgctgcgtagctagcactggccgacacactggcggcagcacccgcagcaccactgatggtcacttgctcctggacaccgtatctcccttcccatctctcttctgtcctgatctgagtagaggttgtcagcgttgtctctctcatctcagcctcagatgaggaggccacgtagccctcttgcttccaagggggaggcacttcaggacctgtggccacggtggatgcctgagtcttacgcatgagcaatggagacctaacagacctgatgggggatgtggagattcttgctgctggagacacggacctgaccggagatggggtcggtgcccgcacgtgtctgaccggggaaggggagtgtcttatgggcgatggggactgctgccgagccagctgtgctttggcagcaatagacggtggtgttggggatcttgactttggcttcggaggaatcctgggaggtgttttatgtggcagctgttgcccagcggcaccatctatgaccatctcaactgttgcaattgatctggcatcaaagtgggcttcaatcttcttttcaattcgggtttgtcttgattctgagatctgagcagtcgaaacaattgtctttgtctttttagcaggtacttcttcttcaccttgaaccagtaattcagcagtcgaagtagctcttccaacgctattggtggcatttactgaataggtccctgagtcctcagggtatgcttctgcaatcagtaagctgtagaggtcgccttcttgtgaaatttggaaatcaagggagctctggatttcggctccatcccggtagaacttcaccacaggtgtagggattccagtcactctcacttggagtctcacttggcttccttgtctcacggtcatgctctgcagtcgttgaacgaagttgggtggtgctgtctcagctttcacgagaagctcagcagtactagtcgcttgtccagatccattggtggctttcagggaatatcgtccactgttggctttagtcacggcggggatcgtcagtttagcgcggccatcgctaaaggagatctgcacgccgggcagagtggaagtggaaatcacctggccatccctaaaccagctcacctcaggaactggaaaaccactaatgtgagcctcaaaggttgcggtactaccctccagtaccacaacgctttgtaacggctgcgtaaacgtcggtgcttgagttgtcatctttctaggcactctgatttctcaagagtgcctaaaaagggtgggactaagcccaaggttgcttctgaaacgacgtcctatggagagttggtttttctgaccatctccgacatgaatcggtgagcctctaatcctaaaaacaaaactacacagtcaagactgtgtagttttgcttttctatgcaatccctacacccgaggcgaggctgggaatgcacgactgctc

SEQ ID NO: 8419 - RNA, 1970 nt, Homo sapiens
  source 1..1970: mol_type = other RNA
aaaactgtaattacttttgtacctacctaatactttgtattctatccttcttttactacatcgttttatctgtccagtcacaaagttaagaggttgcccctacaataagactgttcacatagaacctagctattagaaacactagctggtgggatcatccttgcatccattagggaaggaaggccagtgaggagcactggcatttgttggaatgttacactattctggcacttggcaacgttattcccatggattctaaaaccagggatcagccattctaccagtacctgctgcagaagatcatctttttgaatgcgtccctgagctctgggctccggaaggcatatatgaaggggtcaatgacggcattgcacatgatcaacatgccgttcacctggaagagagacatgtagcaggcgcagtaggggttacttgggcagaatgtcatcaagaggacatgaagcacaaagggggcccagcagaagatgaagaccccgagcaggatggtcagtgtgatggcccctttcatgttggctctggggagggtggagatcttcctggtgtgggatcgagccagcaggaacatgtgcacatagaggcacaggatgaagaccagcatcagcgggaacagcgacgtgaaggtgatcactgtgggcacatgatgggagaagatcaccatggtgatgccagtccccgtgcagaacgtccagatgaccgtaagcaccaccacagtgcggcgcatggtcacgatgctgtggtaccgcagtgcgtggaagatggtgatgtagcggtccgcagcaatcacagacaggctgaagatggagccaagcagggagaggacaaacagggagtcgatgatgtcatcggctgtggtttcaaaactgccacgtggcttgagatagcccatgtttctcaatatgatcaggatattttccaagatcttatataggctgcccagcatatcagatatggccaagctacagatgaaaaagtacatgggtgcctggagattcttattcttgaacacagccagcaggacgatcagattctccaaaactccaacaatggaaattgtgaaaaatatctcctccggcaaaaccacacgaggacagtcggaattatttcttgctgtgttgttgatgttttcatacgagttgataatgtgcttcatttctcctgcttgtggttaaggcggggatgttacttggacttgacttcacggaaaacttgattgattcttcaggatcttttcttccttgtagcacttgctggagatctaagttaaaatctcccaatcacagctctgtacaatctgtttccatgctgttttctcactgtattttctagcattctcctgtgtagaacacgcattccagctggcccaggcctcttattgtctctaagatgccttgctcatttttgcctgtcacattttttagtactgctctccctctgaacttttcgaatctttcctctgtctaaatcatatatttgtttaagcccaaacaagatcaaatgttttgaaggtctctggctccatatcaacccacgcgacctgtctgtgccatcacaacaccacagcgtgttttgttcttggcttgcgtgtggcaggcgacactctctgctcttgggaaaagtctgctttaagtgtagatgtcttgtctcctgagcagccgggcagtgccctgaaaggttggcaaatttgacaccctcttctttgtatcttcccgggtaactgaggtgcacggtaataatttatggatgccttgggatgtgacaatcagcaacttgaacaacccagggtaatctgaatgattcacagcctgtgcttcttcagctctgaagcaggaactttctgggcaaaatgaatgagaaggaatgagctcggagagaaaagcaagcaagtggaccttgggccgggaagggccggaacacatgcatcaccggagatacagctagattgttatcat

SEQ ID NO: 8420 - RNA, 1348 nt, Homo sapiens
  source 1..1348: mol_type = other RNA
aaaactgtaattacttttgtacctacctaatactttgtattctatccttcttttactacatcgttttatctgtccagtcacaaagttaagaggttgcccctacaataagactgttcacatagaacctagctattagaaacactagctggtgggatcatccttgcatccattagggaaggaaggccagtgaggagcactggcatttgttggaatgttacactattctggcacttggcaacgttattcccatggattctaaaaccagggatcagccattctaccagtacctgctgcagaagatcatctttttgaatgcgtccctgagctctgggctccggaaggcatatatgaaggggtcaatgacggcattgcacatgatcaacatgccgttcacctggaagagagacatgtagcaggcgcagtaggggttacttgggcagaatgtcatcaagaggacatgaagcacaaagggggcccagcagaagatgaagaccccgagcaggatggtcagtgtgatggcccctttcatgttggctctggggagggtggagatcttcctggtgtgggatcgagccagcaggaacatgtgcacatagaggcacaggatgaagaccagcatcagcgggaacagcgacgtgaaggtgatcactgtgggcacatgatgggagaagatcaccatggtgatgccagtccccgtgcagaacgtccagatgaccgtaagcaccaccacagtgcggcgcatggtcacgatgctgtggtaccgcagtgcgtggaagatggtgatgtagcggtccgcagcaatcacagacaggctgaagatggagccaagcagggagaggacaaacagggagtcgatgatgtcatcggctgtggtttcaaaactgccacgtggcttgagatagcccatgtttctcaatatgatcaggatattttccaagatcttatataggctgcccagcatatcagatatggccaagctacagatgaaaaagtacatgggtgcctggagattcttattcttgaacacagccagcaggacgatcagattctccaaaactccaacaatggaaattgtgaaaaatatctcctccggcaaaaccacacgaggacagtcggaattatttcttgctgtgttgttgatgttttcatacgagttgataatgtgcttcatttctcctgcttgtggttaaggcggggatgttacttggacttgacttcacggaaaacttgattgattcttcaggatcttttcttccttgtagcacttgctggagatctaagttaaaatctcccaatcaccttcagctctgaagcaggaactttctgggcaaaatgaatgagaaggaat

SEQ ID NO: 8421 - RNA, 1377 nt, Homo sapiens
  source 1..1377: mol_type = other RNA
aaaactgtaattacttttgtacctacctaatactttgtattctatccttcttttactacatcgttttatctgtccagtcacaaagttaagaggttgcccctacaataagactgttcacatagaacctagctattagaaacactagctggtgggatcatccttgcatccattagggaaggaaggccagtgaggagcactggcatttgttggaatgttacactattctggcacttggcaacgttattcccatggattctaaaaccagggatcagccattctaccagtacctgctgcagaagatcatctttttgaatgcgtccctgagctctgggctccggaaggcatatatgaaggggtcaatgacggcattgcacatgatcaacatgccgttcacctggaagagagacatgtagcaggcgcagtaggggttacttgggcagaatgtcatcaagaggacatgaagcacaaagggggcccagcagaagatgaagaccccgagcaggatggtcagtgtgatggcccctttcatgttggctctggggagggtggagatcttcctggtgtgggatcgagccagcaggaacatgtgcacatagaggcacaggatgaagaccagcatcagcgggaacagcgacgtgaaggtgatcactgtgggcacatgatgggagaagatcaccatggtgatgccagtccccgtgcagaacgtccagatgaccgtaagcaccaccacagtgcggcgcatggtcacgatgctgtggtaccgcagtgcgtggaagatggtgatgtagcggtccgcagcaatcacagacaggctgaagatggagccaagcagggagaggacaaacagggagtcgatgatgtcatcggctgtggtttcaaaactgccacgtggcttgagatagcccatgtttctcaatatgatcaggatattttccaagatcttatataggctgcccagcatatcagatatggccaagctacagatgaaaaagtacatgggtgcctggagattcttattcttgaacacagccagcaggacgatcagattctccaaaactccaacaatggaaattgtgaaaaatatctcctccggcaaaaccacacgaggacagtcggaattatttcttgctgtgttgttgatgttttcatacgagttgataatgtgcttcatttctcctgcttgtggttaaggcggggatgttacttggacttgacttcacggaaaacttgattgattcttcaggatcttttcttccttgtagcacttgctggagatctaagttaaaatctcccaatcaccttgaataaatgtcatcccacatgaactgtgcatttctggtaatgtgaagttagagaaatggaaagacacaggcagat

SEQ ID NO: 8422 - RNA, 2688 nt, Homo sapiens
  source 1..2688: mol_type = other RNA
aaaagcacttttctgtctcccagaaatatgaaaggagatgggctgaaaacattaaatcaaaactaataatataataagagcttcagttctttgttacaaaatgtacgtgcttcaaaaaggcatatttttttaagactgagtctcactctcacccagactggagtgcagtggtgcaatctcagctcacttcaacatccgcctcccaggttcaagtgattctcctgcctcagcctcctgtgtagtgagattacaggcgagtccaccatgcctagctaatttgtgtatttttagtagagatggggtttcaaccatgtaggccaggcttgtcttgaactcctgacctcaggcgatccacccggctcagcctcccaaactgctaggattacaggcgtgagccactgtgcctgatcaaaaaaggcataattaaactatgaatattctttctaaacaatgggcaaagtcacagtggattaactttcacctatgttaataatcaaattctagttctgacaaaggccccacgccaacagtgattacaatgaccaaaaatatttacttgttggttctcattcagttctatagatttctccttaatgtgcaggaaagcatctgataatacttttgtaaagtggtctttattgatttaacataaaacttatagaatactccagagaaaacatgtgatataaatgtcattgttagagccatcaaaataattcttattttcattaataatttgtggaggaaattattgagaaatgttgattctcttatcagagctcaggaggagttaatggtgctaactgggggtggtggaaatagtcccgtgagaagcagaggagccaaatctacctcctcacactgatttggtcacctcctttatattcccaagtataacactctacacagacaatgagagagctcaatgcatgtacagaatccccggttatttatgcagtccattggatgaagcccatcttcatttcagagttctattcacaaagtaatttgaggtctctggtgttctcaggcacagatttcttgaagagcaaagcagaagtccttaggaaaattcaggctccacttacggtgccatcccttgactcaacctttagaacaacgggtttttctggttgaagaagtcctcctaagcttaatttcagggggatctgtgtttctttacaaggtttgaaggagaagttctgaaggactctgattagagcaagtttcatgttcatgagagcaaacctcatgccaatgcagtttctgggtccacttccaaagggtgtgtatatgtaaggatctatgttgtccttgttcttcttgctgaatctttcagggaggaacttctcaggctctgtccagtactttgggtcacggtgaagagcatagcttggaatcatcaccaccacccctttgggaatgaacatcccattgatctcaacatcttttttgcagaccctctcaagtctcatagcaattgggaataatctgagcgtttcattcaccaccatgtcaagatactccatctgtagcacagtatcataggtgggtggtgccttattgggtaaaactgcatcaatttcctcctgcagtttctgctggacatcagggtgagtggccagttcatacataatgaaggagagaacactgctcgtggtttcatagccagcaaaaataaagataattgattgggccacgagctccagatcggacagagctttgtgggactcagtttcttttgaattctgagagtcaatcatcagctgaaggaaatccactcggtgcttttgtgtatcttcgaggcgactttctttcatcctttttacagattttcttaaaaaatttgtaacttctcttggaaacacacagatatttaatacttcaagaattgggatgaggaatggaaagactgttattgagagaaagaatggatccaaaaaatcaaatcttaaaagcttcttggtgttttccacaaaggggtcttgtggattgttgagagagtcgatgttcactccaaatgatgtgctagtgatcacatccatgctgtaggccccaaagacgtctttcaaggtgacaggcttgcctgtctctgcttcccgcctcagatttctcaccaacacatctccatactgggcaatgatagggaccatctccttgagttttccactggtgaaggttggagacagcaatgatcgtaatctcttccattcttcatcctcagctatagagatggcacttttcataaatcccactggaccaaaaggcctccggtttgtgaagacagaataacattctttcactagcactgttttgatcatgtcaggatctgtgatagccagcacaggctgttgaccatcataaaagccccacacttttccatactttttatgacattccatgtcaaacatacaaaagcccttatggtaggacaaaatatttcccaaaaaaggcagaggtgtgggccctggaattccaagcttcttaaaaagtccatgtgaatgggttccatatagatagaggagcaccaggctgacagccaggagaagccaggtttccatggccaagtctgggatgagagccatcactactttccttacttatctctctcctctgagtcttcctttcagctctgtgttgctctttgctgggctatgtgcatggagctttcctgccctgcacagcagt

SEQ ID NO: 8423 - RNA, 2685 nt, Homo sapiens
  source 1..2685: mol_type = other RNA
aaaagcacttttctgtctcccagaaatatgaaaggagatgggctgaaaacattaaatcaaaactaataatataataagagcttcagttctttgttacaaaatgtacgtgcttcaaaaaggcatatttttttaagactgagtctcactctcacccagactggagtgcagtggtgcaatctcagctcacttcaacatccgcctcccaggttcaagtgattctcctgcctcagcctcctgtgtagtgagattacaggcgagtccaccatgcctagctaatttgtgtatttttagtagagatggggtttcaaccatgtaggccaggcttgtcttgaactcctgacctcaggcgatccacccggctcagcctcccaaactgctaggattacaggcgtgagccactgtgcctgatcaaaaaaggcataattaaactatgaatattctttctaaacaatgggcaaagtcacagtggattaactttcacctatgttaataatcaaattctagttctgacaaaggccccacgccaacagtgattacaatgaccaaaaatatttacttgttggttctcattcagttctatagatttctccttaatgtgcaggaaagcatctgataatacttttgtaaagtggtctttattgatttaacataaaacttatagaatactccagagaaaacatgtgatataaatgtcattgttagagccatcaaaataattcttattttcattaataatttgtggaggaaattattgagaaatgttgattctcttatcagagctcaggaggagttaatggtgctaactgggggtggtggaaatagtcccgtgagaagcagaggagccaaatctacctcctcacactgatttggtcacctcctttatattcccaagtataacactctacacagacaatgagagagctcaatgcatgtacagaatccccggttatttatgcagtccattggatgaagcccatcttcatttcagagttctattcacaaagtaatttgaggtctctggtgttctcaggcacagatttcttgaagagcaaagcagaagtccttaggaaaattcaggctccacttacggtgccatcccttgactcaacctttagaacaacgggtttttctggttgaagaagtcctcctaagcttaatttcagggggatctgtgtttctttacaaggtttgaaggagaagttctgaaggactctgattagagcaagtttcatgttcatgagagcaaacctcatgccaatgcagtttctgggtccacttccaaagggtgtgtatatgtaaggatctatgttgtccttgttcttcttgctgaatctttcagggaggaacttctcaggctctgtccagtactttgggtcacggtgaagagcatagcttggaatcatcaccaccacccctttgggaatgaacatcccattgatctcaacatcttttttgcagaccctctcaagtctcatagcaattgggaataatctgagcgtttcattcaccaccatgtcaagatactccatctgtagcacagtatcataggtgggtggtgccttattgggtaaaactgcatcaatttcctcctgcagtttctgctggacatcagggtgagtggccagttcatacataatgaaggagagaacactgctcgtggtttcatagccagcaaaaataaagataattgattgggccacgagctccagatcggacagagctttgtgggactcagtttcttttgaattctgagagtcaatcatcagctgaaggaaatccactcggtgcttttgtgtatcttcgaggcgactttctttcatcctttttacagattttcttaaaaaatttgtaacttctcttggaaacacacagatatttaatacttcaagaattgggatgaggaatggaaagattattgagagaaagaatggatccaaaaaatcaaatcttaaaagcttcttggtgttttccacaaaggggtcttgtggattgttgagagagtcgatgttcactccaaatgatgtgctagtgatcacatccatgctgtaggccccaaagacgtctttcaaggtgacaggcttgcctgtctctgcttcccgcctcagatttctcaccaacacatctccatactgggcaatgatagggaccatctccttgagttttccactggtgaaggttggagacagcaatgatcgtaatctcttccattcttcatcctcagctatagagatggcacttttcataaatcccactggaccaaaaggcctccggtttgtgaagacagaataacattctttcactagcactgttttgatcatgtcaggatctgtgatagccagcacaggctgttgaccatcataaaagccccacacttttccatactttttatgacattccatgtcaaacatacaaaagcccttatggtaggacaaaatatttcccaaaaaaggcagaggtgtgggccctggaattccaagcttcttaaaaagtccatgtgaatgggttccatatagatagaggagcaccaggctgacagccaggagaagccaggtttccatggccaagtctgggatgagagccatcactactttccttacttatctctctcctctgagtcttcctttcagctctgtgttgctctttgctgggctatgtgcatggagctttcctgccctgcacagcagt

SEQ ID NO: 8424 - RNA, 370 nt, Homo sapiens
  source 1..370: mol_type = other RNA
aaaagcacttttctgtctcccagtcaccaaccatgttgggtgtgggctccagagatgcttggagtaaatggcactgtccttgtcatctcctgcatgtcttggctcaaatgttaccttttcagtgaaaacttcctgttcagccctattttaaatcacacttcttcccacttgttgggtgctcccaatcccttttcttctttcttctccatggcacttaccaccatctgaacttggggaatggatgccacaagctcatctatctggacctctctggctgcacccaggtttgtctttcagtcttctctttgctgcggtgtgtgaggaagttctccagagaatgggctgcattcagccctcacgttatactaat

SEQ ID NO: 8425 - RNA, 525 nt, Homo sapiens
  source 1..525: mol_type = other RNA
aaaagctgggctgagaggcgactggtgtctaatttgtttgtctctccaactcagactgcctggcccacagccacagctcagccccgagctgctctacatctgtgcacagaatgtcagagagtgtttctttggagaatatctttaagtgctctcaaatggaactacagagccatcagctatgtcccctccgattgcagtaagaactgaatggaagagaaggaccttcagaataaagccagggaagcagaaaccactgaaaaccttctctctggaaccaaccaggcagggcccaagcagtgttttgaatctccttagcctatcattcataagaacacaaactaattatctgcaatccctttggatatcatttcaaacaataaaaataaggacacccgttcattaagtggacttgtctcggtttactgctcccctgcaccttattagaagggccaatgctttgccattattctgctgaacacaggccacagctgtcttcgtaagtcaacacaaacctctccaaccccc

SEQ ID NO: 8426 - RNA, 778 nt, Homo sapiens
  source 1..778: mol_type = other RNA
aaaaggcattgtggtttttggtctcgcattttccctgccttctgatggcttagcaggggaccctttcttctttggctggtggggcttctctggatcagtaatgtccacatgcggcttctgcagcaaggttttctcttttgctgatactgtaactcggggggctctgttttcaaaggaatgagaggcctctggttttcgaagcccccctctgcctttgctcaccactcgaggagtgacctctgaaacgtcagcctcatcatcagattcagaatcagaggagctggaagaggatgaagacgaaggcgacgtcactttccgacccacctgacgagcttctgaatcagagccctgttttctgaatggagacagaactttctgtggaaactctaccaaagtctttcttgacaaaaatttcggaaccccttcatctgtgaatagcacgctgccactgggactgggactagctaccttcctgcccttattcacagctggcgggtaagaactgggtgaagataagtttttagacaattcagctgctgtctgggtggctaggagcttgcccctctcctttggttccactacattttttggtggactttgcttcttggaattctgtggctgacccttttcactcttccctgattccgcagacaaagaaaccgtagaagcaagtcctcgaaacacctgggcttcctggagcatagtcttcagcgccccggctcgtccttgccgcagcaaacacggggcagccatggcggtgacagcgggcgcaccaagc

SEQ ID NO: 8427 - RNA, 816 nt, Homo sapiens
  source 1..816: mol_type = other RNA
aaaaggcattgtggtttttggtctcgcattttccctgccttctgatggcttagcaggggaccctttcttctttggctggtggggcttctctggatcagtaatgtccacatgcggcttctgcagcaaggttttctcttttgctgatactgtaactcggggggctctgttttcaaaggaatgagaggcctctggttttcgaagcccccctctgcctttgctcaccactcgaggagtgacctctgaaacgtcagcctcatcatcagattcagaatcagaggagctggaagaggatgaagacgaaggcgacgtcactttccgacccacctgacgagcttctgaatcagagccctgttttctgaatggagacagaactttctgtggaaactctaccaaagtctttcttgacaaaaatttcggaaccccttcatctgtgaatagcacgctgccactgggactgggactagctaccttcctgcccttattcacagctggcgggtaagaactgggtgaagataagtttttagacaattcagctgctgtctgggtggctaggagcttgcccctctcctttggttccactacattttttggtggactttgcttcttggaattctgtggctgacccttttcactcttccctgattccgcagacaaagaaaccgtagaagcaagtcctcgaaacacctgggcttcctggagcatagtcttcagcgccccggctcgtccttgccgcagcaaacacggggcagccatggcggtgacagcgggcgcaccaagcagggccacagcagctgcgcgcgcacccgcgcctgaaca

SEQ ID NO: 8428 - RNA, 771 nt, Homo sapiens
  source 1..771: mol_type = other RNA
aaaaggcattgtggtttttgtccagagtgaatgtcctagggatctggtaggctgagagtggggtggccggaacatccatattgtctaccaggaggtccccgaactccctgcacagggtgttgctgggcgtcttgaaggtgtacacatcctcattatctgtctcggagcctgtgaggctgcccttggtgtggccatgggaggccaggctgcgggggaggtcgtaggtactgtctctgaattctgtattgtgccggctcggcttgggaaggctatagaagccatggacttgaccactgatcccgttgacacagtgtccattgccctgggcaagtttttgtacagctgtgtcactcctcatgagaaaagaggctctggtgccctgagagaagctggcactcctgtgctctcctcagcctgattgaagccacagatctggcagatgctctggacccacttattcatgtcctcttctgtctcagccaccaggtaaaaggtgcgttcactggtcttgatgtcaaacacaaaactatcctgcagctccttcttgttaaaggtcaggcctgcatctacctgctcacagaagttcaggttgatgatccgcagaggcttcttggagtgatcgttcttgtagtattccagaacatctgggtcaccgctcatccggccactccgcaggataaaccagcgtttcttccaggccagggaaaatccatcagagagttgataattgagggagacttctttttgaggagggagatgagggatcaggag

SEQ ID NO: 8429 - RNA, 1118 nt, Homo sapiens
  source 1..1118: mol_type = other RNA
aaaaggcattgtggtttttgtccagagtgaatgtcctagggatctggtaggctgagagtggggtggccggaacatccatattgtctaccaggaggtccccgaactccctgcacagggtgttgctgggcgtcttgaaggtgtacacatcctcattatctgtctcggagcctgtgaggctgcccttggtgtggccatgggaggccaggctgcgggggaggtcgtaggtactgtctctgaattctgtattgtgccggctcggcttgggaaggctatagaagccatggacttgaccactgatcccgttgacacagtgtccattgccctgggcaagtttttgtacagctgtgtcactcctcatgagaaaagaggctctggtgccctgagagaagctggcactccttgcattttctgctcttcggcttatgcactggtgcaagtagagatactcctgaggtgcgctggtggacaaggtgggctgcatgtggtttgacacagggggttcaaacgtgaacagagttggctggctggagtgtgatggggctgaggacttgcgctctcggagaaggtgctggctagagctgctgagctcagctggagaagagcgggggccatgaccggctgaggaaacatttctcagggagtctgtgctctcctcagcctgattgaagccacagatctggcagatgctctggacccacttattcatgtcctcttctgtctcagccaccaggtaaaaggtgcgttcactggtcttgatgtcaaacacaaaactatcctgcagctccttcttgttaaaggtcaggcctgcatctacctgctcacagaagttcaggttgatgatccgcagaggcttcttggagtgatcgttcttgtagtattccagaacatctgggtcaccgctcatccggccactccgcaggataaaccagcgtttcttccaggcatagcgcctcaacttcttctcgggaggcgatttcctcagccagccggtgcacaccacgtcgccgccgccgctcatgctgccggcctggagccccccgccgggtcgcgcggacgagggcgcgggctcgggcagctggggcagcggccggcggtgcgcagctcgcgggaggccaggg

SEQ ID NO: 8430 - RNA, 1103 nt, Homo sapiens
  source 1..1103: mol_type = other RNA
aaaaggcattgtggtttttgtccagagtgaatgtcctagggatctggtaggctgagagtggggtggccggaacatccatattgtctaccaggaggtccccgaactccctgcacagggtgttgctgggcgtcttgaaggtgtacacatcctcattatctgtctcggagcctgtgaggctgcccttggtgtggccatgggaggccaggctgcgggggaggtcgtaggtactgtctctgaattctgtattgtgccggctcggcttgggaaggctatagaagccatggacttgaccactgatcccgttgacacagtgtccattgccctgggcaagtttttgtacagctgtgtcactcctcatgagaaaagaggctctggtgccctgagagaagctggcactccttgcattttctgctcttcggcttatgcactggtgcaagtagagatactcctgaggtgcgctggtggacaaggtgggctgcatgtggtttgacacagggggttcaaacgtgaacagagttggctggctggagtgtgatggggctgaggacttgcgctctcggagaaggtgctggctagagctgctgagctcagctggagaagagcgggggccatgaccggctgaggaaacatttctcagggagtctgtgctctcctcagcctgattgaagccacagatctggcagatgctctggacccacttattcatgtcctcttctgtctcagccaccaggtaaaaggtgcgttcactggtcttgatgtcaaacacaaaactatcctgcagctccttcttgttaaaggtcaggcctgcatctacctgctcacagaagttcaggttgatgatccgcagaggcttcttggagtgatcgttcttgtagtattccagaacatctgggtcaccgctcatccggccactccgcaggataaaccagcgtttcttccaggccttttcatgatgataccaaaggtctaattccctcacttgtctctctattgctagcctcgcctttgtctcagttactcctctcttcagggatcttcttcatcccaccacttctcaaaatttctgatccaagttatcatctgaatggctaagtgcaatgttt

SEQ ID NO: 8431 - RNA, 1785 nt, Homo sapiens
  source 1..1785: mol_type = other RNA
aaaaggcattgtggtttttgtccagagtgaatgtcctagggatctggtaggctgagagtggggtggccggaacatccatattgtctaccaggaggtccccgaactccctgcacagggtgttgctgggcgtcttgaaggtgtacacatcctcattatctgtctcggagcctgtgaggctgcccttggtgtggccatgggaggccaggctgcgggggaggtcgtaggtactgtctctgaattctgtattgtgccggctcggcttgggaaggctatagaagccatggacttgaccactgatcccgttgacacagtgtccattgccctgggcaagtttttgtacagctgtgtcactcctcatgagaaaagaggctctggtgccctgagagaagctggcactccttgcattttctgctcttcggcttatgcactggtgcaagtagagatactcctgaggtgcgctggtggacaaggtgggctgcatgtggtttgacacagggggttcaaacgtgaacagagttggctggctggagtgtgatggggctgaggacttgcgctctcggagaaggtgctggctagagctgctgagctcagctggagaagagcgggggccatgaccggctgaggaaacatttctcagggagtctgtgctctcctcagcctgattgaagccacagatctggcagatgctctggacccacttattcatgtcctcttctgtctcagccaccaggtaaaaggtgcgttcactggtcttgatgtcaaacacaaaactatcctgcagctccttcttgttaaaggtcaggcctgcatctacctgctcacagaagttcaggttgatgatccgcagaggcttcttggagtgatcgttcttgtagtattccagaacatctgggtcaccgctcatccggccactccgcaggataaaccagcgtttcttccaggccttttcctgtgctgaagccattcgccttccagcatcttcaatctaatagactgaagtgggctgaaatggctcttaggagagaactggggctagtcttttccttaatgctgcctcttcaccactactcaagcagcagcagcattactggtaattacatcattataccataatggaacacatgcggtgcaagtgaaacagcctggcggctccccagttgaggagagaagaaaaggactccactttcactgttcaatttctattaactctctaggttctggcttattttcaaaggcaaaccacctttatgacatttcacaatcttaaaacagagaccacagacgtggagcttacttaaagatcaggagtgaagttaatgcattagtgtaatagagatcctccacgggaatagggattaggagatgtgggtccagttctggctttgctaaaagcactttatgtgacttgagggaaaccatatttacatcttttaggtttcagtttcctcatctataaacaacagcaaagtttctgggcaggggatcccaaaacgtccctgtgggcaatttgagattggcacgaatgatcacaagagctctcccacccaactgtaaccttctgttatcaaaaaagattccatgaacaggagagacaggagtgaaatagtatttggaaggccaactctatttgatcttcaccagttaaccagatgagaattcttgcctctactctgacccatgtatcagtgtcaggtcatctttatcaacatccacagcaacatttcaagagaccaagctcaggcggggcatgatggcgcatgcctgtaatcccagtgctttaagagg

SEQ ID NO: 8432 - RNA, 1165 nt, Homo sapiens
  source 1..1165: mol_type = other RNA
aaaaggcattgtggtttttgtccagagtgaatgtcctagggatctggtaggctgagagtggggtggccggaacatccatattgtctaccaggaggtccccgaactccctgcacagggtgttgctgggcgtcttgaaggtgtacacatcctcattatctgtctcggagcctgtgaggctgcccttggtgtggccatgggaggccaggctgcgggggaggtcgtaggtactgtctctgaattctgtattgtgccggctcggcttgggaaggctatagaagccatggacttgaccactgatcccgttgacacagtgtccattgccctgggcaagtttttgtacagctgtgtcactcctcatgagaaaagaggctctggtgccctgagagaagctggcactccttgcattttctgctcttcggcttatgcactggtgcaagtagagatactcctgaggtgcgctggtggacaaggtgggctgcatgtggtttgacacagggggttcaaacgtgaacagagttggctggctggagtgtgatggggctgaggacttgcgctctcggagaaggtgctggctagagctgctgagctcagctggagaagagcgggggccatgaccggctgaggaaacatttctcagggagtctgtgctctcctcagcctgattgaagccacagatctggcagatgctctggacccacttattcatgtcctcttctgtctcagccaccaggtaaaaggtgcgttcactggtcttgatgtcaaacacaaaactatcctgcagctccttcttgttaaaggtcaggcctgcatctacctgctcacagaagttcaggttgatgatccgcagaggcttcttggagtgatcgttcttgtagtattccagaacatctgggtcaccgctcatccggccactccgcaggataaaccagcgtttcttccaggctgtatgccagaatcaggtaggtgttaagaagagatatttgagttaattcttgtcaagcagatgtggggttgaagtcagacagaaggtaatagcgcctcaacttcttctcgggaggcgatttcctcagccagccggtgcacaccacgtcgccgccgccgctcatgctgccggcctggagccccccgccgggtcgcgcggacgagggcgcgggctcgggcagct

SEQ ID NO: 8433 - RNA, 2767 nt, Homo sapiens
  source 1..2767: mol_type = other RNA
aaaaggcattgtggtttttgtttgcttctttgtttttgggatggagtttcgctcttgtcgcccaggctggagtgcaatggcatggtcttggctcactgcaacctctgcctcctgggttcaagagattctcctgcctcagcctcccgagtaccagggattacaggtgcccaccatcttgcctggctaatttttgtgattttagtagagacaggtttcgccatgttgaccaggctggtctcgaactcctgacctcaagtgattcgcctgcctcggcctccaaaagtgctgggattacaggcatgagccaccacacctggctaaatgtatcgtgttctaaacctgcttcattcactttggctgtgactggagacaacaaacattttgggaaataaatcatgctcatgtcatagacatgtggagtctcagcatggaccccaatctctttccactttaaggttttggagatactagatctgcagccttcattagccagccaagggggttccctagtggagaaagagattggctgtaaaaatgccgtgagtcactagtttgactgtgtcaaagcctgtgaggcagcttttgttttcaccttttcctccaaatgtttgcttcttgtctgattgacaggaggccctaaaactcatgactggtggtcactgagctctcaccctgcttggctattgtagataggcaatactaaactggggaatgcagctacagggcaatagtattacttacctggtatagatccagccttcatgtttttctgacatgtaccaagttaacattagagaaacattccaaaaggtattaataaaatgaaaagttttaccaaaagcaatgaaagttcactgctatggtctaaatgtttgtcctccccaccccaaaatgcatatgtcgaaacctaatccccaaggtgatggtattaggaggtaaggccattgggaggcgattaggtcatgagaccagagccctcatgaatgagattagtgcccttgtaaaagagaccccagaggactagctcaccctttctatcatatgaggacacagcaagaaggtactatctatgagccagaaggctggccctcagcagacactgaacctgccagcaccctgcgcttggacttcccagcctccagaactgtaagaaatgaattcctattgtttataagccattctgtttatggcgttttgttatagcagcctgaacaggctaagacactcacatcatgtctgtattttatgattgatttgagggcatccttagaaaactaaatataattgactaaaattgaatgtggactaaatgttaataatattttatcagtgttaaattctgtgagtttggtatttgtgttgtggttgttagacaacatccttgaccttagaagatacatgctgaggtatgtaggtatacaggtgtaaagggttacaatatctgccactcactctcaaagagttcagcaaaatggtaactgtaatattgtgagagagagaaagtttgaacaaatattaacaatgatagaatctatgtgaaggatatgcaggtgtttgttgtacaattcttgcaacttttatgtaaatgtgaaagttttcaaaatataaagttttaaaaaagcaaagcacaacacttcctcataagggtcaaacactggatttagaacagtcacatgacaaaaaacatcaactggaaaagggtcgccagagtgcagtcagcacatgttttgtgggcctgtttatgctcaggattgtcttggaaagtccaaagcaccagaaaggtgtagcatgtgcattaagggcactgctggctgccagttgtcaagctcctcaacctcttgtatctcatttttcaaactgttggccttctccttcacccagaaaggcaagttgggaatttgtggaagaggctcaagtggaataaatgtatcaaatttcttttcataaggcactattgaaaaattcactggtgggagcattgatcctgctttgtggaagcctttactctgttctgggtacatatatggattgtcgcctggagttaactttgggattccattcctgggatcaatatcgtatttctttctcccaaagcacttgtccaccgtcctctctgatagagacctcttgttgccgaggaagactccattaaagaagcactgctttccgacgtggtaggtgtggatgttgctgctaaaccttgggtaaaatgtccactcaggacgatgcccatctttcgtctgcaacttaagcaggctgaattcctcaggatatttatccttttggacttcaggcaacgacatttcagaggagtgatcagaatgtgagaaggagagtttccgatccaagtcagcagtggtgtctacgtaagcagacactctggggaggccaggaggctcactgacacttgggcctgtttccacagaagatgaggaactgacacttttgccagagggtgttgtgttggcaaaacatcccttagattccagaaaatcactgcaattagcactgtaggtcctctccacctcggtcatgccagagtcccttttttctggaaccttctccagctgtctgccgcaggtcgtgcttgagatggaggggagacggcagccccgtggactgtttccagtgagcatggatggactcatcaacgaaccaactggcaactgaactgccgaacgcacgccgcacgccgaggcctgagaaccgagagcctagggcaaaagggacaccgcagccgcctgcttctcccacagaggcgcgttcc

SEQ ID NO: 8434 - RNA, 2759 nt, Homo sapiens
  source 1..2759: mol_type = other RNA
aaaaggcattgtggtttttgtttgcttctttgtttttgggatggagtttcgctcttgtcgcccaggctggagtgcaatggcatggtcttggctcactgcaacctctgcctcctgggttcaagagattctcctgcctcagcctcccgagtaccagggattacaggtgcccaccatcttgcctggctaatttttgtgattttagtagagacaggtttcgccatgttgaccaggctggtctcgaactcctgacctcaagtgattcgcctgcctcggcctccaaaagtgctgggattacaggcatgagccaccacacctggctaaatgtatcgtgttctaaacctgcttcattcactttggctgtgactggagacaacaaacattttgggaaataaatcatgctcatgtcatagacatgtggagtctcagcatggaccccaatctctttccactttaaggttttggagatactagatctgcagccttcattagccagccaagggggttccctagtggagaaagagattggctgtaaaaatgccgtgagtcactagtttgactgtgtcaaagcctgtgaggcagcttttgttttcaccttttcctccaaatgtttgcttcttgtctgattgacaggaggccctaaaactcatgactggtggtcactgagctctcaccctgcttggctattgtagataggcaatactaaactggggaatgcagctacagggcaatagtattacttacctggtatagatccagccttcatgtttttctgacatgtaccaagttaacattagagaaacattccaaaaggtattaataaaatgaaaagttttaccaaaagcaatgaaagttcactgctatggtctaaatgtttgtcctccccaccccaaaatgcatatgtcgaaacctaatccccaaggtgatggtattaggaggtaaggccattgggaggcgattaggtcatgagaccagagccctcatgaatgagattagtgcccttgtaaaagagaccccagaggactagctcaccctttctatcatatgaggacacagcaagaaggtactatctatgagccagaaggctggccctcagcagacactgaacctgccagcaccctgcgcttggacttcccagcctccagaactgtaagaaatgaattcctattgtttataagccattctgtttatggcgttttgttatagcagcctgaacaggctaagacactcacatcatgtctgtattttatgattgatttgagggcatccttagaaaactaaatataattgactaaaattgaatgtggactaaatgttaataatattttatcagtgttaaattctgtgagtttggtatttgtgttgtggttgttagacaacatccttgaccttagaagatacatgctgaggtatgtaggtatacaggtgtaaagggttacaatatctgccactcactctcaaagagttcagcaaaatggtaactgtaatattgtgagagagagaaagtttgaacaaatattaacaatgatagaatctatgtgaaggatatgcaggtgtttgttgtacaattcttgcaacttttatgtaaatgtgaaagttttcaaaatataaagttttaaaaaagcaaagcacaacacttcctcataagggtcaaacactggatttagaacagtcacatgacaaaaaacatcaactggaaaagggtcgccagagtgcagtcagcacatgttttgtgggcctgtttatgctcaggattgtcttggaaagtccaaagcaccagaaaggtgtagcatgtgcattaagggcactgctggctgccagttgtcaagctcctcaacctcttgtatctcatttttcaaactgttggccttctccttcacccagaaaggcaagttgggaatttgtggaagaggctcaagtggaataaatgtatcaaatttcttttcataaggcactattgaaaaattcactggtgggagcattgatcctgctttgtggaagcctttactctgttctgggtacatatatggattgtcgcctggagttaactttgggattccattcctgggatcaatatcgtatttctttctcccaaagcacttgtccaccgtcctctctgatagagacctcttgttgccgaggaagactccattaaagaagcactgctttccgacgtggtaggtgtggatgttgctgctaaaccttgggtaaaatgtccactcaggacgatgcccatctttcgtctgcaacttaagcaggctgaattcctcaggatatttatccttttggacttcaggcaacgacatttcagaggagtgatcagaatgtgagaaggagagtttccgatccaagtcagcagtggtgtctacgtaagcagacactctggggaggccaggaggctcactgacacttgggcctgtttccacagaagatgaggaactgacacttttgccagagggtgttgtgttggcaaaacatcccttagattccagaaaatcactgcaattagcactgtaggtcctctccacctcggtcatgccagagtcccttttttctggaaccttctccagctgtctgccgcaggtcgtgcttgagatggaggggagacggcagccccgtggactgtttccagtgagcatggatggactcatcaactggcaactgaactgccgaacgcacgccgcacgccgaggcctgagaaccgagagcctagggcaaaagggacaccgcagccgcctgcttctcccacagaggcgcgttcc

SEQ ID NO: 8435 - RNA, 2850 nt, Homo sapiens
  source 1..2850: mol_type = other RNA
aaaagggggctgaggtggagagtagaggggttggcagtgtgcgggtttggcaaagcatcacgaccatctttggggttcaagttcattgacatgtgatctactaggcattatcaataatggtttcacacatcaatattctatagcctaaacagctgtgcaacctgagggaagtccttctcctcccccaggtttcactttgctcctttactaatgagaggactcgactagatgacaccaaaggtcagaaacactccttatctcaggattctacgggtctggccgagggacccctgccatgccgtatgaccccagactgacctccctaacctgctggggtcttaacttgctgatcctcaagcctgttgggagggagaaactcttaaaatcaaatcctacgcactgtagttgacctacacaagtggcttccgcatttggacaaaaatcagttactaacaagtgaacaacacatcagtaacagtcttattaaaactagttgtttaggtcaggcacaaaatctcagaggaggctcaggatgggcctctgggctccctagattgtctttccagagagggcagtaaggtgacaccaccagaatccaccaggaggccccggtcacgcccctgcaggagaattcagttatggaaaatgctttcaggacctgcctggttcagtcaccagtggtctcccaggctgtcaccctggggtgtgggtggcagtgaagaggctctttggagatgcatgtggccaggggagacaatggggacatctgtgcttgttgcacccaagctacgctagtgcccccatcacatgtcccagcacacgccagaatttacaatttacacagccttatagtgtcaggctcaccagagacactggctgccagccactggggctgcgtccccaagtgcccatttgtcatgcctttcgattttcccttcctagtagctccctgtcaatgttgctgagtcatgtacttagggtgaatttgagacaatacttagaggacagcaacagcacgtgagacaggcacatctgacatgcctaatttcccccaaggcccttgcgggacagccttctgcaaaaatgacagctttgttggggggcctccctttgggaatcccagttcatagcaccagtgattccaggaaacaggaacgtgaccgtggagggatggattatggtgggaacccaggtctcctttaacatcttggttggagcggcccttctgcagagctctttgggtagtaagcaagagccagtcacagagacactggcatccacacccagggcccctgggtgggagagcaccactgaataggtcctggggcccttgagtcgccagtcccagggacccctgcctccgggagacccactggagtaacttggcctcagcttcctctgacacccctccagcccaagccctccgctccagcccctccgcccagtctgagggctcctcagcagagagagaacctccgagagttgatgttcatcttggtcacgccaataagcttgagtggtgtggagaggctgaaggaggaggcaagaggggagtcacagaagaggtcggccagctcatcccgctcctccagctcgtaggtggcatcgttgagcatcctcctgtggaggcggcaggtgtgttcgattttcagcttgttgatgtcgccacgcaggcgcatgagctgtctggccagttgctggtcctgcagccgcatctccgtcagttccttcctgagccaggctatagcttcatcgatgctctgaaagccttccagcttgccagtggacaggggtctggcaccttggctggcactcctggcagaaggggggtgctgcccagcctctctcagggggagcaagggctcctgccccccacgctccccctcctccaagctcgcctgtggctccgcagccggcctcgggaagggccaggtatgctcctccagcctggcctgccattccaggtaggagggcctgcgggtctccagcctcagtttctcggtgagggccttcaggctccggaggtggtcatcgggtggtgcggctgctcccgccccctcttctgcacccacttcttccacgtggatctggggcacagacattctacagtctgccctggcagccggacatgcgagggcacggggggcgcagggggaggcttggtgggtggcacagttgggtcccgctctgggatggcctcatccaggtgcccgagggcatttccgggacaggagccggcctcagaggctgggtggcaggggagctgagagggaccgcgcagtgagccgcacagggcgccctcctggaggctcgggtctatgatccgtcctggaagcctgtgggtgccatgctccacagaaggcaggaacagacagcgtcgcaggaatctcggggcagcctgtgccaaggtctatctgtcctgaacgcactcgaagaccagactggcaggaagaaggcccagagctctctcttctcgggaagggcaggtggctggagacccacgcgctcctgctgttccttccagcctcgcattctccactagaaccctttcgtttcttctccataagacacaatctttccaaccccgacccagcactcctgtcccgccggacaccatgctctttcacacccctgactcggcacaagctttcctccagcctggaaagcccttcactcccttctgtgccttagttcagttctcagggattttctcctgggggaagttttgcttgatttgcccaggctgggctgtgtgtacccaggacaacccgagcacatcagagaaacaattatgtcatcgcaacattagctaatgcttacagcacaccacacgagctgtggtgctaaaag

SEQ ID NO: 8436 - RNA, 2651 nt, Homo sapiens
  source 1..2651: mol_type = other RNA
aaaagggggctgaggtggagagtagaggggttggcagtgtgcgggtttggcaaagcatcacgaccatctttggggttcaagttcattgacatgtgatctactaggcattatcaataatggtttcacacatcaatattctatagcctaaacagctgtgcaacctgagggaagtccttctcctcccccaggtttcactttgctcctttactaatgagaggactcgactagatgacaccaaaggtcagaaacactccttatctcaggattctacgggtctggccgagggacccctgccatgccgtatgaccccagactgacctccctaacctgctggggtcttaacttgctgatcctcaagcctgttgggagggagaaactcttaaaatcaaatcctacgcactgtagttgacctacacaagtggcttccgcatttggacaaaaatcagttactaacaagtgaacaacacatcagtaacagtcttattaaaactagttgtttaggtcaggcacaaaatctcagaggaggctcaggatgggcctctgggctccctagattgtctttccagagagggcagtaaggtgacaccaccagaatccaccaggaggccccggtcacgcccctgcaggagaattcagttatggaaaatgctttcaggacctgcctggttcagtcaccagtggtctcccaggctgtcaccctggggtgtgggtggcagtgaagaggctctttggagatgcatgtggccaggggagacaatggggacatctgtgcttgttgcacccaagctacgctagtgcccccatcacatgtcccagcacacgccagaatttacaatttacacagccttatagtgtcaggctcaccagagacactggctgccagccactggggctgcgtccccaagtgcccatttgtcatgcctttcgattttcccttcctagtagctccctgtcaatgttgctgagtcatgtacttagggtgaatttgagacaatacttagaggacagcaacagcacgtgagacaggcacatctgacatgcctaatttcccccaaggcccttgcgggacagccttctgcaaaaatgacagctttgttggggggcctccctttgggaatcccagttcatagcaccagtgattccaggaaacaggaacgtgaccgtggagggatggattatggtgggaacccaggtctcctttaacatcttggttggagcggcccttctgcagagctctttgggtagtaagcaagagccagtcacagagacactggcatccacacccagggcccctgggtgggagagcaccactgaataggtcctggggcccttgagtcgccagtcccagggacccctgcctccgggagacccactggagtaacttggcctcagcttcctctgacacccctccagcccaagccctccgctccagcccctccgcccagtctgagggctcctcagcagagagagaacctccgagagttgatgttcatcttggtcacgccaataagcttgagtggtgtggagaggctgaaggaggaggcaagaggggagtcacagaagaggtcggccagctcatcccgctcctccagctcgtaggtggcatcgttgagcatcctcctgtggaggcggcaggtgtgttcgattttcagcttgttgatgtcgccacgcaggcgcatgagctgtctggccagttgctggtcctgcagccgcatctccgtcagttccttcctgagccaggctatagcttcatcgatgctctgaaagccttccagcttgccagtggacaggggtctggcaccttggctggcactcctggcagaaggggggtgctgcccagcctctctcagggggagcaagggctcctgccccccacgctccccctcctccaagctcgcctgtggctccgcagccggcctcgggaagggccaggtatgctcctccagcctggcctgccattccaggtaggagggcctgcgggtctccagcctcagtttctcggtgagggccttcaggctccggaggtggtcatcgggtggtgcggctgctcccgccccctcttctgcacccacttcttccacgtggatctggggcacagacattctacagtctgccctggcagccggacatgcgagggcacggggggcgcagggggaggcttggtgggtggcacagttgggtcccgctctgggatggcctcatccaggtgcccgagggcatttccgggacaggagccggcctcagaggctgggtggcaggggagctgagagggaccgcgcagtgagccgcacagggcgccctcctggaggctcgggtctatgatccgtcctggaagcctgtgggtgccatgctccacagaaggcaggaacagacagcgtcgcaggaatctcggggcagcctgtgccaaggtctatctgtcctgaacgcactcgaagaccagactggcaggaagaaggcccagagctctctcttctcgggaagggcaggtggctggagacccccagacctcatcaagcacctttcctagatgcccggggctggaagcgtctttcaaagggctccagtctgccattctcacgatagccctgggcgtgcgcgcaggcgccgcctacatggccagacgcgaagctgagtggtggggctgcaaagtg

SEQ ID NO: 8437 - RNA, 2543 nt, Homo sapiens
  source 1..2543: mol_type = other RNA
aaaagggggctgaggtggagagtagaggggttggcagtgtgcgggtttggcaaagcatcacgaccatctttggggttcaagttcattgacatgtgatctactaggcattatcaataatggtttcacacatcaatattctatagcctaaacagctgtgcaacctgagggaagtccttctcctcccccaggtttcactttgctcctttactaatgagaggactcgactagatgacaccaaaggtcagaaacactccttatctcaggattctacgggtctggccgagggacccctgccatgccgtatgaccccagactgacctccctaacctgctggggtcttaacttgctgatcctcaagcctgttgggagggagaaactcttaaaatcaaatcctacgcactgtagttgacctacacaagtggcttccgcatttggacaaaaatcagttactaacaagtgaacaacacatcagtaacagtcttattaaaactagttgtttaggtcaggcacaaaatctcagaggaggctcaggatgggcctctgggctccctagattgtctttccagagagggcagtaaggtgacaccaccagaatccaccaggaggccccggtcacgcccctgcaggagaattcagttatggaaaatgctttcaggacctgcctggttcagtcaccagtggtctcccaggctgtcaccctggggtgtgggtggcagtgaagaggctctttggagatgcatgtggccaggggagacaatggggacatctgtgcttgttgcacccaagctacgctagtgcccccatcacatgtcccagcacacgccagaatttacaatttacacagccttatagtgtcaggctcaccagagacactggctgccagccactggggctgcgtccccaagtgcccatttgtcatgcctttcgattttcccttcctagtagctccctgtcaatgttgctgagtcatgtacttagggtgaatttgagacaatacttagaggacagcaacagcacgtgagacaggcacatctgacatgcctaatttcccccaaggcccttgcgggacagccttctgcaaaaatgacagctttgttggggggcctccctttgggaatcccagttcatagcaccagtgattccaggaaacaggaacgtgaccgtggagggatggattatggtgggaacccaggtctcctttaacatcttggttggagcggcccttctgcagagctctttgggtagtaagcaagagccagtcacagagacactggcatccacacccagggcccctgggtgggagagcaccactgaataggtcctggggcccttgagtcgccagtcccagggacccctgcctccgggagacccactggagtaacttggcctcagcttcctctgacacccctccagcccaagccctccgctccagcccctccgcccagtctgagggctcctcagcagagagagaacctccgagagttgatgttcatcttggtcacgccaataagcttgagtggtgtggagaggctgaaggaggaggcaagaggggagtcacagaagaggtcggccagctcatcccgctcctccagctcgtaggtggcatcgttgagcatcctcctgtggaggcggcaggtgtgttcgattttcagcttgttgatgtcgccacgcaggcgcatgagctgtctggccagttgctggtcctgcagccgcatctccgtcagttccttcctgagccaggctatagcttcatcgatgctctgaaagccttccagcttgccagtggacaggggtctggcaccttggctggcactcctggcagaaggggggtgctgcccagcctctctcagggggagcaagggctcctgccccccacgctccccctcctccaagctcgcctgtggctccgcagccggcctcgggaagggccaggtatgctcctccagcctggcctgccattccaggtaggagggcctgcgggtctccagcctcagtttctcggtgagggccttcaggctccggaggtggtcatcgggtggtgcggctgctcccgccccctcttctgcacccacttcttccacgtggatctggggcacagacattctacagtctgccctggcagccggacatgcgagggcacggggggcgcagggggaggcttggtgggtggcacagttgggtcccgctctgggatggcctcatccaggtgcccgagggcatttccgggacaggagccggcctcagaggctgggtggcaggggagctgagagggaccgcgcagtgagccgcacagggcgccctcctggaggctcgggtctatgatccgtcctggaagcctgtgggtgccatgctccacagaaggcaggaacagacagcgtcgcaggaatctcggggcagcctgtgccaaggtctatctgtcctgaacgcactcgaagaccagactggcaggaagaaggcccagagctctctcttctcgggaagggcaggtggctggagaccccctgtggacgcagacctcttggttatcctcccagtagactacg

SEQ ID NO: 8438 - RNA, 2722 nt, Homo sapiens
  source 1..2722: mol_type = other RNA
aaaagggggctgaggtggagagtagaggggttggcagtgtgcgggtttggcaaagcatcacgaccatctttggggttcaagttcattgacatgtgatctactaggcattatcaataatggtttcacacatcaatattctatagcctaaacagctgtgcaacctgagggaagtccttctcctcccccaggtttcactttgctcctttactaatgagaggactcgactagatgacaccaaaggtcagaaacactccttatctcaggattctacgggtctggccgagggacccctgccatgccgtatgaccccagactgacctccctaacctgctggggtcttaacttgctgatcctcaagcctgttgggagggagaaactcttaaaatcaaatcctacgcactgtagttgacctacacaagtggcttccgcatttggacaaaaatcagttactaacaagtgaacaacacatcagtaacagtcttattaaaactagttgtttaggtcaggcacaaaatctcagaggaggctcaggatgggcctctgggctccctagattgtctttccagagagggcagtaaggtgacaccaccagaatccaccaggaggccccggtcacgcccctgcaggagaattcagttatggaaaatgctttcaggacctgcctggttcagtcaccagtggtctcccaggctgtcaccctggggtgtgggtggcagtgaagaggctctttggagatgcatgtggccaggggagacaatggggacatctgtgcttgttgcacccaagctacgctagtgcccccatcacatgtcccagcacacgccagaatttacaatttacacagccttatagtgtcaggctcaccagagacactggctgccagccactggggctgcgtccccaagtgcccatttgtcatgcctttcgattttcccttcctagtagctccctgtcaatgttgctgagtcatgtacttagggtgaatttgagacaatacttagaggacagcaacagcacgtgagacaggcacatctgacatgcctaatttcccccaaggcccttgcgggacagccttctgcaaaaatgacagctttgttggggggcctccctttgggaatcccagttcatagcaccagtgattccaggaaacaggaacgtgaccgtggagggatggattatggtgggaacccaggtctcctttaacatcttggttggagcggcccttctgcagagctctttgggtagtaagcaagagccagtcacagagacactggcatccacacccagggcccctgggtgggagagcaccactgaataggtcctggggcccttgagtcgccagtcccagggacccctgcctccgggagacccactggagtaacttggcctcagcttcctctgacacccctccagcccaagccctccgctccagcccctccgcccagtctgagggctcctcagcagagagagaacctccgagagttgatgttcatcttggtcacgccaataagcttgagtggtgtggagaggctgaaggaggaggcaagaggggagtcacagaagaggtcggccagctcatcccgctcctccagctcgtaggtggcatcgttgagcatcctcctgtggaggcggcaggtgtgttcgattttcagcttgttgatgtcgccacgcaggcgcatgagctgtctggccagttgctggtcctgcagccgcatctccgtcagttccttcctgagccaggctatagcttcatcgatgctctgaaagccttccagcttgccagtggacaggggtctggcaccttggctggcactcctggcagaaggggggtgctgcccagcctctctcagggggagcaagggctcctgccccccacgctccccctcctccaagctcgcctgtggctccgcagccggcctcgggaagggccaggtatgctcctccagcctggcctgccattccaggtaggagggcctgcgggtctccagcctcagtttctcggtgagggccttcaggctccggaggtggtcatcgggtggtgcggctgctcccgccccctcttctgcacccacttcttccacgtggatctggggcacagacattctacagtctgccctggcagccggacatgcgagggcacggggggcgcagggggaggcttggtgggtggcacagttgggtcccgctctgggatggcctcatccaggtgcccgagggcatttccgggacaggagccggcctcagaggctgggtggcaggggagctgagagggaccgcgcagtgagccgcacagggcgccctcctggaggctcgggtctatgatccgtcctggaagcctgtgggtgccatgctccacagaaggcaggaacagacagcgtcgcaggaatctcggggcagcctgtgccaaggtctatctgtcctgaacgcactcgaagaccagactggcaggaagaaggcccagagctctctcttctcgggaagggcaggtggctggagacccgagatctcccagcaataagttgtggggacaagctcaggctgtctgaatctgaggccacaggtctttcctctctgtggcaacagccggggggtccccagagccagccagcagggaaaccgcaccccacacaggctaaggtgggtctgctccgtccaggtgccactgccccctcaccacctccacccaccacaggtcctgtcctccagcagccgtttctacatc

SEQ ID NO: 8439 - RNA, 3006 nt, Homo sapiens
  source 1..3006: mol_type = other RNA
aaaagggggctgaggtggagagtagaggggttggcagtgtgcgggtttggcaaagcatcacgaccatctttggggttcaagttcattgacatgtgatctactaggcattatcaataatggtttcacacatcaatattctatagcctaaacagctgtgcaacctgagggaagtccttctcctcccccaggtttcactttgctcctttactaatgagaggactcgactagatgacaccaaaggtcagaaacactccttatctcaggattctacgggtctggccgagggacccctgccatgccgtatgaccccagactgacctccctaacctgctggggtcttaacttgctgatcctcaagcctgttgggagggagaaactcttaaaatcaaatcctacgcactgtagttgacctacacaagtggcttccgcatttggacaaaaatcagttactaacaagtgaacaacacatcagtaacagtcttattaaaactagttgtttaggtcaggcacaaaatctcagaggaggctcaggatgggcctctgggctccctagattgtctttccagagagggcagtaaggtgacaccaccagaatccaccaggaggccccggtcacgcccctgcaggagaattcagttatggaaaatgctttcaggacctgcctggttcagtcaccagtggtctcccaggctgtcaccctggggtgtgggtggcagtgaagaggctctttggagatgcatgtggccaggggagacaatggggacatctgtgcttgttgcacccaagctacgctagtgcccccatcacatgtcccagcacacgccagaatttacaatttacacagccttatagtgtcaggctcaccagagacactggctgccagccactggggctgcgtccccaagtgcccatttgtcatgcctttcgattttcccttcctagtagctccctgtcaatgttgctgagtcatgtacttagggtgaatttgagacaatacttagaggacagcaacagcacgtgagacaggcacatctgacatgcctaatttcccccaaggcccttgcgggacagccttctgcaaaaatgacagctttgttggggggcctccctttgggaatcccagttcatagcaccagtgattccaggaaacaggaacgtgaccgtggagggatggattatggtgggaacccaggtctcctttaacatcttggttggagcggcccttctgcagagctctttgggtagtaagcaagagccagtcacagagacactggcatccacacccagggcccctgggtgggagagcaccactgaataggtcctggggcccttgagtcgccagtcccagggacccctgcctccgggagacccactggagtaacttggcctcagcttcctctgacacccctccagcccaagccctccgctccagcccctccgcccagtctgagggctcctcagcagagagagaacctccgagagttgatgttcatcttggtcacgccaataagcttgagtggtgtggagaggctgaaggaggaggcaagaggggagtcacagaagaggtcggccagctcatcccgctcctccagctcgtaggtggcatcgttgagcatcctcctgtggaggcggcaggtgtgttcgattttcagcttgttgatgtcgccacgcaggcgcatgagctgtctggccagttgctggtcctgcagccgcatctccgtcagttccttcctgagccaggctatagcttcatcgatgctctgaaagccttccagcttgccagtggacaggggtctggcaccttggctggcactcctggcagaaggggggtgctgcccagcctctctcagggggagcaagggctcctgccccccacgctccccctcctccaagctcgcctgtggctccgcagccggcctcgggaagggccaggtatgctcctccagcctggcctgccattccaggtaggagggcctgcgggtctccagcctcagtttctcggtgagggccttcaggctccggaggtggtcatcgggtggtgcggctgctcccgccccctcttctgcacccacttcttccacgtggatctggggcacagacattctacagtctgccctggcagccggacatgcgagggcacggggggcgcagggggaggcttggtgggtggcacagttgggtcccgctctgggatggcctcatccaggtgcccgagggcatttccgggacaggagccggcctcagaggctgggtggcaggggagctgagagggaccgcgcagtgagccgcacagggcgccctcctggaggctcgggtctatgatccgtcctggaagcctgtgggtgccatgctccacagaaggcaggaacagacagcgtcgcaggaatctcggggcagcctgtgccaaggtctatctgtcctgaacgcactcgaagaccagactggcaggaagaaggcccagagctctctcttctcgggaagggcaggtggctggagaccctcacctcttcagagacagaagcaaataaacctgcagctgtggagggaagaaggcggtggcacctgggctggatggctaaacaagcaggctgtgactcattgttctagaacgaggcttctcgtgttcacctaagtgcccgcatggcagcacctccagctctgcttggagcaagcgagaatccccctgaggaactggattctgattcaattggtcgagagatgggacttagacagcagtgttcagctcccccgatgatccgagtgtgcagccggggtggagaaccactgtctccagatgcagacactagagttgggatcagatggcctagctctacgtcttgtcaggcttgctaagtctcattttcttcatctgtaaaatgggagtgataaataccaacctcctatgttctagcagattggcagaactaaaattcaccggcactctctgaagacttagcacgctaagtccgcaaatgcgaaatgtactcatgggagtctcctgtgcag

SEQ ID NO: 8440 - RNA, 2627 nt, Homo sapiens
  source 1..2627: mol_type = other RNA
aaaagggggctgaggtggagagtagaggggttggcagtgtgcgggtttggcaaagcatcacgaccatctttggggttcaagttcattgacatgtgatctactaggcattatcaataatggtttcacacatcaatattctatagcctaaacagctgtgcaacctgagggaagtccttctcctcccccaggtttcactttgctcctttactaatgagaggactcgactagatgacaccaaaggtcagaaacactccttatctcaggattctacgggtctggccgagggacccctgccatgccgtatgaccccagactgacctccctaacctgctggggtcttaacttgctgatcctcaagcctgttgggagggagaaactcttaaaatcaaatcctacgcactgtagttgacctacacaagtggcttccgcatttggacaaaaatcagttactaacaagtgaacaacacatcagtaacagtcttattaaaactagttgtttaggtcaggcacaaaatctcagaggaggctcaggatgggcctctgggctccctagattgtctttccagagagggcagtaaggtgacaccaccagaatccaccaggaggccccggtcacgcccctgcaggagaattcagttatggaaaatgctttcaggacctgcctggttcagtcaccagtggtctcccaggctgtcaccctggggtgtgggtggcagtgaagaggctctttggagatgcatgtggccaggggagacaatggggacatctgtgcttgttgcacccaagctacgctagtgcccccatcacatgtcccagcacacgccagaatttacaatttacacagccttatagtgtcaggctcaccagagacactggctgccagccactggggctgcgtccccaagtgcccatttgtcatgcctttcgattttcccttcctagtagctccctgtcaatgttgctgagtcatgtacttagggtgaatttgagacaatacttagaggacagcaacagcacgtgagacaggcacatctgacatgcctaatttcccccaaggcccttgcgggacagccttctgcaaaaatgacagctttgttggggggcctccctttgggaatcccagttcatagcaccagtgattccaggaaacaggaacgtgaccgtggagggatggattatggtgggaacccaggtctcctttaacatcttggttggagcggcccttctgcagagctctttgggtagtaagcaagagccagtcacagagacactggcatccacacccagggcccctgggtgggagagcaccactgaataggtcctggggcccttgagtcgccagtcccagggacccctgcctccgggagacccactggagtaacttggcctcagcttcctctgacacccctccagcccaagccctccgctccagcccctccgcccagtctgagggctcctcagcagagagagaacctccgagagttgatgttcatcttggtcacgccaataagcttgagtggtgtggagaggctgaaggaggaggcaagaggggagtcacagaagaggtcggccagctcatcccgctcctccagctcgtaggtggcatcgttgagcatcctcctgtggaggcggcaggtgtgttcgattttcagcttgttgatgtcgccacgcaggcgcatgagctgtctggccagttgctggtcctgcagccgcatctccgtcagttccttcctgagccaggctatagcttcatcgatgctctgaaagccttccagcttgccagtggacaggggtctggcaccttggctggcactcctggcagaaggggggtgctgcccagcctctctcagggggagcaagggctcctgccccccacgctccccctcctccaagctcgcctgtggctccgcagccggcctcgggaagggccaggtatgctcctccagcctggcctgccattccaggtaggagggcctgcgggtctccagcctcagtttctcggtgagggccttcaggctccggaggtggtcatcgggtggtgcggctgctcccgccccctcttctgcacccacttcttccacgtggatctggggcacagacattctacagtctgccctggcagccggacatgcgagggcacggggggcgcagggggaggcttggtgggtggcacagttgggtcccgctctgggatggcctcatccaggtgcccgagggcatttccgggacaggagccggcctcagaggctgggtggcaggggagctgagagggaccgcgcagtgagccgcacagggcgccctcctggaggctcgggtctatgatccgtcctggaagcctgtgggtgccatgctccacagaaggcaggaacagacagcgtcgcaggaatctcggggcagcctgtgccaaggtctatctgtcctgaacgcactcgaagaccagactggcaggaagaaggcccagagctctctcttctcgggaagggcaggtggctggagacccttccgggagcccaggggccctgctggggactcgccggtgtccccgccgcctcctcctgcgcgggtccgcgctgcccggcctcagctcagggctcccgcctcgcctccccgagctccggtgaattctc

SEQ ID NO: 8441 - RNA, 600 nt, Homo sapiens
  source 1..600: mol_type = other RNA
aaaagtaatcactgtttttgccattttcagaatgtcatataatggaaatcatacagtatcagtcttttcagatgggcttccttcagttaacaacatgcatttaagattcatccatctcttttctggcttaatagctcatttccttttattactaaatagtatttcattctatggctacaccacactttccctatccattcacatattgtagaacatcttggttacttctagtttttagtggttgtgaatcagccttctgtaaacttttgcatgtagattttttgtgtggatgtaaggtttcaactcctttgggtagatatctaggaaagtgattgctggatcatatggtgagagtatgtttagctttttaggaaaccattaaactgccttccaaagttgacagtgtcatttcgcattcccataaacaatgagtgattgctcctattgctctgcttcctccccagtcgttggtatctccagtttgtttttgtatttttgcctttctaaatagtgtgtaatagtacctcattgctttttgttgttgttgttgtttgtttgttttgagatggagttttgctcttgtcgcctagactggagtgc

SEQ ID NO: 8442 - RNA, 3699 nt, Homo sapiens
  source 1..3699: mol_type = other RNA
aaaagtaattgcagtttttgccactgaaagtaatggcaaaaaaaaaaaaaaaaggaagtactggctattatcagatgtgtaattagttgtgtccttctccaccagagggcgcagtcctgcacccgagacttgtcacgaaaacccgataatggggtagatctgaaagtaggttcatgaccccagtcattgataacagcagtcactggtggaatcaggggactctgcagtcacaggactcaaacttggaaatgagacatcatctagaaacctagatgatcacagggcctcaaattgtagtattcaagttcccctttcatgtacatattcagcattttccaagccttcagacaagatttctcccttttggtttgtctccccatggggacaaatgtattctaatttatttttactctggtaaattataaagtaatgaatgacagatagttctaacttaattgacgggctccccaccatattgcaaataaaatgacttgaaaattgtcatctcagaagcctatgtctgcatttaatttttgtaatctaggactcttttccacctaaagccaataaataaggaaactgtatttccacttctttccactgtactttggcaaaaatagattctggacttcttactactatttcattgtgccctttcaggtggatgtgagtctgtgtcatttattggttacatccttacacatgtatcattcttacccatctcttagtcccgtctaccatggaaacagtaggtgatgacaggatggtaataagcatgaaattcaaaaccagaaaggtgagctgatgctggagctacagggtctttactatctgcaactggagtggaccatttctgctgtcttgtccttgatatgacactgacatgaagatacagtaagaacatttgccatttctggtgctcttcattcctttgggcaaattcaagtgtccatctggtataattttccatcagtttgaacaacttcctttagcatttctcgtagtacagttttagtgatgaattctttcatctttagatttcctcagaaagaaatgatggtattgcggtgcctcagctctaccaactagattcaccaaccagtgagctctgcctcaatcatcgtagaatcaggaatcatcatctcggagtcattctgagatgattcatcatagaattgggaatcatctcagagtcattatcagagtctcagatcatcagtattataatccctattgcacttttcttgaagcattttaccttcctgaccggacaccatctgttcctgtgagtagaaaaatcctacggtctctgcaattctccttctgtgaagaggcctggatggaggcagcttcctgcagcctctcagggtggcagggatctcctagcaggttgattgtgtcacgggatccttcaggtgttgcttttccagctagaaagctctgtgaccagtggtgcctttgcctgagttttgatcaggcccgccagacttgttccactgacgtggcctggcaggctgtgctcagctcatgctaccagccaggattccacgcctgccgagggtgagccaggcacggaacagcgaggggtgtgcaggcgagcgaacgcagggtctggccactgcgcagagccggacacaccagctgctgcagctgggcaggcagctccaggcgccggcaaaggtgccggttctatgcaagtctgcagctggatctgatgaaccacaagcggcttctgctgtgggcacctgtgtctggacaaggggaatgcagtggtgcccggaagtttgaagataccagaaaccgcagagccccaaagagggtgtcacagccctggctcagggagcccctaggtctgtgctccctgaagggccacagcacttctctccttcacatcacccgcaacatggcaagtcgcgggggtgtggggacgggaggagggcgtgtttcagccctgtttgtgttactgctctttcagtcccgccattcagtgggtcctgagttctcgtcccacatccaggaagaatgaggtacgcggacaactagagggtgagcaaggcggagaggagccttatcgagtgacagaacagctctcgggaaacttgaagtgggtagctcctttccgcaggcaggttgtcccagtaagtgtccagctctcagtggagaagagacccagagtgggtagctcccttcttcaggcaggttgtcttgatgagtcgaggagacctgaattgggtagctccttcccacagctggtagtcccagcgtctgtgtgagtctggctaggctcagaagggaggaagtgcatgctgattggcccatgggtggccatgggctgacccggaaaaatcaccataagttctcactccgggccacagacttcacccgggactgacagcctagcccctgggcttcaggcctccctggcttgatggtggggctttaccggggacccacctctttccgcccaggagcctgtctgcctcctgccaccatcaatcatgtcatccacagcgcccaggctgttcctgcagaggagtaccggcagcccgcaccgagtgccctcagctcccccaccccacgccgccagcctctctcctgtgcttctcagtgcccaaagcctagagggggccagggtggcagggggctggcatgtcagcggcgccccaggcgcacgcacacccagctgggtctagacagcgcttggcctcagccacaactttgctccaccccagagtgggctccaggagcaaggagaggccaggcagcaggagcaggcacttccaagcctgcgggtcagggggtcttcccagcccccgagagcacagggatgtccaggtctgcagctgtggctgggtggttgcagctgtgccggaaagcgtggggctcccacccggccaactcagaagagggtggggctccggccagctccacggagcacgcagcccccaccgtgcctcccacactacagctggcatcttcacagtagccgctccagacaggccactgctgccatcaattgtttacttgtcttaaactgcaggtgttcataacccatattgcagagctctacttatcagtcctattcttgtgattggggacagggatgcaaagcagaggagaaaggcttacgaagaggaagaggttgaggagactggaactgtcaagagcactcccccaacatcctccaccttcagaatgagttttcaggtaataacttctgttgttgccagcagactatgccaaacattcacttgcaccagggccagaacattggtctgttccttgttcctcaggccagaggctgtttgggtgcagggtactctcgcgtttccttctttgaagcatcctctattttcctggattcacttaggaaattctaaaagaatatacgagctcacattcctttggtcataagagcagtgtcatcattagacatcaggtcgcctctggaaaattccattgtgagtttaaaaggcaaatgacgtctataattctaaaactagttctcccaccgaaactctagaaaggatcttgggatctgcagggtctcccggatcacactttgagaactgctgctttagtcttcctcccatctcctaaggccagagctcctgagtttgcttcccactggccaaggagaaaagagcaaggtcacttgtcggggggctgcagagggaattaccttctttcatttgcaaa

SEQ ID NO: 8443 - RNA, 3703 nt, Homo sapiens
  source 1..3703: mol_type = other RNA
aaaagtaattgcagtttttgccactgaaagtaatggcaaaaaaaaaaaaaaaaggaagtactggctattatcagatgtgtaattagttgtgtccttctccaccagagggcgcagtcctgcacccgagacttgtcacgaaaacccgataatggggtagatctgaaagtaggttcatgaccccagtcattgataacagcagtcactggtggaatcaggggactctgcagtcacaggactcaaacttggaaatgagacatcatctagaaacctagatgatcacagggcctcaaattgtagtattcaagttcccctttcatgtacatattcagcattttccaagccttcagacaagatttctcccttttggtttgtctccccatggggacaaatgtattctaatttatttttactctggtaaattataaagtaatgaatgacagatagttctaacttaattgacgggctccccaccatattgcaaataaaatgacttgaaaattgtcatctcagaagcctatgtctgcatttaatttttgtaatctaggactcttttccacctaaagccaataaataaggaaactgtatttccacttctttccactgtactttggcaaaaatagattctggacttcttactactatttcattgtgccctttcaggtggatgtgagtctgtgtcatttattggttacatccttacacatgtatcattcttacccatctcttagtcccgtctaccatggaaacagtaggtgatgacaggatggtaataagcatgaaattcaaaaccagaaaggtgagctgatgctggagctacagggtctttactatctgcaactggagtggaccatttctgctgtcttgtccttgatatgacactgacatgaagatacagtaagaccacacatttgccatttctggtgctcttcattcctttgggcaaattcaagtgtccatctggtataattttccatcagtttgaacaacttcctttagcatttctcgtagtacagttttagtgatgaattctttcatctttagatttcctcagaaagaaatgatggtattgcggtgcctcagctctaccaactagattcaccaaccagtgagctctgcctcaatcatcgtagaatcaggaatcatcatctcggagtcattctgagatgattcatcatagaattgggaatcatctcagagtcattatcagagtctcagatcatcagtattataatccctattgcacttttcttgaagcattttaccttcctgaccggacaccatctgttcctgtgagtagaaaaatcctacggtctctgcaattctccttctgtgaagaggcctggatggaggcagcttcctgcagcctctcagggtggcagggatctcctagcaggttgattgtgtcacgggatccttcaggtgttgcttttccagctagaaagctctgtgaccagtggtgcctttgcctgagttttgatcaggcccgccagacttgttccactgacgtggcctggcaggctgtgctcagctcatgctaccagccaggattccacgcctgccgagggtgagccaggcacggaacagcgaggggtgtgcaggcgagcgaacgcagggtctggccactgcgcagagccggacacaccagctgctgcagctgggcaggcagctccaggcgccggcaaaggtgccggttctatgcaagtctgcagctggatctgatgaaccacaagcggcttctgctgtgggcacctgtgtctggacaaggggaatgcagtggtgcccggaagtttgaagataccagaaaccgcagagccccaaagagggtgtcacagccctggctcagggagcccctaggtctgtgctccctgaagggccacagcacttctctccttcacatcacccgcaacatggcaagtcgcgggggtgtggggacgggaggagggcgtgtttcagccctgtttgtgttactgctctttcagtcccgccattcagtgggtcctgagttctcgtcccacatccaggaagaatgaggtacgcggacaactagagggtgagcaaggcggagaggagccttatcgagtgacagaacagctctcgggaaacttgaagtgggtagctcctttccgcaggcaggttgtcccagtaagtgtccagctctcagtggagaagagacccagagtgggtagctcccttcttcaggcaggttgtcttgatgagtcgaggagacctgaattgggtagctccttcccacagctggtagtcccagcgtctgtgtgagtctggctaggctcagaagggaggaagtgcatgctgattggcccatgggtggccatgggctgacccggaaaaatcaccataagttctcactccgggccacagacttcacccgggactgacagcctagcccctgggcttcaggcctccctggcttgatggtggggctttaccggggacccacctctttccgcccaggagcctgtctgcctcctgccaccatcaatcatgtcatccacagcgcccaggctgttcctgcagaggagtaccggcagcccgcaccgagtgccctcagctcccccaccccacgccgccagcctctctcctgtgcttctcagtgcccaaagcctagagggggccagggtggcagggggctggcatgtcagcggcgccccaggcgcacgcacacccagctgggtctagacagcgcttggcctcagccacaactttgctccaccccagagtgggctccaggagcaaggagaggccaggcagcaggagcaggcacttccaagcctgcgggtcagggggtcttcccagcccccgagagcacagggatgtccaggtctgcagctgtggctgggtggttgcagctgtgccggaaagcgtggggctcccacccggccaactcagaagagggtggggctccggccagctccacggagcacgcagcccccaccgtgcctcccacactacagctggcatcttcacagtagccgctccagacaggccactgctgccatcaattgtttacttgtcttaaactgcaggtgttcataacccatattgcagagctctacttatcagtcctattcttgtgattggggacagggatgcaaagcagaggagaaaggcttacgaagaggaagaggttgaggagactggaactgtcaagagcactcccccaacatcctccaccttcagaatgagttttcaggtaataacttctgttgttgccagcagactatgccaaacattcacttgcaccagggccagaacattggtctgttccttgttcctcaggccagaggctgtttgggtgcagggtactctcgcgtttccttctttgaagcatcctctattttcctggattcacttaggaaattctaaaagaatatacgagctcacattcctttggtcataagagcagtgtcatcattagacatcaggtcgcctctggaaaattccattgtgagtttaaaaggcaaatgacgtctataattctaaaactagttctcccaccgaaactctagaaaggatcttgggatctgcagggtctcccggatcacactttgagaactgctgctttagtcttcctcccatctcctaaggccagagctcctgagtttgcttcccactggccaaggagaaaagagcaaggtcacttgtcggggggctgcagagggaattaccttctttcatttgcaaa

SEQ ID NO: 8444 - RNA, 56 nt, Homo sapiens
  source 1..56: mol_type = other RNA
aaaagtaattgcagtttttgccactgaaagtaatggcaaaaacagcaattactttc

SEQ ID NO: 8445 - RNA, 10441 nt, Homo sapiens
  source 1..10441: mol_type = other RNA
aaaagtaattgcagtttttgccattaaaagtaatgaacaattcctttagcactaacaataatttagcacctaaaagtcaagcatttagaagtctgaaattctgaggcagcagaaaataacagttactttccaggtaatgtgaaacacacacatatgcaagtatgttcacaggccatacatgcaaattttaatgctattacataaacacataggtaggcatatatttcatatgctacaacatttatatacatatataaaaacttaagacacaggcatgcacatttagttaacaagccaatacgatatttgagtgtttctgggtaatatatcagtgtatctcacaagctactaaactggttaattaaacattagatagctattttcactataaagatggaaaacggctactctgttattctgcctgactcctgagttgaggagaatagagtttaaatttaaaaacttgcaaatcgtacagggcacagtggcccagcactttgggaggccgaggtaatcccagcactttgggaggccaaggcgggtggatcacctaaggtcaggagtttgagaacagcctggccaacatggtgaaaccctgtctctaccaaaaacacaaaaattagccaggcgtggtggcatgcccctgtaatcctagctactcaggaggttgaggcaggagaatcgcttgaacccggaaggcagagattgcagtgagccaagactgtgccactgcactccagcctgggtgacagagcaagactttgtcatcaaacaaacaaaaacatgcaaatgcagttgatataaggatcattttgtaagggcatgatattaattttaaaacatcgatattgattgacagagaaagtatacaatttaagaaatttggatttagccatcataaaattgagtcagttactttgttttccaagcaatatattttcactggaaaaaattgagcccaccattcaaccactgggcatatgttgatttaggcatatagtctctgacttatataaaactaaatataatacaaaccagaagcccaacccccaaattataaatagtaccgtatgcacagatggaataaagaagtcccaagattttctaaattcttcatttgatcttagccaaaaggccgagaagcgataagattttctaaattcttaaactgattttgtcttgaactttccatcgagatctgcttattccagtttagggttgcaggtggcctgagcttctccctgcagcttaggacaccagacaggaaacaaccatccctacacaggtagtatcaccaggtgtactcactgaccccccgcactcactctgactgggaccattagatgaactgaatgtgcataactttggaatgtcagggagacctgggtacccagaaaaaaacccatccagacctggggaaaacatgtagactctacccagacagtgaaccccagtgggaatatatatgtatatatatattctttttttctcatcaacgttataaggaaacaatgttgaatgaaatgactgttattcaaagacctgctgtacctaaatctgcaaacagagaattgaattttgcaaacattcaatcaagcaggattggctacctctggaatcaactgaatatattctgaaatactcctttctttgttcctgatgatcttatttcagaacttctcctactcacgtgctgtggacagaactgatatgatatgatagctgttctatttatattggtgatctacactaatgtagtctcattgcttggaaccttgctttgagccatcataaacgtccaaattgcttccatcaaaggatgcctttagaggacttcattgtgaccgctacatagaatgtgaaagttcacaaatattatccttgtaaacccctagcattatggggttggaatatatgtaacaggtctgtagtgtaagcagccaccttgcatccagcagttttggttgttgtttggaaatgcagatctaaaagtgtttctgaagtttcagtctcttcttacaattgttgtgcaaaatgcttctggcaggctctgattcaaggtaataatgatgtttctgaaaggaagcagagatagctcctatcttctgagtacaactttaaggtattcttattgttgctcttttaaccccatgcctttattgatcaatgtcagtcttcattagatcctctttgccaggaactcttggattcccctgaagcccacagcacaagaagaagatcgcaggtgcttctgtcatcagtcattctgtcttctccaataaacctggaattagcaggaaaggttggagtaaataagtgtaaaatgtgtagcagttcctcttgcaaatcatgctcttctggttcaatgttgacatggataacggcttccactaacttttccttgaaccatttactgatgattcagcattccaatttaggatctgttttcttgatcctctcttgggactaattgtcttaggtctggtgctctaagaaagactctcacgtgcagatttgcatacaggaagtttatgagggcatactctcataaaacaccacctgggagggaatgcaagctgcagatctggcagataaagaagttgaattgagatgcagttacaacagaggccttagctgattataccaggagctcagaagctaagctggctcttcacagatataacaaattgggggaagcgattaagcttgtgtcctgccttattgaccaatcatttcatgttgtcttctcagaatgtaattggctttttaaacagcaatacttgatgtcagacaacaatgaagccatagttaaaaattgccaaccaaattaaaaggagaaaatgaaaatcttttgatatattcaaagctgagaaaaattaatccaatgtgcccttttaaatattttttcttttatcccattatcccttgaaaagttaccaaaaaactttctttgaaggatgtaccaacatcaaggagagaggatgttatgagattccaaccctagaaagcgtcaaaagaaattcctaggtatcagatgagctactacaggttctaacctgcagttcatatacaccgttcctccaagaccccgggaaagagtcatctcactcttggacacaagaaggacaaaagtaaaacttgaataaactgtctgctacctgtaaatatctaacatgcttcataaagaccattatttgtttattttaatgtaaaagtaaaagcaaataccagaagagaaaaatgcccagacacagtggctcacacctatatgttgaaggccaaaagagtaagggtcgtgatcaacccagtataccactggaggctgtatgagtaaacagcaaactgttctcataaatgcagaatgttggcagacggacaaactgcctctgccacccagaaggaatgctgagggcagtcacgacccaggcacaagtgtttcttttgattaggcacatctgaagcctgttagcaataatgtgaacctgtgatcagtcgagcagctgaccaatcattacctcctcctccctgctctttctacccaataaatacaaagggctgtggaagctcaaggttgctgcctttgcttactggaagcagagagccctcttcttcctcccctagccccttcctttaaaatagttacttttgtcttaagtttttatttctacattcgtcctccttccttcagtctcgtaatgactgtctcaagcagtatcagtagtaactgttgtaatgatagtctcaagtagtaaccatggcagtcagccacacctgtaattccagttttggggaggccaaggtggaaggatcacttgaagccaagagtttaagacaagtcaggacaacataaggagactccatttctaggttgggttactggaacaactgggactgtgtgtgcatctctctccatgtggcctgtcaacatagctagctttggtcatcttcacagcaaggtagcctcagcatagtaggacttgttaaagagaggctgttttctcctaagaacaaacattctaggaacacactgactaagccttagaaattctggaatatcacttcaacaatagtctattgatcaactatatcattaaaaactggtcaaattcaagggaatccacatcttgaaagaagagtaaaatatgcaagcatatttaatataccatacctctccttatagtataatctcatataatttggaaagtgttataatattccttaattttagaaaaatttaaaggtgggaaaaaaaggtgtggcataataaaataaaacgattatcttccattttaaggactgtcttactctggtagtccatattgaaataagaataaatataattattggtaaatttgattgtctagtcaataacacgtttactttatgagaaatataaataatatgaaatacaaaatgaaatatataaacatggcatattttgttacatatagaaatgtaaagatttttttgtaaagtaattgtgacctcccaactttctgttttccctcattcaaaacattctgggcctacatagcaaaaggctttaaaatgtcttctattaaaatgttatcgaaatgttctgtgattaaagtagcatctcaagtgtgttctaattgaactgcatctgtgaattctgcaatttggctcctatgaaccttgacaacatgtaaaagcttgcatagaaattatatttattgagcttttagtctgtgctagaaaatattttaaacacttattacctattaattcatttaaatctccaaatggctctaggaaatgaatagtagtattatttcaatttaacaaataagttatctaaagcaaagaccttgcccaagctcagaagccaacgagaagtagagctgggattcaaatccacacagctagctttattgagtgttttaatcactataatacactgtatgagctgcctgagtattcttaaaagtaacagtggagttaaaatcactttatttaatctctctctttctatgacttattcttctgcatttaaaatctctgaggaacaaaatttttactttgtcactgtgacttaaaatccttccaatcacagatagaaaatgtaaactggggaaataaaatatggagtgcattttgtattaactgtcctagtattaagacagactagaacacattttgatcatctgtaattggagccaattgacttggatcttgcactgaaatcctgctgagcatcacagacacacttagcctaaatattattacttagatttaatttctccaaattatggcttttatgggccttaaaagccccataaacaagtgtcaatgattgtagacacatacaatttctgttgacatacacaacaaaatgtgtgggtcactgtacaaagctcaaagtaaaagttgacttttattacctctgtactaataacagttaccattagtagaccatgcctatagaaggacagttattaaatggatgagctttagaaaaaattaaatcaaatttaattctatcagttctagataacaaagcatgggccagatagcataactgtcagcatcaatgtgggcctttaagtaggtactaaattacatgtcatttctccttcagagaaaacagaagaaaagttgcaacagagtgaaaaatcaggaaaacctcatcgagatagatattctgccagagacaaaacgaaacctcatcgagatagatattctgccagagaaaaatgagacatcagatatgtgtgatcacaggtcatagactcagtgaaggtgaacaattctcagacttgggaattttgagaccagcaggcaggtcctatatcagcacattggctgtagccattggtcacagggaataaagcaagcatgagggtttcccgagtccagaggctcttgtaattgctctagagctatgtgcttcatagggtgagtgtgacatctgagagatgtcaggtatggtgacaacaaatttagtggaagccttagcacaaggtcatactgttttagaagaagcctaatcttaatcctctttaaactagcagtttgggtttctggtgagttatttagcttgggcagaaaaccagatccaaacatctaagaacttttccttctggttcaaagaacttttggataaaatcaccctctaacaacctcttctgaggtaggaattttcttttttctctatcttgtggcttcagccatcttgccgtgtgccttcttctagggctccagaacttttttatccaagtcttagcctactcacgattgaagagtaaataggagttgaaacttgtctgttacaaattcagcttatactggtctcctggaagctggaggctccaaataggatgctcttttcaacaaatcaagcaaacaaacaaaacttgtgtctgacaaccacagccaagagaagcagaggccactacccatcactaactttaattacttctaggatagcctaaaaagaaaaaaagaagaaaggaagagacagggagagaaaggaaggaaggaagttagatagttggcagattagatctgttggttattgtggaagtaacgatagggcttagaaaaaagcacatcattttcatactttttctgatatgtgtatctaattttttagtatatgaaaatttattttctcatgttttctactaattgatattcattatgatacagaaataggcaaggctacttgattacaatcaaaaatcaatttttttcagttttgaaatagtttcctgttcttttttcaactaaaaactattttaaactcttcacttatacagtacttgtaaggtaagttcccttgattgctgcctagaagtttcccaccgagaagtataaacatatgcttctacttaaaatagaagcagccctatcttcacctccttcatttttcttaagatcttttatcattagaaatgtccttggaatcagaaattttagcagaacagtattgtactttcccattgaaaaaaaaaagatttttattgctttcctttaattaccagcttctggaacgattttgaacatccctctgaaatattaaaaatttgagattgttgaacaactatgaatattcaccaagcagtcattcgacccctttgcacattcctaagcagaatatgataaagatcagtcaatccaattctgcaattccttgtttgaattttcagatataagtttaagattgatttagtcatagctttcttctcacctgagatggactttggtaaattcaatagaagaatgtaagtattcctgtttacttatttaattttttttgccttgagtttttctaattggcatgtatacccccttttaaaatttccctcaacctgacaatcaattgctataggaccaagccggtgcagtatgcttctcttgctgtttagcacaatacctatatacagtaggagcttgattggtgctcatgaaagaaggaaaggagaagcaggcatgcagcttgttcttaaggaattagattgaattggattaacaagtaggctggaagtaaataccaaacagtaacaacaaacgttccaaagctaaaaatattttatgaccagcaaataattacagcctgaaaaattatctttattgccatttttgctatgattggtatctttaaaagccacgcttattagcatgcaggtttacaattatgctctgagcctggtaatgccctgccatttttacctctagggatttatgtctgattcttgttccattagtaagcgtctgtaggacagaatgacagagccattcgtgctttgccagcacatgataatgatgatattattattttcacagtcagtttggtgatggttgtttgaacctcatcatgtctaatagaggaaaaaatgaaaaaactaatatttgaaacagtgtattgtgtttagcatcattattgccacttttatggcaagtgctttgacatttaagtgagttccatttacaatatcgccaccataatctcctcattttgtaattgcttctggatacctataaggtttaactgctggtattactcttcaataaaaaaaaaagaactcatgcattagatttatggaaagttatcctggggattttagatcgttattttaatgttagcagagctcaatacagcataggtcctattgttagttgctgtagcctgcatgagttatgtggatttcttgggctgtacagacattgaggccagttgtgctatgggggtagcaactcccatcttgggattgtagaataaatgtataataaggtattctgaagtgagcagcttatttggctgctcctcagagaccctctgactctgggatggatacaggatgtctgccccagcacgcttgttttcctcgtcccaacgcctgacagacagcaccactcaagtgtgggattttcactagttggcgtgatgtcagccaactggggaatacatctgagagggcagcatactgagacactactgcctgacaggtttgttttcacgtgatggattggtcaggggatcaacaaggcagagatcagatatggtctaaacatccagctgtaggatttggtgtttaggaagaggggaaattgcttctgtttggcccatagattggaacccactatagagatggatttttgtttttttccctttcatgaacattctttaattaacattataatggcttctgagtagccttgccaagcttagatcctttcttccaactgaaatcattctgcttcaccttctgtaccaaaagcaaagaaatatttccaaacctccacagtgcagtttggtcctcctggagatttcttcttcatcttttgaatctatcaatattccccatgtctaatggaagtattactataacttacagaaagctgagttagctgttacttactttttattcagaccacaaaacgtgagttctgaggacaccaaaaagtaggtgctgaaggcagaaatctgaataggtcagatttttcttcctttcatgattatgcagtgagtcctatagaaagaatttttccttgcagtctggcttccctctatatgacaatctgtccaccaaattctggatataggaatattatgaatcatacaagttatgtaaatacatctttgcaccaaatgttgaaaaactagatttaacaaacaaataggagaggtatgtgatatgattaagcaaaagagtgttcctaagtaaataaaaatcaagtaatttttgtttaaaacagaataacctatgctactggggagcctataccatgatgagtttcagtaaatctaactccacattcatttacctaacttgtgcattctgttgatttcatcaaaagccatctagcaagagaaataaggttgcctgttagcacttactaatctaacaatctggggttttaaaaagttattcctgcttctcagttaatacttcaagatttataagtataatggctttgataatccagtcaataattcacatgtagataacagtataaaaaattctgcaactacccattgagacaagaaatcttcacatttcaataaataaccaagaaaaaaccctgcagctttcagctgccagcttagaggaagtttctgttgaggttctgaggccctcagactactctctcctctgtctgtccatttctatagcagctttgttatgttttatgatgacagtctcacccccttgagaccagccataagaaaggtacaatagcagcattatttgtattgtttggttttgtatgagatgcacattgggaaaccactacttcatggaatagcatttgcaggaggtctccagggggcagctcttaccaatctcgctggctcaacccaaggttgaatgacaataaagaatgggaaaaattaaaagaaaaggtactttaattgaacctgtatttgtggaaatgtgatacagacctagaaaacacctttcttagttcctggaatgagaaagacggcttctccagggaccttgtacagtgacagctgaatctttgctggctaaaacaaatgccctccattagctaaagatgtacttcaaaaatacttctttgagaaaatgctcattctcccattgacaaataaaacagaataagataaaataaaataacaaaataaaacagacgagaccaaaaacaagagatggcaaactttctcagtcaagggctttgcagggcatatggtctctgtggcaactactcagcactgccattatagtgtgaaaggagtcatggaaaataacataatcaaatgtgcgtagctgtgtcccaataaaaccttttttataaaaggaagctgagtttggcccagggagctgtatgctgatcactgatctaaagtattttgcagtctagctgcttactataaagttggagaaaagtctggaataatgaagtcgttatccagcatgtctaaaattcagatcttttaacattcagttctcttgct

SEQ ID NO: 8446 - RNA, 57 nt, Homo sapiens
  source 1..57: mol_type = other RNA
aaaagtaattgcagtttttgccattactttctaatagcaaaaatcacagttaccttt

SEQ ID NO: 8447 - RNA, 62 nt, Homo sapiens
  source 1..62: mol_type = other RNA
aaaagtaattgcagtttttgccattacttttaaatgacaaaaaccacaattacttttgcaca

SEQ ID NO: 8448 - RNA, 4375 nt, Homo sapiens
  source 1..4375: mol_type = other RNA
aaaagtaattgcagtttttgccattacttttagtagcaaaaaccacaattacttttctatcaatgtaatagtagaaacggggtttcactgtgttggccaggctgttcttgaactcctgacctcaagtgatccgcctgcctcagcctcccaaagagctgggattagaagtgtgagtcactgatcctggctgaaataaaaaaaattaaaaaatatattttattgttttgaattttatttaaaactctttgcaagaaatgatgctggaagactacctgtttagaattgtaatccatatatccacaagctctggcagctttaaagagaggcaatagaagaatgaatgcccaaatgtagcagattggcttttactcattttcatagtctcctcaccctagcactggtataatatgattctgagaatgttaggcagctaaagctgtttcttttaattcttgtccactttggtgacatgaggaatcaaactcaccattttatatatttagatactgaatattctggtagctcagcaccagactctgtgaagtcattccttttgcttatctatgacttggattacattccaagtatgaattaacatacagccagactagatgaacagctttagaagaatatgacttgcttttttttttttgacaagctcatttagaaggtgatacattcttttccatgttcatttccaaatgcttatataaagaatgctgagtgaactcttgcctagtgatcttaaacattaacttacacaaagtaccttccttccttgtctcagcatgttaatacatcctgtctctcccatagatatctagggcaatgaagttgatgctagcccagttcttataacctgctgccaagtattttgatggctttatctgaagagtaggtaagatctttgctgacccagctacccagcatgcagctggatgtgtggagagtagaaatatgctggccttgtgcagatggatttcaagtacaatggccaacatttttactgtccctgctatattaaaccaaccaatttaatgccttctttctagttaagctccagttccttgaaaaatatattgtttataatatagttataatagatgtcatttattaaacacaataaatactggctgtcttttaatattttacatctattttctcagtgaatgctcaaaactataagatagacactattattgtaaacattttagagttgacagaggtgagccttagagagatcaagtaactatccccaggtaactttggtagaaagttgaaaatctgggatttgaactaaagcctatgttttaagccactatatgacattgctcccactgtaccataggttttagtagaaatgtgggtgtaggggaacttaatgatttagatgtggctattcaagaacacttcttgttcttgtagtgcattaaatttggaatatattgaatattatcactaatctctagctagcaaccaaagaaaacaagatactcagaatagcaacagctttacataaaatactttttcaaaaatattatacattctccaataccttctgtggctctgataatttgctctcataatcagttcaatccagcttgttccttaaatgcttgagaagtacctcattttactcaacatattaccacatataaagcatgtgaaaataccagattgtgttccacttttaccccaaatagtaacaaagctcctgcaattttttaagatattattaaactgtgtacaaatgctcagattaaaaaaaagtgcttacttccattgaaattggacactaccactacctattcaaattcaagttgtcattgccttgaatccatgtgtaaagtttttggtaggatagtctatttctagttgtttttcaagactcataatttggaacattctagatataagattgcattgacactttatattctttttactttataaaatggtcatccatggtttatgttacaaacgaaagcaaaaatctgggggaaagttaaagaagtagagccagataacagaattttcttttctaatatctaataaagtgaaacaaaaggatgaaaataaaatcatgataggaaggaaaaaattaccagaaactatcaaagagagagaaaacagatctcatgccattaacttaaaatgtcacctaagaaaagaaacaatagattttgtctaggagaatgaaagccttctaaacttgtctctagaaacctgttttaaccataaactagaaaatggacatattaagttgacaaaaatcttaaaaattttctcctcatttggagaaaagtagactaaatatatattctttcattttcctcttatgaaaggagggaagttgcaatggttacatttgaaatatagatgaaaaaatggaggagaagaaaaattattcactcctcgatggaaacatagtctccagggctccatgctgaagaacaatgctgatactacattctcctcaaaacaattctgaaaatttcttgactcatgaaacccagctaactcagtagttgtaattacttacttttatgatctggtttcctttttcactctaaattcttatcctcctactcttctaaataaacaatctgttttgcttcttaaatttcaaataatttatggaaaacagaactaattctttccaactgttccttttcagatccccattcactcttctctaataacaattaaaatattattttgttttttgtaaatttattacataaatttaccatttatatatctttccttgattctagactatagttttcttgaaattaagacatatacttttcctattttaatcttcaagggccaatttagcacttgaaatatagacattcaatgcatatttgttaagtgaaaatgtattttgaagtgtaatctccttttttaaagtttcacaatctttttgactgagtccttgaaagcttgtttcacttgctgatttcttaaagtatatatgaagggattcagtaagggagtaaccgaagtaatgagtacagctattcctttgttgaaagcacctccttcttttgcagaaggattaatgtacataaacatgcagctgccataagagagggagatgacaatcatgtgggaggaacaagtggaaaaggcctttgtcctttgctgggcagaagggatcctcagaatagtcctgataatgtatgtgtaagaaagtgtcaccagcaccagagtaaccatgagagtcacaacggccaagaggatgaccatcagttctaagaggcttgtgtctgagcaggcaagctccacgagaggcccatagtcacagtaatagtgattcagaatgttggagacacagaaatctacctgggtcatcaggatgattggtggtaagattgctaggaatccccccaaccaggagcagaacactagttgtatgcagactctgctgctcataatagtcaggtaatgcaagggtttgcagatggccacataacgatcataagacatggaggccaggaggtaaaactcggtagctccaagaaatatagcaaaaaaatactgagtcaagcagccagcaaagctgataactttatttcctgttgtcatgctggtcagaaatctgggaataaaaatggatgtgaaggaaatttctaagaaggagaaattccggaggaagaaatacatgggggtctggaggtgggggtctagtaaggtgagggtgataatagtcagatttcctaggatacttagcatgtaggtgaggaacagaaagatgaatatcatcacttggagttcaggttgatttgtaaggcccagtagaataaactcaccaaacatggttctgtttttcattgttgaccttcggaaaacctgtggtctttggcaagtactgcattttcttccagattttcacagttgattcatttcatgatccacatttatagaatgataaaatcagtgactttaaaaacatatgttgctcatacctttgacaacctgaatgactatagtatactgtttaccttgttgttcctaagaggtaaatcaaagatgagatgtgccacgtgaatctttgagtagtatatactttaacatgttttctattggcttccatccacattttacctttctcttaatagaagtatccaaacttatggaacttaaccagaaaaaagagcatattattttccattctaagaatccaatccagaatcaaatcatagttcctgagagacagagaacttcacataggtaataaaaaataaaaacaaagcccatagcagttattgaattggaagaaaatactttgagagacagaaaatttctgaaaatttatgttctaagagagattatgttgaagttcttagatggcagaggatgggcatct

SEQ ID NO: 8449 - RNA, 4223 nt, Homo sapiens
  source 1..4223: mol_type = other RNA
aaaagtaattgcagtttttgccattacttttagtagcaaaaaccacaattacttttctatcaatgtaatagtagaaacggggtttcactgtgttggccaggctgttcttgaactcctgacctcaagtgatccgcctgcctcagcctcccaaagagctgggattagaagtgtgagtcactgatcctggctgaaataaaaaaaattaaaaaatatattttattgttttgaattttatttaaaactctttgcaagaaatgatgctggaagactacctgtttagaattgtaatccatatatccacaagctctggcagctttaaagagaggcaatagaagaatgaatgcccaaatgtagcagattggcttttactcattttcatagtctcctcaccctagcactggtataatatgattctgagaatgttaggcagctaaagctgtttcttttaattcttgtccactttggtgacatgaggaatcaaactcaccattttatatatttagatactgaatattctggtagctcagcaccagactctgtgaagtcattccttttgcttatctatgacttggattacattccaagtatgaattaacatacagccagactagatgaacagctttagaagaatatgacttgcttttttttttttgacaagctcatttagaaggtgatacattcttttccatgttcatttccaaatgcttatataaagaatgctgagtgaactcttgcctagtgatcttaaacattaacttacacaaagtaccttccttccttgtctcagcatgttaatacatcctgtctctcccatagatatctagggcaatgaagttgatgctagcccagttcttataacctgctgccaagtattttgatggctttatctgaagagtaggtaagatctttgctgacccagctacccagcatgcagctggatgtgtggagagtagaaatatgctggccttgtgcagatggatttcaagtacaatggccaacatttttactgtccctgctatattaaaccaaccaatttaatgccttctttctagttaagctccagttccttgaaaaatatattgtttataatatagttataatagatgtcatttattaaacacaataaatactggctgtcttttaatattttacatctattttctcagtgaatgctcaaaactataagatagacactattattgtaaacattttagagttgacagaggtgagccttagagagatcaagtaactatccccaggtaactttggtagaaagttgaaaatctgggatttgaactaaagcctatgttttaagccactatatgacattgctcccactgtaccataggttttagtagaaatgtgggtgtaggggaacttaatgatttagatgtggctattcaagaacacttcttgttcttgtagtgcattaaatttggaatatattgaatattatcactaatctctagctagcaaccaaagaaaacaagatactcagaatagcaacagctttacataaaatactttttcaaaaatattatacattctccaataccttctgtggctctgataatttgctctcataatcagttcaatccagcttgttccttaaatgcttgagaagtacctcattttactcaacatattaccacatataaagcatgtgaaaataccagattgtgttccacttttaccccaaatagtaacaaagctcctgcaattttttaagatattattaaactgtgtacaaatgctcagattaaaaaaaagtgcttacttccattgaaattggacactaccactacctattcaaattcaagttgtcattgccttgaatccatgtgtaaagtttttggtaggatagtctatttctagttgtttttcaagactcataatttggaacattctagatataagattgcattgacactttatattctttttactttataaaatggtcatccatggtttatgttacaaacgaaagcaaaaatctgggggaaagttaaagaagtagagccagataacagaattttcttttctaatatctaataaagtgaaacaaaaggatgaaaataaaatcatgataggaaggaaaaaattaccagaaactatcaaagagagagaaaacagatctcatgccattaacttaaaatgtcacctaagaaaagaaacaatagattttgtctaggagaatgaaagccttctaaacttgtctctagaaacctgttttaaccataaactagaaaatggacatattaagttgacaaaaatcttaaaaattttctcctcatttggagaaaagtagactaaatatatattctttcattttcctcttatgaaaggagggaagttgcaatggttacatttgaaatatagatgaaaaaatggaggagaagaaaaattattcactcctcgatggaaacatagtctccagggctccatgctgaagaacaatgctgatactacattctcctcaaaacaattctgaaaatttcttgactcatgaaacccagctaactcagtagttgtaattacttacttttatgatctggtttcctttttcactctaaattcttatcctcctactcttctaaataaacaatctgttttgcttcttaaatttcaaataatttatggaaaacagaactaattctttccaactgttccttttcagatccccattcactcttctctaataacaattaaaatattattttgttttttgtaaatttattacataaatttaccatttatatatctttccttgattctagactatagttttcttgaaattaagacatatacttttcctattttaatcttcaagggccaatttagcacttgaaatatagacattcaatgcatatttgttaagtgaaaatgtattttgaagtgtaatctccttttttaaagtttcacaatctttttgactgagtccttgaaagcttgtttcacttgctgatttcttaaagtatatatgaagggattcagtaagggagtaaccgaagtaatgagtacagctattcctttgttgaaagcacctccttcttttgcagaaggattaatgtacataaacatgcagctgccataagagagggagatgacaatcatgtgggaggaacaagtggaaaaggcctttgtcctttgctgggcagaagggatcctcagaatagtcctgataatgtatgtgtaagaaagtgtcaccagcaccagagtaaccatgagagtcacaacggccaagaggatgaccatcagttctaagaggcttgtgtctgagcaggcaagctccacgagaggcccatagtcacagtaatagtgattcagaatgttggagacacagaaatctacctgggtcatcaggatgattggtggtaagattgctaggaatccccccaaccaggagcagaacactagttgtatgcagactctgctgctcataatagtcaggtaatgcaagggtttgcagatggccacataacgatcataagacatggaggccaggaggtaaaactcggtagctccaagaaatatagcaaaaaaatactgagtcaagcagccagcaaagctgataactttatttcctgttgtcatgctggtcagaaatctgggaataaaaatggatgtgaaggaaatttctaagaaggagaaattccggaggaagaaatacatgggggtctggaggtgggggtctagtaaggtgagggtgataatagtcagatttcctaggatacttagcatgtaggtgaggaacagaaagatgaatatcatcacttggagttcaggttgatttgtaaggcccagtagaataaactcaccaaacatggttctgtttttcattgttgaccttcggaaaaccttgttgttcctaagaggtaaatcaaagatgagatgtgccacgtgaatctttgagtagtatatactttaacatgttttctattggcttccatccacattttacctttctcttaatagaagtatccaaacttatggaacttaaccagaaaaaagagcatattattttccattctaagaatccaatccagaatcaaatcatagttcctgagagacagagaacttcacataggtaataaaaaataaaaacaaagcccatagcagttattgaattggaagaaaatactttgagagacagaaaatttctgaaaatttatgttctaagagagattatgttgaagttcttagatggcagaggatgggcatct

SEQ ID NO: 8450 - RNA, 62 nt, Homo sapiens
  source 1..62: mol_type = other RNA
aaaagtaattgcagtttttgccattataatggcaaaaaccgcaacttaatggcaaaaactgc

SEQ ID NO: 8451 - RNA, 4556 nt, Homo sapiens
  source 1..4556: mol_type = other RNA
aaaagtaattgcagtttttgccattatttttatttttattttttatttttatttttttcaagacagagtcaagtgctgggattacaggcatgagccactgcgcctggcctttgccattacttttaatggcaaaaaatgcagttaacttttacaccaacctaatagaacgtaaagcagcttaaaacaagctgccctgactcagcagttcccaacaacaatcattcatctagaactacccaaggaaagcaacaaaaactttaattcccttaaggtttagaaccaatacaatgctcaaaggtctctgtgcaggaaaaaaaaatgcacagcaaaaagaaaaccttgctaggtacggtcgcttatgtctataatcccagcactttgggaggcccaggcgggagaactgcttgaggtgaggagttaggagatcagtatgggtaacacagtgtgactccatctccacgcgcaaatttttttttaattagttggacatggcgacgcatggctgtagtcccagatactcaggaggctgaggccagaggatcacttgagcccaggaggtcgaggctgcagtgagctatgattgtgccactgtacttcagcctgcgagacagagtaagaccttctctcttaaaacaaagtcacaggttctgagggttagggaaaaaataataaatttaataaagaaaaaagaaaactcaaaaaacaaacagcatttgcttcctatgaaatatttacccctttaccctaaatttaactgctttccagtccaaagctctacacacttcatgtgggcctttataaagcaaccactggctttatgatttgtctagaatacttgaagaaggaagtttatgactttgtcaaaaagctgttgtatattcccacttaacggataaataaagcaggttctattcaattggaagaaacaggaataaagacgtgtgcattttcagatttcctttgagtgccctggccttcagaccattcagtgtggcatttaactagtttagattatggttattgttgatcctctatttactgatgttccatgccttttatgaagaaaaatagctacctaattctctttcacccagtgaactatatattagagttgttgttgtttaattggaacagaaaaatagtttgatgaacaagctctatttttcttacccccaaattaattaccatcacttcaaggaagagagagggcaccaactctatttggaagctattttacgatctagactcccccacacacagtatcataggtgtctcatgtggatcacagaacacaggcaacataacaccagttgtagaggaaaagcctggcagagattccaagaacagcttgtctggggagtcctatggcagtaggccaagcaggaagaccatcgcggtaccttctggatggaggtactttcaaaccgggaggcccatccacatttcagattccactggagttctaagacctggtgtaacaggttctggtagccaacgacaatcccagcctaaaagtaggatttggcaatacagataacattcactctcttctggggcctagcaactcttcaacttttatctgtagtaaaaacagatgccaaatattttagctaacctggaatcaatgaaatatcttctcttacacttgtaccactactaataaggaaaacagataaaggggcatatgcattagatggtaccacagaaccctgaattcaactcggacccaagcaaaaattgaagccatcatcctgattataaaacccagtgagcttgatgcagaaagccactcctctctaggaataatcatgtcctatcacatagggactagcagcaagactgatttatccatgctaacggagggtataaatactcaaacccagaaaaaaactctggtatctgactccaggtctaaaggccagttgcccagggcatacaccacttacacagaaatgggtttccaaaggctacattgaacagccccacatctgctaggggatatgaaactgttcaggtccataggggctgaggtgttgcttgttttgcctcagctttccctaagctttcactgaccagctatcataggtatgagcgtggggacctaagttcaacctggctagagagcaggcaagccttcttaaagcgcagaggctccacagtcattagctaaggcagcaacgcctcctgctcaccagtgttggggaagagacttttgccttaggccagctgattgattacagtagttgggccaagtcctgaactgcatttccacaatgcaataataactactgcaagcaagccattatctggctaatttcctaaaattaaaaaaaaattttgttgttgggtgtggtaagggaggggtggtcctcactatgttgcccaggctggtcttgaactcctggcctcaagtcatcttcccactttggctaagtgctgtaattacaggcatgagccactgtgctcagccctaaaatattgttagagaacatttacagacataaagatgagctcagtctcatccttatcaatctcctaaaaggaaaatttaagatctagtacttataatcctgtcctcaaagcaaacctaaaaataactgtctctctgatttgttttacagaatcatttatagttgtgtctgtcaaatagcaagaatcattcctagccagtgatgtggttatcacttatcttatgtgagggtaaacctgcaatatcttagagtcctttctaaaattatacagaagtcaaaataacctttccaaaaaggagtactaaaaaactgtcactgatagaaaacatcaactgtatgccaaagtactaaaaaacaggcaatcattccatttcagttgtattcacctattttcatcagtaggcagggcagtgctatcagaagagtaggctgcccttctatgacgacagaagctgttcctgatacttagttctgccttgcacatagtagactcaggtatcagtaaaatgaatgaatgaattatgaaatacactgactggtgagtcagacgttttttaacattccaggaaaaaaaagaaggctgaaattcctaatgaaaaaaggatgtctcattgagagatttttgcattactctttctgtatacgaaagcttgttgtttagataaattaccacaacacaggactttcacatacctgtctttattttgcttttatttgtgatttgatttaaataaataagaaggttcacacaggttaataaaaagacaagcaagtttgttgtatggctgagaaataatatgctctcttggtgtatactgatggcattatcggataacaccatgaggaccctcctcttcctcatttcctgggtcagtcctggtcagtgcttcttccgcctagtgctccttttgtatcacttatgtacactggatggagagaaaagaactcttctatgccttagtcaacatagatagcagcaggtgagaaaaagagctgatttctgatgtaacagaagcagactgactcctgctagctccagatacaaaatgctctacaggatgacttactgtaagtcactactgataagttgtttgcgtgactgctgggagacagatttacagagttctgtgacagtctattctggtcttgctcagtttggtcaggagcaggagcccatgtgtcaggagcaggagcccatgtgtttttgctgatcgagtcgaactcggagcccccagggtcttttaagttgttttcatctgattgtcggttcttttggggagaggcaaaagggttgaagtttccttctaccttacgatgcggctgtgtgttgaactccgtttcaaaagatgacagctgctgcgttactcctaaaagtccacccacctccacactgagaatcacccagatgacatctccatagtagagtcctgtagcagtgcacatccgccactgtccctgatacattcctgctctgctggggctgcacatctggacgctgacatctgcaatctcttggggctctagcgatctcaccatcaccatgttcacatgtccaaattggtctcccccgacatatttaagacaaacccctggaggccaggcctctgccccagaattctggatccgccatgtttttacaaactgagtatccggaggtattgactccccttctcctatggtgacatcttcaacaaaggacatagagggcacactgatgtttgggctctcaaagtcataataggcgccaattgctgcttgtaggttccagttggtcatgtccaggaagaaggcgcaaccggcaggattgagctggaagccgagcagcctctggaactcggagatgagcacgtccttgtcggtggtgcccaggcagctgaacttctgcatcagctccgggtccaggtctacgtccatgccctccatggcggggaccggacacccgcttccccgcctcttcacaaccaagccgccgccgcgccgccgggcccggggacctggaggggggccgctgctagctagcttcgcgaccccgctcctttgaggtaggccccgggcctctcacagtctcataggggtaaactcact

SEQ ID NO: 8452 - RNA, 4894 nt, Homo sapiens
  source 1..4894: mol_type = other RNA
aaaagtaattgcagtttttgccattgaaaataatggcaggggagactcttgatcttatcattcaaggctttctgttgctcaatgttatattaaaaacaatgaatttccatactaatttcaaagtcaattcctaagatactgtttcatcccattgtgaacaccaccaaggtcagttatatgtttttcagaatacttgaagtacgagaaaaacagaaatatatagctctggctacattaaatatcttttgccactttctgagatctttcgtaactctaagagaaacatggcatttccattaacgaaaataggagctttttgaataggattgttcaaaattagatacaaatgttctcagctaaaggtctcacatattcagaagtttgggtgccttttgtgatagctcttgtatcatttgataatattgatttttttgaaaaaggcaggctatttacaaggcaaagagtttttgttttgttttgttttgtttttgagatggagtcttgctctgtcgcccaggctggagtgcagtggcgcgatctcggctcactgcaagctctgcctcctgggttcacgccattctccggcctcagcctcctgagtagctgggactacaggcacccgccaccacacctggctaatttttttttgtatttttagtagagacggggtttcaccatgttagccaggatggtctcgatctcctgaccttgtgatccgcccgcctcggcctccaaaagtgctgggattataggcatgagccaccatacccagcaggagtttttaactttcactttctcaagtagagaaggccctcaactgtaaacccctttaccctagtctctgggaaatattcctgcccaccaagcactctatcccccccagcccccagctccactgggttattctagggtgagggagcggacatgatcatccagtagcgtctgaccagccggaaggcaaaagagacaagcaaaagttctgtgttacccaggagagctcagctgtccagaaataattagagctacagccacacgtggttcaaggaaatgtggttgtcagagagagacagagatctgccaagccatctcctcttcaactgcctgggcggagggggctgcagcccacattttagagacacagtattgtttgcagttgatttagaacttgagctggaagaagtcccccatcatgacctgcacaccattagaagaaagtgttgtctccaacaagctcagccacaatgttggctgccaacggtatgtctttccccactcattggaaaggagattatcacactaaagcattgagatgaattccgatgaacaaaggtagtcagaccgttaggctggactgtcactaggacatgatgacaatgaataaacttaggctcttgcaatgtccatcactgacatgttttaataagagttgaacgcacaaattggcttccttgcaatgtttacttcaagcagtaggtctgtctgctctggcctttgatgggatctgccagcttcctccctccttgtctatgtcccctgccttcaccatgggaaaaaaggctccagtaaaccaaatcccagaagtgatgttgcctgcggagaccaactcaaaaccaactggcctcccactgcttcctttgaaaacatatacatttcacacacctgagtcctcccacccctctccactccacggcaggctccatgaatggaactccaggggctgcctttgtgtaatgatcaagacgtccctggacagaggagcagcttcgcatcagggaatcctggtcccctgatccccatgggatgagatggtgggtgtagcatccttctggtttctctgcccattcagctgtctacccatgcacaaaacccaaagccctggattttggattttgtacctgcaaacctgagtaaactttttcccctcaagagtcatcattcaggccgggtgcagtggctcccacctgtaatctcagcactgtgggaggccgaggcgggtggatcacttgaggtcaggagttcgagaccagcctggccaacatggtgaaaccctgtctctactaaaaagtacaggtgggcacctgtaatcccagctactcgggaggctgagacaggagaattgcttgaacccgggaggcagagttgcagtgagccgagatcacgctactgcactccagcctgggcgacagatcaagactccgtctcaaaaaacaataaaagtcaccattcagcctgaccaaggagggggccaggaaagaagtcggaaccgtggccttcgctgcttcagaaggggaggcccgtgctctgacttcagcttgattcactttggcctcagtcctcagttcccagggggtaacggcgttctgaggttgtcacctggtgcaagaccagctgtccccagggacacatctggatctcttggtgccaacaacggcaactccagagggggctgggtgggggcatgtggctccagtttgaatgcaccatgtccatctgccagagaatccactggtcaggctctagggaggcaaaccggggggcccctgccaggaaatagctgctcagaccacacctagatcgcctgcaatttcaaagaagaaagcctggggctgtgagtgtgggagaaacctactgaacaggtccggtgggtggacagcaggtgtcacatgggcctgagcctggacggtatctacagagagatattttggttgttcactgagggtttggccgggtgactctgggtggtgtctgattggttgctggcattaccagaccctcctaatatgggtagtcttcccatgtagatccacaggttatgaacaaagctttcaccacatatacagagaaccccctagagcaaacatctccccatccctgggtggacctcaatgaagatgagcaaactgagtcaagacacaaaaccctgttggtccaggtcatactcttgggtgagttcttgatgtcggcagtgacaatcagtgccccagttggggcctgccagccccccaagctctgcagcctcaaagaccagctcagtcccccatcggtcactattcctgagagccagagttcgacctggtaacacctgcaccgtgcattcctcggccgaccatctcctggccccactcccggtggctggactcctgcagtcctcggcctttggtctcaatgggcaaaaagcaggaggccagggcagccaggaggcagcagccactgtaaactgccagagtcaggtacacagaggattccagcatcacctgggcgatgaacggagtgatgagagcacccactcttgccatgccgctgcaggtgcccaggccgagggcccgcgttgccgtggggtagacctcaggtgtgtaaacatatgccgcttgaaagcctccagaaataaacgctcttgcaatgaagagtaacagagtgagcacatttcttccaacacagataaacagcaggaggctgcagaaggagaagatgacaaagcacagggccatggtcttcttgcgccccaggcggtcaataatccacagagtcacaaggacacctggaaactcagagagggtggtccacagcaagtccatgtaatcctcctcactcaggtactcgcaggccaggctgcattttgcctctacagccttcttccgactggagatgccgcagacatctcctgcctggaagagttctgtggtgagtagaactaacccgtagtaagagaatgcattggaaaaccatataaaccacagcagcaaagttgtccatctaaaatggggtgtgaaaaggtccctcattttgcctcggtcttcctgtctggagatgatgagtttccccagcggcatgggagctccgttttcagttgctatcctctttaaggtggcgattgccttttcctggttccctgacagcacatcataccttgcactttcaggcagccagaaacacagcacggcaaagaggaggagcgggacagctgagaggatgagcagccaacgccagcccaggctgggcatcacgaacacagccaggacgacctcgaacactgtcccgatggcccagaatacctcaatcagcaaaatacatttagctctggctttcatgggaaggaactcggcatacagcgtcaccgactggggaactcctccgatcccgaagcccaccaggccccggagcaccaggatccagctatacacgggcgcaaatgcactaaggatgccatagtacagagtccacagcacgctgatcttcagccctgttttcctgccgtactggtctgagatatttccccagagcgtggagctggacatcatgcctacaaagaccaccgaggtcagcaatgccacctgccagcttgggagcctccactcgcaatgcagctgtggtgccaggatgctgaggatcatcatctccatggcatcagccatccaagccaagccagtgagaacagacagcttccactgaaattttccaaagccaatggcttccactgcatcttccaccatgaaagtatcatcagtgggattggcaaactccttgggcacagctgccccatcatccagctccacagcctctaggcccacgtggaccccttcaatctggacttcatgctctcctgaagccgtgtcgtcctctgaccttgcactctcgcctgtgcgacggaatttcacaaccggcagctgccttagctggaataagtcctcctccatgtccgcgctgcgccaggatgagcccttctcatggcccttacatggtagtggtggatgacgagccctccggttttcagcaccgggaagctggacagcacccgcgccgcttcctccctggagcagcagctgttcggggagggagccgctggggaccagcccacgagacaaagcctccgccgccaggagaccgcggcgagagt

SEQ ID NO: 8453 - RNA, 412 nt, Homo sapiens
  source 1..412: mol_type = other RNA
aaaagtaattgcagtttttgccattgaaagtaatgtcagttacttttgcaccaacctaatacaaaccatcccatatctgtgttctccatcctttcatcctttatcacagtggggttgtgatagatccctgaaaacacaggatcaagtataggtaaatgcaagatggtacatagaatcaagtgtgaaagtgagtcccatcaacccacactctttccatttggcccagttgctgcccttgttgtttagaatggcacgtacctggccttgaaatgcactgaagcctatggggattactttaaaattcggtcctgtaagccagtctgttagtatcattgctcctactaatgatagaaattgctggtgttggccgggtgtggtggctcacaccagtaatccaagcactttggcagac

SEQ ID NO: 8454 - RNA, 84 nt, Homo sapiens
  source 1..84: mol_type = other RNA
aaaagtaattgcagtttttgctattactttcaatgacaaaaaccgcgattacttttgcaccaacctaatacatgcagaatcaga

SEQ ID NO: 8455 - RNA, 6557 nt, Homo sapiens
  source 1..6557: mol_type = other RNA
aaaagtaattgcggtttttgccatacttttcatgacaaaaccacagtaacttttgcaccaatctaacagcatgtagttccttggagttgttaagattgaggtctttattttgtgttgtcttcagctggggaatgctcttgactcctaaagggtctcatacttccttgccaagtggaattctcacaaatggcaactgatttcttcaaaggtggcaggaaatctctctccactgtgctgagatggagtcttatataaagaaacaaacacaggagtgaatattgccgcgcctttgccatataacataacgtaattacgggaatgacatccaccacctctaacacagcaagcctagagttccatctgcagtcaagaggaggggcttatacaaggatgggattcactggggatcagattggaattctgcttaccataattattatacccagagcatttttcttacccctttagatatgggttttcctttgtctagtagggaactactagacatagggtttgcctgtgtctaaaaccatcaccttcacagatgacttgaagtccacccatcctcccgttgaggtttccattatatgtataatcctcttagggcacttgctcactctggaatgtgatacagtttgcagggtcttctcccccaatatacagaaatcttcttccaagcagggaactagattatattcaacctcacatttcctctcactcctcactctgtactgtgcagcatagtgctttctacataggcagtagctggcaaacactagtgaaattcaataaatcaaagcatagaaattacagaatatgcaagctaaaacagagcttcggggtcacctagaccgagctccttcccttatttctcttggctggaggctattggcatctttttgtgtttgtatgttccatctgctatcaaacatttttatgacatttatttcctcattatagtccttattgtgctttatttatatatctgtgaggcacgggagaatttccaattctcctttcccctgcaagcctgctcagactcctaatgcccatgacaggcccccagggctcccgtgacaacactactccccacttccctacgtgtctctctgtctcctctgtccctccatcatcaatttcaaacttcctgccctgacattcaaggcctccttacactttgagtctgtctgtatcacctcccttattttctctgggtctcattccctaactcccactcccaattctgggcatttctccaagtttctccatattcctggaaccatcatcccactctctccctcccccacccctcctatcatctgtcaagacttcccccatttcttttatcttccctaaccctaaaaattttgaaagaactgtcttttgacacactaagtacatgtagatttgatattctatgagcaaatattggcccatgactgttcaaccattgaaacatatacataggacagatgtgagaataccttggtctttgccacagtgaaaatcataagcaaagcttttaatatcagacatggtaaagtgggaaggaagcctaccatcaaacagaattaagctgtcttgatttgcccgcctggccaacttaactcaagaaggatacaaattatttggggcttgatctaacaccctaataggtcttttgctatttcaggtaaagggaaggctaggcattggacagatttttaaggtgagctctcatagttactagctgctgtgattttggataaattatataaactctctaacattgcttccttacttccaaatagaaattatcttaataataatacctgataatgaaacaaattaacatgtacaaaaacatccataacaaattgtaaaatgcatgtaactgacactcgtaacctttcacagcagcatttttgagtgcagcttgtgtcagattctcagtgatcgactgtgggagagcctccaggttccctcaggacctcaatttcctcatctttaatattggggtaataaactcctgccttgcttatctcaataagctgttttgaagataccctaagagaaaagaaatggacaatttaactcaggaaggtgtgagtttgaatcaaattttcagaatttatccatcaacccaacaacctattgtgtcattgagtgagtttagggcataatttgctgatttagggagttcaggtactggtaactgattatggaaaactctgtgatagactcttctccgttctcttcaagtaaagcaatattgcaattctaaattagaatactttaatagattacttggcagttttgcctgccctcagtgtttggaggagggcagaggcaccaaagaagcacaacagcagggaatattagttgtctgttgttgtgtaacaaattaccataaacttacaagcttaaataacaaatttgttatctcacagtgtctgtaagtcggagtcctagtacattgtaacttggttctctgcttagggtctcatgggagaaagtgggtcttgctggccaggcaggggtctcatctagggactctggggaagaaattactcccaaactcacccaggttgttgccaaattagttaccttagattactggttgttggaataaggtccccatttccctgctggctgccagtcaggggttctctctgctcctataggctgcgcatattccccttcatgctttctatagggccctccatctttgtagcagccagggtttattcaggactcacacttcaaatccctccaacttctctttcagcctccagctggaaaaagctctctgctgttaaggactcacatgattatatcaggcccacttggataactcattatttataaaagcaaatgtattgtgatggtttccactgaactgggaaacagggttcccagattaaacattatttctgtgtgtttctttgagagtgtttccagattatatcaaaatttaaattggtggactaggtgaagcaggtgaccctgcccaatgtgagtgagcttcatccaatccagtgagagcctgaatagaacaaaaaggtggaggaagggagaatttattctctctctgcctgacagcttgtgctgagacatcactcctctgccctcgactagaaattgtgccattgaccctccagttctcagaacaacagcaccaactccctgtgtttccagcttgcaggcagcagatcatgggacttctcagcctctgtaattacttgagcagcaaattctttataataaacaggtatcaacttcttttgaaaagtcaaaagatctggcaacactgtgcccatttctccccatgacaataacaggctggtgcctccttgaagcagcttgtgcagctccaattgttgtagttccattactcacttttgtgttgcacctggtctattcactctctcatgtcacttgcctgctccttgaaggcttttgggctggcaccacttgatcttgtttaaccaactcattttaccgataagaaagcacactgaagcatacattcttccagttcatggagaattttcagtatccaagtgatattacatagaaggtgacatctcctcagggtgtttatggattgttgggagaaaggtgggtttctttatcattctgtcatcaaagatagctgctttctacctagactttctgggaacaaggaaggattaaatgaggaattttaataatttcacattttattaagcctattttctttttgtttgttttgttttgtctttacctgataaactactaagatttaaaatgaattggcctacatttttgccaattttttacctctaacttcccaaaaaattctaagatcagtaaaattgattaaagttattaaacaagtagggaggaaaagacacatttaagagcctggataaaacagtgatgggaaaatccacacacgattgacttacttaactgtatttaattaggaaaaatctctagaatttagaggaaactggaattttcatctgagaagctccaggttgtttacagttcaacttgcctcagtttgcctcactgagccactgagccactgagccatgctggtataaaaggagcgaaggcaaagaaaaacaaggacctcacctaagggagagatgggacagaagatccagccacctgcctgagcaagaggagctgtttgctgtgggactctgagcaaagagtagtgacttaccaatgacctttcctcttcacgcttcctgggactgtctccccttttccatactgtggaactgtcccttccacataaatccaaacatggatcaccatttttgcgcctccaaaatgggccagaagacacatccctgaccacatcataacccagaaagccagatgctgatgacacacttcgcagccgagatctcattgccttggtatctgggaccacaactaagtactttccaactgtattgttacctcattattattcaaatttcatctgtattggcacgttaattaagtaaagatttggaaaagaattgtgcatatgcttcaaatctagaaaaagttttgatggctgtattctcaatggaaaagtgatgttttagaaagagggatgacattttataacattagatggcattttcctggggacaggggaacaggaacatatgaatcctgccttaatctcacagctttttcctgtaatgtccccataaaaacaagggaccacagcaaatgagaaattaaagtccgcttcattattagcctggctaatgccaaataaacaaatgcagaactttctggtaatttgcctaggacacatggcatactctcagatcacagtccagaccaccaaactctaaattaaatatcttatcttagaatcttagcatccttgggctgctcacatggaacaggagacagaagtaataaataaggaaagtattgcatggaaaaagaaataaaattaacctggagaaatttcagagacagggtcttttattaaaacaagacaacaaacaaatgaaatgtactctaccataaaaaacagctcttctataaaaagttatctgtcatcaggcagacagatcttctgaacctaatgtctaagtgatagatagagagggagtgtgtgttccagcataaaaccctgagtacaagaagaaaagaagagatggctaaactaaggccctgtcaccaatctagccataagattaaaggagaaagtaaattttagcctatgatgaacttcccactagtgaatatggaccaccccagcagcagagaatccaacatagtttagtacctcagtttcttaggaaaaagtgaagaacagggcaagagggtgaagaaactgtttccccaaccccgtacaagtcaaagattggttaaaagagaaagaaaggcttttatttattttgaggttgttgttttattgtcgtcattaatactagagttgtgagtcccttgcaccttggaggggaatttatacgggaactcctgcaaccatcacatgtacatctttttttagagtaagatattgcaagaagcccacaggtcccagcccatacattgaatggttcaagttaaaaaaataataataatactaacccttgttaacctttgcctagcaatcctgaccctcccagggtgtgagaatccaagcaagaatcacagtgacagctatgcaggtatcaaaaaggagcctcagaaagattaatttgaccaagatctctgtattagtctgttctcacgctgctacgaagaaatacccgacactgggtaatttataaaggaaagaggtttaattgactcacagttctgcaggggtggggaggcctcagaaaacttacaatcatggcagaaggtgccctttcacagggcagcaggagagagaatgagtgccgagcgaagggggatgcctcttataaacccatcagatctcatgagacccactcattatcgtgagaacggcatgatggaaactgcccccatgattcaattatctgcatctggtcctgcccttggcacgcggggattattatatttcaaggtgagatttgggtggggacacagagccaaatcatatctatctcatagctaataaatgtgatcttgggctaagtccagagtctatgctacagtcattaaaaaaaaaaaaaaaaaatctgagattctcataccagaattgtacaattaattacaacaggttttggaaatcacttgattttttttgtctcattagccattgcaatttggcctgcataaaaatattcaaagtagacactgaattactctatgttttctgtatacaaacggagccaagcaagcattgttcaccatgttctttgtagcattctctaaataatttttctttcaatattatttttgattgacaaaccatgattgtatacatttgtgaggtacaacatgatgttttgatttatgtatacaatatagaatgattaaatcaagcaatttaacgtatctatcacttcacttacctgtcacgttttattaagacatttaaaatgtactctgtggccaggtgctgtggctcacgcttataatcccagcacctcgggaggcagtac

SEQ ID NO: 8456 - RNA, 4505 nt, Homo sapiens
  source 1..4505: mol_type = other RNA
aaaagtaattgcggtttttgccatacttttcatgacaaaaccacagtaacttttgcaccaatctaacagcatgtagttccttggagttgttaagattgaggtctttattttgtgttgtcttcagctggggaatgctcttgactcctaaagggtctcatacttccttgccaagtggaattctcacaaatggcaactgatttcttcaaaggtggcaggaaatctctctccactgtgctgagatggagtcttatataaagaaacaaacacaggagtgaatattgccgcgcctttgccatataacataacgtaattacgggaatgacatccaccacctctaacacagcaagcctagagttccatctgcagtcaagaggaggggcttatacaaggatgggattcactggggatcagattggaattctgcttaccataattattatacccagagcatttttcttacccctttagatatgggttttcctttgtctagtagggaactactagacatagggtttgcctgtgtctaaaaccatcaccttcacagatgacttgaagtccacccatcctcccgttgaggtttccattatatgtataatcctcttagggcacttgctcactctggaatgtgatacagtttgcagggtcttctcccccaatatacagaaatcttcttccaagcagggaactagattatattcaacctcacatttcctctcactcctcactctgtactgtgcagcatagtgctttctacataggcagtagctggcaaacactagtgaaattcaataaatcaaagcatagaaattacagaatatgcaagctaaaacagagcttcggggtcacctagaccgagctccttcccttatttctcttggctggaggctattggcatctttttgtgtttgtatgttccatctgctatcaaacatttttatgacatttatttcctcattatagtccttattgtgctttatttatatatctgtgaggcacgggagaatttccaattctcctttcccctgcaagcctgctcagactcctaatgcccatgacaggcccccagggctcccgtgacaacactactccccacttccctacgtgtctctctgtctcctctgtccctccatcatcaatttcaaacttcctgccctgacattcaaggcctccttacactttgagtctgtctgtatcacctcccttattttctctgggtctcattccctaactcccactcccaattctgggcatttctccaagtttctccatattcctggaaccatcatcccactctctccctcccccacccctcctatcatctgtcaagacttcccccatttcttttatcttccctaaccctaaaaattttgaaagaactgtcttttgacacactaagtacatgtagatttgatattctatgagcaaatattggcccatgactgttcaaccattgaaacatatacataggacagatgtgagaataccttggtctttgccacagtgaaaatcataagcaaagcttttaatatcagacatggtaaagtgggaaggaagcctaccatcaaacagaattaagctgtcttgatttgcccgcctggccaacttaactcaagaaggatacaaattatttggggcttgatctaacaccctaataggtcttttgctatttcaggtaaagggaaggctaggcattggacagatttttaaggtgagctctcatagttactagctgctgtgattttggataaattatataaactctctaacattgcttccttacttccaaatagaaattatcttaataataatacctgataatgaaacaaattaacatgtacaaaaacatccataacaaattgtaaaatgcatgtaactgacactcgtaacctttcacagcagcatttttgagtgcagcttgtgtcagattctcagtgatcgactgtgggagagcctccaggttccctcaggacctcaatttcctcatctttaatattggggtaataaactcctgccttgcttatctcaataagctgttttgaagataccctaagagaaaagaaatggacaatttaactcaggaaggtgtgagtttgaatcaaattttcagaatttatccatcaacccaacaacctattgtgtcattgagtgagtttagggcataatttgctgatttagggagttcaggtactggtaactgattatggaaaactctgtgatagactcttctccgttctcttcaagtaaagcaatattgcaattctaaattagaatactttaatagattacttggcagttttgcctgccctcagtgtttggaggagggcagaggcaccaaagaagcacaacagcagggaatattagttgtctgttgttgtgtaacaaattaccataaacttacaagcttaaataacaaatttgttatctcacagtgtctgtaagtcggagtcctagtacattgtaacttggttctctgcttagggtctcatgggagaaagtgggtcttgctggccaggcaggggtctcatctagggactctggggaagaaattactcccaaactcacccaggttgttgccaaattagttaccttagattactggttgttggaataaggtccccatttccctgctggctgccagtcaggggttctctctgctcctataggctgcgcatattccccttcatgctttctatagggccctccatctttgtagcagccagggtttattcaggactcacacttcaaatccctccaacttctctttcagcctccagctggaaaaagctctctgctgttaaggactcacatgattatatcaggcccacttggataactcattatttataaaagcaaatgtattgtgatggtttccactgaactgggaaacagggttcccagattaaacattatttctgtgtgtttctttgagagtgtttccagattatatcaaaatttaaattggtggactaggtgaagcaggtgaccctgcccaatgtgagtgagcttcatccaatccagtgagagcctgaatagaacaaaaaggtggaggaagggagaatttattctctctctgcctgacagcttgtgctgagacatcactcctctgccctcgactagaaattgtgccattgaccctccagttctcagaacaacagcaccaactccctgtgtttccagcttgcaggcagcagatcatgggacttctcagcctctgtaattacttgagcagcaaattctttataataaacaggtatcaacttcttttgaaaagtcaaaagatctggcaacactgtgcccatttctccccatgacaataacaggctggtgcctccttgaagcagcttgtgcagctccaattgttgtagttccattactcacttttgtgttgcacctggtctattcactctctcatgtcacttgcctgctccttgaaggcttttgggctggcaccacttgatcttgtttaaccaactcattttaccgataagaaagctgagtaacagagagattaaatagtatgttcagacagcaaggacaagtctcctaacccatgccacgccaccaaatttcttagtgtaaattttgctgtaagcaatatgtcttttttaaaaaaaaattcaacttgtattatagattaaagggttcatgtgcaggctttttgtacattttcctatttttaaaagtttgtataggccaaacagtatttagtctgtgagtggtcagtttgaaatcctttaaataagtatatctttaagccacctgcaactgaaaaaatatatatatttctgtttttcatttagagatataaacttaggtatgaatactgtaatacggaacatatttattgcatacattgggaaaacatctcctttaaggtatggttgtcctaggtacacaaaatattttttgtcttcccttaggtggtttgtttatccaacactccatttggtttagaaaaacctccttatttgcttcaaggaaatcaataaagactctctaaacctccttatttgcttcaaggaaatcaataaagactctctctctgtctctctctctcttcctatctgtgtaagaataggtgtgtgtatatatacatatatatctcccataggtttctttttctgaaaccccctaatacatgtaccatatagcataacacaaaatcacaagaatatttcatcgtatttacaaatttagggtattatgtcaggatatctcagggaggaagaggtcattttagaaattctgtttaccacactgaagcatacattcttccagttcatggagaattttcagtatccaagtgatattacatagaaggtgacatctcctcagggtgtttatggattgttgggagaaaggtgggtttctttatcattctgtcatcaaagatagctgctttctacctagactttctgtcacgttttattaagacatttaaaatgtactctgtggccaggtgctgtggctcacgcttataatcccagcacctcgggaggcagtac

SEQ ID NO: 8457 - RNA, 86 nt, Homo sapiens
  source 1..86: mol_type = other RNA
aaaagtaattgcggtttttgccattaaaagtaaagcaaaatccgcaagtacttttgcaccaacctaacagcaatacttgagaaaag

SEQ ID NO: 8458 - RNA, 3892 nt, Homo sapiens
  source 1..3892: mol_type = other RNA
aaaagtaattgcggtttttgccattaaaagtaacggcaatgtgccatatatataatacatgtgccatatatataatacagtaatgcattgcttaacaacggggatgtattctgaaaaatacaccaataggtgcatctatctgaacatagaaaaagtagagccaaaatgtagtagtataatcttatgggaccaccattttatatatatatacatatatatgtatatatatatatatgtgtgtgtatatatatgtgtatatatatccatatatatatatatatataatccatatatatatggtctgtcatttactgaaatgttatgcagtgcatgactgtatatatacaattatataatgcacgtaaaagccagatagttagaaattttggtacaagctgaaaaggaaatgaatagggtgatgtcaagaagtgttaatggagtaatcggggagagctggcagaagattctcttgctagggggactggctttccaacttgtagctcaatacaaatgcctgtgaatacaggatgtccccctgcccacatgctaggaagggctgtgtactgtgtctaagggtgcctgaactgttccaaagggtaagaatcagacaggggccctctctgctaagagcatttcttgagaaggaaggtcctcaggaatgcagtgctgtcttccatcctgggatattcctaagagaggaggaggcagcaggaggaactccatagtcacaggtactggaaatgtgctgcttacactgtgaagatcaaaactgtgctcccagacagcatgccgtgctgtgaaattgtaaaacctttctgaagcttgaacctttttataactggatattctctgacataggtgttcaattctttcactgcaaagggcactgaatttactctgaaggtcagtaggaatcacttcatttagagaatttaggctggtacagttttgtacaaaatgctcatcacttttagccagggcttcaagaatcttggcagttaagctgaagaaacctttgggctcaatcatcttttccaccacattgcacttgatgccagctgtgctgtcgtactcatacacgacaccatattccaggtggacattgtccactgtcagactcacatgctccttcttcccatcaatgatggccatagtgttgaatttgtcaataacctcttctactttacagtcaaaagcatcccctgcttcatctccagggggcttggagtgagatttttgaaggtcttcttgagcactctcaatgctattataaacccattgtatggaatcttgcttcgttggccgcctgtacttcctgcaggctgtaacgtgtgcaatgacactggcatgtgtctctttgctgacattgattccattcaccttgataatgcactgtccagggtgaagaccagctgctgcagccacagttcctcttcctacagcatgcacaacagaagggccaaatccccggatctggaagccaagtccatcagctgaatctggaattttcactgtctctcttggctttgtgctcacaagaactcttagaggttttctgctgtttaaacacgatttcaggaagcaatccacttcattgaaaggtctcataaaaactaggtcaccattaatagcaaaaatctttttcccgacttccatgccagccatctcagcattagatcccttttctaccaactttattattggaactttatttttgtcttctaatccaaagccatagctgccttcattggatttaatcaataatgacttagctataacattttccacaacttttaagtcatgtttcataagtcgatgtttcatatttgatccctccatttcctcatccgaaaaaaaacggaaaagtaggggttcatctttgaattcgcttttttcaaggacatggtgcataaatccattgtcacagagtccaacgccaaatatcattgcctcttctctggtgcggcaatctccctgtgcaattaaccagtctatcagtttgttggccatgaccacagatttgtaggtccttaaatggtaatctttatctcttatcactggagtaaaaaggctatgaagacgacaatataatcttacaccctttgaaatcacgtcctgcatctcatttcttggataaaatgttccatcatcatagcgaaatctatataacatctgttctggtttgaattgatgtttatcagtaacatggtgaatgattccattttctaataatgcttgtcccaagtgcacgccttcctcaggcctgtgaatctctccaatttccaacagccatgacacaaattcgcttccaagaaagcatttagggaacgtagtcagttttctctttcggtctttgatcagatttccttgtctgcacatcattttataaagtttctcaccctgttcagagatcatgacccaggtatcttgctccattcctaattttaaacctttccgccgttctctttctttcaaaatagcttcaaaccattcatgcttctcttcaggtgtttttgccatacaaacaaaccatttattttttgctgtgttatgtatcttccatccattaacaacaatgtgtccactgctatggaaatcagcggtgccatcatccacattctccacttccatcacctccgtgttgatccggccacgaaaaaggtaccgatgtccatctgtagatgccttgctgttcttcaaccgtctgtgttttcttttgcagtacaccaaaagattatcgaaaagaaaaaacacccgttcttgaatatttccagaagaaattttcagtaagactccacacattagcatttcagtgcaggtgtcagtgatgttggacccctcccagccttcaatgtgagactgccattcctctaaaacttctaacttctccatctgtctcttggcctcgtttatgttggaacagacagctttcatggcttggagggcttccatcactgctgcatagtcactgtgtttccgtggagtccgcttcagcaactccttcaaaataagagggtacttgcatattctttgtattggtgttactaaatatccttccaagggaacatctgtgttcttccgtcctccaagcagcatgcagttcaaaagaaatgtccggattgttcttattttgttgagttcaagaagtaatttttgtgccttctcatggttactacaatattcatcatagatacgaaacttgtctttaaagtgaagaaagcaggttcccacttcttgttgagcattaggttcggggtgtaagcattcttccacgacttttaagaattctttatgtactgcaaggatgtcttcaatgtttgagaacaacatcttcactgtttcttctgtcacatttttgtcaacttttgatgctgcacactggttcattctgtgtaagaatgccgacaccaggaactccagcgtgcccacatagtcccgctcggtcttctggagctcgctgagcacgcacacgcgcaggcgaagctgcttctccaggtccttggcgctctcggcgcggctgtctccgcggctgtcctcgctcatggtcggcggcggtgcgcagcgcggcgctgcccgccgtgctgagcgctgacccgcgcgcccgctgctgcccggcccccggcggcgagaatggaaagttgccgcctccgccaactccgaggagagacagaagactttacatgctggggagaggctgggcgcagggagaggaggggatcgggctgaaatcccggcgcggggggcgcggggctctgcagaggaaactcctgggagtgggggctccggccaggccctgcgcgcccggccccgctgctctggcctcacacggccggggctggaggggaagcggcttcggcagccacagcagtgacttggacattaatcaaaagct

SEQ ID NO: 8459 - RNA, 6847 nt, Homo sapiens
  source 1..6847: mol_type = other RNA
aaaagtaattgcggtttttgccattaatagtggcaaaaactacaattaattttgtgccaacctaatacattaaagttagggaaggcagctgtcatcagattttcaggtaattttaagattaatgactacagacaagtttagtagtagtcatttatttaatagtcaatgagacccctttcagaaaaccgtattgcaacatgcaatctattttaataaatatacacttagaatatggctgtatatacacatacctacacagccctacacatatacaaacttacacaaatatgttgctctcttttttttttttttttttttttgagacggtctcactctgtcacccaagctggagttgcagtggcgtgatctccactcactgtagcctctgcctcagttcaagcgattctcctgcctcagcctgagtagctgggactacagtggtgcgcctggctaatttttgtatttttagtaaagacagggtctcaccgtgttggccaggctggtctcgaactcctggcctcaagtgatccacccaccttgctcagcctcccaaagtgctgggattacaggcctgagccaccgtgcccggccatgttgcttttataattgagatatttcatttgttttgggggttaggcaaatttaatttgccattcctcaaactcagtaacttcaaatataaacaatgcctagaatgaatatggttcctcattatttctatcaaactactacaaatactgaagaatcccaaagtagttttccacagaggcagaaaagcagttcaggggttgaaaatcttcaatattaataagccctgggacattcaaatggcacttcatatttcaaggtaatgcaatatgaatcataattcattatatattgtccccaagagttacttcaattccgtattcaccagttcttacgatttggaaaaaaaaacttgaatgtttccagatgaaatctaatccccaagccttgtgtgtcaacattctagtgaatctctatttaaatgagaggcgctccaaaacacttcctgcaccactcgacactggcacttggtggagcatcaattttctgcaacctttcaagaatctctgaagacagactattgtatgcaattccatattcattgtcaaatgcctcaatatcaatattctctcttcctagagacactaatgataagaagaggatttctctgtataaactcctttgtcttttcatgcctggcttcatttgctgtgaaagtaggttgatgggtttaagaacattattgtgctgaatactctgcctgatggtttctactaaagtgcttgtttcttgttgttcctctgacaggagagatgatttcttttcagaatctgtacaccttcattacaatgttcagatgtgaggataagtcctggcaagttactaggaaggtccaaacgtctgaaataccaaacgaggttccagaaaatgattggatgttgattgatgaaagaagatgtatgaatcacctgatcaccttcattttctagcaaagattcaagttctttacggagtactagaggactcaagtagggcacagaaacagggggaggattgggtctttttcctaaaggatccacaacttcctgcagactatttggaagactaactgttgagatgccatgaaacggtcgctgggtaaagtcaatattctgcaatgggcctccaacactgtgacttcgagtcaaagacacatttcgctttgataaactattaggcacagatgaaattttcatagtttggacatctccactggctctctttatttcatcacttggttcaactgcagagcctgtttcttcagttatgatctggttatgttttgggaagtccataaagttgatcaagtcaggttctgctaaactggatacaggtttgtgctccaaggattcatttgccaatggaatgcttccactttgtaaactgtcaccagaggtacttggtttcaggaaaaagcttgcagaacctctcaaatctttgaattctatattgagaagaggcaagaagttgcttttacagaatggacaagctgtattcaaatttgagtcatctgctgtccatccagccataatttcttcatcataaactaaagctccacaagctctacactgtgaacaactggacatcaaaacctccattgcacaattctgatagatgctagacatgctggtattttgagaagaaccatgatctgatttttcaaagtcttgccctttcatgcctcttggaaatggaacttcacctgttggataatgcagttttcctacatctccactactgctgctactgccaagacttgtgttgctctgggtaagttcactggggaccaaccctgagatacttgtgttaggcgatatattctcccccaaaatatggtcttctaggccagctgggaagctgtagtctctattagtttcttcctcatcatctgagtagctgtaggcagacgcaacagctacccacatcttactggctactgtcgctgcttgtttcataccagatttcaggacatctatcttgggccctgagagtatattatccagctttagccctgacaaagaatttactacagaacccaacgagccatgtggcgaagaacgcaccagtgctgacaaagaagttgaacgttctttatgagttcgagagggggtttgctgcttgaaacgcccagtaaaagttttagacctggacactgcaggtgagctcttttcactttcaggattttcctgtgctggtgaaccatgatctaaaggtaggcttgatctcctctctagagcatgaataaatgcagtagtcatgccagactctctgttttcctctctgtgtaattccatactagaagatttactacctaggggactttttaggttcatatagctttctatttcatcagccagattacgtgcaataactggagaaaacaacttatcttcagaatcaggagtttttcctcctgtacattcagtggctaaaagagacaaaggatctagtccagtttcaacatcttccctctgaaccaccttagcaataccatataaactacttctcttattcctcagatctttggatactgttttcaagtctctggactgattactgttactatcacttagtagactctcatatgtatctactgttgcagtagttttaggtacgtcatcaaccacaggctcaaggagttcttggctttcctcaagcatctctggcaccggagatgatctgtgctcaggattccaagtgctttcagacatacaagtcctactatcaggtaggtgacagctaacattctcaaagctatgggttcttgcaatatgaagtagagaagtcttaggacatgtcaatgctgctgtgagaatcttggcatctgctcccatcatgatagccatttcacttgaattcgaatccaaactactcttcttaagcaacattcctgctcgactttcagaactaaaactacaactcctctcaggaaaatgcttttgtcttttttctcctctatcaccattcttcttgagattagtagcttcgccaaagactgcatcttcaactggatcttgagtagaaaacagcacatttgatatactaccagtgctacttttcctgctgttgacatcaaatataccagacggaactttcacaatactgctgccccatgcaggaggttcagtaggactgtgaggctctggactaggttgtgaatgttttgccacaatagcagaggcatcacacacctcttctgtttgcatttttgttttagttatcaattctcttgctgcctgttcttcaggcacatgaatttctgcatcatcctttataagttcatccttagacccgtatccttggtcagactgaccacctgatgtggttaacattcaagggtagaattaatgcacacgtgtatccatagcttcacgtcatataagtctgtctgatattgaggagacctgtgacctttgcacagtctttttaagcggctgcctaaactgtgccaagccacgtaccacattccgtaccttcgtccataagaaaataccactgcgggtactgctaggccacgggctctccaagactaccttattataataaccataagtaatagcattaggctttatcctagcagttttcatttcaaataagactctcactgctaaaacaggatgaccccaaagtccacaaagctgcatcactactcgatagcacacctcatctaagggatccacatctgttttcctcatcttaataagtacatcatatgcctgctgaagtgctctgactttaggatgagaaactctaacataggccggaagacaaataaaccataaactgtaacaatgactaaacagacacttggcccactgtggtggatttgtataacatctcttcgccaatttatgagctgtttttatttcctgtttagttctcttagccatgagaggtggactctttgtaatgctattcccagtagggtgtctactaaaacaaagtttcaactcctgcggtctgtcaaaaagcttaaggtccagtcttggaaagtatttgtaactgtactttggtgacaggtcctttccatcatcaggaggtggctctggcggcattataaatacagtatgctcacttttctgtgaatcatctagttctatcaatctggtatcttctgctgaatcaaaatcaaccttatctgttttctctgtgcctttatcaggaaacaacttttctatgcagtcatcaaaaaatgctaatccagtatctttatcacttacaaaactgcattcttcaatgaaacgaataaaaatctgtgttttggataaaagggtatagaattttgcataggcacgatctcgactttttaaaaatccctgtcggtcaaacaatgaatcagcagctgtggctttatttgaaggagcctctgtgattggtctgagatatgttctatatccttttaaaatagacgccataaagcgcaaaaatgcctcttgaatttccatctcaagctgtgtcatcttcttttgccaggagaaatctgcttcaattggagtcatgtcaatcgctgagccttcttgagttttttggtgaactgaagacagctggggatacaatttctttaaggtgctaagtagatttttgcacggctttttgggaagttgcttccagttcatgttcttcttttcatctgatacatataacatgttcgtatccaagtcaatgcaaacaacatcttgtggtgggtcatgaagatcaaaataccttgagtcaactccaactataaatggtaaaggtgcactaagcactgcagccagtgaaagaggacaaaggggaatatatgggcattgccactgaaatggaaagatcatagctacaacagcttcagctaccccagtcaagacagctggcctaagagaatgcagcagaattttactctcaagtaaaacaaagagcagcagtgttgcacaattctcaggacccagattcattagcaaggtgctaaagttggctccacttagtggtaaaggtgtagaaactggctgtgataatattaatgcatcatggactgacagctggacaaggattctcggtctttgtggtgaaggaaaagggatgttttgcataaaatgtgaaatgtgcttttcaatgggaagaggatgtggtccagacacagaaagtttgtagataaacataagaaatttcctaaaagcttcaaaaaaaggccagtgtgagagtaaacaaatgcatttgtttgtattgatggatttggagaccatttttctctccacaggcgtcaacaagcccaggtgcataagctgtttctctgatagaagttcccgagagtaaggttcataaaactgaatggcagctccatatacctttttggctgaagaacctgtcaagacaaaagttgaaaaaactggaagtggatatttggtttcaggatcccagcactcaatagtagctcccataggaaggcagaaaagaggtacatctgattctgagagtggaaatgactcatagtcctcttctggatatctaaaaattaaaccagccttatatgctattgcatttgaagcaggtacagacttcttataacacagaaacacgctggaaccccacattccacaatttaagtttttgtcaactttgcagaaggtatgaggaggagtttctcctttactggttacaataacacagatatcagttacagccaaggaattctggggtcgaactggaggagcccttcgataagtgataaagattctttgtgaagtagttgaactattgttgacattggcacagcgaccatagggtgtggctaggatcacttcacatcctggaataagccgttctttcccttcatatagaactccaatatctgtaagcggtggtttatctctccctctcttataacagaggaaaagttctgggcttttcagacttccatagttcaagtttgcttggagagctgatggagtggcttctacacaggtgtaaccttcaggtactgtttctccagctgatttgataataatggcaatgtctgtaattggagctttaggtccagttgacttagtatctaaacgatttatttcttgatccaaaagagtagatgtgtcagtgagaccagctacgacaaagtagtctgtcactcttggtcctttgtcttctatcatggctgctactgtattttctgctgcctgctcctctgtcagcgcagccccgacacggcttcttcctggggcaagaaagcaccggattcgcggactgggcgcgctcggcagggcagggcgggggactagctccagcggccgccgccgcctcagtccggtct

SEQ ID NO: 8460 - RNA, 6794 nt, Homo sapiens
  source 1..6794: mol_type = other RNA
aaaagtaattgcggtttttgccattaatagtggcaaaaactacaattaattttgtgccaacctaatacattaaagttagggaaggcagctgtcatcagattttcaggtaattttaagattaatgactacagacaagtttagtagtagtcatttatttaatagtcaatgagacccctttcagaaaaccgtattgcaacatgcaatctattttaataaatatacacttagaatatggctgtatatacacatacctacacagccctacacatatacaaacttacacaaatatgttgctctcttttttttttttttttttttttgagacggtctcactctgtcacccaagctggagttgcagtggcgtgatctccactcactgtagcctctgcctcagttcaagcgattctcctgcctcagcctgagtagctgggactacagtggtgcgcctggctaatttttgtatttttagtaaagacagggtctcaccgtgttggccaggctggtctcgaactcctggcctcaagtgatccacccaccttgctcagcctcccaaagtgctgggattacaggcctgagccaccgtgcccggccatgttgcttttataattgagatatttcatttgttttgggggttaggcaaatttaatttgccattcctcaaactcagtaacttcaaatataaacaatgcctagaatgaatatggttcctcattatttctatcaaactactacaaatactgaagaatcccaaagtagttttccacagaggcagaaaagcagttcaggggttgaaaatcttcaatattaataagccctgggacattcaaatggcacttcatatttcaaggtaatgcaatatgaatcataattcattatatattgtccccaagagttacttcaattccgtattcaccagttcttacgatttggaaaaaaaaacttgaatgtttccagatgaaatctaatccccaagccttgtgtgtcaacattctagtgaatctctatttaaatgagaggcgctccaaaacacttcctgcaccactcgacactggcacttggtggagcatcaattttctgcaacctttcaagaatctctgaagacagactattgtatgcaattccatattcattgtcaaatgcctcaatatcaatattctctcttcctagagacactaatgataagaagaggatttctctgtataaactcctttgtcttttcatgcctggcttcatttgctgtgaaagtaggttgatgggtttaagaacattattgtgctgaatactctgcctgatggtttctactaaagtgcttgtttcttgttgttcctctgacaggagagatgatttcttttcagaattaaaattcctccatgagacatacagaggttctcttggttcctgatgaaggttgatattatcccataacagctgaatatacacaagtttgctatcctgggacagagatgacagaggaagcacaacttcctgcagactatttggaagactaactgttgagatgccatgaaacggtcgctgggtaaagtcaatattctgcaatgggcctccaacactgtgacttcgagtcaaagacacatttcgctttgataaactattaggcacagatgaaattttcatagtttggacatctccactggctctctttatttcatcacttggttcaactgcagagcctgtttcttcagttatgatctggttatgttttgggaagtccataaagttgatcaagtcaggttctgctaaactggatacaggtttgtgctccaaggattcatttgccaatggaatgcttccactttgtaaactgtcaccagaggtacttggtttcaggaaaaagcttgcagaacctctcaaatctttgaattctatattgagaagaggcaagaagttgcttttacagaatggacaagctgtattcaaatttgagtcatctgctgtccatccagccataatttcttcatcataaactaaagctccacaagctctacactgtgaacaactggacatcaaaacctccattgcacaattctgatagatgctagacatgctggtattttgagaagaaccatgatctgatttttcaaagtcttgccctttcatgcctcttggaaatggaacttcacctgttggataatgcagttttcctacatctccactactgctgctactgccaagacttgtgttgctctgggtaagttcactggggaccaaccctgagatacttgtgttaggcgatatattctcccccaaaatatggtcttctaggccagctgggaagctgtagtctctattagtttcttcctcatcatctgagtagctgtaggcagacgcaacagctacccacatcttactggctactgtcgctgcttgtttcataccagatttcaggacatctatcttgggccctgagagtatattatccagctttagccctgacaaagaatttactacagaacccaacgagccatgtggcgaagaacgcaccagtgctgacaaagaagttgaacgttctttatgagttcgagagggggtttgctgcttgaaacgcccagtaaaagttttagacctggacactgcaggtgagctcttttcactttcaggattttcctgtgctggtgaaccatgatctaaaggtaggcttgatctcctctctagagcatgaataaatgcagtagtcatgccagactctctgttttcctctctgtgtaattccatactagaagatttactacctaggggactttttaggttcatatagctttctatttcatcagccagattacgtgcaataactggagaaaacaacttatcttcagaatcaggagtttttcctcctgtacattcagtggctaaaagagacaaaggatctagtccagtttcaacatcttccctctgaaccaccttagcaataccatataaactacttctcttattcctcagatctttggatactgttttcaagtctctggactgattactgttactatcacttagtagactctcatatgtatctactgttgcagtagttttaggtacgtcatcaaccacaggctcaaggagttcttggctttcctcaagcatctctggcaccggagatgatctgtgctcaggattccaagtgctttcagacatacaagtcctactatcaggtaggtgacagctaacattctcaaagctatgggttcttgcaatatgaagtagagaagtcttaggacatgtcaatgctgctgtgagaatcttggcatctgctcccatcatgatagccatttcacttgaattcgaatccaaactactcttcttaagcaacattcctgctcgactttcagaactaaaactacaactcctctcaggaaaatgcttttgtcttttttctcctctatcaccattcttcttgagattagtagcttcgccaaagactgcatcttcaactggatcttgagtagaaaacagcacatttgatatactaccagtgctacttttcctgctgttgacatcaaatataccagacggaactttcacaatactgctgccccatgcaggaggttcagtaggactgtgaggctctggactaggttgtgaatgttttgccacaatagcagaggcatcacacacctcttctgtttgcatttttgttttagttatcaattctcttgctgcctgttcttcaggcacatgaatttctgcatcatcctttataagttcatccttagacccgtatccttggtcagactgaccacctgtgctagagtgattatcaatggactcaagcctgattaaatctctgacgaagactgtgtgctccccattgttagcatcattagaactatccacactaccgtggctcaccgtgtccccatcacttccacctgtgacattttgaagagctgatattgaggagacctgtgacctttgcacagtctttttaagcggctgcctaaactgtgccaagccacgtaccacattccgtaccttcgtccataagaaaataccactgcgggtactgctaggccacgggctctccaagactaccttattataataaccataagtaatagcattaggctttatcctagcagttttcatttcaaataagactctcactgctaaaacaggatgaccccaaagtccacaaagctgcatcactactcgatagcacacctcatctaagggatccacatctgttttcctcatcttaataagtacatcatatgcctgctgaagtgctctgactttaggatgagaaactctaacataggccggaagacaaataaaccataaactgtaacaatgactaaacagacacttggcccactgtggtggatttgtataacatctcttcgccaatttatgagctgtttttatttcctgtttagttctcttagccatgagaggtggactctttgtaatgctattcccagtagggtgtctactaaaacaaagtttcaactcctgcggtctgtcaaaaagcttaaggtccagtcttggaaagtatttgtaactgtactttggtgacaggtcctttccatcatcaggaggtggctctggcggcattataaatacagtatgctcacttttctgtgaatcatctagttctatcaatctggtatcttctgctgaatcaaaatcaaccttatctgttttctctgtgcctttatcaggaaacaacttttctatgcagtcatcaaaaaatgctaatccagtatctttatcacttacaaaactgcattcttcaatgaaacgaataaaaatctgtgttttggataaaagggtatagaattttgcataggcacgatctcgactttttaaaaatccctgtcggtcaaacaatgaatcagcagctgtggctttatttgaaggagcctctgtgattggtctgagatatgttctatatccttttaaaatagacgccataaagcgcaaaaatgcctcttgaatttccatctcaagctgtgtcatcttcttttgccaggagaaatctgcttcaattggagtcatgtcaatcgctgagccttcttgagttttttggtgaactgaagacagctggggatacaatttctttaaggtgctaagtagatttttgcacggctttttgggaagttgcttccagttcatgttcttcttttcatctgatacatataacatgttcgtatccaagtcaatgcaaacaacatcttgtggtgggtcatgaagatcaaaataccttgagtcaactccaactataaatggtaaaggtgcactaagcactgcagccagtgaaagaggacaaaggggaatatatgggcattgccactgaaatggaaagatcatagctacaacagcttcagctaccccagtcaagacagctggcctaagagaatgcagcagaattttactctcaagtaaaacaaagagcagcagtgttgcacaattctcaggacccagattcattagcaaggtgctaaagttggctccacttagtggtaaaggtgtagaaactggctgtgataatattaatgcatcatggactgacagctggacaaggattctcggtctttgtggtgaaggaaaagggatgttttgcataaaatgtgaaatgtgcttttcaatgggaagaggatgtggtccagacacagaaagtttgtagataaacataagaaatttcctaaaagcttcaaaaaaaggccagtgtgagagtaaacaaatgcatttgtttgtattgatggatttggagaccatttttctctccacaggcgtcaacaagcccaggtgcataagctgtttctctgatagaagttcccgagagtaaggttcataaaactgaatggcagctccatatacctttttggctgaagaacctgtcaagacaaaagttgaaaaaactggaagtggatatttggtttcaggatcccagcactcaatagtagctcccataggaaggcagaaaagaggtacatctgattctgagagtggaaatgactcatagtcctcttctggatatctaaaaattaaaccagccttatatgctattgcatttgaagcaggtacagacttcttataacacagaaacacgctggaaccccacattccacaatttaagtttttgtcaactttgcagaaggtatgaggaggagtttctcctttactggttacaataacacagatatcagttacagccaaggaattctggggtcgaactggaggagcccttcgataagtgataaagattctttgtgaagtagttgaactattgttgacattggcacagcgaccatagggtgtggctaggatcacttcacatcctggaataagccgttctttcccttcatatagaactccaatatctgtaagcggtggtttatctctccctctcttataacagaggaaaagttctgggcttttcagacttccatagttcaagtttgcttggagagctgatggagtggcttctacacaggtgtaaccttcaggtactgtttctccagctgatttgataataatggcaatgtctgtaattggagctttaggtccagttgacttagtatctaaacgatttatttcttgatccaaaagagtagatgtgtcagtgagaccagctacgacaaagtagtctgtcactcttggtcctttgtcttctatcatggctgctactgtattttctgctgcctgctcctctgtcagcgcagccccgacacggcttcttcctggggcaagaaagcaccggattcgcggactgggcgcgctcggcagggcagggcgggggactagctccagcggccgccgccgcctcagtccggtct

SEQ ID NO: 8461 - RNA, 6478 nt, Homo sapiens
  source 1..6478: mol_type = other RNA
aaaagtaattgcggtttttgccattaatagtggcaaaaactacaattaattttgtgccaacctaatacattaaagttagggaaggcagctgtcatcagattttcaggtaattttaagattaatgactacagacaagtttagtagtagtcatttatttaatagtcaatgagacccctttcagaaaaccgtattgcaacatgcaatctattttaataaatatacacttagaatatggctgtatatacacatacctacacagccctacacatatacaaacttacacaaatatgttgctctcttttttttttttttttttttttgagacggtctcactctgtcacccaagctggagttgcagtggcgtgatctccactcactgtagcctctgcctcagttcaagcgattctcctgcctcagcctgagtagctgggactacagtggtgcgcctggctaatttttgtatttttagtaaagacagggtctcaccgtgttggccaggctggtctcgaactcctggcctcaagtgatccacccaccttgctcagcctcccaaagtgctgggattacaggcctgagccaccgtgcccggccatgttgcttttataattgagatatttcatttgttttgggggttaggcaaatttaatttgccattcctcaaactcagtaacttcaaatataaacaatgcctagaatgaatatggttcctcattatttctatcaaactactacaaatactgaagaatcccaaagtagttttccacagaggcagaaaagcagttcaggggttgaaaatcttcaatattaataagccctgggacattcaaatggcacttcatatttcaaggtaatgcaatatgaatcataattcattatatattgtccccaagagttacttcaattccgtattcaccagttcttacgatttggaaaaaaaaacttgaatgtttccagatgaaatctaatccccaagccttgtgtgtcaacattctagtgaatctctatttaaatgagaggcgctccaaaacacttcctgcaccactcgacactggcacttggtggagcatcaattttctgcaacctttcaagaatctctgaagacagactattgtatgcaattccatattcattgtcaaatgcctcaatatcaatattctctcttcctagagacactaatgataagaagaggatttctctgtataaactcctttgtcttttcatgcctggcttcatttgctgtgaaagtaggttgatgggtttaagaacattattgtgctgaatactctgcctgatggtttctactaaagtgcttgtttcttgttgttcctctgacaggagagatgatttcttttcagaattaaaattcctccatgagacatacagaggttctcttggttcctgatgaaggttgatattatcccataacagctgaatatacacaagtttgctatcctgggacagagatgacagaggaagctgtacaccttcattacaatgttcagatgtgaggataagtcctggcaagttactaggaaggtccaaacgtcacaacttcctgcagactatttggaagactaactgttgagatgccatgaaacggtcgctgggtaaagtcaatattctgcaatgggcctccaacactgtgacttcgagtcaaagacacatttcgctttgataaactattaggcacagatgaaattttcatagtttggacatctccactggctctctttatttcatcacttggttcaactgcagagcctgtttcttcagttatgatctggttatgttttgggaagtccataaagttgatcaagtcaggttctgctaaactggatacaggtttgtgctccaaggattcatttgccaatggaatgcttccactttgtaaactgtcaccagaggtacttggtttcaggaaaaagcttgcagaacctctcaaatctttgaattctatattgagaagaggcaagaagttgcttttacagaatggacaagctgtattcaaatttgagtcatctgctgtccatccagccataatttcttcatcataaactaaagctccacaagctctacactgtgaacaactggacatcaaaacctccattgcacaattctgatagatgctagacatgctggtattttgagaagaaccatgatctgatttttcaaagtcttgccctttcatgcctcttggaaatggaacttcacctgttggataatgcagttttcctacatctccactactgctgctactgccaagacttgtgttgctctgggtaagttcactggggaccaaccctgagatacttgtgttaggcgatatattctcccccaaaatatggtcttctaggccagctgggaagctgtagtctctattagtttcttcctcatcatctgagtagctgtaggcagacgcaacagctacccacatcttactggctactgtcgctgcttgtttcataccagatttcaggacatctatcttgggccctgagagtatattatccagctttagccctgacaaagaatttactacagaacccaacgagccatgtggcgaagaacgcaccagtgctgacaaagaagttgaacgttctttatgagttcgagagggggtttgctgcttgaaacgcccagtaaaagttttagacctggacactgcaggtgagctcttttcactttcaggattttcctgtgctggtgaaccatgatctaaaggtaggcttgatctcctctctagagcatgaataaatgcagtagtcatgccagactctctgttttcctctctgtgtaattccatactagaagatttactacctaggggactttttaggttcatatagctttctatttcatcagccagattacgtgcaataactggagaaaacaacttatcttcagaatcaggagtttttcctcctgtacattcagtggctaaaagagacaaaggatctagtccagtttcaacatcttccctctgaaccaccttagcaataccatataaactacttctcttattcctcagatctttggatactgttttcaagtctctggactgattactgttactatcacttagtagactctcatatgtatctactgttgcagtagttttaggtacgtcatcaaccacaggctcaaggagttcttggctttcctcaagcatctctggcaccggagatgatctgtgctcaggattccaagtgctttcagacatacaagtcctactatcaggtaggtgacagctaacattctcaaagctatgggttcttgcaatatgaagtagagaagtcttaggacatgtcaatgctgctgtgagaatcttggcatctgctcccatcatgatagccatttcacttgaattcgaatccaaactactcttcttaagcaacattcctgctcgactttcagaactaaaactacaactcctctcaggaaaatgcttttgtcttttttctcctctatcaccattcttcttgagattagtagcttcgccaaagactgcatcttcaactggatcttgagtagaaaacagcacatttgatatactaccagtgctacttttcctgctgttgacatcaaatataccagacggaactttcacaatactgctgccccatgcaggaggttcagtaggactgtgaggctctggactaggttgtgaatgttttgccacaatagcagaggcatcacacacctcttctgtttgcatttttgttttagttatcaattctcttgctgcctgttcttcaggcacatgaatttctgcatcatcctttataagttcatccttagacccgtatccttggtcagactgaccacctgatattgaggagacctgtgacctttgcacagtctttttaagcggctgcctaaactgtgccaagccacgtaccacattccgtaccttcgtccataagaaaataccactgcgggtactgctaggccacgggctctccaagactaccttattataataaccataagtaatagcattaggctttatcctagcagttttcatttcaaataagactctcactgctaaaacaggatgaccccaaagtccacaaagctgcatcactactcgatagcacacctcatctaagggatccacatctgttttcctcatcttaataagtacatcatatgcctgctgaagtgctctgactttaggatgagaaactctaacataggccggaagacaaataaaccataaactgtaacaatgactaaacagacacttggcccactgtggtggatttgtataacatctcttcgccaatttatgagctgtttttatttcctgtttagttctcttagccatgagaggtggactctttgtaatgctattcccagtagggtgtctactaaaacaaagtttcaactcctgcggtctgtcaaaaagcttaaggtccagtcttggaaagtatttgtaactgtactttggtgacaggtcctttccatcatcaggaggtggctctggcggcattataaatacagtatgctcacttttctgtgaatcatctagttctatcaatctggtatcttctgctgaatcaaaatcaaccttatctgttttctctgtgcctttatcaggaaacaacttttctatgcagtcatcaaaaaatgctaatccagtatctttatcacttacaaaactgcattcttcaatgaaacgaataaaaatctgtgttttggataaaagggtatagaattttgcataggcacgatctcgactttttaaaaatccctgtcggtcaaacaatgaatcagcagctgtggctttatttgaaggagcctctgtgattggtctgagatatgttctatatccttttaaaatagacgccataaagcgcaaaaatgcctcttgaatttccatctcaagctgtgtcatcttcttttgccaggagaaatctgcttcaattggagtcatgtcaatcgctgagccttcttgagttttttggtgaactgaagacagctggggatacaatttctttaaggtgctaagtagatttttgcacggctttttgggaagttgcttccagttcatgttcttcttttcatctgatacatataacatgttcgtatccaagtcaatgcaaacaacatcttgtggtgggtcatgaagatcaaaataccttgagtcaactccaactataaatggtaaaggtgcactaagcactgcagccagtgaaagaggacaaaggggaatatatgggcattgccactgaaatggaaagatcatagctacaacagcttcagctaccccagtcaagacagctggcctaagagaatgcagcagaattttactctcaagtaaaacaaagagcagcagtgttgcacaattctcaggacccagattcattagcaaggtgctaaagttggctccacttagtggtaaaggtgtagaaactggctgtgataatattaatgcatcatggactgacagctggacaaggattctcggtctttgtggtgaaggaaaagggatgttttgcataaaatgtgaaatgtgcctttttggctgaagaacctgtcaagacaaaagttgaaaaaactggaagtggatatttggtttcaggatcccagcactcaatagtagctcccataggaaggcagaaaagaggtacatctgattctgagagtggaaatgactcatagtcctcttctggatatctaaaaattaaaccagccttatatgctattgcatttgaagcaggtacagacttcttataacacagaaacacgctggaaccccacattccacaatttaagtttttgtcaactttgcagaaggtatgaggaggagtttctcctttactggttacaataacacagatatcagttacagccaaggaattctggggtcgaactggaggagcccttcgataagtgataaagattctttgtgaagtagttgaactattgttgacattggcacagcgaccatagggtgtggctaggatcacttcacatcctggaataagccgttctttcccttcatatagaactccaatatctgtaagcggtggtttatctctccctctcttataacagaggaaaagttctgggcttttcagacttccatagttcaagtttgcttggagagctgatggagtggcttctacacaggtgtaaccttcaggtactgtttctccagctgatttgataataatggcaatgtctgtaattggagctttaggtccagttgacttagtatctaaacgatttatttcttgatccaaaagagtagatgtgtcagtgagaccagctacgacaaagtagtctgtcactcttggtcctttgtcttctatcatggctgctactgtattttctgctgcctgctcctctgtcagcgcagccccgacacggcttcttcctggggcaagaaagcaccggattcgcggactgggcgcgctcggcagggcagggcgggggactagctccagcggccgccgccgcctcagtccggtct

SEQ ID NO: 8462 - RNA, 7050 nt, Homo sapiens
  source 1..7050: mol_type = other RNA
aaaagtaattgcggtttttgccattaatagtggcaaaaactacaattaattttgtgccaacctaatacattaaagttagggaaggcagctgtcatcagattttcaggtaattttaagattaatgactacagacaagtttagtagtagtcatttatttaatagtcaatgagacccctttcagaaaaccgtattgcaacatgcaatctattttaataaatatacacttagaatatggctgtatatacacatacctacacagccctacacatatacaaacttacacaaatatgttgctctcttttttttttttttttttttttgagacggtctcactctgtcacccaagctggagttgcagtggcgtgatctccactcactgtagcctctgcctcagttcaagcgattctcctgcctcagcctgagtagctgggactacagtggtgcgcctggctaatttttgtatttttagtaaagacagggtctcaccgtgttggccaggctggtctcgaactcctggcctcaagtgatccacccaccttgctcagcctcccaaagtgctgggattacaggcctgagccaccgtgcccggccatgttgcttttataattgagatatttcatttgttttgggggttaggcaaatttaatttgccattcctcaaactcagtaacttcaaatataaacaatgcctagaatgaatatggttcctcattatttctatcaaactactacaaatactgaagaatcccaaagtagttttccacagaggcagaaaagcagttcaggggttgaaaatcttcaatattaataagccctgggacattcaaatggcacttcatatttcaaggtaatgcaatatgaatcataattcattatatattgtccccaagagttacttcaattccgtattcaccagttcttacgatttggaaaaaaaaacttgaatgtttccagatgaaatctaatccccaagccttgtgtgtcaacattctagtgaatctctatttaaatgagaggcgctccaaaacacttcctgcaccactcgacactggcacttggtggagcatcaattttctgcaacctttcaagaatctctgaagacagactattgtatgcaattccatattcattgtcaaatgcctcaatatcaatattctctcttcctagagacactaatgataagaagaggatttctctgtataaactcctttgtcttttcatgcctggcttcatttgctgtgaaagtaggttgatgggtttaagaacattattgtgctgaatactctgcctgatggtttctactaaagtgcttgtttcttgttgttcctctgacaggagagatgatttcttttcagaattaaaattcctccatgagacatacagaggttctcttggttcctgatgaaggttgatattatcccataacagctgaatatacacaagtttgctatcctgggacagagatgacagaggaagctgtacaccttcattacaatgttcagatgtgaggataagtcctggcaagttactaggaaggtccaaacgtctgaaataccaaacgaggttccagaaaatgattggatgttgattgatgaaagaagatgtatgaatcacctgatcaccttcattttctagcaaagattcaagttctttacggagtactagaggactcaagtagggcacagaaacagggggaggattgggtctttttcctaaaggatccacaacttcctgcagactatttggaagactaactgttgagatgccatgaaacggtcgctgggtaaagtcaatattctgcaatgggcctccaacactgtgacttcgagtcaaagacacatttcgctttgataaactattaggcacagatgaaattttcatagtttggacatctccactggctctctttatttcatcacctttgataccttggttcaactgcagagcctgtttcttcagttatgatctggttatgttttgggaagtccataaagttgatcaagtcaggttctgctaaactggatacaggtttgtgctccaaggattcatttgccaatggaatgcttccactttgtaaactgtcaccagaggtacttggtttcaggaaaaagcttgcagaacctctcaaatctttgaattctatattgagaagaggcaagaagttgcttttacagaatggacaagctgtattcaaatttgagtcatctgctgtccatccagccataatttcttcatcataaactaaagctccacaagctctacactgtgaacaactggacatcaaaacctccattgcacaattctgatagatgctagacatgctggtattttgagaagaaccatgatctgatttttcaaagtcttgccctttcatgcctcttggaaatggaacttcacctgttggataatgcagttttcctacatctccactactgctgctactgccaagacttgtgttgctctgggtaagttcactggggaccaaccctgagatacttgtgttaggcgatatattctcccccaaaatatggtcttctaggccagctgggaagctgtagtctctattagtttcttcctcatcatctgagtagctgtaggcagacgcaacagctacccacatcttactggctactgtcgctgcttgtttcataccagatttcaggacatctatcttgggccctgagagtatattatccagctttagccctgacaaagaatttactacagaacccaacgagccatgtggcgaagaacgcaccagtgctgacaaagaagttgaacgttctttatgagttcgagagggggtttgctgcttgaaacgcccagtaaaagttttagacctggacactgcaggtgagctcttttcactttcaggattttcctgtgctggtgaaccatgatctaaaggtaggcttgatctcctctctagagcatgaataaatgcagtagtcatgccagactctctgttttcctctctgtgtaattccatactagaagatttactacctaggggactttttaggttcatatagctttctatttcatcagccagattacgtgcaataactggagaaaacaacttatcttcagaatcaggagtttttcctcctgtacattcagtggctaaaagagacaaaggatctagtccagtttcaacatcttccctctgaaccaccttagcaataccatataaactacttctcttattcctcagatctttggatactgttttcaagtctctggactgattactgttactatcacttagtagactctcatatgtatctactgttgcagtagttttaggtacgtcatcaaccacaggctcaaggagttcttggctttcctcaagcatctctggcaccggagatgatctgtgctcaggattccaagtgctttcagacatacaagtcctactatcaggtaggtgacagctaacattctcaaagctatgggttcttgcaatatgaagtagagaagtcttaggacatgtcaatgctgctgtgagaatcttggcatctgctcccatcatgatagccatttcacttgaattcgaatccaaactactcttcttaagcaacattcctgctcgactttcagaactaaaactacaactcctctcaggaaaatgcttttgtcttttttctcctctatcaccattcttcttgagattagtagcttcgccaaagactgcatcttcaactggatcttgagtagaaaacagcacatttgatatactaccagtgctacttttcctgctgttgacatcaaatataccagacggaactttcacaatactgctgccccatgcaggaggttcagtaggactgtgaggctctggactaggttgtgaatgttttgccacaatagcagaggcatcacacacctcttctgtttgcatttttgttttagttatcaattctcttgctgcctgttcttcaggcacatgaatttctgcatcatcctttataagttcatccttagacccgtatccttggtcagactgaccacctgtgctagagtgattatcaatggactcaagcctgattaaatctctgacgaagactgtgtgctccccattgttagcatcattagaactatccacactaccgtggctcaccgtgtccccatcacttccacctgtgacattttgaagagctgatattgaggagacctgtgacctttgcacagtctttttaagcggctgcctaaactgtgccaagccacgtaccacattccgtaccttcgtccataagaaaataccactgcgggtactgctaggccacgggctctccaagactaccttattataataaccataagtaatagcattaggctttatcctagcagttttcatttcaaataagactctcactgctaaaacaggatgaccccaaagtccacaaagctgcatcactactcgatagcacacctcatctaagggatccacatctgttttcctcatcttaataagtacatcatatgcctgctgaagtgctctgactttaggatgagaaactctaacataggccggaagacaaataaaccataaactgtaacaatgactaaacagacacttggcccactgtggtggatttgtataacatctcttcgccaatttatgagctgtttttatttcctgtttagttctcttagccatgagaggtggactctttgtaatgctattcccagtagggtgtctactaaaacaaagtttcaactcctgcggtctgtcaaaaagcttaaggtccagtcttggaaagtatttgtaactgtactttggtgacaggtcctttccatcatcaggaggtggctctggcggcattataaatacagtatgctcacttttctgtgaatcatctagttctatcaatctggtatcttctgctgaatcaaaatcaaccttatctgttttctctgtgcctttatcaggaaacaacttttctatgcagtcatcaaaaaatgctaatccagtatctttatcacttacaaaactgcattcttcaatgaaacgaataaaaatctgtgttttggataaaagggtatagaattttgcataggcacgatctcgactttttaaaaatccctgtcggtcaaacaatgaatcagcagctgtggctttatttgaaggagcctctgtgattggtctgagatatgttctatatccttttaaaatagacgccataaagcgcaaaaatgcctcttgaatttccatctcaagctgtgtcatcttcttttgccaggagaaatctgcttcaattggagtcatgtcaatcgctgagccttcttgagttttttggtgaactgaagacagctggggatacaatttctttaaggtgctaagtagatttttgcacggctttttgggaagttgcttccagttcatgttcttcttttcatctgatacatataacatgttcgtatccaagtcaatgcaaacaacatcttgtggtgggtcatgaagatcaaaataccttgagtcaactccaactataaatggtaaaggtgcactaagcactgcagccagtgaaagaggacaaaggggaatatatgggcattgccactgaaatggaaagatcatagctacaacagcttcagctaccccagtcaagacagctggcctaagagaatgcagcagaattttactctcaagtaaaacaaagagcagcagtgttgcacaattctcaggacccagattcattagcaaggtgctaaagttggctccacttagtggtaaaggtgtagaaactggctgtgataatattaatgcatcatggactgacagctggacaaggattctcggtctttgtggtgaaggaaaagggatgttttgcataaaatgtgaaatgtgcttttcaatgggaagaggatgtggtccagacacagaaagtttgtagataaacataagaaatttcctaaaagcttcaaaaaaaggccagtgtgagagtaaacaaatgcatttgtttgtattgatggatttggagaccatttttctctccacaggcgtcaacaagcccaggtgcataagctgtttctctgatagaagttcccgagagtaaggttcataaaactgaatggcagctccatatacctttttggctgaagaacctgtcaagacaaaagttgaaaaaactggaagtggatatttggtttcaggatcccagcactcaatagtagctcccataggaaggcagaaaagaggtacatctgattctgagagtggaaatgactcatagtcctcttctggatatctaaaaattaaaccagccttatatgctattgcatttgaagcaggtacagacttcttataacacagaaacacgctggaaccccacattccacaatttaagtttttgtcaactttgcagaaggtatgaggaggagtttctcctttactggttacaataacacagatatcagttacagccaaggaattctggggtcgaactggaggagcccttcgataagtgataaagattctttgtgaagtagttgaactattgttgacattggcacagcgaccatagggtgtggctaggatcacttcacatcctggaataagccgttctttcccttcatatagaactccaatatctgtaagcggtggtttatctctccctctcttataacagaggaaaagttctgggcttttcagacttccatagttcaagtttgcttggagagctgatggagtggcttctacacaggtgtaaccttcaggtactgtttctccagctgatttgataataatggcaatgtctgtaattggagctttaggtccagttgacttagtatctaaacgatttatttcttgatccaaaagagtagatgtgtcagtgagaccagctacgacaaagtagtctgtcactcttggtcctttgtcttctatcatggctgctactgtattttctgctgcctgctcctctgtcagcgcagccccgacacggcttcttcctggggcaagaaagcaccggattcgcggactgggcgcgctcggcagggcagggcgggggactagctccagcggccgccgccgcctcagtccggtct

SEQ ID NO: 8463 - RNA, 7136 nt, Homo sapiens
  source 1..7136: mol_type = other RNA
aaaagtaattgcggtttttgccattaatagtggcaaaaactacaattaattttgtgccaacctaatacattaaagttagggaaggcagctgtcatcagattttcaggtaattttaagattaatgactacagacaagtttagtagtagtcatttatttaatagtcaatgagacccctttcagaaaaccgtattgcaacatgcaatctattttaataaatatacacttagaatatggctgtatatacacatacctacacagccctacacatatacaaacttacacaaatatgttgctctcttttttttttttttttttttttgagacggtctcactctgtcacccaagctggagttgcagtggcgtgatctccactcactgtagcctctgcctcagttcaagcgattctcctgcctcagcctgagtagctgggactacagtggtgcgcctggctaatttttgtatttttagtaaagacagggtctcaccgtgttggccaggctggtctcgaactcctggcctcaagtgatccacccaccttgctcagcctcccaaagtgctgggattacaggcctgagccaccgtgcccggccatgttgcttttataattgagatatttcatttgttttgggggttaggcaaatttaatttgccattcctcaaactcagtaacttcaaatataaacaatgcctagaatgaatatggttcctcattatttctatcaaactactacaaatactgaagaatcccaaagtagttttccacagaggcagaaaagcagttcaggggttgaaaatcttcaatattaataagccctgggacattcaaatggcacttcatatttcaaggtaatgcaatatgaatcataattcattatatattgtccccaagagttacttcaattccgtattcaccagttcttacgatttggaaaaaaaaacttgaatgtttccagatgaaatctaatccccaagccttgtgtgtcaacattctagtgaatctctatttaaatgagaggcgctccaaaacacttcctgcaccactcgacactggcacttggtggagcatcaattttctgcaacctttcaagaatctctgaagacagactattgtatgcaattccatattcattgtcaaatgcctcaatatcaatattctctcttcctagagacactaatgataagaagaggatttctctgtataaactcctttgtcttttcatgcctggcttcatttgctgtgaaagtaggttgatgggtttaagaacattattgtgctgaatactctgcctgatggtttctactaaagtgcttgtttcttgttgttcctctgacaggagagatgatttcttttcagaattaaaattcctccatgagacatacagaggttctcttggttcctgatgaaggttgatattatcccataacagctgaatatacacaagtttgctatcctgggacagagatgacagaggaagctgtacaccttcattacaatgttcagatgtgaggataagtcctggcaagttactaggaaggtccaaacgtctgaaataccaaacgaggttccagaaaatgattggatgttgattgatgaaagaagatgtatgaatcacctgatcaccttcattttctagcaaagattcaagttctttacggagtactagaggactcaagtagggcacagaaacagggggaggattgggtctttttcctaaaggatccacaacttcctgcagactatttggaagactaactgttgagatgccatgaaacggtcgctgggtaaagtcaatattctgcaatgggcctccaacactgtgacttcgagtcaaagacacatttcgctttgataaactattaggcacagatgaaattttcatagtttggacatctccactggctctctttatttcatcacttggttcaactgcagagcctgtttcttcagttatgatctggttatgttttgggaagtccataaagttgatcaagtcaggttctgctaaactggatacaggtttgtgctccaaggattcatttgccaatggaatgcttccactttgtaaactgtcaccagaggtacttggtttcaggaaaaagctccattgcacaattctgatagatgctagacatgctggtattttgagaagaaccatgatctgatttttcaaagtcttgccctttcatgcctcttggaaatggaacttcacctgttggataatgcagttttcctacatctccactactgctgctactgccaagacttgtgttgctctgggtaagttcactggggaccaaccctgagatacttgtgttaggcgatatattctcccccaaaatatggtcttctaggccagctgggaagctgtagtctctattagtttcttcctcatcatctgagtagctgtaggcagacgcaacagctacccacatcttactggctactgtcgctgcttgtttcataccagatttcaggacatctatcttgggccctgagagtatattatccagctttagccctgacaaagaatttactacagaacccaacgagccatgtggcgaagaacgcaccagtgctgacaaagaagttgaacgttctttatgagttcgagagggggtttgctgcttgaaacgcccagtaaaagttttagacctggacactgcaggtgagctcttttcactttcaggattttcctgtgctggtgaaccatgatctaaaggtaggcttgatctcctctctagagcatgaataaatgcagtagtcatgccagactctctgttttcctctctgtgtaattccatactagaagatttactacctaggggactttttaggttcatatagctttctatttcatcagccagattacgtgcaataactggagaaaacaacttatcttcagaatcaggagtttttcctcctgtacattcagtggctaaaagagacaaaggatctagtccagtttcaacatcttccctctgaaccaccttagcaataccatataaactacttctcttattcctcagatctttggatactgttttcaagtctctggactgattactgttactatcacttagtagactctcatatgtatctactgttgcagtagttttaggtacgtcatcaaccacaggctcaaggagttcttggctttcctcaagcatctctggcaccggagatgatctgtgctcaggattccaagtgctttcagacatacaagtcctactatcaggtaggtgacagctaacattctcaaagctatgggttcttgcaatatgaagtagagaagtcttaggacatgtcaatgctgctgtgagaatcttggcatctgctcccatcatgatagccatttcacttgaattcgaatccaaactactcttcttaagcaacattcctgctcgactttcagaactaaaactacaactcctctcaggaaaatgcttttgtcttttttctcctctatcaccattcttcttgagattagtagcttcgccaaagactgcatcttcaactggatcttgagtagaaaacagcacatttgatatactaccagtgctacttttcctgctgttgacatcaaatataccagacggaactttcacaatactgctgccccatgcaggaggttcagtaggactgtgaggctctggactaggttgtgaatgttttgccacaatagcagaggcatcacacacctcttctgtttgcatttttgttttagttatcaattctcttgctgcctgttcttcaggcacatgaatttctgcatcatcctttataagttcatccttagacccgtatccttggtcagactgaccacctgatgtggttaacattcaagggtagaattaatgcacacgtgtatccatagcttcacgtcatataagtctgtctgtgctagagtgattatcaatggactcaagcctgattaaatctctgacgaagactgtgtgctccccattgttagcatcattagaactatccacactaccgtggctcaccgtgtccccatcacttccacctgtgacattttgaagagctgatattgaggagacctgtgacctttgcacagtctttttaagcggctgcctaaactgtgccaagccacgtaccacattccgtaccttcgtccataagaaaataccactgcgggtactgctaggccacgggctctccaagactaccttattataataaccataagtaatagcattaggctttatcctagcagttttcatttcaaataagactctcactgctaaaacaggatgaccccaaagtccacaaagctgcatcactactcgatagcacacctcatctaagggatccacatctgttttcctcatcttaataagtacatcatatgcctgctgaagtgctctgactttaggatgagaaactctaacataggccggaagacaaataaaccataaactgtaacaatgactaaacagacacttggcccactgtggtggatttgtataacatctcttcgccaatttatgagctgtttttatttcctgtttagttctcttagccatgagaggtggactctttgtaatgctattcccagtagggtgtctactaaaacaaagtttcaactcctgcggtctgtcaaaaagcttaaggtccagtcttggaaagtatttgtaactgtactttggtgacaggtcctttccatcatcaggaggtggctctggcggcattataaatacagtatgctcacttttctgtgaatcatctagttctatcaatctggtatcttctgctgaatcaaaatcaaccttatctgttttctctgtgcctttatcaggaaacaacttttctatgcagtcatcaaaaaatgctaatccagtatctttatcacttacaaaactgcattcttcaatgaaacgaataaaaatctgtgttttggataaaagggtatagaattttgcataggcacgatctcgactttttaaaaatccctgtcggtcaaacaatgaatcagcagctgtggctttatttgaaggagcctctgtgattggtctgagatatgttctatatccttttaaaatagacgccataaagcgcaaaaatgcctcttgaatttccatctcaagctgtgtcatcttcttttgccaggagaaatctgcttcaattggagtcatgtcaatcgctgagccttcttgagttttttggtgaactgaagacagctggggatacaatttctttaaggtgctaagtagatttttgcacggctttttgggaagttgcttccagttcatgttcttcttttcatctgatacatataacatgttcgtatccaagtcaatgcaaacaacatcttgtggtgggtcatgaagatcaaaataccttgagtcaactccaactataaatggtaaaggtgcactaagcactgcagccagtgaaagaggacaaaggggaatatatgggcattgccactgaaatggaaagatcatagctacaacagcttcagctaccccagtcaagacagctggcctaagagaatgcagcagaattttactctcaagtaaaacaaagagcagcagtgttgcacaattctcaggacccagattcattagcaaggtgctaaagttggctccacttagtggtaaaggtgtagaaactggctgtgataatattaatgcatcatggactgacagctggacaaggattctcggtctttgtggtgaaggaaaagggatgttttgcataaaatgtgaaatgtgcttttcaatgggaagaggatgtggtccagacacagaaagtttgtagataaacataagaaatttcctaaaagcttcaaaaaaaggccagtgtgagagtaaacaaatgcatttgtttgtattgatggatttggagaccatttttctctccacaggcgtcaacaagcccaggtgcataagctgtttctctgatagaagttcccgagagtaaggttcataaaactgaatggcagctccatatacctttttggctgaagaacctgtcaagacaaaagttgaaaaaactggaagtggatatttggtttcaggatcccagcactcaatagtagctcccataggaaggcagaaaagaggtacatctgattctgagagtggaaatgactcatagtcctcttctggatatctaaaaattaaacctgtattttcagtttttatcccaccataccagtggaatgaagacgtgacacttaaatctttacagcccttgacactttaatgtgcagtaagaatgtggcgatagatttctcaaacacttcatggcagaaaagtttctcaggccctcctctcctccatatagctgattctttgcaacaaaggagaaaggaagcaagtccaccagccttatatgctattgcatttgaagcaggtacagacttcttataacacagaaacacgctggaaccccacattccacaatttaagtttttgtcaactttgcagaaggtatgaggaggagtttctcctttactggttacaataacacagatatcagttacagccaaggaattctggggtcgaactggaggagcccttcgataagtgataaagattctttgtgaagtagttgaactattgttgacattggcacagcgaccatagggtgtggctaggatcacttcacatcctggaataagccgttctttcccttcatatagaactccaatatctgtaagcggtggtttatctctccctctcttataacagaggaaaagttctgggcttttcagacttccatagttcaagtttgcttggagagctgatggagtggcttctacacaggtgtaaccttcaggtactgtttctccagctgatttgataataatggcaatgtctgtaattggagctttaggtccagttgacttagtatctaaacgatttatttcttgatccaaaagagtagatgtgtcagtgagaccagctacgacaaagtagtctgtcactcttggtcctttgtcttctatcatggctgctactgtattttctgctgcctgctcctctgtcagcgcagccccgacacggcttcttcctggggcaagaaagcaccggattcgcggactgggcgcgctcggcagggcagggcgggggactagctccagcggccgccgccgcctcagtccggtct

SEQ ID NO: 8464 - RNA, 6688 nt, Homo sapiens
  source 1..6688: mol_type = other RNA
aaaagtaattgcggtttttgccattaatagtggcaaaaactacaattaattttgtgccaacctaatacattaaagttagggaaggcagctgtcatcagattttcaggtaattttaagattaatgactacagacaagtttagtagtagtcatttatttaatagtcaatgagacccctttcagaaaaccgtattgcaacatgcaatctattttaataaatatacacttagaatatggctgtatatacacatacctacacagccctacacatatacaaacttacacaaatatgttgctctcttttttttttttttttttttttgagacggtctcactctgtcacccaagctggagttgcagtggcgtgatctccactcactgtagcctctgcctcagttcaagcgattctcctgcctcagcctgagtagctgggactacagtggtgcgcctggctaatttttgtatttttagtaaagacagggtctcaccgtgttggccaggctggtctcgaactcctggcctcaagtgatccacccaccttgctcagcctcccaaagtgctgggattacaggcctgagccaccgtgcccggccatgttgcttttataattgagatatttcatttgttttgggggttaggcaaatttaatttgccattcctcaaactcagtaacttcaaatataaacaatgcctagaatgaatatggttcctcattatttctatcaaactactacaaatactgaagaatcccaaagtagttttccacagaggcagaaaagcagttcaggggttgaaaatcttcaatattaataagccctgggacattcaaatggcacttcatatttcaaggtaatgcaatatgaatcataattcattatatattgtccccaagagttacttcaattccgtattcaccagttcttacgatttggaaaaaaaaacttgaatgtttccagatgaaatctaatccccaagccttgtgtgtcaacattctagtgaatctctatttaaatgagaggcgctccaaaacacttcctgcaccactcgacactggcacttggtggagcatcaattttctgcaacctttcaagaatctctgaagacagactattgtatgcaattccatattcattgtcaaatgcctcaatatcaatattctctcttcctagagacactaatgataagaagaggatttctctgtataaactcctttgtcttttcatgcctggcttcatttgctgtgaaagtaggttgatgggtttaagaacattattgtgctgaatactctgcctgatggtttctactaaagtgcttgtttcttgttgttcctctgacaggagagatgatttcttttcagaattaaaattcctccatgagacatacagaggttctcttggttcctgatgaaggttgatattatcccataacagctgaatatacacaagtttgctatcctgggacagagatgacagaggaagctgtacaccttcattacaatgttcagatgtgaggataagtcctggcaagttactaggaaggtccaaacgtctgaaataccaaacgaggttccagaaaatgattggatgttgattgatgaaagaagatgtatgaatcacctgatcaccttcattttctagcaaagattcaagttctttacggagtactagaggactcaagtagggcacagaaacagggggaggattgggtctttttcctaaaggatccacaacttcctgcagactatttggaagactaactgttgagatgccatgaaacggtcgctgggtaaagtcaatattctgcaatgggcctccaacactgtgacttcgagtcaaagacacatttcgctttgataaactattaggcacagatgaaattttcatagtttggacatctccactggctctctttatttcatcacttggttcaactgcagagcctgtttcttcagttatgatctggttatgttttgggaagtccataaagttgatcaagtcaggttctgctaaactggatacaggtttgtgctccaaggattcatttgccaatggaatgcttccactttgtaaactgtcaccagaggtacttggtttcaggaaaaagctccattgcacaattctgatagatgctagacatgctggtattttgagaagaaccatgatctgatttttcaaagtcttgccctttcatgcctcttggaaatggaacttcacctgttggataatgcagttttcctacatctccactactgctgctactgccaagacttgtgttgctctgggtaagttcactggggaccaaccctgagatacttgtgttaggcgatatattctcccccaaaatatggtcttctaggccagctgggaagctgtagtctctattagtttcttcctcatcatctgagtagctgtaggcagacgcaacagctacccacatcttactggctactgtcgctgcttgtttcataccagatttcaggacatctatcttgggccctgagagtatattatccagctttagccctgacaaagaatttactacagaacccaacgagccatgtggcgaagaacgcaccagtgctgacaaagaagttgaacgttctttatgagttcgagagggggtttgctgcttgaaacgcccagtaaaagttttagacctggacactgcaggtgagctcttttcactttcaggattttcctgtgctggtgaaccatgatctaaaggtaggcttgatctcctctctagagcatgaataaatgcagtagtcatgccagactctctgttttcctctctgtgtaattccatactagaagatttactacctaggggactttttaggttcatatagctttctatttcatcagccagattacgtgcaataactggagaaaacaacttatcttcagaatcaggagtttttcctcctgtacattcagtggctaaaagagacaaaggatctagtccagtttcaacatcttccctctgaaccaccttagcaataccatataaactacttctcttattcctcagatctttggatactgttttcaagtctctggactgattactgttactatcacttagtagactctcatatgtatctactgttgcagtagttttaggtacgtcatcaaccacaggctcaaggagttcttggctttcctcaagcatctctggcaccggagatgatctgtgctcaggattccaagtgctttcagacatacaagtcctactatcaggtaggtgacagctaacattctcaaagctatgggttcttgcaatatgaagtagagaagtcttaggacatgtcaatgctgctgtgagaatcttggcatctgctcccatcatgatagccatttcacttgaattcgaatccaaactactcttcttaagcaacattcctgctcgactttcagaactaaaactacaactcctctcaggaaaatgcttttgtcttttttctcctctatcaccattcttcttgagattagtagcttcgccaaagactgcatcttcaactggatcttgagtagaaaacagcacatttgatatactaccagtgctacttttcctgctgttgacatcaaatataccagacggaactttcacaatactgctgccccatgcaggaggttcagtaggactgtgaggctctggactaggttgtgaatgttttgccacaatagcagaggcatcacacacctcttctgtttgcatttttgttttagttatcaattctcttgctgcctgttcttcaggcacatgaatttctgcatcatcctttataagttcatccttagacccgtatccttggtcagactgaccacctgtgctagagtgattatcaatggactcaagcctgattaaatctctgacgaagactgtgtgctccccattgttagcatcattagaactatccacactaccgtggctcaccgtgtccccatcacttccacctgtgacattttgaagagctgatattgaggagacctgtgacctttgcacagtctttttaagcggctgcctaaactgtgccaagccacgtaccacattccgtaccttcgtccataagaaaataccactgcgggtactgctaggccacgggctctccaagactaccttattataataaccataagtaatagcattaggctttatcctagcagttttcatttcaaataagactctcactgctaaaacaggatgaccccaaagtccacaaagctgcatcactactcgatagcacacctcatctaagggatccacatctgttttcctcatcttaataagtacatcatatgcctgctgaagtgctctgactttaggatgagaaactctaacataggccggaagacaaataaaccataaactgtaacaatgactaaacagacacttggcccactgtggtggatttgtataacatctcttcgccaatttatgagctgtttttatttcctgtttagttctcttagccatgagaggtggactctttgtaatgctattcccagtagggtgtctactaaaacaaagtttcaactcctgcggtctgtcaaaaagcttaaggtccagtcttggaaagtatttgtaactgtactttggtgacaggtcctttccatcatcaggaggtggctctggcggcattataaatacagtatgctcacttttctgtgaatcatctagttctatcaatctggtatcttctgctgaatcaaaatcaaccttatctgttttctctgtgcctttatcaggaaacaacttttctatgcagtcatcaaaaaatgctaatccagtatctttatcacttacaaaactgcattcttcaatgaaacgaataaaaatctgtgttttggataaaagggtatagaattttgcataggcacgatctcgactttttaaaaatccctgtcggtcaaacaatgaatcagcagctgtggctttatttgaaggagcctctgtgattggtctgagatatgttctatatccttttaaaatagacgccataaagcgcaaaaatgcctcttgaatttccatctcaagctgtgtcatcttcttttgccaggagaaatctgcttcaattggagtcatgtcaatcgctgagccttcttgagttttttggtgaactgaagacagctggggatacaatttctttaaggtgctaagtagatttttgcacggctttttgggaagttgcttccagttcatgttcttcttttcatctgatagctacaacagcttcagctaccccagtcaagacagctggcctaagagaatgcagcagaattttactctcaagtaaaacaaagagcagcagtgttgcacaattctcaggacccagattcattagcaaggtgctaaagttggctccacttagtggtaaaggtgtagaaactggctgtgataatattaatgcatcatggactgacagctggacaaggattctcggtctttgtggtgaaggaaaagggatgttttgcataaaatgtgaaatgtgcttttcaatgggaagaggatgtggtccagacacagaaagtttgtagataaacataagaaatttcctaaaagcttcaaaaaaaggccagtgtgagagtaaacaaatgcatttgtttgtattgatggatttggagaccatttttctctccacaggcgtcaacaagcccaggtgcataagctgtttctctgatagaagttcccgagagtaaggttcataaaactgaatggcagctccatatacctttttggctgaagaacctgtcaagacaaaagttgaaaaaactggaagtggatatttggtttcaggatcccagcactcaatagtagctcccataggaaggcagaaaagaggtacatctgattctgagagtggaaatgactcatagtcctcttctggatatctaaaaattaaaccagccttatatgctattgcatttgaagcaggtacagacttcttataacacagaaacacgctggaaccccacattccacaatttaagtttttgtcaactttgcagaaggtatgaggaggagtttctcctttactggttacaataacacagatatcagttacagccaaggaattctggggtcgaactggaggagcccttcgataagtgataaagattctttgtgaagtagttgaactattgttgacattggcacagcgaccatagggtgtggctaggatcacttcacatcctggaataagccgttctttcccttcatatagaactccaatatctgtaagcggtggtttatctctccctctcttataacagaggaaaagttctgggcttttcagacttccatagttcaagtttgcttggagagctgatggagtggcttctacacaggtgtaaccttcaggtactgtttctccagctgatttgataataatggcaatgtctgtaattggagctttaggtccagttgacttagtatctaaacgatttatttcttgatccaaaagagtagatgtgtcagtgagaccagctacgacaaagtagtctgtcactcttggtcctttgtcttctatcatggctgctactgtattttctgctgcctgctcctctgtcagcgcagccccgacacggcttcttcctggggcaagaaagcaccggattcgcggactgggcgcgctcggcagggcagggcgggggactagctccagcggccgccgccgcctcagtccggtct

SEQ ID NO: 8465 - RNA, 6650 nt, Homo sapiens
  source 1..6650: mol_type = other RNA
aaaagtaattgcggtttttgccattaatagtggcaaaaactacaattaattttgtgccaacctaatacattaaagttagggaaggcagctgtcatcagattttcaggtaattttaagattaatgactacagacaagtttagtagtagtcatttatttaatagtcaatgagacccctttcagaaaaccgtattgcaacatgcaatctattttaataaatatacacttagaatatggctgtatatacacatacctacacagccctacacatatacaaacttacacaaatatgttgctctcttttttttttttttttttttttgagacggtctcactctgtcacccaagctggagttgcagtggcgtgatctccactcactgtagcctctgcctcagttcaagcgattctcctgcctcagcctgagtagctgggactacagtggtgcgcctggctaatttttgtatttttagtaaagacagggtctcaccgtgttggccaggctggtctcgaactcctggcctcaagtgatccacccaccttgctcagcctcccaaagtgctgggattacaggcctgagccaccgtgcccggccatgttgcttttataattgagatatttcatttgttttgggggttaggcaaatttaatttgccattcctcaaactcagtaacttcaaatataaacaatgcctagaatgaatatggttcctcattatttctatcaaactactacaaatactgaagaatcccaaagtagttttccacagaggcagaaaagcagttcaggggttgaaaatcttcaatattaataagccctgggacattcaaatggcacttcatatttcaaggtaatgcaatatgaatcataattcattatatattgtccccaagagttacttcaattccgtattcaccagttcttacgatttggaaaaaaaaacttgaatgtttccagatgaaatctaatccccaagccttgtgtgtcaacattctagtgaatctctatttaaatgagaggcgctccaaaacacttcctgcaccactcgacactggcacttggtggagcatcaattttctgcaacctttcaagaatctctgaagacagactattgtatgcaattccatattcattgtcaaatgcctcaatatcaatattctctcttcctagagacactaatgataagaagaggatttctctgtataaactcctttgtcttttcatgcctggcttcatttgctgtgaaagtaggttgatgggtttaagaacattattgtgctgaatactctgcctgatggtttctactaaagtgcttgtttcttgttgttcctctgacaggagagatgatttcttttcagaattaaaattcctccatgagacatacagaggttctcttggttcctgatgaaggttgatattatcccataacagctgaatatacacaagtttgctatcctgggacagagatgacagaggaagctgtacaccttcattacaatgttcagatgtgaggataagtcctggcaagttactaggaaggtccaaacgtctgaaataccaaacgaggttccagaaaatgattggatgttgattgatgaaagaagatgtatgaatcacctgatcaccttcattttctagcaaagattcaagttctttacggagtactagaggactcaagtagggcacagaaacagggggaggattgggtctttttcctaaaggatccacaacttcctgcagactatttggaagactaactgttgagatgccatgaaacggtcgctgggtaaagtcaatattctgcaatgggcctccaacactgtgacttcgagtcaaagacacatttcgctttgataaactattaggcacagatgaaattttcatagtttggacatctccactggctctctttatttcatcacttggttcaactgcagagcctgtttcttcagttatgatctggttatgttttgggaagtccataaagttgatcaagtcaggttctgctaaactggatacaggtttgtgctccaaggattcatttgccaatggaatgcttccactttgtaaactgtcaccagaggtacttggtttcaggaaaaagcttgcagaacctctcaaatctttgaattctatattgagaagaggcaagaagttgcttttacagaatggacaagctgtattcaaatttgagtcatctgctgtccatccagccataatttcttcatcataaactaaagctccacaagctctacactgtgaacaactggacatcaaaacctccattgcacaattctgatagatgctagacatgctggtattttgagaagaaccatgatctgatttttcaaagtcttgccctttcatgcctcttggaaatggaacttcacctgttggataatgcagttttcctacatctccactactgctgctactgccaagacttgtgttgctctgggtaagttcactggggaccaaccctgagatacttgtgttaggcgatatattctcccccaaaatatggtcttctaggccagctgggaagctgtagtctctattagtttcttccagtgctgacaaagaagttgaacgttctttatgagttcgagagggggtttgctgcttgaaacgcccagtaaaagttttagacctggacactgcaggtgagctcttttcactttcaggattttcctgtgctggtgaaccatgatctaaaggtaggcttgatctcctctctagagcatgaataaatgcagtagtcatgccagactctctgttttcctctctgtgtaattccatactagaagatttactacctaggggactttttaggttcatatagctttctatttcatcagccagattacgtgcaataactggagaaaacaacttatcttcagaatcaggagtttttcctcctgtacattcagtggctaaaagagacaaaggatctagtccagtttcaacatcttccctctgaaccaccttagcaataccatataaactacttctcttattcctcagatctttggatactgttttcaagtctctggactgattactgttactatcacttagtagactctcatatgtatctactgttgcagtagttttaggtacgtcatcaaccacaggctcaaggagttcttggctttcctcaagcatctctggcaccggagatgatctgtgctcaggattccaagtgctttcagacatacaagtcctactatcaggtaggtgacagctaacattctcaaagctatgggttcttgcaatatgaagtagagaagtcttaggacatgtcaatgctgctgtgagaatcttggcatctgctcccatcatgatagccatttcacttgaattcgaatccaaactactcttcttaagcaacattcctgctcgactttcagaactaaaactacaactcctctcaggaaaatgcttttgtcttttttctcctctatcaccattcttcttgagattagtagcttcgccaaagactgcatcttcaactggatcttgagtagaaaacagcacatttgatatactaccagtgctacttttcctgctgttgacatcaaatataccagacggaactttcacaatactgctgccccatgcaggaggttcagtaggactgtgaggctctggactaggttgtgaatgttttgccacaatagcagaggcatcacacacctcttctgtttgcatttttgttttagttatcaattctcttgctgcctgttcttcaggcacatgaatttctgcatcatcctttataagttcatccttagacccgtatccttggtcagactgaccacctgtgctagagtgattatcaatggactcaagcctgattaaatctctgacgaagactgtgtgctccccattgttagcatcattagaactatccacactaccgtggctcaccgtgtccccatcacttccacctgtgacattttgaagagctgatattgaggagacctgtgacctttgcacagtctttttaagcggctgcctaaactgtgccaagccacgtaccacattccgtaccttcgtccataagaaaataccactgcgggtactgctaggccacgggctctccaagactaccttattataataaccataagtaatagcattaggctttatcctagcagttttcatttcaaataagactctcactgctaaaacaggatgaccccaaagtccacaaagctgcatcactactcgatagcacacctgtttagttctcttagccatgagaggtggactctttgtaatgctattcccagtagggtgtctactaaaacaaagtttcaactcctgcggtctgtcaaaaagcttaaggtccagtcttggaaagtatttgtaactgtactttggtgacaggtcctttccatcatcaggaggtggctctggcggcattataaatacagtatgctcacttttctgtgaatcatctagttctatcaatctggtatcttctgctgaatcaaaatcaaccttatctgttttctctgtgcctttatcaggaaacaacttttctatgcagtcatcaaaaaatgctaatccagtatctttatcacttacaaaactgcattcttcaatgaaacgaataaaaatctgtgttttggataaaagggtatagaattttgcataggcacgatctcgactttttaaaaatccctgtcggtcaaacaatgaatcagcagctgtggctttatttgaaggagcctctgtgattggtctgagatatgttctatatccttttaaaatagacgccataaagcgcaaaaatgcctcttgaatttccatctcaagctgtgtcatcttcttttgccaggagaaatctgcttcaattggagtcatgtcaatcgctgagccttcttgagttttttggtgaactgaagacagctggggatacaatttctttaaggtgctaagtagatttttgcacggctttttgggaagttgcttccagttcatgttcttcttttcatctgatacatataacatgttcgtatccaagtcaatgcaaacaacatcttgtggtgggtcatgaagatcaaaataccttgagtcaactccaactataaatggtaaaggtgcactaagcactgcagccagtgaaagaggacaaaggggaatatatgggcattgccactgaaatggaaagatcatagctacaacagcttcagctaccccagtcaagacagctggcctaagagaatgcagcagaattttactctcaagtaaaacaaagagcagcagtgttgcacaattctcaggacccagattcattagcaaggtgctaaagttggctccacttagtggtaaaggtgtagaaactggctgtgataatattaatgcatcatggactgacagctggacaaggattctcggtctttgtggtgaaggaaaagggatgttttgcataaaatgtgaaatgtgcttttcaatgggaagaggatgtggtccagacacagaaagtttgtagataaacataagaaatttcctaaaagcttcaaaaaaaggccagtgtgagagtaaacaaatgcatttgtttgtattgatggatttggagaccatttttctctccacaggcgtcaacaagcccaggtgcataagctgtttctctgatagaagttcccgagagtaaggttcataaaactgaatggcagctccatatacctttttggctgaagaacctgtcaagacaaaagttgaaaaaactggaagtggatatttggtttcaggatcccagcactcaatagtagctcccataggaaggcagaaaagaggtacatctgattctgagagtggaaatgactcatagtcctcttctggatatctaaaaattaaaccagccttatatgctattgcatttgaagcaggtacagacttcttataacacagaaacacgctggaaccccacattccacaatttaagtttttgtcaactttgcagaaggtatgaggaggagtttctcctttactggttacaataacacagatatcagttacagccaaggaattctggggtcgaactggaggagcccttcgataagtgataaagattctttgtgaagtagttgaactattgttgacattggcacagcgaccatagggtgtggctaggatcacttcacatcctggaataagccgttctttcccttcatatagaactccaatatctgtaagcggtggtttatctctccctctcttataacagaggaaaagttctgggcttttcagacttccatagttcaagtttgcttggagagctgatggagtggcttctacacaggtgtaaccttcaggtactgtttctccagctgatttgataataatggcaatgtctgtaattggagctttaggtccagttgacttagtatctaaacgatttatttcttgatccaaaagagtagatgtgtcagtgagaccagctacgacaaagtagtctgtcactcttggtcctttgtcttctatcatggctgctactgtattttctgctgcctgctcctctgtcagcgcagccccgacacggcttcttcctggggcaagaaagcaccggattcgcggactgggcgcgctcggcagggcagggcgggggactagctccagcggccgccgccgcctcagtccggtct

SEQ ID NO: 8466 - RNA, 7001 nt, Homo sapiens
  source 1..7001: mol_type = other RNA
aaaagtaattgcggtttttgccattaatagtggcaaaaactacaattaattttgtgccaacctaatacattaaagttagggaaggcagctgtcatcagattttcaggtaattttaagattaatgactacagacaagtttagtagtagtcatttatttaatagtcaatgagacccctttcagaaaaccgtattgcaacatgcaatctattttaataaatatacacttagaatatggctgtatatacacatacctacacagccctacacatatacaaacttacacaaatatgttgctctcttttttttttttttttttttttgagacggtctcactctgtcacccaagctggagttgcagtggcgtgatctccactcactgtagcctctgcctcagttcaagcgattctcctgcctcagcctgagtagctgggactacagtggtgcgcctggctaatttttgtatttttagtaaagacagggtctcaccgtgttggccaggctggtctcgaactcctggcctcaagtgatccacccaccttgctcagcctcccaaagtgctgggattacaggcctgagccaccgtgcccggccatgttgcttttataattgagatatttcatttgttttgggggttaggcaaatttaatttgccattcctcaaactcagtaacttcaaatataaacaatgcctagaatgaatatggttcctcattatttctatcaaactactacaaatactgaagaatcccaaagtagttttccacagaggcagaaaagcagttcaggggttgaaaatcttcaatattaataagccctgggacattcaaatggcacttcatatttcaaggtaatgcaatatgaatcataattcattatatattgtccccaagagttacttcaattccgtattcaccagttcttacgatttggaaaaaaaaacttgaatgtttccagatgaaatctaatccccaagccttgtgtgtcaacattctagtgaatctctatttaaatgagaggcgctccaaaacacttcctgcaccactcgacactggcacttggtggagcatcaattttctgcaacctttcaagaatctctgaagacagactattgtatgcaattccatattcattgtcaaatgcctcaatatcaatattctctcttcctagagacactaatgataagaagaggatttctctgtataaactcctttgtcttttcatgcctggcttcatttgctgtgaaagtaggttgatgggtttaagaacattattgtgctgaatactctgcctgatggtttctactaaagtgcttgtttcttgttgttcctctgacaggagagatgatttcttttcagaattaaaattcctccatgagacatacagaggttctcttggttcctgatgaaggttgatattatcccataacagctgaatatacacaagtttgctatcctgggacagagatgacagaggaagctgtacaccttcattacaatgttcagatgtgaggataagtcctggcaagttactaggaaggtccaaacgtctgaaataccaaacgaggttccagaaaatgattggatgttgattgatgaaagaagatgtatgaatcacctgatcaccttcattttctagcaaagattcaagttctttacggagtactagaggactcaagtagggcacagaaacagggggaggattgggtctttttcctaaaggatccacaacttcctgcagactatttggaagactaactgttgagatgccatgaaacggtcgctgggtaaagtcaatattctgcaatgggcctccaacactgtgacttcgagtcaaagacacatttcgctttgataaactattaggcacagatgaaattttcatagtttggacatctccactggctctctttatttcatcacttggttcaactgcagagcctgtttcttcagttatgatctggttatgttttgggaagtccataaagttgatcaagtcaggttctgctaaactggatacaggtttgtgctccaaggattcatttgccaatggaatgcttccactttgtaaactgtcaccagaggtacttggtttcaggaaaaagcttgcagaacctctcaaatctttgaattctatattgagaagaggcaagaagttgcttttacagaatggacaagctgtattcaaatttgagtcatctgctgtccatccagccataatttcttcatcataaactaaagctccacaagctctacactgtgaacaactggacatcaaaacctccattgcacaattctgatagatgctagacatgctggtattttgagaagaaccatgatctgatttttcaaagtcttgccctttcatgcctcttggaaatggaacttcacctgttggataatgcagttttcctacatctccactactgctgctactgccaagacttgtgttgctctgggtaagttcactggggaccaaccctgagatacttgtgttaggcgatatattctcccccaaaatatggtcttctaggccagctgggaagctgtagtctctattagtttcttcccacatcttactggctactgtcgctgcttgtttcataccagatttcaggacatctatcttgggccctgagagtatattatccagctttagccctgacaaagaatttactacagaacccaacgagccatgtggcgaagaacgcaccagtgctgacaaagaagttgaacgttctttatgagttcgagagggggtttgctgcttgaaacgcccagtaaaagttttagacctggacactgcaggtgagctcttttcactttcaggattttcctgtgctggtgaaccatgatctaaaggtaggcttgatctcctctctagagcatgaataaatgcagtagtcatgccagactctctgttttcctctctgtgtaattccatactagaagatttactacctaggggactttttaggttcatatagctttctatttcatcagccagattacgtgcaataactggagaaaacaacttatcttcagaatcaggagtttttcctcctgtacattcagtggctaaaagagacaaaggatctagtccagtttcaacatcttccctctgaaccaccttagcaataccatataaactacttctcttattcctcagatctttggatactgttttcaagtctctggactgattactgttactatcacttagtagactctcatatgtatctactgttgcagtagttttaggtacgtcatcaaccacaggctcaaggagttcttggctttcctcaagcatctctggcaccggagatgatctgtgctcaggattccaagtgctttcagacatacaagtcctactatcaggtaggtgacagctaacattctcaaagctatgggttcttgcaatatgaagtagagaagtcttaggacatgtcaatgctgctgtgagaatcttggcatctgctcccatcatgatagccatttcacttgaattcgaatccaaactactcttcttaagcaacattcctgctcgactttcagaactaaaactacaactcctctcaggaaaatgcttttgtcttttttctcctctatcaccattcttcttgagattagtagcttcgccaaagactgcatcttcaactggatcttgagtagaaaacagcacatttgatatactaccagtgctacttttcctgctgttgacatcaaatataccagacggaactttcacaatactgctgccccatgcaggaggttcagtaggactgtgaggctctggactaggttgtgaatgttttgccacaatagcagaggcatcacacacctcttctgtttgcatttttgttttagttatcaattctcttgctgcctgttcttcaggcacatgaatttctgcatcatcctttataagttcatccttagacccgtatccttggtcagactgaccacctgtgctagagtgattatcaatggactcaagcctgattaaatctctgacgaagactgtgtgctccccattgttagcatcattagaactatccacactaccgtggctcaccgtgtccccatcacttccacctgtgacattttgaagagctgatattgaggagacctgtgacctttgcacagtctttttaagcggctgcctaaactgtgccaagccacgtaccacattccgtaccttcgtccataagaaaataccactgcgggtactgctaggccacgggctctccaagactaccttattataataaccataagtaatagcattaggctttatcctagcagttttcatttcaaataagactctcactgctaaaacaggatgaccccaaagtccacaaagctgcatcactactcgatagcacacctcatctaagggatccacatctgttttcctcatcttaataagtacatcatatgcctgctgaagtgctctgactttaggatgagaaactctaacataggccggaagacaaataaaccataaactgtaacaatgactaaacagacacttggcccactgtggtggatttgtataacatctcttcgccaatttatgagctgtttttatttcctgtttagttctcttagccatgagaggtggactctttgtaatgctattcccagtagggtgtctactaaaacaaagtttcaactcctgcggtctgtcaaaaagcttaaggtccagtcttggaaagtatttgtaactgtactttggtgacaggtcctttccatcatcaggaggtggctctggcggcattataaatacagtatgctcacttttctgtgaatcatctagttctatcaatctggtatcttctgctgaatcaaaatcaaccttatctgttttctctgtgcctttatcaggaaacaacttttctatgcagtcatcaaaaaatgctaatccagtatctttatcacttacaaaactgcattcttcaatgaaacgaataaaaatctgtgttttggataaaagggtatagaattttgcataggcacgatctcgactttttaaaaatccctgtcggtcaaacaatgaatcagcagctgtggctttatttgaaggagcctctgtgattggtctgagatatgttctatatccttttaaaatagacgccataaagcgcaaaaatgcctcttgaatttccatctcaagctgtgtcatcttcttttgccaggagaaatctgcttcaattggagtcatgtcaatcgctgagccttcttgagttttttggtgaactgaagacagctggggatacaatttctttaaggtgctaagtagatttttgcacggctttttgggaagttgcttccagttcatgttcttcttttcatctgatacatataacatgttcgtatccaagtcaatgcaaacaacatcttgtggtgggtcatgaagatcaaaataccttgagtcaactccaactataaatggtaaaggtgcactaagcactgcagccagtgaaagaggacaaaggggaatatatgggcattgccactgaaatggaaagatcatagctacaacagcttcagctaccccagtcaagacagctggcctaagagaatgcagcagaattttactctcaagtaaaacaaagagcagcagtgttgcacaattctcaggacccagattcattagcaaggtgctaaagttggctccacttagtggtaaaggtgtagaaactggctgtgataatattaatgcatcatggactgacagctggacaaggattctcggtctttgtggtgaaggaaaagggatgttttgcataaaatgtgaaatgtgcttttcaatgggaagaggatgtggtccagacacagaaagtttgtagataaacataagaaatttcctaaaagcttcaaaaaaaggccagtgtgagagtaaacaaatgcatttgtttgtattgatggatttggagaccatttttctctccacaggcgtcaacaagcccaggtgcataagctgtttctctgatagaagttcccgagagtaaggttcataaaactgaatggcagctccatatacctttttggctgaagaacctgtcaagacaaaagttgaaaaaactggaagtggatatttggtttcaggatcccagcactcaatagtagctcccataggaaggcagaaaagaggtacatctgattctgagagtggaaatgactcatagtcctcttctggatatctaaaaattaaaccagccttatatgctattgcatttgaagcaggtacagacttcttataacacagaaacacgctggaaccccacattccacaatttaagtttttgtcaactttgcagaaggtatgaggaggagtttctcctttactggttacaataacacagatatcagttacagccaaggaattctggggtcgaactggaggagcccttcgataagtgataaagattctttgtgaagtagttgaactattgttgacattggcacagcgaccatagggtgtggctaggatcacttcacatcctggaataagccgttctttcccttcatatagaactccaatatctgtaagcggtggtttatctctccctctcttataacagaggaaaagttctgggcttttcagacttccatagttcaagtttgcttggagagctgatggagtggcttctacacaggtgtaaccttcaggtactgtttctccagctgatttgataataatggcaatgtctgtaattggagctttaggtccagttgacttagtatctaaacgatttatttcttgatccaaaagagtagatgtgtcagtgagaccagctacgacaaagtagtctgtcactcttggtcctttgtcttctatcatggctgctactgtattttctgctgcctgctcctctgtcagcgcagccccgacacggcttcttcctggggcaagaaagcaccggattcgcggactgggcgcgctcggcagggcagggcgggggactagctccagcggccgccgccgcctcagtccggtct

SEQ ID NO: 8467 - RNA, 6893 nt, Homo sapiens
  source 1..6893: mol_type = other RNA
aaaagtaattgcggtttttgccattaatagtggcaaaaactacaattaattttgtgccaacctaatacattaaagttagggaaggcagctgtcatcagattttcaggtaattttaagattaatgactacagacaagtttagtagtagtcatttatttaatagtcaatgagacccctttcagaaaaccgtattgcaacatgcaatctattttaataaatatacacttagaatatggctgtatatacacatacctacacagccctacacatatacaaacttacacaaatatgttgctctcttttttttttttttttttttttgagacggtctcactctgtcacccaagctggagttgcagtggcgtgatctccactcactgtagcctctgcctcagttcaagcgattctcctgcctcagcctgagtagctgggactacagtggtgcgcctggctaatttttgtatttttagtaaagacagggtctcaccgtgttggccaggctggtctcgaactcctggcctcaagtgatccacccaccttgctcagcctcccaaagtgctgggattacaggcctgagccaccgtgcccggccatgttgcttttataattgagatatttcatttgttttgggggttaggcaaatttaatttgccattcctcaaactcagtaacttcaaatataaacaatgcctagaatgaatatggttcctcattatttctatcaaactactacaaatactgaagaatcccaaagtagttttccacagaggcagaaaagcagttcaggggttgaaaatcttcaatattaataagccctgggacattcaaatggcacttcatatttcaaggtaatgcaatatgaatcataattcattatatattgtccccaagagttacttcaattccgtattcaccagttcttacgatttggaaaaaaaaacttgaatgtttccagatgaaatctaatccccaagccttgtgtgtcaacattctagtgaatctctatttaaatgagaggcgctccaaaacacttcctgcaccactcgacactggcacttggtggagcatcaattttctgcaacctttcaagaatctctgaagacagactattgtatgcaattccatattcattgtcaaatgcctcaatatcaatattctctcttcctagagacactaatgataagaagaggatttctctgtataaactcctttgtcttttcatgcctggcttcatttgctgtgaaagtaggttgatgggtttaagaacattattgtgctgaatactctgcctgatggtttctactaaagtgcttgtttcttgttgttcctctgacaggagagatgatttcttttcagaattaaaattcctccatgagacatacagaggttctcttggttcctgatgaaggttgatattatcccataacagctgaatatacacaagtttgctatcctgggacagagatgacagaggaagctgtacaccttcattacaatgttcagatgtgaggataagtcctggcaagttactaggaaggtccaaacgtctgaaataccaaacgaggttccagaaaatgattggatgttgattgatgaaagaagatgtatgaatcacctgatcaccttcattttctagcaaagattcaagttctttacggagtactagaggactcaagtagggcacagaaacagggggaggattgggtctttttcctaaaggatccacaacttcctgcagactatttggaagactaactgttgagatgccatgaaacggtcgctgggtaaagtcaatattctgcaatgggcctccaacactgtgacttcgagtcaaagacacatttcgctttgataaactattaggcacagatgaaattttcatagtttggacatctccactggctctctttatttcatcacttggttcaactgcagagcctgtttcttcagttatgatctggttatgttttgggaagtccataaagttgatcaagtcaggttctgctaaactggatacaggtttgtgctccaaggattcatttgccaatggaatgcttccactttgtaaactgtcaccagaggtacttggtttcaggaaaaagcttgcagaacctctcaaatctttgaattctatattgagaagaggcaagaagttgcttttacagaatggacaagctgtattcaaatttgagtcatctgctgtccatccagccataatttcttcatcataaactaaagctccacaagctctacactgtgaacaactggacatcaaaacctccattgcacaattctgatagatgctagacatgctggtattttgagaagaaccatgatctgatttttcaaagtcttgccctttcatgcctcttggaaatggaacttcacctgttggataatgcagttttcctacatctccactactgctgctactgccaagacttgtgttgctctgggtaagttcactggggaccaaccctgagatacttgtgttaggcgatatattctcccccaaaatatggtcttctaggccagctgggaagctgtagtctctattagtttcttcctcatcatctgagtagctgtaggcagacgcaacagctacccacatcttactggctactgtcgctgcttgtttcataccagatttcaggacatctatcttgggccctgagagtatattatccagctttagccctgacaaagaatttactacagaacccaacgagccatgtggcgaagaacgcaccagtgctgacaaagaagttgaacgttctttatgagttcgagagggggtttgctgcttgaaacgcccagtaaaagttttagacctggacactgcaggtgagctcttttcactttcaggattttcctgtgctggtgaaccatgatctaaaggtaggcttgatctcctctctagagcatgaataaatgcagtagtcatgccagactctctgttttcctctctgtgtaattccatactagaagatttactacctaggggactttttaggttcatatagctttctatttcatcagccagattacgtgcaataactggagaaaacaacttatcttcagaatcaggagtttttcctcctgtacattcagtggctaaaagagacaaaggatctagtccagtttcaacatcttccctctgaaccaccttagcaataccatataaactacttctcttattcctcagatctttggatactgttttcaagtctctggactgattactgttactatcacttagtagactctcatatgtatctactgttgcagtagttttaggtacgtcatcaaccacaggctcaaggagttcttggctttcctcaagcatctctggcaccggagatgatctgtgctcaggattccaagtgctttcagacatacaagtcctactatcaggtaggtgacagctaacattctcaaagctatgggttcttgcaatatgaagtagagaagtcttaggacatgtcaatgctgctgtgagaatcttggcatctgctcccatcatgatagccatttcacttgaattcgaatccaaactactcttcttaagcaacattcctgctcgactttcagaactaaaactacaactcctctcaggaaaatgcttttgtcttttttctcctctatcaccattcttcttgagattagtagcttcgccaaagactgcatcttcaactggatcttgagtagaaaacagcacatttgatatactaccagtgctacttttcctgctgttgacatcaaatataccagacggaactttcacaatactgctgccccatgcaggaggttcagtaggactgtgaggctctggactaggttgtgaatgttttgccacaatagcagaggcatcacacacctcttctgtttgcatttttgttttagttatcaattctcttgctgcctgttcttcaggcacatgaatttctgcatcatcctttataagttcatccttagacccgtatccttggtcagactgaccacctgatattgaggagacctgtgacctttgcacagtctttttaagcggctgcctaaactgtgccaagccacgtaccacattccgtaccttcgtccataagaaaataccactgcgggtactgctaggccacgggctctccaagactaccttattataataaccataagtaatagcattaggctttatcctagcagttttcatttcaaataagactctcactgctaaaacaggatgaccccaaagtccacaaagctgcatcactactcgatagcacacctcatctaagggatccacatctgttttcctcatcttaataagtacatcatatgcctgctgaagtgctctgactttaggatgagaaactctaacataggccggaagacaaataaaccataaactgtaacaatgactaaacagacacttggcccactgtggtggatttgtataacatctcttcgccaatttatgagctgtttttatttcctgtttagttctcttagccatgagaggtggactctttgtaatgctattcccagtagggtgtctactaaaacaaagtttcaactcctgcggtctgtcaaaaagcttaaggtccagtcttggaaagtatttgtaactgtactttggtgacaggtcctttccatcatcaggaggtggctctggcggcattataaatacagtatgctcacttttctgtgaatcatctagttctatcaatctggtatcttctgctgaatcaaaatcaaccttatctgttttctctgtgcctttatcaggaaacaacttttctatgcagtcatcaaaaaatgctaatccagtatctttatcacttacaaaactgcattcttcaatgaaacgaataaaaatctgtgttttggataaaagggtatagaattttgcataggcacgatctcgactttttaaaaatccctgtcggtcaaacaatgaatcagcagctgtggctttatttgaaggagcctctgtgattggtctgagatatgttctatatccttttaaaatagacgccataaagcgcaaaaatgcctcttgaatttccatctcaagctgtgtcatcttcttttgccaggagaaatctgcttcaattggagtcatgtcaatcgctgagccttcttgagttttttggtgaactgaagacagctggggatacaatttctttaaggtgctaagtagatttttgcacggctttttgggaagttgcttccagttcatgttcttcttttcatctgatacatataacatgttcgtatccaagtcaatgcaaacaacatcttgtggtgggtcatgaagatcaaaataccttgagtcaactccaactataaatggtaaaggtgcactaagcactgcagccagtgaaagaggacaaaggggaatatatgggcattgccactgaaatggaaagatcatagctacaacagcttcagctaccccagtcaagacagctggcctaagagaatgcagcagaattttactctcaagtaaaacaaagagcagcagtgttgcacaattctcaggacccagattcattagcaaggtgctaaagttggctccacttagtggtaaaggtgtagaaactggctgtgataatattaatgcatcatggactgacagctggacaaggattctcggtctttgtggtgaaggaaaagggatgttttgcataaaatgtgaaatgtgcttttcaatgggaagaggatgtggtccagacacagaaagtttgtagataaacataagaaatttcctaaaagcttcaaaaaaaggccagtgtgagagtaaacaaatgcatttgtttgtattgatggatttggagaccatttttctctccacaggcgtcaacaagcccaggtgcataagctgtttctctgatagaagttcccgagagtaaggttcataaaactgaatggcagctccatatacctttttggctgaagaacctgtcaagacaaaagttgaaaaaactggaagtggatatttggtttcaggatcccagcactcaatagtagctcccataggaaggcagaaaagaggtacatctgattctgagagtggaaatgactcatagtcctcttctggatatctaaaaattaaaccagccttatatgctattgcatttgaagcaggtacagacttcttataacacagaaacacgctggaaccccacattccacaatttaagtttttgtcaactttgcagaaggtatgaggaggagtttctcctttactggttacaataacacagatatcagttacagccaaggaattctggggtcgaactggaggagcccttcgataagtgataaagattctttgtgaagtagttgaactattgttgacattggcacagcgaccatagggtgtggctaggatcacttcacatcctggaataagccgttctttcccttcatatagaactccaatatctgtaagcggtggtttatctctccctctcttataacagaggaaaagttctgggcttttcagacttccatagttcaagtttgcttggagagctgatggagtggcttctacacaggtgtaaccttcaggtactgtttctccagctgatttgataataatggcaatgtctgtaattggagctttaggtccagttgacttagtatctaaacgatttatttcttgatccaaaagagtagatgtgtcagtgagaccagctacgacaaagtagtctgtcactcttggtcctttgtcttctatcatggctgctactgtattttctgctgcctgctcctctgtcagcgcagccccgacacggcttcttcctggggcaagaaagcaccggattcgcggactgggcgcgctcggcagggcagggcgggggactagctccagcggccgccgccgcctcagtccggtct

SEQ ID NO: 8468 - RNA, 6788 nt, Homo sapiens
  source 1..6788: mol_type = other RNA
aaaagtaattgcggtttttgccattaatagtggcaaaaactacaattaattttgtgccaacctaatacattaaagttagggaaggcagctgtcatcagattttcaggtaattttaagattaatgactacagacaagtttagtagtagtcatttatttaatagtcaatgagacccctttcagaaaaccgtattgcaacatgcaatctattttaataaatatacacttagaatatggctgtatatacacatacctacacagccctacacatatacaaacttacacaaatatgttgctctcttttttttttttttttttttttgagacggtctcactctgtcacccaagctggagttgcagtggcgtgatctccactcactgtagcctctgcctcagttcaagcgattctcctgcctcagcctgagtagctgggactacagtggtgcgcctggctaatttttgtatttttagtaaagacagggtctcaccgtgttggccaggctggtctcgaactcctggcctcaagtgatccacccaccttgctcagcctcccaaagtgctgggattacaggcctgagccaccgtgcccggccatgttgcttttataattgagatatttcatttgttttgggggttaggcaaatttaatttgccattcctcaaactcagtaacttcaaatataaacaatgcctagaatgaatatggttcctcattatttctatcaaactactacaaatactgaagaatcccaaagtagttttccacagaggcagaaaagcagttcaggggttgaaaatcttcaatattaataagccctgggacattcaaatggcacttcatatttcaaggtaatgcaatatgaatcataattcattatatattgtccccaagagttacttcaattccgtattcaccagttcttacgatttggaaaaaaaaacttgaatgtttccagatgaaatctaatccccaagccttgtgtgtcaacattctagtgaatctctatttaaatgagaggcgctccaaaacacttcctgcaccactcgacactggcacttggtggagcatcaattttctgcaacctttcaagaatctctgaagacagactattgtatgcaattccatattcattgtcaaatgcctcaatatcaatattctctcttcctagagacactaatgataagaagaggatttctctgtataaactcctttgtcttttcatgcctggcttcatttgctgtgaaagtaggttgatgggtttaagaacattattgtgctgaatactctgcctgatggtttctactaaagtgcttgtttcttgttgttcctctgacaggagagatgatttcttttcagaattaaaattcctccatgagacatacagaggttctcttggttcctgatgaaggttgatattatcccataacagctgaatatacacaagtttgctatcctgggacagagatgacagaggaagctgtacaccttcattacaatgttcagatgtgaggataagtcctggcaagttactaggaaggtccaaacgtctgaaataccaaacgaggttccagaaaatgattggatgttgattgatgaaagaagatgtatgaatcacctgatcaccttcattttctagcaaagattcaagttctttacggagtactagaggactcaagtagggcacagaaacagggggaggattgggtctttttcctaaaggatccacaacttcctgcagactatttggaagactaactgttgagatgccatgaaacggtcgctgggtaaagtcaatattctgcaatgggcctccaacactgtgacttcgagtcaaagacacatttcgctttgataaactattaggcacagatgaaattttcatagtttggacatctccactggctctctttatttcatcacttggttcaactgcagagcctgtttcttcagttatgatctggttatgttttgggaagtccataaagttgatcaagtcaggttctgctaaactggatacaggtttgtgctccaaggattcatttgccaatggaatgcttccactttgtaaactgtcaccagaggtacttggtttcaggaaaaagcttgcagaacctctcaaatctttgaattctatattgagaagaggcaagaagttgcttttacagaatggacaagctgtattcaaatttgagtcatctgctgtccatccagccataatttcttcatcataaactaaagctccacaagctctacactgtgaacaactggacatcaaaacctccattgcacaattctgatagatgctagacatgctggtattttgagaagaaccatgatctgatttttcaaagtcttgccctttcatgcctcttggaaatggaacttcacctgttggataatgcagttttcctacatctccactactgctgctactgccaagacttgtgttgctctgggtaagttcactggggaccaaccctgagatacttgtgttaggcgatatattctcccccaaaatatggtcttctaggccagctgggaagctgtagtctctattagtttcttcctcatcatctgagtagctgtaggcagacgcaacagctacccacatcttactggctactgtcgctgcttgtttcataccagatttcaggacatctatcttgggccctgagagtatattatccagctttagccctgacaaagaatttactacagaacccaacgagccatgtggcgaagaacgcaccagtgctgacaaagaagttgaacgttctttatgagttcgagagggggtttgctgcttgaaacgcccagtaaaagttttagacctggacactgcaggtgagctcttttcactttcaggattttcctgtgctggtgaaccatgatctaaaggtaggcttgatctcctctctagagcatgaataaatgcagtagtcatgccagactctctgttttcctctctgtgtaattccatactagaagatttactacctaggggactttttaggttcatatagctttctatttcatcagccagattacgtgcaataactggagaaaacaacttatcttcagaatcaggagtttttcctcctgtacattcagtggctaaaagagacaaaggatctagtccagtttcaacatcttccctctgaaccaccttagcaataccatataaactacttctcttattcctcagatctttggatactgttttcaagtctctggactgattactgttactatcacttagtagactctcatatgtatctactgttgcagtagttttaggtacgtcatcaaccacaggctcaaggagttcttggctttcctcaagcatctctggcaccggagatgatctgtgctcaggattccaagtgctttcagacatacaagtcctactatcaggtaggtgacagctaacattctcaaagctatgggttcttgcaatatgaagtagagaagtcttaggacatgtcaatgctgctgtgagaatcttggcatctgctcccatcatgatagccatttcacttgaattcgaatccaaactactcttcttaagcaacattcctgctcgactttcagaactaaaactacaactcctctcaggaaaatgcttttgtcttttttctcctctatcaccattcttcttgagattagtagcttcgccaaagactgcatcttcaactggatcttgagtagaaaacagcacatttgatatactaccagtgctacttttcctgctgttgacatcaaatataccagacggaactttcacaatactgctgccccatgcaggaggttcagtaggactgtgaggctctggactaggttgtgaatgttttgccacaatagcagaggcatcacacacctcttctgtttgcatttttgttttagttatcaattctcttgctgcctgttcttcaggcacatgaatttctgcatcatcctttataagttcatccttagacccgtatccttggtcagactgaccacctgatattgaggagacctgtgacctttgcacagtctttttaagcggctgcctaaactgtgccaagccacgtaccacattccgtaccttcgtccataagaaaataccactgcgggtactgctaggccacgggctctccaagactaccttattataataaccataagtaatagcattaggctttatcctagcagttttcatttcaaataagactctcactgctaaaacaggatgaccccaaagtccacaaagctgcatcactactcgatagcacacctcatctaagggatccacatctgttttcctcatcttaataagtacatcatatgcctgctgaagtgctctgactttaggatgagaaactctaacataggccggaagacaaataaaccataaactgtaacaatgactaaacagacacttggcccactgtggtggatttgtataacatctcttcgccaatttatgagctgtttttatttcctgtttagttctcttagccatgagaggtggactctttgtaatgctattcccagtagggtgtctactaaaacaaagtttcaactcctgcggtctgtcaaaaagcttaaggtccagtcttggaaagtatttgtaactgtactttggtgacaggtcctttccatcatcaggaggtggctctggcggcattataaatacagtatgctcacttttctgtgaatcatctagttctatcaatctggtatcttctgctgaatcaaaatcaaccttatctgttttctctgtgcctttatcaggaaacaacttttctatgcagtcatcaaaaaatgctaatccagtatctttatcacttacaaaactgcattcttcaatgaaacgaataaaaatctgtgttttggataaaagggtatagaattttgcataggcacgatctcgactttttaaaaatccctgtcggtcaaacaatgaatcagcagctgtggctttatttgaaggagcctctgtgattggtctgagatatgttctatatccttttaaaatagacgccataaagcgcaaaaatgcctcttgaatttccatctcaagctgtgtcatcttcttttgccaggagaaatctgcttcaattggagtcatgtcaatcgctgagccttcttgagttttttggtgaactgaagacagctggggatacaatttctttaaggtgctaagtagatttttgcacggctttttgggaagttgcttccagttcatgttcttcttttcatctgatacatataacatgttcgtatccaagtcaatgcaaacaacatcttgtggtgggtcatgaagatcaaaataccttgagtcaactccaactataaatggtaaaggtgcactaagcactgcagccagtgaaagaggacaaaggggaatatatgggcattgccactgaaatggaaagatcatagctacaacagcttcagctaccccagtcaagacagctggccttagtggtaaaggtgtagaaactggctgtgataatattaatgcatcatggactgacagctggacaaggattctcggtctttgtggtgaaggaaaagggatgttttgcataaaatgtgaaatgtgcttttcaatgggaagaggatgtggtccagacacagaaagtttgtagataaacataagaaatttcctaaaagcttcaaaaaaaggccagtgtgagagtaaacaaatgcatttgtttgtattgatggatttggagaccatttttctctccacaggcgtcaacaagcccaggtgcataagctgtttctctgatagaagttcccgagagtaaggttcataaaactgaatggcagctccatatacctttttggctgaagaacctgtcaagacaaaagttgaaaaaactggaagtggatatttggtttcaggatcccagcactcaatagtagctcccataggaaggcagaaaagaggtacatctgattctgagagtggaaatgactcatagtcctcttctggatatctaaaaattaaaccagccttatatgctattgcatttgaagcaggtacagacttcttataacacagaaacacgctggaaccccacattccacaatttaagtttttgtcaactttgcagaaggtatgaggaggagtttctcctttactggttacaataacacagatatcagttacagccaaggaattctggggtcgaactggaggagcccttcgataagtgataaagattctttgtgaagtagttgaactattgttgacattggcacagcgaccatagggtgtggctaggatcacttcacatcctggaataagccgttctttcccttcatatagaactccaatatctgtaagcggtggtttatctctccctctcttataacagaggaaaagttctgggcttttcagacttccatagttcaagtttgcttggagagctgatggagtggcttctacacaggtgtaaccttcaggtactgtttctccagctgatttgataataatggcaatgtctgtaattggagctttaggtccagttgacttagtatctaaacgatttatttcttgatccaaaagagtagatgtgtcagtgagaccagctacgacaaagtagtctgtcactcttggtcctttgtcttctatcatggctgctactgtattttctgctgcctgctcctctgtcagcgcagccccgacacggcttcttcctggggcaagaaagcaccggattcgcggactgggcgcgctcggcagggcagggcgggggactagctccagcggccgccgccgcctcagtccggtct

SEQ ID NO: 8469 - RNA, 7136 nt, Homo sapiens
  source 1..7136: mol_type = other RNA
aaaagtaattgcggtttttgccattaatagtggcaaaaactacaattaattttgtgccaacctaatacattaaagttagggaaggcagctgtcatcagattttcaggtaattttaagattaatgactacagacaagtttagtagtagtcatttatttaatagtcaatgagacccctttcagaaaaccgtattgcaacatgcaatctattttaataaatatacacttagaatatggctgtatatacacatacctacacagccctacacatatacaaacttacacaaatatgttgctctcttttttttttttttttttttttgagacggtctcactctgtcacccaagctggagttgcagtggcgtgatctccactcactgtagcctctgcctcagttcaagcgattctcctgcctcagcctgagtagctgggactacagtggtgcgcctggctaatttttgtatttttagtaaagacagggtctcaccgtgttggccaggctggtctcgaactcctggcctcaagtgatccacccaccttgctcagcctcccaaagtgctgggattacaggcctgagccaccgtgcccggccatgttgcttttataattgagatatttcatttgttttgggggttaggcaaatttaatttgccattcctcaaactcagtaacttcaaatataaacaatgcctagaatgaatatggttcctcattatttctatcaaactactacaaatactgaagaatcccaaagtagttttccacagaggcagaaaagcagttcaggggttgaaaatcttcaatattaataagccctgggacattcaaatggcacttcatatttcaaggtaatgcaatatgaatcataattcattatatattgtccccaagagttacttcaattccgtattcaccagttcttacgatttggaaaaaaaaacttgaatgtttccagatgaaatctaatccccaagccttgtgtgtcaacattctagtgaatctctatttaaatgagaggcgctccaaaacacttcctgcaccactcgacactggcacttggtggagcatcaattttctgcaacctttcaagaatctctgaagacagactattgtatgcaattccatattcattgtcaaatgcctcaatatcaatattctctcttcctagagacactaatgataagaagaggatttctctgtataaactcctttgtcttttcatgcctggcttcatttgctgtgaaagtaggttgatgggtttaagaacattattgtgctgaatactctgcctgatggtttctactaaagtgcttgtttcttgttgttcctctgacaggagagatgatttcttttcagaattaaaattcctccatgagacatacagaggttctcttggttcctgatgaaggttgatattatcccataacagctgaatatacacaagtttgctatcctgggacagagatgacagaggaagctgtacaccttcattacaatgttcagatgtgaggataagtcctggcaagttactaggaaggtccaaacgtctgaaataccaaacgaggttccagaaaatgattggatgttgattgatgaaagaagatgtatgaatcacctgatcaccttcattttctagcaaagattcaagttctttacggagtactagaggactcaagtagggcacagaaacagggggaggattgggtctttttcctaaaggatccacaacttcctgcagactatttggaagactaactgttgagatgccatgaaacggtcgctgggtaaagtcaatattctgcaatgggcctccaacactgtgacttcgagtcaaagacacatttcgctttgataaactattaggcacagatgaaattttcatagtttggacatctccactggctctctttatttcatcacttggttcaactgcagagcctgtttcttcagttatgatctggttatgttttgggaagtccataaagttgatcaagtcaggttctgctaaactggatacaggtttgtgctccaaggattcatttgccaatggaatgcttccactttgtaaactgtcaccagaggtacttggtttcaggaaaaagcttgcagaacctctcaaatctttgaattctatattgagaagaggcaagaagttgcttttacagaatggacaagctgtattcaaatttgagtcatctgctgtccatccagccataatttcttcatcataaactaaagctccacaagctctacactgtgaacaactggacatcaaaacctccattgcacaattctgatagatgctagacatgctggtattttgagaagaaccatgatctgatttttcaaagtcttgccctttcatgcctcttggaaatggaacttcacctgttggataatgcagttttcctacatctccactactgctgctactgccaagacttgtgttgctctgggtaagttcactggggaccaaccctgagatacttgtgttaggcgatatattctcccccaaaatatggtcttctaggccagctgggaagctgtagtctctattagtttcttcctcatcatctgagtagctgtaggcagacgcaacagctacccacatcttactggctactgtcgctgcttgtttcataccagatttcaggacatctatcttgggccctgagagtatattatccagctttagccctgacaaagaatttactacagaacccaacgagccatgtggcgaagaacgcaccagtgctgacaaagaagttgaacgttctttatgagttcgagagggggtttgctgcttgaaacgcccagtaaaagttttagacctggacactgcaggtgagctcttttcactttcaggattttcctgtgctggtgaaccatgatctaaaggtaggcttgatctcctctctagagcatgaataaatgcagtagtcatgccagactctctgttttcctctctgtgtaattccatactagaagatttactacctaggggactttttaggttcatatagctttctatttcatcagccagattacgtgcaataactggagaaaacaacttatcttcagaatcaggagtttttcctcctgtacattcagtggctaaaagagacaaaggatctagtccagtttcaacatcttccctctgaaccaccttagcaataccatataaactacttctcttattcctcagatctttggatactgttttcaagtctctggactgattactgttactatcacttagtagactctcatatgtatctactgttgcagtagttttaggtacgtcatcaaccacaggctcaaggagttcttggctttcctcaagcatctctggcaccggagatgatctgtgctcaggattccaagtgctttcagacatacaagtcctactatcaggtaggtgacagctaacattctcaaagctatgggttcttgcaatatgaagtagagaagtcttaggacatgtcaatgctgctgtgagaatcttggcatctgctcccatcatgatagccatttcacttgaattcgaatccaaactactcttcttaagcaacattcctgctcgactttcagaactaaaactacaactcctctcaggaaaatgcttttgtcttttttctcctctatcaccattcttcttgagattagtagcttcgccaaagactgcatcttcaactggatcttgagtagaaaacagcacatttgatatactaccagtgctacttttcctgctgttgacatcaaatataccagacggaactttcacaatactgctgccccatgcaggaggttcagtaggactgtgaggctctggactaggttgtgaatgttttgccacaatagcagaggcatcacacacctcttctgtttgcatttttgttttagttatcaattctcttgctgcctgttcttcaggcacatgaatttctgcatcatcctttataagttcatccttagacccgtatccttggtcagactgaccacctgatgtggttaacattcaagggtagaattaatgcacacgtgtatccatagcttcacgtcatataagtctgtctgtgctagagtgattatcaatggactcaagcctgattaaatctctgacgaagactgtgtgctccccattgttagcatcattagaactatccacactaccgtggctcaccgtgtccccatcacttccacctgtgacattttgaagagctgatattgaggagacctgtgacctttgcacagtctttttaagcggctgcctaaactgtgccaagccacgtaccacattccgtaccttcgtccataagaaaataccactgcgggtactgctaggccacgggctctccaagactaccttattataataaccataagtaatagcattaggctttatcctagcagttttcatttcaaataagactctcactgctaaaacaggatgaccccaaagtccacaaagctgcatcactactcgatagcacacctcatctaagggatccacatctgttttcctcatcttaataagtacatcatatgcctgctgaagtgctctgactttaggatgagaaactctaacataggccggaagacaaataaaccataaactgtaacaatgactaaacagacacttggcccactgtggtggatttgtataacatctcttcgccaatttatgagctgtttttatttcctgtttagttctcttagccatgagaggtggactctttgtaatgctattcccagtagggtgtctactaaaacaaagtttcaactcctgcggtctgtcaaaaagcttaaggtccagtcttggaaagtatttgtaactgtactttggtgacaggtcctttccatcatcaggaggtggctctggcggcattataaatacagtatgctcacttttctgtgaatcatctagttctatcaatctggtatcttctgctgaatcaaaatcaaccttatctgttttctctgtgcctttatcaggaaacaacttttctatgcagtcatcaaaaaatgctaatccagtatctttatcacttacaaaactgcattcttcaatgaaacgaataaaaatctgtgttttggataaaagggtatagaattttgcataggcacgatctcgactttttaaaaatccctgtcggtcaaacaatgaatcagcagctgtggctttatttgaaggagcctctgtgattggtctgagatatgttctatatccttttaaaatagacgccataaagcgcaaaaatgcctcttgaatttccatctcaagctgtgtcatcttcttttgccaggagaaatctgcttcaattggagtcatgtcaatcgctgagccttcttgagttttttggtgaactgaagacagctggggatacaatttctttaaggtgctaagtagatttttgcacggctttttgggaagttgcttccagttcatgttcttcttttcatctgatagctacaacagcttcagctaccccagtcaagacagctggcctaagagaatgcagcagaattttactctcaagtaaaacaaagagcagcagtgttgcacaattctcaggacccagattcattagcaaggtgctaaagttggctccacttagtggtaaaggtgtagaaactggctgtgataatattaatgcatcatggactgacagctggacaaggattctcggtctttgtggtgaaggaaaagggatgttttgcataaaatgtgaaatgtgcttttcaatgggaagaggatgtggtccagacacagaaagtttgtagataaacataagaaatttcctaaaagcttcaaaaaaaggccagtgtgagagtaaacaaatgcatttgtttgtattgatggatttggagaccatttttctctccacaggcgtcaacaagcccaggtgcataagctgtttctctgatagaagttcccgagagtaaggttcataaaactgaatggcagctccatatacctttttggctgaagaacctgtcaagacaaaagttgaaaaaactggaagtggatatttggtttcaggatcccagcactcaatagtagctcccataggaaggcagaaaagaggtacatctgattctgagagtggaaatgactcatagtcctcttctggatatctaaaaattaaacctgtattttcagtttttatcccaccataccagtggaatgaagacgtgacacttaaatctttacagcccttgacactttaatgtgcagtaagaatgtggcgatagatttctcaaacacttcatggcagaaaagtttctcaggccctcctctcctccatatagctgattctttgcaacaaaggagaaaggaagcaagtccaccagccttatatgctattgcatttgaagcaggtacagacttcttataacacagaaacacgctggaaccccacattccacaatttaagtttttgtcaactttgcagaaggtatgaggaggagtttctcctttactggttacaataacacagatatcagttacagccaaggaattctggggtcgaactggaggagcccttcgataagtgataaagattctttgtgaagtagttgaactattgttgacattggcacagcgaccatagggtgtggctaggatcacttcacatcctggaataagccgttctttcccttcatatagaactccaatatctgtaagcggtggtttatctctccctctcttataacagaggaaaagttctgggcttttcagacttccatagttcaagtttgcttggagagctgatggagtggcttctacacaggtgtaaccttcaggtactgtttctccagctgatttgataataatggcaatgtctgtaattggagctttaggtccagttgacttagtatctaaacgatttatttcttgatccaaaagagtagatgtgtcagtgagaccagctacgacaaagtagtctgtcactcttggtcctttgtcttctatcatggctgctactgtattttctgctgcctgctcctctgtcagcgcagccccgacacggcttcttcctggggcaagaaagcaccggattcgcggactgggcgcgctcggcagggcagggcgggggactagctccagcggccgccgccgcctcagtccggtct

SEQ ID NO: 8470 - RNA, 6759 nt, Homo sapiens
  source 1..6759: mol_type = other RNA
aaaagtaattgcggtttttgccattaatagtggcaaaaactacaattaattttgtgccaacctaatacattaaagttagggaaggcagctgtcatcagattttcaggtaattttaagattaatgactacagacaagtttagtagtagtcatttatttaatagtcaatgagacccctttcagaaaaccgtattgcaacatgcaatctattttaataaatatacacttagaatatggctgtatatacacatacctacacagccctacacatatacaaacttacacaaatatgttgctctcttttttttttttttttttttttgagacggtctcactctgtcacccaagctggagttgcagtggcgtgatctccactcactgtagcctctgcctcagttcaagcgattctcctgcctcagcctgagtagctgggactacagtggtgcgcctggctaatttttgtatttttagtaaagacagggtctcaccgtgttggccaggctggtctcgaactcctggcctcaagtgatccacccaccttgctcagcctcccaaagtgctgggattacaggcctgagccaccgtgcccggccatgttgcttttataattgagatatttcatttgttttgggggttaggcaaatttaatttgccattcctcaaactcagtaacttcaaatataaacaatgcctagaatgaatatggttcctcattatttctatcaaactactacaaatactgaagaatcccaaagtagttttccacagaggcagaaaagcagttcaggggttgaaaatcttcaatattaataagccctgggacattcaaatggcacttcatatttcaaggtaatgcaatatgaatcataattcattatatattgtccccaagagttacttcaattccgtattcaccagttcttacgatttggaaaaaaaaacttgaatgtttccagatgaaatctaatccccaagccttgtgtgtcaacattctagtgaatctctatttaaatgagaggcgctccaaaacacttcctgcaccactcgacactggcacttggtggagcatcaattttctgcaacctttcaagaatctctgaagacagactattgtatgcaattccatattcattgtcaaatgcctcaatatcaatattctctcttcctagagacactaatgataagaagaggatttctctgtataaactcctttgtcttttcatgcctggcttcatttgctgtgaaagtaggttgatgggtttaagaacattattgtgctgaatactctgcctgatggtttctactaaagtgcttgtttcttgttgttcctctgacaggagagatgatttcttttcagaattaaaattcctccatgagacatacagaggttctcttggttcctgatgaaggttgatattatcccataacagctgaatatacacaagtttgctatcctgggacagagatgacagaggaagctgtacaccttcattacaatgttcagatgtgaggataagtcctggcaagttactaggaaggtccaaacgtctgaaataccaaacgaggttccagaaaatgattggatgttgattgatgaaagaagatgtatgaatcacctgatcaccttcattttctagcaaagattcaagttctttacggagtactagaggactcaagtagggcacagaaacagggggaggattgggtctttttcctaaaggatccacaacttcctgcagactatttggaagactaactgttgagatgccatgaaacggtcgctgggtaaagtcaatattctgcaatgggcctccaacactgtgacttcgagtcaaagacacatttcgctttgataaactattaggcacagatgaaattttcatagtttggacatctccactggctctctttatttcatcacttggttcaactgcagagcctgtttcttcagttatgatctggttatgttttgggaagtccataaagttgatcaagtcaggttctgctaaactggatacaggtttgtgctccaaggattcatttgccaatggaatgcttccactttgtaaactgtcaccagaggtacttggtttcaggaaaaagcttgcagaacctctcaaatctttgaattctatattgagaagaggcaagaagttgcttttacagaatggacaagctgtattcaaatttgagtcatctgctgtccatccagccataatttcttcatcataaactaaagctccacaagctctacactgtgaacaactggacatcaaaacctccattgcacaattctgatagatgctagacatgctggtattttgagaagaaccatgatctgatttttcaaagtcttgccctttcatgcctcttggaaatggaacttcacctgttggataatgcagttttcctacatctccactactgctgctactgccaagacttgtgttgctctgggtaagttcactggggaccaaccctgagatacttgtgttaggcgatatattctcccccaaaatatggtcttctaggccagctgggaagctgtagtctctattagtttcttcctcatcatctgagtagctgtaggcagacgcaacagctacccacatcttactggctactgtcgctgcttgtttcataccagatttcaggacatctatcttgggccctgagagtatattatccagctttagccctgacaaagaatttactacagaacccaacgagccatgtggcgaagaacgcaccagtgctgacaaagaagttgaacgttctttatgagttcgagagggggtttgctgcttgaaacgcccagtaaaagttttagacctggacactgcaggtgagctcttttcactttcaggattttcctgtgctggtgaaccatgatctaaaggtaggcttgatctcctctctagagcatgaataaatgcagtagtcatgccagactctctgttttcctctctgtgtaattccatactagaagatttactacctaggggactttttaggttcatatagctttctatttcatcagccagattacgtgcaataactggagaaaacaacttatcttcagaatcaggagtttttcctcctgtacattcagtggctaaaagagacaaaggatctagtccagtttcaacatcttccctctgaaccaccttagcaataccatataaactacttctcttattcctcagatctttggatactgttttcaagtctctggactgattactgttactatcacttagtagactctcatatgtatctactgttgcagtagttttaggtacgtcatcaaccacaggctcaaggagttcttggctttcctcaagcatctctggcaccggagatgatctgtgctcaggattccaagtgctttcagacatacaagtcctactatcaggtaggtgacagctaacattctcaaagctatgggttcttgcaatatgaagtagagaagtcttaggacatgtcaatgctgctgtgagaatcttggcatctgctcccatcatgatagccatttcacttgaattcgaatccaaactactcttcttaagcaacattcctgctcgactttcagaactaaaactacaactcctctcaggaaaatgcttttgtcttttttctcctctatcaccattcttcttgagattagtagcttcgccaaagactgcatcttcaactggatcttgagtagaaaacagcacatttgatatactaccagtgctacttttcctgctgttgacatcaaatataccagacggaactttcacaatactgctgccccatgcaggaggttcagtaggactgtgaggctctggactaggttgtgaatgttttgccacaatagcagaggcatcacacacctcttctgtttgcatttttgttttagttatcaattctcttgctgcctgttcttcaggcacatgaatttctgcatcatcctttataagttcatccttagacccgtatccttggtcagactgaccacctgatgtggttaacattcaagggtagaattaatgcacacgtgtatccatagcttcacgtcatataagtctgtctgtgctagagtgattatcaatggactcaagcctgattaaatctctgacgaagactgtgtgctccccattgttagcatcattagaactatccacactaccgtggctcaccgtgtccccatcacttccacctgtgacattttgaagagctgatattgaggagacctgtgacctttgcacagtctttttaagcggctgcctaaactgtgccaagccacgtaccacattccgtaccttcgtccataagaaaataccactgcgggtactgctaggccacgggctctccaagactaccttattataataaccataagtaatagcattaggctttatcctagcagttttcatttcaaataagactctcactgctaaaacaggatgaccccaaagtccacaaagctgcatcactactcgatagcacacctgtttagttctcttagccatgagaggtggactctttgtaatgctattcccagtagggtgtctactaaaacaaagtttcaactcctgcggtctgtcaaaaagcttaaggtccagtcttggaaagtatttgtaactgtactttggtgacaggtcctttccatcatcaggaggtggctctggcggcattataaatacagtatgctcacttttctgtgaatcatctagttctatcaatctggtatcttctgctgaatcaaaatcaaccttatctgttttctctgtgcctttatcaggaaacaacctgtcggtcaaacaatgaatcagcagctgtggctttatttgaaggagcctctgtgattggtctgagatatgttctatatccttttaaaatagacgccataaagcgcaaaaatgcctcttgaatttccatctcaagctgtgtcatcttcttttgccaggagaaatctgcttcaattggagtcatgtcaatcgctgagccttcttgagttttttggtgaactgaagacagctggggatacaatttctttaaggtgctaagtagatttttgcacggctttttgggaagttgcttccagttcatgttcttcttttcatctgatacatataacatgttcgtatccaagtcaatgcaaacaacatcttgtggtgggtcatgaagatcaaaataccttgagtcaactccaactataaatggtaaaggtgcactaagcactgcagccagtgaaagaggacaaaggggaatatatgggcattgccactgaaatggaaagatcatagctacaacagcttcagctaccccagtcaagacagctggcctaagagaatgcagcagaattttactctcaagtaaaacaaagagcagcagtgttgcacaattctcaggacccagattcattagcaaggtgctaaagttggctccacttagtggtaaaggtgtagaaactggctgtgataatattaatgcatcatggactgacagctggacaaggattctcggtctttgtggtgaaggaaaagggatgttttgcataaaatgtgaaatgtgcttttcaatgggaagaggatgtggtccagacacagaaagtttgtagataaacataagaaatttcctaaaagcttcaaaaaaaggccagtgtgagagtaaacaaatgcatttgtttgtattgatggatttggagaccatttttctctccacaggcgtcaacaagcccaggtgcataagctgtttctctgatagaagttcccgagagtaaggttcataaaactgaatggcagctccatatacctttttggctgaagaacctgtcaagacaaaagttgaaaaaactggaagtggatatttggtttcaggatcccagcactcaatagtagctcccataggaaggcagaaaagaggtacatctgattctgagagtggaaatgactcatagtcctcttctggatatctaaaaattaaaccagccttatatgctattgcatttgaagcaggtacagacttcttataacacagaaacacgctggaaccccacattccacaatttaagtttttgtcaactttgcagaaggtatgaggaggagtttctcctttactggttacaataacacagatatcagttacagccaaggaattctggggtcgaactggaggagcccttcgataagtgataaagattctttgtgaagtagttgaactattgttgacattggcacagcgaccatagggtgtggctaggatcacttcacatcctggaataagccgttctttcccttcatatagaactccaatatctgtaagcggtggtttatctctccctctcttataacagaggaaaagttctgggcttttcagacttccatagttcaagtttgcttggagagctgatggagtggcttctacacaggtgtaaccttcaggtactgtttctccagctgatttgataataatggcaatgtctgtaattggagctttaggtccagttgacttagtatctaaacgatttatttcttgatccaaaagagtagatgtgtcagtgagaccagctacgacaaagtagtctgtcactcttggtcctttgtcttctatcatggctgctactgtattttctgctgcctgctcctctgtcagcgcagccccgacacggcttcttcctggggcaagaaagcaccggattcgcggactgggcgcgctcggcagggcagggcgggggactagctccagcggccgccgccgcctcagtccggtct

SEQ ID NO: 8471 - RNA, 7022 nt, Homo sapiens
  source 1..7022: mol_type = other RNA
aaaagtaattgcggtttttgccattaatagtggcaaaaactacaattaattttgtgccaacctaatacattaaagttagggaaggcagctgtcatcagattttcaggtaattttaagattaatgactacagacaagtttagtagtagtcatttatttaatagtcaatgagacccctttcagaaaaccgtattgcaacatgcaatctattttaataaatatacacttagaatatggctgtatatacacatacctacacagccctacacatatacaaacttacacaaatatgttgctctcttttttttttttttttttttttgagacggtctcactctgtcacccaagctggagttgcagtggcgtgatctccactcactgtagcctctgcctcagttcaagcgattctcctgcctcagcctgagtagctgggactacagtggtgcgcctggctaatttttgtatttttagtaaagacagggtctcaccgtgttggccaggctggtctcgaactcctggcctcaagtgatccacccaccttgctcagcctcccaaagtgctgggattacaggcctgagccaccgtgcccggccatgttgcttttataattgagatatttcatttgttttgggggttaggcaaatttaatttgccattcctcaaactcagtaacttcaaatataaacaatgcctagaatgaatatggttcctcattatttctatcaaactactacaaatactgaagaatcccaaagtagttttccacagaggcagaaaagcagttcaggggttgaaaatcttcaatattaataagccctgggacattcaaatggcacttcatatttcaaggtaatgcaatatgaatcataattcattatatattgtccccaagagttacttcaattccgtattcaccagttcttacgatttggaaaaaaaaacttgaatgtttccagatgaaatctaatccccaagccttgtgtgtcaacattctagtgaatctctatttaaatgagaggcgctccaaaacacttcctgcaccactcgacactggcacttggtggagcatcaattttctgcaacctttcaagaatctctgaagacagactattgtatgcaattccatattcattgtcaaatgcctcaatatcaatattctctcttcctagagacactaatgataagaagaggatttctctgtataaactcctttgtcttttcatgcctggcttcatttgctgtgaaagtaggttgatgggtttaagaacattattgtgctgaatactctgcctgatggtttctactaaagtgcttgtttcttgttgttcctctgacaggagagatgatttcttttcagaattaaaattcctccatgagacatacagaggttctcttggttcctgatgaaggttgatattatcccataacagctgaatatacacaagtttgctatcctgggacagagatgacagaggaagctgtacaccttcattacaatgttcagatgtgaggataagtcctggcaagttactaggaaggtccaaacgtctgaaataccaaacgaggttccagaaaatgattggatgttgattgatgaaagaagatgtatgaatcacctgatcaccttcattttctagcaaagattcaagttctttacggagtactagaggactcaagtagggcacagaaacagggggaggattgggtctttttcctaaaggatccacaacttcctgcagactatttggaagactaactgttgagatgccatgaaacggtcgctgggtaaagtcaatattctgcaatgggcctccaacactgtgacttcgagtcaaagacacatttcgctttgataaactattaggcacagatgaaattttcatagtttggacatctccactggctctctttatttcatcacttggttcaactgcagagcctgtttcttcagttatgatctggttatgttttgggaagtccataaagttgatcaagtcaggttctgctaaactggatacaggtttgtgctccaaggattcatttgccaatggaatgcttccactttgtaaactgtcaccagaggtacttggtttcaggaaaaagcttgcagaacctctcaaatctttgaattctatattgagaagaggcaagaagttgcttttacagaatggacaagctgtattcaaatttgagtcatctgctgtccatccagccataatttcttcatcataaactaaagctccacaagctctacactgtgaacaactggacatcaaaacctccattgcacaattctgatagatgctagacatgctggtattttgagaagaaccatgatctgatttttcaaagtcttgccctttcatgcctcttggaaatggaacttcacctgttggataatgcagttttcctacatctccactactgctgctactgccaagacttgtgttgctctgggtaagttcactggggaccaaccctgagatacttgtgttaggcgatatattctcccccaaaatatggtcttctaggccagctgggaagctgtagtctctattagtttcttcctcatcatctgagtagctgtaggcagacgcaacagctacccacatcttactggctactgtcgctgcttgtttcataccagatttcaggacatctatcttgggccctgagagtatattatccagctttagccctgacaaagaatttactacagaacccaacgagccatgtggcgaagaacgcaccagtgctgacaaagaagttgaacgttctttatgagttcgagagggggtttgctgcttgaaacgcccagtaaaagttttagacctggacactgcaggtgagctcttttcactttcaggattttcctgtgctggtgaaccatgatctaaaggtaggcttgatctcctctctagagcatgaataaatgcagtagtcatgccagactctctgttttcctctctgtgtaattccatactagaagatttactacctaggggactttttaggttcatatagctttctatttcatcagccagattacgtgcaataactggagaaaacaacttatcttcagaatcaggagtttttcctcctgtacattcagtggctaaaagagacaaaggatctagtccagtttcaacatcttccctctgaaccaccttagcaataccatataaactacttctcttattcctcagatctttggatactgttttcaagtctctggactgattactgttactatcacttagtagactctcatatgtatctactgttgcagtagttttaggtacgtcatcaaccacaggctcaaggagttcttggctttcctcaagcatctctggcaccggagatgatctgtgctcaggattccaagtgctttcagacatacaagtcctactatcaggtaggtgacagctaacattctcaaagctatgggttcttgcaatatgaagtagagaagtcttaggacatgtcaatgctgctgtgagaatcttggcatctgctcccatcatgatagccatttcacttgaattcgaatccaaactactcttcttaagcaacattcctgctcgactttcagaactaaaactacaactcctctcaggaaaatgcttttgtcttttttctcctctatcaccattcttcttgagattagtagcttcgccaaagactgcatcttcaactggatcttgagtagaaaacagcacatttgatatactaccagtgctacttttcctgctgttgacatcaaatataccagacggaactttcacaatactgctgccccatgcaggaggttcagtaggactgtgaggctctggactaggttgtgaatgttttgccacaatagcagaggcatcacacacctcttctgtttgcatttttgttttagttatcaattctcttgctgcctgttcttcaggcacatgaatttctgcatcatcctttataagttcatccttagacccgtatccttggtcagactgaccacctgtgctagagtgattatcaatggactcaagcctgattaaatctctgacgaagactgtgtgctccccattgttagcatcattagaactatccacactaccgtggctcaccgtgtccccatcacttccacctgatattgaggagacctgtgacctttgcacagtctttttaagcggctgcctaaactgtgccaagccacgtaccacattccgtaccttcgtccataagaaaataccactgcgggtactgctaggccacgggctctccaagactaccttattataataaccataagtaatagcattaggctttatcctagcagttttcatttcaaataagactctcactgctaaaacaggatgaccccaaagtccacaaagctgcatcactactcgatagcacacctcatctaagggatccacatctgttttcctcatcttaataagtacatcatatgcctgctgaagtgctctgactttaggatgagaaactctaacataggccggaagacaaataaaccataaactgtaacaatgactaaacagacacttggcccactgtggtggatttgtataacatctcttcgccaatttatgagctgtttttatttcctgtttagttctcttagccatgagaggtggactctttgtaatgctattcccagtagggtgtctactaaaacaaagtttcaactcctgcggtctgtcaaaaagcttaaggtccagtcttggaaagtatttgtaactgtactttggtgacaggtcctttccatcatcaggaggtggctctggcggcattataaatacagtatgctcacttttctgtgaatcatctagttctatcaatctggtatcttctgctgaatcaaaatcaaccttatctgttttctctgtgcctttatcaggaaacaacttttctatgcagtcatcaaaaaatgctaatccagtatctttatcacttacaaaactgcattcttcaatgaaacgaataaaaatctgtgttttggataaaagggtatagaattttgcataggcacgatctcgactttttaaaaatccctgtcggtcaaacaatgaatcagcagctgtggctttatttgaaggagcctctgtgattggtctgagatatgttctatatccttttaaaatagacgccataaagcgcaaaaatgcctcttgaatttccatctcaagctgtgtcatcttcttttgccaggagaaatctgcttcaattggagtcatgtcaatcgctgagccttcttgagttttttggtgaactgaagacagctggggatacaatttctttaaggtgctaagtagatttttgcacggctttttgggaagttgcttccagttcatgttcttcttttcatctgatacatataacatgttcgtatccaagtcaatgcaaacaacatcttgtggtgggtcatgaagatcaaaataccttgagtcaactccaactataaatggtaaaggtgcactaagcactgcagccagtgaaagaggacaaaggggaatatatgggcattgccactgaaatggaaagatcatagctacaacagcttcagctaccccagtcaagacagctggcctaagagaatgcagcagaattttactctcaagtaaaacaaagagcagcagtgttgcacaattctcaggacccagattcattagcaaggtgctaaagttggctccacttagtggtaaaggtgtagaaactggctgtgataatattaatgcatcatggactgacagctggacaaggattctcggtctttgtggtgaaggaaaagggatgttttgcataaaatgtgaaatgtgcttttcaatgggaagaggatgtggtccagacacagaaagtttgtagataaacataagaaatttcctaaaagcttcaaaaaaaggccagtgtgagagtaaacaaatgcatttgtttgtattgatggatttggagaccatttttctctccacaggcgtcaacaagcccaggtgcataagctgtttctctgatagaagttcccgagagtaaggttcataaaactgaatggcagctccatatacctttttggctgaagaacctgtcaagacaaaagttgaaaaaactggaagtggatatttggtttcaggatcccagcactcaatagtagctcccataggaaggcagaaaagaggtacatctgattctgagagtggaaatgactcatagtcctcttctggatatctaaaaattaaaccagccttatatgctattgcatttgaagcaggtacagacttcttataacacagaaacacgctggaaccccacattccacaatttaagtttttgtcaactttgcagaaggtatgaggaggagtttctcctttactggttacaataacacagatatcagttacagccaaggaattctggggtcgaactggaggagcccttcgataagtgataaagattctttgtgaagtagttgaactattgttgacattggcacagcgaccatagggtgtggctaggatcacttcacatcctggaataagccgttctttcccttcatatagaactccaatatctgtaagcggtggtttatctctccctctcttataacagaggaaaagttctgggcttttcagacttccatagttcaagtttgcttggagagctgatggagtggcttctacacaggtgtaaccttcaggtactgtttctccagctgatttgataataatggcaatgtctgtaattggagctttaggtccagttgacttagtatctaaacgatttatttcttgatccaaaagagtagatgtgtcagtgagaccagctacgacaaagtagtctgtcactcttggtcctttgtcttctatcatggctgctactgtattttctgctgcctgctcctctgtcagcgcagccccgacacggcttcttcctggggcaagaaagcaccggattcgcggactgggcgcgctcggcagggcagggcgggggactagctccagcggccgccgccgcctcagtccggtct

SEQ ID NO: 8472 - RNA, 5345 nt, Homo sapiens
  source 1..5345: mol_type = other RNA
aaaagtaattgcggtttttgccattaatagtggcaaaaactacaattaattttgtgccaacctaatacattaaagttagggaaggcagctgtcatcagattttcaggtaattttaagattaatgactacagacaagtttagtagtagtcatttatttaatagtcaatgagacccctttcagaaaaccgtattgcaacatgcaatctattttaataaatatacacttagaatatggctgtatatacacatacctacacagccctacacatatacaaacttacacaaatatgttgctctcttttttttttttttttttttttgagacggtctcactctgtcacccaagctggagttgcagtggcgtgatctccactcactgtagcctctgcctcagttcaagcgattctcctgcctcagcctgagtagctgggactacagtggtgcgcctggctaatttttgtatttttagtaaagacagggtctcaccgtgttggccaggctggtctcgaactcctggcctcaagtgatccacccaccttgctcagcctcccaaagtgctgggattacaggcctgagccaccgtgcccggccatgttgcttttataattgagatatttcatttgttttgggggttaggcaaatttaatttgccattcctcaaactcagtaacttcaaatataaacaatgcctagaatgaatatggttcctcattatttctatcaaactactacaaatactgaagaatcccaaagtagttttccacagaggcagaaaagcagttcaggggttgaaaatcttcaatattaataagccctgggacattcaaatggcacttcatatttcaaggtaatgcaatatgaatcataattcattatatattgtccccaagagttacttcaattccgtattcaccagttcttacgatttggaaaaaaaaacttgaatgtttccagatgaaatctaatccccaagccttgtgtgtcaacattctagtgaatctctatttaaatgagaggcgctccaaaacacttcctgcaccactcgacactggcacttggtggagcatcaattttctgcaacctttcaagaatctctgaagacagactattgtatgcaattccatattcattgtcaaatgcctcaatatcaatattctctcttcctagagacactaatgataagaagaggatttctctgtataaactcctttgtcttttcatgcctggcttcatttgctgtgaaagtaggttgatgggtttaagaacattattgtgctgaatactctgcctgatggtttctactaaagtgcttgtttcttgttgttcctctgacaggagagatgatttcttttcagaattaaaattcctccatgagacatacagaggttctcttggttcctgatgaaggttgatattatcccataacagctgaatatacacaagtttgctatcctgggacagagatgacagaggaagctgtacaccttcattacaatgttcagatgtgaggataagtcctggcaagttactaggaaggtccaaacgtctgaaataccaaacgaggttccagaaaatgattggatgttgattgatgaaagaagatgtatgaatcacctgatcaccttcattttctagcaaagattcaagttctttacggagtactagaggactcaagtagggcacagaaacagggggaggattgggtctttttcctaaaggatccacaacttcctgcagactatttggaagactaactgttgagatgccatgaaacggtcgctgggtaaagtcaatattctgcaatgggcctccaacactgtgacttcgagtcaaagacacatttcgctttgataaactattaggcacagatgaaattttcatagtttggacatctccactggctctctttatttcatcacttggttcaactgcagagcctgtttcttcagttatgatctggttatgttttgggaagtccataaagttgatcaagtcaggttctgctaaactggatacaggtttgtgctccaaggattcatttgccaatggaatgcttccactttgtaaactgtcaccagaggtacttggtttcaggaaaaagcttgcagaacctctcaaatctttgaattctatattgagaagaggcaagaagttgcttttacagaatggacaagctgtattcaaatttgagtcatctgctgtccatccagccataatttcttcatcataaactaaagctccacaagctctacactgtgaacaactggacatcaaaacctccattgcacaattctgatagatgctagacatgctggtattttgagaagaaccatgatctgatttttcaaagtcttgccctttcatgcctcttggaaatggaacttcacctgttggataatgcagttttcctacatctccactactgctgctactgccaagacttgtgttgctctgggtaagttcactggggaccaaccctgagatacttgtgttaggcgatatattctcccccaaaatatggtcttctaggccagctgggaagctgtagtctctattagtttcttcctcatcatctgagtagctgtaggcagacgcaacagctacccacatcttactggctactgtcgctgcttgtttcataccagatttcaggacatctatcttgggccctgagagtatattatccagctttagccctgacaaagaatttactacagaacccaacgagccatgtggcgaagaacgcaccagtgctgacaaagaagttgaacgttctttatgagttcgagagggggtttgctgcttgaaacgcccagtaaaagttttagacctggacactgcaggtgagctcttttcactttcaggattttcctgtgctggtgaaccatgatctaaaggtaggcttgatctcctctctagagcatgaataaatgcagtagtcatgccagactctctgttttcctctctgtgtaattccatactagaagatttactacctaggggactttttaggttcatatagctttctatttcatcagccagattacgtgcaataactggagaaaacaacttatcttcagaatcaggagtttttcctcctgtacattcagtggctaaaagagacaaaggatctagtccagtttcaacatcttccctctgaaccaccttagcaataccatataaactacttctcttattcctcagatctttggatactgttttcaagtctctggactgattactgttactatcacttagtagactctcatatgtatctactgttgcagtagttttaggtacgtcatcaaccacaggctcaaggagttcttggctttcctcaagcatctctggcaccggagatgatctgtgctcaggattccaagtgctttcagacatacaagtcctactatcaggtaggtgacagctaacattctcaaagctatgggttcttgcaatatgaagtagagaagtcttaggacatgtcaatgctgctgtgagaatcttggcatctgctcccatcatgatagccatttcacttgaattcgaatccaaactactcttcttaagcaacattcctgctcgactttcagaactaaaactacaactcctctcaggaaaatgcttttgtcttttttctcctctatcaccattcttcttgagattagtagcttcgccaaagactgcatcttcaactggatcttgagtagaaaacagcacatttgatatactaccagtgctacttttcctgctgttgacatcaaatataccagacggaactttcacaatactgctgccccatgcaggaggttcagtaggactgtgaggctctggactaggttgtgaatgttttgccacaatagcagaggcatcacacacctcttctgtttgcatttttgttttagttatcaattctcttgctgcctgttcttcaggcacatgaatttctgcatcatcctttataagttcatccttagacccgtatccttggtcagactgaccacctgtgctagagtgattatcaatggactcaagcctgattaaatctctgacgaagactgtgtgctccccattgttagcatcattagaactatccacactaccgtggctcaccgtgtccccatcacttccacctgtgacattttgaagagctgatattgaggagacctgtgacctttgcacagtctttttaagcggctgcctaaactgtgccaagccacgtaccacattccgtaccttcgtccataagaaaataccactgcgggtactgctaggccacgggctctccaagactaccttattataataaccataagtaatagcattaggctttatcctagcagttttcatttcaaataagactctcactgctaaaacaggatgaccccaaagtccacaaagctgcatcactactcgatagcacacctcatctaagggatccacatctgttttcctcatcttaataagtacatcatatgcctgctgaagtgctctgactttaggatgagaaactctaacataggccggaagacaaataaaccataaactgtaacaatgactaaacagacacttggcccactgtggtggatttgtataacatctcttcgccaatttatgagctgtttttatttccattccacaatttaagtttttgtcaactttgcagaaggtatgaggaggagtttctcctttactggttacaataacacagatatcagttacagccaaggaattctggggtcgaactggaggagcccttcgataagtgataaagattctttgtgaagtagttgaactattgttgacattggcacagcgaccatagggtgtggctaggatcacttcacatcctggaataagccgttctttcccttcatatagaactccaatatctgtaagcggtggtttatctctccctctcttataacagaggaaaagttctgggcttttcagacttccatagttcaagtttgcttggagagctgatggagtggcttctacacaggtgtaaccttcaggtactgtttctccagctgatttgataataatggcaatgtctgtaattggagctttaggtccagttgacttagtatctaaacgatttatttcttgatccaaaagagtagatgtgtcagtgagaccagctacgacaaagtagtctgtcactcttggtcctttgtcttctatcatggctgctactgtattttctgctgcctgctcctctgtcagcgcagccccgacacggcttcttcctggggcaagaaagcaccggattcgcggactgggcgcgctcggcagggcagggcgggggactagctccagcggccgccgccgcctcagtccggtct

SEQ ID NO: 8473 - RNA, 6801 nt, Homo sapiens
  source 1..6801: mol_type = other RNA
aaaagtaattgcggtttttgccattaatagtggcaaaaactacaattaattttgtgccaacctaatacattaaagttagggaaggcagctgtcatcagattttcaggtaattttaagattaatgactacagacaagtttagtagtagtcatttatttaatagtcaatgagacccctttcagaaaaccgtattgcaacatgcaatctattttaataaatatacacttagaatatggctgtatatacacatacctacacagccctacacatatacaaacttacacaaatatgttgctctcttttttttttttttttttttttgagacggtctcactctgtcacccaagctggagttgcagtggcgtgatctccactcactgtagcctctgcctcagttcaagcgattctcctgcctcagcctgagtagctgggactacagtggtgcgcctggctaatttttgtatttttagtaaagacagggtctcaccgtgttggccaggctggtctcgaactcctggcctcaagtgatccacccaccttgctcagcctcccaaagtgctgggattacaggcctgagccaccgtgcccggccatgttgcttttataattgagatatttcatttgttttgggggttaggcaaatttaatttgccattcctcaaactcagtaacttcaaatataaacaatgcctagaatgaatatggttcctcattatttctatcaaactactacaaatactgaagaatcccaaagtagttttccacagaggcagaaaagcagttcaggggttgaaaatcttcaatattaataagccctgggacattcaaatggcacttcatatttcaaggtaatgcaatatgaatcataattcattatatattgtccccaagagttacttcaattccgtattcaccagttcttacgatttggaaaaaaaaacttgaatgtttccagatgaaatctaatccccaagccttgtgtgtcaacattctagtgaatctctatttaaatgagaggcgctccaaaacacttcctgcaccactcgacactggcacttggtggagcatcaattttctgcaacctttcaagaatctctgaagacagactattgtatgcaattccatattcattgtcaaatgcctcaatatcaatattctctcttcctagagacactaatgataagaagaggatttctctgtataaactcctttgtcttttcatgcctggcttcatttgctgtgaaagtaggttgatgggtttaagaacattattgtgctgaatactctgcctgatggtttctactaaagtgcttgtttcttgttgttcctctgacaggagagatgatttcttttcagaattaaaattcctccatgagacatacagaggttctcttggttcctgatgaaggttgatattatcccataacagctgaatatacacaagtttgctatcctgggacagagatgacagaggaagctgtacaccttcattacaatgttcagatgtgaggataagtcctggcaagttactaggaaggtccaaacgtctgaaataccaaacgaggttccagaaaatgattggatgttgattgatgaaagaagatgtatgaatcacctgatcaccttcattttctagcaaagattcaagttctttacggagtactagaggactcaagtagggcacagaaacagggggaggattgggtctttttcctaaaggatccacaacttcctgcagactatttggaagactaactgttgagatgccatgaaacggtcgctgggtaaagtcaatattctgcaatgggcctccaacactgtgacttcgagtcaaagacacatttcgctttgataaactattaggcacagatgaaattttcatagtttggacatctccactggctctctttatttcatcacttggttcaactgcagagcctgtttcttcagttatgatctggttatgttttgggaagtccataaagttgatcaagtcaggttctgctaaactggatacaggtttgtgctccaaggattcatttgccaatggaatgcttccactttgtaaactgtcaccagaggtacttggtttcaggaaaaagcttgcagaacctctcaaatctttgaattctatattgagaagaggcaagaagttgcttttacagaatggacaagctgtattcaaatttgagtcatctgctgtccatccagccataatttcttcatcataaactaaagctccacaagctctacactgtgaacaactggacatcaaaacctccattgcacaattctgatagatgctagacatgctggtattttgagaagaaccatgatctgatttttcaaagtcttgccctttcatgcctcttggaaatggaacttcacctgttggataatgcagttttcctacatctccactactgctgctactgccaagacttgtgttgctctgggtaagttcactggggaccaaccctgagatacttgtgttaggcgatatattctcccccaaaatatggtcttctaggccagctgggaagctgtagtctctattagtttcttcctcatcatctgagtagctgtaggcagacgcaacagctacccacatcttactggctactgtcgctgcttgtttcataccagatttcaggacatctatcttgggccctgagagtatattatccagctttagccctgacaaagaatttactacagaacccaacgagccatgtggcgaagaacgcaccagtgctgacaaagaagttgaacgttctttatgagttcgagagggggtttgctgcttgaaacgcccagtaaaagttttagacctggacactgcaggtgagctcttttcactttcaggattttcctgtgctggtgaaccatgatctaaaggtaggcttgatctcctctctagagcatgaataaatgcagtagtcatgccagactctctgttttcctctctgtgtaattccatactagaagatttactacctaggggactttttaggttcatatagctttctatttcatcagccagattacgtgcaataactggagaaaacaacttatcttcagaatcaggagtttttcctcctgtacattcagtggctaaaagagacaaaggatctagtccagtttcaacatcttccctctgaaccaccttagcaataccatataaactacttctcttattcctcagatctttggatactgttttcaagtctctggactgattactgttactatcacttagtagactctcatatgtatctactgttgcagtagttttaggtacgtcatcaaccacaggctcaaggagttcttggctttcctcaagcatctctggcaccggagatgatctgtgctcaggattccaagtgctttcagacatacaagtcctactatcaggtaggtgacagctaacattctcaaagctatgggttcttgcaatatgaagtagagaagtcttaggacatgtcaatgctgctgtgagaatcttggcatctgctcccatcatgatagccatttcacttgaattcgaatccaaactactcttcttaagcaacattcctgctcgactttcagaactaaaactacaactcctctcaggaaaatgcttttgtcttttttctcctctatcaccattcttcttgagattagtagcttcgccaaagactgcatcttcaactggatcttgagtagaaaacagcacatttgatatactaccagtgctacttttcctgctgttgacatcaaatataccagacggaactttcacaatactgctgccccatgcaggaggttcagtaggactgtgaggctctggactaggttgtgaatgttttgccacaatagcagaggcatcacacacctcttctgtttgcatttttgttttagttatcaattctcttgctgcctgttcttcaggcacatgaatttctgcatcatcctttataagttcatccttagacccgtatccttggtcagactgaccacctgtgctagagtgattatcaatggactcaagcctgattaaatctctgacgaagactgtgtgctccccattgttagcatcattagaactatccacactaccgtggctcaccgtgtccccatcacttccacctgtgacattttgaagagctgatattgaggagacctgtgacctttgcacagtctttttaagcggctgcctaaactgtgccaagccacgtaccacattccgtaccttcgtccataagaaaataccactgcgggtactgctaggccacgggctctccaagactaccttattataataaccataagtaatagcattaggctttatcctagcagttttcatttcaaataagactctcactgctaaaacaggatgaccccaaagtccacaaagctgcatcactactcgatagcacacctcatctaagggatccacatctgttttcctcatcttaataagtacatcatatgcctgctgaagtgctctgactttaggatgagaaactctaacataggccggaagacaaataaaccataaactgtaacaatgactaaacagacacttggcccactgtggtggatttgtataacatctcttcgccaatttatgagctgtttttatttcctgtttagttctcttagccatgagaggtggactctttgtaatgctattcccagtagggtgtctactaaaacaaagtttcaactcctgcggtctgtcaaaaagcttaaggtccagtcttggaaagtatttgtaactgtactttggtgacaggtcctttccatcatcaggaggtggctctggcggcattataaatacagtatgctcacttttctgtgaatcatctagttctatcaatctggtatcttctgctgaatcaaaatcaaccttatctgttttctctgtgcctttatcaggaaacaacttttctatgcagtcatcaaaaaatgctaatccagtatctttatcacttacaaaactgcattcttcaatgaaacgaataaaaatctgtgttttggataaaagggtatagaattttgcataggcacgatctcgactttttaaaaatccctgtcggtcaaacaatgaatcagcagctgtggctttatttgaaggagcctctgtgattggtctgagatatgttctatatccttttaaaatagacgccataaagcgcaaaaatgcctcttgaatttccatctcaagctgtgtcatcttcttttgccaggagaaatctgcttcaattggagtcatgtcaatcgctgagccttcttgagttttttggtgaactgaagacagctggggatacaatttctttaaggtgctaagtagatttttgcacggctttttgggaagttgcttccagttcatgttcttcttttcatctgatacatataacatgttcgtatccaagtcaatgcaaacaacatcttgtggtgggtcatgaagatcaaaataccttgagtcaactccaactataaatggtaaaggtgcactaagcactgcagccagtgaaagaggacaaaggggaatatatgggcattgccactgaaatggaaagatcatagctacaacagcttcagctaccccagtcaagacagctggcctaagagaatgcagcagaattttactctcaagtaaaacaaagagcagcagtgttgcacaattctcaggacccagattcattagcaaggtgctaaagttggctccacttagtggtaaaggtgtagaaactggctgtgataatattaatgcatcatggactgacagctggacaaggattctcggtctttgtggtgaaggaaaagggatgttttgcataaaatgtgaaatgtgcctttttggctgaagaacctgtcaagacaaaagttgaaaaaactggaagtggatatttggtttcaggatcccagcactcaatagtagctcccataggaaggcagaaaagaggtacatctgattctgagagtggaaatgactcatagtcctcttctggatatctaaaaattaaaccagccttatatgctattgcatttgaagcaggtacagacttcttataacacagaaacacgctggaaccccacattccacaatttaagtttttgtcaactttgcagaaggtatgaggaggagtttctcctttactggttacaataacacagatatcagttacagccaaggaattctggggtcgaactggaggagcccttcgataagtgataaagattctttgtgaagtagttgaactattgttgacattggcacagcgaccatagggtgtggctaggatcacttcacatcctggaataagccgttctttcccttcatatagaactccaatatctgtaagcggtggtttatctctccctctcttataacagaggaaaagttctgggcttttcagacttccatagttcaagtttgcttggagagctgatggagtggcttctacacaggtgtaaccttcaggtactgtttctccagctgatttgataataatggcaatgtctgtaattggagctttaggtccagttgacttagtatctaaacgatttatttcttgatccaaaagagtagatgtgtcagtgagaccagctacgacaaagtagtctgtcactcttggtcctttgtcttctatcatggctgctactgtattttctgctgcctgctcctctgtcagcgcagccccgacacggcttcttcctggggcaagaaagcaccggattcgcggactgggcgcgctcggcagggcagggcgggggactagctccagcggccgccgccgcctcagtccggtct

SEQ ID NO: 8474 - RNA, 7040 nt, Homo sapiens
  source 1..7040: mol_type = other RNA
aaaagtaattgcggtttttgccattaatagtggcaaaaactacaattaattttgtgccaacctaatacattaaagttagggaaggcagctgtcatcagattttcaggtaattttaagattaatgactacagacaagtttagtagtagtcatttatttaatagtcaatgagacccctttcagaaaaccgtattgcaacatgcaatctattttaataaatatacacttagaatatggctgtatatacacatacctacacagccctacacatatacaaacttacacaaatatgttgctctcttttttttttttttttttttttgagacggtctcactctgtcacccaagctggagttgcagtggcgtgatctccactcactgtagcctctgcctcagttcaagcgattctcctgcctcagcctgagtagctgggactacagtggtgcgcctggctaatttttgtatttttagtaaagacagggtctcaccgtgttggccaggctggtctcgaactcctggcctcaagtgatccacccaccttgctcagcctcccaaagtgctgggattacaggcctgagccaccgtgcccggccatgttgcttttataattgagatatttcatttgttttgggggttaggcaaatttaatttgccattcctcaaactcagtaacttcaaatataaacaatgcctagaatgaatatggttcctcattatttctatcaaactactacaaatactgaagaatcccaaagtagttttccacagaggcagaaaagcagttcaggggttgaaaatcttcaatattaataagccctgggacattcaaatggcacttcatatttcaaggtaatgcaatatgaatcataattcattatatattgtccccaagagttacttcaattccgtattcaccagttcttacgatttggaaaaaaaaacttgaatgtttccagatgaaatctaatccccaagccttgtgtgtcaacattctagtgaatctctatttaaatgagaggcgctccaaaacacttcctgcaccactcgacactggcacttggtggagcatcaattttctgcaacctttcaagaatctctgaagacagactattgtatgcaattccatattcattgtcaaatgcctcaatatcaatattctctcttcctagagacactaatgataagaagaggatttctctgtataaactcctttgtcttttcatgcctggcttcatttgctgtgaaagtaggttgatgggtttaagaacattattgtgctgaatactctgcctgatggtttctactaaagtgcttgtttcttgttgttcctctgacaggagagatgatttcttttcagaattaaaattcctccatgagacatacagaggttctcttggttcctgatgaaggttgatattatcccataacagctgaatatacacaagtttgctatcctgggacagagatgacagaggaagctgtacaccttcattacaatgttcagatgtgaggataagtcctggcaagttactaggaaggtccaaacgtctgaaataccaaacgaggttccagaaaatgattggatgttgattgatgaaagaagatgtatgaatcacctgatcaccttcattttctagcaaagattcaagttctttacggagtactagaggactcaagtagggcacagaaacagggggaggattgggtctttttcctaaaggatccacaacttcctgcagactatttggaagactaactgttgagatgccatgaaacggtcgctgggtaaagtcaatattctgcaatgggcctccaacactgtgacttcgagtcaaagacacatttcgctttgataaactattaggcacagatgaaattttcatagtttggacatctccactggctctctttatttcatcacttggttcaactgcagagcctgtttcttcagttatgatctggttatgttttgggaagtccataaagttgatcaagtcaggttctgctaaactggatacaggtttgtgctccaaggattcatttgccaatggaatgcttccactttgtaaactgtcaccagaggtacttggtttcaggaaaaagcttgcagaacctctcaaatctttgaattctatattgagaagaggcaagaagttgcttttacagaatggacaagctgtattcaaatttgagtcatctgctgtccatccagccataatttcttcatcataaactaaagctccacaagctctacactgtgaacaactggacatcaaaacctccattgcacaattctgatagatgctagacatgctggtattttgagaagaaccatgatctgatttttcaaagtcttgccctttcatgcctcttggaaatggaacttcacctgttggataatgcagttttcctacatctccactactgctgctactgccaagacttgtgttgctctgggtaagttcactggggaccaaccctgagatacttgtgttaggcgatatattctcccccaaaatatggtcttctaggccagctgggaagctgtagtctctattagtttcttcctcatcatctgagtagctgtaggcagacgcaacagctacccacatcttactggctactgtcgctgcttgtttcataccagatttcaggacatctatcttgggccctgagagtatattatccagctttagccctgacaaagaatttactacagaacccaacgagccatgtggcgaagaacgcaccagtgctgacaaagaagttgaacgttctttatgagttcgagagggggtttgctgcttgaaacgcccagtaaaagttttagacctggacactgcaggtgagctcttttcactttcaggattttcctgtgctggtgaaccatgatctaaaggtaggcttgatctcctctctagagcatgaataaatgcagtagtcatgccagactctctgttttcctctctgtgtaattccatactagaagatttactacctaggggactttttaggttcatatagctttctatttcatcagccagattacgtgcaataactggagaaaacaacttatcttcagaatcaggagtttttcctcctgtacattcagtggctaaaagagacaaaggatctagtccagtttcaacatcttccctctgaaccaccttagcaataccatataaactacttctcttattcctcagatctttggatactgttttcaagtctctggactgattactgttactatcacttagtagactctcatatgtatctactgttgcagtagttttaggtacgtcatcaaccacaggctcaaggagttcttggctttcctcaagcatctctggcaccggagatgatctgtgctcaggattccaagtgctttcagacatacaagtcctactatcaggtaggtgacagctaacattctcaaagctatgggttcttgcaatatgaagtagagaagtcttaggacatgtcaatgctgctgtgagaatcttggcatctgctcccatcatgatagccatttcacttgaattcgaatccaaactactcttcttaagcaacattcctgctcgactttcagaactaaaactacaactcctctcaggaaaatgcttttgtcttttttctcctctatcaccattcttcttgagattagtagcttcgccaaagactgcatcttcaactggatcttgagtagaaaacagcacatttgatatactaccagtgctacttttcctgctgttgacatcaaatataccagacggaactttcacaatactgctgccccatgcaggaggttcagtaggactgtgaggctctggactaggttgtgaatgttttgccacaatagcagaggcatcacacacctcttctgtttgcatttttgttttagttatcaattctcttgctgcctgttcttcaggcacatgaatttctgcatcatcctttataagttcatccttagacccgtatccttggtcagactgaccacctgtgctagagtgattatcaatggactcaagcctgattaaatctctgacgaagactgtgtgctccccattgttagcatcattagaactatccacactaccgtggctcaccgtgtccccatcacttccacctgtgacattttgaagagctgatattgaggagacctgtgacctttgcacagtctttttaagcggctgcctaaactgtgccaagccacgtaccacattccgtaccttcgtccataagaaaataccactgcgggtactgctaggccacgggctctccaagactaccttattataataaccataagtaatagcattaggctttatcctagcagttttcatttcaaataagactctcactgctaaaacaggatgaccccaaagtccacaaagctgcatcactactcgatagcacacctcatctaagggatccacatctgttttcctcatcttaataagtacatcatatgcctgctgaagtgctctgactttaggatgagaaactctaacataggccggaagacaaataaaccataaactgtaacaatgactaaacagacacttggcccactgtggtggatttgtataacatctcttcgccaatttatgagctgtttttatttcctgtttagttctcttagccatgagaggtggactctttgtaatgctattcccagtagggtgtctactaaaacaaagtttcaactcctgcggtctgtcaaaaagcttaaggtccagtcttggaaagtatttgtaactgtactttggtgacaggtcctttccatcatcaggaggtggctctggcggcattataaatacagtatgctcacttttctgtgaatcatctagttctatcaatctggtatcttctgctgaatcaaaatcaaccttatctgttttctctgtgcctttatcaggaaacaacttttctatgcagtcatcaaaaaatgctaatccagtatctttatcacttacaaaactgcattcttcaatgaaacgaataaaaatctgtgttttggataaaagggtatagaattttgcataggcacgatctcgactttttaaaaatccctgtcggtcaaacaatgaatcagcagctgtggctttatttgaaggagcctctgtgattggtctgagatatgttctatatccttttaaaatagacgccataaagcgcaaaaatgcctcttgaatttccatctcaagctgtgtcatcttcttttgccaggagaaatctgcttcaattggagtcatgtcaatcgctgagccttcttgagttttttggtgaactgaagacagctggggatacaatttctttaaggtgctaagtagatttttgcacggctttttgggaagttgcttccagttcatgttcttcttttcatctgatacatataacatgttcgtatccaagtcaatgcaaacaacatcttgtggtgggtcatgaagatcaaaataccttgagtcaactccaactataaatggtaaaggtgcactaagcactgcagccagtgaaagaggacaaaggggaatatatgggcattgccactgaaatggaaagatcatagctacaacagcttcagctaccccagtcaagacagctggcctaagagaatgcagcagaattttactctcaagtaaaacaaagagcagcagtgttgcacaattctcaggacccagattcattagcaaggtgctaaagttggctccacttagtggtaaaggtgtagaaactggctgtgataatattaatgcatcatggactgacagctggacaaggattctcggtctttgtggtgaaggaaaagggatgttttgcataaaatgtgaaatgtgcttttcaatgggaagaggatgtggtccagacacagaaagtttgtagataaacataagaaatttcctaaaagcttcaaaaaaaggccagtgtgagagtaaacaaatgcatttgtttgtattgatggatttggagaccatttttctctccacaggcgtcaacaagcccaggtgcataagctgtttctctgatagaagttcccgagagtaaggttcataaaactgaatggcagctccatatacctttttggctgaagaacctgtcaagacaaaagttgaaaaaactggaagtggatatttggtttcaggatcccagcactcaatagtagctcccataggaaggcagaaaagaggtacatctgattctgagagtggaaatgactcatagtcctcttctggatatctaaaaattaaaccagccttatatgctattgcatttgaagcaggtacagacttcttataacacagaaacacgctggaaccccacattccacaatttaagtttttgtcaactttgcagaaggtatgaggaggagtttctcctttactggttacaataacacagatatcagttacagccaaggaattctggggtcgaactggaggagcccttcgataagtgataaagattctttgtgaagtagttgaactattgttgacattggcacagcgaccatagggtgtggctaggatcacttcacatcctggaataagccgttctttcccttcatatagaactccaatatctgtaagcggtggtttatctctccctctcttataacagaggaaaagttctgggcttttcagacttccatagttcaagtttgcttggagagctgatggagtggcttctacacaggtgtaaccttcaggtactgtttctccagctgatttgataataatggcaatgtctgtaattggagctttaggtccagttgacttagtatctaaacgatttatttcttgatccaaaagagtagatgtgtcagtgagaccagctacgacaaagtagtctgtcactcttggtcctttgtcttctatcatggctgctactgtattttctgctgcctgctcctctgtcagcgcagccccgacacggcttcttcctggggcaagaaagcaccggattcgcggactgggcgcgctcggcagggcagggcgggggactagctccagcggccgccgccgcctcagtccggtct

SEQ ID NO: 8475 - RNA, 7130 nt, Homo sapiens
  source 1..7130: mol_type = other RNA
aaaagtaattgcggtttttgccattaatagtggcaaaaactacaattaattttgtgccaacctaatacattaaagttagggaaggcagctgtcatcagattttcaggtaattttaagattaatgactacagacaagtttagtagtagtcatttatttaatagtcaatgagacccctttcagaaaaccgtattgcaacatgcaatctattttaataaatatacacttagaatatggctgtatatacacatacctacacagccctacacatatacaaacttacacaaatatgttgctctcttttttttttttttttttttttgagacggtctcactctgtcacccaagctggagttgcagtggcgtgatctccactcactgtagcctctgcctcagttcaagcgattctcctgcctcagcctgagtagctgggactacagtggtgcgcctggctaatttttgtatttttagtaaagacagggtctcaccgtgttggccaggctggtctcgaactcctggcctcaagtgatccacccaccttgctcagcctcccaaagtgctgggattacaggcctgagccaccgtgcccggccatgttgcttttataattgagatatttcatttgttttgggggttaggcaaatttaatttgccattcctcaaactcagtaacttcaaatataaacaatgcctagaatgaatatggttcctcattatttctatcaaactactacaaatactgaagaatcccaaagtagttttccacagaggcagaaaagcagttcaggggttgaaaatcttcaatattaataagccctgggacattcaaatggcacttcatatttcaaggtaatgcaatatgaatcataattcattatatattgtccccaagagttacttcaattccgtattcaccagttcttacgatttggaaaaaaaaacttgaatgtttccagatgaaatctaatccccaagccttgtgtgtcaacattctagtgaatctctatttaaatgagaggcgctccaaaacacttcctgcaccactcgacactggcacttggtggagcatcaattttctgcaacctttcaagaatctctgaagacagactattgtatgcaattccatattcattgtcaaatgcctcaatatcaatattctctcttcctagagacactaatgataagaagaggatttctctgtataaactcctttgtcttttcatgcctggcttcatttgctgtgaaagtaggttgatgggtttaagaacattattgtgctgaatactctgcctgatggtttctactaaagtgcttgtttcttgttgttcctctgacaggagagatgatttcttttcagaattaaaattcctccatgagacatacagaggttctcttggttcctgatgaaggttgatattatcccataacagctgaatatacacaagtttgctatcctgggacagagatgacagaggaagctgtacaccttcattacaatgttcagatgtgaggataagtcctggcaagttactaggaaggtccaaacgtctgaaataccaaacgaggttccagaaaatgattggatgttgattgatgaaagaagatgtatgaatcacctgatcaccttcattttctagcaaagattcaagttctttacggagtactagaggactcaagtagggcacagaaacagggggaggattgggtctttttcctaaaggatccacaacttcctgcagactatttggaagactaactgttgagatgccatgaaacggtcgctgggtaaagtcaatattctgcaatgggcctccaacactgtgacttcgagtcaaagacacatttcgctttgataaactattaggcacagatgaaattttcatagtttggacatctccactggctctctttatttcatcacttggttcaactgcagagcctgtttcttcagttatgatctggttatgttttgggaagtccataaagttgatcaagtcaggttctgctaaactggatacaggtttgtgctccaaggattcatttgccaatggaatgcttccactttgtaaactgtcaccagaggtacttggtttcaggaaaaagcttgcagaacctctcaaatctttgaattctatattgagaagaggcaagaagttgcttttacagaatggacaagctgtattcaaatttgagtcatctgctgtccatccagccataatttcttcatcataaactaaagctccacaagctctacactgtgaacaactggacatcaaaacctccattgcacaattctgatagatgctagacatgctggtattttgagaagaaccatgatctgatttttcaaagtcttgccctttcatgcctcttggaaatggaacttcacctgttggataatgcagttttcctacatctccactactgctgctactgccaagacttgtgttgctctgggtaagttcactggggaccaaccctgagatacttgtgttaggcgatatattctcccccaaaatatggtcttctaggccagctgggaagctgtagtctctattagtttcttcctcatcatctgagtagctgtaggcagacgcaacagctacccacatcttactggctactgtcgctgcttgtttcataccagatttcaggacatctatcttgggccctgagagtatattatccagctttagccctgacaaagaatttactacagaacccaacgagccatgtggcgaagaacgcaccagtgctgacaaagaagttgaacgttctttatgagttcgagagggggtttgctgcttgaaacgcccagtaaaagttttagacctggacactgcaggtgagctcttttcactttcaggattttcctgtgctggtgaaccatgatctaaaggtaggcttgatctcctctctagagcatgaataaatgcagtagtcatgccagactctctgttttcctctctgtgtaattccatactagaagatttactacctaggggactttttaggttcatatagctttctatttcatcagccagattacgtgcaataactggagaaaacaacttatcttcagaatcaggagtttttcctcctgtacattcagtggctaaaagagacaaaggatctagtccagtttcaacatcttccctctgaaccaccttagcaataccatataaactacttctcttattcctcagatctttggatactgttttcaagtctctggactgattactgttactatcacttagtagactctcatatgtatctactgttgcagtagttttaggtacgtcatcaaccacaggctcaaggagttcttggctttcctcaagcatctctggcaccggagatgatctgtgctcaggattccaagtgctttcagacatacaagtcctactatcaggtaggtgacagctaacattctcaaagctatgggttcttgcaatatgaagtagagaagtcttaggacatgtcaatgctgctgtgagaatcttggcatctgctcccatcatgatagccatttcacttgaattcgaatccaaactactcttcttaagcaacattcctgctcgactttcagaactaaaactacaactcctctcaggaaaatgcttttgtcttttttctcctctatcaccattcttcttgagattagtagcttcgccaaagactgcatcttcaactggatcttgagtagaaaacagcacatttgatatactaccagtgctacttttcctgctgttgacatcaaatataccagacggaactttcacaatactgctgccccatgcaggaggttcagtaggactgtgaggctctggactaggttgtgaatgttttgccacaatagcagaggcatcacacacctcttctgtttgcatttttgttttagttatcaattctcttgctgcctgttcttcaggcacatgaatttctgcatcatcctttataagttcatccttagacccgtatccttggtcagactgaccacctgtgctagagtgattatcaatggactcaagcctgattaaatctctgacgaagactgtgtgctccccattgttagcatcattagaactatccacactaccgtggctcaccgtgtccccatcacttccacctgtgacattttgaagagctgatattgaggagacctgtgacctttgcacagtctttttaagcggctgcctaaactgtgccaagccacgtaccacattccgtaccttcgtccataagaaaataccactgcgggtactgctaggccacgggctctccaagactaccttattataataaccataagtaatagcattaggctttatcctagcagttttcatttcaaataagactctcactgctaaaacaggatgaccccaaagtccacaaagctgcatcactactcgatagcacacctcatctaagggatccacatctgttttcctcatcttaataagtacatcatatgcctgctgaagtgctctgactttaggatgagaaactctaacataggccggaagacaaataaaccataaactgtaacaatgactaaacagacacttggcccactgtggtggatttgtataacatctcttcgccaatttatgagctgtttttatttcctgtttagttctcttagccatgagaggtggactctttgtaatgctattcccagtagggtgtctactaaaacaaagtttcaactcctgcggtctgtcaaaaagcttaaggtccagtcttggaaagtatttgtaactgtactttggtgacaggtcctttccatcatcaggaggtggctctggcggcattataaatacagtatgctcacttttctgtgaatcatctagttctatcaatctggtatcttctgctgaatcaaaatcaaccttatctgttttctctgtgcctttatcaggaaacaacttttctatgcagtcatcaaaaaatgctaatccagtatctttatcacttacaaaactgcattcttcaatgaaacgaataaaaatctgtgttttggataaaagggtatagaattttgcataggcacgatctcgactttttaaaaatccctgtcggtcaaacaatgaatcagcagctgtggctttatttgaaggagcctctgtgattggtctgagatatgttctatatccttttaaaatagacgccataaagcgcaaaaatgcctcttgaatttccatctcaagctgtgtcatcttcttttgccaggagaaatctgcttcaattggagtcatgtcaatcgctgagccttcttgagttttttggtgaactgaagacagctggggatacaatttctttaaggtgctaagtagatttttgcacggctttttgggaagttgcttccagttcatgttcttcttttcatctgatacatataacatgttcgtatccaagtcaatgcaaacaacatcttgtggtgggtcatgaagatcaaaataccttgagtcaactccaactataaatggtaaaggtgcactaagcactgcagccagtgaaagaggacaaaggggaatatatgggcattgccactgaaatggaaagatcatagctacaacagcttcagctaccccagtcaagacagctggcctaagagaatgcagcagaattttactctcaagtaaaacaaagagcagcagtgttgcacaattctcaggacccagattcattagcaaggtgctaaagttggctccacttagtggtaaaggtgtagaaactggctgtgataatattaatgcatcatggactgacagctggacaaggattctcggtctttgtggtgaaggaaaagggatgttttgcataaaatgtgaaatgtgcttttcaatgggaagaggatgtggtccagacacagaaagtttgtagataaacataagaaatttcctaaaagcttcaaaaaaaggccagtgtgagagtaaacaaatgcatttgtttgtattgatggatttggagaccatttttctctccacaggcgtcaacaagcccaggtgcataagctgtttctctgatagaagttcccgagagtaaggttcataaaactgaatggcagctccatatacctttttggctgaagaacctgtcaagacaaaagttgaaaaaactggaagtggatatttggtttcaggatcccagcactcaatagtagctcccataggaaggcagaaaagaggtacatctgattctgagagtggaaatgactcatagtcctcttctggatatctaaaaattaaaccagccttatatgctattgcatttgaagcaggtacagacttcttataacacagaaacacgctggaaccccacattccacaatttaagtttttgtcaactttgcagaaggtatgaggaggagtttctcctttactggttacaataacacagatatcagttacagccaaggaattctggggtcgaactggaggagcccttcgataagtgataaagattctttgtgaagtagttgaactattgttgacattggcacagcgaccatagggtgtggctaggatcacttcacatcctggaataagccgttctttcccttcatatagaactccaatatctgtaagcggtggtttatctctccctctcttataacagaggaaaagttctgggcttttcagacttccatagttcaagtttgcttggagagctgatggagtggcttctacacaggtgtaaccttcaggtactgtttctccagctgatttgataataatggcaatgtctgtaattggagctttaggtccagttgacttagtatctaaacgatttatttcttgatccaaaagagtagatgtgtcagtgagaccagctacgacaaagtagtctgtcactcttggtcctttgtcttctatcatggctgctactgtattttctgtcccgcgccctcccagccttgcagcgcaggccccgcgagggcacggcgcaggcttcctccgccaaaggccccgcgccgcagcctcacctgctgcctgctcctctgtcagcgcagccccgacacggcttcttcctggggcaagaaagcaccggattcgcggactgggcgcgctcggcagggcagggcgggggactagctccagcggccgccgccgcctcagtccggtct

SEQ ID NO: 8476 - RNA, 6970 nt, Homo sapiens
  source 1..6970: mol_type = other RNA
aaaagtaattgcggtttttgccattaatagtggcaaaaactacaattaattttgtgccaacctaatacattaaagttagggaaggcagctgtcatcagattttcaggtaattttaagattaatgactacagacaagtttagtagtagtcatttatttaatagtcaatgagacccctttcagaaaaccgtattgcaacatgcaatctattttaataaatatacacttagaatatggctgtatatacacatacctacacagccctacacatatacaaacttacacaaatatgttgctctcttttttttttttttttttttttgagacggtctcactctgtcacccaagctggagttgcagtggcgtgatctccactcactgtagcctctgcctcagttcaagcgattctcctgcctcagcctgagtagctgggactacagtggtgcgcctggctaatttttgtatttttagtaaagacagggtctcaccgtgttggccaggctggtctcgaactcctggcctcaagtgatccacccaccttgctcagcctcccaaagtgctgggattacaggcctgagccaccgtgcccggccatgttgcttttataattgagatatttcatttgttttgggggttaggcaaatttaatttgccattcctcaaactcagtaacttcaaatataaacaatgcctagaatgaatatggttcctcattatttctatcaaactactacaaatactgaagaatcccaaagtagttttccacagaggcagaaaagcagttcaggggttgaaaatcttcaatattaataagccctgggacattcaaatggcacttcatatttcaaggtaatgcaatatgaatcataattcattatatattgtccccaagagttacttcaattccgtattcaccagttcttacgatttggaaaaaaaaacttgaatgtttccagatgaaatctaatccccaagccttgtgtgtcaacattctagtgaatctctatttaaatgagaggcgctccaaaacacttcctgcaccactcgacactggcacttggtggagcatcaattttctgcaacctttcaagaatctctgaagacagactattgtatgcaattccatattcattgtcaaatgcctcaatatcaatattctctcttcctagagacactaatgataagaagaggatttctctgtataaactcctttgtcttttcatgcctggcttcatttgctgtgaaagtaggttgatgggtttaagaacattattgtgctgaatactctgcctgatggtttctactaaagtgcttgtttcttgttgttcctctgacaggagagatgatttcttttcagaattaaaattcctccatgagacatacagaggttctcttggttcctgatgaaggttgatattatcccataacagctgaatatacacaagtttgctatcctgggacagagatgacagaggaagctgtacaccttcattacaatgttcagatgtgaggataagtcctggcaagttactaggaaggtccaaacgtctgaaataccaaacgaggttccagaaaatgattggatgttgattgatgaaagaagatgtatgaatcacctgatcaccttcattttctagcaaagattcaagttctttacggagtactagaggactcaagtagggcacagaaacagggggaggattgggtctttttcctaaaggatccacaacttcctgcagactatttggaagactaactgttgagatgccatgaaacggtcgctgggtaaagtcaatattctgcaatgggcctccaacactgtgacttcgagtcaaagacacatttcgctttgataaactattaggcacagatgaaattttcatagtttggacatctccactggctctctttatttcatcacttggttcaactgcagagcctgtttcttcagttatgatctggttatgttttgggaagtccataaagttgatcaagtcaggttctgctaaactggatacaggtttgtgctccaaggattcatttgccaatggaatgcttccactttgtaaactgtcaccagaggtacttggtttcaggaaaaagcttgcagaacctctcaaatctttgaattctatattgagaagaggcaagaagttgcttttacagaatggacaagctgtattcaaatttgagtcatctgctgtccatccagccataatttcttcatcataaactaaagctccacaagctctacactgtgaacaactggacatcaaaacctccattgcacaattctgatagatgctagacatgctggtattttgagaagaaccatgatctgatttttcaaagtcttgccctttcatgcctcttggaaatggaacttcacctgttggataatgcagttttcctacatctccactactgctgctactgccaagacttgtgttgctctgggtaagttcactggggaccaaccctgagatacttgtgttaggcgatatattctcccccaaaatatggtcttctaggccagctgggaagctgtagtctctattagtttcttcctcatcatctgagtagctgtaggcagacgcaacagctacccacatcttactggctactgtcgctgcttgtttcataccagatttcaggacatctatcttgggccctgagagtatattatccagctttagccctgacaaagaatttactacagaacccaacgagccatgtggcgaagaacgcaccagtgctgacaaagaagttgaacgttctttatgagttcgagagggggtttgctgcttgaaacgcccagtaaaagttttagacctggacactgcaggtgagctcttttcactttcaggattttcctgtgctggtgaaccatgatctaaaggtaggcttgatctcctctctagagcatgaataaatgcagtagtcatgccagactctctgttttcctctctgtgtaattccatactagaagatttactacctaggggactttttaggttcatatagctttctatttcatcagccagattacgtgcaataactggagaaaacaacttatcttcagaatcaggagtttttcctcctgtacattcagtggctaaaagagacaaaggatctagtccagtttcaacatcttccctctgaaccaccttagcaataccatataaactacttctcttattcctcagatctttggatactgttttcaagtctctggactgattactgttactatcacttagtagactctcatatgtatctactgttgcagtagttttaggtacgtcatcaaccacaggctcaaggagttcttggctttcctcaagcatctctggcaccggagatgatctgtgctcaggattccaagtgctttcagacatacaagtcctactatcaggtaggtgacagctaacattctcaaagctatgggttcttgcaatatgaagtagagaagtcttaggacatgtcaatgctgctgtgagaatcttggcatctgctcccatcatgatagccatttcacttgaattcgaatccaaactactcttcttaagcaacattcctgctcgactttcagaactaaaactacaactcctctcaggaaaatgcttttgtcttttttctcctctatcaccattcttcttgagattagtagcttcgccaaagactgcatcttcaactggatcttgagtagaaaacagcacatttgatatactaccagtgctacttttcctgctgttgacatcaaatataccagacggaactttcacaatactgctgccccatgcaggaggttcagtaggactgtgaggctctggactaggttgtgaatgttttgccacaatagcagaggcatcacacacctcttctgtttgcatttttgttttagttatcaattctcttgctgcctgttcttcaggcacatgaatttctgcatcatcctttataagttcatccttagacccgtatccttggtcagactgaccacctgtgctagagtgattatcaatggactcaagcctgattaaatctctgacgaagactgtgtgctccccattgttagcatcattagaactatccacactaccgtggctcaccgtgtccccatcacttccacctgtgacattttgaagagctgatattgaggagacctgtgacctttgcacagtctttttaagcggctgcctaaactgtgccaagccacgtaccacattccgtaccttcgtccataagaaaataccactgcgggtactgctaggccacgggctctccaagactaccttattataataaccataagtaatagcattaggctttatcctagcagttttcatttcaaataagactctcactgctaaaacaggatgaccccaaagtccacaaagctgcatcactactcgatagcacacctcatctaagggatccacatctgttttcctcatcttaataagtacatcatatgcctgctgaagtgctctgactttaggatgagaaactctaacataggccggaagacaaataaaccataaactgtaacaatgactaaacagacacttggcccactgtggtggatttgtataacatctcttcgccaatttatgagctgtttttatttcctgtttagttctcttagccatgagaggtggactctttgtaatgctattcccagtagggtgtctactaaaacaaagtttcaactcctgcggtctgtcaaaaagcttaaggtccagtcttggaaagtatttgtaactgtactttggtgacaggtcctttccatcatcaggaggtggctctggcggcattataaatacagtatgctcacttttctgtgaatcatctagttctatcaatctggtatcttctgctgaatcaaaatcaaccttatctgttttctctgtgcctttatcaggaaacaacttttctatgcagtcatcaaaaaatgctaatccagtatctttatcacttacaaaactgcattcttcaatgaaacgaataaaaatctgtgttttggataaaagggtatagaattttgcataggcacgatctcgactttttaaaaatccctgtcggtcaaacaatgaatcagcagctgtggctttatttgaaggagcctctgtgattggtctgagatatgttctatatccttttaaaatagacgccataaagcgcaaaaatgcctcttgaatttccatctcaagctgtgtcatcttcttttgccaggagaaatctgcttcaattggagtcatgtcaatcgctgagccttcttgagttttttggtgaactgaagacagctggggatacaatttctttaaggtgctaagtagatttttgcacggctttttgggaagttgcttccagttcatgttcttcttttcatctgatacatataacatgttcgtatccaagtcaatgcaaacaacatcttgtggtgggtcatgaagatcaaaataccttgagtcaactccaactataaatggtaaaggtgcactaagcactgcagccagtgaaagaggacaaaggggaatatatgggcattgccactgaaatggaaagatcatagctacaacagcttcagctaccccagtcaagacagctggcctaagagaatgcagcagaattttactctcaagtaaaacaaagagcagcagtgttgcacaattctcaggacccagattcattagcaaggtgctaaagttggctccacttagtggtaaaggtgtagaaactggctgtgataatattaatgcatcatggactgacagctggacaaggattctcggtctttgtggtgaaggaaaagggatgttttgcataaaatgtgaaatgtgcttttcaatgggaagaggatgtggtccagacacagaaagtttgtagataaacataagaaatttcctaaaagcttcaaaaaaaggccagtgtgagagtaaacaaatgcatttgtttgtattgatggatttggagaccatttttctctccacaggcgtcaacaagcccaggtgcataagctgtttctctgatagaagttcccgagagtaaggttcataaaactgaatggcagctccatatacctttttggctgaagaacctgtcaagacaaaagttgaaaaaactggaagtggatatttggtttcaggatcccagcactcaatagtagctcccataggaaggcagaaaagaggtacatctgattctgagagtggaaatgactcatagtcctcttctggatatctaaaaattaaaccattccacaatttaagtttttgtcaactttgcagaaggtatgaggaggagtttctcctttactggttacaataacacagatatcagttacagccaaggaattctggggtcgaactggaggagcccttcgataagtgataaagattctttgtgaagtagttgaactattgttgacattggcacagcgaccatagggtgtggctaggatcacttcacatcctggaataagccgttctttcccttcatatagaactccaatatctgtaagcggtggtttatctctccctctcttataacagaggaaaagttctgggcttttcagacttccatagttcaagtttgcttggagagctgatggagtggcttctacacaggtgtaaccttcaggtactgtttctccagctgatttgataataatggcaatgtctgtaattggagctttaggtccagttgacttagtatctaaacgatttatttcttgatccaaaagagtagatgtgtcagtgagaccagctacgacaaagtagtctgtcactcttggtcctttgtcttctatcatggctgctactgtattttctgctgcctgctcctctgtcagcgcagccccgacacggcttcttcctggggcaagaaagcaccggattcgcggactgggcgcgctcggcagggcagggcgggggactagctccagcggccgccgccgcctcagtccggtct

SEQ ID NO: 8477 - RNA, 6717 nt, Homo sapiens
  source 1..6717: mol_type = other RNA
aaaagtaattgcggtttttgccattaatagtggcaaaaactacaattaattttgtgccaacctaatacattaaagttagggaaggcagctgtcatcagattttcaggtaattttaagattaatgactacagacaagtttagtagtagtcatttatttaatagtcaatgagacccctttcagaaaaccgtattgcaacatgcaatctattttaataaatatacacttagaatatggctgtatatacacatacctacacagccctacacatatacaaacttacacaaatatgttgctctcttttttttttttttttttttttgagacggtctcactctgtcacccaagctggagttgcagtggcgtgatctccactcactgtagcctctgcctcagttcaagcgattctcctgcctcagcctgagtagctgggactacagtggtgcgcctggctaatttttgtatttttagtaaagacagggtctcaccgtgttggccaggctggtctcgaactcctggcctcaagtgatccacccaccttgctcagcctcccaaagtgctgggattacaggcctgagccaccgtgcccggccatgttgcttttataattgagatatttcatttgttttgggggttaggcaaatttaatttgccattcctcaaactcagtaacttcaaatataaacaatgcctagaatgaatatggttcctcattatttctatcaaactactacaaatactgaagaatcccaaagtagttttccacagaggcagaaaagcagttcaggggttgaaaatcttcaatattaataagccctgggacattcaaatggcacttcatatttcaaggtaatgcaatatgaatcataattcattatatattgtccccaagagttacttcaattccgtattcaccagttcttacgatttggaaaaaaaaacttgaatgtttccagatgaaatctaatccccaagccttgtgtgtcaacattctagtgaatctctatttaaatgagaggcgctccaaaacacttcctgcaccactcgacactggcacttggtggagcatcaattttctgcaacctttcaagaatctctgaagacagactattgtatgcaattccatattcattgtcaaatgcctcaatatcaatattctctcttcctagagacactaatgataagaagaggatttctctgtataaactcctttgtcttttcatgcctggcttcatttgctgtgaaagtaggttgatgggtttaagaacattattgtgctgaatactctgcctgatggtttctactaaagtgcttgtttcttgttgttcctctgacaggagagatgatttcttttcagaattaaaattcctccatgagacatacagaggttctcttggttcctgatgaaggttgatattatcccataacagctgaatatacacaagtttgctatcctgggacagagatgacagaggaagctgtacaccttcattacaatgttcagatgtgaggataagtcctggcaagttactaggaaggtccaaacgtctgaaataccaaacgaggttccagaaaatgattggatgttgattgatgaaagaagatgtatgaatcacctgatcaccttcattttctagcaaagattcaagttctttacggagtactagaggactcaagtagggcacagaaacagggggaggattgggtctttttcctaaaggatccacaacttcctgcagactatttggaagactaactgttgagatgccatgaaacggtcgctgggtaaagtcaatattctgcaatgggcctccaacactgtgacttcgagtcaaagacacatttcgctttgataaactattaggcacagatgaaattttcatagtttggacatctccactggctctctttatttcatcacttggttcaactgcagagcctgtttcttcagttatgatctggttatgttttgggaagtccataaagttgatcaagtcaggttctgctaaactggatacaggtttgtgctccaaggattcatttgccaatggaatgcttccactttgtaaactgtcaccagaggtacttggtttcaggaaaaagcttgcagaacctctcaaatctttgaattctatattgagaagaggcaagaagttgcttttacagaatggacaagctgtattcaaatttgagtcatctgctgtccatccagccataatttcttcatcataaactaaagctccacaagctctacactgtgaacaactggacatcaaaacctccattgcacaattctgatagatgctagacatgctggtattttgagaagaaccatgatctgatttttcaaagtcttgccctttcatgcctcttggaaatggaacttcacctgttggataatgcagttttcctacatctccactactgctgctactgccaagacttgtgttgctctgggtaagttcactggggaccaaccctgagatacttgtgttaggcgatatattctcccccaaaatatggtcttctaggccagctgggaagctgtagtctctattagtttcttcctcatcatctgagtagctgtaggcagacgcaacagctacccacatcttactggctactgtcgctgcttgtttcataccagatttcaggacatctatcttgggccctgagagtatattatccagctttagccctgacaaagaatttactacagaacccaacgagccatgtggcgaagaacgcaccagtgctgacaaagaagttgaacgttctttatgagttcgagagggggtttgctgcttgaaacgcccagtaaaagttttagacctggacactgcaggtgagctcttttcactttcaggattttcctgtgctggtgaaccatgatctaaaggtaggcttgatctcctctctagagcatgaataaatgcagtagtcatgccagactctctgttttcctctctgtgtaattccatactagaagatttactacctaggggactttttaggttcatatagctttctatttcatcagccagattacgtgcaataactggagaaaacaacttatcttcagaatcaggagtttttcctcctgtacattcagtggctaaaagagacaaaggatctagtccagtttcaacatcttccctctgaaccaccttagcaataccatataaactacttctcttattcctcagatctttggatactgttttcaagtctctggactgattactgttactatcacttagtagactctcatatgtatctactgttgcagtagttttaggtacgtcatcaaccacaggctcaaggagttcttggctttcctcaagcatctctggcaccggagatgatctgtgctcaggattccaagtgctttcagacatacaagtcctactatcaggtaggtgacagctaacattctcaaagctatgggttcttgcaatatgaagtagagaagtcttaggacatgtcaatgctgctgtgagaatcttggcatctgctcccatcatgatagccatttcacttgaattcgaatccaaactactcttcttaagcaacattcctgctcgactttcagaactaaaactacaactcctctcaggaaaatgcttttgtcttttttctcctctatcaccattcttcttgagattagtagcttcgccaaagactgcatcttcaactggatcttgagtagaaaacagcacatttgatatactaccagtgctacttttcctgctgttgacatcaaatataccagacggaactttcacaatactgctgccccatgcaggaggttcagtaggactgtgaggctctggactaggttgtgaatgttttgccacaatagcagaggcatcacacacctcttctgtttgcatttttgttttagttatcaattctcttgctgcctgttcttcaggcacatgaatttctgcatcatcctttataagttcatccttagacccgtatccttggtcagactgaccacctgtgctagagtgattatcaatggactcaagcctgattaaatctctgacgaagactgtgtgctccccattgttagcatcattagaactatccacactaccgtggctcaccgtgtccccatcacttccacctgtgacattttgaagagctgatattgaggagacctgtgacctttgcacagtctttttaagcggctgcctaaactgtgccaagccacgtaccacattccgtaccttcgtccataagaaaataccactgcgggtactgctaggccacgggctctccaagactaccttattataataaccataagtaatagcattaggctttatcctagcagttttcatttcaaataagactctcactgctaaaacaggatgaccccaaagtccacaaagctgcatcactactcgatagcacacctcatctaagggatccacatctgttttcctcatcttaataagtacatcatatgcctgctgaagtgctctgactttaggatgagaaactctaacataggccggaagacaaataaaccataaactgtaacaatgactaaacagacacttggcccactgtggtggatttgtataacatctcttcgccaatttatgagctgtttttatttcctgtttagttctcttagccatgagaggtggactctttgtaatgctattcccagtagggtgtctactaaaacaaagtttcaactcctgcggtctgtcaaaaagcttaaggtccagtcttggaaagtatttgtaactgtactttggtgacaggtcctttccatcatcaggaggtggctctggcggcattataaatacagtatgctcacttttctgtgaatcatctagttctatcaatctggtatcttctgctgaatcaaaatcaaccttatctgttttctctgtgcctttatcaggaaacaacttttctatgcagtcatcaaaaaatgctaatccagtatctttatcacttacaaaactgcattcttcaatgaaacgaataaaaatctgtgttttggataaaagggtatagaattttgcataggcacgatctcgactttttaaaaatccctgtcggtcaaacaatgaatcagcagctgtggctttatttgaaggagcctctgtgattggtctgagatatgttctatatccttttaaaatagacgccataaagcgcaaaaatgcctcttgaatttccatctcaagctgtgtcatcttcttttgccaggagaaatctgcttcaattggagtcatgtcaatcgctgagccttcttgagttttttggtgaactgaagacagctggggatacaatttctttaaggtgctaagtagatttttgcacggctttttgggaagttgcttccagttcatgttcttcttttcatctgatacatataacatgttcgtatccaagtcaatgcaaacaacatcttgtggtgggtcatgaagatcaaaataccttgagtcaactccaactataaatggtaaaggtgcactaagcactgcagccagtgaaagaggacaaaggggaatatatgggcattgccactgaaatggaaagatcatagctacaacagcttcagctaccccagtcaagacagctggcctaagagaatgcagcagaattttactctcaagtaaaacaaagagcagcagtgttgcacaattctcaggacccagattcattagcaaggtgctaaagttggctccacttagtggtaaaggtgtagaaactggctgtgataatattaatgcatcatggactgacagctggacaaggattctcggtctttgtggtgaaggaaaagggatgttttgcataaaatgtgaaatgtgcttttcaatgggaagaggatgtggtccagacacagaaagtttgtagataaacataagaaatttcctaaaagcttcaaaaaaaggccagtgtgagagtaaacaaatgcatttgtttgtattgatggatttggagaccatttttctctccacaggcgtcaacaagcccaggtgcataagctgtttctctgatagaagttcccgagagtaaggttcataaaactgaatggcagctccatatacctttttggctgaagaacctgtcaagacaaaagttgaaaaaactggaagtggatatttggtttcaggatcccagcactcaatagtagctcccataggaaggcagaaaagaggtacatctgattctgagagtggaaatgactcatagtcctcttctggatatctaaaaattaaacccaatatctgtaagcggtggtttatctctccctctcttataacagaggaaaagttctgggcttttcagacttccatagttcaagtttgcttggagagctgatggagtggcttctacacaggtgtaaccttcaggtactgtttctccagctgatttgataataatggcaatgtctgtaattggagctttaggtccagttgacttagtatctaaacgatttatttcttgatccaaaagagtagatgtgtcagtgagaccagctacgacaaagtagtctgtcactcttggtcctttgtcttctatcatggctgctactgtattttctgctgcctgctcctctgtcagcgcagccccgacacggcttcttcctggggcaagaaagcaccggattcgcggactgggcgcgctcggcagggcagggcgggggactagctccagcggccgccgccgcctcagtccggtct

SEQ ID NO: 8478 - RNA, 7103 nt, Homo sapiens
  source 1..7103: mol_type = other RNA
aaaagtaattgcggtttttgccattaatagtggcaaaaactacaattaattttgtgccaacctaatacattaaagttagggaaggcagctgtcatcagattttcaggtaattttaagattaatgactacagacaagtttagtagtagtcatttatttaatagtcaatgagacccctttcagaaaaccgtattgcaacatgcaatctattttaataaatatacacttagaatatggctgtatatacacatacctacacagccctacacatatacaaacttacacaaatatgttgctctcttttttttttttttttttttttgagacggtctcactctgtcacccaagctggagttgcagtggcgtgatctccactcactgtagcctctgcctcagttcaagcgattctcctgcctcagcctgagtagctgggactacagtggtgcgcctggctaatttttgtatttttagtaaagacagggtctcaccgtgttggccaggctggtctcgaactcctggcctcaagtgatccacccaccttgctcagcctcccaaagtgctgggattacaggcctgagccaccgtgcccggccatgttgcttttataattgagatatttcatttgttttgggggttaggcaaatttaatttgccattcctcaaactcagtaacttcaaatataaacaatgcctagaatgaatatggttcctcattatttctatcaaactactacaaatactgaagaatcccaaagtagttttccacagaggcagaaaagcagttcaggggttgaaaatcttcaatattaataagccctgggacattcaaatggcacttcatatttcaaggtaatgcaatatgaatcataattcattatatattgtccccaagagttacttcaattccgtattcaccagttcttacgatttggaaaaaaaaacttgaatgtttccagatgaaatctaatccccaagccttgtgtgtcaacattctagtgaatctctatttaaatgagaggcgctccaaaacacttcctgcaccactcgacactggcacttggtggagcatcaattttctgcaacctttcaagaatctctgaagacagactattgtatgcaattccatattcattgtcaaatgcctcaatatcaatattctctcttcctagagacactaatgataagaagaggatttctctgtataaactcctttgtcttttcatgcctggcttcatttgctgtgaaagtaggttgatgggtttaagaacattattgtgctgaatactctgcctgatggtttctactaaagtgcttgtttcttgttgttcctctgacaggagagatgatttcttttcagaattaaaattcctccatgagacatacagaggttctcttggttcctgatgaaggttgatattatcccataacagctgaatatacacaagtttgctatcctgggacagagatgacagaggaagctgtacaccttcattacaatgttcagatgtgaggataagtcctggcaagttactaggaaggtccaaacgtctgaaataccaaacgaggttccagaaaatgattggatgttgattgatgaaagaagatgtatgaatcacctgatcaccttcattttctagcaaagattcaagttctttacggagtactagaggactcaagtagggcacagaaacagggggaggattgggtctttttcctaaaggatccacaacttcctgcagactatttggaagactaactgttgagatgccatgaaacggtcgctgggtaaagtcaatattctgcaatgggcctccaacactgtgacttcgagtcaaagacacatttcgctttgataaactattaggcacagatgaaattttcatagtttggacatctccactggctctctttatttcatcacttggttcaactgcagagcctgtttcttcagttatgatctggttatgttttgggaagtccataaagttgatcaagtcaggttctgctaaactggatacaggtttgtgctccaaggattcatttgccaatggaatgcttccactttgtaaactgtcaccagaggtacttggtttcaggaaaaagcttgcagaacctctcaaatctttgaattctatattgagaagaggcaagaagttgcttttacagaatggacaagctgtattcaaatttgagtcatctgctgtccatccagccataatttcttcatcataaactaaagctccacaagctctacactgtgaacaactggacatcaaaacctccattgcacaattctgatagatgctagacatgctggtattttgagaagaaccatgatctgatttttcaaagtcttgccctttcatgcctcttggaaatggaacttcacctgttggataatgcagttttcctacatctccactactgctgctactgccaagacttgtgttgctctgggtaagttcactggggaccaaccctgagatacttgtgttaggcgatatattctcccccaaaatatggtcttctaggccagctgggaagctgtagtctctattagtttcttcctcatcatctgagtagctgtaggcagacgcaacagctacccacatcttactggctactgtcgctgcttgtttcataccagatttcaggacatctatcttgggccctgagagtatattatccagctttagccctgacaaagaatttactacagaacccaacgagccatgtggcgaagaacgcaccagtgctgacaaagaagttgaacgttctttatgagttcgagagggggtttgctgcttgaaacgcccagtaaaagttttagacctggacactgcaggtgagctcttttcactttcaggattttcctgtgctggtgaaccatgatctaaaggtaggcttgatctcctctctagagcatgaataaatgcagtagtcatgccagactctctgttttcctctctgtgtaattccatactagaagatttactacctaggggactttttaggttcatatagctttctatttcatcagccagattacgtgcaataactggagaaaacaacttatcttcagaatcaggagtttttcctcctgtacattcagtggctaaaagagacaaaggatctagtccagtttcaacatcttccctctgaaccaccttagcaataccatataaactacttctcttattcctcagatctttggatactgttttcaagtctctggactgattactgttactatcacttagtagactctcatatgtatctactgttgcagtagttttaggtacgtcatcaaccacaggctcaaggagttcttggctttcctcaagcatctctggcaccggagatgatctgtgctcaggattccaagtgctttcagacatacaagtcctactatcaggtaggtgacagctaacattctcaaagctatgggttcttgcaatatgaagtagagaagtcttaggacatgtcaatgctgctgtgagaatcttggcatctgctcccatcatgatagccatttcacttgaattcgaatccaaactactcttcttaagcaacattcctgctcgactttcagaactaaaactacaactcctctcaggaaaatgcttttgtcttttttctcctctatcaccattcttcttgagattagtagcttcgccaaagactgcatcttcaactggatcttgagtagaaaacagcacatttgatatactaccagtgctacttttcctgctgttgacatcaaatataccagacggaactttcacaatactgctgccccatgcaggaggttcagtaggactgtgaggctctggactaggttgtgaatgttttgccacaatagcagaggcatcacacacctcttctgtttgcatttttgttttagttatcaattctcttgctgcctgttcttcaggcacatgaatttctgcatcatcctttataagttcatccttagacccgtatccttggtcagactgaccacctgtgctagagtgattatcaatggactcaagcctgattaaatctctgacgaagactgtgtgctccccattgttagcatcattagaactatccacactaccgtggctcaccgtgtccccatcacttccacctgtgacattttgaagagctgatattgaggagacctgtgacctttgcacagtctttttaagcggctgcctaaactgtgccaagccacgtaccacattccgtaccttcgtccataagaaaataccactgcgggtactgctaggccacgggctctccaagactaccttattataataaccataagtaatagcattaggctttatcctagcagttttcatttcaaataagactctcactgctaaaacaggatgaccccaaagtccacaaagctgcatcactactcgatagcacacctcatctaagggatccacatctgttttcctcatcttaataagtacatcatatgcctgctgaagtgctctgactttaggatgagaaactctaacataggccggaagacaaataaaccataaactgtaacaatgactaaacagacacttggcccactgtggtggatttgtataacatctcttcgccaatttatgagctgtttttatttcctgtttagttctcttagccatgagaggtggactctttgtaatgctattcccagtagggtgtctactaaaacaaagtttcaactcctgcggtctgtcaaaaagcttaaggtccagtcttggaaagtatttgtaactgtactttggtgacaggtcctttccatcatcaggaggtggctctggcggcattataaatacagtatgctcacttttctgtgaatcatctagttctatcaatctggtatcttctgctgaatcaaaatcaaccttatctgttttctctgtgcctttatcaggaaacaacttttctatgcagtcatcaaaaaatgctaatccagtatctttatcacttacaaaactgcattcttcaatgaaacgaataaaaatctgtgttttggataaaagggtatagaattttgcataggcacgatctcgactttttaaaaatccctgtcggtcaaacaatgaatcagcagctgtggctttatttgaaggagcctctgtgattggtctgagatatgttctatatccttttaaaatagacgccataaagcgcaaaaatgcctcttgaatttccatctcaagctgtgtcatcttcttttgccaggagaaatctgcttcaattggagtcatgtcaatcgctgagccttcttgagttttttggtgaactgaagacagctggggatacaatttctttaaggtgctaagtagatttttgcacggctttttgggaagttgcttccagttcatgttcttcttttcatctgatacatataacatgttcgtatccaagtcaatgcaaacaacatcttgtggtgggtcatgaagatcaaaataccttgagtcaactccaactataaatggtaaaggtgcactaagcactgcagccagtgaaagaggacaaaggggaatatatgggcattgccactgaaatggaaagatcatagctacaacagcttcagctaccccagtcaagacagctggcctaagagaatgcagcagaattttactctcaagtaaaacaaagagcagcagtgttgcacaattctcaggacccagattcattagcaaggtgctaaagttggctccacttagtggtaaaggtgtagaaactggctgtgataatattaatgcatcatggactgacagctggacaaggattctcggtctttgtggtgaaggaaaagggatgttttgcataaaatgtgaaatgtgcttttcaatgggaagaggatgtggtccagacacagaaagtttgtagataaacataagaaatttcctaaaagcttcaaaaaaaggccagtgtgagagtaaacaaatgcatttgtttgtattgatggatttggagaccatttttctctccacaggcgtcaacaagcccaggtgcataagctgtttctctgatagaagttcccgagagtaaggttcataaaactgaatggcagctccatatacctttttggctgaagaacctgtcaagacaaaagttgaaaaaactggaagtggatatttggtttcaggatcccagcactcaatagtagctcccataggaaggcagaaaagaggtacatctgattctgagagtggaaatgactcatagtcctcttctggatatctaaaaattaaacctgtattttcagtttttatcccaccataccagtggaatgaagacgtgacacttaaatctttacagcccttgacactttaatgtgcagtaagaatgtggcgatagatttctcaaacacttcatggcagaaaagtttctcaggccctcctctcctccatatagctgattcagccttatatgctattgcatttgaagcaggtacagacttcttataacacagaaacacgctggaaccccacattccacaatttaagtttttgtcaactttgcagaaggtatgaggaggagtttctcctttactggttacaataacacagatatcagttacagccaaggaattctggggtcgaactggaggagcccttcgataagtgataaagattctttgtgaagtagttgaactattgttgacattggcacagcgaccatagggtgtggctaggatcacttcacatcctggaataagccgttctttcccttcatatagaactccaatatctgtaagcggtggtttatctctccctctcttataacagaggaaaagttctgggcttttcagacttccatagttcaagtttgcttggagagctgatggagtggcttctacacaggtgtaaccttcaggtactgtttctccagctgatttgataataatggcaatgtctgtaattggagctttaggtccagttgacttagtatctaaacgatttatttcttgatccaaaagagtagatgtgtcagtgagaccagctacgacaaagtagtctgtcactcttggtcctttgtcttctatcatggctgctactgtattttctgctgcctgctcctctgtcagcgcagccccgacacg

SEQ ID NO: 8479 - RNA, 7240 nt, Homo sapiens
  source 1..7240: mol_type = other RNA
aaaagtaattgcggtttttgccattaatagtggcaaaaactacaattaattttgtgccaacctaatacattaaagttagggaaggcagctgtcatcagattttcaggtaattttaagattaatgactacagacaagtttagtagtagtcatttatttaatagtcaatgagacccctttcagaaaaccgtattgcaacatgcaatctattttaataaatatacacttagaatatggctgtatatacacatacctacacagccctacacatatacaaacttacacaaatatgttgctctcttttttttttttttttttttttgagacggtctcactctgtcacccaagctggagttgcagtggcgtgatctccactcactgtagcctctgcctcagttcaagcgattctcctgcctcagcctgagtagctgggactacagtggtgcgcctggctaatttttgtatttttagtaaagacagggtctcaccgtgttggccaggctggtctcgaactcctggcctcaagtgatccacccaccttgctcagcctcccaaagtgctgggattacaggcctgagccaccgtgcccggccatgttgcttttataattgagatatttcatttgttttgggggttaggcaaatttaatttgccattcctcaaactcagtaacttcaaatataaacaatgcctagaatgaatatggttcctcattatttctatcaaactactacaaatactgaagaatcccaaagtagttttccacagaggcagaaaagcagttcaggggttgaaaatcttcaatattaataagccctgggacattcaaatggcacttcatatttcaaggtaatgcaatatgaatcataattcattatatattgtccccaagagttacttcaattccgtattcaccagttcttacgatttggaaaaaaaaacttgaatgtttccagatgaaatctaatccccaagccttgtgtgtcaacattctagtgaatctctatttaaatgagaggcgctccaaaacacttcctgcaccactcgacactggcacttggtggagcatcaattttctgcaacctttcaagaatctctgaagacagactattgtatgcaattccatattcattgtcaaatgcctcaatatcaatattctctcttcctagagacactaatgataagaagaggatttctctgtataaactcctttgtcttttcatgcctggcttcatttgctgtgaaagtaggttgatgggtttaagaacattattgtgctgaatactctgcctgatggtttctactaaagtgcttgtttcttgttgttcctctgacaggagagatgatttcttttcagaattaaaattcctccatgagacatacagaggttctcttggttcctgatgaaggttgatattatcccataacagctgaatatacacaagtttgctatcctgggacagagatgacagaggaagctgtacaccttcattacaatgttcagatgtgaggataagtcctggcaagttactaggaaggtccaaacgtctgaaataccaaacgaggttccagaaaatgattggatgttgattgatgaaagaagatgtatgaatcacctgatcaccttcattttctagcaaagattcaagttctttacggagtactagaggactcaagtagggcacagaaacagggggaggattgggtctttttcctaaaggatccacaacttcctgcagactatttggaagactaactgttgagatgccatgaaacggtcgctgggtaaagtcaatattctgcaatgggcctccaacactgtgacttcgagtcaaagacacatttcgctttgataaactattaggcacagatgaaattttcatagtttggacatctccactggctctctttatttcatcacttggttcaactgcagagcctgtttcttcagttatgatctggttatgttttgggaagtccataaagttgatcaagtcaggttctgctaaactggatacaggtttgtgctccaaggattcatttgccaatggaatgcttccactttgtaaactgtcaccagaggtacttggtttcaggaaaaagcttgcagaacctctcaaatctttgaattctatattgagaagaggcaagaagttgcttttacagaatggacaagctgtattcaaatttgagtcatctgctgtccatccagccataatttcttcatcataaactaaagctccacaagctctacactgtgaacaactggacatcaaaacctccattgcacaattctgatagatgctagacatgctggtattttgagaagaaccatgatctgatttttcaaagtcttgccctttcatgcctcttggaaatggaacttcacctgttggataatgcagttttcctacatctccactactgctgctactgccaagacttgtgttgctctgggtaagttcactggggaccaaccctgagatacttgtgttaggcgatatattctcccccaaaatatggtcttctaggccagctgggaagctgtagtctctattagtttcttcctcatcatctgagtagctgtaggcagacgcaacagctacccacatcttactggctactgtcgctgcttgtttcataccagatttcaggacatctatcttgggccctgagagtatattatccagctttagccctgacaaagaatttactacagaacccaacgagccatgtggcgaagaacgcaccagtgctgacaaagaagttgaacgttctttatgagttcgagagggggtttgctgcttgaaacgcccagtaaaagttttagacctggacactgcaggtgagctcttttcactttcaggattttcctgtgctggtgaaccatgatctaaaggtaggcttgatctcctctctagagcatgaataaatgcagtagtcatgccagactctctgttttcctctctgtgtaattccatactagaagatttactacctaggggactttttaggttcatatagctttctatttcatcagccagattacgtgcaataactggagaaaacaacttatcttcagaatcaggagtttttcctcctgtacattcagtggctaaaagagacaaaggatctagtccagtttcaacatcttccctctgaaccaccttagcaataccatataaactacttctcttattcctcagatctttggatactgttttcaagtctctggactgattactgttactatcacttagtagactctcatatgtatctactgttgcagtagttttaggtacgtcatcaaccacaggctcaaggagttcttggctttcctcaagcatctctggcaccggagatgatctgtgctcaggattccaagtgctttcagacatacaagtcctactatcaggtaggtgacagctaacattctcaaagctatgggttcttgcaatatgaagtagagaagtcttaggacatgtcaatgctgctgtgagaatcttggcatctgctcccatcatgatagccatttcacttgaattcgaatccaaactactcttcttaagcaacattcctgctcgactttcagaactaaaactacaactcctctcaggaaaatgcttttgtcttttttctcctctatcaccattcttcttgagattagtagcttcgccaaagactgcatcttcaactggatcttgagtagaaaacagcacatttgatatactaccagtgctacttttcctgctgttgacatcaaatataccagacggaactttcacaatactgctgccccatgcaggaggttcagtaggactgtgaggctctggactaggttgtgaatgttttgccacaatagcagaggcatcacacacctcttctgtttgcatttttgttttagttatcaattctcttgctgcctgttcttcaggcacatgaatttctgcatcatcctttataagttcatccttagacccgtatccttggtcagactgaccacctgtgctagagtgattatcaatggactcaagcctgattaaatctctgacgaagactgtgtgctccccattgttagcatcattagaactatccacactaccgtggctcaccgtgtccccatcacttccacctgtgacattttgaagagctgatattgaggagacctgtgacctttgcacagtctttttaagcggctgcctaaactgtgccaagccacgtaccacattccgtaccttcgtccataagaaaataccactgcgggtactgctaggccacgggctctccaagactaccttattataataaccataagtaatagcattaggctttatcctagcagttttcatttcaaataagactctcactgctaaaacaggatgaccccaaagtccacaaagctgcatcactactcgatagcacacctcatctaagggatccacatctgttttcctcatcttaataagtacatcatatgcctgctgaagtgctctgactttaggatgagaaactctaacataggccggaagacaaataaaccataaactgtaacaatgactaaacagacacttggcccactgtggtggatttgtataacatctcttcgccaatttatgagctgtttttatttcctgtttagttctcttagccatgagaggtggactctttgtaatgctattcccagtagggtgtctactaaaacaaagtttcaactcctgcggtctgtcaaaaagcttaaggtccagtcttggaaagtatttgtaactgtactttggtgacaggtcctttccatcatcaggaggtggctctggcggcattataaatacagtatgctcacttttctgtgaatcatctagttctatcaatctggtatcttctgctgaatcaaaatcaaccttatctgttttctctgtgcctttatcaggaaacaacttttctatgcagtcatcaaaaaatgctaatccagtatctttatcacttacaaaactgcattcttcaatgaaacgaataaaaatctgtgttttggataaaagggtatagaattttgcataggcacgatctcgactttttaaaaatccctgtcggtcaaacaatgaatcagcagctgtggctttatttgaaggagcctctgtgattggtctgagatatgttctatatccttttaaaatagacgccataaagcgcaaaaatgcctcttgaatttccatctcaagctgtgtcatcttcttttgccaggagaaatctgcttcaattggagtcatgtcaatcgctgagccttcttgagttttttggtgaactgaagacagctggggatacaatttctttaaggtgctaagtagatttttgcacggctttttgggaagttgcttccagttcatgttcttcttttcatctgatacatataacatgttcgtatccaagtcaatgcaaacaacatcttgtggtgggtcatgaagatcaaaataccttgagtcaactccaactataaatggtaaaggtgcactaagcactgcagccagtgaaagaggacaaaggggaatatatgggcattgccactgaaatggaaagatcatagctacaacagcttcagctaccccagtcaagacagctggcctaagagaatgcagcagaattttactctcaagtaaaacaaagagcagcagtgttgcacaattctcaggacccagattcattagcaaggtgctaaagttggctccacttagtggtaaaggtgtagaaactggctgtgataatattaatgcatcatggactgacagctggacaaggattctcggtctttgtggtgaaggaaaagggatgttttgcataaaatgtgaaatgtgcttttcaatgggaagaggatgtggtccagacacagaaagtttgtagataaacataagaaatttcctaaaagcttcaaaaaaaggccagtgtgagagtaaacaaatgcatttgtttgtattgatggatttggagaccatttttctctccacaggcgtcaacaagcccaggtgcataagctgtttctctgatagaagttcccgagagtaaggttcataaaactgaatggcagctccatatacctttttggctgaagaacctgtcaagacaaaagttgaaaaaactggaagtggatatttggtttcaggatcccagcactcaatagtagctcccataggaaggcagaaaagaggtacatctgattctgagagtggaaatgactcatagtcctcttctggatatctaaaaattaaacctgtattttcagtttttatcccaccataccagtggaatgaagacgtgacacttaaatctttacagcccttgacactttaatgtgcagtaagaatgtggcgatagatttctcaaacacttcatggcagaaaagtttctcaggccctcctctcctccatatagctgattctttgcaacaaaggagaaaggaagcaagtccaccagccttatatgctattgcatttgaagcaggtacagacttcttataacacagaaacacgctggaaccccacattccacaatttaagtttttgtcaactttgcagaaggtatgaggaggagtttctcctttactggttacaataacacagatatcagttacagccaaggaattctggggtcgaactggaggagcccttcgataagtgataaagattctttgtgaagtagttgaactattgttgacattggcacagcgaccatagggtgtggctaggatcacttcacatcctggaataagccgttctttcccttcatatagaactccaatatctgtaagcggtggtttatctctccctctcttataacagaggaaaagttctgggcttttcagacttccatagttcaagtttgcttggagagctgatggagtggcttctacacaggtgtaaccttcaggtactgtttctccagctgatttgataataatggcaatgtctgtaattggagctttaggtccagttgacttagtatctaaacgatttatttcttgatccaaaagagtagatgtgtcagtgagaccagctacgacaaagtagtctgtcactcttggtcctttgtcttctatcatggctgctactgtattttctgctgcctgctcctctgtcagcgcagccccgacacggcttcttcctggggcaagaaagcaccggattcgcggactgggcgcgctcggcagggcagggcgggggactagctccagcggccgccgccgcctcagtccggtct

SEQ ID NO: 8480 - RNA, 6625 nt, Homo sapiens
  source 1..6625: mol_type = other RNA
aaaagtaattgcggtttttgccattaatagtggcaaaaactacaattaattttgtgccaacctaatacattaaagttagggaaggcagctgtcatcagattttcaggtaattttaagattaatgactacagacaagtttagtagtagtcatttatttaatagtcaatgagacccctttcagaaaaccgtattgcaacatgcaatctattttaataaatatacacttagaatatggctgtatatacacatacctacacagccctacacatatacaaacttacacaaatatgttgctctcttttttttttttttttttttttgagacggtctcactctgtcacccaagctggagttgcagtggcgtgatctccactcactgtagcctctgcctcagttcaagcgattctcctgcctcagcctgagtagctgggactacagtggtgcgcctggctaatttttgtatttttagtaaagacagggtctcaccgtgttggccaggctggtctcgaactcctggcctcaagtgatccacccaccttgctcagcctcccaaagtgctgggattacaggcctgagccaccgtgcccggccatgttgcttttataattgagatatttcatttgttttgggggttaggcaaatttaatttgccattcctcaaactcagtaacttcaaatataaacaatgcctagaatgaatatggttcctcattatttctatcaaactactacaaatactgaagaatcccaaagtagttttccacagaggcagaaaagcagttcaggggttgaaaatcttcaatattaataagccctgggacattcaaatggcacttcatatttcaaggtaatgcaatatgaatcataattcattatatattgtccccaagagttacttcaattccgtattcaccagttcttacgatttggaaaaaaaaacttgaatgtttccagatgaaatctaatccccaagccttgtgtgtcaacattctagtgaatctctatttaaatgagaggcgctccaaaacacttcctgcaccactcgacactggcacttggtggagcatcaattttctgcaacctttcaagaatctctgaagacagactattgtatgcaattccatattcattgtcaaatgcctcaatatcaatattctctcttcctagagacactaatgataagaagaggatttctctgtataaactcctttgtcttttcatgcctggcttcatttgctgtgaaagtaggttgatgggtttaagaacattattgtgctgaatactctgcctgatggtttctactaaagtgcttgtttcttgttgttcctctgacaggagagatgatttcttttcagaattaaaattcctccatgagacatacagaggttctcttggttcctgatgaaggttgatattatcccataacagctgaatatacacaagtttgctatcctgggacagagatgacagaggaagctgtacaccttcattacaatgttcagatgtgaggataagtcctggcaagttactaggaaggtccaaacgtctgaaataccaaacgaggttccagaaaatgattggatgttgattgatgaaagaagatgtatgaatcacctgatcaccttcattttctagcaaagattcaagttctttacggagtactagaggactcaagtagggcacagaaacagggggaggattgggtctttttcctaaaggatccacaacttcctgcagactatttggaagactaactgttgagatgccatgaaacggtcgctgggtaaagtcaatattctgcaatgggcctccaacactgtgacttcgagtcaaagacacatttcgctttgataaactattaggcacagatgaaattttcatagtttggacatctccactggctctctttatttcatcacttggttcaactgcagagcctgtttcttcagttatgatctggttatgttttgggaagtccataaagttgatcaagtcaggttctgctaaactggatacaggtttgtgctccaaggattcatttgccaatggaatgcttccactttgtaaactgtcaccagaggtacttggtttcaggaaaaagcttgcagaacctctcaaatctttgaattctatattgagaagaggcaagaagttgcttttacagaatggacaagctgtattcaaatttgagtcatctgctgtccatccagccataatttcttcatcataaactaaagctccacaagctctacactgtgaacaactggacatcaaaacctccattgcacaattctgatagatgctagacatgctggtattttgagaagaaccatgatctgatttttcaaagtcttgccctttcatgcctcttggaaatggaacttcacctgttggataatgcagttttcctacatctccactactgctgctactgccaagacttgtgttgctctgggtaagttcactggggaccaaccctgagatacttgtgttaggcgatatattctcccccaaaatatggtcttctaggccagctgggaagctgtagtctctattagtttcttcctcatcatctgagtagctgtaggcagacgcaacagctacccacatcttactggctactgtcgctgcttgtttcataccagatttcaggacatctatcttgggccctgagagtatattatccagctttagccctgacaaagaatttactacagaacccaacgagccatgtggcgaagaacgcaccagtgctgacaaagaagttgaacgttctttatgagttcgagagggggtttgctgcttgaaacgcccagtaaaagttttagacctggacactgcaggtgagctcttttcactttcaggattttcctgtgctggtgaaccatgatctaaaggtaggcttgatctcctctctagagcatgaataaatgcagtagtcatgccagactctctgttttcctctctgtgtaattccatactagaagatttactacctaggggactttttaggttcatatagctttctatttcatcagccagattacgtgcaataactggagaaaacaacttatcttcagaatcaggagtttttcctcctgtacattcagtggctaaaagagacaaaggatctagtccagtttcaacatcttccctctgaaccaccttagcaataccatataaactacttctcttattcctcagatctttggatactgttttcaagtctctggactgattactgttactatcacttagtagactctcatatgtatctactgttgcagtagttttaggtacgtcatcaaccacaggctcaaggagttcttggctttcctcaagcatctctggcaccggagatgatctgtgctcaggattccaagtgctttcagacatacaagtcctactatcaggtaggtgacagctaacattctcaaagctatgggttcttgcaatatgaagtagagaagtcttaggacatgtcaatgctgctgtgagaatcttggcatctgctcccatcatgatagccatttcacttgaattcgaatccaaactactcttcttaagcaacattcctgctcgactttcagaactaaaactacaactcctctcaggaaaatgcttttgtcttttttctcctctatcaccattcttcttgagattagtagcttcgccaaagactgcatcttcaactggatcttgagtagaaaacagcacatttgatatactaccagtgctacttttcctgctgttgacatcaaatataccagacggaactttcacaatactgctgccccatgcaggaggttcagtaggactgtgaggctctggactaggttgtgaatgttttgccacaatagcagaggcatcacacacctcttctgtttgcatttttgttttagttatcaattctcttgctgcctgttcttcaggcacatgaatttctgcatcatcctttataagttcatccttagacccgtatccttggtcagactgaccacctgtgctagagtgattatcaatggactcaagcctgattaaatctctgacgaagactgtgtgctccccattgttagcatcattagaactatccacactaccgtggctcaccgtgtccccatcacttccacctgtgacattttgaagagctgatattgaggagacctgtgacctttgcacagtctttttaagcggctgcctaaactgtgccaagccacgtaccacattccgtaccttcgtccataagaaaataccactgcgggtactgctaggccacgggctctccaagactaccttattataataaccataagtaatagcattaggctttatcctagcagttttcatttcaaataagactctcactgctaaaacaggatgaccccaaagtccacaaagctgcatcactactcgatagcacacctcatctaagggatccacatctgttttcctcatcttaataagtacatcatatgcctgctgaagtgctctgactttaggatgagaaactctaacataggccggaagacaaataaaccataaactgtaacaatgactaaacagacacttggcccactgtggtggatttgtataacatctcttcgccaatttatgagctgtttttatttcctgtttagttctcttagccatgagaggtggactctttgtaatgctattcccagtagggtgtctactaaaacaaagtttcaactcctgcggtctgtcaaaaagcttaaggtccagtcttggaaagtatttgtaactgtactttggtgacaggtcctttccatcatcaggaggtggctctggcggcattataaatacagtatgctcacttttctgtgaatcatctagttctatcaatctggtatcttctgctgaatcaaaatcaaccttatctgttttctctgtgcctttatcaggaaacaacttttctatgcagtcatcaaaaaatgctaatccagtatctttatcacttacaaaactgcattcttcaatgaaacgaataaaaatctgtgttttggataaaagggtatagaattttgcataggcacgatctcgactttttaaaaatccctgtcggtcaaacaatgaatcagcagctgtggctttatttgaaggagcctctgtgattggtctgagatatgttctatatccttttaaaatagacgccataaagcgcaaaaatgcctcttgaatttccatctcaagctgtgtcatcttcttttgccaggagaaatctgcttcaattggagtcatgtcaatcgctgagccttcttgagttttttggtgaactgaagacagctggggatacaatttctttaaggtgctaagtagatttttgcacggctttttgggaagttgcttccagttcatgttcttcttttcatctgatagctacaacagcttcagctaccccagtcaagacagctggcctaagagaatgcagcagaattttactctcaagtaaaacaaagagcagcagtgttgcacaattctcaggacccagattcattagcaaggtgctaaagttggctccacttagtggtaaaggtgtagaaactggctgtgataatattaatgcatcatggactgacagctggacaaggattctcggtctttgtggtgaaggaaaagggatgttttgcataaaatgtgaaatgtgcctttttggctgaagaacctgtcaagacaaaagttgaaaaaactggaagtggatatttggtttcaggatcccagcactcaatagtagctcccataggaaggcagaaaagaggtacatctgattctgagagtggaaatgactcatagtcctcttctggatatctaaaaattaaaccagccttatatgctattgcatttgaagcaggtacagacttcttataacacagaaacacgctggaaccccacattccacaatttaagtttttgtcaactttgcagaaggtatgaggaggagtttctcctttactggttacaataacacagatatcagttacagccaaggaattctggggtcgaactggaggagcccttcgataagtgataaagattctttgtgaagtagttgaactattgttgacattggcacagcgaccatagggtgtggctaggatcacttcacatcctggaataagccgttctttcccttcatatagaactccaatatctgtaagcggtggtttatctctccctctcttataacagaggaaaagttctgggcttttcagacttccatagttcaagtttgcttggagagctgatggagtggcttctacacaggtgtaaccttcaggtactgtttctccagctgatttgataataatggcaatgtctgtaattggagctttaggtccagttgacttagtatctaaacgatttatttcttgatccaaaagagtagatgtgtcagtgagaccagctacgacaaagtagtctgtcactcttggtcctttgtcttctatcatggctgctactgtattttctgctgcctgctcctctgtcagcgcagccccgacacggcttcttcctggggcaagaaagcaccggattcgcggactgggcgcgctcggcagggcagggcgggggactagctccagcggccgccgccgcctcagtccggtct

SEQ ID NO: 8481 - RNA, 6864 nt, Homo sapiens
  source 1..6864: mol_type = other RNA
aaaagtaattgcggtttttgccattaatagtggcaaaaactacaattaattttgtgccaacctaatacattaaagttagggaaggcagctgtcatcagattttcaggtaattttaagattaatgactacagacaagtttagtagtagtcatttatttaatagtcaatgagacccctttcagaaaaccgtattgcaacatgcaatctattttaataaatatacacttagaatatggctgtatatacacatacctacacagccctacacatatacaaacttacacaaatatgttgctctcttttttttttttttttttttttgagacggtctcactctgtcacccaagctggagttgcagtggcgtgatctccactcactgtagcctctgcctcagttcaagcgattctcctgcctcagcctgagtagctgggactacagtggtgcgcctggctaatttttgtatttttagtaaagacagggtctcaccgtgttggccaggctggtctcgaactcctggcctcaagtgatccacccaccttgctcagcctcccaaagtgctgggattacaggcctgagccaccgtgcccggccatgttgcttttataattgagatatttcatttgttttgggggttaggcaaatttaatttgccattcctcaaactcagtaacttcaaatataaacaatgcctagaatgaatatggttcctcattatttctatcaaactactacaaatactgaagaatcccaaagtagttttccacagaggcagaaaagcagttcaggggttgaaaatcttcaatattaataagccctgggacattcaaatggcacttcatatttcaaggtaatgcaatatgaatcataattcattatatattgtccccaagagttacttcaattccgtattcaccagttcttacgatttggaaaaaaaaacttgaatgtttccagatgaaatctaatccccaagccttgtgtgtcaacattctagtgaatctctatttaaatgagaggcgctccaaaacacttcctgcaccactcgacactggcacttggtggagcatcaattttctgcaacctttcaagaatctctgaagacagactattgtatgcaattccatattcattgtcaaatgcctcaatatcaatattctctcttcctagagacactaatgataagaagaggatttctctgtataaactcctttgtcttttcatgcctggcttcatttgctgtgaaagtaggttgatgggtttaagaacattattgtgctgaatactctgcctgatggtttctactaaagtgcttgtttcttgttgttcctctgacaggagagatgatttcttttcagaattaaaattcctccatgagacatacagaggttctcttggttcctgatgaaggttgatattatcccataacagctgaatatacacaagtttgctatcctgggacagagatgacagaggaagctgtacaccttcattacaatgttcagatgtgaggataagtcctggcaagttactaggaaggtccaaacgtctgaaataccaaacgaggttccagaaaatgattggatgttgattgatgaaagaagatgtatgaatcacctgatcaccttcattttctagcaaagattcaagttctttacggagtactagaggactcaagtagggcacagaaacagggggaggattgggtctttttcctaaaggatccacaacttcctgcagactatttggaagactaactgttgagatgccatgaaacggtcgctgggtaaagtcaatattctgcaatgggcctccaacactgtgacttcgagtcaaagacacatttcgctttgataaactattaggcacagatgaaattttcatagtttggacatctccactggctctctttatttcatcacttggttcaactgcagagcctgtttcttcagttatgatctggttatgttttgggaagtccataaagttgatcaagtcaggttctgctaaactggatacaggtttgtgctccaaggattcatttgccaatggaatgcttccactttgtaaactgtcaccagaggtacttggtttcaggaaaaagcttgcagaacctctcaaatctttgaattctatattgagaagaggcaagaagttgcttttacagaatggacaagctgtattcaaatttgagtcatctgctgtccatccagccataatttcttcatcataaactaaagctccacaagctctacactgtgaacaactggacatcaaaacctccattgcacaattctgatagatgctagacatgctggtattttgagaagaaccatgatctgatttttcaaagtcttgccctttcatgcctcttggaaatggaacttcacctgttggataatgcagttttcctacatctccactactgctgctactgccaagacttgtgttgctctgggtaagttcactggggaccaaccctgagatacttgtgttaggcgatatattctcccccaaaatatggtcttctaggccagctgggaagctgtagtctctattagtttcttcctcatcatctgagtagctgtaggcagacgcaacagctacccacatcttactggctactgtcgctgcttgtttcataccagatttcaggacatctatcttgggccctgagagtatattatccagctttagccctgacaaagaatttactacagaacccaacgagccatgtggcgaagaacgcaccagtgctgacaaagaagttgaacgttctttatgagttcgagagggggtttgctgcttgaaacgcccagtaaaagttttagacctggacactgcaggtgagctcttttcactttcaggattttcctgtgctggtgaaccatgatctaaaggtaggcttgatctcctctctagagcatgaataaatgcagtagtcatgccagactctctgttttcctctctgtgtaattccatactagaagatttactacctaggggactttttaggttcatatagctttctatttcatcagccagattacgtgcaataactggagaaaacaacttatcttcagaatcaggagtttttcctcctgtacattcagtggctaaaagagacaaaggatctagtccagtttcaacatcttccctctgaaccaccttagcaataccatataaactacttctcttattcctcagatctttggatactgttttcaagtctctggactgattactgttactatcacttagtagactctcatatgtatctactgttgcagtagttttaggtacgtcatcaaccacaggctcaaggagttcttggctttcctcaagcatctctggcaccggagatgatctgtgctcaggattccaagtgctttcagacatacaagtcctactatcaggtaggtgacagctaacattctcaaagctatgggttcttgcaatatgaagtagagaagtcttaggacatgtcaatgctgctgtgagaatcttggcatctgctcccatcatgatagccatttcacttgaattcgaatccaaactactcttcttaagcaacattcctgctcgactttcagaactaaaactacaactcctctcaggaaaatgcttttgtcttttttctcctctatcaccattcttcttgagattagtagcttcgccaaagactgcatcttcaactggatcttgagtagaaaacagcacatttgatatactaccagtgctacttttcctgctgttgacatcaaatataccagacggaactttcacaatactgctgccccatgcaggaggttcagtaggactgtgaggctctggactaggttgtgaatgttttgccacaatagcagaggcatcacacacctcttctgtttgcatttttgttttagttatcaattctcttgctgcctgttcttcaggcacatgaatttctgcatcatcctttataagttcatccttagacccgtatccttggtcagactgaccacctgtgctagagtgattatcaatggactcaagcctgattaaatctctgacgaagactgtgtgctccccattgttagcatcattagaactatccacactaccgtggctcaccgtgtccccatcacttccacctgtgacattttgaagagctgatattgaggagacctgtgacctttgcacagtctttttaagcggctgcctaaactgtgccaagccacgtaccacattccgtaccttcgtccataagaaaataccactgcgggtactgctaggccacgggctctccaagactaccttattataataaccataagtaatagcattaggctttatcctagcagttttcatttcaaataagactctcactgctaaaacaggatgaccccaaagtccacaaagctgcatcactactcgatagcacacctcatctaagggatccacatctgttttcctcatcttaataagtacatcatatgcctgctgaagtgctctgactttaggatgagaaactctaacataggccggaagacaaataaaccataaactgtaacaatgactaaacagacacttggcccactgtggtggatttgtataacatctcttcgccaatttatgagctgtttttatttcctgtttagttctcttagccatgagaggtggactctttgtaatgctattcccagtagggtgtctactaaaacaaagtttcaactcctgcggtctgtcaaaaagcttaaggtccagtcttggaaagtatttgtaactgtactttggtgacaggtcctttccatcatcaggaggtggctctggcggcattataaatacagtatgctcacttttctgtgaatcatctagttctatcaatctggtatcttctgctgaatcaaaatcaaccttatctgttttctctgtgcctttatcaggaaacaacttttctatgcagtcatcaaaaaatgctaatccagtatctttatcacttacaaaactgcattcttcaatgaaacgaataaaaatctgtgttttggataaaagggtatagaattttgcataggcacgatctcgactttttaaaaatccctgtcggtcaaacaatgaatcagcagctgtggctttatttgaaggagcctctgtgattggtctgagatatgttctatatccttttaaaatagacgccataaagcgcaaaaatgcctcttgaatttccatctcaagctgtgtcatcttcttttgccaggagaaatctgcttcaattggagtcatgtcaatcgctgagccttcttgagttttttggtgaactgaagacagctggggatacaatttctttaaggtgctaagtagatttttgcacggctttttgggaagttgcttccagttcatgttcttcttttcatctgatagctacaacagcttcagctaccccagtcaagacagctggcctaagagaatgcagcagaattttactctcaagtaaaacaaagagcagcagtgttgcacaattctcaggacccagattcattagcaaggtgctaaagttggctccacttagtggtaaaggtgtagaaactggctgtgataatattaatgcatcatggactgacagctggacaaggattctcggtctttgtggtgaaggaaaagggatgttttgcataaaatgtgaaatgtgcttttcaatgggaagaggatgtggtccagacacagaaagtttgtagataaacataagaaatttcctaaaagcttcaaaaaaaggccagtgtgagagtaaacaaatgcatttgtttgtattgatggatttggagaccatttttctctccacaggcgtcaacaagcccaggtgcataagctgtttctctgatagaagttcccgagagtaaggttcataaaactgaatggcagctccatatacctttttggctgaagaacctgtcaagacaaaagttgaaaaaactggaagtggatatttggtttcaggatcccagcactcaatagtagctcccataggaaggcagaaaagaggtacatctgattctgagagtggaaatgactcatagtcctcttctggatatctaaaaattaaaccagccttatatgctattgcatttgaagcaggtacagacttcttataacacagaaacacgctggaaccccacattccacaatttaagtttttgtcaactttgcagaaggtatgaggaggagtttctcctttactggttacaataacacagatatcagttacagccaaggaattctggggtcgaactggaggagcccttcgataagtgataaagattctttgtgaagtagttgaactattgttgacattggcacagcgaccatagggtgtggctaggatcacttcacatcctggaataagccgttctttcccttcatatagaactccaatatctgtaagcggtggtttatctctccctctcttataacagaggaaaagttctgggcttttcagacttccatagttcaagtttgcttggagagctgatggagtggcttctacacaggtgtaaccttcaggtactgtttctccagctgatttgataataatggcaatgtctgtaattggagctttaggtccagttgacttagtatctaaacgatttatttcttgatccaaaagagtagatgtgtcagtgagaccagctacgacaaagtagtctgtcactcttggtcctttgtcttctatcatggctgctactgtattttctgctgcctgctcctctgtcagcgcagccccgacacggcttcttcctggggcaagaaagcaccggattcgcggactgggcgcgctcggcagggcagggcgggggactagctccagcggccgccgccgcctcagtccggtct

SEQ ID NO: 8482 - RNA, 5858 nt, Homo sapiens
  source 1..5858: mol_type = other RNA
aaaagtaattgcggtttttgccattaatagtggcaaaaactacaattaattttgtgccaacctaatacattaaagttagggaaggcagctgtcatcagattttcaggtaattttaagattaatgactacagacaagtttagtagtagtcatttatttaatagtcaatgagacccctttcagaaaaccgtattgcaacatgcaatctattttaataaatatacacttagaatatggctgtatatacacatacctacacagccctacacatatacaaacttacacaaatatgttgctctcttttttttttttttttttttttgagacggtctcactctgtcacccaagctggagttgcagtggcgtgatctccactcactgtagcctctgcctcagttcaagcgattctcctgcctcagcctgagtagctgggactacagtggtgcgcctggctaatttttgtatttttagtaaagacagggtctcaccgtgttggccaggctggtctcgaactcctggcctcaagtgatccacccaccttgctcagcctcccaaagtgctgggattacaggcctgagccaccgtgcccggccatgttgcttttataattgagatatttcatttgttttgggggttaggcaaatttaatttgccattcctcaaactcagtaacttcaaatataaacaatgcctagaatgaatatggttcctcattatttctatcaaactactacaaatactgaagaatcccaaagtagttttccacagaggcagaaaagcagttcaggggttgaaaatcttcaatattaataagccctgggacattcaaatggcacttcatatttcaaggtaatgcaatatgaatcataattcattatatattgtccccaagagttacttcaattccgtattcaccagttcttacgatttggaaaaaaaaacttgaatgtttccagatgaaatctaatccccaagccttgtgtgtcaacattctagtgaatctctatttaaatgagaggcgctccaaaacacttcctgcaccactcgacactggcacttggtggagcatcaattttctgcaacctttcaagaatctctgaagacagactattgtatgcaattccatattcattgtcaaatgcctcaatatcaatattctctcttcctagagacactaatgataagaagaggatttctctgtataaactcctttgtcttttcatgcctggcttcatttgctgtgaaagtaggttgatgggtttaagaacattattgtgctgaatactctgcctgatggtttctactaaagtgcttgtttcttgttgttcctctgacaggagagatgatttcttttcagaattaaaattcctccatgagacatacagaggttctcttggttcctgatgaaggttgatattatcccataacagctgaatatacacaagtttgctatcctgggacagagatgacagaggaagctgtacaccttcattacaatgttcagatgtgaggataagtcctggcaagttactaggaaggtccaaacgtctgaaataccaaacgaggttccagaaaatgattggatgttgattgatgaaagaagatgtatgaatcacctgatcaccttcattttctagcaaagattcaagttctttacggagtactagaggactcaagtagggcacagaaacagggggaggattgggtctttttcctaaaggatccacaacttcctgcagactatttggaagactaactgttgagatgccatgaaacggtcgctgggtaaagtcaatattctgcaatgggcctccaacactgtgacttcgagtcaaagacacatttcgctttgataaactattaggcacagatgaaattttcatagtttggacatctccactggctctctttatttcatcacttggttcaactgcagagcctgtttcttcagttatgatctggttatgttttgggaagtccataaagttgatcaagtcaggttctgctaaactggatacaggtttgtgctccaaggattcatttgccaatggaatgcttccactttgtaaactgtcaccagaggtacttggtttcaggaaaaagcttgcagaacctctcaaatctttgaattctatattgagaagaggcaagaagttgcttttacagaatggacaagctgtattcaaatttgagtcatctgctgtccatccagccataatttcttcatcataaactaaagctccacaagctctacactgtgaacaactggacatcaaaacctccattgcacaattctgatagatgctagacatgctggtattttgagaagaaccatgatctgatttttcaaagtcttgccctttcatgcctcttggaaatggaacttcacctgttggataatgcagttttcctacatctccactactgctgctactgccaagacttgtgttgctctgggtaagttcactggggaccaaccctgagatacttgtgttaggcgatatattctcccccaaaatatggtcttctaggccagctgggaagctgtagtctctattagtttcttcctcatcatctgagtagctgtaggcagacgcaacagctacccacatcttactggctactgtcgctgcttgtttcataccagatttcaggacatctatcttgggccctgagagtatattatccagctttagccctgacaaagaatttactacagaacccaacgagccatgtggcgaagaacgcaccagtgctgacaaagaagttgaacgttctttatgagttcgagagggggtttgctgcttgaaacgcccagtaaaagttttagacctggacactgcaggtgagctcttttcactttcaggattttcctgtgctggtgaaccatgatctaaaggtaggcttgatctcctctctagagcatgaataaatgcagtagtcatgccagactctctgttttcctctctgtgtaattccatactagaagatttactacctaggggactttttaggttcatatagctttctatttcatcagccagattacgtgcaataactggagaaaacaacttatcttcagaatcaggagtttttcctcctgtacattcagtggctaaaagagacaaaggatctagtccagtttcaacatcttccctctgaaccaccttagcaataccatataaactacttctcttattcctcagatctttggatactgttttcaagtctctggactgattactgttactatcacttagtagactctcatatgtatctactgttgcagtagttttaggtacgtcatcaaccacaggctcaaggagttcttggctttcctcaagcatctctggcaccggagatgatctgtgctcaggattccaagtgctttcagacatacaagtcctactatcaggtaggtgacagctaacattctcaaagctatgggttcttgcaatatgaagtagagaagtcttaggacatgtcaatgctgctgtgagaatcttggcatctgctcccatcatgatagccatttcacttgaattcgaatccaaactactcttcttaagcaacattcctgctcgactttcagaactaaaactacaactcctctcaggaaaatgcttttgtcttttttctcctctatcaccattcttcttgagattagtagcttcgccaaagactgcatcttcaactggatcttgagtagaaaacagcacatttgatatactaccagtgctacttttcctgctgttgacatcaaatataccagacggaactttcacaatactgctgccccatgcaggaggttcagtaggactgtgaggctctggactaggttgtgaatgttttgccacaatagcagaggcatcacacacctcttctgtttgcatttttgttttagttatcaattctcttgctgcctgttcttcaggcacatgaatttctgcatcatcctttataagttcatccttagacccgtatccttggtcagactgaccacctgtgctagagtgattatcaatggactcaagcctgattaaatctctgacgaagactgtgtgctccccattgttagcatcattagaactatccacactaccgtggctcaccgtgtccccatcacttccacctgtgacattttgaagagctgatattgaggagacctgtgacctttgcacagtctttttaagcggctgcctaaactgtgccaagccacgtaccacattccgtaccttcgtccataagaaaataccactgcgggtactgctaggccacgggctctccaagactaccttattataataaccataagtaatagcattaggctttatcctagcagttttcatttcaaataagactctcactgctaaaacaggatgaccccaaagtccacaaagctgcatcactactcgatagcacacctcatctaagggatccacatctgttttcctcatcttaataagtacatcatatgcctgctgaagtgctctgactttaggatgagaaactctaacataggccggaagacaaataaaccataaactgtaacaatgactaaacagacacttggcccactgtggtggatttgtataacatctcttcgccaatttatgagctgtttttatttcctgtttagttctcttagccatgagaggtggactctttgtaatgctattcccagtagggtgtctactaaaacaaagtttcaactcctgcggtctgtcaaaaagcttaaggtccagtcttggaaagtatttgtaactgtactttggtgacaggtcctttccatcatcaggaggtggctctggcggcattataaatacagtatgctcacttttctgtgaatcatctagttctatcaatctggtatcttctgctgaatcaaaatcaaccttatctgttttctctgtgcctttatcaggaaacaacttttctatgcagtcatcaaaaaatgctaatccagtatctttatcacttacaaaactgcattcttcaatgaaacgaataaaaatctgtgttttggataaaagggtatagaattttgcataggcacgatctcgactttttaaaaatccctgtcggtcaaacaatgaatcagcagctgtggctttatttgaaggagcctctgtgattggtctgagatatgttctatatccttttaaaatagacgccataaagcgcaaaaatgcctcttgaatttccatctcaagctgtgtcatcttcttttgccaggagaaatctgcttcaattggagtcatgtcaatcgctgagccttcttgagttttttggtgaactgaagacagctggggatacaatttctttaaggtgctaagtagatttttgcacggctttttgggaagttgcttccagttcatgttcttcttttcatctgatccaatatctgtaagcggtggtttatctctccctctcttataacagaggaaaagttctgggcttttcagacttccatagttcaagtttgcttggagagctgatggagtggcttctacacaggtgtaaccttcaggtactgtttctccagctgatttgataataatggcaatgtctgtaattggagctttaggtccagttgacttagtatctaaacgatttatttcttgatccaaaagagtagatgtgtcagtgagaccagctacgacaaagtagtctgtcactcttggtcctttgtcttctatcatggctgctactgtattttctgctgcctgctcctctgtcagcgcagccccgacacggcttcttcctggggcaagaaagcaccggattcgcggactgggcgcgctcggcagggcagggcgggggactagctccagcggccgccgccgcctcagtccggtct

SEQ ID NO: 8483 - RNA, 6833 nt, Homo sapiens
  source 1..6833: mol_type = other RNA
aaaagtaattgcggtttttgccattaatagtggcaaaaactacaattaattttgtgccaacctaatacattaaagttagggaaggcagctgtcatcagattttcaggtaattttaagattaatgactacagacaagtttagtagtagtcatttatttaatagtcaatgagacccctttcagaaaaccgtattgcaacatgcaatctattttaataaatatacacttagaatatggctgtatatacacatacctacacagccctacacatatacaaacttacacaaatatgttgctctcttttttttttttttttttttttgagacggtctcactctgtcacccaagctggagttgcagtggcgtgatctccactcactgtagcctctgcctcagttcaagcgattctcctgcctcagcctgagtagctgggactacagtggtgcgcctggctaatttttgtatttttagtaaagacagggtctcaccgtgttggccaggctggtctcgaactcctggcctcaagtgatccacccaccttgctcagcctcccaaagtgctgggattacaggcctgagccaccgtgcccggccatgttgcttttataattgagatatttcatttgttttgggggttaggcaaatttaatttgccattcctcaaactcagtaacttcaaatataaacaatgcctagaatgaatatggttcctcattatttctatcaaactactacaaatactgaagaatcccaaagtagttttccacagaggcagaaaagcagttcaggggttgaaaatcttcaatattaataagccctgggacattcaaatggcacttcatatttcaaggtaatgcaatatgaatcataattcattatatattgtccccaagagttacttcaattccgtattcaccagttcttacgatttggaaaaaaaaacttgaatgtttccagatgaaatctaatccccaagccttgtgtgtcaacattctagtgaatctctatttaaatgagaggcgctccaaaacacttcctgcaccactcgacactggcacttggtggagcatcaattttctgcaacctttcaagaatctctgaagacagactattgtatgcaattccatattcattgtcaaatgcctcaatatcaatattctctcttcctagagacactaatgataagaagaggatttctctgtataaactcctttgtcttttcatgcctggcttcatttgctgtgaaagtaggttgatgggtttaagaacattattgtgctgaatactctgcctgatggtttctactaaagtgcttgtttcttgttgttcctctgacaggagagatgatttcttttcagaattaaaattcctccatgagacatacagaggttctcttggttcctgatgaaggttgatattatcccataacagctgaatatacacaagtttgctatcctgggacagagatgacagaggaagctgtacaccttcattacaatgttcagatgtgaggataagtcctggcaagttactaggaaggtccaaacgtctgaaataccaaacgaggttccagaaaatgattggatgttgattgatgaaagaagatgtatgaatcacctgatcaccttcattttctagcaaagattcaagttctttacggagtactagaggactcaagtagggcacagaaacagggggaggattgggtctttttcctaaaggatccacaacttcctgcagactatttggaagactaactgttgagatgccatgaaacggtcgctgggtaaagtcaatattctgcaatgggcctccaacactgtgacttcgagtcaaagacacatttcgctttgataaactattaggcacagatgaaattttcatagtttggacatctccactggctctctttatttcatcacttggttcaactgcagagcctgtttcttcagttatgatctggttatgttttgggaagtccataaagttgatcaagtcaggttctgctaaactggatacaggtttgtgctccaaggattcatttgccaatggaatgcttccactttgtaaactgtcaccagaggtacttggtttcaggaaaaagcttgcagaacctctcaaatctttgaattctatattgagaagaggcaagaagttgcttttacagaatggacaagctgtattcaaatttgagtcatctgctgtccatccagccataatttcttcatcataaactaaagctccacaagctctacactgtgaacaactggacatcaaaacctccattgcacaattctgatagatgctagacatgctggtattttgagaagaaccatgatctgatttttcaaagtcttgccctttcatgcctcttggaaatggaacttcacctgttggataatgcagttttcctacatctccactactgctgctactgccaagacttgtgttgctctgggtaagttcactggggaccaaccctgagatacttgtgttaggcgatatattctcccccaaaatatggtcttctaggccagctgggaagctgtagtctctattagtttcttcctcatcatctgagtagctgtaggcagacgcaacagctacccacatcttactggctactgtcgctgcttgtttcataccagatttcaggacatctatcttgggccctgagagtatattatccagctttagccctgacaaagaatttactacagaacccaacgagccatgtggcgaagaacgcaccagtgctgacaaagaagttgaacgttctttatgagttcgagagggggtttgctgcttgaaacgcccagtaaaagttttagacctggacactgcaggtgagctcttttcactttcaggattttcctgtgctggtgaaccatgatctaaaggtaggcttgatctcctctctagagcatgaataaatgcagtagtcatgccagactctctgttttcctctctgtgtaattccatactagaagatttactacctaggggactttttaggttcatatagctttctatttcatcagccagattacgtgcaataactggagaaaacaacttatcttcagaatcaggagtttttcctcctgtacattcagtggctaaaagagacaaaggatctagtccagtttcaacatcttccctctgaaccaccttagcaataccatataaactacttctcttattcctcagatctttggatactgttttcaagtctctggactgattactgttactatcacttagtagactctcatatgtatctactgttgcagtagttttaggtacgtcatcaaccacaggctcaaggagttcttggctttcctcaagcatctctggcaccggagatgatctgtgctcaggattccaagtgctttcagacatacaagtcctactatcaggtaggtgacagctaacattctcaaagctatgggttcttgcaatatgaagtagagaagtcttaggacatgtcaatgctgctgtgagaatcttggcatctgctcccatcatgatagccatttcacttgaattcgaatccaaactactcttcttaagcaacattcctgctcgactttcagaactaaaactacaactcctctcaggaaaatgcttttgtcttttttctcctctatcaccattcttcttgagattagtagcttcgccaaagactgcatcttcaactggatcttgagtagaaaacagcacatttgatatactaccagtgctacttttcctgctgttgacatcaaatataccagacggaactttcacaatactgctgccccatgcaggaggttcagtaggactgtgaggctctggactaggttgtgaatgttttgccacaatagcagaggcatcacacacctcttctgtttgcatttttgttttagttatcaattctcttgctgcctgttcttcaggcacatgaatttctgcatcatcctttataagttcatccttagacccgtatccttggtcagactgaccacctgtgctagagtgattatcaatggactcaagcctgattaaatctctgacgaagactgtgtgctccccattgttagcatcattagaactatccacactaccgtggctcaccgtgtccccatcacttccacctgtgacattttgaagagctgatattgaggagacctgtgacctttgcacagtctttttaagcggctgcctaaactgtgccaagccacgtaccacattccgtaccttcgtccataagaaaataccactgcgggtactgctaggccacgggctctccaagactaccttattataataaccataagtaatagcattaggctttatcctagcagttttcatttcaaataagactctcactgctaaaacaggatgaccccaaagtccacaaagctgcatcactactcgatagcacacctgtttagttctcttagccatgagaggtggactctttgtaatgctattcccagtagggtgtctactaaaacaaagtttcaactcctgcggtctgtcaaaaagcttaaggtccagtcttggaaagtatttgtaactgtactttggtgacaggtcctttccatcatcaggaggtggctctggcggcattataaatacagtatgctcacttttctgtgaatcatctagttctatcaatctggtatcttctgctgaatcaaaatcaaccttatctgttttctctgtgcctttatcaggaaacaacttttctatgcagtcatcaaaaaatgctaatccagtatctttatcacttacaaaactgcattcttcaatgaaacgaataaaaatctgtgttttggataaaagggtatagaattttgcataggcacgatctcgactttttaaaaatccctgtcggtcaaacaatgaatcagcagctgtggctttatttgaaggagcctctgtgattggtctgagatatgttctatatccttttaaaatagacgccataaagcgcaaaaatgcctcttgaatttccatctcaagctgtgtcatcttcttttgccaggagaaatctgcttcaattggagtcatgtcaatcgctgagccttcttgagttttttggtgaactgaagacagctggggatacaatttctttaaggtgctaagtagatttttgcacggctttttgggaagttgcttccagttcatgttcttcttttcatctgatacatataacatgttcgtatccaagtcaatgcaaacaacatcttgtggtgggtcatgaagatcaaaataccttgagtcaactccaactataaatggtaaaggtgcactaagcactgcagccagtgaaagaggacaaaggggaatatatgggcattgccactgaaatggaaagatcatagctacaacagcttcagctaccccagtcaagacagctggcctaagagaatgcagcagaattttactctcaagtaaaacaaagagcagcagtgttgcacaattctcaggacccagattcattagcaaggtgctaaagttggctccacttagtggtaaaggtgtagaaactggctgtgataatattaatgcatcatggactgacagctggacaaggattctcggtctttgtggtgaaggaaaagggatgttttgcataaaatgtgaaatgtgcttttcaatgggaagaggatgtggtccagacacagaaagtttgtagataaacataagaaatttcctaaaagcttcaaaaaaaggccagtgtgagagtaaacaaatgcatttgtttgtattgatggatttggagaccatttttctctccacaggcgtcaacaagcccaggtgcataagctgtttctctgatagaagttcccgagagtaaggttcataaaactgaatggcagctccatatacctttttggctgaagaacctgtcaagacaaaagttgaaaaaactggaagtggatatttggtttcaggatcccagcactcaatagtagctcccataggaaggcagaaaagaggtacatctgattctgagagtggaaatgactcatagtcctcttctggatatctaaaaattaaaccagccttatatgctattgcatttgaagcaggtacagacttcttataacacagaaacacgctggaaccccacattccacaatttaagtttttgtcaactttgcagaaggtatgaggaggagtttctcctttactggttacaataacacagatatcagttacagccaaggaattctggggtcgaactggaggagcccttcgataagtgataaagattctttgtgaagtagttgaactattgttgacattggcacagcgaccatagggtgtggctaggatcacttcacatcctggaataagccgttctttcccttcatatagaactccaatatctgtaagcggtggtttatctctccctctcttataacagaggaaaagttctgggcttttcagacttccatagttcaagtttgcttggagagctgatggagtggcttctacacaggtgtaaccttcaggtactgtttctccagctgatttgataataatggcaatgtctgtaattggagctttaggtccagttgacttagtatctaaacgatttatttcttgatccaaaagagtagatgtgtcagtgagaccagctacgacaaagtagtctgtcactcttggtcctttgtcttctatcatggctgctactgtattttctgctgcctgctcctctgtcagcgcagccccgacacggcttcttcctggggcaagaaagcaccggattcgcggactgggcgcgctcggcagggcagggcgggggactagctccagcggccgccgccgcctcagtccggtct

SEQ ID NO: 8484 - RNA, 6866 nt, Homo sapiens
  source 1..6866: mol_type = other RNA
aaaagtaattgcggtttttgccattaatagtggcaaaaactacaattaattttgtgccaacctaatacattaaagttagggaaggcagctgtcatcagattttcaggtaattttaagattaatgactacagacaagtttagtagtagtcatttatttaatagtcaatgagacccctttcagaaaaccgtattgcaacatgcaatctattttaataaatatacacttagaatatggctgtatatacacatacctacacagccctacacatatacaaacttacacaaatatgttgctctcttttttttttttttttttttttgagacggtctcactctgtcacccaagctggagttgcagtggcgtgatctccactcactgtagcctctgcctcagttcaagcgattctcctgcctcagcctgagtagctgggactacagtggtgcgcctggctaatttttgtatttttagtaaagacagggtctcaccgtgttggccaggctggtctcgaactcctggcctcaagtgatccacccaccttgctcagcctcccaaagtgctgggattacaggcctgagccaccgtgcccggccatgttgcttttataattgagatatttcatttgttttgggggttaggcaaatttaatttgccattcctcaaactcagtaacttcaaatataaacaatgcctagaatgaatatggttcctcattatttctatcaaactactacaaatactgaagaatcccaaagtagttttccacagaggcagaaaagcagttcaggggttgaaaatcttcaatattaataagccctgggacattcaaatggcacttcatatttcaaggtaatgcaatatgaatcataattcattatatattgtccccaagagttacttcaattccgtattcaccagttcttacgatttggaaaaaaaaacttgaatgtttccagatgaaatctaatccccaagccttgtgtgtcaacattctagtgaatctctatttaaatgagaggcgctccaaaacacttcctgcaccactcgacactggcacttggtggagcatcaattttctgcaacctttcaagaatctctgaagacagactattgtatgcaattccatattcattgtcaaatgcctcaatatcaatattctctcttcctagagacactaatgataagaagaggatttctctgtataaactcctttgtcttttcatgcctggcttcatttgctgtgaaagtaggttgatgggtttaagaacattattgtgctgaatactctgcctgatggtttctactaaagtgcttgtttcttgttgttcctctgacaggagagatgatttcttttcagaattaaaattcctccatgagacatacagaggttctcttggttcctgatgaaggttgatattatcccataacagctgaatatacacaagtttgctatcctgggacagagatgacagaggaagctgtacaccttcattacaatgttcagatgtgaggataagtcctggcaagttactaggaaggtccaaacgtctgaaataccaaacgaggttccagaaaatgattggatgttgattgatgaaagaagatgtatgaatcacctgatcaccttcattttctagcaaagattcaagttctttacggagtactagaggactcaagtagggcacagaaacagggggaggattgggtctttttcctaaaggatccacaacttcctgcagactatttggaagactaactgttgagatgccatgaaacggtcgctgggtaaagtcaatattctgcaatgggcctccaacactgtgacttcgagtcaaagacacatttcgctttgataaactattaggcacagatgaaattttcatagtttggacatctccactggctctctttatttcatcacttggttcaactgcagagcctgtttcttcagttatgatctggttatgttttgggaagtccataaagttgatcaagtcaggttctgctaaactggatacaggtttgtgctccaaggattcatttgccaatggaatgcttccactttgtaaactgtcaccagaggtacttggtttcaggaaaaagcttgcagaacctctcaaatctttgaattctatattgagaagaggcaagaagttgcttttacagaatggacaagctgtattcaaatttgagtcatctgctgtccatccagccataatttcttcatcataaactaaagctccacaagctctacactgtgaacaactggacatcaaaacctccattgcacaattctgatagatgctagacatgctggtattttgagaagaaccatgatctgatttttcaaagtcttgccctttcatgcctcttggaaatggaacttcacctgttggataatgcagttttcctacatctccactactgctgctactgccaagacttgtgttgctctgggtaagttcactggggaccaaccctgagatacttgtgttaggcgatatattctcccccaaaatatggtcttctaggccagctgggaagctgtagtctctattagtttcttcctcatcatctgagtagctgtaggcagacgcaacagctacccacatcttactggctactgtcgctgcttgtttcataccagatttcaggacatctatcttgggccctgagagtatattatccagctttagccctgacaaagaatttactacagaacccaacgagccatgtggcgaagaacgcaccagtgctgacaaagaagttgaacgttctttatgagttcgagagggggtttgctgcttgaaacgcccagtaaaagttttagacctggacactgcaggtgagctcttttcactttcaggattttcctgtgctggtgaaccatgatctaaaggtaggcttgatctcctctctagagcatgaataaatgcagtagtcatgccagactctctgttttcctctctgtgtaattccatactagaagatttactacctaggggactttttaggttcatatagctttctatttcatcagccagattacgtgcaataactggagaaaacaacttatcttcagaatcaggagtttttcctcctgtacattcagtggctaaaagagacaaaggatctagtccagtttcaacatcttccctctgaaccaccttagcaataccatataaactacttctcttattcctcagatctttggatactgttttcaagtctctggactgattactgttactatcacttagtagactctcatatgtatctactgttgcagtagttttaggtacgtcatcaaccacaggctcaaggagttcttggctttcctcaagcatctctggcaccggagatgatctgtgctcaggattccaagtgctttcagacatacaagtcctactatcaggtaggtgacagctaacattctcaaagctatgggttcttgcaatatgaagtagagaagtcttaggacatgtcaatgctgctgtgagaatcttggcatctgctcccatcatgatagccatttcacttgaattcgaatccaaactactcttcttaagcaacattcctgctcgactttcagaactaaaactacaactcctctcaggaaaatgcttttgtcttttttctcctctatcaccattcttcttgagattagtagcttcgccaaagactgcatcttcaactggatcttgagtagaaaacagcacatttgatatactaccagtgctacttttcctgctgttgacatcaaatataccagacggaactttcacaatactgctgccccatgcaggaggttcagtaggactgtgaggctctggactaggttgtgaatgttttgccacaatagcagaggcatcacacacctcttctgtttgcatttttgttttagttatcaattctcttgctgcctgttcttcaggcacatgaatttctgcatcatcctttataagttcatccttagacccgtatccttggtcagactgaccacctgtgctagagtgattatcaatggactcaagcctgattaaatctctgacgaagactgtgtgctccccattgttagcatcattagaactatccacactaccgtggctcaccgtgtccccatcacttccacctgtgacattttgaagagcttcgtccataagaaaataccactgcgggtactgctaggccacgggctctccaagactaccttattataataaccataagtaatagcattaggctttatcctagcagttttcatttcaaataagactctcactgctaaaacaggatgaccccaaagtccacaaagctgcatcactactcgatagcacacctgtaatcccagctacttgggaagctgaggcacgagaatcgcttgaagccaggaggtagaggttgtaatgagcccagatcacgccactgcactccagcctgggcaacagagtgagactctgtttagttctcttagccatgagaggtggactctttgtaatgctattcccagtagggtgtctactaaaacaaagtttcaactcctgcggtctgtcaaaaagcttaaggtccagtcttggaaagtatttgtaactgtactttggtgacaggtcctttccatcatcaggaggtggctctggcggcattataaatacagtatgctcacttttctgtgaatcatctagttctatcaatctggtatcttctgctgaatcaaaatcaaccttatctgttttctctgtgcctttatcaggaaacaacttttctatgcagtcatcaaaaaatgctaatccagtatctttatcacttacaaaactgcattcttcaatgaaacgaataaaaatctgtgttttggataaaagggtatagaattttgcataggcacgatctcgactttttaaaaatccctgtcggtcaaacaatgaatcagcagctgtggctttatttgaaggagcctctgtgattggtctgagatatgttctatatccttttaaaatagacgccataaagcgcaaaaatgcctcttgaatttccatctcaagctgtgtcatcttcttttgccaggagaaatctgcttcaattggagtcatgtcaatcgctgagccttcttgagttttttggtgaactgaagacagctggggatacaatttctttaaggtgctaagtagatttttgcacggctttttgggaagttgcttccagttcatgttcttcttttcatctgatacatataacatgttcgtatccaagtcaatgcaaacaacatcttgtggtgggtcatgaagatcaaaataccttgagtcaactccaactataaatggtaaaggtgcactaagcactgcagccagtgaaagaggacaaaggggaatatatgggcattgccactgaaatggaaagatcatagctacaacagcttcagctaccccagtcaagacagctggcctaagagaatgcagcagaattttactctcaagtaaaacaaagagcagcagtgttgcacaattctcaggacccagattcattagcaaggtgctaaagttggctccacttagtggtaaaggtgtagaaactggctgtgataatattaatgcatcatggactgacagctggacaaggattctcggtctttgtggtgaaggaaaagggatgttttgcataaaatgtgaaatgtgcttttcaatgggaagaggatgtggtccagacacagaaagtttgtagataaacataagaaatttcctaaaagcttcaaaaaaaggccagtgtgagagtaaacaaatgcatttgtttgtattgatggatttggagaccatttttctctccacaggcgtcaacaagcccaggtgcataagctgtttctctgatagaagttcccgagagtaaggttcataaaactgaatggcagctccatatacctttttggctgaagaacctgtcaagacaaaagttgaaaaaactggaagtggatatttggtttcaggatcccagcactcaatagtagctcccataggaaggcagaaaagaggtacatctgattctgagagtggaaatgactcatagtcctcttctggatatctaaaaattaaaccagccttatatgctattgcatttgaagcaggtacagacttcttataacacagaaacacgctggaaccccacattccacaatttaagtttttgtcaactttgcagaaggtatgaggaggagtttctcctttactggttacaataacacagatatcagttacagccaaggaattctggggtcgaactggaggagcccttcgataagtgataaagattctttgtgaagtagttgaactattgttgacattggcacagcgaccatagggtgtggctaggatcacttcacatcctggaataagccgttctttcccttcatatagaactccaatatctgtaagcggtggtttatctctccctctcttataacagaggaaaagttctgggcttttcagacttccatagttcaagtttgcttggagagctgatggagtggcttctacacaggtgtaaccttcaggtactgtttctccagctgatttgataataatggcaatgtctgtaattggagctttaggtccagttgacttagtatctaaacgatttatttcttgatccaaaagagtagatgtgtcagtgagaccagctacgacaaagtagtctgtcactcttggtcctttgtcttctatcatggctgctactgtattttctgctgcctgctcctctgtcagcgcagccccgacacggcttcttcctggggcaagaaagcaccggattcgcggactgggcgcgctcggcagggcagggcgggggactagctccagcggccgccgccgcctcagtccggtct

SEQ ID NO: 8485 - RNA, 7136 nt, Homo sapiens
  source 1..7136: mol_type = other RNA
aaaagtaattgcggtttttgccattaatagtggcaaaaactacaattaattttgtgccaacctaatacattaaagttagggaaggcagctgtcatcagattttcaggtaattttaagattaatgactacagacaagtttagtagtagtcatttatttaatagtcaatgagacccctttcagaaaaccgtattgcaacatgcaatctattttaataaatatacacttagaatatggctgtatatacacatacctacacagccctacacatatacaaacttacacaaatatgttgctctcttttttttttttttttttttttgagacggtctcactctgtcacccaagctggagttgcagtggcgtgatctccactcactgtagcctctgcctcagttcaagcgattctcctgcctcagcctgagtagctgggactacagtggtgcgcctggctaatttttgtatttttagtaaagacagggtctcaccgtgttggccaggctggtctcgaactcctggcctcaagtgatccacccaccttgctcagcctcccaaagtgctgggattacaggcctgagccaccgtgcccggccatgttgcttttataattgagatatttcatttgttttgggggttaggcaaatttaatttgccattcctcaaactcagtaacttcaaatataaacaatgcctagaatgaatatggttcctcattatttctatcaaactactacaaatactgaagaatcccaaagtagttttccacagaggcagaaaagcagttcaggggttgaaaatcttcaatattaataagccctgggacattcaaatggcacttcatatttcaaggtaatgcaatatgaatcataattcattatatattgtccccaagagttacttcaattccgtattcaccagttcttacgatttggaaaaaaaaacttgaatgtttccagatgaaatctaatccccaagccttgtgtgtcaacattctagtgaatctctatttaaatgagaggcgctccaaaacacttcctgcaccactcgacactggcacttggtggagcatcaattttctgcaacctttcaagaatctctgaagacagactattgtatgcaattccatattcattgtcaaatgcctcaatatcaatattctctcttcctagagacactaatgataagaagaggatttctctgtataaactcctttgtcttttcatgcctggcttcatttgctgtgaaagtaggttgatgggtttaagaacattattgtgctgaatactctgcctgatggtttctactaaagtgcttgtttcttgttgttcctctgacaggagagatgatttcttttcagaattaaaattcctccatgagacatacagaggttctcttggttcctgatgaaggttgatattatcccataacagctgaatatacacaagtttgctatcctgggacagagatgacagaggaagctgtacaccttcattacaatgttcagatgtgaggataagtcctggcaagttactaggaaggtccaaacgtctgaaataccaaacgaggttccagaaaatgattggatgttgattgatgaaagaagatgtatgaatcacctgatcaccttcattttctagcaaagattcaagttctttacggagtactagaggactcaagtagggcacagaaacagggggaggattgggtctttttcctaaaggatccacaacttcctgcagactatttggaagactaactgttgagatgccatgaaacggtcgctgggtaaagtcaatattctgcaatgggcctccaacactgtgacttcgagtcaaagacacatttcgctttgataaactattaggcacagatgaaattttcatagtttggacatctccactggctctctttatttcatcacttggttcaactgcagagcctgtttcttcagttatgatctggttatgttttgggaagtccataaagttgatcaagtcaggttctgctaaactggatacaggtttgtgctccaaggattcatttgccaatggaatgcttccactttgtaaactgtcaccagaggtacttggtttcaggaaaaagttcttgagagagcttttataagactaaccttgcagaacctctcaaatctttgaattctatattgagaagaggcaagaagttgcttttacagaatggacaagctgtattcaaatttgagtcatctgctgtccatccagccataatttcttcatcataaactaaagctccacaagctctacactgtgaacaactggacatcaaaacctccattgcacaattctgatagatgctagacatgctggtattttgagaagaaccatgatctgatttttcaaagtcttgccctttcatgcctcttggaaatggaacttcacctgttggataatgcagttttcctacatctccactactgctgctactgccaagacttgtgttgctctgggtaagttcactggggaccaaccctgagatacttgtgttaggcgatatattctcccccaaaatatggtcttctaggccagctgggaagctgtagtctctattagtttcttcctcatcatctgagtagctgtaggcagacgcaacagctacccacatcttactggctactgtcgctgcttgtttcataccagatttcaggacatctatcttgggccctgagagtatattatccagctttagccctgacaaagaatttactacagaacccaacgagccatgtggcgaagaacgcaccagtgctgacaaagaagttgaacgttctttatgagttcgagagggggtttgctgcttgaaacgcccagtaaaagttttagacctggacactgcaggtgagctcttttcactttcaggattttcctgtgctggtgaaccatgatctaaaggtaggcttgatctcctctctagagcatgaataaatgcagtagtcatgccagactctctgttttcctctctgtgtaattccatactagaagatttactacctaggggactttttaggttcatatagctttctatttcatcagccagattacgtgcaataactggagaaaacaacttatcttcagaatcaggagtttttcctcctgtacattcagtggctaaaagagacaaaggatctagtccagtttcaacatcttccctctgaaccaccttagcaataccatataaactacttctcttattcctcagatctttggatactgttttcaagtctctggactgattactgttactatcacttagtagactctcatatgtatctactgttgcagtagttttaggtacgtcatcaaccacaggctcaaggagttcttggctttcctcaagcatctctggcaccggagatgatctgtgctcaggattccaagtgctttcagacatacaagtcctactatcaggtaggtgacagctaacattctcaaagctatgggttcttgcaatatgaagtagagaagtcttaggacatgtcaatgctgctgtgagaatcttggcatctgctcccatcatgatagccatttcacttgaattcgaatccaaactactcttcttaagcaacattcctgctcgactttcagaactaaaactacaactcctctcaggaaaatgcttttgtcttttttctcctctatcaccattcttcttgagattagtagcttcgccaaagactgcatcttcaactggatcttgagtagaaaacagcacatttgatatacagtgctacttttcctgctgttgacatcaaatataccagacggaactttcacaatactgctgccccatgcaggaggttcagtaggactgtgaggctctggactaggttgtgaatgttttgccacaatagcagaggcatcacacacctcttctgtttgcatttttgttttagttatcaattctcttgctgcctgttcttcaggcacatgaatttctgcatcatcctttataagttcatccttagacccgtatccttggtcagactgaccacctgatgtggttaacattcaagggtagaattaatgcacacgtgtatccatagcttcacgtcatataagtctgtctgtgctagagtgattatcaatggactcaagcctgattaaatctctgacgaagactgtgtgctccccattgttagcatcattagaactatccacactaccgtggctcaccgtgtccccatcacttccacctgtgacattttgaagagctgatattgaggagacctgtgacctttgcacagtctttttaagcggctgcctaaactgtgccaagccacgtaccacattccgtaccttcgtccataagaaaataccactgcgggtactgctaggccacgggctctccaagactaccttattataataaccataagtaatagcattaggctttatcctagcagttttcatttcaaataagactctcactgctaaaacaggatgaccccaaagtccacaaagctgcatcactactcgatagcacacctcatctaagggatccacatctgttttcctcatcttaataagtacatcatatgcctgctgaagtgctctgactttaggatgagaaactctaacataggccggaagacaaataaaccataaactgtaacaatgactaaacagacacttggcccactgtggtggatttgtataacatctcttcgccaatttatgagctgtttttatttcctgtttagttctcttagccatgagaggtggactctttgtaatgctattcccagtagggtgtctactaaaacaaagtttcaactcctgcggtctgtcaaaaagcttaaggtccagtcttggaaagtatttgtaactgtactttggtgacaggtcctttccatcatcaggaggtggctctggcggcattataaatacagtatgctcacttttctgtgaatcatctagttctatcaatctggtatcttctgctgaatcaaaatcaaccttatctgttttctctgtgcctttatcaggaaacaacttttctatgcagtcatcaaaaaatgctaatccagtatctttatcacttacaaaactgcattcttcaatgaaacgaataaaaatctgtgttttggataaaagggtatagaattttgcataggcacgatctcgactttttaaaaatccctgtcggtcaaacaatgaatcagcagctgtggctttatttgaaggagcctctgtgattggtctgagatatgttctatatccttttaaaatagacgccataaagcgcaaaaatgcctcttgaatttccatctcaagctgtgtcatcttcttttgccaggagaaatctgcttcaattggagtcatgtcaatcgctgagccttcttgagttttttggtgaactgaagacagctggggatacaatttctttaaggtgctaagtagatttttgcacggctttttgggaagttgcttccagttcatgttcttcttttcatctgatacatataacatgttcgtatccaagtcaatgcaaacaacatcttgtggtgggtcatgaagatcaaaataccttgagtcaactccaactataaatggtaaaggtgcactaagcactgcagccagtgaaagaggacaaaggggaatatatgggcattgccactgaaatggaaagatcatagctacaacagcttcagctaccccagtcaagacagctggcctaagagaatgcagcagaattttactctcaagtaaaacaaagagcagcagtgttgcacaattctcaggacccagattcattagcaaggtgctaaagttggctccacttagtggtaaaggtgtagaaactggctgtgataatattaatgcatcatggactgacagctggacaaggattctcggtctttgtggtgaaggaaaagggatgttttgcataaaatgtgaaatgtgcttttcaatgggaagaggatgtggtccagacacagaaagtttgtagataaacataagaaatttcctaaaagcttcaaaaaaaggccagtgtgagagtaaacaaatgcatttgtttgtattgatggatttggagaccatttttctctccacaggcgtcaacaagcccaggtgcataagctgtttctctgatagaagttcccgagagtaaggttcataaaactgaatggcagctccatatacctttttggctgaagaacctgtcaagacaaaagttgaaaaaactggaagtggatatttggtttcaggatcccagcactcaatagtagctcccataggaaggcagaaaagaggtacatctgattctgagagtggaaatgactcatagtcctcttctggatatctaaaaattaaaccagccttatatgctattgcatttgaagcaggtacagacttcttataacacagaaacacgctggaaccccacattccacaatttaagtttttgtcaactttgcagaaggtatgaggaggagtttctcctttactggttacaataacacagatatcagttacagccaaggaattctggggtcgaactggaggagcccttcgataagtgataaagattctttgtgaagtagttgaactattgttgacattggcacagcgaccatagggtgtggctaggatcacttcacatcctggaataagccgttctttcccttcatatagaactccaatatctgtaagcggtggtttatctctccctctcttataacagaggaaaagttctgggcttttcagacttccatagttcaagtttgcttggagagctgatggagtggcttctacacaggtgtaaccttcaggtactgtttctccagctgatttgataataatggcaatgtctgtaattggagctttaggtccagttgacttagtatctaaacgatttatttcttgatccaaaagagtagatgtgtcagtgagaccagctacgacaaagtagtctgtcactcttggtcctttgtcttctatcatggctgctactgtattttctgctgcctgctcctctgtcagcgcagccccgacacggcttcttcctggggcaagaaagcaccggattcgcggactgggcgcgctcggcagggcagggcgggggactagctccagcggccgccgccgcctcagtccggtct

SEQ ID NO: 8486 - RNA, 6921 nt, Homo sapiens
  source 1..6921: mol_type = other RNA
aaaagtaattgcggtttttgccattaatagtggcaaaaactacaattaattttgtgccaacctaatacattaaagttagggaaggcagctgtcatcagattttcaggtaattttaagattaatgactacagacaagtttagtagtagtcatttatttaatagtcaatgagacccctttcagaaaaccgtattgcaacatgcaatctattttaataaatatacacttagaatatggctgtatatacacatacctacacagccctacacatatacaaacttacacaaatatgttgctctcttttttttttttttttttttttgagacggtctcactctgtcacccaagctggagttgcagtggcgtgatctccactcactgtagcctctgcctcagttcaagcgattctcctgcctcagcctgagtagctgggactacagtggtgcgcctggctaatttttgtatttttagtaaagacagggtctcaccgtgttggccaggctggtctcgaactcctggcctcaagtgatccacccaccttgctcagcctcccaaagtgctgggattacaggcctgagccaccgtgcccggccatgttgcttttataattgagatatttcatttgttttgggggttaggcaaatttaatttgccattcctcaaactcagtaacttcaaatataaacaatgcctagaatgaatatggttcctcattatttctatcaaactactacaaatactgaagaatcccaaagtagttttccacagaggcagaaaagcagttcaggggttgaaaatcttcaatattaataagccctgggacattcaaatggcacttcatatttcaaggtaatgcaatatgaatcataattcattatatattgtccccaagagttacttcaattccgtattcaccagttcttacgatttggaaaaaaaaacttgaatgtttccagatgaaatctaatccccaagccttgtgtgtcaacattctagtgaatctctatttaaatgagaggcgctccaaaacacttcctgcaccactcgacactggcacttggtggagcatcaattttctgcaacctttcaagaatctctgaagacagactattgtatgcaattccatattcattgtcaaatgcctcaatatcaatattctctcttcctagagacactaatgataagaagaggatttctctgtataaactcctttgtcttttcatgcctggcttcatttgctgtgaaagtaggttgatgggtttaagaacattattgtgctgaatactctgcctgatggtttctactaaagtgcttgtttcttgttgttcctctgacaggagagatgatttcttttcagaattaaaattcctccatgagacatacagaggttctcttggttcctgatgaaggttgatattatcccataacagctgaatatacacaagtttgctatcctgggacagagatgacagaggaagctgtacaccttcattacaatgttcagatgtgaggataagtcctggcaagttactaggaaggtccaaacgtctgaaataccaaacgaggttccagaaaatgattggatgttgattgatgaaagaagatgtatgaatcacctgatcaccttcattttctagcaaagattcaagttctttacggagtactagaggactcaagtagggcacagaaacagggggaggattgggtctttttcctaaaggatccacaacttcctgcagactatttggaagactaactgttgagatgccatgaaacggtcgctgggtaaagtcaatattctgcaatgggcctccaacactgtgacttcgagtcaaagacacatttcgctttgataaactattaggcacagatgaaattttcatagtttggacatctccactggctctctttatttcatcacttggttcaactgcagagcctgtttcttcagttatgatctggttatgttttgggaagtccataaagttgatcaagtcaggttctgctaaactggatacaggtttgtgctccaaggattcatttgccaatggaatgcttccactttgtaaactgtcaccagaggtacttggtttcaggaaaaagttcttgagagagcttttataagactaaccttgcagaacctctcaaatctttgaattctatattgagaagaggcaagaagttgcttttacagaatggacaagctgtattcaaatttgagtcatctgctgtccatccagccataatttcttcatcataaactaaagctccacaagctctacactgtgaacaactggacatcaaaacctccattgcacaattctgatagatgctagacatgctggtattttgagaagaaccatgatctgatttttcaaagtcttgccctttcatgcctcttggaaatggaacttcacctgttggataatgcagttttcctacatctccactactgctgctactgccaagacttgtgttgctctgggtaagttcactggggaccaaccctgagatacttgtgttaggcgatatattctcccccaaaatatggtcttctaggccagctgggaagctgtagtctctattagtttcttcctcatcatctgagtagctgtaggcagacgcaacagctacccacatcttactggctactgtcgctgcttgtttcataccagatttcaggacatctatcttgggccctgagagtatattatccagctttagccctgacaaagaatttactacagaacccaacgagccatgtggcgaagaacgcaccagtgctgacaaagaagttgaacgttctttatgagttcgagagggggtttgctgcttgaaacgcccagtaaaagttttagacctggacactgcaggtgagctcttttcactttcaggattttcctgtgctggtgaaccatgatctaaaggtaggcttgatctcctctctagagcatgaataaatgcagtagtcatgccagactctctgttttcctctctgtgtaattccatactagaagatttactacctaggggactttttaggttcatatagctttctatttcatcagccagattacgtgcaataactggagaaaacaacttatcttcagaatcaggagtttttcctcctgtacattcagtggctaaaagagacaaaggatctagtccagtttcaacatcttccctctgaaccaccttagcaataccatataaactacttctcttattcctcagatctttggatactgttttcaagtctctggactgattactgttactatcacttagtagactctcatatgtatctactgttgcagtagttttaggtacgtcatcaaccacaggctcaaggagttcttggctttcctcaagcatctctggcaccggagatgatctgtgctcaggattccaagtgctttcagacatacaagtcctactatcaggtaggtgacagctaacattctcaaagctatgggttcttgcaatatgaagtagagaagtcttaggacatgtcaatgctgctgtgagaatcttggcatctgctcccatcatgatagccatttcacttgaattcgaatccaaactactcttcttaagcaacattcctgctcgactttcagaactaaaactacaactcctctcaggaaaatgcttttgtcttttttctcctctatcaccattcttcttgagattagtagcttcgccaaagactgcatcttcaactggatcttgagtagaaaacagcacatttgatatactaccagtgctacttttcctgctgttgacatcaaatataccagacggaactttcacaatactgctgccccatgcaggaggttcagtaggactgtgaggctctggactaggttgtgaatgttttgccacaatagcagaggcatcacacacctcttctgtttgcatttttgttttagttatcaattctcttgctgcctgttcttcaggcacatgaatttctgcatcatcctttataagttcatccttagacccgtatccttggtcagactgaccacctgatattgaggagacctgtgacctttgcacagtctttttaagcggctgcctaaactgtgccaagccacgtaccacattccgtaccttcgtccataagaaaataccactgcgggtactgctaggccacgggctctccaagactaccttattataataaccataagtaatagcattaggctttatcctagcagttttcatttcaaataagactctcactgctaaaacaggatgaccccaaagtccacaaagctgcatcactactcgatagcacacctcatctaagggatccacatctgttttcctcatcttaataagtacatcatatgcctgctgaagtgctctgactttaggatgagaaactctaacataggccggaagacaaataaaccataaactgtaacaatgactaaacagacacttggcccactgtggtggatttgtataacatctcttcgccaatttatgagctgtttttatttcctgtttagttctcttagccatgagaggtggactctttgtaatgctattcccagtagggtgtctactaaaacaaagtttcaactcctgcggtctgtcaaaaagcttaaggtccagtcttggaaagtatttgtaactgtactttggtgacaggtcctttccatcatcaggaggtggctctggcggcattataaatacagtatgctcacttttctgtgaatcatctagttctatcaatctggtatcttctgctgaatcaaaatcaaccttatctgttttctctgtgcctttatcaggaaacaacttttctatgcagtcatcaaaaaatgctaatccagtatctttatcacttacaaaactgcattcttcaatgaaacgaataaaaatctgtgttttggataaaagggtatagaattttgcataggcacgatctcgactttttaaaaatccctgtcggtcaaacaatgaatcagcagctgtggctttatttgaaggagcctctgtgattggtctgagatatgttctatatccttttaaaatagacgccataaagcgcaaaaatgcctcttgaatttccatctcaagctgtgtcatcttcttttgccaggagaaatctgcttcaattggagtcatgtcaatcgctgagccttcttgagttttttggtgaactgaagacagctggggatacaatttctttaaggtgctaagtagatttttgcacggctttttgggaagttgcttccagttcatgttcttcttttcatctgatacatataacatgttcgtatccaagtcaatgcaaacaacatcttgtggtgggtcatgaagatcaaaataccttgagtcaactccaactataaatggtaaaggtgcactaagcactgcagccagtgaaagaggacaaaggggaatatatgggcattgccactgaaatggaaagatcatagctacaacagcttcagctaccccagtcaagacagctggcctaagagaatgcagcagaattttactctcaagtaaaacaaagagcagcagtgttgcacaattctcaggacccagattcattagcaaggtgctaaagttggctccacttagtggtaaaggtgtagaaactggctgtgataatattaatgcatcatggactgacagctggacaaggattctcggtctttgtggtgaaggaaaagggatgttttgcataaaatgtgaaatgtgcttttcaatgggaagaggatgtggtccagacacagaaagtttgtagataaacataagaaatttcctaaaagcttcaaaaaaaggccagtgtgagagtaaacaaatgcatttgtttgtattgatggatttggagaccatttttctctccacaggcgtcaacaagcccaggtgcataagctgtttctctgatagaagttcccgagagtaaggttcataaaactgaatggcagctccatatacctttttggctgaagaacctgtcaagacaaaagttgaaaaaactggaagtggatatttggtttcaggatcccagcactcaatagtagctcccataggaaggcagaaaagaggtacatctgattctgagagtggaaatgactcatagtcctcttctggatatctaaaaattaaaccagccttatatgctattgcatttgaagcaggtacagacttcttataacacagaaacacgctggaaccccacattccacaatttaagtttttgtcaactttgcagaaggtatgaggaggagtttctcctttactggttacaataacacagatatcagttacagccaaggaattctggggtcgaactggaggagcccttcgataagtgataaagattctttgtgaagtagttgaactattgttgacattggcacagcgaccatagggtgtggctaggatcacttcacatcctggaataagccgttctttcccttcatatagaactccaatatctgtaagcggtggtttatctctccctctcttataacagaggaaaagttctgggcttttcagacttccatagttcaagtttgcttggagagctgatggagtggcttctacacaggtgtaaccttcaggtactgtttctccagctgatttgataataatggcaatgtctgtaattggagctttaggtccagttgacttagtatctaaacgatttatttcttgatccaaaagagtagatgtgtcagtgagaccagctacgacaaagtagtctgtcactcttggtcctttgtcttctatcatggctgctactgtattttctgctgcctgctcctctgtcagcgcagccccgacacggcttcttcctggggcaagaaagcaccggattcgcggactgggcgcgctcggcagggcagggcgggggactagctccagcggccgccgccgcctcagtccggtct

SEQ ID NO: 8487 - RNA, 7268 nt, Homo sapiens
  source 1..7268: mol_type = other RNA
aaaagtaattgcggtttttgccattaatagtggcaaaaactacaattaattttgtgccaacctaatacattaaagttagggaaggcagctgtcatcagattttcaggtaattttaagattaatgactacagacaagtttagtagtagtcatttatttaatagtcaatgagacccctttcagaaaaccgtattgcaacatgcaatctattttaataaatatacacttagaatatggctgtatatacacatacctacacagccctacacatatacaaacttacacaaatatgttgctctcttttttttttttttttttttttgagacggtctcactctgtcacccaagctggagttgcagtggcgtgatctccactcactgtagcctctgcctcagttcaagcgattctcctgcctcagcctgagtagctgggactacagtggtgcgcctggctaatttttgtatttttagtaaagacagggtctcaccgtgttggccaggctggtctcgaactcctggcctcaagtgatccacccaccttgctcagcctcccaaagtgctgggattacaggcctgagccaccgtgcccggccatgttgcttttataattgagatatttcatttgttttgggggttaggcaaatttaatttgccattcctcaaactcagtaacttcaaatataaacaatgcctagaatgaatatggttcctcattatttctatcaaactactacaaatactgaagaatcccaaagtagttttccacagaggcagaaaagcagttcaggggttgaaaatcttcaatattaataagccctgggacattcaaatggcacttcatatttcaaggtaatgcaatatgaatcataattcattatatattgtccccaagagttacttcaattccgtattcaccagttcttacgatttggaaaaaaaaacttgaatgtttccagatgaaatctaatccccaagccttgtgtgtcaacattctagtgaatctctatttaaatgagaggcgctccaaaacacttcctgcaccactcgacactggcacttggtggagcatcaattttctgcaacctttcaagaatctctgaagacagactattgtatgcaattccatattcattgtcaaatgcctcaatatcaatattctctcttcctagagacactaatgataagaagaggatttctctgtataaactcctttgtcttttcatgcctggcttcatttgctgtgaaagtaggttgatgggtttaagaacattattgtgctgaatactctgcctgatggtttctactaaagtgcttgtttcttgttgttcctctgacaggagagatgatttcttttcagaattaaaattcctccatgagacatacagaggttctcttggttcctgatgaaggttgatattatcccataacagctgaatatacacaagtttgctatcctgggacagagatgacagaggaagctgtacaccttcattacaatgttcagatgtgaggataagtcctggcaagttactaggaaggtccaaacgtctgaaataccaaacgaggttccagaaaatgattggatgttgattgatgaaagaagatgtatgaatcacctgatcaccttcattttctagcaaagattcaagttctttacggagtactagaggactcaagtagggcacagaaacagggggaggattgggtctttttcctaaaggatccacaacttcctgcagactatttggaagactaactgttgagatgccatgaaacggtcgctgggtaaagtcaatattctgcaatgggcctccaacactgtgacttcgagtcaaagacacatttcgctttgataaactattaggcacagatgaaattttcatagtttggacatctccactggctctctttatttcatcacttggttcaactgcagagcctgtttcttcagttatgatctggttatgttttgggaagtccataaagttgatcaagtcaggttctgctaaactggatacaggtttgtgctccaaggattcatttgccaatggaatgcttccactttgtaaactgtcaccagaggtacttggtttcaggaaaaagttcttgagagagcttttataagactaaccttgcagaacctctcaaatctttgaattctatattgagaagaggcaagaagttgcttttacagaatggacaagctgtattcaaatttgagtcatctgctgtccatccagccataatttcttcatcataaactaaagctccacaagctctacactgtgaacaactggacatcaaaacctccattgcacaattctgatagatgctagacatgctggtattttgagaagaaccatgatctgatttttcaaagtcttgccctttcatgcctcttggaaatggaacttcacctgttggataatgcagttttcctacatctccactactgctgctactgccaagacttgtgttgctctgggtaagttcactggggaccaaccctgagatacttgtgttaggcgatatattctcccccaaaatatggtcttctaggccagctgggaagctgtagtctctattagtttcttcctcatcatctgagtagctgtaggcagacgcaacagctacccacatcttactggctactgtcgctgcttgtttcataccagatttcaggacatctatcttgggccctgagagtatattatccagctttagccctgacaaagaatttactacagaacccaacgagccatgtggcgaagaacgcaccagtgctgacaaagaagttgaacgttctttatgagttcgagagggggtttgctgcttgaaacgcccagtaaaagttttagacctggacactgcaggtgagctcttttcactttcaggattttcctgtgctggtgaaccatgatctaaaggtaggcttgatctcctctctagagcatgaataaatgcagtagtcatgccagactctctgttttcctctctgtgtaattccatactagaagatttactacctaggggactttttaggttcatatagctttctatttcatcagccagattacgtgcaataactggagaaaacaacttatcttcagaatcaggagtttttcctcctgtacattcagtggctaaaagagacaaaggatctagtccagtttcaacatcttccctctgaaccaccttagcaataccatataaactacttctcttattcctcagatctttggatactgttttcaagtctctggactgattactgttactatcacttagtagactctcatatgtatctactgttgcagtagttttaggtacgtcatcaaccacaggctcaaggagttcttggctttcctcaagcatctctggcaccggagatgatctgtgctcaggattccaagtgctttcagacatacaagtcctactatcaggtaggtgacagctaacattctcaaagctatgggttcttgcaatatgaagtagagaagtcttaggacatgtcaatgctgctgtgagaatcttggcatctgctcccatcatgatagccatttcacttgaattcgaatccaaactactcttcttaagcaacattcctgctcgactttcagaactaaaactacaactcctctcaggaaaatgcttttgtcttttttctcctctatcaccattcttcttgagattagtagcttcgccaaagactgcatcttcaactggatcttgagtagaaaacagcacatttgatatactaccagtgctacttttcctgctgttgacatcaaatataccagacggaactttcacaatactgctgccccatgcaggaggttcagtaggactgtgaggctctggactaggttgtgaatgttttgccacaatagcagaggcatcacacacctcttctgtttgcatttttgttttagttatcaattctcttgctgcctgttcttcaggcacatgaatttctgcatcatcctttataagttcatccttagacccgtatccttggtcagactgaccacctgtgctagagtgattatcaatggactcaagcctgattaaatctctgacgaagactgtgtgctccccattgttagcatcattagaactatccacactaccgtggctcaccgtgtccccatcacttccacctgtgacattttgaagagctgatattgaggagacctgtgacctttgcacagtctttttaagcggctgcctaaactgtgccaagccacgtaccacattccgtaccttcgtccataagaaaataccactgcgggtactgctaggccacgggctctccaagactaccttattataataaccataagtaatagcattaggctttatcctagcagttttcatttcaaataagactctcactgctaaaacaggatgaccccaaagtccacaaagctgcatcactactcgatagcacacctcatctaagggatccacatctgttttcctcatcttaataagtacatcatatgcctgctgaagtgctctgactttaggatgagaaactctaacataggccggaagacaaataaaccataaactgtaacaatgactaaacagacacttggcccactgtggtggatttgtataacatctcttcgccaatttatgagctgtttttatttcctgtttagttctcttagccatgagaggtggactctttgtaatgctattcccagtagggtgtctactaaaacaaagtttcaactcctgcggtctgtcaaaaagcttaaggtccagtcttggaaagtatttgtaactgtactttggtgacaggtcctttccatcatcaggaggtggctctggcggcattataaatacagtatgctcacttttctgtgaatcatctagttctatcaatctggtatcttctgctgaatcaaaatcaaccttatctgttttctctgtgcctttatcaggaaacaacttttctatgcagtcatcaaaaaatgctaatccagtatctttatcacttacaaaactgcattcttcaatgaaacgaataaaaatctgtgttttggataaaagggtatagaattttgcataggcacgatctcgactttttaaaaatccctgtcggtcaaacaatgaatcagcagctgtggctttatttgaaggagcctctgtgattggtctgagatatgttctatatccttttaaaatagacgccataaagcgcaaaaatgcctcttgaatttccatctcaagctgtgtcatcttcttttgccaggagaaatctgcttcaattggagtcatgtcaatcgctgagccttcttgagttttttggtgaactgaagacagctggggatacaatttctttaaggtgctaagtagatttttgcacggctttttgggaagttgcttccagttcatgttcttcttttcatctgatacatataacatgttcgtatccaagtcaatgcaaacaacatcttgtggtgggtcatgaagatcaaaataccttgagtcaactccaactataaatggtaaaggtgcactaagcactgcagccagtgaaagaggacaaaggggaatatatgggcattgccactgaaatggaaagatcatagctacaacagcttcagctaccccagtcaagacagctggcctaagagaatgcagcagaattttactctcaagtaaaacaaagagcagcagtgttgcacaattctcaggacccagattcattagcaaggtgctaaagttggctccacttagtggtaaaggtgtagaaactggctgtgataatattaatgcatcatggactgacagctggacaaggattctcggtctttgtggtgaaggaaaagggatgttttgcataaaatgtgaaatgtgcttttcaatgggaagaggatgtggtccagacacagaaagtttgtagataaacataagaaatttcctaaaagcttcaaaaaaaggccagtgtgagagtaaacaaatgcatttgtttgtattgatggatttggagaccatttttctctccacaggcgtcaacaagcccaggtgcataagctgtttctctgatagaagttcccgagagtaaggttcataaaactgaatggcagctccatatacctttttggctgaagaacctgtcaagacaaaagttgaaaaaactggaagtggatatttggtttcaggatcccagcactcaatagtagctcccataggaaggcagaaaagaggtacatctgattctgagagtggaaatgactcatagtcctcttctggatatctaaaaattaaacctgtattttcagtttttatcccaccataccagtggaatgaagacgtgacacttaaatctttacagcccttgacactttaatgtgcagtaagaatgtggcgatagatttctcaaacacttcatggcagaaaagtttctcaggccctcctctcctccatatagctgattctttgcaacaaaggagaaaggaagcaagtccaccagccttatatgctattgcatttgaagcaggtacagacttcttataacacagaaacacgctggaaccccacattccacaatttaagtttttgtcaactttgcagaaggtatgaggaggagtttctcctttactggttacaataacacagatatcagttacagccaaggaattctggggtcgaactggaggagcccttcgataagtgataaagattctttgtgaagtagttgaactattgttgacattggcacagcgaccatagggtgtggctaggatcacttcacatcctggaataagccgttctttcccttcatatagaactccaatatctgtaagcggtggtttatctctccctctcttataacagaggaaaagttctgggcttttcagacttccatagttcaagtttgcttggagagctgatggagtggcttctacacaggtgtaaccttcaggtactgtttctccagctgatttgataataatggcaatgtctgtaattggagctttaggtccagttgacttagtatctaaacgatttatttcttgatccaaaagagtagatgtgtcagtgagaccagctacgacaaagtagtctgtcactcttggtcctttgtcttctatcatggctgctactgtattttctgctgcctgctcctctgtcagcgcagccccgacacggcttcttcctggggcaagaaagcaccggattcgcggactgggcgcgctcggcagggcagggcgggggactagctccagcggccgccgccgcctcagtccggtct

SEQ ID NO: 8488 - RNA, 6622 nt, Homo sapiens
  source 1..6622: mol_type = other RNA
aaaagtaattgcggtttttgccattaatagtggcaaaaactacaattaattttgtgccaacctaatacattaaagttagggaaggcagctgtcatcagattttcaggtaattttaagattaatgactacagacaagtttagtagtagtcatttatttaatagtcaatgagacccctttcagaaaaccgtattgcaacatgcaatctattttaataaatatacacttagaatatggctgtatatacacatacctacacagccctacacatatacaaacttacacaaatatgttgctctcttttttttttttttttttttttgagacggtctcactctgtcacccaagctggagttgcagtggcgtgatctccactcactgtagcctctgcctcagttcaagcgattctcctgcctcagcctgagtagctgggactacagtggtgcgcctggctaatttttgtatttttagtaaagacagggtctcaccgtgttggccaggctggtctcgaactcctggcctcaagtgatccacccaccttgctcagcctcccaaagtgctgggattacaggcctgagccaccgtgcccggccatgttgcttttataattgagatatttcatttgttttgggggttaggcaaatttaatttgccattcctcaaactcagtaacttcaaatataaacaatgcctagaatgaatatggttcctcattatttctatcaaactactacaaatactgaagaatcccaaagtagttttccacagaggcagaaaagcagttcaggggttgaaaatcttcaatattaataagccctgggacattcaaatggcacttcatatttcaaggtaatgcaatatgaatcataattcattatatattgtccccaagagttacttcaattccgtattcaccagttcttacgatttggaaaaaaaaacttgaatgtttccagatgaaatctaatccccaagccttgtgtgtcaacattctagtgaatctctatttaaatgagaggcgctccaaaacacttcctgcaccactcgacactggcacttggtggagcatcaattttctgcaacctttcaagaatctctgaagacagactattgtatgcaattccatattcattgtcaaatgcctcaatatcaatattctctcttcctagagacactaatgataagaagaggatttctctgtataaactcctttgtcttttcatgcctggcttcatttgctgtgaaagtaggttgatgggtttaagaacattattgtgctgaatactctgcctgatggtttctactaaagtgcttgtttcttgttgttcctctgacaggagagatgatttcttttcagaattaaaattcctccatgagacatacagaggttctcttggttcctgatgaaggttgatattatcccataacagctgaatatacacaagtttgctatcctgggacagagatgacagaggaagctgtacaccttcattacaatgttcagatgtgaggataagtcctggcaagttactaggaaggtccaaacgtctgaaataccaaacgaggttccagaaaatgattggatgttgattgatgaaagaagatgtatgaatcacctgatcaccttcattttctagcaaagattcaagttctttacggagtactagaggactcaagtagggcacagaaacagggggaggattgggtctttttcctaaaggatccttgcagaacctctcaaatctttgaattctatattgagaagaggcaagaagttgcttttacagaatggacaagctgtattcaaatttgagtcatctgctgtccatccagccataatttcttcatcataaactaaagctccacaagctctacactgtgaacaactggacatcaaaacctccattgcacaattctgatagatgctagacatgctggtattttgagaagaaccatgatctgatttttcaaagtcttgccctttcatgcctcttggaaatggaacttcacctgttggataatgcagttttcctacatctccactactgctgctactgccaagacttgtgttgctctgggtaagttcactggggaccaaccctgagatacttgtgttaggcgatatattctcccccaaaatatggtcttctaggccagctgggaagctgtagtctctattagtttcttcctcatcatctgagtagctgtaggcagacgcaacagctacccacatcttactggctactgtcgctgcttgtttcataccagatttcaggacatctatcttgggccctgagagtatattatccagctttagccctgacaaagaatttactacagaacccaacgagccatgtggcgaagaacgcaccagtgctgacaaagaagttgaacgttctttatgagttcgagagggggtttgctgcttgaaacgcccagtaaaagttttagacctggacactgcaggtgagctcttttcactttcaggattttcctgtgctggtgaaccatgatctaaaggtaggcttgatctcctctctagagcatgaataaatgcagtagtcatgccagactctctgttttcctctctgtgtaattccatactagaagatttactacctaggggactttttaggttcatatagctttctatttcatcagccagattacgtgcaataactggagaaaacaacttatcttcagaatcaggagtttttcctcctgtacattcagtggctaaaagagacaaaggatctagtccagtttcaacatcttccctctgaaccaccttagcaataccatataaactacttctcttattcctcagatctttggatactgttttcaagtctctggactgattactgttactatcacttagtagactctcatatgtatctactgttgcagtagttttaggtacgtcatcaaccacaggctcaaggagttcttggctttcctcaagcatctctggcaccggagatgatctgtgctcaggattccaagtgctttcagacatacaagtcctactatcaggtaggtgacagctaacattctcaaagctatgggttcttgcaatatgaagtagagaagtcttaggacatgtcaatgctgctgtgagaatcttggcatctgctcccatcatgatagccatttcacttgaattcgaatccaaactactcttcttaagcaacattcctgctcgactttcagaactaaaactacaactcctctcaggaaaatgcttttgtcttttttctcctctatcaccattcttcttgagattagtagcttcgccaaagactgcatcttcaactggatcttgagtagaaaacagcacatttgatatactaccagtgctacttttcctgctgttgacatcaaatataccagacggaactttcacaatactgctgccccatgcaggaggttcagtaggactgtgaggctctggactaggttgtgaatgttttgccacaatagcagaggcatcacacacctcttctgtttgcatttttgttttagttatcaattctcttgctgcctgttcttcaggcacatgaatttctgcatcatcctttataagttcatccttagacccgtatccttggtcagactgaccacctgtgctagagtgattatcaatggactcaagcctgattaaatctctgacgaagactgtgtgctccccattgttagcatcattagaactatccacactaccgtggctcaccgtgtccccatcacttccacctgtgacattttgaagagctgatattgaggagacctgtgacctttgcacagtctttttaagcggctgcctaaactgtgccaagccacgtaccacattccgtaccttcgtccataagaaaataccactgcgggtactgctaggccacgggctctccaagactaccttattataataaccataagtaatagcattaggctttatcctagcagttttcatttcaaataagactctcactgctaaaacaggatgaccccaaagtccacaaagctgcatcactactcgatagcacacctcatctaagggatccacatctgttttcctcatcttaataagtacatcatatgcctgctgaagtgctctgactttaggatgagaaactctaacataggccggaagacaaataaaccataaactgtaacaatgactaaacagacacttggcccactgtggtggatttgtataacatctcttcgccaatttatgagctgtttttatttcctgtttagttctcttagccatgagaggtggactctttgtaatgctattcccagtagggtgtctactaaaacaaagtttcaactcctgcggtctgtcaaaaagcttaaggtccagtcttggaaagtatttgtaactgtactttggtgacaggtcctttccatcatcaggaggtggctctggcggcattataaatacagtatgctcacttttctgtgaatcatctagttctatcaatctggtatcttctgctgaatcaaaatcaaccttatctgttttctctgtgcctttatcaggaaacaacttttctatgcagtcatcaaaaaatgctaatccagtatctttatcacttacaaaactgcattcttcaatgaaacgaataaaaatctgtgttttggataaaagggtatagaattttgcataggcacgatctcgactttttaaaaatccctgtcggtcaaacaatgaatcagcagctgtggctttatttgaaggagcctctgtgattggtctgagatatgttctatatccttttaaaatagacgccataaagcgcaaaaatgcctcttgaatttccatctcaagctgtgtcatcttcttttgccaggagaaatctgcttcaattggagtcatgtcaatcgctgagccttcttgagttttttggtgaactgaagacagctggggatacaatttctttaaggtgctaagtagatttttgcacggctttttgggaagttgcttccagttcatgttcttcttttcatctgatacatataacatgttcgtatccaagtcaatgcaaacaacatcttgtggtgggtcatgaagatcaaaataccttgagtcaactccaactataaatggtaaaggtgcactaagcactgcagccagtgaaagaggacaaaggggaatatatgggcattgccactgaaatggaaagatcatagctacaacagcttcagctaccccagtcaagacagctggcctaagagaatgcagcagaattttactctcaagtaaaacaaagagcagcagtgttgcacaattctcaggacccagattcattagcaaggtgctaaagttggctccacttagtggtaaaggtgtagaaactggctgtgataatattaatgcatcatggactgacagctggacaaggattctcggtctttgtggtgaaggaaaagggatgttttgcataaaatgtgaaatgtgcctttttggctgaagaacctgtcaagacaaaagttgaaaaaactggaagtggatatttggtttcaggatcccagcactcaatagtagctcccataggaaggcagaaaagaggtacatctgattctgagagtggaaatgactcatagtcctcttctggatatctaaaaattaaacctgtattttcagtttttatcccaccataccagtggaatgaagacgtgacacttaaatctttacagcccttgacactttaatgtgcagtaagaatgtggcgatagatttctcaaacacttcatggcagaaaagtttctcaggccctcctctcctccatatagctgattctttgcaacaaaggagaaaggaagcaagtccaccagccttatatgctattgcatttgaagcaggtacagacttcttataacacagaaacacgctggaaccccacattccacaatttaagtttttgtcaactttgcagaaggtatgaggaggagtttctcctttactggttacaataacacagatatcagttacagccaaggaattctggggtcgaactggaggagcccttcgataagtgataaagattctttgtgaagtagttgaactattgttgacattggcacagcgaccatagggtgtggctaggatcacttcacatcctggaataagccgttctttcccttcatatagaactccaatatctgtaagcggtggtttatctctccctctcttataacagaggaaaagttctgggcttttcagacttccatagttcaagtttgcttggagagctgatggagtggcttctacacaggtgtaaccttcaggtactgtttctccagctgatttgataataatggcaatgtctgtaattggagctttaggtccagttgacttagtatctaaacgatttatttcttgatccaaaagagtagatgtgtcagtgagaccagctacgacaaagtagtctgtcactcttggtcctttgtcttctatcatggctgctactgtattttctgctgcctgctcctctgtcagcgcagccccgacacggcttcttcctggggcaagaaagcaccggattcgcggactgggcgcgctcggcagggcagggcgggggactagctccagcggccgccgccgcctcagtccggtct

SEQ ID NO: 8489 - RNA, 7024 nt, Homo sapiens
  source 1..7024: mol_type = other RNA
aaaagtaattgcggtttttgccattaatagtggcaaaaactacaattaattttgtgccaacctaatacattaaagttagggaaggcagctgtcatcagattttcaggtaattttaagattaatgactacagacaagtttagtagtagtcatttatttaatagtcaatgagacccctttcagaaaaccgtattgcaacatgcaatctattttaataaatatacacttagaatatggctgtatatacacatacctacacagccctacacatatacaaacttacacaaatatgttgctctcttttttttttttttttttttttgagacggtctcactctgtcacccaagctggagttgcagtggcgtgatctccactcactgtagcctctgcctcagttcaagcgattctcctgcctcagcctgagtagctgggactacagtggtgcgcctggctaatttttgtatttttagtaaagacagggtctcaccgtgttggccaggctggtctcgaactcctggcctcaagtgatccacccaccttgctcagcctcccaaagtgctgggattacaggcctgagccaccgtgcccggccatgttgcttttataattgagatatttcatttgttttgggggttaggcaaatttaatttgccattcctcaaactcagtaacttcaaatataaacaatgcctagaatgaatatggttcctcattatttctatcaaactactacaaatactgaagaatcccaaagtagttttccacagaggcagaaaagcagttcaggggttgaaaatcttcaatattaataagccctgggacattcaaatggcacttcatatttcaaggtaatgcaatatgaatcataattcattatatattgtccccaagagttacttcaattccgtattcaccagttcttacgatttggaaaaaaaaacttgaatgtttccagatgaaatctaatccccaagccttgtgtgtcaacattctagtgaatctctatttaaatgagaggcgctccaaaacacttcctgcaccactcgacactggcacttggtggagcatcaattttctgcaacctttcaagaatctctgaagacagactattgtatgcaattccatattcattgtcaaatgcctcaatatcaatattctctcttcctagagacactaatgataagaagaggatttctctgtataaactcctttgtcttttcatgcctggcttcatttgctgtgaaagtaggttgatgggtttaagaacattattgtgctgaatactctgcctgatggtttctactaaagtgcttgtttcttgttgttcctctgacaggagagatgatttcttttcagaattaaaattcctccatgagacatacagaggttctcttggttcctgatgaaggttgatattatcccataacagctgaatatacacaagtttgctatcctgggacagagatgacagaggaagctgtacaccttcattacaatgttcagatgtgaggataagtcctggcaagttactaggaaggtccaaacgtctgaaataccaaacgaggttccagaaaatgattggatgttgattgatgaaagaagatgtatgaatcacctgatcaccttcattttctagcaaagattcaagttctttacggagtactagaggactcaagtagggcacagaaacagggggaggattgggtctttttcctaaaggatccttggttcaactgcagagcctgtttcttcagttatgatctggttatgttttgggaagtccataaagttgatcaagtcaggttctgctaaactggatacaggtttgtgctccaaggattcatttgccaatggaatgcttccactttgtaaactgtcaccagaggtacttggtttcaggaaaaagcttgcagaacctctcaaatctttgaattctatattgagaagaggcaagaagttgcttttacagaatggacaagctgtattcaaatttgagtcatctgctgtccatccagccataatttcttcatcataaactaaagctccacaagctctacactgtgaacaactggacatcaaaacctccattgcacaattctgatagatgctagacatgctggtattttgagaagaaccatgatctgatttttcaaagtcttgccctttcatgcctcttggaaatggaacttcacctgttggataatgcagttttcctacatctccactactgctgctactgccaagacttgtgttgctctgggtaagttcactggggaccaaccctgagatacttgtgttaggcgatatattctcccccaaaatatggtcttctaggccagctgggaagctgtagtctctattagtttcttcctcatcatctgagtagctgtaggcagacgcaacagctacccacatcttactggctactgtcgctgcttgtttcataccagatttcaggacatctatcttgggccctgagagtatattatccagctttagccctgacaaagaatttactacagaacccaacgagccatgtggcgaagaacgcaccagtgctgacaaagaagttgaacgttctttatgagttcgagagggggtttgctgcttgaaacgcccagtaaaagttttagacctggacactgcaggtgagctcttttcactttcaggattttcctgtgctggtgaaccatgatctaaaggtaggcttgatctcctctctagagcatgaataaatgcagtagtcatgccagactctctgttttcctctctgtgtaattccatactagaagatttactacctaggggactttttaggttcatatagctttctatttcatcagccagattacgtgcaataactggagaaaacaacttatcttcagaatcaggagtttttcctcctgtacattcagtggctaaaagagacaaaggatctagtccagtttcaacatcttccctctgaaccaccttagcaataccatataaactacttctcttattcctcagatctttggatactgttttcaagtctctggactgattactgttactatcacttagtagactctcatatgtatctactgttgcagtagttttaggtacgtcatcaaccacaggctcaaggagttcttggctttcctcaagcatctctggcaccggagatgatctgtgctcaggattccaagtgctttcagacatacaagtcctactatcaggtaggtgacagctaacattctcaaagctatgggttcttgcaatatgaagtagagaagtcttaggacatgtcaatgctgctgtgagaatcttggcatctgctcccatcatgatagccatttcacttgaattcgaatccaaactactcttcttaagcaacattcctgctcgactttcagaactaaaactacaactcctctcaggaaaatgcttttgtcttttttctcctctatcaccattcttcttgagattagtagcttcgccaaagactgcatcttcaactggatcttgagtagaaaacagcacatttgatatactaccagtgctacttttcctgctgttgacatcaaatataccagacggaactttcacaatactgctgccccatgcaggaggttcagtaggactgtgaggctctggactaggttgtgaatgttttgccacaatagcagaggcatcacacacctcttctgtttgcatttttgttttagttatcaattctcttgctgcctgttcttcaggcacatgaatttctgcatcatcctttataagttcatccttagacccgtatccttggtcagactgaccacctgtgctagagtgattatcaatggactcaagcctgattaaatctctgacgaagactgtgtgctccccattgttagcatcattagaactatccacactaccgtggctcaccgtgtccccatcacttccacctgtgacattttgaagagctgatattgaggagacctgtgacctttgcacagtctttttaagcggctgcctaaactgtgccaagccacgtaccacattccgtaccttcgtccataagaaaataccactgcgggtactgctaggccacgggctctccaagactaccttattataataaccataagtaatagcattaggctttatcctagcagttttcatttcaaataagactctcactgctaaaacaggatgaccccaaagtccacaaagctgcatcactactcgatagcacacctcatctaagggatccacatctgttttcctcatcttaataagtacatcatatgcctgctgaagtgctctgactttaggatgagaaactctaacataggccggaagacaaataaaccataaactgtaacaatgactaaacagacacttggcccactgtggtggatttgtataacatctcttcgccaatttatgagctgtttttatttcctgtttagttctcttagccatgagaggtggactctttgtaatgctattcccagtagggtgtctactaaaacaaagtttcaactcctgcggtctgtcaaaaagcttaaggtccagtcttggaaagtatttgtaactgtactttggtgacaggtcctttccatcatcaggaggtggctctggcggcattataaatacagtatgctcacttttctgtgaatcatctagttctatcaatctggtatcttctgctgaatcaaaatcaaccttatctgttttctctgtgcctttatcaggaaacaacttttctatgcagtcatcaaaaaatgctaatccagtatctttatcacttacaaaactgcattcttcaatgaaacgaataaaaatctgtgttttggataaaagggtatagaattttgcataggcacgatctcgactttttaaaaatccctgtcggtcaaacaatgaatcagcagctgtggctttatttgaaggagcctctgtgattggtctgagatatgttctatatccttttaaaatagacgccataaagcgcaaaaatgcctcttgaatttccatctcaagctgtgtcatcttcttttgccaggagaaatctgcttcaattggagtcatgtcaatcgctgagccttcttgagttttttggtgaactgaagacagctggggatacaatttctttaaggtgctaagtagatttttgcacggctttttgggaagttgcttccagttcatgttcttcttttcatctgatacatataacatgttcgtatccaagtcaatgcaaacaacatcttgtggtgggtcatgaagatcaaaataccttgagtcaactccaactataaatggtaaaggtgcactaagcactgcagccagtgaaagaggacaaaggggaatatatgggcattgccactgaaatggaaagatcatagctacaacagcttcagctaccccagtcaagacagctggcctaagagaatgcagcagaattttactctcaagtaaaacaaagagcagcagtgttgcacaattctcaggacccagattcattagcaaggtgctaaagttggctccacttagtggtaaaggtgtagaaactggctgtgataatattaatgcatcatggactgacagctggacaaggattctcggtctttgtggtgaaggaaaagggatgttttgcataaaatgtgaaatgtgcttttcaatgggaagaggatgtggtccagacacagaaagtttgtagataaacataagaaatttcctaaaagcttcaaaaaaaggccagtgtgagagtaaacaaatgcatttgtttgtattgatggatttggagaccatttttctctccacaggcgtcaacaagcccaggtgcataagctgtttctctgatagaagttcccgagagtaaggttcataaaactgaatggcagctccatatacctttttggctgaagaacctgtcaagacaaaagttgaaaaaactggaagtggatatttggtttcaggatcccagcactcaatagtagctcccataggaaggcagaaaagaggtacatctgattctgagagtggaaatgactcatagtcctcttctggatatctaaaaattaaaccagccttatatgctattgcatttgaagcaggtacagacttcttataacacagaaacacgctggaaccccacattccacaatttaagtttttgtcaactttgcagaaggtatgaggaggagtttctcctttactggttacaataacacagatatcagttacagccaaggaattctggggtcgaactggaggagcccttcgataagtgataaagattctttgtgaagtagttgaactattgttgacattggcacagcgaccatagggtgtggctaggatcacttcacatcctggaataagccgttctttcccttcatatagaactccaatatctgtaagcggtggtttatctctccctctcttataacagaggaaaagttctgggcttttcagacttccatagttcaagtttgcttggagagctgatggagtggcttctacacaggtgtaaccttcaggtactgtttctccagctgatttgataataatggcaatgtctgtaattggagctttaggtccagttgacttagtatctaaacgatttatttcttgatccaaaagagtagatgtgtcagtgagaccagctacgacaaagtagtctgtcactcttggtcctttgtcttctatcatggctgctactgtattttctgctgcctgctcctctgtcagcgcagccccgacacggcttcttcctggggcaagaaagcaccggattcgcggactgggcgcgctcggcagggcagggcgggggactagctccagcggccgccgccgcctcagtccggtctgcgcctgcgccgcctcgcgggcagggtctccgaggggcgccgcctacagccaggggcgatggccggagcgctggcccgcgcgggtgcctccgcgctgtgagccgtcggacagtgcgggcggcgcgtcgcctaggagctgcccgcggcgcagccgtcccaagacctgaccgccatgtttct

SEQ ID NO: 8490 - RNA, 6575 nt, Homo sapiens
  source 1..6575: mol_type = other RNA
aaaagtaattgcggtttttgccattaatagtggcaaaaactacaattaattttgtgccaacctaatacattaaagttagggaaggcagctgtcatcagattttcaggtaattttaagattaatgactacagacaagtttagtagtagtcatttatttaatagtcaatgagacccctttcagaaaaccgtattgcaacatgcaatctattttaataaatatacacttagaatatggctgtatatacacatacctacacagccctacacatatacaaacttacacaaatatgttgctctcttttttttttttttttttttttgagacggtctcactctgtcacccaagctggagttgcagtggcgtgatctccactcactgtagcctctgcctcagttcaagcgattctcctgcctcagcctgagtagctgggactacagtggtgcgcctggctaatttttgtatttttagtaaagacagggtctcaccgtgttggccaggctggtctcgaactcctggcctcaagtgatccacccaccttgctcagcctcccaaagtgctgggattacaggcctgagccaccgtgcccggccatgttgcttttataattgagatatttcatttgttttgggggttaggcaaatttaatttgccattcctcaaactcagtaacttcaaatataaacaatgcctagaatgaatatggttcctcattatttctatcaaactactacaaatactgaagaatcccaaagtagttttccacagaggcagaaaagcagttcaggggttgaaaatcttcaatattaataagccctgggacattcaaatggcacttcatatttcaaggtaatgcaatatgaatcataattcattatatattgtccccaagagttacttcaattccgtattcaccagttcttacgatttggaaaaaaaaacttgaatgtttccagatgaaatctaatccccaagccttgtgtgtcaacattctagtgaatctctatttaaatgagaggcgctccaaaacacttcctgcaccactcgacactggcacttggtggagcatcaattttctgcaacctttcaagaatctctgaagacagactattgtatgcaattccatattcattgtcaaatgcctcaatatcaatattctctcttcctagagacactaatgataagaagaggatttctctgtataaactctaaaattcctccatgagacatacagaggttctcttggttcctgatgaaggttgatattatcccataacagctgaatatacacaagtttgctatcctgggacagagatgacagaggaagctgtacaccttcattacaatgttcagatgtgaggataagtcctggcaagttactaggaaggtccaaacgtctgaaataccaaacgaggttccagaaaatgattggatgttgattgatgaaagaagatgtatgaatcacctgatcaccttcattttctagcaaagattcaagttctttacggagtactagaggactcaagtagggcacagaaacagggggaggattgggtctttttcctaaaggatccacaacttcctgcagactatttggaagactaactgttgagatgccatgaaacggtcgctgggtaaagtcaatattctgcaatgggcctccaacactgtgacttcgagtcaaagacacatttcgctttgataaactattaggcacagatgaaattttcatagtttggacatctccactggctctctttatttcatcacttggttcaactgcagagcctgtttcttcagttatgatctggttatgttttgggaagtccataaagttgatcaagtcaggttctgctaaactggatacaggtttgtgctccaaggattcatttgccaatggaatgcttccactttgtaaactgtcaccagaggtacttggtttcaggaaaaagcttgcagaacctctcaaatctttgaattctatattgagaagaggcaagaagttgcttttacagaatggacaagctgtattcaaatttgagtcatctgctgtccatccagccataatttcttcatcataaactaaagctccacaagctctacactgtgaacaactggacatcaaaacctccattgcacaattctgatagatgctagacatgctggtattttgagaagaaccatgatctgatttttcaaagtcttgccctttcatgcctcttggaaatggaacttcacctgttggataatgcagttttcctacatctccactactgctgctactgccaagacttgtgttgctctgggtaagttcactggggaccaaccctgagatacttgtgttaggcgatatattctcccccaaaatatggtcttctaggccagctgggaagctgtagtctctattagtttcttcctcatcatctgagtagctgtaggcagacgcaacagctacccacatcttactggctactgtcgctgcttgtttcataccagatttcaggacatctatcttgggccctgagagtatattatccagctttagccctgacaaagaatttactacagaacccaacgagccatgtggcgaagaacgcaccagtgctgacaaagaagttgaacgttctttatgagttcgagagggggtttgctgcttgaaacgcccagtaaaagttttagacctggacactgcaggtgagctcttttcactttcaggattttcctgtgctggtgaaccatgatctaaaggtaggcttgatctcctctctagagcatgaataaatgcagtagtcatgccagactctctgttttcctctctgtgtaattccatactagaagatttactacctaggggactttttaggttcatatagctttctatttcatcagccagattacgtgcaataactggagaaaacaacttatcttcagaatcaggagtttttcctcctgtacattcagtggctaaaagagacaaaggatctagtccagtttcaacatcttccctctgaaccaccttagcaataccatataaactacttctcttattcctcagatctttggatactgttttcaagtctctggactgattactgttactatcacttagtagactctcatatgtatctactgttgcagtagttttaggtacgtcatcaaccacaggctcaaggagttcttggctttcctcaagcatctctggcaccggagatgatctgtgctcaggattccaagtgctttcagacatacaagtcctactatcaggtaggtgacagctaacattctcaaagctatgggttcttgcaatatgaagtagagaagtcttaggacatgtcaatgctgctgtgagaatcttggcatctgctcccatcatgatagccatttcacttgaattcgaatccaaactactcttcttaagcaacattcctgctcgactttcagaactaaaactacaactcctctcaggaaaatgcttttgtcttttttctcctctatcaccattcttcttgagattagtagcttcgccaaagactgcatcttcaactggatcttgagtagaaaacagcacatttgatatactaccagtgctacttttcctgctgttgacatcaaatataccagacggaactttcacaatactgctgccccatgcaggaggttcagtaggactgtgaggctctggactaggttgtgaatgttttgccacaatagcagaggcatcacacacctcttctgtttgcatttttgttttagttatcaattctcttgctgcctgttcttcaggcacatgaatttctgcatcatcctttataagttcatccttagacccgtatccttggtcagactgaccacctgatgtggttaacattcaagggtagaattaatgcacacgtgtatccatagcttcacgtcatataagtctgtctgatattgaggagacctgtgacctttgcacagtctttttaagcggctgcctaaactgtgccaagccacgtaccacattccgtaccttcgtccataagaaaataccactgcgggtactgctaggccacgggctctccaagactaccttattataataaccataagtaatagcattaggctttatcctagcagttttcatttcaaataagactctcactgctaaaacaggatgaccccaaagtccacaaagctgcatcactactcgatagcacacctcatctaagggatccacatctgttttcctcatcttaataagtacatcatatgcctgctgaagtgctctgactttaggatgagaaactctaacataggccggaagacaaataaaccataaactgtaacaatgactaaacagacacttggcccactgtggtggatttgtataacatctcttcgccaatttatgagctgtttttatttcctgtttagttctcttagccatgagaggtggactctttgtaatgctattcccagtagggtgtctactaaaacaaagtttcaactcctgcggtctgtcaaaaagcttaaggtccagtcttggaaagtatttgtaactgtactttggtgacaggtcctttccatcatcaggaggtggctctggcggcattataaatacagtatgctcacttttctgtgaatcatctagttctatcaatctggtatcttctgctgaatcaaaatcaaccttatctgttttctctgtgcctttatcaggaaacaacttttctatgcagtcatcaaaaaatgctaatccagtatctttatcacttacaaaactgcattcttcaatgaaacgaataaaaatctgtgttttggataaaagggtatagaattttgcataggcacgatctcgactttttaaaaatccctgtcggtcaaacaatgaatcagcagctgtggctttatttgaaggagcctctgtgattggtctgagatatgttctatatccttttaaaatagacgccataaagcgcaaaaatgcctcttgaatttccatctcaagctgtgtcatcttcttttgccaggagaaatctgcttcaattggagtcatgtcaatcgctgagccttcttgagttttttggtgaactgaagacagctggggatacaatttctttaaggtgctaagtagatttttgcacggctttttgggaagttgcttccagttcatgttcttcttttcatctgatacatataacatgttcgtatccaagtcaatgcaaacaacatcttgtggtgggtcatgaagatcaaaataccttgagtcaactccaactataaatggtaaaggtgcactaagcactgcagccagtgaaagaggacaaaggggaatatatgggcattgccactgaaatggaaagatcatagctacaacagcttcagctaccccagtcaagacagctggcctaagagaatgcagcagaattttactctcaagtaaaacaaagagcagcagtgttgcacaattctcaggacccagattcattagcaaggtgctaaagttggctccacttagtggtaaaggtgtagaaactggctgtgataatattaatgcatcatggactgacagctggacaaggattctcggtctttgtggtgaaggaaaagggatgttttgcataaaatgtgaaatgtgcctttttggctgaagaacctgtcaagacaaaagttgaaaaaactggaagtggatatttggtttcaggatcccagcactcaatagtagctcccataggaaggcagaaaagaggtacatctgattctgagagtggaaatgactcatagtcctcttctggatatctaaaaattaaaccagccttatatgctattgcatttgaagcaggtacagacttcttataacacagaaacacgctggaaccccacattccacaatttaagtttttgtcaactttgcagaaggtatgaggaggagtttctcctttactggttacaataacacagatatcagttacagccaaggaattctggggtcgaactggaggagcccttcgataagtgataaagattctttgtgaagtagttgaactattgttgacattggcacagcgaccatagggtgtggctaggatcacttcacatcctggaataagccgttctttcccttcatatagaactccaatatctgtaagcggtggtttatctctccctctcttataacagaggaaaagttctgggcttttcagacttccatagttcaagtttgcttggagagctgatggagtggcttctacacaggtgtaaccttcaggtactgtttctccagctgatttgataataatggcaatgtctgtaattggagctttaggtccagttgacttagtatctaaacgatttatttcttgatccaaaagagtagatgtgtcagtgagaccagctacgacaaagtagtctgtcactcttggtcctttgtcttctatcatggctgctactgtattttctgctgcctgctcctctgtcagcgcagccccgacacggcttcttcctggggcaagaaagcaccggattcgcggactgggcgcgctcggcagggcagggcgggggactagctccagcggccgccgccgcctcagtccggtct

SEQ ID NO: 8491 - RNA, 6682 nt, Homo sapiens
  source 1..6682: mol_type = other RNA
aaaagtaattgcggtttttgccattaatagtggcaaaaactacaattaattttgtgccaacctaatacattaaagttagggaaggcagctgtcatcagattttcaggtaattttaagattaatgactacagacaagtttagtagtagtcatttatttaatagtcaatgagacccctttcagaaaaccgtattgcaacatgcaatctattttaataaatatacacttagaatatggctgtatatacacatacctacacagccctacacatatacaaacttacacaaatatgttgctctcttttttttttttttttttttttgagacggtctcactctgtcacccaagctggagttgcagtggcgtgatctccactcactgtagcctctgcctcagttcaagcgattctcctgcctcagcctgagtagctgggactacagtggtgcgcctggctaatttttgtatttttagtaaagacagggtctcaccgtgttggccaggctggtctcgaactcctggcctcaagtgatccacccaccttgctcagcctcccaaagtgctgggattacaggcctgagccaccgtgcccggccatgttgcttttataattgagatatttcatttgttttgggggttaggcaaatttaatttgccattcctcaaactcagtaacttcaaatataaacaatgcctagaatgaatatggttcctcattatttctatcaaactactacaaatactgaagaatcccaaagtagttttccacagaggcagaaaagcagttcaggggttgaaaatcttcaatattaataagccctgggacattcaaatggcacttcatatttcaaggtaatgcaatatgaatcataattcattatatattgtccccaagagttacttcaattccgtattcaccagttcttacgatttggaaaaaaaaacttgaatgtttccagatgaaatctaatccccaagccttgtgtgtcaacattctagtgaatctctatttaaatgagaggcgctccaaaacacttcctgcaccactcgacactggcacttggtggagcatcaattttctgcaacctttcaagaatctctgaagacagactattgtatgcaattccatattcattgtcaaatgcctcaatatcaatattctctcttcctagagacactaatgataagaagaggatttctctgtataaactctaaaattcctccatgagacatacagaggttctcttggttcctgatgaaggttgatattatcccataacagctgaatatacacaagtttgctatcctgggacagagatgacagaggaagctgtacaccttcattacaatgttcagatgtgaggataagtcctggcaagttactaggaaggtccaaacgtctgaaataccaaacgaggttccagaaaatgattggatgttgattgatgaaagaagatgtatgaatcacctgatcaccttcattttctagcaaagattcaagttctttacggagtactagaggactcaagtagggcacagaaacagggggaggattgggtctttttcctaaaggatccacaacttcctgcagactatttggaagactaactgttgagatgccatgaaacggtcgctgggtaaagtcaatattctgcaatgggcctccaacactgtgacttcgagtcaaagacacatttcgctttgataaactattaggcacagatgaaattttcatagtttggacatctccactggctctctttatttcatcacttggttcaactgcagagcctgtttcttcagttatgatctggttatgttttgggaagtccataaagttgatcaagtcaggttctgctaaactggatacaggtttgtgctccaaggattcatttgccaatggaatgcttccactttgtaaactgtcaccagaggtacttggtttcaggaaaaagcttgcagaacctctcaaatctttgaattctatattgagaagaggcaagaagttgcttttacagaatggacaagctgtattcaaatttgagtcatctgctgtccatccagccataatttcttcatcataaactaaagctccacaagctctacactgtgaacaactggacatcaaaacctccattgcacaattctgatagatgctagacatgctggtattttgagaagaaccatgatctgatttttcaaagtcttgccctttcatgcctcttggaaatggaacttcacctgttggataatgcagttttcctacatctccactactgctgctactgccaagacttgtgttgctctgggtaagttcactggggaccaaccctgagatacttgtgttaggcgatatattctcccccaaaatatggtcttctaggccagctgggaagctgtagtctctattagtttcttcctcatcatctgagtagctgtaggcagacgcaacagctacccacatcttactggctactgtcgctgcttgtttcataccagatttcaggacatctatcttgggccctgagagtatattatccagctttagccctgacaaagaatttactacagaacccaacgagccatgtggcgaagaacgcaccagtgctgacaaagaagttgaacgttctttatgagttcgagagggggtttgctgcttgaaacgcccagtaaaagttttagacctggacactgcaggtgagctcttttcactttcaggattttcctgtgctggtgaaccatgatctaaaggtaggcttgatctcctctctagagcatgaataaatgcagtagtcatgccagactctctgttttcctctctgtgtaattccatactagaagatttactacctaggggactttttaggttcatatagctttctatttcatcagccagattacgtgcaataactggagaaaacaacttatcttcagaatcaggagtttttcctcctgtacattcagtggctaaaagagacaaaggatctagtccagtttcaacatcttccctctgaaccaccttagcaataccatataaactacttctcttattcctcagatctttggatactgttttcaagtctctggactgattactgttactatcacttagtagactctcatatgtatctactgttgcagtagttttaggtacgtcatcaaccacaggctcaaggagttcttggctttcctcaagcatctctggcaccggagatgatctgtgctcaggattccaagtgctttcagacatacaagtcctactatcaggtaggtgacagctaacattctcaaagctatgggttcttgcaatatgaagtagagaagtcttaggacatgtcaatgctgctgtgagaatcttggcatctgctcccatcatgatagccatttcacttgaattcgaatccaaactactcttcttaagcaacattcctgctcgactttcagaactaaaactacaactcctctcaggaaaatgcttttgtcttttttctcctctatcaccattcttcttgagattagtagcttcgccaaagactgcatcttcaactggatcttgagtagaaaacagcacatttgatatactaccagtgctacttttcctgctgttgacatcaaatataccagacggaactttcacaatactgctgccccatgcaggaggttcagtaggactgtgaggctctggactaggttgtgaatgttttgccacaatagcagaggcatcacacacctcttctgtttgcatttttgttttagttatcaattctcttgctgcctgttcttcaggcacatgaatttctgcatcatcctttataagttcatccttagacccgtatccttggtcagactgaccacctgtgctagagtgattatcaatggactcaagcctgattaaatctctgacgaagactgtgtgctccccattgttagcatcattagaactatccacactaccgtggctcaccgtgtccccatcacttccacctgtgacattttgaagagctgatattgaggagacctgtgacctttgcacagtctttttaagcggctgcctaaactgtgccaagccacgtaccacattccgtaccttcgtccataagaaaataccactgcgggtactgctaggccacgggctctccaagactaccttattataataaccataagtaatagcattaggctttatcctagcagttttcatttcaaataagactctcactgctaaaacaggatgaccccaaagtccacaaagctgcatcactactcgatagcacacctgtttagttctcttagccatgagaggtggactctttgtaatgctattcccagtagggtgtctactaaaacaaagtttcaactcctgcggtctgtcaaaaagcttaaggtccagtcttggaaagtatttgtaactgtactttggtgacaggtcctttccatcatcaggaggtggctctggcggcattataaatacagtatgctcacttttctgtgaatcatctagttctatcaatctggtatcttctgctgaatcaaaatcaaccttatctgttttctctgtgcctttatcaggaaacaacttttctatgcagtcatcaaaaaatgctaatccagtatctttatcacttacaaaactgcattcttcaatgaaacgaataaaaatctgtgttttggataaaagggtatagaattttgcataggcacgatctcgactttttaaaaatccctgtcggtcaaacaatgaatcagcagctgtggctttatttgaaggagcctctgtgattggtctgagatatgttctatatccttttaaaatagacgccataaagcgcaaaaatgcctcttgaatttccatctcaagctgtgtcatcttcttttgccaggagaaatctgcttcaattggagtcatgtcaatcgctgagccttcttgagttttttggtgaactgaagacagctggggatacaatttctttaaggtgctaagtagatttttgcacggctttttgggaagttgcttccagttcatgttcttcttttcatctgatacatataacatgttcgtatccaagtcaatgcaaacaacatcttgtggtgggtcatgaagatcaaaataccttgagtcaactccaactataaatggtaaaggtgcactaagcactgcagccagtgaaagaggacaaaggggaatatatgggcattgccactgaaatggaaagatcatagctacaacagcttcagctaccccagtcaagacagctggcctaagagaatgcagcagaattttactctcaagtaaaacaaagagcagcagtgttgcacaattctcaggacccagattcattagcaaggtgctaaagttggctccacttagtggtaaaggtgtagaaactggctgtgataatattaatgcatcatggactgacagctggacaaggattctcggtctttgtggtgaaggaaaagggatgttttgcataaaatgtgaaatgtgcttttcaatgggaagaggatgtggtccagacacagaaagtttgtagataaacataagaaatttcctaaaagcttcaaaaaaaggccagtgtgagagtaaacaaatgcatttgtttgtattgatggatttggagaccatttttctctccacaggcgtcaacaagcccaggtgcataagctgtttctctgatagaagttcccgagagtaaggttcataaaactgaatggcagctccatatacctttttggctgaagaacctgtcaagacaaaagttgaaaaaactggaagtggatatttggtttcaggatcccagcactcaatagtagctcccataggaaggcagaaaagaggtacatctgattctgagagtggaaatgactcatagtcctcttctggatatctaaaaattaaaccagccttatatgctattgcatttgaagcaggtacagacttcttataacacagaaacacgctggaaccccacattccacaatttaagtttttgtcaactttgcagaaggtatgaggaggagtttctcctttactggttacaataacacagatatcagttacagccaaggaattctggggtcgaactggaggagcccttcgataagtgataaagattctttgtgaagtagttgaactattgttgacattggcacagcgaccatagggtgtggctaggatcacttcacatcctggaataagccgttctttcccttcatatagaactccaatatctgtaagcggtggtttatctctccctctcttataacagaggaaaagttctgggcttttcagacttccatagttcaagtttgcttggagagctgatggagtggcttctacacaggtgtaaccttcaggtactgtttctccagctgatttgataataatggcaatgtctgtaattggagctttaggtccagttgacttagtatctaaacgatttatttcttgatccaaaagagtagatgtgtcagtgagaccagctacgacaaagtagtctgtcactcttggtcctttgtcttctatcatggctgctactgtattttctgctgcctgctcctctgtcagcgcagccccgacacggcttcttcctggggcaagaaagcaccggattcgcggactgggcgcgctcggcagggcagggcgggggactagctccagcggccgccgccgcctcagtccggtct

SEQ ID NO: 8492 - RNA, 6828 nt, Homo sapiens
  source 1..6828: mol_type = other RNA
aaaagtaattgcggtttttgccattaatagtggcaaaaactacaattaattttgtgccaacctaatacattaaagttagggaaggcagctgtcatcagattttcaggtaattttaagattaatgactacagacaagtttagtagtagtcatttatttaatagtcaatgagacccctttcagaaaaccgtattgcaacatgcaatctattttaataaatatacacttagaatatggctgtatatacacatacctacacagccctacacatatacaaacttacacaaatatgttgctctcttttttttttttttttttttttgagacggtctcactctgtcacccaagctggagttgcagtggcgtgatctccactcactgtagcctctgcctcagttcaagcgattctcctgcctcagcctgagtagctgggactacagtggtgcgcctggctaatttttgtatttttagtaaagacagggtctcaccgtgttggccaggctggtctcgaactcctggcctcaagtgatccacccaccttgctcagcctcccaaagtgctgggattacaggcctgagccaccgtgcccggccatgttgcttttataattgagatatttcatttgttttgggggttaggcaaatttaatttgccattcctcaaactcagtaacttcaaatataaacaatgcctagaatgaatatggttcctcattatttctatcaaactactacaaatactgaagaatcccaaagtagttttccacagaggcagaaaagcagttcaggggttgaaaatcttcaatattaataagccctgggacattcaaatggcacttcatatttcaaggtaatgcaatatgaatcataattcattatatattgtccccaagagttacttcaattccgtattcaccagttcttacgatttggaaaaaaaaacttgaatgtttccagatgaaatctaatccccaagccttgtgtgtcaacattctagtgaatctctatttaaatgagaggcgctccaaaacacttcctgcaccactcgacactggcacttggtggagcatcaattttctgcaacctttcaagaatctctgaagacagactattgtatgcaattccatattcattgtcaaatgcctctttgtcttttcatgcctggcttcatttgctgtgaaagtaggttgatgggtttaagaacattattgtgctgaatactctgcctgatggtttctactaaagtgcttgtttcttgttgttcctctgacaggagagatgatttcttttcagaattaaaattcctccatgagacatacagaggttctcttggttcctgatgaaggttgatattatcccataacagctgaatatacacaagtttgctatcctgggacagagatgacagaggaagctgtacaccttcattacaatgttcagatgtgaggataagtcctggcaagttactaggaaggtccaaacgtctgaaataccaaacgaggttccagaaaatgattggatgttgattgatgaaagaagatgtatgaatcacctgatcaccttcattttctagcaaagattcaagttctttacggagtactagaggactcaagtagggcacagaaacagggggaggattgggtctttttcctaaaggatccacaacttcctgcagactatttggaagactaactgttgagatgccatgaaacggtcgctgggtaaagtcaatattctgcaatgggcctccaacactgtgacttcgagtcaaagacacatttcgctttgataaactattaggcacagatgaaattttcatagtttggacatctccactggctctctttatttcatcacttggttcaactgcagagcctgtttcttcagttatgatctggttatgttttgggaagtccataaagttgatcaagtcaggttctgctaaactggatacaggtttgtgctccaaggattcatttgccaatggaatgcttccactttgtaaactgtcaccagaggtacttggtttcaggaaaaagcttgcagaacctctcaaatctttgaattctatattgagaagaggcaagaagttgcttttacagaatggacaagctgtattcaaatttgagtcatctgctgtccatccagccataatttcttcatcataaactaaagctccacaagctctacactgtgaacaactggacatcaaaacctccattgcacaattctgatagatgctagacatgctggtattttgagaagaaccatgatctgatttttcaaagtcttgccctttcatgcctcttggaaatggaacttcacctgttggataatgcagttttcctacatctccactactgctgctactgccaagacttgtgttgctctgggtaagttcactggggaccaaccctgagatacttgtgttaggcgatatattctcccccaaaatatggtcttctaggccagctgggaagctgtagtctctattagtttcttcctcatcatctgagtagctgtaggcagacgcaacagctacccacatcttactggctactgtcgctgcttgtttcataccagatttcaggacatctatcttgggccctgagagtatattatccagctttagccctgacaaagaatttactacagaacccaacgagccatgtggcgaagaacgcaccagtgctgacaaagaagttgaacgttctttatgagttcgagagggggtttgctgcttgaaacgcccagtaaaagttttagacctggacactgcaggtgagctcttttcactttcaggattttcctgtgctggtgaaccatgatctaaaggtaggcttgatctcctctctagagcatgaataaatgcagtagtcatgccagactctctgttttcctctctgtgtaattccatactagaagatttactacctaggggactttttaggttcatatagctttctatttcatcagccagattacgtgcaataactggagaaaacaacttatcttcagaatcaggagtttttcctcctgtacattcagtggctaaaagagacaaaggatctagtccagtttcaacatcttccctctgaaccaccttagcaataccatataaactacttctcttattcctcagatctttggatactgttttcaagtctctggactgattactgttactatcacttagtagactctcatatgtatctactgttgcagtagttttaggtacgtcatcaaccacaggctcaaggagttcttggctttcctcaagcatctctggcaccggagatgatctgtgctcaggattccaagtgctttcagacatacaagtcctactatcaggtaggtgacagctaacattctcaaagctatgggttcttgcaatatgaagtagagaagtcttaggacatgtcaatgctgctgtgagaatcttggcatctgctcccatcatgatagccatttcacttgaattcgaatccaaactactcttcttaagcaacattcctgctcgactttcagaactaaaactacaactcctctcaggaaaatgcttttgtcttttttctcctctatcaccattcttcttgagattagtagcttcgccaaagactgcatcttcaactggatcttgagtagaaaacagcacatttgatatactaccagtgctacttttcctgctgttgacatcaaatataccagacggaactttcacaatactgctgccccatgcaggaggttcagtaggactgtgaggctctggactaggttgtgaatgttttgccacaatagcagaggcatcacacacctcttctgtttgcatttttgttttagttatcaattctcttgctgcctgttcttcaggcacatgaatttctgcatcatcctttataagttcatccttagacccgtatccttggtcagactgaccacctgatattgaggagacctgtgacctttgcacagtctttttaagcggctgcctaaactgtgccaagccacgtaccacattccgtaccttcgtccataagaaaataccactgcgggtactgctaggccacgggctctccaagactaccttattataataaccataagtaatagcattaggctttatcctagcagttttcatttcaaataagactctcactgctaaaacaggatgaccccaaagtccacaaagctgcatcactactcgatagcacacctcatctaagggatccacatctgttttcctcatcttaataagtacatcatatgcctgctgaagtgctctgactttaggatgagaaactctaacataggccggaagacaaataaaccataaactgtaacaatgactaaacagacacttggcccactgtggtggatttgtataacatctcttcgccaatttatgagctgtttttatttcctgtttagttctcttagccatgagaggtggactctttgtaatgctattcccagtagggtgtctactaaaacaaagtttcaactcctgcggtctgtcaaaaagcttaaggtccagtcttggaaagtatttgtaactgtactttggtgacaggtcctttccatcatcaggaggtggctctggcggcattataaatacagtatgctcacttttctgtgaatcatctagttctatcaatctggtatcttctgctgaatcaaaatcaaccttatctgttttctctgtgcctttatcaggaaacaacttttctatgcagtcatcaaaaaatgctaatccagtatctttatcacttacaaaactgcattcttcaatgaaacgaataaaaatctgtgttttggataaaagggtatagaattttgcataggcacgatctcgactttttaaaaatccctgtcggtcaaacaatgaatcagcagctgtggctttatttgaaggagcctctgtgattggtctgagatatgttctatatccttttaaaatagacgccataaagcgcaaaaatgcctcttgaatttccatctcaagctgtgtcatcttcttttgccaggagaaatctgcttcaattggagtcatgtcaatcgctgagccttcttgagttttttggtgaactgaagacagctggggatacaatttctttaaggtgctaagtagatttttgcacggctttttgggaagttgcttccagttcatgttcttcttttcatctgatacatataacatgttcgtatccaagtcaatgcaaacaacatcttgtggtgggtcatgaagatcaaaataccttgagtcaactccaactataaatggtaaaggtgcactaagcactgcagccagtgaaagaggacaaaggggaatatatgggcattgccactgaaatggaaagatcatagctacaacagcttcagctaccccagtcaagacagctggcctaagagaatgcagcagaattttactctcaagtaaaacaaagagcagcagtgttgcacaattctcaggacccagattcattagcaaggtgctaaagttggctccacttagtggtaaaggtgtagaaactggctgtgataatattaatgcatcatggactgacagctggacaaggattctcggtctttgtggtgaaggaaaagggatgttttgcataaaatgtgaaatgtgcttttcaatgggaagaggatgtggtccagacacagaaagtttgtagataaacataagaaatttcctaaaagcttcaaaaaaaggccagtgtgagagtaaacaaatgcatttgtttgtattgatggatttggagaccatttttctctccacaggcgtcaacaagcccaggtgcataagctgtttctctgatagaagttcccgagagtaaggttcataaaactgaatggcagctccatatacctttttggctgaagaacctgtcaagacaaaagttgaaaaaactggaagtggatatttggtttcaggatcccagcactcaatagtagctcccataggaaggcagaaaagaggtacatctgattctgagagtggaaatgactcatagtcctcttctggatatctaaaaattaaaccagccttatatgctattgcatttgaagcaggtacagacttcttataacacagaaacacgctggaaccccacattccacaatttaagtttttgtcaactttgcagaaggtatgaggaggagtttctcctttactggttacaataacacagatatcagttacagccaaggaattctggggtcgaactggaggagcccttcgataagtgataaagattctttgtgaagtagttgaactattgttgacattggcacagcgaccatagggtgtggctaggatcacttcacatcctggaataagccgttctttcccttcatatagaactccaatatctgtaagcggtggtttatctctccctctcttataacagaggaaaagttctgggcttttcagacttccatagttcaagtttgcttggagagctgatggagtggcttctacacaggtgtaaccttcaggtactgtttctccagctgatttgataataatggcaatgtctgtaattggagctttaggtccagttgacttagtatctaaacgatttatttcttgatccaaaagagtagatgtgtcagtgagaccagctacgacaaagtagtctgtcactcttggtcctttgtcttctatcatggctgctactgtattttctgctgcctgctcctctgtcagcgcagccccgacacggcttcttcctggggcaagaaagcaccggattcgcggactgggcgcgctcggcagggcagggcgggggactagctccagcggccgccgccgcctcagtccggtct

SEQ ID NO: 8493 - RNA, 6975 nt, Homo sapiens
  source 1..6975: mol_type = other RNA
aaaagtaattgcggtttttgccattaatagtggcaaaaactacaattaattttgtgccaacctaatacattaaagttagggaaggcagctgtcatcagattttcaggtaattttaagattaatgactacagacaagtttagtagtagtcatttatttaatagtcaatgagacccctttcagaaaaccgtattgcaacatgcaatctattttaataaatatacacttagaatatggctgtatatacacatacctacacagccctacacatatacaaacttacacaaatatgttgctctcttttttttttttttttttttttgagacggtctcactctgtcacccaagctggagttgcagtggcgtgatctccactcactgtagcctctgcctcagttcaagcgattctcctgcctcagcctgagtagctgggactacagtggtgcgcctggctaatttttgtatttttagtaaagacagggtctcaccgtgttggccaggctggtctcgaactcctggcctcaagtgatccacccaccttgctcagcctcccaaagtgctgggattacaggcctgagccaccgtgcccggccatgttgcttttataattgagatatttcatttgttttgggggttaggcaaatttaatttgccattcctcaaactcagtaacttcaaatataaacaatgcctagaatgaatatggttcctcattatttctatcaaactactacaaatactgaagaatcccaaagtagttttccacagaggcagaaaagcagttcaggggttgaaaatcttcaatattaataagccctgggacattcaaatggcacttcatatttcaaggtaatgcaatatgaatcataattcattatatattgtccccaagagttacttcaattccgtattcaccagttcttacgatttggaaaaaaaaacttgaatgtttccagatgaaatctaatccccaagccttgtgtgtcaacattctagtgaatctctatttaaatgagaggcgctccaaaacacttcctgcaccactcgacactggcacttggtggagcatcaattttctgcaacctttcaagaatctctgaagacagactattgtatgcaattccatattcattgtcaaatgcctctttgtcttttcatgcctggcttcatttgctgtgaaagtaggttgatgggtttaagaacattattgtgctgaatactctgcctgatggtttctactaaagtgcttgtttcttgttgttcctctgacaggagagatgatttcttttcagaattaaaattcctccatgagacatacagaggttctcttggttcctgatgaaggttgatattatcccataacagctgaatatacacaagtttgctatcctgggacagagatgacagaggaagctgtacaccttcattacaatgttcagatgtgaggataagtcctggcaagttactaggaaggtccaaacgtctgaaataccaaacgaggttccagaaaatgattggatgttgattgatgaaagaagatgtatgaatcacctgatcaccttcattttctagcaaagattcaagttctttacggagtactagaggactcaagtagggcacagaaacagggggaggattgggtctttttcctaaaggatccacaacttcctgcagactatttggaagactaactgttgagatgccatgaaacggtcgctgggtaaagtcaatattctgcaatgggcctccaacactgtgacttcgagtcaaagacacatttcgctttgataaactattaggcacagatgaaattttcatagtttggacatctccactggctctctttatttcatcacttggttcaactgcagagcctgtttcttcagttatgatctggttatgttttgggaagtccataaagttgatcaagtcaggttctgctaaactggatacaggtttgtgctccaaggattcatttgccaatggaatgcttccactttgtaaactgtcaccagaggtacttggtttcaggaaaaagcttgcagaacctctcaaatctttgaattctatattgagaagaggcaagaagttgcttttacagaatggacaagctgtattcaaatttgagtcatctgctgtccatccagccataatttcttcatcataaactaaagctccacaagctctacactgtgaacaactggacatcaaaacctccattgcacaattctgatagatgctagacatgctggtattttgagaagaaccatgatctgatttttcaaagtcttgccctttcatgcctcttggaaatggaacttcacctgttggataatgcagttttcctacatctccactactgctgctactgccaagacttgtgttgctctgggtaagttcactggggaccaaccctgagatacttgtgttaggcgatatattctcccccaaaatatggtcttctaggccagctgggaagctgtagtctctattagtttcttcctcatcatctgagtagctgtaggcagacgcaacagctacccacatcttactggctactgtcgctgcttgtttcataccagatttcaggacatctatcttgggccctgagagtatattatccagctttagccctgacaaagaatttactacagaacccaacgagccatgtggcgaagaacgcaccagtgctgacaaagaagttgaacgttctttatgagttcgagagggggtttgctgcttgaaacgcccagtaaaagttttagacctggacactgcaggtgagctcttttcactttcaggattttcctgtgctggtgaaccatgatctaaaggtaggcttgatctcctctctagagcatgaataaatgcagtagtcatgccagactctctgttttcctctctgtgtaattccatactagaagatttactacctaggggactttttaggttcatatagctttctatttcatcagccagattacgtgcaataactggagaaaacaacttatcttcagaatcaggagtttttcctcctgtacattcagtggctaaaagagacaaaggatctagtccagtttcaacatcttccctctgaaccaccttagcaataccatataaactacttctcttattcctcagatctttggatactgttttcaagtctctggactgattactgttactatcacttagtagactctcatatgtatctactgttgcagtagttttaggtacgtcatcaaccacaggctcaaggagttcttggctttcctcaagcatctctggcaccggagatgatctgtgctcaggattccaagtgctttcagacatacaagtcctactatcaggtaggtgacagctaacattctcaaagctatgggttcttgcaatatgaagtagagaagtcttaggacatgtcaatgctgctgtgagaatcttggcatctgctcccatcatgatagccatttcacttgaattcgaatccaaactactcttcttaagcaacattcctgctcgactttcagaactaaaactacaactcctctcaggaaaatgcttttgtcttttttctcctctatcaccattcttcttgagattagtagcttcgccaaagactgcatcttcaactggatcttgagtagaaaacagcacatttgatatactaccagtgctacttttcctgctgttgacatcaaatataccagacggaactttcacaatactgctgccccatgcaggaggttcagtaggactgtgaggctctggactaggttgtgaatgttttgccacaatagcagaggcatcacacacctcttctgtttgcatttttgttttagttatcaattctcttgctgcctgttcttcaggcacatgaatttctgcatcatcctttataagttcatccttagacccgtatccttggtcagactgaccacctgtgctagagtgattatcaatggactcaagcctgattaaatctctgacgaagactgtgtgctccccattgttagcatcattagaactatccacactaccgtggctcaccgtgtccccatcacttccacctgtgacattttgaagagctgatattgaggagacctgtgacctttgcacagtctttttaagcggctgcctaaactgtgccaagccacgtaccacattccgtaccttcgtccataagaaaataccactgcgggtactgctaggccacgggctctccaagactaccttattataataaccataagtaatagcattaggctttatcctagcagttttcatttcaaataagactctcactgctaaaacaggatgaccccaaagtccacaaagctgcatcactactcgatagcacacctcatctaagggatccacatctgttttcctcatcttaataagtacatcatatgcctgctgaagtgctctgactttaggatgagaaactctaacataggccggaagacaaataaaccataaactgtaacaatgactaaacagacacttggcccactgtggtggatttgtataacatctcttcgccaatttatgagctgtttttatttcctgtttagttctcttagccatgagaggtggactctttgtaatgctattcccagtagggtgtctactaaaacaaagtttcaactcctgcggtctgtcaaaaagcttaaggtccagtcttggaaagtatttgtaactgtactttggtgacaggtcctttccatcatcaggaggtggctctggcggcattataaatacagtatgctcacttttctgtgaatcatctagttctatcaatctggtatcttctgctgaatcaaaatcaaccttatctgttttctctgtgcctttatcaggaaacaacttttctatgcagtcatcaaaaaatgctaatccagtatctttatcacttacaaaactgcattcttcaatgaaacgaataaaaatctgtgttttggataaaagggtatagaattttgcataggcacgatctcgactttttaaaaatccctgtcggtcaaacaatgaatcagcagctgtggctttatttgaaggagcctctgtgattggtctgagatatgttctatatccttttaaaatagacgccataaagcgcaaaaatgcctcttgaatttccatctcaagctgtgtcatcttcttttgccaggagaaatctgcttcaattggagtcatgtcaatcgctgagccttcttgagttttttggtgaactgaagacagctggggatacaatttctttaaggtgctaagtagatttttgcacggctttttgggaagttgcttccagttcatgttcttcttttcatctgatacatataacatgttcgtatccaagtcaatgcaaacaacatcttgtggtgggtcatgaagatcaaaataccttgagtcaactccaactataaatggtaaaggtgcactaagcactgcagccagtgaaagaggacaaaggggaatatatgggcattgccactgaaatggaaagatcatagctacaacagcttcagctaccccagtcaagacagctggcctaagagaatgcagcagaattttactctcaagtaaaacaaagagcagcagtgttgcacaattctcaggacccagattcattagcaaggtgctaaagttggctccacttagtggtaaaggtgtagaaactggctgtgataatattaatgcatcatggactgacagctggacaaggattctcggtctttgtggtgaaggaaaagggatgttttgcataaaatgtgaaatgtgcttttcaatgggaagaggatgtggtccagacacagaaagtttgtagataaacataagaaatttcctaaaagcttcaaaaaaaggccagtgtgagagtaaacaaatgcatttgtttgtattgatggatttggagaccatttttctctccacaggcgtcaacaagcccaggtgcataagctgtttctctgatagaagttcccgagagtaaggttcataaaactgaatggcagctccatatacctttttggctgaagaacctgtcaagacaaaagttgaaaaaactggaagtggatatttggtttcaggatcccagcactcaatagtagctcccataggaaggcagaaaagaggtacatctgattctgagagtggaaatgactcatagtcctcttctggatatctaaaaattaaaccagccttatatgctattgcatttgaagcaggtacagacttcttataacacagaaacacgctggaaccccacattccacaatttaagtttttgtcaactttgcagaaggtatgaggaggagtttctcctttactggttacaataacacagatatcagttacagccaaggaattctggggtcgaactggaggagcccttcgataagtgataaagattctttgtgaagtagttgaactattgttgacattggcacagcgaccatagggtgtggctaggatcacttcacatcctggaataagccgttctttcccttcatatagaactccaatatctgtaagcggtggtttatctctccctctcttataacagaggaaaagttctgggcttttcagacttccatagttcaagtttgcttggagagctgatggagtggcttctacacaggtgtaaccttcaggtactgtttctccagctgatttgataataatggcaatgtctgtaattggagctttaggtccagttgacttagtatctaaacgatttatttcttgatccaaaagagtagatgtgtcagtgagaccagctacgacaaagtagtctgtcactcttggtcctttgtcttctatcatggctgctactgtattttctgctgcctgctcctctgtcagcgcagccccgacacggcttcttcctggggcaagaaagcaccggattcgcggactgggcgcgctcggcagggcagggcgggggactagctccagcggccgccgccgcctcagtccggtct

SEQ ID NO: 8494 - RNA, 6999 nt, Homo sapiens
  source 1..6999: mol_type = other RNA
aaaagtaattgcggtttttgccattaatagtggcaaaaactacaattaattttgtgccaacctaatacattaaagttagggaaggcagctgtcatcagattttcaggtaattttaagattaatgactacagacaagtttagtagtagtcatttatttaatagtcaatgagacccctttcagaaaaccgtattgcaacatgcaatctattttaataaatatacacttagaatatggctgtatatacacatacctacacagccctacacatatacaaacttacacaaatatgttgctctcttttttttttttttttttttttgagacggtctcactctgtcacccaagctggagttgcagtggcgtgatctccactcactgtagcctctgcctcagttcaagcgattctcctgcctcagcctgagtagctgggactacagtggtgcgcctggctaatttttgtatttttagtaaagacagggtctcaccgtgttggccaggctggtctcgaactcctggcctcaagtgatccacccaccttgctcagcctcccaaagtgctgggattacaggcctgagccaccgtgcccggccatgttgcttttataattgagatatttcatttgttttgggggttaggcaaatttaatttgccattcctcaaactcagtaacttcaaatataaacaatgcctagaatgaatatggttcctcattatttctatcaaactactacaaatactgaagaatcccaaagtagttttccacagaggcagaaaagcagttcaggggttgaaaatcttcaatattaataagccctgggacattcaaatggcacttcatatttcaaggtaatgcaatatgaatcataattcattatatattgtccccaagagttacttcaattccgtattcaccagttcttacgatttggaaaaaaaaacttgaatgtttccagatgaaatctaatccccaagccttgtgtgtcaacattctagtgaatctctatttaaatgagaggcgctccaaaacacttcctgcaccactcgacactggcacttggtggagcatcaattttctgcaacctttcaagaatctctgaagacagactattgtatgcaattccatattcattgtcaaatgcctctttgtcttttcatgcctggcttcatttgctgtgaaagtaggttgatgggtttaagaacattattgtgctgaatactctgcctgatggtttctactaaagtgcttgtttcttgttgttcctctgacaggagagatgatttcttttcagaattaaaattcctccatgagacatacagaggttctcttggttcctgatgaaggttgatattatcccataacagctgaatatacacaagtttgctatcctgggacagagatgacagaggaagctgtacaccttcattacaatgttcagatgtgaggataagtcctggcaagttactaggaaggtccaaacgtctgaaataccaaacgaggttccagaaaatgattggatgttgattgatgaaagaagatgtatgaatcacctgatcaccttcattttctagcaaagattcaagttctttacggagtactagaggactcaagtagggcacagaaacagggggaggattgggtctttttcctaaaggatccacaacttcctgcagactatttggaagactaactgttgagatgccatgaaacggtcgctgggtaaagtcaatattctgcaatgggcctccaacactgtgacttcgagtcaaagacacatttcgctttgataaactattaggcacagatgaaattttcatagtttggacatctccactggctctctttatttcatcacttggttcaactgcagagcctgtttcttcagttatgatctggttatgttttgggaagtccataaagttgatcaagtcaggttctgctaaactggatacaggtttgtgctccaaggattcatttgccaatggaatgcttccactttgtaaactgtcaccagaggtacttggtttcaggaaaaagcttgcagaacctctcaaatctttgaattctatattgagaagaggcaagaagttgcttttacagaatggacaagctgtattcaaatttgagtcatctgctgtccatccagccataatttcttcatcataaactaaagctccacaagctctacactgtgaacaactggacatcaaaacctccattgcacaattctgatagatgctagacatgctggtattttgagaagaaccatgatctgatttttcaaagtcttgccctttcatgcctcttggaaatggaacttcacctgttggataatgcagttttcctacatctccactactgctgctactgccaagacttgtgttgctctgggtaagttcactggggaccaaccctgagatacttgtgttaggcgatatattctcccccaaaatatggtcttctaggccagctgggaagctgtagtctctattagtttcttcctcatcatctgagtagctgtaggcagacgcaacagctacccacatcttactggctactgtcgctgcttgtttcataccagatttcaggacatctatcttgggccctgagagtatattatccagctttagccctgacaaagaatttactacagaacccaacgagccatgtggcgaagaacgcaccagtgctgacaaagaagttgaacgttctttatgagttcgagagggggtttgctgcttgaaacgcccagtaaaagttttagacctggacactgcaggtgagctcttttcactttcaggattttcctgtgctggtgaaccatgatctaaaggtaggcttgatctcctctctagagcatgaataaatgcagtagtcatgccagactctctgttttcctctctgtgtaattccatactagaagatttactacctaggggactttttaggttcatatagctttctatttcatcagccagattacgtgcaataactggagaaaacaacttatcttcagaatcaggagtttttcctcctgtacattcagtggctaaaagagacaaaggatctagtccagtttcaacatcttccctctgaaccaccttagcaataccatataaactacttctcttattcctcagatctttggatactgttttcaagtctctggactgattactgttactatcacttagtagactctcatatgtatctactgttgcagtagttttaggtacgtcatcaaccacaggctcaaggagttcttggctttcctcaagcatctctggcaccggagatgatctgtgctcaggattccaagtgctttcagacatacaagtcctactatcaggtaggtgacagctaacattctcaaagctatgggttcttgcaatatgaagtagagaagtcttaggacatgtcaatgctgctgtgagaatcttggcatctgctcccatcatgatagccatttcacttgaattcgaatccaaactactcttcttaagcaacattcctgctcgactttcagaactaaaactacaactcctctcaggaaaatgcttttgtcttttttctcctctatcaccattcttcttgagattagtagcttcgccaaagactgcatcttcaactggatcttgagtagaaaacagcacatttgatatactaccagtgctacttttcctgctgttgacatcaaatataccagacggaactttcacaatactgctgccccatgcaggaggttcagtaggactgtgaggctctggactaggttgtgaatgttttgccacaatagcagaggcatcacacacctcttctgtttgcatttttgttttagttatcaattctcttgctgcctgttcttcaggcacatgaatttctgcatcatcctttataagttcatccttagacccgtatccttggtcagactgaccacctgtgctagagtgattatcaatggactcaagcctgattaaatctctgacgaagactgtgtgctccccattgttagcatcattagaactatccacactaccgtggctcaccgtgtccccatcacttccacctgtgacattttgaagagctgatattgaggagacctgtgacctttgcacagtctttttaagcggctgcctaaactgtgccaagccacgtaccacattccgtaccttcgtccataagaaaataccactgcgggtactgctaggccacgggctctccaagactaccttattataataaccataagtaatagcattaggctttatcctagcagttttcatttcaaataagactctcactgctaaaacaggatgaccccaaagtccacaaagctgcatcactactcgatagcacacctcatctaagggatccacatctgttttcctcatcttaataagtacatcatatgcctgctgaagtgctctgactttaggatgagaaactctaacataggccggaagacaaataaaccataaactgtaacaatgactaaacagacacttggcccactgtggtggatttgtataacatctcttcgccaatttatgagctgtttttatttcctgtttagttctcttagccatgagaggtggactctttgtaatgctattcccagtagggtgtctactaaaacaaagtttcaactcctgcggtctgtcaaaaagcttaaggtccagtcttggaaagtatttgtaactgtactttggtgacaggtcctttccatcatcaggaggtggctctggcggcattataaatacagtatgctcacttttctgtgaatcatctagttctatcaatctggtatcttctgctgaatcaaaatcaaccttatctgttttctctgtgcctttatcaggaaacaacttttctatgcagtcatcaaaaaatgctaatccagtatctttatcacttacaaaactgcattcttcaatgaaacgaataaaaatctgtgttttggataaaagggtatagaattttgcataggcacgatctcgactttttaaaaatccctgtcggtcaaacaatgaatcagcagctgtggctttatttgaaggagcctctgtgattggtctgagatatgttctatatccttttaaaatagacgccataaagcgcaaaaatgcctcttgaatttccatctcaagctgtgtcatcttcttttgccaggagaaatctgcttcaattggagtcatgtcaatcgctgagccttcttgagttttttggtgaactgaagacagctggggatacaatttctttaaggtgctaagtagatttttgcacggctttttgggaagttgcttccagttcatgttcttcttttcatctgatagctacaacagcttcagctaccccagtcaagacagctggcctaagagaatgcagcagaattttactctcaagtaaaacaaagagcagcagtgttgcacaattctcaggacccagattcattagcaaggtgctaaagttggctccacttagtggtaaaggtgtagaaactggctgtgataatattaatgcatcatggactgacagctggacaaggattctcggtctttgtggtgaaggaaaagggatgttttgcataaaatgtgaaatgtgcttttcaatgggaagaggatgtggtccagacacagaaagtttgtagataaacataagaaatttcctaaaagcttcaaaaaaaggccagtgtgagagtaaacaaatgcatttgtttgtattgatggatttggagaccatttttctctccacaggcgtcaacaagcccaggtgcataagctgtttctctgatagaagttcccgagagtaaggttcataaaactgaatggcagctccatatacctttttggctgaagaacctgtcaagacaaaagttgaaaaaactggaagtggatatttggtttcaggatcccagcactcaatagtagctcccataggaaggcagaaaagaggtacatctgattctgagagtggaaatgactcatagtcctcttctggatatctaaaaattaaacctgtattttcagtttttatcccaccataccagtggaatgaagacgtgacacttaaatctttacagcccttgacactttaatgtgcagtaagaatgtggcgatagatttctcaaacacttcatggcagaaaagtttctcaggccctcctctcctccatatagctgattctttgcaacaaaggagaaaggaagcaagtccaccagccttatatgctattgcatttgaagcaggtacagacttcttataacacagaaacacgctggaaccccacattccacaatttaagtttttgtcaactttgcagaaggtatgaggaggagtttctcctttactggttacaataacacagatatcagttacagccaaggaattctggggtcgaactggaggagcccttcgataagtgataaagattctttgtgaagtagttgaactattgttgacattggcacagcgaccatagggtgtggctaggatcacttcacatcctggaataagccgttctttcccttcatatagaactccaatatctgtaagcggtggtttatctctccctctcttataacagaggaaaagttctgggcttttcagacttccatagttcaagtttgcttggagagctgatggagtggcttctacacaggtgtaaccttcaggtactgtttctccagctgatttgataataatggcaatgtctgtaattggagctttaggtccagttgacttagtatctaaacgatttatttcttgatccaaaagagtagatgtgtcagtgagaccagctacgacaaagtagtctgtcactcttggtcctttgtcttctatcatggctgctactgtattttctgctgcctgctcctctgtcagcgcagccccgacacggcttcttcctggggcaagaaagcaccggattcgcggactgggcgcgctcggcagggcagggcgggggactagctccagcggccgccgccgcctcagtccggtct

SEQ ID NO: 8495 - RNA, 73 nt, Homo sapiens
  source 1..73: mol_type = other RNA
aaaagtaattgcggtttttgccattactttcagtagcaaaaatctcaattacttttgcaccaacttaatactt

SEQ ID NO: 8496 - RNA, 1917 nt, Homo sapiens
  source 1..1917: mol_type = other RNA
aaaagtaattgcggtttttgccattacttttaatagaacaatgttttcaaacttaagtttgcatcagaatcacttgattctgattttaacagtcgttaaaataaagattgctgggacccatccgcagtttctggttttggcagggtgcaagaacttccatttctaataagttcctgggtggtgatgatgctgttggttgaaggaccacactttgagaaccacttatctagaagttcaaaggttgaggtgagagaatcgcttgatcccaggaggtcgaggctccagtgagctgtgatcacaccactgcactccagcctaggtgacagagcaagaccctgtaatcccagctactcggaaggctgaggcaggagaattgcttgaacccgggaggcagaggttgcggtgggctaagattgcgccactgcactccagcctgggtgacagagagagactccatctcaaaaaaagaaaagaaaagaaaacaacattaattctcacttttgaagggatagcaggaagatgcatattaatattacagcatctttgataaaaaccaatctatttggccgggcatggtggctcatgcctgttaccctagcactttgggaggctgaagaaggaagatcccttgagtccaggagtccgagaccagcctaggaatacagtaagaccttgtctctacaataaatacacaaaattagtgagcatagtggcaggcacctatagttgcagctactctagaggctgaagtgggaggatcccttgagtgctggaggtcaaggctgcagtgagccaaaaaaaagaccaatgaattcaagtgtctaccccctaacccaaacagaagcagaccctaaatctttcagggtgtcatcctaagctaagtagaaatctaaaagtttcctagagcacagataagagtgacctagcactccagccaaccagaaagggaaaagcagaacataagcttactttctacaaaggaagcagctatacaaattatgccagagaactagaaaaacactaatttgagtatccaaaaggggggaagtagttccaaatatttctaataaagagcattctgtaagccttccaacaagctattaaaggttgagaaaacctatctggcaacccagttaatttcaggacacataattacaggaacttagtccctcaagtcagagatgcctgtgaggaattgcacggtttgaatcacagcagatttgcagcctatttaagtttttggaccactagaaaactggaaaaacaattcatttaatatagttgagagaatacttaaaaatcctacatcaattcaattatatactgacttagaattatatgattacttcctatggagggttaattccctggcatttaggttgagcccctacatataccttcaattatcaaaaaaaaaatcaaaactttatttgaactcaaagttttacttatgagaataatgaaatcttacttagattaacactcaaaacatttcttggggataggctttttaaaatgaaacccataatttatttttgttacaaaaggaaatgtttacgtccctgttaaagtataaaaagggtctcattagtgtatctgaagagtactacattgtacattgtcttccagaggtggaaaaaaaaagaagttaacttttacatatacttgaaagggaaagtctgcattctgcactaagttttcttgaatggaataagtttaaattgtcctcagttctagcaaagaatgttcttaaatatctgtctttaaaaatccaatagtagggccgggtgaggtggctcacgtctgtaatcccagcattttgggaggcagatggatcatctgaggtcaggagttcgaaaacagcccggccaacatggtgaaaacagcatggccaacatggtgaaaccctgtctccgt

SEQ ID NO: 8497 - RNA, 70 nt, Homo sapiens
  source 1..70: mol_type = other RNA
aaaagtaattgcggtttttgccattacttttataggcaaaaaccacaatgccttttgcaccaacctaatg

SEQ ID NO: 8498 - RNA, 3040 nt, Homo sapiens
  source 1..3040: mol_type = other RNA
aaaagtaattgcggtttttgccattccttttgatggtaaaaaccgcaattacttttgcacaaatctaattttaaaaattagagtatgtcggacagtgtcagtgctaaggaggaaaataaagtacaagtagtgaatagggactacggaatggtggtgcaggattttaaatagggtagccaggaaggggtttgcgaggaccacgtttgagcaaaccgaaaggtgagggagcgagctgtgcagatgtgggggtcggggaggacactgtcccagagacagaagagcaggttcaaaggccctgagacagaaacaatcgcctggtgatccccattttacagaagagagatctgaggctcagaaagatggagtcactcatccaaacttgcacagctgtaagtggcagagctgggattcgaatgccaggcccgataccaccaaaacctgcatttgtttctcattttctcatatttttcaattcagacactgaggatgtaggtgttggggcatcggcagagtgcttaagagctagacgtgatgtgaaccagacctgggttcaggttttgtggtgccacttacctccttgggtggctgacttgaactgtctgagcctcagtttccacatgctggtatttatcatatgcctcggctcctcaaactgcagcaaacaaactccatggaagagaaaaaaatgggactccagagacttgaaaccacggccacttgtcagatgcagcccccaactcagctgcaggagcttagccaaatttctagtcctctctgagcctcaatttccttatctataaaatgtggctctggatacctctcttgtagagttcttgtttagattacatgtgagcacttctataaaacactgaagacatgagctagccgttattctttataaacagtcatcaggagaattttgattttccacctcacagatttcccacaggaatgtgctgtcctgaaatgtgtctaaaggtcaacatttgaaaaacagaaagaatggaaaagaaagtcagcaaagtccagcatcatgacttggcagtgtccccagtggccaggtgcaaaggagcacccagagaggtgttttcagaccactgtaaatagtgtgagtgctatttaggacttacacacactcagacacatgcacacacacacaaatatagatacagccacacacatctgcagtttcactgccacacatagacactcacacatgcaagcacacacaaatatctagtcacacttctagacactcacacacatgaatacacacagttacacttacaatcttatgcacatgccaaactcataaacagatacatagacatacacttaactacagagctacatatacatgacagtcacacacatagttacatacacagtctcacacatacattcacacacatccacatctaccaacacacatgcatgcatgtaagtatacataaacacctgtacacctgcgcatacagctctacacacacttgcacacatgtacacatacacagtctcacatacatccatgtactgacacataggcacacatgggcacaaacatgcacaaccttacacacatgtctttacacacagaaccgcacacacataacagctatacatacatcccacagtcacatgtgcacacacaaaaacatacatgcatgcacttaggctatctcacatacacagctatgtacttcacacaggcacacacattataacaacatgttttcttttctttacagcccttattcattctctcagctatttactgaatgtttactgtgtgctagctaccgttaaaagtccttgagctaaatcattgaacaaaatgagcaaaaatatctgccctcatgaagcttagattctaatggaaggagagagaggcaaaaatagtaagtaagtatgttagcaggtagtgagtattagagacaatagtgcctagtaatgaggaggaggaagaaccaacttggaggtgggttgccgttttgagaaggtggtcaaggtaagcttcattgagaagttgacaaaaatatttagcaaggaaataaagtaggagagggagttatccatgtagatatctatgaaaaatcagtctgagaagaggaaacagcaagtgcagataccctaaaggcagagtgtgacttcaaggaacaggaagaaagcccttgtagttgacatgcagtgaataagggggtaaaggaacaggacatcaaaccagagatgaagagagtgtgtgaaaatcttaccagaccttgaataatgaggtaaaaactctgaagttaattttgcatgaaactgagattcaccggtaggttgtgagcagaggtgtgacatgatctgacctctgacttatcctttacagtatataaaatgaacttcattactttacatgttattatctgtgtcacttctgaacaggaatgaatctgtcatggtcacctctgtgtctacctgagagtaacactcagtcaatatttgttgactacttgataaggacagacatttccaaggagaaaagtgttctgaggtgctccagtttggatgtttgctctcaataaaactcatattgaaatttgagatggaaccttacaggaggtatttgagtcatgagggagaatccctcatgaataaattaatgccctccctagggagtgagtgagtcctaatcctattattccccacaagagctggttgttgcaaagagcctggcatctccccactatctctcttgcttcctctctcaccatgtcatccatgcacacgccagctccctttcaccttctaccatgaatagaagcatcccgaggcccttgccagctgcagatgcccaatcttgaaatttccagctatcagaatcatgggcctaataaacatttctgaaataaattacccagcctcagatatttctttatagcaatgaaaaatggactacaacaggaaattgttgccagggagtagggtattgctataaagatacctgaaaatatgacagcagctttggaactgggcaatggaaaaggttggaagagtttgg

SEQ ID NO: 8499 - RNA, 3421 nt, Homo sapiens
  source 1..3421: mol_type = other RNA
aaaagtaattgcggtttttgccattgaaagtaatggaaaaaccacaattacttttgcaccaacccattacaaacaagttttaacaatcacaagactaatgttttagtgacggctcctaaaacttcagggaaaaaaaaagtgcatttctgactggcaatagtttgcaaaataatcgtaatgaaactacttatttctttattttaaaagttaataaaaggaaacctctcaatttttaggaagaattcaattacaataaaatcatgatgtcttatgatctggcatcttataatctgtgtctcagaaagaagggcaatttacagcatcagatgaatactggagtttaggtcagacttaagttatctgaaaagaacataaggcatttacagtttttagcagggaaaaataatcaaatctctttttttaaaaaaaaccttcttagtatcttggttaaatgtccaaaaagctgtattatttttagttttaaaccagtaggcactattcgaaactgagaattcaggatgttatcaaatacaaatttttaaaagcttgaccattaaagcataaattgcctaatgagacacatgtaatcataaaaactaacgccaggatcatttacttgtgattggatatatgccatttatttttctggcttctttctaatgtgtaattcctgctgaattgagtgagcatgtcagatttctatctttatcttagtgtgtgtaaaagttctcaacctagacaaggacaaattttagaattttccaatgaacatcattcactatgtatgatgctgttttgttaaactagctgtttggaaaacaataaagatttcatttgttttgcgttagccacagagagtggacttgtttagaatgtaaaagtatttatctcaaatactaaaatcaaactcaagaaaaatcaaacaatgctggagctgagaaaaataatggctatatatctggttgaacatgttgaaagaaaagtgaaaacacagccaggcatggtggtgcgcacctgtaatcccagctacttgggaggctgagacaggagaattgcttgaatctaggaggcagaggttgcagtgagccaagatcaaccactgcactacacagcctgggtgacacagactccttcacgcacacacaaaaaagtgaaaacaaacttggaagtctagaatgaagaattacatctaatgcagtaatattcttcccacctttccatattaaatgtaagaagcaccagcaaaaaatactaaagacagagaaatgacctggcaaaatgattcaaataccacagagcgtgagaatattcctcagtaaagctcaagatattatgaagtagctagcagaagaaatggcaggggtagcggaagtaaaaattctaaccatatgacagactctaacagtaagtcataaattctaaaggtttaattagtaaattcattatttcctccaaaatatactgtcattcttctcttaacaatgaatgtttgacacaaatccaattttgatgttaaaagtcaacatacatagataggtccctcatgttgacagagcacagaattggaaaaaaaaactgcaaatgagaaataggggtatttctaaatcttctgtattcctaaaatatcacactgcgcccttgcttcagcctccctgatagactggtttgggtgtgcaatattaatgcaggaatacgtggaataccagcacaaagccggggagggagactagcaaactctcgccatcaattatttctcaactacatttagtattcttcgcagttttagatttttttttcctttaagcgaaaaccactccactgaaaaaaattccaaacttgttttttaaaaattgcaggaatttcttcgtattttatcaacaaaaataccagaaattaaagagctgacagaaattcaagcagatccaaattcaaccatccatttttcatacttctccaagtctgcagcagagacagacttagcaattttctttagggccaattcaaagtctcctttggtaacaggcatctgaagttcctctttagaaagtgcacggatttcttctggacttaagccattgatacgccgtctcattgccattaaagaggcatccctgcaaacattagtgatgtcagcaccagaatagccctcaatcttctcggctatatcttccagttgaatatcaggatctaattcgacctcacgaaggttgatcttcagaagctcagctcttccttttgctgttgggagaggtatatatatccttttttctaaccttcttcgcaaagcttcatcaatgtcccacgggaaattagtagcagccaataccataaccattttggaaggatcatcattttctaaagctcctccaactccatccatctgaatgagcagttcagacttgaccctgcgacttgcctcatgttcatcagaggttcctcttcgactgcagatagaatctatctcatcaatgaagatcgtggtaggggcataaaatctagccatctcaaacaacagacgaactaacttctcagattcacctctgtatttagatgtcagtgtagaagacgaaacgttgaagaatgttgtaccacattcagtggcaacagctttagctagcatagttttaccagtgcctgggggtccaaccatcagtacacccttccatggccttctaatccctttgaaaaagtcaggcatccacattggaagaacaacagcttcccttagcaacttcttagcttcttccagatctgctatgtcatcccaatgaatgctaggattcctggatacaatgtctctttcaagggcttccaccagatccttatcataaccagcaccatcaaattttggcatttcaccatcacttgcaccatcttgcatattcttccttccctgtgttctgcaggaacagggggtggccaaacagcaggatctctaaatggttcatcttgacaggacacagggaaatctggaggcttgtcaattttaaaactttctaaagtgctgacaatacttttaacttgttcatattcctccaataattcctgccgaacctgttgccatttgcctttgatagctggatctctgactgactggcaatgtctctgaatctgctgcatcaccccctggtaatataccattgatgagtcgtaatttccaagaagggcatattctcttcctttctttgcattatcacaaatctcagccaaattcatcttctttcagagacccagaaataaacgtatccaggaaaggagaaaaacctgttaaaacacggtttctcaggtctcacatccaatgtgtgacatacatacggttctgcaccgaaaggcagcaacctgcgagggtcagaggcgccgaagacccgaggccctgcagcttgggcggctgctcatccctgagactgtgcagggcggtggc

SEQ ID NO: 8500 - RNA, 3401 nt, Homo sapiens
  source 1..3401: mol_type = other RNA
aaaagtaattgcggtttttgccattgaaagtaatggaaaaaccacaattacttttgcaccaacccattacaaacaagttttaacaatcacaagactaatgttttagtgacggctcctaaaacttcagggaaaaaaaaagtgcatttctgactggcaatagtttgcaaaataatcgtaatgaaactacttatttctttattttaaaagttaataaaaggaaacctctcaatttttaggaagaattcaattacaataaaatcatgatgtcttatgatctggcatcttataatctgtgtctcagaaagaagggcaatttacagcatcagatgaatactggagtttaggtcagacttaagttatctgaaaagaacataaggcatttacagtttttagcagggaaaaataatcaaatctctttttttaaaaaaaaccttcttagtatcttggttaaatgtccaaaaagctgtattatttttagttttaaaccagtaggcactattcgaaactgagaattcaggatgttatcaaatacaaatttttaaaagcttgaccattaaagcataaattgcctaatgagacacatgtaatcataaaaactaacgccaggatcatttacttgtgattggatatatgccatttatttttctggcttctttctaatgtgtaattcctgctgaattgagtgagcatgtcagatttctatctttatcttagtgtgtgtaaaagttctcaacctagacaaggacaaattttagaattttccaatgaacatcattcactatgtatgatgctgttttgttaaactagctgtttggaaaacaataaagatttcatttgttttgcgttagccacagagagtggacttgtttagaatgtaaaagtatttatctcaaatactaaaatcaaactcaagaaaaatcaaacaatgctggagctgagaaaaataatggctatatatctggttgaacatgttgaaagaaaagtgaaaacacagccaggcatggtggtgcgcacctgtaatcccagctacttgggaggctgagacaggagaattgcttgaatctaggaggcagaggttgcagtgagccaagatcaaccactgcactacacagcctgggtgacacagactccttcacgcacacacaaaaaagtgaaaacaaacttggaagtctagaatgaagaattacatctaatgcagtaatattcttcccacctttccatattaaatgtaagaagcaccagcaaaaaatactaaagacagagaaatgacctggcaaaatgattcaaataccacagagcgtgagaatattcctcagtaaagctcaagatattatgaagtagctagcagaagaaatggcaggggtagcggaagtaaaaattctaaccatatgacagactctaacagtaagtcataaattctaaaggtttaattagtaaattcattatttcctccaaaatatactgtcattcttctcttaacaatgaatgtttgacacaaatccaattttgatgttaaaagtcaacatacatagataggtccctcatgttgacagagcacagaattggaaaaaaaaactgcaaatgagaaataggggtatttctaaatcttctgtattcctaaaatatcacactgcgcccttgcttcagcctccctgatagactggtttgggtgtgcaatattaatgcaggaatacgtggaataccagcacaaagccggggagggagactagcaaactctcgccatcaattatttctcaactacatttagtattcttcgcagttttagatttttttttcctttaagcgaaaaccactccactgaaaaaaattccaaacttgttttttaaaaattgcaggaatttcttcgtattttatcaacaaaaataccagaaattaaagagctgacagaaattcaagcagatccaaattcaaccatccatttttcatacttctccaagtctgcagcagagacagacttagcaattttctttagggccaattcaaagtctcctttggtaacaggcatctgaagttcctctttagaaagtgcacggatttcttctggacttaagccattgatacgccgtctcattgccattaaagaggcatccctgcaaacattagtgatgtcagcaccagaatagccctcaatcttctcggctatatcttccagttgaatatcaggatctaattcgacctcacgaaggttgatcttcagaagctcagctcttccttttgctgttgggagaggtatatatatccttttttctaaccttcttcgcaaagcttcatcaatgtcccacgggaaattagtagcagccaataccataaccattttggaaggatcatcattttctaaagctcctccaactccatccatctgaatgagcagttcagacttgaccctgcgacttgcctcatgttcatcagaggttcctcttcgactgcagatagaatctatctcatcaatgaagatcgtggtaggggcataaaatctagccatctcaaacaacagacgaactaacttctcagattcacctctgtatttagatgtcagtgtagaagacgaaacgttgaagaatgttgtaccacattcagtggcaacagctttagctagcatagttttaccagtgcctgggggtccaaccatcagtacacccttccatggccttctaatccctttgaaaaagtcaggcatccacattggaagaacaacagcttcccttagcaacttcttagcttcttccagatctgctatgtcatcccaatgaatgctaggattcctggatacaatgtctctttcaagggcttccaccagatccttatcataaccagcaccatcaaattttggcatttcaccatcacttgcaccatcttgcatattcttccttccctgtgttctgcaggaacagggggtggccaaacagcaggatctctaaatggttcatcttgacaggacacagggaaatctggaggcttgtcaattttaaaactttctaaagtgctgacaatacttttaacttgttcatattcctccaataattcctgccgaacctgttgccatttgcctttgatagctggatctctgactgactggcaatgtctctgaatctgctgcatcaccccctggtaatataccattgatgagtcgtaatttccaagaagggcatattctcttcctttctttgcattatcacaaatctcagccaaattcatcttctttcagagacccagaaggcgcaggtccgggcacattcagcgatgcggtccagatggggtgcgggtggggcgcaggccgccgccgccgccgccgccgagtccgttagctcgcgacgtgcgtgaaaaggcggcggcggcgtagtgttgccatggcagccgcggccgcgcggtgggcgcagcgc

SEQ ID NO: 8501 - RNA, 3529 nt, Homo sapiens
  source 1..3529: mol_type = other RNA
aaaagtaattgcggtttttgccattgaaagtaatggaaaaaccacaattacttttgcaccaacccattacaaacaagttttaacaatcacaagactaatgttttagtgacggctcctaaaacttcagggaaaaaaaaagtgcatttctgactggcaatagtttgcaaaataatcgtaatgaaactacttatttctttattttaaaagttaataaaaggaaacctctcaatttttaggaagaattcaattacaataaaatcatgatgtcttatgatctggcatcttataatctgtgtctcagaaagaagggcaatttacagcatcagatgaatactggagtttaggtcagacttaagttatctgaaaagaacataaggcatttacagtttttagcagggaaaaataatcaaatctctttttttaaaaaaaaccttcttagtatcttggttaaatgtccaaaaagctgtattatttttagttttaaaccagtaggcactattcgaaactgagaattcaggatgttatcaaatacaaatttttaaaagcttgaccattaaagcataaattgcctaatgagacacatgtaatcataaaaactaacgccaggatcatttacttgtgattggatatatgccatttatttttctggcttctttctaatgtgtaattcctgctgaattgagtgagcatgtcagatttctatctttatcttagtgtgtgtaaaagttctcaacctagacaaggacaaattttagaattttccaatgaacatcattcactatgtatgatgctgttttgttaaactagctgtttggaaaacaataaagatttcatttgttttgcgttagccacagagagtggacttgtttagaatgtaaaagtatttatctcaaatactaaaatcaaactcaagaaaaatcaaacaatgctggagctgagaaaaataatggctatatatctggttgaacatgttgaaagaaaagtgaaaacacagccaggcatggtggtgcgcacctgtaatcccagctacttgggaggctgagacaggagaattgcttgaatctaggaggcagaggttgcagtgagccaagatcaaccactgcactacacagcctgggtgacacagactccttcacgcacacacaaaaaagtgaaaacaaacttggaagtctagaatgaagaattacatctaatgcagtaatattcttcccacctttccatattaaatgtaagaagcaccagcaaaaaatactaaagacagagaaatgacctggcaaaatgattcaaataccacagagcgtgagaatattcctcagtaaagctcaagatattatgaagtagctagcagaagaaatggcaggggtagcggaagtaaaaattctaaccatatgacagactctaacagtaagtcataaattctaaaggtttaattagtaaattcattatttcctccaaaatatactgtcattcttctcttaacaatgaatgtttgacacaaatccaattttgatgttaaaagtcaacatacatagataggtccctcatgttgacagagcacagaattggaaaaaaaaactgcaaatgagaaataggggtatttctaaatcttctgtattcctaaaatatcacactgcgcccttgcttcagcctccctgatagactggtttgggtgtgcaatattaatgcaggaatacgtggaataccagcacaaagccggggagggagactagcaaactctcgccatcaattatttctcaactacatttagtattcttcgcagttttagatttttttttcctttaagcgaaaaccactccactgaaaaaaattccaaacttgttttttaaaaattgcaggaatttcttcgtattttatcaacaaaaataccagaaattaaagagctgacagaaattcaagcagatccaaattcaaccatccatttttcatacttctccaagtctgcagcagagacagacttagcaattttctttagggccaattcaaagtctcctttggtaacaggcatctgaagttcctctttagaaagtgcacggatttcttctggacttaagccattgatacgccgtctcattgccattaaagaggcatccctgcaaacattagtgatgtcagcaccagaatagccctcaatcttctcggctatatcttccagttgaatatcaggatctaattcgacctcacgaaggttgatcttcagaagctcagctcttccttttgctgttgggagaggtatatatatccttttttctaaccttcttcgcaaagcttcatcaatgtcccacgggaaattagtagcagccaataccataaccattttggaaggatcatcattttctaaagctcctccaactccatccatctgaatgagcagttcagacttgaccctgcgacttgcctcatgttcatcagaggttcctcttcgactgcagatagaatctatctcatcaatgaagatcgtggtaggggcataaaatctagccatctcaaacaacagacgaactaacttctcagattcacctctgtatttagatgtcagtgtagaagacgaaacgttgaagaatgttgtaccacattcagtggcaacagctttagctagcatagttttaccagtgcctgggggtccaaccatcagtacacccttccatggccttctaatccctttgaaaaagtcaggcatccacattggaagaacaacagcttcccttagcaacttcttagcttcttccagatctgctatgtcatcccaatgaatgctaggattcctggatacaatgtctctttcaagggcttccaccagatccttatcataaccagcaccatcaaattttggcatttcaccatcacttgcaccatcttgcatattcttccttccctgtgttctgcaggaacagggggtggccaaacagcaggatctctaaatggttcatcttgacaggacacagggaaatctggaggcttgtcaattttaaaactttctaaagtgctgacaatacttttaacttgttcatattcctccaataattcctgccgaacctgttgccatttgcctttgatagctggatctctgactgactggcaatgtctctgaatctgctgcatcaccccctggtaatataccattgatgagtcgtaatttccaagaagggcatattctcttcctttctttgcattatcacaaatctcagccaaattcatcttctttcagagacctgttaaaacacggtttctcaggtctcacatccaatgtgtgacatacatacggttctgcaccgaaaggcagcaacctgcgagggtcagaggcgccgaagacccgaggccctgcagcttgggcggctgctcatccctgagactgtgcagggcggtggcccagccggggtggggctgagcgctgcaactggggcgggcccagctacagggcgggaagcccgaggctcacctccacttccctttcccaacgcacagagcccaggtccgcgaccactcaacagccccctcaagacaaagagag

SEQ ID NO: 8502 - RNA, 3511 nt, Homo sapiens
  source 1..3511: mol_type = other RNA
aaaagtaattgcggtttttgccattgaaagtaatggaaaaaccacaattacttttgcaccaacccattacaaacaagttttaacaatcacaagactaatgttttagtgacggctcctaaaacttcagggaaaaaaaaagtgcatttctgactggcaatagtttgcaaaataatcgtaatgaaactacttatttctttattttaaaagttaataaaaggaaacctctcaatttttaggaagaattcaattacaataaaatcatgatgtcttatgatctggcatcttataatctgtgtctcagaaagaagggcaatttacagcatcagatgaatactggagtttaggtcagacttaagttatctgaaaagaacataaggcatttacagtttttagcagggaaaaataatcaaatctctttttttaaaaaaaaccttcttagtatcttggttaaatgtccaaaaagctgtattatttttagttttaaaccagtaggcactattcgaaactgagaattcaggatgttatcaaatacaaatttttaaaagcttgaccattaaagcataaattgcctaatgagacacatgtaatcataaaaactaacgccaggatcatttacttgtgattggatatatgccatttatttttctggcttctttctaatgtgtaattcctgctgaattgagtgagcatgtcagatttctatctttatcttagtgtgtgtaaaagttctcaacctagacaaggacaaattttagaattttccaatgaacatcattcactatgtatgatgctgttttgttaaactagctgtttggaaaacaataaagatttcatttgttttgcgttagccacagagagtggacttgtttagaatgtaaaagtatttatctcaaatactaaaatcaaactcaagaaaaatcaaacaatgctggagctgagaaaaataatggctatatatctggttgaacatgttgaaagaaaagtgaaaacacagccaggcatggtggtgcgcacctgtaatcccagctacttgggaggctgagacaggagaattgcttgaatctaggaggcagaggttgcagtgagccaagatcaaccactgcactacacagcctgggtgacacagactccttcacgcacacacaaaaaagtgaaaacaaacttggaagtctagaatgaagaattacatctaatgcagtaatattcttcccacctttccatattaaatgtaagaagcaccagcaaaaaatactaaagacagagaaatgacctggcaaaatgattcaaataccacagagcgtgagaatattcctcagtaaagctcaagatattatgaagtagctagcagaagaaatggcaggggtagcggaagtaaaaattctaaccatatgacagactctaacagtaagtcataaattctaaaggtttaattagtaaattcattatttcctccaaaatatactgtcattcttctcttaacaatgaatgtttgacacaaatccaattttgatgttaaaagtcaacatacatagataggtccctcatgttgacagagcacagaattggaaaaaaaaactgcaaatgagaaataggggtatttctaaatcttctgtattcctaaaatatcacactgcgcccttgcttcagcctccctgatagactggtttgggtgtgcaatattaatgcaggaatacgtggaataccagcacaaagccggggagggagactagcaaactctcgccatcaattatttctcaactacatttagtattcttcgcagttttagatttttttttcctttaagcgaaaaccactccactgaaaaaaattccaaacttgttttttaaaaattgcaggaatttcttcgtattttatcaacaaaaataccagaaattaaagagctgacagaaattcaagcagatccaaattcaaccatccatttttcatacttctccaagtctgcagcagagacagacttagcaattttctttagggccaattcaaagtctcctttggtaacaggcatctgaagttcctctttagaaagtgcacggatttcttctggacttaagccattgatacgccgtctcattgccattaaagaggcatccctgcaaacattagtgatgtcagcaccagaatagccctcaatcttctcggctatatcttccagttgaatatcaggatctaattcgacctcacgaaggttgatcttcagaagctcagctcttccttttgctgttgggagaggtatatatatccttttttctaaccttcttcgcaaagcttcatcaatgtcccacgggaaattagtagcagccaataccataaccattttggaaggatcatcattttctaaagctcctccaactccatccatctgaatgagcagttcagacttgaccctgcgacttgcctcatgttcatcagaggttcctcttcgactgcagatagaatctatctcatcaatgaagatcgtggtaggggcataaaatctagccatctcaaacaacagacgaactaacttctcagattcacctctgtatttagatgtcagtgtagaagacgaaacgttgaagaatgttgtaccacattcagtggcaacagctttagctagcatagttttaccagtgcctgggggtccaaccatcagtacacccttccatggccttctaatccctttgaaaaagtcaggcatccacattggaagaacaacagcttcccttagcaacttcttagcttcttccagatctgctatgtcatcccaatgaatgctaggattcctggatacaatgtctctttcaagggcttccaccagatccttatcataaccagcaccatcaaattttggcatttcaccatcacttgcaccatcttgcatattcttccttcccttgtcatctctccctcttgctctatagtccttgtccctacttgtagaaggcttttcactctttgatataggatgtgctcggcctacaggtccccgggctcctactcctgccatttctttcctcagaggtcttacttctcgattgggacgcctgatctgaggtggagctctgtgttctgcaggaacagggggtggccaaacagcaggatctctaaatggttcatcttgacaggacacagggaaatctggaggcttgtcaattttaaaactttctaaagtgctgacaatacttttaacttgttcatattcctccaataattcctgccgaacctgttgccatttgcctttgatagctggatctctgactgactggcaatgtctctgaatctgctgcatcaccccctggtaatataccattgatgagtcgtaatttccaagaagggcatattctcttcctttctttgcattatcacaaatctcagccaaattcatcttctttcagagacatacggttctgcaccgaaaggcagcaacctgcgagggtcagaggcgccgaagacccgaggccctgcagcttgggcggctgctcatccctgagactgtgcagggcggtggccc

SEQ ID NO: 8503 - RNA, 3592 nt, Homo sapiens
  source 1..3592: mol_type = other RNA
aaaagtaattgcggtttttgccattgaaagtaatggaaaaaccacaattacttttgcaccaacccattacaaacaagttttaacaatcacaagactaatgttttagtgacggctcctaaaacttcagggaaaaaaaaagtgcatttctgactggcaatagtttgcaaaataatcgtaatgaaactacttatttctttattttaaaagttaataaaaggaaacctctcaatttttaggaagaattcaattacaataaaatcatgatgtcttatgatctggcatcttataatctgtgtctcagaaagaagggcaatttacagcatcagatgaatactggagtttaggtcagacttaagttatctgaaaagaacataaggcatttacagtttttagcagggaaaaataatcaaatctctttttttaaaaaaaaccttcttagtatcttggttaaatgtccaaaaagctgtattatttttagttttaaaccagtaggcactattcgaaactgagaattcaggatgttatcaaatacaaatttttaaaagcttgaccattaaagcataaattgcctaatgagacacatgtaatcataaaaactaacgccaggatcatttacttgtgattggatatatgccatttatttttctggcttctttctaatgtgtaattcctgctgaattgagtgagcatgtcagatttctatctttatcttagtgtgtgtaaaagttctcaacctagacaaggacaaattttagaattttccaatgaacatcattcactatgtatgatgctgttttgttaaactagctgtttggaaaacaataaagatttcatttgttttgcgttagccacagagagtggacttgtttagaatgtaaaagtatttatctcaaatactaaaatcaaactcaagaaaaatcaaacaatgctggagctgagaaaaataatggctatatatctggttgaacatgttgaaagaaaagtgaaaacacagccaggcatggtggtgcgcacctgtaatcccagctacttgggaggctgagacaggagaattgcttgaatctaggaggcagaggttgcagtgagccaagatcaaccactgcactacacagcctgggtgacacagactccttcacgcacacacaaaaaagtgaaaacaaacttggaagtctagaatgaagaattacatctaatgcagtaatattcttcccacctttccatattaaatgtaagaagcaccagcaaaaaatactaaagacagagaaatgacctggcaaaatgattcaaataccacagagcgtgagaatattcctcagtaaagctcaagatattatgaagtagctagcagaagaaatggcaggggtagcggaagtaaaaattctaaccatatgacagactctaacagtaagtcataaattctaaaggtttaattagtaaattcattatttcctccaaaatatactgtcattcttctcttaacaatgaatgtttgacacaaatccaattttgatgttaaaagtcaacatacatagataggtccctcatgttgacagagcacagaattggaaaaaaaaactgcaaatgagaaataggggtatttctaaatcttctgtattcctaaaatatcacactgcgcccttgcttcagcctccctgatagactggtttgggtgtgcaatattaatgcaggaatacgtggaataccagcacaaagccggggagggagactagcaaactctcgccatcaattatttctcaactacatttagtattcttcgcagttttagatttttttttcctttaagcgaaaaccactccactgaaaaaaattccaaacttgttttttaaaaattgcaggaatttcttcgtattttatcaacaaaaataccagaaattaaagagctgacagaaattcaagcagatccaaattcaaccatccatttttcatacttctccaagtctgcagcagagacagacttagcaattttctttagggccaattcaaagtctcctttggtaacaggcatctgaagttcctctttagaaagtgcacggatttcttctggacttaagccattgatacgccgtctcattgccattaaagaggcatccctgcaaacattagtgatgtcagcaccagaatagccctcaatcttctcggctatatcttccagttgaatatcaggatctaattcgacctcacgaaggttgatcttcagaagctcagctcttccttttgctgttgggagaggtatatatatccttttttctaaccttcttcgcaaagcttcatcaatgtcccacgggaaattagtagcagccaataccataaccattttggaaggatcatcattttctaaagctcctccaactccatccatctgaatgagcagttcagacttgaccctgcgacttgcctcatgttcatcagaggttcctcttcgactgcagatagaatctatctcatcaatgaagatcgtggtaggggcataaaatctagccatctcaaacaacagacgaactaacttctcagattcacctctgtatttagatgtcagtgtagaagacgaaacgttgaagaatgttgtaccacattcagtggcaacagctttagctagcatagttttaccagtgcctgggggtccaaccatcagtacacccttccatggccttctaatccctttgaaaaagtcaggcatccacattggaagaacaacagcttcccttagcaacttcttagcttcttccagatctgctatgtcatcccaatgaatgctaggattcctggatacaatgtctctttcaagggcttccaccagatccttatcataaccagcaccatcaaattttggcatttcaccatcacttgcaccatcttgcatattcttccttcccttgtcatctctccctcttgctctatagtccttgtccctacttgtagaaggcttttcactctttgatataggatgtgctcggcctacaggtccccgggctcctactcctgccatttctttcctcagaggtcttacttctcgattgggacgcctgatctgaggtggagctctgtgttctgcaggaacagggggtggccaaacagcaggatctctaaatggttcatcttgacaggacacagggaaatctggaggcttgtcaattttaaaactttctaaagtgctgacaatacttttaacttgttcatattcctccaataattcctgccgaacctgttgccatttgcctttgatagctggatctctgactgactggcaatgtctctgaatctgctgcatcaccccctggtaatataccattgatgagtcgtaatttccaagaagggcatattctcttcctttctttgcattatcacaaatctcagccaaattcatcttctttcagagacccagaaataaacgtatccaggaaaggagaaaaacctgttaaaacacggtttctcaggtctcacatccaatgtgtgacatacatacggttctgcaccgaaaggcagcaacctgcgagggtcagaggcgccgaagacccgaggccctgcagcttgggcggctgctcatccctgagactgtgcagggcggtggccc

SEQ ID NO: 8504 - RNA, 3620 nt, Homo sapiens
  source 1..3620: mol_type = other RNA
aaaagtaattgcggtttttgccattgaaagtaatggaaaaaccacaattacttttgcaccaacccattacaaacaagttttaacaatcacaagactaatgttttagtgacggctcctaaaacttcagggaaaaaaaaagtgcatttctgactggcaatagtttgcaaaataatcgtaatgaaactacttatttctttattttaaaagttaataaaaggaaacctctcaatttttaggaagaattcaattacaataaaatcatgatgtcttatgatctggcatcttataatctgtgtctcagaaagaagggcaatttacagcatcagatgaatactggagtttaggtcagacttaagttatctgaaaagaacataaggcatttacagtttttagcagggaaaaataatcaaatctctttttttaaaaaaaaccttcttagtatcttggttaaatgtccaaaaagctgtattatttttagttttaaaccagtaggcactattcgaaactgagaattcaggatgttatcaaatacaaatttttaaaagcttgaccattaaagcataaattgcctaatgagacacatgtaatcataaaaactaacgccaggatcatttacttgtgattggatatatgccatttatttttctggcttctttctaatgtgtaattcctgctgaattgagtgagcatgtcagatttctatctttatcttagtgtgtgtaaaagttctcaacctagacaaggacaaattttagaattttccaatgaacatcattcactatgtatgatgctgttttgttaaactagctgtttggaaaacaataaagatttcatttgttttgcgttagccacagagagtggacttgtttagaatgtaaaagtatttatctcaaatactaaaatcaaactcaagaaaaatcaaacaatgctggagctgagaaaaataatggctatatatctggttgaacatgttgaaagaaaagtgaaaacacagccaggcatggtggtgcgcacctgtaatcccagctacttgggaggctgagacaggagaattgcttgaatctaggaggcagaggttgcagtgagccaagatcaaccactgcactacacagcctgggtgacacagactccttcacgcacacacaaaaaagtgaaaacaaacttggaagtctagaatgaagaattacatctaatgcagtaatattcttcccacctttccatattaaatgtaagaagcaccagcaaaaaatactaaagacagagaaatgacctggcaaaatgattcaaataccacagagcgtgagaatattcctcagtaaagctcaagatattatgaagtagctagcagaagaaatggcaggggtagcggaagtaaaaattctaaccatatgacagactctaacagtaagtcataaattctaaaggtttaattagtaaattcattatttcctccaaaatatactgtcattcttctcttaacaatgaatgtttgacacaaatccaattttgatgttaaaagtcaacatacatagataggtccctcatgttgacagagcacagaattggaaaaaaaaactgcaaatgagaaataggggtatttctaaatcttctgtattcctaaaatatcacactgcgcccttgcttcagcctccctgatagactggtttgggtgtgcaatattaatgcaggaatacgtggaataccagcacaaagccggggagggagactagcaaactctcgccatcaattatttctcaactacatttagtattcttcgcagttttagatttttttttcctttaagcgaaaaccactccactgaaaaaaattccaaacttgttttttaaaaattgcaggaatttcttcgtattttatcaacaaaaataccagaaattaaagagctgacagaaattcaagcagatccaaattcaaccatccatttttcatacttctccaagtctgcagcagagacagacttagcaattttctttagggccaattcaaagtctcctttggtaacaggcatctgaagttcctctttagaaagtgcacggatttcttctggacttaagccattgatacgccgtctcattgccattaaagaggcatccctgcaaacattagtgatgtcagcaccagaatagccctcaatcttctcggctatatcttccagttgaatatcaggatctaattcgacctcacgaaggttgatcttcagaagctcagctcttccttttgctgttgggagaggtatatatatccttttttctaaccttcttcgcaaagcttcatcaatgtcccacgggaaattagtagcagccaataccataaccattttggaaggatcatcattttctaaagctcctccaactccatccatctgaatgagcagttcagacttgaccctgcgacttgcctcatgttcatcagaggttcctcttcgactgcagatagaatctatctcatcaatgaagatcgtggtaggggcataaaatctagccatctcaaacaacagacgaactaacttctcagattcacctctgtatttagatgtcagtgtagaagacgaaacgttgaagaatgttgtaccacattcagtggcaacagctttagctagcatagttttaccagtgcctgggggtccaaccatcagtacacccttccatggccttctaatccctttgaaaaagtcaggcatccacattggaagaacaacagcttcccttagcaacttcttagcttcttccagatctgctatgtcatcccaatgaatgctaggattcctggatacaatgtctctttcaagggcttccaccagatccttatcataaccagcaccatcaaattttggcatttcaccatcacttgcaccatcttgcatattcttccttcccttgtcatctctccctcttgctctatagtccttgtccctacttgtagaaggcttttcactctttgatataggatgtgctcggcctacaggtccccgggctcctactcctgccatttctttcctcagaggtcttacttctcgattgggacgcctgatctgaggtggagctctgtgttctgcaggaacagggggtggccaaacagcaggatctctaaatggttcatcttgacaggacacagggaaatctggaggcttgtcaattttaaaactttctaaagtgctgacaatacttttaacttgttcatattcctccaataattcctgccgaacctgttgccatttgcctttgatagctggatctctgactgactggcaatgtctctgaatctgctgcatcaccccctggtaatataccattgatgagtcgtaatttccaagaagggcatattctcttcctttctttgcattatcacaaatctcagccaaattcatcttctttcagagacccagaaggcgcaggtccgggcacattcagcgatgcggtccagatggggtgcgggtggggcgcaggccgccgccgccgccgccgccgagtccgttagctcgcgacgtgcgtgaaaaggcggcggcggcgtagtgttgccatggcagccgcggccgcgcggtgggcgcagcgcgggagggagcgcgggggctgtgagtccgctctggggcggagcttgggact

SEQ ID NO: 8505 - RNA, 3471 nt, Homo sapiens
  source 1..3471: mol_type = other RNA
aaaagtaattgcggtttttgccattgaaagtaatggaaaaaccacaattacttttgcaccaacccattacaaacaagttttaacaatcacaagactaatgttttagtgacggctcctaaaacttcagggaaaaaaaaagtgcatttctgactggcaatagtttgcaaaataatcgtaatgaaactacttatttctttattttaaaagttaataaaaggaaacctctcaatttttaggaagaattcaattacaataaaatcatgatgtcttatgatctggcatcttataatctgtgtctcagaaagaagggcaatttacagcatcagatgaatactggagtttaggtcagacttaagttatctgaaaagaacataaggcatttacagtttttagcagggaaaaataatcaaatctctttttttaaaaaaaaccttcttagtatcttggttaaatgtccaaaaagctgtattatttttagttttaaaccagtaggcactattcgaaactgagaattcaggatgttatcaaatacaaatttttaaaagcttgaccattaaagcataaattgcctaatgagacacatgtaatcataaaaactaacgccaggatcatttacttgtgattggatatatgccatttatttttctggcttctttctaatgtgtaattcctgctgaattgagtgagcatgtcagatttctatctttatcttagtgtgtgtaaaagttctcaacctagacaaggacaaattttagaattttccaatgaacatcattcactatgtatgatgctgttttgttaaactagctgtttggaaaacaataaagatttcatttgttttgcgttagccacagagagtggacttgtttagaatgtaaaagtatttatctcaaatactaaaatcaaactcaagaaaaatcaaacaatgctggagctgagaaaaataatggctatatatctggttgaacatgttgaaagaaaagtgaaaacacagccaggcatggtggtgcgcacctgtaatcccagctacttgggaggctgagacaggagaattgcttgaatctaggaggcagaggttgcagtgagccaagatcaaccactgcactacacagcctgggtgacacagactccttcacgcacacacaaaaaagtgaaaacaaacttggaagtctagaatgaagaattacatctaatgcagtaatattcttcccacctttccatattaaatgtaagaagcaccagcaaaaaatactaaagacagagaaatgacctggcaaaatgattcaaataccacagagcgtgagaatattcctcagtaaagctcaagatattatgaagtagctagcagaagaaatggcaggggtagcggaagtaaaaattctaaccatatgacagactctaacagtaagtcataaattctaaaggtttaattagtaaattcattatttcctccaaaatatactgtcattcttctcttaacaatgaatgtttgacacaaatccaattttgatgttaaaagtcaacatacatagataggtccctcatgttgacagagcacagaattggaaaaaaaaactgcaaatgagaaataggggtatttctaaatcttctgtattcctaaaatatcacactgcgcccttgcttcagcctccctgatagactggtttgggtgtgcaatattaatgcaggaatacgtggaataccagcacaaagccggggagggagactagcaaactctcgccatcaattatttctcaactacatttagtattcttcgcagttttagatttttttttcctttaagcgaaaaccactccactgaaaaaaattccaaacttgttttttaaaaattgcaggaatttcttcgtattttatcaacaaaaataccagaaattaaagagctgacagaaattcaagcagatccaaattcaaccatccatttttcatacttctccaagtctgcagcagagacagacttagcaattttctttagggccaattcaaagtctcctttggtaacaggcatctgaagttcctctttagaaagtgcacggatttcttctggacttaagccattgatacgccgtctcattgccattaaagaggcatccctgcaaacattagtgatgtcagcaccagaatagccctcaatcttctcggctatatcttccagttgaatatcaggatctaattcgacctcacgaaggttgatcttcagaagctcagctcttccttttgctgttgggagaggtatatatatccttttttctaaccttcttcgcaaagcttcatcaatgtcccacgggaaattagtagcagccaataccataaccattttggaaggatcatcattttctaaagctcctccaactccatccatctgaatgagcagttcagacttgaccctgcgacttgcctcatgttcatcagaggttcctcttcgactgcagatagaatctatctcatcaatgaagatcgtggtaggggcataaaatctagccatctcaaacaacagacgaactaacttctcagattcacctctgtatttagatgtcagtgtagaagacgaaacgttgaagaatgttgtaccacattcagtggcaacagctttagctagcatagttttaccagtgcctgggggtccaaccatcagtacacccttccatggccttctaatccctttgaaaaagtcaggcatccacattggaagaacaacagcttcccttagcaacttcttagcttcttccagatctgctatgtcatcccaatgaatgctaggattcctggatacaatgtctctttcaagggcttccaccagatccttatcataaccagcaccatcaaattttggcatttcaccatcacttgcaccatcttgcatattcttccttcccttgtcatctctccctcttgctctatagtccttgtccctacttgtagaaggcttttcactctttgatataggatgtgctcggcctacaggtccccgggctcctactcctgccatttctttcctcagaggtcttacttctcgattgggacgcctgatctgaggtggagctctgtgttctgcaggaacagggggtggccaaacagcaggatctctaaatggttcatcttgacaggacacagggaaatctggaggcttgtcaattttaaaactttctaaagtgctgacaatacttttaacttgttcatattcctccaataattcctgccgaacctgttgccatttgcctttgatagctggatctctgactgactggcaatgtctctgaatctgctgcatcaccccctggtaatataccattgatgagtcgtaatttccaagaagggcatattctcttcctttctttgcattatcacaaatctcagccaaattcatcttctttcagagacctccacttccctttcccaacgcacagagcccaggtccgcgaccactcaacagccccctcaagacaaagagag

SEQ ID NO: 8506 - RNA, 3698 nt, Homo sapiens
  source 1..3698: mol_type = other RNA
aaaagtaattgcggtttttgccattgaaagtaatggaaaaaccacaattacttttgcaccaacccattacaaacaagttttaacaatcacaagactaatgttttagtgacggctcctaaaacttcagggaaaaaaaaagtgcatttctgactggcaatagtttgcaaaataatcgtaatgaaactacttatttctttattttaaaagttaataaaaggaaacctctcaatttttaggaagaattcaattacaataaaatcatgatgtcttatgatctggcatcttataatctgtgtctcagaaagaagggcaatttacagcatcagatgaatactggagtttaggtcagacttaagttatctgaaaagaacataaggcatttacagtttttagcagggaaaaataatcaaatctctttttttaaaaaaaaccttcttagtatcttggttaaatgtccaaaaagctgtattatttttagttttaaaccagtaggcactattcgaaactgagaattcaggatgttatcaaatacaaatttttaaaagcttgaccattaaagcataaattgcctaatgagacacatgtaatcataaaaactaacgccaggatcatttacttgtgattggatatatgccatttatttttctggcttctttctaatgtgtaattcctgctgaattgagtgagcatgtcagatttctatctttatcttagtgtgtgtaaaagttctcaacctagacaaggacaaattttagaattttccaatgaacatcattcactatgtatgatgctgttttgttaaactagctgtttggaaaacaataaagatttcatttgttttgcgttagccacagagagtggacttgtttagaatgtaaaagtatttatctcaaatactaaaatcaaactcaagaaaaatcaaacaatgctggagctgagaaaaataatggctatatatctggttgaacatgttgaaagaaaagtgaaaacacagccaggcatggtggtgcgcacctgtaatcccagctacttgggaggctgagacaggagaattgcttgaatctaggaggcagaggttgcagtgagccaagatcaaccactgcactacacagcctgggtgacacagactccttcacgcacacacaaaaaagtgaaaacaaacttggaagtctagaatgaagaattacatctaatgcagtaatattcttcccacctttccatattaaatgtaagaagcaccagcaaaaaatactaaagacagagaaatgacctggcaaaatgattcaaataccacagagcgtgagaatattcctcagtaaagctcaagatattatgaagtagctagcagaagaaatggcaggggtagcggaagtaaaaattctaaccatatgacagactctaacagtaagtcataaattctaaaggtttaattagtaaattcattatttcctccaaaatatactgtcattcttctcttaacaatgaatgtttgacacaaatccaattttgatgttaaaagtcaacatacatagataggtccctcatgttgacagagcacagaattggaaaaaaaaactgcaaatgagaaataggggtatttctaaatcttctgtattcctaaaatatcacactgcgcccttgcttcagcctccctgatagactggtttgggtgtgcaatattaatgcaggaatacgtggaataccagcacaaagccggggagggagactagcaaactctcgccatcaattatttctcaactacatttagtattcttcgcagttttagatttttttttcctttaagcgaaaaccactccactgaaaaaaattccaaacttgttttttaaaaattgcaggaatttcttcgtattttatcaacaaaaataccagaaattaaagagctgacagaaattcaagcagatccaaattcaaccatccatttttcatacttctccaagtctgcagcagagacagacttagcaattttctttagggccaattcaaagtctcctttggtaacaggcatctgaagttcctctttagaaagtgcacggatttcttctggacttaagccattgatacgccgtctcattgccattaaagaggcatccctgcaaacattagtgatgtcagcaccagaatagccctcaatcttctcggctatatcttccagttgaatatcaggatctaattcgacctcacgaaggttgatcttcagaagctcagctcttccttttgctgttgggagaggtatatatatccttttttctaaccttcttcgcaaagcttcatcaatgtcccacgggaaattagtagcagccaataccataaccattttggaaggatcatcattttctaaagctcctccaactccatccatctgaatgagcagttcagacttgaccctgcgacttgcctcatgttcatcagaggttcctcttcgactgcagatagaatctatctcatcaatgaagatcgtggtaggggcataaaatctagccatctcaaacaacagacgaactaacttctcagattcacctctgtatttagatgtcagtgtagaagacgaaacgttgaagaatgttgtaccacattcagtggcaacagctttagctagcatagttttaccagtgcctgggggtccaaccatcagtacacccttccatggccttctaatccctttgaaaaagtcaggcatccacattggaagaacaacagcttcccttagcaacttcttagcttcttccagatctgctatgtcatcccaatgaatgctaggattcctggatacaatgtctctttcaagggcttccaccagatccttatcataaccagcaccatcaaattttggcatttcaccatcacttgcaccatcttgcatattcttccttcccttgtcatctctccctcttgctctatagtccttgtccctacttgtagaaggcttttcactctttgatataggatgtgctcggcctacaggtccccgggctcctactcctgccatttctttcctcagaggtcttacttctcgattgggacgcctgatctgaggtggagctctgtgttctgcaggaacagggggtggccaaacagcaggatctctaaatggttcatcttgacaggacacagggaaatctggaggcttgtcaattttaaaactttctaaagtgctgacaatacttttaacttgttcatattcctccaataattcctgccgaacctgttgccatttgcctttgatagctggatctctgactgactggcaatgtctctgaatctgctgcatcaccccctggtaatataccattgatgagtcgtaatttccaagaagggcatattctcttcctttctttgcattatcacaaatctcagccaaattcatcttctttcagagacctgttaaaacacggtttctcaggtctcacatccaatgtgtgacatacatacggttctgcaccgaaaggcagcaacctgcgagggtcagaggcgccgaagacccgaggccctgcagcttgggcggctgctcatccctgagactgtgcagggcggtggcccagccggggtggggctgagcgctgcaactggggcgggcccagctacagggcgggaagcccgaggctcacctccacttccctttcccaacgcacagagcccaggtccgcgaccactcaacagccccctcaagacaaagagag

SEQ ID NO: 8507 - RNA, 3730 nt, Homo sapiens
  source 1..3730: mol_type = other RNA
aaaagtaattgcggtttttgccattgaaagtaatggaaaaaccacaattacttttgcaccaacccattacaaacaagttttaacaatcacaagactaatgttttagtgacggctcctaaaacttcagggaaaaaaaaagtgcatttctgactggcaatagtttgcaaaataatcgtaatgaaactacttatttctttattttaaaagttaataaaaggaaacctctcaatttttaggaagaattcaattacaataaaatcatgatgtcttatgatctggcatcttataatctgtgtctcagaaagaagggcaatttacagcatcagatgaatactggagtttaggtcagacttaagttatctgaaaagaacataaggcatttacagtttttagcagggaaaaataatcaaatctctttttttaaaaaaaaccttcttagtatcttggttaaatgtccaaaaagctgtattatttttagttttaaaccagtaggcactattcgaaactgagaattcaggatgttatcaaatacaaatttttaaaagcttgaccattaaagcataaattgcctaatgagacacatgtaatcataaaaactaacgccaggatcatttacttgtgattggatatatgccatttatttttctggcttctttctaatgtgtaattcctgctgaattgagtgagcatgtcagatttctatctttatcttagtgtgtgtaaaagttctcaacctagacaaggacaaattttagaattttccaatgaacatcattcactatgtatgatgctgttttgttaaactagctgtttggaaaacaataaagatttcatttgttttgcgttagccacagagagtggacttgtttagaatgtaaaagtatttatctcaaatactaaaatcaaactcaagaaaaatcaaacaatgctggagctgagaaaaataatggctatatatctggttgaacatgttgaaagaaaagtgaaaacacagccaggcatggtggtgcgcacctgtaatcccagctacttgggaggctgagacaggagaattgcttgaatctaggaggcagaggttgcagtgagccaagatcaaccactgcactacacagcctgggtgacacagactccttcacgcacacacaaaaaagtgaaaacaaacttggaagtctagaatgaagaattacatctaatgcagtaatattcttcccacctttccatattaaatgtaagaagcaccagcaaaaaatactaaagacagagaaatgacctggcaaaatgattcaaataccacagagcgtgagaatattcctcagtaaagctcaagatattatgaagtagctagcagaagaaatggcaggggtagcggaagtaaaaattctaaccatatgacagactctaacagtaagtcataaattctaaaggtttaattagtaaattcattatttcctccaaaatatactgtcattcttctcttaacaatgaatgtttgacacaaatccaattttgatgttaaaagtcaacatacatagataggtccctcatgttgacagagcacagaattggaaaaaaaaactgcaaatgagaaataggggtatttctaaatcttctgtattcctaaaatatcacactgcgcccttgcttcagcctccctgatagactggtttgggtgtgcaatattaatgcaggaatacgtggaataccagcacaaagccggggagggagactagcaaactctcgccatcaattatttctcaactacatttagtattcttcgcagttttagatttttttttcctttaagcgaaaaccactccactgaaaaaaattccaaacttgttttttaaaaattgcaggaatttcttcgtattttatcaacaaaaataccagaaattaaagagctgacagaaattcaagcagatccaaattcaaccatccatttttcatacttctccaagtctgcagcagagacagacttagcaattttctttagggccaattcaaagtctcctttggtaacaggcatctgaagttcctctttagaaagtgcacggatttcttctggacttaagccattgatacgccgtctcattgccattaaagaggcatccctgcaaacattagtgatgtcagcaccagaatagccctcaatcttctcggctatatcttccagttgaatatcaggatctaattcgacctcacgaaggttgatcttcagaagctcagctcttccttttgctgttgggagaggtatatatatccttttttctaaccttcttcgcaaagcttcatcaatgtcccacgggaaattagtagcagccaataccataaccattttggaaggatcatcattttctaaagctcctccaactccatccatctgaatgagcagttcagacttgaccctgcgacttgcctcatgttcatcagaggttcctcttcgactgcagatagaatctatctcatcaatgaagatcgtggtaggggcataaaatctagccatctcaaacaacagacgaactaacttctcagattcacctctgtatttagatgtcagtgtagaagacgaaacgttgaagaatgttgtaccacattcagtggcaacagctttagctagcatagttttaccagtgcctgggggtccaaccatcagtacacccttccatggccttctaatccctttgaaaaagtcaggcatccacattggaagaacaacagcttcccttagcaacttcttagcttcttccagatctgctatgtcatcccaatgaatgctaggattcctggatacaatgtctctttcaagggcttccaccagatccttatcataaccagcaccatcaaattttggcatttcaccatcacttgcaccatcttgcatattcttccttcctgaaaaacagcattttaagcttggatctaacctgaagcctgtcagtaattttaaaaaagaaaaagaaaaaagacataatcagtctcagaaaataaactcgtattattataagaagacagtaagcattttcaaataagagtctgtatagcataatgattaaaaaactcaggtattacacatagacaaggttcaaatcctagttcaccatctatttgcagttaagacttcagtgtctcaatttctctacacataaaacaggaaaaataatgctgagctcacaggattatgcagggatcaaataaaccaataaatgtaaaaagcttcaaagcgggctttttttgtagaaagcttcaaaaaggataagtgcgctcaaggaagactaacatttgctactactgctattattagttgttccatcatacagttcccaacaccaaattaaaaatccaaaaatataccagggaccttaagcaagatatgtctaacttctcttatcctcaattttttttacatctataaagttaagtacatagttagagtgctgcagcagctttcaaaattctgacccaggcacaaagtaataaatgcattctggatcatgagctggtgtacataaacatatgaataaatttgtatatatttttatcaaaataatactgtacttatgggcaataaactgagttttctgttctactctgcttcaattttaaagctggcagcaatacacaaaactgatcttaagaaaaacaaatacaataaacactggggactcccatatctctgagggtacttccaaacaacactaattttcctttcttttttttttttttgagacca

SEQ ID NO: 8508 - RNA, 2984 nt, Homo sapiens
  source 1..2984: mol_type = other RNA
aaaagtaattgcggtttttgctgcaattaaaggttatggcaaaaaccacaattacttttgcaccaacctaatagctatctatctagggctagggctatctatctagggctagggctatcgatctagggctgttaaaagtgtattcaacccaaggtatctaatacacatagtttataatggcatgtgagaaataaactccttccttaaaagattaaatattacttctttttccaaaacctaaattgtttcatcaatttccactagaaatgtatcttcaataagcaggctgggcacagtagctcatgcctataatcccagcactttcgacggccaagttgggaggactgcctgagctcaagagttcgagaccagctggggcaatatagtgagactctgtctctatttaataaataaaaaggataattaaaaaaataataagcataatggtgtagacctggtaaatcttttgacagcaacgtttataacccacatgccatgtatttcactacattcataaaggggcttggggatttatccagaatgacataccattcatttcaaaataacatacatcttttctctagacagctaagaatatttatagttgttaaagcaaaaagaaattcttggtaacaagttcttggtgtatggattgctttggctttgatggaaatatctactttctccaaagattggtccctgggcctcaaagcatttaccccaagaaataactgctatgacttaggtcttcaaggcagcttccagtgctcgagctttctctgtgatgttcttctgaaaaggcatcataaaatcgtcgaagtccacctcatgtgtaaacctctctcgccgtagttccctcttcctgatcagctctgctgttgtggcttcaggactccaaatcctccgtggaataaatgtgatatccactttcttagtataaccactggtaatcaatgaattcagatgaaccacattacccttctgtactttctttccctctgatgtggttggtacaccataaattgatgacagcagttcctcttctttcttaatttcagggccttcagtcttcagtataggaggtgtcttgccttttagtttttgattttctgctggtttcggcaagttatctagcttttctttaatcagatcaattattctataatcagcatatgcctttgcaacgtccatggcactatgcccttttctattttccagctggaatttagcaccaatatcaagtaggtattttactgtatccagtctgcagctttcaatggctctatttaaaggagttgagttgttgattgaagctgcatctattaaagctccagattcaacaagaagctcaacaatgtcttgttggcctgcatggcatgcaaaatgaagtggagtccacagaaagttatctgttgcattaacgttagctcctttttcaagaagaaacttgaccacatctatgtttccacttgcacacgccgtcattagcggagttttgtaataattatccttcatatccacaggtattcctgattcaaaggcctttttcagagaagccagatcccctgctttggtgataatattaatgtttgaaaataccttctctgaatcatcaatgtaccaaacagagtcatcctgaatgggatgttctgggggatgatctctattaaaccggctgctatcagtgacattcttgtaggtctcaatcatgtaatacggtggcccaccatcctgccggcgtggaaacgcgtactcaggaatgacacagattggaaggggtaagacaaatttccctttctttccttttttgcccatccctttttcctttttcttaggtccatacgatcctaagacaaaagacttgtttaaatatctggttcctttaaagaattcattaatattgacccctcctccccgggttttctcatgaaggtgagcgatggcagccagctgttctgagcttgcataatcctgcctttcctccaacaccatcacgaagtcgttcttgctgatgcttccatcacccctgtctaaaaccgcaaaggcttcccggaggaaagcctcacgttctacggaccaatcgtgcagtctaagggcccacagtggatttggatttttggctcctggcctggctagtttattagcgattctctctgctcggcgtatttctttgcttgctgctttgaagccgccttccttagccacagccctgggcgttttatgatctaaattcttccatttcaggtcacatcctcgctgagctatatatttacagcagtctgcaaaaccacccatggcagcataatgaagtggtgtgttcccatttatcgaaatcagccccacgtctccattgtaggcaaaaagaagcttcaatatatcgaaaaagcctcctttagcagcaaaatgagcagcgtgatgcctgtcgttgtcaaatgcattcacttcacctcctctttccaatatgcctcgaactatttccactaccccttctcttgacgcttccattaaagctgtgcggcctgtggatgagttgattgcattaggattggctcctttttccaaaaatgtcaggcacacatctttaacatcatgtgcatcttcacaagctctaaggaatattggctttccttcataggtagaattgttgacatctgcaccatgttcaagggcgatcagagcacagcgataatgccgcttagtcggtaaaatgcagtaaaacaaaacacctcttagtcttccgggcgatcagaagccagggatctctgggcacctatgtgcctgggcctgctggggcgaccggggaggcccctgctctcgtcctctgacgctcagcgctggcccagccgcgaccttgggctcccggagcccggcggaggcgcccaggcgtgaatgatgtcccttgggtagggctggtgagctggcgcgcgggacagcagggctgggtgtatgtgtccatgggccccgggtccccggaaggcgagcgc

SEQ ID NO: 8509 - RNA, 3509 nt, Homo sapiens
  source 1..3509: mol_type = other RNA
aaaagtaattgcggtttttgctgcaattaaaggttatggcaaaaaccacaattacttttgcaccaacctaatagctatctatctagggctagggctatctatctagggctagggctatcgatctagggctgttaaaagtgtattcaacccaaggtatctaatacacatagtttataatggcatgtgagaaataaactccttccttaaaagattaaatattacttctttttccaaaacctaaattgtttcatcaatttccactagaaatgtatcttcaataagcaggctgggcacagtagctcatgcctataatcccagcactttcgacggccaagttgggaggactgcctgagctcaagagttcgagaccagctggggcaatatagtgagactctgtctctatttaataaataaaaaggataattaaaaaaataataagcataatggtgtagacctggtaaatcttttgacagcaacgtttataacccacatgccatgtatttcactacattcataaaggggcttggggatttatccagaatgacataccattcatttcaaaataacatacatcttttctctagacagctaagaatatttatagttgttaaagcaaaaagaaattcttggtaacaagttcttggtgtatggattgctttggctttgatggaaatatctactttctccaaagattggtccctgggcctcaaagcatttaccccaagaaataactgctatgacttaggtcttcaaggcagcttccagtgctcgagctttctctgtgatgttcttctgaaaaggcatcataaaatcgtcgaagtccacctcatgtgtaaacctctctcgccgtagttccctcttcctgatcagctctgctgttgtggcttcaggactccaaatcctccgtggaataaatgtgatatccactttcttagtataaccactggtaatcaatgaattcagatgaaccacattacccttctgtactttctttccctctgatgtggttggtacaccataaattgatgacagcagttcctcttctttcttaatttcagggccttcagtcttcagtataggaggtgtcttgccttttagtttttgattttctgctggtttcggcaagttatctagcttttctttaatcagatcaattattctataatcagcatatgcctttgcaacgtccatggcactatgcccttttctattttccagctggaatttagcaccaatatcaagtaggtattttactgtatccagtctgcagctttcaatggctctatttaaaggagttgagttgttgattgaagctgcatctattaaagctccagattcaacaagaagctcaacaatgtcttgttggcctgcatggcatgcaaaatgaagtggagtccacagaaagttatctgttgcattaacgttagctcctttttcaagaagaaacttgaccacatctatgtttccacttgcacacgccgtcattagcggagttttgtaataattatccttcatatccacaggtattcctgattcaaaggcctttttcagagaagccagatcccctgctttggtgataatattaatgtttgaaaataccttctctgaatcatcaatgtaccaaacagagtcatcctgaatgggatgttctgggggatgatctctattaaaccggctgctatcagtgacattcttgtaggtctcaatcatgtaatacggtggcccaccatcctgccggcgtggaaacgcgtactcaggaatgacacagattggaaggggtaagacaaatttccctttctttccttttttgcccatccctttttcctttttcttaggtccatacgatcctaagacaaaagacttgtttaaatatctggttcctttaaagaattcattaatattgacccctcctccccgggttttctcatgaaggtgagcgatggcagccagctgttctgagcttgcataatcctgcctttcctccaacaccatcacgaagtcgttcttgctgatgcttccatcacccctgtctaaaaccgcaaaggcttcccggaggaaagcctcacgttctacggaccaatcgtgcagtctaagggcccacagtggatttggatttttggctcctggcctggctagtttattagcgattctctctgctcggcgtatttctttgcttgctgctttgaagccgccttccttagccacagccctgggcgttttatgatctaaattcttccatttcaggtcacatcctcgctgagctatatatttacagcagtctgcaaaaccacccatggcagcataatgaagtggtgtgttcccatttatcgaaatcagccccacgtctccattgtaggcaaaaagaagcttcaatatatcgaaaaagcctcctttagcagcaaaatgagcagcgtgatgcctgtcgttgtcaaatgcattcacttcacctcctctttccaatatgcctcgaactatttccactaccccttctcttgacgcttccattaaagctgtgcggcctgtggatgagttgattgcattaggattggctcctttttccaaaaatgtcaggcacacatctttaacatcatgtgcatcttcacaagctctaaggaatattggctttccttcataggtagaattgttgacatctgcaccatgttcaagggcgatcagagcacagcgataatgccgcttagtcggtaaaatgcagtaaaacaaaacaccttatcatagaactggcatacggcattgaggactgagtacacatgccttttccttcattatcaactatagtcatatcagcctttgcctttgctaatatttccattgacaattcatggcccagttctgcagccctcattgtgggagtacagcccattcggtcttgcacatcagggtgagcaccaaggtcaaggagaaagctgaccatatcaatatcattggaaactgaggctaagtgcaaagcactaagtccattaatgggttctgtataattgattagttcagggtatccaagcttggtcagcttctctatctgcttcttgtctttgttccgcacacattgaagaactttgtagatctgtaagttctcaagtctcttatctgctaaagccatgcttgaccagctccttgaaaatgctttctggaccaaaactaaagctcttagtcttccgggcgatcagaagccagggatctctgggcacctatgtgcctgggcctgctggggcgaccggggaggcccctgctctcgtcctctgacgctcagcgctggcccagccgcgaccttgggctcccggagcccggcggaggcgcccaggcgtgaatgatgtcccttgggtagggctggtgagctggcgcgcgggacagcagggctgggtgtatgtgtccatgggccccgggtccccggaaggcgagcgcgcgggcaggtgagcgcagggggcggggtggaagccggagggaccgggctgattgtgagcttccgccacgcagggcgcggctgccggggc

SEQ ID NO: 8510 - RNA, 3527 nt, Homo sapiens
  source 1..3527: mol_type = other RNA
aaaagtaattgcggtttttgctgcaattaaaggttatggcaaaaaccacaattacttttgcaccaacctaatagctatctatctagggctagggctatctatctagggctagggctatcgatctagggctgttaaaagtgtattcaacccaaggtatctaatacacatagtttataatggcatgtgagaaataaactccttccttaaaagattaaatattacttctttttccaaaacctaaattgtttcatcaatttccactagaaatgtatcttcaataagcaggctgggcacagtagctcatgcctataatcccagcactttcgacggccaagttgggaggactgcctgagctcaagagttcgagaccagctggggcaatatagtgagactctgtctctatttaataaataaaaaggataattaaaaaaataataagcataatggtgtagacctggtaaatcttttgacagcaacgtttataacccacatgccatgtatttcactacattcataaaggggcttggggatttatccagaatgacataccattcatttcaaaataacatacatcttttctctagacagctaagaatatttatagttgttaaagcaaaaagaaattcttggtaacaagttcttggtgtatggattgctttggctttgatggaaatatctactttctccaaagattggtccctgggcctcaaagcatttaccccaagaaataactgctatgacttaggtcttcaaggcagcttccagtgctcgagctttctctgtgatgttcttctgaaaaggcatcataaaatcgtcgaagtccacctcatgtgtaaacctctctcgccgtagttccctcttcctgatcagctctgctgttgtggcttcaggactccaaatcctccgtggaataaatgtgatatccactttcttagtataaccactggtaatcaatgaattcagatgaaccacattacccttctgtactttctttccctctgatgtggttggtacaccataaattgatgacagcagttcctcttctttcttaatttcagggccttcagtcttcagtataggaggtgtcttgccttttagtttttgattttctgctggtttcggcaagttatctagcttttctttaatcagatcaattattctataatcagcatatgcctttgcaacgtccatggcactatgcccttttctattttccagctggaatttagcaccaatatcaagtaggtattttactgtatccagtctgcagctttcaatggctctatttaaaggagttgagttgttgattgaagctgcatctattaaagctccagattcaacaagaagctcaacaatgtcttgttggcctgcatggcatgcaaaatgaagtggagtccacagaaagttatctgttgcattaacgttagctcctttttcaagaagaaacttgaccacatctatgtttccacttgcacacgccgtcattagcggagttttgtaataattatccttcatatccacaggtattcctgattcaaaggcctttttcagagaagccagatcccctgctttggtgataatattaatgtttgaaaataccttctctgaatcatcaatgtaccaaacagagtcatcctgaatgggatgttctgggggatgatctctattaaaccggctgctatcagtgacattcttgtaggtctcaatcatgtaatacggtggcccaccatcctgccggcgtggaaacgcgtactcaggaatgacacagattggaaggggtaagacaaatttccctttctttccttttttgcccatccctttttcctttttcttaggtccatacgatcctaagacaaaagacttgtttaaatatctggttcctttaaagaattcattaatattgacccctcctccccgggttttctcatgaaggtgagcgatggcagccagctgttctgagcttgcataatcctgcctttcctccaacaccatcacgaagtcgttcttgctgatgcttccatcacccctgtctaaaaccgcaaaggcttcccggaggaaagcctcacgttctacggaccaatcgtgcagtctaagggcccacagtggatttggatttttggctcctggcctggctagtttattagcgattctctctgctcggcgtatttctttgcttgctgctttgaagccgccttccttagccacagccctgggcgttttatgatctaaattcttccatttcaggtcacatcctcgctgagctatatatttacagcagtctgcaaaaccacccatggcagcataatgaagtggtgtgttcccatttatcgaaatcagccccacgtctccattgtaggcaaaaagaagcttcaatatatcgaaaaagcctcctttagcagcaaaatgagcagcgtgatgcctgtcgttgtcaaatgcattcacttcacctcctctttccaatatgcctcgaactatttccactaccccttctcttgacgcttccattaaagctgtgcggcctgtggatgagttgattgcattaggattggctcctttttccaaaaatgtcaggcacacatctttaacatcatgtgcatcttcacaagctctaaggaatattggctttccttcataggtagaattgttgacatctgcaccatgttcaagggcgatcagagcacagcgataatgccgcttagtcggtaaaatgcagtaaaacaaaacaccttttccttcattatcaactatagtcatatcagcctttgcctttgctaatatttccattgacaattcatggcccagttctgcagccctcattgtgggagtacagcccattcggtcttgcacatcagggtgagcaccaaggtcaaggagaaagctgaccatatcaatatcattggaaactgaggctaagtgcaaagcactaagtccattaatgggttctgtataattgattagttcagggtatccaagcttggtcagcttctctatctgcttcttgtctttgttccgcacacattgaagaactttgtagatctgtaagttctcaagtctcttatctgctaaagccatgcttgaccagctccttgaaaatgctttctggaccaaaactaaagctagtttttacctcagtttctgcatctgtgaactggcaatagcaatggtgcccacttcatgggactcttagtcttccgggcgatcagaagccagggatctctgggcacctatgtgcctgggcctgctggggcgaccggggaggcccctgctctcgtcctctgacgctcagcgctggcccagccgcgaccttgggctcccggagcccggcggaggcgcccaggcgtgaatgatgtcccttgggtagggctggtgagctggcgcgcgggacagcagggctgggtgtatgtgtccatgggccccgggtccccggaaggcgagcgcgcgggcaggtgagcgcagggggcggggtggaagccggagggaccgggctgattgtgagcttccgccacgcagggcgcggctgccggggc

SEQ ID NO: 8511 - RNA, 3463 nt, Homo sapiens
  source 1..3463: mol_type = other RNA
aaaagtaattgcggtttttgctgcaattaaaggttatggcaaaaaccacaattacttttgcaccaacctaatagctatctatctagggctagggctatctatctagggctagggctatcgatctagggctgttaaaagtgtattcaacccaaggtatctaatacacatagtttataatggcatgtgagaaataaactccttccttaaaagattaaatattacttctttttccaaaacctaaattgtttcatcaatttccactagaaatgtatcttcaataagcaggctgggcacagtagctcatgcctataatcccagcactttcgacggccaagttgggaggactgcctgagctcaagagttcgagaccagctggggcaatatagtgagactctgtctctatttaataaataaaaaggataattaaaaaaataataagcataatggtgtagacctggtaaatcttttgacagcaacgtttataacccacatgccatgtatttcactacattcataaaggggcttggggatttatccagaatgacataccattcatttcaaaataacatacatcttttctctagacagctaagaatatttatagttgttaaagcaaaaagaaattcttggtaacaagttcttggtgtatggattgctttggctttgatggaaatatctactttctccaaagattggtccctgggcctcaaagcatttaccccaagaaataactgctatgacttaggtcttcaaggcagcttccagtgctcgagctttctctgtgatgttcttctgaaaaggcatcataaaatcgtcgaagtccacctcatgtgtaaacctctctcgccgtagttccctcttcctgatcagctctgctgttgtggcttcaggactccaaatcctccgtggaataaatgtgatatccactttcttagtataaccactggtaatcaatgaattcagatgaaccacattacccttctgtactttctttccctctgatgtggttggtacaccataaattgatgacagcagttcctcttctttcttaatttcagggccttcagtcttcagtataggaggtgtcttgccttttagtttttgattttctgctggtttcggcaagttatctagcttttctttaatcagatcaattattctataatcagcatatgcctttgcaacgtccatggcactatgcccttttctattttccagctggaatttagcaccaatatcaagtaggtattttactgtatccagtctgcagctttcaatggctctatttaaaggagttgagttgttgattgaagctgcatctattaaagctccagattcaacaagaagctcaacaatgtcttgttggcctgcatggcatgcaaaatgaagtggagtccacagaaagttatctgttgcattaacgttagctcctttttcaagaagaaacttgaccacatctatgtttccacttgcacacgccgtcattagcggagttttgtaataattatccttcatatccacaggtattcctgattcaaaggcctttttcagagaagccagatcccctgctttggtgataatattaatgtttgaaaataccttctctgaatcatcaatgtaccaaacagagtcatcctgaatgggatgttctgggggatgatctctattaaaccggctgctatcagtgacattcttgtaggtctcaatcatgtaatacggtggcccaccatcctgccggcgtggaaacgcgtactcaggaatgacacagattggaaggggtaagacaaatttccctttctttccttttttgcccatccctttttcctttttcttaggtccatacgatcctaagacaaaagacttgtttaaatatctggttcctttaaagaattcattaatattgacccctcctccccgggttttctcatgaaggtgagcgatggcagccagctgttctgagcttgcataatcctgcctttcctccaacaccatcacgaagtcgttcttgctgatgcttccatcacccctgtctaaaaccgcaaaggcttcccggaggaaagcctcacgttctacggaccaatcgtgcagtctaagggcccacagtggatttggatttttggctcctggcctggctagtttattagcgattctctctgctcggcgtatttctttgcttgctgctttgaagccgccttccttagccacagccctgggcgttttatgatctaaattcttccatttcaggtcacatcctcgctgagctatatatttacagcagtctgcaaaaccacccatggcagcataatgaagtggtgtgttcccatttatcgaaatcagccccacgtctccattgtaggcaaaaagaagcttcaatatatcgaaaaagcctcctttagcagcaaaatgagcagcgtgatgcctgtcgttgtcaaatgcattcacttcacctcctctttccaatatgcctcgaactatttccactaccccttctcttgacgcttccattaaagctgtgcggcctgtggatgagttgattgcattaggattggctcctttttccaaaaatgtcaggcacacatctttaacatcatgtgcatcttcacaagctctaaggaatattggctttccttcataggtagaattgttgacatctgcaccatgttcaagggcgatcagagcacagcgataatgccgcttagtcggtaaaatgcagtaaaacaaaacaccttttccttcattatcaactatagtcatatcagcctttgcctttgctaatatttccattgacaattcatggcccagttctgcagccctcattgtgggagtacagcccattcggtcttgcacatcagggtgagcaccaaggtcaaggagaaagctgaccatatcaatatcattggaaactgaggctaagtgcaaagcactaagtccattaatgggttctgtataattgattagttcagggtatccaagcttggtcagcttctctatctgcttcttgtctttgttccgcacacattgaagaactttgtagatctgtaagttctcaagtctcttatctgctaaagccatgcttgaccagctccttgaaaatgctttctggaccaaaactaaagctcttagtcttccgggcgatcagaagccagggatctctgggcacctatgtgcctgggcctgctggggcgaccggggaggcccctgctctcgtcctctgacgctcagcgctggcccagccgcgaccttgggctcccggagcccggcggaggcgcccaggcgtgaatgatgtcccttgggtagggctggtgagctggcgcgcgggacagcagggctgggtgtatgtgtccatgggccccgggtccccggaaggcgagcgcgcgggcaggtgagcgcagggggcggggtggaagccggagggaccgggctgattgtgagcttccgccacgcagggcgcggctgccggggc

SEQ ID NO: 8512 - RNA, 461 nt, Homo sapiens
  source 1..461: mol_type = other RNA
aaaagtaattgtggttttggccaaaattttcagtggcctataatttttaggccaactgttgacatgaaccccaaaattttcaccctctagatagtggagaccaagagaaagtatccccatatactcacaaggtcaagctcccaaggacataaaacaagacgagaaggaaactttacctactttttgtttcaggaatctgcaacaaactttgtaactggtcagtttgctggtacagcttaaatagaaggcttataggtaaccccttttataacagaactacacacaaagacaaattcatagtgcaaagtacaccagatttgctacagcctaagactagtctcacaaatcctttttcccattaatcaaaattttatagaggagataaatagtgatttttaccattcattcaacctgtttgcacagaaagagtgagagagaaaacgagagagagagagagatat

SEQ ID NO: 8513 - RNA, 4888 nt, Homo sapiens
  source 1..4888: mol_type = other RNA
aaaagtaattgtggtttttgccatacttaatggcaatacattaagtatggcaaaaacttacttttgcaccaacctaacagatctgttttggtttgtaaacttttagacaagttcttatcccagtaactccccaccactgtttaatacaatttggcacagtatatagtacatgaggccatcgagtgtaactactatgggactccattttggcaccagcccctagagaccagtactgcttcaaagactaatactgtgtggcttaatcctttctccctttccaaaaagactagtttgtgctttccttggggaagtttaatattgaaaacactgccttgtacattttcaattgttattttcctgggcccaggggtttggttaaaatttagatcttcacccagctctagattcatcttcccttatcagaagggcagacatggtttcctggacccaactcacacaggtgggcagcacttcagctgctgagacaaccagctgaagcatagcaaagccccttacaggaggtggggttaagaacgatacattgagatttggcaaagatgggggaaagagcaattcaatgaagcagcacgtcatctcataccatctttccaataaactgctaaagaaacatcacaaaagctgacaaagccagttgtcaaaactgagttatttcttatttcccaacacacttgtttgttgttgccctcagatgttgccgatttccaaagtggcgtccacatcctgcccctctccacatcaccctgatgttctgttgctaagcaaggagtgtactggcttatctgaggggcatgcattcagcctcttacacagacttactgctcactcattaagtggcaaacctatttctaggttgaaaggaacaagacttttcacttcccagaagtataacttcaaaccctacacacacctcaccttggatccctttgcagaaaaactgcatttcttgtggtcatgaaagagtcaagcattggcccagagctactgcagaagcttgaaatctttgctgagcatcaagtactcaaacttgaaaggaacttgtaagtccctccctgactgctcccttttctggcttctcatttgcaaatggatcaatataaccaaaaaataactaaatggcttttttggtgggggatgaggaggctaaatagttaatttaaaaaacaacaaaatacatccactctagtacatctaatgcacggaatgtcttcttaaagggtggggaaggaacctagtttctccagagtactcagggtcctgggctgcctgcctcttttgtgcagctttctctgatacactctgatctgggatggaaagggccttatctggccaagagcagcctggcttttccctcagtcaaccactacccaatccagaaccggggaaaatgagttgcaaactggcttaatgaaaaagcagtctttttaaaacctcagtctgggtacccagctacaactgatcccacagaacctgctgggacccctggagacttattcaagagtcttatttagctagaacagaagccaggcatctggcccaagacccccttcagctttctagcagtactataccgtgggtgatcttaaagtttcccatttgcccctctgaaggaggaactgtcaggtttaggatttaaaaaaaaaaacaaattccaagtatgttccctatggtcaatatcagttttagaaaaataccaactgccaaaactctttaataatccttaagatgggagcccagagctgtaaggctgctcacaatggaactcaaaacatgcaattcctgcccaggctgagaaacatacctgggacgcagcggggtattaggttaagggagaaacctccaaatgtttaacagacaaagtctcattacctcaagagtataaatatttttatacgtttttatttaaaagattccctttttaatctgttccaaagtgttggaagctgaactatacaagttcctgccacccatccttccagtacagttttctgaggacatactttttaaatggaaaaataacaggaggaccctctaactgaaaccaggtaggcccagagtgagctcctcaggcccctgtggcagcctggccaaagctggcctttatggagccagcgcgtggagaagtctggggaaccggggccctccctcttgtgaggaaagggctgagcaaactcatgttctctttagtgaaatggtccaaattcagatccaaaagcctccattatggcattccctggcactcttcttatactttatacattgaaggcagctccctcttttatggccagtataagcaggcaaagaaacaaaggaatatagatacatatatgtgtatatatatatattttatataggtaaaatatatacatattttatatatgtatatatacatatttgggggtagggaaaggagaggagggtcatgtaaacctaaacagtcatcacattaccccaaatgagcctgactttaacaaaaagataataaataactcctgggggttaagtgacaacatgggtgcagcaagaagggaaagggcacaaatttaactattaaatacactttgatatttgtttggcagagttcaggccaaccccaggcttctgcccttgccagacaagtaagctgatgatattcaaagaaaaaaataaaaatattaaaaaaaaaaaaattcaagcagagctccataccacagttttccttcaagtcagttggccggcaggcagtttcccgaccaccaggaacagaaactttggctccaaggcaaatgaaacaaacaaacaaaaaaaagtatttccacttacaacatgaaaatacagaaacttcatcaaagaaagaaaactatcaaagaagtctacttccagcaaaactgaggtagcactgctttctccgcattcaatgcttaagtggttctcagtacaatgtgttcttaaaaaatgctcacttgactgacaggtgcagcatgttgatggaaaaactcaacatgaaatgcaataggtcaaagaaggaatgagcaagaagtgagggaaatcagggttctggataaattagcttaaaagggggttgtcaccagactacaaatgctcttggctggccttggctctccaagagctctaaatcgcctgggaattaatgcaatgtggttaacagttaacactgctattcaaatctgtgtaaatctttaaaaataattattacaacctaaattcatctatgtaaacagcactacacacagtacagacctgccctgaaaaacaatatgcgaaactgagatctggcactgtatcattttgtaatgttaattcaacctaacagtcccatccccccgccctgctctatgccctcccctaccaaaaaaaaaaaaaaaaaaacaaaaaaaaacaaaaaaaaaacctaaatttgtgcaagaaatggcaggcttattctatctgaaggcttcaaaaaaagatacacaacatgtaaccaggttcaaatattctgggagatccccccaaaaaggaaataaccaaaataaccaaaaaaatgaagaaagtgcctaaaacatgatacagcattttagagccctttcagatacaaggcagagaaaggtgtaaagtagaaaatatccggatcttcagtaatttccaaaatggtccaattcctcagttggctgcagggcagctggcagatccttgctgctgctcctgggacagagccactaagtctgctcctcgggacacaagccctcaggccctgagctgagtgcacctctcccttccccttctcttttccttcgctccatttcccactccacaaaggtgtcaaagagacttggccaggcctcatcttcactgtagttgctgaggtcagggccaatcacctgagtgaagttaaggaacatgttccaagtgtcccgggagatgcccttgatccccgaggggttctctgttaggaagtttagccattggtccaataccggaggattgttctgggtaaagactagtttccacagggcaatggctatttcccgatgcagtgaccgctgcccttcttcagagtccaggccaaactgaaatgtaaaccggtagagatccttgaatttatcctcttgtttggcttctgttaagaggctagggaaccgtgcacagattccgtcaatgctgtctgcacttattgctttgcagccatcaaaaaactccttcctggtgaatttgcacatggttgcagcctggaacttccaagccaagagcagcactcgaaattctgtggggtcaacacacaggtcattgcaaaagcgctccatgccttcctccaaaattgcatcttcccgctcatccttgtagcgcctgaacagttcttccaatctttgcaaggaagactcctcggcattggacttggactccctcccagcatctcccgaggacgttggcagctggcaggcctcagtggcagcctcggccttcttggtcccgttgacgaggatatctccacctggcttgccacagggtggtacctgctcctcacggtggcctgcacccctcctgctatgtgacttgttgctgggctcacggtctccatttttgctgcccagggtcgatgagggattcttacacttggtgacacactggcccatggtgctggtggcctggcctctagagtggacccctctggattggatgccctcgctgccgctggcccatgtacctcaacatgccatcagccagaggagccagccaacagctgctccagaggttcctccagtcaaaccctttctggaaacgacggcggcccggcgggtccaaaccacctaccatccccgctcgcgtttccaggctccctacccccgccgccgccgcctcttcttccaccactgccaccgcctcctcttcatct

SEQ ID NO: 8514 - RNA, 2844 nt, Homo sapiens
  source 1..2844: mol_type = other RNA
aaaagtaattgtggtttttgccattactgtctacggcaaaaaccgcaattacttttgcaccaaccaatataaattgtaacagatttgagacaaaatataaaatttttcaaattgagcagaatttatcaacccagaatctataatgtatgaaataaattaatagagaacccaacagatcatgttatgttgtaaatataacatctatctttaggttaaagtaacatagcaaaaatatatatttatgggtgcaagacacatacataatttgtaccaatctcacagaactaattcaattcaaaacaacaaaaaacttactctattatctaatggatgcaataaaaattaaccatttgaagataagttctcttgcacttcccctacttacgtttttcctggcacctgctatactgtgtatgtatttcttcaccgctttactgcctgactcccctactagatcataagttccaagagggcaagccctctgaaacactgctatgtctccagcacctagaacttggcatgtagtaggcatccaatacataagtgttaaatgagtgaatttaaaacacgtacatgccaggaatggtggctcaggcctgtaatcccagcactttgggaggccgaggcgggggatggcctgaggtcaggagttccagaccagcctggctaatatggtgaaaccccgactctactaaaaatacaaaaattagctcttcctttctctgccattgtggtgtgtgcttgactctgcttcttgccatgtcttctcataagacttccaggattaagtgattcctgaccgagaaattaaaacaaaatcgccccactccccagtggattcagatgaaaactggtaataaaatcaggtacaactccaaaaggagacattgaagaagaaccaagctagccctataaggaattgcacatgagagggcacacatatttatgctgtctgaaggtcacagtcatgttaccacatcaagctgaaaatgtcaccgctctctggagaattgtacatgttttattgggaatatattttttctttctgaatctgttatgaatgcattggttggctgggttcagtaataaatatgtgagacctttcattaaaaaaaaatacaaaaattagctgggcatggtggcgcacacctgtagtaccagctactctggaggctgaggcgggagaattgcttcaacccagaaggcggaggttgcagtgagctgagatcgcgccactgcactccagcctgtgtgacagagtgagactttgtctcaaaaaacaaacaaaacatgcacacatttaatcaatataaaatattatttctgcgaagtcacttcaagctgatactgcatactccatatatgctaaacttcacaaggtctttacctcatacctgactctctttcctgaccccctgcggggtaagtcaatgccctggggttgcttagccacttggtactaccagctttgggcaccaggtctgtttcagctcattggtgtatgccccggctggcttttcccatagggcagagttgcacaagttgtgggtgtgaagctgagaggtgagcagaggaggaagggaggtagacagtcctcatcccagtgtccctctgaactgccgcgtgtgttgctccagcttctcagcctccgcctggaggtgccccagcgcggcagggctggggtacgtgagcacggcattcttagtggccagcgctacgtccttgagcaggctgcagaggtgactgctgccacggaggatctcgttgcgcacgtccctctcctgggtctccatgcacagcgtgtccaccagcttctgtcccaccatgatgaccagcttgctctgagtgatgatctccgcgggctggctgctgctgaggctgccgtgaaatgcgctgatggctttgaagagcgccccaaagtagagccggcagtgttcagataagcggggtttcctctcaggagtctgttgactcgaaggctgaggtataagagggccaggattacttgcttggctgtctgggggatggagtcctgccttcttggggctggctggtatgtcatataactgctgcttctctggctccttcaggaccacggggccccggtgctgggtaggcacgtcatacacctgggaaggcagagtcggcagtgaggcccggacaggtctgggaagcgtgaggatggcctgttttggaaagctgagagtcttttcacagatgattctggcactggtgggagggtcggggaattcatagacttgggcagtagggggctggggcccctccgcccaactcctcatctgctcataaacggggcctggagtgggagggcggggtagagtgggcacctgataggtctcctctgagctggcaggagcttcttccaggcctctcaggaatggggggcacggcctgtctgcagcgacctccgtgaggatttggaggcggttggcaggggccaggccttgcctcccatggagcaaacacttccaccaaccctcgctttctggcacgtgttgctccagaatggtcaggatgtcccctctgctgaaagccagctcgtcagagcagtcagggcagttgtcataaagtgccctggccaggagtgccttgggcgcacagtccatgatgcctgttcccttcatgtcggtgatgtggagcagctcccctgagctctgcagctagtatctccagcttcagaggcagattgtgcaatgtcactgcatgcttctggctggttctcagaaactgaattctatggagctatctgacaacacatgggaaacgatcaaaaagactctcccagcaggcaaactttctggaaagcacgataagagtaaaatg

SEQ ID NO: 8515 - RNA, 3993 nt, Homo sapiens
  source 1..3993: mol_type = other RNA
aaaagtaattgtggtttttgccattactgtctacggcaaaaaccgcaattacttttgcaccaaccaatataaattgtaacagatttgagacaaaatataaaatttttcaaattgagcagaatttatcaacccagaatctataatgtatgaaataaattaatagagaacccaacagatcatgttatgttgtaaatataacatctatctttaggttaaagtaacatagcaaaaatatatatttatgggtgcaagacacatacataatttgtaccaatctcacagaactaattcaattcaaaacaacaaaaaacttactctattatctaatggatgcaataaaaattaaccatttgaagataagttctcttgcacttcccctacttacgtttttcctggcacctgctatactgtgtatgtatttcttcaccgctttactgcctgactcccctactagatcataagttccaagagggcaagccctctgaaacactgctatgtctccagcacctagaacttggcatgtagtaggcatccaatacataagtgttaaatgagtgaatttaaaacacgtacatgccaggaatggtggctcaggcctgtaatcccagcactttgggaggccgaggcgggggatggcctgaggtcaggagttccagaccagcctggctaatatggtgaaaccccgactctactaaaaatacaaaaattagctcttcctttctctgccattgtggtgtgtgcttgactctgcttcttgccatgtcttctcataagacttccaggattaagtgattcctgaccgagaaattaaaacaaaatcgccccactccccagtggattcagatgaaaactggtaataaaatcaggtacaactccaaaaggagacattgaagaagaaccaagctagccctataaggaattgcacatgagagggcacacatatttatgctgtctgaaggtcacagtcatgttaccacatcaagctgaaaatgtcaccgctctctggagaattgtacatgttttattgggaatatattttttctttctgaatctgttatgaatgcattggttggctgggttcagtaataaatatgtgagacctttcattaaaaaaaaatacaaaaattagctgggcatggtggcgcacacctgtagtaccagctactctggaggctgaggcgggagaattgcttcaacccagaaggcggaggttgcagtgagctgagatcgcgccactgcactccagcctgtgtgacagagtgagactttgtctcaaaaaacaaacaaaacatgcacacatttaatcaatataaaatattatttctgcgaagtcacttcaagctgatactgcatactccatatatgctaaacttcacaaggtctttacctcatacctgactctctttcctgaccccctgcggggtaagtcaatgccctggggttgcttagccacttggtactaccagctttgggcaccaggtctgtttcagctcattggtgtatgccccggctggcttttcccatagggcagagttgcacaagttgtgggtgtgaagctgagaggtgagcagaggaggaagggaggtagacagtcctcatcccagtgtccctctgaactgccgcgtgtgttgctccagcttctcagcctccgcctggaggtgccccagcgcggcagggctggggtacgtgagcacggcattcttagtggccagcgctacgtccttgagcaggctgcagaggtgactgctgccacggaggatctcgttgcgcacgtccctctcctgggtctccatgcacagcgtgtccaccagcttctgtcccaccatgatgaccagcttgctctgagtgatgatctccgcgggctggctgctgctgaggctgccgtgaaatgcgctgatggctttgaagagcgccccaaagtagagccggcagtgttcagataagcggggtttcctctcaggagtctgttgactcgaaggctgaggtataagagggccaggattctgtccacagatatttgccctatttttctttaatagttcagaagagtgttcatcttccctttgcttagtggaaggggtactcttttggtgtgattcagtttctctttggggaggctggatgtatttttcacacttaaattctgcatttggggtcaactgcacagtctcttccttttcacagttccgcttaaaaaggagccttccattggcaatgacaatggaggcaaacctcttgatgtcttctggaagcatccgtgccaccatgacaaacctctcaaggtcatctgggctgttctggacactgtcagtcacaagaacttccagaggccaattgcgattatccaagctttcctttgtttcaagcaggatgcggtaggagttggagatggtctgcatctggtcccgaattctgttctgaaggttactgtcagtgaggttacaggcagtcccatggactcctcgggcaaaatccagaaattctcttacagattcttctatgtgatcagtggacctgtggattgcatcaatgttggcctccagatagtctcggaatctccacttcctgctgacaaagagcatcaggccagcgacagagctgaccaccttgtgctgcagagccatcactgtctccttggccacatccaggtccaaggagagctcctttgctgactcctccgaggaagagctggaggagtcgtcggtggatgtggtggagcacgaggaaacgatgctagctctgctgtcagaactggaacctgataatctgtccggttcaggagatggggaagttgtccgtctggagaaccatgaggaattatggcccgcggaattctctgacacctccttggctttctccagctccttcccagcctgagaaacactcgacgttgctttagggatgtcataaatattgggcttggtgttctgctgttccactcggggaatcagaaagcttgaaggaaccttgtagctgacatcttcatccaaaggaaatgtgcctctgggtacaagaaagccataagaaggaatttctggaaggctgagttttttctgcatgggcacattgttattcagttgtggagtgagggacctggatctgccacttggaggattgtagaaagtggagctggaactggggagagcgtggggccttgattcttccgcaaagctggtgagaggcgtgtttctgacgctggcctttcctggagacactggagtgtcataaatccattccgatttctgaggatttggtaatgtgctgtaaccgcctcttcttaaggtagtcactgatatcaggggaacaccctgcccacttgcttggctgtctgggggatggagtcctgccttcttggggctggctggtatgtcatataactgctgcttctctggctccttcaggaccacggggccccggtgctgggtaggcacgtcatacacctgggaaggcagagtcggcagtgaggcccggacaggtctgggaagcgtgaggatggcctgataggtctcctctgagctggcaggagcttcttccaggcctctcaggaatggggggcacggcctgtctgcagcgacctccgtgaggatttggaggcggttggcaggggccaggccttgcctcccatggagcaaacacttccaccaaccctcgctttctggcacgtgttgctccagaatggtcaggatgtcccctctgctgaaagccagctcgtcagagcagtcagggcagttgtcataaagtgccctggccaggagtgccttgggcgcacagtccatgatgcctgttcccttcatgtcggtgatgtggagcagctcccctgagctctgcagctagtatctccagcttcagaggcagattgtgcaatgtcactgcatgcttctggctggttctcagaaactgaattctatggagctatctgacaacacatgggaaacgatcaaaaagactctcccagcaggcaaactttctggaaagcacgataagagtaaaatg

SEQ ID NO: 8516 - RNA, 4155 nt, Homo sapiens
  source 1..4155: mol_type = other RNA
aaaagtaattgtggtttttgccattactgtctacggcaaaaaccgcaattacttttgcaccaaccaatataaattgtaacagatttgagacaaaatataaaatttttcaaattgagcagaatttatcaacccagaatctataatgtatgaaataaattaatagagaacccaacagatcatgttatgttgtaaatataacatctatctttaggttaaagtaacatagcaaaaatatatatttatgggtgcaagacacatacataatttgtaccaatctcacagaactaattcaattcaaaacaacaaaaaacttactctattatctaatggatgcaataaaaattaaccatttgaagataagttctcttgcacttcccctacttacgtttttcctggcacctgctatactgtgtatgtatttcttcaccgctttactgcctgactcccctactagatcataagttccaagagggcaagccctctgaaacactgctatgtctccagcacctagaacttggcatgtagtaggcatccaatacataagtgttaaatgagtgaatttaaaacacgtacatgccaggaatggtggctcaggcctgtaatcccagcactttgggaggccgaggcgggggatggcctgaggtcaggagttccagaccagcctggctaatatggtgaaaccccgactctactaaaaatacaaaaattagctcttcctttctctgccattgtggtgtgtgcttgactctgcttcttgccatgtcttctcataagacttccaggattaagtgattcctgaccgagaaattaaaacaaaatcgccccactccccagtggattcagatgaaaactggtaataaaatcaggtacaactccaaaaggagacattgaagaagaaccaagctagccctataaggaattgcacatgagagggcacacatatttatgctgtctgaaggtcacagtcatgttaccacatcaagctgaaaatgtcaccgctctctggagaattgtacatgttttattgggaatatattttttctttctgaatctgttatgaatgcattggttggctgggttcagtaataaatatgtgagacctttcattaaaaaaaaatacaaaaattagctgggcatggtggcgcacacctgtagtaccagctactctggaggctgaggcgggagaattgcttcaacccagaaggcggaggttgcagtgagctgagatcgcgccactgcactccagcctgtgtgacagagtgagactttgtctcaaaaaacaaacaaaacatgcacacatttaatcaatataaaatattatttctgcgaagtcacttcaagctgatactgcatactccatatatgctaaacttcacaaggtctttacctcatacctgactctctttcctgaccccctgcggggtaagtcaatgccctggggttgcttagccacttggtactaccagctttgggcaccaggtctgtttcagctcattggtgtatgccccggctggcttttcccatagggcagagttgcacaagttgtgggtgtgaagctgagaggtgagcagaggaggaagggaggtagacagtcctcatcccagtgtccctctgaactgccgcgtgtgttgctccagcttctcagcctccgcctggaggtgccccagcgcggcagggctggggtacgtgagcacggcattcttagtggccagcgctacgtccttgagcaggctgcagaggtgactgctgccacggaggatctcgttgcgcacgtccctctcctgggtctccatgcacagcgtgtccaccagcttctgtcccaccatgatgaccagcttgctctgagtgatgatctccgcgggctggctgctgctgaggctgccgtgaaatgcgctgatggctttgaagagcgccccaaagtagagccggcagtgttcagataagcggggtttcctctcaggagtctgttgactcgaaggctgaggtataagagggccaggattctgtccacagatatttgccctatttttctttaatagttcagaagagtgttcatcttccctttgcttagtggaaggggtactcttttggtgtgattcagtttctctttggggaggctggatgtatttttcacacttaaattctgcatttggggtcaactgcacagtctcttccttttcacagttccgcttaaaaaggagccttccattggcaatgacaatggaggcaaacctcttgatgtcttctggaagcatccgtgccaccatgacaaacctctcaaggtcatctgggctgttctggacactgtcagtcacaagaacttccagaggccaattgcgattatccaagctttcctttgtttcaagcaggatgcggtaggagttggagatggtctgcatctggtcccgaattctgttctgaaggttactgtcagtgaggttacaggcagtcccatggactcctcgggcaaaatccagaaattctcttacagattcttctatgtgatcagtggacctgtggattgcatcaatgttggcctccagatagtctcggaatctccacttcctgctgacaaagagcatcaggccagcgacagagctgaccaccttgtgctgcagagccatcactgtctccttggccacatccaggtccaaggagagctcctttgctgactcctccgaggaagagctggaggagtcgtcggtggatgtggtggagcacgaggaaacgatgctagctctgctgtcagaactggaacctgataatctgtccggttcaggagatggggaagttgtccgtctggagaaccatgaggaattatggcccgcggaattctctgacacctccttggctttctccagctccttcccagcctgagaaacactcgacgttgctttagggatgtcataaatattgggcttggtgttctgctgttccactcggggaatcagaaagcttgaaggaaccttgtagctgacatcttcatccaaaggaaatgtgcctctgggtacaagaaagccataagaaggaatttctggaaggctgagttttttctgcatgggcacattgttattcagttgtggagtgagggacctggatctgccacttggaggattgtagaaagtggagctggaactggggagagcgtggggccttgattcttccgcaaagctggtgagaggcgtgtttctgacgctggcctttcctggagacactggagtgtcataaatccattccgatttctgaggatttggtaatgtgctgtaaccgcctcttcttaaggtagtcactgatatcaggggaacaccctgcccacttgcttggctgtctgggggatggagtcctgccttcttggggctggctggtatgtcatataactgctgcttctctggctccttcaggaccacggggccccggtgctgggtaggcacgtcatacacctgggaaggcagagtcggcagtgaggcccggacaggtctgggaagcgtgaggatggcctgttttggaaagctgagagtcttttcacagatgattctggcactggtgggagggtcggggaattcatagacttgggcagtagggggctggggcccctccgcccaactcctcatctgctcataaacggggcctggagtgggagggcggggtagagtgggcacctgataggtctcctctgagctggcaggagcttcttccaggcctctcaggaatggggggcacggcctgtctgcagcgacctccgtgaggatttggaggcggttggcaggggccaggccttgcctcccatggagcaaacacttccaccaaccctcgctttctggcacgtgttgctccagaatggtcaggatgtcccctctgctgaaagccagctcgtcagagcagtcagggcagttgtcataaagtgccctggccaggagtgccttgggcgcacagtccatgatgcctgttcccttcatgtcggtgatgtggagcagctcccctgagctctgcagctagtatctccagcttcagaggcagattgtgcaatgtcactgcatgcttctggctggttctcagaaactgaattctatggagctatctgacaacacatgggaaacgatcaaaaagactctcccagcaggcaaactttctggaaagcacgataagagtaaaatg

SEQ ID NO: 8517 - RNA, 4257 nt, Homo sapiens
  source 1..4257: mol_type = other RNA
aaaagtaattgtggtttttgccattactgtctacggcaaaaaccgcaattacttttgcaccaaccaatataaattgtaacagatttgagacaaaatataaaatttttcaaattgagcagaatttatcaacccagaatctataatgtatgaaataaattaatagagaacccaacagatcatgttatgttgtaaatataacatctatctttaggttaaagtaacatagcaaaaatatatatttatgggtgcaagacacatacataatttgtaccaatctcacagaactaattcaattcaaaacaacaaaaaacttactctattatctaatggatgcaataaaaattaaccatttgaagataagttctcttgcacttcccctacttacgtttttcctggcacctgctatactgtgtatgtatttcttcaccgctttactgcctgactcccctactagatcataagttccaagagggcaagccctctgaaacactgctatgtctccagcacctagaacttggcatgtagtaggcatccaatacataagtgttaaatgagtgaatttaaaacacgtacatgccaggaatggtggctcaggcctgtaatcccagcactttgggaggccgaggcgggggatggcctgaggtcaggagttccagaccagcctggctaatatggtgaaaccccgactctactaaaaatacaaaaattagctcttcctttctctgccattgtggtgtgtgcttgactctgcttcttgccatgtcttctcataagacttccaggattaagtgattcctgaccgagaaattaaaacaaaatcgccccactccccagtggattcagatgaaaactggtaataaaatcaggtacaactccaaaaggagacattgaagaagaaccaagctagccctataaggaattgcacatgagagggcacacatatttatgctgtctgaaggtcacagtcatgttaccacatcaagctgaaaatgtcaccgctctctggagaattgtacatgttttattgggaatatattttttctttctgaatctgttatgaatgcattggttggctgggttcagtaataaatatgtgagacctttcattaaaaaaaaatacaaaaattagctgggcatggtggcgcacacctgtagtaccagctactctggaggctgaggcgggagaattgcttcaacccagaaggcggaggttgcagtgagctgagatcgcgccactgcactccagcctgtgtgacagagtgagactttgtctcaaaaaacaaacaaaacatgcacacatttaatcaatataaaatattatttctgcgaagtcacttcaagctgatactgcatactccatatatgctaaacttcacaaggtctttacctcatacctgactctctttcctgaccccctgcggggtaagtcaatgccctggggttgcttagccacttggtactaccagctttgggcaccaggtctgtttcagctcattggtgtatgccccggctggcttttcccatagggcagagttgcacaagttgtgggtgtgaagctgagaggtgagcagaggaggaagggaggtagacagtcctcatcccagtgtccctctgaactgccgcgtgtgttgctccagcttctcagcctccgcctggaggtgccccagcgcggcagggctggggtacgtgagcacggcattcttagtggccagcgctacgtccttgagcaggctgcagaggtgactgctgccacggaggatctcgttgcgcacgtccctctcctgggtctccatgcacagcgtgtccaccagcttctgtcccaccatgatgaccagcttgctctgagtgatgatctccgcgggctggctgctgctgaggctgccgtgaaatgcgctgatggctttgaagagcgccccaaagtagagccggcagtgttcagataagcggggtttcctctcaggagtctgttgactcgaaggctgaggtataagagggccaggattctgtccacagatatttgccctatttttctttaatagttcagaagagtgttcatcttccctttgcttagtggaaggggtactcttttggtgtgattcagtttctctttggggaggctggatgtatttttcacacttaaattctgcatttggggtcaactgcacagtctcttccttttcacagttccgcttaaaaaggagccttccattggcaatgacaatggaggcaaacctcttgatgtcttctggaagcatccgtgccaccatgacaaacctctcaaggtcatctgggctgttctggacactgtcagtcacaagaacttccagaggccaattgcgattatccaagctttcctttgtttcaagcaggatgcggtaggagttggagatggtctgcatctggtcccgaattctgttctgaaggttactgtcagtgaggttacaggcagtcccatggactcctcgggcaaaatccagaaattctcttacagattcttctatgtgatcagtggacctgtggattgcatcaatgttggcctccagatagtctcggaatctccacttcctgctgacaaagagcatcaggccagcgacagagctgaccaccttgtgctgcagagccatcactgtctccttggccacatccaggtccaaggagagctcctttgctgactcctccgaggaagagctggaggagtcgtcggtggatgtggtggagcacgaggaaacgatgctagctctgctgtcagaactggaacctgataatctgtccggttcaggagatggggaagttgtccgtctggagaaccatgaggaattatggcccgcggaattctctgacacctccttggctttctccagctccttcccagcctgagaaacactcgacgttgctttagggatgtcataaatattgggcttggtgttctgctgttccactcggggaatcagaaagcttgaaggaaccttgtagctgacatcttcatccaaaggaaatgtgcctctgggtacaagaaagccataagaaggaatttctggaaggctgagttttttctgcatgggcacattgttattcagttgtggagtgagggacctggatctgccacttggaggattgtagaaagtggagctggaactggggagagcgtggggccttgattcttccgcaaagctggtgagaggcgtgtttctgacgctggcctttcctggagacactggagtgtcataaatccattccgatttctgaggatttggtaatgtgctgtaaccgcctcttcttaaggtagtcactgatatcaggggaacaccctgcccacttgcttggctgtctgggggatggagtcctgccttcttggggctggctggtatgtcatataactgctgcttctctggctccttcaggaccacggggccccggtgctgggtaggcacgtcatacacctgggaaggcagagtcggcagtgaggcccggacaggtctgggaagcgtgaggatggcctgttttggaaagctgagagtcttttcacagatgattctggcactggtgggagggtcggggaattcatagacttgggcagtagggggctggggcccctccgcccaactcctcatctgctcataaacggggcctggagtgggagggcggggtagagtgggcacctgataggtctcctctgagctggcaggagcttcttccaggcctctcaggaatggggggcacggcctgtctgcagcgacctccgtgaggatttggaggcggttggcaggggccaggccttgcctcccatggagcaaacacttccaccaaccctcgctttctggcacgtgttgctccagaatggtcaggatgtcccctctgctgaaagccagctcgtcagagcagtcagggcagttgtcataaagtgccctggccaggagtgccttgggcgcacagtccatgatgcctgttcccttcatgtcggtgatgtggagcagctcccctgagctctgcagctagtatctccagcttcagaggcagattgtgcaatgtcactgcatgcttctggctggttctcagaaactgaattctatggagctatgtctcaatgcctgacgtctcactttgtctgtaagtagagactgtcactcatttgctatgtgaaaccacaaaagaagaagaagaagaaaaaaacaccactcttctgctttatagggcgaagttcctacttcgaagagctcagtgtatgaacacacagcattcttgtcctttgaactctgt

SEQ ID NO: 8518 - RNA, 2280 nt, Homo sapiens
  source 1..2280: mol_type = other RNA
aaaagtaattgtggtttttgccattacttttgcaccatcctactacaagtttggtctccagaatatattgtatatcggatgaaacacaggctgaacatcccttttccggcacccttggcctattgatcatgatcttctttcctggcatgcttggactcaacttcagaatgtttcttgatactgtgtttcaggcaactgccaccaatcaattggtgttggcacaatccagaggaccgctaccggtctccagtagatttcacctggtgtagagagatctgaggcgtattatcgctggcaaaacgcgatggggagttcccggctgggcaccagggtgcctgagtgtagcatctcaacaggctcattgtctgtggcctggatgtcgtatttgcggacaatccaacaaagagccaaatgcagttgaagctctgctaatcggcgaccaatgcacattctttttccaacgccaaatggaagatgcgcaaaaggattaattttttccttctcctgaagccaacgttcaggtctaaactgacttgaatcttcaaaattgtcttcactggatcccaacacctgggtatttagcatgagcactgttcctttgggtaaagcatattcacccagaactgttgccttgtcaagagtccgagttgtaaatggtacactcggcgtaagcctcatagattctttcagacaggcttttaaatacggcatattcctcaaatcttctgcccgtggcacctgattctcaggtaatacactttgaatttccttaagaagcttttgttgcacttggggattacgggataaattgtagagaatccacattagactgtttgctgtcgtttccaccgcagccagctggagctctgtgacagcagcatacaattctttctttgaaagccgattctggtgataaatgtcacaaaggaaatctgcactaggctgctgagaatacttctctaaccggttgtcgatacaagctttgactgatttgaaaatggtgtcccaggccagagtgtggtcctgccagaccttggtgttgaggctcttgtgcagctcgactggagtgaccatcatcctcccaaacgtgctcatcattgttttgatggccatgatgaagttcacagcttcatcccctgcattcttctggagaagcccaaatctcttctcatacaacacgaggcagatactttcaaacgaccatttgttcagttcgctgtacaagtcttcaacgtggcctctttcatcacagagctcatctattctgcccataaaatcggccaagacctcattgattttgttgtccagcttcatcacttcccctggtttcattagtttcttttgaaaggcactccggacccgctgccagtcttccccttccaggatcagcagcccgtagccttctttgcggtagtcgcgataggccttccacggtttgatctccagccgctgcgggtacgcgctctcggtgcggtacagcgcttccagcaggcatggcgagcccaggtgcaccgactcaaaggaacccaacttcatgcggaaaatcttgccatacttcttgtggtactccaccagggtgtcgtgctgtttcttgagaccccctttccagagaatctgcagcaggctgcccagcagtggccagctggtggggcccggcagggcggccgcgttctgagtctcgccaccagctgtcagcgggcagactggcacctctcgcggctgaggggacgtgtacgccgtagatgtcaccagtctcgggggctgcctcggactgcgcagctgctgcaggaaggcggcaagcgagcggctcttgctgatgggggagctcatggcagcgggggacaccggagcgcgggaaggcaggaggatggggtggggcgaggttggtacgaggtgctagtgggagtcggggcttaacgattctgggaaaaggaagcaaagagggccagctggtgtgatggagcggggtgaggcgggacaggcagcagaaaggacctcggcgaggatgctcgacgctgcaccacgcgacagcctcagagcattggtgcctccttgcactggccgcaggggctggaagagggtggccggtgtctggggacctcttgaaaagggaaagctgggagtcctcctgttggtccgcaaggctgacctctagggtctggctggagccacggggaggtgtcaaggagggtagatgagatgctgctggcgctgcgtttcctcctgtccctctccatgttcctatgcccagggaccatgcatttatggagacagagcatg

SEQ ID NO: 8519 - RNA, 7883 nt, Homo sapiens
  source 1..7883: mol_type = other RNA
aaaagtaattgtggtttttgccattacttttttttttttttttttttggagacagagtctctgtcactcatgctggagtgcagtggtgcgatctcggctcactgcaacctccgcctcccgggttcaagccattctcctgcctcagcctcccaagtagctggaattacaggtgtacgtcaccacaccaggctaatttttgtatttttgagtagagacagagtttcaccatgttgaccaggctgctcttgaacacctggcctcaagtgatccacccgcctcagcctcccaaagtgctgggattacaggcgtgagccaccgaggcttttgccattattattattattatgagatggagtcttgctctgtcacccaggctggagtgcagtggcacaatctcagctcactgcaacctccgcctcccgggttcaagtgattctcctgactcagcctcctgagtaactgagattacaggcactcaccaccatgcctggctgatttttgtatttttagtagagaagggtttcaccatgttgtccaggctggtctcaaactcctgacctcaggtgatccacctgcctcggccttccaaagagctgggaccacaggtgtgagccactgtgcccagccagtttttgccattatttttaatatttttaatggcgaaaaccacagttactttttgcaccaaccttagtaatcttcaacaccttagaagctgctgcccaatacatccaagcatacatcttaaaattacagtttaaaatatttttaaatgaaatttgacactaacatttgcagaactaccaaaacctgccttggaaaactggtttggaaaatggatgaataagacagcagtagggtcttgttcagctcaaaagcctctgtttctaaggttgcttttattgagactctatcaggaattccacggaggggagaagggatagccaccttgaagatttagactatcctagcattaaagtaaaagcctgagaagactgagaagggcttttagaaggctgtgggcaaagaagaaagatccacttaagtggaatgaaaacagtttgactgttgaacttgcacaaggcagacagttcaaaagcaaagcagggagagatcagcagctctttctacttccaagagcctccagtttttaagattaaaaacccacatctttatcccaaaagtttgggagccaaggaatagagagggatgaactataacatgttgattgttttactgccagcgtgagtcctgaagtcagctcattaaccaaagacgcacatgccaaatgcactatagatataaattcaaccaatcgccaactttaaaagtcagaacatttttgcataaaagtctggatttctggctttgcttattacaactggaagcactgacagcagtgggcttgtttggccatggtgattctgggctacagtcaggctgctcatacccaccctagacacaatctctgccttccacatgtccagtctctgtctctccctgctgctcacccaggtgcatggaagtgtctagattagtcactagctcctgtgagcatttgagtgtggtgcctgtggaagagatggttgtgctctgcagactgaaattggagtgaggtctaacaggaatgggacagaaggctcactctcagagctcttgcaccttggacttgtgacctgaatcaaattataactacttccgcaaggctcagtttcctcatctgtaaaatagatacagaaactcctgccctccctaaagtatgagttgtgatgaggatcagatgacagcacctacagctttataaactgtgaggttctgtggtccacatcagtgatttgctgtatctcacattcatccgttcccccttcatctggtaccagaactccagtttgcatctcaggagtaatctcttctattctcagtcccagtggtggacattggatcagtctagccgattagagctctgcattctcccagatataataattggtttagggctaggcgtatgggccaattgggaccagtagagttgaggctaggactgttgggaaagagaagctctcttttctattgaaattggagacagcagcatattggccaccatgttgctaacctgggggtggcaagtctgagaatgaaaatgaaaaagaggaaagaataatggaaagatgagaagagacaaggtctgaagccataatctgaagccatgggtccagatatacaccagcaaacgtattctttttgctttaactagattaaatggggctaactcactggagccccatacccccacagggtttttttatttttatttttttacactatcaggcacacttgtgagcatttgtttgatttggtttcatttccctgggcactttctgactccaagtcctggggagctcctgcagctgcaactagctcctctctctgcctggatttgaccatccacattgccttcttgaagttcttaagagggtcctgcggtgaggcttttgctgaaaggcactggaaattctctcggatcagataaccatgcctggtgggggcaatgaagccactggtggttgggatgattctgtttaccacagcatggacaaactggactgtcagcagggtgccatccagcacactccaaacaagtatagagcgatcctttaagcccacgtacacatacttgtcatccttggagaagcaagcacattggacccctctgcagtaagaactcgtgtagctcatctcgaatttccacttgcgtgcctgcaggtcccagagacacagcagggcatcctcagacccgctgaccaccagctgctccttgtggctgacctccacacaggcaactcggctcctgtgggtctccaagggaaacgctttggaagttgcacactcgtaaagaaagaggtccccattggtcatgctgtagaccacgcggtagtccgtcagaatggccacgctggagagggtctcgggcagctgagtgtaaaaggtgtatcttggcccatcgatgaccgggcaggggtccccggaggtgatgtccagcaccaggacgatgttgtcataggcgatggccaggcggtcctcgcacttgctcagggacatgcagttgattgctttccgggcctcgggagggggaatgcatatcacgtcctgcctggaattcagggggaacacaaggacgacccccgacacgaggcccgtaaataggagcttgcgctgctcagcaacctccagacacctgatctcactggaggtgtccagggaatcttgttcctcgccttctgccaagtcccaaatagtgactttgtttttgtccccaattttggggaagtagacgtagcttccattgtgggacactgcggtgaggccggtgcggtccagaaatggtgcaggcacccgggacctatgagcatcgctgagatcccagaccttgaaagatgaggactgtggggaagcagatgccaccaaagccccgccgcgggccagcaggctcacgggggccccgacgccttccaggatgtccagaagggtcccctgttctgacagactccacacctgaatgagcgcatcaagggaccccgtgatgatcaggttgttctcagtaccaaaaacagccgtctccaccatgtcttcatgttccagatccatggccatgaatcggcgaaagcccctcgagtccgccaagaatatccgcaccgatcttccaaagcctgcggcgaggagggactcatcttcagagaccaccaggaacctcacagcatctggaagcttctccagcaatctgtcccctttggaggaaaccaaagagatggagccattgctaaacccggtaacaagctttccttgcttctggactgagacggcacaggtaggtgtttcttctttgatgctggacatatgttgcttcccctgaagttttcccgtagctgagctccacagactgaccacaccatccctggacactgtcagcagtgtggcctgggaggccagcacggccatgcacatccaaggatcagaggcatctcccaggatatggaataccggctctgcagtttccagattccaagcattgatctttgagccagatgctgaatacacaactttgtgtgcctcatccacatgaaggttccagatctgaggttcagcgggattttttgagcctccatcccaaatggtaaatttctcctggccagagagtaagttccacaagtgcagcgtgtaatcctttgaagcagagttggcgagggtccctttggcaaatattttcacacacctcacctctcctgtgtgtccagttagcatgtggatcacatgctgctcttccatgtcccacacagccatgatgccatcctgggtgccaatcaccagcagcttctcctccacaccccatgccatggcggtgatgcctttgtgacagccgctgagagttgcccggaggggtcctcccgggggctggaggaatcctccgaggggcaccagcacagggtgtgcgcacaactggaaccagctctgggcctgttggcatagctgtcccaccagtgctggatgtgaggtggcgaagaaatggagtctggccagcagttctgtgtacaggaggctcctctccatgcctcggagctccacagcagggcggcagagctggagggcttcacggaccaggccaacctcaggggagtccaggtgaggggcacacaggtcaaagtcatccagcaggtcttcaatgcccccagagatgccccggcaggaaatccagctcatgctgcccagaacctcctgtttcagctcctccaggcggcccgagtgaagcaggtgatagggcaactccttcagcttccgcaggtttgcaaccgtatgtgagaaccacagaggctgcggggccacctttcggtccaagttcagtggtttccccacaagtggcagagtgatgagcttcttggtaccctggctccaggtccctgagaagaagtcggccaggacgccatgcctcttggctctctcggatcctgacaggtagcgctcacggaccacctcgaccagctgtctgtgggcaatggccaggagggtgaagccatccacgggccgccgggccaagtagtatcccagatcccgacgaagccgcacccacagcaggggcgggaagcgcagcagctccttgctgggcggggtccaatctcggtacacatcctgcaggacctcgtcgtccagggacaaaacatccttcagctccgcctccgagagaccgtgtcgggaagacacaatgtagcccagcacgtgggccacgaggagctgcccgtgtgtctgctccaggcgggtgcagagttggtgcgtggcttcctctgcggtggtggccagcgggacaggcacggtgaaagaggcccatttccgggcttcctcaaacgccagcctcagccgccctgggttcccacactctgggaggctggcccagagcaaatctgtgtgcaccgggctcagcgtcctccttgcagctgccagcaggagttggatcatctgctggccttggtttccggaaaggggcttcacctcccagtaggcctccgggtccaggagcacccgctgcaaggtgtccaaaacccccagtgcccccgagcaagctgagaggatgaggtgcaccctcggggggcagttgagaggcagccagggaaccctccgagcatggcggacagagtccaggtcatccatagcatccagcaggagcacgagagactcgaagtttctgcaagagacagtgtggaggagggtatggaaaaactggaccaccctggtgtgggcgtccagaacctgggcagggggcaagggcagcccataggccaggcacacctggaagcagatgctcttcagcaggccacgggcatctgagctcatttgtgacgtccccagcagccgcaggacggtcactgtcttgtgccccagcagccttggcatctgctcagccagcttgcacatcagggctgtctttccaatgcctgggggcccaaagagtaccaggggggtgtgctgcttgctgtcatcgtgcctgagctgctgcccaagccgggccaggagttcctggcgtccgcagaaggtctgaatgacctccgagctctgccaaaggtggtggcggatctcttggtagagccacgccaactcctgtccggccgtatccagctcacggaggcgtgtgaggacctggtgattggccctcaccacaaactgctcacccagctccttcaggtagcaggcgtgagtcttgttcttggggttcaccaagtcgcggctccacggcaggcggtgggtcttgaggacccctgggtgcatgtcagtgatgtgacttttgaggctgctgagaaggttctgggcatcagcgtccaggcagccatccgcgagccggtccaccatcctaagggcgcagtcttcaaggatgtgtttgtggaggtcttggatctctctaaggaagacggtggctccctgttcccggtcctctgagctcagcaggctccgctctatctcccactcaatgactgaccggtggtagtgctgccactgctcctgggtgatgagccccagcctccgggcctcctgggctccagagcgtaggacagaagttaaggtggcctcctctggttcacaggcctccccagtacctggtgcctgcaggacgtaggtgggaggaaacgcattctcgtccctctggaagtatcgtgccaccagctccaggtcacttggcctggcagtcagatggtccctcaatacctcccactccttctcatcgatccgcgagggaatcagacaggggccgtactgatcaccgatgagggcaacaaaagctggccctatggatgttttccaacaccggtcaacctcctccaagcagagttctgtggtcaagtggtcagtggcttcaatgttccgaataccccacctcagatcaacgacctcaaacatcaagccgtgcctctggcagaaggtctggcacttcagggtaggcagtgctctgcagggcttccctctctgcatccatatcttggcatccgtgagcctggttggaatgccggctcctccatcgccctcctggaggacttaagcaagtggtctccctcccagggcatcggccgcatggtcaacagctgatatgtttctacatgttattgtttgtctgtcccacgagaaagtgaattccatgagcccaaggatcttgtctggtaaggctggcgtgcctggcacatagtaggtgctcagtaaattatcatcacaacagcttcctccacaactgtttctctttctggacttctgtttgttgctgaagaagacagctgagcaggactgggcttccccagtaaggacagaggccctttgcagtgtcagcgttctggctgtcctgggggctccagcctctctttagcctttgctggtagttgaacgaccaatttagactcctctggggaaataggttagagaggacagtttcctggcctcggcgccacccggaagacaagcccctggctatcctagtaactttcgtcttaggtattttatgggtctctccttgcccaattctcccagcaactgggataatgaaagcgattgtttgcactagggcaccagcttagccgggcattcagcccagacttagtggttaactattgtgtgccaggctgatacggctcctcgtaaaagatgccatttgctgacagtctaggaggtgcagttggttggcatttggcattagcagtccacattattaccccaagagacagacattatgatcctgtttcacagatgaagaaaacaagatgcagaaaggtgaagtcccttgcctgtgacgcttcactactctgcacttgaattttctcactaacttcctgtgttggtgagacaatgaaaagcat

SEQ ID NO: 8520 - RNA, 8103 nt, Homo sapiens
  source 1..8103: mol_type = other RNA
aaaagtaattgtggtttttgccattacttttttttttttttttttttggagacagagtctctgtcactcatgctggagtgcagtggtgcgatctcggctcactgcaacctccgcctcccgggttcaagccattctcctgcctcagcctcccaagtagctggaattacaggtgtacgtcaccacaccaggctaatttttgtatttttgagtagagacagagtttcaccatgttgaccaggctgctcttgaacacctggcctcaagtgatccacccgcctcagcctcccaaagtgctgggattacaggcgtgagccaccgaggcttttgccattattattattattatgagatggagtcttgctctgtcacccaggctggagtgcagtggcacaatctcagctcactgcaacctccgcctcccgggttcaagtgattctcctgactcagcctcctgagtaactgagattacaggcactcaccaccatgcctggctgatttttgtatttttagtagagaagggtttcaccatgttgtccaggctggtctcaaactcctgacctcaggtgatccacctgcctcggccttccaaagagctgggaccacaggtgtgagccactgtgcccagccagtttttgccattatttttaatatttttaatggcgaaaaccacagttactttttgcaccaaccttagtaatcttcaacaccttagaagctgctgcccaatacatccaagcatacatcttaaaattacagtttaaaatatttttaaatgaaatttgacactaacatttgcagaactaccaaaacctgccttggaaaactggtttggaaaatggatgaataagacagcagtagggtcttgttcagctcaaaagcctctgtttctaaggttgcttttattgagactctatcaggaattccacggaggggagaagggatagccaccttgaagatttagactatcctagcattaaagtaaaagcctgagaagactgagaagggcttttagaaggctgtgggcaaagaagaaagatccacttaagtggaatgaaaacagtttgactgttgaacttgcacaaggcagacagttcaaaagcaaagcagggagagatcagcagctctttctacttccaagagcctccagtttttaagattaaaaacccacatctttatcccaaaagtttgggagccaaggaatagagagggatgaactataacatgttgattgttttactgccagcgtgagtcctgaagtcagctcattaaccaaagacgcacatgccaaatgcactatagatataaattcaaccaatcgccaactttaaaagtcagaacatttttgcataaaagtctggatttctggctttgcttattacaactggaagcactgacagcagtgggcttgtttggccatggtgattctgggctacagtcaggctgctcatacccaccctagacacaatctctgccttccacatgtccagtctctgtctctccctgctgctcacccaggtgcatggaagtgtctagattagtcactagctcctgtgagcatttgagtgtggtgcctgtggaagagatggttgtgctctgcagactgaaattggagtgaggtctaacaggaatgggacagaaggctcactctcagagctcttgcaccttggacttgtgacctgaatcaaattataactacttccgcaaggctcagtttcctcatctgtaaaatagatacagaaactcctgccctccctaaagtatgagttgtgatgaggatcagatgacagcacctacagctttataaactgtgaggttctgtggtccacatcagtgatttgctgtatctcacattcatccgttcccccttcatctggtaccagaactccagtttgcatctcaggagtaatctcttctattctcagtcccagtggtggacattggatcagtctagccgattagagctctgcattctcccagatataataattggtttagggctaggcgtatgggccaattgggaccagtagagttgaggctaggactgttgggaaagagaagctctcttttctattgaaattggagacagcagcatattggccaccatgttgctaacctgggggtggcaagtctgagaatgaaaatgaaaaagaggaaagaataatggaaagatgagaagagacaaggtctgaagccataatctgaagccatgggtccagatatacaccagcaaacgtattctttttgctttaactagattaaatggggctaactcactggagccccatacccccacagggtttttttatttttatttttttacactatcaggcacacttgtgagcatttgtttgatttggtttcatttccctgggcactttctgactccaagtcctggggagctcctgcagctgcaactagctcctctctctgcctggatttgaccatccacattgccttcttgaagttcttaagagggtcctgcggtgaggcttttgctgaaaggcactggaaattctctcggatcagataaccatgcctggtgggggcaatgaagccactggtggttgggatgattctgtttaccacagcatggacaaactggactgtcagcagggtgccatccagcacactccaaacaagtatagagcgatcctttaagcccacgtacacatacttgtcatccttggagaagcaagcacattggacccctctgcagtaagaactcgtgtagctcatctcgaatttccacttgcgtgcctgcaggtcccagagacacagcagggcatcctcagacccgctgaccaccagctgctccttgtggctgacctccacacaggcaactcggctcctgtgggtctccaagggaaacgctttggaagttgcacactcgtaaagaaagaggtccccattggtcatgctgtagaccacgcggtagtccgtcagaatggccacgctggagagggtctcgggcagctgagtgtaaaaggtgtatcttggcccatcgatgaccgggcaggggtccccggaggtgatgtccagcaccaggacgatgttgtcataggcgatggccaggcggtcctcgcacttgctcagggacatgcagttgattgctttccgggcctcgggagggggaatgcatatcacgtcctgcctggaattcagggggaacacaaggacgacccccgacacgaggcccgtaaataggagcttgcgctgctcagcaacctccagacacctgatctcactggaggtgtccagggaatcttgttcctcgccttctgccaagtcccaaatagtgactttgtttttgtccccaattttggggaagtagacgtagcttccattgtgggacactgcggtgaggccggtgcggtccagaaatggtgcaggcacccgggacctatgagcatcgctgagatcccagaccttgaaagatgaggactgtggggaagcagatgccaccaaagccccgccgcgggccagcaggctcacgggggccccgacgccttccaggatgtccagaagggtcccctgttctgacagactccacacctgaatgagcgcatcaagggaccccgtgatgatcaggttgttctcagtaccaaaaacagccgtctccaccatgtcttcatgttccagatccatggccatgaatcggcgaaagcccctcgagtccgccaagaatatccgcaccgatcttccaaagcctgcggcgaggagggactcatcttcagagaccaccaggaacctcacagcatctggaagcttctccagcaatctgtcccctttggaggaaaccaaagagatggagccattgctaaacccggtaacaagctttccttgcttctggactgagacggcacaggtaggtgtttcttctttgatgctggacatatgttgcttcccctgaagttttcccgtagctgagctccacagactgaccacaccatccctggacactgtcagcagtgtggcctgggaggccagcacggccatgcacatccaaggatcagaggcatctcccaggatatggaataccggctctgcagtttccagattccaagcattgatctttgagccagatgctgaatacacaactttgtgtgcctcatccacatgaaggttccagatctgaggttcagcgggattttttgagcctccatcccaaatggtaaatttctcctggccagagagtaagttccacaagtgcagcgtgtaatcctttgaagcagagttggcgagggtccctttggcaaatattttcacacacctcacctctcctgtgtgtccagttagcatgtggatcacatgctgctcttccatgtcccacacagccatgatgccatcctgggtgccaatcaccagcagcttctcctccacaccccatgccatggcggtgatgcctttgtgacagccgctgagagttgcccggaggggtcctcccgggggctggaggaatcctccgaggggcaccagcacagggtgtgcgcacaactggaaccagctctgggcctgttggcatagctgtcccaccagtgctggatgtgaggtggcgaagaaatggagtctggccagcagttctgtgtacaggaggctcctctccatgcctcggagctccacagcagggcggcagagctggagggcttcacggaccaggccaacctcaggggagtccaggtgaggggcacacaggtcaaagtcatccagcaggtcttcaatgcccccagagatgccccggcaggaaatccagctcatgctgcccagaacctcctgtttcagctcctccaggcggcccgagtgaagcaggtgatagggcaactccttcagcttccgcaggtttgcaaccgtatgtgagaaccacagaggctgcggggccacctttcggtccaagttcagtggtttccccacaagtggcagagtgatgagcttcttggtaccctggctccaggtccctgagaagaagtcggccaggacgccatgcctcttggctctctcggatcctgacaggtagcgctcacggaccacctcgaccagctgtctgtgggcaatggccaggagggtgaagccatccacgggccgccgggccaagtagtatcccagatcccgacgaagccgcacccacagcaggggcgggaagcgcagcagctccttgctgggcggggtccaatctcggtacacatcctgcaggacctcgtcgtccagggacaaaacatccttcagctccgcctccgagagaccgtgtcgggaagacacaatgtagcccagcacgtgggccacgaggagctgcccgtgtgtctgctccaggcgggtgcagagttggtgcgtggcttcctctgcggtggtggccagcgggacaggcacggtgaaagaggcccatttccgggcttcctcaaacgccagcctcagccgccctgggttcccacactctgggaggctggcccagagcaaatctgtgtgcaccgggctcagcgtcctccttgcagctgccagcaggagttggatcatctgctggccttggtttccggaaaggggcttcacctcccagtaggcctccgggtccaggagcacccgctgcaaggtgtccaaaacccccagtgcccccgagcaagctgagaggatgaggtgcaccctcggggggcagttgagaggcagccagggaaccctccgagcatggcggacagagtccaggtcatccatagcatccagcaggagcacgagagactcgaagtttctgcaagagacagtgtggaggagggtatggaaaaactggaccaccctggtgtgggcgtccagaacctgggcagggggcaagggcagcccataggccaggcacacctggaagcagatgctcttcagcaggccacgggcatctgagctcatttgtgacgtccccagcagccgcaggacggtcactgtcttgtgccccagcagccttggcatctgctcagccagcttgcacatcagggctgtctttccaatgcctgggggcccaaagagtaccaggggggtgtgctgcttgctgtcatcgtgcctgagctgctgcccaagccgggccaggagttcctggcgtccgcagaaggtctgaatgacctccgagctctgccaaaggtggtggcggatctcttggtagagccacgccaactcctgtccggccgtatccagctcacggaggcgtgtgaggacctggtgattggccctcaccacaaactgctcacccagctccttcaggtagcaggcgtgagtcttgttcttggggttcaccaagtcgcggctccacggcaggcggtgggtcttgaggacccctgggtgcatgtcagtgatgtgacttttgaggctgctgagaaggttctgggcatcagcgtccaggcagccatccgcgagccggtccaccatcctaagggcgcagtcttcaaggatgtgtttgtggaggtcttggatctctctaaggaagacggtggctccctgttcccggtcctctgagctcagcaggctccgctctatctcccactcaatgactgaccggtggtagtgctgccactgctcctgggtgatgagccccagcctccgggcctcctgggctccagagcgtaggacagaagttaaggtggcctcctctggttcacaggcctccccagtacctggtgcctgcaggacgtaggtgggaggaaacgcattctcgtccctctggaagtatcgtgccaccagctccaggtcacttggcctggcagtcagatggtccctcaatacctcccactccttctcatcgatccgcgagggaatcagacaggggccgtactgatcaccgatgagggcaacaaaagctggccctatggatgttttccaacaccggtcaacctcctccaagcagagttctgtggtcaagtggtcagtggcttcaatgttccgaataccccacctcagatcaacgacctcaaacatcaagccgtgcctctggcagaaggtctggcacttcagggtaggcagtgctctgcagggcttccctctctgcatccatatcttggcatccgtgagcctggttggaatgccggctcctccatcgccctcctggaggacttaagcaagtggtctccctcccagggcatcggccgcatggtctggataccacagtttagctgcagcctgctgatctcactgaggccccagttctgggtcccagcatctctccagacctctcttagcacctcctccccaatcttctgatcttgaatttgcctccaccacaatttctgttccttctctcgttttcctgggtcccagcaggctccttggacccgaattcacttcagcgcctggccacgctcccttggttactgccaacagctgatatgtttctacatgttattgtttgtctgtcccacgagaaagtgaattccatgagcccaaggatcttgtctggtaaggctggcgtgcctggcacatagtaggtgctcagtaaattatcatcacaacagcttcctccacaactgtttctctttctggacttctgtttgttgctgaagaagacagctgagcaggactgggcttccccagtaaggacagaggccctttgcagtgtcagcgttctggctgtcctgggggctccagcctctctttagcctttgctggtagttgaacgaccaatttagactcctctggggaaataggttagagaggacagtttcctggcctcggcgccacccggaagacaagcccctggctatcctagtaactttcgtcttaggtattttatgggtctctccttgcccaattctcccagcaactgggataatgaaagcgattgtttgcactagggcaccagcttagccgggcattcagcccagacttagtggttaactattgtgtgccaggctgatacggctcctcgtaaaagatgccatttgctgacagtctaggaggtgcagttggttggcatttggcattagcagtccacattattaccccaagagacagacattatgatcctgtttcacagatgaagaaaacaagatgcagaaaggtgaagtcccttgcctgtgacgcttcactactctgcacttgaattttctcactaacttcctgtgttggtgagacaatgaaaagcat

SEQ ID NO: 8521 - RNA, 7617 nt, Homo sapiens
  source 1..7617: mol_type = other RNA
aaaagtaattgtggtttttgccattacttttttttttttttttttttggagacagagtctctgtcactcatgctggagtgcagtggtgcgatctcggctcactgcaacctccgcctcccgggttcaagccattctcctgcctcagcctcccaagtagctggaattacaggtgtacgtcaccacaccaggctaatttttgtatttttgagtagagacagagtttcaccatgttgaccaggctgctcttgaacacctggcctcaagtgatccacccgcctcagcctcccaaagtgctgggattacaggcgtgagccaccgaggcttttgccattattattattattatgagatggagtcttgctctgtcacccaggctggagtgcagtggcacaatctcagctcactgcaacctccgcctcccgggttcaagtgattctcctgactcagcctcctgagtaactgagattacaggcactcaccaccatgcctggctgatttttgtatttttagtagagaagggtttcaccatgttgtccaggctggtctcaaactcctgacctcaggtgatccacctgcctcggccttccaaagagctgggaccacaggtgtgagccactgtgcccagccagtttttgccattatttttaatatttttaatggcgaaaaccacagttactttttgcaccaaccttagtaatcttcaacaccttagaagctgctgcccaatacatccaagcatacatcttaaaattacagtttaaaatatttttaaatgaaatttgacactaacatttgcagaactaccaaaacctgccttggaaaactggtttggaaaatggatgaataagacagcagtagggtcttgttcagctcaaaagcctctgtttctaaggttgcttttattgagactctatcaggaattccacggaggggagaagggatagccaccttgaagatttagactatcctagcattaaagtaaaagcctgagaagactgagaagggcttttagaaggctgtgggcaaagaagaaagatccacttaagtggaatgaaaacagtttgactgttgaacttgcacaaggcagacagttcaaaagcaaagcagggagagatcagcagctctttctacttccaagagcctccagtttttaagattaaaaacccacatctttatcccaaaagtttgggagccaaggaatagagagggatgaactataacatgttgattgttttactgccagcgtgagtcctgaagtcagctcattaaccaaagacgcacatgccaaatgcactatagatataaattcaaccaatcgccaactttaaaagtcagaacatttttgcataaaagtctggatttctggctttgcttattacaactggaagcactgacagcagtgggcttgtttggccatggtgattctgggctacagtcaggctgctcatacccaccctagacacaatctctgccttccacatgtccagtctctgtctctccctgctgctcacccaggtgcatggaagtgtctagattagtcactagctcctgtgagcatttgagtgtggtgcctgtggaagagatggttgtgctctgcagactgaaattggagtgaggtctaacaggaatgggacagaaggctcactctcagagctcttgcaccttggacttgtgacctgaatcaaattataactacttccgcaaggctcagtttcctcatctgtaaaatagatacagaaactcctgccctccctaaagtatgagttgtgatgaggatcagatgacagcacctacagctttataaactgtgaggttctgtggtccacatcagtgatttgctgtatctcacattcatccgttcccccttcatctggtaccagaactccagtttgcatctcaggagtaatctcttctattctcagtcccagtggtggacattggatcagtctagccgattagagctctgcattctcccagatataataattggtttagggctaggcgtatgggccaattgggaccagtagagttgaggctaggactgttgggaaagagaagctctcttttctattgaaattggagacagcagcatattggccaccatgttgctaacctgggggtggcaagtctgagaatgaaaatgaaaaagaggaaagaataatggaaagatgagaagagacaaggtctgaagccataatctgaagccatgggtccagatatacaccagcaaacgtattctttttgctttaactagattaaatggggctaactcactggagccccatacccccacagggtttttttatttttatttttttacactatcaggcacacttgtgagcatttgtttgatttggtttcatttccctgggcactttctgactccaagtcctggggagctcctgcagctgcaactagctcctctctctgcctggatttgaccatccacattgccttcttgaagttcttaagagggtcctgcggtgaggcttttgctgaaaggcactggaaattctctcggatcagataaccatgcctggtgggggcaatgaagccactggtggttgggatgattctgtttaccacagcatggacaaactggactgtcagcagggtgccatccagcacactccaaacaagtatagagcgatcctttaagcccacgtacacatacttgtcatccttggagaagcaagcacattggacccctctgcagtaagaactcgtgtagctcatctcgaatttccacttgcgtgcctgcaggtcccagagacacagcagggcatcctcagacccgctgaccaccagctgctccttgtggctgacctccacacaggcaactcggctcctgtgggtctccaagggaaacgctttggaagttgcacactcgtaaagaaagaggtccccattggtcatgctgtagaccacgcggtagtccgtcagaatggccacgctggagagggtctcgggcagctgagtgtaaaaggtgtatcttggcccatcgatgaccgggcaggggtccccggaggtgatgtccagcaccaggacgatgttgtcataggcgatggccaggcggtcctcgcacttgctcagggacatgcagttgattgctttccgggcctcgggagggggaatgcatatcacgtcctgcctggaattcagggggaacacaaggacgacccccgacacgaggcccgtaaataggagcttgcgctgctcagcaacctccagacacctgatctcactggaggtgtccagggaatcttgttcctcgccttctgccaagtcccaaatagtgactttgtttttgtccccaattttggggaagtagacgtagcttccattgtgggacactgcggtgaggccggtgcggtccagaaatggtgcaggcacccgggacctatgagcatcgctgagatcccagaccttgaaagatgaggactgtggggaagcagatgccaccaaagccccgccgcgggccagcaggctcacgggggccccgacgccttccaggatgtccagaagggtcccctgttctgacagactccacacctgaatgagcgcatcaagggaccccgtgatgatcaggttgttctcagtaccaaaaacagccgtctccaccatgtcttcatgttccagatccatggccatgaatcggcgaaagcccctcgagtccgccaagaatatccgcaccgatcttccaaagcctgcggcgaggagggactcatcttcagagaccaccaggaacctcacagcatctggaagcttctccagcaatctgtcccctttggaggaaaccaaagagatggagccattgctaaacccggtaacaagctttccttgcttctggactgagacggcacaggtaggtgtttcttctttgatgctggacatatgttgcttcccctgaagttttcccgtagctgagctccacagactgaccacaccatccctggacactgtcagcagtgtggcctgggaggccagcacggccatgcacatccaaggatcagaggcatctcccaggatatggaataccggctctgcagtttccagattccaagcattgatctttgagccagatgctgaatacacaactttgtgtgcctcatccacatgaaggttccagatctgaggttcagcgggattttttgagcctccatcccaaatggtaaatttctcctggccagagagtaagttccacaagtgcagcgtgtaatcctttgaagcagagttggcgagggtccctttggcaaatattttcacacacctcacctctcctgtgtgtccagttagcatgtggatcacatgctgctcttccatgtcccacacagccatgatgccatcctgggtgccaatcaccagcagcttctcctccacaccccatgccatggcggtgatgcctttgtgacagccgctgagagttgcccggaggggtcctcccgggggctggaggaatcctccgaggggcaccagcacagggtgtgcgcacaactggaaccagctctgggcctgttggcatagctgtcccaccagtgctggatgtgaggtggcgaagaaatggagtctggccagcagttctgtgtacaggaggctcctctccatgcctcggagctccacagcagggcggcagagctggagggcttcacggaccaggccaacctcaggggagtccaggtgaggggcacacaggtcaaagtcatccagcaggtcttcaatgcccccagagatgccccggcaggaaatccagctcatgctgcccagaacctcctgtttcagctcctccaggcggcccgagtgaagcaggtgatagggcaactccttcagcttccgcaggtttgcaaccgtatgtgagaaccacagaggctgcggggccacctttcggtccaagttcagtggtttccccacaagtggcagagtgatgagcttcttggtaccctggctccaggtccctgagaagaagtcggccaggacgccatgcctcttggctctctcggatcctgacaggtagcgctcacggaccacctcgaccagctgtctgtgggcaatggccaggagggtgaagccatccacgggccgccgggccaagtagtatcccagatcccgacgaagccgcacccacagcaggggcgggaagcgcagcagctccttgctgggcggggtccaatctcggtacacatcctgcaggacctcgtcgtccagggacaaaacatccttcagctccgcctccgagagaccgtgtcgggaagacacaatgtagcccagcacgtgggccacgaggagctgcccgtgtgtctgctccaggcgggtgcagagttggtgcgtggcttcctctgcggtggtggccagcgggacaggcacggtgaaagaggcccatttccgggcttcctcaaacgccagcctcagccgccctgggttcccacactctgggaggctggcccagagcaaatctgtgtgcaccgggctcagcgtcctccttgcagctgccagcaggagttggatcatctgctggccttggtttccggaaaggggcttcacctcccagtaggcctccgggtccaggagcacccgctgcaaggtgtccaaaacccccagtgcccccgagcaagctgagaggatgaggtgcaccctcggggggcagttgagaggcagccagggaaccctccgagcatggcggacagagtccaggtcatccatagcatccagcaggagcacgagagactcgaagtttctgcaagagacagtgtggaggagggtatggaaaaactggaccaccctggtgtgggcgtccagaacctgggcagggggcaagggcagcccataggccaggcacacctggaagcagatgctcttcagcaggccacgggcatctgagctcatttgtgacgtccccagcagccgcaggacggtcactgtcttgtgccccagcagccttggcatctgctcagccagcttgcacatcagggctgtctttccaatgcctgggggcccaaagagtaccaggggggtgtgctgcttgctgtcatcgtgcctgagctgctgcccaagccgggccaggagttcctggcgtccgcagaaggtctgaatgacctccgagctctgccaaaggtggtggcggatctcttggtagagccacgccaactcctgtccggccgtatccagctcacggaggcgtgtgaggacctggtgattggccctcaccacaaactgctcacccagctccttcaggtagcaggcgtgagtcttgttcttggggttcaccaagtcgcggctccacggcaggcggtgggtcttgaggacccctgggtgcatgtcagtgatgtgacttttgaggctgctgagaaggttctgggcatcagcgtccaggcagccatccgcgagccggtccaccatcctaagggcgcagtcttcaaggatgtgtttgtggaggtcttggatctctctaaggaagacggtggctccctgttcccggtcctctgagctcagcaggctccgctctatctcccactcaatgactgaccggtggtagtgctgccactgctcctgggtgatgagccccagcctccgggcctcctgggctccagagcgtaggacagaagttaaggtggcctcctctggttcacaggcctccccagtacctggtgcctgcaggacgtaggtgggaggaaacgcattctcgtccctctggaagtatcgtgccaccagctccaggtcacttggcctggcagtcagatggtccctcaatacctcccactccttctcatcgatccgcgagggaatcagacaggggccgtactgatcaccgatgagggcaacaaaagctggccctatggatgttttccaacaccggtcaacctcctccaagcagagttctgtggtcaagtggtcagtggcttcaatgttccgaataccccacctcagatcaacgacctcaaacatcaagccgtgcctctggcagaaggtctggcacttcagggtaggcagtgctctgcagggcttccctctctgcatccatatcttggcatccgtgagcctggttggaatgccggctcctccatcgccctcctggaggacttaagcaagtggtctccctcccagggcatcggccgcatggtctggataccacagtttagctgcagcctgctgatctcactgaggccccagttctgggtcccagcatctctccagacctctcttagcacctcctccccaatcttctgatcttgaatttgcctccaccacaatttctgttccttctctcgttttcctgggtcccagcaggctccttggacccgaattcacttcagcgcctggccacgctcccttggttactgcctgcaacagctgatatgtttctacatgttattgtttgtctgtcccacgagaaagtgaattccatgagcccaaggatcttgtctggtaaggctggcgtgcctggcacatagtaggtgctcagtaaattatcatcacaacagcttcctccacaactgtttctctttctggacttctgtttgttgctgaagaagacagctgagcaggactgggcttccccagtaaggacagaggccctttgcagtgtcagcgttctggctgtcctgggggctccagcctctcttt

SEQ ID NO: 8522 - RNA, 7084 nt, Homo sapiens
  source 1..7084: mol_type = other RNA
aaaagtaattgtggtttttgccattacttttttttttttttttttttggagacagagtctctgtcactcatgctggagtgcagtggtgcgatctcggctcactgcaacctccgcctcccgggttcaagccattctcctgcctcagcctcccaagtagctggaattacaggtgtacgtcaccacaccaggctaatttttgtatttttgagtagagacagagtttcaccatgttgaccaggctgctcttgaacacctggcctcaagtgatccacccgcctcagcctcccaaagtgctgggattacaggcgtgagccaccgaggcttttgccattattattattattatgagatggagtcttgctctgtcacccaggctggagtgcagtggcacaatctcagctcactgcaacctccgcctcccgggttcaagtgattctcctgactcagcctcctgagtaactgagattacaggcactcaccaccatgcctggctgatttttgtatttttagtagagaagggtttcaccatgttgtccaggctggtctcaaactcctgacctcaggtgatccacctgcctcggccttccaaagagctgggaccacaggtgtgagccactgtgcccagccagtttttgccattatttttaatatttttaatggcgaaaaccacagttactttttgcaccaaccttagtaatcttcaacaccttagaagctgctgcccaatacatccaagcatacatcttaaaattacagtttaaaatatttttaaatgaaatttgacactaacatttgcagaactaccaaaacctgccttggaaaactggtttggaaaatggatgaataagacagcagtagggtcttgttcagctcaaaagcctctgtttctaaggttgcttttattgagactctatcaggaattccacggaggggagaagggatagccaccttgaagatttagactatcctagcattaaagtaaaagcctgagaagactgagaagggcttttagaaggctgtgggcaaagaagaaagatccacttaagtggaatgaaaacagtttgactgttgaacttgcacaaggcagacagttcaaaagcaaagcagggagagatcagcagctctttctacttccaagagcctccagtttttaagattaaaaacccacatctttatcccaaaagtttgggagccaaggaatagagagggatgaactataacatgttgattgttttactgccagcgtgagtcctgaagtcagctcattaaccaaagacgcacatgccaaatgcactatagatataaattcaaccaatcgccaactttaaaagtcagaacatttttgcataaaagtctggatttctggctttgcttattacaactggaagcactgacagcagtgggcttgtttggccatggtgattctgggctacagtcaggctgctcatacccaccctagacacaatctctgccttccacatgtccagtctctgtctctccctgctgctcacccaggtgcatggaagtgtctagattagtcactagctcctgtgagcatttgagtgtggtgcctgtggaagagatggttgtgctctgcagactgaaattggagtgaggtctaacaggaatgggacagaaggctcactctcagagctcttgcaccttggacttgtgacctgaatcaaattataactacttccgcaaggctcagtttcctcatctgtaaaatagatacagaaactcctgccctccctaaagtatgagttgtgatgaggatcagatgacagcacctacagctttataaactgtgaggttctgtggtccacatcagtgatttgctgtatctcacattcatccgttcccccttcatctggtaccagaactccagtttgcatctcaggagtaatctcttctattctcagtcccagtggtggacattggatcagtctagccgattagagctctgcattctcccagatataataattggtttagggctaggcgtatgggccaattgggaccagtagagttgaggctaggactgttgggaaagagaagctctcttttctattgaaattggagacagcagcatattggccaccatgttgctaacctgggggtggcaagtctgagaatgaaaatgaaaaagaggaaagaataatggaaagatgagaagagacaaggtctgaagccataatctgaagccatgggtccagatatacaccagcaaacgtattctttttgctttaactagattaaatggggctaactcactggagccccatacccccacagggtttttttatttttatttttttacactatcaggcacacttgtgagcatttgtttgatttggtttcatttccctgggcactttctgactccaagtcctggggagctcctgcagctgcaactagctcctctctctgcctggatttgaccatccacattgccttcttgaagttcttaagagggtcctgcggtgaggcttttgctgaaaggcactggaaattctctcggatcagataaccatgcctggtgggggcaatgaagccactggtggttgggatgattctgtttaccacagcatggacaaactggactgtcagcagggtgccatccagcacactccaaacaagtatagagcgatcctttaagcccacgtacacatacttgtcatccttggagaagcaagcacattggacccctctgcagtaagaactcgtgtagctcatctcgaatttccacttgcgtgcctgcaggtcccagagacacagcagggcatcctcagacccgctgaccaccagctgctccttgtggctgacctccacacaggcaactcggctcctgtgggtctccaagggaaacgctttggaagttgcacactcgtaaagaaagaggtccccattggtcatgctgtagaccacgcggtagtccgtcagaatggccacgctggagagggtctcgggcagctgagtgtaaaaggtgtatcttggcccatcgatgaccgggcaggggtccccggaggtgatgtccagcaccaggacgatgttgtcataggcgatggccaggcggtcctcgcacttgctcagggacatgcagttgattgctttccgggcctcgggagggggaatgcatatcacgtcctgcctggaattcagggggaacacaaggacgacccccgacacgaggcccgtaaataggagcttgcgctgctcagcaacctccagacacctgatctcactggaggtgtccagggaatcttgttcctcgccttctgccaagtcccaaatagtgactttgtttttgtccccaattttggggaagtagacgtagcttccattgtgggacactgcggtgaggccggtgcggtccagaaatggtgcaggcacccgggacctatgagcatcgctgagatcccagaccttgaaagatgaggactgtggggaagcagatgccaccaaagccccgccgcgggccagcaggctcacgggggccccgacgccttccaggatgtccagaagggtcccctgttctgacagactccacacctgaatgagcgcatcaagggaccccgtgatgatcaggttgttctcagtaccaaaaacagccgtctccaccatgtcttcatgttccagatccatggccatgaatcggcgaaagcccctcgagtccgccaagaatatccgcaccgatcttccaaagcctgcggcgaggagggactcatcttcagagaccaccaggaacctcacagcatctggaagcttctccagcaatctgtcccctttggaggaaaccaaagagatggagccattgctaaacccggtaacaagctttccttgcttctggactgagacggcacaggtaggtgtttcttctttgatgctggacatatgttgcttcccctgaagttttcccgtagctgagctccacagactgaccacaccatccctggacactgtcagcagtgtggcctgggaggccagcacggccatgcacatccaaggatcagaggcatctcccaggatatggaataccggctctgcagtttccagattccaagcattgatctttgagccagatgctgaatacacaactttgtgtgcctcatccacatgaaggttccagatctgaggttcagcgggattttttgagcctccatcccaaatggtaaatttctcctggccagagagtaagttccacaagtgcagcgtgtaatcctttgaagcagagttggcgagggtccctttggcaaatattttcacacacctcacctctcctgtgtgtccagttagcatgtggatcacatgctgctcttccatgtcccacacagccatgatgccatcctgggtgccaatcaccagcagcttctcctccacaccccatgccatggcggtgatgcctttgtgacagccgctgagagttgcccggaggggtcctcccgggggctggaggaatcctccgaggggcaccagcacagggtgtgcgcacaactggaaccagctctgggcctgttggcatagctgtcccaccagtgctggatgtgaggtggcgaagaaatggagtctggccagcagttctgtgtacaggaggctcctctccatgcctcggagctccacagcagggcggcagagctggagggcttcacggaccaggccaacctcaggggagtccaggtgaggggcacacaggtcaaagtcatccagcaggtcttcaatgcccccagagatgccccggcaggaaatccagctcatgctgcccagaacctcctgtttcagctcctccaggcggcccgagtgaagcaggtgatagggcaactccttcagcttccgcaggtttgcaaccgtatgtgagaaccacagaggctgcggggccacctttcggtccaagttcagtggtttccccacaagtggcagagtgatgagcttcttggtaccctggctccaggtccctgagaagaagtcggccaggacgccatgcctcttggctctctcggatcctgacaggtagcgctcacggaccacctcgaccagctgtctgtgggcaatggccaggagggtgaagccatccacgggccgccgggccaagtagtatcccagatcccgacgaagccgcacccacagcaggggcgggaagcgcagcagctccttgctgggcggggtccaatctcggtacacatcctgcaggacctcgtcgtccagggacaaaacatccttcagctccgcctccgagagaccgtgtcgggaagacacaatgtagcccagcacgtgggccacgaggagctgcccgtgtgtctgctccaggcgggtgcagagttggtgcgtggcttcctctgcggtggtggccagcgggacaggcacggtgaaagaggcccatttccgggcttcctcaaacgccagcctcagccgccctgggttcccacactctgggaggctggcccagagcaaatctgtgtgcaccgggctcagcgtcctccttgcagctgccagcaggagttggatcatctgctggccttggtttccggaaaggggcttcacctcccagtaggcctccgggtccaggagcacccgctgcaaggtgtccaaaacccccagtgcccccgagcaagctgagaggatgaggtgcaccctcggggggcagttgagaggcagccagggaaccctccgagcatggcggacagagtccaggtcatccatagcatccagcaggagcacgagagactcgaagtttctgcaagagacagtgtggaggagggtatggaaaaactggaccaccctggtgtgggcgtccagaacctgggcagggggcaagggcagcccataggccaggcacacctggaagcagatgctcttcagcaggccacgggcatctgagctcatttgtgacgtccccagcagccgcaggacggtcactgtcttgtgccccagcagccttggcatctgctcagccagcttgcacatcagggctgtctttccaatgcctgggggcccaaagagtaccaggggggtgtgctgcttgctgtcatcgtgcctgagctgctgcccaagccgggccaggagttcctggcgtccgcagaaggtctgaatgacctccgagctctgccaaaggtggtggcggatctcttggtagagccacgccaactcctgtccggccgtatccagctcacggaggcgtgtgaggacctggtgattggccctcaccacaaactgctcacccagctccttcaggtagcaggcgtgagtcttgttcttggggttcaccaagtcgcggctccacggcaggcggtgggtcttgaggacccctgggtgcatgtcagtgatgtgacttttgaggctgctgagaaggttctgggcatcagcgtccaggcagccatccgcgagccggtccaccatcctaagggcgcagtcttcaaggatgtgtttgtggaggtcttggatctctctaaggaagacggtggctccctgttcccggtcctctgagctcagcaggctccgctctatctcccactcaatgactgaccggtggtagtgctgccactgctcctgggtgatgagccccagcctccgggcctcctgggctccagagcgtaggacagaagttaaggtggcctcctctggttcacaggcctccccagtacctggtgcctgcaggacgtaggtgggaggaaacgcattctcgtccctctggaagtatcgtgccaccagctccaggtcacttggcctggcagtcagatggtccctcaatacctcccactccttctcatcgatccgcgagggaatcagacaggggccgtactgatcaccgatgagggcctggccatggtacttttctttactttttccctctttactgtccaggacagggatcagcacatttctcaacaaaagctggccctatggatgttttccaacaccggtcaacctcctccaagcagagttctgtggtcaagtggtcagtggcttcaatgttccgaataccccacctcagatcaacgacctcaaacatcaagccgtgcctctggcagaaggtctggcacttcagggtaggcagtgctctgcagggcttccctctctgcatccatat

SEQ ID NO: 8523 - RNA, 8170 nt, Homo sapiens
  source 1..8170: mol_type = other RNA
aaaagtaattgtggtttttgccattacttttttttttttttttttttggagacagagtctctgtcactcatgctggagtgcagtggtgcgatctcggctcactgcaacctccgcctcccgggttcaagccattctcctgcctcagcctcccaagtagctggaattacaggtgtacgtcaccacaccaggctaatttttgtatttttgagtagagacagagtttcaccatgttgaccaggctgctcttgaacacctggcctcaagtgatccacccgcctcagcctcccaaagtgctgggattacaggcgtgagccaccgaggcttttgccattattattattattatgagatggagtcttgctctgtcacccaggctggagtgcagtggcacaatctcagctcactgcaacctccgcctcccgggttcaagtgattctcctgactcagcctcctgagtaactgagattacaggcactcaccaccatgcctggctgatttttgtatttttagtagagaagggtttcaccatgttgtccaggctggtctcaaactcctgacctcaggtgatccacctgcctcggccttccaaagagctgggaccacaggtgtgagccactgtgcccagccagtttttgccattatttttaatatttttaatggcgaaaaccacagttactttttgcaccaaccttagtaatcttcaacaccttagaagctgctgcccaatacatccaagcatacatcttaaaattacagtttaaaatatttttaaatgaaatttgacactaacatttgcagaactaccaaaacctgccttggaaaactggtttggaaaatggatgaataagacagcagtagggtcttgttcagctcaaaagcctctgtttctaaggttgcttttattgagactctatcaggaattccacggaggggagaagggatagccaccttgaagatttagactatcctagcattaaagtaaaagcctgagaagactgagaagggcttttagaaggctgtgggcaaagaagaaagatccacttaagtggaatgaaaacagtttgactgttgaacttgcacaaggcagacagttcaaaagcaaagcagggagagatcagcagctctttctacttccaagagcctccagtttttaagattaaaaacccacatctttatcccaaaagtttgggagccaaggaatagagagggatgaactataacatgttgattgttttactgccagcgtgagtcctgaagtcagctcattaaccaaagacgcacatgccaaatgcactatagatataaattcaaccaatcgccaactttaaaagtcagaacatttttgcataaaagtctggatttctggctttgcttattacaactggaagcactgacagcagtgggcttgtttggccatggtgattctgggctacagtcaggctgctcatacccaccctagacacaatctctgccttccacatgtccagtctctgtctctccctgctgctcacccaggtgcatggaagtgtctagattagtcactagctcctgtgagcatttgagtgtggtgcctgtggaagagatggttgtgctctgcagactgaaattggagtgaggtctaacaggaatgggacagaaggctcactctcagagctcttgcaccttggacttgtgacctgaatcaaattataactacttccgcaaggctcagtttcctcatctgtaaaatagatacagaaactcctgccctccctaaagtatgagttgtgatgaggatcagatgacagcacctacagctttataaactgtgaggttctgtggtccacatcagtgatttgctgtatctcacattcatccgttcccccttcatctggtaccagaactccagtttgcatctcaggagtaatctcttctattctcagtcccagtggtggacattggatcagtctagccgattagagctctgcattctcccagatataataattggtttagggctaggcgtatgggccaattgggaccagtagagttgaggctaggactgttgggaaagagaagctctcttttctattgaaattggagacagcagcatattggccaccatgttgctaacctgggggtggcaagtctgagaatgaaaatgaaaaagaggaaagaataatggaaagatgagaagagacaaggtctgaagccataatctgaagccatgggtccagatatacaccagcaaacgtattctttttgctttaactagattaaatggggctaactcactggagccccatacccccacagggtttttttatttttatttttttacactatcaggcacacttgtgagcatttgtttgatttggtttcatttccctgggcactttctgactccaagtcctggggagctcctgcagctgcaactagctcctctctctgcctggatttgaccatccacattgccttcttgaagttcttaagagggtcctgcggtgaggcttttgctgaaaggcactggaaattctctcggatcagataaccatgcctggtgggggcaatgaagccactggtggttgggatgattctgtttaccacagcatggacaaactggactgtcagcagggtgccatccagcacactccaaacaagtatagagcgatcctttaagcccacgtacacatacttgtcatccttggagaagcaagcacattggacccctctgcagtaagaactcgtgtagctcatctcgaatttccacttgcgtgcctgcaggtcccagagacacagcagggcatcctcagacccgctgaccaccagctgctccttgtggctgacctccacacaggcaactcggctcctgtgggtctccaagggaaacgctttggaagttgcacactcgtaaagaaagaggtccccattggtcatgctgtagaccacgcggtagtccgtcagaatggccacgctggagagggtctcgggcagctgagtgtaaaaggtgtatcttggcccatcgatgaccgggcaggggtccccggaggtgatgtccagcaccaggacgatgttgtcataggcgatggccaggcggtcctcgcacttgctcagggacatgcagttgattgctttccgggcctcgggagggggaatgcatatcacgtcctgcctggaattcagggggaacacaaggacgacccccgacacgaggcccgtaaataggagcttgcgctgctcagcaacctccagacacctgatctcactggaggtgtccagggaatcttgttcctcgccttctgccaagtcccaaatagtgactttgtttttgtccccaattttggggaagtagacgtagcttccattgtgggacactgcggtgaggccggtgcggtccagaaatggtgcaggcacccgggacctatgagcatcgctgagatcccagaccttgaaagatgaggactgtggggaagcagatgccaccaaagccccgccgcgggccagcaggctcacgggggccccgacgccttccaggatgtccagaagggtcccctgttctgacagactccacacctgaatgagcgcatcaagggaccccgtgatgatcaggttgttctcagtaccaaaaacagccgtctccaccatgtcttcatgttccagatccatggccatgaatcggcgaaagcccctcgagtccgccaagaatatccgcaccgatcttccaaagcctgcggcgaggagggactcatcttcagagaccaccaggaacctcacagcatctggaagcttctccagcaatctgtcccctttggaggaaaccaaagagatggagccattgctaaacccggtaacaagctttccttgcttctggactgagacggcacaggtaggtgtttcttctttgatgctggacatatgttgcttcccctgaagttttcccgtagctgagctccacagactgaccacaccatccctggacactgtcagcagtgtggcctgggaggccagcacggccatgcacatccaaggatcagaggcatctcccaggatatggaataccggctctgcagtttccagattccaagcattgatctttgagccagatgctgaatacacaactttgtgtgcctcatccacatgaaggttccagatctgaggttcagcgggattttttgagcctccatcccaaatggtaaatttctcctggccagagagtaagttccacaagtgcagcgtgtaatcctttgaagcagagttggcgagggtccctttggcaaatattttcacacacctcacctctcctgtgtgtccagttagcatgtggatcacatgctgctcttccatgtcccacacagccatgatgccatcctgggtgccaatcaccagcagcttctcctccacaccccatgccatggcggtgatgcctttgtgacagccgctgagagttgcccggaggggtcctcccgggggctggaggaatcctccgaggggcaccagcacagggtgtgcgcacaactggaaccagctctgggcctgttggcatagctgtcccaccagtgctggatgtgaggtggcgaagaaatggagtctggccagcagttctgtgtacaggaggctcctctccatgcctcggagctccacagcagggcggcagagctggagggcttcacggaccaggccaacctcaggggagtccaggtgaggggcacacaggtcaaagtcatccagcaggtcttcaatgcccccagagatgccccggcaggaaatccagctcatgctgcccagaacctcctgtttcagctcctccaggcggcccgagtgaagcaggtgatagggcaactccttcagcttccgcaggtttgcaaccgtatgtgagaaccacagaggctgcggggccacctttcggtccaagttcagtggtttccccacaagtggcagagtgatgagcttcttggtaccctggctccaggtccctgagaagaagtcggccaggacgccatgcctcttggctctctcggatcctgacaggtagcgctcacggaccacctcgaccagctgtctgtgggcaatggccaggagggtgaagccatccacgggccgccgggccaagtagtatcccagatcccgacgaagccgcacccacagcaggggcgggaagcgcagcagctccttgctgggcggggtccaatctcggtacacatcctgcaggacctcgtcgtccagggacaaaacatccttcagctccgcctccgagagaccgtgtcgggaagacacaatgtagcccagcacgtgggccacgaggagctgcccgtgtgtctgctccaggcgggtgcagagttggtgcgtggcttcctctgcggtggtggccagcgggacaggcacggtgaaagaggcccatttccgggcttcctcaaacgccagcctcagccgccctgggttcccacactctgggaggctggcccagagcaaatctgtgtgcaccgggctcagcgtcctccttgcagctgccagcaggagttggatcatctgctggccttggtttccggaaaggggcttcacctcccagtaggcctccgggtccaggagcacccgctgcaaggtgtccaaaacccccagtgcccccgagcaagctgagaggatgaggtgcaccctcggggggcagttgagaggcagccagggaaccctccgagcatggcggacagagtccaggtcatccatagcatccagcaggagcacgagagactcgaagtttctgcaagagacagtgtggaggagggtatggaaaaactggaccaccctggtgtgggcgtccagaacctgggcagggggcaagggcagcccataggccaggcacacctggaagcagatgctcttcagcaggccacgggcatctgagctcatttgtgacgtccccagcagccgcaggacggtcactgtcttgtgccccagcagccttggcatctgctcagccagcttgcacatcagggctgtctttccaatgcctgggggcccaaagagtaccaggggggtgtgctgcttgctgtcatcgtgcctgagctgctgcccaagccgggccaggagttcctggcgtccgcagaaggtctgaatgacctccgagctctgccaaaggtggtggcggatctcttggtagagccacgccaactcctgtccggccgtatccagctcacggaggcgtgtgaggacctggtgattggccctcaccacaaactgctcacccagctccttcaggtagcaggcgtgagtcttgttcttggggttcaccaagtcgcggctccacggcaggcggtgggtcttgaggacccctgggtgcatgtcagtgatgtgacttttgaggctgctgagaaggttctgggcatcagcgtccaggcagccatccgcgagccggtccaccatcctaagggcgcagtcttcaaggatgtgtttgtggaggtcttggatctctctaaggaagacggtggctccctgttcccggtcctctgagctcagcaggctccgctctatctcccactcaatgactgaccggtggtagtgctgccactgctcctgggtgatgagccccagcctccgggcctcctgggctccagagcgtaggacagaagttaaggtggcctcctctggttcacaggcctccccagtacctggtgcctgcaggacgtaggtgggaggaaacgcattctcgtccctctggaagtatcgtgccaccagctccaggtcacttggcctggcagtcagatggtccctcaatacctcccactccttctcatcgatccgcgagggaatcagacaggggccgtactgatcaccgatgagggcctggccatggtacttttctttactttttccctctttactgtccaggacagggatcagcacatttctcaacaaaagctggccctatggatgttttccaacaccggtcaacctcctccaagcagagttctgtggtcaagtggtcagtggcttcaatgttccgaataccccacctcagatcaacgacctcaaacatcaagccgtgcctctggcagaaggtctggcacttcagggtaggcagtgctctgcagggcttccctctctgcatccatatcttggcatccgtgagcctggttggaatgccggctcctccatcgccctcctggaggacttaagcaagtggtctccctcccagggcatcggccgcatggtctggataccacagtttagctgcagcctgctgatctcactgaggccccagttctgggtcccagcatctctccagacctctcttagcacctcctccccaatcttctgatcttgaatttgcctccaccacaatttctgttccttctctcgttttcctgggtcccagcaggctccttggacccgaattcacttcagcgcctggccacgctcccttggttactgccaacagctgatatgtttctacatgttattgtttgtctgtcccacgagaaagtgaattccatgagcccaaggatcttgtctggtaaggctggcgtgcctggcacatagtaggtgctcagtaaattatcatcacaacagcttcctccacaactgtttctctttctggacttctgtttgttgctgaagaagacagctgagcaggactgggcttccccagtaaggacagaggccctttgcagtgtcagcgttctggctgtcctgggggctccagcctctctttagcctttgctggtagttgaacgaccaatttagactcctctggggaaataggttagagaggacagtttcctggcctcggcgccacccggaagacaagcccctggctatcctagtaactttcgtcttaggtattttatgggtctctccttgcccaattctcccagcaactgggataatgaaagcgattgtttgcactagggcaccagcttagccgggcattcagcccagacttagtggttaactattgtgtgccaggctgatacggctcctcgtaaaagatgccatttgctgacagtctaggaggtgcagttggttggcatttggcattagcagtccacattattaccccaagagacagacattatgatcctgtttcacagatgaagaaaacaagatgcagaaaggtgaagtcccttgcctgtgacgcttcactactctgcacttgaattttctcactaacttcctgtgttggtgagacaatgaaaagcat

SEQ ID NO: 8524 - RNA, 8214 nt, Homo sapiens
  source 1..8214: mol_type = other RNA
aaaagtaattgtggtttttgccattacttttttttttttttttttttggagacagagtctctgtcactcatgctggagtgcagtggtgcgatctcggctcactgcaacctccgcctcccgggttcaagccattctcctgcctcagcctcccaagtagctggaattacaggtgtacgtcaccacaccaggctaatttttgtatttttgagtagagacagagtttcaccatgttgaccaggctgctcttgaacacctggcctcaagtgatccacccgcctcagcctcccaaagtgctgggattacaggcgtgagccaccgaggcttttgccattattattattattatgagatggagtcttgctctgtcacccaggctggagtgcagtggcacaatctcagctcactgcaacctccgcctcccgggttcaagtgattctcctgactcagcctcctgagtaactgagattacaggcactcaccaccatgcctggctgatttttgtatttttagtagagaagggtttcaccatgttgtccaggctggtctcaaactcctgacctcaggtgatccacctgcctcggccttccaaagagctgggaccacaggtgtgagccactgtgcccagccagtttttgccattatttttaatatttttaatggcgaaaaccacagttactttttgcaccaaccttagtaatcttcaacaccttagaagctgctgcccaatacatccaagcatacatcttaaaattacagtttaaaatatttttaaatgaaatttgacactaacatttgcagaactaccaaaacctgccttggaaaactggtttggaaaatggatgaataagacagcagtagggtcttgttcagctcaaaagcctctgtttctaaggttgcttttattgagactctatcaggaattccacggaggggagaagggatagccaccttgaagatttagactatcctagcattaaagtaaaagcctgagaagactgagaagggcttttagaaggctgtgggcaaagaagaaagatccacttaagtggaatgaaaacagtttgactgttgaacttgcacaaggcagacagttcaaaagcaaagcagggagagatcagcagctctttctacttccaagagcctccagtttttaagattaaaaacccacatctttatcccaaaagtttgggagccaaggaatagagagggatgaactataacatgttgattgttttactgccagcgtgagtcctgaagtcagctcattaaccaaagacgcacatgccaaatgcactatagatataaattcaaccaatcgccaactttaaaagtcagaacatttttgcataaaagtctggatttctggctttgcttattacaactggaagcactgacagcagtgggcttgtttggccatggtgattctgggctacagtcaggctgctcatacccaccctagacacaatctctgccttccacatgtccagtctctgtctctccctgctgctcacccaggtgcatggaagtgtctagattagtcactagctcctgtgagcatttgagtgtggtgcctgtggaagagatggttgtgctctgcagactgaaattggagtgaggtctaacaggaatgggacagaaggctcactctcagagctcttgcaccttggacttgtgacctgaatcaaattataactacttccgcaaggctcagtttcctcatctgtaaaatagatacagaaactcctgccctccctaaagtatgagttgtgatgaggatcagatgacagcacctacagctttataaactgtgaggttctgtggtccacatcagtgatttgctgtatctcacattcatccgttcccccttcatctggtaccagaactccagtttgcatctcaggagtaatctcttctattctcagtcccagtggtggacattggatcagtctagccgattagagctctgcattctcccagatataataattggtttagggctaggcgtatgggccaattgggaccagtagagttgaggctaggactgttgggaaagagaagctctcttttctattgaaattggagacagcagcatattggccaccatgttgctaacctgggggtggcaagtctgagaatgaaaatgaaaaagaggaaagaataatggaaagatgagaagagacaaggtctgaagccataatctgaagccatgggtccagatatacaccagcaaacgtattctttttgctttaactagattaaatggggctaactcactggagccccatacccccacagggtttttttatttttatttttttacactatcaggcacacttgtgagcatttgtttgatttggtttcatttccctgggcactttctgactccaagtcctggggagctcctgcagctgcaactagctcctctctctgcctggatttgaccatccacattgccttcttgaagttcttaagagggtcctgcggtgaggcttttgctgaaaggcactggaaattctctcggatcagataaccatgcctggtgggggcaatgaagccactggtggttgggatgattctgtttaccacagcatggacaaactggactgtcagcagggtgccatccagcacactccaaacaagtatagagcgatcctttaagcccacgtacacatacttgtcatccttggagaagcaagcacattggacccctctgcagtaagaactcgtgtagctcatctcgaatttccacttgcgtgcctgcaggtcccagagacacagcagggcatcctcagacccgctgaccaccagctgctccttgtggctgacctccacacaggcaactcggctcctgtgggtctccaagggaaacgctttggaagttgcacactcgtaaagaaagaggtccccattggtcatgctgtagaccacgcggtagtccgtcagaatggccacgctggagagggtctcgggcagctgagtgtaaaaggtgtatcttggcccatcgatgaccgggcaggggtccccggaggtgatgtccagcaccaggacgatgttgtcataggcgatggccaggcggtcctcgcacttgctcagggacatgcagttgattgctttccgggcctcgggagggggaatgcatatcacgtcctgcctggaattcagggggaacacaaggacgacccccgacacgaggcccgtaaataggagcttgcgctgctcagcaacctccagacacctgatctcactggaggtgtccagggaatcttgttcctcgccttctgccaagtcccaaatagtgactttgtttttgtccccaattttggggaagtagacgtagcttccattgtgggacactgcggtgaggccggtgcggtccagaaatggtgcaggcacccgggacctatgagcatcgctgagatcccagaccttgaaagatgaggactgtggggaagcagatgccaccaaagccccgccgcgggccagcaggctcacgggggccccgacgccttccaggatgtccagaagggtcccctgttctgacagactccacacctgaatgagcgcatcaagggaccccgtgatgatcaggttgttctcagtaccaaaaacagccgtctccaccatgtcttcatgttccagatccatggccatgaatcggcgaaagcccctcgagtccgccaagaatatccgcaccgatcttccaaagcctgcggcgaggagggactcatcttcagagaccaccaggaacctcacagcatctggaagcttctccagcaatctgtcccctttggaggaaaccaaagagatggagccattgctaaacccggtaacaagctttccttgcttctggactgagacggcacaggtaggtgtttcttctttgatgctggacatatgttgcttcccctgaagttttcccgtagctgagctccacagactgaccacaccatccctggacactgtcagcagtgtggcctgggaggccagcacggccatgcacatccaaggatcagaggcatctcccaggatatggaataccggctctgcagtttccagattccaagcattgatctttgagccagatgctgaatacacaactttgtgtgcctcatccacatgaaggttccagatctgaggttcagcgggattttttgagcctccatcccaaatggtaaatttctcctggccagagagtaagttccacaagtgcagcgtgtaatcctttgaagcagagttggcgagggtccctttggcaaatattttcacacacctcacctctcctgtgtgtccagttagcatgtggatcacatgctgctcttccatgtcccacacagccatgatgccatcctgggtgccaatcaccagcagcttctcctccacaccccatgccatggcggtgatgcctttgtgacagccgctgagagttgcccggaggggtcctcccgggggctggaggaatcctccgaggggcaccagcacagggtgtgcgcacaactggaaccagctctgggcctgttggcatagctgtcccaccagtgctggatgtgaggtggcgaagaaatggagtctggccagcagttctgtgtacaggaggctcctctccatgcctcggagctccacagcagggcggcagagctggagggcttcacggaccaggccaacctcaggggagtccaggtgaggggcacacaggtcaaagtcatccagcaggtcttcaatgcccccagagatgccccggcaggaaatccagctcatgctgcccagaacctcctgtttcagctcctccaggcggcccgagtgaagcaggtgatagggcaactccttcagcttccgcaggtttgcaaccgtatgtgagaaccacagaggctgcggggccacctttcggtccaagttcagtggtttccccacaagtggcagagtgatgagcttcttggtaccctggctccaggtccctgagaagaagtcggccaggacgccatgcctcttggctctctcggatcctgacaggtagcgctcacggaccacctcgaccagctgtctgtgggcaatggccaggagggtgaagccatccacgggccgccgggccaagtagtatcccagatcccgacgaagccgcacccacagcaggggcgggaagcgcagcagctccttgctgggcggggtccaatctcggtacacatcctgcaggacctcgtcgtccagggacaaaacatccttcagctccgcctccgagagaccgtgtcgggaagacacaatgtagcccagcacgtgggccacgaggagctgcccgtgtgtctgctccaggcgggtgcagagttggtgcgtggcttcctctgcggtggtggccagcgggacaggcacggtgaaagaggcccatttccgggcttcctcaaacgccagcctcagccgccctgggttcccacactctgggaggctggcccagagcaaatctgtgtgcaccgggctcagcgtcctccttgcagctgccagcaggagttggatcatctgctggccttggtttccggaaaggggcttcacctcccagtaggcctccgggtccaggagcacccgctgcaaggtgtccaaaacccccagtgcccccgagcaagctgagaggatgaggtgcaccctcggggggcagttgagaggcagccagggaaccctccgagcatggcggacagagtccaggtcatccatagcatccagcaggagcacgagagactcgaagtttctgcaagagacagtgtggaggagggtatggaaaaactggaccaccctggtgtgggcgtccagaacctgggcagggggcaagggcagcccataggccaggcacacctggaagcagatgctcttcagcaggccacgggcatctgagctcatttgtgacgtccccagcagccgcaggacggtcactgtcttgtgccccagcagccttggcatctgctcagccagcttgcacatcagggctgtctttccaatgcctgggggcccaaagagtaccaggggggtgtgctgcttgctgtcatcgtgcctgagctgctgcccaagccgggccaggagttcctggcgtccgcagaaggtctgaatgacctccgagctctgccaaaggtggtggcggatctcttggtagagccacgccaactcctgtccggccgtatccagctcacggaggcgtgtgaggacctggtgattggccctcaccacaaactgctcacccagctccttcaggtagcaggcgtgagtcttgttcttggggttcaccaagtcgcggctccacggcaggcggtgggtcttgaggacccctgggtgcatgtcagtgatgtgacttttgaggctgctgagaaggttctgggcatcagcgtccaggcagccatccgcgagccggtccaccatcctaagggcgcagtcttcaaggatgtgtttgtggaggtcttggatctctctaaggaagacggtggctccctgttcccggtcctctgagctcagcaggctccgctctatctcccactcaatgactgccaccatgtaagatgtgcctctttgcttctcctttgccttcagccatgattgtgaggcctccccagccatgtggaattgtgagtccattaaacctctttcctttgtaaattacccagcctcaagtatgcctttattagtggcatgagaacagactaatacggcccctgtgccaggaacctccctgggagacaagaagaaagagccagcgaggagaggaagatcctgagaccaagattgatcaggaacatggctgaactatcttggatcagtaaaacagcctttctcagagccgagggaccagaggttgactggtttggcatttgcaagaaatgcagactgttgcatttttgccaacaggggatggatattctgaacacgtggtcagtttcttgtgggtctccagaggggagtccctgcggcctcacctgaccggtggtagtgctgccactgctcctgggtgatgagccccagcctccgggcctcctgggctccagagcgtaggacagaagttaaggtggcctcctctggttcacaggcctccccagtacctggtgcctgcaggacgtaggtgggaggaaacgcattctcgtccctctggaagtatcgtgccaccagctccaggtcacttggcctggcagtcagatggtccctcaatacctcccactccttctcatcgatccgcgagggaatcagacaggggccgtactgatcaccgatgagggcaacaaaagctggccctatggatgttttccaacaccggtcaacctcctccaagcagagttctgtggtcaagtggtcagtggcttcaatgttccgaataccccacctcagatcaacgacctcaaacatcaagccgtgcctctggcagaaggtctggcacttcagggtaggcagtgctctgcagggcttccctctctgcatccatatcttggcatccgtgagcctggttggaatgccggctcctccatcgccctcctggaggacttaagcaagtggtctccctcccagggcatcggccgcatggtctggataccacagtttagctgcagcctgctgatctcactgaggccccagttctgggtcccagcatctctccagacctctcttagcacctcctccccaatcttctgatcttgaatttgcctccaccacaatttctgttccttctctcgttttcctgggtcccagcaggctccttggacccgaattcacttcagcgcctggccacgctcccttggttactgcctgcaacagctgatatgtttctacatgttattgtttgtctgtcccacgagaaagtgaattccatgagcccaaggatcttgtctggtaaggctggcgtgcctggcacatagtaggtgctcagtaaattatcatcacaacagcttcctccacaactgtttctctttctggacttctgtttgttgctgaagaagacagctgagcaggactgggcttccccagtaaggacagaggccctttgcagtgtcagcgttctggctgtcctgggggctccagcctctctttagcctttgctggtagttgaacgaccaatttagactcctctggggaaataggttagagaggacagtttcctggcctcggcgccacccggaagacaagcccctggctatcctagtaactttcgtcttaggtattttatgggtctctccttgcccaattctcccagcaact

SEQ ID NO: 8525 - RNA, 5822 nt, Homo sapiens
  source 1..5822: mol_type = other RNA
aaaagtaattgtggtttttgccattacttttttttttttttttttttggagacagagtctctgtcactcatgctggagtgcagtggtgcgatctcggctcactgcaacctccgcctcccgggttcaagccattctcctgcctcagcctcccaagtagctggaattacaggtgtacgtcaccacaccaggctaatttttgtatttttgagtagagacagagtttcaccatgttgaccaggctgctcttgaacacctggcctcaagtgatccacccgcctcagcctcccaaagtgctgggattacaggcgtgagccaccgaggcttttgccattattattattattatgagatggagtcttgctctgtcacccaggctggagtgcagtggcacaatctcagctcactgcaacctccgcctcccgggttcaagtgattctcctgactcagcctcctgagtaactgagattacaggcactcaccaccatgcctggctgatttttgtatttttagtagagaagggtttcaccatgttgtccaggctggtctcaaactcctgacctcaggtgatccacctgcctcggccttccaaagagctgggaccacaggtgtgagccactgtgcccagccagtttttgccattatttttaatatttttaatggcgaaaaccacagttactttttgcaccaaccttagtaatcttcaacaccttagaagctgctgcccaatacatccaagcatacatcttaaaattacagtttaaaatatttttaaatgaaatttgacactaacatttgcagaactaccaaaacctgccttggaaaactggtttggaaaatggatgaataagacagcagtagggtcttgttcagctcaaaagcctctgtttctaaggttgcttttattgagactctatcaggaattccacggaggggagaagggatagccaccttgaagatttagactatcctagcattaaagtaaaagcctgagaagactgagaagggcttttagaaggctgtgggcaaagaagaaagatccacttaagtggaatgaaaacagtttgactgttgaacttgcacaaggcagacagttcaaaagcaaagcagggagagatcagcagctctttctacttccaagagcctccagtttttaagattaaaaacccacatctttatcccaaaagtttgggagccaaggaatagagagggatgaactataacatgttgattgttttactgccagcgtgagtcctgaagtcagctcattaaccaaagacgcacatgccaaatgcactatagatataaattcaaccaatcgccaactttaaaagtcagaacatttttgcataaaagtctggatttctggctttgcttattacaactggaagcactgacagcagtgggcttgtttggccatggtgattctgggctacagtcaggctgctcatacccaccctagacacaatctctgccttccacatgtccagtctctgtctctccctgctgctcacccaggtgcatggaagtgtctagattagtcactagctcctgtgagcatttgagtgtggtgcctgtggaagagatggttgtgctctgcagactgaaattggagtgaggtctaacaggaatgggacagaaggctcactctcagagctcttgcaccttggacttgtgacctgaatcaaattataactacttccgcaaggctcagtttcctcatctgtaaaatagatacagaaactcctgccctccctaaagtatgagttgtgatgaggatcagatgacagcacctacagctttataaactgtgaggttctgtggtccacatcagtgatttgctgtatctcacattcatccgttcccccttcatctggtaccagaactccagtttgcatctcaggagtaatctcttctattctcagtcccagtggtggacattggatcagtctagccgattagagctctgcattctcccagatataataattggtttagggctaggcgtatgggccaattgggaccagtagagttgaggctaggactgttgggaaagagaagctctcttttctattgaaattggagacagcagcatattggccaccatgttgctaacctgggggtggcaagtctgagaatgaaaatgaaaaagaggaaagaataatggaaagatgagaagagacaaggtctgaagccataatctgaagccatgggtccagatatacaccagcaaacgtattctttttgctttaactagattaaatggggctaactcactggagccccatacccccacagggtttttttatttttatttttttacactatcaggcacacttgtgagcatttgtttgatttggtttcatttccctgggcactttctgactccaagtcctggggagctcctgcagctgcaactagctcctctctctgcctggatttgaccatccacattgccttcttgaagttcttaagagggtcctgcggtgaggcttttgctgaaaggcactggaaattctctcggatcagataaccatgcctggtgggggcaatgaagccactggtggttgggatgattctgtttaccacagcatggacaaactggactgtcagcagggtgccatccagcacactccaaacaagtatagagcgatcctttaagcccacgtacacatacttgtcatccttggagaagcaagcacattggacccctctgcagtaagaactcgtgtagctcatctcgaatttccacttgcgtgcctgcaggtcccagagacacagcagggcatcctcagacccgctgaccaccagctgctccttgtggctgacctccacacaggcaactcggctcctgtgggtctccaagggaaacgctttggaagttgcacactcgtaaagaaagaggtccccattggtcatgctgtagaccacgcggtagtccgtcagaatggccacgctggagagggtctcgggcagctgagtgtaaaaggtgtatcttggcccatcgatgaccgggcaggggtccccggaggtgatgtccagcaccaggacgatgttgtcataggcgatggccaggcggtcctcgcacttgctcagggacatgcagttgattgctttccgggcctcgggagggggaatgcatatcacgtcctgcctggaattcagggggaacacaaggacgacccccgacacgaggcccgtaaataggagcttgcgctgctcagcaacctccagacacctgatctcactggaggtgtccagggaatcttgttcctcgccttctgccaagtcccaaatagtgactttgtttttgtccccaattttggggaagtagacgtagcttccattgtgggacactgcggtgaggccggtgcggtccagaaatggtgcaggcacccgggacctatgagcatcgctgagatcccagaccttgaaagatgaggactgtggggaagcagatgccaccaaagccccgccgcgggccagcaggctcacgggggccccgacgccttccaggatgtccagaagggtcccctgttctgacagactccacacctgaatgagcgcatcaagggaccccgtgatgatcaggttgttctcagtaccaaaaacagccgtctccaccatgtcttcatgttccagatccatggccatgaatcggcgaaagcccctcgagtccgccaagaatatccgcaccgatcttccaaagcctgcggcgaggagggactcatcttcagagaccaccaggaacctcacagcatctggaagcttctccagcaatctgtcccctttggaggaaaccaaagagatggagccattgctaaacccggtaacaagctttccttgcttctggactgagacggcacaggtaggtgtttcttctttgatgctggacatatgttgcttcccctgaagttttcccgtagctgagctccacagactgaccacaccatccctggacactgtcagcagtgtggcctgggaggccagcacggccatgcacatccaaggatcagaggcatctcccaggatatggaataccggctctgcagtttccagattccaagcattgatctttgagccagatgctgaatacacaactttgtgtgcctcatccacatgaaggttccagatctgaggttcagcgggattttttgagcctccatcccaaatggtaaatttctcctggccagagagtaagttccacaagtgcagcgtgtaatcctttgaagcagagttggcgagggtccctttggcaaatattttcacacacctcacctctcctgtgtgtccagttagcatgtggatcacatgctgctcttccatgtcccacacagccatgatgccatcctgggtgccaatcaccagcagcttctcctccacaccccatgccatggcggtgatgcctttgtgacagccgctgagagttgcccggaggggtcctcccgggggctggaggaatcctccgaggggcaccagcacagggtgtgcgcacaactggaaccagctctgggcctgttggcatagctgtcccaccagtgctggatgtgaggtggcgaagaaatggagtctggccagcagttctgtgtacaggaggctcctctccatgcctcggagctccacagcagggcggcagagctggagggcttcacggaccaggccaacctcaggggagtccaggtgaggggcacacaggtcaaagtcatccagcaggtcttcaatgcccccagagatgccccggcaggaaatccagctcatgctgcccagaacctcctgtttcagctcctccaggcggcccgagtgaagcaggtgatagggcaactccttcagcttccgcaggtttgcaaccgtatgtgagaaccacagaggctgcggggccacctttcggtccaagttcagtggtttccccacaagtggcagagtgatgagcttcttggtaccctggctccaggtccctgagaagaagtcggccaggacgccatgcctcttggctctctcggatcctgacaggtagcgctcacggaccacctcgaccagctgtctgtgggcaatggccaggagggtgaagccatccacgggccgccgggccaagtagtatcccagatcccgacgaagccgcacccacagcaggggcgggaagcgcagcagctccttgctgggcggggtccaatctcggtacacatcctgcaggacctcgtcgtccagggacaaaacatccttcagctccgcctccgagagaccgtgtcgggaagacacaatgtagcccagcacgtgggccacgaggagctgcccgtgtgtctgctccaggcgggtgcagagttggtgcgtggcttcctctgcggtggtggccagcgggacaggcacggtgaaagaggcccatttccgggcttcctcaaacgccagcctcagccgccctgggttcccacactctgggaggctggcccagagcaaatctgtgtgcaccgggctcagcgtcctccttgcagctgccagcaggagttggatcatctgctggccttggtttccggaaaggggcttcacctcccagtaggcctccgggtccaggagcacccgctgcaaggtgtccaaaacccccagtgcccccgagcaagctgagaggatgaggtgcaccctcggggggcagttgagaggcagccagggaaccctccgagcatggcggacagagtccaggtcatccatagcatccagcaggagcacgagagactcgaagtttctggaagcagatgctcttcagcaggccacgggcatctgagctcatttgtgacgtccccagcagccgcaggacggtcactgtcttgtgcccc

SEQ ID NO: 8526 - RNA, 7456 nt, Homo sapiens
  source 1..7456: mol_type = other RNA
aaaagtaattgtggtttttgccattacttttttttttttttttttttggagacagagtctctgtcactcatgctggagtgcagtggtgcgatctcggctcactgcaacctccgcctcccgggttcaagccattctcctgcctcagcctcccaagtagctggaattacaggtgtacgtcaccacaccaggctaatttttgtatttttgagtagagacagagtttcaccatgttgaccaggctgctcttgaacacctggcctcaagtgatccacccgcctcagcctcccaaagtgctgggattacaggcgtgagccaccgaggcttttgccattattattattattatgagatggagtcttgctctgtcacccaggctggagtgcagtggcacaatctcagctcactgcaacctccgcctcccgggttcaagtgattctcctgactcagcctcctgagtaactgagattacaggcactcaccaccatgcctggctgatttttgtatttttagtagagaagggtttcaccatgttgtccaggctggtctcaaactcctgacctcaggtgatccacctgcctcggccttccaaagagctgggaccacaggtgtgagccactgtgcccagccagtttttgccattatttttaatatttttaatggcgaaaaccacagttactttttgcaccaaccttagtaatcttcaacaccttagaagctgctgcccaatacatccaagcatacatcttaaaattacagtttaaaatatttttaaatgaaatttgacactaacatttgcagaactaccaaaacctgccttggaaaactggtttggaaaatggatgaataagacagcagtagggtcttgttcagctcaaaagcctctgtttctaaggttgcttttattgagactctatcaggaattccacggaggggagaagggatagccaccttgaagatttagactatcctagcattaaagtaaaagcctgagaagactgagaagggcttttagaaggctgtgggcaaagaagaaagatccacttaagtggaatgaaaacagtttgactgttgaacttgcacaaggcagacagttcaaaagcaaagcagggagagatcagcagctctttctacttccaagagcctccagtttttaagattaaaaacccacatctttatcccaaaagtttgggagccaaggaatagagagggatgaactataacatgttgattgttttactgccagcgtgagtcctgaagtcagctcattaaccaaagacgcacatgccaaatgcactatagatataaattcaaccaatcgccaactttaaaagtcagaacatttttgcataaaagtctggatttctggctttgcttattacaactggaagcactgacagcagtgggcttgtttggccatggtgattctgggctacagtcaggctgctcatacccaccctagacacaatctctgccttccacatgtccagtctctgtctctccctgctgctcacccaggtgcatggaagtgtctagattagtcactagctcctgtgagcatttgagtgtggtgcctgtggaagagatggttgtgctctgcagactgaaattggagtgaggtctaacaggaatgggacagaaggctcactctcagagctcttgcaccttggacttgtgacctgaatcaaattataactacttccgcaaggctcagtttcctcatctgtaaaatagatacagaaactcctgccctccctaaagtatgagttgtgatgaggatcagatgacagcacctacagctttataaactgtgaggttctgtggtccacatcagtgatttgctgtatctcacattcatccgttcccccttcatctggtaccagaactccagtttgcatctcaggagtaatctcttctattctcagtcccagtggtggacattggatcagtctagccgattagagctctgcattctcccagatataataattggtttagggctaggcgtatgggccaattgggaccagtagagttgaggctaggactgttgggaaagagaagctctcttttctattgaaattggagacagcagcatattggccaccatgttgctaacctgggggtggcaagtctgagaatgaaaatgaaaaagaggaaagaataatggaaagatgagaagagacaaggtctgaagccataatctgaagccatgggtccagatatacaccagcaaacgtattctttttgctttaactagattaaatggggctaactcactggagccccatacccccacagggtttttttatttttatttttttacactatcaggcacacttgtgagcatttgtttgatttggtttcatttccctgggcactttctgactccaagtcctggggagctcctgcagctgcaactagctcctctctctgcctggatttgaccatccacattgccttcttgaagttcttaagagggtcctgcggtgaggcttttgctgaaaggcactggaaattctctcggatcagataaccatgcctggtgggggcaatgaagccactggtggttgggatgattctgtttaccacagcatggacaaactggactgtcagcagggtgccgtgtagctcatctcgaatttccacttgcgtgcctgcaggtcccagagacacagcagggcatcctcagacccgctgaccaccagctgctccttgtggctgacctccacacaggcaactcggctcctgtgggtctccaagggaaacgctttggaagttgcacactcgtaaagaaagaggtccccattggtcatgctgtagaccacgcggtagtccgtcagaatggccacgctggagagggtctcgggcagctgagtgtaaaaggtgtatcttggcccatcgatgaccgggcaggggtccccggaggtgatgtccagcaccaggacgatgttgtcataggcgatggccaggcggtcctcgcacttgctcagggacatgcagttgattgctttccgggcctcgggagggggaatgcatatcacgtcctgcctggaattcagggggaacacaaggacgacccccgacacgaggcccgtaaataggagcttgcgctgctcagcaacctccagacacctgatctcactggaggtgtccagggaatcttgttcctcgccttctgccaagtcccaaatagtgactttgtttttgtccccaattttggggaagtagacgtagcttccattgtgggacactgcggtgaggccggtgcggtccagaaatggtgcaggcacccgggacctatgagcatcgctgagatcccagaccttgaaagatgaggactgtggggaagcagatgccaccaaagccccgccgcgggccagcaggctcacgggggccccgacgccttccaggatgtccagaagggtcccctgttctgacagactccacacctgaatgagcgcatcaagggaccccgtgatgatcaggttgttctcagtaccaaaaacagccgtctccaccatgtcttcatgttccagatccatggccatgaatcggcgaaagcccctcgagtccgccaagaatatccgcaccgatcttccaaagcctgcggcgaggagggactcatcttcagagaccaccaggaacctcacagcatctggaagcttctccagcaatctgtcccctttggaggaaaccaaagagatggagccattgctaaacccggtaacaagctttccttgcttctggactgagacggcacaggtaggtgtttcttctttgatgctggacatatgttgcttcccctgaagttttcccgtagctgagctccacagactgaccacaccatccctggacactgtcagcagtgtggcctgggaggccagcacggccatgcacatccaaggatcagaggcatctcccaggatatggaataccggctctgcagtttccagattccaagcattgatctttgagccagatgctgaatacacaactttgtgtgcctcatccacatgaaggttccagatctgaggttcagcgggattttttgagcctccatcccaaatggtaaatttctcctggccagagagtaagttccacaagtgcagcgtgtaatcctttgaagcagagttggcgagggtccctttggcaaatattttcacacacctcacctctcctgtgtgtccagttagcatgtggatcacatgctgctcttccatgtcccacacagccatgatgccatcctgggtgccaatcaccagcagcttctcctccacaccccatgccatggcggtgatgcctttgtgacagccgctgagagttgcccggaggggtcctcccgggggctggaggaatcctccgaggggcaccagcacagggtgtgcgcacaactggaaccagctctgggcctgttggcatagctgtcccaccagtgctggatgtgaggtggcgaagaaatggagtctggccagcagttctgtgtacaggaggctcctctccatgcctcggagctccacagcagggcggcagagctggagggcttcacggaccaggccaacctcaggggagtccaggtgaggggcacacaggtcaaagtcatccagcaggtcttcaatgcccccagagatgccccggcaggaaatccagctcatgctgcccagaacctcctgtttcagctcctccaggcggcccgagtgaagcaggtgatagggcaactccttcagcttccgcaggtttgcaaccgtatgtgagaaccacagaggctgcggggccacctttcggtccaagttcagtggtttccccacaagtggcagagtgatgagcttcttggtaccctggctccaggtccctgagaagaagtcggccaggacgccatgcctcttggctctctcggatcctgacaggtagcgctcacggaccacctcgaccagctgtctgtgggcaatggccaggagggtgaagccatccacgggccgccgggccaagtagtatcccagatcccgacgaagccgcacccacagcaggggcgggaagcgcagcagctccttgctgggcggggtccaatctcggtacacatcctgcaggacctcgtcgtccagggacaaaacatccttcagctccgcctccgagagaccgtgtcgggaagacacaatgtagcccagcacgtgggccacgaggagctgcccgtgtgtctgctccaggcgggtgcagagttggtgcgtggcttcctctgcggtggtggccagcgggacaggcacggtgaaagaggcccatttccgggcttcctcaaacgccagcctcagccgccctgggttcccacactctgggaggctggcccagagcaaatctgtgtgcaccgggctcagcgtcctccttgcagctgccagcaggagttggatcatctgctggccttggtttccggaaaggggcttcacctcccagtaggcctccgggtccaggagcacccgctgcaaggtgtccaaaacccccagtgcccccgagcaagctgagaggatgaggtgcaccctcggggggcagttgagaggcagccagggaaccctccgagcatggcggacagagtccaggtcatccatagcatccagcaggagcacgagagactcgaagtttctgcaagagacagtgtggaggagggtatggaaaaactggaccaccctggtgtgggcgtccagaacctgggcagggggcaagggcagcccataggccaggcacacctggaagcagatgctcttcagcaggccacgggcatctgagctcatttgtgacgtccccagcagccgcaggacggtcactgtcttgtgccccagcagccttggcatctgctcagccagcttgcacatcagggctgtctttccaatgcctgggggcccaaagagtaccaggggggtgtgctgcttgctgtcatcgtgcctgagctgctgcccaagccgggccaggagttcctggcgtccgcagaaggtctgaatgacctccgagctctgccaaaggtggtggcggatctcttggtagagccacgccaactcctgtccggccgtatccagctcacggaggcgtgtgaggacctggtgattggccctcaccacaaactgctcacccagctccttcaggtagcaggcgtgagtcttgttcttggggttcaccaagtcgcggctccacggcaggcggtgggtcttgaggacccctgggtgcatgtcagtgatgtgacttttgaggctgctgagaaggttctgggcatcagcgtccaggcagccatccgcgagccggtccaccatcctaagggcgcagtcttcaaggatgtgtttgtggaggtcttggatctctctaaggaagacggtggctccctgttcccggtcctctgagctcagcaggctccgctctatctcccactcaatgactgaccggtggtagtgctgccactgctcctgggtgatgagccccagcctccgggcctcctgggctccagagcgtaggacagaagttaaggtggcctcctctggttcacaggcctccccagtacctggtgcctgcaggacgtaggtgggaggaaacgcattctcgtccctctggaagtatcgtgccaccagctccaggtcacttggcctggcagtcagatggtccctcaatacctcccactccttctcatcgatccgcgagggaatcagacaggggccgtactgatcaccgatgagggcaacaaaagctggccctatggatgttttccaacaccggtcaacctcctccaagcagagttctgtggtcaagtggtcagtggcttcaatgttccgaataccccacctcagatcaacgacctcaaacatcaagccgtgcctctggcagaaggtctggcacttcagggtaggcagtgctctgcagggcttccctctctgcatccatatcttggcatccgtgagcctggttggaatgccggctcctccatcgccctcctggaggacttaagcaagtggtctccctcccagggcatcggccgcatggtcaacagctgatatgtttctacatgttattgtttgtctgtcccacgagaaagtgaattccatgagcccaaggatcttgtctggtaaggctggcgtgcctggcacatagtaggtgctcagtaaattatcatcacaacagcttcctccacaactgtttctctttctggacttctgtttgttgctgaagaagacagctgagcaggactgggcttccccagtaaggacagaggccctttgcagtgtcagcgttctggctgtcctgggggctccagcctctctttagcctttgctggtagttgaacgaccaatttagactcctctggggaaataggttagagaggacagtttcctggcctcggcgccacccggaagacaagcccctggctatcctagtaactttcgtcttaggtattttatgggtctctccttgcccaattctcccagcaact

SEQ ID NO: 8527 - RNA, 7511 nt, Homo sapiens
  source 1..7511: mol_type = other RNA
aaaagtaattgtggtttttgccattacttttttttttttttttttttggagacagagtctctgtcactcatgctggagtgcagtggtgcgatctcggctcactgcaacctccgcctcccgggttcaagccattctcctgcctcagcctcccaagtagctggaattacaggtgtacgtcaccacaccaggctaatttttgtatttttgagtagagacagagtttcaccatgttgaccaggctgctcttgaacacctggcctcaagtgatccacccgcctcagcctcccaaagtgctgggattacaggcgtgagccaccgaggcttttgccattattattattattatgagatggagtcttgctctgtcacccaggctggagtgcagtggcacaatctcagctcactgcaacctccgcctcccgggttcaagtgattctcctgactcagcctcctgagtaactgagattacaggcactcaccaccatgcctggctgatttttgtatttttagtagagaagggtttcaccatgttgtccaggctggtctcaaactcctgacctcaggtgatccacctgcctcggccttccaaagagctgggaccacaggtgtgagccactgtgcccagccagtttttgccattatttttaatatttttaatggcgaaaaccacagttactttttgcaccaaccttagtaatcttcaacaccttagaagctgctgcccaatacatccaagcatacatcttaaaattacagtttaaaatatttttaaatgaaatttgacactaacatttgcagaactaccaaaacctgccttggaaaactggtttggaaaatggatgaataagacagcagtagggtcttgttcagctcaaaagcctctgtttctaaggttgcttttattgagactctatcaggaattccacggaggggagaagggatagccaccttgaagatttagactatcctagcattaaagtaaaagcctgagaagactgagaagggcttttagaaggctgtgggcaaagaagaaagatccacttaagtggaatgaaaacagtttgactgttgaacttgcacaaggcagacagttcaaaagcaaagcagggagagatcagcagctctttctacttccaagagcctccagtttttaagattaaaaacccacatctttatcccaaaagtttgggagccaaggaatagagagggatgaactataacatgttgattgttttactgccagcgtgagtcctgaagtcagctcattaaccaaagacgcacatgccaaatgcactatagatataaattcaaccaatcgccaactttaaaagtcagaacatttttgcataaaagtctggatttctggctttgcttattacaactggaagcactgacagcagtgggcttgtttggccatggtgattctgggctacagtcaggctgctcatacccaccctagacacaatctctgccttccacatgtccagtctctgtctctccctgctgctcacccaggtgcatggaagtgtctagattagtcactagctcctgtgagcatttgagtgtggtgcctgtggaagagatggttgtgctctgcagactgaaattggagtgaggtctaacaggaatgggacagaaggctcactctcagagctcttgcaccttggacttgtgacctgaatcaaattataactacttccgcaaggctcagtttcctcatctgtaaaatagatacagaaactcctgccctccctaaagtatgagttgtgatgaggatcagatgacagcacctacagctttataaactgtgaggttctgtggtccacatcagtgatttgctgtatctcacattcatccgttcccccttcatctggtaccagaactccagtttgcatctcaggagtaatctcttctattctcagtcccagtggtggacattggatcagtctagccgattagagctctgcattctcccagatataataattggtttagggctaggcgtatgggccaattgggaccagtagagttgaggctaggactgttgggaaagagaagctctcttttctattgaaattggagacagcagcatattggccaccatgttgctaacctgggggtggcaagtctgagaatgaaaatgaaaaagaggaaagaataatggaaagatgagaagagacaaggtctgaagccataatctgaagccatgggtccagatatacaccagcaaacgtattctttttgctttaactagattaaatggggctaactcactggagccccatacccccacagggtttttttatttttatttttttacactatcaggcacacttgtgagcatttgtttgatttggtttcatttccctgggcactttctgactccaagtcctggggagctcctgcagctgcaactagctcctctctctgcctggatttgaccatccacattgccttcttgaagttcttaagagggtcctgcggtgaggcttttgctgaaaggcactggaaattctctcggatcagataaccatgcctggtgggggcaatgaagccactggtggttgggatgattctgtttaccacagcatggacaaactggactgtcagcagggtgccgtgtagctcatctcgaatttccacttgcgtgcctgcaggtcccagagacacagcagggcatcctcagacccgctgaccaccagctgctccttgtggctgacctccacacaggcaactcggctcctgtgggtctccaagggaaacgctttggaagttgcacactcgtaaagaaagaggtccccattggtcatgctgtagaccacgcggtagtccgtcagaatggccacgctggagagggtctcgggcagctgagtgtaaaaggtgtatcttggcccatcgatgaccgggcaggggtccccggaggtgatgtccagcaccaggacgatgttgtcataggcgatggccaggcggtcctcgcacttgctcagggacatgcagttgattgctttccgggcctcgggagggggaatgcatatcacgtcctgcctggaattcagggggaacacaaggacgacccccgacacgaggcccgtaaataggagcttgcgctgctcagcaacctccagacacctgatctcactggaggtgtccagggaatcttgttcctcgccttctgccaagtcccaaatagtgactttgtttttgtccccaattttggggaagtagacgtagcttccattgtgggacactgcggtgaggccggtgcggtccagaaatggtgcaggcacccgggacctatgagcatcgctgagatcccagaccttgaaagatgaggactgtggggaagcagatgccaccaaagccccgccgcgggccagcaggctcacgggggccccgacgccttccaggatgtccagaagggtcccctgttctgacagactccacacctgaatgagcgcatcaagggaccccgtgatgatcaggttgttctcagtaccaaaaacagccgtctccaccatgtcttcatgttccagatccatggccatgaatcggcgaaagcccctcgagtccgccaagaatatccgcaccgatcttccaaagcctgcggcgaggagggactcatcttcagagaccaccaggaacctcacagcatctggaagcttctccagcaatctgtcccctttggaggaaaccaaagagatggagccattgctaaacccggtaacaagctttccttgcttctggactgagacggcacaggtaggtgtttcttctttgatgctggacatatgttgcttcccctgaagttttcccgtagctgagctccacagactgaccacaccatccctggacactgtcagcagtgtggcctgggaggccagcacggccatgcacatccaaggatcagaggcatctcccaggatatggaataccggctctgcagtttccagattccaagcattgatctttgagccagatgctgaatacacaactttgtgtgcctcatccacatgaaggttccagatctgaggttcagcgggattttttgagcctccatcccaaatggtaaatttctcctggccagagagtaagttccacaagtgcagcgtgtaatcctttgaagcagagttggcgagggtccctttggcaaatattttcacacacctcacctctcctgtgtgtccagttagcatgtggatcacatgctgctcttccatgtcccacacagccatgatgccatcctgggtgccaatcaccagcagcttctcctccacaccccatgccatggcggtgatgcctttgtgacagccgctgagagttgcccggaggggtcctcccgggggctggaggaatcctccgaggggcaccagcacagggtgtgcgcacaactggaaccagctctgggcctgttggcatagctgtcccaccagtgctggatgtgaggtggcgaagaaatggagtctggccagcagttctgtgtacaggaggctcctctccatgcctcggagctccacagcagggcggcagagctggagggcttcacggaccaggccaacctcaggggagtccaggtgaggggcacacaggtcaaagtcatccagcaggtcttcaatgcccccagagatgccccggcaggaaatccagctcatgctgcccagaacctcctgtttcagctcctccaggcggcccgagtgaagcaggtgatagggcaactccttcagcttccgcaggtttgcaaccgtatgtgagaaccacagaggctgcggggccacctttcggtccaagttcagtggtttccccacaagtggcagagtgatgagcttcttggtaccctggctccaggtccctgagaagaagtcggccaggacgccatgcctcttggctctctcggatcctgacaggtagcgctcacggaccacctcgaccagctgtctgtgggcaatggccaggagggtgaagccatccacgggccgccgggccaagtagtatcccagatcccgacgaagccgcacccacagcaggggcgggaagcgcagcagctccttgctgggcggggtccaatctcggtacacatcctgcaggacctcgtcgtccagggacaaaacatccttcagctccgcctccgagagaccgtgtcgggaagacacaatgtagcccagcacgtgggccacgaggagctgcccgtgtgtctgctccaggcgggtgcagagttggtgcgtggcttcctctgcggtggtggccagcgggacaggcacggtgaaagaggcccatttccgggcttcctcaaacgccagcctcagccgccctgggttcccacactctgggaggctggcccagagcaaatctgtgtgcaccgggctcagcgtcctccttgcagctgccagcaggagttggatcatctgctggccttggtttccggaaaggggcttcacctcccagtaggcctccgggtccaggagcacccgctgcaaggtgtccaaaacccccagtgcccccgagcaagctgagaggatgaggtgcaccctcggggggcagttgagaggcagccagggaaccctccgagcatggcggacagagtccaggtcatccatagcatccagcaggagcacgagagactcgaagtttctgcaagagacagtgtggaggagggtatggaaaaactggaccaccctggtgtgggcgtccagaacctgggcagggggcaagggcagcccataggccaggcacacctggaagcagatgctcttcagcaggccacgggcatctgagctcatttgtgacgtccccagcagccgcaggacggtcactgtcttgtgccccagcagccttggcatctgctcagccagcttgcacatcagggctgtctttccaatgcctgggggcccaaagagtaccaggggggtgtgctgcttgctgtcatcgtgcctgagctgctgcccaagccgggccaggagttcctggcgtccgcagaaggtctgaatgacctccgagctctgccaaaggtggtggcggatctcttggtagagccacgccaactcctgtccggccgtatccagctcacggaggcgtgtgaggacctggtgattggccctcaccacaaactgctcacccagctccttcaggtagcaggcgtgagtcttgttcttggggttcaccaagtcgcggctccacggcaggcggtgggtcttgaggacccctgggtgcatgtcagtgatgtgacttttgaggctgctgagaaggttctgggcatcagcgtccaggcagccatccgcgagccggtccaccatcctaagggcgcagtcttcaaggatgtgtttgtggaggtcttggatctctctaaggaagacggtggctccctgttcccggtcctctgagctcagcaggctccgctctatctcccactcaatgactgaccggtggtagtgctgccactgctcctgggtgatgagccccagcctccgggcctcctgggctccagagcgtaggacagaagttaaggtggcctcctctggttcacaggcctccccagtacctggtgcctgcaggacgtaggtgggaggaaacgcattctcgtccctctggaagtatcgtgccaccagctccaggtcacttggcctggcagtcagatggtccctcaatacctcccactccttctcatcgatccgcgagggaatcagacaggggccgtactgatcaccgatgagggcaacaaaagctggccctatggatgttttccaacaccggtcaacctcctccaagcagagttctgtggtcaagtggtcagtggcttcaatgttccgaataccccacctcagatcaacgacctcaaacatcaagccgtgcctctggcagaaggtctggcacttcagggtaggcagtgctctgcagggcttccctctctgcatccatatcttggcatccgtgagcctggttggaatgccggctcctccatcgccctcctggaggacttaagcaagtggtctccctcccagggcatcggccgcatggtctggataccacagtttagctgcagcctgctgatctcactgaggccccagttctgggtcccagcatctctccagacctctcttagcacctcctccccaatcttctgatcttgaatttgcctccaccacaatttctgttccttctctcgttttcctgggtcccagcaggctccttggacccgaattcacttcagcgcctggccacgctcccttggttactgcctgcaacagctgatatgtttctacatgttattgtttgtctgtcccacgagaaagtgaattccatgagcccaaggatcttgtctggtaaggctggcgtgcctggcacatagtaggtgctcagtaaattatcatcacaacagcttcctccacaactgtttctctttctggacttctgtttgttgctgaagaagacagctgagcaggactgggcttccccagtaaggacagaggccctttgcagtgtcagcgttctggctgtcctgggggctccagcctctcttt

SEQ ID NO: 8528 - RNA, 73 nt, Homo sapiens
  source 1..73: mol_type = other RNA
aaaagtaattgtggtttttgccattgaaagtaatggcaaaaaccacagtttcttttgcaccaacctaataaaa

SEQ ID NO: 8529 - RNA, 8608 nt, Homo sapiens
  source 1..8608: mol_type = other RNA
aaaagtaattgtggtttttgcctgcacttttaatggtaaaaaccgcaattactttttcagcaacctaataattacaattctaagtaatggagatacatatcttttataggcttcaatgagcaatacattagcataatgttttatttcatactgactttgaatattccttgtcaaaaatgcacttatactttggagttactatgtatgtttaggttactgtgttgtcatcagaaggctggagttatcatagcagagctttaatgacaaaatattatgagccttgtaaatagttttaaaaattgtccactaatatctatttgtcttgcaaaatttgcaattttactagtaattttcatcacttgctctttctacctctaatgtttctcagtctcctccattagatcttactgacttatcacatataaacaccttcctcagaaacagtccaataaaaattaaagaccaagaggtagaatctactggagccatcatgaattccagttctttttgttgttattgatttttcttttttttttttaaaaggcacacccttgacttttttttattgttaaaataaccagattctaatttcaggcagcaaaatcagttactgcaaaaagtcaataatcaaaaatcaatgtataattggttttcatcacctatagaattagtgaggtttatacccctcaagtgtttagtgattctattcagtcaacctaaaaaaaattgcctcttttctacttaaataaataatttatttatttattttgagacagagtttcgctctgttgcccaggccggagtgcagtggcacaatctcagctcactgcaacctccgcctcccaggtcaagcgattgattctcatgcctcagcctcccaaatagctgggattataggtgcccgccaccatgctcagctaatttttgtatttttagtagagatggcgtttcaccatgttggccaggctggtcttgaactgacctcaagtgatccgcccaccttggcctcccaaagtgtggggattactagtgtgagccaccacgcctggcctgcctgttttcattattacctgcctgttctcagtatgcaacatggcagtactattgacagtgaggtgctttggcatatcagataacttttccagttggtcaaggatcccttttctcttttcctcatttctgaactgcagaacaggaagtactaaagaagtggctcaggacaatgttgtcacatcaggagtggcagaggtgtttactaggattatgatcctttcagctgtgtgtcttagaaggatctcctgaagccctgggtttgatatagaaaccataagaaaaagacttggggcagttctatatctggctcttctcccacttctcccataaaagattaagaaaaactgatgggatgatttcagatgtttcattgccaccaaactacagccatgagttttttttctttaagtgatcttatgaggccagtaaaggcctctgtcttgattaatgatgatcatcctataatatctggatatggtggcttgacatgagttttcaacaaagaaaattagtctctgaaagacatttctcatctgaaactctcaatatattaaaatgcatttaaaagttacttctgggaaacatactaaataggccaatcagttaatcattagctaattgtcaaaccctataaaatcatggtataatgtcaccctgacataaagcaacatcaaaattagtgcatcatctataaagtgaagtattattttctcccaagtgacaaattctattgccaaaaaataccactgtacttctaataagtgacactcattttaatagaccctacaaaaatacaatattttcaatgtccccataaaacagttaacttacaaatattattctcagagctctggtgacatcattcagtgatactattgtgaaaatcctcatacaatacttgaaacactagcatgtaaagtaaattcattatataacaaaagaactatgtaaaattatgaaagataatgcatgcaaccaactccgggaaattatcctggaaattcaaattaatattgtaattaaattaatgactaatatgaaagataagtattttaaaggattataaaataaattttgatcatttatgcaggaaaatagtttcaatggaaaagtaaataattctacattaaccatgcttgtctttctcttcagtgaaaaagcattcaggattttacataccttgaaactgtttttggaaaaaaagtattttatctatttctgcccagaaaaacagccattgaaattaatgatacaggtagaccacagctctgagaaattatatttgaagtttcatatttaaataccaaggatttaaaatcacctaccataactttctaacagcagtctttcgtaatgataaattttatcaatttccaaaattcgttttaaataatttaaaaagcagcaaattagattaagcaacacacaaataaattccacatttacaagtaaagaaatcacaggggctacagtttataatcaacatgaacttgaaagaaataaagcaatacctttcctgccacccatcatccactgcttaaatttgtggtgaaaaagacttaactacaatgacctttagtctgtttctaaactctgcatgtattgtaattagctaaaggcattgaacaaattagttcatcctatttttatttgggtcccagagataaatggctaatttatgaaatatttcactctgtgtcatgagaatttagcaaatgaatatggaaccaaatataaacactttataccatatgtacagttactttcataaggcattatcatgtaatttttattgaaaaagattcaatatagtaaagtcttattttaagatatattttttctctatctgagatgtttagtttatgaaaatattgtttttctctatattctttttgtatatatgccaacatataccttgtgctagaaatattttatgggaattacaattctttatatttgtattttctatataaaggcatatacaactttgaggcagtgtttctgatggagagcagaattcataaagagcttgtgtgtgcttccgtgctccgaaattatatgaaatccattttgagaagaaacttatttgattaaaaacaaaaacaaaaacagaaacaaaactgcaccaatgcacagccagaggctgacaattaaaactaatacataaccacatgaacatcatatttatagagttaacattttttaaggatggtcagtgctaacatatagtattatacatttggcactaatgtttgccattggtccagcaattggcaaaatttgtttctatgtataaatttatttttgaacattaggtctggctagacgtatcttcactatttataaaaaatatttagacagtaagctcacgttgaataactaggtctactgtgttctggaaactcttcagtagtaatacagctttttcatgttccatatgtacaaaactgtgtccatttgcctgaaggatcttatcaccaggctgcagtaggtttgatgctggcccatcaggctgaaccctagtaacaaagatacccttgtcagaaggtttgaatggatttccttgtccactaattccaccactgatactaaatccaaggccaggattcttttctattctcacacaaaactgctctggatatccatccatactcctttgccctttagtttgaattaagcaccgtccaggctgaggtccccgggtggcctgtgaagaggggatctgaataggcaatggtgactgaaattgctggatggtcactttgtttatatttccttcatacggctgctgctcccggctgcgatgctgaaggctttgggaccccatcaacgtctggatgtggctgcctgccctgtctaaccgtctagcttctatatgtctaagcagctgttgtctccagtctgcaggcattttaccacagctctcctctcccttcacaggagtaggcctcgtctttaaatcactgttatctgatggcttgtcaccatagttacccaagttatagtcagatggtattttttccaaaagagctgccatagtaggcctagctgaaactggcctggtttgggaggcaccgtaactctctgtactgtagcttctcgcagacaatggcctcctttgggtaaggtttttaaccggaaaacttcccgcctgagctttcacttcttgatatgaagggtgttcatcttcatacctgccattccttttcaggaactgggactcagtcactgtaacgctgctttggcgatccagccctcccctatatgggggtctgccgtacctatcagttgggggcagctcatgaggctcattgacccttctaaacatggccatttctgtggcgctcaccagggagtcggcccttctcaggaagcccgccctggccccttggcttgcgaactgggcattcaccacagcatcctcattcacagatggctgagaaaatgaaaacatttgctccatcggtgggtatcctctgtaagctctaggactaatcaaatccttggcgatgtttttgctggcctgttgcacgtactcgggattgtgttgaaaagggggtggtatcctcttttcggctttcacttccactgatccttgaggattgaagctttggtcaaactgatagactttttttgtcatagaagctttttgttgttgtggccccttactacttccgtaggtgagcatctcatcatccagcattgggactgactggcttcgagacatactggacataccatgctctggtcccagcatcttatccggtcgttcgtggcttcctaagtgatcactcccagaagcatagttttctaatggtatgttatacaccttatatgtaccaatgtcaatctcatcgatactctgtgactttttgaatttattagacttgatatctttcattaggggggaaagcctctctgtgcttttgctaattgaaataacacctttagaagattccgggcggcagtggatttgagaaaagacattactaagactcctgttgggattggaatcatgatactcccatggtacgcctggagaaaaaggactaggtatttcagtagattcctttatatgttctttcctttcaggcaatgggctggtagtgggggttgtctctaatttggaaggaaaagcggtcctgtcttcaaacggactaggggttctggtccaattctgccaaggattggaaggaggcacttctgtttctggtgtgtgtctgtgtgtagactgctcgagttccaggggaacaccaacaatcctgtcttgcctgatcaaaggcctgcgtccatgcgaagatgtgcttctagatttcgaacttaagagaggattactgttggcattctcggctgtggtttcctcagcaacaaaccctgtgttgtcataatgcgagccatcagtccagttgtcagtgaaagtatcactcatgggcagccggtcaggacgctgtggtatattgcctgggggaacagcctcccgctggctgagtaatggctttgaatcaagaggctgtgggaaagatggtgcaatcctgttaccccacaaagaattatgtactgcatctttagctgttgtctgcaaggaccccactttaacccgggtattagaggatcctgaggaagcctgggaaggcgagtagtctgagtaagtgccttttttgtccttccctagcagaacaagtttgggtgggtacagaggggtctcagctaatgaagggtgaagttccccaatcctcatttcattagctggatgaacaaaagaatcctccactgtaatctcctttggggctaccggccacttgtgttcatatttttctttcacagtttgctccgtgttagcagttggatttgaattctcaacacgcactccatggcttggcttacccaccaaattttgaacagattttaccatattctttaaatcctctgggtaaggagttggatatcgttttaggtttatttcaacctgtctgccacttagagagggaagagtggtggattgtgctgcaactggcaatggagtacacatgctcctttcctgctggaggccacttatacaaccccatgccagctgtgggtcattctgggggacgggcatatcttggatctgctgatcacacctggcccatggtgtgcagcaatcgccagacagtctggcaggttggagagtaatcccacgctggcccctttcccagggggcttggcaggagagatccttaactttcccagcattttcgtcatcttcttttttgtcttcaaattcaaaggcaacagtcatgcgttgttgtctctgctcttcccacagtgtagggttaaagctgtcactgtctgactggaaatcttcatcaccacgaggctgctggggaaacatgtagttagtcaatactctttgctttgtttctggatgggcttctgtttgtaaagggataagggctttggactgattgtcagaaagccacaaagctgcaagctctttaagtttggtaaatgagaatggtaaattcttcaatctgttgtcactcaaatttaggactcttagtttctgcatctgtccaatctcttcaggaagaaattctaatttgttggagcgtagagacatgactgttacattcttacaacttccaatttctctgggtaattctggaaggaaattctcatcaactgctaatgtccgaagactatgaaggtagccaatagtagaaggtagtgactccagttcattacagctacagtcaaattcttctaataaagataaatttccaattgtattgggtagcattgtaagttgattgtcatctacttttagagttgttagttttttcaaaagtcctatagaatcaggcaattgttgcaacatattggatgacaataagaggtcctcaagggcttcacatccagaaatgtccatgtcaactgtttctattctgttttttgacatatccaggtataccaacatctttaacttccctatagacccaggtaacacttgtaatgcattattatccatccataactccctcaaattttgtatttgatccagaacttcaggcagctcaccgaattcattattgcctaggtcaagtctttccaactgggccagtttgtgcattgactttggtagagttttcaagtgattttctcttaactccaagatccgcaatttgacaagtcttccaaaattggctggaagaaattcaagaaaggcgtcattcaggtagagctgggtcaggtttaggagctgtgtgaagccatcaggtagtttagaaatgggattgacactggcttcaataattgttaaacacttacagcactttatgttttctggaaattcttgtacaccatttttactgatgtcgagttctttaagattaactaaactagcaatagtggttggcagatttgaaaggtcgttatcaggaatacttagttttcgtagagcttgacagttgaacaattgcttgggtagttcttcaatttgattggcatctagataaagctcctctaatgttcgttcgaagttaaagacctcctttggcacctgctgaagactgcagtgggagtaatctaaaactgagatgatttcttcttcacctcggaaacatcggcatggcaccagacggccgatgattttccgtttggtggtcatctccaggcactgcattgctagttattcctgtctctgcagacttctaggttgtgaccactttgacttgcattttttttcatgtagcgggctcactcctcttcaggcctcttccgaagtgctgcacgaacctctttacaaggacttctctggtattgcgggggattccttccccttattaggttctccatcatcgccggcgggagaaactgcccatgaggtttcggagagcgtagtcgtgcagctgccaagggttattccttaagtgttcaggggtccgcagtggagtgggcgccagggtcttcggaggagaagaggagggaaggagtagaaggtaggaagaacaggagatagaggggaatccaggaaggtgccacgttagaccatgatgccagtgcccttcaggtggacggctggagaggttcccgcgggaagcggctgaggggaagcccgaagcgccggcgggggaggcaggagcgcgtccactccccagcctcagcctgcccagcgcgccgcgctagcgaccgcagcagcagcggcggcggcggcggcggtggcggaggcgcagctccctccccgcccccagaaggctccacagacaataaatcctgggcggagaagagacaagcaggaaaggcgaatcctgcacccaactccgtaacaacccctgcccgttgccgcgcctgtgcagggcgaggatccccaggggccagggcgcagcgggcgtctcggaggggctgagcgctccgcaactgcaggaggcggtggcggtggcccgagtgggcggctgcaggtcccgccggcgagaacccgctgcactggggctgggtgtccgtggcttcaagcccggtgttcacccggagtagggtcctcctcggtgcagtggctcggcgcacaggtgccaggattggc

SEQ ID NO: 8530 - RNA, 8711 nt, Homo sapiens
  source 1..8711: mol_type = other RNA
aaaagtaattgtggtttttgcctgcacttttaatggtaaaaaccgcaattactttttcagcaacctaataattacaattctaagtaatggagatacatatcttttataggcttcaatgagcaatacattagcataatgttttatttcatactgactttgaatattccttgtcaaaaatgcacttatactttggagttactatgtatgtttaggttactgtgttgtcatcagaaggctggagttatcatagcagagctttaatgacaaaatattatgagccttgtaaatagttttaaaaattgtccactaatatctatttgtcttgcaaaatttgcaattttactagtaattttcatcacttgctctttctacctctaatgtttctcagtctcctccattagatcttactgacttatcacatataaacaccttcctcagaaacagtccaataaaaattaaagaccaagaggtagaatctactggagccatcatgaattccagttctttttgttgttattgatttttcttttttttttttaaaaggcacacccttgacttttttttattgttaaaataaccagattctaatttcaggcagcaaaatcagttactgcaaaaagtcaataatcaaaaatcaatgtataattggttttcatcacctatagaattagtgaggtttatacccctcaagtgtttagtgattctattcagtcaacctaaaaaaaattgcctcttttctacttaaataaataatttatttatttattttgagacagagtttcgctctgttgcccaggccggagtgcagtggcacaatctcagctcactgcaacctccgcctcccaggtcaagcgattgattctcatgcctcagcctcccaaatagctgggattataggtgcccgccaccatgctcagctaatttttgtatttttagtagagatggcgtttcaccatgttggccaggctggtcttgaactgacctcaagtgatccgcccaccttggcctcccaaagtgtggggattactagtgtgagccaccacgcctggcctgcctgttttcattattacctgcctgttctcagtatgcaacatggcagtactattgacagtgaggtgctttggcatatcagataacttttccagttggtcaaggatcccttttctcttttcctcatttctgaactgcagaacaggaagtactaaagaagtggctcaggacaatgttgtcacatcaggagtggcagaggtgtttactaggattatgatcctttcagctgtgtgtcttagaaggatctcctgaagccctgggtttgatatagaaaccataagaaaaagacttggggcagttctatatctggctcttctcccacttctcccataaaagattaagaaaaactgatgggatgatttcagatgtttcattgccaccaaactacagccatgagttttttttctttaagtgatcttatgaggccagtaaaggcctctgtcttgattaatgatgatcatcctataatatctggatatggtggcttgacatgagttttcaacaaagaaaattagtctctgaaagacatttctcatctgaaactctcaatatattaaaatgcatttaaaagttacttctgggaaacatactaaataggccaatcagttaatcattagctaattgtcaaaccctataaaatcatggtataatgtcaccctgacataaagcaacatcaaaattagtgcatcatctataaagtgaagtattattttctcccaagtgacaaattctattgccaaaaaataccactgtacttctaataagtgacactcattttaatagaccctacaaaaatacaatattttcaatgtccccataaaacagttaacttacaaatattattctcagagctctggtgacatcattcagtgatactattgtgaaaatcctcatacaatacttgaaacactagcatgtaaagtaaattcattatataacaaaagaactatgtaaaattatgaaagataatgcatgcaaccaactccgggaaattatcctggaaattcaaattaatattgtaattaaattaatgactaatatgaaagataagtattttaaaggattataaaataaattttgatcatttatgcaggaaaatagtttcaatggaaaagtaaataattctacattaaccatgcttgtctttctcttcagtgaaaaagcattcaggattttacataccttgaaactgtttttggaaaaaaagtattttatctatttctgcccagaaaaacagccattgaaattaatgatacaggtagaccacagctctgagaaattatatttgaagtttcatatttaaataccaaggatttaaaatcacctaccataactttctaacagcagtctttcgtaatgataaattttatcaatttccaaaattcgttttaaataatttaaaaagcagcaaattagattaagcaacacacaaataaattccacatttacaagtaaagaaatcacaggggctacagtttataatcaacatgaacttgaaagaaataaagcaatacctttcctgccacccatcatccactgcttaaatttgtggtgaaaaagacttaactacaatgacctttagtctgtttctaaactctgcatgtattgtaattagctaaaggcattgaacaaattagttcatcctatttttatttgggtcccagagataaatggctaatttatgaaatatttcactctgtgtcatgagaatttagcaaatgaatatggaaccaaatataaacactttataccatatgtacagttactttcataaggcattatcatgtaatttttattgaaaaagattcaatatagtaaagtcttattttaagatatattttttctctatctgagatgtttagtttatgaaaatattgtttttctctatattctttttgtatatatgccaacatataccttgtgctagaaatattttatgggaattacaattctttatatttgtattttctatataaaggcatatacaactttgaggcagtgtttctgatggagagcagaattcataaagagcttgtgtgtgcttccgtgctccgaaattatatgaaatccattttgagaagaaacttatttgattaaaaacaaaaacaaaaacagaaacaaaactgcaccaatgcacagccagaggctgacaattaaaactaatacataaccacatgaacatcatatttatagagttaacattttttaaggatggtcagtgctaacatatagtattatacatttggcactaatgtttgccattggtccagcaattggcaaaatttgtttctatgtataaatttatttttgaacattaggtctggctagacgtatcttcactatttataaaaaatatttagacagtaagctcacgttgaataactaggtctactgtgttctggaaactcttcagtagtaatacagctttttcatgttccatatgtacaaaactgtgtccatttgcctgaaggatcttatcaccaggctgcagtaggtttgatgctggcccatcaggctgaaccctagtaacaaagatacccttgtcagaaggtttgaatggatttccttgtccactaattccaccactgatactaaatccaaggccaggattcttttctattctcacacaaaactgctctggatatccatccatactcctttgccctttagtttgaattaagcaccgtccaggctgaggtccccgggtggcctgtgaagaggggatctgaataggcaatggtgactgaaattgctggatggtcactttgtttatatttccttcatacggctgctgctcccggctgcgatgctgaaggctttgggaccccatcaacgtctggatgtggctgcctgccttcttagtaatggtgtccggaggtacatcccgcctcccaagtggataaggattccattggccactaggagatacatcttcttgtccattgtctaaaatgttgctttgctgggacggggtcctgtctaaccgtctagcttctatatgtctaagcagctgttgtctccagtctgcaggcattttaccacagctctcctctcccttcacaggagtaggcctcgtctttaaatcactgttatctgatggcttgtcaccatagttacccaagttatagtcagatggtattttttccaaaagagctgccatagtaggcctagctgaaactggcctggtttgggaggcaccgtaactctctgtactgtagcttctcgcagacaatggcctcctttgggtaaggtttttaaccggaaaacttcccgcctgagctttcacttcttgatatgaagggtgttcatcttcatacctgccattccttttcaggaactgggactcagtcactgtaacgctgctttggcgatccagccctcccctatatgggggtctgccgtacctatcagttgggggcagctcatgaggctcattgacccttctaaacatggccatttctgtggcgctcaccagggagtcggcccttctcaggaagcccgccctggccccttggcttgcgaactgggcattcaccacagcatcctcattcacagatggctgagaaaatgaaaacatttgctccatcggtgggtatcctctgtaagctctaggactaatcaaatccttggcgatgtttttgctggcctgttgcacgtactcgggattgtgttgaaaagggggtggtatcctcttttcggctttcacttccactgatccttgaggattgaagctttggtcaaactgatagactttttttgtcatagaagctttttgttgttgtggccccttactacttccgtaggtgagcatctcatcatccagcattgggactgactggcttcgagacatactggacataccatgctctggtcccagcatcttatccggtcgttcgtggcttcctaagtgatcactcccagaagcatagttttctaatggtatgttatacaccttatatgtaccaatgtcaatctcatcgatactctgtgactttttgaatttattagacttgatatctttcattaggggggaaagcctctctgtgcttttgctaattgaaataacacctttagaagattccgggcggcagtggatttgagaaaagacattactaagactcctgttgggattggaatcatgatactcccatggtacgcctggagaaaaaggactaggtatttcagtagattcctttatatgttctttcctttcaggcaatgggctggtagtgggggttgtctctaatttggaaggaaaagcggtcctgtcttcaaacggactaggggttctggtccaattctgccaaggattggaaggaggcacttctgtttctggtgtgtgtctgtgtgtagactgctcgagttccaggggaacaccaacaatcctgtcttgcctgatcaaaggcctgcgtccatgcgaagatgtgcttctagatttcgaacttaagagaggattactgttggcattctcggctgtggtttcctcagcaacaaaccctgtgttgtcataatgcgagccatcagtccagttgtcagtgaaagtatcactcatgggcagccggtcaggacgctgtggtatattgcctgggggaacagcctcccgctggctgagtaatggctttgaatcaagaggctgtgggaaagatggtgcaatcctgttaccccacaaagaattatgtactgcatctttagctgttgtctgcaaggaccccactttaacccgggtattagaggatcctgaggaagcctgggaaggcgagtagtctgagtaagtgcctgaggaaacactgttattcagacagtgagttttgtcaacttcagactcatcagttgattcttttttgtccttccctagcagaacaagtttgggtgggtacagaggggtctcagctaatgaagggtgaagttccccaatcctcatttcattagctggatgaacaaaagaatcctccactgtaatctcctttggggctaccggccacttgtgttcatatttttctttcacagtttgctccgtgttagcagttggatttgaattctcaacacgcactccatggcttggcttacccaccaaattttgaacagattttaccatattctttaaatcctctgggtaaggagttggatatcgttttaggtttatttcaacctgtctgccacttagagagggaagagtggtggattgtgctgcaactggcaatggagtacacatgctcctttcctgctggaggccacttatacaaccccatgccagctgtgggtcattctgggggacgggcatatcttggatctgctgatcacacctggcccatggtgtgcagcaatcgccagacagtctggcaggttggagagtaatcccacgctggcccctttcccagggggcttggcaggagagatccttaactttcccagcattttcgtcatcttcttttttgtcttcaaattcaaaggcaacagtcatgcgttgttgtctctgctcttcccacagtgtagggttaaagctgtcactgtctgactggaaatcttcatcaccacgaggctgctggggaaacatgtagttagtcaatactctttgctttgtttctggatgggcttctgtttgtaaagggataagggctttggactgattgtcagaaagccacaaagctgcaagctctttaagtttggtaaatgagaatggtaaattcttcaatctgttgtcactcaaatttaggactcttagtttctgcatctgtccaatctcttcaggaagaaattctaatttgttggagcgtagagacatgactgttacattcttacaacttccaatttctctgggtaattctggaaggaaattctcatcaactgctaatgtccgaagactatgaaggtagccaatagtagaaggtagtgactccagttcattacagctacagtcaaattcttctaataaagataaatttccaattgtattgggtagcattgtaagttgattgtcatctacttttagagttgttagttttttcaaaagtcctatagaatcaggcaattgttgcaacatattggatgacaataagaggtcctcaagggcttcacatccagaaatgtccatgtcaactgtttctattctgttttttgacatatccaggtataccaacatctttaacttccctatagacccaggtaacacttgtaatgcattattatccatccataactccctcaaattttgtatttgatccagaacttcaggcagctcaccgaattcattattgcctaggtcaagtctttccaactgggccagtttgtgcattgactttggtagagttttcaagtgattttctcttaactccaagatccgcaatttgacaagtcttccaaaattggctggaagaaattcaagaaaggcgtcattcaggtagagctgggtcaggtttaggagctgtgtgaagccatcaggtagtttagaaatgggattgacactggcttcaataattgttaaacacttacagcactttatgttttctggaaattcttgtacaccatttttactgatgtcgagttctttaagattaactaaactagcaatagtggttggcagatttgaaaggtcgttatcaggaatacttagttttcgtagagcttgacagttgaacaattgcttgggtagttcttcaatttgattggcatctagataaagctcctctaatgttcgttcgaagttaaagacctcctttggcacctgctgaagactgcagtgggagtaatctaaaactgagatgatttcttcttcacctcggaaacatcggcatggcaccagacggccgatgattttccgtttggtggtcatctccaggcactgcaactcctcttcaggcctcttccgaagtgctgcacgaacctctttacaaggacttctctggtattgcgggggattccttccccttattaggttctccatcatcgccggcgggagaaactgcccatgaggtttcggagagcgtagtcgtgcagctgccaagggttattccttaagtgttcaggggtccgcagtggagtgggcgccagggtcttcggaggagaagaggagggaaggagtagaaggtaggaagaacaggagatagaggggaatccaggaaggtgccacgttagaccatgatgccagtgcccttcaggtggacggctggagaggttcccgcgggaagcggctgaggggaagcccgaagcgccggcgggggaggcaggagcgcgtccactccccagcctcagcctgcccagcgcgccgcgctagcgaccgcagcagcagcggcggcggcggcggcggtggcggaggcgcagctccctccccgcccccagaaggctccacagacaataaatcctgggcggagaagagacaagcaggaaaggcgaatcctgcacccaactccgtaacaacccctgcccgttgccgcgcctgtgcagggcgaggatccccaggggccagggcgcagcgggcgtctcggaggggctgagcgctccgcaactgcaggaggcggtggcggtggcccgagtgggcggctgcaggtcccgccggcgagaacccgctgcactggggctgggtgtccgtggcttcaagcccggtgttcacccggagtagggtcctcctcggtgcagtggctcggcgcacaggtgccaggattggc

SEQ ID NO: 8531 - RNA, 8788 nt, Homo sapiens
  source 1..8788: mol_type = other RNA
aaaagtaattgtggtttttgcctgcacttttaatggtaaaaaccgcaattactttttcagcaacctaataattacaattctaagtaatggagatacatatcttttataggcttcaatgagcaatacattagcataatgttttatttcatactgactttgaatattccttgtcaaaaatgcacttatactttggagttactatgtatgtttaggttactgtgttgtcatcagaaggctggagttatcatagcagagctttaatgacaaaatattatgagccttgtaaatagttttaaaaattgtccactaatatctatttgtcttgcaaaatttgcaattttactagtaattttcatcacttgctctttctacctctaatgtttctcagtctcctccattagatcttactgacttatcacatataaacaccttcctcagaaacagtccaataaaaattaaagaccaagaggtagaatctactggagccatcatgaattccagttctttttgttgttattgatttttcttttttttttttaaaaggcacacccttgacttttttttattgttaaaataaccagattctaatttcaggcagcaaaatcagttactgcaaaaagtcaataatcaaaaatcaatgtataattggttttcatcacctatagaattagtgaggtttatacccctcaagtgtttagtgattctattcagtcaacctaaaaaaaattgcctcttttctacttaaataaataatttatttatttattttgagacagagtttcgctctgttgcccaggccggagtgcagtggcacaatctcagctcactgcaacctccgcctcccaggtcaagcgattgattctcatgcctcagcctcccaaatagctgggattataggtgcccgccaccatgctcagctaatttttgtatttttagtagagatggcgtttcaccatgttggccaggctggtcttgaactgacctcaagtgatccgcccaccttggcctcccaaagtgtggggattactagtgtgagccaccacgcctggcctgcctgttttcattattacctgcctgttctcagtatgcaacatggcagtactattgacagtgaggtgctttggcatatcagataacttttccagttggtcaaggatcccttttctcttttcctcatttctgaactgcagaacaggaagtactaaagaagtggctcaggacaatgttgtcacatcaggagtggcagaggtgtttactaggattatgatcctttcagctgtgtgtcttagaaggatctcctgaagccctgggtttgatatagaaaccataagaaaaagacttggggcagttctatatctggctcttctcccacttctcccataaaagattaagaaaaactgatgggatgatttcagatgtttcattgccaccaaactacagccatgagttttttttctttaagtgatcttatgaggccagtaaaggcctctgtcttgattaatgatgatcatcctataatatctggatatggtggcttgacatgagttttcaacaaagaaaattagtctctgaaagacatttctcatctgaaactctcaatatattaaaatgcatttaaaagttacttctgggaaacatactaaataggccaatcagttaatcattagctaattgtcaaaccctataaaatcatggtataatgtcaccctgacataaagcaacatcaaaattagtgcatcatctataaagtgaagtattattttctcccaagtgacaaattctattgccaaaaaataccactgtacttctaataagtgacactcattttaatagaccctacaaaaatacaatattttcaatgtccccataaaacagttaacttacaaatattattctcagagctctggtgacatcattcagtgatactattgtgaaaatcctcatacaatacttgaaacactagcatgtaaagtaaattcattatataacaaaagaactatgtaaaattatgaaagataatgcatgcaaccaactccgggaaattatcctggaaattcaaattaatattgtaattaaattaatgactaatatgaaagataagtattttaaaggattataaaataaattttgatcatttatgcaggaaaatagtttcaatggaaaagtaaataattctacattaaccatgcttgtctttctcttcagtgaaaaagcattcaggattttacataccttgaaactgtttttggaaaaaaagtattttatctatttctgcccagaaaaacagccattgaaattaatgatacaggtagaccacagctctgagaaattatatttgaagtttcatatttaaataccaaggatttaaaatcacctaccataactttctaacagcagtctttcgtaatgataaattttatcaatttccaaaattcgttttaaataatttaaaaagcagcaaattagattaagcaacacacaaataaattccacatttacaagtaaagaaatcacaggggctacagtttataatcaacatgaacttgaaagaaataaagcaatacctttcctgccacccatcatccactgcttaaatttgtggtgaaaaagacttaactacaatgacctttagtctgtttctaaactctgcatgtattgtaattagctaaaggcattgaacaaattagttcatcctatttttatttgggtcccagagataaatggctaatttatgaaatatttcactctgtgtcatgagaatttagcaaatgaatatggaaccaaatataaacactttataccatatgtacagttactttcataaggcattatcatgtaatttttattgaaaaagattcaatatagtaaagtcttattttaagatatattttttctctatctgagatgtttagtttatgaaaatattgtttttctctatattctttttgtatatatgccaacatataccttgtgctagaaatattttatgggaattacaattctttatatttgtattttctatataaaggcatatacaactttgaggcagtgtttctgatggagagcagaattcataaagagcttgtgtgtgcttccgtgctccgaaattatatgaaatccattttgagaagaaacttatttgattaaaaacaaaaacaaaaacagaaacaaaactgcaccaatgcacagccagaggctgacaattaaaactaatacataaccacatgaacatcatatttatagagttaacattttttaaggatggtcagtgctaacatatagtattatacatttggcactaatgtttgccattggtccagcaattggcaaaatttgtttctatgtataaatttatttttgaacattaggtctggctagacgtatcttcactatttataaaaaatatttagacagtaagctcacgttgaataactaggtctactgtgttctggaaactcttcagtagtaatacagctttttcatgttccatatgtacaaaactgtgtccatttgcctgaaggatcttatcaccaggctgcagtaggtttgatgctggcccatcaggctgaaccctagtaacaaagatacccttgtcagaaggtttgaatggatttccttgtccactaattccaccactgatactaaatccaaggccaggattcttttctattctcacacaaaactgctctggatatccatccatactcctttgccctttagtttgaattaagcaccgtccaggctgaggtccccgggtggcctgtgaagaggggatctgaataggcaatggtgactgaaattgctggatggtcactttgtttatatttccttcatacggctgctgctcccggctgcgatgctgaaggctttgggaccccatcaacgtctggatgtggctgcctgccttcttagtaatggtgtccggaggtacatcccgcctcccaagtggataaggattccattggccactaggagatacatcttcttgtccattgtctaaaatgttgctttgctgggacggggtcctgtctaaccgtctagcttctatatgtctaagcagctgttgtctccagtctgcaggcattttaccacagctctcctctcccttcacaggagtaggcctcgtctttaaatcactgttatctgatggcttgtcaccatagttacccaagttatagtcagatggtattttttccaaaagagctgccatagtaggcctagctgaaactggcctggtttgggaggcaccgtaactctctgtactgtagcttctcgcagacaatggcctcctttgggtaaggtttttaaccggaaaacttcccgcctgagctttcacttcttgatatgaagggtgttcatcttcatacctgccattccttttcaggaactgggactcagtcactgtaacgctgctttggcgatccagccctcccctatatgggggtctgccgtacctatcagttgggggcagctcatgaggctcattgacccttctaaacatggccatttctgtggcgctcaccagggagtcggcccttctcaggaagcccgccctggccccttggcttgcgaactgggcattcaccacagcatcctcattcacagatggctgagaaaatgaaaacatttgctccatcggtgggtatcctctgtaagctctaggactaatcaaatccttggcgatgtttttgctggcctgttgcacgtactcgggattgtgttgaaaagggggtggtatcctcttttcggctttcacttccactgatccttgaggattgaagctttggtcaaactgatagactttttttgtcatagaagctttttgttgttgtggccccttactacttccgtaggtgagcatctcatcatccagcattgggactgactggcttcgagacatactggacataccatgctctggtcccagcatcttatccggtcgttcgtggcttcctaagtgatcactcccagaagcatagttttctaatggtatgttatacaccttatatgtaccaatgtcaatctcatcgatactctgtgactttttgaatttattagacttgatatctttcattaggggggaaagcctctctgtgcttttgctaattgaaataacacctttagaagattccgggcggcagtggatttgagaaaagacattactaagactcctgttgggattggaatcatgatactcccatggtacgcctggagaaaaaggactaggtatttcagtagattcctttatatgttctttcctttcaggcaatgggctggtagtgggggttgtctctaatttggaaggaaaagcggtcctgtcttcaaacggactaggggttctggtccaattctgccaaggattggaaggaggcacttctgtttctggtgtgtgtctgtgtgtagactgctcgagttccaggggaacaccaacaatcctgtcttgcctgatcaaaggcctgcgtccatgcgaagatgtgcttctagatttcgaacttaagagaggattactgttggcattctcggctgtggtttcctcagcaacaaaccctgtgttgtcataatgcgagccatcagtccagttgtcagtgaaagtatcactcatgggcagccggtcaggacgctgtggtatattgcctgggggaacagcctcccgctggctgagtaatggctttgaatcaagaggctgtgggaaagatggtgcaatcctgttaccccacaaagaattatgtactgcatctttagctgttgtctgcaaggaccccactttaacccgggtattagaggatcctgaggaagcctgggaaggcgagtagtctgagtaagtgcctgaggaaacactgttattcagacagtgagttttgtcaacttcagactcatcagttgattcttttttgtccttccctagcagaacaagtttgggtgggtacagaggggtctcagctaatgaagggtgaagttccccaatcctcatttcattagctggatgaacaaaagaatcctccactgtaatctcctttggggctaccggccacttgtgttcatatttttctttcacagtttgctccgtgttagcagttggatttgaattctcaacacgcactccatggcttggcttacccaccaaattttgaacagattttaccatattctttaaatcctctgggtaaggagttggatatcgttttaggtttatttcaacctgtctgccacttagagagggaagagtggtggattgtgctgcaactggcaatggagtacacatgctcctttcctgctggaggccacttatacaaccccatgccagctgtgggtcattctgggggacgggcatatcttggatctgctgatcacacctggcccatggtgtgcagcaatcgccagacagtctggcaggttggagagtaatcccacgctggcccctttcccagggggcttggcaggagagatccttaactttcccagcattttcgtcatcttcttttttgtcttcaaattcaaaggcaacagtcatgcgttgttgtctctgctcttcccacagtgtagggttaaagctgtcactgtctgactggaaatcttcatcaccacgaggctgctggggaaacatgtagttagtcaatactctttgctttgtttctggatgggcttctgtttgtaaagggataagggctttggactgattgtcagaaagccacaaagctgcaagctctttaagtttggtaaatgagaatggtaaattcttcaatctgttgtcactcaaatttaggactcttagtttctgcatctgtccaatctcttcaggaagaaattctaatttgttggagcgtagagacatgactgttacattcttacaacttccaatttctctgggtaattctggaaggaaattctcatcaactgctaatgtccgaagactatgaaggtagccaatagtagaaggtagtgactccagttcattacagctacagtcaaattcttctaataaagataaatttccaattgtattgggtagcattgtaagttgattgtcatctacttttagagttgttagttttttcaaaagtcctatagaatcaggcaattgttgcaacatattggatgacaataagaggtcctcaagggcttcacatccagaaatgtccatgtcaactgtttctattctgttttttgacatatccaggtataccaacatctttaacttccctatagacccaggtaacacttgtaatgcattattatccatccataactccctcaaattttgtatttgatccagaacttcaggcagctcaccgaattcattattgcctaggtcaagtctttccaactgggccagtttgtgcattgactttggtagagttttcaagtgattttctcttaactccaagatccgcaatttgacaagtcttccaaaattggctggaagaaattcaagaaaggcgtcattcaggtagagctgggtcaggtttaggagctgtgtgaagccatcaggtagtttagaaatgggattgacactggcttcaataattgttaaacacttacagcactttatgttttctggaaattcttgtacaccatttttactgatgtcgagttctttaagattaactaaactagcaatagtggttggcagatttgaaaggtcgttatcaggaatacttagttttcgtagagcttgacagttgaacaattgcttgggtagttcttcaatttgattggcatctagataaagctcctctaatgttcgttcgaagttaaagacctcctttggcacctgctgaagactgcagtgggagtaatctaaaactgagatgatttcttcttcacctcggaaacatcggcatggcaccagacggccgatgattttccgtttggtggtcatctccaggcactgcattgctagttattcctgtctctgcagacttctaggttgtgaccactttgacttgcattttttttcatgtagcgggctcactcctcttcaggcctcttccgaagtgctgcacgaacctctttacaaggacttctctggtattgcgggggattccttccccttattaggttctccatcatcgccggcgggagaaactgcccatgaggtttcggagagcgtagtcgtgcagctgccaagggttattccttaagtgttcaggggtccgcagtggagtgggcgccagggtcttcggaggagaagaggagggaaggagtagaaggtaggaagaacaggagatagaggggaatccaggaaggtgccacgttagaccatgatgccagtgcccttcaggtggacggctggagaggttcccgcgggaagcggctgaggggaagcccgaagcgccggcgggggaggcaggagcgcgtccactccccagcctcagcctgcccagcgcgccgcgctagcgaccgcagcagcagcggcggcggcggcggcggtggcggaggcgcagctccctccccgcccccagaaggctccacagacaataaatcctgggcggagaagagacaagcaggaaaggcgaatcctgcacccaactccgtaacaacccctgcccgttgccgcgcctgtgcagggcgaggatccccaggggccagggcgcagcgggcgtctcggaggggctgagcgctccgcaactgcaggaggcggtggcggtggcccgagtgggcggctgcaggtcccgccggcgagaacccgctgcactggggctgggtgtccgtggcttcaagcccggtgttcacccggagtagggtcctcctcggtgcagtggctcggcgcacaggtgccaggattggc

SEQ ID NO: 8532 - RNA, 8852 nt, Homo sapiens
  source 1..8852: mol_type = other RNA
aaaagtaattgtggtttttgcctgcacttttaatggtaaaaaccgcaattactttttcagcaacctaataattacaattctaagtaatggagatacatatcttttataggcttcaatgagcaatacattagcataatgttttatttcatactgactttgaatattccttgtcaaaaatgcacttatactttggagttactatgtatgtttaggttactgtgttgtcatcagaaggctggagttatcatagcagagctttaatgacaaaatattatgagccttgtaaatagttttaaaaattgtccactaatatctatttgtcttgcaaaatttgcaattttactagtaattttcatcacttgctctttctacctctaatgtttctcagtctcctccattagatcttactgacttatcacatataaacaccttcctcagaaacagtccaataaaaattaaagaccaagaggtagaatctactggagccatcatgaattccagttctttttgttgttattgatttttcttttttttttttaaaaggcacacccttgacttttttttattgttaaaataaccagattctaatttcaggcagcaaaatcagttactgcaaaaagtcaataatcaaaaatcaatgtataattggttttcatcacctatagaattagtgaggtttatacccctcaagtgtttagtgattctattcagtcaacctaaaaaaaattgcctcttttctacttaaataaataatttatttatttattttgagacagagtttcgctctgttgcccaggccggagtgcagtggcacaatctcagctcactgcaacctccgcctcccaggtcaagcgattgattctcatgcctcagcctcccaaatagctgggattataggtgcccgccaccatgctcagctaatttttgtatttttagtagagatggcgtttcaccatgttggccaggctggtcttgaactgacctcaagtgatccgcccaccttggcctcccaaagtgtggggattactagtgtgagccaccacgcctggcctgcctgttttcattattacctgcctgttctcagtatgcaacatggcagtactattgacagtgaggtgctttggcatatcagataacttttccagttggtcaaggatcccttttctcttttcctcatttctgaactgcagaacaggaagtactaaagaagtggctcaggacaatgttgtcacatcaggagtggcagaggtgtttactaggattatgatcctttcagctgtgtgtcttagaaggatctcctgaagccctgggtttgatatagaaaccataagaaaaagacttggggcagttctatatctggctcttctcccacttctcccataaaagattaagaaaaactgatgggatgatttcagatgtttcattgccaccaaactacagccatgagttttttttctttaagtgatcttatgaggccagtaaaggcctctgtcttgattaatgatgatcatcctataatatctggatatggtggcttgacatgagttttcaacaaagaaaattagtctctgaaagacatttctcatctgaaactctcaatatattaaaatgcatttaaaagttacttctgggaaacatactaaataggccaatcagttaatcattagctaattgtcaaaccctataaaatcatggtataatgtcaccctgacataaagcaacatcaaaattagtgcatcatctataaagtgaagtattattttctcccaagtgacaaattctattgccaaaaaataccactgtacttctaataagtgacactcattttaatagaccctacaaaaatacaatattttcaatgtccccataaaacagttaacttacaaatattattctcagagctctggtgacatcattcagtgatactattgtgaaaatcctcatacaatacttgaaacactagcatgtaaagtaaattcattatataacaaaagaactatgtaaaattatgaaagataatgcatgcaaccaactccgggaaattatcctggaaattcaaattaatattgtaattaaattaatgactaatatgaaagataagtattttaaaggattataaaataaattttgatcatttatgcaggaaaatagtttcaatggaaaagtaaataattctacattaaccatgcttgtctttctcttcagtgaaaaagcattcaggattttacataccttgaaactgtttttggaaaaaaagtattttatctatttctgcccagaaaaacagccattgaaattaatgatacaggtagaccacagctctgagaaattatatttgaagtttcatatttaaataccaaggatttaaaatcacctaccataactttctaacagcagtctttcgtaatgataaattttatcaatttccaaaattcgttttaaataatttaaaaagcagcaaattagattaagcaacacacaaataaattccacatttacaagtaaagaaatcacaggggctacagtttataatcaacatgaacttgaaagaaataaagcaatacctttcctgccacccatcatccactgcttaaatttgtggtgaaaaagacttaactacaatgacctttagtctgtttctaaactctgcatgtattgtaattagctaaaggcattgaacaaattagttcatcctatttttatttgggtcccagagataaatggctaatttatgaaatatttcactctgtgtcatgagaatttagcaaatgaatatggaaccaaatataaacactttataccatatgtacagttactttcataaggcattatcatgtaatttttattgaaaaagattcaatatagtaaagtcttattttaagatatattttttctctatctgagatgtttagtttatgaaaatattgtttttctctatattctttttgtatatatgccaacatataccttgtgctagaaatattttatgggaattacaattctttatatttgtattttctatataaaggcatatacaactttgaggcagtgtttctgatggagagcagaattcataaagagcttgtgtgtgcttccgtgctccgaaattatatgaaatccattttgagaagaaacttatttgattaaaaacaaaaacaaaaacagaaacaaaactgcaccaatgcacagccagaggctgacaattaaaactaatacataaccacatgaacatcatatttatagagttaacattttttaaggatggtcagtgctaacatatagtattatacatttggcactaatgtttgccattggtccagcaattggcaaaatttgtttctatgtataaatttatttttgaacattaggtctggctagacgtatcttcactatttataaaaaatatttagacagtaagctcacgttgaataactaggtctactgtgttctggaaactcttcagtagtaatacagctttttcatgttccatatgtacaaaactgtgtccatttgcctgaaggatcttatcaccaggctgcagtaggtttgatgctggcccatcaggctgaaccctagtaacaaagatacccttgtcagaaggtttgaatggatttccttgtccactaattccaccactgatactaaatccaaggccaggattcttttctattctcacacaaaactgctctggatatccatccatactcctttgccctttagtttgaattaagcaccgtccaggctgaggtccccgggtggcctgtgaagaggggatctgaataggcaatggtgactgaaattgctggatggtcactttgtttatatttccttcatacggctgctgctcccggctgcgatgctgaaggctttgggaccccatcaacgtctggatgtggctgcctgccttcttagtaatggtgtccggaggtacatcccgcctcccaagtggataaggattccattggccactaggagatacatcttcttgtccattgtctaaaatgttgctttgctgggacggggttttctgaagaggtagttcttgatgatcaaatttagacttagtctgcaagtttaaagtcatgcttctgcctgcatgcattgctgaaatacctccatagggcagcatgccaaggttaactgtattgtgtttgtaagcagcattcctgtctaaccgtctagcttctatatgtctaagcagctgttgtctccagtctgcaggcattttaccacagctctcctctcccttcacaggagtaggcctcgtctttaaatcactgttatctgatggcttgtcaccatagttacccaagttatagtcagatggtattttttccaaaagagctgccatagtaggcctagctgaaactggcctggtttgggaggcaccgtaactctctgtactgtagcttctcgcagacaatggcctcctttgggtaaggtttttaaccggaaaacttcccgcctgagctttcacttcttgatatgaagggtgttcatcttcatacctgccattccttttcaggaactgggactcagtcactgtaacgctgctttggcgatccagccctcccctatatgggggtctgccgtacctatcagttgggggcagctcatgaggctcattgacccttctaaacatggccatttctgtggcgctcaccagggagtcggcccttctcaggaagcccgccctggccccttggcttgcgaactgggcattcaccacagcatcctcattcacagatggctgagaaaatgaaaacatttgctccatcggtgggtatcctctgtaagctctaggactaatcaaatccttggcgatgtttttgctggcctgttgcacgtactcgggattgtgttgaaaagggggtggtatcctcttttcggctttcacttccactgatccttgaggattgaagctttggtcaaactgatagactttttttgtcatagaagctttttgttgttgtggccccttactacttccgtaggtgagcatctcatcatccagcattgggactgactggcttcgagacatactggacataccatgctctggtcccagcatcttatccggtcgttcgtggcttcctaagtgatcactcccagaagcatagttttctaatggtatgttatacaccttatatgtaccaatgtcaatctcatcgatactctgtgactttttgaatttattagacttgatatctttcattaggggggaaagcctctctgtgcttttgctaattgaaataacacctttagaagattccgggcggcagtggatttgagaaaagacattactaagactcctgttgggattggaatcatgatactcccatggtacgcctggagaaaaaggactaggtatttcagtagattcctttatatgttctttcctttcaggcaatgggctggtagtgggggttgtctctaatttggaaggaaaagcggtcctgtcttcaaacggactaggggttctggtccaattctgccaaggattggaaggaggcacttctgtttctggtgtgtgtctgtgtgtagactgctcgagttccaggggaacaccaacaatcctgtcttgcctgatcaaaggcctgcgtccatgcgaagatgtgcttctagatttcgaacttaagagaggattactgttggcattctcggctgtggtttcctcagcaacaaaccctgtgttgtcataatgcgagccatcagtccagttgtcagtgaaagtatcactcatgggcagccggtcaggacgctgtggtatattgcctgggggaacagcctcccgctggctgagtaatggctttgaatcaagaggctgtgggaaagatggtgcaatcctgttaccccacaaagaattatgtactgcatctttagctgttgtctgcaaggaccccactttaacccgggtattagaggatcctgaggaagcctgggaaggcgagtagtctgagtaagtgcctgaggaaacactgttattcagacagtgagttttgtcaacttcagactcatcagttgattcttttttgtccttccctagcagaacaagtttgggtgggtacagaggggtctcagctaatgaagggtgaagttccccaatcctcatttcattagctggatgaacaaaagaatcctccactgtaatctcctttggggctaccggccacttgtgttcatatttttctttcacagtttgctccgtgttagcagttggatttgaattctcaacacgcactccatggcttggcttacccaccaaattttgaacagattttaccatattctttaaatcctctgggtaaggagttggatatcgttttaggtttatttcaacctgtctgccacttagagagggaagagtggtggattgtgctgcaactggcaatggagtacacatgctcctttcctgctggaggccacttatacaaccccatgccagctgtgggtcattctgggggacgggcatatcttggatctgctgatcacacctggcccatggtgtgcagcaatcgccagacagtctggcaggttggagagtaatcccacgctggcccctttcccagggggcttggcaggagagatccttaactttcccagcattttcgtcatcttcttttttgtcttcaaattcaaaggcaacagtcatgcgttgttgtctctgctcttcccacagtgtagggttaaagctgtcactgtctgactggaaatcttcatcaccacgaggctgctggggaaacatgtagttagtcaatactctttgctttgtttctggatgggcttctgtttgtaaagggataagggctttggactgattgtcagaaagccacaaagctgcaagctctttaagtttggtaaatgagaatggtaaattcttcaatctgttgtcactcaaatttaggactcttagtttctgcatctgtccaatctcttcaggaagaaattctaatttgttggagcgtagagacatgactgttacattcttacaacttccaatttctctgggtaattctggaaggaaattctcatcaactgctaatgtccgaagactatgaaggtagccaatagtagaaggtagtgactccagttcattacagctacagtcaaattcttctaataaagataaatttccaattgtattgggtagcattgtaagttgattgtcatctacttttagagttgttagttttttcaaaagtcctatagaatcaggcaattgttgcaacatattggatgacaataagaggtcctcaagggcttcacatccagaaatgtccatgtcaactgtttctattctgttttttgacatatccaggtataccaacatctttaacttccctatagacccaggtaacacttgtaatgcattattatccatccataactccctcaaattttgtatttgatccagaacttcaggcagctcaccgaattcattattgcctaggtcaagtctttccaactgggccagtttgtgcattgactttggtagagttttcaagtgattttctcttaactccaagatccgcaatttgacaagtcttccaaaattggctggaagaaattcaagaaaggcgtcattcaggtagagctgggtcaggtttaggagctgtgtgaagccatcaggtagtttagaaatgggattgacactggcttcaataattgttaaacacttacagcactttatgttttctggaaattcttgtacaccatttttactgatgtcgagttctttaagattaactaaactagcaatagtggttggcagatttgaaaggtcgttatcaggaatacttagttttcgtagagcttgacagttgaacaattgcttgggtagttcttcaatttgattggcatctagataaagctcctctaatgttcgttcgaagttaaagacctcctttggcacctgctgaagactgcagtgggagtaatctaaaactgagatgatttcttcttcacctcggaaacatcggcatggcaccagacggccgatgattttccgtttggtggtcatctccaggcactgcaactcctcttcaggcctcttccgaagtgctgcacgaacctctttacaaggacttctctggtattgcgggggattccttccccttattaggttctccatcatcgccggcgggagaaactgcccatgaggtttcggagagcgtagtcgtgcagctgccaagggttattccttaagtgttcaggggtccgcagtggagtgggcgccagggtcttcggaggagaagaggagggaaggagtagaaggtaggaagaacaggagatagaggggaatccaggaaggtgccacgttagaccatgatgccagtgcccttcaggtggacggctggagaggttcccgcgggaagcggctgaggggaagcccgaagcgccggcgggggaggcaggagcgcgtccactccccagcctcagcctgcccagcgcgccgcgctagcgaccgcagcagcagcggcggcggcggcggcggtggcggaggcgcagctccctccccgcccccagaaggctccacagacaataaatcctgggcggagaagagacaagcaggaaaggcgaatcctgcacccaactccgtaacaacccctgcccgttgccgcgcctgtgcagggcgaggatccccaggggccagggcgcagcgggcgtctcggaggggctgagcgctccgcaactgcaggaggcggtggcggtggcccgagtgggcggctgcaggtcccgccggcgagaacccgctgcactggggctgggtgtccgtggcttcaagcccggtgttcacccggagtagggtcctcctcggtgcagtggctcggcgcacaggtgccaggattggc

SEQ ID NO: 8533 - RNA, 8042 nt, Homo sapiens
  source 1..8042: mol_type = other RNA
aaaagtaattgtggtttttgcctgcacttttaatggtaaaaaccgcaattactttttcagcaacctaataattacaattctaagtaatggagatacatatcttttataggcttcaatgagcaatacattagcataatgttttatttcatactgactttgaatattccttgtcaaaaatgcacttatactttggagttactatgtatgtttaggttactgtgttgtcatcagaaggctggagttatcatagcagagctttaatgacaaaatattatgagccttgtaaatagttttaaaaattgtccactaatatctatttgtcttgcaaaatttgcaattttactagtaattttcatcacttgctctttctacctctaatgtttctcagtctcctccattagatcttactgacttatcacatataaacaccttcctcagaaacagtccaataaaaattaaagaccaagaggtagaatctactggagccatcatgaattccagttctttttgttgttattgatttttcttttttttttttaaaaggcacacccttgacttttttttattgttaaaataaccagattctaatttcaggcagcaaaatcagttactgcaaaaagtcaataatcaaaaatcaatgtataattggttttcatcacctatagaattagtgaggtttatacccctcaagtgtttagtgattctattcagtcaacctaaaaaaaattgcctcttttctacttaaataaataatttatttatttattttgagacagagtttcgctctgttgcccaggccggagtgcagtggcacaatctcagctcactgcaacctccgcctcccaggtcaagcgattgattctcatgcctcagcctcccaaatagctgggattataggtgcccgccaccatgctcagctaatttttgtatttttagtagagatggcgtttcaccatgttggccaggctggtcttgaactgacctcaagtgatccgcccaccttggcctcccaaagtgtggggattactagtgtgagccaccacgcctggcctgcctgttttcattattacctgcctgttctcagtatgcaacatggcagtactattgacagtgaggtgctttggcatatcagataacttttccagttggtcaaggatcccttttctcttttcctcatttctgaactgcagaacaggaagtactaaagaagtggctcaggacaatgttgtcacatcaggagtggcagaggtgtttactaggattatgatcctttcagctgtgtgtcttagaaggatctcctgaagccctgggtttgatatagaaaccataagaaaaagacttggggcagttctatatctggctcttctcccacttctcccataaaagattaagaaaaactgatgggatgatttcagatgtttcattgccaccaaactacagccatgagttttttttctttaagtgatcttatgaggccagtaaaggcctctgtcttgattaatgatgatcatcctataatatctggatatggtggcttgacatgagttttcaacaaagaaaattagtctctgaaagacatttctcatctgaaactctcaatatattaaaatgcatttaaaagttacttctgggaaacatactaaataggccaatcagttaatcattagctaattgtcaaaccctataaaatcatggtataatgtcaccctgacataaagcaacatcaaaattagtgcatcatctataaagtgaagtattattttctcccaagtgacaaattctattgccaaaaaataccactgtacttctaataagtgacactcattttaatagaccctacaaaaatacaatattttcaatgtccccataaaacagttaacttacaaatattattctcagagctctggtgacatcattcagtgatactattgtgaaaatcctcatacaatacttgaaacactagcatgtaaagtaaattcattatataacaaaagaactatgtaaaattatgaaagataatgcatgcaaccaactccgggaaattatcctggaaattcaaattaatattgtaattaaattaatgactaatatgaaagataagtattttaaaggattataaaataaattttgatcatttatgcaggaaaatagtttcaatggaaaagtaaataattctacattaaccatgcttgtctttctcttcagtgaaaaagcattcaggattttacataccttgaaactgtttttggaaaaaaagtattttatctatttctgcccagaaaaacagccattgaaattaatgatacaggtagaccacagctctgagaaattatatttgaagtttcatatttaaataccaaggatttaaaatcacctaccataactttctaacagcagtctttcgtaatgataaattttatcaatttccaaaattcgttttaaataatttaaaaagcagcaaattagattaagcaacacacaaataaattccacatttacaagtaaagaaatcacaggggctacagtttataatcaacatgaacttgaaagaaataaagcaatacctttcctgccacccatcatccactgcttaaatttgtggtgaaaaagacttaactacaatgacctttagtctgtttctaaactctgcatgtattgtaattagctaaaggcattgaacaaattagttcatcctatttttatttgggtcccagagataaatggctaatttatgaaatatttcactctgtgtcatgagaatttagcaaatgaatatggaaccaaatataaacactttataccatatgtacagttactttcataaggcattatcatgtaatttttattgaaaaagattcaatatagtaaagtcttattttaagatatattttttctctatctgagatgtttagtttatgaaaatattgtttttctctatattctttttgtatatatgccaacatataccttgtgctagaaatattttatgggaattacaattctttatatttgtattttctatataaaggcatatacaactttgaggcagtgtttctgatggagagcagaattcataaagagcttgtgtgtgcttccgtgctccgaaattatatgaaatccattttgagaagaaacttatttgattaaaaacaaaaacaaaaacagaaacaaaactgcaccaatgcacagccagaggctgacaattaaaactaatacataaccacatgaacatcatatttatagagttaacattttttaaggatggtcagtgctaacatatagtattatacatttggcactaatgtttgccattggtccagcaattggcaaaatttgtttctatgtataaatttatttttgaacattaggtctggctagacgtatcttcactatttataaaaaatatttagacagtaagctcacgttgaataactaggtctactgtgttctggaaactcttcagtagtaatacagctttttcatgttccatatgtacaaaactgtgtccatttgcctgaaggatcttatcaccaggctgcagtaggtttgatgctggcccatcaggctgaacccttgtcagaaggtttgaatggatttccttgtccactaattccaccactgatactaaatccaaggccaggattcttttctattctcacacaaaactgctctggatatccatccatactcctttgccctttagtttgaattaagcaccgtccaggctgaggtccccgggtggcctgtgaagaggggatctgaataggcaatggtgactgaaattgctggatggtcactttgtttatatttccttcatacggctgctgctcccggctgcgatgctgaaggctttgggaccccatcaacgtctggatgtggctgcctgccttcttagtaatggtgtccggaggtacatcccgcctcccaagtggataaggattccattggccactaggagatacatcttcttgtccattgtctaaaatgttgctttgctgggacggggtcctgtctaaccgtctagcttctatatgtctaagcagctgttgtctccagtctgcaggcattttaccacagctctcctctcccttcacaggagtaggcctcgtctttaaatcactgttatctgatggcttgtcaccatagttacccaagttatagtcagatggtattttttccaaaagagctgccatagtaggcctagctgaaactggcctggtttgggaggcaccgtaactctctgtactgtagcttctcgcagacaatggcctcctttgggtaaggtttttaaccggaaaacttcccgcctgagctttcacttcttgatatgaagggtgttcatcttcatacctgccattccttttcaggaactgggactcagtcactgtaacgctgctttggcgatccagccctcccctatatgggggtctgccgtacctatcagttgggggcagctcatgaggctcattgacccttctaaacatggccatttctgtggcgctcaccagggagtcggcccttctcaggaagcccgccctggccccttggcttgcgaactgggcattcaccacagcatcctcattcacagatggctgagaaaatgaaaacatttgctccatcggtgggtatcctctgtaagctctaggactaatcaaatccttggcgatgtttttgctggcctgttgcacgtactcgggattgtgttgaaaagggggtggtatcctcttttcggctttcacttccactgatccttgaggattgaagctttggtcaaactgatagactttttttgtcatagaagctttttgttgttgtggccccttactacttccgtaggtgagcatctcatcatccagcattgggactgactggcttcgagacatactggacataccatgctctggtcccagcatcttatccggtcgttcgtggcttcctaagtgatcactcccagaagcatagttttctaatggtatgttatacaccttatatgtaccaatgtcaatctcatcgatactctgtgactttttgaatttattagacttgatatctttcattaggggggaaagcctctctgtgcttttgctaattgaaataacacctttagaagattccgggcggcagtggatttgagaaaagacattactaagactcctgttgggattggaatcatgatactcccatggtacgcctggagaaaaaggactaggtatttcagtagattcctttatatgttctttcctttcaggcaatgggctggtagtgggggttgtctctaatttggaaggaaaagcggtcctgtcttcaaacggactaggggttctggtccaattctgccaaggattggaaggaggcacttctgtttctggtgtgtgtctgtgtgtagactgctcgagttccaggggaacaccaacaatcctgtcttgcctgatcaaaggcctgcgtccatgcgaagatgtgcttctagatttcgaacttaagagaggattactgttggcattctcggctgtggtttcctcagcaacaaaccctgtgttgtcataatgcgagccatcagtccagttgtcagtgaaagtatcactcatgggcagccggtcaggacgctgtggtatattgcctgggggaacagcctcccgctggctgagtaatggctttgaatcaagaggctgtgggaaagatggtgcaatcctgttaccccacaaagaattatgtactgcatctttagctgttgtctgcaaggaccccactttaacccgggtattagaggatcctgaggaagcctgggaaggcgagtagtctgagtaagtgcctgaggaaacactgttattcagacagtgagttttgtcaacttcagactcatcagttgattcttttttgtccttccctagcagaacaagtttgggtgggtacagaggggtctcagctaatgaagggtgaagttccccaatcctcatttcattagctggatgaacaaaagaatcctccactgtaatctcctttggggctaccggccacttgtgttcatatttttctttcacagtttgctccgtgttagcagttggatttgaattctcaacacgcactccatggcttggcttacccaccaaattttgaacagattttaccatattctttaaatcctctgggtaaggagttggatatcgttttaggtttatttcaacctgtctgccacttagagagggaagagtggtggattgtgctgcaactggcaatggagtacacatgctcctttcctgctggaggccacttatacaaccccatgccagctgtgggtcattctgggggacgggcatatcttggatctgctgatcacacctggcccatggtgtgcagcaatcgccagacagtctggcaggttggagagtaatcccacgctggcccctttcccagggggcttggcaggagagatccttaactttcccagcattttcgtcatcttcttttttgtcttcaaattcaaaggcaacagtcatgcgttgttgtctctgctcttcccacagtgtagggttaaagctgtcactgtctgactggaaatcttcatcaccacgaggctgctggggaaacatgtagttagtcaatactctttgctttgtttctggatgggcttctgtttgtaaagggataagggctttggactgattgtcagaaagccacaaagctgcaagctctttaagtttggtaaatgagaatggtaaattcttcaatctgttgtcactcaaatttaggactcttagtttctgcatctgtccaatctcttcaggaagaaattctaatttgttggagcgtagagacatgactgttacattcttacaacttccaatttctctgggtaattctggaaggaaattctcatcaactgctaatgtccgaagactatgaaggtagccaatagtagaaggtagtgactccagttcattacagctacagtcaaattcttctaataaagataaatttccaattgtattgggtagcattgtaagttgattgtcatctacttttagagttgttagttttttcaaaagtcctatagaatcaggcaattgttgcaacatattggatgacaataagaggtcctcaagggcttcacatccagaaatgtccatgtcaactgtttctattctgttttttgacatatccaggtataccaacatctttaacttccctatagacccaggtaacacttgtaatgcattattatccatccataactccctcaaattttgtatttgatccagaacttcaggcagctcaccgaattcattattgcctaggtcaagtctttccaactgggccagtttgtgcattgactttggtagagttttcaagtgattttctcttaactccaagatccgcaatttgacaagtcttccaaaattggctggaagaaattcaagaaaggcgtcattcaggtagagctgggtcaggtttaggagctgtgtgaagccatcaggtagtttagaaatgggattgacactggcttcaataattgttaaacacttacagcactttatgttttctggaaattcttgtacaccatttttactgatgtcgagttctttaagattaactaaactagcaatagtggttggcagatttgaaaggtcgttatcaggaatacttagttttcgtagagcttgacagttgaacaattgcttgggtagttcttcaatttgattggcatctagataaagctcctctaatgttcgttcgaagttaaagacctcctttggcacctgctgaagactgcagtgggagtaatctaaaactgagatgatttcttcttcacctcggaaacatcggcatggcaccagacggccgatgattttccgtttggtggtcatctccaggcactgcaactcctcttcaggcctcttccgaagtgctgcacgaacctctttacaaggacttctctggtattgcgggggattccttccccttattaggttctccatccacatcttcgccgcctccctcggccaccgcacaagcagctccccgcgagcgccgaagcctcccgccct

SEQ ID NO: 8534 - RNA, 8119 nt, Homo sapiens
  source 1..8119: mol_type = other RNA
aaaagtaattgtggtttttgcctgcacttttaatggtaaaaaccgcaattactttttcagcaacctaataattacaattctaagtaatggagatacatatcttttataggcttcaatgagcaatacattagcataatgttttatttcatactgactttgaatattccttgtcaaaaatgcacttatactttggagttactatgtatgtttaggttactgtgttgtcatcagaaggctggagttatcatagcagagctttaatgacaaaatattatgagccttgtaaatagttttaaaaattgtccactaatatctatttgtcttgcaaaatttgcaattttactagtaattttcatcacttgctctttctacctctaatgtttctcagtctcctccattagatcttactgacttatcacatataaacaccttcctcagaaacagtccaataaaaattaaagaccaagaggtagaatctactggagccatcatgaattccagttctttttgttgttattgatttttcttttttttttttaaaaggcacacccttgacttttttttattgttaaaataaccagattctaatttcaggcagcaaaatcagttactgcaaaaagtcaataatcaaaaatcaatgtataattggttttcatcacctatagaattagtgaggtttatacccctcaagtgtttagtgattctattcagtcaacctaaaaaaaattgcctcttttctacttaaataaataatttatttatttattttgagacagagtttcgctctgttgcccaggccggagtgcagtggcacaatctcagctcactgcaacctccgcctcccaggtcaagcgattgattctcatgcctcagcctcccaaatagctgggattataggtgcccgccaccatgctcagctaatttttgtatttttagtagagatggcgtttcaccatgttggccaggctggtcttgaactgacctcaagtgatccgcccaccttggcctcccaaagtgtggggattactagtgtgagccaccacgcctggcctgcctgttttcattattacctgcctgttctcagtatgcaacatggcagtactattgacagtgaggtgctttggcatatcagataacttttccagttggtcaaggatcccttttctcttttcctcatttctgaactgcagaacaggaagtactaaagaagtggctcaggacaatgttgtcacatcaggagtggcagaggtgtttactaggattatgatcctttcagctgtgtgtcttagaaggatctcctgaagccctgggtttgatatagaaaccataagaaaaagacttggggcagttctatatctggctcttctcccacttctcccataaaagattaagaaaaactgatgggatgatttcagatgtttcattgccaccaaactacagccatgagttttttttctttaagtgatcttatgaggccagtaaaggcctctgtcttgattaatgatgatcatcctataatatctggatatggtggcttgacatgagttttcaacaaagaaaattagtctctgaaagacatttctcatctgaaactctcaatatattaaaatgcatttaaaagttacttctgggaaacatactaaataggccaatcagttaatcattagctaattgtcaaaccctataaaatcatggtataatgtcaccctgacataaagcaacatcaaaattagtgcatcatctataaagtgaagtattattttctcccaagtgacaaattctattgccaaaaaataccactgtacttctaataagtgacactcattttaatagaccctacaaaaatacaatattttcaatgtccccataaaacagttaacttacaaatattattctcagagctctggtgacatcattcagtgatactattgtgaaaatcctcatacaatacttgaaacactagcatgtaaagtaaattcattatataacaaaagaactatgtaaaattatgaaagataatgcatgcaaccaactccgggaaattatcctggaaattcaaattaatattgtaattaaattaatgactaatatgaaagataagtattttaaaggattataaaataaattttgatcatttatgcaggaaaatagtttcaatggaaaagtaaataattctacattaaccatgcttgtctttctcttcagtgaaaaagcattcaggattttacataccttgaaactgtttttggaaaaaaagtattttatctatttctgcccagaaaaacagccattgaaattaatgatacaggtagaccacagctctgagaaattatatttgaagtttcatatttaaataccaaggatttaaaatcacctaccataactttctaacagcagtctttcgtaatgataaattttatcaatttccaaaattcgttttaaataatttaaaaagcagcaaattagattaagcaacacacaaataaattccacatttacaagtaaagaaatcacaggggctacagtttataatcaacatgaacttgaaagaaataaagcaatacctttcctgccacccatcatccactgcttaaatttgtggtgaaaaagacttaactacaatgacctttagtctgtttctaaactctgcatgtattgtaattagctaaaggcattgaacaaattagttcatcctatttttatttgggtcccagagataaatggctaatttatgaaatatttcactctgtgtcatgagaatttagcaaatgaatatggaaccaaatataaacactttataccatatgtacagttactttcataaggcattatcatgtaatttttattgaaaaagattcaatatagtaaagtcttattttaagatatattttttctctatctgagatgtttagtttatgaaaatattgtttttctctatattctttttgtatatatgccaacatataccttgtgctagaaatattttatgggaattacaattctttatatttgtattttctatataaaggcatatacaactttgaggcagtgtttctgatggagagcagaattcataaagagcttgtgtgtgcttccgtgctccgaaattatatgaaatccattttgagaagaaacttatttgattaaaaacaaaaacaaaaacagaaacaaaactgcaccaatgcacagccagaggctgacaattaaaactaatacataaccacatgaacatcatatttatagagttaacattttttaaggatggtcagtgctaacatatagtattatacatttggcactaatgtttgccattggtccagcaattggcaaaatttgtttctatgtataaatttatttttgaacattaggtctggctagacgtatcttcactatttataaaaaatatttagacagtaagctcacgttgaataactaggtctactgtgttctggaaactcttcagtagtaatacagctttttcatgttccatatgtacaaaactgtgtccatttgcctgaaggatcttatcaccaggctgcagtaggtttgatgctggcccatcaggctgaacccttgtcagaaggtttgaatggatttccttgtccactaattccaccactgatactaaatccaaggccaggattcttttctattctcacacaaaactgctctggatatccatccatactcctttgccctttagtttgaattaagcaccgtccaggctgaggtccccgggtggcctgtgaagaggggatctgaataggcaatggtgactgaaattgctggatggtcactttgtttatatttccttcatacggctgctgctcccggctgcgatgctgaaggctttgggaccccatcaacgtctggatgtggctgcctgccttcttagtaatggtgtccggaggtacatcccgcctcccaagtggataaggattccattggccactaggagatacatcttcttgtccattgtctaaaatgttgctttgctgggacggggtcctgtctaaccgtctagcttctatatgtctaagcagctgttgtctccagtctgcaggcattttaccacagctctcctctcccttcacaggagtaggcctcgtctttaaatcactgttatctgatggcttgtcaccatagttacccaagttatagtcagatggtattttttccaaaagagctgccatagtaggcctagctgaaactggcctggtttgggaggcaccgtaactctctgtactgtagcttctcgcagacaatggcctcctttgggtaaggtttttaaccggaaaacttcccgcctgagctttcacttcttgatatgaagggtgttcatcttcatacctgccattccttttcaggaactgggactcagtcactgtaacgctgctttggcgatccagccctcccctatatgggggtctgccgtacctatcagttgggggcagctcatgaggctcattgacccttctaaacatggccatttctgtggcgctcaccagggagtcggcccttctcaggaagcccgccctggccccttggcttgcgaactgggcattcaccacagcatcctcattcacagatggctgagaaaatgaaaacatttgctccatcggtgggtatcctctgtaagctctaggactaatcaaatccttggcgatgtttttgctggcctgttgcacgtactcgggattgtgttgaaaagggggtggtatcctcttttcggctttcacttccactgatccttgaggattgaagctttggtcaaactgatagactttttttgtcatagaagctttttgttgttgtggccccttactacttccgtaggtgagcatctcatcatccagcattgggactgactggcttcgagacatactggacataccatgctctggtcccagcatcttatccggtcgttcgtggcttcctaagtgatcactcccagaagcatagttttctaatggtatgttatacaccttatatgtaccaatgtcaatctcatcgatactctgtgactttttgaatttattagacttgatatctttcattaggggggaaagcctctctgtgcttttgctaattgaaataacacctttagaagattccgggcggcagtggatttgagaaaagacattactaagactcctgttgggattggaatcatgatactcccatggtacgcctggagaaaaaggactaggtatttcagtagattcctttatatgttctttcctttcaggcaatgggctggtagtgggggttgtctctaatttggaaggaaaagcggtcctgtcttcaaacggactaggggttctggtccaattctgccaaggattggaaggaggcacttctgtttctggtgtgtgtctgtgtgtagactgctcgagttccaggggaacaccaacaatcctgtcttgcctgatcaaaggcctgcgtccatgcgaagatgtgcttctagatttcgaacttaagagaggattactgttggcattctcggctgtggtttcctcagcaacaaaccctgtgttgtcataatgcgagccatcagtccagttgtcagtgaaagtatcactcatgggcagccggtcaggacgctgtggtatattgcctgggggaacagcctcccgctggctgagtaatggctttgaatcaagaggctgtgggaaagatggtgcaatcctgttaccccacaaagaattatgtactgcatctttagctgttgtctgcaaggaccccactttaacccgggtattagaggatcctgaggaagcctgggaaggcgagtagtctgagtaagtgcctgaggaaacactgttattcagacagtgagttttgtcaacttcagactcatcagttgattcttttttgtccttccctagcagaacaagtttgggtgggtacagaggggtctcagctaatgaagggtgaagttccccaatcctcatttcattagctggatgaacaaaagaatcctccactgtaatctcctttggggctaccggccacttgtgttcatatttttctttcacagtttgctccgtgttagcagttggatttgaattctcaacacgcactccatggcttggcttacccaccaaattttgaacagattttaccatattctttaaatcctctgggtaaggagttggatatcgttttaggtttatttcaacctgtctgccacttagagagggaagagtggtggattgtgctgcaactggcaatggagtacacatgctcctttcctgctggaggccacttatacaaccccatgccagctgtgggtcattctgggggacgggcatatcttggatctgctgatcacacctggcccatggtgtgcagcaatcgccagacagtctggcaggttggagagtaatcccacgctggcccctttcccagggggcttggcaggagagatccttaactttcccagcattttcgtcatcttcttttttgtcttcaaattcaaaggcaacagtcatgcgttgttgtctctgctcttcccacagtgtagggttaaagctgtcactgtctgactggaaatcttcatcaccacgaggctgctggggaaacatgtagttagtcaatactctttgctttgtttctggatgggcttctgtttgtaaagggataagggctttggactgattgtcagaaagccacaaagctgcaagctctttaagtttggtaaatgagaatggtaaattcttcaatctgttgtcactcaaatttaggactcttagtttctgcatctgtccaatctcttcaggaagaaattctaatttgttggagcgtagagacatgactgttacattcttacaacttccaatttctctgggtaattctggaaggaaattctcatcaactgctaatgtccgaagactatgaaggtagccaatagtagaaggtagtgactccagttcattacagctacagtcaaattcttctaataaagataaatttccaattgtattgggtagcattgtaagttgattgtcatctacttttagagttgttagttttttcaaaagtcctatagaatcaggcaattgttgcaacatattggatgacaataagaggtcctcaagggcttcacatccagaaatgtccatgtcaactgtttctattctgttttttgacatatccaggtataccaacatctttaacttccctatagacccaggtaacacttgtaatgcattattatccatccataactccctcaaattttgtatttgatccagaacttcaggcagctcaccgaattcattattgcctaggtcaagtctttccaactgggccagtttgtgcattgactttggtagagttttcaagtgattttctcttaactccaagatccgcaatttgacaagtcttccaaaattggctggaagaaattcaagaaaggcgtcattcaggtagagctgggtcaggtttaggagctgtgtgaagccatcaggtagtttagaaatgggattgacactggcttcaataattgttaaacacttacagcactttatgttttctggaaattcttgtacaccatttttactgatgtcgagttctttaagattaactaaactagcaatagtggttggcagatttgaaaggtcgttatcaggaatacttagttttcgtagagcttgacagttgaacaattgcttgggtagttcttcaatttgattggcatctagataaagctcctctaatgttcgttcgaagttaaagacctcctttggcacctgctgaagactgcagtgggagtaatctaaaactgagatgatttcttcttcacctcggaaacatcggcatggcaccagacggccgatgattttccgtttggtggtcatctccaggcactgcattgctagttattcctgtctctgcagacttctaggttgtgaccactttgacttgcattttttttcatgtagcgggctcactcctcttcaggcctcttccgaagtgctgcacgaacctctttacaaggacttctctggtattgcgggggattccttccccttattaggttctccatccacatcttcgccgcctccctcggccaccgcacaagcagctccccgcgagcgccgaagcctcccgccct

SEQ ID NO: 8535 - RNA, 73 nt, Homo sapiens
  source 1..73: mol_type = other RNA
aaaagtaattgtggtttttgcctgtaaaagtaatggcaaaaaccacagtttcttttgcaccagactaataaag

SEQ ID NO: 8536 - RNA, 64 nt, Homo sapiens
  source 1..64: mol_type = other RNA
aaaagtaattgtggtttttgtcattaaaaaattgcaaaaaccacgatcacttttgcaccaccct

SEQ ID NO: 8537 - RNA, 76 nt, Homo sapiens
  source 1..76: mol_type = other RNA
aaaagtaattgtggtttttgttattggttttaatgacaaagaccgcaattacttttgcaccaacctaggaattggt

SEQ ID NO: 8538 - RNA, 4635 nt, Homo sapiens
  source 1..4635: mol_type = other RNA
aaaagtgcttacagtgcaggtagaaactctgtaaccttaagcatgtaaactacatagaataaaactgtttccactgcatttctgtccttcaaagtggccaacctgattaagtcagccttaatcactgctgctgtcagtttcacgactaaaggtcatattgactaagtagtcatcagctgaccacctcgctgtatcagccagcaacgaggggaaggtgaagaaacatgataggccatatagaatctgccctatgtttacttttttaacccagataattatttttgtgtgcagtatctaagctcctgattgtgtaacctgggacttctggcaccttttgttccattcattttatgtataaaatgcatgccaaagcacactgtgccctctggtacccttgcttccaatcgccaaccatgctcatttccttcctttttttgtggtccctttttgtggtgatcattttaaaccacgtcatccaacaaatgttttatggtcaaccttagcttgttcataagccatagcaactgaaagattaaactcttaaatatgtgtctgggcagtggctattaaatagcaaaaaacaatcagattttagtattttattatttccttgtaaaatggctgaactaaattaaacccttgtttcccatttgttctataatttatagtgaaactgagaacaaaactatctttataaatgatagctaaaagtatttccagatatttaaacaatttaaaataaatttcttctgcagagatgcaaagcatctcaacactggaatgaacaaatgccttaaattcaatggagtaaacctttagaatgaagaggaactgtcatttcacccaagccgaagacaacagccttatgcacttgtgtgctctgtctttgctgcttctcgtgtttcaagcctttcctgtgggatcagcacagcaaagtgcaacttaccaaatggtttaatgactggttaattctttcttctcccaatggaaaagcaatggcaacacaacagtagactgctggcttgacaatcttaaacgtgagcctttgcacatgtaggtttatcatcatttgagtatacgactaagcaagtcaatgaactttttttttttttttagcagtttaatttggtcctgagaatgttgcagtctttattaccccttttgcattaatccacttttctaaccaccttttaagctttaatttttaacactatacaccaagtctttgaaatcagtgatctgttatttaactctaaagcatttgacacttcttgccttaacagttttaaaaaccacacacaaaaaaactctgtaagtaatacagtaggccaaaagtttcatcctatctatcttgcagtttacctatctgatctgatctctgtaattatagttctgtcatttaaaatatactatttaaatctaatttttacatttcaaaaattatcttcagtagtaactaagtatattttctgtggattctgagaatgttatttttcagaatgtgagaatatatatgtacatttataatcttgtgactttaaagtctgttttcagatacagtatgtaaatacttgtaaaaaaatttgtataattttgtgataatgtagtttcccaaaaaaattatttagaaggcattatgttattagtaaatgagagcactgtatagaactgttcctattttctgcacttgccattccagctgcctccactgtccatacccacctcattcatcctgtcacagaaggcaggaaaactgggaactttaccaaagtagcactcagcctgagaggcctgtataatcatgcttttcaaactaaattcacttaaaaattaaaaagcagaattgaatattttaagcagcctcagtacctttggccaatgctgttttcatggtggattatgaacattatataatctttgggaaaagtgaaagtagtacaatttttagaataatgacaactgcctcactgcatctctccactcacacagcaaccgtgtagccccctaagctgcagtaccatgactaaccatgatgtcaatttcatatgctgatcctcacaacagcagtgcacaaacatgccccaaatattttaacagaatttagctcttccttaagctgtcttttcatagtaaaaacaaaacaaaaacacccaatgttaaaaccacataataaacttacaaacttgaaaaattagacacttcagatagataggcaataaaacttcatattatgaaagcaatatattccaagtttcaaagatttgacaagttctgtagagtatctttcatcagtacatgaaaacttccaaactgcatgatcttctgccaggcaggactgggtgctattcgctggtttgaggtcgaatccatttcaaggcatgtcgtggtgggacattaatggtgggatggtagaatgtgcagtccggtcttgtacattgagtgttaaacctacaatgttttggatgatagaagggacattccatcttcttacaagcagggaagtaacggcagagctgactactggaaggtggtgctggtggtgcaactgctggttttggagacagtactggaattcttctactcacatgagtgaagggacaatctggtttagtacactttgcatcatatttacaatttgggtgaacaaacaaacatttttcagcaaatttacaattggggaaggctttgcagggtgagatggggtgatggtaggcacactcatccccatttttacaagcaggccagtacttgcagcgctccaaaagtttttctggtttctgtgccacactcagttcactcatctcagcatttgggtcctcaagctgcctgctcagcaagtgcaactgctgtgggtggaggagacctctgagtcccttgtttgaggctgcagtttggtttacgggtttcattccttcaaagcacatgtcctcctcttgatctgacatgtatcctggggggctggggacaccatccagcgtcactataaacttgggacttgcaggtttatctggttgtacaagatctcgtgtctgcataaggtgtcctgaaagtacccgaagggaatctgcagtcttcatccccgactcttggtttggtgccactactacttcctcagacagctttggcttcttcagaataaatgatcttgtgtctgcatggaccatggattccatgtcatagtaatcttgactcatctgcagagtttctgccattactgggtcgatttgcagtcgggataataattgcctctgttgagttccttgatttttttctacagaatctccttttgtttcctcttctttaatggggggacttattctgggggtcctactttgtccctggaccacttctgctagcaattcttcttgagaagttcgagttctgggagcaactggaagtgtctgtttctgtggaactgtagagtagttagttgtttttgttacggattcttgagcttcagatatagccttcaaaatcagattcttgttagcttgtttagaaggtggaagagaaggtctcctttcaggctttgcaggcacagacacactgctggagatgcttcctgttcgagacccgtaatcatcatcttcttcctcctcttctccatcatgattgaatttttttactttaacaactgaacttaccacaggcaactttctcttccgaaagttttcatcctccatactcattttctccgagttgtttctaaagaacggactatacgtttcttctaagctgttaagcacctctggttcacacaaacgtcctgtttcatatacccaactactctgcatatcaagctgcttggcagcatgaatactattctgctgctgttgaaattgcaacctgtttaaatgaacaccactatctgcatttctacttgcaggtggtcgataaatttcaatagaagggcgagaagaaccatatgtaagtgtcactgtaggttttttctgagataagggattctcctgcacaaagttgaggtcttcgtcaatgagatcatctggttctggcttaatatcaatcacatcttcagagggtgctggctccctcaaaggtttcactgttgacattagtcgggttgcagctccatcatcgtaagtctgtctgacatttgtggtttttgactcctgcgaacttgtagaaactctggaatctcttttttcaggtctcgcgctaggaatggcaagtggtggcactgcagcttcatgcctcctctcatctccccgactgaaattgctcttgtttgaaggcacgttactatcaaagatgttggtatcagaagacttcagactagagggttcagttgtaacagagcgaagtttatctaatacaccatgaagccatacggtgaatcgaattgtgttgttccctagaaacagggacagatcctctgtcatttggtcctgacttttcttgttggccaccatcaccataatgtaatcaggaagttcttcatcaacataagctcctaattcttgtaatttccccttaatggcactccggatcttgcggctgatctcggtgccgatctccatggctctgcggcgtgcgggaactcagcactgcgcggcgcttggcttacccggaggctgccgcggactcctaccccgcagccgggacaccaccgcctcc

SEQ ID NO: 8539 - RNA, 4560 nt, Homo sapiens
  source 1..4560: mol_type = other RNA
aaaagtgcttacagtgcaggtagaaactctgtaaccttaagcatgtaaactacatagaataaaactgtttccactgcatttctgtccttcaaagtggccaacctgattaagtcagccttaatcactgctgctgtcagtttcacgactaaaggtcatattgactaagtagtcatcagctgaccacctcgctgtatcagccagcaacgaggggaaggtgaagaaacatgataggccatatagaatctgccctatgtttacttttttaacccagataattatttttgtgtgcagtatctaagctcctgattgtgtaacctgggacttctggcaccttttgttccattcattttatgtataaaatgcatgccaaagcacactgtgccctctggtacccttgcttccaatcgccaaccatgctcatttccttcctttttttgtggtccctttttgtggtgatcattttaaaccacgtcatccaacaaatgttttatggtcaaccttagcttgttcataagccatagcaactgaaagattaaactcttaaatatgtgtctgggcagtggctattaaatagcaaaaaacaatcagattttagtattttattatttccttgtaaaatggctgaactaaattaaacccttgtttcccatttgttctataatttatagtgaaactgagaacaaaactatctttataaatgatagctaaaagtatttccagatatttaaacaatttaaaataaatttcttctgcagagatgcaaagcatctcaacactggaatgaacaaatgccttaaattcaatggagtaaacctttagaatgaagaggaactgtcatttcacccaagccgaagacaacagccttatgcacttgtgtgctctgtctttgctgcttctcgtgtttcaagcctttcctgtgggatcagcacagcaaagtgcaacttaccaaatggtttaatgactggttaattctttcttctcccaatggaaaagcaatggcaacacaacagtagactgctggcttgacaatcttaaacgtgagcctttgcacatgtaggtttatcatcatttgagtatacgactaagcaagtcaatgaactttttttttttttttagcagtttaatttggtcctgagaatgttgcagtctttattaccccttttgcattaatccacttttctaaccaccttttaagctttaatttttaacactatacaccaagtctttgaaatcagtgatctgttatttaactctaaagcatttgacacttcttgccttaacagttttaaaaaccacacacaaaaaaactctgtaagtaatacagtaggccaaaagtttcatcctatctatcttgcagtttacctatctgatctgatctctgtaattatagttctgtcatttaaaatatactatttaaatctaatttttacatttcaaaaattatcttcagtagtaactaagtatattttctgtggattctgagaatgttatttttcagaatgtgagaatatatatgtacatttataatcttgtgactttaaagtctgttttcagatacagtatgtaaatacttgtaaaaaaatttgtataattttgtgataatgtagtttcccaaaaaaattatttagaaggcattatgttattagtaaatgagagcactgtatagaactgttcctattttctgcacttgccattccagctgcctccactgtccatacccacctcattcatcctgtcacagaaggcaggaaaactgggaactttaccaaagtagcactcagcctgagaggcctgtataatcatgcttttcaaactaaattcacttaaaaattaaaaagcagaattgaatattttaagcagcctcagtacctttggccaatgctgttttcatggtggattatgaacattatataatctttgggaaaagtgaaagtagtacaatttttagaataatgacaactgcctcactgcatctctccactcacacagcaaccgtgtagccccctaagctgcagtaccatgactaaccatgatgtcaatttcatatgctgatcctcacaacagcagtgcacaaacatgccccaaatattttaacagaatttagctcttccttaagctgtcttttcatagtaaaaacaaaacaaaaacacccaatgttaaaaccacataataaacttacaaacttgaaaaattagacacttcagatagataggcaataaaacttcatattatgaaagcaatatattccaagtttcaaagatttgacaagttctgtagagtatctttcatcagtacatgaaaacttccaaactgcatgatcttctgccaggcaggactgggtgctattcgctggtttgaggtcgaatccatttcaaggcatgtcgtggtgggacattaatggtgggatggtagaatgtgcagtccggtcttgtacattgagtgttaaacctacaatgttttggatgatagaagggacattccatcttcttacaagcagggaagtaacggcagagctgactactggaaggtggtgctggtggtgcaactgctggttttggagacagtactggaattcttctactcacatgagtgaagggacaatctggtttagtacactttgcatcatatttacaatttgggtgaacaaacaaacatttttcagcaaatttacaattggggaaggctttgcagggtgagatggggtgatggtaggcacactcatccccatttttacaagcaggccagtacttgcagcgctccaaaagtttttctggtttctgtgccacactcagttcactcatctcagcatttgggtcctcaagctgcctgctcagcaagtgcaactgctgtgggtggaggagacctctgagtcccttgtttgaggctgcagtttggtttacgggtttcattccttcaaagcacatgtcctcctcttgatctgacatgtatcctggggggctggggacaccatccagcgtcactataaacttgggacttgcaggtttatctggttgtacaagatctcgtgtctgcataaggtgtcctgaaagtacccgaagggaatctgcagtcttcatccccgactcttggtttggtgccactactacttcctcagacagctttggcttcttcagaataaatgatcttgtgtctgcatggaccatggattccatgtcatagtaatcttgatttttttctacagaatctccttttgtttcctcttctttaatggggggacttattctgggggtcctactttgtccctggaccacttctgctagcaattcttcttgagaagttcgagttctgggagcaactggaagtgtctgtttctgtggaactgtagagtagttagttgtttttgttacggattcttgagcttcagatatagccttcaaaatcagattcttgttagcttgtttagaaggtggaagagaaggtctcctttcaggctttgcaggcacagacacactgctggagatgcttcctgttcgagacccgtaatcatcatcttcttcctcctcttctccatcatgattgaatttttttactttaacaactgaacttaccacaggcaactttctcttccgaaagttttcatcctccatactcattttctccgagttgtttctaaagaacggactatacgtttcttctaagctgttaagcacctctggttcacacaaacgtcctgtttcatatacccaactactctgcatatcaagctgcttggcagcatgaatactattctgctgctgttgaaattgcaacctgtttaaatgaacaccactatctgcatttctacttgcaggtggtcgataaatttcaatagaagggcgagaagaaccatatgtaagtgtcactgtaggttttttctgagataagggattctcctgcacaaagttgaggtcttcgtcaatgagatcatctggttctggcttaatatcaatcacatcttcagagggtgctggctccctcaaaggtttcactgttgacattagtcgggttgcagctccatcatcgtaagtctgtctgacatttgtggtttttgactcctgcgaacttgtagaaactctggaatctcttttttcaggtctcgcgctaggaatggcaagtggtggcactgcagcttcatgcctcctctcatctccccgactgaaattgctcttgtttgaaggcacgttactatcaaagatgttggtatcagaagacttcagactagagggttcagttgtaacagagcgaagtttatctaatacaccatgaagccatacggtgaatcgaattgtgttgttccctagaaacagggacagatcctctgtcatttggtcctgacttttcttgttggccaccatcaccataatgtaatcaggaagttcttcatcaacataagctcctaattcttgtaatttccccttaatggcactccggatcttgcggctgatctcggtgccgatctccatggctctgcggcgtgcgggaactcagcactgcgcggcgcttggcttacccggaggctgccgcggactcctaccccgcagccgggacaccaccgcctcc

SEQ ID NO: 8540 - RNA, 4535 nt, Homo sapiens
  source 1..4535: mol_type = other RNA
aaaagtgcttacagtgcaggtagaaactctgtaaccttaagcatgtaaactacatagaataaaactgtttccactgcatttctgtccttcaaagtggccaacctgattaagtcagccttaatcactgctgctgtcagtttcacgactaaaggtcatattgactaagtagtcatcagctgaccacctcgctgtatcagccagcaacgaggggaaggtgaagaaacatgataggccatatagaatctgccctatgtttacttttttaacccagataattatttttgtgtgcagtatctaagctcctgattgtgtaacctgggacttctggcaccttttgttccattcattttatgtataaaatgcatgccaaagcacactgtgccctctggtacccttgcttccaatcgccaaccatgctcatttccttcctttttttgtggtccctttttgtggtgatcattttaaaccacgtcatccaacaaatgttttatggtcaaccttagcttgttcataagccatagcaactgaaagattaaactcttaaatatgtgtctgggcagtggctattaaatagcaaaaaacaatcagattttagtattttattatttccttgtaaaatggctgaactaaattaaacccttgtttcccatttgttctataatttatagtgaaactgagaacaaaactatctttataaatgatagctaaaagtatttccagatatttaaacaatttaaaataaatttcttctgcagagatgcaaagcatctcaacactggaatgaacaaatgccttaaattcaatggagtaaacctttagaatgaagaggaactgtcatttcacccaagccgaagacaacagccttatgcacttgtgtgctctgtctttgctgcttctcgtgtttcaagcctttcctgtgggatcagcacagcaaagtgcaacttaccaaatggtttaatgactggttaattctttcttctcccaatggaaaagcaatggcaacacaacagtagactgctggcttgacaatcttaaacgtgagcctttgcacatgtaggtttatcatcatttgagtatacgactaagcaagtcaatgaactttttttttttttttagcagtttaatttggtcctgagaatgttgcagtctttattaccccttttgcattaatccacttttctaaccaccttttaagctttaatttttaacactatacaccaagtctttgaaatcagtgatctgttatttaactctaaagcatttgacacttcttgccttaacagttttaaaaaccacacacaaaaaaactctgtaagtaatacagtaggccaaaagtttcatcctatctatcttgcagtttacctatctgatctgatctctgtaattatagttctgtcatttaaaatatactatttaaatctaatttttacatttcaaaaattatcttcagtagtaactaagtatattttctgtggattctgagaatgttatttttcagaatgtgagaatatatatgtacatttataatcttgtgactttaaagtctgttttcagatacagtatgtaaatacttgtaaaaaaatttgtataattttgtgataatgtagtttcccaaaaaaattatttagaaggcattatgttattagtaaatgagagcactgtatagaactgttcctattttctgcacttgccattccagctgcctccactgtccatacccacctcattcatcctgtcacagaaggcaggaaaactgggaactttaccaaagtagcactcagcctgagaggcctgtataatcatgcttttcaaactaaattcacttaaaaattaaaaagcagaattgaatattttaagcagcctcagtacctttggccaatgctgttttcatggtggattatgaacattatataatctttgggaaaagtgaaagtagtacaatttttagaataatgacaactgcctcactgcatctctccactcacacagcaaccgtgtagccccctaagctgcagtaccatgactaaccatgatgtcaatttcatatgctgatcctcacaacagcagtgcacaaacatgccccaaatattttaacagaatttagctcttccttaagctgtcttttcatagtaaaaacaaaacaaaaacacccaatgttaaaaccacataataaacttacaaacttgaaaaattagacacttcagatagataggcaataaaacttcatattatgaaagcaatatattccaagtttcaaagatttgacaagttctgtagagtatctttcatcagtacatgaaaacttccaaactgcatgatcttctgccaggcaggactgggtgctattcgctggtttgaggtcgaatccatttcaaggcatgtcgtggtgggacattaatggtgggatggtagaatgtgcagtccggtcttgtacattgagtgttaaacctacaatgttttggatgatagaagggacattccatcttcttacaagcagggaagtaacggcagagctgactactggaaggtggtgctggtggtgcaactgctggttttggagacagtactggaattcttctactcacatgagtgaagggacaatctggtttagtacactttgcatcatatttacaatttgggtgaacaaacaaacatttttcagcaaatttacaattggggaaggctttgcagggtgagatggggtgatggtaggcacactcatccccatttttacaagcaggccagtacttgcagcgctccaaaagtttttctggtttctgtgccacactcagttcactcatctcagcgttagaaaagctaccatttgggtcctcaagctgcctgctcagcaagtgcaactgctgtgggtggaggagacctctgagtcccttgtttgaggctgcagtttggtttacgggtttcattccttcaaagcacatgtcctcctcttgatctgacatgtatcctggggggctggggacaccatccagcgtcactataaacttgggacttgcaggtttatctggttgtacaagatctcgtgtctgcataaggtgtcctgaaagtacccgaagggaatctgcagtcttcatccccgactcttggtttggtgccactactacttcctcagacagctttggcttcttcagaataaatgatcttgtgtctgcatggaccatggattccatgtcatagtaatcttgactcatctgcagagtttctgccattactgggtcgatttgcagtcgggataataattgcctctgttgagttccttgatttttttctacagaatctccttttgtttcctcttctttaatggggggacttattctgggggtcctactttgtccctggaccacttctgctagcaattcttcttgagaagttcgagttctgggagcaactggaagtgtctgtttctgtggaactgtagagtagttagttgtttttgttacggattcttgagcttcagatatagccttcaaaatcagattcttgttagcttgtttagaaggtggaagagaaggtctcctttcaggctttgcaggcacagacacactgctggagatgcttcctgttcgagacccgtaatcatcatcttcttcctcctcttctccatcatgattgaatttttttactttaacaactgaacttaccacaggcaactttctcttccgaaagttttcatcctccatactcattttctccgagttgtttctaaagaacggactatacgtttcttctaagctgttaagcacctctggttcacacaaacgtcctgtttcatatacccaactactctgcatatcaagctgcttggcagcatgaatactattctgctgctgttgaaattgcaacctgtttaaatgaacaccactatctgcatttctacttgcaggtggtcgataaatttcaatagaagggcgagaagaaccatatgtaagtgtcactgtaggttttttctgagataagggattctcctgcacaaagttgaggtcttcgtcaatgagatcatctggttctggcttaatatcaatcacatcttcagagggtgctggctccctcaaaggtttcactgttgacattagtcgggttgcagctccatcatcgtaagtctgtctgacatttgtggtttttgactcctgcgaacttgtagaaactctggaatctcttttttcaggtctcgcgctaggaatggcaagtggtggcactgcagcttcatgcctcctctcatctccccgactgaaattgctcttgtttgaaggcacgttactatcaaagatgttggtatcagaagacttcagactagagggttcagttgtaacagagcgaagtttatctaatacaccatgaagccaacataagctcctaattcttgtaatttccccttaatggcactccggatcttgcggctgatctcggtgccgatctccatggctctgcggcgtgcgggaactcagcactgcgcggcgcttggcttacccggaggctgccgcggactcctaccccgcagccgggacaccaccgcctcc

SEQ ID NO: 8541 - RNA, 4650 nt, Homo sapiens
  source 1..4650: mol_type = other RNA
aaaagtgcttacagtgcaggtagaaactctgtaaccttaagcatgtaaactacatagaataaaactgtttccactgcatttctgtccttcaaagtggccaacctgattaagtcagccttaatcactgctgctgtcagtttcacgactaaaggtcatattgactaagtagtcatcagctgaccacctcgctgtatcagccagcaacgaggggaaggtgaagaaacatgataggccatatagaatctgccctatgtttacttttttaacccagataattatttttgtgtgcagtatctaagctcctgattgtgtaacctgggacttctggcaccttttgttccattcattttatgtataaaatgcatgccaaagcacactgtgccctctggtacccttgcttccaatcgccaaccatgctcatttccttcctttttttgtggtccctttttgtggtgatcattttaaaccacgtcatccaacaaatgttttatggtcaaccttagcttgttcataagccatagcaactgaaagattaaactcttaaatatgtgtctgggcagtggctattaaatagcaaaaaacaatcagattttagtattttattatttccttgtaaaatggctgaactaaattaaacccttgtttcccatttgttctataatttatagtgaaactgagaacaaaactatctttataaatgatagctaaaagtatttccagatatttaaacaatttaaaataaatttcttctgcagagatgcaaagcatctcaacactggaatgaacaaatgccttaaattcaatggagtaaacctttagaatgaagaggaactgtcatttcacccaagccgaagacaacagccttatgcacttgtgtgctctgtctttgctgcttctcgtgtttcaagcctttcctgtgggatcagcacagcaaagtgcaacttaccaaatggtttaatgactggttaattctttcttctcccaatggaaaagcaatggcaacacaacagtagactgctggcttgacaatcttaaacgtgagcctttgcacatgtaggtttatcatcatttgagtatacgactaagcaagtcaatgaactttttttttttttttagcagtttaatttggtcctgagaatgttgcagtctttattaccccttttgcattaatccacttttctaaccaccttttaagctttaatttttaacactatacaccaagtctttgaaatcagtgatctgttatttaactctaaagcatttgacacttcttgccttaacagttttaaaaaccacacacaaaaaaactctgtaagtaatacagtaggccaaaagtttcatcctatctatcttgcagtttacctatctgatctgatctctgtaattatagttctgtcatttaaaatatactatttaaatctaatttttacatttcaaaaattatcttcagtagtaactaagtatattttctgtggattctgagaatgttatttttcagaatgtgagaatatatatgtacatttataatcttgtgactttaaagtctgttttcagatacagtatgtaaatacttgtaaaaaaatttgtataattttgtgataatgtagtttcccaaaaaaattatttagaaggcattatgttattagtaaatgagagcactgtatagaactgttcctattttctgcacttgccattccagctgcctccactgtccatacccacctcattcatcctgtcacagaaggcaggaaaactgggaactttaccaaagtagcactcagcctgagaggcctgtataatcatgcttttcaaactaaattcacttaaaaattaaaaagcagaattgaatattttaagcagcctcagtacctttggccaatgctgttttcatggtggattatgaacattatataatctttgggaaaagtgaaagtagtacaatttttagaataatgacaactgcctcactgcatctctccactcacacagcaaccgtgtagccccctaagctgcagtaccatgactaaccatgatgtcaatttcatatgctgatcctcacaacagcagtgcacaaacatgccccaaatattttaacagaatttagctcttccttaagctgtcttttcatagtaaaaacaaaacaaaaacacccaatgttaaaaccacataataaacttacaaacttgaaaaattagacacttcagatagataggcaataaaacttcatattatgaaagcaatatattccaagtttcaaagatttgacaagttctgtagagtatctttcatcagtacatgaaaacttccaaactgcatgatcttctgccaggcaggactgggtgctattcgctggtttgaggtcgaatccatttcaaggcatgtcgtggtgggacattaatggtgggatggtagaatgtgcagtccggtcttgtacattgagtgttaaacctacaatgttttggatgatagaagggacattccatcttcttacaagcagggaagtaacggcagagctgactactggaaggtggtgctggtggtgcaactgctggttttggagacagtactggaattcttctactcacatgagtgaagggacaatctggtttagtacactttgcatcatatttacaatttgggtgaacaaacaaacatttttcagcaaatttacaattggggaaggctttgcagggtgagatggggtgatggtaggcacactcatccccatttttacaagcaggccagtacttgcagcgctccaaaagtttttctggtttctgtgccacactcagttcactcatctcagcgttagaaaagctaccatttgggtcctcaagctgcctgctcagcaagtgcaactgctgtgggtggaggagacctctgagtcccttgtttgaggctgcagtttggtttacgggtttcattccttcaaagcacatgtcctcctcttgatctgacatgtatcctggggggctggggacaccatccagcgtcactataaacttgggacttgcaggtttatctggttgtacaagatctcgtgtctgcataaggtgtcctgaaagtacccgaagggaatctgcagtcttcatccccgactcttggtttggtgccactactacttcctcagacagctttggcttcttcagaataaatgatcttgtgtctgcatggaccatggattccatgtcatagtaatcttgactcatctgcagagtttctgccattactgggtcgatttgcagtcgggataataattgcctctgttgagttccttgatttttttctacagaatctccttttgtttcctcttctttaatggggggacttattctgggggtcctactttgtccctggaccacttctgctagcaattcttcttgagaagttcgagttctgggagcaactggaagtgtctgtttctgtggaactgtagagtagttagttgtttttgttacggattcttgagcttcagatatagccttcaaaatcagattcttgttagcttgtttagaaggtggaagagaaggtctcctttcaggctttgcaggcacagacacactgctggagatgcttcctgttcgagacccgtaatcatcatcttcttcctcctcttctccatcatgattgaatttttttactttaacaactgaacttaccacaggcaactttctcttccgaaagttttcatcctccatactcattttctccgagttgtttctaaagaacggactatacgtttcttctaagctgttaagcacctctggttcacacaaacgtcctgtttcatatacccaactactctgcatatcaagctgcttggcagcatgaatactattctgctgctgttgaaattgcaacctgtttaaatgaacaccactatctgcatttctacttgcaggtggtcgataaatttcaatagaagggcgagaagaaccatatgtaagtgtcactgtaggttttttctgagataagggattctcctgcacaaagttgaggtcttcgtcaatgagatcatctggttctggcttaatatcaatcacatcttcagagggtgctggctccctcaaaggtttcactgttgacattagtcgggttgcagctccatcatcgtaagtctgtctgacatttgtggtttttgactcctgcgaacttgtagaaactctggaatctcttttttcaggtctcgcgctaggaatggcaagtggtggcactgcagcttcatgcctcctctcatctccccgactgaaattgctcttgtttgaaggcacgttactatcaaagatgttggtatcagaagacttcagactagagggttcagttgtaacagagcgaagtttatctaatacaccatgaagccatacggtgaatcgaattgtgttgttccctagaaacagggacagatcctctgtcatttggtcctgacttttcttgttggccaccatcaccataatgtaatcaggaagttcttcatcaacataagctcctaattcttgtaatttccccttaatggcactccggatcttgcggctgatctcggtgccgatctccatggctctgcggcgtgcgggaactcagcactgcgcggcgcttggcttacccggaggctgccgcggactcctaccccgcagccgggacaccaccgcctcc

SEQ ID NO: 8542 - RNA, 4831 nt, Homo sapiens
  source 1..4831: mol_type = other RNA
aaaagtgcttacagtgcaggtagaaactctgtaaccttaagcatgtaaactacatagaataaaactgtttccactgcatttctgtccttcaaagtggccaacctgattaagtcagccttaatcactgctgctgtcagtttcacgactaaaggtcatattgactaagtagtcatcagctgaccacctcgctgtatcagccagcaacgaggggaaggtgaagaaacatgataggccatatagaatctgccctatgtttacttttttaacccagataattatttttgtgtgcagtatctaagctcctgattgtgtaacctgggacttctggcaccttttgttccattcattttatgtataaaatgcatgccaaagcacactgtgccctctggtacccttgcttccaatcgccaaccatgctcatttccttcctttttttgtggtccctttttgtggtgatcattttaaaccacgtcatccaacaaatgttttatggtcaaccttagcttgttcataagccatagcaactgaaagattaaactcttaaatatgtgtctgggcagtggctattaaatagcaaaaaacaatcagattttagtattttattatttccttgtaaaatggctgaactaaattaaacccttgtttcccatttgttctataatttatagtgaaactgagaacaaaactatctttataaatgatagctaaaagtatttccagatatttaaacaatttaaaataaatttcttctgcagagatgcaaagcatctcaacactggaatgaacaaatgccttaaattcaatggagtaaacctttagaatgaagaggaactgtcatttcacccaagccgaagacaacagccttatgcacttgtgtgctctgtctttgctgcttctcgtgtttcaagcctttcctgtgggatcagcacagcaaagtgcaacttaccaaatggtttaatgactggttaattctttcttctcccaatggaaaagcaatggcaacacaacagtagactgctggcttgacaatcttaaacgtgagcctttgcacatgtaggtttatcatcatttgagtatacgactaagcaagtcaatgaactttttttttttttttagcagtttaatttggtcctgagaatgttgcagtctttattaccccttttgcattaatccacttttctaaccaccttttaagctttaatttttaacactatacaccaagtctttgaaatcagtgatctgttatttaactctaaagcatttgacacttcttgccttaacagttttaaaaaccacacacaaaaaaactctgtaagtaatacagtaggccaaaagtttcatcctatctatcttgcagtttacctatctgatctgatctctgtaattatagttctgtcatttaaaatatactatttaaatctaatttttacatttcaaaaattatcttcagtagtaactaagtatattttctgtggattctgagaatgttatttttcagaatgtgagaatatatatgtacatttataatcttgtgactttaaagtctgttttcagatacagtatgtaaatacttgtaaaaaaatttgtataattttgtgataatgtagtttcccaaaaaaattatttagaaggcattatgttattagtaaatgagagcactgtatagaactgttcctattttctgcacttgccattccagctgcctccactgtccatacccacctcattcatcctgtcacagaaggcaggaaaactgggaactttaccaaagtagcactcagcctgagaggcctgtataatcatgcttttcaaactaaattcacttaaaaattaaaaagcagaattgaatattttaagcagcctcagtacctttggccaatgctgttttcatggtggattatgaacattatataatctttgggaaaagtgaaagtagtacaatttttagaataatgacaactgcctcactgcatctctccactcacacagcaaccgtgtagccccctaagctgcagtaccatgactaaccatgatgtcaatttcatatgctgatcctcacaacagcagtgcacaaacatgccccaaatattttaacagaatttagctcttccttaagctgtcttttcatagtaaaaacaaaacaaaaacacccaatgttaaaaccacataataaacttacaaacttgaaaaattagacacttcagatagataggcaataaaacttcatattatgaaagcaatatattccaagtttcaaagatttgacaagttctgtagagtatctttcatcagtacatgaaaacttccaaactgcatgatcttctgccaggcaggactgggtgctattcgctggtttgaggtcgaatccatttcaaggcatgtcgtggtgggacattaatggtgggatggtagaatgtgcagtccggtcttgtacattgagtgttaaacctacaatgttttggatgatagaagggacattccatcttcttacaagcagggaagtaacggcagagctgactactggaaggtggtgctggtggtgcaactgctggttttggagacagtactggaattcttctactcacatgagtgaagggacaatctggtttagtacactttgcatcatatttacaatttgggtgaacaaacaaacatttttcagcaaatttacaattggggaaggctttgcagggtgagatggggtgatggtaggcacactcatccccatttttacaagcaggccagtacttgcagcgctccaaaagtttttctggtttctgtgccacactcagttcactcatctcagcgttagaaaagctaccatttgggtcctcaagctgcctgctcagcaagtgcaactgctgtgggtggaggagacctctgagtcccttgtttgaggctgcagtttggtttacgggtttcattccttcaaagcacatgtcctcctcttgatctgacatgtatcctggggggctggggacaccatccagcgtcactataaacttgggacttgcaggtttatctggttgtacaagatctcgtgtctgcataaggtgtcctgaaagtacccgaagggaatctgcagtcttcatccccgactcttggtttggtgccactactacttcctcagacagctttggcttcttcagaataaatgatcttgtgtctgcatggaccatggattccatgtcatagtaatcttgactcatctgcagagtttctgccattactgggtcgatttgcagtcgggataataattgcctctgttgagttccttgatttttttctacagaatctccttttgtttcctcttctttaatggggggacttattctgggggtcctactttgtccctggaccacttctgctagcaattcttcttgagaagttcgagttctgggagcaactggaagtgtctgtttctgtggaactgtagagtagttagttgtttttgttacggattcttgagcttcagatatagccttcaaaatcagattcttgttagcttgtttagaaggtggaagagaaggtctcctttcaggctttgcaggcacagacacactgctggagatgcttcctgttcgagacccgtaatcatcatcttcttcctcctcttctccatcatgattgaatttttttactttaacaactgaacttaccacaggcaactttctcttccgaaagttttcatcctccatactcattttctccgagttgtttctaaagaacggactatacgtttcttctaagctgttaagcacctctggttcacacaaacgtcctgtttcatatacccaactactctgcatatcaagctgcttggcagcatgaatactattctgctgctgttgaaattgcaacctgtttaaatgaacaccactatctgcatttctacttgcaggtggtcgataaatttcaatagaagggcgagaagaaccatatgtaagtgtcactgtaggttttttctgagataagggattctcctgcacaaagttgaggtcttcgtcaatgagatcatctggttctggcttaatatcaatcacatcttcagagggtgctggctccctcaaaggtttcactgttgacattagtcgggttgcagctccatcatcgtaagtctgtctgacatttgtggtttttgactcctgcgaacttgtagaaactctggaatctcttttttcaggtctcgcgctaggaatggcaagtggtggcactgcagcttcatgcctcctctcatctccccgactgaaattgctcttgtttgaaggcacgttactatcaaagatgttggtatcagaagacttcagactagagggttcagttgtaacagagcgaagtttatctaatacaccatgaagccatacggtgaatcgaattgtgttgttccctagaaacagggacagatcctctgtcatttggtcctgacttttcttgttggccaccatcaccataatgtaatcaggaagttcttcatctatttaaaaggaaaggtagatcaaaactttgtttcctcaaaactttcttcttaaagttgatgtgcttgaaaatatagatgtagctctaagctttagagtcgcagagctctactggaattacattggacaagatggcttagctttaatttttttctcttcattccacaggtatttcaaatacaacataagctcctaattcttgtaatttccccttaatggcactccggatcttgcggctgatctcggtgccgatctccatggctctgcggcgtgcgggaactcagcactgcgcggcgcttggcttacccggaggctgccgcggactcctaccccgcagccgggacaccaccgcctcc

SEQ ID NO: 8543 - RNA, 4460 nt, Homo sapiens
  source 1..4460: mol_type = other RNA
aaaagtgcttacagtgcaggtagaaactctgtaaccttaagcatgtaaactacatagaataaaactgtttccactgcatttctgtccttcaaagtggccaacctgattaagtcagccttaatcactgctgctgtcagtttcacgactaaaggtcatattgactaagtagtcatcagctgaccacctcgctgtatcagccagcaacgaggggaaggtgaagaaacatgataggccatatagaatctgccctatgtttacttttttaacccagataattatttttgtgtgcagtatctaagctcctgattgtgtaacctgggacttctggcaccttttgttccattcattttatgtataaaatgcatgccaaagcacactgtgccctctggtacccttgcttccaatcgccaaccatgctcatttccttcctttttttgtggtccctttttgtggtgatcattttaaaccacgtcatccaacaaatgttttatggtcaaccttagcttgttcataagccatagcaactgaaagattaaactcttaaatatgtgtctgggcagtggctattaaatagcaaaaaacaatcagattttagtattttattatttccttgtaaaatggctgaactaaattaaacccttgtttcccatttgttctataatttatagtgaaactgagaacaaaactatctttataaatgatagctaaaagtatttccagatatttaaacaatttaaaataaatttcttctgcagagatgcaaagcatctcaacactggaatgaacaaatgccttaaattcaatggagtaaacctttagaatgaagaggaactgtcatttcacccaagccgaagacaacagccttatgcacttgtgtgctctgtctttgctgcttctcgtgtttcaagcctttcctgtgggatcagcacagcaaagtgcaacttaccaaatggtttaatgactggttaattctttcttctcccaatggaaaagcaatggcaacacaacagtagactgctggcttgacaatcttaaacgtgagcctttgcacatgtaggtttatcatcatttgagtatacgactaagcaagtcaatgaactttttttttttttttagcagtttaatttggtcctgagaatgttgcagtctttattaccccttttgcattaatccacttttctaaccaccttttaagctttaatttttaacactatacaccaagtctttgaaatcagtgatctgttatttaactctaaagcatttgacacttcttgccttaacagttttaaaaaccacacacaaaaaaactctgtaagtaatacagtaggccaaaagtttcatcctatctatcttgcagtttacctatctgatctgatctctgtaattatagttctgtcatttaaaatatactatttaaatctaatttttacatttcaaaaattatcttcagtagtaactaagtatattttctgtggattctgagaatgttatttttcagaatgtgagaatatatatgtacatttataatcttgtgactttaaagtctgttttcagatacagtatgtaaatacttgtaaaaaaatttgtataattttgtgataatgtagtttcccaaaaaaattatttagaaggcattatgttattagtaaatgagagcactgtatagaactgttcctattttctgcacttgccattccagctgcctccactgtccatacccacctcattcatcctgtcacagaaggcaggaaaactgggaactttaccaaagtagcactcagcctgagaggcctgtataatcatgcttttcaaactaaattcacttaaaaattaaaaagcagaattgaatattttaagcagcctcagtacctttggccaatgctgttttcatggtggattatgaacattatataatctttgggaaaagtgaaagtagtacaatttttagaataatgacaactgcctcactgcatctctccactcacacagcaaccgtgtagccccctaagctgcagtaccatgactaaccatgatgtcaatttcatatgctgatcctcacaacagcagtgcacaaacatgccccaaatattttaacagaatttagctcttccttaagctgtcttttcatagtaaaaacaaaacaaaaacacccaatgttaaaaccacataataaacttacaaacttgaaaaattagacacttcagatagataggcaataaaacttcatattatgaaagcaatatattccaagtttcaaagatttgacaagttctgtagagtatctttcatcagtacatgaaaacttccaaactgcatgatcttctgccaggcaggactgggtgctattcgctggtttgaggtcgaatccatttcaaggcatgtcgtggtgggacattaatggtgggatggtagaatgtgcagtccggtcttgtacattgagtgttaaacctacaatgttttggatgatagaagggacattccatcttcttacaagcagggaagtaacggcagagctgactactggaaggtggtgctggtggtgcaactgctggttttggagacagtactggaattcttctactcacatgagtgaagggacaatctggtttagtacactttgcatcatatttacaatttgggtgaacaaacaaacatttttcagcaaatttacaattggggaaggctttgcagggtgagatggggtgatggtaggcacactcatccccatttttacaagcaggccagtacttgcagcgctccaaaagtttttctggtttctgtgccacactcagttcactcatctcagcgttagaaaagctaccatttgggtcctcaagctgcctgctcagcaagtgcaactgctgtgggtggaggagacctctgagtcccttgtttgaggctgcagtttggtttacgggtttcattccttcaaagcacatgtcctcctcttgatctgacatgtatcctggggggctggggacaccatccagcgtcactataaacttgggacttgcaggtttatctggttgtacaagatctcgtgtctgcataaggtgtcctgaaagtacccgaagggaatctgcagtcttcatccccgactcttggtttggtgccactactacttcctcagacagctttggcttcttcagaataaatgatcttgtgtctgcatggaccatggattccatgtcatagtaatcttgatttttttctacagaatctccttttgtttcctcttctttaatggggggacttattctgggggtcctactttgtccctggaccacttctgctagcaattcttcttgagaagttcgagttctgggagcaactggaagtgtctgtttctgtggaactgtagagtagttagttgtttttgttacggattcttgagcttcagatatagccttcaaaatcagattcttgttagcttgtttagaaggtggaagagaaggtctcctttcaggctttgcaggcacagacacactgctggagatgcttcctgttcgagacccgtaatcatcatcttcttcctcctcttctccatcatgattgaatttttttactttaacaactgaacttaccacaggcaactttctcttccgaaagttttcatcctccatactcattttctccgagttgtttctaaagaacggactatacgtttcttctaagctgttaagcacctctggttcacacaaacgtcctgtttcatatacccaactactctgcatatcaagctgcttggcagcatgaatactattctgctgctgttgaaattgcaacctgtttaaatgaacaccactatctgcatttctacttgcaggtggtcgataaatttcaatagaagggcgagaagaaccatatgtaagtgtcactgtaggttttttctgagataagggattctcctgcacaaagttgaggtcttcgtcaatgagatcatctggttctggcttaatatcaatcacatcttcagagggtgctggctccctcaaaggtttcactgttgacattagtcgggttgcagctccatcatcgtaagtctgtctgacatttgtggtttttgactcctgcgaacttgtagaaactctggaatctcttttttcaggtctcgcgctaggaatggcaagtggtggcactgcagcttcatgcctcctctcatctccccgactgaaattgctcttgtttgaaggcacgttactatcaaagatgttggtatcagaagacttcagactagagggttcagttgtaacagagcgaagtttatctaatacaccatgaagccaacataagctcctaattcttgtaatttccccttaatggcactccggatcttgcggctgatctcggtgccgatctccatggctctgcggcgtgcgggaactcagcactgcgcggcgcttggcttacccggaggctgccgcggactcctaccccgcagccgggacaccaccgcctcc

SEQ ID NO: 8544 - RNA, 4575 nt, Homo sapiens
  source 1..4575: mol_type = other RNA
aaaagtgcttacagtgcaggtagaaactctgtaaccttaagcatgtaaactacatagaataaaactgtttccactgcatttctgtccttcaaagtggccaacctgattaagtcagccttaatcactgctgctgtcagtttcacgactaaaggtcatattgactaagtagtcatcagctgaccacctcgctgtatcagccagcaacgaggggaaggtgaagaaacatgataggccatatagaatctgccctatgtttacttttttaacccagataattatttttgtgtgcagtatctaagctcctgattgtgtaacctgggacttctggcaccttttgttccattcattttatgtataaaatgcatgccaaagcacactgtgccctctggtacccttgcttccaatcgccaaccatgctcatttccttcctttttttgtggtccctttttgtggtgatcattttaaaccacgtcatccaacaaatgttttatggtcaaccttagcttgttcataagccatagcaactgaaagattaaactcttaaatatgtgtctgggcagtggctattaaatagcaaaaaacaatcagattttagtattttattatttccttgtaaaatggctgaactaaattaaacccttgtttcccatttgttctataatttatagtgaaactgagaacaaaactatctttataaatgatagctaaaagtatttccagatatttaaacaatttaaaataaatttcttctgcagagatgcaaagcatctcaacactggaatgaacaaatgccttaaattcaatggagtaaacctttagaatgaagaggaactgtcatttcacccaagccgaagacaacagccttatgcacttgtgtgctctgtctttgctgcttctcgtgtttcaagcctttcctgtgggatcagcacagcaaagtgcaacttaccaaatggtttaatgactggttaattctttcttctcccaatggaaaagcaatggcaacacaacagtagactgctggcttgacaatcttaaacgtgagcctttgcacatgtaggtttatcatcatttgagtatacgactaagcaagtcaatgaactttttttttttttttagcagtttaatttggtcctgagaatgttgcagtctttattaccccttttgcattaatccacttttctaaccaccttttaagctttaatttttaacactatacaccaagtctttgaaatcagtgatctgttatttaactctaaagcatttgacacttcttgccttaacagttttaaaaaccacacacaaaaaaactctgtaagtaatacagtaggccaaaagtttcatcctatctatcttgcagtttacctatctgatctgatctctgtaattatagttctgtcatttaaaatatactatttaaatctaatttttacatttcaaaaattatcttcagtagtaactaagtatattttctgtggattctgagaatgttatttttcagaatgtgagaatatatatgtacatttataatcttgtgactttaaagtctgttttcagatacagtatgtaaatacttgtaaaaaaatttgtataattttgtgataatgtagtttcccaaaaaaattatttagaaggcattatgttattagtaaatgagagcactgtatagaactgttcctattttctgcacttgccattccagctgcctccactgtccatacccacctcattcatcctgtcacagaaggcaggaaaactgggaactttaccaaagtagcactcagcctgagaggcctgtataatcatgcttttcaaactaaattcacttaaaaattaaaaagcagaattgaatattttaagcagcctcagtacctttggccaatgctgttttcatggtggattatgaacattatataatctttgggaaaagtgaaagtagtacaatttttagaataatgacaactgcctcactgcatctctccactcacacagcaaccgtgtagccccctaagctgcagtaccatgactaaccatgatgtcaatttcatatgctgatcctcacaacagcagtgcacaaacatgccccaaatattttaacagaatttagctcttccttaagctgtcttttcatagtaaaaacaaaacaaaaacacccaatgttaaaaccacataataaacttacaaacttgaaaaattagacacttcagatagataggcaataaaacttcatattatgaaagcaatatattccaagtttcaaagatttgacaagttctgtagagtatctttcatcagtacatgaaaacttccaaactgcatgatcttctgccaggcaggactgggtgctattcgctggtttgaggtcgaatccatttcaaggcatgtcgtggtgggacattaatggtgggatggtagaatgtgcagtccggtcttgtacattgagtgttaaacctacaatgttttggatgatagaagggacattccatcttcttacaagcagggaagtaacggcagagctgactactggaaggtggtgctggtggtgcaactgctggttttggagacagtactggaattcttctactcacatgagtgaagggacaatctggtttagtacactttgcatcatatttacaatttgggtgaacaaacaaacatttttcagcaaatttacaattggggaaggctttgcagggtgagatggggtgatggtaggcacactcatccccatttttacaagcaggccagtacttgcagcgctccaaaagtttttctggtttctgtgccacactcagttcactcatctcagcgttagaaaagctaccatttgggtcctcaagctgcctgctcagcaagtgcaactgctgtgggtggaggagacctctgagtcccttgtttgaggctgcagtttggtttacgggtttcattccttcaaagcacatgtcctcctcttgatctgacatgtatcctggggggctggggacaccatccagcgtcactataaacttgggacttgcaggtttatctggttgtacaagatctcgtgtctgcataaggtgtcctgaaagtacccgaagggaatctgcagtcttcatccccgactcttggtttggtgccactactacttcctcagacagctttggcttcttcagaataaatgatcttgtgtctgcatggaccatggattccatgtcatagtaatcttgatttttttctacagaatctccttttgtttcctcttctttaatggggggacttattctgggggtcctactttgtccctggaccacttctgctagcaattcttcttgagaagttcgagttctgggagcaactggaagtgtctgtttctgtggaactgtagagtagttagttgtttttgttacggattcttgagcttcagatatagccttcaaaatcagattcttgttagcttgtttagaaggtggaagagaaggtctcctttcaggctttgcaggcacagacacactgctggagatgcttcctgttcgagacccgtaatcatcatcttcttcctcctcttctccatcatgattgaatttttttactttaacaactgaacttaccacaggcaactttctcttccgaaagttttcatcctccatactcattttctccgagttgtttctaaagaacggactatacgtttcttctaagctgttaagcacctctggttcacacaaacgtcctgtttcatatacccaactactctgcatatcaagctgcttggcagcatgaatactattctgctgctgttgaaattgcaacctgtttaaatgaacaccactatctgcatttctacttgcaggtggtcgataaatttcaatagaagggcgagaagaaccatatgtaagtgtcactgtaggttttttctgagataagggattctcctgcacaaagttgaggtcttcgtcaatgagatcatctggttctggcttaatatcaatcacatcttcagagggtgctggctccctcaaaggtttcactgttgacattagtcgggttgcagctccatcatcgtaagtctgtctgacatttgtggtttttgactcctgcgaacttgtagaaactctggaatctcttttttcaggtctcgcgctaggaatggcaagtggtggcactgcagcttcatgcctcctctcatctccccgactgaaattgctcttgtttgaaggcacgttactatcaaagatgttggtatcagaagacttcagactagagggttcagttgtaacagagcgaagtttatctaatacaccatgaagccatacggtgaatcgaattgtgttgttccctagaaacagggacagatcctctgtcatttggtcctgacttttcttgttggccaccatcaccataatgtaatcaggaagttcttcatcaacataagctcctaattcttgtaatttccccttaatggcactccggatcttgcggctgatctcggtgccgatctccatggctctgcggcgtgcgggaactcagcactgcgcggcgcttggcttacccggaggctgccgcggactcctaccccgcagccgggacaccaccgcctcc

SEQ ID NO: 8545 - RNA, 4756 nt, Homo sapiens
  source 1..4756: mol_type = other RNA
aaaagtgcttacagtgcaggtagaaactctgtaaccttaagcatgtaaactacatagaataaaactgtttccactgcatttctgtccttcaaagtggccaacctgattaagtcagccttaatcactgctgctgtcagtttcacgactaaaggtcatattgactaagtagtcatcagctgaccacctcgctgtatcagccagcaacgaggggaaggtgaagaaacatgataggccatatagaatctgccctatgtttacttttttaacccagataattatttttgtgtgcagtatctaagctcctgattgtgtaacctgggacttctggcaccttttgttccattcattttatgtataaaatgcatgccaaagcacactgtgccctctggtacccttgcttccaatcgccaaccatgctcatttccttcctttttttgtggtccctttttgtggtgatcattttaaaccacgtcatccaacaaatgttttatggtcaaccttagcttgttcataagccatagcaactgaaagattaaactcttaaatatgtgtctgggcagtggctattaaatagcaaaaaacaatcagattttagtattttattatttccttgtaaaatggctgaactaaattaaacccttgtttcccatttgttctataatttatagtgaaactgagaacaaaactatctttataaatgatagctaaaagtatttccagatatttaaacaatttaaaataaatttcttctgcagagatgcaaagcatctcaacactggaatgaacaaatgccttaaattcaatggagtaaacctttagaatgaagaggaactgtcatttcacccaagccgaagacaacagccttatgcacttgtgtgctctgtctttgctgcttctcgtgtttcaagcctttcctgtgggatcagcacagcaaagtgcaacttaccaaatggtttaatgactggttaattctttcttctcccaatggaaaagcaatggcaacacaacagtagactgctggcttgacaatcttaaacgtgagcctttgcacatgtaggtttatcatcatttgagtatacgactaagcaagtcaatgaactttttttttttttttagcagtttaatttggtcctgagaatgttgcagtctttattaccccttttgcattaatccacttttctaaccaccttttaagctttaatttttaacactatacaccaagtctttgaaatcagtgatctgttatttaactctaaagcatttgacacttcttgccttaacagttttaaaaaccacacacaaaaaaactctgtaagtaatacagtaggccaaaagtttcatcctatctatcttgcagtttacctatctgatctgatctctgtaattatagttctgtcatttaaaatatactatttaaatctaatttttacatttcaaaaattatcttcagtagtaactaagtatattttctgtggattctgagaatgttatttttcagaatgtgagaatatatatgtacatttataatcttgtgactttaaagtctgttttcagatacagtatgtaaatacttgtaaaaaaatttgtataattttgtgataatgtagtttcccaaaaaaattatttagaaggcattatgttattagtaaatgagagcactgtatagaactgttcctattttctgcacttgccattccagctgcctccactgtccatacccacctcattcatcctgtcacagaaggcaggaaaactgggaactttaccaaagtagcactcagcctgagaggcctgtataatcatgcttttcaaactaaattcacttaaaaattaaaaagcagaattgaatattttaagcagcctcagtacctttggccaatgctgttttcatggtggattatgaacattatataatctttgggaaaagtgaaagtagtacaatttttagaataatgacaactgcctcactgcatctctccactcacacagcaaccgtgtagccccctaagctgcagtaccatgactaaccatgatgtcaatttcatatgctgatcctcacaacagcagtgcacaaacatgccccaaatattttaacagaatttagctcttccttaagctgtcttttcatagtaaaaacaaaacaaaaacacccaatgttaaaaccacataataaacttacaaacttgaaaaattagacacttcagatagataggcaataaaacttcatattatgaaagcaatatattccaagtttcaaagatttgacaagttctgtagagtatctttcatcagtacatgaaaacttccaaactgcatgatcttctgccaggcaggactgggtgctattcgctggtttgaggtcgaatccatttcaaggcatgtcgtggtgggacattaatggtgggatggtagaatgtgcagtccggtcttgtacattgagtgttaaacctacaatgttttggatgatagaagggacattccatcttcttacaagcagggaagtaacggcagagctgactactggaaggtggtgctggtggtgcaactgctggttttggagacagtactggaattcttctactcacatgagtgaagggacaatctggtttagtacactttgcatcatatttacaatttgggtgaacaaacaaacatttttcagcaaatttacaattggggaaggctttgcagggtgagatggggtgatggtaggcacactcatccccatttttacaagcaggccagtacttgcagcgctccaaaagtttttctggtttctgtgccacactcagttcactcatctcagcgttagaaaagctaccatttgggtcctcaagctgcctgctcagcaagtgcaactgctgtgggtggaggagacctctgagtcccttgtttgaggctgcagtttggtttacgggtttcattccttcaaagcacatgtcctcctcttgatctgacatgtatcctggggggctggggacaccatccagcgtcactataaacttgggacttgcaggtttatctggttgtacaagatctcgtgtctgcataaggtgtcctgaaagtacccgaagggaatctgcagtcttcatccccgactcttggtttggtgccactactacttcctcagacagctttggcttcttcagaataaatgatcttgtgtctgcatggaccatggattccatgtcatagtaatcttgatttttttctacagaatctccttttgtttcctcttctttaatggggggacttattctgggggtcctactttgtccctggaccacttctgctagcaattcttcttgagaagttcgagttctgggagcaactggaagtgtctgtttctgtggaactgtagagtagttagttgtttttgttacggattcttgagcttcagatatagccttcaaaatcagattcttgttagcttgtttagaaggtggaagagaaggtctcctttcaggctttgcaggcacagacacactgctggagatgcttcctgttcgagacccgtaatcatcatcttcttcctcctcttctccatcatgattgaatttttttactttaacaactgaacttaccacaggcaactttctcttccgaaagttttcatcctccatactcattttctccgagttgtttctaaagaacggactatacgtttcttctaagctgttaagcacctctggttcacacaaacgtcctgtttcatatacccaactactctgcatatcaagctgcttggcagcatgaatactattctgctgctgttgaaattgcaacctgtttaaatgaacaccactatctgcatttctacttgcaggtggtcgataaatttcaatagaagggcgagaagaaccatatgtaagtgtcactgtaggttttttctgagataagggattctcctgcacaaagttgaggtcttcgtcaatgagatcatctggttctggcttaatatcaatcacatcttcagagggtgctggctccctcaaaggtttcactgttgacattagtcgggttgcagctccatcatcgtaagtctgtctgacatttgtggtttttgactcctgcgaacttgtagaaactctggaatctcttttttcaggtctcgcgctaggaatggcaagtggtggcactgcagcttcatgcctcctctcatctccccgactgaaattgctcttgtttgaaggcacgttactatcaaagatgttggtatcagaagacttcagactagagggttcagttgtaacagagcgaagtttatctaatacaccatgaagccatacggtgaatcgaattgtgttgttccctagaaacagggacagatcctctgtcatttggtcctgacttttcttgttggccaccatcaccataatgtaatcaggaagttcttcatctatttaaaaggaaaggtagatcaaaactttgtttcctcaaaactttcttcttaaagttgatgtgcttgaaaatatagatgtagctctaagctttagagtcgcagagctctactggaattacattggacaagatggcttagctttaatttttttctcttcattccacaggtatttcaaatacaacataagctcctaattcttgtaatttccccttaatggcactccggatcttgcggctgatctcggtgccgatctccatggctctgcggcgtgcgggaactcagcactgcgcggcgcttggcttacccggaggctgccgcggactcctaccccgcagccgggacaccaccgcctcc

SEQ ID NO: 8546 - RNA, 4490 nt, Homo sapiens
  source 1..4490: mol_type = other RNA
aaaagtgcttacagtgcaggtagaaactctgtaaccttaagcatgtaaactacatagaataaaactgtttccactgcatttctgtccttcaaagtggccaacctgattaagtcagccttaatcactgctgctgtcagtttcacgactaaaggtcatattgactaagtagtcatcagctgaccacctcgctgtatcagccagcaacgaggggaaggtgaagaaacatgataggccatatagaatctgccctatgtttacttttttaacccagataattatttttgtgtgcagtatctaagctcctgattgtgtaacctgggacttctggcaccttttgttccattcattttatgtataaaatgcatgccaaagcacactgtgccctctggtacccttgcttccaatcgccaaccatgctcatttccttcctttttttgtggtccctttttgtggtgatcattttaaaccacgtcatccaacaaatgttttatggtcaaccttagcttgttcataagccatagcaactgaaagattaaactcttaaatatgtgtctgggcagtggctattaaatagcaaaaaacaatcagattttagtattttattatttccttgtaaaatggctgaactaaattaaacccttgtttcccatttgttctataatttatagtgaaactgagaacaaaactatctttataaatgatagctaaaagtatttccagatatttaaacaatttaaaataaatttcttctgcagagatgcaaagcatctcaacactggaatgaacaaatgccttaaattcaatggagtaaacctttagaatgaagaggaactgtcatttcacccaagccgaagacaacagccttatgcacttgtgtgctctgtctttgctgcttctcgtgtttcaagcctttcctgtgggatcagcacagcaaagtgcaacttaccaaatggtttaatgactggttaattctttcttctcccaatggaaaagcaatggcaacacaacagtagactgctggcttgacaatcttaaacgtgagcctttgcacatgtaggtttatcatcatttgagtatacgactaagcaagtcaatgaactttttttttttttttagcagtttaatttggtcctgagaatgttgcagtctttattaccccttttgcattaatccacttttctaaccaccttttaagctttaatttttaacactatacaccaagtctttgaaatcagtgatctgttatttaactctaaagcatttgacacttcttgccttaacagttttaaaaaccacacacaaaaaaactctgtaagtaatacagtaggccaaaagtttcatcctatctatcttgcagtttacctatctgatctgatctctgtaattatagttctgtcatttaaaatatactatttaaatctaatttttacatttcaaaaattatcttcagtagtaactaagtatattttctgtggattctgagaatgttatttttcagaatgtgagaatatatatgtacatttataatcttgtgactttaaagtctgttttcagatacagtatgtaaatacttgtaaaaaaatttgtataattttgtgataatgtagtttcccaaaaaaattatttagaaggcattatgttattagtaaatgagagcactgtatagaactgttcctattttctgcacttgccattccagctgcctccactgtccatacccacctcattcatcctgtcacagaaggcaggaaaactgggaactttaccaaagtagcactcagcctgagaggcctgtataatcatgcttttcaaactaaattcacttaaaaattaaaaagcagaattgaatattttaagcagcctcagtacctttggccaatgctgttttcatggtggattatgaacattatataatctttgggaaaagtgaaagtagtacaatttttagaataatgacaactgcctcactgcatctctccactcacacagcaaccgtgtagccccctaagctgcagtaccatgactaaccatgatgtcaatttcatatgctgatcctcacaacagcagtgcacaaacatgccccaaatattttaacagaatttagctcttccttaagctgtcttttcatagtaaaaacaaaacaaaaacacccaatgttaaaaccacataataaacttacaaacttgaaaaattagacacttcagatagataggcaataaaacttcatattatgaaagcaatatattccaagtttcaaagatttgacaagttctgtagagtatctttcatcagtacatgaaaacttccaaactgcatgatcttctgccaggcaggactgggtgctattcgctggtttgaggtcgaatccatttcaaggcatgtcgtggtgggacattaatggtgggatggtagaatgtgcagtccggtcttgtacattgagtgttaaacctacaatgttttggatgatagaagggacattccatcttcttacaagcagggaagtaacggcagagctgactactggaaggtggtgctggtggtgcaactgctggttttggagacagtactggaattcttctactcacatgagtgaagggacaatctggtttagtacactttgcatcatatttacaatttgggtgaacaaacaaacatttttcagcaaatttacaattggggaaggctttgcagggtgagatggggtgatggtaggcacactcatccccatttttacaagcaggccagtacttgcagcgctccaaaagtttttctggtttctgtgccacactcagttcactcatctcagcgttagaaaagctaccatttgggtcctcaagctgcctgctcagcaagtgcaactgctgtgggtggaggagacctctgagtcccttgtttgaggctgcagtttggtttacgggtttcattccttcaaagcacatgtcctcctcttgatctgacatgtatcctggggggctggggacaccatccagcgtcactataaacttgggacttgcaggtttatctggttgtacaagatctcttgactcatctgcagagtttctgccattactgggtcgatttgcagtcgggataataattgcctctgttgagttccttgatttttttctacagaatctccttttgtttcctcttctttaatggggggacttattctgggggtcctactttgtccctggaccacttctgctagcaattcttcttgagaagttcgagttctgggagcaactggaagtgtctgtttctgtggaactgtagagtagttagttgtttttgttacggattcttgagcttcagatatagccttcaaaatcagattcttgttagcttgtttagaaggtggaagagaaggtctcctttcaggctttgcaggcacagacacactgctggagatgcttcctgttcgagacccgtaatcatcatcttcttcctcctcttctccatcatgattgaatttttttactttaacaactgaacttaccacaggcaactttctcttccgaaagttttcatcctccatactcattttctccgagttgtttctaaagaacggactatacgtttcttctaagctgttaagcacctctggttcacacaaacgtcctgtttcatatacccaactactctgcatatcaagctgcttggcagcatgaatactattctgctgctgttgaaattgcaacctgtttaaatgaacaccactatctgcatttctacttgcaggtggtcgataaatttcaatagaagggcgagaagaaccatatgtaagtgtcactgtaggttttttctgagataagggattctcctgcacaaagttgaggtcttcgtcaatgagatcatctggttctggcttaatatcaatcacatcttcagagggtgctggctccctcaaaggtttcactgttgacattagtcgggttgcagctccatcatcgtaagtctgtctgacatttgtggtttttgactcctgcgaacttgtagaaactctggaatctcttttttcaggtctcgcgctaggaatggcaagtggtggcactgcagcttcatgcctcctctcatctccccgactgaaattgctcttgtttgaaggcacgttactatcaaagatgttggtatcagaagacttcagactagagggttcagttgtaacagagcgaagtttatctaatacaccatgaagccatacggtgaatcgaattgtgttgttccctagaaacagggacagatcctctgtcatttggtcctgacttttcttgttggccaccatcaccataatgtaatcaggaagttcttcatcaacataagctcctaattcttgtaatttccccttaatggcactccggatcttgcggctgatctcggtgccgatctccatggctctgcggcgtgcgggaactcagcactgcgcggcgcttggcttacccggaggctgccgcggactcctaccccgcagccgggacaccaccgcctcc

SEQ ID NO: 8547 - RNA, 4026 nt, Homo sapiens
  source 1..4026: mol_type = other RNA
aaaagtgcttacagtgcaggtagaaactctgtaaccttaagcatgtaaactacatagaataaaactgtttccactgcatttctgtccttcaaagtggccaacctgattaagtcagccttaatcactgctgctgtcagtttcacgactaaaggtcatattgactaagtagtcatcagctgaccacctcgctgtatcagccagcaacgaggggaaggtgaagaaacatgataggccatatagaatctgccctatgtttacttttttaacccagataattatttttgtgtgcagtatctaagctcctgattgtgtaacctgggacttctggcaccttttgttccattcattttatgtataaaatgcatgccaaagcacactgtgccctctggtacccttgcttccaatcgccaaccatgctcatttccttcctttttttgtggtccctttttgtggtgatcattttaaaccacgtcatccaacaaatgttttatggtcaaccttagcttgttcataagccatagcaactgaaagattaaactcttaaatatgtgtctgggcagtggctattaaatagcaaaaaacaatcagattttagtattttattatttccttgtaaaatggctgaactaaattaaacccttgtttcccatttgttctataatttatagtgaaactgagaacaaaactatctttataaatgatagctaaaagtatttccagatatttaaacaatttaaaataaatttcttctgcagagatgcaaagcatctcaacactggaatgaacaaatgccttaaattcaatggagtaaacctttagaatgaagaggaactgtcatttcacccaagccgaagacaacagccttatgcacttgtgtgctctgtctttgctgcttctcgtgtttcaagcctttcctgtgggatcagcacagcaaagtgcaacttaccaaatggtttaatgactggttaattctttcttctcccaatggaaaagcaatggcaacacaacagtagactgctggcttgacaatcttaaacgtgagcctttgcacatgtaggtttatcatcatttgagtatacgactaagcaagtcaatgaactttttttttttttttagcagtttaatttggtcctgagaatgttgcagtctttattaccccttttgcattaatccacttttctaaccaccttttaagctttaatttttaacactatacaccaagtctttgaaatcagtgatctgttatttaactctaaagcatttgacacttcttgccttaacagttttaaaaaccacacacaaaaaaactctgtaagtaatacagtaggccaaaagtttcatcctatctatcttgcagtttacctatctgatctgatctctgtaattatagttctgtcatttaaaatatactatttaaatctaatttttacatttcaaaaattatcttcagtagtaactaagtatattttctgtggattctgagaatgttatttttcagaatgtgagaatatatatgtacatttataatcttgtgactttaaagtctgttttcagatacagtatgtaaatacttgtaaaaaaatttgtataattttgtgataatgtagtttcccaaaaaaattatttagaaggcattatgttattagtaaatgagagcactgtatagaactgttcctattttctgcacttgccattccagctgcctccactgtccatacccacctcattcatcctgtcacagaaggcaggaaaactgggaactttaccaaagtagcactcagcctgagaggcctgtataatcatgcttttcaaactaaattcacttaaaaattaaaaagcagaattgaatattttaagcagcctcagtacctttggccaatgctgttttcatggtggattatgaacattatataatctttgggaaaagtgaaagtagtacaatttttagaataatgacaactgcctcactgcatctctccactcacacagcaaccgtgtagccccctaagctgcagtaccatgactaaccatgatgtcaatttcatatgctgatcctcacaacagcagtgcacaaacatgccccaaatattttaacagaatttagctcttccttaagctgtcttttcatagtaaaaacaaaacaaaaacacccaatgttaaaaccacataataaacttacaaacttgaaaaattagacacttcagatagataggcaataaaacttcatattatgaaagcaatatattccaagtttcaaagatttgacaagttctgtagagtatctttcatcagtacatgaaaacttccaaactgcatgatcttctgccaggcaggactgggtgctattcgctggtttgaggtcgaatccatttcaaggcatgtcgtggtgggacattaatggtgggatggtagaatgtgcagtccggtcttgtacattgagtgttaaacctacaatgttttggatgatagaagggacattccatcttcttacaagcagggaagtaacggcagagctgactactggaaggtggtgctggtggtgcaactgctggttttggagacagtactggaattcttctactcacatgagtgaagggacaatctggtttagtacactttgcatcatatttacaatttgggtgaacaaacaaacatttttcagcaaatttacaattggggaaggctttgcagggtgagatggggtgatggtaggcacactcatccccatttttacaagcaggccagtacttgcagcgctccaaaagtttttctggtttctgtgccacactcagttcactcatctcagctgtagagtagttagttgtttttgttacggattcttgagcttcagatatagccttcaaaatcagattcttgttagcttgtttagaaggtggaagagaaggtctcctttcaggctttgcaggcacagacacactgctggagatgcttcctgttcgagacccgtaatcatcatcttcttcctcctcttctccatcatgattgaatttttttactttaacaactgaacttaccacaggcaactttctcttccgaaagttttcatcctccatactcattttctccgagttgtttctaaagaacggactatacgtttcttctaagctgttaagcacctctggttcacacaaacgtcctgtttcatatacccaactactctgcatatcaagctgcttggcagcatgaatactattctgctgctgttgaaattgcaacctgtttaaatgaacaccactatctgcatttctacttgcaggtggtcgataaatttcaatagaagggcgagaagaaccatatgtaagtgtcactgtaggttttttctgagataagggattctcctgcacaaagttgaggtcttcgtcaatgagatcatctggttctggcttaatatcaatcacatcttcagagggtgctggctccctcaaaggtttcactgttgacattagtcgggttgcagctccatcatcgtaagtctgtctgacatttgtggtttttgactcctgcgaacttgtagaaactctggaatctcttttttcaggtctcgcgctaggaatggcaagtggtggcactgcagcttcatgcctcctctcatctccccgactgaaattgctcttgtttgaaggcacgttactatcaaagatgttggtatcagaagacttcagactagagggttcagttgtaacagagcgaagtttatctaatacaccatgaagccatacggtgaatcgaattgtgttgttccctagaaacagggacagatcctctgtcatttggtcctgacttttcttgttggccaccatcaccataatgtaatcaggaagttcttcatcaacataagctcctaattcttgtaatttccccttaatggcactccggatcttgcggctgatctcggtgccgatctccatggctctgcggcgtgcgggaactcagcactgcgcggcgcttggcttacccggaggctgccgcggactcctaccccgcagccgggacaccaccgcctcc

SEQ ID NO: 8548 - RNA, 4142 nt, Homo sapiens
  source 1..4142: mol_type = other RNA
aaaagtgcttacagtgcaggtagaaactctgtaaccttaagcatgtaaactacatagaataaaactgtttccactgcatttctgtccttcaaagtggccaacctgattaagtcagccttaatcactgctgctgtcagtttcacgactaaaggtcatattgactaagtagtcatcagctgaccacctcgctgtatcagccagcaacgaggggaaggtgaagaaacatgataggccatatagaatctgccctatgtttacttttttaacccagataattatttttgtgtgcagtatctaagctcctgattgtgtaacctgggacttctggcaccttttgttccattcattttatgtataaaatgcatgccaaagcacactgtgccctctggtacccttgcttccaatcgccaaccatgctcatttccttcctttttttgtggtccctttttgtggtgatcattttaaaccacgtcatccaacaaatgttttatggtcaaccttagcttgttcataagccatagcaactgaaagattaaactcttaaatatgtgtctgggcagtggctattaaatagcaaaaaacaatcagattttagtattttattatttccttgtaaaatggctgaactaaattaaacccttgtttcccatttgttctataatttatagtgaaactgagaacaaaactatctttataaatgatagctaaaagtatttccagatatttaaacaatttaaaataaatttcttctgcagagatgcaaagcatctcaacactggaatgaacaaatgccttaaattcaatggagtaaacctttagaatgaagaggaactgtcatttcacccaagccgaagacaacagccttatgcacttgtgtgctctgtctttgctgcttctcgtgtttcaagcctttcctgtgggatcagcacagcaaagtgcaacttaccaaatggtttaatgactggttaattctttcttctcccaatggaaaagcaatggcaacacaacagtagactgctggcttgacaatcttaaacgtgagcctttgcacatgtaggtttatcatcatttgagtatacgactaagcaagtcaatgaactttttttttttttttagcagtttaatttggtcctgagaatgttgcagtctttattaccccttttgcattaatccacttttctaaccaccttttaagctttaatttttaacactatacaccaagtctttgaaatcagtgatctgttatttaactctaaagcatttgacacttcttgccttaacagttttaaaaaccacacacaaaaaaactctgtaagtaatacagtaggccaaaagtttcatcctatctatcttgcagtttacctatctgatctgatctctgtaattatagttctgtcatttaaaatatactatttaaatctaatttttacatttcaaaaattatcttcagtagtaactaagtatattttctgtggattctgagaatgttatttttcagaatgtgagaatatatatgtacatttataatcttgtgactttaaagtctgttttcagatacagtatgtaaatacttgtaaaaaaatttgtataattttgtgataatgtagtttcccaaaaaaattatttagaaggcattatgttattagtaaatgagagcactgtatagaactgttcctattttctgcacttgccattccagctgcctccactgtccatacccacctcattcatcctgtcacagaaggcaggaaaactgggaactttaccaaagtagcactcagcctgagaggcctgtataatcatgcttttcaaactaaattcacttaaaaattaaaaagcagaattgaatattttaagcagcctcagtacctttggccaatgctgttttcatggtggattatgaacattatataatctttgggaaaagtgaaagtagtacaatttttagaataatgacaactgcctcactgcatctctccactcacacagcaaccgtgtagccccctaagctgcagtaccatgactaaccatgatgtcaatttcatatgctgatcctcacaacagcagtgcacaaacatgccccaaatattttaacagaatttagctcttccttaagctgtcttttcatagtaaaaacaaaacaaaaacacccaatgttaaaaccacataataaacttacaaacttgaaaaattagacacttcagatagataggcaataaaacttcatattatgaaagcaatatattccaagtttcaaagatttgacaagttctgtagagtatctttcatcagtacatgaaaacttccaaactgcatgatcttctgccaggcaggactgggtgctattcgctggtttgaggtcgaatccatttcaaggcatgtcgtggtgggacattaatggtgggatggtagaatgtgcagtccggtcttgtacattgagtgttaaacctacaatgttttggatgatagaagggacattccatcttcttacaagcagggaagtaacggcagagctgactactggaaggtggtgctggtggtgcaactgctggttttggagacagtactggaattcttctactcacatgagtgaagggacaatctggtttagtacactttgcatcatatttacaatttgggtgaacaaacaaacatttttcagcaaatttacaattggggaaggctttgcagggtgagatggggtgatggtaggcacactcatccccatttttacaagcaggccagtacttgcagcgctccaaaagtttttctggtttctgtgccacactcagttcactcatctcagcttgactcatctgcagagtttctgccattactgggtcgatttgcagtcgggataataattgcctctgttgagttccttgatttttttctacagaatctccttttgtttcctcttctttaatggggggacttattctgggggtcctactttgtccctggaccacttctgctagcaattcttcttgagaagttcgagttctgggagcaactggaagtgtctgtttctgtggaactgtagagtagttagttgtttttgttacggattcttgagcttcagatatagccttcaaaatcagattcttgttagcttgtttagaaggtggaagagaaggtctcctttcaggctttgcaggcacagacacactgctggagatgcttcctgttcgagacccgtaatcatcatcttcttcctcctcttctccatcatgattgaatttttttactttaacaactgaacttaccacaggcaactttctcttccgaaagttttcatcctccatactcattttctccgagttgtttctaaagaacggactatacgtttcttctaagctgttaagcacctctggttcacacaaacgtcctgtttcatatacccaactactctgcatatcaagctgcttggcagcatgaatactattctgctgctgttgaaattgcaacctgtttaaatgaacaccactatctgcatttctacttgcaggtggtcgataaatttcaatagaagggcgagaagaaccatatgtaagtgtcactgtaggttttttctgagataagggattctcctgcacaaagttgaggtcttcgtcaatgagatcatctggttctggcttaatatcaatcacatcttcagagggtgctggctccctcaaaggtttcactgttgacattagtcgggttgcagctccatcatcgtaagtctgtctgacatttgtggtttttgactcctgcgaacttgtagaaactctggaatctcttttttcaggtctcgcgctaggaatggcaagtggtggcactgcagcttcatgcctcctctcatctccccgactgaaattgctcttgtttgaaggcacgttactatcaaagatgttggtatcagaagacttcagactagagggttcagttgtaacagagcgaagtttatctaatacaccatgaagccaacataagctcctaattcttgtaatttccccttaatggcactccggatcttgcggctgatctcggtgccgatctccatggctctgcggcgtgcgggaactcagcactgcgcggcgcttggcttacccggaggctgccgcggactcctaccccgcagccgggacaccaccgcctcc

SEQ ID NO: 8549 - RNA, 4257 nt, Homo sapiens
  source 1..4257: mol_type = other RNA
aaaagtgcttacagtgcaggtagaaactctgtaaccttaagcatgtaaactacatagaataaaactgtttccactgcatttctgtccttcaaagtggccaacctgattaagtcagccttaatcactgctgctgtcagtttcacgactaaaggtcatattgactaagtagtcatcagctgaccacctcgctgtatcagccagcaacgaggggaaggtgaagaaacatgataggccatatagaatctgccctatgtttacttttttaacccagataattatttttgtgtgcagtatctaagctcctgattgtgtaacctgggacttctggcaccttttgttccattcattttatgtataaaatgcatgccaaagcacactgtgccctctggtacccttgcttccaatcgccaaccatgctcatttccttcctttttttgtggtccctttttgtggtgatcattttaaaccacgtcatccaacaaatgttttatggtcaaccttagcttgttcataagccatagcaactgaaagattaaactcttaaatatgtgtctgggcagtggctattaaatagcaaaaaacaatcagattttagtattttattatttccttgtaaaatggctgaactaaattaaacccttgtttcccatttgttctataatttatagtgaaactgagaacaaaactatctttataaatgatagctaaaagtatttccagatatttaaacaatttaaaataaatttcttctgcagagatgcaaagcatctcaacactggaatgaacaaatgccttaaattcaatggagtaaacctttagaatgaagaggaactgtcatttcacccaagccgaagacaacagccttatgcacttgtgtgctctgtctttgctgcttctcgtgtttcaagcctttcctgtgggatcagcacagcaaagtgcaacttaccaaatggtttaatgactggttaattctttcttctcccaatggaaaagcaatggcaacacaacagtagactgctggcttgacaatcttaaacgtgagcctttgcacatgtaggtttatcatcatttgagtatacgactaagcaagtcaatgaactttttttttttttttagcagtttaatttggtcctgagaatgttgcagtctttattaccccttttgcattaatccacttttctaaccaccttttaagctttaatttttaacactatacaccaagtctttgaaatcagtgatctgttatttaactctaaagcatttgacacttcttgccttaacagttttaaaaaccacacacaaaaaaactctgtaagtaatacagtaggccaaaagtttcatcctatctatcttgcagtttacctatctgatctgatctctgtaattatagttctgtcatttaaaatatactatttaaatctaatttttacatttcaaaaattatcttcagtagtaactaagtatattttctgtggattctgagaatgttatttttcagaatgtgagaatatatatgtacatttataatcttgtgactttaaagtctgttttcagatacagtatgtaaatacttgtaaaaaaatttgtataattttgtgataatgtagtttcccaaaaaaattatttagaaggcattatgttattagtaaatgagagcactgtatagaactgttcctattttctgcacttgccattccagctgcctccactgtccatacccacctcattcatcctgtcacagaaggcaggaaaactgggaactttaccaaagtagcactcagcctgagaggcctgtataatcatgcttttcaaactaaattcacttaaaaattaaaaagcagaattgaatattttaagcagcctcagtacctttggccaatgctgttttcatggtggattatgaacattatataatctttgggaaaagtgaaagtagtacaatttttagaataatgacaactgcctcactgcatctctccactcacacagcaaccgtgtagccccctaagctgcagtaccatgactaaccatgatgtcaatttcatatgctgatcctcacaacagcagtgcacaaacatgccccaaatattttaacagaatttagctcttccttaagctgtcttttcatagtaaaaacaaaacaaaaacacccaatgttaaaaccacataataaacttacaaacttgaaaaattagacacttcagatagataggcaataaaacttcatattatgaaagcaatatattccaagtttcaaagatttgacaagttctgtagagtatctttcatcagtacatgaaaacttccaaactgcatgatcttctgccaggcaggactgggtgctattcgctggtttgaggtcgaatccatttcaaggcatgtcgtggtgggacattaatggtgggatggtagaatgtgcagtccggtcttgtacattgagtgttaaacctacaatgttttggatgatagaagggacattccatcttcttacaagcagggaagtaacggcagagctgactactggaaggtggtgctggtggtgcaactgctggttttggagacagtactggaattcttctactcacatgagtgaagggacaatctggtttagtacactttgcatcatatttacaatttgggtgaacaaacaaacatttttcagcaaatttacaattggggaaggctttgcagggtgagatggggtgatggtaggcacactcatccccatttttacaagcaggccagtacttgcagcgctccaaaagtttttctggtttctgtgccacactcagttcactcatctcagcttgactcatctgcagagtttctgccattactgggtcgatttgcagtcgggataataattgcctctgttgagttccttgatttttttctacagaatctccttttgtttcctcttctttaatggggggacttattctgggggtcctactttgtccctggaccacttctgctagcaattcttcttgagaagttcgagttctgggagcaactggaagtgtctgtttctgtggaactgtagagtagttagttgtttttgttacggattcttgagcttcagatatagccttcaaaatcagattcttgttagcttgtttagaaggtggaagagaaggtctcctttcaggctttgcaggcacagacacactgctggagatgcttcctgttcgagacccgtaatcatcatcttcttcctcctcttctccatcatgattgaatttttttactttaacaactgaacttaccacaggcaactttctcttccgaaagttttcatcctccatactcattttctccgagttgtttctaaagaacggactatacgtttcttctaagctgttaagcacctctggttcacacaaacgtcctgtttcatatacccaactactctgcatatcaagctgcttggcagcatgaatactattctgctgctgttgaaattgcaacctgtttaaatgaacaccactatctgcatttctacttgcaggtggtcgataaatttcaatagaagggcgagaagaaccatatgtaagtgtcactgtaggttttttctgagataagggattctcctgcacaaagttgaggtcttcgtcaatgagatcatctggttctggcttaatatcaatcacatcttcagagggtgctggctccctcaaaggtttcactgttgacattagtcgggttgcagctccatcatcgtaagtctgtctgacatttgtggtttttgactcctgcgaacttgtagaaactctggaatctcttttttcaggtctcgcgctaggaatggcaagtggtggcactgcagcttcatgcctcctctcatctccccgactgaaattgctcttgtttgaaggcacgttactatcaaagatgttggtatcagaagacttcagactagagggttcagttgtaacagagcgaagtttatctaatacaccatgaagccatacggtgaatcgaattgtgttgttccctagaaacagggacagatcctctgtcatttggtcctgacttttcttgttggccaccatcaccataatgtaatcaggaagttcttcatcaacataagctcctaattcttgtaatttccccttaatggcactccggatcttgcggctgatctcggtgccgatctccatggctctgcggcgtgcgggaactcagcactgcgcggcgcttggcttacccggaggctgccgcggactcctaccccgcagccgggacaccaccgcctcc

SEQ ID NO: 8550 - RNA, 4233 nt, Homo sapiens
  source 1..4233: mol_type = other RNA
aaaagtgcttacagtgcaggtagaaactctgtaaccttaagcatgtaaactacatagaataaaactgtttccactgcatttctgtccttcaaagtggccaacctgattaagtcagccttaatcactgctgctgtcagtttcacgactaaaggtcatattgactaagtagtcatcagctgaccacctcgctgtatcagccagcaacgaggggaaggtgaagaaacatgataggccatatagaatctgccctatgtttacttttttaacccagataattatttttgtgtgcagtatctaagctcctgattgtgtaacctgggacttctggcaccttttgttccattcattttatgtataaaatgcatgccaaagcacactgtgccctctggtacccttgcttccaatcgccaaccatgctcatttccttcctttttttgtggtccctttttgtggtgatcattttaaaccacgtcatccaacaaatgttttatggtcaaccttagcttgttcataagccatagcaactgaaagattaaactcttaaatatgtgtctgggcagtggctattaaatagcaaaaaacaatcagattttagtattttattatttccttgtaaaatggctgaactaaattaaacccttgtttcccatttgttctataatttatagtgaaactgagaacaaaactatctttataaatgatagctaaaagtatttccagatatttaaacaatttaaaataaatttcttctgcagagatgcaaagcatctcaacactggaatgaacaaatgccttaaattcaatggagtaaacctttagaatgaagaggaactgtcatttcacccaagccgaagacaacagccttatgcacttgtgtgctctgtctttgctgcttctcgtgtttcaagcctttcctgtgggatcagcacagcaaagtgcaacttaccaaatggtttaatgactggttaattctttcttctcccaatggaaaagcaatggcaacacaacagtagactgctggcttgacaatcttaaacgtgagcctttgcacatgtaggtttatcatcatttgagtatacgactaagcaagtcaatgaactttttttttttttttagcagtttaatttggtcctgagaatgttgcagtctttattaccccttttgcattaatccacttttctaaccaccttttaagctttaatttttaacactatacaccaagtctttgaaatcagtgatctgttatttaactctaaagcatttgacacttcttgccttaacagttttaaaaaccacacacaaaaaaactctgtaagtaatacagtaggccaaaagtttcatcctatctatcttgcagtttacctatctgatctgatctctgtaattatagttctgtcatttaaaatatactatttaaatctaatttttacatttcaaaaattatcttcagtagtaactaagtatattttctgtggattctgagaatgttatttttcagaatgtgagaatatatatgtacatttataatcttgtgactttaaagtctgttttcagatacagtatgtaaatacttgtaaaaaaatttgtataattttgtgataatgtagtttcccaaaaaaattatttagaaggcattatgttattagtaaatgagagcactgtatagaactgttcctattttctgcacttgccattccagctgcctccactgtccatacccacctcattcatcctgtcacagaaggcaggaaaactgggaactttaccaaagtagcactcagcctgagaggcctgtataatcatgcttttcaaactaaattcacttaaaaattaaaaagcagaattgaatattttaagcagcctcagtacctttggccaatgctgttttcatggtggattatgaacattatataatctttgggaaaagtgaaagtagtacaatttttagaataatgacaactgcctcactgcatctctccactcacacagcaaccgtgtagccccctaagctgcagtaccatgactaaccatgatgtcaatttcatatgctgatcctcacaacagcagtgcacaaacatgccccaaatattttaacagaatttagctcttccttaagctgtcttttcatagtaaaaacaaaacaaaaacacccaatgttaaaaccacataataaacttacaaacttgaaaaattagacacttcagatagataggcaataaaacttcatattatgaaagcaatatattccaagtttcaaagatttgacaagttctgtagagtatctttcatcagtacatgaaaacttccaaactgcatgatcttctgccaggcaggactgggtgctattcgctggtttgaggtcgaatccatttcaaggcatgtcgtggtgggacattaatggtgggatggtagaatgtgcagtccggtcttgtacattgagtgttaaacctacaatgttttggatgatagaagggacattccatcttcttacaagcagggaagtaacggcagagctgactactggaaggtggtgctggtggtgcaactgctggttttggagacagtactggaattcttctactcacatgagtgaagggacaatctggtttagtacactttgcatcatatttacaatttgggtgaacaaacaaacatttttcagcaaatttacaattggggaaggctttgcagggtgagatggggtgatggtaggcacactcatccccatttttacaagcaggccagtacttgcagcgctccaaaagtttttctggtttctgtgccacactcagttcactcatctcagcttgactcatctgcagagtttctgccattactgggtcgatttgcagtcgggataataattgcctctgttgagttccttgatttttttctacagaatctccttttgtttcctcttctttaatggggggacttattctgggggtcctactttgtccctggaccacttctgctagcaattcttcttgagaagttcgagttctgggagcaactggaagtgtctgtttctgtggaactgtagagtagttagttgtttttgttacggattcttgagcttcagatatagccttcaaaatcagattcttgttagcttgtttagaaggtggaagagaaggtctcctttcaggctttgcaggcacagacacactgctggagatgcttcctgttcgagacccgtaatcatcatcttcttcctcctcttctccatcatgattgaatttttttactttaacaactgaacttaccacaggcaactttctcttccgaaagttttcatcctccatactcattttctccgagttgtttctaaagaacggactatacgtttcttctaagctgttaagcacctctggttcacacaaacgtcctgtttcatatacccaactactctgcatatcaagctgcttggcagcatgaatactattctgctgctgttgaaattgcaacctgtttaaatgaacaccactatctgcatttctacttgcaggtggtcgataaatttcaatagaagggcgagaagaaccatatgtaagtgtcactgtaggttttttctgagataagggattctcctgcacaaagttgaggtcttcgtcaatgagatcatctggttctggcttaatatcaatcacatcttcagagggtgctggctccctcaaaggtttcactgttgacattagtcgggttgcagctccatcatcgtaagtctgtctgacatttgtggtttttgactcctgcgaacttgtagaaactctggaatctcttttttcaggtctcgcgctaggaatggcaagtggtggcactgcagcttcatgcctcctctcatctccccgactgaaattgctcttgtttgaaggcacgttactatcaaagatgttggtatcagaagacttcagactagagggttcagttgtaacagagcgaagtttatctaatacaccatgaagccatacggtgaatcgaattgtgttgttccctagaaacagggacagatcctctgtcatttggtcctgacttttcttgttggccaccatcaccataatgtaatcaggaagttcttcatcaacataagctcctaattcttgtaatttccccttaatggcactctcccgcagcggatccaaagcggcgccgtgcgccgcggtggtggctccagccgggcctgcgcctgtccttccatttcccggcggctacttcagccgcagccacgctccg

SEQ ID NO: 8551 - RNA, 4067 nt, Homo sapiens
  source 1..4067: mol_type = other RNA
aaaagtgcttacagtgcaggtagaaactctgtaaccttaagcatgtaaactacatagaataaaactgtttccactgcatttctgtccttcaaagtggccaacctgattaagtcagccttaatcactgctgctgtcagtttcacgactaaaggtcatattgactaagtagtcatcagctgaccacctcgctgtatcagccagcaacgaggggaaggtgaagaaacatgataggccatatagaatctgccctatgtttacttttttaacccagataattatttttgtgtgcagtatctaagctcctgattgtgtaacctgggacttctggcaccttttgttccattcattttatgtataaaatgcatgccaaagcacactgtgccctctggtacccttgcttccaatcgccaaccatgctcatttccttcctttttttgtggtccctttttgtggtgatcattttaaaccacgtcatccaacaaatgttttatggtcaaccttagcttgttcataagccatagcaactgaaagattaaactcttaaatatgtgtctgggcagtggctattaaatagcaaaaaacaatcagattttagtattttattatttccttgtaaaatggctgaactaaattaaacccttgtttcccatttgttctataatttatagtgaaactgagaacaaaactatctttataaatgatagctaaaagtatttccagatatttaaacaatttaaaataaatttcttctgcagagatgcaaagcatctcaacactggaatgaacaaatgccttaaattcaatggagtaaacctttagaatgaagaggaactgtcatttcacccaagccgaagacaacagccttatgcacttgtgtgctctgtctttgctgcttctcgtgtttcaagcctttcctgtgggatcagcacagcaaagtgcaacttaccaaatggtttaatgactggttaattctttcttctcccaatggaaaagcaatggcaacacaacagtagactgctggcttgacaatcttaaacgtgagcctttgcacatgtaggtttatcatcatttgagtatacgactaagcaagtcaatgaactttttttttttttttagcagtttaatttggtcctgagaatgttgcagtctttattaccccttttgcattaatccacttttctaaccaccttttaagctttaatttttaacactatacaccaagtctttgaaatcagtgatctgttatttaactctaaagcatttgacacttcttgccttaacagttttaaaaaccacacacaaaaaaactctgtaagtaatacagtaggccaaaagtttcatcctatctatcttgcagtttacctatctgatctgatctctgtaattatagttctgtcatttaaaatatactatttaaatctaatttttacatttcaaaaattatcttcagtagtaactaagtatattttctgtggattctgagaatgttatttttcagaatgtgagaatatatatgtacatttataatcttgtgactttaaagtctgttttcagatacagtatgtaaatacttgtaaaaaaatttgtataattttgtgataatgtagtttcccaaaaaaattatttagaaggcattatgttattagtaaatgagagcactgtatagaactgttcctattttctgcacttgccattccagctgcctccactgtccatacccacctcattcatcctgtcacagaaggcaggaaaactgggaactttaccaaagtagcactcagcctgagaggcctgtataatcatgcttttcaaactaaattcacttaaaaattaaaaagcagaattgaatattttaagcagcctcagtacctttggccaatgctgttttcatggtggattatgaacattatataatctttgggaaaagtgaaagtagtacaatttttagaataatgacaactgcctcactgcatctctccactcacacagcaaccgtgtagccccctaagctgcagtaccatgactaaccatgatgtcaatttcatatgctgatcctcacaacagcagtgcacaaacatgccccaaatattttaacagaatttagctcttccttaagctgtcttttcatagtaaaaacaaaacaaaaacacccaatgttaaaaccacataataaacttacaaacttgaaaaattagacacttcagatagataggcaataaaacttcatattatgaaagcaatatattccaagtttcaaagatttgacaagttctgtagagtatctttcatcagtacatgaaaacttccaaactgcatgatcttctgccaggcaggactgggtgctattcgctggtttgaggtcgaatccatttcaaggcatgtcgtggtgggacattaatggtgggatggtagaatgtgcagtccggtcttgtacattgagtgttaaacctacaatgttttggatgatagaagggacattccatcttcttacaagcagggaagtaacggcagagctgactactggaaggtggtgctggtggtgcaactgctggttttggagacagtactggaattcttctactcacatgagtgaagggacaatctggtttagtacactttgcatcatatttacaatttgggtgaacaaacaaacatttttcagcaaatttacaattggggaaggctttgcagggtgagatggggtgatggtaggcacactcatccccatttttacaagcaggccagtacttgcagcgctccaaaagtttttctggtttctgtgccacactcagttcactcatctcagcttgatttttttctacagaatctccttttgtttcctcttctttaatggggggacttattctgggggtcctactttgtccctggaccacttctgctagcaattcttcttgagaagttcgagttctgggagcaactggaagtgtctgtttctgtggaactgtagagtagttagttgtttttgttacggattcttgagcttcagatatagccttcaaaatcagattcttgttagcttgtttagaaggtggaagagaaggtctcctttcaggctttgcaggcacagacacactgctggagatgcttcctgttcgagacccgtaatcatcatcttcttcctcctcttctccatcatgattgaatttttttactttaacaactgaacttaccacaggcaactttctcttccgaaagttttcatcctccatactcattttctccgagttgtttctaaagaacggactatacgtttcttctaagctgttaagcacctctggttcacacaaacgtcctgtttcatatacccaactactctgcatatcaagctgcttggcagcatgaatactattctgctgctgttgaaattgcaacctgtttaaatgaacaccactatctgcatttctacttgcaggtggtcgataaatttcaatagaagggcgagaagaaccatatgtaagtgtcactgtaggttttttctgagataagggattctcctgcacaaagttgaggtcttcgtcaatgagatcatctggttctggcttaatatcaatcacatcttcagagggtgctggctccctcaaaggtttcactgttgacattagtcgggttgcagctccatcatcgtaagtctgtctgacatttgtggtttttgactcctgcgaacttgtagaaactctggaatctcttttttcaggtctcgcgctaggaatggcaagtggtggcactgcagcttcatgcctcctctcatctccccgactgaaattgctcttgtttgaaggcacgttactatcaaagatgttggtatcagaagacttcagactagagggttcagttgtaacagagcgaagtttatctaatacaccatgaagccaacataagctcctaattcttgtaatttccccttaatggcactccggatcttgcggctgatctcggtgccgatctccatggctctgcggcgtgcgggaactcagcactgcgcggcgcttggcttacccggaggctgccgcggactcctaccccgcagccgggacaccaccgcctcc

SEQ ID NO: 8552 - RNA, 4182 nt, Homo sapiens
  source 1..4182: mol_type = other RNA
aaaagtgcttacagtgcaggtagaaactctgtaaccttaagcatgtaaactacatagaataaaactgtttccactgcatttctgtccttcaaagtggccaacctgattaagtcagccttaatcactgctgctgtcagtttcacgactaaaggtcatattgactaagtagtcatcagctgaccacctcgctgtatcagccagcaacgaggggaaggtgaagaaacatgataggccatatagaatctgccctatgtttacttttttaacccagataattatttttgtgtgcagtatctaagctcctgattgtgtaacctgggacttctggcaccttttgttccattcattttatgtataaaatgcatgccaaagcacactgtgccctctggtacccttgcttccaatcgccaaccatgctcatttccttcctttttttgtggtccctttttgtggtgatcattttaaaccacgtcatccaacaaatgttttatggtcaaccttagcttgttcataagccatagcaactgaaagattaaactcttaaatatgtgtctgggcagtggctattaaatagcaaaaaacaatcagattttagtattttattatttccttgtaaaatggctgaactaaattaaacccttgtttcccatttgttctataatttatagtgaaactgagaacaaaactatctttataaatgatagctaaaagtatttccagatatttaaacaatttaaaataaatttcttctgcagagatgcaaagcatctcaacactggaatgaacaaatgccttaaattcaatggagtaaacctttagaatgaagaggaactgtcatttcacccaagccgaagacaacagccttatgcacttgtgtgctctgtctttgctgcttctcgtgtttcaagcctttcctgtgggatcagcacagcaaagtgcaacttaccaaatggtttaatgactggttaattctttcttctcccaatggaaaagcaatggcaacacaacagtagactgctggcttgacaatcttaaacgtgagcctttgcacatgtaggtttatcatcatttgagtatacgactaagcaagtcaatgaactttttttttttttttagcagtttaatttggtcctgagaatgttgcagtctttattaccccttttgcattaatccacttttctaaccaccttttaagctttaatttttaacactatacaccaagtctttgaaatcagtgatctgttatttaactctaaagcatttgacacttcttgccttaacagttttaaaaaccacacacaaaaaaactctgtaagtaatacagtaggccaaaagtttcatcctatctatcttgcagtttacctatctgatctgatctctgtaattatagttctgtcatttaaaatatactatttaaatctaatttttacatttcaaaaattatcttcagtagtaactaagtatattttctgtggattctgagaatgttatttttcagaatgtgagaatatatatgtacatttataatcttgtgactttaaagtctgttttcagatacagtatgtaaatacttgtaaaaaaatttgtataattttgtgataatgtagtttcccaaaaaaattatttagaaggcattatgttattagtaaatgagagcactgtatagaactgttcctattttctgcacttgccattccagctgcctccactgtccatacccacctcattcatcctgtcacagaaggcaggaaaactgggaactttaccaaagtagcactcagcctgagaggcctgtataatcatgcttttcaaactaaattcacttaaaaattaaaaagcagaattgaatattttaagcagcctcagtacctttggccaatgctgttttcatggtggattatgaacattatataatctttgggaaaagtgaaagtagtacaatttttagaataatgacaactgcctcactgcatctctccactcacacagcaaccgtgtagccccctaagctgcagtaccatgactaaccatgatgtcaatttcatatgctgatcctcacaacagcagtgcacaaacatgccccaaatattttaacagaatttagctcttccttaagctgtcttttcatagtaaaaacaaaacaaaaacacccaatgttaaaaccacataataaacttacaaacttgaaaaattagacacttcagatagataggcaataaaacttcatattatgaaagcaatatattccaagtttcaaagatttgacaagttctgtagagtatctttcatcagtacatgaaaacttccaaactgcatgatcttctgccaggcaggactgggtgctattcgctggtttgaggtcgaatccatttcaaggcatgtcgtggtgggacattaatggtgggatggtagaatgtgcagtccggtcttgtacattgagtgttaaacctacaatgttttggatgatagaagggacattccatcttcttacaagcagggaagtaacggcagagctgactactggaaggtggtgctggtggtgcaactgctggttttggagacagtactggaattcttctactcacatgagtgaagggacaatctggtttagtacactttgcatcatatttacaatttgggtgaacaaacaaacatttttcagcaaatttacaattggggaaggctttgcagggtgagatggggtgatggtaggcacactcatccccatttttacaagcaggccagtacttgcagcgctccaaaagtttttctggtttctgtgccacactcagttcactcatctcagcttgatttttttctacagaatctccttttgtttcctcttctttaatggggggacttattctgggggtcctactttgtccctggaccacttctgctagcaattcttcttgagaagttcgagttctgggagcaactggaagtgtctgtttctgtggaactgtagagtagttagttgtttttgttacggattcttgagcttcagatatagccttcaaaatcagattcttgttagcttgtttagaaggtggaagagaaggtctcctttcaggctttgcaggcacagacacactgctggagatgcttcctgttcgagacccgtaatcatcatcttcttcctcctcttctccatcatgattgaatttttttactttaacaactgaacttaccacaggcaactttctcttccgaaagttttcatcctccatactcattttctccgagttgtttctaaagaacggactatacgtttcttctaagctgttaagcacctctggttcacacaaacgtcctgtttcatatacccaactactctgcatatcaagctgcttggcagcatgaatactattctgctgctgttgaaattgcaacctgtttaaatgaacaccactatctgcatttctacttgcaggtggtcgataaatttcaatagaagggcgagaagaaccatatgtaagtgtcactgtaggttttttctgagataagggattctcctgcacaaagttgaggtcttcgtcaatgagatcatctggttctggcttaatatcaatcacatcttcagagggtgctggctccctcaaaggtttcactgttgacattagtcgggttgcagctccatcatcgtaagtctgtctgacatttgtggtttttgactcctgcgaacttgtagaaactctggaatctcttttttcaggtctcgcgctaggaatggcaagtggtggcactgcagcttcatgcctcctctcatctccccgactgaaattgctcttgtttgaaggcacgttactatcaaagatgttggtatcagaagacttcagactagagggttcagttgtaacagagcgaagtttatctaatacaccatgaagccatacggtgaatcgaattgtgttgttccctagaaacagggacagatcctctgtcatttggtcctgacttttcttgttggccaccatcaccataatgtaatcaggaagttcttcatcaacataagctcctaattcttgtaatttccccttaatggcactccggatcttgcggctgatctcggtgccgatctccatggctctgcggcgtgcgggaactcagcactgcgcggcgcttggcttacccggaggctgccgcggactcctaccccgcagccgggacaccaccgcctcc

SEQ ID NO: 8553 - RNA, 4632 nt, Homo sapiens
  source 1..4632: mol_type = other RNA
aaaagtgcttacagtgcaggtagaaactctgtaaccttaagcatgtaaactacatagaataaaactgtttccactgcatttctgtccttcaaagtggccaacctgattaagtcagccttaatcactgctgctgtcagtttcacgactaaaggtcatattgactaagtagtcatcagctgaccacctcgctgtatcagccagcaacgaggggaaggtgaagaaacatgataggccatatagaatctgccctatgtttacttttttaacccagataattatttttgtgtgcagtatctaagctcctgattgtgtaacctgggacttctggcaccttttgttccattcattttatgtataaaatgcatgccaaagcacactgtgccctctggtacccttgcttccaatcgccaaccatgctcatttccttcctttttttgtggtccctttttgtggtgatcattttaaaccacgtcatccaacaaatgttttatggtcaaccttagcttgttcataagccatagcaactgaaagattaaactcttaaatatgtgtctgggcagtggctattaaatagcaaaaaacaatcagattttagtattttattatttccttgtaaaatggctgaactaaattaaacccttgtttcccatttgttctataatttatagtgaaactgagaacaaaactatctttataaatgatagctaaaagtatttccagatatttaaacaatttaaaataaatttcttctgcagagatgcaaagcatctcaacactggaatgaacaaatgccttaaattcaatggagtaaacctttagaatgaagaggaactgtcatttcacccaagccgaagacaacagccttatgcacttgtgtgctctgtctttgctgcttctcgtgtttcaagcctttcctgtgggatcagcacagcaaagtgcaacttaccaaatggtttaatgactggttaattctttcttctcccaatggaaaagcaatggcaacacaacagtagactgctggcttgacaatcttaaacgtgagcctttgcacatgtaggtttatcatcatttgagtatacgactaagcaagtcaatgaactttttttttttttttagcagtttaatttggtcctgagaatgttgcagtctttattaccccttttgcattaatccacttttctaaccaccttttaagctttaatttttaacactatacaccaagtctttgaaatcagtgatctgttatttaactctaaagcatttgacacttcttgccttaacagttttaaaaaccacacacaaaaaaactctgtaagtaatacagtaggccaaaagtttcatcctatctatcttgcagtttacctatctgatctgatctctgtaattatagttctgtcatttaaaatatactatttaaatctaatttttacatttcaaaaattatcttcagtagtaactaagtatattttctgtggattctgagaatgttatttttcagaatgtgagaatatatatgtacatttataatcttgtgactttaaagtctgttttcagatacagtatgtaaatacttgtaaaaaaatttgtataattttgtgataatgtagtttcccaaaaaaattatttagaaggcattatgttattagtaaatgagagcactgtatagaactgttcctattttctgcacttgccattccagctgcctccactgtccatacccacctcattcatcctgtcacagaaggcaggaaaactgggaactttaccaaagtagcactcagcctgagaggcctgtataatcatgcttttcaaactaaattcacttaaaaattaaaaagcagaattgaatattttaagcagcctcagtacctttggccaatgctgttttcatggtggattatgaacattatataatctttgggaaaagtgaaagtagtacaatttttagaataatgacaactgcctcactgcatctctccactcacacagcaaccgtgtagccccctaagctgcagtaccatgactaaccatgatgtcaatttcatatgctgatcctcacaacagcagtgcacaaacatgccccaaatattttaacagaatttagctcttccttaagctgtcttttcatagtaaaaacaaaacaaaaacacccaatgttaaaaccacataataaacttacaaacttgaaaaattagacacttcagatagataggcaataaaacttcatattatgaaagcaatatattccaagtttcaaagatttgacaagttctgtagagtatctttcatcagtacatgaaaacttccaaactgcatgatcttctgccaggcaggactgggtgctattcgctggtttgaggtcgaatccatttcaaggcatgtcgtggtgggacattaatggtgggatggtagaatgtgcagtccggtcttgtacattgagtgttaaacctacaatgttttggatgatagaagggacattccatcttcttacaagcagggaagtaacggcagagctgactactggaaggtggtgctggtggtgcaactggttttggagacagtactggaattcttctactcacatgagtgaagggacaatctggtttagtacactttgcatcatatttacaatttgggtgaacaaacaaacatttttcagcaaatttacaattggggaaggctttgcagggtgagatggggtgatggtaggcacactcatccccatttttacaagcaggccagtacttgcagcgctccaaaagtttttctggtttctgtgccacactcagttcactcatctcagcatttgggtcctcaagctgcctgctcagcaagtgcaactgctgtgggtggaggagacctctgagtcccttgtttgaggctgcagtttggtttacgggtttcattccttcaaagcacatgtcctcctcttgatctgacatgtatcctggggggctggggacaccatccagcgtcactataaacttgggacttgcaggtttatctggttgtacaagatctcgtgtctgcataaggtgtcctgaaagtacccgaagggaatctgcagtcttcatccccgactcttggtttggtgccactactacttcctcagacagctttggcttcttcagaataaatgatcttgtgtctgcatggaccatggattccatgtcatagtaatcttgactcatctgcagagtttctgccattactgggtcgatttgcagtcgggataataattgcctctgttgagttccttgatttttttctacagaatctccttttgtttcctcttctttaatggggggacttattctgggggtcctactttgtccctggaccacttctgctagcaattcttcttgagaagttcgagttctgggagcaactggaagtgtctgtttctgtggaactgtagagtagttagttgtttttgttacggattcttgagcttcagatatagccttcaaaatcagattcttgttagcttgtttagaaggtggaagagaaggtctcctttcaggctttgcaggcacagacacactgctggagatgcttcctgttcgagacccgtaatcatcatcttcttcctcctcttctccatcatgattgaatttttttactttaacaactgaacttaccacaggcaactttctcttccgaaagttttcatcctccatactcattttctccgagttgtttctaaagaacggactatacgtttcttctaagctgttaagcacctctggttcacacaaacgtcctgtttcatatacccaactactctgcatatcaagctgcttggcagcatgaatactattctgctgctgttgaaattgcaacctgtttaaatgaacaccactatctgcatttctacttgcaggtggtcgataaatttcaatagaagggcgagaagaaccatatgtaagtgtcactgtaggttttttctgagataagggattctcctgcacaaagttgaggtcttcgtcaatgagatcatctggttctggcttaatatcaatcacatcttcagagggtgctggctccctcaaaggtttcactgttgacattagtcgggttgcagctccatcatcgtaagtctgtctgacatttgtggtttttgactcctgcgaacttgtagaaactctggaatctcttttttcaggtctcgcgctaggaatggcaagtggtggcactgcagcttcatgcctcctctcatctccccgactgaaattgctcttgtttgaaggcacgttactatcaaagatgttggtatcagaagacttcagactagagggttcagttgtaacagagcgaagtttatctaatacaccatgaagccatacggtgaatcgaattgtgttgttccctagaaacagggacagatcctctgtcatttggtcctgacttttcttgttggccaccatcaccataatgtaatcaggaagttcttcatcaacataagctcctaattcttgtaatttccccttaatggcactccggatcttgcggctgatctcggtgccgatctccatggctctgcggcgtgcgggaactcagcactgcgcggcgcttggcttacccggaggctgccgcggactcctaccccgcagccgggacaccaccgcctcc

SEQ ID NO: 8554 - RNA, 4557 nt, Homo sapiens
  source 1..4557: mol_type = other RNA
aaaagtgcttacagtgcaggtagaaactctgtaaccttaagcatgtaaactacatagaataaaactgtttccactgcatttctgtccttcaaagtggccaacctgattaagtcagccttaatcactgctgctgtcagtttcacgactaaaggtcatattgactaagtagtcatcagctgaccacctcgctgtatcagccagcaacgaggggaaggtgaagaaacatgataggccatatagaatctgccctatgtttacttttttaacccagataattatttttgtgtgcagtatctaagctcctgattgtgtaacctgggacttctggcaccttttgttccattcattttatgtataaaatgcatgccaaagcacactgtgccctctggtacccttgcttccaatcgccaaccatgctcatttccttcctttttttgtggtccctttttgtggtgatcattttaaaccacgtcatccaacaaatgttttatggtcaaccttagcttgttcataagccatagcaactgaaagattaaactcttaaatatgtgtctgggcagtggctattaaatagcaaaaaacaatcagattttagtattttattatttccttgtaaaatggctgaactaaattaaacccttgtttcccatttgttctataatttatagtgaaactgagaacaaaactatctttataaatgatagctaaaagtatttccagatatttaaacaatttaaaataaatttcttctgcagagatgcaaagcatctcaacactggaatgaacaaatgccttaaattcaatggagtaaacctttagaatgaagaggaactgtcatttcacccaagccgaagacaacagccttatgcacttgtgtgctctgtctttgctgcttctcgtgtttcaagcctttcctgtgggatcagcacagcaaagtgcaacttaccaaatggtttaatgactggttaattctttcttctcccaatggaaaagcaatggcaacacaacagtagactgctggcttgacaatcttaaacgtgagcctttgcacatgtaggtttatcatcatttgagtatacgactaagcaagtcaatgaactttttttttttttttagcagtttaatttggtcctgagaatgttgcagtctttattaccccttttgcattaatccacttttctaaccaccttttaagctttaatttttaacactatacaccaagtctttgaaatcagtgatctgttatttaactctaaagcatttgacacttcttgccttaacagttttaaaaaccacacacaaaaaaactctgtaagtaatacagtaggccaaaagtttcatcctatctatcttgcagtttacctatctgatctgatctctgtaattatagttctgtcatttaaaatatactatttaaatctaatttttacatttcaaaaattatcttcagtagtaactaagtatattttctgtggattctgagaatgttatttttcagaatgtgagaatatatatgtacatttataatcttgtgactttaaagtctgttttcagatacagtatgtaaatacttgtaaaaaaatttgtataattttgtgataatgtagtttcccaaaaaaattatttagaaggcattatgttattagtaaatgagagcactgtatagaactgttcctattttctgcacttgccattccagctgcctccactgtccatacccacctcattcatcctgtcacagaaggcaggaaaactgggaactttaccaaagtagcactcagcctgagaggcctgtataatcatgcttttcaaactaaattcacttaaaaattaaaaagcagaattgaatattttaagcagcctcagtacctttggccaatgctgttttcatggtggattatgaacattatataatctttgggaaaagtgaaagtagtacaatttttagaataatgacaactgcctcactgcatctctccactcacacagcaaccgtgtagccccctaagctgcagtaccatgactaaccatgatgtcaatttcatatgctgatcctcacaacagcagtgcacaaacatgccccaaatattttaacagaatttagctcttccttaagctgtcttttcatagtaaaaacaaaacaaaaacacccaatgttaaaaccacataataaacttacaaacttgaaaaattagacacttcagatagataggcaataaaacttcatattatgaaagcaatatattccaagtttcaaagatttgacaagttctgtagagtatctttcatcagtacatgaaaacttccaaactgcatgatcttctgccaggcaggactgggtgctattcgctggtttgaggtcgaatccatttcaaggcatgtcgtggtgggacattaatggtgggatggtagaatgtgcagtccggtcttgtacattgagtgttaaacctacaatgttttggatgatagaagggacattccatcttcttacaagcagggaagtaacggcagagctgactactggaaggtggtgctggtggtgcaactggttttggagacagtactggaattcttctactcacatgagtgaagggacaatctggtttagtacactttgcatcatatttacaatttgggtgaacaaacaaacatttttcagcaaatttacaattggggaaggctttgcagggtgagatggggtgatggtaggcacactcatccccatttttacaagcaggccagtacttgcagcgctccaaaagtttttctggtttctgtgccacactcagttcactcatctcagcatttgggtcctcaagctgcctgctcagcaagtgcaactgctgtgggtggaggagacctctgagtcccttgtttgaggctgcagtttggtttacgggtttcattccttcaaagcacatgtcctcctcttgatctgacatgtatcctggggggctggggacaccatccagcgtcactataaacttgggacttgcaggtttatctggttgtacaagatctcgtgtctgcataaggtgtcctgaaagtacccgaagggaatctgcagtcttcatccccgactcttggtttggtgccactactacttcctcagacagctttggcttcttcagaataaatgatcttgtgtctgcatggaccatggattccatgtcatagtaatcttgatttttttctacagaatctccttttgtttcctcttctttaatggggggacttattctgggggtcctactttgtccctggaccacttctgctagcaattcttcttgagaagttcgagttctgggagcaactggaagtgtctgtttctgtggaactgtagagtagttagttgtttttgttacggattcttgagcttcagatatagccttcaaaatcagattcttgttagcttgtttagaaggtggaagagaaggtctcctttcaggctttgcaggcacagacacactgctggagatgcttcctgttcgagacccgtaatcatcatcttcttcctcctcttctccatcatgattgaatttttttactttaacaactgaacttaccacaggcaactttctcttccgaaagttttcatcctccatactcattttctccgagttgtttctaaagaacggactatacgtttcttctaagctgttaagcacctctggttcacacaaacgtcctgtttcatatacccaactactctgcatatcaagctgcttggcagcatgaatactattctgctgctgttgaaattgcaacctgtttaaatgaacaccactatctgcatttctacttgcaggtggtcgataaatttcaatagaagggcgagaagaaccatatgtaagtgtcactgtaggttttttctgagataagggattctcctgcacaaagttgaggtcttcgtcaatgagatcatctggttctggcttaatatcaatcacatcttcagagggtgctggctccctcaaaggtttcactgttgacattagtcgggttgcagctccatcatcgtaagtctgtctgacatttgtggtttttgactcctgcgaacttgtagaaactctggaatctcttttttcaggtctcgcgctaggaatggcaagtggtggcactgcagcttcatgcctcctctcatctccccgactgaaattgctcttgtttgaaggcacgttactatcaaagatgttggtatcagaagacttcagactagagggttcagttgtaacagagcgaagtttatctaatacaccatgaagccatacggtgaatcgaattgtgttgttccctagaaacagggacagatcctctgtcatttggtcctgacttttcttgttggccaccatcaccataatgtaatcaggaagttcttcatcaacataagctcctaattcttgtaatttccccttaatggcactccggatcttgcggctgatctcggtgccgatctccatggctctgcggcgtgcgggaactcagcactgcgcggcgcttggcttacccggaggctgccgcggactcctaccccgcagccgggacaccaccgcctcc

SEQ ID NO: 8555 - RNA, 4532 nt, Homo sapiens
  source 1..4532: mol_type = other RNA
aaaagtgcttacagtgcaggtagaaactctgtaaccttaagcatgtaaactacatagaataaaactgtttccactgcatttctgtccttcaaagtggccaacctgattaagtcagccttaatcactgctgctgtcagtttcacgactaaaggtcatattgactaagtagtcatcagctgaccacctcgctgtatcagccagcaacgaggggaaggtgaagaaacatgataggccatatagaatctgccctatgtttacttttttaacccagataattatttttgtgtgcagtatctaagctcctgattgtgtaacctgggacttctggcaccttttgttccattcattttatgtataaaatgcatgccaaagcacactgtgccctctggtacccttgcttccaatcgccaaccatgctcatttccttcctttttttgtggtccctttttgtggtgatcattttaaaccacgtcatccaacaaatgttttatggtcaaccttagcttgttcataagccatagcaactgaaagattaaactcttaaatatgtgtctgggcagtggctattaaatagcaaaaaacaatcagattttagtattttattatttccttgtaaaatggctgaactaaattaaacccttgtttcccatttgttctataatttatagtgaaactgagaacaaaactatctttataaatgatagctaaaagtatttccagatatttaaacaatttaaaataaatttcttctgcagagatgcaaagcatctcaacactggaatgaacaaatgccttaaattcaatggagtaaacctttagaatgaagaggaactgtcatttcacccaagccgaagacaacagccttatgcacttgtgtgctctgtctttgctgcttctcgtgtttcaagcctttcctgtgggatcagcacagcaaagtgcaacttaccaaatggtttaatgactggttaattctttcttctcccaatggaaaagcaatggcaacacaacagtagactgctggcttgacaatcttaaacgtgagcctttgcacatgtaggtttatcatcatttgagtatacgactaagcaagtcaatgaactttttttttttttttagcagtttaatttggtcctgagaatgttgcagtctttattaccccttttgcattaatccacttttctaaccaccttttaagctttaatttttaacactatacaccaagtctttgaaatcagtgatctgttatttaactctaaagcatttgacacttcttgccttaacagttttaaaaaccacacacaaaaaaactctgtaagtaatacagtaggccaaaagtttcatcctatctatcttgcagtttacctatctgatctgatctctgtaattatagttctgtcatttaaaatatactatttaaatctaatttttacatttcaaaaattatcttcagtagtaactaagtatattttctgtggattctgagaatgttatttttcagaatgtgagaatatatatgtacatttataatcttgtgactttaaagtctgttttcagatacagtatgtaaatacttgtaaaaaaatttgtataattttgtgataatgtagtttcccaaaaaaattatttagaaggcattatgttattagtaaatgagagcactgtatagaactgttcctattttctgcacttgccattccagctgcctccactgtccatacccacctcattcatcctgtcacagaaggcaggaaaactgggaactttaccaaagtagcactcagcctgagaggcctgtataatcatgcttttcaaactaaattcacttaaaaattaaaaagcagaattgaatattttaagcagcctcagtacctttggccaatgctgttttcatggtggattatgaacattatataatctttgggaaaagtgaaagtagtacaatttttagaataatgacaactgcctcactgcatctctccactcacacagcaaccgtgtagccccctaagctgcagtaccatgactaaccatgatgtcaatttcatatgctgatcctcacaacagcagtgcacaaacatgccccaaatattttaacagaatttagctcttccttaagctgtcttttcatagtaaaaacaaaacaaaaacacccaatgttaaaaccacataataaacttacaaacttgaaaaattagacacttcagatagataggcaataaaacttcatattatgaaagcaatatattccaagtttcaaagatttgacaagttctgtagagtatctttcatcagtacatgaaaacttccaaactgcatgatcttctgccaggcaggactgggtgctattcgctggtttgaggtcgaatccatttcaaggcatgtcgtggtgggacattaatggtgggatggtagaatgtgcagtccggtcttgtacattgagtgttaaacctacaatgttttggatgatagaagggacattccatcttcttacaagcagggaagtaacggcagagctgactactggaaggtggtgctggtggtgcaactggttttggagacagtactggaattcttctactcacatgagtgaagggacaatctggtttagtacactttgcatcatatttacaatttgggtgaacaaacaaacatttttcagcaaatttacaattggggaaggctttgcagggtgagatggggtgatggtaggcacactcatccccatttttacaagcaggccagtacttgcagcgctccaaaagtttttctggtttctgtgccacactcagttcactcatctcagcgttagaaaagctaccatttgggtcctcaagctgcctgctcagcaagtgcaactgctgtgggtggaggagacctctgagtcccttgtttgaggctgcagtttggtttacgggtttcattccttcaaagcacatgtcctcctcttgatctgacatgtatcctggggggctggggacaccatccagcgtcactataaacttgggacttgcaggtttatctggttgtacaagatctcgtgtctgcataaggtgtcctgaaagtacccgaagggaatctgcagtcttcatccccgactcttggtttggtgccactactacttcctcagacagctttggcttcttcagaataaatgatcttgtgtctgcatggaccatggattccatgtcatagtaatcttgactcatctgcagagtttctgccattactgggtcgatttgcagtcgggataataattgcctctgttgagttccttgatttttttctacagaatctccttttgtttcctcttctttaatggggggacttattctgggggtcctactttgtccctggaccacttctgctagcaattcttcttgagaagttcgagttctgggagcaactggaagtgtctgtttctgtggaactgtagagtagttagttgtttttgttacggattcttgagcttcagatatagccttcaaaatcagattcttgttagcttgtttagaaggtggaagagaaggtctcctttcaggctttgcaggcacagacacactgctggagatgcttcctgttcgagacccgtaatcatcatcttcttcctcctcttctccatcatgattgaatttttttactttaacaactgaacttaccacaggcaactttctcttccgaaagttttcatcctccatactcattttctccgagttgtttctaaagaacggactatacgtttcttctaagctgttaagcacctctggttcacacaaacgtcctgtttcatatacccaactactctgcatatcaagctgcttggcagcatgaatactattctgctgctgttgaaattgcaacctgtttaaatgaacaccactatctgcatttctacttgcaggtggtcgataaatttcaatagaagggcgagaagaaccatatgtaagtgtcactgtaggttttttctgagataagggattctcctgcacaaagttgaggtcttcgtcaatgagatcatctggttctggcttaatatcaatcacatcttcagagggtgctggctccctcaaaggtttcactgttgacattagtcgggttgcagctccatcatcgtaagtctgtctgacatttgtggtttttgactcctgcgaacttgtagaaactctggaatctcttttttcaggtctcgcgctaggaatggcaagtggtggcactgcagcttcatgcctcctctcatctccccgactgaaattgctcttgtttgaaggcacgttactatcaaagatgttggtatcagaagacttcagactagagggttcagttgtaacagagcgaagtttatctaatacaccatgaagccaacataagctcctaattcttgtaatttccccttaatggcactccggatcttgcggctgatctcggtgccgatctccatggctctgcggcgtgcgggaactcagcactgcgcggcgcttggcttacccggaggctgccgcggactcctaccccgcagccgggacaccaccgcctcc

SEQ ID NO: 8556 - RNA, 4647 nt, Homo sapiens
  source 1..4647: mol_type = other RNA
aaaagtgcttacagtgcaggtagaaactctgtaaccttaagcatgtaaactacatagaataaaactgtttccactgcatttctgtccttcaaagtggccaacctgattaagtcagccttaatcactgctgctgtcagtttcacgactaaaggtcatattgactaagtagtcatcagctgaccacctcgctgtatcagccagcaacgaggggaaggtgaagaaacatgataggccatatagaatctgccctatgtttacttttttaacccagataattatttttgtgtgcagtatctaagctcctgattgtgtaacctgggacttctggcaccttttgttccattcattttatgtataaaatgcatgccaaagcacactgtgccctctggtacccttgcttccaatcgccaaccatgctcatttccttcctttttttgtggtccctttttgtggtgatcattttaaaccacgtcatccaacaaatgttttatggtcaaccttagcttgttcataagccatagcaactgaaagattaaactcttaaatatgtgtctgggcagtggctattaaatagcaaaaaacaatcagattttagtattttattatttccttgtaaaatggctgaactaaattaaacccttgtttcccatttgttctataatttatagtgaaactgagaacaaaactatctttataaatgatagctaaaagtatttccagatatttaaacaatttaaaataaatttcttctgcagagatgcaaagcatctcaacactggaatgaacaaatgccttaaattcaatggagtaaacctttagaatgaagaggaactgtcatttcacccaagccgaagacaacagccttatgcacttgtgtgctctgtctttgctgcttctcgtgtttcaagcctttcctgtgggatcagcacagcaaagtgcaacttaccaaatggtttaatgactggttaattctttcttctcccaatggaaaagcaatggcaacacaacagtagactgctggcttgacaatcttaaacgtgagcctttgcacatgtaggtttatcatcatttgagtatacgactaagcaagtcaatgaactttttttttttttttagcagtttaatttggtcctgagaatgttgcagtctttattaccccttttgcattaatccacttttctaaccaccttttaagctttaatttttaacactatacaccaagtctttgaaatcagtgatctgttatttaactctaaagcatttgacacttcttgccttaacagttttaaaaaccacacacaaaaaaactctgtaagtaatacagtaggccaaaagtttcatcctatctatcttgcagtttacctatctgatctgatctctgtaattatagttctgtcatttaaaatatactatttaaatctaatttttacatttcaaaaattatcttcagtagtaactaagtatattttctgtggattctgagaatgttatttttcagaatgtgagaatatatatgtacatttataatcttgtgactttaaagtctgttttcagatacagtatgtaaatacttgtaaaaaaatttgtataattttgtgataatgtagtttcccaaaaaaattatttagaaggcattatgttattagtaaatgagagcactgtatagaactgttcctattttctgcacttgccattccagctgcctccactgtccatacccacctcattcatcctgtcacagaaggcaggaaaactgggaactttaccaaagtagcactcagcctgagaggcctgtataatcatgcttttcaaactaaattcacttaaaaattaaaaagcagaattgaatattttaagcagcctcagtacctttggccaatgctgttttcatggtggattatgaacattatataatctttgggaaaagtgaaagtagtacaatttttagaataatgacaactgcctcactgcatctctccactcacacagcaaccgtgtagccccctaagctgcagtaccatgactaaccatgatgtcaatttcatatgctgatcctcacaacagcagtgcacaaacatgccccaaatattttaacagaatttagctcttccttaagctgtcttttcatagtaaaaacaaaacaaaaacacccaatgttaaaaccacataataaacttacaaacttgaaaaattagacacttcagatagataggcaataaaacttcatattatgaaagcaatatattccaagtttcaaagatttgacaagttctgtagagtatctttcatcagtacatgaaaacttccaaactgcatgatcttctgccaggcaggactgggtgctattcgctggtttgaggtcgaatccatttcaaggcatgtcgtggtgggacattaatggtgggatggtagaatgtgcagtccggtcttgtacattgagtgttaaacctacaatgttttggatgatagaagggacattccatcttcttacaagcagggaagtaacggcagagctgactactggaaggtggtgctggtggtgcaactggttttggagacagtactggaattcttctactcacatgagtgaagggacaatctggtttagtacactttgcatcatatttacaatttgggtgaacaaacaaacatttttcagcaaatttacaattggggaaggctttgcagggtgagatggggtgatggtaggcacactcatccccatttttacaagcaggccagtacttgcagcgctccaaaagtttttctggtttctgtgccacactcagttcactcatctcagcgttagaaaagctaccatttgggtcctcaagctgcctgctcagcaagtgcaactgctgtgggtggaggagacctctgagtcccttgtttgaggctgcagtttggtttacgggtttcattccttcaaagcacatgtcctcctcttgatctgacatgtatcctggggggctggggacaccatccagcgtcactataaacttgggacttgcaggtttatctggttgtacaagatctcgtgtctgcataaggtgtcctgaaagtacccgaagggaatctgcagtcttcatccccgactcttggtttggtgccactactacttcctcagacagctttggcttcttcagaataaatgatcttgtgtctgcatggaccatggattccatgtcatagtaatcttgactcatctgcagagtttctgccattactgggtcgatttgcagtcgggataataattgcctctgttgagttccttgatttttttctacagaatctccttttgtttcctcttctttaatggggggacttattctgggggtcctactttgtccctggaccacttctgctagcaattcttcttgagaagttcgagttctgggagcaactggaagtgtctgtttctgtggaactgtagagtagttagttgtttttgttacggattcttgagcttcagatatagccttcaaaatcagattcttgttagcttgtttagaaggtggaagagaaggtctcctttcaggctttgcaggcacagacacactgctggagatgcttcctgttcgagacccgtaatcatcatcttcttcctcctcttctccatcatgattgaatttttttactttaacaactgaacttaccacaggcaactttctcttccgaaagttttcatcctccatactcattttctccgagttgtttctaaagaacggactatacgtttcttctaagctgttaagcacctctggttcacacaaacgtcctgtttcatatacccaactactctgcatatcaagctgcttggcagcatgaatactattctgctgctgttgaaattgcaacctgtttaaatgaacaccactatctgcatttctacttgcaggtggtcgataaatttcaatagaagggcgagaagaaccatatgtaagtgtcactgtaggttttttctgagataagggattctcctgcacaaagttgaggtcttcgtcaatgagatcatctggttctggcttaatatcaatcacatcttcagagggtgctggctccctcaaaggtttcactgttgacattagtcgggttgcagctccatcatcgtaagtctgtctgacatttgtggtttttgactcctgcgaacttgtagaaactctggaatctcttttttcaggtctcgcgctaggaatggcaagtggtggcactgcagcttcatgcctcctctcatctccccgactgaaattgctcttgtttgaaggcacgttactatcaaagatgttggtatcagaagacttcagactagagggttcagttgtaacagagcgaagtttatctaatacaccatgaagccatacggtgaatcgaattgtgttgttccctagaaacagggacagatcctctgtcatttggtcctgacttttcttgttggccaccatcaccataatgtaatcaggaagttcttcatcaacataagctcctaattcttgtaatttccccttaatggcactccggatcttgcggctgatctcggtgccgatctccatggctctgcggcgtgcgggaactcagcactgcgcggcgcttggcttacccggaggctgccgcggactcctaccccgcagccgggacaccaccgcctcc

SEQ ID NO: 8557 - RNA, 4623 nt, Homo sapiens
  source 1..4623: mol_type = other RNA
aaaagtgcttacagtgcaggtagaaactctgtaaccttaagcatgtaaactacatagaataaaactgtttccactgcatttctgtccttcaaagtggccaacctgattaagtcagccttaatcactgctgctgtcagtttcacgactaaaggtcatattgactaagtagtcatcagctgaccacctcgctgtatcagccagcaacgaggggaaggtgaagaaacatgataggccatatagaatctgccctatgtttacttttttaacccagataattatttttgtgtgcagtatctaagctcctgattgtgtaacctgggacttctggcaccttttgttccattcattttatgtataaaatgcatgccaaagcacactgtgccctctggtacccttgcttccaatcgccaaccatgctcatttccttcctttttttgtggtccctttttgtggtgatcattttaaaccacgtcatccaacaaatgttttatggtcaaccttagcttgttcataagccatagcaactgaaagattaaactcttaaatatgtgtctgggcagtggctattaaatagcaaaaaacaatcagattttagtattttattatttccttgtaaaatggctgaactaaattaaacccttgtttcccatttgttctataatttatagtgaaactgagaacaaaactatctttataaatgatagctaaaagtatttccagatatttaaacaatttaaaataaatttcttctgcagagatgcaaagcatctcaacactggaatgaacaaatgccttaaattcaatggagtaaacctttagaatgaagaggaactgtcatttcacccaagccgaagacaacagccttatgcacttgtgtgctctgtctttgctgcttctcgtgtttcaagcctttcctgtgggatcagcacagcaaagtgcaacttaccaaatggtttaatgactggttaattctttcttctcccaatggaaaagcaatggcaacacaacagtagactgctggcttgacaatcttaaacgtgagcctttgcacatgtaggtttatcatcatttgagtatacgactaagcaagtcaatgaactttttttttttttttagcagtttaatttggtcctgagaatgttgcagtctttattaccccttttgcattaatccacttttctaaccaccttttaagctttaatttttaacactatacaccaagtctttgaaatcagtgatctgttatttaactctaaagcatttgacacttcttgccttaacagttttaaaaaccacacacaaaaaaactctgtaagtaatacagtaggccaaaagtttcatcctatctatcttgcagtttacctatctgatctgatctctgtaattatagttctgtcatttaaaatatactatttaaatctaatttttacatttcaaaaattatcttcagtagtaactaagtatattttctgtggattctgagaatgttatttttcagaatgtgagaatatatatgtacatttataatcttgtgactttaaagtctgttttcagatacagtatgtaaatacttgtaaaaaaatttgtataattttgtgataatgtagtttcccaaaaaaattatttagaaggcattatgttattagtaaatgagagcactgtatagaactgttcctattttctgcacttgccattccagctgcctccactgtccatacccacctcattcatcctgtcacagaaggcaggaaaactgggaactttaccaaagtagcactcagcctgagaggcctgtataatcatgcttttcaaactaaattcacttaaaaattaaaaagcagaattgaatattttaagcagcctcagtacctttggccaatgctgttttcatggtggattatgaacattatataatctttgggaaaagtgaaagtagtacaatttttagaataatgacaactgcctcactgcatctctccactcacacagcaaccgtgtagccccctaagctgcagtaccatgactaaccatgatgtcaatttcatatgctgatcctcacaacagcagtgcacaaacatgccccaaatattttaacagaatttagctcttccttaagctgtcttttcatagtaaaaacaaaacaaaaacacccaatgttaaaaccacataataaacttacaaacttgaaaaattagacacttcagatagataggcaataaaacttcatattatgaaagcaatatattccaagtttcaaagatttgacaagttctgtagagtatctttcatcagtacatgaaaacttccaaactgcatgatcttctgccaggcaggactgggtgctattcgctggtttgaggtcgaatccatttcaaggcatgtcgtggtgggacattaatggtgggatggtagaatgtgcagtccggtcttgtacattgagtgttaaacctacaatgttttggatgatagaagggacattccatcttcttacaagcagggaagtaacggcagagctgactactggaaggtggtgctggtggtgcaactggttttggagacagtactggaattcttctactcacatgagtgaagggacaatctggtttagtacactttgcatcatatttacaatttgggtgaacaaacaaacatttttcagcaaatttacaattggggaaggctttgcagggtgagatggggtgatggtaggcacactcatccccatttttacaagcaggccagtacttgcagcgctccaaaagtttttctggtttctgtgccacactcagttcactcatctcagcgttagaaaagctaccatttgggtcctcaagctgcctgctcagcaagtgcaactgctgtgggtggaggagacctctgagtcccttgtttgaggctgcagtttggtttacgggtttcattccttcaaagcacatgtcctcctcttgatctgacatgtatcctggggggctggggacaccatccagcgtcactataaacttgggacttgcaggtttatctggttgtacaagatctcgtgtctgcataaggtgtcctgaaagtacccgaagggaatctgcagtcttcatccccgactcttggtttggtgccactactacttcctcagacagctttggcttcttcagaataaatgatcttgtgtctgcatggaccatggattccatgtcatagtaatcttgactcatctgcagagtttctgccattactgggtcgatttgcagtcgggataataattgcctctgttgagttccttgatttttttctacagaatctccttttgtttcctcttctttaatggggggacttattctgggggtcctactttgtccctggaccacttctgctagcaattcttcttgagaagttcgagttctgggagcaactggaagtgtctgtttctgtggaactgtagagtagttagttgtttttgttacggattcttgagcttcagatatagccttcaaaatcagattcttgttagcttgtttagaaggtggaagagaaggtctcctttcaggctttgcaggcacagacacactgctggagatgcttcctgttcgagacccgtaatcatcatcttcttcctcctcttctccatcatgattgaatttttttactttaacaactgaacttaccacaggcaactttctcttccgaaagttttcatcctccatactcattttctccgagttgtttctaaagaacggactatacgtttcttctaagctgttaagcacctctggttcacacaaacgtcctgtttcatatacccaactactctgcatatcaagctgcttggcagcatgaatactattctgctgctgttgaaattgcaacctgtttaaatgaacaccactatctgcatttctacttgcaggtggtcgataaatttcaatagaagggcgagaagaaccatatgtaagtgtcactgtaggttttttctgagataagggattctcctgcacaaagttgaggtcttcgtcaatgagatcatctggttctggcttaatatcaatcacatcttcagagggtgctggctccctcaaaggtttcactgttgacattagtcgggttgcagctccatcatcgtaagtctgtctgacatttgtggtttttgactcctgcgaacttgtagaaactctggaatctcttttttcaggtctcgcgctaggaatggcaagtggtggcactgcagcttcatgcctcctctcatctccccgactgaaattgctcttgtttgaaggcacgttactatcaaagatgttggtatcagaagacttcagactagagggttcagttgtaacagagcgaagtttatctaatacaccatgaagccatacggtgaatcgaattgtgttgttccctagaaacagggacagatcctctgtcatttggtcctgacttttcttgttggccaccatcaccataatgtaatcaggaagttcttcatcaacataagctcctaattcttgtaatttccccttaatggcactctcccgcagcggatccaaagcggcgccgtgcgccgcggtggtggctccagccgggcctgcgcctgtccttccatttcccggcggctacttcagccgcagccacgctccg

SEQ ID NO: 8558 - RNA, 4828 nt, Homo sapiens
  source 1..4828: mol_type = other RNA
aaaagtgcttacagtgcaggtagaaactctgtaaccttaagcatgtaaactacatagaataaaactgtttccactgcatttctgtccttcaaagtggccaacctgattaagtcagccttaatcactgctgctgtcagtttcacgactaaaggtcatattgactaagtagtcatcagctgaccacctcgctgtatcagccagcaacgaggggaaggtgaagaaacatgataggccatatagaatctgccctatgtttacttttttaacccagataattatttttgtgtgcagtatctaagctcctgattgtgtaacctgggacttctggcaccttttgttccattcattttatgtataaaatgcatgccaaagcacactgtgccctctggtacccttgcttccaatcgccaaccatgctcatttccttcctttttttgtggtccctttttgtggtgatcattttaaaccacgtcatccaacaaatgttttatggtcaaccttagcttgttcataagccatagcaactgaaagattaaactcttaaatatgtgtctgggcagtggctattaaatagcaaaaaacaatcagattttagtattttattatttccttgtaaaatggctgaactaaattaaacccttgtttcccatttgttctataatttatagtgaaactgagaacaaaactatctttataaatgatagctaaaagtatttccagatatttaaacaatttaaaataaatttcttctgcagagatgcaaagcatctcaacactggaatgaacaaatgccttaaattcaatggagtaaacctttagaatgaagaggaactgtcatttcacccaagccgaagacaacagccttatgcacttgtgtgctctgtctttgctgcttctcgtgtttcaagcctttcctgtgggatcagcacagcaaagtgcaacttaccaaatggtttaatgactggttaattctttcttctcccaatggaaaagcaatggcaacacaacagtagactgctggcttgacaatcttaaacgtgagcctttgcacatgtaggtttatcatcatttgagtatacgactaagcaagtcaatgaactttttttttttttttagcagtttaatttggtcctgagaatgttgcagtctttattaccccttttgcattaatccacttttctaaccaccttttaagctttaatttttaacactatacaccaagtctttgaaatcagtgatctgttatttaactctaaagcatttgacacttcttgccttaacagttttaaaaaccacacacaaaaaaactctgtaagtaatacagtaggccaaaagtttcatcctatctatcttgcagtttacctatctgatctgatctctgtaattatagttctgtcatttaaaatatactatttaaatctaatttttacatttcaaaaattatcttcagtagtaactaagtatattttctgtggattctgagaatgttatttttcagaatgtgagaatatatatgtacatttataatcttgtgactttaaagtctgttttcagatacagtatgtaaatacttgtaaaaaaatttgtataattttgtgataatgtagtttcccaaaaaaattatttagaaggcattatgttattagtaaatgagagcactgtatagaactgttcctattttctgcacttgccattccagctgcctccactgtccatacccacctcattcatcctgtcacagaaggcaggaaaactgggaactttaccaaagtagcactcagcctgagaggcctgtataatcatgcttttcaaactaaattcacttaaaaattaaaaagcagaattgaatattttaagcagcctcagtacctttggccaatgctgttttcatggtggattatgaacattatataatctttgggaaaagtgaaagtagtacaatttttagaataatgacaactgcctcactgcatctctccactcacacagcaaccgtgtagccccctaagctgcagtaccatgactaaccatgatgtcaatttcatatgctgatcctcacaacagcagtgcacaaacatgccccaaatattttaacagaatttagctcttccttaagctgtcttttcatagtaaaaacaaaacaaaaacacccaatgttaaaaccacataataaacttacaaacttgaaaaattagacacttcagatagataggcaataaaacttcatattatgaaagcaatatattccaagtttcaaagatttgacaagttctgtagagtatctttcatcagtacatgaaaacttccaaactgcatgatcttctgccaggcaggactgggtgctattcgctggtttgaggtcgaatccatttcaaggcatgtcgtggtgggacattaatggtgggatggtagaatgtgcagtccggtcttgtacattgagtgttaaacctacaatgttttggatgatagaagggacattccatcttcttacaagcagggaagtaacggcagagctgactactggaaggtggtgctggtggtgcaactggttttggagacagtactggaattcttctactcacatgagtgaagggacaatctggtttagtacactttgcatcatatttacaatttgggtgaacaaacaaacatttttcagcaaatttacaattggggaaggctttgcagggtgagatggggtgatggtaggcacactcatccccatttttacaagcaggccagtacttgcagcgctccaaaagtttttctggtttctgtgccacactcagttcactcatctcagcgttagaaaagctaccatttgggtcctcaagctgcctgctcagcaagtgcaactgctgtgggtggaggagacctctgagtcccttgtttgaggctgcagtttggtttacgggtttcattccttcaaagcacatgtcctcctcttgatctgacatgtatcctggggggctggggacaccatccagcgtcactataaacttgggacttgcaggtttatctggttgtacaagatctcgtgtctgcataaggtgtcctgaaagtacccgaagggaatctgcagtcttcatccccgactcttggtttggtgccactactacttcctcagacagctttggcttcttcagaataaatgatcttgtgtctgcatggaccatggattccatgtcatagtaatcttgactcatctgcagagtttctgccattactgggtcgatttgcagtcgggataataattgcctctgttgagttccttgatttttttctacagaatctccttttgtttcctcttctttaatggggggacttattctgggggtcctactttgtccctggaccacttctgctagcaattcttcttgagaagttcgagttctgggagcaactggaagtgtctgtttctgtggaactgtagagtagttagttgtttttgttacggattcttgagcttcagatatagccttcaaaatcagattcttgttagcttgtttagaaggtggaagagaaggtctcctttcaggctttgcaggcacagacacactgctggagatgcttcctgttcgagacccgtaatcatcatcttcttcctcctcttctccatcatgattgaatttttttactttaacaactgaacttaccacaggcaactttctcttccgaaagttttcatcctccatactcattttctccgagttgtttctaaagaacggactatacgtttcttctaagctgttaagcacctctggttcacacaaacgtcctgtttcatatacccaactactctgcatatcaagctgcttggcagcatgaatactattctgctgctgttgaaattgcaacctgtttaaatgaacaccactatctgcatttctacttgcaggtggtcgataaatttcaatagaagggcgagaagaaccatatgtaagtgtcactgtaggttttttctgagataagggattctcctgcacaaagttgaggtcttcgtcaatgagatcatctggttctggcttaatatcaatcacatcttcagagggtgctggctccctcaaaggtttcactgttgacattagtcgggttgcagctccatcatcgtaagtctgtctgacatttgtggtttttgactcctgcgaacttgtagaaactctggaatctcttttttcaggtctcgcgctaggaatggcaagtggtggcactgcagcttcatgcctcctctcatctccccgactgaaattgctcttgtttgaaggcacgttactatcaaagatgttggtatcagaagacttcagactagagggttcagttgtaacagagcgaagtttatctaatacaccatgaagccatacggtgaatcgaattgtgttgttccctagaaacagggacagatcctctgtcatttggtcctgacttttcttgttggccaccatcaccataatgtaatcaggaagttcttcatctatttaaaaggaaaggtagatcaaaactttgtttcctcaaaactttcttcttaaagttgatgtgcttgaaaatatagatgtagctctaagctttagagtcgcagagctctactggaattacattggacaagatggcttagctttaatttttttctcttcattccacaggtatttcaaatacaacataagctcctaattcttgtaatttccccttaatggcactccggatcttgcggctgatctcggtgccgatctccatggctctgcggcgtgcgggaactcagcactgcgcggcgcttggcttacccggaggctgccgcggactcctaccccgcagccgggacaccaccgcctcc

SEQ ID NO: 8559 - RNA, 4457 nt, Homo sapiens
  source 1..4457: mol_type = other RNA
aaaagtgcttacagtgcaggtagaaactctgtaaccttaagcatgtaaactacatagaataaaactgtttccactgcatttctgtccttcaaagtggccaacctgattaagtcagccttaatcactgctgctgtcagtttcacgactaaaggtcatattgactaagtagtcatcagctgaccacctcgctgtatcagccagcaacgaggggaaggtgaagaaacatgataggccatatagaatctgccctatgtttacttttttaacccagataattatttttgtgtgcagtatctaagctcctgattgtgtaacctgggacttctggcaccttttgttccattcattttatgtataaaatgcatgccaaagcacactgtgccctctggtacccttgcttccaatcgccaaccatgctcatttccttcctttttttgtggtccctttttgtggtgatcattttaaaccacgtcatccaacaaatgttttatggtcaaccttagcttgttcataagccatagcaactgaaagattaaactcttaaatatgtgtctgggcagtggctattaaatagcaaaaaacaatcagattttagtattttattatttccttgtaaaatggctgaactaaattaaacccttgtttcccatttgttctataatttatagtgaaactgagaacaaaactatctttataaatgatagctaaaagtatttccagatatttaaacaatttaaaataaatttcttctgcagagatgcaaagcatctcaacactggaatgaacaaatgccttaaattcaatggagtaaacctttagaatgaagaggaactgtcatttcacccaagccgaagacaacagccttatgcacttgtgtgctctgtctttgctgcttctcgtgtttcaagcctttcctgtgggatcagcacagcaaagtgcaacttaccaaatggtttaatgactggttaattctttcttctcccaatggaaaagcaatggcaacacaacagtagactgctggcttgacaatcttaaacgtgagcctttgcacatgtaggtttatcatcatttgagtatacgactaagcaagtcaatgaactttttttttttttttagcagtttaatttggtcctgagaatgttgcagtctttattaccccttttgcattaatccacttttctaaccaccttttaagctttaatttttaacactatacaccaagtctttgaaatcagtgatctgttatttaactctaaagcatttgacacttcttgccttaacagttttaaaaaccacacacaaaaaaactctgtaagtaatacagtaggccaaaagtttcatcctatctatcttgcagtttacctatctgatctgatctctgtaattatagttctgtcatttaaaatatactatttaaatctaatttttacatttcaaaaattatcttcagtagtaactaagtatattttctgtggattctgagaatgttatttttcagaatgtgagaatatatatgtacatttataatcttgtgactttaaagtctgttttcagatacagtatgtaaatacttgtaaaaaaatttgtataattttgtgataatgtagtttcccaaaaaaattatttagaaggcattatgttattagtaaatgagagcactgtatagaactgttcctattttctgcacttgccattccagctgcctccactgtccatacccacctcattcatcctgtcacagaaggcaggaaaactgggaactttaccaaagtagcactcagcctgagaggcctgtataatcatgcttttcaaactaaattcacttaaaaattaaaaagcagaattgaatattttaagcagcctcagtacctttggccaatgctgttttcatggtggattatgaacattatataatctttgggaaaagtgaaagtagtacaatttttagaataatgacaactgcctcactgcatctctccactcacacagcaaccgtgtagccccctaagctgcagtaccatgactaaccatgatgtcaatttcatatgctgatcctcacaacagcagtgcacaaacatgccccaaatattttaacagaatttagctcttccttaagctgtcttttcatagtaaaaacaaaacaaaaacacccaatgttaaaaccacataataaacttacaaacttgaaaaattagacacttcagatagataggcaataaaacttcatattatgaaagcaatatattccaagtttcaaagatttgacaagttctgtagagtatctttcatcagtacatgaaaacttccaaactgcatgatcttctgccaggcaggactgggtgctattcgctggtttgaggtcgaatccatttcaaggcatgtcgtggtgggacattaatggtgggatggtagaatgtgcagtccggtcttgtacattgagtgttaaacctacaatgttttggatgatagaagggacattccatcttcttacaagcagggaagtaacggcagagctgactactggaaggtggtgctggtggtgcaactggttttggagacagtactggaattcttctactcacatgagtgaagggacaatctggtttagtacactttgcatcatatttacaatttgggtgaacaaacaaacatttttcagcaaatttacaattggggaaggctttgcagggtgagatggggtgatggtaggcacactcatccccatttttacaagcaggccagtacttgcagcgctccaaaagtttttctggtttctgtgccacactcagttcactcatctcagcgttagaaaagctaccatttgggtcctcaagctgcctgctcagcaagtgcaactgctgtgggtggaggagacctctgagtcccttgtttgaggctgcagtttggtttacgggtttcattccttcaaagcacatgtcctcctcttgatctgacatgtatcctggggggctggggacaccatccagcgtcactataaacttgggacttgcaggtttatctggttgtacaagatctcgtgtctgcataaggtgtcctgaaagtacccgaagggaatctgcagtcttcatccccgactcttggtttggtgccactactacttcctcagacagctttggcttcttcagaataaatgatcttgtgtctgcatggaccatggattccatgtcatagtaatcttgatttttttctacagaatctccttttgtttcctcttctttaatggggggacttattctgggggtcctactttgtccctggaccacttctgctagcaattcttcttgagaagttcgagttctgggagcaactggaagtgtctgtttctgtggaactgtagagtagttagttgtttttgttacggattcttgagcttcagatatagccttcaaaatcagattcttgttagcttgtttagaaggtggaagagaaggtctcctttcaggctttgcaggcacagacacactgctggagatgcttcctgttcgagacccgtaatcatcatcttcttcctcctcttctccatcatgattgaatttttttactttaacaactgaacttaccacaggcaactttctcttccgaaagttttcatcctccatactcattttctccgagttgtttctaaagaacggactatacgtttcttctaagctgttaagcacctctggttcacacaaacgtcctgtttcatatacccaactactctgcatatcaagctgcttggcagcatgaatactattctgctgctgttgaaattgcaacctgtttaaatgaacaccactatctgcatttctacttgcaggtggtcgataaatttcaatagaagggcgagaagaaccatatgtaagtgtcactgtaggttttttctgagataagggattctcctgcacaaagttgaggtcttcgtcaatgagatcatctggttctggcttaatatcaatcacatcttcagagggtgctggctccctcaaaggtttcactgttgacattagtcgggttgcagctccatcatcgtaagtctgtctgacatttgtggtttttgactcctgcgaacttgtagaaactctggaatctcttttttcaggtctcgcgctaggaatggcaagtggtggcactgcagcttcatgcctcctctcatctccccgactgaaattgctcttgtttgaaggcacgttactatcaaagatgttggtatcagaagacttcagactagagggttcagttgtaacagagcgaagtttatctaatacaccatgaagccaacataagctcctaattcttgtaatttccccttaatggcactccggatcttgcggctgatctcggtgccgatctccatggctctgcggcgtgcgggaactcagcactgcgcggcgcttggcttacccggaggctgccgcggactcctaccccgcagccgggacaccaccgcctcc

SEQ ID NO: 8560 - RNA, 4572 nt, Homo sapiens
  source 1..4572: mol_type = other RNA
aaaagtgcttacagtgcaggtagaaactctgtaaccttaagcatgtaaactacatagaataaaactgtttccactgcatttctgtccttcaaagtggccaacctgattaagtcagccttaatcactgctgctgtcagtttcacgactaaaggtcatattgactaagtagtcatcagctgaccacctcgctgtatcagccagcaacgaggggaaggtgaagaaacatgataggccatatagaatctgccctatgtttacttttttaacccagataattatttttgtgtgcagtatctaagctcctgattgtgtaacctgggacttctggcaccttttgttccattcattttatgtataaaatgcatgccaaagcacactgtgccctctggtacccttgcttccaatcgccaaccatgctcatttccttcctttttttgtggtccctttttgtggtgatcattttaaaccacgtcatccaacaaatgttttatggtcaaccttagcttgttcataagccatagcaactgaaagattaaactcttaaatatgtgtctgggcagtggctattaaatagcaaaaaacaatcagattttagtattttattatttccttgtaaaatggctgaactaaattaaacccttgtttcccatttgttctataatttatagtgaaactgagaacaaaactatctttataaatgatagctaaaagtatttccagatatttaaacaatttaaaataaatttcttctgcagagatgcaaagcatctcaacactggaatgaacaaatgccttaaattcaatggagtaaacctttagaatgaagaggaactgtcatttcacccaagccgaagacaacagccttatgcacttgtgtgctctgtctttgctgcttctcgtgtttcaagcctttcctgtgggatcagcacagcaaagtgcaacttaccaaatggtttaatgactggttaattctttcttctcccaatggaaaagcaatggcaacacaacagtagactgctggcttgacaatcttaaacgtgagcctttgcacatgtaggtttatcatcatttgagtatacgactaagcaagtcaatgaactttttttttttttttagcagtttaatttggtcctgagaatgttgcagtctttattaccccttttgcattaatccacttttctaaccaccttttaagctttaatttttaacactatacaccaagtctttgaaatcagtgatctgttatttaactctaaagcatttgacacttcttgccttaacagttttaaaaaccacacacaaaaaaactctgtaagtaatacagtaggccaaaagtttcatcctatctatcttgcagtttacctatctgatctgatctctgtaattatagttctgtcatttaaaatatactatttaaatctaatttttacatttcaaaaattatcttcagtagtaactaagtatattttctgtggattctgagaatgttatttttcagaatgtgagaatatatatgtacatttataatcttgtgactttaaagtctgttttcagatacagtatgtaaatacttgtaaaaaaatttgtataattttgtgataatgtagtttcccaaaaaaattatttagaaggcattatgttattagtaaatgagagcactgtatagaactgttcctattttctgcacttgccattccagctgcctccactgtccatacccacctcattcatcctgtcacagaaggcaggaaaactgggaactttaccaaagtagcactcagcctgagaggcctgtataatcatgcttttcaaactaaattcacttaaaaattaaaaagcagaattgaatattttaagcagcctcagtacctttggccaatgctgttttcatggtggattatgaacattatataatctttgggaaaagtgaaagtagtacaatttttagaataatgacaactgcctcactgcatctctccactcacacagcaaccgtgtagccccctaagctgcagtaccatgactaaccatgatgtcaatttcatatgctgatcctcacaacagcagtgcacaaacatgccccaaatattttaacagaatttagctcttccttaagctgtcttttcatagtaaaaacaaaacaaaaacacccaatgttaaaaccacataataaacttacaaacttgaaaaattagacacttcagatagataggcaataaaacttcatattatgaaagcaatatattccaagtttcaaagatttgacaagttctgtagagtatctttcatcagtacatgaaaacttccaaactgcatgatcttctgccaggcaggactgggtgctattcgctggtttgaggtcgaatccatttcaaggcatgtcgtggtgggacattaatggtgggatggtagaatgtgcagtccggtcttgtacattgagtgttaaacctacaatgttttggatgatagaagggacattccatcttcttacaagcagggaagtaacggcagagctgactactggaaggtggtgctggtggtgcaactggttttggagacagtactggaattcttctactcacatgagtgaagggacaatctggtttagtacactttgcatcatatttacaatttgggtgaacaaacaaacatttttcagcaaatttacaattggggaaggctttgcagggtgagatggggtgatggtaggcacactcatccccatttttacaagcaggccagtacttgcagcgctccaaaagtttttctggtttctgtgccacactcagttcactcatctcagcgttagaaaagctaccatttgggtcctcaagctgcctgctcagcaagtgcaactgctgtgggtggaggagacctctgagtcccttgtttgaggctgcagtttggtttacgggtttcattccttcaaagcacatgtcctcctcttgatctgacatgtatcctggggggctggggacaccatccagcgtcactataaacttgggacttgcaggtttatctggttgtacaagatctcgtgtctgcataaggtgtcctgaaagtacccgaagggaatctgcagtcttcatccccgactcttggtttggtgccactactacttcctcagacagctttggcttcttcagaataaatgatcttgtgtctgcatggaccatggattccatgtcatagtaatcttgatttttttctacagaatctccttttgtttcctcttctttaatggggggacttattctgggggtcctactttgtccctggaccacttctgctagcaattcttcttgagaagttcgagttctgggagcaactggaagtgtctgtttctgtggaactgtagagtagttagttgtttttgttacggattcttgagcttcagatatagccttcaaaatcagattcttgttagcttgtttagaaggtggaagagaaggtctcctttcaggctttgcaggcacagacacactgctggagatgcttcctgttcgagacccgtaatcatcatcttcttcctcctcttctccatcatgattgaatttttttactttaacaactgaacttaccacaggcaactttctcttccgaaagttttcatcctccatactcattttctccgagttgtttctaaagaacggactatacgtttcttctaagctgttaagcacctctggttcacacaaacgtcctgtttcatatacccaactactctgcatatcaagctgcttggcagcatgaatactattctgctgctgttgaaattgcaacctgtttaaatgaacaccactatctgcatttctacttgcaggtggtcgataaatttcaatagaagggcgagaagaaccatatgtaagtgtcactgtaggttttttctgagataagggattctcctgcacaaagttgaggtcttcgtcaatgagatcatctggttctggcttaatatcaatcacatcttcagagggtgctggctccctcaaaggtttcactgttgacattagtcgggttgcagctccatcatcgtaagtctgtctgacatttgtggtttttgactcctgcgaacttgtagaaactctggaatctcttttttcaggtctcgcgctaggaatggcaagtggtggcactgcagcttcatgcctcctctcatctccccgactgaaattgctcttgtttgaaggcacgttactatcaaagatgttggtatcagaagacttcagactagagggttcagttgtaacagagcgaagtttatctaatacaccatgaagccatacggtgaatcgaattgtgttgttccctagaaacagggacagatcctctgtcatttggtcctgacttttcttgttggccaccatcaccataatgtaatcaggaagttcttcatcaacataagctcctaattcttgtaatttccccttaatggcactccggatcttgcggctgatctcggtgccgatctccatggctctgcggcgtgcgggaactcagcactgcgcggcgcttggcttacccggaggctgccgcggactcctaccccgcagccgggacaccaccgcctcc

SEQ ID NO: 8561 - RNA, 4023 nt, Homo sapiens
  source 1..4023: mol_type = other RNA
aaaagtgcttacagtgcaggtagaaactctgtaaccttaagcatgtaaactacatagaataaaactgtttccactgcatttctgtccttcaaagtggccaacctgattaagtcagccttaatcactgctgctgtcagtttcacgactaaaggtcatattgactaagtagtcatcagctgaccacctcgctgtatcagccagcaacgaggggaaggtgaagaaacatgataggccatatagaatctgccctatgtttacttttttaacccagataattatttttgtgtgcagtatctaagctcctgattgtgtaacctgggacttctggcaccttttgttccattcattttatgtataaaatgcatgccaaagcacactgtgccctctggtacccttgcttccaatcgccaaccatgctcatttccttcctttttttgtggtccctttttgtggtgatcattttaaaccacgtcatccaacaaatgttttatggtcaaccttagcttgttcataagccatagcaactgaaagattaaactcttaaatatgtgtctgggcagtggctattaaatagcaaaaaacaatcagattttagtattttattatttccttgtaaaatggctgaactaaattaaacccttgtttcccatttgttctataatttatagtgaaactgagaacaaaactatctttataaatgatagctaaaagtatttccagatatttaaacaatttaaaataaatttcttctgcagagatgcaaagcatctcaacactggaatgaacaaatgccttaaattcaatggagtaaacctttagaatgaagaggaactgtcatttcacccaagccgaagacaacagccttatgcacttgtgtgctctgtctttgctgcttctcgtgtttcaagcctttcctgtgggatcagcacagcaaagtgcaacttaccaaatggtttaatgactggttaattctttcttctcccaatggaaaagcaatggcaacacaacagtagactgctggcttgacaatcttaaacgtgagcctttgcacatgtaggtttatcatcatttgagtatacgactaagcaagtcaatgaactttttttttttttttagcagtttaatttggtcctgagaatgttgcagtctttattaccccttttgcattaatccacttttctaaccaccttttaagctttaatttttaacactatacaccaagtctttgaaatcagtgatctgttatttaactctaaagcatttgacacttcttgccttaacagttttaaaaaccacacacaaaaaaactctgtaagtaatacagtaggccaaaagtttcatcctatctatcttgcagtttacctatctgatctgatctctgtaattatagttctgtcatttaaaatatactatttaaatctaatttttacatttcaaaaattatcttcagtagtaactaagtatattttctgtggattctgagaatgttatttttcagaatgtgagaatatatatgtacatttataatcttgtgactttaaagtctgttttcagatacagtatgtaaatacttgtaaaaaaatttgtataattttgtgataatgtagtttcccaaaaaaattatttagaaggcattatgttattagtaaatgagagcactgtatagaactgttcctattttctgcacttgccattccagctgcctccactgtccatacccacctcattcatcctgtcacagaaggcaggaaaactgggaactttaccaaagtagcactcagcctgagaggcctgtataatcatgcttttcaaactaaattcacttaaaaattaaaaagcagaattgaatattttaagcagcctcagtacctttggccaatgctgttttcatggtggattatgaacattatataatctttgggaaaagtgaaagtagtacaatttttagaataatgacaactgcctcactgcatctctccactcacacagcaaccgtgtagccccctaagctgcagtaccatgactaaccatgatgtcaatttcatatgctgatcctcacaacagcagtgcacaaacatgccccaaatattttaacagaatttagctcttccttaagctgtcttttcatagtaaaaacaaaacaaaaacacccaatgttaaaaccacataataaacttacaaacttgaaaaattagacacttcagatagataggcaataaaacttcatattatgaaagcaatatattccaagtttcaaagatttgacaagttctgtagagtatctttcatcagtacatgaaaacttccaaactgcatgatcttctgccaggcaggactgggtgctattcgctggtttgaggtcgaatccatttcaaggcatgtcgtggtgggacattaatggtgggatggtagaatgtgcagtccggtcttgtacattgagtgttaaacctacaatgttttggatgatagaagggacattccatcttcttacaagcagggaagtaacggcagagctgactactggaaggtggtgctggtggtgcaactggttttggagacagtactggaattcttctactcacatgagtgaagggacaatctggtttagtacactttgcatcatatttacaatttgggtgaacaaacaaacatttttcagcaaatttacaattggggaaggctttgcagggtgagatggggtgatggtaggcacactcatccccatttttacaagcaggccagtacttgcagcgctccaaaagtttttctggtttctgtgccacactcagttcactcatctcagctgtagagtagttagttgtttttgttacggattcttgagcttcagatatagccttcaaaatcagattcttgttagcttgtttagaaggtggaagagaaggtctcctttcaggctttgcaggcacagacacactgctggagatgcttcctgttcgagacccgtaatcatcatcttcttcctcctcttctccatcatgattgaatttttttactttaacaactgaacttaccacaggcaactttctcttccgaaagttttcatcctccatactcattttctccgagttgtttctaaagaacggactatacgtttcttctaagctgttaagcacctctggttcacacaaacgtcctgtttcatatacccaactactctgcatatcaagctgcttggcagcatgaatactattctgctgctgttgaaattgcaacctgtttaaatgaacaccactatctgcatttctacttgcaggtggtcgataaatttcaatagaagggcgagaagaaccatatgtaagtgtcactgtaggttttttctgagataagggattctcctgcacaaagttgaggtcttcgtcaatgagatcatctggttctggcttaatatcaatcacatcttcagagggtgctggctccctcaaaggtttcactgttgacattagtcgggttgcagctccatcatcgtaagtctgtctgacatttgtggtttttgactcctgcgaacttgtagaaactctggaatctcttttttcaggtctcgcgctaggaatggcaagtggtggcactgcagcttcatgcctcctctcatctccccgactgaaattgctcttgtttgaaggcacgttactatcaaagatgttggtatcagaagacttcagactagagggttcagttgtaacagagcgaagtttatctaatacaccatgaagccatacggtgaatcgaattgtgttgttccctagaaacagggacagatcctctgtcatttggtcctgacttttcttgttggccaccatcaccataatgtaatcaggaagttcttcatcaacataagctcctaattcttgtaatttccccttaatggcactccggatcttgcggctgatctcggtgccgatctccatggctctgcggcgtgcgggaactcagcactgcgcggcgcttggcttacccggaggctgccgcggactcctaccccgcagccgggacaccaccgcctcc

SEQ ID NO: 8562 - RNA, 4139 nt, Homo sapiens
  source 1..4139: mol_type = other RNA
aaaagtgcttacagtgcaggtagaaactctgtaaccttaagcatgtaaactacatagaataaaactgtttccactgcatttctgtccttcaaagtggccaacctgattaagtcagccttaatcactgctgctgtcagtttcacgactaaaggtcatattgactaagtagtcatcagctgaccacctcgctgtatcagccagcaacgaggggaaggtgaagaaacatgataggccatatagaatctgccctatgtttacttttttaacccagataattatttttgtgtgcagtatctaagctcctgattgtgtaacctgggacttctggcaccttttgttccattcattttatgtataaaatgcatgccaaagcacactgtgccctctggtacccttgcttccaatcgccaaccatgctcatttccttcctttttttgtggtccctttttgtggtgatcattttaaaccacgtcatccaacaaatgttttatggtcaaccttagcttgttcataagccatagcaactgaaagattaaactcttaaatatgtgtctgggcagtggctattaaatagcaaaaaacaatcagattttagtattttattatttccttgtaaaatggctgaactaaattaaacccttgtttcccatttgttctataatttatagtgaaactgagaacaaaactatctttataaatgatagctaaaagtatttccagatatttaaacaatttaaaataaatttcttctgcagagatgcaaagcatctcaacactggaatgaacaaatgccttaaattcaatggagtaaacctttagaatgaagaggaactgtcatttcacccaagccgaagacaacagccttatgcacttgtgtgctctgtctttgctgcttctcgtgtttcaagcctttcctgtgggatcagcacagcaaagtgcaacttaccaaatggtttaatgactggttaattctttcttctcccaatggaaaagcaatggcaacacaacagtagactgctggcttgacaatcttaaacgtgagcctttgcacatgtaggtttatcatcatttgagtatacgactaagcaagtcaatgaactttttttttttttttagcagtttaatttggtcctgagaatgttgcagtctttattaccccttttgcattaatccacttttctaaccaccttttaagctttaatttttaacactatacaccaagtctttgaaatcagtgatctgttatttaactctaaagcatttgacacttcttgccttaacagttttaaaaaccacacacaaaaaaactctgtaagtaatacagtaggccaaaagtttcatcctatctatcttgcagtttacctatctgatctgatctctgtaattatagttctgtcatttaaaatatactatttaaatctaatttttacatttcaaaaattatcttcagtagtaactaagtatattttctgtggattctgagaatgttatttttcagaatgtgagaatatatatgtacatttataatcttgtgactttaaagtctgttttcagatacagtatgtaaatacttgtaaaaaaatttgtataattttgtgataatgtagtttcccaaaaaaattatttagaaggcattatgttattagtaaatgagagcactgtatagaactgttcctattttctgcacttgccattccagctgcctccactgtccatacccacctcattcatcctgtcacagaaggcaggaaaactgggaactttaccaaagtagcactcagcctgagaggcctgtataatcatgcttttcaaactaaattcacttaaaaattaaaaagcagaattgaatattttaagcagcctcagtacctttggccaatgctgttttcatggtggattatgaacattatataatctttgggaaaagtgaaagtagtacaatttttagaataatgacaactgcctcactgcatctctccactcacacagcaaccgtgtagccccctaagctgcagtaccatgactaaccatgatgtcaatttcatatgctgatcctcacaacagcagtgcacaaacatgccccaaatattttaacagaatttagctcttccttaagctgtcttttcatagtaaaaacaaaacaaaaacacccaatgttaaaaccacataataaacttacaaacttgaaaaattagacacttcagatagataggcaataaaacttcatattatgaaagcaatatattccaagtttcaaagatttgacaagttctgtagagtatctttcatcagtacatgaaaacttccaaactgcatgatcttctgccaggcaggactgggtgctattcgctggtttgaggtcgaatccatttcaaggcatgtcgtggtgggacattaatggtgggatggtagaatgtgcagtccggtcttgtacattgagtgttaaacctacaatgttttggatgatagaagggacattccatcttcttacaagcagggaagtaacggcagagctgactactggaaggtggtgctggtggtgcaactggttttggagacagtactggaattcttctactcacatgagtgaagggacaatctggtttagtacactttgcatcatatttacaatttgggtgaacaaacaaacatttttcagcaaatttacaattggggaaggctttgcagggtgagatggggtgatggtaggcacactcatccccatttttacaagcaggccagtacttgcagcgctccaaaagtttttctggtttctgtgccacactcagttcactcatctcagcttgactcatctgcagagtttctgccattactgggtcgatttgcagtcgggataataattgcctctgttgagttccttgatttttttctacagaatctccttttgtttcctcttctttaatggggggacttattctgggggtcctactttgtccctggaccacttctgctagcaattcttcttgagaagttcgagttctgggagcaactggaagtgtctgtttctgtggaactgtagagtagttagttgtttttgttacggattcttgagcttcagatatagccttcaaaatcagattcttgttagcttgtttagaaggtggaagagaaggtctcctttcaggctttgcaggcacagacacactgctggagatgcttcctgttcgagacccgtaatcatcatcttcttcctcctcttctccatcatgattgaatttttttactttaacaactgaacttaccacaggcaactttctcttccgaaagttttcatcctccatactcattttctccgagttgtttctaaagaacggactatacgtttcttctaagctgttaagcacctctggttcacacaaacgtcctgtttcatatacccaactactctgcatatcaagctgcttggcagcatgaatactattctgctgctgttgaaattgcaacctgtttaaatgaacaccactatctgcatttctacttgcaggtggtcgataaatttcaatagaagggcgagaagaaccatatgtaagtgtcactgtaggttttttctgagataagggattctcctgcacaaagttgaggtcttcgtcaatgagatcatctggttctggcttaatatcaatcacatcttcagagggtgctggctccctcaaaggtttcactgttgacattagtcgggttgcagctccatcatcgtaagtctgtctgacatttgtggtttttgactcctgcgaacttgtagaaactctggaatctcttttttcaggtctcgcgctaggaatggcaagtggtggcactgcagcttcatgcctcctctcatctccccgactgaaattgctcttgtttgaaggcacgttactatcaaagatgttggtatcagaagacttcagactagagggttcagttgtaacagagcgaagtttatctaatacaccatgaagccaacataagctcctaattcttgtaatttccccttaatggcactccggatcttgcggctgatctcggtgccgatctccatggctctgcggcgtgcgggaactcagcactgcgcggcgcttggcttacccggaggctgccgcggactcctaccccgcagccgggacaccaccgcctcc

SEQ ID NO: 8563 - RNA, 3570 nt, Homo sapiens
  source 1..3570: mol_type = other RNA
aaaagtgcttacagtgcaggtagaaactctgtaaccttaagcatgtaaactacatagaataaaactgtttccactgcatttctgtccttcaaagtggccaacctgattaagtcagccttaatcactgctgctgtcagtttcacgactaaaggtcatattgactaagtagtcatcagctgaccacctcgctgtatcagccagcaacgaggggaaggtgaagaaacatgataggccatatagaatctgccctatgtttacttttttaacccagataattatttttgtgtgcagtatctaagctcctgattgtgtaacctgggacttctggcaccttttgttccattcattttatgtataaaatgcatgccaaagcacactgtgccctctggtacccttgcttccaatcgccaaccatgctcatttccttcctttttttgtggtccctttttgtggtgatcattttaaaccacgtcatccaacaaatgttttatggtcaaccttagcttgttcataagccatagcaactgaaagattaaactcttaaatatgtgtctgggcagtggctattaaatagcaaaaaacaatcagattttagtattttattatttccttgtaaaatggctgaactaaattaaacccttgtttcccatttgttctataatttatagtgaaactgagaacaaaactatctttataaatgatagctaaaagtatttccagatatttaaacaatttaaaataaatttcttctgcagagatgcaaagcatctcaacactggaatgaacaaatgccttaaattcaatggagtaaacctttagaatgaagaggaactgtcatttcacccaagccgaagacaacagccttatgcacttgtgtgctctgtctttgctgcttctcgtgtttcaagcctttcctgtgggatcagcacagcaaagtgcaacttaccaaatggtttaatgactggttaattctttcttctcccaatggaaaagcaatggcaacacaacagtagactgctggcttgacaatcttaaacgtgagcctttgcacatgtaggtttatcatcatttgagtatacgactaagcaagtcaatgaactttttttttttttttagcagtttaatttggtcctgagaatgttgcagtctttattaccccttttgcattaatccacttttctaaccaccttttaagctttaatttttaacactatacaccaagtctttgaaatcagtgatctgttatttaactctaaagcatttgacacttcttgccttaacagttttaaaaaccacacacaaaaaaactctgtaagtaatacagtaggccaaaagtttcatcctatctatcttgcagtttacctatctgatctgatctctgtaattatagttctgtcatttaaaatatactatttaaatctaatttttacatttcaaaaattatcttcagtagtaactaagtatattttctgtggattctgagaatgttatttttcagaatgtgagaatatatatgtacatttataatcttgtgactttaaagtctgttttcagatacagtatgtaaatacttgtaaaaaaatttgtataattttgtgataatgtagtttcccaaaaaaattatttagaaggcattatgttattagtaaatgagagcactgtatagaactgttcctattttctgcacttgccattccagctgcctccactgtccatacccacctcattcatcctgtcacagaaggcaggaaaactgggaactttaccaaagtagcactcagcctgagaggcctgtataatcatgcttttcaaactaaattcacttaaaaattaaaaagcagaattgaatattttaagcagcctcagtacctttggccaatgctgttttcatggtggattatgaacattatataatctttgggaaaagtgaaagtagtacaatttttagaataatgacaactgcctcactgcatctctccactcacacagcaaccgtgtagccccctaagctgcagtaccatgactaaccatgatgtcaatttcatatgctgatcctcacaacagcagtgcacaaacatgccccaaatattttaacagaatttagctcttccttaagctgtcttttcatagtaaaaacaaaacaaaaacacccaatgttaaaaccacataataaacttacaaacttgaaaaattagacacttcagatagataggcaataaaacttcatattatgaaagcaatatattccaagtttcaaagatttgacaagttctgtagagtatctttcatcagtacatgaaaacttccaaactgcatgatcttctgccaggcaggactgggtgctattcgctggtttgaggtcgaatccatttcaaggcatgtcgtggtgggacattaatggtgggatggtagaatgtgcagtccggtcttgtacattgagtgttaaacctacaatgttttggatgatagaagggacattccatcttcttacaagcagggaagtaacggcagagctgactactggaaggtggtgctggtggtgcaactggttttggagacagtactggaattcttctactcacatgagtgaagggacaatctggtttagtacactttgcatcatatttacaatttgggtgaacaaacaaacatttttcagcaaatttacaattggggaaggctttgcagggtgagatggggtgatggtaggcacactcatccccatttttacaagcaggccagtacttgcagcgctccaaaagtttttctggtttctgtgccacactcagttcactcatctcagcttgactcatctgcagagtttctgccattactgggtcgatttgcagtcgggataataattgcctctgttgagttcctttctcaacgtttctaaggaagccgattatttttacatcagtagttcttgactgtgattcagtatcttcttcttgatcttcaaactgtctgttgcattcatatgttgttgaatattcattcattttaacctccaaagatgaaatttttgcttcattcttggacactctaacatttagatcaaaaagatttgcttccactgtcaaaatagctgctttcattcctttaatttcattgatatcagctgatattttccttaaaaggtgggaaatattgtctagctcattcagtgaacaagaggagcttgttatggaacctaagtccactggctccggtggaagaaaaattggtagaggtggtgatggaaactttgaagacattctcataaaggtgacaggaacctcaaagacattttcataaaattctctcccttaaaatctgataattttttcttcacagctcattaagttatttcatcgaaagtaaaagcagtgatcaaggctgttaccttaagacgtattaagagcaaataacatcttaaaacctgtaattcaaaagatggggttgtacatttctagagtcagaattcaaaactaaatgtgaaaaagctaaacgtaccagaccaattgctcttcgctacaactaagaagccctaatacgtagggccctacatcctctaagtaccatctgtat

SEQ ID NO: 8564 - RNA, 4064 nt, Homo sapiens
  source 1..4064: mol_type = other RNA
aaaagtgcttacagtgcaggtagaaactctgtaaccttaagcatgtaaactacatagaataaaactgtttccactgcatttctgtccttcaaagtggccaacctgattaagtcagccttaatcactgctgctgtcagtttcacgactaaaggtcatattgactaagtagtcatcagctgaccacctcgctgtatcagccagcaacgaggggaaggtgaagaaacatgataggccatatagaatctgccctatgtttacttttttaacccagataattatttttgtgtgcagtatctaagctcctgattgtgtaacctgggacttctggcaccttttgttccattcattttatgtataaaatgcatgccaaagcacactgtgccctctggtacccttgcttccaatcgccaaccatgctcatttccttcctttttttgtggtccctttttgtggtgatcattttaaaccacgtcatccaacaaatgttttatggtcaaccttagcttgttcataagccatagcaactgaaagattaaactcttaaatatgtgtctgggcagtggctattaaatagcaaaaaacaatcagattttagtattttattatttccttgtaaaatggctgaactaaattaaacccttgtttcccatttgttctataatttatagtgaaactgagaacaaaactatctttataaatgatagctaaaagtatttccagatatttaaacaatttaaaataaatttcttctgcagagatgcaaagcatctcaacactggaatgaacaaatgccttaaattcaatggagtaaacctttagaatgaagaggaactgtcatttcacccaagccgaagacaacagccttatgcacttgtgtgctctgtctttgctgcttctcgtgtttcaagcctttcctgtgggatcagcacagcaaagtgcaacttaccaaatggtttaatgactggttaattctttcttctcccaatggaaaagcaatggcaacacaacagtagactgctggcttgacaatcttaaacgtgagcctttgcacatgtaggtttatcatcatttgagtatacgactaagcaagtcaatgaactttttttttttttttagcagtttaatttggtcctgagaatgttgcagtctttattaccccttttgcattaatccacttttctaaccaccttttaagctttaatttttaacactatacaccaagtctttgaaatcagtgatctgttatttaactctaaagcatttgacacttcttgccttaacagttttaaaaaccacacacaaaaaaactctgtaagtaatacagtaggccaaaagtttcatcctatctatcttgcagtttacctatctgatctgatctctgtaattatagttctgtcatttaaaatatactatttaaatctaatttttacatttcaaaaattatcttcagtagtaactaagtatattttctgtggattctgagaatgttatttttcagaatgtgagaatatatatgtacatttataatcttgtgactttaaagtctgttttcagatacagtatgtaaatacttgtaaaaaaatttgtataattttgtgataatgtagtttcccaaaaaaattatttagaaggcattatgttattagtaaatgagagcactgtatagaactgttcctattttctgcacttgccattccagctgcctccactgtccatacccacctcattcatcctgtcacagaaggcaggaaaactgggaactttaccaaagtagcactcagcctgagaggcctgtataatcatgcttttcaaactaaattcacttaaaaattaaaaagcagaattgaatattttaagcagcctcagtacctttggccaatgctgttttcatggtggattatgaacattatataatctttgggaaaagtgaaagtagtacaatttttagaataatgacaactgcctcactgcatctctccactcacacagcaaccgtgtagccccctaagctgcagtaccatgactaaccatgatgtcaatttcatatgctgatcctcacaacagcagtgcacaaacatgccccaaatattttaacagaatttagctcttccttaagctgtcttttcatagtaaaaacaaaacaaaaacacccaatgttaaaaccacataataaacttacaaacttgaaaaattagacacttcagatagataggcaataaaacttcatattatgaaagcaatatattccaagtttcaaagatttgacaagttctgtagagtatctttcatcagtacatgaaaacttccaaactgcatgatcttctgccaggcaggactgggtgctattcgctggtttgaggtcgaatccatttcaaggcatgtcgtggtgggacattaatggtgggatggtagaatgtgcagtccggtcttgtacattgagtgttaaacctacaatgttttggatgatagaagggacattccatcttcttacaagcagggaagtaacggcagagctgactactggaaggtggtgctggtggtgcaactggttttggagacagtactggaattcttctactcacatgagtgaagggacaatctggtttagtacactttgcatcatatttacaatttgggtgaacaaacaaacatttttcagcaaatttacaattggggaaggctttgcagggtgagatggggtgatggtaggcacactcatccccatttttacaagcaggccagtacttgcagcgctccaaaagtttttctggtttctgtgccacactcagttcactcatctcagcttgatttttttctacagaatctccttttgtttcctcttctttaatggggggacttattctgggggtcctactttgtccctggaccacttctgctagcaattcttcttgagaagttcgagttctgggagcaactggaagtgtctgtttctgtggaactgtagagtagttagttgtttttgttacggattcttgagcttcagatatagccttcaaaatcagattcttgttagcttgtttagaaggtggaagagaaggtctcctttcaggctttgcaggcacagacacactgctggagatgcttcctgttcgagacccgtaatcatcatcttcttcctcctcttctccatcatgattgaatttttttactttaacaactgaacttaccacaggcaactttctcttccgaaagttttcatcctccatactcattttctccgagttgtttctaaagaacggactatacgtttcttctaagctgttaagcacctctggttcacacaaacgtcctgtttcatatacccaactactctgcatatcaagctgcttggcagcatgaatactattctgctgctgttgaaattgcaacctgtttaaatgaacaccactatctgcatttctacttgcaggtggtcgataaatttcaatagaagggcgagaagaaccatatgtaagtgtcactgtaggttttttctgagataagggattctcctgcacaaagttgaggtcttcgtcaatgagatcatctggttctggcttaatatcaatcacatcttcagagggtgctggctccctcaaaggtttcactgttgacattagtcgggttgcagctccatcatcgtaagtctgtctgacatttgtggtttttgactcctgcgaacttgtagaaactctggaatctcttttttcaggtctcgcgctaggaatggcaagtggtggcactgcagcttcatgcctcctctcatctccccgactgaaattgctcttgtttgaaggcacgttactatcaaagatgttggtatcagaagacttcagactagagggttcagttgtaacagagcgaagtttatctaatacaccatgaagccaacataagctcctaattcttgtaatttccccttaatggcactccggatcttgcggctgatctcggtgccgatctccatggctctgcggcgtgcgggaactcagcactgcgcggcgcttggcttacccggaggctgccgcggactcctaccccgcagccgggacaccaccgcctcc

SEQ ID NO: 8565 - RNA, 4179 nt, Homo sapiens
  source 1..4179: mol_type = other RNA
aaaagtgcttacagtgcaggtagaaactctgtaaccttaagcatgtaaactacatagaataaaactgtttccactgcatttctgtccttcaaagtggccaacctgattaagtcagccttaatcactgctgctgtcagtttcacgactaaaggtcatattgactaagtagtcatcagctgaccacctcgctgtatcagccagcaacgaggggaaggtgaagaaacatgataggccatatagaatctgccctatgtttacttttttaacccagataattatttttgtgtgcagtatctaagctcctgattgtgtaacctgggacttctggcaccttttgttccattcattttatgtataaaatgcatgccaaagcacactgtgccctctggtacccttgcttccaatcgccaaccatgctcatttccttcctttttttgtggtccctttttgtggtgatcattttaaaccacgtcatccaacaaatgttttatggtcaaccttagcttgttcataagccatagcaactgaaagattaaactcttaaatatgtgtctgggcagtggctattaaatagcaaaaaacaatcagattttagtattttattatttccttgtaaaatggctgaactaaattaaacccttgtttcccatttgttctataatttatagtgaaactgagaacaaaactatctttataaatgatagctaaaagtatttccagatatttaaacaatttaaaataaatttcttctgcagagatgcaaagcatctcaacactggaatgaacaaatgccttaaattcaatggagtaaacctttagaatgaagaggaactgtcatttcacccaagccgaagacaacagccttatgcacttgtgtgctctgtctttgctgcttctcgtgtttcaagcctttcctgtgggatcagcacagcaaagtgcaacttaccaaatggtttaatgactggttaattctttcttctcccaatggaaaagcaatggcaacacaacagtagactgctggcttgacaatcttaaacgtgagcctttgcacatgtaggtttatcatcatttgagtatacgactaagcaagtcaatgaactttttttttttttttagcagtttaatttggtcctgagaatgttgcagtctttattaccccttttgcattaatccacttttctaaccaccttttaagctttaatttttaacactatacaccaagtctttgaaatcagtgatctgttatttaactctaaagcatttgacacttcttgccttaacagttttaaaaaccacacacaaaaaaactctgtaagtaatacagtaggccaaaagtttcatcctatctatcttgcagtttacctatctgatctgatctctgtaattatagttctgtcatttaaaatatactatttaaatctaatttttacatttcaaaaattatcttcagtagtaactaagtatattttctgtggattctgagaatgttatttttcagaatgtgagaatatatatgtacatttataatcttgtgactttaaagtctgttttcagatacagtatgtaaatacttgtaaaaaaatttgtataattttgtgataatgtagtttcccaaaaaaattatttagaaggcattatgttattagtaaatgagagcactgtatagaactgttcctattttctgcacttgccattccagctgcctccactgtccatacccacctcattcatcctgtcacagaaggcaggaaaactgggaactttaccaaagtagcactcagcctgagaggcctgtataatcatgcttttcaaactaaattcacttaaaaattaaaaagcagaattgaatattttaagcagcctcagtacctttggccaatgctgttttcatggtggattatgaacattatataatctttgggaaaagtgaaagtagtacaatttttagaataatgacaactgcctcactgcatctctccactcacacagcaaccgtgtagccccctaagctgcagtaccatgactaaccatgatgtcaatttcatatgctgatcctcacaacagcagtgcacaaacatgccccaaatattttaacagaatttagctcttccttaagctgtcttttcatagtaaaaacaaaacaaaaacacccaatgttaaaaccacataataaacttacaaacttgaaaaattagacacttcagatagataggcaataaaacttcatattatgaaagcaatatattccaagtttcaaagatttgacaagttctgtagagtatctttcatcagtacatgaaaacttccaaactgcatgatcttctgccaggcaggactgggtgctattcgctggtttgaggtcgaatccatttcaaggcatgtcgtggtgggacattaatggtgggatggtagaatgtgcagtccggtcttgtacattgagtgttaaacctacaatgttttggatgatagaagggacattccatcttcttacaagcagggaagtaacggcagagctgactactggaaggtggtgctggtggtgcaactggttttggagacagtactggaattcttctactcacatgagtgaagggacaatctggtttagtacactttgcatcatatttacaatttgggtgaacaaacaaacatttttcagcaaatttacaattggggaaggctttgcagggtgagatggggtgatggtaggcacactcatccccatttttacaagcaggccagtacttgcagcgctccaaaagtttttctggtttctgtgccacactcagttcactcatctcagcttgatttttttctacagaatctccttttgtttcctcttctttaatggggggacttattctgggggtcctactttgtccctggaccacttctgctagcaattcttcttgagaagttcgagttctgggagcaactggaagtgtctgtttctgtggaactgtagagtagttagttgtttttgttacggattcttgagcttcagatatagccttcaaaatcagattcttgttagcttgtttagaaggtggaagagaaggtctcctttcaggctttgcaggcacagacacactgctggagatgcttcctgttcgagacccgtaatcatcatcttcttcctcctcttctccatcatgattgaatttttttactttaacaactgaacttaccacaggcaactttctcttccgaaagttttcatcctccatactcattttctccgagttgtttctaaagaacggactatacgtttcttctaagctgttaagcacctctggttcacacaaacgtcctgtttcatatacccaactactctgcatatcaagctgcttggcagcatgaatactattctgctgctgttgaaattgcaacctgtttaaatgaacaccactatctgcatttctacttgcaggtggtcgataaatttcaatagaagggcgagaagaaccatatgtaagtgtcactgtaggttttttctgagataagggattctcctgcacaaagttgaggtcttcgtcaatgagatcatctggttctggcttaatatcaatcacatcttcagagggtgctggctccctcaaaggtttcactgttgacattagtcgggttgcagctccatcatcgtaagtctgtctgacatttgtggtttttgactcctgcgaacttgtagaaactctggaatctcttttttcaggtctcgcgctaggaatggcaagtggtggcactgcagcttcatgcctcctctcatctccccgactgaaattgctcttgtttgaaggcacgttactatcaaagatgttggtatcagaagacttcagactagagggttcagttgtaacagagcgaagtttatctaatacaccatgaagccatacggtgaatcgaattgtgttgttccctagaaacagggacagatcctctgtcatttggtcctgacttttcttgttggccaccatcaccataatgtaatcaggaagttcttcatcaacataagctcctaattcttgtaatttccccttaatggcactccggatcttgcggctgatctcggtgccgatctccatggctctgcggcgtgcgggaactcagcactgcgcggcgcttggcttacccggaggctgccgcggactcctaccccgcagccgggacaccaccgcctcc

SEQ ID NO: 8566 - RNA, 4360 nt, Homo sapiens
  source 1..4360: mol_type = other RNA
aaaagtgcttacagtgcaggtagaaactctgtaaccttaagcatgtaaactacatagaataaaactgtttccactgcatttctgtccttcaaagtggccaacctgattaagtcagccttaatcactgctgctgtcagtttcacgactaaaggtcatattgactaagtagtcatcagctgaccacctcgctgtatcagccagcaacgaggggaaggtgaagaaacatgataggccatatagaatctgccctatgtttacttttttaacccagataattatttttgtgtgcagtatctaagctcctgattgtgtaacctgggacttctggcaccttttgttccattcattttatgtataaaatgcatgccaaagcacactgtgccctctggtacccttgcttccaatcgccaaccatgctcatttccttcctttttttgtggtccctttttgtggtgatcattttaaaccacgtcatccaacaaatgttttatggtcaaccttagcttgttcataagccatagcaactgaaagattaaactcttaaatatgtgtctgggcagtggctattaaatagcaaaaaacaatcagattttagtattttattatttccttgtaaaatggctgaactaaattaaacccttgtttcccatttgttctataatttatagtgaaactgagaacaaaactatctttataaatgatagctaaaagtatttccagatatttaaacaatttaaaataaatttcttctgcagagatgcaaagcatctcaacactggaatgaacaaatgccttaaattcaatggagtaaacctttagaatgaagaggaactgtcatttcacccaagccgaagacaacagccttatgcacttgtgtgctctgtctttgctgcttctcgtgtttcaagcctttcctgtgggatcagcacagcaaagtgcaacttaccaaatggtttaatgactggttaattctttcttctcccaatggaaaagcaatggcaacacaacagtagactgctggcttgacaatcttaaacgtgagcctttgcacatgtaggtttatcatcatttgagtatacgactaagcaagtcaatgaactttttttttttttttagcagtttaatttggtcctgagaatgttgcagtctttattaccccttttgcattaatccacttttctaaccaccttttaagctttaatttttaacactatacaccaagtctttgaaatcagtgatctgttatttaactctaaagcatttgacacttcttgccttaacagttttaaaaaccacacacaaaaaaactctgtaagtaatacagtaggccaaaagtttcatcctatctatcttgcagtttacctatctgatctgatctctgtaattatagttctgtcatttaaaatatactatttaaatctaatttttacatttcaaaaattatcttcagtagtaactaagtatattttctgtggattctgagaatgttatttttcagaatgtgagaatatatatgtacatttataatcttgtgactttaaagtctgttttcagatacagtatgtaaatacttgtaaaaaaatttgtataattttgtgataatgtagtttcccaaaaaaattatttagaaggcattatgttattagtaaatgagagcactgtatagaactgttcctattttctgcacttgccattccagctgcctccactgtccatacccacctcattcatcctgtcacagaaggcaggaaaactgggaactttaccaaagtagcactcagcctgagaggcctgtataatcatgcttttcaaactaaattcacttaaaaattaaaaagcagaattgaatattttaagcagcctcagtacctttggccaatgctgttttcatggtggattatgaacattatataatctttgggaaaagtgaaagtagtacaatttttagaataatgacaactgcctcactgcatctctccactcacacagcaaccgtgtagccccctaagctgcagtaccatgactaaccatgatgtcaatttcatatgctgatcctcacaacagcagtgcacaaacatgccccaaatattttaacagaatttagctcttccttaagctgtcttttcatagtaaaaacaaaacaaaaacacccaatgttaaaaccacataataaacttacaaacttgaaaaattagacacttcagatagataggcaataaaacttcatattatgaaagcaatatattccaagtttcaaagatttgacaagttctgtagagtatctttcatcagtacatgaaaacttccaaactgcatgatcttctgccaggcaggactgggtgctattcgctggtttgaggtcgaatccatttcaaggcatgtcgtggtgggacattaatggtgggatggtagaatgtgcagtccggtcttgtacattgagtgttaaacctacaatgttttggatgatagaagggacattccatcttcttacaagcagggaagtaacggcagagctgactactggaaggtggtgctggtggtgcaactggttttggagacagtactggaattcttctactcacatgagtgaagggacaatctggtttagtacactttgcatcatatttacaatttgggtgaacaaacaaacatttttcagcaaatttacaattggggaaggctttgcagggtgagatggggtgatggtaggcacactcatccccatttttacaagcaggccagtacttgcagcgctccaaaagtttttctggtttctgtgccacactcagttcactcatctcagcttgatttttttctacagaatctccttttgtttcctcttctttaatggggggacttattctgggggtcctactttgtccctggaccacttctgctagcaattcttcttgagaagttcgagttctgggagcaactggaagtgtctgtttctgtggaactgtagagtagttagttgtttttgttacggattcttgagcttcagatatagccttcaaaatcagattcttgttagcttgtttagaaggtggaagagaaggtctcctttcaggctttgcaggcacagacacactgctggagatgcttcctgttcgagacccgtaatcatcatcttcttcctcctcttctccatcatgattgaatttttttactttaacaactgaacttaccacaggcaactttctcttccgaaagttttcatcctccatactcattttctccgagttgtttctaaagaacggactatacgtttcttctaagctgttaagcacctctggttcacacaaacgtcctgtttcatatacccaactactctgcatatcaagctgcttggcagcatgaatactattctgctgctgttgaaattgcaacctgtttaaatgaacaccactatctgcatttctacttgcaggtggtcgataaatttcaatagaagggcgagaagaaccatatgtaagtgtcactgtaggttttttctgagataagggattctcctgcacaaagttgaggtcttcgtcaatgagatcatctggttctggcttaatatcaatcacatcttcagagggtgctggctccctcaaaggtttcactgttgacattagtcgggttgcagctccatcatcgtaagtctgtctgacatttgtggtttttgactcctgcgaacttgtagaaactctggaatctcttttttcaggtctcgcgctaggaatggcaagtggtggcactgcagcttcatgcctcctctcatctccccgactgaaattgctcttgtttgaaggcacgttactatcaaagatgttggtatcagaagacttcagactagagggttcagttgtaacagagcgaagtttatctaatacaccatgaagccatacggtgaatcgaattgtgttgttccctagaaacagggacagatcctctgtcatttggtcctgacttttcttgttggccaccatcaccataatgtaatcaggaagttcttcatctatttaaaaggaaaggtagatcaaaactttgtttcctcaaaactttcttcttaaagttgatgtgcttgaaaatatagatgtagctctaagctttagagtcgcagagctctactggaattacattggacaagatggcttagctttaatttttttctcttcattccacaggtatttcaaatacaacataagctcctaattcttgtaatttccccttaatggcactccggatcttgcggctgatctcggtgccgatctccatggctctgcggcgtgcgggaactcagcactgcgcggcgcttggcttacccggaggctgccgcggactcctaccccgcagccgggacaccaccgcctcc

SEQ ID NO: 8567 - RNA, 35 nt, Homo sapiens
  source 1..35: mol_type = other RNA
aaacaccattgtcacactccacagctctgctaagg

SEQ ID NO: 8568 - RNA, 435 nt, Homo sapiens
  source 1..435: mol_type = other RNA
aaacaccattgtcacactccacagctctgctaaggaaactctgtagccacgaaggtgttaacttcacctccacattccaccattgtcactgataataggggaaccttgtcagctccacatattgtgaccagggctatcgctgaccatccacaagaggctctagaagtctcttagctctgctgggaagaaacagtgagaggtgaacaattcactgattaaaagggtccccggaggatgcgcttggagcgctctatcctgggcaagggcttggacccatttcacttctcagggctccatagcagtatctgagcatcctccacttctccatgggggctctgttggcttttggctttgaataatccccagtcagctccggtcctctcagtccaaggcccttcctgtggcaggcaggatggcgccttccacagcttctgt

SEQ ID NO: 8569 - RNA, 597 nt, Homo sapiens
  source 1..597: mol_type = other RNA
aaacaccattgtcacactccacagctctgctaaggaaactctgtagccacgaaggtgttaacttcacctccacattccaccattgtcactgataataggggaaccttgtcagctccacatattgtgacctaagcagagaaaagaagcatcacgggtacaagcatcttgagcaatgggaagagctgaacactctcaatgaaaggcttctgtgttctggaacagtagagtagtagaggggtccactgcctgtgttccactgccacccagcaaaccccttctgcaaaaacttccagggctatcgctgaccatccacaagaggctctagaagtctcttagctctgctgggaagaaacagtgagaggtgaacaattcactgattaaaagggtccccggaggatgcgcttggagcgctctatcctgggcaagggcttggacccatttcacttctcagggctccatagcagtatctgagcatcctccacttctccatgggggctctgttggcttttggctttgaataatccccagtcagctccggtcctctcagtccaaggcccttcctgtggcaggcaggatggcgccttccacagcttctgt

SEQ ID NO: 8570 - RNA, 152 nt, Homo sapiens
  source 1..152: mol_type = other RNA
aaacaccattgtcacactccacattttcaagaggtgcatcctcaggcagatccacatcaagcataagatcatcatcctcaaggtcacatgattcaagattattcaaaatatcattaggaccatctcaactttctataagctgtccctccact

SEQ ID NO: 8571 - RNA, 165 nt, Homo sapiens
  source 1..165: mol_type = other RNA
aaacaccattgtcacactccacattttcaagaggtgcatcctcaggcagatccacatcaagcataagatcatcatcctcaaggtcacatgattcaagattattcaaaatatcctacattaggaccatctcaactttctataagctgtccctccactaccacatct

SEQ ID NO: 8572 - RNA, 207 nt, Homo sapiens
  source 1..207: mol_type = other RNA
aaacaccattgtcacactccacattttcaagaggtgcatcctcaggcagatccacatcaagcataagatcatcatcctcaaggtcacatgattcaagattattcaaaatatcctgaaagtatcaatatcagtttgagatttctatttacctacattaggaccatctcaactttctataagctgtccctccactaccacatctatgct

SEQ ID NO: 8573 - RNA, 1905 nt, Homo sapiens
  source 1..1905: mol_type = other RNA
aaacaccattgtcacactccacattttcaagaggtgcatcctcaggcagatccacatcaagcataagatcatcatcctcaaggtcacatgattcaagattattcaaaatatctatgctgttcatttcagaggactcatagctcccaactggatggacatttccaatgggttccaagccttcttcatcccacatgtatgttccatcagagctatcagatggagagagttcaaacgaagaaccagctctgtagtctgtatctggtgaaaccaaattattcccagaagtatgttttgtacattcactcctgtcagagacacttatatctatccattcatcagttttactgaaggctttttcattttccttgggggaatcaaacatatcctgtggtggcccattttcatgtttctcttctttgagagacatttcctctggagttattctagttctgttggagtcttctatatctataaaatcatcactaaagtcttcacttaaatcattcttatcagaagatgacaaagacgacaaggaaatgtcatccacatcatcactcaggtatctcattttagcatcatgtttcatggtctggttgttttttgttctataactttcattttcaatcagttcttggtccttattagcagctctgtccttagccaaaactgtagcatcttcctctacacatgtgtcagcaggtgaatttttatttccatcaactgtcatagtcccagaaaatggagatcggctagatttcagtagagagggatgaaccattctataacctaaagtagaagttacacctgggccatttggtaaagccaacttctttccaccagcagcataaggcctattaaatccataccccaaatgttcattcccattgagtacttctggctgccgggaatttcttgttagcatacttgaccgtagaggcactctaatggatagctgttggttctgataaggctttgtaagatccacagctctattaaaggaatgtgatctggttatagatgaaggtggaaggaatgaattctgaatggaatgtgaaaaactttgtgaccttaccattttttcacaattaatagatttactactgtctggggattgagctaagctttctccagaactgcttctggtggcacaggagttcgctctaggcctttgcatgctaccagctgatcggtttccataaaatccattcaactgtgattttggagtattgatcgaagaatatgaagtccttcctaataatgtgcctttggtgaatttacccaaattagatggtccagaaaaagacttttggtttaactcctctgtagatgacacaaacatagtggatggctttgctaactttgatgtgaataaagaaacacttttcaaacctccctttatcccatttttatcaaacattccttgagtaggaacacgtttttcaggatcaattattttatcatgtgaattttgagtattgttaggctcttcgacaccttgtgcacaaagctgatatttatttgctttcctccaattaaatgaatgagatgatggacaatcagagccattatttttgatgtaacttttgacattactattcttggaagttcctaataaattaacaggtgtcccatttggcattggctgcaatgtacttcttacagattttgttccatactttggcaacttggaacccaaaaatgtcttgatttgtgttttttcttccatgagctataaggtgcatttgttcttaaaagttgaaagaatatttagtgtaagaggtgctgtgtggccaagtgctatgtggctcactcttgtaatcccagcactttgagaggtcgaagcagaaggatcacttgaggctaggagtttgagaccagcccaggcaagatagcaaaactccgcct

SEQ ID NO: 8574 - RNA, 1985 nt, Homo sapiens
  source 1..1985: mol_type = other RNA
aaacaccattgtcacactccacattttcaagaggtgcatcctcaggcagatccacatcaagcataagatcatcatcctcaaggtcacatgattcaagattattcaaaatatctatgctgttcatttcagaggactcatagctcccaactggatggacatttccaatgggttccaagccttcttcatcccacatgtatgttccatcagagctatcagatggagagagttcaaacgaagaaccagctctgtagtctgtatctggtgaaaccaaattattcccagaagtatgttttgtacattcactcctgtcagagacacttatatctatccattcatcagttttactgaaggctttttcattttccttgggggaatcaaacatatcctgtggtggcccattttcatgtttctcttctttgagagacatttcctctggagttattctagttctgttggagtcttctatatctataaaatcatcactaaagtcttcacttaaatcattcttatcagaagatgacaaagacgacaaggaaatgtcatccacatcatcactcaggtatctcattttagcatcatgtttcatggtctggttgttttttgttctataactttcattttcaatcagttcttggtccttattagcagctctgtccttagccaaaactgtagcatcttcctctacacatgtgtcagcaggtgaatttttatttccatcaactgtcatagtcccagaaaatggagatcggctagatttcagtagagagggatgaaccattctataacctaaagtagaagttacacctgggccatttggtaaagccaacttctttccaccagcagcataaggcctattaaatccataccccaaatgttcattcccattgagtacttctggctgccgggaatttcttgttagcatacttgaccgtagaggcactctaatggatagctgttggttctgataaggctttgtaagatccacagctctattaaaggaatgtgatctggttatagatgaaggtggaaggaatgaattctgaatggaatgtgaaaaactttgtgaccttaccattttttcacaattaatagatttactactgtctggggattgagctaagctttctccagaactgcttctggtggcacaggagttcgctctaggcctttgcatgctaccagctgatcggtttccataaaatccattcaactgtgattttggagtattgatcgaagaatatgaagtccttcctaataatgtgcctttggtgaatttacccaaattagatggtccagaaaaagacttttggtttaactcctctgtagatgacacaaacatagtggatggctttgctaactttgatgtgaataaagaaacacttttcaaacctccctttatcccatttttatcaaacattccttgagtaggaacacgtttttcaggatcaattattttatcatgtgaattttgagtattgttaggctcttcgacaccttgtgcacaaagctgatatttatttgctttcctccaattaaatgaatgagatgatggacaatcagagccattatttttgatgtaacttttgacattactattcttggaagttcctaataaattaacaggtgtcccatttggcattggctgcaatgtacttcttacagattttgttccatactttggcaacttggaacccaaaaatgtcttgatttgtgttttttcttccatgagctataaggtgcatttgttcttaaaagttgaaagaatcgtgcggaggtcgcgctgcctcctcggccgcggcccagctgcaggccgccctgcgacctgcgggcccgaggacggaaggtgagacgaagggccgcccgtcacatccccgccagccccgccgcccgagccgcagcaaccagcatcgcgtccgcggcctgagggagcgccggactccaaagccgccgcgccccctccctcggccggcgcccgcccggactcc

SEQ ID NO: 8575 - RNA, 2001 nt, Homo sapiens
  source 1..2001: mol_type = other RNA
aaacaccattgtcacactccacattttcaagaggtgcatcctcaggcagatccacatcaagcataagatcatcatcctcaaggtcacatgattcaagattattcaaaatatctatgctgttcatttcagaggactcatagctcccaactggatggacatttccaatgggttccaagccttcttcatcccacatgtatgttccatcagagctatcagatggagagagttcaaacgaagaaccagctctgtagtctgtatctggtgaaaccaaattattcccagaagtatgttttgtacattcactcctgtcagagacacttatatctatccattcatcagttttactgaaggctttttcattttccttgggggaatcaaacatatcctgtggtggcccattttcatgtttctcttctttgagagacatttcctctggagttattctagttctgttggagtcttctatatctataaaatcatcactaaagtcttcacttaaatcattcttatcagaagatgacaaagacgacaaggaaatgtcatccacatcatcactcaggtatctcattttagcatcatgtttcatggtctggttgttttttgttctataactttcattttcaatcagttcttggtccttattagcagctctgtccttagccaaaactgtagcatcttcctctacacatgtgtcagcaggtgaatttttatttccatcaactgtcatagtcccagaaaatggagatcggctagatttcagtagagagggatgaaccattctataacctaaagtagaagttacacctgggccatttggtaaagccaacttctttccaccagcagcataaggcctattaaatccataccccaaatgttcattcccattgagtacttctggctgccgggaatttcttgttagcatacttgaccgtagaggcactctaatggatagctgttggttctgataaggctttgtaagatccacagctctattaaaggaatgtgatctggttatagatgaaggtggaaggaatgaattctgaatggaatgtgaaaaactttgtgaccttaccattttttcacaattaatagatttactactgtctggggattgagctaagctttctccagaactgcttctggtggcacaggagttcgctctaggcctttgcatgctaccagctgatcggtttccataaaatccattcaactgtgattttggagtattgatcgaagaatatgaagtccttcctaataatgtgcctttggtgaatttacccaaattagatggtccagaaaaagacttttggtttaactcctctgtagatgacacaaacatagtggatggctttgctaactttgatgtgaataaagaaacacttttcaaacctccctttatcccatttttatcaaacattccttgagtaggaacacgtttttcaggatcaattattttatcatgtgaattttgagtattgttaggctcttcgacaccttgtgcacaaagctgatatttatttgctttcctccaattaaatgaatgagatgatggacaatcagagccattatttttgatgtaacttttgacattactattcttggaagttcctaataaattaacaggtgtcccatttggcattggctgcaatgtacttcttacagattttgttccatactttggcaacttggaacccaaaaatgtcttgatttgtgttttttcttccatgagctataaggtgcatttgttcttaaaagttgaaagaatcgtgcggaggtcgcgctgcctcctcggccgcggcccagctgcaggccgccctgcgacctgcgggcccgaggacggaaggtgagacgaagggccgcccgtcacatccccgccagccccgccgcccgagccgcagcaaccagcatcgcgtccgcggcctgagggagcgccggactccaaagccgccgcgccccctccctcggccggcgcccgcccggactccgccctccagggccggc

SEQ ID NO: 8576 - RNA, 2022 nt, Homo sapiens
  source 1..2022: mol_type = other RNA
aaacaccattgtcacactccacattttcaagaggtgcatcctcaggcagatccacatcaagcataagatcatcatcctcaaggtcacatgattcaagattattcaaaatatctatgctgttcatttcagaggactcatagctcccaactggatggacatttccaatgggttccaagccttcttcatcccacatgtatgttccatcagagctatcagatggagagagttcaaacgaagaaccagctctgtagtctgtatctggtgaaaccaaattattcccagaagtatgttttgtacattcactcctgtcagagacacttatatctatccattcatcagttttactgaaggctttttcattttccttgggggaatcaaacatatcctgtggtggcccattttcatgtttctcttctttgagagacatttcctctggagttattctagttctgttggagtcttctatatctataaaatcatcactaaagtcttcacttaaatcattcttatcagaagatgacaaagacgacaaggaaatgtcatccacatcatcactcaggtatctcattttagcatcatgtttcatggtctggttgttttttgttctataactttcattttcaatcagttcttggtccttattagcagctctgtccttagccaaaactgtagcatcttcctctacacatgtgtcagcaggtgaatttttatttccatcaactgtcatagtcccagaaaatggagatcggctagatttcagtagagagggatgaaccattctataacctaaagtagaagttacacctgggccatttggtaaagccaacttctttccaccagcagcataaggcctattaaatccataccccaaatgttcattcccattgagtacttctggctgccgggaatttcttgttagcatacttgaccgtagaggcactctaatggatagctgttggttctgataaggctttgtaagatccacagctctattaaaggaatgtgatctggttatagatgaaggtggaaggaatgaattctgaatggaatgtgaaaaactttgtgaccttaccattttttcacaattaatagatttactactgtctggggattgagctaagctttctccagaactgcttctggtggcacaggagttcgctctaggcctttgcatgctaccagctgatcggtttccataaaatccattcaactgtgattttggagtattgatcgaagaatatgaagtccttcctaataatgtgcctttggtgaatttacccaaattagatggtccagaaaaagacttttggtttaactcctctgtagatgacacaaacatagtggatggctttgctaactttgatgtgaataaagaaacacttttcaaacctccctttatcccatttttatcaaacattccttgagtaggaacacgtttttcaggatcaattattttatcatgtgaattttgagtattgttaggctcttcgacaccttgtgcacaaagctgatatttatttgctttcctccaattaaatgaatgagatgatggacaatcagagccattatttttgatgtaacttttgacattactattcttggaagttcctaataaattaacaggtgtcccatttggcattggctgcaatgtacttcttacagattttgttccatactttggcaacttggaacccaaaaatgtcttgatttgtgttttttcttccatgagctataaggtgcatttgttcttaaaagttgaaagaatcgtgcggaggtcgcgctgcctcctcggccgcggcccagctgcaggccgccctgcgacctgcgggcccgaggacggaaggtgagacgaagggccgcccgtcacatccccgccagccccgccgcccgagccgcagcaaccagcatcgcgtccgcggcctgagggagcgccggactccaaagccgccgcgccccctccctcggccggcgcccgcccggactccgccctccagggccggcgcaccgcgcacgcgcagtccc

SEQ ID NO: 8577 - RNA, 131 nt, Homo sapiens
  source 1..131: mol_type = other RNA
aaacaccattgtcacactccaccaaatactttttcctcacatatctgagcactcactaagagagttactttgcacaagggagacattgtgttaccggctgcctactcagacatagttgtacccaaggcact

SEQ ID NO: 8578 - RNA, 2028 nt, Homo sapiens
  source 1..2028: mol_type = other RNA
aaaccgttaccattactgagtttaaaaaaaaaaagaaagaaaaaacaaagaaaataaaagaaagaaaagagaagagaaaaaaagaaaagaaaaccgaaacagtttcaccaatagtttacggctccagatgtttgctacaaacattgaatgacaaacttggacaacaagatatgtaaacacaaaaagtgaagagaaaaaaacaataatgagcaaaaacataagtaaaacatgtcaataaatcatcacgtatgaaaagattataaaataagctatttttgttttaaaacaaggtagaaattttacaaaatcaaaacttcgcagattgttggagaatatttagacaaatttcataacgtgtttacctcagtaacttggatgggttagaaatatataaaagaataagcaagcttgttaaaattgtaggaaaacttacttaaagaatatacctagagtacatagctttccaacacagcaaaaataaaaggagaaaaaaacaatgtttaatccaagaggaggcaaaagaaaaaaagtcattggtagtgttttgctgttttggaaactgaataaaaactgagtgacatttttatcaagtccttaaggatgtcactttatcaattatgagagacatattggaggaatttctaatagcatgacaatctgaaatcaaaaacatatttataagctaaagtgagcatataaaatcaataatttattagacaaaaatgataaagtttaaattcctagctttaagttgtaaatacttctgtgataagcaatttgcaatataagttatgctcaaaaatgatttataacatttagttagcacttacaatccctcaagagctagaccaagcacttcatatattatacattagctcatttaatcctcacagcgacccaacaagctatacaactattaaatgaagaaaccaagaatcacacctaggcagattcattctaaactctgcagtcttgaccacaacactccacagctttaaatattattctcttgttagttgtcaggctccagtatcttcatgtgttcactctcaatcactcttctgtcctttactgtatgatgtcattctgctttataaagtgtgctgatcaaagaggttgtggtggattgatttgtcactttttttggcctccctgccacagtgggtgacatctatttccttcccctttcttttttttcaaatttatttatgtatttatttactataaattaacatatagaattgcatgtatttatcacaaacaacataatgttgtaaattggatatacctgtggataagttaaatctagctaattaacaaatgcatcccttcacatcattatcattttgtggtgagaacacttaataggtatactcaacatttttcaaaattacaatatgttgtcattaactatagtcaccatgctatccaataaatctattccctttccttttgaatcttggatggcattctttaaccaatagaatatgcccttttagaatcccaacactcttattctgcaaataagcacagtttagcctccttgaagatgataaatcacatggagagagacactgcacagacaaagaatgtccagacactccagcgaaggtccagacatgtaattgaggtcatctaggatcattccgtctcacatagctgcataaggtactacaggcaagacctgataagctatccaaaagatgcagcagacaaagaacagtgaaaggtgactgggctgatgccttgtttttgtaccttgtcagaatgcatctagctacacgctgataagagagaaaggagggccaaggagcaattcctgaggttcagctgtgaggttttgtgtctctggtagttactggtgcccatgtctctcactacgaggagaaacctaatcaacataacatagaataagttggagtcctgagcttgttttcctgcaactaggcagtctcatcaatgcaggcagtcatcgtccaatcttctgggggcaaaatatccatatactctgcactcctcccagcccag

SEQ ID NO: 8579 - RNA, 54 nt, Homo sapiens
  source 1..54: mol_type = other RNA
aaaccgttaccattactgagtttagtaatggtaatggttctcttgctataccca

SEQ ID NO: 8580 - RNA, 57 nt, Homo sapiens
  source 1..57: mol_type = other RNA
aaactaatatacccatattctgatgatcacctagccagaatatgggtatattagttt

SEQ ID NO: 8581 - RNA, 57 nt, Homo sapiens
  source 1..57: mol_type = other RNA
aaactaatatacccatattctggctaggtgatcatcagaatatgggtatattagttt

SEQ ID NO: 8582 - RNA, 7801 nt, Homo sapiens
  source 1..7801: mol_type = other RNA
aaactactgaaaatcaaagattaacctatgccatctgatccatgcagcaagtgataaattcagtattttcaaaagaaatattgaatttttttcttgagtcaaattgaaacctttcagaaacttgtttaaatgcgccaagtccctacgcacctttttagtatgtatgagcaaaatactgttgaatttcacactcaactaatcctttaataattttctttcagccagaatgaaaaaggctagtattaatttcctaataaaattttttttcaaaagttatcgaggatatgactataaccttggaccagtttcaatttctttttattttttctgagaatacaccaaagattaatgtcaatggcaagtgagaaattgtccctagagaactattcaaggactttttcttactacatttgattggactggagtgaactgacattatagcatctttatcatcacctttaaaattctattttctcttagtagcaacagtgaagactttagaactattacttactttaaattattaaagtatatcacagacaaaatattcaattttacattaaagcaacattaagggtctcaatttcattgaacagaaacaaatgctgaagaaatttacaggtatgatttaattttagagagtgttctttctttagggaacaaaatgaaactagatctctcatttgtctgtatgggcaagatatggtaaacctcatgatcaaaacacatgccagttagaaacttgatcacagaaatgatgctcagtgttgaaacccaacaataaacaaacaaacaaaaacccccactctaaccagaggcatttaagcctctccactgaagttcctgtttcccaccagtttacgacccttaatgttactgcatgtatggttgcatatttgagatgattaaaaataaaagactggcttaaaagcacctcctcctctagtgtgtaattacatacaaactaaagattccttctgacgtcctaggaaccccatttgttaccgtttcatgtgtaagcaccattgaaccaatttttaaagcacatttgcagttatcaaatgtttagtgtgtcctcaagtttcattgatttgtttgcctttaagcaagaaaagagtaaagtgtattattttcccctgcttcttttcatatctgaattgtcaaaaaatgttaattttggaagtgcttttaatcactattttccccaacagactagaatggctccatgaaatttgacaattaagtaaggaaatctttatccccaaaagaagcacgtatcttaccctctaaactgcatgcaaagtaagggtctgtgtgagagtattttccccaaactcctaatggacatggcagacaatgtgtagaaaaatctgagttttgaactgaccaacttcaagtcttttaaaatctttgggcaaaaaaaaatatcatgtagcagttaaaaaaattattgacttacaaattatagaaaagatatgttatctacaatatatgccaggtgacccattaaatttaaaaaatgtgtgcgaatgagtaactacattaaaactaccatcttggatcttggtgctttccaaaattctgaaatcactattaaggagggaccataccagatttttttgttgttcttttccttggagaatggggaagaagttggaaagagaaggaagtaaaccttcactctttggtacagccctgtatagcaaacttcagcctggggcacatttttatggtcaaattaaaaacctttgagaataggagtttatcatagaaatgctgacagatcctaacccagagaagggctaagagcaacacagtaatattaagaaagctctccctcagcacgattgagcttcagcgcaagggatagagttgtctagtggacgcccttggccagtaaacaaccatgatttaatgtgcttgagacttggtcatatgggagctctgtgaccctctaagccaaattttcttttctttttgttttcaactgaaatatgcctcaaagggtaaaggattgcaattttagccttcattcatggatatattgctttctttcaacaatatctgatgggcctgttaactgccacccatggggagcaggttgcaggaaggtctcattgaacacaaaacaccaagtgttttcagtagtttattcacatttttttttctctgcttattttaatatgcaccacgtgtaagttagatgagggctacggtaaaaacatttttgatgactgaaatcttacttttccttctaacgatctggagcaaatcacatattcattgatcatgacgaataaaatgatttctgctacaatgttgagaaaaaatgtgttcattaatatgaacacatgtctacagagatgatttacacgatgcaagtaatgaaagagttcttccttaactagtctactatcaaactgaaaagatgaatcttaaaattcccttgaaaataccatatgattggtcatgtgtcagtaaaagaaagacggtccccatcaccaggccaccaccataagagagctatattaaatacttgggaaaaaatatggaaacaccggtggtgatgattaaattgataattacatagatacactgccataatgatacatatttgttctatgataagtgaaatcaaaaataagatcaatttggttatagaaattccttaaagaacaccaccacttaattatttcaaacttgaactatcccaagaatgtcgagaaaaaaattagaaagcactggctaaaagcaaagcaatctggatacaccaatgtagtcagcatgccttgtgcttgtctgttaaccctctgagtacatctctgacattcaggatcttggtagcttaatgttagaaagattgcattccatctgattactcaagatttctacttgactggtcacattccactgtttattcagcatagatcactcaaattctacagtgatgtgctgggatccccatgctgaatgggccctgcattcttctgagctgcccttctgcagtgtgctgagaaacaccccctagcttcacacggtccagagtccccctagacgtcgatgggaaaaggcctgagccatgcaccgcaggctcagtacactagatgctgtagcaatatagttaatgcccacagaaaaagcagtaattcagagaaagaaaggaaaatgacagtccactgcaggtaggtctctgcccattgcattcttcacacttttagagttgaggccaggctgtagagctactccatagccttggaatagtgctttgctttatatttctagagaaagcagtaatttccaactagttcagtgttcctcattaatatggaatctacctacacaccaacactctttctggtgttctgtgccccctacccccacctcccccccaaaaacaactcaactaatttactgatttatgctactttgtgattttgcgtgttatcacttccggatgctctaaaagggggggaaaaaaacctcaataaacgatatgctttttacatgtcaggacaacacagaccacagagatgaacctaaatgtaaaagagcaaaaaattttggtgatggtgttgcaaaagtaatgacatgtgatttaaaaatccatattaatgtagaccatagtttcagggttgaagagtaaaaatgcagcaagtgaagatcaatgtgcatttgaaaataaaggactatagaaacgttgttcacaaattttaagactctcaggtattaaagtatattcaaaacagagaacataggtactgttcagccaccagatgcaaatttcatgagatatccctctctggttgtctcgtggatcccagagcccagcaaaccttgggaatacatttgagttgggcacctgcctctaagacaccccaggagaatcctctctgagcactgtggtgatgcacagaacctgtgaatccccattctaaaatggaatctgttccagaagaaactcaggcctggagacactgcactagggagatagatttggtaacaagagtgaaaatacaggtctcagacaggacttggcccaaagacagaaaaaacactctgacctcctggacagctaaagacagtggtatttaaaaaaaatcattttaggggatggaggttttatcctcaggggtatcatctaggtctttcatcctgatcttcctaggagactatataggtaacctaaaggtgcacatggaattgtcttgccagtggtttattcactgaaaacttattgttagaacattctggattgtgttcccagtgtgctttctcctcagccatcttgcaaagcaactgcctccagtccccttgtgccccagctctcctatgtgtggatttcatactagatgtagattgcacagtgatgaccacagtgcgtggaaaagcaggtgagaaaaatcacaggatcttattccctctttctgtttgaaattccagccctgcagagcaccgggcaatttattgctcttttccaccagttgtttctttcctgtagatgtctgacactgagtagagagaccctcactcaccaagcacaagacaagctgtggtgactccctgagagtctgcgctggcgctagcagcagctgatatggaagcagcatttctggggcgtcatcagtacatcttcatgtggagacaatttggggggcaccatctatttcctgggtcaagctctttgccacaaacccaattccctccacttgggatgcagaactcactgcaactgacagtcatatctctaatgaaaaaaaaaatctgtttctgaataggattgtgaagaagaaagaaccgtgcgtgtgtcgaagttataaacctgccacgttctaaacccacagaaaaggacaaacaagatatcattctaaatgtccttcttttctggacatttcagcatctaacaacaccccttgatctgcagtaaaatcaagaaacatgtgtgtatacatccaaaggcctgaaaaattcccaaacaagaattctcaataaaattctatgcactcagagggttaacaagtgctatattacatactgcagatcctagcttgactgatgaaaacattcattgcttctaagtttaaaaaaaaattgcaaattggccttaaccctttgaggactctattagcagcaaattaccatcttcacaatcaccacgtgtcatcttattcagtaaagggaaaccgctacaaagatacctgaaaacactttcagttctgccattcaagcattgagcgctagatagatcagatgaaactgttttacacaaatttgggggaaaaaaatctcagagtctcaaagggttaagctaggactttgagtaaaagggtcttattaaaagggcgagttaggggagcgaacagtctcggaggagcttggggagtagtcttccgattccgagttgagttcgggaggagctggctgcgccttgtaccggctcctcacatcctggttgcgtcttcgtcggaaaacctgcctctccttatcaagagcggtggtctagcaggggctgctatgacagaaactccagctgctgtgctattcggcttggggcctgtgttgaaatgcttctttatctttccagctactgacagctgatgttcattttctgggaggccatcatcattaacccagggatgctcaagtacttgaacagcagaaaatcgctgatctacatcgaccaacagcatcatggtaatgagctcctttgcagaatcggaaacattatcccagtatggagaaggaaagtccacctgccccatcaaaatctgatcaaaaagcacctcctggtcatcaccacttccacggaatggagggaaaccacacagcaggatataagtgattacacctgctgcccagatgtccaccttgaggccgtatccagtctctgcaatgatttctggagccacgtatgttggggtgccacagactgtgtacagggggccgtctacaatggtggccagtccaaagtcacccagcttcagtgatttgctgccatcttggtgctcatacaccagcaggttctctggcttgatatcacggtggacgatgttcaggctatgcaggtatttgatggcgctggctaggttgtacagcatcccactggcgtctctctcggtgtatttgttagtggaagtaatggcatcaaaaaggtctcccccctttactaattccatgacaagatacagttcagttggcacatccatctcctcaatcagaagaacgatattgggatgcttcactcttcttaaaatagacacttcattctggatcatgtgctctttgcctcgacatttgcttttcttgataattttcagagcatactctctagcagtcgatctttctacacattccttgacaacagcaaaatttccatctcctattgttcttccgactttatatcgttctgttattgtagctggaatctggaagccttcctccgacacttcttctccagggccatcgttctcatccatcgagctgcagactttggtggacgcaagtgacgtagaggagccgccatgctgagagctcctctgcttccgcaggcttcctgggctggtgggtgatgggcttggcgacttgcctgagcgcggagtagagagctgactaccaggggttccattaactgagctggtggaggcaggggacttgctacgcctggacggtcctgggctcttggtggtgctcctgcgggatgatgaagctattttggtgtaagaagtggactttaccactcgacattcactttcatctagcaagaaatcatcctggtaacggaacttctccggtccacatgcaataaaaatgtcatcatcaccaaaaaagtcctgaaggcacatcacctgtttcccatccaacgtgtacaggcgtttcaccactcccgagtccagcttgatggcatcggtgatatcggtgaggacctgctcaaaggaatgagccgttttcttgttcagcagaatcctgacagctttccgtggcttcacgccacttctgatgatggtgaccagcttgggccgaatgaaatccttattctctcgcacctctgaagggcttcctttggcagtggccagtgaagacactgcccgagaagccgaggtggtcttgacgttcaccgaccagttggggttcacattcttggtgtactccagtttcttgaagggctctatggagccacatacataactctctccttccaccagttggtccaggctggaaatcttcttgagcccatcaatggtgtagattgttctcactccctggggcaaattcacgttatccgacagagttcgggtcaaatcagccagcagggcctcaaaagatcggaaccggtctggggagatggcatacacaatccctttgaagtatcgatctccgtttcgatagaaacgaactttcttggccttcttctcggagctgagcgtctgcagcgtgcgggtgcggtagaagctgcagtgggcgctgtgcgtcgggctcggcaggccgttcacccgcgaccctcggctgtatctctgcgccttatcccgctcgtcgaagtgctccagctccatgtctctgccgaaggacatgatggacttcaagtaggaccggtccgcggagagacgccgccgggggtctttgtggccgcgctgggggccgcctcctggtgctgtcctcgccgggctgggcgcggccggggctgcggggctgcagggctggggggcggcggcggggccgggctgggcggcagcagctgctggagcgcggcgcctcggttgcggccactagtgcagggatgtgcctcggcccgtcctcattgaaatgc

SEQ ID NO: 8583 - RNA, 7916 nt, Homo sapiens
  source 1..7916: mol_type = other RNA
aaactactgaaaatcaaagattaacctatgccatctgatccatgcagcaagtgataaattcagtattttcaaaagaaatattgaatttttttcttgagtcaaattgaaacctttcagaaacttgtttaaatgcgccaagtccctacgcacctttttagtatgtatgagcaaaatactgttgaatttcacactcaactaatcctttaataattttctttcagccagaatgaaaaaggctagtattaatttcctaataaaattttttttcaaaagttatcgaggatatgactataaccttggaccagtttcaatttctttttattttttctgagaatacaccaaagattaatgtcaatggcaagtgagaaattgtccctagagaactattcaaggactttttcttactacatttgattggactggagtgaactgacattatagcatctttatcatcacctttaaaattctattttctcttagtagcaacagtgaagactttagaactattacttactttaaattattaaagtatatcacagacaaaatattcaattttacattaaagcaacattaagggtctcaatttcattgaacagaaacaaatgctgaagaaatttacaggtatgatttaattttagagagtgttctttctttagggaacaaaatgaaactagatctctcatttgtctgtatgggcaagatatggtaaacctcatgatcaaaacacatgccagttagaaacttgatcacagaaatgatgctcagtgttgaaacccaacaataaacaaacaaacaaaaacccccactctaaccagaggcatttaagcctctccactgaagttcctgtttcccaccagtttacgacccttaatgttactgcatgtatggttgcatatttgagatgattaaaaataaaagactggcttaaaagcacctcctcctctagtgtgtaattacatacaaactaaagattccttctgacgtcctaggaaccccatttgttaccgtttcatgtgtaagcaccattgaaccaatttttaaagcacatttgcagttatcaaatgtttagtgtgtcctcaagtttcattgatttgtttgcctttaagcaagaaaagagtaaagtgtattattttcccctgcttcttttcatatctgaattgtcaaaaaatgttaattttggaagtgcttttaatcactattttccccaacagactagaatggctccatgaaatttgacaattaagtaaggaaatctttatccccaaaagaagcacgtatcttaccctctaaactgcatgcaaagtaagggtctgtgtgagagtattttccccaaactcctaatggacatggcagacaatgtgtagaaaaatctgagttttgaactgaccaacttcaagtcttttaaaatctttgggcaaaaaaaaatatcatgtagcagttaaaaaaattattgacttacaaattatagaaaagatatgttatctacaatatatgccaggtgacccattaaatttaaaaaatgtgtgcgaatgagtaactacattaaaactaccatcttggatcttggtgctttccaaaattctgaaatcactattaaggagggaccataccagatttttttgttgttcttttccttggagaatggggaagaagttggaaagagaaggaagtaaaccttcactctttggtacagccctgtatagcaaacttcagcctggggcacatttttatggtcaaattaaaaacctttgagaataggagtttatcatagaaatgctgacagatcctaacccagagaagggctaagagcaacacagtaatattaagaaagctctccctcagcacgattgagcttcagcgcaagggatagagttgtctagtggacgcccttggccagtaaacaaccatgatttaatgtgcttgagacttggtcatatgggagctctgtgaccctctaagccaaattttcttttctttttgttttcaactgaaatatgcctcaaagggtaaaggattgcaattttagccttcattcatggatatattgctttctttcaacaatatctgatgggcctgttaactgccacccatggggagcaggttgcaggaaggtctcattgaacacaaaacaccaagtgttttcagtagtttattcacatttttttttctctgcttattttaatatgcaccacgtgtaagttagatgagggctacggtaaaaacatttttgatgactgaaatcttacttttccttctaacgatctggagcaaatcacatattcattgatcatgacgaataaaatgatttctgctacaatgttgagaaaaaatgtgttcattaatatgaacacatgtctacagagatgatttacacgatgcaagtaatgaaagagttcttccttaactagtctactatcaaactgaaaagatgaatcttaaaattcccttgaaaataccatatgattggtcatgtgtcagtaaaagaaagacggtccccatcaccaggccaccaccataagagagctatattaaatacttgggaaaaaatatggaaacaccggtggtgatgattaaattgataattacatagatacactgccataatgatacatatttgttctatgataagtgaaatcaaaaataagatcaatttggttatagaaattccttaaagaacaccaccacttaattatttcaaacttgaactatcccaagaatgtcgagaaaaaaattagaaagcactggctaaaagcaaagcaatctggatacaccaatgtagtcagcatgccttgtgcttgtctgttaaccctctgagtacatctctgacattcaggatcttggtagcttaatgttagaaagattgcattccatctgattactcaagatttctacttgactggtcacattccactgtttattcagcatagatcactcaaattctacagtgatgtgctgggatccccatgctgaatgggccctgcattcttctgagctgcccttctgcagtgtgctgagaaacaccccctagcttcacacggtccagagtccccctagacgtcgatgggaaaaggcctgagccatgcaccgcaggctcagtacactagatgctgtagcaatatagttaatgcccacagaaaaagcagtaattcagagaaagaaaggaaaatgacagtccactgcaggtaggtctctgcccattgcattcttcacacttttagagttgaggccaggctgtagagctactccatagccttggaatagtgctttgctttatatttctagagaaagcagtaatttccaactagttcagtgttcctcattaatatggaatctacctacacaccaacactctttctggtgttctgtgccccctacccccacctcccccccaaaaacaactcaactaatttactgatttatgctactttgtgattttgcgtgttatcacttccggatgctctaaaagggggggaaaaaaacctcaataaacgatatgctttttacatgtcaggacaacacagaccacagagatgaacctaaatgtaaaagagcaaaaaattttggtgatggtgttgcaaaagtaatgacatgtgatttaaaaatccatattaatgtagaccatagtttcagggttgaagagtaaaaatgcagcaagtgaagatcaatgtgcatttgaaaataaaggactatagaaacgttgttcacaaattttaagactctcaggtattaaagtatattcaaaacagagaacataggtactgttcagccaccagatgcaaatttcatgagatatccctctctggttgtctcgtggatcccagagcccagcaaaccttgggaatacatttgagttgggcacctgcctctaagacaccccaggagaatcctctctgagcactgtggtgatgcacagaacctgtgaatccccattctaaaatggaatctgttccagaagaaactcaggcctggagacactgcactagggagatagatttggtaacaagagtgaaaatacaggtctcagacaggacttggcccaaagacagaaaaaacactctgacctcctggacagctaaagacagtggtatttaaaaaaaatcattttaggggatggaggttttatcctcaggggtatcatctaggtctttcatcctgatcttcctaggagactatataggtaacctaaaggtgcacatggaattgtcttgccagtggtttattcactgaaaacttattgttagaacattctggattgtgttcccagtgtgctttctcctcagccatcttgcaaagcaactgcctccagtccccttgtgccccagctctcctatgtgtggatttcatactagatgtagattgcacagtgatgaccacagtgcgtggaaaagcaggtgagaaaaatcacaggatcttattccctctttctgtttgaaattccagccctgcagagcaccgggcaatttattgctcttttccaccagttgtttctttcctgtagatgtctgacactgagtagagagaccctcactcaccaagcacaagacaagctgtggtgactccctgagagtctgcgctggcgctagcagcagctgatatggaagcagcatttctggggcgtcatcagtacatcttcatgtggagacaatttggggggcaccatctatttcctgggtcaagctctttgccacaaacccaattccctccacttgggatgcagaactcactgcaactgacagtcatatctctaatgaaaaaaaaaatctgtttctgaataggattgtgaagaagaaagaaccgtgcgtgtgtcgaagttataaacctgccacgttctaaacccacagaaaaggacaaacaagatatcattctaaatgtccttcttttctggacatttcagcatctaacaacaccccttgatctgcagtaaaatcaagaaacatgtgtgtatacatccaaaggcctgaaaaattcccaaacaagaattctcaataaaattctatgcactcagagggttaacaagtgctatattacatactgcagatcctagcttgactgatgaaaacattcattgcttctaagtttaaaaaaaaattgcaaattggccttaaccctttgaggactctattagcagcaaattaccatcttcacaatcaccacgtgtcatcttattcagtaaagggaaaccgctacaaagatacctgaaaacactttcagttctgccattcaagcattgagcgctagatagatcagatgaaactgttttacacaaatttgggggaaaaaaatctcagagtctcaaagggttaagctaggactttgagtaaaagggtcttattaaaagggcgagttaggggagcgaacagtctcggaggagcttggggagtagtcttccgattccgagttgagttcgggaggagctggctgcgccttgtaccggctcctcacatcctggttgcgtcttcgtcggaaaacctgcctctccttatcaagagcggtggtcttatccaatacattcctggttgctggtagtagtccaaagaccctgatctcttgatggtaaacccgtggtccagtgctatgacagaaactccagctgctgtgctattcggcttggggcctgtgttgaaatgcttctttatctttccagctactgacagctgatgttcattttctgggaggccatcatcattaacccagggatgctcaagtacttgaacagcagaaaatcgctgatctacatcgaccaacagcatcatggtaatgagctcctttgcagaatcggaaacattatcccagtatggagaaggaaagtccacctgccccatcaaaatctgatcaaaaagcacctcctggtcatcaccacttccacggaatggagggaaaccacacagcaggatataagtgattacacctgctgcccagatgtccaccttgaggccgtatccagtctctgcaatgatttctggagccacgtatgttggggtgccacagactgtgtacagggggccgtctacaatggtggccagtccaaagtcacccagcttcagtgatttgctgccatcttggtgctcatacaccagcaggttctctggcttgatatcacggtggacgatgttcaggctatgcaggtatttgatggcgctggctaggttgtacagcatcccactggcgtctctctcggtgtatttgttagtggaagtaatggcatcaaaaaggtctcccccctttactaattccatgacaagatacagttcagttggcacatccatctcctcaatcagaagaacgatattgggatgcttcactcttcttaaaatagacacttcattctggatcatgtgctctttgcctcgacatttgcttttcttgataattttcagagcatactctctagcagtcgatctttctacacattccttgacaacagcaaaatttccatctcctattgttcttccgactttatatcgttctgttattgtagctggaatctggaagccttcctccgacacttcttctccagggccatcgttctcatccatcgagctgcagactttggtggacgcaagtgacgtagaggagccgccatgctgagagctcctctgcttccgcaggcttcctgggctggtgggtgatgggcttggcgacttgcctgagcgcggagtagagagctgactaccaggggttccattaactgagctggtggaggcaggggacttgctacgcctggacggtcctgggctcttggtggtgctcctgcgggatgatgaagctattttggtgtaagaagtggactttaccactcgacattcactttcatctagcaagaaatcatcctggtaacggaacttctccggtccacatgcaataaaaatgtcatcatcaccaaaaaagtcctgaaggcacatcacctgtttcccatccaacgtgtacaggcgtttcaccactcccgagtccagcttgatggcatcggtgatatcggtgaggacctgctcaaaggaatgagccgttttcttgttcagcagaatcctgacagctttccgtggcttcacgccacttctgatgatggtgaccagcttgggccgaatgaaatccttattctctcgcacctctgaagggcttcctttggcagtggccagtgaagacactgcccgagaagccgaggtggtcttgacgttcaccgaccagttggggttcacattcttggtgtactccagtttcttgaagggctctatggagccacatacataactctctccttccaccagttggtccaggctggaaatcttcttgagcccatcaatggtgtagattgttctcactccctggggcaaattcacgttatccgacagagttcgggtcaaatcagccagcagggcctcaaaagatcggaaccggtctggggagatggcatacacaatccctttgaagtatcgatctccgtttcgatagaaacgaactttcttggccttcttctcggagctgagcgtctgcagcgtgcgggtgcggtagaagctgcagtgggcgctgtgcgtcgggctcggcaggccgttcacccgcgaccctcggctgtatctctgcgccttatcccgctcgtcgaagtgctccagctccatgtctctgccgaaggacatgatggacttcaagtaggaccggtccgcggagagacgccgccgggggtctttgtggccgcgctgggggccgcctcctggtgctgtcctcgccgggctgggcgcggccggggctgcggggctgcagggctggggggcggcggcggggccgggctgggcggcagcagctgctggagcgcggcgcctcggttgcggccactagtgcagggatgtgcctcggcccgtcctcattgaaatgcggcgcttcgcacagcctcactccagcctctctctccagaggagggcggcggc

SEQ ID NO: 8584 - RNA, 6846 nt, Homo sapiens
  source 1..6846: mol_type = other RNA
aaactactgaaaatcaaagattaacctatgccatctgatccatgcagcaagtgataaattcagtattttcaaaagaaatattgaatttttttcttgagtcaaattgaaacctttcagaaacttgtttaaatgcgccaagtccctacgcacctttttagtatgtatgagcaaaatactgttgaatttcacactcaactaatcctttaataattttctttcagccagaatgaaaaaggctagtattaatttcctaataaaattttttttcaaaagttatcgaggatatgactataaccttggaccagtttcaatttctttttattttttctgagaatacaccaaagattaatgtcaatggcaagtgagaaattgtccctagagaactattcaaggactttttcttactacatttgattggactggagtgaactgacattatagcatctttatcatcacctttaaaattctattttctcttagtagcaacagtgaagactttagaactattacttactttaaattattaaagtatatcacagacaaaatattcaattttacattaaagcaacattaagggtctcaatttcattgaacagaaacaaatgctgaagaaatttacaggtatgatttaattttagagagtgttctttctttagggaacaaaatgaaactagatctctcatttgtctgtatgggcaagatatggtaaacctcatgatcaaaacacatgccagttagaaacttgatcacagaaatgatgctcagtgttgaaacccaacaataaacaaacaaacaaaaacccccactctaaccagaggcatttaagcctctccactgaagttcctgtttcccaccagtttacgacccttaatgttactgcatgtatggttgcatatttgagatgattaaaaataaaagactggcttaaaagcacctcctcctctagtgtgtaattacatacaaactaaagattccttctgacgtcctaggaaccccatttgttaccgtttcatgtgtaagcaccattgaaccaatttttaaagcacatttgcagttatcaaatgtttagtgtgtcctcaagtttcattgatttgtttgcctttaagcaagaaaagagtaaagtgtattattttcccctgcttcttttcatatctgaattgtcaaaaaatgttaattttggaagtgcttttaatcactattttccccaacagactagaatggctccatgaaatttgacaattaagtaaggaaatctttatccccaaaagaagcacgtatcttaccctctaaactgcatgcaaagtaagggtctgtgtgagagtattttccccaaactcctaatggacatggcagacaatgtgtagaaaaatctgagttttgaactgaccaacttcaagtcttttaaaatctttgggcaaaaaaaaatatcatgtagcagttaaaaaaattattgacttacaaattatagaaaagatatgttatctacaatatatgccaggtgacccattaaatttaaaaaatgtgtgcgaatgagtaactacattaaaactaccatcttggatcttggtgctttccaaaattctgaaatcactattaaggagggaccataccagatttttttgttgttcttttccttggagaatggggaagaagttggaaagagaaggaagtaaaccttcactctttggtacagccctgtatagcaaacttcagcctggggcacatttttatggtcaaattaaaaacctttgagaataggagtttatcatagaaatgctgacagatcctaacccagagaagggctaagagcaacacagtaatattaagaaagctctccctcagcacgattgagcttcagcgcaagggatagagttgtctagtggacgcccttggccagtaaacaaccatgatttaatgtgcttgagacttggtcatatgggagctctgtgaccctctaagccaaattttcttttctttttgttttcaactgaaatatgcctcaaagggtaaaggattgcaattttagccttcattcatggatatattgctttctttcaacaatatctgatgggcctgttaactgccacccatggggagcaggttgcaggaaggtctcattgaacacaaaacaccaagtgttttcagtagtttattcacatttttttttctctgcttattttaatatgcaccacgtgtaagttagatgagggctacggtaaaaacatttttgatgactgaaatcttacttttccttctaacgatctggagcaaatcacatattcattgatcatgacgaataaaatgatttctgctacaatgttgagaaaaaatgtgttcattaatatgaacacatgtctacagagatgatttacacgatgcaagtaatgaaagagttcttccttaactagtctactatcaaactgaaaagatgaatcttaaaattcccttgaaaataccatatgattggtcatgtgtcagtaaaagaaagacggtccccatcaccaggccaccaccataagagagctatattaaatacttgggaaaaaatatggaaacaccggtggtgatgattaaattgataattacatagatacactgccataatgatacatatttgttctatgataagtgaaatcaaaaataagatcaatttggttatagaaattccttaaagaacaccaccacttaattatttcaaacttgaactatcccaagaatgtcgagaaaaaaattagaaagcactggctaaaagcaaagcaatctggatacaccaatgtagtcagcatgccttgtgcttgtctgttaaccctctgagtacatctctgacattcaggatcttggtagcttaatgttagaaagattgcattccatctgattactcaagatttctacttgactggtcacattccactgtttattcagcatagatcactcaaattctacagtgatgtgctgggatccccatgctgaatgggccctgcattcttctgagctgcccttctgcagtgtgctgagaaacaccccctagcttcacacggtccagagtccccctagacgtcgatgggaaaaggcctgagccatgcaccgcaggctcagtacactagatgctgtagcaatatagttaatgcccacagaaaaagcagtaattcagagaaagaaaggaaaatgacagtccactgcaggtaggtctctgcccattgcattcttcacacttttagagttgaggccaggctgtagagctactccatagccttggaatagtgctttgctttatatttctagagaaagcagtaatttccaactagttcagtgttcctcattaatatggaatctacctacacaccaacactctttctggtgttctgtgccccctacccccacctcccccccaaaaacaactcaactaatttactgatttatgctactttgtgattttgcgtgttatcacttccggatgctctaaaagggggggaaaaaaacctcaataaacgatatgctttttacatgtcaggacaacacagaccacagagatgaacctaaatgtaaaagagcaaaaaattttggtgatggtgttgcaaaagtaatgacatgtgatttaaaaatccatattaatgtagaccatagtttcagggttgaagagtaaaaatgcagcaagtgaagatcaatgtgcatttgaaaataaaggactatagaaacgttgttcacaaattttaagactctcaggtattaaagtatattcaaaacagagaacataggtactgttcagccaccagatgcaaatttcatgagatatccctctctggttgtctcgtggatcccagagcccagcaaaccttgggaatacatttgagttgggcacctgcctctaagacaccccaggagaatcctctctgagcactgtggtgatgcacagaacctgtgaatccccattctaaaatggaatctgttccagaagaaactcaggcctggagacactgcactagggagatagatttggtaacaagagtgaaaatacaggtctcagacaggacttggcccaaagacagaaaaaacactctgacctcctggacagctaaagacagtggtatttaaaaaaaatcattttaggggatggaggttttatcctcaggggtatcatctaggtctttcatcctgatcttcctaggagactatataggtaacctaaaggtgcacatggaattgtcttgccagtggtttattcactgaaaacttattgttagaacattctggattgtgttcccagtgtgctttctcctcagccatcttgcaaagcaactgcctccagtccccttgtgccccagctctcctatgtgtggatttcatactagatgtagattgcacagtgatgaccacagtgcgtggaaaagcaggtgagaaaaatcacaggatcttattccctctttctgtttgaaattccagccctgcagagcaccgggcaatttattgctcttttccaccagttgtttctttcctgtagatgtctgacactgagtagagagaccctcactcaccaagcacaagacaagctgtggtgactccctgagagtctgcgctggcgctagcagcagctgatatggaagcagcatttctggggcgtcatcagtacatcttcatgtggagacaatttggggggcaccatctatttcctgggtcaagctctttgccacaaacccaattccctccacttgggatgcagaactcactgcaactgacagtcatatctctaatgaaaaaaaaaatctgtttctgaataggattgtgaagaagaaagaaccgtgcgtgtgtcgaagttataaacctgccacgttctaaacccacagaaaaggacaaacaagatatcattctaaatgtccttcttttctggacatttcagcatctaacaacaccccttgatctgcagtaaaatcaagaaacatgtgtgtatacatccaaaggcctgaaaaattcccaaacaagaattctcaataaaattctatgcactcagagggttaacaagtgctatattacatactgcagatcctagcttgactgatgaaaacattcattgcttctaagtttaaaaaaaaattgcaaattggccttaaccctttgaggactctattagcagcaaattaccatcttcacaatcaccacgtgtcatcttattcagtaaagggaaaccgctacaaagatacctgaaaacactttcagttctgccattcaagcattgagcgctagatagatcagatgaaactgttttacacaaatttgggggaaaaaaatctcagagtctcaaagggttaagctaggactttgagtaaaagggtcttattaaaagggcgagttaggggagcgaacagtctcggaggagcttggggagtagtcttccgattccgagttgagttcgggaggagctggctgcgccttgtaccggctcctcacatcctggttgcgtcttcgtcggaaaacctgcctctccttatcaagagcggtggtcttatccaatacattcctggttgctggtagtagtccaaagaccctgatctcttgatggtaaacccgtggtccagtgctatgacagaaactccagctgctgtgctattcggcttggggcctgtgttgaaatgcttctttatctttccagctactgacagctgatgttcattttctgggaggccatcatcattaacccagggatgctcaagtacttgaacagcagaaaatcgctgatctacatcgaccaacagcatcatggtaatgagctcctttgcagaatcggaaacattatcccagtatggagaaggaaagtccacctgccccatcaaaatctgatcaaaaagcacctcctggtcatcaccacttccacggaatggagggaaaccacacagcaggatataagtgattacacctgctgcccagatgtccaccttgaggccgtatccagtctctgcaatgatttctggagccacgtatgttggggtgccacagactgtgtacagggggccgtctacaatggtggccagtccaaagtcacccagcttcagtgatttgctgccatcttggtgctcatacaccagcaggttctctggcttgatatcacggtggacgatgttcaggctatgcaggtatttgatggcgctggctaggttgtacagcatcccactggcgtctctctcggtgtatttgttagtggaagtaatggcatcaaaaaggtctcccccctttactaattccatgacaagatacagttcagttggcacatccatctcctcaatcagaagaacgatattgggatgcttcactcttcttaaaatagacacttcattctggatcatgtgctctttgcctcgacatttgcttttcttgataattttcagagcatactctctagcagtcgatctttctacacattccttgacaacagcaaaatttccatctcctattgttcttccgactttatatcgttctgttattgtagctggaatctggaagccttcctccgacacttcttctccagggccatcgttctcatccatcgagctgcagactttggtggacgcaagtgacgtagaggagccgccatgctgagagctcctctgcttccgcaggcttcctgggctggtgggtgatgggcttggcgacttgcctgagcgcggagtagagagctgactaccaggggttccattaacttctatgagttctaacatggacacagtcttagtgttggacctgaataccaacggcggaatcccgtctcagcactaagccaagcacccgcggaaatgggaatcggttggatgagtttaaggatggctaaggctgctcccagagcaggctgaatgagat

SEQ ID NO: 8585 - RNA, 7842 nt, Homo sapiens
  source 1..7842: mol_type = other RNA
aaactactgaaaatcaaagattaacctatgccatctgatccatgcagcaagtgataaattcagtattttcaaaagaaatattgaatttttttcttgagtcaaattgaaacctttcagaaacttgtttaaatgcgccaagtccctacgcacctttttagtatgtatgagcaaaatactgttgaatttcacactcaactaatcctttaataattttctttcagccagaatgaaaaaggctagtattaatttcctaataaaattttttttcaaaagttatcgaggatatgactataaccttggaccagtttcaatttctttttattttttctgagaatacaccaaagattaatgtcaatggcaagtgagaaattgtccctagagaactattcaaggactttttcttactacatttgattggactggagtgaactgacattatagcatctttatcatcacctttaaaattctattttctcttagtagcaacagtgaagactttagaactattacttactttaaattattaaagtatatcacagacaaaatattcaattttacattaaagcaacattaagggtctcaatttcattgaacagaaacaaatgctgaagaaatttacaggtatgatttaattttagagagtgttctttctttagggaacaaaatgaaactagatctctcatttgtctgtatgggcaagatatggtaaacctcatgatcaaaacacatgccagttagaaacttgatcacagaaatgatgctcagtgttgaaacccaacaataaacaaacaaacaaaaacccccactctaaccagaggcatttaagcctctccactgaagttcctgtttcccaccagtttacgacccttaatgttactgcatgtatggttgcatatttgagatgattaaaaataaaagactggcttaaaagcacctcctcctctagtgtgtaattacatacaaactaaagattccttctgacgtcctaggaaccccatttgttaccgtttcatgtgtaagcaccattgaaccaatttttaaagcacatttgcagttatcaaatgtttagtgtgtcctcaagtttcattgatttgtttgcctttaagcaagaaaagagtaaagtgtattattttcccctgcttcttttcatatctgaattgtcaaaaaatgttaattttggaagtgcttttaatcactattttccccaacagactagaatggctccatgaaatttgacaattaagtaaggaaatctttatccccaaaagaagcacgtatcttaccctctaaactgcatgcaaagtaagggtctgtgtgagagtattttccccaaactcctaatggacatggcagacaatgtgtagaaaaatctgagttttgaactgaccaacttcaagtcttttaaaatctttgggcaaaaaaaaatatcatgtagcagttaaaaaaattattgacttacaaattatagaaaagatatgttatctacaatatatgccaggtgacccattaaatttaaaaaatgtgtgcgaatgagtaactacattaaaactaccatcttggatcttggtgctttccaaaattctgaaatcactattaaggagggaccataccagatttttttgttgttcttttccttggagaatggggaagaagttggaaagagaaggaagtaaaccttcactctttggtacagccctgtatagcaaacttcagcctggggcacatttttatggtcaaattaaaaacctttgagaataggagtttatcatagaaatgctgacagatcctaacccagagaagggctaagagcaacacagtaatattaagaaagctctccctcagcacgattgagcttcagcgcaagggatagagttgtctagtggacgcccttggccagtaaacaaccatgatttaatgtgcttgagacttggtcatatgggagctctgtgaccctctaagccaaattttcttttctttttgttttcaactgaaatatgcctcaaagggtaaaggattgcaattttagccttcattcatggatatattgctttctttcaacaatatctgatgggcctgttaactgccacccatggggagcaggttgcaggaaggtctcattgaacacaaaacaccaagtgttttcagtagtttattcacatttttttttctctgcttattttaatatgcaccacgtgtaagttagatgagggctacggtaaaaacatttttgatgactgaaatcttacttttccttctaacgatctggagcaaatcacatattcattgatcatgacgaataaaatgatttctgctacaatgttgagaaaaaatgtgttcattaatatgaacacatgtctacagagatgatttacacgatgcaagtaatgaaagagttcttccttaactagtctactatcaaactgaaaagatgaatcttaaaattcccttgaaaataccatatgattggtcatgtgtcagtaaaagaaagacggtccccatcaccaggccaccaccataagagagctatattaaatacttgggaaaaaatatggaaacaccggtggtgatgattaaattgataattacatagatacactgccataatgatacatatttgttctatgataagtgaaatcaaaaataagatcaatttggttatagaaattccttaaagaacaccaccacttaattatttcaaacttgaactatcccaagaatgtcgagaaaaaaattagaaagcactggctaaaagcaaagcaatctggatacaccaatgtagtcagcatgccttgtgcttgtctgttaaccctctgagtacatctctgacattcaggatcttggtagcttaatgttagaaagattgcattccatctgattactcaagatttctacttgactggtcacattccactgtttattcagcatagatcactcaaattctacagtgatgtgctgggatccccatgctgaatgggccctgcattcttctgagctgcccttctgcagtgtgctgagaaacaccccctagcttcacacggtccagagtccccctagacgtcgatgggaaaaggcctgagccatgcaccgcaggctcagtacactagatgctgtagcaatatagttaatgcccacagaaaaagcagtaattcagagaaagaaaggaaaatgacagtccactgcaggtaggtctctgcccattgcattcttcacacttttagagttgaggccaggctgtagagctactccatagccttggaatagtgctttgctttatatttctagagaaagcagtaatttccaactagttcagtgttcctcattaatatggaatctacctacacaccaacactctttctggtgttctgtgccccctacccccacctcccccccaaaaacaactcaactaatttactgatttatgctactttgtgattttgcgtgttatcacttccggatgctctaaaagggggggaaaaaaacctcaataaacgatatgctttttacatgtcaggacaacacagaccacagagatgaacctaaatgtaaaagagcaaaaaattttggtgatggtgttgcaaaagtaatgacatgtgatttaaaaatccatattaatgtagaccatagtttcagggttgaagagtaaaaatgcagcaagtgaagatcaatgtgcatttgaaaataaaggactatagaaacgttgttcacaaattttaagactctcaggtattaaagtatattcaaaacagagaacataggtactgttcagccaccagatgcaaatttcatgagatatccctctctggttgtctcgtggatcccagagcccagcaaaccttgggaatacatttgagttgggcacctgcctctaagacaccccaggagaatcctctctgagcactgtggtgatgcacagaacctgtgaatccccattctaaaatggaatctgttccagaagaaactcaggcctggagacactgcactagggagatagatttggtaacaagagtgaaaatacaggtctcagacaggacttggcccaaagacagaaaaaacactctgacctcctggacagctaaagacagtggtatttaaaaaaaatcattttaggggatggaggttttatcctcaggggtatcatctaggtctttcatcctgatcttcctaggagactatataggtaacctaaaggtgcacatggaattgtcttgccagtggtttattcactgaaaacttattgttagaacattctggattgtgttcccagtgtgctttctcctcagccatcttgcaaagcaactgcctccagtccccttgtgccccagctctcctatgtgtggatttcatactagatgtagattgcacagtgatgaccacagtgcgtggaaaagcaggtgagaaaaatcacaggatcttattccctctttctgtttgaaattccagccctgcagagcaccgggcaatttattgctcttttccaccagttgtttctttcctgtagatgtctgacactgagtagagagaccctcactcaccaagcacaagacaagctgtggtgactccctgagagtctgcgctggcgctagcagcagctgatatggaagcagcatttctggggcgtcatcagtacatcttcatgtggagacaatttggggggcaccatctatttcctgggtcaagctctttgccacaaacccaattccctccacttgggatgcagaactcactgcaactgacagtcatatctctaatgaaaaaaaaaatctgtttctgaataggattgtgaagaagaaagaaccgtgcgtgtgtcgaagttataaacctgccacgttctaaacccacagaaaaggacaaacaagatatcattctaaatgtccttcttttctggacatttcagcatctaacaacaccccttgatctgcagtaaaatcaagaaacatgtgtgtatacatccaaaggcctgaaaaattcccaaacaagaattctcaataaaattctatgcactcagagggttaacaagtgctatattacatactgcagatcctagcttgactgatgaaaacattcattgcttctaagtttaaaaaaaaattgcaaattggccttaaccctttgaggactctattagcagcaaattaccatcttcacaatcaccacgtgtcatcttattcagtaaagggaaaccgctacaaagatacctgaaaacactttcagttctgccattcaagcattgagcgctagatagatcagatgaaactgttttacacaaatttgggggaaaaaaatctcagagtctcaaagggttaagctaggactttgagtaaaagggtcttattaaaagggcgagttaggggagcgaacagtctcggaggagcttggggagtagtcttccgattccgagttgagttcgggaggagctggctgcgccttgtaccggctcctcacatcctggttgcgtcttcgtcggaaaacctgcctctccttatcaagagcggtggttgctatgacagaaactccagctgctgtgctattcggcttggggcctgtgttgaaatgcttctttatctttccagctactgacagctgatgttcattttctgggaggccatcatcattaacccagggatgctcaagtacttgaacagcagaaaatcgctgatctacatcgaccaacagcatcatggtaatgagctcctttgcagaatcggaaacattatcccagtatggagaaggaaagtccacctgccccatcaaaatctgatcaaaaagcacctcctggtcatcaccacttccacggaatggagggaaaccacacagcaggatataagtgattacacctgctgcccagatgtccaccttgaggccgtatccagtctctgcaatgatttctggagccacgtatgttggggtgccacagactgtgtacagggggccgtctacaatggtggccagtccaaagtcacccagcttcagtgatttgctgccatcttggtgctcatacaccagcaggttctctggcttgatatcacggtggacgatgttcaggctatgcaggtatttgatggcgctggctaggttgtacagcatcccactggcgtctctctcggtgtatttgttagtggaagtaatggcatcaaaaaggtctcccccctttactaattccatgacaagatacagttcagttggcacatccatctcctcaatcagaagaacgatattgggatgcttcactcttcttaaaatagacacttcattctggatcatgtgctctttgcctcgacatttgcttttcttgataattttcagagcatactctctagcagtcgatctttctacacattccttgacaacagcaaaatttccatctcctattgttcttccgactttatatcgttctgttattgtagctggaatctggaagccttcctccgacacttcttctccagggccatcgttctcatccatcgagctgcagactttggtggacgcaagtgacgtagaggagccgccatgctgagagctcctctgcttccgcaggcttcctgggctggtgggtgatgggcttggcgacttgcctgagcgcggagtagagagctgactaccaggggttccattaactgagctggtggaggcaggggacttgctacgcctggacggtcctgggctcttggtggtgctcctgcgggatgatgaagctattttggtgtaagaagtggactttaccactcgacattcactttcatctagcaagaaatcatcctggtaacggaacttctccggtccacatgcaataaaaatgtcatcatcaccaaaaaagtcctgaaggcacatcacctgtttcccatccaacgtgtacaggcgtttcaccactcccgagtccagcttgatggcatcggtgatatcggtgaggacctgctcaaaggaatgagccgttttcttgttcagcagaatcctgacagctttccgtggcttcacgccacttctgatgatggtgaccagcttgggccgaatgaaatccttattctctcgcacctctgaagggcttcctttggcagtggccagtgaagacactgcccgagaagccgaggtggtcttgacgttcaccgaccagttggggttcacattcttggtgtactccagtttcttgaagggctctatggagccacatacataactctctccttccaccagttggtccaggctggaaatcttcttgagcccatcaatggtgtagattgttctcactccctggggcaaattcacgttatccgacagagttcgggtcaaatcagccagcagggcctcaaaagatcggaaccggtctggggagatggcatacacaatccctttgaagtatcgatctccgtttcgatagaaacgaactttcttggccttcttctcggagctgagcgtctgcagcgtgcgggtgcggtagaagctgcagtgggcgctgtgcgtcgggctcggcaggccgttcacccgcgaccctcggctgtatctctgcgccttatcccgctcgtcgaagtgctccagctccatgtctctgccgaaggacatgatggacttcaagtaggaccggtccgcggagagacgccgccgggggtctttgtggccgcgctgggggccgcctcctggtgctgtcctcgccgggctgggcgcggccggggctgcggggctgcagggctggggggcggcggcggggccgggctgggcggcagcagctgctggagcgcggcgcctcggttgcggccactagtgcagggatgtgcctcggcccgtcctcattgaaatgcggcgcttcgcacagcctcactccagcctctctctccagaggagggcggcggc

SEQ ID NO: 8586 - RNA, 7743 nt, Homo sapiens
  source 1..7743: mol_type = other RNA
aaactactgaaaatcaaagattaacctatgccatctgatccatgcagcaagtgataaattcagtattttcaaaagaaatattgaatttttttcttgagtcaaattgaaacctttcagaaacttgtttaaatgcgccaagtccctacgcacctttttagtatgtatgagcaaaatactgttgaatttcacactcaactaatcctttaataattttctttcagccagaatgaaaaaggctagtattaatttcctaataaaattttttttcaaaagttatcgaggatatgactataaccttggaccagtttcaatttctttttattttttctgagaatacaccaaagattaatgtcaatggcaagtgagaaattgtccctagagaactattcaaggactttttcttactacatttgattggactggagtgaactgacattatagcatctttatcatcacctttaaaattctattttctcttagtagcaacagtgaagactttagaactattacttactttaaattattaaagtatatcacagacaaaatattcaattttacattaaagcaacattaagggtctcaatttcattgaacagaaacaaatgctgaagaaatttacaggtatgatttaattttagagagtgttctttctttagggaacaaaatgaaactagatctctcatttgtctgtatgggcaagatatggtaaacctcatgatcaaaacacatgccagttagaaacttgatcacagaaatgatgctcagtgttgaaacccaacaataaacaaacaaacaaaaacccccactctaaccagaggcatttaagcctctccactgaagttcctgtttcccaccagtttacgacccttaatgttactgcatgtatggttgcatatttgagatgattaaaaataaaagactggcttaaaagcacctcctcctctagtgtgtaattacatacaaactaaagattccttctgacgtcctaggaaccccatttgttaccgtttcatgtgtaagcaccattgaaccaatttttaaagcacatttgcagttatcaaatgtttagtgtgtcctcaagtttcattgatttgtttgcctttaagcaagaaaagagtaaagtgtattattttcccctgcttcttttcatatctgaattgtcaaaaaatgttaattttggaagtgcttttaatcactattttccccaacagactagaatggctccatgaaatttgacaattaagtaaggaaatctttatccccaaaagaagcacgtatcttaccctctaaactgcatgcaaagtaagggtctgtgtgagagtattttccccaaactcctaatggacatggcagacaatgtgtagaaaaatctgagttttgaactgaccaacttcaagtcttttaaaatctttgggcaaaaaaaaatatcatgtagcagttaaaaaaattattgacttacaaattatagaaaagatatgttatctacaatatatgccaggtgacccattaaatttaaaaaatgtgtgcgaatgagtaactacattaaaactaccatcttggatcttggtgctttccaaaattctgaaatcactattaaggagggaccataccagatttttttgttgttcttttccttggagaatggggaagaagttggaaagagaaggaagtaaaccttcactctttggtacagccctgtatagcaaacttcagcctggggcacatttttatggtcaaattaaaaacctttgagaataggagtttatcatagaaatgctgacagatcctaacccagagaagggctaagagcaacacagtaatattaagaaagctctccctcagcacgattgagcttcagcgcaagggatagagttgtctagtggacgcccttggccagtaaacaaccatgatttaatgtgcttgagacttggtcatatgggagctctgtgaccctctaagccaaattttcttttctttttgttttcaactgaaatatgcctcaaagggtaaaggattgcaattttagccttcattcatggatatattgctttctttcaacaatatctgatgggcctgttaactgccacccatggggagcaggttgcaggaaggtctcattgaacacaaaacaccaagtgttttcagtagtttattcacatttttttttctctgcttattttaatatgcaccacgtgtaagttagatgagggctacggtaaaaacatttttgatgactgaaatcttacttttccttctaacgatctggagcaaatcacatattcattgatcatgacgaataaaatgatttctgctacaatgttgagaaaaaatgtgttcattaatatgaacacatgtctacagagatgatttacacgatgcaagtaatgaaagagttcttccttaactagtctactatcaaactgaaaagatgaatcttaaaattcccttgaaaataccatatgattggtcatgtgtcagtaaaagaaagacggtccccatcaccaggccaccaccataagagagctatattaaatacttgggaaaaaatatggaaacaccggtggtgatgattaaattgataattacatagatacactgccataatgatacatatttgttctatgataagtgaaatcaaaaataagatcaatttggttatagaaattccttaaagaacaccaccacttaattatttcaaacttgaactatcccaagaatgtcgagaaaaaaattagaaagcactggctaaaagcaaagcaatctggatacaccaatgtagtcagcatgccttgtgcttgtctgttaaccctctgagtacatctctgacattcaggatcttggtagcttaatgttagaaagattgcattccatctgattactcaagatttctacttgactggtcacattccactgtttattcagcatagatcactcaaattctacagtgatgtgctgggatccccatgctgaatgggccctgcattcttctgagctgcccttctgcagtgtgctgagaaacaccccctagcttcacacggtccagagtccccctagacgtcgatgggaaaaggcctgagccatgcaccgcaggctcagtacactagatgctgtagcaatatagttaatgcccacagaaaaagcagtaattcagagaaagaaaggaaaatgacagtccactgcaggtaggtctctgcccattgcattcttcacacttttagagttgaggccaggctgtagagctactccatagccttggaatagtgctttgctttatatttctagagaaagcagtaatttccaactagttcagtgttcctcattaatatggaatctacctacacaccaacactctttctggtgttctgtgccccctacccccacctcccccccaaaaacaactcaactaatttactgatttatgctactttgtgattttgcgtgttatcacttccggatgctctaaaagggggggaaaaaaacctcaataaacgatatgctttttacatgtcaggacaacacagaccacagagatgaacctaaatgtaaaagagcaaaaaattttggtgatggtgttgcaaaagtaatgacatgtgatttaaaaatccatattaatgtagaccatagtttcagggttgaagagtaaaaatgcagcaagtgaagatcaatgtgcatttgaaaataaaggactatagaaacgttgttcacaaattttaagactctcaggtattaaagtatattcaaaacagagaacataggtactgttcagccaccagatgcaaatttcatgagatatccctctctggttgtctcgtggatcccagagcccagcaaaccttgggaatacatttgagttgggcacctgcctctaagacaccccaggagaatcctctctgagcactgtggtgatgcacagaacctgtgaatccccattctaaaatggaatctgttccagaagaaactcaggcctggagacactgcactagggagatagatttggtaacaagagtgaaaatacaggtctcagacaggacttggcccaaagacagaaaaaacactctgacctcctggacagctaaagacagtggtatttaaaaaaaatcattttaggggatggaggttttatcctcaggggtatcatctaggtctttcatcctgatcttcctaggagactatataggtaacctaaaggtgcacatggaattgtcttgccagtggtttattcactgaaaacttattgttagaacattctggattgtgttcccagtgtgctttctcctcagccatcttgcaaagcaactgcctccagtccccttgtgccccagctctcctatgtgtggatttcatactagatgtagattgcacagtgatgaccacagtgcgtggaaaagcaggtgagaaaaatcacaggatcttattccctctttctgtttgaaattccagccctgcagagcaccgggcaatttattgctcttttccaccagttgtttctttcctgtagatgtctgacactgagtagagagaccctcactcaccaagcacaagacaagctgtggtgactccctgagagtctgcgctggcgctagcagcagctgatatggaagcagcatttctggggcgtcatcagtacatcttcatgtggagacaatttggggggcaccatctatttcctgggtcaagctctttgccacaaacccaattccctccacttgggatgcagaactcactgcaactgacagtcatatctctaatgaaaaaaaaaatctgtttctgaataggattgtgaagaagaaagaaccgtgcgtgtgtcgaagttataaacctgccacgttctaaacccacagaaaaggacaaacaagatatcattctaaatgtccttcttttctggacatttcagcatctaacaacaccccttgatctgcagtaaaatcaagaaacatgtgtgtatacatccaaaggcctgaaaaattcccaaacaagaattctcaataaaattctatgcactcagagggttaacaagtgctatattacatactgcagatcctagcttgactgatgaaaacattcattgcttctaagtttaaaaaaaaattgcaaattggccttaaccctttgaggactctattagcagcaaattaccatcttcacaatcaccacgtgtcatcttattcagtaaagggaaaccgctacaaagatacctgaaaacactttcagttctgccattcaagcattgagcgctagatagatcagatgaaactgttttacacaaatttgggggaaaaaaatctcagagtctcaaagggttaagctaggactttgagtaaaagggtcttattaaaagggcgagttaggggagcgaacagtctcggaggagcttggggagtagtcttccgattccgagttgagttcgggaggagctggctgcgccttgtaccggctcctcacatcctggttgcgtcttcgtcggaaaacctgcctctccttatcaagagcggtggttgctatgacagaaactccagctgctgtgctattcggcttggggcctgtgttgaaatgcttctttatctttccagctactgacagctgatgttcattttctgggaggccatcatcattaacccagggatgctcaagtacttgaacagcagaaaatcgctgatctacatcgaccaacagcatcatggtaatgagctcctttgcagaatcggaaacattatcccagtatggagaaggaaagtccacctgccccatcaaaatctgatcaaaaagcacctcctggtcatcaccacttccacggaatggagggaaaccacacagcaggatataagtgattacacctgctgcccagatgtccaccttgaggccgtatccagtctctgcaatgatttctggagccacgtatgttggggtgccacagactgtgtacagggggccgtctacaatggtggccagtccaaagtcacccagcttcagtgatttgctgccatcttggtgctcatacaccagcaggttctctggcttgatatcacggtggacgatgttcaggctatgcaggtatttgatggcgctggctaggttgtacagcatcccactggcgtctctctcggtgtatttgttagtggaagtaatggcatcaaaaaggtctcccccctttactaattccatgacaagatacagttcagttggcacatccatctcctcaatcagaagaacgatattgggatgcttcactcttcttaaaatagacacttcattctggatcatgtgctctttgcctcgacatttgcttttcttgataattttcagagcatactctctagcagtcgatctttctacacattccttgacaacagcaaaatttccatctcctattgttcttccgactttatatcgttctgttattgtagctggaatctggaagccttcctccgacacttcttctccagggccatcgttctcatccatcgagctgcagactttggtggacgcaagtgacgtagaggagccgccatgctgagagctcctctgcttccgcaggcttcctgggctggtgggtgatgggcttggcgacttgcctgagcgcggagtagagagctgactaccaggggttccattaactgagctggtggaggcaggggacttgctacgcctggacggtcctgggctcttggtggtgctcctgcgggatgatgaagctattttggtgtaagaagtggactttaccactcgacattcactttcatctagcaagaaatcatcctggtaacggaacttctccggtccacatgcaataaaaatgtcatcatcaccaaaaaagtcctgaaggcacatcacctgtttcccatccaacgtgtacaggcgtttcaccactcccgagtccagcttgatggcatcggtgatatcggtgaggacctgctcaaaggaatgagccgttttcttgttcagcagaatcctgacagctttccgtggcttcacgccacttctgatgatggtgaccagcttgggccgaatgaaatccttattctctcgcacctctgaagggcttcctttggcagtggccagtgaagacactgcccgagaagccgaggtggtcttgacgttcaccgaccagttggggttcacattcttggtgtactccagtttcttgaagggctctatggagccacatacataactctctccttccaccagttggtccaggctggaaatcttcttgagcccatcaatggtgtagattgttctcactccctggggcaaattcacgttatccgacagagttcgggtcaaatcagccagcagggcctcaaaagatcggaaccggtctggggagatggcatacacaatccctttgaagtatcgatctccgtttcgatagaaacgaactttcttggccttcttctcggagctgagcgtctgcagcgtgcgggtgcggtagaagctgcagtgggcgctgtgcgtcgggctcggcaggccgttcacccgcgaccctcggctgtatctctgcgccttatcccgctcgtcgaagtgctccagctccatgtctctgccgaaggacatgatggacttcaagtaggaccttttgatgtgacctcacggtctgacacctttcccagggtatggaagccagtggatcaccttctcatcctttttgcccgggatgcacccacgcagtgcctcttcggatgaccaaccctcccaagctatgcactctggtgccccccacattgggaagagctggatctgttc

SEQ ID NO: 8587 - RNA, 6772 nt, Homo sapiens
  source 1..6772: mol_type = other RNA
aaactactgaaaatcaaagattaacctatgccatctgatccatgcagcaagtgataaattcagtattttcaaaagaaatattgaatttttttcttgagtcaaattgaaacctttcagaaacttgtttaaatgcgccaagtccctacgcacctttttagtatgtatgagcaaaatactgttgaatttcacactcaactaatcctttaataattttctttcagccagaatgaaaaaggctagtattaatttcctaataaaattttttttcaaaagttatcgaggatatgactataaccttggaccagtttcaatttctttttattttttctgagaatacaccaaagattaatgtcaatggcaagtgagaaattgtccctagagaactattcaaggactttttcttactacatttgattggactggagtgaactgacattatagcatctttatcatcacctttaaaattctattttctcttagtagcaacagtgaagactttagaactattacttactttaaattattaaagtatatcacagacaaaatattcaattttacattaaagcaacattaagggtctcaatttcattgaacagaaacaaatgctgaagaaatttacaggtatgatttaattttagagagtgttctttctttagggaacaaaatgaaactagatctctcatttgtctgtatgggcaagatatggtaaacctcatgatcaaaacacatgccagttagaaacttgatcacagaaatgatgctcagtgttgaaacccaacaataaacaaacaaacaaaaacccccactctaaccagaggcatttaagcctctccactgaagttcctgtttcccaccagtttacgacccttaatgttactgcatgtatggttgcatatttgagatgattaaaaataaaagactggcttaaaagcacctcctcctctagtgtgtaattacatacaaactaaagattccttctgacgtcctaggaaccccatttgttaccgtttcatgtgtaagcaccattgaaccaatttttaaagcacatttgcagttatcaaatgtttagtgtgtcctcaagtttcattgatttgtttgcctttaagcaagaaaagagtaaagtgtattattttcccctgcttcttttcatatctgaattgtcaaaaaatgttaattttggaagtgcttttaatcactattttccccaacagactagaatggctccatgaaatttgacaattaagtaaggaaatctttatccccaaaagaagcacgtatcttaccctctaaactgcatgcaaagtaagggtctgtgtgagagtattttccccaaactcctaatggacatggcagacaatgtgtagaaaaatctgagttttgaactgaccaacttcaagtcttttaaaatctttgggcaaaaaaaaatatcatgtagcagttaaaaaaattattgacttacaaattatagaaaagatatgttatctacaatatatgccaggtgacccattaaatttaaaaaatgtgtgcgaatgagtaactacattaaaactaccatcttggatcttggtgctttccaaaattctgaaatcactattaaggagggaccataccagatttttttgttgttcttttccttggagaatggggaagaagttggaaagagaaggaagtaaaccttcactctttggtacagccctgtatagcaaacttcagcctggggcacatttttatggtcaaattaaaaacctttgagaataggagtttatcatagaaatgctgacagatcctaacccagagaagggctaagagcaacacagtaatattaagaaagctctccctcagcacgattgagcttcagcgcaagggatagagttgtctagtggacgcccttggccagtaaacaaccatgatttaatgtgcttgagacttggtcatatgggagctctgtgaccctctaagccaaattttcttttctttttgttttcaactgaaatatgcctcaaagggtaaaggattgcaattttagccttcattcatggatatattgctttctttcaacaatatctgatgggcctgttaactgccacccatggggagcaggttgcaggaaggtctcattgaacacaaaacaccaagtgttttcagtagtttattcacatttttttttctctgcttattttaatatgcaccacgtgtaagttagatgagggctacggtaaaaacatttttgatgactgaaatcttacttttccttctaacgatctggagcaaatcacatattcattgatcatgacgaataaaatgatttctgctacaatgttgagaaaaaatgtgttcattaatatgaacacatgtctacagagatgatttacacgatgcaagtaatgaaagagttcttccttaactagtctactatcaaactgaaaagatgaatcttaaaattcccttgaaaataccatatgattggtcatgtgtcagtaaaagaaagacggtccccatcaccaggccaccaccataagagagctatattaaatacttgggaaaaaatatggaaacaccggtggtgatgattaaattgataattacatagatacactgccataatgatacatatttgttctatgataagtgaaatcaaaaataagatcaatttggttatagaaattccttaaagaacaccaccacttaattatttcaaacttgaactatcccaagaatgtcgagaaaaaaattagaaagcactggctaaaagcaaagcaatctggatacaccaatgtagtcagcatgccttgtgcttgtctgttaaccctctgagtacatctctgacattcaggatcttggtagcttaatgttagaaagattgcattccatctgattactcaagatttctacttgactggtcacattccactgtttattcagcatagatcactcaaattctacagtgatgtgctgggatccccatgctgaatgggccctgcattcttctgagctgcccttctgcagtgtgctgagaaacaccccctagcttcacacggtccagagtccccctagacgtcgatgggaaaaggcctgagccatgcaccgcaggctcagtacactagatgctgtagcaatatagttaatgcccacagaaaaagcagtaattcagagaaagaaaggaaaatgacagtccactgcaggtaggtctctgcccattgcattcttcacacttttagagttgaggccaggctgtagagctactccatagccttggaatagtgctttgctttatatttctagagaaagcagtaatttccaactagttcagtgttcctcattaatatggaatctacctacacaccaacactctttctggtgttctgtgccccctacccccacctcccccccaaaaacaactcaactaatttactgatttatgctactttgtgattttgcgtgttatcacttccggatgctctaaaagggggggaaaaaaacctcaataaacgatatgctttttacatgtcaggacaacacagaccacagagatgaacctaaatgtaaaagagcaaaaaattttggtgatggtgttgcaaaagtaatgacatgtgatttaaaaatccatattaatgtagaccatagtttcagggttgaagagtaaaaatgcagcaagtgaagatcaatgtgcatttgaaaataaaggactatagaaacgttgttcacaaattttaagactctcaggtattaaagtatattcaaaacagagaacataggtactgttcagccaccagatgcaaatttcatgagatatccctctctggttgtctcgtggatcccagagcccagcaaaccttgggaatacatttgagttgggcacctgcctctaagacaccccaggagaatcctctctgagcactgtggtgatgcacagaacctgtgaatccccattctaaaatggaatctgttccagaagaaactcaggcctggagacactgcactagggagatagatttggtaacaagagtgaaaatacaggtctcagacaggacttggcccaaagacagaaaaaacactctgacctcctggacagctaaagacagtggtatttaaaaaaaatcattttaggggatggaggttttatcctcaggggtatcatctaggtctttcatcctgatcttcctaggagactatataggtaacctaaaggtgcacatggaattgtcttgccagtggtttattcactgaaaacttattgttagaacattctggattgtgttcccagtgtgctttctcctcagccatcttgcaaagcaactgcctccagtccccttgtgccccagctctcctatgtgtggatttcatactagatgtagattgcacagtgatgaccacagtgcgtggaaaagcaggtgagaaaaatcacaggatcttattccctctttctgtttgaaattccagccctgcagagcaccgggcaatttattgctcttttccaccagttgtttctttcctgtagatgtctgacactgagtagagagaccctcactcaccaagcacaagacaagctgtggtgactccctgagagtctgcgctggcgctagcagcagctgatatggaagcagcatttctggggcgtcatcagtacatcttcatgtggagacaatttggggggcaccatctatttcctgggtcaagctctttgccacaaacccaattccctccacttgggatgcagaactcactgcaactgacagtcatatctctaatgaaaaaaaaaatctgtttctgaataggattgtgaagaagaaagaaccgtgcgtgtgtcgaagttataaacctgccacgttctaaacccacagaaaaggacaaacaagatatcattctaaatgtccttcttttctggacatttcagcatctaacaacaccccttgatctgcagtaaaatcaagaaacatgtgtgtatacatccaaaggcctgaaaaattcccaaacaagaattctcaataaaattctatgcactcagagggttaacaagtgctatattacatactgcagatcctagcttgactgatgaaaacattcattgcttctaagtttaaaaaaaaattgcaaattggccttaaccctttgaggactctattagcagcaaattaccatcttcacaatcaccacgtgtcatcttattcagtaaagggaaaccgctacaaagatacctgaaaacactttcagttctgccattcaagcattgagcgctagatagatcagatgaaactgttttacacaaatttgggggaaaaaaatctcagagtctcaaagggttaagctaggactttgagtaaaagggtcttattaaaagggcgagttaggggagcgaacagtctcggaggagcttggggagtagtcttccgattccgagttgagttcgggaggagctggctgcgccttgtaccggctcctcacatcctggttgcgtcttcgtcggaaaacctgcctctccttatcaagagcggtggttgctatgacagaaactccagctgctgtgctattcggcttggggcctgtgttgaaatgcttctttatctttccagctactgacagctgatgttcattttctgggaggccatcatcattaacccagggatgctcaagtacttgaacagcagaaaatcgctgatctacatcgaccaacagcatcatggtaatgagctcctttgcagaatcggaaacattatcccagtatggagaaggaaagtccacctgccccatcaaaatctgatcaaaaagcacctcctggtcatcaccacttccacggaatggagggaaaccacacagcaggatataagtgattacacctgctgcccagatgtccaccttgaggccgtatccagtctctgcaatgatttctggagccacgtatgttggggtgccacagactgtgtacagggggccgtctacaatggtggccagtccaaagtcacccagcttcagtgatttgctgccatcttggtgctcatacaccagcaggttctctggcttgatatcacggtggacgatgttcaggctatgcaggtatttgatggcgctggctaggttgtacagcatcccactggcgtctctctcggtgtatttgttagtggaagtaatggcatcaaaaaggtctcccccctttactaattccatgacaagatacagttcagttggcacatccatctcctcaatcagaagaacgatattgggatgcttcactcttcttaaaatagacacttcattctggatcatgtgctctttgcctcgacatttgcttttcttgataattttcagagcatactctctagcagtcgatctttctacacattccttgacaacagcaaaatttccatctcctattgttcttccgactttatatcgttctgttattgtagctggaatctggaagccttcctccgacacttcttctccagggccatcgttctcatccatcgagctgcagactttggtggacgcaagtgacgtagaggagccgccatgctgagagctcctctgcttccgcaggcttcctgggctggtgggtgatgggcttggcgacttgcctgagcgcggagtagagagctgactaccaggggttccattaacttctatgagttctaacatggacacagtcttagtgttggacctgaataccaacggcggaatcccgtctcagcactaagccaagcacccgcggaaatgggaatcggttggatgagtttaaggatggctaaggctgctcccagagcaggctgaatgagat

SEQ ID NO: 8588 - RNA, 4193 nt, Homo sapiens
  source 1..4193: mol_type = other RNA
aaactctacttgtccttctgagtgtaattacgtacatgcagtagctcaggagacaagcaggtttaccctgtggatgagtctgaaaaaattcatcagcagctcatggaaaatctataaccaagagatgatgggttattggcatcaccactgagcataaagtcaatatatataaatattgttctccgtatcttattcaaatatgattaattactttcattattaaactgatgaaggaaaaggttctaaaaatttcccttcaaaaaaggtgcatttttaaagaggcaacccagtattacatatctgggtcctagctgcaactctgatactcactctgcatacatcagcctctctggacatcagattctctctgtgccacatcaggagtttgaattagatgattctaacactgtgcagctttagcagtctataattcaattaattagagttaggactcagtttttggtcacctactgggagattttccagatcacctctctcccaggctgctttggtaccctttgatgcgctctaaattgacttgctgctttggccccattaaagcatttatcacactctgttgcatttgtctatccctattggatagaactccgtgagggaagagaccatttctaaattcatctttgaattctcagtgtctgctatagtccctgactcacagtacaataaaaaaataatgttaagttggtgtaagtaaactcaggatagcagtaacttaagcaatgttaaaatatagtgatttcctagtgaactgaggtgcatttcatagattcacagtattttaaccatggaaaggatgatagtgataacataggccagagattctcaacctagctttcccctatacacttgatggattgccgtcagtaacaatagctcactaaaactgtgatgtttaaccaagaggaattgtggcaggtgggcaaaggagaggaagggaagaaggtgcttgacaaagcctcccaagggcatcccagcaaatctgaatatataatccacaattttagagctgctagttcttttttggtatcttcattttacaaatgaaaaagcatgaaaatgtgatgataagagatattttcaagttgctctactatttagtggagatttttatattacaattgaattatttttgtttgctaccttttgacatcatacatggatatagtcttcagggcaaatgttttaagcaaacaaatcaaagctagggatcgaaattaagatttactgctttccaaatttgaaagatatatctgaaagtaagaaactcagaagtctgcacctagcttcctgggtctgctctgggaagtaagctttttcaaggtctaggctgggccccaaaaggatgaacaaggtgattacagattttcatggccctgtgcctatccaaaactctttttgatctgccattaagatctgagatcaaccctgtaaaggtctctgggtggctatggtcattgtaagttcttattgactttggtcccagtccttgatatccttcacttaatgagtacctatcataagccagaccctattgtgggattggtacacactggtgtgataaagagacataattctactttttgtggtaattagaacctactaggagagggagattaaaatacacacagaggcaaatattaattcattcaatattcatttatcaccttctatatgcaagatgctggaggaataccagaaacaaaagtttctgcttttgtggtccttacgagtctaatgggagagatggatgataagtaagggcttaattaattaatttaacaaataaatattgtgcaccagacttacgccaaacattgttttatacactgtgccagtgctaatggacaaaataaataaaatctaatggcatttgcatgctaatgagagtcacacaatgaacacacacataaacaactacaagtgccaaggagaagaaataaaactgggtaaaggagagtgctataaatgggggctgctgttttagatgtgttagtaaaggaacaccctcctgagtcagtgacatttgagaagagtcctgtagaaagtgaggaggcaaagttgcagatacctggggaaatgtcctcaggagggggaactcctgtgcatactgggaacagccaggaaggtcagtgtgaaaaagtgagagagggaagaatatgaaaaatgggatgtgtaaagttggtagccgggggtcagatgatgtaactcataattagaatttcagattagttgaaatttgaagtgctctgaagaaaataaacatgtggttggaatagagaataacagagaagggcctgtttggttagcattggtcgaggaaggctcactgagaaagcaaaatttaaactacgttttggtgtattagattaataagatctttaggaaaagcattctggagagagtgaagagtatacataaaagcaggtccacagtcacaacttatctgtctttcagtttttacatttataaccaagaaaatgatcaaaaactgaaattaccaagaaataataacgcattaattatgcatcctggggtagaaatttaattatatattaagaaaatctatagatcagctttttgcttctttgtattacaaggctaaaacatcatatattataattcgatttttagaaatatactgagcactgtaatttacatgtcactatgcataaatctacatgttgaatccaagtggtcataagaggagatatattcaattttagtccaatattttatgttagacagtggtatagaaagtagtacatgtcatttacccttgtaacaaagagaagatactgataaggagattagtgtggaattcttctcttccagaccttaaaatgttcatagcaactcttctctacatcagaggttagtttgctcagattttaatctttaaaaccaggaatgaccttcagctaaactcaagggaacaaagaagaatgcaatccttaatacttaacacgtggatattaaagaacatagaaatgcttcaggaattaaagaccgcatggatttagggactttctaaagtatggtagctccaattctccttcacttttcatctcaaggtcagagaagataatacaaaataactcttcaaattttacttttgcttactctgttcccttaatttttaagccaaatggctcttgaatactcatggcttatgaaggaataatacaaaaccaactcttggagaaaaatgaataattaaaacatttctaatactttccttatgacatgattagtagcttccaatctgcatttaaatgcttacataagatacaaggttggtattactatcatctaacttttccgtgagttaaattcattttggacaagttgcaaaaatgaaaatggaaatctttatttcttggcttctaaaataagtcgtaatttaaaatattgattaaacaaatcctagtgtgcttttcatttaagacaaatcaaacttttgtcctttaaaaaatctgctataaaaccaagaacttttattttgtggatttcaaccttatggaaaacaagtataagaacaaaaattgaatgcaaataactatcccatgggtgccacacttgtcatagaatttgtgatacattacaatttttctcttttcccttttcacttttcaaggcaggcagagcttattacttcatgcgtcttccgattcaagccctgggaagcctataggttttctaatcagctttattcactggtttttataaaatctgtatttgccagaaaattgcttttgcttacactccagaggggtttgccccttctcttgctcctagtttgtttgtttgttttaatttgacacggagaaagattaaggaagaaggaaaataaaaattaggttagtctttatgtcgttttcaagatgtatgccctggtgttttgatcaggggtagaaaagaggagggctgactatattttatgtctcttgtcctaaatccttcccatagcagcagccgcatgtgttttagtgtacaaacaagtaagcgcttgcttgctctctcatattttctctgggctccagcaaatattaaaaaattgaactgaacttttttatttctttgtaaatcaatgagtgtttcctttcacactatatagttacaaaacactccaggagttttccattttttttttttttttctttttgacagagtct

SEQ ID NO: 8589 - RNA, 10206 nt, Homo sapiens
  source 1..10206: mol_type = other RNA
aaagactctgcaagatgccttgaagtctttttgctcaaattctccctttgcatgttggggctaaagcaaatctgggacaggagagagactggggaggcagtgggtgtggttattgaagaagttaatgtgggtaacaccagagatcctggaggtgatgacagtgttctgtaacatgacaatggtggtgaatactagaacctacatgtgataaaactgtatagaattaacacacacatacaaatgaagtaaagctaaggaaatatgaataagatcggagaattttatcaacctcaatatcctggttttgatattgtactatcattttgcaagatgttaccattaggcaaaactgggtaaagggtatatgagggctctattttttcttgcaactgcatgtcaacctacaattatctcaatacaaatgtcaattatacaaaatagaagttagatttaatgtctttcttttttatatgtgcagtctcaggttatacctgcagaaccatatacttgtattatgctgctgacaaaaaagtgtgaaagaacccaatgccttcattttaaagatgagtcacataaaggttaggcgactatccaagctgataaagcttgtttatattaagcatttatcatggtttctgcctttccataagttataatgatggagaattttatggcaatgttaagacgtccagtcctgggttcagacaactttgggatatatcctatcaggattcaaacggtctcaccatgtgatcttagaaaaataatgtttgcattttctactcattgaaatgagataataaaataatcccatacaccgatgggatttcaagatactgaaataaaataattcatgctggtacagtggatgcgtgataggagactctcaaaataatgcctgttttccggcatattaagtgctggacactagagctaaaggctttgaatacaaagagataaaaggtacagcttctgcttccataaacagagtctaggagagagaataacacaaagataattgcacagattaaaatgtgaaaaataggagagtacagggaattggtggttgatgaggctggataagtaaatgcagcaggtgaggaaggcacctttttaggaatccacactttggctaggtttatgtcatcaaagagcctaacagcctgtttttttgttttttggtttttttttttcacgtgacaggatcttgctttattgcccaggctggagtgcagtgatgtgatcatagctcactgctgcctcaaatggtggggctcaagtgatcttctcacctcagcctcccaagtagcctggactataggcacatgccaccatacctggaattttaaaagtgtttgtagagacaaggtcttgctatgttgcccaggatggtctcagacttctggcctcaggaaatcctcctgcctcagccctgtaaagtgctaggattacaggtatgagccgccatggctggccgagagcctggtcttttagagttagatggatttgaggatggagctcagtgctatccctcaccagctgtgttactgtgggcaaaattgcttatttttctaatcctcccttttctcaaccccaaaataagaagattgcaatagaataattccctctagggtggctgtgtcagttaatgagatcatgaatatggacatgcttagcactcagtatcttcctgcagcttgctaaaatagccacagtgtatgcaaaaatgtaaatatctttcggtataactgggctacaaatgatggtagaaaacataatcataccactccaaggtcatttcacatcttcatgtttaaaacagactattctgaaatagtcatttgattgagaaattaaattatctgatttcaacattcacatgtgctctctggtacattctctcctctcaagcactctctctccctttcctctgattttgtctcagaattatagttgtcaatgaaaagagtcaaaccctgtaaaacatttgaagagatttattctgagccaaatatgagtgaccaatggcccacaacacagccttcaggagatcccaaacacatgtgcctaaggtggtcaggctacaacttggttttatacattttagggacacaaaagacattaatcagtacaaaaaagatgtacactggttcagtctggaaaggtgggacaactggaaggcaagggcttccaggtcataagcagattcaaatactttctgactggcaattggttgaaaggattaagttattacctaaagacttagaatcaatggaaaggaacgtctgggctaaggggttgtgaagaccaagtttttatcatgcaggcaaagtctccaggtagctggctttagagagaatacattataaattattcttatcagacttagagagtctgttctctcagtaatttcaaaagggaggagggtataatgaggcatgtccgaccccacttcccatcatggcctgaactagtttttcaggttaacttcggaatttactttgctgagaggagaggtccattgcagtggttggagggcttagaattttatttttggtttacatagtctttgtgcaggggaacacttaacaaaaaatgaaggagcaagggaatatgtgtcaggtctgggtgctggtggctgggccctgctggcttctgtaggggcatttcaccccgttgggtctttggtttaggcttcagtcctgctgcatcccctgctggggtcatttggtccccctggcctttggatgcaagtgagcatctgggcccactgtcctcctacaaggcctctggtccagatgtcctcaccctgtgctcacctcaccccatccctggccaccctcagtctctggccctctgtatcagttatttattgctgctggaacaaatgcctgcaaacttagtggctcaaaataaaaacttttcttagaggtctggaggttagaagtccaaagcaggtctcatggggctaaaatcaaggtgctggagagactgtgctctttctgaaggctctaggggggaacctgtctccttgccttttcttgcttctggaggctcctacctgtcttttattatctgattttcttgcctccctcttttaaggacccttttgattatatcagacccacccggataatccaggataattgtcccaactcaggattctgtaagccaaaacaaaaatcccaggccccccaacagactgaacagagccaagagaaacctgaaaaatgaaattcacaatcatcatgggaagggaggttggacacacctcgttataccctctcccttttggagttcagcacaactgaccagcattaacactaaaatagagatcacaagactgacaaaacagactctgtggcaataagagatcaaattccatcctgactctagtgtagcatcacatgacagatatcagaccctgaaggaaatcaaagtattttaccccaaaatacatttctctgacactttgaaatggccctgcaaagctgtcttgtgtggggaaaattctacatctgtagagaacctccattaatgcagcccagtctttctgggatctaggagagattaactaagagtctgacacctttaaggtatgaaaagacacatttaccatctattcccactgaagcctgctacctggaggcttcatctacataataagaaccttggcttccacaactctccccacccgcttaccttaaccaaagcatttctttctactgatttcaaatagtttaactctttcaaacaattgccaatcagataatttttgaatccatctatgacctgtaagctcccccactctttgagatgtctcacctttccaggccaaatcaatatattccttacatgtattgatctatgtctttgcctgtaacttgtctccctaaactatataaaaccaaactgtaatctgacctccttgggcaccctttctcaggaccccctgaggctcttcctggagccatggtcactcatattggcttagaataaactcctttaaatattttacagagtttgggttttttgttcacaattattaatcacacatttgccaagtaaggtcacatactcacaggttctgggggttaggatgtggacatgtttggggggcaattgttctgctttccataccctcctatcattcccaacccctttctgggacaagcagcacacactggattcccccatgtcactgatgggccatgggaaagtggagatgctactttacgccgtcccgctgctgaaagcgccaaactgcctctcctcctccatgcagctgcctcatgggggtgggaggcaccaggtgaggccccttatctcagagattgaagtggaaagagtggcacaaacctatctgggtgtgtgttatatgacatcattcctggggtacataggaggcatgaataaagagcactggggaattttcagcctaagccttgatgtgacaatcctgcattccccaatccttcctgttcccactataatcaggaccaaaagagctgaatcctgcaggtagtgagctgggcttgattaggaaatgagaaggttctgggtgtgatgatctaagttccatataggtaggctcagatgcatgctgggcttgctagctgtatcggagttgatctttctgagaaggtgagttcaagctctgtttcactgggtggcagggaaagttttgttcaaggcagaaatggaaagtagagtctcacactttgacacatagggagagaccccagtatccaaaatcccagctgctgcagcatacccgtgggctctcttgagggcccaggaggagaaagaacctgaaagccaaggttggtacgctgttatggattcctggtttcctctgtgtgtgtggttgggggtaggggttggagtacctgttctcacatgcttctgtcctcaattttaaggtgtggcttctcaggagtctgtgttccctgagaacaggaggtgaagaatgaaaaggaaaatggctcggtcatttctagaggtgatatcacaggtgaactgcttacttctgatttccttcctaaaataccaatttacagggctaaagacattttgcatttgttccacaaggatgcagctccccattctggtgatgaggtgacagtcagagaggcaacagaggggacctaaataacccagaagctttctttagtgacccaagatttagtattcattcaacaaactgctcaaggtctgacccaagatttagtattcattcaacaaactgctcaacgactgacccaagatttaggattcattcaacaaactactcaaggactgactgaccaagaggagtcattagcacaggtcttctaggcatgaatttgtttgaaaacttttaagctgaagaataggagtccctggggatagtgagttcagtttgaagttggacagcttgcatgtgttggcagcgcagggagcaatggcttaacttgctctcaaatctatgggagagctggagcagggcacaggcagtcaggtggatgggatgaaggtggagggatgccaccatatttctgggtaacaaaagggcactcgtcctgacagacttaaaatccaacacatcaaactatgctaattaaaataatatagaaatgataatacgttgatgggtaaacagaagaaaatagaaggccagatacacattgtggtagaatgaacaatctcccccacccattgcaaaatgtccccatcctagtccctggaagctgtgaatgtgttaccttacatggtaaaagggactttgcaggtgtcattaagttgaggatcttcagatggggggtttctcctgggttgtctgggtgggcctgaaatgtaatcactgggtctcttgcgtctttgggtaaggaaggtcttgttagttcacaactgcccatgggagaattttctccttctgtgcaaatatctgcaacactccctgaaaatgccagttgaattttctaacttcatattcttcagtaaagcatcgtagctcatctagttggaaagagacgactaccttcattaacagaaggtagaactcgccagaatgtaagatgatccagagatttcagagaaacttgtttctcgagtttcagtgctgacatcagggaaggcagctcattcataggctccctttgctaaactcgagatcaatgtagaaagaatcttagtcgaagcctaattcttcgtggattcatgctgtatggagtatcttggaaatataaatatgtaaatgttgaagaaatggagatgtgatcagaaatgtactttttttattgcactgacttgaatctttggccaaggcaggtggttcatgaggtcaagagttccagaccagcctggtcaacatagtgaaaccccatctctcctgctggttcttgttggcatggctcagtagatgagcctgtggctgctctcctttccccaggatctcctccagctctttcagctcctgggctaggtgtgtgcttagcaacaccacaaatggcaccaacctctgtaggacacccacatcgtttaggtagaagacagtaaaaactgccacagctttgtctgtgggttccagcttgtctttattctcttagtgttcactttcactacttgcttggcagtttagcattgtgtaagttatttgatttgttgctttgttggaatttattactttgttggaacttattccttgtgggatttctgatgtaaaagaaagtttgatttgtggcgaaatgttttctcacatttgttacattcataaggtttctctcctgtgtgtattttctgatgttcagtgagagtccacaggcgacggtaggttttcccacattgattacattcatatggtttctctcctgtgtgaattcttctatggactctgaaggctgacttatggcagaaggatttcccacattcattacattcatatggtttctccccagtgtgagttcgctgatgttcaacaaaggagaacttctgacagaaggttttcccacattcattacactcatagggtctctgtcctgtgtgtgttctctgatggtgagtcagggctgacttcctgcagtaggttctcccacattcattgcattcatatggtctctcccatatagttctctgatgtacaatgaggtgtgagtttttgctgacggcatgcccatgttcactacactcataaagattctcctttgtgttcattctcttacactgactgcagtttgacttcacaatggagattctaccacatttattaaacacaccatgtttctctcctgtgtgtgttctctgatgtatagtgagtgttgacttatggcagaaaaatttcccacattcattacattcataagacttctttcctctatgagttatctgatgtgcaatgagggctgatttcgtacataaaaattttccacattgactgcattcatagggcttctctcctgtatgacttcttcgatgcacattgagggcagattgacaaaagaaggttttctcacattcactacattcatagggtttttcccctgtgtgaattctctgatgcgcagtaagggctgactgacagaagaaggttttcccacattccttacattcatttggcttctctcctctgtgagttctttgatgtacaacaagatacgatttcttgctgaaggcatttccacattccttgcattcgtaaggcttctcccctgtgtgtgacctgaaatgttcagccagggctgacttccgaaaaaaggtctttccacattcattacactcataggatttctcccctccatgaattttctggtgtacaataagggcagatttgtcaatgaaggttttcctgcattcactgcattcatagggtctctctccagtatgaattcttcggtgtcgagtgaggcttgtcttcacacgaaaagttttcctacaatcactacaaacatacggtttctcccctgtatgaattctctgatgtacaatgagggtagatctcttagaaaaggttttcctacattcattacattcatttggtttcctttcagtctgtctccccttttgtgtaatgagaattgccctcttgaagaaggttttcccacatttattatagtcaaacggttgtttcaaaatctgaatgttctggtgcagaataagattttcgttttgattgctggctttcctcattggattgtatctgtattttttcattcccaaatgacttttctcatgcttcccaaatccactgtatccatcaggaatctttctgttttctttgcttttctttgcaacaattacttctgaattagttttcaaactgtttcctcctggattacatttatagggcatttttcttgagggaacactattcatgcccagattaagtgttttcccaaatacattctctctttctgtaatcagtgttttgttgctgaagaatacagtttgtgtcaaatgtttatcttggatttccttgttcttctctaaggcatcatcaatgtctgggtagttctgatttgagaattcctccactatccatggctcttctccttgctccaatttgaaaatcacatctggtttgctaacatgataccccacagagaccaagttgctgtagttctccagcatcacatccctgtacaggagcctctgagcagggtccagttgctgccattcctcttgggtgaagttcacagtcaggtcctggaatgaaactggtatctccttctcattttccatttcccttcattcaaggttcacccacggtgagttaacttgcgcacacttccaggttgcatcatctggctccaccatctggcccctcaggaagctggtaccacacctcatggtgtgtggtttcatccaagtctaaaacaggaggcagcctggtgtgggtgggtggcattaactgaaattttttcattttcatgttctcttgagaaagggccaagagtgttgaaagcagagctgggtaaggaagaatggcgaatggaatcatgagcgatttggctcacacagcagctctacaattacctacaaagccacacacccatttaaaaacatggccctttgaccagtctggttcaggaagcaacatgttgaggaaacgttcacttgtccatttatagttctagaatggtctcatagagcttttcttactgagtgagtgtcaacaaatgttttctactgaattactgtcaatctatgcctcctttgaaaaaaattgaaaacgtctgagtccaattaataggagactaggtcaacgaaagttagtatatacaaagcctggaacactattttggcattaaaatggactctaggattaaaagatttcttggaataggaaaatgatattatgtcacttacctgttttcctactaatgtgtttagccacttgagatgacagaatccagagagaatgaatgaaagtgctttaaggtgtttgtctttttgacagtttggtttcccttagctgcagtttcacaagaggaccttttactaagaaacttcttgtggtaggtaacgtaaatgtggtagatgacaaaagccctgacctggtactcaaaggaccagaattcagttattggatctgtcactagcaaactgcattactgaaaaaaatatttactaagtcgtaattttaatataagataaattggtttttagtctttcctttacccctatcgtgtagctctgtaaggggtaaactcagtaaatcccaggtgaggtgatgaacatggttggtgcagctctgaataaacagagggtggagatggtagggaatgacatgtatgtgtttaggaagtgatgaagacatcatttccttatttataaccagtactccttccctccaacccaggactctcgcagatacctccagtgaagtgtcttttcctgtcaaatcttgaccctgcccattccagctcacatccttcttccgaaagttgaactgaactttgctgagctataataatcaatggctgcaagactaagtgcatcagcagaagttctggaaagaggttctagctacttggatgcgtaaacctttcaccttcaccaagcgccttcttcgggcaaatcagggccctagagagagctcgcccgtggcctgcaggtcaggagcccaatcctgccctggctgcctcgcctcccgaccacaggaaaccctccctccaaagacagggagagcgcgcgtccaccctccgcagacccgaggcccgctccgcccgg

SEQ ID NO: 8590 - RNA, 9959 nt, Homo sapiens
  source 1..9959: mol_type = other RNA
aaagactctgcaagatgccttgaagtctttttgctcaaattctccctttgcatgttggggctaaagcaaatctgggacaggagagagactggggaggcagtgggtgtggttattgaagaagttaatgtgggtaacaccagagatcctggaggtgatgacagtgttctgtaacatgacaatggtggtgaatactagaacctacatgtgataaaactgtatagaattaacacacacatacaaatgaagtaaagctaaggaaatatgaataagatcggagaattttatcaacctcaatatcctggttttgatattgtactatcattttgcaagatgttaccattaggcaaaactgggtaaagggtatatgagggctctattttttcttgcaactgcatgtcaacctacaattatctcaatacaaatgtcaattatacaaaatagaagttagatttaatgtctttcttttttatatgtgcagtctcaggttatacctgcagaaccatatacttgtattatgctgctgacaaaaaagtgtgaaagaacccaatgccttcattttaaagatgagtcacataaaggttaggcgactatccaagctgataaagcttgtttatattaagcatttatcatggtttctgcctttccataagttataatgatggagaattttatggcaatgttaagacgtccagtcctgggttcagacaactttgggatatatcctatcaggattcaaacggtctcaccatgtgatcttagaaaaataatgtttgcattttctactcattgaaatgagataataaaataatcccatacaccgatgggatttcaagatactgaaataaaataattcatgctggtacagtggatgcgtgataggagactctcaaaataatgcctgttttccggcatattaagtgctggacactagagctaaaggctttgaatacaaagagataaaaggtacagcttctgcttccataaacagagtctaggagagagaataacacaaagataattgcacagattaaaatgtgaaaaataggagagtacagggaattggtggttgatgaggctggataagtaaatgcagcaggtgaggaaggcacctttttaggaatccacactttggctaggtttatgtcatcaaagagcctaacagcctgtttttttgttttttggtttttttttttcacgtgacaggatcttgctttattgcccaggctggagtgcagtgatgtgatcatagctcactgctgcctcaaatggtggggctcaagtgatcttctcacctcagcctcccaagtagcctggactataggcacatgccaccatacctggaattttaaaagtgtttgtagagacaaggtcttgctatgttgcccaggatggtctcagacttctggcctcaggaaatcctcctgcctcagccctgtaaagtgctaggattacaggtatgagccgccatggctggccgagagcctggtcttttagagttagatggatttgaggatggagctcagtgctatccctcaccagctgtgttactgtgggcaaaattgcttatttttctaatcctcccttttctcaaccccaaaataagaagattgcaatagaataattccctctagggtggctgtgtcagttaatgagatcatgaatatggacatgcttagcactcagtatcttcctgcagcttgctaaaatagccacagtgtatgcaaaaatgtaaatatctttcggtataactgggctacaaatgatggtagaaaacataatcataccactccaaggtcatttcacatcttcatgtttaaaacagactattctgaaatagtcatttgattgagaaattaaattatctgatttcaacattcacatgtgctctctggtacattctctcctctcaagcactctctctccctttcctctgattttgtctcagaattatagttgtcaatgaaaagagtcaaaccctgtaaaacatttgaagagatttattctgagccaaatatgagtgaccaatggcccacaacacagccttcaggagatcccaaacacatgtgcctaaggtggtcaggctacaacttggttttatacattttagggacacaaaagacattaatcagtacaaaaaagatgtacactggttcagtctggaaaggtgggacaactggaaggcaagggcttccaggtcataagcagattcaaatactttctgactggcaattggttgaaaggattaagttattacctaaagacttagaatcaatggaaaggaacgtctgggctaaggggttgtgaagaccaagtttttatcatgcaggcaaagtctccaggtagctggctttagagagaatacattataaattattcttatcagacttagagagtctgttctctcagtaatttcaaaagggaggagggtataatgaggcatgtccgaccccacttcccatcatggcctgaactagtttttcaggttaacttcggaatttactttgctgagaggagaggtccattgcagtggttggagggcttagaattttatttttggtttacatagtctttgtgcaggggaacacttaacaaaaaatgaaggagcaagggaatatgtgtcaggtctgggtgctggtggctgggccctgctggcttctgtaggggcatttcaccccgttgggtctttggtttaggcttcagtcctgctgcatcccctgctggggtcatttggtccccctggcctttggatgcaagtgagcatctgggcccactgtcctcctacaaggcctctggtccagatgtcctcaccctgtgctcacctcaccccatccctggccaccctcagtctctggccctctgtatcagttatttattgctgctggaacaaatgcctgcaaacttagtggctcaaaataaaaacttttcttagaggtctggaggttagaagtccaaagcaggtctcatggggctaaaatcaaggtgctggagagactgtgctctttctgaaggctctaggggggaacctgtctccttgccttttcttgcttctggaggctcctacctgtcttttattatctgattttcttgcctccctcttttaaggacccttttgattatatcagacccacccggataatccaggataattgtcccaactcaggattctgtaagccaaaacaaaaatcccaggccccccaacagactgaacagagccaagagaaacctgaaaaatgaaattcacaatcatcatgggaagggaggttggacacacctcgttataccctctcccttttggagttcagcacaactgaccagcattaacactaaaatagagatcacaagactgacaaaacagactctgtggcaataagagatcaaattccatcctgactctagtgtagcatcacatgacagatatcagaccctgaaggaaatcaaagtattttaccccaaaatacatttctctgacactttgaaatggccctgcaaagctgtcttgtgtggggaaaattctacatctgtagagaacctccattaatgcagcccagtctttctgggatctaggagagattaactaagagtctgacacctttaaggtatgaaaagacacatttaccatctattcccactgaagcctgctacctggaggcttcatctacataataagaaccttggcttccacaactctccccacccgcttaccttaaccaaagcatttctttctactgatttcaaatagtttaactctttcaaacaattgccaatcagataatttttgaatccatctatgacctgtaagctcccccactctttgagatgtctcacctttccaggccaaatcaatatattccttacatgtattgatctatgtctttgcctgtaacttgtctccctaaactatataaaaccaaactgtaatctgacctccttgggcaccctttctcaggaccccctgaggctcttcctggagccatggtcactcatattggcttagaataaactcctttaaatattttacagagtttgggttttttgttcacaattattaatcacacatttgccaagtaaggtcacatactcacaggttctgggggttaggatgtggacatgtttggggggcaattgttctgctttccataccctcctatcattcccaacccctttctgggacaagcagcacacactggattcccccatgtcactgatgggccatgggaaagtggagatgctactttacgccgtcccgctgctgaaagcgccaaactgcctctcctcctccatgcagctgcctcatgggggtgggaggcaccaggtgaggccccttatctcagagattgaagtggaaagagtggcacaaacctatctgggtgtgtgttatatgacatcattcctggggtacataggaggcatgaataaagagcactggggaattttcagcctaagccttgatgtgacaatcctgcattccccaatccttcctgttcccactataatcaggaccaaaagagctgaatcctgcaggtagtgagctgggcttgattaggaaatgagaaggttctgggtgtgatgatctaagttccatataggtaggctcagatgcatgctgggcttgctagctgtatcggagttgatctttctgagaaggtgagttcaagctctgtttcactgggtggcagggaaagttttgttcaaggcagaaatggaaagtagagtctcacactttgacacatagggagagaccccagtatccaaaatcccagctgctgcagcatacccgtgggctctcttgagggcccaggaggagaaagaacctgaaagccaaggttggtacgctgttatggattcctggtttcctctgtgtgtgtggttgggggtaggggttggagtacctgttctcacatgcttctgtcctcaattttaaggtgtggcttctcaggagtctgtgttccctgagaacaggaggtgaagaatgaaaaggaaaatggctcggtcatttctagaggtgatatcacaggtgaactgcttacttctgatttccttcctaaaataccaatttacagggctaaagacattttgcatttgttccacaaggatgcagctccccattctggtgatgaggtgacagtcagagaggcaacagaggggacctaaataacccagaagctttctttagtgacccaagatttagtattcattcaacaaactgctcaaggtctgacccaagatttagtattcattcaacaaactgctcaacgactgacccaagatttaggattcattcaacaaactactcaaggactgactgaccaagaggagtcattagcacaggtcttctaggcatgaatttgtttgaaaacttttaagctgaagaataggagtccctggggatagtgagttcagtttgaagttggacagcttgcatgtgttggcagcgcagggagcaatggcttaacttgctctcaaatctatgggagagctggagcagggcacaggcagtcaggtggatgggatgaaggtggagggatgccaccatatttctgggtaacaaaagggcactcgtcctgacagacttaaaatccaacacatcaaactatgctaattaaaataatatagaaatgataatacgttgatgggtaaacagaagaaaatagaaggccagatacacattgtggtagaatgaacaatctcccccacccattgcaaaatgtccccatcctagtccctggaagctgtgaatgtgttaccttacatggtaaaagggactttgcaggtgtcattaagttgaggatcttcagatggggggtttctcctgggttgtctgggtgggcctgaaatgtaatcactgggtctcttgcgtctttgggtaaggaaggtcttgttagttcacaactgcccatgggagaattttctccttctgtgcaaatatctgcaacactccctgaaaatgccagttgaattttctaacttcatattcttcagtaaagcatcgtagctcatctagttggaaagagacgactaccttcattaacagaaggtagaactcgccagaatgtaagatgatccagagatttcagagaaacttgtttctcgagtttcagtgctgacatcagggaaggcagctcattcataggctccctttgctaaactcgagatcaatgtagaaagaatcttagtcgaagcctaattcttcgtggattcatgctgtatggagtatcttggaaatataaatatgtaaatgttgaagaaatggagatgtgatcagaaatgtactttttttattgcactgacttgaatctttggccaaggcaggtggttcatgaggtcaagagttccagaccagcctggtcaacatagtgaaaccccatctctcctgctggttcttgttggcatggctcagtagatgagcctgtggctgctctcctttccccaggatctcctccagctctttcagctcctgggctaggtgtgtgcttagcaacaccacaaatggcaccaacctctgtaggacacccacatcgtttaggtagaagacagtaaaaactgccacagctttgtctgtgggttccagcttgtctttattctcttagtgttcactttcactacttgcttggcagtttagcattgtgtaagttatttgatttgttgctttgttggaatttattactttgttggaacttattccttgtgggatttctgatgtaaaagaaagtttgatttgtggcgaaatgttttctcacatttgttacattcataaggtttctctcctgtgtgtattttctgatgttcagtgagagtccacaggcgacggtaggttttcccacattgattacattcatatggtttctctcctgtgtgaattcttctatggactctgaaggctgacttatggcagaaggatttcccacattcattacattcatatggtttctccccagtgtgagttcgctgatgttcaacaaaggagaacttctgacagaaggttttcccacattcattacactcatagggtctctgtcctgtgtgtgttctctgatggtgagtcagggctgacttcctgcagtaggttctcccacattcattgcattcatatggtctctcccatatagttctctgatgtacaatgaggtgtgagtttttgctgacggcatgcccatgttcactacactcataaagattctcctttgtgttcattctcttacactgactgcagtttgacttcacaatggagattctaccacatttattaaacacaccatgtttctctcctgtgtgtgttctctgatgtatagtgagtgttgacttatggcagaaaaatttcccacattcattacattcataagacttctttcctctatgagttatctgatgtgcaatgagggctgatttcgtacataaaaattttccacattgactgcattcatagggcttctctcctgtatgacttcttcgatgcacattgagggcagattgacaaaagaaggttttctcacattcactacattcatagggtttttcccctgtgtgaattctctgatgcgcagtaagggctgactgacagaagaaggttttcccacattccttacattcatttggcttctctcctctgtgagttctttgatgtacaacaagatacgatttcttgctgaaggcatttccacattccttgcattcgtaaggcttctcccctgtgtgtgacctgaaatgttcagccagggctgacttccgaaaaaaggtctttccacattcattacactcataggatttctcccctccatgaattttctggtgtacaataagggcagatttgtcaatgaaggttttcctgcattcactgcattcatagggtctctctccagtatgaattcttcggtgtcgagtgaggcttgtcttcacacgaaaagttttcctacaatcactacaaacatacggtttctcccctgtatgaattctctgatgtacaatgagggtagatctcttagaaaaggttttcctacattcattacattcatttggtttcctttcagtctgtctccccttttgtgtaatgagaattgccctcttgaagaaggttttcccacatttattatagtcaaacggttgtttcaaaatctgaatgttctggtgcagaataagattttcgttttgattgctggctttcctcattggattgtatctgtattttttcattcccaaatgacttttctcatgcttcccaaatccactgtatccatcaggaatctttctgttttctttgcttttctttgcaacaattacttctgaattagttttcaaactgtttcctcctggattacatttatagggcatttttcttgagggaacactattcatgcccagattaagtgttttcccaaatacattctctctttctgtaatcagtgttttgttgctgaagaatacagtttgtgtcaaatgtttatcttggatttccttgttcttctctaaggcatcatcaatgtctgggtagttctgatttgagaattcctccactatccatggctcttctccttgctccaatttgaaaatcacatctggtttgctaacatgataccccacagagaccaagttgctgtagttctccagcatcacatccctgtacaggagcctctgagcagggtccagttgctgccattcctcttgggtgaagttcacagtcaggtcctggaatgaaactggtatctccttctcattttccatttcccttcattcaaggttcacccacggtgagttaacttgcgcacacttccaggttgcatcatctggctccaccatctggcccctcaggaagctggtaccacacctcatggtgtgtggtttcatccaagtctaaaacaggaggcagcctggtgtgggtgggtggcattaactgaaattttttcattttcatgttctcttgagaaagggccaagagtgttgaaagcagagctgttttcctactaatgtgtttagccacttgagatgacagaatccagagagaatgaatgaaagtgctttaaggtgtttgtctttttgacagtttggtttcccttagctgcagtttcacaagaggaccttttactaagaaacttcttgtggtaggtaacgtaaatgtggtagatgacaaaagccctgacctggtactcaaaggaccagaattcagttattggatctgtcactagcaaactgcattactgaaaaaaatatttactaagtcgtaattttaatataagataaattggtttttagtctttcctttacccctatcgtgtagctctgtaaggggtaaactcagtaaatcccaggtgaggtgatgaacatggttggtgcagctctgaataaacagagggtggagatggtagggaatgacatgtatgtgtttaggaagtgatgaagacatcatttccttatttataaccagtactccttccctccaacccaggactctcgcagatacctccagtgaagtgtcttttcctgtcaaatcttgaccctgcccattccagctcacatccttcttccgaaagttgaactgaactttgctgagctataataatcaatggctgcaagactaagtgcatcagcagaagttctggaaagaggttctagctacttggatgcgtaaacctttcaccttcaccaagcgccttcttcgggcaaatcagggccctagagagagctcgcccgtggcctgcaggtcaggagcccaatcctgccctggctgcctcgcctcccgaccacaggaaaccctccctccaaagacagggagagcgcgcgtccaccctccgcagacccgaggcccgctccgcccggccccaccgttccctccgacgcccgagtgctcagagctcgccgccagcccttcctataggttgtgggtgcacccgcttcgcctccagttcgcaccaggtccaagtctcggcgggaccagggattcacgggctgcaggaccctcacccggaaga

SEQ ID NO: 8591 - RNA, 9053 nt, Homo sapiens
  source 1..9053: mol_type = other RNA
aaagactctgcaagatgccttgaagtctttttgctcaaattctccctttgcatgttggggctaaagcaaatctgggacaggagagagactggggaggcagtgggtgtggttattgaagaagttaatgtgggtaacaccagagatcctggaggtgatgacagtgttctgtaacatgacaatggtggtgaatactagaacctacatgtgataaaactgtatagaattaacacacacatacaaatgaagtaaagctaaggaaatatgaataagatcggagaattttatcaacctcaatatcctggttttgatattgtactatcattttgcaagatgttaccattaggcaaaactgggtaaagggtatatgagggctctattttttcttgcaactgcatgtcaacctacaattatctcaatacaaatgtcaattatacaaaatagaagttagatttaatgtctttcttttttatatgtgcagtctcaggttatacctgcagaaccatatacttgtattatgctgctgacaaaaaagtgtgaaagaacccaatgccttcattttaaagatgagtcacataaaggttaggcgactatccaagctgataaagcttgtttatattaagcatttatcatggtttctgcctttccataagttataatgatggagaattttatggcaatgttaagacgtccagtcctgggttcagacaactttgggatatatcctatcaggattcaaacggtctcaccatgtgatcttagaaaaataatgtttgcattttctactcattgaaatgagataataaaataatcccatacaccgatgggatttcaagatactgaaataaaataattcatgctggtacagtggatgcgtgataggagactctcaaaataatgcctgttttccggcatattaagtgctggacactagagctaaaggctttgaatacaaagagataaaaggtacagcttctgcttccataaacagagtctaggagagagaataacacaaagataattgcacagattaaaatgtgaaaaataggagagtacagggaattggtggttgatgaggctggataagtaaatgcagcaggtgaggaaggcacctttttaggaatccacactttggctaggtttatgtcatcaaagagcctaacagcctgtttttttgttttttggtttttttttttcacgtgacaggatcttgctttattgcccaggctggagtgcagtgatgtgatcatagctcactgctgcctcaaatggtggggctcaagtgatcttctcacctcagcctcccaagtagcctggactataggcacatgccaccatacctggaattttaaaagtgtttgtagagacaaggtcttgctatgttgcccaggatggtctcagacttctggcctcaggaaatcctcctgcctcagccctgtaaagtgctaggattacaggtatgagccgccatggctggccgagagcctggtcttttagagttagatggatttgaggatggagctcagtgctatccctcaccagctgtgttactgtgggcaaaattgcttatttttctaatcctcccttttctcaaccccaaaataagaagattgcaatagaataattccctctagggtggctgtgtcagttaatgagatcatgaatatggacatgcttagcactcagtatcttcctgcagcttgctaaaatagccacagtgtatgcaaaaatgtaaatatctttcggtataactgggctacaaatgatggtagaaaacataatcataccactccaaggtcatttcacatcttcatgtttaaaacagactattctgaaatagtcatttgattgagaaattaaattatctgatttcaacattcacatgtgctctctggtacattctctcctctcaagcactctctctccctttcctctgattttgtctcagaattatagttgtcaatgaaaagagtcaaaccctgtaaaacatttgaagagatttattctgagccaaatatgagtgaccaatggcccacaacacagccttcaggagatcccaaacacatgtgcctaaggtggtcaggctacaacttggttttatacattttagggacacaaaagacattaatcagtacaaaaaagatgtacactggttcagtctggaaaggtgggacaactggaaggcaagggcttccaggtcataagcagattcaaatactttctgactggcaattggttgaaaggattaagttattacctaaagacttagaatcaatggaaaggaacgtctgggctaaggggttgtgaagaccaagtttttatcatgcaggcaaagtctccaggtagctggctttagagagaatacattataaattattcttatcagacttagagagtctgttctctcagtaatttcaaaagggaggagggtataatgaggcatgtccgaccccacttcccatcatggcctgaactagtttttcaggttaacttcggaatttactttgctgagaggagaggtccattgcagtggttggagggcttagaattttatttttggtttacatagtctttgtgcaggggaacacttaacaaaaaatgaaggagcaagggaatatgtgtcaggtctgggtgctggtggctgggccctgctggcttctgtaggggcatttcaccccgttgggtctttggtttaggcttcagtcctgctgcatcccctgctggggtcatttggtccccctggcctttggatgcaagtgagcatctgggcccactgtcctcctacaaggcctctggtccagatgtcctcaccctgtgctcacctcaccccatccctggccaccctcagtctctggccctctgtatcagttatttattgctgctggaacaaatgcctgcaaacttagtggctcaaaataaaaacttttcttagaggtctggaggttagaagtccaaagcaggtctcatggggctaaaatcaaggtgctggagagactgtgctctttctgaaggctctaggggggaacctgtctccttgccttttcttgcttctggaggctcctacctgtcttttattatctgattttcttgcctccctcttttaaggacccttttgattatatcagacccacccggataatccaggataattgtcccaactcaggattctgtaagccaaaacaaaaatcccaggccccccaacagactgaacagagccaagagaaacctgaaaaatgaaattcacaatcatcatgggaagggaggttggacacacctcgttataccctctcccttttggagttcagcacaactgaccagcattaacactaaaatagagatcacaagactgacaaaacagactctgtggcaataagagatcaaattccatcctgactctagtgtagcatcacatgacagatatcagaccctgaaggaaatcaaagtattttaccccaaaatacatttctctgacactttgaaatggccctgcaaagctgtcttgtgtggggaaaattctacatctgtagagaacctccattaatgcagcccagtctttctgggatctaggagagattaactaagagtctgacacctttaaggtatgaaaagacacatttaccatctattcccactgaagcctgctacctggaggcttcatctacataataagaaccttggcttccacaactctccccacccgcttaccttaaccaaagcatttctttctactgatttcaaatagtttaactctttcaaacaattgccaatcagataatttttgaatccatctatgacctgtaagctcccccactctttgagatgtctcacctttccaggccaaatcaatatattccttacatgtattgatctatgtctttgcctgtaacttgtctccctaaactatataaaaccaaactgtaatctgacctccttgggcaccctttctcaggaccccctgaggctcttcctggagccatggtcactcatattggcttagaataaactcctttaaatattttacagagtttgggttttttgttcacaattattaatcacacatttgccaagtaaggtcacatactcacaggttctgggggttaggatgtggacatgtttggggggcaattgttctgctttccataccctcctatcattcccaacccctttctgggacaagcagcacacactggattcccccatgtcactgatgggccatgggaaagtggagatgctactttacgccgtcccgctgctgaaagcgccaaactgcctctcctcctccatgcagctgcctcatgggggtgggaggcaccaggtgaggccccttatctcagagattgaagtggaaagagtggcacaaacctatctgggtgtgtgttatatgacatcattcctggggtacataggaggcatgaataaagagcactggggaattttcagcctaagccttgatgtgacaatcctgcattccccaatccttcctgttcccactataatcaggaccaaaagagctgaatcctgcaggtagtgagctgggcttgattaggaaatgagaaggttctgggtgtgatgatctaagttccatataggtaggctcagatgcatgctgggcttgctagctgtatcggagttgatctttctgagaaggtgagttcaagctctgtttcactgggtggcagggaaagttttgttcaaggcagaaatggaaagtagagtctcacactttgacacatagggagagaccccagtatccaaaatcccagctgctgcagcatacccgtgggctctcttgagggcccaggaggagaaagaacctgaaagccaaggttggtacgctgttatggattcctggtttcctctgtgtgtgtggttgggggtaggggttggagtacctgttctcacatgcttctgtcctcaattttaaggtgtggcttctcaggagtctgtgttccctgagaacaggaggtgaagaatgaaaaggaaaatggctcggtcatttctagaggtgatatcacaggtgaactgcttacttctgatttccttcctaaaataccaatttacagggctaaagacattttgcatttgttccacaaggatgcagctccccattctggtgatgaggtgacagtcagagaggcaacagaggggacctaaataacccagaagctttctttagtgacccaagatttagtattcattcaacaaactgctcaaggtctgacccaagatttagtattcattcaacaaactgctcaacgactgacccaagatttaggattcattcaacaaactactcaaggactgactgaccaagaggagtcattagcacaggtcttctaggcatgaatttgtttgaaaacttttaagctgaagaataggagtccctggggatagtgagttcagtttgaagttggacagcttgcatgtgttggcagcgcagggagcaatggcttaacttgctctcaaatctatgggagagctggagcagggcacaggcagtcaggtggatgggatgaaggtggagggatgccaccatatttctgggtaacaaaagggcactcgtcctgacagacttaaaatccaacacatcaaactatgctaattaaaataatatagaaatgataatacgttgatgggtaaacagaagaaaatagaaggccagatacacattgtggtagaatgaacaatctcccccacccattgcaaaatgtccccatcctagtccctggaagctgtgaatgtgttaccttacatggtaaaagggactttgcaggtgtcattaagttgaggatcttcagatggggggtttctcctgggttgtctgggtgggcctgaaatgtaatcactgggtctcttgcgtctttgggtaaggaaggtcttgttagttcacaactgcccatgggagaattttctccttctgtgcaaatatctgcaacactccctgaaaatgccagttgaattttctaacttcatattcttcagtaaagcatcgtagctcatctagttggaaagagacgactaccttcattaacagaaggtagaactcgccagaatgtaagatgatccagagatttcagagaaacttgtttctcgagtttcagtgctgacatcagggaaggcagctcattcataggctccctttgctaaactcgagatcaatgtagaaagaatcttagtcgaagcctaattcttcgtggattcatgctgtatggagtatcttggaaatataaatatgtaaatgttgaagaaatggagatgtgatcagaaatgtactttttttattgcactgacttgaatctttggccaaggcaggtggttcatgaggtcaagagttccagaccagcctggtcaacatagtgaaaccccatctctcctgctggttcttgttggcatggctcagtagatgagcctgtggctgctctcctttccccaggatctcctccagctctttcagctcctgggctaggtgtgtgcttagcaacaccacaaatggcaccaacctctgtaggacacccacatcgtttaggtagaagacagtaaaaactgccacagctttgtctgtgggttccagcttgtctttattctcttagtgttcactttcactacttgcttggcagtttagcattgtgtaagttatttgatttgttgctttgttggaatttattactttgttggaacttattccttgtgggatttctgatgtaaaagaaagtttgatttgtggcgaaatgttttctcacatttgttacattcataaggtttctctcctgtgtgtattttctgatgttcagtgagagtccacaggcgacggtaggttttcccacattgattacattcatatggtttctctcctgtgtgaattcttctatggactctgaaggctgacttatggcagaaggatttcccacattcattacattcatatggtttctccccagtgtgagttcgctgatgttcaacaaaggagaacttctgacagaaggttttcccacattcattacactcatagggtctctgtcctgtgtgtgttctctgatggtgagtcagggctgacttcctgcagtaggttctcccacattcattgcattcatatggtctctcccatatagttctctgatgtacaatgaggtgtgagtttttgctgacggcatgcccatgttcactacactcataaagattctcctttgtgttcattctcttacactgactgcagtttgacttcacaatggagattctaccacatttattaaacacaccatgtttctctcctgtgtgtgttctctgatgtatagtgagtgttgacttatggcagaaaaatttcccacattcattacattcataagacttctttcctctatgagttatctgatgtgcaatgagggctgatttcgtacataaaaattttccacattgactgcattcatagggcttctctcctgtatgacttcttcgatgcacattgagggcagattgacaaaagaaggttttctcacattcactacattcatagggtttttcccctgtgtgaattctctgatgcgcagtaagggctgactgacagaagaaggttttcccacattccttacattcatttggcttctctcctctgtgagttctttgatgtacaacaagatacgatttcttgctgaaggcatttccacattccttgcattcgtaaggcttctcccctgtgtgtgacctgaaatgttcagccagggctgacttccgaaaaaaggtctttccacattcattacactcataggatttctcccctccatgaattttctggtgtacaataagggcagatttgtcaatgaaggttttcctgcattcactgcattcatagggtctctctccagtatgaattcttcggtgtcgagtgaggcttgtcttcacacgaaaagttttcctacaatcactacaaacatacggtttctcccctgtatgaattctctgatgtacaatgagggtagatctcttagaaaaggttttcctacattcattacattcatttggtttcctttcagtctgtctccccttttgtgtaatgagaattgccctcttgaagaaggttttcccacatttattatagtcaaacggttgtttcaaaatctgaatgttctggtgcagaataagattttcgttttgattgctggctttcctcattggattgtatctgtattttttcattcccaaatgacttttctcatgcttcccaaatccactgtatccatcaggaatctttctgttttctttgcttttctttgcaacaattacttctgaattagttttcaaactgtttcctcctggattacatttatagggcatttttcttgagggaacactattcatgcccagattaagtgttttcccaaatacattctctctttctgtaatcagtgttttgttgctgaagaatacagtttgtgtcaaatgtttatcttggatttccttgttcttctctaaggcatcatcaatgtctgggtagttctgatttgagaattcctccactatccatggctcttctccttgctccaatttgaaaatcacatctggtttgctaacatgataccccacagagaccaagttgctgtagttctccagcatcacatccctgtacaggagcctctgagcagggtccagttgctgccattcctcttgggtgaagttcacagtcaggtcctggaatgaaactggtatctccttctcattttccatttcccttcattcaaggttcacccacggtgagttaacttgcgcacacttccaggttgcatcatctggctccaccatctggcccctcaggaagctggtaccacacctcatggtgtgtggtttcatccaagtctgaaattttttcattttcatgttctcttgagaaagggccaagagtgttgaaagcagagcgttccctccgacgcccgagtgctcagagctcgccgccagcccttcctataggttgtgggtgcacccgcttcgcctccagttcgcaccaggtccaagtctcggcgggaccagggattcacgggctgcaggaccctcacccggaagagcct

SEQ ID NO: 8592 - RNA, 8819 nt, Homo sapiens
  source 1..8819: mol_type = other RNA
aaagactctgcaagatgccttgaagtctttttgctcaaattctccctttgcatgttggggctaaagcaaatctgggacaggagagagactggggaggcagtgggtgtggttattgaagaagttaatgtgggtaacaccagagatcctggaggtgatgacagtgttctgtaacatgacaatggtggtgaatactagaacctacatgtgataaaactgtatagaattaacacacacatacaaatgaagtaaagctaaggaaatatgaataagatcggagaattttatcaacctcaatatcctggttttgatattgtactatcattttgcaagatgttaccattaggcaaaactgggtaaagggtatatgagggctctattttttcttgcaactgcatgtcaacctacaattatctcaatacaaatgtcaattatacaaaatagaagttagatttaatgtctttcttttttatatgtgcagtctcaggttatacctgcagaaccatatacttgtattatgctgctgacaaaaaagtgtgaaagaacccaatgccttcattttaaagatgagtcacataaaggttaggcgactatccaagctgataaagcttgtttatattaagcatttatcatggtttctgcctttccataagttataatgatggagaattttatggcaatgttaagacgtccagtcctgggttcagacaactttgggatatatcctatcaggattcaaacggtctcaccatgtgatcttagaaaaataatgtttgcattttctactcattgaaatgagataataaaataatcccatacaccgatgggatttcaagatactgaaataaaataattcatgctggtacagtggatgcgtgataggagactctcaaaataatgcctgttttccggcatattaagtgctggacactagagctaaaggctttgaatacaaagagataaaaggtacagcttctgcttccataaacagagtctaggagagagaataacacaaagataattgcacagattaaaatgtgaaaaataggagagtacagggaattggtggttgatgaggctggataagtaaatgcagcaggtgaggaaggcacctttttaggaatccacactttggctaggtttatgtcatcaaagagcctaacagcctgtttttttgttttttggtttttttttttcacgtgacaggatcttgctttattgcccaggctggagtgcagtgatgtgatcatagctcactgctgcctcaaatggtggggctcaagtgatcttctcacctcagcctcccaagtagcctggactataggcacatgccaccatacctggaattttaaaagtgtttgtagagacaaggtcttgctatgttgcccaggatggtctcagacttctggcctcaggaaatcctcctgcctcagccctgtaaagtgctaggattacaggtatgagccgccatggctggccgagagcctggtcttttagagttagatggatttgaggatggagctcagtgctatccctcaccagctgtgttactgtgggcaaaattgcttatttttctaatcctcccttttctcaaccccaaaataagaagattgcaatagaataattccctctagggtggctgtgtcagttaatgagatcatgaatatggacatgcttagcactcagtatcttcctgcagcttgctaaaatagccacagtgtatgcaaaaatgtaaatatctttcggtataactgggctacaaatgatggtagaaaacataatcataccactccaaggtcatttcacatcttcatgtttaaaacagactattctgaaatagtcatttgattgagaaattaaattatctgatttcaacattcacatgtgctctctggtacattctctcctctcaagcactctctctccctttcctctgattttgtctcagaattatagttgtcaatgaaaagagtcaaaccctgtaaaacatttgaagagatttattctgagccaaatatgagtgaccaatggcccacaacacagccttcaggagatcccaaacacatgtgcctaaggtggtcaggctacaacttggttttatacattttagggacacaaaagacattaatcagtacaaaaaagatgtacactggttcagtctggaaaggtgggacaactggaaggcaagggcttccaggtcataagcagattcaaatactttctgactggcaattggttgaaaggattaagttattacctaaagacttagaatcaatggaaaggaacgtctgggctaaggggttgtgaagaccaagtttttatcatgcaggcaaagtctccaggtagctggctttagagagaatacattataaattattcttatcagacttagagagtctgttctctcagtaatttcaaaagggaggagggtataatgaggcatgtccgaccccacttcccatcatggcctgaactagtttttcaggttaacttcggaatttactttgctgagaggagaggtccattgcagtggttggagggcttagaattttatttttggtttacatagtctttgtgcaggggaacacttaacaaaaaatgaaggagcaagggaatatgtgtcaggtctgggtgctggtggctgggccctgctggcttctgtaggggcatttcaccccgttgggtctttggtttaggcttcagtcctgctgcatcccctgctggggtcatttggtccccctggcctttggatgcaagtgagcatctgggcccactgtcctcctacaaggcctctggtccagatgtcctcaccctgtgctcacctcaccccatccctggccaccctcagtctctggccctctgtatcagttatttattgctgctggaacaaatgcctgcaaacttagtggctcaaaataaaaacttttcttagaggtctggaggttagaagtccaaagcaggtctcatggggctaaaatcaaggtgctggagagactgtgctctttctgaaggctctaggggggaacctgtctccttgccttttcttgcttctggaggctcctacctgtcttttattatctgattttcttgcctccctcttttaaggacccttttgattatatcagacccacccggataatccaggataattgtcccaactcaggattctgtaagccaaaacaaaaatcccaggccccccaacagactgaacagagccaagagaaacctgaaaaatgaaattcacaatcatcatgggaagggaggttggacacacctcgttataccctctcccttttggagttcagcacaactgaccagcattaacactaaaatagagatcacaagactgacaaaacagactctgtggcaataagagatcaaattccatcctgactctagtgtagcatcacatgacagatatcagaccctgaaggaaatcaaagtattttaccccaaaatacatttctctgacactttgaaatggccctgcaaagctgtcttgtgtggggaaaattctacatctgtagagaacctccattaatgcagcccagtctttctgggatctaggagagattaactaagagtctgacacctttaaggtatgaaaagacacatttaccatctattcccactgaagcctgctacctggaggcttcatctacataataagaaccttggcttccacaactctccccacccgcttaccttaaccaaagcatttctttctactgatttcaaatagtttaactctttcaaacaattgccaatcagataatttttgaatccatctatgacctgtaagctcccccactctttgagatgtctcacctttccaggccaaatcaatatattccttacatgtattgatctatgtctttgcctgtaacttgtctccctaaactatataaaaccaaactgtaatctgacctccttgggcaccctttctcaggaccccctgaggctcttcctggagccatggtcactcatattggcttagaataaactcctttaaatattttacagagtttgggttttttgttcacaattattaatcacacatttgccaagtaaggtcacatactcacaggttctgggggttaggatgtggacatgtttggggggcaattgttctgctttccataccctcctatcattcccaacccctttctgggacaagcagcacacactggattcccccatgtcactgatgggccatgggaaagtggagatgctactttacgccgtcccgctgctgaaagcgccaaactgcctctcctcctccatgcagctgcctcatgggggtgggaggcaccaggtgaggccccttatctcagagattgaagtggaaagagtggcacaaacctatctgggtgtgtgttatatgacatcattcctggggtacataggaggcatgaataaagagcactggggaattttcagcctaagccttgatgtgacaatcctgcattccccaatccttcctgttcccactataatcaggaccaaaagagctgaatcctgcaggtagtgagctgggcttgattaggaaatgagaaggttctgggtgtgatgatctaagttccatataggtaggctcagatgcatgctgggcttgctagctgtatcggagttgatctttctgagaaggtgagttcaagctctgtttcactgggtggcagggaaagttttgttcaaggcagaaatggaaagtagagtctcacactttgacacatagggagagaccccagtatccaaaatcccagctgctgcagcatacccgtgggctctcttgagggcccaggaggagaaagaacctgaaagccaaggttggtacgctgttatggattcctggtttcctctgtgtgtgtggttgggggtaggggttggagtacctgttctcacatgcttctgtcctcaattttaaggtgtggcttctcaggagtctgtgttccctgagaacaggaggtgaagaatgaaaaggaaaatggctcggtcatttctagaggtgatatcacaggtgaactgcttacttctgatttccttcctaaaataccaatttacagggctaaagacattttgcatttgttccacaaggatgcagctccccattctggtgatgaggtgacagtcagagaggcaacagaggggacctaaataacccagaagctttctttagtgacccaagatttagtattcattcaacaaactgctcaaggtctgacccaagatttagtattcattcaacaaactgctcaacgactgacccaagatttaggattcattcaacaaactactcaaggactgactgaccaagaggagtcattagcacaggtcttctaggcatgaatttgtttgaaaacttttaagctgaagaataggagtccctggggatagtgagttcagtttgaagttggacagcttgcatgtgttggcagcgcagggagcaatggcttaacttgctctcaaatctatgggagagctggagcagggcacaggcagtcaggtggatgggatgaaggtggagggatgccaccatatttctgggtaacaaaagggcactcgtcctgacagacttaaaatccaacacatcaaactatgctaattaaaataatatagaaatgataatacgttgatgggtaaacagaagaaaatagaaggccagatacacattgtggtagaatgaacaatctcccccacccattgcaaaatgtccccatcctagtccctggaagctgtgaatgtgttaccttacatggtaaaagggactttgcaggtgtcattaagttgaggatcttcagatggggggtttctcctgggttgtctgggtgggcctgaaatgtaatcactgggtctcttgcgtctttgggtaaggaaggtcttgttagttcacaactgcccatgggagaattttctccttctgtgcaaatatctgcaacactccctgaaaatgccagttgaattttctaacttcatattcttcagtaaagcatcgtagctcatctagttggaaagagacgactaccttcattaacagaaggtagaactcgccagaatgtaagatgatccagagatttcagagaaacttgtttctcgagtttcagtgctgacatcagggaaggcagctcattcataggctccctttgctaaactcgagatcaatgtagaaagaatcttagtcgaagcctaattcttcgtggattcatgctgtatggagtatcttggaaatataaatatgtaaatgttgaagaaatggagatgtgatcagaaatgtactttttttattgcactgacttgaatctttggccaaggcaggtggttcatgaggtcaagagttccagaccagcctggtcaacatagtgaaaccccatctctcctgctggttcttgttggcatggctcagtagatgagcctgtggctgctctcctttccccaggatctcctccagctctttcagctcctgggctaggtgtgtgcttagcaacaccacaaatggcaccaacctctgtaggacacccacatcgtttaggtagaagacagtaaaaactgccacagctttgtctgtgggttccagcttgtctttattctcttagtgttcactttcactacttgcttggcagtttagcattgtgtaagttatttgatttgttgctttgttggaatttattactttgttggaacttattccttgtgggatttctgatgtaaaagaaagtttgatttgtggcgaaatgttttctcacatttgttacattcataaggtttctctcctgtgtgtattttctgatgttcagtgagagtccacaggcgacggtaggttttcccacattgattacattcatatggtttctctcctgtgtgaattcttctatggactctgaaggctgacttatggcagaaggatttcccacattcattacattcatatggtttctccccagtgtgagttcgctgatgttcaacaaaggagaacttctgacagaaggttttcccacattcattacactcatagggtctctgtcctgtgtgtgttctctgatggtgagtcagggctgacttcctgcagtaggttctcccacattcattgcattcatatggtctctcccatatagttctctgatgtacaatgaggtgtgagtttttgctgacggcatgcccatgttcactacactcataaagattctcctttgtgttcattctcttacactgactgcagtttgacttcacaatggagattctaccacatttattaaacacaccatgtttctctcctgtgtgtgttctctgatgtatagtgagtgttgacttatggcagaaaaatttcccacattcattacattcataagacttctttcctctatgagttatctgatgtgcaatgagggctgatttcgtacataaaaattttccacattgactgcattcatagggcttctctcctgtatgacttcttcgatgcacattgagggcagattgacaaaagaaggttttctcacattcactacattcatagggtttttcccctgtgtgaattctctgatgcgcagtaagggctgactgacagaagaaggttttcccacattccttacattcatttggcttctctcctctgtgagttctttgatgtacaacaagatacgatttcttgctgaaggcatttccacattccttgcattcgtaaggcttctcccctgtgtgtgacctgaaatgttcagccagggctgacttccgaaaaaaggtctttccacattcattacactcataggatttctcccctccatgaattttctggtgtacaataagggcagatttgtcaatgaaggttttcctgcattcactgcattcatagggtctctctccagtatgaattcttcggtgtcgagtgaggcttgtcttcacacgaaaagttttcctacaatcactacaaacatacggtttctcccctgtatgaattctctgatgtacaatgagggtagatctcttagaaaaggttttcctacattcattacattcatttggtttcctttcagtctgtctccccttttgtgtaatgagaattgccctcttgaagaaggttttcccacatttattatagtcaaacggttgtttcaaaatctgaatgttctggtgcagaataagattttcgttttgattgctggctttcctcattggattgtatctgtattttttcattcccaaatgacttttctcatgcttcccaaatccactgtatccatcaggaatctttctgttttctttgcttttctttgcaacaattacttctgaattagttttcaaactgtttcctcctggattacatttatagggcatttttcttgagggaacactattcatgcccagattaagtgttttcccaaatacattctctctttctgtaatcagtgttttgttgctgaagaatacagtttgtgtcaaatgtttatcttggatttccttgttcttctctaaggcatcatcaatgtctgggtagttctgatttgagaattcctccactatccatggctcttctccttgctccaatttgaaaatcacatctggtttgctaacatgataccccacagagaccaagttgctgtagttctccagcatcacatccctgtacaggagcctctgagcagggtccagttgctgccattcctcttgggtgaagttcacagtcaggtcctggaatgaaactggtatctgaaattttttcattttcatgttctcttgagaaagggccaagagtgttgaaagcagagcaggtccaagtctcggcgggaccagggattcacgggctgcaggaccctcacccggaagagcct

SEQ ID NO: 8593 - RNA, 8902 nt, Homo sapiens
  source 1..8902: mol_type = other RNA
aaagactctgcaagatgccttgaagtctttttgctcaaattctccctttgcatgttggggctaaagcaaatctgggacaggagagagactggggaggcagtgggtgtggttattgaagaagttaatgtgggtaacaccagagatcctggaggtgatgacagtgttctgtaacatgacaatggtggtgaatactagaacctacatgtgataaaactgtatagaattaacacacacatacaaatgaagtaaagctaaggaaatatgaataagatcggagaattttatcaacctcaatatcctggttttgatattgtactatcattttgcaagatgttaccattaggcaaaactgggtaaagggtatatgagggctctattttttcttgcaactgcatgtcaacctacaattatctcaatacaaatgtcaattatacaaaatagaagttagatttaatgtctttcttttttatatgtgcagtctcaggttatacctgcagaaccatatacttgtattatgctgctgacaaaaaagtgtgaaagaacccaatgccttcattttaaagatgagtcacataaaggttaggcgactatccaagctgataaagcttgtttatattaagcatttatcatggtttctgcctttccataagttataatgatggagaattttatggcaatgttaagacgtccagtcctgggttcagacaactttgggatatatcctatcaggattcaaacggtctcaccatgtgatcttagaaaaataatgtttgcattttctactcattgaaatgagataataaaataatcccatacaccgatgggatttcaagatactgaaataaaataattcatgctggtacagtggatgcgtgataggagactctcaaaataatgcctgttttccggcatattaagtgctggacactagagctaaaggctttgaatacaaagagataaaaggtacagcttctgcttccataaacagagtctaggagagagaataacacaaagataattgcacagattaaaatgtgaaaaataggagagtacagggaattggtggttgatgaggctggataagtaaatgcagcaggtgaggaaggcacctttttaggaatccacactttggctaggtttatgtcatcaaagagcctaacagcctgtttttttgttttttggtttttttttttcacgtgacaggatcttgctttattgcccaggctggagtgcagtgatgtgatcatagctcactgctgcctcaaatggtggggctcaagtgatcttctcacctcagcctcccaagtagcctggactataggcacatgccaccatacctggaattttaaaagtgtttgtagagacaaggtcttgctatgttgcccaggatggtctcagacttctggcctcaggaaatcctcctgcctcagccctgtaaagtgctaggattacaggtatgagccgccatggctggccgagagcctggtcttttagagttagatggatttgaggatggagctcagtgctatccctcaccagctgtgttactgtgggcaaaattgcttatttttctaatcctcccttttctcaaccccaaaataagaagattgcaatagaataattccctctagggtggctgtgtcagttaatgagatcatgaatatggacatgcttagcactcagtatcttcctgcagcttgctaaaatagccacagtgtatgcaaaaatgtaaatatctttcggtataactgggctacaaatgatggtagaaaacataatcataccactccaaggtcatttcacatcttcatgtttaaaacagactattctgaaatagtcatttgattgagaaattaaattatctgatttcaacattcacatgtgctctctggtacattctctcctctcaagcactctctctccctttcctctgattttgtctcagaattatagttgtcaatgaaaagagtcaaaccctgtaaaacatttgaagagatttattctgagccaaatatgagtgaccaatggcccacaacacagccttcaggagatcccaaacacatgtgcctaaggtggtcaggctacaacttggttttatacattttagggacacaaaagacattaatcagtacaaaaaagatgtacactggttcagtctggaaaggtgggacaactggaaggcaagggcttccaggtcataagcagattcaaatactttctgactggcaattggttgaaaggattaagttattacctaaagacttagaatcaatggaaaggaacgtctgggctaaggggttgtgaagaccaagtttttatcatgcaggcaaagtctccaggtagctggctttagagagaatacattataaattattcttatcagacttagagagtctgttctctcagtaatttcaaaagggaggagggtataatgaggcatgtccgaccccacttcccatcatggcctgaactagtttttcaggttaacttcggaatttactttgctgagaggagaggtccattgcagtggttggagggcttagaattttatttttggtttacatagtctttgtgcaggggaacacttaacaaaaaatgaaggagcaagggaatatgtgtcaggtctgggtgctggtggctgggccctgctggcttctgtaggggcatttcaccccgttgggtctttggtttaggcttcagtcctgctgcatcccctgctggggtcatttggtccccctggcctttggatgcaagtgagcatctgggcccactgtcctcctacaaggcctctggtccagatgtcctcaccctgtgctcacctcaccccatccctggccaccctcagtctctggccctctgtatcagttatttattgctgctggaacaaatgcctgcaaacttagtggctcaaaataaaaacttttcttagaggtctggaggttagaagtccaaagcaggtctcatggggctaaaatcaaggtgctggagagactgtgctctttctgaaggctctaggggggaacctgtctccttgccttttcttgcttctggaggctcctacctgtcttttattatctgattttcttgcctccctcttttaaggacccttttgattatatcagacccacccggataatccaggataattgtcccaactcaggattctgtaagccaaaacaaaaatcccaggccccccaacagactgaacagagccaagagaaacctgaaaaatgaaattcacaatcatcatgggaagggaggttggacacacctcgttataccctctcccttttggagttcagcacaactgaccagcattaacactaaaatagagatcacaagactgacaaaacagactctgtggcaataagagatcaaattccatcctgactctagtgtagcatcacatgacagatatcagaccctgaaggaaatcaaagtattttaccccaaaatacatttctctgacactttgaaatggccctgcaaagctgtcttgtgtggggaaaattctacatctgtagagaacctccattaatgcagcccagtctttctgggatctaggagagattaactaagagtctgacacctttaaggtatgaaaagacacatttaccatctattcccactgaagcctgctacctggaggcttcatctacataataagaaccttggcttccacaactctccccacccgcttaccttaaccaaagcatttctttctactgatttcaaatagtttaactctttcaaacaattgccaatcagataatttttgaatccatctatgacctgtaagctcccccactctttgagatgtctcacctttccaggccaaatcaatatattccttacatgtattgatctatgtctttgcctgtaacttgtctccctaaactatataaaaccaaactgtaatctgacctccttgggcaccctttctcaggaccccctgaggctcttcctggagccatggtcactcatattggcttagaataaactcctttaaatattttacagagtttgggttttttgttcacaattattaatcacacatttgccaagtaaggtcacatactcacaggttctgggggttaggatgtggacatgtttggggggcaattgttctgctttccataccctcctatcattcccaacccctttctgggacaagcagcacacactggattcccccatgtcactgatgggccatgggaaagtggagatgctactttacgccgtcccgctgctgaaagcgccaaactgcctctcctcctccatgcagctgcctcatgggggtgggaggcaccaggtgaggccccttatctcagagattgaagtggaaagagtggcacaaacctatctgggtgtgtgttatatgacatcattcctggggtacataggaggcatgaataaagagcactggggaattttcagcctaagccttgatgtgacaatcctgcattccccaatccttcctgttcccactataatcaggaccaaaagagctgaatcctgcaggtagtgagctgggcttgattaggaaatgagaaggttctgggtgtgatgatctaagttccatataggtaggctcagatgcatgctgggcttgctagctgtatcggagttgatctttctgagaaggtgagttcaagctctgtttcactgggtggcagggaaagttttgttcaaggcagaaatggaaagtagagtctcacactttgacacatagggagagaccccagtatccaaaatcccagctgctgcagcatacccgtgggctctcttgagggcccaggaggagaaagaacctgaaagccaaggttggtacgctgttatggattcctggtttcctctgtgtgtgtggttgggggtaggggttggagtacctgttctcacatgcttctgtcctcaattttaaggtgtggcttctcaggagtctgtgttccctgagaacaggaggtgaagaatgaaaaggaaaatggctcggtcatttctagaggtgatatcacaggtgaactgcttacttctgatttccttcctaaaataccaatttacagggctaaagacattttgcatttgttccacaaggatgcagctccccattctggtgatgaggtgacagtcagagaggcaacagaggggacctaaataacccagaagctttctttagtgacccaagatttagtattcattcaacaaactgctcaaggtctgacccaagatttagtattcattcaacaaactgctcaacgactgacccaagatttaggattcattcaacaaactactcaaggactgactgaccaagaggagtcattagcacaggtcttctaggcatgaatttgtttgaaaacttttaagctgaagaataggagtccctggggatagtgagttcagtttgaagttggacagcttgcatgtgttggcagcgcagggagcaatggcttaacttgctctcaaatctatgggagagctggagcagggcacaggcagtcaggtggatgggatgaaggtggagggatgccaccatatttctgggtaacaaaagggcactcgtcctgacagacttaaaatccaacacatcaaactatgctaattaaaataatatagaaatgataatacgttgatgggtaaacagaagaaaatagaaggccagatacacattgtggtagaatgaacaatctcccccacccattgcaaaatgtccccatcctagtccctggaagctgtgaatgtgttaccttacatggtaaaagggactttgcaggtgtcattaagttgaggatcttcagatggggggtttctcctgggttgtctgggtgggcctgaaatgtaatcactgggtctcttgcgtctttgggtaaggaaggtcttgttagttcacaactgcccatgggagaattttctccttctgtgcaaatatctgcaacactccctgaaaatgccagttgaattttctaacttcatattcttcagtaaagcatcgtagctcatctagttggaaagagacgactaccttcattaacagaaggtagaactcgccagaatgtaagatgatccagagatttcagagaaacttgtttctcgagtttcagtgctgacatcagggaaggcagctcattcataggctccctttgctaaactcgagatcaatgtagaaagaatcttagtcgaagcctaattcttcgtggattcatgctgtatggagtatcttggaaatataaatatgtaaatgttgaagaaatggagatgtgatcagaaatgtactttttttattgcactgacttgaatctttggccaaggcaggtggttcatgaggtcaagagttccagaccagcctggtcaacatagtgaaaccccatctctcctgctggttcttgttggcatggctcagtagatgagcctgtggctgctctcctttccccaggatctcctccagctctttcagctcctgggctaggtgtgtgcttagcaacaccacaaatggcaccaacctctgtaggacacccacatcgtttaggtagaagacagtaaaaactgccacagctttgtctgtgggttccagcttgtctttattctcttagtgttcactttcactacttgcttggcagtttagcattgtgtaagttatttgatttgttgctttgttggaatttattactttgttggaacttattccttgtgggatttctgatgtaaaagaaagtttgatttgtggcgaaatgttttctcacatttgttacattcataaggtttctctcctgtgtgtattttctgatgttcagtgagagtccacaggcgacggtaggttttcccacattgattacattcatatggtttctctcctgtgtgaattcttctatggactctgaaggctgacttatggcagaaggatttcccacattcattacattcatatggtttctccccagtgtgagttcgctgatgttcaacaaaggagaacttctgacagaaggttttcccacattcattacactcatagggtctctgtcctgtgtgtgttctctgatggtgagtcagggctgacttcctgcagtaggttctcccacattcattgcattcatatggtctctcccatatagttctctgatgtacaatgaggtgtgagtttttgctgacggcatgcccatgttcactacactcataaagattctcctttgtgttcattctcttacactgactgcagtttgacttcacaatggagattctaccacatttattaaacacaccatgtttctctcctgtgtgtgttctctgatgtatagtgagtgttgacttatggcagaaaaatttcccacattcattacattcataagacttctttcctctatgagttatctgatgtgcaatgagggctgatttcgtacataaaaattttccacattgactgcattcatagggcttctctcctgtatgacttcttcgatgcacattgagggcagattgacaaaagaaggttttctcacattcactacattcatagggtttttcccctgtgtgaattctctgatgcgcagtaagggctgactgacagaagaaggttttcccacattccttacattcatttggcttctctcctctgtgagttctttgatgtacaacaagatacgatttcttgctgaaggcatttccacattccttgcattcgtaaggcttctcccctgtgtgtgacctgaaatgttcagccagggctgacttccgaaaaaaggtctttccacattcattacactcataggatttctcccctccatgaattttctggtgtacaataagggcagatttgtcaatgaaggttttcctgcattcactgcattcatagggtctctctccagtatgaattcttcggtgtcgagtgaggcttgtcttcacacgaaaagttttcctacaatcactacaaacatacggtttctcccctgtatgaattctctgatgtacaatgagggtagatctcttagaaaaggttttcctacattcattacattcatttggtttcctttcagtctgtctccccttttgtgtaatgagaattgccctcttgaagaaggttttcccacatttattatagtcaaacggttgtttcaaaatctgaatgttctggtgcagaataagattttcgttttgattgctggctttcctcattggattgtatctgtattttttcattcccaaatgacttttctcatgcttcccaaatccactgtatccatcaggaatctttctgttttctttgcttttctttgcaacaattacttctgaattagttttcaaactgtttcctcctggattacatttatagggcatttttcttgagggaacactattcatgcccagattaagtgttttcccaaatacattctctctttctgtaatcagtgttttgttgctgaagaatacagtttgtgtcaaatgtttatcttggatttccttgttcttctctaaggcatcatcaatgtctgggtagttctgatttgagaattcctccactatccatggctcttctccttgctccaatttgaaaatcacatctggtttgctaacatgataccccacagagaccaagttgctgtagttctccagcatcacatccctgtacaggagcctctgagcagggtccagttgctgccattcctcttgggtgaagttcacagtcaggtcctggaatgaaactggtatctgaaattttttcattttcatgttctcttgagaaagggccaagagtgttgaaagcagagcgttccctccgacgcccgagtgctcagagctcgccgccagcccttcctataggttgtgggtgcacccgcttcgcctccagttcgcaccaggtccaagtctcggcgggaccagggattcacgggctgcaggaccctcacccggaaga

SEQ ID NO: 8594 - RNA, 10019 nt, Homo sapiens
  source 1..10019: mol_type = other RNA
aaagactctgcaagatgccttgaagtctttttgctcaaattctccctttgcatgttggggctaaagcaaatctgggacaggagagagactggggaggcagtgggtgtggttattgaagaagttaatgtgggtaacaccagagatcctggaggtgatgacagtgttctgtaacatgacaatggtggtgaatactagaacctacatgtgataaaactgtatagaattaacacacacatacaaatgaagtaaagctaaggaaatatgaataagatcggagaattttatcaacctcaatatcctggttttgatattgtactatcattttgcaagatgttaccattaggcaaaactgggtaaagggtatatgagggctctattttttcttgcaactgcatgtcaacctacaattatctcaatacaaatgtcaattatacaaaatagaagttagatttaatgtctttcttttttatatgtgcagtctcaggttatacctgcagaaccatatacttgtattatgctgctgacaaaaaagtgtgaaagaacccaatgccttcattttaaagatgagtcacataaaggttaggcgactatccaagctgataaagcttgtttatattaagcatttatcatggtttctgcctttccataagttataatgatggagaattttatggcaatgttaagacgtccagtcctgggttcagacaactttgggatatatcctatcaggattcaaacggtctcaccatgtgatcttagaaaaataatgtttgcattttctactcattgaaatgagataataaaataatcccatacaccgatgggatttcaagatactgaaataaaataattcatgctggtacagtggatgcgtgataggagactctcaaaataatgcctgttttccggcatattaagtgctggacactagagctaaaggctttgaatacaaagagataaaaggtacagcttctgcttccataaacagagtctaggagagagaataacacaaagataattgcacagattaaaatgtgaaaaataggagagtacagggaattggtggttgatgaggctggataagtaaatgcagcaggtgaggaaggcacctttttaggaatccacactttggctaggtttatgtcatcaaagagcctaacagcctgtttttttgttttttggtttttttttttcacgtgacaggatcttgctttattgcccaggctggagtgcagtgatgtgatcatagctcactgctgcctcaaatggtggggctcaagtgatcttctcacctcagcctcccaagtagcctggactataggcacatgccaccatacctggaattttaaaagtgtttgtagagacaaggtcttgctatgttgcccaggatggtctcagacttctggcctcaggaaatcctcctgcctcagccctgtaaagtgctaggattacaggtatgagccgccatggctggccgagagcctggtcttttagagttagatggatttgaggatggagctcagtgctatccctcaccagctgtgttactgtgggcaaaattgcttatttttctaatcctcccttttctcaaccccaaaataagaagattgcaatagaataattccctctagggtggctgtgtcagttaatgagatcatgaatatggacatgcttagcactcagtatcttcctgcagcttgctaaaatagccacagtgtatgcaaaaatgtaaatatctttcggtataactgggctacaaatgatggtagaaaacataatcataccactccaaggtcatttcacatcttcatgtttaaaacagactattctgaaatagtcatttgattgagaaattaaattatctgatttcaacattcacatgtgctctctggtacattctctcctctcaagcactctctctccctttcctctgattttgtctcagaattatagttgtcaatgaaaagagtcaaaccctgtaaaacatttgaagagatttattctgagccaaatatgagtgaccaatggcccacaacacagccttcaggagatcccaaacacatgtgcctaaggtggtcaggctacaacttggttttatacattttagggacacaaaagacattaatcagtacaaaaaagatgtacactggttcagtctggaaaggtgggacaactggaaggcaagggcttccaggtcataagcagattcaaatactttctgactggcaattggttgaaaggattaagttattacctaaagacttagaatcaatggaaaggaacgtctgggctaaggggttgtgaagaccaagtttttatcatgcaggcaaagtctccaggtagctggctttagagagaatacattataaattattcttatcagacttagagagtctgttctctcagtaatttcaaaagggaggagggtataatgaggcatgtccgaccccacttcccatcatggcctgaactagtttttcaggttaacttcggaatttactttgctgagaggagaggtccattgcagtggttggagggcttagaattttatttttggtttacatagtctttgtgcaggggaacacttaacaaaaaatgaaggagcaagggaatatgtgtcaggtctgggtgctggtggctgggccctgctggcttctgtaggggcatttcaccccgttgggtctttggtttaggcttcagtcctgctgcatcccctgctggggtcatttggtccccctggcctttggatgcaagtgagcatctgggcccactgtcctcctacaaggcctctggtccagatgtcctcaccctgtgctcacctcaccccatccctggccaccctcagtctctggccctctgtatcagttatttattgctgctggaacaaatgcctgcaaacttagtggctcaaaataaaaacttttcttagaggtctggaggttagaagtccaaagcaggtctcatggggctaaaatcaaggtgctggagagactgtgctctttctgaaggctctaggggggaacctgtctccttgccttttcttgcttctggaggctcctacctgtcttttattatctgattttcttgcctccctcttttaaggacccttttgattatatcagacccacccggataatccaggataattgtcccaactcaggattctgtaagccaaaacaaaaatcccaggccccccaacagactgaacagagccaagagaaacctgaaaaatgaaattcacaatcatcatgggaagggaggttggacacacctcgttataccctctcccttttggagttcagcacaactgaccagcattaacactaaaatagagatcacaagactgacaaaacagactctgtggcaataagagatcaaattccatcctgactctagtgtagcatcacatgacagatatcagaccctgaaggaaatcaaagtattttaccccaaaatacatttctctgacactttgaaatggccctgcaaagctgtcttgtgtggggaaaattctacatctgtagagaacctccattaatgcagcccagtctttctgggatctaggagagattaactaagagtctgacacctttaaggtatgaaaagacacatttaccatctattcccactgaagcctgctacctggaggcttcatctacataataagaaccttggcttccacaactctccccacccgcttaccttaaccaaagcatttctttctactgatttcaaatagtttaactctttcaaacaattgccaatcagataatttttgaatccatctatgacctgtaagctcccccactctttgagatgtctcacctttccaggccaaatcaatatattccttacatgtattgatctatgtctttgcctgtaacttgtctccctaaactatataaaaccaaactgtaatctgacctccttgggcaccctttctcaggaccccctgaggctcttcctggagccatggtcactcatattggcttagaataaactcctttaaatattttacagagtttgggttttttgttcacaattattaatcacacatttgccaagtaaggtcacatactcacaggttctgggggttaggatgtggacatgtttggggggcaattgttctgctttccataccctcctatcattcccaacccctttctgggacaagcagcacacactggattcccccatgtcactgatgggccatgggaaagtggagatgctactttacgccgtcccgctgctgaaagcgccaaactgcctctcctcctccatgcagctgcctcatgggggtgggaggcaccaggtgaggccccttatctcagagattgaagtggaaagagtggcacaaacctatctgggtgtgtgttatatgacatcattcctggggtacataggaggcatgaataaagagcactggggaattttcagcctaagccttgatgtgacaatcctgcattccccaatccttcctgttcccactataatcaggaccaaaagagctgaatcctgcaggtagtgagctgggcttgattaggaaatgagaaggttctgggtgtgatgatctaagttccatataggtaggctcagatgcatgctgggcttgctagctgtatcggagttgatctttctgagaaggtgagttcaagctctgtttcactgggtggcagggaaagttttgttcaaggcagaaatggaaagtagagtctcacactttgacacatagggagagaccccagtatccaaaatcccagctgctgcagcatacccgtgggctctcttgagggcccaggaggagaaagaacctgaaagccaaggttggtacgctgttatggattcctggtttcctctgtgtgtgtggttgggggtaggggttggagtacctgttctcacatgcttctgtcctcaattttaaggtgtggcttctcaggagtctgtgttccctgagaacaggaggtgaagaatgaaaaggaaaatggctcggtcatttctagaggtgatatcacaggtgaactgcttacttctgatttccttcctaaaataccaatttacagggctaaagacattttgcatttgttccacaaggatgcagctccccattctggtgatgaggtgacagtcagagaggcaacagaggggacctaaataacccagaagctttctttagtgacccaagatttagtattcattcaacaaactgctcaaggtctgacccaagatttagtattcattcaacaaactgctcaacgactgacccaagatttaggattcattcaacaaactactcaaggactgactgaccaagaggagtcattagcacaggtcttctaggcatgaatttgtttgaaaacttttaagctgaagaataggagtccctggggatagtgagttcagtttgaagttggacagcttgcatgtgttggcagcgcagggagcaatggcttaacttgctctcaaatctatgggagagctggagcagggcacaggcagtcaggtggatgggatgaaggtggagggatgccaccatatttctgggtaacaaaagggcactcgtcctgacagacttaaaatccaacacatcaaactatgctaattaaaataatatagaaatgataatacgttgatgggtaaacagaagaaaatagaaggccagatacacattgtggtagaatgaacaatctcccccacccattgcaaaatgtccccatcctagtccctggaagctgtgaatgtgttaccttacatggtaaaagggactttgcaggtgtcattaagttgaggatcttcagatggggggtttctcctgggttgtctgggtgggcctgaaatgtaatcactgggtctcttgcgtctttgggtaaggaaggtcttgttagttcacaactgcccatgggagaattttctccttctgtgcaaatatctgcaacactccctgaaaatgccagttgaattttctaacttcatattcttcagtaaagcatcgtagctcatctagttggaaagagacgactaccttcattaacagaaggtagaactcgccagaatgtaagatgatccagagatttcagagaaacttgtttctcgagtttcagtgctgacatcagggaaggcagctcattcataggctccctttgctaaactcgagatcaatgtagaaagaatcttagtcgaagcctaattcttcgtggattcatgctgtatggagtatcttggaaatataaatatgtaaatgttgaagaaatggagatgtgatcagaaatgtactttttttattgcactgacttgaatctttggccaaggcaggtggttcatgaggtcaagagttccagaccagcctggtcaacatagtgaaaccccatctctcctgctggttcttgttggcatggctcagtagatgagcctgtggctgctctcctttccccaggatctcctccagctctttcagctcctgggctaggtgtgtgcttagcaacaccacaaatggcaccaacctctgtaggacacccacatcgtttaggtagaagacagtaaaaactgccacagctttgtctgtgggttccagcttgtctttattctcttagtgttcactttcactacttgcttggcagtttagcattgtgtaagttatttgatttgttgctttgttggaatttattactttgttggaacttattccttgtgggatttctgatgtaaaagaaagtttgatttgtggcgaaatgttttctcacatttgttacattcataaggtttctctcctgtgtgtattttctgatgttcagtgagagtccacaggcgacggtaggttttcccacattgattacattcatatggtttctctcctgtgtgaattcttctatggactctgaaggctgacttatggcagaaggatttcccacattcattacattcatatggtttctccccagtgtgagttcgctgatgttcaacaaaggagaacttctgacagaaggttttcccacattcattacactcatagggtctctgtcctgtgtgtgttctctgatggtgagtcagggctgacttcctgcagtaggttctcccacattcattgcattcatatggtctctcccatatagttctctgatgtacaatgaggtgtgagtttttgctgacggcatgcccatgttcactacactcataaagattctcctttgtgttcattctcttacactgactgcagtttgacttcacaatggagattctaccacatttattaaacacaccatgtttctctcctgtgtgtgttctctgatgtatagtgagtgttgacttatggcagaaaaatttcccacattcattacattcataagacttctttcctctatgagttatctgatgtgcaatgagggctgatttcgtacataaaaattttccacattgactgcattcatagggcttctctcctgtatgacttcttcgatgcacattgagggcagattgacaaaagaaggttttctcacattcactacattcatagggtttttcccctgtgtgaattctctgatgcgcagtaagggctgactgacagaagaaggttttcccacattccttacattcatttggcttctctcctctgtgagttctttgatgtacaacaagatacgatttcttgctgaaggcatttccacattccttgcattcgtaaggcttctcccctgtgtgtgacctgaaatgttcagccagggctgacttccgaaaaaaggtctttccacattcattacactcataggatttctcccctccatgaattttctggtgtacaataagggcagatttgtcaatgaaggttttcctgcattcactgcattcatagggtctctctccagtatgaattcttcggtgtcgagtgaggcttgtcttcacacgaaaagttttcctacaatcactacaaacatacggtttctcccctgtatgaattctctgatgtacaatgagggtagatctcttagaaaaggttttcctacattcattacattcatttggtttcctttcagtctgtctccccttttgtgtaatgagaattgccctcttgaagaaggttttcccacatttattatagtcaaacggttgtttcaaaatctgaatgttctggtgcagaataagattttcgttttgattgctggctttcctcattggattgtatctgtattttttcattcccaaatgacttttctcatgcttcccaaatccactgtatccatcaggaatctttctgttttctttgcttttctttgcaacaattacttctgaattagttttcaaactgtttcctcctggattacatttatagggcatttttcttgagggaacactattcatgcccagattaagtgttttcccaaatacattctctctttctgtaatcagtgttttgttgctgaagaatacagtttgtgtcaaatgtttatcttggatttccttgttcttctctaaggcatcatcaatgtctgggtagttctgatttgagaattcctccactatccatggctcttctccttgctccaatttgaaaatcacatctggtttgctaacatgataccccacagagaccaagttgctgtagttctccagcatcacatccctgtacaggagcctctgagcagggtccagttgctgccattcctcttgggtgaagttcacagtcaggtcctggaatgaaactggtatctgaaattttttcattttcatgttctcttgagaaagggccaagagtgttgaaagcagagctgggtaaggaagaatggcgaatggaatcatgagcgatttggctcacacagcagctctacaattacctacaaagccacacacccatttaaaaacatggccctttgaccagtctggttcaggaagcaacatgttgaggaaacgttcacttgtccatttatagttctagaatggtctcatagagcttttcttactgagtgagtgtcaacaaatgttttctactgaattactgtcaatctatgcctcctttgaaaaaaattgaaaacgtctgagtccaattaataggagactaggtcaacgaaagttagtatatacaaagcctggaacactattttggcattaaaatggactctaggattaaaagatttcttggaataggaaaatgatattatgtcacttacctgttttcctactaatgtgtttagccacttgagatgacagaatccagagagaatgaatgaaagtgctttaaggtgtttgtctttttgacagtttggtttcccttagctgcagtttcacaagaggaccttttactaagaaacttcttgtggtaggtaacgtaaatgtggtagatgacaaaagccctgacctggtactcaaaggaccagaattcagttattggatctgtcactagcaaactgcattactgaaaaaaatatttactaagtcgtaattttaatataagataaattggtttttagtctttcctttacccctatcgtgtagctctgtaaggggtaaactcagtaaatcccaggtgaggtgatgaacatggttggtgcagctctgaataaacagagggtggagatggtagggaatgacatgtatgtgtttaggaagtgatgaagacatcatttccttatttataaccagtactccttccctccaacccaggactctcgcagatacctccagtgaagtgtcttttcctgtcaaatcttgaccctgcccattccagctcacatccttcttccgaaagttgaactgaactttgctgagctataataatcaatggctgcaagactaagtgcatcagcagaagttctggaaagaggttctagctacttggatgcgtaaacctttcaccttcaccaagcgccttcttcgggcaaatcagggccctagagagagctcgcccgtggcctgcaggtcaggagcccaatcctgccctggctgcctcgcctcccgaccacaggaaaccctccctccaaagacagggagagcgcgcgtccaccctccgcagacccgaggcccgctccgcccgg

SEQ ID NO: 8595 - RNA, 10256 nt, Homo sapiens
  source 1..10256: mol_type = other RNA
aaagactctgcaagatgccttgaagtctttttgctcaaattctccctttgcatgttggggctaaagcaaatctgggacaggagagagactggggaggcagtgggtgtggttattgaagaagttaatgtgggtaacaccagagatcctggaggtgatgacagtgttctgtaacatgacaatggtggtgaatactagaacctacatgtgataaaactgtatagaattaacacacacatacaaatgaagtaaagctaaggaaatatgaataagatcggagaattttatcaacctcaatatcctggttttgatattgtactatcattttgcaagatgttaccattaggcaaaactgggtaaagggtatatgagggctctattttttcttgcaactgcatgtcaacctacaattatctcaatacaaatgtcaattatacaaaatagaagttagatttaatgtctttcttttttatatgtgcagtctcaggttatacctgcagaaccatatacttgtattatgctgctgacaaaaaagtgtgaaagaacccaatgccttcattttaaagatgagtcacataaaggttaggcgactatccaagctgataaagcttgtttatattaagcatttatcatggtttctgcctttccataagttataatgatggagaattttatggcaatgttaagacgtccagtcctgggttcagacaactttgggatatatcctatcaggattcaaacggtctcaccatgtgatcttagaaaaataatgtttgcattttctactcattgaaatgagataataaaataatcccatacaccgatgggatttcaagatactgaaataaaataattcatgctggtacagtggatgcgtgataggagactctcaaaataatgcctgttttccggcatattaagtgctggacactagagctaaaggctttgaatacaaagagataaaaggtacagcttctgcttccataaacagagtctaggagagagaataacacaaagataattgcacagattaaaatgtgaaaaataggagagtacagggaattggtggttgatgaggctggataagtaaatgcagcaggtgaggaaggcacctttttaggaatccacactttggctaggtttatgtcatcaaagagcctaacagcctgtttttttgttttttggtttttttttttcacgtgacaggatcttgctttattgcccaggctggagtgcagtgatgtgatcatagctcactgctgcctcaaatggtggggctcaagtgatcttctcacctcagcctcccaagtagcctggactataggcacatgccaccatacctggaattttaaaagtgtttgtagagacaaggtcttgctatgttgcccaggatggtctcagacttctggcctcaggaaatcctcctgcctcagccctgtaaagtgctaggattacaggtatgagccgccatggctggccgagagcctggtcttttagagttagatggatttgaggatggagctcagtgctatccctcaccagctgtgttactgtgggcaaaattgcttatttttctaatcctcccttttctcaaccccaaaataagaagattgcaatagaataattccctctagggtggctgtgtcagttaatgagatcatgaatatggacatgcttagcactcagtatcttcctgcagcttgctaaaatagccacagtgtatgcaaaaatgtaaatatctttcggtataactgggctacaaatgatggtagaaaacataatcataccactccaaggtcatttcacatcttcatgtttaaaacagactattctgaaatagtcatttgattgagaaattaaattatctgatttcaacattcacatgtgctctctggtacattctctcctctcaagcactctctctccctttcctctgattttgtctcagaattatagttgtcaatgaaaagagtcaaaccctgtaaaacatttgaagagatttattctgagccaaatatgagtgaccaatggcccacaacacagccttcaggagatcccaaacacatgtgcctaaggtggtcaggctacaacttggttttatacattttagggacacaaaagacattaatcagtacaaaaaagatgtacactggttcagtctggaaaggtgggacaactggaaggcaagggcttccaggtcataagcagattcaaatactttctgactggcaattggttgaaaggattaagttattacctaaagacttagaatcaatggaaaggaacgtctgggctaaggggttgtgaagaccaagtttttatcatgcaggcaaagtctccaggtagctggctttagagagaatacattataaattattcttatcagacttagagagtctgttctctcagtaatttcaaaagggaggagggtataatgaggcatgtccgaccccacttcccatcatggcctgaactagtttttcaggttaacttcggaatttactttgctgagaggagaggtccattgcagtggttggagggcttagaattttatttttggtttacatagtctttgtgcaggggaacacttaacaaaaaatgaaggagcaagggaatatgtgtcaggtctgggtgctggtggctgggccctgctggcttctgtaggggcatttcaccccgttgggtctttggtttaggcttcagtcctgctgcatcccctgctggggtcatttggtccccctggcctttggatgcaagtgagcatctgggcccactgtcctcctacaaggcctctggtccagatgtcctcaccctgtgctcacctcaccccatccctggccaccctcagtctctggccctctgtatcagttatttattgctgctggaacaaatgcctgcaaacttagtggctcaaaataaaaacttttcttagaggtctggaggttagaagtccaaagcaggtctcatggggctaaaatcaaggtgctggagagactgtgctctttctgaaggctctaggggggaacctgtctccttgccttttcttgcttctggaggctcctacctgtcttttattatctgattttcttgcctccctcttttaaggacccttttgattatatcagacccacccggataatccaggataattgtcccaactcaggattctgtaagccaaaacaaaaatcccaggccccccaacagactgaacagagccaagagaaacctgaaaaatgaaattcacaatcatcatgggaagggaggttggacacacctcgttataccctctcccttttggagttcagcacaactgaccagcattaacactaaaatagagatcacaagactgacaaaacagactctgtggcaataagagatcaaattccatcctgactctagtgtagcatcacatgacagatatcagaccctgaaggaaatcaaagtattttaccccaaaatacatttctctgacactttgaaatggccctgcaaagctgtcttgtgtggggaaaattctacatctgtagagaacctccattaatgcagcccagtctttctgggatctaggagagattaactaagagtctgacacctttaaggtatgaaaagacacatttaccatctattcccactgaagcctgctacctggaggcttcatctacataataagaaccttggcttccacaactctccccacccgcttaccttaaccaaagcatttctttctactgatttcaaatagtttaactctttcaaacaattgccaatcagataatttttgaatccatctatgacctgtaagctcccccactctttgagatgtctcacctttccaggccaaatcaatatattccttacatgtattgatctatgtctttgcctgtaacttgtctccctaaactatataaaaccaaactgtaatctgacctccttgggcaccctttctcaggaccccctgaggctcttcctggagccatggtcactcatattggcttagaataaactcctttaaatattttacagagtttgggttttttgttcacaattattaatcacacatttgccaagtaaggtcacatactcacaggttctgggggttaggatgtggacatgtttggggggcaattgttctgctttccataccctcctatcattcccaacccctttctgggacaagcagcacacactggattcccccatgtcactgatgggccatgggaaagtggagatgctactttacgccgtcccgctgctgaaagcgccaaactgcctctcctcctccatgcagctgcctcatgggggtgggaggcaccaggtgaggccccttatctcagagattgaagtggaaagagtggcacaaacctatctgggtgtgtgttatatgacatcattcctggggtacataggaggcatgaataaagagcactggggaattttcagcctaagccttgatgtgacaatcctgcattccccaatccttcctgttcccactataatcaggaccaaaagagctgaatcctgcaggtagtgagctgggcttgattaggaaatgagaaggttctgggtgtgatgatctaagttccatataggtaggctcagatgcatgctgggcttgctagctgtatcggagttgatctttctgagaaggtgagttcaagctctgtttcactgggtggcagggaaagttttgttcaaggcagaaatggaaagtagagtctcacactttgacacatagggagagaccccagtatccaaaatcccagctgctgcagcatacccgtgggctctcttgagggcccaggaggagaaagaacctgaaagccaaggttggtacgctgttatggattcctggtttcctctgtgtgtgtggttgggggtaggggttggagtacctgttctcacatgcttctgtcctcaattttaaggtgtggcttctcaggagtctgtgttccctgagaacaggaggtgaagaatgaaaaggaaaatggctcggtcatttctagaggtgatatcacaggtgaactgcttacttctgatttccttcctaaaataccaatttacagggctaaagacattttgcatttgttccacaaggatgcagctccccattctggtgatgaggtgacagtcagagaggcaacagaggggacctaaataacccagaagctttctttagtgacccaagatttagtattcattcaacaaactgctcaaggtctgacccaagatttagtattcattcaacaaactgctcaacgactgacccaagatttaggattcattcaacaaactactcaaggactgactgaccaagaggagtcattagcacaggtcttctaggcatgaatttgtttgaaaacttttaagctgaagaataggagtccctggggatagtgagttcagtttgaagttggacagcttgcatgtgttggcagcgcagggagcaatggcttaacttgctctcaaatctatgggagagctggagcagggcacaggcagtcaggtggatgggatgaaggtggagggatgccaccatatttctgggtaacaaaagggcactcgtcctgacagacttaaaatccaacacatcaaactatgctaattaaaataatatagaaatgataatacgttgatgggtaaacagaagaaaatagaaggccagatacacattgtggtagaatgaacaatctcccccacccattgcaaaatgtccccatcctagtccctggaagctgtgaatgtgttaccttacatggtaaaagggactttgcaggtgtcattaagttgaggatcttcagatggggggtttctcctgggttgtctgggtgggcctgaaatgtaatcactgggtctcttgcgtctttgggtaaggaaggtcttgttagttcacaactgcccatgggagaattttctccttctgtgcaaatatctgcaacactccctgaaaatgccagttgaattttctaacttcatattcttcagtaaagcatcgtagctcatctagttggaaagagacgactaccttcattaacagaaggtagaactcgccagaatgtaagatgatccagagatttcagagaaacttgtttctcgagtttcagtgctgacatcagggaaggcagctcattcataggctccctttgctaaactcgagatcaatgtagaaagaatcttagtcgaagcctaattcttcgtggattcatgctgtatggagtatcttggaaatataaatatgtaaatgttgaagaaatggagatgtgatcagaaatgtactttttttattgcactgacttgaatctttggccaaggcaggtggttcatgaggtcaagagttccagaccagcctggtcaacatagtgaaaccccatctctcctgctggttcttgttggcatggctcagtagatgagcctgtggctgctctcctttccccaggatctcctccagctctttcagctcctgggctaggtgtgtgcttagcaacaccacaaatggcaccaacctctgtaggacacccacatcgtttaggtagaagacagtaaaaactgccacagctttgtctgtgggttccagcttgtctttattctcttagtgttcactttcactacttgcttggcagtttagcattgtgtaagttatttgatttgttgctttgttggaatttattactttgttggaacttattccttgtgggatttctgatgtaaaagaaagtttgatttgtggcgaaatgttttctcacatttgttacattcataaggtttctctcctgtgtgtattttctgatgttcagtgagagtccacaggcgacggtaggttttcccacattgattacattcatatggtttctctcctgtgtgaattcttctatggactctgaaggctgacttatggcagaaggatttcccacattcattacattcatatggtttctccccagtgtgagttcgctgatgttcaacaaaggagaacttctgacagaaggttttcccacattcattacactcatagggtctctgtcctgtgtgtgttctctgatggtgagtcagggctgacttcctgcagtaggttctcccacattcattgcattcatatggtctctcccatatagttctctgatgtacaatgaggtgtgagtttttgctgacggcatgcccatgttcactacactcataaagattctcctttgtgttcattctcttacactgactgcagtttgacttcacaatggagattctaccacatttattaaacacaccatgtttctctcctgtgtgtgttctctgatgtatagtgagtgttgacttatggcagaaaaatttcccacattcattacattcataagacttctttcctctatgagttatctgatgtgcaatgagggctgatttcgtacataaaaattttccacattgactgcattcatagggcttctctcctgtatgacttcttcgatgcacattgagggcagattgacaaaagaaggttttctcacattcactacattcatagggtttttcccctgtgtgaattctctgatgcgcagtaagggctgactgacagaagaaggttttcccacattccttacattcatttggcttctctcctctgtgagttctttgatgtacaacaagatacgatttcttgctgaaggcatttccacattccttgcattcgtaaggcttctcccctgtgtgtgacctgaaatgttcagccagggctgacttccgaaaaaaggtctttccacattcattacactcataggatttctcccctccatgaattttctggtgtacaataagggcagatttgtcaatgaaggttttcctgcattcactgcattcatagggtctctctccagtatgaattcttcggtgtcgagtgaggcttgtcttcacacgaaaagttttcctacaatcactacaaacatacggtttctcccctgtatgaattctctgatgtacaatgagggtagatctcttagaaaaggttttcctacattcattacattcatttggtttcctttcagtctgtctccccttttgtgtaatgagaattgccctcttgaagaaggttttcccacatttattatagtcaaacggttgtttcaaaatctgaatgttctggtgcagaataagattttcgttttgattgctggctttcctcattggattgtatctgtattttttcattcccaaatgacttttctcatgcttcccaaatccactgtatccatcaggaatctttctgttttctttgcttttctttgcaacaattacttctgaattagttttcaaactgtttcctcctggattacatttatagggcatttttcttgagggaacactattcatgcccagattaagtgttttcccaaatacattctctctttctgtaatcagtgttttgttgctgaagaatacagtttgtgtcaaatgtttatcttggatttccttgttcttctctaaggcatcatcaatgtctgggtagttctgatttgagaattcctccactatccatggctcttctccttgctccaatttgaaaatcacatctggtttgctaacatgataccccacagagaccaagttgctgtagttctccagcatcacatccctgtacaggagcctctgagcagggtccagttgctgccattcctcttgggtgaagttcacagtcaggtcctggaatgaaactggtatcttgaaatagtgcacagaatagagaaaggatggggaattcatctgcccacctccttctcattttccatttcccttcattcaaggttcacccacggtgagttaacttgcgcacacttccaggttgcatcatctggctccaccatctggcccctcaggaagctggtaccacacctcatggtgtgtggtttcatccaagtctaaaacaggaggcagcctggtgtgggtgggtggcattaactgaaattttttcattttcatgttctcttgagaaagggccaagagtgttgaaagcagagctgggtaaggaagaatggcgaatggaatcatgagcgatttggctcacacagcagctctacaattacctacaaagccacacacccatttaaaaacatggccctttgaccagtctggttcaggaagcaacatgttgaggaaacgttcacttgtccatttatagttctagaatggtctcatagagcttttcttactgagtgagtgtcaacaaatgttttctactgaattactgtcaatctatgcctcctttgaaaaaaattgaaaacgtctgagtccaattaataggagactaggtcaacgaaagttagtatatacaaagcctggaacactattttggcattaaaatggactctaggattaaaagatttcttggaataggaaaatgatattatgtcacttacctgttttcctactaatgtgtttagccacttgagatgacagaatccagagagaatgaatgaaagtgctttaaggtgtttgtctttttgacagtttggtttcccttagctgcagtttcacaagaggaccttttactaagaaacttcttgtggtaggtaacgtaaatgtggtagatgacaaaagccctgacctggtactcaaaggaccagaattcagttattggatctgtcactagcaaactgcattactgaaaaaaatatttactaagtcgtaattttaatataagataaattggtttttagtctttcctttacccctatcgtgtagctctgtaaggggtaaactcagtaaatcccaggtgaggtgatgaacatggttggtgcagctctgaataaacagagggtggagatggtagggaatgacatgtatgtgtttaggaagtgatgaagacatcatttccttatttataaccagtactccttccctccaacccaggactctcgcagatacctccagtgaagtgtcttttcctgtcaaatcttgaccctgcccattccagctcacatccttcttccgaaagttgaactgaactttgctgagctataataatcaatggctgcaagactaagtgcatcagcagaagttctggaaagaggttctagctacttggatgcgtaaacctttcaccttcaccaagcgccttcttcgggcaaatcagggccctagagagagctcgcccgtggcctgcaggtcaggagcccaatcctgccctggctgcctcgcctcccgaccacaggaaaccctccctccaaagacagggagagcgcgcgtccaccctccgcagacccgaggcccgctccgcccgg

SEQ ID NO: 8596 - RNA, 10259 nt, Homo sapiens
  source 1..10259: mol_type = other RNA
aaagactctgcaagatgccttgaagtctttttgctcaaattctccctttgcatgttggggctaaagcaaatctgggacaggagagagactggggaggcagtgggtgtggttattgaagaagttaatgtgggtaacaccagagatcctggaggtgatgacagtgttctgtaacatgacaatggtggtgaatactagaacctacatgtgataaaactgtatagaattaacacacacatacaaatgaagtaaagctaaggaaatatgaataagatcggagaattttatcaacctcaatatcctggttttgatattgtactatcattttgcaagatgttaccattaggcaaaactgggtaaagggtatatgagggctctattttttcttgcaactgcatgtcaacctacaattatctcaatacaaatgtcaattatacaaaatagaagttagatttaatgtctttcttttttatatgtgcagtctcaggttatacctgcagaaccatatacttgtattatgctgctgacaaaaaagtgtgaaagaacccaatgccttcattttaaagatgagtcacataaaggttaggcgactatccaagctgataaagcttgtttatattaagcatttatcatggtttctgcctttccataagttataatgatggagaattttatggcaatgttaagacgtccagtcctgggttcagacaactttgggatatatcctatcaggattcaaacggtctcaccatgtgatcttagaaaaataatgtttgcattttctactcattgaaatgagataataaaataatcccatacaccgatgggatttcaagatactgaaataaaataattcatgctggtacagtggatgcgtgataggagactctcaaaataatgcctgttttccggcatattaagtgctggacactagagctaaaggctttgaatacaaagagataaaaggtacagcttctgcttccataaacagagtctaggagagagaataacacaaagataattgcacagattaaaatgtgaaaaataggagagtacagggaattggtggttgatgaggctggataagtaaatgcagcaggtgaggaaggcacctttttaggaatccacactttggctaggtttatgtcatcaaagagcctaacagcctgtttttttgttttttggtttttttttttcacgtgacaggatcttgctttattgcccaggctggagtgcagtgatgtgatcatagctcactgctgcctcaaatggtggggctcaagtgatcttctcacctcagcctcccaagtagcctggactataggcacatgccaccatacctggaattttaaaagtgtttgtagagacaaggtcttgctatgttgcccaggatggtctcagacttctggcctcaggaaatcctcctgcctcagccctgtaaagtgctaggattacaggtatgagccgccatggctggccgagagcctggtcttttagagttagatggatttgaggatggagctcagtgctatccctcaccagctgtgttactgtgggcaaaattgcttatttttctaatcctcccttttctcaaccccaaaataagaagattgcaatagaataattccctctagggtggctgtgtcagttaatgagatcatgaatatggacatgcttagcactcagtatcttcctgcagcttgctaaaatagccacagtgtatgcaaaaatgtaaatatctttcggtataactgggctacaaatgatggtagaaaacataatcataccactccaaggtcatttcacatcttcatgtttaaaacagactattctgaaatagtcatttgattgagaaattaaattatctgatttcaacattcacatgtgctctctggtacattctctcctctcaagcactctctctccctttcctctgattttgtctcagaattatagttgtcaatgaaaagagtcaaaccctgtaaaacatttgaagagatttattctgagccaaatatgagtgaccaatggcccacaacacagccttcaggagatcccaaacacatgtgcctaaggtggtcaggctacaacttggttttatacattttagggacacaaaagacattaatcagtacaaaaaagatgtacactggttcagtctggaaaggtgggacaactggaaggcaagggcttccaggtcataagcagattcaaatactttctgactggcaattggttgaaaggattaagttattacctaaagacttagaatcaatggaaaggaacgtctgggctaaggggttgtgaagaccaagtttttatcatgcaggcaaagtctccaggtagctggctttagagagaatacattataaattattcttatcagacttagagagtctgttctctcagtaatttcaaaagggaggagggtataatgaggcatgtccgaccccacttcccatcatggcctgaactagtttttcaggttaacttcggaatttactttgctgagaggagaggtccattgcagtggttggagggcttagaattttatttttggtttacatagtctttgtgcaggggaacacttaacaaaaaatgaaggagcaagggaatatgtgtcaggtctgggtgctggtggctgggccctgctggcttctgtaggggcatttcaccccgttgggtctttggtttaggcttcagtcctgctgcatcccctgctggggtcatttggtccccctggcctttggatgcaagtgagcatctgggcccactgtcctcctacaaggcctctggtccagatgtcctcaccctgtgctcacctcaccccatccctggccaccctcagtctctggccctctgtatcagttatttattgctgctggaacaaatgcctgcaaacttagtggctcaaaataaaaacttttcttagaggtctggaggttagaagtccaaagcaggtctcatggggctaaaatcaaggtgctggagagactgtgctctttctgaaggctctaggggggaacctgtctccttgccttttcttgcttctggaggctcctacctgtcttttattatctgattttcttgcctccctcttttaaggacccttttgattatatcagacccacccggataatccaggataattgtcccaactcaggattctgtaagccaaaacaaaaatcccaggccccccaacagactgaacagagccaagagaaacctgaaaaatgaaattcacaatcatcatgggaagggaggttggacacacctcgttataccctctcccttttggagttcagcacaactgaccagcattaacactaaaatagagatcacaagactgacaaaacagactctgtggcaataagagatcaaattccatcctgactctagtgtagcatcacatgacagatatcagaccctgaaggaaatcaaagtattttaccccaaaatacatttctctgacactttgaaatggccctgcaaagctgtcttgtgtggggaaaattctacatctgtagagaacctccattaatgcagcccagtctttctgggatctaggagagattaactaagagtctgacacctttaaggtatgaaaagacacatttaccatctattcccactgaagcctgctacctggaggcttcatctacataataagaaccttggcttccacaactctccccacccgcttaccttaaccaaagcatttctttctactgatttcaaatagtttaactctttcaaacaattgccaatcagataatttttgaatccatctatgacctgtaagctcccccactctttgagatgtctcacctttccaggccaaatcaatatattccttacatgtattgatctatgtctttgcctgtaacttgtctccctaaactatataaaaccaaactgtaatctgacctccttgggcaccctttctcaggaccccctgaggctcttcctggagccatggtcactcatattggcttagaataaactcctttaaatattttacagagtttgggttttttgttcacaattattaatcacacatttgccaagtaaggtcacatactcacaggttctgggggttaggatgtggacatgtttggggggcaattgttctgctttccataccctcctatcattcccaacccctttctgggacaagcagcacacactggattcccccatgtcactgatgggccatgggaaagtggagatgctactttacgccgtcccgctgctgaaagcgccaaactgcctctcctcctccatgcagctgcctcatgggggtgggaggcaccaggtgaggccccttatctcagagattgaagtggaaagagtggcacaaacctatctgggtgtgtgttatatgacatcattcctggggtacataggaggcatgaataaagagcactggggaattttcagcctaagccttgatgtgacaatcctgcattccccaatccttcctgttcccactataatcaggaccaaaagagctgaatcctgcaggtagtgagctgggcttgattaggaaatgagaaggttctgggtgtgatgatctaagttccatataggtaggctcagatgcatgctgggcttgctagctgtatcggagttgatctttctgagaaggtgagttcaagctctgtttcactgggtggcagggaaagttttgttcaaggcagaaatggaaagtagagtctcacactttgacacatagggagagaccccagtatccaaaatcccagctgctgcagcatacccgtgggctctcttgagggcccaggaggagaaagaacctgaaagccaaggttggtacgctgttatggattcctggtttcctctgtgtgtgtggttgggggtaggggttggagtacctgttctcacatgcttctgtcctcaattttaaggtgtggcttctcaggagtctgtgttccctgagaacaggaggtgaagaatgaaaaggaaaatggctcggtcatttctagaggtgatatcacaggtgaactgcttacttctgatttccttcctaaaataccaatttacagggctaaagacattttgcatttgttccacaaggatgcagctccccattctggtgatgaggtgacagtcagagaggcaacagaggggacctaaataacccagaagctttctttagtgacccaagatttagtattcattcaacaaactgctcaaggtctgacccaagatttagtattcattcaacaaactgctcaacgactgacccaagatttaggattcattcaacaaactactcaaggactgactgaccaagaggagtcattagcacaggtcttctaggcatgaatttgtttgaaaacttttaagctgaagaataggagtccctggggatagtgagttcagtttgaagttggacagcttgcatgtgttggcagcgcagggagcaatggcttaacttgctctcaaatctatgggagagctggagcagggcacaggcagtcaggtggatgggatgaaggtggagggatgccaccatatttctgggtaacaaaagggcactcgtcctgacagacttaaaatccaacacatcaaactatgctaattaaaataatatagaaatgataatacgttgatgggtaaacagaagaaaatagaaggccagatacacattgtggtagaatgaacaatctcccccacccattgcaaaatgtccccatcctagtccctggaagctgtgaatgtgttaccttacatggtaaaagggactttgcaggtgtcattaagttgaggatcttcagatggggggtttctcctgggttgtctgggtgggcctgaaatgtaatcactgggtctcttgcgtctttgggtaaggaaggtcttgttagttcacaactgcccatgggagaattttctccttctgtgcaaatatctgcaacactccctgaaaatgccagttgaattttctaacttcatattcttcagtaaagcatcgtagctcatctagttggaaagagacgactaccttcattaacagaaggtagaactcgccagaatgtaagatgatccagagatttcagagaaacttgtttctcgagtttcagtgctgacatcagggaaggcagctcattcataggctccctttgctaaactcgagatcaatgtagaaagaatcttagtcgaagcctaattcttcgtggattcatgctgtatggagtatcttggaaatataaatatgtaaatgttgaagaaatggagatgtgatcagaaatgtactttttttattgcactgacttgaatctttggccaaggcaggtggttcatgaggtcaagagttccagaccagcctggtcaacatagtgaaaccccatctctcctgctggttcttgttggcatggctcagtagatgagcctgtggctgctctcctttccccaggatctcctccagctctttcagctcctgggctaggtgtgtgcttagcaacaccacaaatggcaccaacctctgtaggacacccacatcgtttaggtagaagacagtaaaaactgccacagctttgtctgtgggttccagcttgtctttattctcttagtgttcactttcactacttgcttggcagtttagcattgtgtaagttatttgatttgttgctttgttggaatttattactttgttggaacttattccttgtgggatttctgatgtaaaagaaagtttgatttgtggcgaaatgttttctcacatttgttacattcataaggtttctctcctgtgtgtattttctgatgttcagtgagagtccacaggcgacggtaggttttcccacattgattacattcatatggtttctctcctgtgtgaattcttctatggactctgaaggctgacttatggcagaaggatttcccacattcattacattcatatggtttctccccagtgtgagttcgctgatgttcaacaaaggagaacttctgacagaaggttttcccacattcattacactcatagggtctctgtcctgtgtgtgttctctgatggtgagtcagggctgacttcctgcagtaggttctcccacattcattgcattcatatggtctctcccatatagttctctgatgtacaatgaggtgtgagtttttgctgacggcatgcccatgttcactacactcataaagattctcctttgtgttcattctcttacactgactgcagtttgacttcacaatggagattctaccacatttattaaacacaccatgtttctctcctgtgtgtgttctctgatgtatagtgagtgttgacttatggcagaaaaatttcccacattcattacattcataagacttctttcctctatgagttatctgatgtgcaatgagggctgatttcgtacataaaaattttccacattgactgcattcatagggcttctctcctgtatgacttcttcgatgcacattgagggcagattgacaaaagaaggttttctcacattcactacattcatagggtttttcccctgtgtgaattctctgatgcgcagtaagggctgactgacagaagaaggttttcccacattccttacattcatttggcttctctcctctgtgagttctttgatgtacaacaagatacgatttcttgctgaaggcatttccacattccttgcattcgtaaggcttctcccctgtgtgtgacctgaaatgttcagccagggctgacttccgaaaaaaggtctttccacattcattacactcataggatttctcccctccatgaattttctggtgtacaataagggcagatttgtcaatgaaggttttcctgcattcactgcattcatagggtctctctccagtatgaattcttcggtgtcgagtgaggcttgtcttcacacgaaaagttttcctacaatcactacaaacatacggtttctcccctgtatgaattctctgatgtacaatgagggtagatctcttagaaaaggttttcctacattcattacattcatttggtttcctttcagtctgtctccccttttgtgtaatgagaattgccctcttgaagaaggttttcccacatttattatagtcaaacggttgtttcaaaatctgaatgttctggtgcagaataagattttcgttttgattgctggctttcctcattggattgtatctgtattttttcattcccaaatgacttttctcatgcttcccaaatccactgtatccatcaggaatctttctgttttctttgcttttctttgcaacaattacttctgaattagttttcaaactgtttcctcctggattacatttatagggcatttttcttgagggaacactattcatgcccagattaagtgttttcccaaatacattctctctttctgtaatcagtgttttgttgctgaagaatacagtttgtgtcaaatgtttatcttggatttccttgttcttctctaaggcatcatcaatgtctgggtagttctgatttgagaattcctccactatccatggctcttctccttgctccaatttgaaaatcacatctggtttgctaacatgataccctgttaatgggaaattacagaacttggaccaagatctttggacatcagagactccacagagaccaagttgctgtagttctccagcatcacatccctgtacaggagcctctgagcagggtccagttgctgccattcctcttgggtgaagttcacagtcaggtcctggaatgaaactggtatctccttctcattttccatttcccttcattcaaggttcacccacggtgagttaacttgcgcacacttccaggttgcatcatctggctccaccatctggcccctcaggaagctggtaccacacctcatggtgtgtggtttcatccaagtctaaaacaggaggcagcctggtgtgggtgggtggcattaactgaaattttttcattttcatgttctcttgagaaagggccaagagtgttgaaagcagagctgggtaaggaagaatggcgaatggaatcatgagcgatttggctcacacagcagctctacaattacctacaaagccacacacccatttaaaaacatggccctttgaccagtctggttcaggaagcaacatgttgaggaaacgttcacttgtccatttatagttctagaatggtctcatagagcttttcttactgagtgagtgtcaacaaatgttttctactgaattactgtcaatctatgcctcctttgaaaaaaattgaaaacgtctgagtccaattaataggagactaggtcaacgaaagttagtatatacaaagcctggaacactattttggcattaaaatggactctaggattaaaagatttcttggaataggaaaatgatattatgtcacttacctgttttcctactaatgtgtttagccacttgagatgacagaatccagagagaatgaatgaaagtgctttaaggtgtttgtctttttgacagtttggtttcccttagctgcagtttcacaagaggaccttttactaagaaacttcttgtggtaggtaacgtaaatgtggtagatgacaaaagccctgacctggtactcaaaggaccagaattcagttattggatctgtcactagcaaactgcattactgaaaaaaatatttactaagtcgtaattttaatataagataaattggtttttagtctttcctttacccctatcgtgtagctctgtaaggggtaaactcagtaaatcccaggtgaggtgatgaacatggttggtgcagctctgaataaacagagggtggagatggtagggaatgacatgtatgtgtttaggaagtgatgaagacatcatttccttatttataaccagtactccttccctccaacccaggactctcgcagatacctccagtgaagtgtcttttcctgtcaaatcttgaccctgcccattccagctcacatccttcttccgaaagttgaactgaactttgctgagctataataatcaatggctgcaagactaagtgcatcagcagaagttctggaaagaggttctagctacttggatgcgtaaacctttcaccttcaccaagcgccttcttcgggcaaatcagggccctagagagagctcgcccgtggcctgcaggtcaggagcccaatcctgccctggctgcctcgcctcccgaccacaggaaaccctccctccaaagacagggagagcgcgcgtccaccctccgcagacccgaggcccgctccgcccgg

SEQ ID NO: 8597 - RNA, 10072 nt, Homo sapiens
  source 1..10072: mol_type = other RNA
aaagactctgcaagatgccttgaagtctttttgctcaaattctccctttgcatgttggggctaaagcaaatctgggacaggagagagactggggaggcagtgggtgtggttattgaagaagttaatgtgggtaacaccagagatcctggaggtgatgacagtgttctgtaacatgacaatggtggtgaatactagaacctacatgtgataaaactgtatagaattaacacacacatacaaatgaagtaaagctaaggaaatatgaataagatcggagaattttatcaacctcaatatcctggttttgatattgtactatcattttgcaagatgttaccattaggcaaaactgggtaaagggtatatgagggctctattttttcttgcaactgcatgtcaacctacaattatctcaatacaaatgtcaattatacaaaatagaagttagatttaatgtctttcttttttatatgtgcagtctcaggttatacctgcagaaccatatacttgtattatgctgctgacaaaaaagtgtgaaagaacccaatgccttcattttaaagatgagtcacataaaggttaggcgactatccaagctgataaagcttgtttatattaagcatttatcatggtttctgcctttccataagttataatgatggagaattttatggcaatgttaagacgtccagtcctgggttcagacaactttgggatatatcctatcaggattcaaacggtctcaccatgtgatcttagaaaaataatgtttgcattttctactcattgaaatgagataataaaataatcccatacaccgatgggatttcaagatactgaaataaaataattcatgctggtacagtggatgcgtgataggagactctcaaaataatgcctgttttccggcatattaagtgctggacactagagctaaaggctttgaatacaaagagataaaaggtacagcttctgcttccataaacagagtctaggagagagaataacacaaagataattgcacagattaaaatgtgaaaaataggagagtacagggaattggtggttgatgaggctggataagtaaatgcagcaggtgaggaaggcacctttttaggaatccacactttggctaggtttatgtcatcaaagagcctaacagcctgtttttttgttttttggtttttttttttcacgtgacaggatcttgctttattgcccaggctggagtgcagtgatgtgatcatagctcactgctgcctcaaatggtggggctcaagtgatcttctcacctcagcctcccaagtagcctggactataggcacatgccaccatacctggaattttaaaagtgtttgtagagacaaggtcttgctatgttgcccaggatggtctcagacttctggcctcaggaaatcctcctgcctcagccctgtaaagtgctaggattacaggtatgagccgccatggctggccgagagcctggtcttttagagttagatggatttgaggatggagctcagtgctatccctcaccagctgtgttactgtgggcaaaattgcttatttttctaatcctcccttttctcaaccccaaaataagaagattgcaatagaataattccctctagggtggctgtgtcagttaatgagatcatgaatatggacatgcttagcactcagtatcttcctgcagcttgctaaaatagccacagtgtatgcaaaaatgtaaatatctttcggtataactgggctacaaatgatggtagaaaacataatcataccactccaaggtcatttcacatcttcatgtttaaaacagactattctgaaatagtcatttgattgagaaattaaattatctgatttcaacattcacatgtgctctctggtacattctctcctctcaagcactctctctccctttcctctgattttgtctcagaattatagttgtcaatgaaaagagtcaaaccctgtaaaacatttgaagagatttattctgagccaaatatgagtgaccaatggcccacaacacagccttcaggagatcccaaacacatgtgcctaaggtggtcaggctacaacttggttttatacattttagggacacaaaagacattaatcagtacaaaaaagatgtacactggttcagtctggaaaggtgggacaactggaaggcaagggcttccaggtcataagcagattcaaatactttctgactggcaattggttgaaaggattaagttattacctaaagacttagaatcaatggaaaggaacgtctgggctaaggggttgtgaagaccaagtttttatcatgcaggcaaagtctccaggtagctggctttagagagaatacattataaattattcttatcagacttagagagtctgttctctcagtaatttcaaaagggaggagggtataatgaggcatgtccgaccccacttcccatcatggcctgaactagtttttcaggttaacttcggaatttactttgctgagaggagaggtccattgcagtggttggagggcttagaattttatttttggtttacatagtctttgtgcaggggaacacttaacaaaaaatgaaggagcaagggaatatgtgtcaggtctgggtgctggtggctgggccctgctggcttctgtaggggcatttcaccccgttgggtctttggtttaggcttcagtcctgctgcatcccctgctggggtcatttggtccccctggcctttggatgcaagtgagcatctgggcccactgtcctcctacaaggcctctggtccagatgtcctcaccctgtgctcacctcaccccatccctggccaccctcagtctctggccctctgtatcagttatttattgctgctggaacaaatgcctgcaaacttagtggctcaaaataaaaacttttcttagaggtctggaggttagaagtccaaagcaggtctcatggggctaaaatcaaggtgctggagagactgtgctctttctgaaggctctaggggggaacctgtctccttgccttttcttgcttctggaggctcctacctgtcttttattatctgattttcttgcctccctcttttaaggacccttttgattatatcagacccacccggataatccaggataattgtcccaactcaggattctgtaagccaaaacaaaaatcccaggccccccaacagactgaacagagccaagagaaacctgaaaaatgaaattcacaatcatcatgggaagggaggttggacacacctcgttataccctctcccttttggagttcagcacaactgaccagcattaacactaaaatagagatcacaagactgacaaaacagactctgtggcaataagagatcaaattccatcctgactctagtgtagcatcacatgacagatatcagaccctgaaggaaatcaaagtattttaccccaaaatacatttctctgacactttgaaatggccctgcaaagctgtcttgtgtggggaaaattctacatctgtagagaacctccattaatgcagcccagtctttctgggatctaggagagattaactaagagtctgacacctttaaggtatgaaaagacacatttaccatctattcccactgaagcctgctacctggaggcttcatctacataataagaaccttggcttccacaactctccccacccgcttaccttaaccaaagcatttctttctactgatttcaaatagtttaactctttcaaacaattgccaatcagataatttttgaatccatctatgacctgtaagctcccccactctttgagatgtctcacctttccaggccaaatcaatatattccttacatgtattgatctatgtctttgcctgtaacttgtctccctaaactatataaaaccaaactgtaatctgacctccttgggcaccctttctcaggaccccctgaggctcttcctggagccatggtcactcatattggcttagaataaactcctttaaatattttacagagtttgggttttttgttcacaattattaatcacacatttgccaagtaaggtcacatactcacaggttctgggggttaggatgtggacatgtttggggggcaattgttctgctttccataccctcctatcattcccaacccctttctgggacaagcagcacacactggattcccccatgtcactgatgggccatgggaaagtggagatgctactttacgccgtcccgctgctgaaagcgccaaactgcctctcctcctccatgcagctgcctcatgggggtgggaggcaccaggtgaggccccttatctcagagattgaagtggaaagagtggcacaaacctatctgggtgtgtgttatatgacatcattcctggggtacataggaggcatgaataaagagcactggggaattttcagcctaagccttgatgtgacaatcctgcattccccaatccttcctgttcccactataatcaggaccaaaagagctgaatcctgcaggtagtgagctgggcttgattaggaaatgagaaggttctgggtgtgatgatctaagttccatataggtaggctcagatgcatgctgggcttgctagctgtatcggagttgatctttctgagaaggtgagttcaagctctgtttcactgggtggcagggaaagttttgttcaaggcagaaatggaaagtagagtctcacactttgacacatagggagagaccccagtatccaaaatcccagctgctgcagcatacccgtgggctctcttgagggcccaggaggagaaagaacctgaaagccaaggttggtacgctgttatggattcctggtttcctctgtgtgtgtggttgggggtaggggttggagtacctgttctcacatgcttctgtcctcaattttaaggtgtggcttctcaggagtctgtgttccctgagaacaggaggtgaagaatgaaaaggaaaatggctcggtcatttctagaggtgatatcacaggtgaactgcttacttctgatttccttcctaaaataccaatttacagggctaaagacattttgcatttgttccacaaggatgcagctccccattctggtgatgaggtgacagtcagagaggcaacagaggggacctaaataacccagaagctttctttagtgacccaagatttagtattcattcaacaaactgctcaaggtctgacccaagatttagtattcattcaacaaactgctcaacgactgacccaagatttaggattcattcaacaaactactcaaggactgactgaccaagaggagtcattagcacaggtcttctaggcatgaatttgtttgaaaacttttaagctgaagaataggagtccctggggatagtgagttcagtttgaagttggacagcttgcatgtgttggcagcgcagggagcaatggcttaacttgctctcaaatctatgggagagctggagcagggcacaggcagtcaggtggatgggatgaaggtggagggatgccaccatatttctgggtaacaaaagggcactcgtcctgacagacttaaaatccaacacatcaaactatgctaattaaaataatatagaaatgataatacgttgatgggtaaacagaagaaaatagaaggccagatacacattgtggtagaatgaacaatctcccccacccattgcaaaatgtccccatcctagtccctggaagctgtgaatgtgttaccttacatggtaaaagggactttgcaggtgtcattaagttgaggatcttcagatggggggtttctcctgggttgtctgggtgggcctgaaatgtaatcactgggtctcttgcgtctttgggtaaggaaggtcttgttagttcacaactgcccatgggagaattttctccttctgtgcaaatatctgcaacactccctgaaaatgccagttgaattttctaacttcatattcttcagtaaagcatcgtagctcatctagttggaaagagacgactaccttcattaacagaaggtagaactcgccagaatgtaagatgatccagagatttcagagaaacttgtttctcgagtttcagtgctgacatcagggaaggcagctcattcataggctccctttgctaaactcgagatcaatgtagaaagaatcttagtcgaagcctaattcttcgtggattcatgctgtatggagtatcttggaaatataaatatgtaaatgttgaagaaatggagatgtgatcagaaatgtactttttttattgcactgacttgaatctttggccaaggcaggtggttcatgaggtcaagagttccagaccagcctggtcaacatagtgaaaccccatctctcctgctggttcttgttggcatggctcagtagatgagcctgtggctgctctcctttccccaggatctcctccagctctttcagctcctgggctaggtgtgtgcttagcaacaccacaaatggcaccaacctctgtaggacacccacatcgtttaggtagaagacagtaaaaactgccacagctttgtctgtgggttccagcttgtctttattctcttagtgttcactttcactacttgcttggcagtttagcattgtgtaagttatttgatttgttgctttgttggaatttattactttgttggaacttattccttgtgggatttctgatgtaaaagaaagtttgatttgtggcgaaatgttttctcacatttgttacattcataaggtttctctcctgtgtgtattttctgatgttcagtgagagtccacaggcgacggtaggttttcccacattgattacattcatatggtttctctcctgtgtgaattcttctatggactctgaaggctgacttatggcagaaggatttcccacattcattacattcatatggtttctccccagtgtgagttcgctgatgttcaacaaaggagaacttctgacagaaggttttcccacattcattacactcatagggtctctgtcctgtgtgtgttctctgatggtgagtcagggctgacttcctgcagtaggttctcccacattcattgcattcatatggtctctcccatatagttctctgatgtacaatgaggtgtgagtttttgctgacggcatgcccatgttcactacactcataaagattctcctttgtgttcattctcttacactgactgcagtttgacttcacaatggagattctaccacatttattaaacacaccatgtttctctcctgtgtgtgttctctgatgtatagtgagtgttgacttatggcagaaaaatttcccacattcattacattcataagacttctttcctctatgagttatctgatgtgcaatgagggctgatttcgtacataaaaattttccacattgactgcattcatagggcttctctcctgtatgacttcttcgatgcacattgagggcagattgacaaaagaaggttttctcacattcactacattcatagggtttttcccctgtgtgaattctctgatgcgcagtaagggctgactgacagaagaaggttttcccacattccttacattcatttggcttctctcctctgtgagttctttgatgtacaacaagatacgatttcttgctgaaggcatttccacattccttgcattcgtaaggcttctcccctgtgtgtgacctgaaatgttcagccagggctgacttccgaaaaaaggtctttccacattcattacactcataggatttctcccctccatgaattttctggtgtacaataagggcagatttgtcaatgaaggttttcctgcattcactgcattcatagggtctctctccagtatgaattcttcggtgtcgagtgaggcttgtcttcacacgaaaagttttcctacaatcactacaaacatacggtttctcccctgtatgaattctctgatgtacaatgagggtagatctcttagaaaaggttttcctacattcattacattcatttggtttcctttcagtctgtctccccttttgtgtaatgagaattgccctcttgaagaaggttttcccacatttattatagtcaaacggttgtttcaaaatctgaatgttctggtgcagaataagattttcgttttgattgctggctttcctcattggattgtatctgtattttttcattcccaaatgacttttctcatgcttcccaaatccactgtatccatcaggaatctttctgttttctttgcttttctttgcaacaattacttctgaattagttttcaaactgtttcctcctggattacatttatagggcatttttcttgagggaacactattcatgcccagattaagtgttttcccaaatacattctctctttctgtaatcagtgttttgttgctgaagaatacagtttgtgtcaaatgtttatcttggatttccttgttcttctctaaggcatcatcaatgtctgggtagttctgatttgagaattcctccactatccatggctcttctccttgctccaatttgaaaatcacatctggtttgctaacatgataccctgttaatgggaaattacagaacttggaccaagatctttggacatcagagactccacagagaccaagttgctgtagttctccagcatcacatccctgtacaggagcctctgagcagggtccagttgctgccattcctcttgggtgaagttcacagtcaggtcctggaatgaaactggtatctgaaattttttcattttcatgttctcttgagaaagggccaagagtgttgaaagcagagctgggtaaggaagaatggcgaatggaatcatgagcgatttggctcacacagcagctctacaattacctacaaagccacacacccatttaaaaacatggccctttgaccagtctggttcaggaagcaacatgttgaggaaacgttcacttgtccatttatagttctagaatggtctcatagagcttttcttactgagtgagtgtcaacaaatgttttctactgaattactgtcaatctatgcctcctttgaaaaaaattgaaaacgtctgagtccaattaataggagactaggtcaacgaaagttagtatatacaaagcctggaacactattttggcattaaaatggactctaggattaaaagatttcttggaataggaaaatgatattatgtcacttacctgttttcctactaatgtgtttagccacttgagatgacagaatccagagagaatgaatgaaagtgctttaaggtgtttgtctttttgacagtttggtttcccttagctgcagtttcacaagaggaccttttactaagaaacttcttgtggtaggtaacgtaaatgtggtagatgacaaaagccctgacctggtactcaaaggaccagaattcagttattggatctgtcactagcaaactgcattactgaaaaaaatatttactaagtcgtaattttaatataagataaattggtttttagtctttcctttacccctatcgtgtagctctgtaaggggtaaactcagtaaatcccaggtgaggtgatgaacatggttggtgcagctctgaataaacagagggtggagatggtagggaatgacatgtatgtgtttaggaagtgatgaagacatcatttccttatttataaccagtactccttccctccaacccaggactctcgcagatacctccagtgaagtgtcttttcctgtcaaatcttgaccctgcccattccagctcacatccttcttccgaaagttgaactgaactttgctgagctataataatcaatggctgcaagactaagtgcatcagcagaagttctggaaagaggttctagctacttggatgcgtaaacctttcaccttcaccaagcgccttcttcgggcaaatcagggccctagagagagctcgcccgtggcctgcaggtcaggagcccaatcctgccctggctgcctcgcctcccgaccacaggaaaccctccctccaaagacagggagagcgcgcgtccaccctccgcagacccgaggcccgctccgcccgg

SEQ ID NO: 8598 - RNA, 3221 nt, Homo sapiens
  source 1..3221: mol_type = other RNA
aaagactctgcaagatgccttgaagtctttttgctcaaattctccctttgcatgttggggctaaagcaaatctgggacaggagagagactggggaggcagtgggtgtggttattgaagaagttaatgtgggtaacaccagagatcctggaggtgatgacagtgttcttgcgtctttgggtaaggaaggtcttgttagttcacaactgcccatgggagaattttctccttctgtgcaaatatctgcaacactccctgaaaatgccagttgaattttctaacttcatattcttcagtaaagcatcgtagctcatctagttggaaagagacgactaccttcattaacagaaggtagaactcgccagaatgtaagatgatccagagatttcagagaaacttgtttctcgagtttcagtgctgacatcagggaaggcagctcattcataggctccctttgctaaactcgagatcaatgtagaaagaatcttagtcgaagcctaattcttcgtggattcatgctgtatggagtatcttggaaatataaatatgtaaatgttgaagaaatggagatgtgatcagaaatgtactttttttattgcactgacttgaatctttggccaaggcaggtggttcatgaggtcaagagttccagaccagcctggtcaacatagtgaaaccccatctctcctgctggttcttgttggcatggctcagtagatgagcctgtggctgctctcctttccccaggatctcctccagctctttcagctcctgggctaggtgtgtgcttagcaacaccacaaatggcaccaacctctgtaggacacccacatcgtttaggtagaagacagtaaaaactgccacagctttgtctgtgggttccagcttgtctttattctcttagtgttcactttcactacttgcttggcagtttagcattgtgtaagttatttgatttgttgctttgttggaatttattactttgttggaacttattccttgtgggatttctgatgtaaaagaaagtttgatttgtggcgaaatgttttctcacatttgttacattcataaggtttctctcctgtgtgtattttctgatgttcagtgagagtccacaggcgacggtaggttttcccacattgattacattcatatggtttctctcctgtgtgaattcttctatggactctgaaggctgacttatggcagaaggatttcccacattcattacattcatatggtttctccccagtgtgagttcgctgatgttcaacaaaggagaacttctgacagaaggttttcccacattcattacactcatagggtctctgtcctgtgtgtgttctctgatggtgagtcagggctgacttcctgcagtaggttctcccacattcattgcattcatatggtctctcccatatagttctctgatgtacaatgaggtgtgagtttttgctgacggcatgcccatgttcactacactcataaagattctcctttgtgttcattctcttacactgactgcagtttgacttcacaatggagattctaccacatttattaaacacaccatgtttctctcctgtgtgtgttctctgatgtatagtgagtgttgacttatggcagaaaaatttcccacattcattacattcataagacttctttcctctatgagttatctgatgtgcaatgagggctgatttcgtacataaaaattttccacattgactgcattcatagggcttctctcctgtatgacttcttcgatgcacattgagggcagattgacaaaagaaggttttctcacattcactacattcatagggtttttcccctgtgtgaattctctgatgcgcagtaagggctgactgacagaagaaggttttcccacattccttacattcatttggcttctctcctctgtgagttctttgatgtacaacaagatacgatttcttgctgaaggcatttccacattccttgcattcgtaaggcttctcccctgtgtgtgacctgaaatgttcagccagggctgacttccgaaaaaaggtctttccacattcattacactcataggatttctcccctccatgaattttctggtgtacaataagggcagatttgtcaatgaaggttttcctgcattcactgcattcatagggtctctctccagtatgaattcttcggtgtcgagtgaggcttgtcttcacacgaaaagttttcctacaatcactacaaacatacggtttctcccctgtatgaattctctgatgtacaatgagggtagatctcttagaaaaggttttcctacattcattacattcatttggtttcctttcagtctgtctccccttttgtgtaatgagaattgccctcttgaagaaggttttcccacatttattatagtcaaacggttgtttcaaaatctgaatgttctggtgcagaataagattttcgttttgattgctggctttcctcattggattgtatctgtattttttcattcccaaatgacttttctcatgcttcccaaatccactgtatccatcaggaatctttctgttttctttgcttttctttgcaacaattacttctgaattagttttcaaactgtttcctcctggattacatttatagggcatttttcttgagggaacactattcatgcccagattaagtgttttcccaaatacattctctctttctgtaatcagtgttttgttgctgaagaatacagtttgtgtcaaatgtttatcttggatttccttgttcttctctaaggcatcatcaatgtctgggtagttctgatttgagaattcctccactatccatggctcttctccttgctccaatttgaaaatcacatctggtttgctaacatgataccccacagagaccaagttgctgtagttctccagcatcacatccctgtacaggagcctctgagcagggtccagttgctgccattcctcttgggtgaagttcacagtcaggtcctggaatgaaactggtatctgaaagaaaatgtttaatcttgggtgaccaaaattgagtgatatcaaatgtatggtaacataaactataagaagaccactgccatggctaatggaaagctatagagagatgtaattgtgggagggcagaaaattaaaaatctgtcactgtgttcattttttaaaatgaattttaaaaatgtgctgagcttataccatgtcctggagct

SEQ ID NO: 8599 - RNA, 25 nt, Homo sapiens
  source 1..25: mol_type = other RNA
aaagatagacaattggctaaataga

SEQ ID NO: 8600 - RNA, 32 nt, Homo sapiens
  source 1..32: mol_type = other RNA
aaagatagacaattggctaaatagaaattgtg

SEQ ID NO: 8601 - RNA, 4598 nt, Homo sapiens
  source 1..4598: mol_type = other RNA
aaagatctggaagtgggagacagtatccgggtgttgtcacgtggttatggctttgactccttcttcattctattcttagctatcgaacttttctgatacatgacttaatgaaatgcaaaatttaatctaaatgcttttatggttcagagttgcattttttatggatagtgactgggcaatttttccacctcttggagcacaaacagaatctcacagggggcagtggcaagagtgagaggtggcagctgggcttctcaataaggctgtgcattaaaaacccataacctagcaaagggagtacaggtcagaccacacattttactttctttctcccatcaccgtatactcagtaccaagcacacacagcacctagtatctggcatgtagtatctgcttccacatgtatttgtaggctcttcattgtgatgaaattgagttgtaacaatgatggatcttatacttgatttctgtttgaatcgttttaaaatcccatattgctgattaaattatggggagaatccatagaaaggctgattaataagggcatgtcatgaattgattaattttaatgagcattttctgtgcccaaagcaactaagctttaactgggccctccctgacaattccagctcttctggattcccacggaatctggttcaagtactacctgctgttttcaaataaacttccccctctttgcagggaaaatgaagccacttcactgtgttccaactttcatgcaattctaccaacaatttctttattctgtctcatcacatcacaagagattaatccatttacctgtctctgatcttcatcctctctcaacttcttagggacctccctcctctatgttttccttccattttttctgctgatttcctctatcacatccactcatactcaaatgtttatcctctttcaaaaacaaaattaaacctacatcaatcttttacagccatcgtcccaccaatcccctcttctcatcacactcagaccaactggaaatactgtctttttaaacttacttatgcagacctaattttgctttaatctggcttccacctccactgctccactgaaatggctctgaccaagctaatgtcaatctccctcttgctaagtccattaatttagagcaagccttccctcactctctgcagcatctggtacagctgattatttcctcctccttgagctcttctcctcccctgctttccacaataccatactctcaagtttatccccctccttctgttccttcttggtctcctctccaggctcatttttctccttccatttctcaagtgttgatgttccacacagtttcgttgtaggctcactccccactaaccctatccactcttgttttgtccactcggctcatatcatccacttccaaggcctgagttaccacatgctccataaattaatgactttcatcgttatcttcagtccaaactgatcttctggcatccagatccaaaatgatgtcactacagagcagctccacttaggtatctcatcagtgcctcaagctcaacatttaaaacaaaattcatcatcctcccaaaacctgatctccacaatgactcctctatttcagtaaaaaaccattagtatcaagccaatcatccaaatagcattatcacctacttcatattcatgagtctcgggtttgtggtagttatcattagtaaacatttcctaaccccccaaacccagatgagctgctcttcctgtgtgcttccaggctttctgcagttcccctatcttagaacttaccccactgtattgtaactgcccatttccatgttcatattccccactcatctataacctccttgaggacaaggacatcgtctaacccagtatctctttattttatagatagatccaggacctagcacagtgcctggcttaatgtggtagaagttccataaatatttgttgaatgagattgctgacaccaaatgcaatgtaaataagagacacagcatctgctccaaaacagcagctgaacatttactattaaaaatacaaatttccaagcataacttaagacgtaccacattaaaatctttggggaagtcctgggaatccgtatttataatgaacataggagaataatttcacattaggtaagttgtggaactgtgctctgaaagaatttgattttttctgttggtacttatttaattacatctgacatatctgagggcgtacctattttgtaaatagtgagtgaagtaatagagcttcaaaatcagtacacagatctgccaggaatctaacaaggatctcaagaaagtagaaattcatgctatggaaaaagaaaggctggctattattttgcagtcttgaaaagatgagaattatatgctaatagtgatttctattaaaacaaaaccttgtcgacttgaaatcaatctcactgactgagatggtcaaattaagaaatataatctgttattcttaaaagtatttccttattagacacaaggtttcaaaaaaaaccttaaaatgaaactaaattcacagtcccattatcacaatgcctgtcctgtccagagttcccaaattgattctgtttttgtttttttttcttgttattttcacctacacttgagccattgagctgacagccaaagtaatcccaaggcagtctcctgacttgtcaccaaagctgtccagggacaatcgcaggcatgagtgctgaagaaagtggcatctgcctcattgtccctggcctccaacaactccaaccctataatgttgtttaatagtaaatcaaaagataatggagagccagcaggaagagtatcagagcaattagatacttggacaactctgctgcgagcaaaactggtcgtctttgagatgtgaactattttgaaccaatatcacaaatacaggatagaggaggactgtcttgatagcagttgaaaatggaaagagcctccaaatttcagggcgttcatacgtggcaacaatgtgatgtagcttgatcagtgcgtccatcatgaagggtggaaatggggatgcctgggccgtagcagacaagtgcatagtacttggcgtagtcgctgaaacttgctgtgtaatattggcacctttctttccttagatggcaagtaacacacttcttgcttggaggatagcttccaatgctaattctgtagatgtttcttcttccagggtattcttcaaattcattgctagaataaaacagtgaatcctgtgttactctgaatatatttatggcctcccacttgccacttgtaatttgaatagcattttccacagtgtctttgatatagtgaatatgtttgtagccatccttgtcactaaatattttgtagtacgaaatggcatcatagctgaaaactggtgttgaaacaaagaatccaccagcccatccagttctgctttcttctatatgctcctgggtctttggacaatcccatgtctgccagtcttccctgaagtcacatatagacaggaccgaaacattctggactctttttagccactgcaaacatactcgttcatcagtaacccacgtgagccaactgaaataataatcacttgaggctatcattgctggaacaggcacttcctggggacctacatacgcagggtaagtggtatcgataataaatatccgaacaacgggattcttagctccagcctttgggtatggaatatttattgttctaggatattgttcatcgccataataggaataggcaataactggtatatccgtatcattaaattccgcatatgccaaaaattttccattaggagaccaccagagagcatattttgtagcaagcatttcctcttcataaacccagtctgggattccattaaatattttattttctcttccattaaatgttatttgaaaaggtggatctcctggtctttgtttcaaatagatattgttttgatagacatatgctaatttactcccaacaggcgaccagcataaatactgaattggacgaggaagctcatttcctcttacaaattctccattgctaaggtcatagatgtaatatgttgctgtgtaagagtatctccaaagctttgaataatcactttctagatatacaaattgccgatcaggtgataagccgtaatttgaagcattcacacttttcatggttctattactcaaaatggtatatgattgtcctgtttcaatattataaagtactatattgttatctgcagattgatgaagatattcttgtcctgaaatccagtttggaaaaaatgttttataagaaaatgttccatttaaaatatccttcagtgtgagtgctctcattgtattttcttcagagttatgaactcttgaagggcgtaagacaatgcacatcaccaataaggcaagcacagcagaggtggcaactccaaatacgatttttacccaagtcttcatttttccagatgtttttgaaagttagctaattctgtcttcagagcgtgggtcactggatctgtgaaaaccgttgaaaaggaccaagtctgtctttgtagttggaagctgaagccaggacaaggtttttttctttccacggactttt

SEQ ID NO: 8602 - RNA, 25 nt, Homo sapiens
  source 1..25: mol_type = other RNA
aaagatggacaattggctaaataga

SEQ ID NO: 8603 - RNA, 32 nt, Homo sapiens
  source 1..32: mol_type = other RNA
aaagatggacaattggctaaatagaaattgtg

SEQ ID NO: 8604 - RNA, 1846 nt, Homo sapiens
  source 1..1846: mol_type = other RNA
aaagcgcttcccttcagagtgaggttcccgagggatgctggagggagggaggagctaccttgaggtgagagtgtgtccctgctcgcgtccactgggagatgcactgttaactcccatggtgtttctaaggacgcatgcttcaggggaggtctccacacaggtgtggattcttcgctgctttctggttctgactcagggtgtggagcacctcttctgtgggctttctcttttgggggttgtttggtgtggtaatgaatctccaccggtaagatgaagagctctgttgggggctcattggctttaaattggctcttcaggggctccaagactctgggtggttcttctgagataggaggtaatttcaaagcctttggtgcctttttcttcttcacttccccaggggtgattattctggagccagtggcagatgctacaggagggaagaggcttctttcagcaggaagcacctgtaacaagtggctgcttctggccttgtggagtttcacgttcctttgtttatcgctgagatctgccttcctattagggaaggcgcctccacagaatgtaatgtgggatttgtcacttgggagccaagagtgatcgatgcggccatgcccaaaggccttcctggaggtttgctgtgtcttttcattgtagctctcctttgaagcatataaacaaaggtgattctctattgacgtgtcctctgcctgcgtttcatcttcctgccagggctgcttcctgcgtggtggcaagcgagtcccctgactgccatggttcttggctagagggccctggtccacgtgtccagcagctccagcttccccttcatccaggccctgttgacgttgttcaaaagattttccttgttgaatccaaaatgaagggaagacaggcaggagatggtattttgggggtacacctgaaagatcttgttgtggcctgagcttctttggtacattaagttgactgtcctggagtagcacagaatccttgatgtatcctgcgcaccagagcctatacatggcgtctgggggccaagtccgcaggaggcctcggaggtatctcttggctgaatgccctggctggatctgccgttgggcctggctctccagctggcttcggaagtggaggtatggttgccaggctctgtcctgctctccctgctgccttccatatgccaggatggcttctttgaggtcttgaagtgtgtgcagttcaagatccagcttcctccagggacctctggggcagtaggggccttttctcctctctttgggtgtccatgccgaaatggcaaaaccttctgagtacaggatcagggcaccctttctagtactgaaagttttagggagaaagaggctccaggagtgctgactggcattgttcttatcttgaggtttgctgacaggaacatagtcttctggggacctccagttcaagtaatcctctggttcaaagtagacttctaacttctgtttgtcctggcccagcttcccgtggccccggctcaggagggagagcgtgaacatgtttccctctgaccaccccttctcaagggcagtccatcttggttttgaaggctgaaatctggtcacacctcaagatttccagagctcacagcaagcccaagaagaccacaaacacagggccttttattaaatacatttttccctctcgcagcagcttcttagtaacaaccagccacacagtttagacagtgtgtgtctttgtggagagaaaaaataaaccgcacagccagcctcctcaagccctggattgtctactctctgggcgacctgtctctccccttctcctgagctcttgttgtcccttggtcccggtt

SEQ ID NO: 8605 - RNA, 3603 nt, Homo sapiens
  source 1..3603: mol_type = other RNA
aaagctgggttgagaagggaaaaggaaaattgcagaggaagcagcaggagtgtgggggccatctcctctccccctttcctcagtttcccctggggtagggtgttccgtggaacaaggaacaagaagaagtttctacattaccacaaaatcagaatgaatattgaatacaagaagatggagtagacagggtccagattccaaagccactataccttggcatctagccagatggcttggccatttcattcgtcaaccatttatgctataactatgcattacaagctcaataaaagtctcaagagatgctaaaatttattaattccttaaacatttacttactgagcttccactataggccagatgttgtgctaattttggggataacatagtaaggaacgactcaaaccaacaaacaccaccaatacaagactgcggccctcttgagtctacagaaagtcaaggaagcaaaacacatgcacaggtaagtgtaaaaacgcacagctgtagtttaagtgccacaaagtagaggtacatgaacatttattctaagagcaatggggagccctatctgtgtccaatgcatggggacacaagaaggtatagtatatggggacattgcaggaatgtctctatggctggaagtcagagagtgctgggggcagagagatgctgaccatggaagacttctaagctaagctaatgtatttttgctttatacccaggaaattaagaggcatttactttaaacaaggagtgaatataaccatatttgtacaacataaaattcatcttggttgctgaatgaaggagggattatgatcccataagaaaagaagcaggagcccagttgggagaaaatgcaatagctgaagttgtgaatgaggatcctgctaaagtcacatcaatggggatagagaagtggatatgctagaaagacagtgaggaagaggatgggaggagagggaaggggaagggaagggagcggagcggaggggacgggagaggaggggaggaggagcaggttatggaggggaagtggggcagtgagattagagaggaggtggtgatgggtgaggacatccctgcttctggcatggtgtcttatgggatggtgagcttctcttttagcaagagaggtgattatgacagagagagagagacagagaatgaagcaaagctgggggcttctcaagtgttaaaaataccctacatcccacacacctccattaactcatcagaaaactcaaaacccaagacaaacttctgctcctctctgtaatttggctgtgagctcccttttctgggtcatgtatgagtccatgggtattttaaacatgagaaggacaaagggataaacctttatttctttttccagtcgtactatattgatttcaggtaagtgaaatgcggtgtcattttcttgtatgtgtcttgcaggatgcccatgggtgatggttagaggagatgatgggtgttggttggtaatcgtgaaagctacactgtgcagggatagggatgaggacaggaaccaagggtggcatatactggtgcttttagcttcttgggacatttgtccgtatttagacaggctgaaaaatttgaaatttcccttggttaattttttcaggaaaacaaaaacaaaacaagctccaatgccacattcaactctcaaatgccatagtcaggttggacttgtttggagtcatctcttttctagcactctgacatctttgggatgaactcagcttagaaaacaccttagaaaattcctttcctcttctctggtgattaatcaagggttttcctttccagacactgtgtggcttcagtctcctccttccaagtgcataggaatccccaatgtcctctgaggcttaatgcatcttaatcagtaaaaagaacgatcattaggaatcatacccataaaattgaagccacttaatcagcaccctgatacagtgtgcacacttaattacgatgattgccaagactggattcattgtcatgcatgttaacgacttgccttggtagctaactgatgtctgagatgactctagcgtaaaatggagagccagccaaccagtttccatggaaggctccaggtgccaatggacgatccccttcctcaagaggacccttgggcatttctcaaagatactcaggcagccctgctgaggaagaacaaggatggccatcagactttcagaggagaaattcataccccacgccgtacgagctgtcagactggaatatagatttcttatttagagaccgctttcctcctctgcaaggtgacttcacaaggacaactttctctgcactttgtggagttttccactaggattgatctacagccatcgaaaaccagaaatgtgaactctaaactaagataccaagcctctgcggtaaactttactcatagcaaaaggcaagatgggtccaaggcttcagaacaaaaagagaagagttccagagttccaggcaggaggctttgtttggcttctgtcaagactcatactttgaattttgattagtagaaaattacaaagtcttgctcaagtcttgtcttcattatatggtaagagctcttctcatagaattttctcctggatttctatatcaaatctgcaaagcttcaaggcagggaagaatatgttacaggtattgtcgctatctttacacaaagttatgaacgaacatatttgttggtttgacattttacgtttcaatcccccgggtgtttttgaggcagatgttggaggtctggacttcaataaacctggtggtaatgcactgggctgtgactccagaaaggaattttctgaaggccagaagtaaacagtgtgggacagcaggctgctctgccctcatgaaggagcattgcaggaggctagcttctgagtcagccctcactgcaaaacctgggagctgcccttctcgtcctgtccatctcagacaaatgtaggacatggacttgcctaattaagctctggtagcagacaggcacccctggcctctccactgccattttcttctcttcttctttgatgtggcttgataattcccactcctttcttctccctacctcttcccaaaatctgcagtttccaaaaatcagtgtgggctgtgctcacagggaagccacaacacacatactccggtgtgttcagaagaaattccttttctggctctgtttctagaaggtttctttgtcaatattgcagggatctttagggtttgctctccagatactagacttagagttcatcccagttgtgtgtgtccaaatcataagtggcagattaactcaggtacaaacctcaaagactggactaaatggatagttgaaaccaaaccttgttcgaggcacagttctgagaactttacaagtgtttcctcgtttagccttcataacagcccagctaggtaggtcctattatccccaatctgagctggcaaggacaggaggtgaagcccagccgatttctcaggtggtgcaggaaggcgcggcccagtcaatcacgttcatgccagaataactgattaaggtagcagcccttgaaacagccttgcctgtaggacgtgacctcccagaccctgtct

SEQ ID NO: 8606 - RNA, 3606 nt, Homo sapiens
  source 1..3606: mol_type = other RNA
aaagctgggttgagaagggaaaaggaaaattgcagaggaagcagcaggagtgtgggggccatctcctctccccctttcctcagtttcccctggggtagggtgttccgtggaacaaggaacaagaagaagtttctacattaccacaaaatcagaatgaatattgaatacaagaagatggagtagacagggtccagattccaaagccactataccttggcatctagccagatggcttggccatttcattcgtcaaccatttatgctataactatgcattacaagctcaataaaagtctcaagagatgctaaaatttattaattccttaaacatttacttactgagcttccactataggccagatgttgtgctaattttggggataacatagtaaggaacgactcaaaccaacaaacaccaccaatacaagactgcggccctcttgagtctacagaaagtcaaggaagcaaaacacatgcacaggtaagtgtaaaaacgcacagctgtagtttaagtgccacaaagtagaggtacatgaacatttattctaagagcaatggggagccctatctgtgtccaatgcatggggacacaagaaggtatagtatatggggacattgcaggaatgtctctatggctggaagtcagagagtgctgggggcagagagatgctgaccatggaagacttctaagctaagctaatgtatttttgctttatacccaggaaattaagaggcatttactttaaacaaggagtgaatataaccatatttgtacaacataaaattcatcttggttgctgaatgaaggagggattatgatcccataagaaaagaagcaggagcccagttgggagaaaatgcaatagctgaagttgtgaatgaggatcctgctaaagtcacatcaatggggatagagaagtggatatgctagaaagacagtgaggaagaggatgggaggagagggaaggggaagggaagggagcggagcggaggggacgggagaggaggggaggaggagcaggttatggaggggaagtggggcagtgagattagagaggaggtggtgatgggtgaggacatccctgcttctggcatggtgtcttatgggatggtgagcttctcttttagcaagagaggtgattatgacagagagagagagacagagaatgaagcaaagctgggggcttctcaagtgttaaaaataccctacatcccacacacctccattaactcatcagaaaactcaaaacccaagacaaacttctgctcctctctgtaatttggctgtgagctcccttttctgggtcatgtatgagtccatgggtattttaaacatgagaaggacaaagggataaacctttatttctttttccagtcgtactatattgatttcaggtaagtgaaatgcggtgtcattttcttgtatgtgtcttgcaggatgcccatgggtgatggttagaggagatgatgggtgttggttggtaatcgtgaaagctacactgtgcagggatagggatgaggacaggaaccaagggtggcatatactggtgcttttagcttcttgggacatttgtccgtatttagacaggctgaaaaatttgaaatttcccttggttaattttttcaggaaaacaaaaacaaaacaagctccaatgccacattcaactctcaaatgccatagtcaggttggacttgtttggagtcatctcttttctagcactctgacatctttgggatgaactcagcttagaaaacaccttagaaaattcctttcctcttctctggtgattaatcaagggttttcctttccagacactgtgtggcttcagtctcctccttccaagtgcataggaatccccaatgtcctctgaggcttaatgcatcttaatcagtaaaaagaacgatcattaggaatcatacccataaaattgaagccacttaatcagcaccctgatacagtgtgcacacttaattacgatgattgccaagactggattcattgtcatgcatgttaacgacttgccttggtagctaactgatgtctgagatgactctagcgtaaaatggagagccagccaaccagtttccatggaaggctccaggtgccaatggacgatccccttcctcaagaggacccttgggcatttctcaaagatactcaggcagccctgctgaggaagaacaaggatggccatcagactttcagaggagaaattcataccccacgccgtacgagctgtcagactggaatatagatttcttatttagagaccgctttcctcctctgcaaggtgacttcacaaggacaactttctctgcactttgtggagttttccactaggattgatctacagccatcgaaaaccagaaatgtgaactctaaactaagataccaagcctctgcggtaaactttactcatagcaaaaggcaagatgggtccaaggcttcagaacaaaaagagaagagttccagagttccaggcaggaggctttgtttggcttctgtcaagactcatactttgaattttgattagtagaaaattacaaagtcttgctcaagtcttgtcttcattatatggtaagagctcttctcatagaattttctcctggatttctatatcaaatctgcaaagcttcaaggcagggaagaatatgttacaggtattgtcgctatctttacacaaagttatgaacgaacatatttgttggtttgacattttacgtttcaatcccccgggtgtttttgaggcagatgttggaggtctggacttcaataaacctggtggtaatgcactgggctgtgactccagaaaggaattttctgaaggccagaagtaaacagtgtgggacagcaggctgctctgccctcatgaaggagcattgcaggaggctagcttctgagtcagccctcactgcaaaacctgggagctgcccttctcgtcctgtccatctcagacaaatgtaggacatggacttgcctaattaagctctggtagcagacaggcacccctggcctctccactgccattttcttctcttcttctttgatgtggcttgataattcccactcctttcttctccctacctcttcccaaaatctgcagtttccaaaaatcagtgtgggctgtgctcacagggaagccacaacacacatactccggtgtgttcagaagaaattccttttctggctctgtttctagaaggtttctttgtcaatattgcagggatctttagggtttgctctccagatactagacttagagttcatcccagttgtgtgtgtccaaatcataagtggcagattaactcaggtacaaacctcaaagactggactaaatggatagttgaaaccaaaccttgttcgaggcacagttctgagaactttacaagtgtttcctcgtttagccttcataacagcccagctaggtaggtcctattatccccacctgcagagcttccactctcctgaggaaggtcactgtgtgtcacccagcaggggtggctggattccatcctgaggcccagcacctggctatctgtgtccctggacatcccattgcgccacaagttttcctcttctacaagaccccctcaagtggccccagt

SEQ ID NO: 8607 - RNA, 3571 nt, Homo sapiens
  source 1..3571: mol_type = other RNA
aaagctgggttgagaagggaaaaggaaaattgcagaggaagcagcaggagtgtgggggccatctcctctccccctttcctcagtttcccctggggtagggtgttccgtggaacaaggaacaagaagaagtttctacattaccacaaaatcagaatgaatattgaatacaagaagatggagtagacagggtccagattccaaagccactataccttggcatctagccagatggcttggccatttcattcgtcaaccatttatgctataactatgcattacaagctcaataaaagtctcaagagatgctaaaatttattaattccttaaacatttacttactgagcttccactataggccagatgttgtgctaattttggggataacatagtaaggaacgactcaaaccaacaaacaccaccaatacaagactgcggccctcttgagtctacagaaagtcaaggaagcaaaacacatgcacaggtaagtgtaaaaacgcacagctgtagtttaagtgccacaaagtagaggtacatgaacatttattctaagagcaatggggagccctatctgtgtccaatgcatggggacacaagaaggtatagtatatggggacattgcaggaatgtctctatggctggaagtcagagagtgctgggggcagagagatgctgaccatggaagacttctaagctaagctaatgtatttttgctttatacccaggaaattaagaggcatttactttaaacaaggagtgaatataaccatatttgtacaacataaaattcatcttggttgctgaatgaaggagggattatgatcccataagaaaagaagcaggagcccagttgggagaaaatgcaatagctgaagttgtgaatgaggatcctgctaaagtcacatcaatggggatagagaagtggatatgctagaaagacagtgaggaagaggatgggaggagagggaaggggaagggaagggagcggagcggaggggacgggagaggaggggaggaggagcaggttatggaggggaagtggggcagtgagattagagaggaggtggtgatgggtgaggacatccctgcttctggcatggtgtcttatgggatggtgagcttctcttttagcaagagaggtgattatgacagagagagagagacagagaatgaagcaaagctgggggcttctcaagtgttaaaaataccctacatcccacacacctccattaactcatcagaaaactcaaaacccaagacaaacttctgctcctctctgtaatttggctgtgagctcccttttctgggtcatgtatgagtccatgggtattttaaacatgagaaggacaaagggataaacctttatttctttttccagtcgtactatattgatttcaggtaagtgaaatgcggtgtcattttcttgtatgtgtcttgcaggatgcccatgggtgatggttagaggagatgatgggtgttggttggtaatcgtgaaagctacactgtgcagggatagggatgaggacaggaaccaagggtggcatatactggtgcttttagcttcttgggacatttgtccgtatttagacaggctgaaaaatttgaaatttcccttggttaattttttcaggaaaacaaaaacaaaacaagctccaatgccacattcaactctcaaatgccatagtcaggttggacttgtttggagtcatctcttttctagcactctgacatctttgggatgaactcagcttagaaaacaccttagaaaattcctttcctcttctctggtgattaatcaagggttttcctttccagacactgtgtggcttcagtctcctccttccaagtgcataggaatccccaatgtcctctgaggcttaatgcatcttaatcagtaaaaagaacgatcattaggaatcatacccataaaattgaagccacttaatcagcaccctgatacagtgtgcacacttaattacgatgattgccaagactggattcattgtcatgcatgttaacgacttgccttggtagctaactgatgtctgagatgactctagcgtaaaatggagagccagccaaccagtttccatggaaggctccaggtgccaatggacgatccccttcctcaagaggacccttgggcatttctcaaagatactcaggcagccctgctgaggaagaacaaggatggccatcagactttcagaggagaaattcataccccacgccgtacgagctgtcagactggaatatagatttcttatttagagaccgctttcctcctctgcaaggtgacttcacaaggacaactttctctgcactttgtggagttttccactaggattgatctacagccatcgaaaaccagaaatgtgaactctaaactaagataccaagcctctgcggtaaactttactcatagcaaaaggcaagatgggtccaaggcttcagaacaaaaagagaagagttccagagttccaggcaggaggctttgtttggcttctgtcaagactcatactttgaattttgattagtagaaaattacaaagtcttgctcaagtcttgtcttcattatatggtaagagctcttctcatagaattttctcctggatttctatatcaaatctgcaaagcttcaaggcagggaagaatatgttacaggtattgtcgctatctttacacaaagttatgaacgaacatatttgttggtttgacattttacgtttcaatcccccgggtgtttttgaggcagatgttggaggtctggacttcaataaacctggtggtaatgcactgggctgtgactccagaaaggaattttctgaaggccagaagtaaacagtgtgggacagcaggctgctctgccctcatgaaggagcattgcaggaggctagcttctgagtcagccctcactgcaaaacctgggagctgcccttctcgtcctgtccatctcagacaaatgtaggacatggacttgcctaattaagctctggtagcagacaggcacccctggcctctccactgccattttcttctcttcttctttgatgtggcttgataattcccactcctttcttctccctacctcttcccaaaatctgcagtttccaaaaatcagtgtgggctgtgctcacagggaagccacaacacacatactccggtgtgttcagaagaaattccttttctggctctgtttctagaaggtttctttgtcaatattgcagggatctttagggtttgctctccagatactagacttagagttcatcccagttgtgtgtgtccaaatcataagtggcagattaactcaggtacaaacctcaaagactggactaaatggatagttgaaaccaaaccttgttcgaggcacagttctgagaactttacaagtgtttcctcgtttagccttcataacagcccagctaggtaggtcctattatccccacctgcagagcttccactctcctgaggaaggtcactgtgtgtcacctggctatctgtgtccctggacatcccattgcgccacaagttttcctcttctacaagaccccctcaagtggccccagttcag

SEQ ID NO: 8608 - RNA, 3631 nt, Homo sapiens
  source 1..3631: mol_type = other RNA
aaagctgggttgagaagggaaaaggaaaattgcagaggaagcagcaggagtgtgggggccatctcctctccccctttcctcagtttcccctggggtagggtgttccgtggaacaaggaacaagaagaagtttctacattaccacaaaatcagaatgaatattgaatacaagaagatggagtagacagggtccagattccaaagccactataccttggcatctagccagatggcttggccatttcattcgtcaaccatttatgctataactatgcattacaagctcaataaaagtctcaagagatgctaaaatttattaattccttaaacatttacttactgagcttccactataggccagatgttgtgctaattttggggataacatagtaaggaacgactcaaaccaacaaacaccaccaatacaagactgcggccctcttgagtctacagaaagtcaaggaagcaaaacacatgcacaggtaagtgtaaaaacgcacagctgtagtttaagtgccacaaagtagaggtacatgaacatttattctaagagcaatggggagccctatctgtgtccaatgcatggggacacaagaaggtatagtatatggggacattgcaggaatgtctctatggctggaagtcagagagtgctgggggcagagagatgctgaccatggaagacttctaagctaagctaatgtatttttgctttatacccaggaaattaagaggcatttactttaaacaaggagtgaatataaccatatttgtacaacataaaattcatcttggttgctgaatgaaggagggattatgatcccataagaaaagaagcaggagcccagttgggagaaaatgcaatagctgaagttgtgaatgaggatcctgctaaagtcacatcaatggggatagagaagtggatatgctagaaagacagtgaggaagaggatgggaggagagggaaggggaagggaagggagcggagcggaggggacgggagaggaggggaggaggagcaggttatggaggggaagtggggcagtgagattagagaggaggtggtgatgggtgaggacatccctgcttctggcatggtgtcttatgggatggtgagcttctcttttagcaagagaggtgattatgacagagagagagagacagagaatgaagcaaagctgggggcttctcaagtgttaaaaataccctacatcccacacacctccattaactcatcagaaaactcaaaacccaagacaaacttctgctcctctctgtaatttggctgtgagctcccttttctgggtcatgtatgagtccatgggtattttaaacatgagaaggacaaagggataaacctttatttctttttccagtcgtactatattgatttcaggtaagtgaaatgcggtgtcattttcttgtatgtgtcttgcaggatgcccatgggtgatggttagaggagatgatgggtgttggttggtaatcgtgaaagctacactgtgcagggatagggatgaggacaggaaccaagggtggcatatactggtgcttttagcttcttgggacatttgtccgtatttagacaggctgaaaaatttgaaatttcccttggttaattttttcaggaaaacaaaaacaaaacaagctccaatgccacattcaactctcaaatgccatagtcaggttggacttgtttggagtcatctcttttctagcactctgacatctttgggatgaactcagcttagaaaacaccttagaaaattcctttcctcttctctggtgattaatcaagggttttcctttccagacactgtgtggcttcagtctcctccttccaagtgcataggaatccccaatgtcctctgaggcttaatgcatcttaatcagtaaaaagaacgatcattaggaatcatacccataaaattgaagccacttaatcagcaccctgatacagtgtgcacacttaattacgatgattgccaagactggattcattgtcatgcatgttaacgacttgccttggtagctaactgatgtctgagatgactctagcgtaaaatggagagccagccaaccagtttccatggaaggctccaggtgccaatggacgatccccttcctcaagaggacccttgggcatttctcaaagatactcaggcagccctgctgaggaagaacaaggatggccatcagactttcagaggagaaattcataccccacgccgtacgagctgtcagactggaatatagatttcttatttagagaccgctttcctcctctgcaaggtgacttcacaaggacaactttctctgcactttgtggagttttccactaggattgatctacagccatcgaaaaccagaaatgtgaactctaaactaagataccaagcctctgcggtaaactttactcatagcaaaaggcaagatgggtccaaggcttcagaacaaaaagagaagagttccagagttccaggcaggaggctttgtttggcttctgtcaagactcatactttgaattttgattagtagaaaattacaaagtcttgctcaagtcttgtcttcattatatggtaagagctcttctcatagaattttctcctggatttctatatcaaatctgcaaagcttcaaggcagggaagaatatgttacaggtattgtcgctatctttacacaaagttatgaacgaacatatttgttggtttgacattttacgtttcaatcccccgggtgtttttgaggcagatgttggaggtctggacttcaataaacctggtggtaatgcactgggctgtgactccagaaaggaattttctgaaggccagaagtaaacagtgtgggacagcaggctgctctgccctcatgaaggagcattgcaggaggctagcttctgagtcagccctcactgcaaaacctgggagctgcccttctcgtcctgtccatctcagacaaatgtaggacatggacttgcctaattaagctctggtagcagacaggcacccctggcctctccactgccattttcttctcttcttctttgatgtggcttgataattcccactcctttcttctccctacctcttcccaaaatctgcagtttccaaaaatcagtgtgggctgtgctcacagggaagccacaacacacatactccggtgtgttcagaagaaattccttttctggctctgtttctagaaggtttctttgtcaatattgcagggatctttagggtttgctctccagatactagacttagagttcatcccagttgtgtgtgtccaaatcataagtggcagattaactcaggtacaaacctcaaagactggactaaatggatagttgaaaccaaaccttgttcgaggcacagttctgagaactttacaagtgtttcctcgtttagccttcataacagcccagctaggtaggtcctattatccccactgaccacccatgtttcattctcaccctgcagagcttccactctcctgaggaaggtcactgtgtgtcacccagcaggggtggctggattccatcctgaggcccagcacctggctatctgtgtccctggacatcccattgcgccacaagttttcctcttctacaagaccccctcaagtggccccagt

SEQ ID NO: 8609 - RNA, 2910 nt, Homo sapiens
  source 1..2910: mol_type = other RNA
aaagctgggttgagaagggaaaaggaaaattgcagaggaagcagcaggagtgtgggggccatctcctctccccctttcctcagtttcccctggggtagggtgttccgtggaacaaggaacaagaagaagtttctacattaccacaaaatcagaatgaatattgaatacaagaagatggagtagacagggtccagattccaaagccactataccttggcatctagccagatggcttggccatttcattcgtcaaccatttatgctataactatgcattacaagctcaataaaagtctcaagagatgctaaaatttattaattccttaaacatttacttactgagcttccactataggccagatgttgtgctaattttggggataacatagtaaggaacgactcaaaccaacaaacaccaccaatacaagactgcggccctcttgagtctacagaaagtcaaggaagcaaaacacatgcacaggtaagtgtaaaaacgcacagctgtagtttaagtgccacaaagtagaggtacatgaacatttattctaagagcaatggggagccctatctgtgtccaatgcatggggacacaagaaggtatagtatatggggacattgcaggaatgtctctatggctggaagtcagagagtgctgggggcagagagatgctgaccatggaagacttctaagctaagctaatgtatttttgctttatacccaggaaattaagaggcatttactttaaacaaggagtgaatataaccatatttgtacaacataaaattcatcttggttgctgaatgaaggagggattatgatcccataagaaaagaagcaggagcccagttgggagaaaatgcaatagctgaagttgtgaatgaggatcctgctaaagtcacatcaatggggatagagaagtggatatgctagaaagacagtgaggaagaggatgggaggagagggaaggggaagggaagggagcggagcggaggggacgggagaggaggggaggaggagcaggttatggaggggaagtggggcagtgagattagagaggaggtggtgatgggtgaggacatccctgcttctggcatggtgtcttatgggatggtgagcttctcttttagcaagagaggtgattatgacagagagagagagacagagaatgaagcaaagctgggggcttctcaagtgttaaaaataccctacatcccacacacctccattaactcatcagaaaactcaaaacccaagacaaacttctgctcctctctgtaatttggctgtgagctcccttttctgggtcatgtatgagtccatgggtattttaaacatgagaaggacaaagggataaacctttatttctttttccagtcgtactatattgatttcaggtaagtgaaatgcggtgtcattttcttgtatgtgtcttgcaggatgcccatgggtgatggttagaggagatgatgggtgttggttggtaatcgtgaaagctacactgtgcagggatagggatgaggacaggaaccaagggtggcatatactggtgcttttagcttcttgggacatttgtccgtatttagacaggctgaaaaatttgaaatttcccttggttaattttttcaggaaaacaaaaacaaaacaagctccaatgccacattcaactctcaaatgccatagtcaggttggacttgtttggagtcatctcttttctagcactctgacatctttgggatgaactcagcttagaaaacaccttagaaaattcctttcctcttctctggtgattaatcaagggttttcctttccagacactgtgtggcttcagtctcctccttccaagtgcataggaatccccaatgtcctctgaggcttaatgcatcttaatcagtaaaaagaacgatcattaggaatcatacccataaaattgaagccacttaatcagcaccctgatacagtgtgcacacttaattacgatgattgccaagactggattcattgtcatgcatgttaacgacttgccttggtagctaactgatgtctgagatgactctagcgtaaaatggagagccagccaaccagtttccatggaaggctccaggtgccaatggacgatccccttcctcaagaggacccttgggcatttctcaaagatactcaggcagccctgctgaggaagaacaaggatggccatcagactttcagaggagaaattcataccccacgccgtacgagctgtcagactggaatatagatttcttatttagagaccgctttcctcctctgcaaggtgacttcacaaggacaactttctctgcactttgtggagttttccactaggattgatctacagccatcgaaaaccagaaatgtgaactctaaactaagataccaagcctctgcggtaaactttactcatagcaaaaggcaagatgggtccaaggcttcagaacaaaaagagaagagttccagagttccaggcaggaggctttgtttggcttctgtcaagactcatactttgaattttgattagtagaaaattacaaagtcttgctcaagtcttgtcttcattatatggtaagagctcttctcatagaattttctcctggatttctatatcaaatctgcaaagcttgttcgaggcacagttctgagaactttacaagtgtttcctcgtttagccttcataacagcccagctaggtaggtcctattatccccacctgcagagcttccactctcctgaggaaggtcactgtgtgtcacccagcaggggtggctggattccatcctgaggcccagcacctggctatctgtgtccctggacatcccattgcgccacaagttttcctcttctacaagaccccctcaagtggccccagttcagactcccattgtagattgggtttt

SEQ ID NO: 8610 - RNA, 2848 nt, Homo sapiens
  source 1..2848: mol_type = other RNA
aaagctgggttgagaagggaaaaggaaaattgcagaggaagcagcaggagtgtgggggccatctcctctccccctttcctcagtttcccctggggtagggtgttccgtggaacaaggaacaagaagaagtttctacattaccacaaaatcagaatgaatattgaatacaagaagatggagtagacagggtccagattccaaagccactataccttggcatctagccagatggcttggccatttcattcgtcaaccatttatgctataactatgcattacaagctcaataaaagtctcaagagatgctaaaatttattaattccttaaacatttacttactgagcttccactataggccagatgttgtgctaattttggggataacatagtaaggaacgactcaaaccaacaaacaccaccaatacaagactgcggccctcttgagtctacagaaagtcaaggaagcaaaacacatgcacaggtaagtgtaaaaacgcacagctgtagtttaagtgccacaaagtagaggtacatgaacatttattctaagagcaatggggagccctatctgtgtccaatgcatggggacacaagaaggtatagtatatggggacattgcaggaatgtctctatggctggaagtcagagagtgctgggggcagagagatgctgaccatggaagacttctaagctaagctaatgtatttttgctttatacccaggaaattaagaggcatttactttaaacaaggagtgaatataaccatatttgtacaacataaaattcatcttggttgctgaatgaaggagggattatgatcccataagaaaagaagcaggagcccagttgggagaaaatgcaatagctgaagttgtgaatgaggatcctgctaaagtcacatcaatggggatagagaagtggatatgctagaaagacagtgaggaagaggatgggaggagagggaaggggaagggaagggagcggagcggaggggacgggagaggaggggaggaggagcaggttatggaggggaagtggggcagtgagattagagaggaggtggtgatgggtgaggacatccctgcttctggcatggtgtcttatgggatggtgagcttctcttttagcaagagaggtgattatgacagagagagagagacagagaatgaagcaaagctgggggcttctcaagtgttaaaaataccctacatcccacacacctccattaactcatcagaaaactcaaaacccaagacaaacttctgctcctctctgtaatttggctgtgagctcccttttctgggtcatgtatgagtccatgggtattttaaacatgagaaggacaaagggataaacctttatttctttttccagtcgtactatattgatttcaggtaagtgaaatgcggtgtcattttcttgtatgtgtcttgcaggatgcccatgggtgatggttagaggagatgatgggtgttggttggtaatcgtgaaagctacactgtgcagggatagggatgaggacaggaaccaagggtggcatatactggtgcttttagcttcttgggacatttgtccgtatttagacaggctgaaaaatttgaaatttcccttggttaattttttcaggaaaacaaaaacaaaacaagctccaatgccacattcaactctcaaatgccatagtcaggttggacttgtttggagtcatctcttttctagcactctgacatctttgggatgaactcagcttagaaaacaccttagaaaattcctttcctcttctctggtgattaatcaagggttttcctttccagacactgtgtggcttcagtctcctccttccaagtgcataggaatccccaatgtcctctgaggcttaatgcatcttaatcagtaaaaagaacgatcattaggaatcatacccataaaattgaagccacttaatcagcaccctgatacagtgtgcacacttaattacgatgattgccaagactggattcattgtcatgcatgttaacgacttgccttggtagctaactgatgtctgagatgactctagcgtaaaatggagagccagccaaccagtttccatggaaggctccaggtgccaatggacgatccccttcctcaagaggacccttgggcatttctcaaagatactcaggcagccctgctgaggaagaacaaggatggccatcagactttcagaggagaaattcataccccacgccgtacgagctgtcagactggaatatagatttcttatttagagaccgctttcctcctctgcaaggtgacttcacaaggacaactttctctgcactttgtggagttttccactaggattgatctacagccatcgaaaaccagaaatgtgaactctaaactaagataccaagcctctgcggtaaactttactcatagcaaaaggcaagatgggtccaaggcttcagaacaaaaagagaagagttccagagttccaggcaggaggctttgtttggcttctgtcaagactcatactttgaattttgattagtagaaaattacaaagtcttgctcaagtcttgtcttcattatatggtaagagctcttctcatagaattttctcctggatttctatatcaaatctgcaaagcttgttcgaggcacagttctgagaactttacaagtgtttcctcgtttagccttcataacagcccagctaggtaggtcctattatccccacctgcagagcttccactctcctgaggaaggtcactgtgtgtcacctggctatctgtgtccctggacatcccattgcgccacaagttttcctcttctacaagaccccctcaagtggccccagttcag

SEQ ID NO: 8611 - RNA, 2908 nt, Homo sapiens
  source 1..2908: mol_type = other RNA
aaagctgggttgagaagggaaaaggaaaattgcagaggaagcagcaggagtgtgggggccatctcctctccccctttcctcagtttcccctggggtagggtgttccgtggaacaaggaacaagaagaagtttctacattaccacaaaatcagaatgaatattgaatacaagaagatggagtagacagggtccagattccaaagccactataccttggcatctagccagatggcttggccatttcattcgtcaaccatttatgctataactatgcattacaagctcaataaaagtctcaagagatgctaaaatttattaattccttaaacatttacttactgagcttccactataggccagatgttgtgctaattttggggataacatagtaaggaacgactcaaaccaacaaacaccaccaatacaagactgcggccctcttgagtctacagaaagtcaaggaagcaaaacacatgcacaggtaagtgtaaaaacgcacagctgtagtttaagtgccacaaagtagaggtacatgaacatttattctaagagcaatggggagccctatctgtgtccaatgcatggggacacaagaaggtatagtatatggggacattgcaggaatgtctctatggctggaagtcagagagtgctgggggcagagagatgctgaccatggaagacttctaagctaagctaatgtatttttgctttatacccaggaaattaagaggcatttactttaaacaaggagtgaatataaccatatttgtacaacataaaattcatcttggttgctgaatgaaggagggattatgatcccataagaaaagaagcaggagcccagttgggagaaaatgcaatagctgaagttgtgaatgaggatcctgctaaagtcacatcaatggggatagagaagtggatatgctagaaagacagtgaggaagaggatgggaggagagggaaggggaagggaagggagcggagcggaggggacgggagaggaggggaggaggagcaggttatggaggggaagtggggcagtgagattagagaggaggtggtgatgggtgaggacatccctgcttctggcatggtgtcttatgggatggtgagcttctcttttagcaagagaggtgattatgacagagagagagagacagagaatgaagcaaagctgggggcttctcaagtgttaaaaataccctacatcccacacacctccattaactcatcagaaaactcaaaacccaagacaaacttctgctcctctctgtaatttggctgtgagctcccttttctgggtcatgtatgagtccatgggtattttaaacatgagaaggacaaagggataaacctttatttctttttccagtcgtactatattgatttcaggtaagtgaaatgcggtgtcattttcttgtatgtgtcttgcaggatgcccatgggtgatggttagaggagatgatgggtgttggttggtaatcgtgaaagctacactgtgcagggatagggatgaggacaggaaccaagggtggcatatactggtgcttttagcttcttgggacatttgtccgtatttagacaggctgaaaaatttgaaatttcccttggttaattttttcaggaaaacaaaaacaaaacaagctccaatgccacattcaactctcaaatgccatagtcaggttggacttgtttggagtcatctcttttctagcactctgacatctttgggatgaactcagcttagaaaacaccttagaaaattcctttcctcttctctggtgattaatcaagggttttcctttccagacactgtgtggcttcagtctcctccttccaagtgcataggaatccccaatgtcctctgaggcttaatgcatcttaatcagtaaaaagaacgatcattaggaatcatacccataaaattgaagccacttaatcagcaccctgatacagtgtgcacacttaattacgatgattgccaagactggattcattgtcatgcatgttaacgacttgccttggtagctaactgatgtctgagatgactctagcgtaaaatggagagccagccaaccagtttccatggaaggctccaggtgccaatggacgatccccttcctcaagaggacccttgggcatttctcaaagatactcaggcagccctgctgaggaagaacaaggatggccatcagactttcagaggagaaattcataccccacgccgtacgagctgtcagactggaatatagatttcttatttagagaccgctttcctcctctgcaaggtgacttcacaaggacaactttctctgcactttgtggagttttccactaggattgatctacagccatcgaaaaccagaaatgtgaactctaaactaagataccaagcctctgcggtaaactttactcatagcaaaaggcaagatgggtccaaggcttcagaacaaaaagagaagagttccagagttccaggcaggaggctttgtttggcttctgtcaagactcatactttgaattttgattagtagaaaattacaaagtcttgctcaagtcttgtcttcattatatggtaagagctcttctcatagaattttctcctggatttctatatcaaatctgcaaagcttgttcgaggcacagttctgagaactttacaagtgtttcctcgtttagccttcataacagcccagctaggtaggtcctattatccccactgaccacccatgtttcattctcaccctgcagagcttccactctcctgaggaaggtcactgtgtgtcacccagcaggggtggctggattccatcctgaggcccagcacctggctatctgtgtccctggacatcccattgcgccacaagttttcctcttctacaagaccccctcaagtggccccagt

SEQ ID NO: 8612 - RNA, 2383 nt, Homo sapiens
  source 1..2383: mol_type = other RNA
aaagctgggttgagaagggaaaaggaaaattgcagaggaagcagcaggagtgtgggggccatctcctctccccctttcctcagtttcccctggggtagggtgttccgtggaacaaggaacaagaagaagtttctacattaccacaaaatcagaatgaatattgaatacaagaagatggagtagacagggtccagattccaaagccactataccttggcatctagccagatggcttggccatttcattcgtcaaccatttatgctataactatgcattacaagctcaataaaagtctcaagagatgctaaaatttattaattccttaaacatttacttactgagcttccactataggccagatgttgtgctaattttggggataacatagtaaggaacgactcaaaccaacaaacaccaccaatacaagactgcggccctcttgagtctacagaaagtcaaggaagcaaaacacatgcacaggtaagtgtaaaaacgcacagctgtagtttaagtgccacaaagtagaggtacatgaacatttattctaagagcaatggggagccctatctgtgtccaatgcatggggacacaagaaggtatagtatatggggacattgcaggaatgtctctatggctggaagtcagagagtgctgggggcagagagatgctgaccatggaagacttctaagctaagctaatgtatttttgctttatacccaggaaattaagaggcatttactttaaacaaggagtgaatataaccatatttgtacaacataaaattcatcttggttgctgaatgaaggagggattatgatcccataagaaaagaagcaggagcccagttgggagaaaatgcaatagctgaagttgtgaatgaggatcctgctaaagtcacatcaatggggatagagaagtggatatgctagaaagacagtgaggaagaggatgggaggagagggaaggggaagggaagggagcggagcggaggggacgggagaggaggggaggaggagcaggttatggaggggaagtggggcagtgagattagagaggaggtggtgatgggtgaggacatccctgcttctggcatggtgtcttatgggatggtgagcttctcttttagcaagagaggtgattatgacagagagagagagacagagaatgaagcaaagctgggggcttctcaagtgttaaaaataccctacatcccacacacctccattaactcatcagaaaactcaaaacccaagacaaacttctgctcctctctgtaatttggctgtgagctcccttttctgggtcatgtatgagtccatgggtattttaaacatgagaaggacaaagggataaacctttatttctttttccagtcgtactatattgatttcaggtaagtgaaatgcggtgtcattttcttgtatgtgtcttgcaggatgcccatgggtgatggttagaggagatgatgggtgttggttggtaatcgtgaaagctacactgtgcagggatagggatgaggacaggaaccaagggtggcatatactggtgcttttagcttcttgggacatttgtccgtatttagacaggctgaaaaatttgaaatttcccttggttaattttttcaggaaaacaaaaacaaaacaagctccaatgccacattcaactctcaaatgccatagtcaggttggacttgtttggagtcatctcttttctagcactctgacatctttgggatgaactcagcttagaaaacaccttagaaaattcctttcctcttctctggtgattaatcaagggttttcctttccagacactgtgtggcttcagtctcctccttccaagtgcataggaatccccaatgtcctctgaggcttaatgcatcttaatcagtaaaaagaacgatcattaggaatcatacccataaaattgaagccacttaatcagcaccctgatacagtgtgcacacttaattacgatgattgccaagactggattcattgtcatgcatgttaacgacttgccttggtagctaactgatgtctgagatgactctagcgtaaaatggagagccagccaaccagtttccatggaaggctccaggtgccaatggacgatccccttcctcaagaggacccttgggcatttctcaaagatactcaggcagcccttgttcgaggcacagttctgagaactttacaagtgtttcctcgtttagccttcataacagcccagctaggtaggtcctattatccccacctgcagagcttccactctcctgaggaaggtcactgtgtgtcacctggctatctgtgtccctggacatcccattgcgccacaagttttcctcttctacaagaccccctcaagtggccccagttcag

SEQ ID NO: 8613 - RNA, 2004 nt, Homo sapiens
  source 1..2004: mol_type = other RNA
aaagctgggttgagaaggtttatggaggtttggccagtgttgggactcaaagcttcaggcatcttttctgacacactagggaactctggggacttagccatctgctgccatcggctgctgcaataatgctttttgtgcactagataattatccaaattattgaatgttatgttacactcaaaacaagtagcccccttgggcatcaaagggctgtaaatgacgggagggtagctactactgccatgcctcagtcgccgatgcaccagttcagacatcttagctaagatctctgaagcttgagggaccatggtgatatcttgggggaaagaaaactgagataggaaagggcccacagggaaagaaggcccaatattaggctgaactggagatgaggcaagtcttgggctagagggctcagactttatttttgtgtaagaaaagctttgtttatttgttgtaggctgtatctctggtctctggttcgtgagaaagagctgagtctttttctcacacttgtccagctctgtgtcagagctcgcatctttagtctgcatggccttttggctctggggaagttcgcttctggtcaataagtctgtggctggctgtaagctgtcttcagttgcacttggagagtgttccatgtcactttctctgggaagtttgccgctagggacatggagctcctggtgctgcaataactccctctgagtctggaagccgaaatggcagtgattacatcggaaggcagcttgagtgagatgggagaacaggtgttggtgaaagttgatcacggaatcagcagtgtagctacagacggtgcattttagactagcaccagggggcaggaattcttccattttcactccactgtgtgaattcaggtgcatttctagagctcgagcatttgaaaagctcttggtgcactgtgggaaggggcacaggctggaaatctgatgggcactgtcttcattttcctctgacaccggagcagcttctctttgcctcccactgcagtagtacatcaaatgggcctgcagattccgctcactccgataccagatgccacaggacttgcaagggaatatatccttattgacaatagctgtgggcaaaatagaagccatggcagcttgctgaggaagcagctgaattgagtccagcaggcgtgcagggtacatcccttctgtgagagtcatctgactggcagcttgtagccttgagtcaaaatccaccacaaaggcaattagctcttcaccctcagagatggccttcgtagttgtacaccaaagctgaccccctttgctgtacacaatgcagttgtttttgttgtcttccactccttgccaagtcacatccagcaaccacttgggaccagcagtcagcaccattgggacctgagcctttgtcttcaaagaattattattcaagtccatcttcccaggaaacggcccccaggttgttcccactggaagttgctgtcgactctgaatttttcgttccccatctttctgaaacacctccagctctcctggtccatcccagtcgtctgtctcaactccaggttgccccggtttctctgactgtgtgtccccatctgattctgctgtctcctggattccttcatcatcacctttgttacaaaagtattccacttcttcgcagctcagattttcaggcccaaattctgtggaaaagctttcctccaatggaaagtctcctttggagatgatgtctgtttcctctgatggacattcttcttcctcatcttcaatggcatcttcaagcggccagcttccgcgctgggaagtgactggcggcccctcccagggaggactccgcgcgccaccagggccagacaccacccgaatccccgctcggctgagcgtcctggcggcgtgagccggacccgcccgaagtcccaggacacgacctgccagccaccagcccgcgcccgcagggcagagacgcacggccgcccgccgcagaggcgcgaacttttac

SEQ ID NO: 8614 - RNA, 2336 nt, Homo sapiens
  source 1..2336: mol_type = other RNA
aaagctgggttgagaaggtttatggaggtttggccagtgttgggactcaaagcttcaggcatcttttctgacacactagggaactctggggacttagccatctgctgccatcggctgctgcaataatgctttttgtgcactagataattatccaaattattgaatgttatgttacactcaaaacaagtagcccccttgggcatcaaagggctgtaaatgacgggagggtagctactactgccatgcctcagtcgccgatgcaccagttcagacatcttagctaagatctctgaagcttgagggaccatggtgatatcttgggggaaagaaaactgagataggaaagggcccacagggaaagaaggcccaatattaggctgaactggagatgaggcaagtcttgggctagagggctcagactttatttttgtgtaagaaaagctttgtttatttgttgtaggctgtatctctggtctctggttcgtgagaaagagctgagtctttttctcacacttgtccagctctgtgtcagagctcgcatctttagtctgcatggccttttggctctggggaagttcgcttctggtcaataagtctgtggctggctgtaagctgtcttcagttgcacttggagagtgttccatgtcactttctctgggaagtttgccgctagggacatggagctcctggtgctgcaataactccctctgagtctggaagccgaaatggcagtgattacatcggaaggcagcttgagtgagatgggagaacaggtgttggtgaaagttgatcacggaatcagcagtgtagctacagacggtgcattttagactagcaccagggggcaggaattcttccattttcactccactgtgtgaattcaggtgcatttctagagctcgagcatttgaaaagctcttggtgcactgtgggaaggggcacaggctggaaatctgatgggcactgtcttcattttcctctgacaccggagcagcttctctttgcctcccactgcagtagtacatcaaatgggcctgcagattccgctcactccgataccagatgccacaggacttgcaagggaatatatccttattgacaatagctgtgggcaaaatagaagccatggcagcttgctgaggaagcagctgaattgagtccagcaggcgtgcagggtacatcccttctgtgagagtcatctgactggcagcttgtagccttgagtcaaaatccaccacaaaggcaattagctcttcaccctcagagatggccttcgtagttgtacaccaaagctgaccccctttgctgtacacaatgcagttgtttttgttgtcttccactccttgccaagtcacatccagcaaccacttgggaccagcagtcagcaccattgggacctgagcctttgtcttcaaagaattattattcaagtccatcttcccaggaaacggcccccaggttgttcccactggaagttgctgtcgactctgaatttttcgttccccatctttctgaaacacctccagctctcctggtccatcccagtcgtctgtctcaactccaggttgccccggtttctctgactgtgtgtccccatctgattctgctgtctcctggattccttcatcatcacctttgttacaaaagtattccacttcttcgcagctcagattttcaggcccaaattctgtggaaaagctttcctccaatggaaagtctcctttggagatgatgtctgtttcctctgatggacattcttcttcctcatcttcaatggcatcttcaagcggccgtttgatctgccggggtttgctttgctttcgccgggacatctcggcggcggctgctgccgctggggctcccgcggtgcccgcggtcgcggctgccgctccctcggctcccgccgccgccgccgccgccgccgccgctggccaggctcggcccgccgccggccggactccaggtgctccgggcgctgggctcctccgggagccgcggattcacgttcggagatgagcaagcaaatgagagaagagagacgggggcacagagagtgtgacagtgaggaggggagggggagaggagagcgacggggggagaatgggaatgtacaagcgaacggtcagggagagagaaaaggggaaagagaagagaaaaataacacggaaagaaggaagagaaggagggagggacgggagagcgagcagcgaggagagggggagcgcgggggcgcagggcgcgggaggaggagcgcgctcgctcgcccctcgccccggcgtgcgggacggatactccggcgccgccgccgccgctccgggccgcgcagctcctgttct

SEQ ID NO: 8615 - RNA, 9151 nt, Homo sapiens
  source 1..9151: mol_type = other RNA
aaagctgggttgagaaggtttatggaggtttggccagtgttgggactcaaagcttcaggcatcttttctgacacactagggaactctggggacttagccatctgctgccatcggctgctgcaataatgctttttgtgcactagataattatccaaattattgaatgttatgttacactcaaaacaagtagcccccttgggcatcaaagggctgtaaatgacgggagggtagctactactgccatgcctcagtcgccgatgcaccagttcagacatcttagctaagatctctgaagcttgagggaccatggtgatatcttgggggaaagaaaactgagataggaaagggcccacagggaaagaaggcccaatattaggctgaactggagatgaggcaagtcttgggctagagggctcagactttatttttgtgtaagaaaagctttgtttatttgttgtaggctgtatctctggtctctggttcgtgagaaagagctgagtctttttctcacacttgtccagctctgtgtcagagctcgcatctttagtctgcatggccttttggctctggggaagttcgcttctggtcaataagtctgtggctggctgtaagctgtcttcagttgcacttggagagtgttccatgtcactttctctgggaagtttgccgctagggacatggagctcctggtgctgcaataactccctctgagtctggaagccgaaatggcagtgattacatcggaaggcagcttgagtgagatgggagaacaggtgttggtgaaagttgatcacggaatcagcagtgtagctacagacggtgcattttagactagcaccagggggcaggaattcttccattttcactccactgtgtgaattcaggtgcatttctagagctcgagcatttgaaaagctcttggtgcactgtgggaaggggcacaggctggaaatctgatgggcactgtcttcattttcctctgacaccggagcagcttctctttgcctcccactgcagtagtacatcaaatgggcctgcagattccgctcactccgataccagatgccacaggacttgcaagggaatatatccttattgacaatagctgtgggcaaaatagaagccatggcagcttgctgaggaagcagctgaattgagtccagcaggcgtgcagggtacatcccttctgtgagagtcatctgactggcagcttgtagccttgagtcaaaatccaccacaaaggcaattagctcttcaccctcagagatggccttcgtagttgtacaccaaagctgaccccctttgctgtacacaatgcagttgtttttgttgtcttccactccttgccaagtcacatccagcaaccacttgggaccagcagtcagcaccattgggacctgagcctttgtcttcaaagaattattattcaagtccatcttcccaggaaacggcccccaggttgttcccactggaagttgctgtcgactctgaatttttcgttccccatctttctgaaacacctccagctctcctggtccatcccagtcgtctgtctcaactccaggttgccccggtttctctgactgtgtgtccccatctgattctgctgtctcctggattccttcatcatcacctttgttacaaaagtattccacttcttcgcagctcagattttcaggcccaaattctgtggaaaagctttcctccaatggaaagtctcctttggagatgatgtctgtttcctctgatggacattcttcttcctcatcttcaatggcatcttcaagcggcctccacagcatcctaggatccacacacagagattctgtgtcagtgggtctgaggcaaatcccaccattctgctttgctaaccagcttcgaagtcatgttgatagctttggtccgtgcactgaccacactttgattagcactgccatcattgtctctgattctgggattggccacctctgcattctaggactgcatcacaattcagctctagtgacaactaagtcacatgaaagaatcctagcaaaagttgagaaatatgcattaaaaataaaccttggggccaggcatggtgagctgagatcatgccactgcactccagcctgggcgacagagcaagactccacctcagaaaaaaaaaaaaaatgaatcttgggatccctttgtaacatagttactgaaaccaaccctataaatgctgattttctagctccagttttacgacacactaggttatctccaattatctccaggggtgatataacagcttcacaaaattaattttactccattttaatttaacaaggttcacatctggaaaatgaatgcagaatttgttggttgaagtgaaagtaaagaacagctgaatccattaactctgctcctataacctaaagctctttgcttaattttgttaaattcattaaggattttgcttttaacttggaccttgtgcctcattctaatagagtggcaaaatgctatggtcaagttgcaaactatttatggaagggtaattataaatatgtaaaggctctgatgaacccagtaacaggcagtggcaggggtggcatcatcattctatggttaaggagatggatgacttacacgtccttccttttactaacgtgttcacttccaaagtcagttattgaaagtgaaaacgatagcccttaaaaactgatggtttatctctatttatctttaggttactggtaattgttttttaagggaatatacatttttttctaagtggcaaaaaattttctagaagaaacataaaccaactgactttgaaaaaaaaagtttgttataaatatatgacaaaatattcaataatgtctcccaattcatctctgtagctagttatggtttttaaatttgtagtctgattttataaatcaaacaagacctgaagtaaacgcttaccatctgcttaccacattgctatgagatgtaaggtttacataaaagcaaaaaggcataagaactctttgtgtgtacatgtgtgtccttaaaatgcttacattcttcatagggagaaaaagctaatatatatgtagaaaaaatacagaaaatgtgtcaaactgtctgacactattagtgaaacaagtataaaaaggaaaaattgctgtggattaggagaatactgaaaagcctcttgaaggatgtggaacttccactggaccttttcaatcagaaagatttatatgatggagaaaagacaggggcatcatatgaacaaaggcaagaggcagggactcacgtgtgtgtgctgggagatggggtctccagggagcagtactacttcaccggaacagaagccaggggcttgacagtaggagaaatagtttgcaaaaagcaaagtattgcaaattatgggaagtcctaaaacagggtagacaaattggacttgataaagtaggtaataaagagctatagcagactttcagcaatggcaatgacatgctgttaattgtttttagaagatcagcctggtagacttgaggaaggcaaaattacaagcaggatgaagcagtaagaggaggaaaacaggcaaatcagtgagtggtgccacttctcgaaaaggcaggcaagaaatagaaatggattgggtaaagaaatacatgctaaaaacattatagtcatcaactgtcgggggaaggagtaagcctcaacaactacagagaaaacaaaacaaactaaatatggaccagaaaggcacttctttgctgtcttttgaagtagaacattatttctgcacatgcaaactgtatatatatatcagtttctaagcatagctgtgaaaagggtcaatattcacagcatctggctttataggaagtgcaggcctgaagatgaaaagcaacacaactgcttacagtgtctcagattacagatccttttgatcttacaaaataaaaagcaataaatgggaaagaatccactgactatgtgtaatgaatcaaatagagctgtgtataacttttattgattgccagtcagccatttattaatatttaattaggaccaactatgtacaagccaatgtgttaggtgccatggatgatgggaacatagaagaggtcagctgacaacttccccaagcaccacaaatacatagaaacctgtcttggccttctaaagcagtcatgaacttgaaaaccaagtgccaaagggaaatcactgtactctctcgaacaataacaaaactgctttatcctttactaaagaaagtttgaattacaggatgacaagaaaaggaggaattctgaaagtggaaagtttaaccactgtgtttgttacaattccctttcacaaaaacttccatgtaaggagttataattctatagcttttatagttcaaaaagaagtaatcaaaccaggtgttgattacaggagagaaaagagggaaggagagagatggggcgtgctttatcttttcccagtattatactttcagtacaagaagcatacattttcaccagttcattacaaaatctgatgacatctacatgttcaaacacatattccatttaaatgaatgcattgtgattattataattaagttcgtacctgaaatttataaaatatgctgcaacacacactgtagttttttttatttaggaatcacctaaactatgttggtcaaaatgcctttggacatattccctacatatacaaatataaatggcaatacatgaatgggcttgtgagcaatctcttgtcatttcctcttttccatccaacagagggaaattaaataagaaaacaaaagcaagtaaaaatagataatattaacagcatcttaaaattttaagtactctccgatcataaaattaaaaagcatgcttgtttgttaaaaggcacagtaaatggaattattactgtaaaatgttaaggtacacagctctataatggcccaacttccttcaagttttcaagtaggaaattttctagaatttaaaagaacaaaactattacccaacatgaacacattaattagccagcaaaaaaagataccataagaaaggattaaagaatttgtgtctgaagaattttcagtgcaaaactccttagcatagtatgacaggagaataagaatgaaaaatgacagttcttaccagttagaataaaaatagcttgtcaatagtgacttctaaaactaaaacttcaaacatccttagcgatatattttattttgccaaataaaagcatagtaggaatgcaacaaactgttaatacagagaaagaatttttaaatgattttacaacaacactgaattgttcatattttccgtgaataaattctcatgttaaaaaacagtgtcaatttttatattatgaaaattgcaataaaatagcatgttacatctgaaaatatagaaactttagaacatttgattttttgttgccgctgttttttgtgtttttcttttttttcttttgagacagagtcttgctctgtcgcccaggctggagtgcagtggcgccatctcggctcacttcaagctccgccacccgggttcatgccattctcctgcctcagcctcccgagtaggtgggaccacaggtgcgtgccaccatgcccagctaattttttgtatttttagtagagacagggtttcaccatgttagccaagatggtctcgatctcctgacctcatgataaaatatcatcctactacatacaatgttcaaaactcaaaattgcgttgcttctcattttactgtgtgtggttttgtactaaaattaaatgcatcagacagaacacaattaaggaatggaagagtagttatctgttttatcctctttgaacatacagatgttcaatgatcatacctcaccaatacatgcctactgccactcatgtttcactttccaaatactcagggtttaaaacagagcagactgcacttttgataacatctgctacaacaaataacaaaaaaagagtgtgaagtctgatgaatgtttaaacagaacattttttatggatcagctaaatcttttctgctttttaattaaaagtaaagaaaatggaacttaattatcctgtaaagattagcttgtgggcatcttcctgtaaattacttctaattgaaagcaaattgtcaagtgacattcaaagtactgtcctttaaaacacagctgttctactgctgatttcagtgcattgcagtgttttcttgttacaatacggcatatttgaatattttaacaatttcactggtttgtatagatttccgtttaacatatcttaatcacatttcttcgtgtaaaaaagttagcatccttaagtggtttgcagcctccttaagtaagctatcatgagtgctctccactgaggtttacttttttttatttgcttgcttagagtaccacatctggacaacgatgatccaggaagtgggtggtcatactccttagaatacagccacaatccaactctttatgatacctgtataattaagccacagtttattgatgttttaaaacatactacaagttcaagtgaaattcttactagaaactaaaaacaaacaacttttcataatttagcacttagaataaaactccggtccttttaaaaaattttaagcaaacactaaagggcaatgtgaagactgctaacataggagttctaatgataaacgttaatatgaagatggataagaagcaaataaggagtataaatgcattaacccactaaaatatatttctgcttctatccagttatatatttaactatccactaactattgctaattagctactattgcctagcactgtattcagttctggagatgtagccaaaaaataaaagagtcacagttctaatggaatttacattccagaaaaggagaaaagaaaattaaacctacatagttttttggtgtcagggactacctggattcctgggcataggttgtttaaaacatctaacaacaacaacaacaaaaatccttgcctgtgtagtgttcttatttcagttgatggtaagtgctttgaaaaaaatatcagaatatggtgataaccagtcacacaaaaggaggcactatcgtatatggggtgaccaggaaaggactctctactagggggacatctgaacagaacacagagtgaattgagtgccagggagacccaagcacagtgcagtatgagagtatggggtggggggatcccttcagaagcattagggaagtctctaggaaggagacctctgatacccaagaaagtagtgtgaaaaaggtgaaagttaggaaggtaaaagattattcatcataatgttggaaggtttatgtttttgcttagacagtaggatgactcaaaccacaaacccaactaataacactttaattctctaggtagtatgttttcaagctgtgtacttagctcaaagcctatacaacacatttatcttatttttacatattgatgtgctaatgttgtgctccacagtgaaacaatctgtatgagttgctctcactgtaactgactggtatagacgaataggtaggtaggtaggttagctggtaatcaagcaggcaggtaggcaggcaggcaggcaggcatacagataaggtttaaatgttaaatgttaacatttttcagtaagcaaaaagccaccttacaacaatgcaggacaaaaatctgaaccacaatttgggctctgcttctcatggcaatatttatggagacatctgagaaaggataaccagaaagcaaacttctgagtcttattttcatctgctcgagcaaatcagcagatccagataataaaagggtcaaagacaggtaaaaaaaaaaaaacggtaaaatgggaacttctggatgtcttttagtcgtgccaaaagaactgaaaaaacaatgtaaaaaaggaggatgttctggactcttttccaattaaaatcatgttcttcattaatactgaattaatgtgggctaatgggttaatataaatgctattacttttaacaaaattcactgaagaatgttaagaaaaactatgtcctagtaatcatataaattataattgatattgttattgtgtattaaataagcagtttagagcatataatgaaagaacagggatattttaattcggtatttaaaacttgtcaaaataagtttctactatggtttcaaagttaaaatgtcattttcataaagaaacatttaaaccatccaacaatgtgcaaaatcaacacaacactatatattttgtaaccaaggcttagttccaaacgtaagatgcatgaagtttaggaagtgatgcatccattggccataattaagctcagcttaaaaaactcattctaaattagtggctttctcatttcggcatgcaaccatttgcagggcatcttaaaaccctgaatcctgggtgcccctctcaagattctggctccaagtctggaatgtacttcagtaatgtgcatttctaacgagctctgaggggatgctgatgctactgccagaccctagaaaaatgcccatctttttagttaaataatttctccattgattaaatatcgaaagttttgcttttaatataaaatagagccttttttccaaagggaaaaatgacctcccatctttttcacagcaatgaatttgaatattaaaaaaaaaacaacatatatttggttcagagaataaagaattatttcttccctatgaatagcccagatttcatcatttacacttttaatcagcaatattatctgtaaaccaaatttagtcattaaaaggaggataaccagaaagcaaaattctgagtcttattctcatctgctcaagcaaatcaggagaaccagttaatgtatctcatggcaattctgattccaatgaaaggattctgagtcaggatcttttacgtaagtacaaagttgaatttgcacctaaaaattctagttaaatttgatgtacagtcagccctccttatctgaggtttccacatcccagaattcaatcaatcatggattggaaatatttacatacacacacacacacaaacacacacacacacacacacacacacacgaaataatgcaactataaaagagaacactaattttaaaatatagtatagcaactatttacatagtatttacattgtattaggtaccataagtaata

SEQ ID NO: 8616 - RNA, 2177 nt, Homo sapiens
  source 1..2177: mol_type = other RNA
aaagctgggttgagaaggtttatggaggtttggccagtgttgggactcaaagcttcaggcatcttttctgacacactagggaactctggggacttagccatctgctgccatcggctgctgcaataatgctttttgtgcactagataattatccaaattattgaatgttatgttacactcaaaacaagtagcccccttgggcatcaaagggctgtaaatgacgggagggtagctactactgccatgcctcagtcgccgatgcaccagttcagacatcttagctaagatctctgaagcttgagggaccatggtgatatcttgggggaaagaaaactgagataggaaagggcccacagggaaagaaggcccaatattaggctgaactggagatgaggcaagtcttgggctagagggctcagactttatttttgtgtaagaaaagctttgtttatttgttgtaggctgtatctctggtctctggttcgtgagaaagagctgagtctttttctcacacttgtccagctctgtgtcagagctcgcatctttagtctgcatggccttttggctctggggaagttcgcttctggtcaataagtctgtggctggctgtaagctgtcttcagttgcacttggagagtgttccatgtcactttctctgggaagtttgccgctagggacatggagctcctggtgctgcaataactccctctgagtctggaagccgaaatggcagtgattacatcggaaggcagcttgagtgagatgggagaacaggtgttggtgaaagttgatcacggaatcagcagtgtagctacagacggtgcattttagactagcaccagggggcaggaattcttccattttcactccactgtgtgaattcaggtgcatttctagagctcgagcatttgaaaagctcttggtgcactgtgggaaggggcacaggctggaaatctgatgggcactgtcttcattttcctctgacaccggagcagcttctctttgcctcccactgcagtagtacatcaaatgggcctgcagattccgctcactccgataccagatgccacaggacttgcaagggaatatatccttattgacaatagctgtgggcaaaatagaagccatggcagcttgctgaggaagcagctgaattgagtccagcaggcgtgcagggtacatcccttctgtgagagtcatctgactggcagcttgtagccttgagtcaaaatccaccacaaaggcaattagctcttcaccctcagagatggccttcgtagttgtacaccaaagctgaccccctttgctgtacacaatgcagttgtttttgttgtcttccactccttgccaagtcacatccagcaaccacttgggaccagcagtcagcaccattgggacctgagcctttgtcttcaaagaattattattcaagtccatcttcccaggaaacggcccccaggttgttcccactggaagttgctgtcgactctgaatttttcgttccccatctttctgaaacacctccagctctcctggtccatcccagtcgtctgtctcaactccaggttgccccggtttctctgactgtgtgtccccatctgattctgctgtctcctggattccttcatcatcacgtttgatctgccggggtttgctttgctttcgccgggacatctcggcggcggctgctgccgctggggctcccgcggtgcccgcggtcgcggctgccgctccctcggctcccgccgccgccgccgccgccgccgccgctggccaggctcggcccgccgccggccggactccaggtgctccgggcgctgggctcctccgggagccgcggattcacgttcggagatgagcaagcaaatgagagaagagagacgggggcacagagagtgtgacagtgaggaggggagggggagaggagagcgacggggggagaatgggaatgtacaagcgaacggtcagggagagagaaaaggggaaagagaagagaaaaataacacggaaagaaggaagagaaggagggagggacgggagagcgagcagcgaggagagggggagcgcgggggcgcagggcgcgggaggaggagcgcgctcgctcgcccctcgccccggcgtgcgggacggatactccggcgccgccgccgccgctccgggccgcgcagctcctgttct

SEQ ID NO: 8617 - RNA, 3456 nt, Homo sapiens
  source 1..3456: mol_type = other RNA
aaaggaaagtgtatcctaaaagtcaagggggtaaaacatcgtttcaaataaaaggcaatgactaactttgtgttgattaccgcagataggttaagtaaggtgaggactaagaactacacattgaaattggcagcaagaaagtccttgatgacactgacatgagcggtgttcctagagtggttggcttgagaagatgatttgagaggaaaagagaacaaagttatgggggtagctggtggggaagagagccaagaaaaattcttgttaagacagaaaaataacatgtttttatgtcaatggaaatgacccggtagaggggaaaatttgatgagaaaaaaattgataaaacaaaaatcatgagtaggaaatggggatgtcatctggcagaggagtttggttttagataggcatgtccagcggttctttattctcagtctacatgttctctctggttaattccggggcactaaaatcaaactaaatgcctccattggactgtggtgagcagaagggcacctacgttgtataaaagcatcattttgtggacaactcagctccagccagttgctgacaggtcaggagtaaggacacagctttgccagatctactttgtcaaaagaaccctggaaccctgattttatgtgagagttcccaatttttaaatgttcacaactaactcagaattaaatgaataaattttttaaatgcaccctgaaggccagagcacattagcaggttgaatcaaattgtggtctttatcctaggaaatcacatcgaggctcactattttaattaacatctcattttccacacagtagctggaatgagtttttaaaatacaaatctgattgtatcactaccctgctaaaaaatccttaagtggctttctcttgcacactagataaagtttaagttctataaaatagcttgtgccatgatcatgccaaagctaactttcccagcttcagctcttgctgttctccttttagacttgacactccagcgatggaacattccacaatttctcaggtacgccatgcccattatcgcttcctggtcatggcacatgggactttcactgcttgaaaaatttctgtattcctttttttctggttcatttctactaggtctttagatgtcagcttacacttttttttttctctaacctgcctggcctgctgccctctctccatgctaccttatgccaagtctttgttaagaacccttctctatgctctcgtcacaccgtatacttcctctagtagtgtaattaaataactcagtgttctataattacatgcaccttctttggagattactgagactctgagacctttggggttaggagtgactactatgaggcaagcatcaaataaataagtgatggaatttggtgctcttcatatctttacaccagcagtccctctcgattatttcctgctatgtagatgtctactggcccctcagattcaacatgcttccttctccatggaccagagaacttgaagtctctctcacacctcacatcagtcatcaccagattctattgaatatttcttgactatctcttaagtcttgctgctgttttctttccactaccactgtcttaggcaagactctctttatttctcactatttctgattactcaaaaatatatatctgtgtctataattcacttatttctgtcttccaacttattctcaacgctgctggcaaacccattcctggtttcttctgctttgaatgcttcactttctcctcctaggcatttgggtatagttcagatgctttaagagacatttctatccattcataatctaccctaccctacgtttacgttttttatctcctcccattttctcccctcaccacttacacaaaatgctctaaagataccaagcttatgacaatatcctaaacatagtttccatgctttgttctaaatgtattcacatatactattatttctgccaaaatggtgtttttatttctccagaaggacttttattcatcttcagaattcagttcaaacatcctctcatccagaaatcctttatttaatattttcctctaagagttactcacttcccctgagctacctttggttcttgtttatatttctattgtacttacttatatgtctttttcttcttctaaaccctgaggtccttaagaacagagactgagctttacctgtctctgatatttcagtgaccagaccatcacctaatgcatggtagtcatttacagactttgttagaatgaatggatgaataatggttatcccttgtcacacacagcttgaacttgccattgattctaagggcactgaatacccctgccctttgtatttacagcacttgccaaagcatttagtttttaacttacaaagaaataattaaacagaaaggatcctgttgccttgatcttgaaatcaataagcatttatcttatcatgccttctgcagagtagccaggaaaatctaagtgaaattgtgaggacgttgacattgcctttgctatcatcccagcttcccttttagaggtcatttcttcccttctgaaattgttcgctttctaaccttctttttatccccaacacttactgcatttcctcttctgggacacttcattttcttgtctcaaagtcatttatactctggcatcttgcctttcgcctggtgtctacctcatcaaggagcttttagtttttgaaggatggtgtttccttagtgttattctcattagatccatcttccaattctactgtagattttatacatgtaacttttttctcttgacaatcttgctcggggacattctgcttcctccagttgctgccactccacacagttcttctggttctgaggaacaatccagagagaggctctaatcttgctgagccagccactcctttctctctcatgacagagataacacacttcccacagctccacggtgtgctgaatcctggagagagacctcctccaggcacagggcatccttcctgtcatcccagggatgctattttctgttcctagagctctgacgcttaaaaatgtgctttggatctcaagcaagtcagtttgaaaattaggtttaaatgtaaccacactaacttctaaaaatagaattcatctacagctggacaatattgaaatgagtaaaaagagtaagaaacttgaggatcaagagaaaataatggtgggggcacctcaaattatagaactgatatctgggcttagcctttgttatttagttggtaacttgacctaagcatttacattctcagagtcccatttgcaggttagggtaagggtatgtttcccggtgcctcaaagccccatttagagatccctgatctcaattgttttgaaaccattacaacttccttttgaacctcaattttaaaaggtacacaaaatagttagaaagaatgaatagacctaatcttt

SEQ ID NO: 8618 - RNA, 3452 nt, Homo sapiens
  source 1..3452: mol_type = other RNA
aaaggaaagtgtatcctaaaagtcaagggggtaaaacatcgtttcaaataaaaggcaatgactaactttgtgttgattaccgcagataggttaagtaaggtgaggactaagaactacacattgaaattggcagcaagaaagtccttgatgacactgacatgagcggtgttcctagagtggttggcttgagaagatgatttgagaggaaaagagaacaaagttatgggggtagctggtggggaagagagccaagaaaaattcttgttaagacagaaaaataacatgtttttatgtcaatggaaatgacccggtagaggggaaaatttgatgagaaaaaaattgataaaacaaaaatcatgagtaggaaatggggatgtcatctggcagaggagtttggttttagataggcatgtccagcggttctttattctcagtctacatgttctctctggttaattccggggcactaaaatcaaactaaatgcctccattggactgtggtgagcagaagggcacctacgttgtataaaagcatcattttgtggacaactcagctccagccagttgctgacaggtcaggagtaaggacacagctttgccagatctactttgtcaaaagaaccctggaaccctgattttatgtgagagttcccaatttttaaatgttcacaactaactcagaattaaatgaataaattttttaaatgcaccctgaaggccagagcacattagcaggttgaatcaaattgtggtctttatcctaggaaatcacatcgaggctcactattttaattaacatctcattttccacacagtagctggaatgagtttttaaaatacaaatctgattgtatcactaccctgctaaaaaatccttaagtggctttctcttgcacactagataaagtttaagttctataaaatagcttgtgccatgatcatgccaaagctaactttcccagcttcagctcttgctgttctccttttagacttgacactccagcgatggaacattccacaatttctcaggtacgccatgcccattatcgcttcctggtcatggcacatgggactttcactgcttgaaaaatttctgtattcctttttttctggttcatttctactaggtctttagatgtcagcttacacttttttttttctctaacctgcctggcctgctgccctctctccatgctaccttatgccaagtctttgttaagaacccttctctatgctctcgtcacaccgtatacttcctctagtagtgtaattaaataactcagtgttctataattacatgcaccttctttggagattactgagactctgagacctttggggttaggagtgactactatgaggcaagcatcaaataaataagtgatggaatttggtgctcttcatatctttacaccagcagtccctctcgattatttcctgctatgtagatgtctactggcccctcagattcaacatgcttccttctccatggaccagagaacttgaagtctctctcacacctcacatcagtcatcaccagattctattgaatatttcttgactatctcttaagtcttgctgctgttttctttccactaccactgtcttaggcaagactctctttatttctcactatttctgattactcaaaaatatatatctgtgtctataattcacttatttctgtcttccaacttattctcaacgctgctggcaaacccattcctggtttcttctgctttgaatgcttcactttctcctcctaggcatttgggtatagttcagatgctttaagagacatttctatccattcataatctaccctaccctacgtttacgttttttatctcctcccattttctcccctcaccacttacacaaaatgctctaaagataccaagcttatgacaatatcctaaacatagtttccatgctttgttctaaatgtattcacatatactattatttctgccaaaatggtgtttttatttctccagaaggacttttattcatcttcagaattcagttcaaacatcctctcatccagaaatcctttatttaatattttcctctaagagttactcacttcccctgagctacctttggttcttgtttatatttctattgtacttacttatatgtctttttcttcttctaaaccctgaggtccttaagaacagagactgagctttacctgtctctgatatttcagtgaccagaccatcacctaatgcatggtagtcatttacagactttgttagaatgaatggatgaataatggttatcccttgtcacacacagcttgaacttgccattgattctaagggcactgaatacccctgccctttgtatttacagcacttgccaaagcatttagtttttaacttacaaagaaataattaaacagaaaggatcctgttgccttgatcttgaaatcaataagcatttatcttatcatgccttctgcagagtagccaggaaaatctaagtgaaattgtgaggacgttgacattgcctttgctatcatcccagcttcccttttagaggtcatttcttcccttctgaaattgttcgctttctaaccttctttttatccccaacacttactgcatttcctcttctgggacacttcattttcttgtctcaaagtcatttatactctggcatcttgcctttcgcctggtgtctcatcaaggagcttttagtttttgaaggatggtgtttccttagtgttattctcattagatccatcttccaattctactgtagattttatacatgtaacttttttctcttgacaatcttgctcggggacattctgcttcctccagttgctgccactccacacagttcttctggttctgaggaacaatccagagagaggctctaatcttgctgagccagccactcctttctctctcatgacagagataacacacttcccacagctccacggtgtgctgaatcctggagagagacctcctccaggcacagggcatccttcctgtcatcccagggatgctattttctgttcctagagctctgacgcttaaaaatgtgctttggatctcaagcaagtcagtttgaaaattaggtttaaatgtaaccacactaacttctaaaaatagaattcatctacagctggacaatattgaaatgagtaaaaagagtaagaaacttgaggatcaagagaaaataatggtgggggcacctcaaattatagaactgatatctgggcttagcctttgttatttagttggtaacttgacctaagcatttacattctcagagtcccatttgcaggttagggtaagggtatgtttcccggtgcctcaaagccccatttagagatccctgatctcaattgttttgaaaccattacaacttccttttgaacctcaattttaaaaggtacacaaaatagttagaaagaatgaatagacctaatcttt

SEQ ID NO: 8619 - RNA, 4366 nt, Homo sapiens
  source 1..4366: mol_type = other RNA
aaaggaaagtgtatcctaaaagtcaagggggtaaaacatcgtttcaaataaaaggcaatgactaactttgtgttgattaccgcagataggttaagtaaggtgaggactaagaactacacattgaaattggcagcaagaaagtccttgatgacactgacatgagcggtgttcctagagtggttggcttgagaagatgatttgagaggaaaagagaacaaagttatgggggtagctggtggggaagagagccaagaaaaattcttgttaagacagaaaaataacatgtttttatgtcaatggaaatgacccggtagaggggaaaatttgatgagaaaaaaattgataaaacaaaaatcatgagtaggaaatggggatgtcatctggcagaggagtttggttttagataggcatgtccagcggttctttattctcagtctacatgttctctctggttaattccggggcactaaaatcaaactaaatgcctccattggactgtggtgagcagaagggcacctacgttgtataaaagcatcattttgtggacaactcagctccagccagttgctgacaggtcaggagtaaggacacagctttgccagatctactttgtcaaaagaaccctggaaccctgattttatgtgagagttcccaatttttaaatgttcacaactaactcagaattaaatgaataaattttttaaatgcaccctgaaggccagagcacattagcaggttgaatcaaattgtggtctttatcctaggaaatcacatcgaggctcactattttaattaacatctcattttccacacagtagctggaatgagtttttaaaatacaaatctgattgtatcactaccctgctaaaaaatccttaagtggctttctcttgcacactagataaagtttaagttctataaaatagcttgtgccatgatcatgccaaagctaactttcccagcttcagctcttgctgttctccttttagacttgacactccagcgatggaacattccacaatttctcaggtacgccatgcccattatcgcttcctggtcatggcacatgggactttcactgcttgaaaaatttctgtattcctttttttctggttcatttctactaggtctttagatgtcagcttacacttttttttttctctaacctgcctggcctgctgccctctctccatgctaccttatgccaagtctttgttaagaacccttctctatgctctcgtcacaccgtatacttcctctagtagtgtaattaaataactcagtgttctataattacatgcaccttctttggagattactgagactctgagacctttggggttaggagtgactactatgaggcaagcatcaaataaataagtgatggaatttggtgctcttcatatctttacaccagcagtccctctcgattatttcctgctatgtagatgtctactggcccctcagattcaacatgcttccttctccatggaccagagaacttgaagtctctctcacacctcacatcagtcatcaccagattctattgaatatttcttgactatctcttaagtcttgctgctgttttctttccactaccactgtcttaggcaagactctctttatttctcactatttctgattactcaaaaatatatatctgtgtctataattcacttatttctgtcttccaacttattctcaacgctgctggcaaacccattcctggtttcttctgctttgaatgcttcactttctcctcctaggcatttgggtatagttcagatgctttaagagacatttctatccattcataatctaccctaccctacgtttacgttttttatctcctcccattttctcccctcaccacttacacaaaatgctctaaagataccaagcttatgacaatatcctaaacatagtttccatgctttgttctaaatgtattcacatatactattatttctgccaaaatggtgtttttatttctccagaaggacttttattcatcttcagaattcagttcaaacatcctctcatccagaaatcctttatttaatattttcctctaagagttactcacttcccctgagctacctttggttcttgtttatatttctattgtacttacttatatgtctttttcttcttctaaaccctgaggtccttaagaacagagactgagctttacctgtctctgatatttcagtgaccagaccatcacctaatgcatggtagtcatttacagactttgttagaatgaatggatgaataatggttatcccttgtcacacacagcttgaacttgccattgattctaagggcactgaatacccctgccctttgtatttacagcacttgccaaagcatttagtttttaacttacaaagaaataattaaacagaaaggatcctgttgccttgatcttgaaatcaataagcatttatcttatcatgccttctgcagagtagccaggaaaatctaagtgaaattgtgaggacgttgacattgcctttgctatcatcccagcttcccttttagaggtcatttcttcccttctgaaattgttcgctttctaaccttctttttatccccaacacttactgcatttcctcttctgggacacttcattttcttgtctcatcaaggagcttttagtttttgaaggatggtgtttccttagtgttattctcattagatccatcttccaattctactgtagattttatacatgtaacttttttctcttgacaatcttcctccaaacatttaattcagaattctcaaggtttccaactgtcattttcattgcttcagcatgggtatttattgccatctgctcctgttccattcttcaattttacaattatatttccctgacaactttgtcagaaatctcaattgttctatcttgcctctatcaaatcatccagttaggttaacaaccaggtcaattccagcacaaagaacattggtgggttcacttctactattcagatggtatcaagttgggtttgcccagagaaacagaaccacaggaagtgatgtagaatcaattgtttattgcaaatattttacttttcccaattatgggagctgactaaacagtttatgtgtggctgttgcttctatgtcttgcattggagactgaagttagcagagcaggacatcgagaaggaaagacagacatgaaatgttggagagaaatgataaattggaattcagggggacaggctggaaatcacagaggcaaactgtttttcagcctctgtcttgaagcctccaaattcaatgatgccagtgacctgcaagagaaactgctttgcttcatcatgttgctaaacatgtaactgacccaggagctggagaaactgaaggaagcaaatctggtgagagctgatgaagctgcatgcccggcttctgctcaatgtcaataatgtgagccagagagcagaaatcacttggtgagctgcagtggtgcctgtgctctgcacttttgcctgcaccgatcttcagtgctttaaaggaatgtgattgacgcttaacttcagccttccaaatcccatcatgtgtgtttctggtggcccacgctaacctgaaattatgcagagacagggatcctgggaaacatagctcctgcttagctaaatttgcacagtgcaaatctaccatacaaactcattttttttaccctagagtcagtctgaattcatagttctatagtttttttctctcattctaaatctttaccaggttcctgaggtccactcttcagctctgttttggggagcacaggcctgatggctcttccctggcattgcagacacagattcagaaagacatgctgtggaggatggaaggaaaatgccatgttggaatcacagccttccccggattaggttgcttctccccttccccacttggggctgcagcatggttctcattgtagtttccaagtaaaccgcccttacttcctggcttcctctaatcagggtggcagggggatgtgtccacctctacagcagccttcctgtgttgacaacactgtttgttcttcccatctccctagggagaagctgccttatcttttccgtgcaatatgtttggaaaaaaacacatttttctctcttaaaggaattgattattgtgcttctcaagactataaagagaatatcttctggacccaaatactggctttaaaaaaataatctagattcctagattattcttagattattgcaagagaaggggatattttggtgattattggtagtgcattttgaatcactctatgcactaaaatatggcatttgagtatgtgtgtgtatgaaaaagagacagagagagacaaatacgaacagat

SEQ ID NO: 8620 - RNA, 3408 nt, Homo sapiens
  source 1..3408: mol_type = other RNA
aaaggaaagtgtatcctaaaagtcaagggggtaaaacatcgtttcaaataaaaggcaatgactaactttgtgttgattaccgcagataggttaagtaaggtgaggactaagaactacacattgaaattggcagcaagaaagtccttgatgacactgacatgagcggtgttcctagagtggttggcttgagaagatgatttgagaggaaaagagaacaaagttatgggggtagctggtggggaagagagccaagaaaaattcttgttaagacagaaaaataacatgtttttatgtcaatggaaatgacccggtagaggggaaaatttgatgagaaaaaaattgataaaacaaaaatcatgagtaggaaatggggatgtcatctggcagaggagtttggttttagataggcatgtccagcggttctttattctcagtctacatgttctctctggttaattccggggcactaaaatcaaactaaatgcctccattggactgtggtgagcagaagggcacctacgttgtataaaagcatcattttgtggacaactcagctccagccagttgctgacaggtcaggagtaaggacacagctttgccagatctactttgtcaaaagaaccctggaaccctgattttatgtgagagttcccaatttttaaatgttcacaactaactcagaattaaatgaataaattttttaaatgcaccctgaaggccagagcacattagcaggttgaatcaaattgtggtctttatcctaggaaatcacatcgaggctcactattttaattaacatctcattttccacacagtagctggaatgagtttttaaaatacaaatctgattgtatcactaccctgctaaaaaatccttaagtggctttctcttgcacactagataaagtttaagttctataaaatagcttgtgccatgatcatgccaaagctaactttcccagcttcagctcttgctgttctccttttagacttgacactccagcgatggaacattccacaatttctcaggtacgccatgcccattatcgcttcctggtcatggcacatgggactttcactgcttgaaaaatttctgtattcctttttttctggttcatttctactaggtctttagatgtcagcttacacttttttttttctctaacctgcctggcctgctgccctctctccatgctaccttatgccaagtctttgttaagaacccttctctatgctctcgtcacaccgtatacttcctctagtagtgtaattaaataactcagtgttctataattacatgcaccttctttggagattactgagactctgagacctttggggttaggagtgactactatgaggcaagcatcaaataaataagtgatggaatttggtgctcttcatatctttacaccagcagtccctctcgattatttcctgctatgtagatgtctactggcccctcagattcaacatgcttccttctccatggaccagagaacttgaagtctctctcacacctcacatcagtcatcaccagattctattgaatatttcttgactatctcttaagtcttgctgctgttttctttccactaccactgtcttaggcaagactctctttatttctcactatttctgattactcaaaaatatatatctgtgtctataattcacttatttctgtcttccaacttattctcaacgctgctggcaaacccattcctggtttcttctgctttgaatgcttcactttctcctcctaggcatttgggtatagttcagatgctttaagagacatttctatccattcataatctaccctaccctacgtttacgttttttatctcctcccattttctcccctcaccacttacacaaaatgctctaaagataccaagcttatgacaatatcctaaacatagtttccatgctttgttctaaatgtattcacatatactattatttctgccaaaatggtgtttttatttctccagaaggacttttattcatcttcagaattcagttcaaacatcctctcatccagaaatcctttatttaatattttcctctaagagttactcacttcccctgagctacctttggttcttgtttatatttctattgtacttacttatatgtctttttcttcttctaaaccctgaggtccttaagaacagagactgagctttacctgtctctgatatttcagtgaccagaccatcacctaatgcatggtagtcatttacagactttgttagaatgaatggatgaataatggttatcccttgtcacacacagcttgaacttgccattgattctaagggcactgaatacccctgccctttgtatttacagcacttgccaaagcatttagtttttaacttacaaagaaataattaaacagaaaggatcctgttgccttgatcttgaaatcaataagcatttatcttatcatgccttctgcagagtagccaggaaaatctaagtgaaattgtgaggacgttgacattgcctttgctatcatcccagcttcccttttagaggtcatttcttcccttctgaaattgttcgctttctaaccttctttttatccccaacacttactgcatttcctcttctgggacacttcattttcttgtctcatcaaggagcttttagtttttgaaggatggtgtttccttagtgttattctcattagatccatcttccaattctactgtagattttatacatgtaacttttttctcttgacaatcttgctcggggacattctgcttcctccagttgctgccactccacacagttcttctggttctgaggaacaatccagagagaggctctaatcttgctgagccagccactcctttctctctcatgacagagataacacacttcccacagctccacggtgtgctgaatcctggagagagacctcctccaggcacagggcatccttcctgtcatcccagggatgctattttctgttcctagagctctgacgcttaaaaatgtgctttggatctcaagcaagtcagtttgaaaattaggtttaaatgtaaccacactaacttctaaaaatagaattcatctacagctggacaatattgaaatgagtaaaaagagtaagaaacttgaggatcaagagaaaataatggtgggggcacctcaaattatagaactgatatctgggcttagcctttgttatttagttggtaacttgacctaagcatttacattctcagagtcccatttgcaggttagggtaagggtatgtttcccggtgcctcaaagccccatttagagatccctgatctcaattgttttgaaaccattacaacttccttttgaacctcaattttaaaaggtacacaaaatagttagaaagaatgaatagacctaatcttt

SEQ ID NO: 8621 - RNA, 33 nt, Homo sapiens
  source 1..33: mol_type = other RNA
aaaggcataaaaccaagacaagcaacaaaaaaa

SEQ ID NO: 8622 - RNA, 46 nt, Homo sapiens
  source 1..46: mol_type = other RNA
aaaggcataaaaccaagacaagcaacagaaaaactgacagcaaaag

SEQ ID NO: 8623 - RNA, 4060 nt, Homo sapiens
  source 1..4060: mol_type = other RNA
aaagtctcgctctctgcccctcagaaggacacagagccctggatgcagggaggctgtgagattgaaactggaagaacgcaagctccagctcacctcctagaagacttgcttgttaacagcaaagagaggagctccagaatccaggcagagccagggaaggaagtagataatgccagaactcatccctgagcagaaggaaggaacaacagattgaaagtgtcctctgattaccaaacatgatgaatgaggaacaaaaaggaaaaaaaaaaaaatctgtacctagttgcattgcagtgaaatttcagaactgtatggataaaagggggaaaatgtgaaagcttttagagagataaattaaaaaaagaaaaaaaattgctcccaacaaagggagaagagacaatagagtttctggtgaatgtaataataacagaacaatttgctgagaacattctttggacccaggtaatcggcatgggatttgtggaagccccatattttctccacttgaattgagaacagtttgaaagattagtaaaaggagtaaagcagatggagattaatgttttgcctttattactgcaaaaggttagtttggaggacttggcaaaaatgggtattttcccacccagggtaagtgctgagtgcctggcaccctctcacatgggaatctgttatcacaaaacagaaggggtggcagggcagagcagaaggctgcttttggagggcagctggttcctacggcaaaagaagcaatgaagggaaagagttatgcaagctcacagcctcattccagatccagtctaccttagtggggaggagtaaaggatgttgggcaagagagagatttgggggaaatttatcttgatcaaaacctggggtataaagaagaaacatttcctaatactatccagagtgtttacatgcacatcttcacttaatcctcaaaacaagacaatacactcatgggaccctcatgatgcccattaaacggatgagtaaaatgaggctcctagatgcttttgtaattgacagttaccttttgctgttacttttgtagcagcacttaccctgggtggcttttgtaattttgttatacagccccatggaggtggcagggtgaagacagttactccagctctgtctccacagatcttctaatccccttctgggctgcttccccgagtgcagggccctaagctgctaccatgttttagatgatgcctcctgagttctttagaagcccagcctgggatgtctgtttcagtagtcagtggcacgatgagccccagaatactggaaatctgctttgaccaagttcttgcaataaaacttgaatctcattaagccatttgtaattaatcctgagtagaagatggatggaaggattgattaggctaggatactgttgctgctgctgctgacaacagctgatttctaccactcttctgggaacttgccatgaattgtgtcatttatacctcacaataaccctatgaggtgtgtactaatgttatccctactgtacagaggaggagaccaaagcaaagaggggttaagtaacttgctcaaggtaacacagctggagtatggctgagtcaggtgaaaactccaacatgagagctattgtagtaagatgcagagctgggatttgaactcactacaccacactgaggttcgtaatccttgggacggcaatgagctcttaaaagcttagggagagctaatgcacagcaaccatgggcttgcttcactcacaaatctgggaataaaaaataggtaatcaacatgtgttccctgaagaaggaagctgttacacagtaattctgagctcctaaattggcagaaggaactttgcagcagggagatcctattgtttgggagtgtttcgagtggtccccaagggtgcagggaactcatgtttggtgtcaatagatcactctagggtgtcagaaacagagaagctgtttgttaactcacccttctgacaccccctgtgaatgtcatgtaaatttcatctttgtgtagcatttcatgaattttcagagctctttcagagtcaacaccttattcaatgtcttatcttggtgttcaagcttcttcacaatgaggctctagcctaagtttccagactcctcgccttcacccctgcttcccaccctatgaccgtccattcctcttcaagccacatcaatcttcctgacatccccacaattacctcatcctcacatacctacttattggtcttcctgcttttatcccatcctcttcctcccttctccacactgcagccactctgttgtgatcactccagtcacaacagtcccaacttaaagttgccctccatgctccagacacaatggcctcttctctgttcttcagacttgctaaccttcttctcctatgccctttgtatgtgccatgattatctttgcctggaaaactaccctctttccttccccaatctgtcagggcatggatggctctctctcatcattctgatctcagtttaaatctcatttcttcagacaaacctcttttctctatgtgagttcctctcttttgtcttctgtcaactttactatttgttcttgtaatagtactttttattatttggatttgttaagtattttaattatcttagtaggctgaaggttccatgagatcagtaccaagtttgttctgtgcttaaaacaatccctggcacatagcaggtgttaataaatatgctgggtcagtggatagaggaataaatgagtgaatgaatgaatgaatgaatgaatggactgatggatattttagtctttccactgattggtaacctctatgtgttctttgtcttttctctgcactggacaaatcttgtttagcattttcaagtcaatgatttgttgaatctttgcatctatctcataaagaatgtattatccttatcaaaatctagatatcatctcaaatttatacaactacaaataatggaaccagaatttgaacccagctttatctgatacccaagtccaagcatgtgctggagataacacaacatgtattactcctgtccatttatatgagcaggagaggaaagacattagcttagatgtcagcaagctaagtctcttagagctatgtttatccacaacgttgaacagcagacataatcaaaactatgttttatacagtgagcctgcacatattcacgtgtgaatgtgtgtgcgcacatctctaaaataagttttgcaaaataatacacattgtcattacatgggaccatgttctgatagcttctattcttttgatggcatttttgtaatgctgatggagccactgaattgatttcacagtttgagagtgggtcataaccttaagtttaaaaacctctttcttagaggagctaataaagtgccagaggccacagtgggaacaggtgcatgacaactggatctgaggtggcttgcaggagacatttctttcccagagatctgaaggatgaagataattcaagggcttcagtttgaggggttggtggaggaactggaaatggtacctgagccaggcaaggcccacatgagggttttaggtcttacccctgccatttctatggccagccacttgtgtcttttacccaaccctataggccactgggcccatcatttccacatttgctcttatgaaatgtgctcaacctgccctttcttgtgccttgtgcctcagatcttatcttatttctgtacgatgctctatcttccctggggaaaggaaaaacaacaacaacaacaacaccctgccctctgctccctgcatgggaattactgcccatctttaagccatactctgttctgaggccccagatgccagttttcagagagcctggggaactcccttactaacagcagctcccatttgactgtgccttgagggtgctgccaggagcacgtgcagggcaaggggaagatagaatgggcagaattgttttaacaaaagcaagactgctttaaagtggttgcatgtgggattatttttgaaacataggccctctaggatgaaaagaagaaaaatttggaaa

SEQ ID NO: 8624 - RNA, 39 nt, Homo sapiens
  source 1..39: mol_type = other RNA
aaagtctcgctctctgcccctcagcctaacttcctttat

SEQ ID NO: 8625 - RNA, 148 nt, Homo sapiens
  source 1..148: mol_type = other RNA
aaagtctcgctctctgcccctcagctgcataattcttctcagtgcagttaactaatgttatcagtttcttgtgtatcctttatttcttcttgagcatcttagtcactttgagttgctgtaacaaattaccatagactagatggcttat

SEQ ID NO: 8626 - RNA, 351 nt, Homo sapiens
  source 1..351: mol_type = other RNA
aaagtctcgctctctgcccctcaggtctcccagaggcattcaccagcatgaaagaacctgatggcatccatggatcagaagtcggtttagtcaaggtgttcacttgctcccaattgaagtcatcaccttcagattgactatatccacatgtgctatacggctcatcaaagaggcagccacccctgtgcaagtggaacactagagggagaacaagttttgtgttgaaaactgtatgaccacagcagcctctcagcttaaaagtccatagtcttcaaactctcaccttagctgcccgcacagcgagcagcaggtaaaggaccagtgcaaaatagaaaatctgtagaacagcac

SEQ ID NO: 8627 - RNA, 751 nt, Homo sapiens
  source 1..751: mol_type = other RNA
aaagtctcgctctctgcccctcaggtctcccagaggcattcaccagcatgaaagaacctgatggcatccatggatcagaagtcggtttagtcaaggtgttcacttgctcccaattgaagtcatcaccttcagattgactatatccacatgtgctatacggctcatcaaagaggcagccacctgagaacgtctcgcccgccgcagttagcaaaagtccggccaaagtcgccaggcaagtcccaagtcccctcatggtgctgagtgcgggccgggccgctccccggcggcggtgggtgggcgcgcgagggcggagggggccgggagctttggttccgaggcagcgaggagagacgggtaaacagcagagcgctaagccaagcccccaaagtgccaacagttgcagaagtccgaactccagcggctccaggggcgcgggcacagggtcctgggtcctcctcccctgtccctggccccactcggcgtctggcgccgctggcagagggagcggagggcgagcccgcggagccaaaatcttccctcggttccggttgctgagctcgccgcctctccccttcccctgcccgggacccgggacccgagctgccggccgtggccgtggcggtggccgtggccgtggccgcgcgcgttccgcccgccgcctctccacaggcagccccaagcccagccccgggcggcggcgcgccgatgaccgagcccgcgccggctgcgcgcggggctcttgctccccgac

SEQ ID NO: 8628 - RNA, 756 nt, Homo sapiens
  source 1..756: mol_type = other RNA
aaagtctcgctctctgcccctcaggtctcccagaggcattcaccagcatgaaagaacctgatggcatccatggatcagaagtcggtttagtcaaggtgttcacttgctcccaattgaagtcatcaccttcagattgactatatccacatgtgctatacggctcatcaaagaggcagccacctgagaacgtctcgcccgccgcagttagcaaaagtccggccaaagtcgccaggcaagtcccaagtcccctcatggtgctgagtgcgggccgggccgctccccggcggcggtgggtgggcgcgcgagggcggagggggccgggagctttggttccgaggcagcgaggagagacgggtaaacagcagagcgctaagccaagcccccaaagtgccaacagttgcagaagtccgaactccagcggctccaggggcgcgggcacagggtcctgggtcctcctcccctgtccctggccccactcggcgtctggcgccgctggcagagggagcggagggcgagcccgcggagccaaaatcttccctcggttccggttgctgagctcgccgcctctccccttcccctgcccgggacccgggacccgagctgccggccgtggccgtggcggtggccgtggccgtggccgcgcgcgttccgcccgccgcctctccacaggcagccccaagcccagccccgggcggcggcgcgccgatgaccgagcccgcgccggctgcgcgcggggctcttgctccccgactgact

SEQ ID NO: 8629 - RNA, 295 nt, Homo sapiens
  source 1..295: mol_type = other RNA
aaagtctcgctctctgcccctcaggtctcccagaggcattcaccagcatgaaagaacctgatggcatccatggatcagaagtcggtttagtcaaggtgttcacttgctcccaattgaagtcatcaccttcagattgactatatccacatgtgctatacggctcatcaaagaggcagccacctgtggtacagtcctcatcgtcactgtcaggagggggctccagccagcacatccacatcccacgcagaaggacagaggaaggggaggaagaagggggcactccctcctcacaagg

SEQ ID NO: 8630 - RNA, 184 nt, Homo sapiens
  source 1..184: mol_type = other RNA
aaagtgcttccctttggactgtcaccatggaaaaggaggggtcagatatgatatactcctgcttgatctttccctcttcatcctggtctgataacctcgattctgtggtggtacctgtagaaggttttactgtagtgctggtttcccagatgaggaaactgagactccgaagagctccagcagc

SEQ ID NO: 8631 - RNA, 316 nt, Homo sapiens
  source 1..316: mol_type = other RNA
aaagtgcttccctttggactgtcaccatggaaaaggaggggtcagatatgatatactcctgcttgatctttccctcttcatcctggtctgataacctggagtccggctcctcctccgactccgccgccgtctcgtcctcctcgccctccgactcctcctcggtctccagctcccgggtcgcctcctcgtccccgtcggagccgagaaagctctcgccagcgtggttgctatcgcggctcgccatcgcctctcccgggcctgggccggggccggagccggagccgcccgcgccgcgcctggtgttctccctccgact

SEQ ID NO: 8632 - RNA, 445 nt, Homo sapiens
  source 1..445: mol_type = other RNA
aaagtgcttccctttggactgtcaccatggaaaaggaggggtcagatatgatatactcctgcttgatctttccctcttcatcctggtctgataacctggagtccggctcctcctccgactccgccgccgtctcgtcctcctcgccctccgactcctcctcggtctccagctcccgggtcgcctcctcgtccccgtcggagccgagaaagctctcgccagcgtggttgctatcgcggctcgccatcgcctctcccgggcctgggccggggccggagccggagccgcccgcgccgcgcctggtgttctccctccgactgctctggcccctgccctccccagccctgcccctgcgggggcggctcgggttcccggcgccgggggcgggcgagccccgcgactttaaatagaaggcgtcaaagtttcgccaccgagcttctggggcccg

SEQ ID NO: 8633 - RNA, 1864 nt, Homo sapiens
  source 1..1864: mol_type = other RNA
aaagtgcttcctttttgagggagtggttacatgtctccatggcttccaataatcgcttctcatcaataaaagggattaacaccacagcttcccattcctgttgtttcccatttaggtcagttttaaaatcaggtgggtaatattctataattggtgagtcttcattggtcatcaaatgctggtagcatgcaggaagtaaatttttgctggctgctggaagtacagcaagaagctgttcaaatggcttaaaaggttttcctagttcaaaatggattttgagtgtactgatgttgtgtatatcagacaggaaaggtgcataatgataaggataataccagctccaggactgaactccatgatagtaatagtgcaaaatccactgtattgcctgaacataacatgcagcttgatcagccagaaagtcatcagatactacgtcaacccccatcttcgtcatgtaatatgttcttttatattgtctaaactcagtttcaaataggtcatcatcttcagtctcatcttctaaattatccttagaagttatcatttcgccttcatttttgtctaaagcagtccaacacagagaattttcctggccctttaactttttcttttccttgtagttcctggcttcttctgctgcgacacctgctgcttcattgaggtacttgttaccaactttgctttcaaaccattttaggtccacaaaaacttcactgaagtgctcccgatcaaaatctgatagtttcacaaggtatttctcaaatcgaggtaagttgaggtgcccactttcattaatataacccccaagttctggcaggatggtaacatatgttccataaagaagaggcagtgcatcatgattaatatgtaaatgaggtagatgagggataaaatcattaccaacaagaaaccccatcaaaatccaatcatctattatcctttcaatatcatatttaaatgtgatcttttcttttaatactgaaaactcatagtcaatatactctctcattaaagacaagtgtagaaggtgaaatgtagtttcttctggagcacatacccgttgtgtttttttgccaccaaatcgaacttcttctcttaagagagaaaaatgtgcctcatgacttgttaatccaagcataatcaagtcagcatctaaaccataaagacagtgtctggtgtttggatcatgatctggctttgctttctcggatctgataaattccatgattttatgctctccttctccaggagtctcatggcctgagaagtagatggtaactccttgccatgacttgtctgtggaaattttcatatttacaaaatacttcagatgttcatgtaacctggccataaattcagttcctggtgtgatacagttggaatcaaatctggcctctgtaggaagagtttctcccttctctattgcctttttaattttgtcttctgcctcctttgctgacctaaaacgcctcccacgctgctggttcatttttgctcgaggagccacaccatctacagccataaagaacactttcctgggtttaataatgcgaaacaacacctccaggtagtgaaaaatatcagtaaagattttatcatctgaaattctaaagtgaacatcatcatcattaggatgggagcactgatgtataattccattcatatccaggtacaagttgtcaaattcaggaatctgatgctctttcaccacttcgctgagacagggataccgctctgagatccatctgtaaaacttggggactcccatttcgatcgtcaacactaatcccagtcagggccaaaccgaaaccaaacgccccgccggggctccgccgcagcctccggtcgtcgctccgcggat

SEQ ID NO: 8634 - RNA, 1889 nt, Homo sapiens
  source 1..1889: mol_type = other RNA
aaagtgcttcctttttgagggagtggttacatgtctccatggcttccaataatcgcttctcatcaataaaagggattaacaccacagcttcccattcctgttgtttcccatttaggtcagttttaaaatcaggtgggtaatattctataattggtgagtcttcattggtcatcaaatgctggtagcatgcaggaagtaaatttttgctggctgctggaagtacagcaagaagctgttcaaatggcttaaaaggttttcctagttcaaaatggattttgagtgtactgatgttgtgtatatcagacaggaaaggtgcataatgataaggataataccagctccaggactgaactccatgatagtaatagtgcaaaatccactgtattgcctgaacataacatgcagcttgatcagccagaaagtcatcagatactacgtcaacccccatcttcgtcatgtaatatgttcttttatattgtctaaactcagtttcaaataggtcatcatcttcagtctcatcttctaaattatccttagaagttatcatttcgccttcatttttgtctaaagcagtccaacacagagaattttcctggccctttaactttttcttttccttgtagttcctggcttcttctgctgcgacacctgctgcttcattgaggtacttgttaccaactttgctttcaaaccattttaggtccacaaaaacttcactgaagtgctcccgatcaaaatctgatagtttcacaaggtatttctcaaatcgaggtaagttgaggtgcccactttcattaatataacccccaagttctggcaggatggtaacatatgttccataaagaagaggcagtgcatcatgattaatatgtaaatgaggtagatgagggataaaatcattaccaacaagaaaccccatcaaaatccaatcatctattatcctttcaatatcatatttaaatgtgatcttttcttttaatactgaaaactcatagtcaatatactctctcattaaagacaagtgtagaaggtgaaatgtagtttcttctggagcacatacccgttgtgtttttttgccaccaaatcgaacttcttctcttaagagagaaaaatgtgcctcatgacttgttaatccaagcataatcaagtcagcatctaaaccataaagacagtgtctggtgtttggatcatgatctggctttgctttctcggatctgataaattccatgattttatgctctccttctccaggagtctcatggcctgagaagtagatggtaactccttgccatgacttgtctgtggaaattttcatatttacaaaatacttcagatgttcatgtaacctggccataaattcagttcctggtgtgatacagttggaatcaaatctggcctctgtaggaagagtttctcccttctctattgcctttttaattttgtcttctgcctcctttgctgacctaaaacgcctcccacgctgctggttcatttttgctcgaggagccacaccatctacagccataaagaacactttcctgggtttaataatgcgaaacaacacctccaggtagtgaaaaatatcagtaaagattttatcatctgaaattctaaagtgaacatcatcatcattaggatgggagcactgatgtataattccattcatatccaggtacaagttgtcaaattcaggaatctgatgctctttcaccacttcgctgagacagggataccgctctgagatccatctgtaaaacttggggactcccatttcgatcgtcaacactaatcccagtcagggccaaaccgaaaccaaacgccccgccggggctccgccgcagcctccggtcgtcgctccgcggatgacaacacaccgcccggccgaccat

SEQ ID NO: 8635 - RNA, 1520 nt, Homo sapiens
  source 1..1520: mol_type = other RNA
aaagtgcttcctttttgagggagtggttacatgtctccatggcttccaataatcgcttctcatcaataaaagggattaacaccacagcttcccattcctgttgtttcccatttaggtcagttttaaaatcaggtgggtaatattctataattggtgagtcttcattggtcatcaaatgctggtagcatgcaggaagtaaatttttgctggctgctggaagtacagcaagaagctgttcaaatggcttaaaaggttttcctagttcaaaatggattttgagtgtactgatgttgtgtatatcagacaggaaaggtgcataatgataaggataataccagctccaggactgaactccatgatagtaatagtgcaaaatccactgtattgcctgaacataacatgcagcttgatcagccagaaagtcatcagatactacgtcaacccccatcttcgtcatgtaatatgttcttttatattgtctaaactcagtttcaaataggtcatcatcttcagtctcatcttctaaattatccttagaagttatcatttcgccttcatttttgtctaaagcagtccaacacagagaattttcctggccctttaactttttcttttccttgtagttcctggcttcttctgctgcgacacctgctgcttcattgaggtacttgttaccaactttgctttcaaaccattttaggtccacaaaaacttcactgaagtgctcccgatcaaaatctgatagtttcacaaggtatttctcaaatcgaggtaagttgaggtgcccactttcattaatataacccccaagttctggcaggatggtaacatatgttccataaagaagaggcagtgcatcatgattaatatgtaaatgaggtagatgagggataaaatcattaccaacaagaaaccccatcaaaatccaatcatctattatcctttcaatatcatatttaaatgtgatcttttcttttaatactgaaaactcatagtcaatatactctctcattaaagacaagtgtagaaggtgaaatgtagtttcttctggagcacatacccgttgtgtttttttgccaccaaatcgaacttcttctcttaagagagaaaaatgtgcctcatgacttgttaatccaagcataatctaaaacgcctcccacgctgctggttcatttttgctcgaggagccacaccatctacagccataaagaacactttcctgggtttaataatgcgaaacaacacctccaggtagtgaaaaatatcagtaaagattttatcatctgaaattctaaagtgaacatcatcatcattaggatgggagcactgatgtataattccattcatatccaggtacaagttgtcaaattcaggaatctgatgctctttcaccacttcgctgagacagggataccgctctgagatccatctgtaaaacttggggactcccatttcgatcgtcaacactaatcccagtcagggccaaaccgaaaccaaacgccccgccggggctccgccgc

SEQ ID NO: 8636 - RNA, 1677 nt, Homo sapiens
  source 1..1677: mol_type = other RNA
aaagtgcttcctttttgagggcatgaggaaggcaaagctgcagtcaagcgttcatgaagcagtctatgccccatgtaaacagcgtggctggttagttaacctctctgagcccttctcattggctgaattcatgactgatgagtagtgagagaatatgagtgaaggtgatttgtaaactatgatgtgtcaaacacatttaagggacaatgatgatactagagaaaaaacactggactcaggctcagatgtgggtttgagatctgtctgccatttacagtgggtgacttttgggaaagtcagttaacttctctgggtctccaataccatctgaaacctctctagagttgtaggcactgggcctatttgaggggttgtttttgctaagaccctgggaatgcctcctgtagctcagcagaaggaccagggccaggtgggtattcctggtggaagcaaagtcagctgactgggcaccctcaaatgaacttttgtggttgtcaggaacgtgtgacgacggctggaggccaacagagtccctacaggtggtgctcacggtaatgcaccgacaatgagtggctgttttccagtttctggcctccgctgcctatctagggtaagtgggtccctccaggggtctcctaggatgaggcctcagcccccagtttcccatcacctttccatagggccttgggagaggccctatccagcccgttttaggtttaccctcacctctactggggcttcattaattcctagaagcttccatcccaggtgtggggtcctgatgctttatatctgcaatttgaaggatcctgggccactgaaatgcccactggatgttgatgagaccagagggtgactctagggatgaggtggaagggacagcttggttagggaggcagatagccaatcgaaatcccagctccgaaatgaggagcttgggtttctgtttcacaaggtgtgccaggccataagcacaccaggaatatgagagaggggcttaggaagaaaccagaaagagaaacaatcccatctcaattaactggggtgggagctgggcgggagaaaagcagtgtgtgggtatctggaagctgcatgtcacctgctcactgcccctctgcgcctctcacacactggcaggcaaaggtgatggaaacttgctgccaagggctcttgctgcctccattgcttgcctttccttgtgcccagacatgtcccctcttgtcctctgtcctctcccatgctgcctaccaccctcccctccaacaagaatctggcccaaggtctccgcttcctggaactcccttatccctacccctactctgtcttcctgtccagcagtctgtctccaagatcccctagaatgacctcctctcagccctctcctccacaccccccaagtccccactacctggcccctcccactcctctgccttttcagccactgctgctctcttctcttctcccttacctgtctcccaggtgtgtcatggcctggtgcgggaggctcttacctccccaagccccactgcttctcctgctgcccgcttgcttcggactctggcagaaaccccacctgctgacacgttcctcctgggcgagcagggcgtgcggccgcgggacctgagcgccatctacgaagccatccctttgtcgccaggcatgagcgacctgctgcag

SEQ ID NO: 8637 - RNA, 1678 nt, Homo sapiens
  source 1..1678: mol_type = other RNA
aaagtgcttcctttttgagggcatgaggaaggcaaagctgcagtcaagcgttcatgaagcagtctatgccccatgtaaacagcgtggctggttagttaacctctctgagcccttctcattggctgaattcatgactgatgagtagtgagagaatatgagtgaaggtgatttgtaaactatgatgtgtcaaacacatttaagggacaatgatgatactagagaaaaaacactggactcaggctcagatgtgggtttgagatctgtctgccatttacagtgggtgacttttgggaaagtcagttaacttctctgggtctccaataccatctgaaacctctctagagttgtaggcactgggcctatttgaggggttgtttttgctaagaccctgggaatgcctcctgtagctcagcagaaggaccagggccaggtgggtattcctggtggaagcaaagtcagctgactgggcaccctcaaatgaacttttgtggttgtcaggaacgtgtgacgacggctggaggccaacagagtccctacaggtggtgctcacggtaatgcaccgacaatgagtggctgttttccagtttctggcctccgctgcctatctagggtaagtgggtccctccaggggtctcctaggatgaggcctcagcccccagtttcccatcacctttccatagggccttgggagaggccctatccagcccgttttaggtttaccctcacctctactggggcttcattaattcctagaagcttccatcccaggtgtggggtcctgatgctttatatctgcaatttgaaggatcctgggccactgaaatgcccactggatgttgatgagaccagagggtgactctagggatgaggtggaagggacagcttggttagggaggcagatagccaatcgaaatcccagctccgaaatgaggagcttgggtttctgtttcacaaggtgtgccaggccataagcacaccaggaatatgagagaggggcttaggaagaaaccagaaagagaaacaatcccatctcaattaactggggtgggagctgggcgggagaaaagcagtgtgtgggtatctggaagctgcatgtcacctgctcactgcccctctgcgcctctcacacactggcaggcaaaggtgatggaaacttgctgccaagggctcttgctgcctccattgcttgcctttccttgtgcccagacatgtcccctcttgtcctctgtcctctcccatgctgcctaccaccctcccctccaacaagaatctggcccaaggtctccgcttcctggaactcccttatccctacccctactctgtcttcctgtccagcagtctgtctccaagatcccctagaatgacctcctctcagccctctcctccacaccccccaagtccccactacctggcccctcccactcctctgccttttcagccactgctgctctcttctcttctcccttacctgtctcccaggtgtgtcatggcctggtgcgggaggctcttacctccccaagccccactgcttctcctgctgcccgcttgcttcggactctggcagaaaccccacctgctgacacgttcctccttcgacttcgacgagactatcgtggacgaaaacagcgacgattcgatcgtgcgcgccgcgccgggccagcggctcccggagagcctg

SEQ ID NO: 8638 - RNA, 6231 nt, Homo sapiens
  source 1..6231: mol_type = other RNA
aaagtgcttctctttggtgggtggcacagcagagaaagactccatcttttgtgaagaaagctgtgcttgagaagtacttgcaggtagaaatgtggtgggagcttgcccgctagtgataggtgcagaggagacagaaggcagggaactacaagtgcttgtcacagaagaaatcactgttgctggaggacttgtcttaggcacacaggcaaacaactgctttctgactgatgaaggagtccgggtattagtgacacacagttgctgactggcagcaactacagaagagacagtgataggacaactggcagtagctagtccagcagactctgagggtaaaacagtcccgttctggttaggtagacggcttgtgttattatgctttggagagctatttgtgttgccaggattcacaggtctcactgggaatggtccccatgtgttaggagaaggtgagaaggttcctccaaactgggccatgggtaagcgaggatgccgaatctgttgcatagtttgagcagccagcagggcaaaatgagggtgaggataagctaagggtagagaaactgggaaagaagaacgtacatttgttggaacattcttattaagtttattagcgggctggaacgtagataacgttgttgcctgtgaagttacaagagttggagcacccaaaggaaatgcatttttactggaagctgctgtggtacctactccagatgagaagttagcatgaattgatttggtgctggcaggtgttctgatatgatttttaggaatcaagtcttccagttccttagcaggatcttgaatgagtgcattgattagttgaactgcatatcttgttgattctgtgccaccccttattgtgatcattctctcgccattcttatctttttgtttatccacatcaatatgggcaccagtaacatcctgtattgcagtgatgttgcatcctcctcttcccattatcctcgacaccactgaggctggaacagacaatttctttgaccttcgtacaacttctttccacccttcttctcttttctgaccccttttagggctagtgagattcagctttatgtttggagagcttaatggcaatgacactgtcttgtagctggttgacaaggaattaggagtcacttcaccttcaagtcgtgtctgagttttggaagtagcagtacttgtcttttcttcttgggaatgaaggagcagtgaggggtatttagaggaattcacatccatcacaaaatttaactcttggcttttaccaccactgctactctcactgttgcagtctgtgctgtccaagttatctgaatcactattcccacctgcaccaccacctctaggttctccatttattttatttttatctgccttttgttgggctaaagacatatgttgttctggtaaaattaaatgtgctgtaggaggggtttcttttgttttgttcttcttatttttccgattggtgctgggagttgtcaccacattggccctttttttcccaaacacatttgtgaatgttgcagatgttgcagagattccaatcgtagtggtggtggttgcactaggaggttctatgggaacttcttgctccacatcttcatcattctcctcttcatcttcatcctctggtagttccgaattctccttaggtttgttttcttcatcttcttcctgtttccttttctgttcctcttttttcttttttctcttttcttttcttttttctcttttagcagcaagagcctgctttctgctctcttctcttgacttttccagatcaagttcctttaaaagaatactcgcattcttatttgcttctgcagcttgctggtctttagccttcacaatggtttcgacacattgatgacattttttcaacagttccttatctgtaattgttgctatgtatctcatgcattctatatcagaagggaactgatttacttcctttaccaaatattgaacaacttttacatgacccttgcgaaatgctgacataagaggtgtgattttccggttatctgctgcatccacatcagcacctgcttgcactagcaactgcacaacatcaaaatgacctccattggatgccagccaaagtggcgtatttccctttttgttacgaacatcaatgtgggctcccctatgaatcaggagttcacaaaatttgtagtgacctttgtctgctgctattgttaaagcagtatctcttgaggaaggcacagggggagcattaacatctgctcctttatcaagaagaactcttccaacctctgcataccctccagaagctgcttccatcaagggggtaagacccgtctttgccctatgttcaacattggcttttcggtccagaagcaaactcactacttctgctcggccctggaaacaggccagggtgagagccgtgttccgattggtctctatttgggcattaatgtctgaacccatatcgagcagcaattttactgcaggaacatgtccattcattgcagccaacatcaggggagaaatacctagtttactcccagtccttgaattaatttctgccccagcattaagcagaatcttaatgatattaacatatcctccagacgcagctagactcagtggtgtataatcagatacgttcctatgttctttatttgcacctcgagccagcagcaagtctaccacctcctgacgtccaccagaacatgccaatgaaagcggagtatccttagttcgttcagactgtgcttctatatctccacctttatccaaaaggatttcaacaactccaacatgccctgctgttgctgccaggattagtggtgtgaaaccttttttgtctctgtgttcaattttggcatcccgtgcaatgagcacagatacaagttcttcatgaccacctgcacaagctagtgttaatgctgtgtcatgattgctctcagtatgtgcatcaatgtcaactgaaggatacacaggaggcatcgattgggaagccacattgcttgtagtctgcgaacaggattcaggtgtaagacactctgtggtctgagaagaactgttggaaccagtgggcactctggtactcacagctgctatcaggtcatcaagagtgtcggtaagcgtctgagctggagttgcaaccattagtccatctggttcttgaactaacagcccctgatcatgtccagtaatagcaatctgaggctgtcctacaatctgctgattacctgatactttctgaagttcaagagaatttgtcccattagaacctaagtcactggaaaagttacactgtggagatgataaaggctggactgggacaaaatcaatctgttctgccgatggtggagactgttgctcatcatcaacatcattatctttaaataagattgtgtcaacctgaggtaactctgaaaagtgatcctctgggagactaccatctccttccccttctgggaagactcctctatgagagcactgttggtgtagagacactgtgtctttctgacctttggtttccaagtattctttggtaaattgctgctgtgttttcatctgcaactgcctttccactttctgcagttctttcaatattttcttcttcttctggacttgctcttctctgttctttttaagttcttctatcttatctttgttcagaggttcaccttgaattaactccagtgacttaagctgtgctttttcaatagcactaattctttgtcccagttcattcagcttgccttcagtctcctctactatgcactccaaaggctggtatgggtgaaaagatggcagtaggtcctgatctgctacctggagggaactggacttctgcttggatgtacctttttgcactcctaaaagggcaggagagttctcctgtgaagttctgtcaggttcctggggaggtacaaccatggcaagtgtatgcgttggcacacgtggcacctgagactgatcttgagaaggtggagggagctgagacacatctgtggtgggaactgacagaacattatttggataatccaacagataagaaactacattagtatggccaccctttgcagcttcaatgagcattgttgaaccatccttgagtcgatgagtagggtcagccccatgagccaagagaagctcaacaactgccaggtggcctcctgcacatgccagcgacactactgtatgatcattattggctgtagccctgttaacattggcacctttgctaataagaaactgcacagtgcacaaatgaccagctcttgcagctttcatcaaaggtgttcttccaccttcagattcatgttctaaatcagcccctgcttgaagtaaaacatctgcaacatccgtatgtccattttcacaagcataggttaaggctgtgtctcctgttgctgttgtagcatgcacattagcgccagaagccagcaaatatttaaccaattccaggtgtccctcctgagatgcctccatcagaggtgtggagcagccaagttctatatcagcccctgccttaataagaaagtctgcaacttcagaaaatcctccacagcaagccaaagtaagagcagtttcttgagtttcttctgtctgggcatttatatttgctccttgtgctaagagtagtgccaccatttcttcatgtccttcccgggcagcttccatcaagggagtgtatccttcatcattaacttcttcaagatttgctcccctttcaataagtagagctgccaattcaacatgtcctccacaggcagctagcgtcaatggagattcaaatgaatctgcaggcatgttcacttgagcaccactatccaaaagcaaacgtgccacctctacatgtccatccatgcaggcctccattaaggcagtgtgcatctcatctgttttgtgctcttgatctgcaccagcttcaagtagaaagcgaaccatatccaaatggcctttgtagcaagcaagtgttagagcactttctttgaattcattagaatgagtgttgatgcctgcaccatgatctaaaagaactcttgcaacttccacatgacctgcactggctgcttccattaagggagtatgtccattttcattatgatcttctatatttgcaccttcattaaggagcactttaacaatgtcaacaaatcctccagcacatgcataagttagcgcagtgtttcctgttgcagactgggagttgacatcagcatcatgaagaagtaataatttcacaatatctaagtaacctccactggaagctgccatcaggggagttatgtctcctttattccctcgatcttcaacattagcatgcatagcaagcaatacttgtgctaattcataataccctgctgaacaagccaaacacagcaggctttctccttcttctgtatgttcatttacacttctgccttcatctagcaatttacgaacagcattaacatccccatctgaacaagcttctgctagactgcgagtgtccacttgtcctgcattgtggctgttttctgctttcatccgtgtcagtgcagcagcagcttcatccagtgcacaactaactgaggatgtcagtctccggagtacctcaggatctgcaaaagctttaccatcagcagttgacaatttgccaattcctgctgcttctagcaatgcttctagtcgtgcctgtgtctctggatccacagtgcgtaagtctgctccttctgcagtacttgataagaatatctctgatgttgttttaagcactgggttatccagatcttcttggtccaaaataaatgattcaacctcggacacttcgtcctcgtcactgccagaggcaccacctccacccccggtcctcagcacggcagccgccaacttgaaatccagcgccgcgtcccctccgcccgtaccgctgccgctgccgccgccgccgctgctgccgactcccgacgctggcccggcctccccaaagagcctcacggtgcggatccccagaccgacccctcccggcggaggcggctccgaggccccagctggggcggatcgcggagccacagagtccaggtcctcctcaaaggaggtgccgccgcctccgctatcagtcagcattgttcgcacccggagccggagacggtgccgacccactcgcggtcaccgccgccgctgatctcgggaacgagaagagcagcaagaggaagaagcgtctcctttcccccgtcccagcagcgccactaacttctcact

SEQ ID NO: 8639 - RNA, 2329 nt, Homo sapiens
  source 1..2329: mol_type = other RNA
aaatatatatatatatgtacgtatgtataaaaaccgtgcccttgttcactgccaacacaacatctgggtggacatgaactcattacaacaaattcttatgtggatgttgtaagaagtcactcaatgtctgtggatttaataagtcacttcacaccacagaaaatatttaataaatccaaaaaaaggaaagaagaatataacgacagaagagcttctgtctcagttctctgaaactgagtcccctataggaaactggtcccaaagttctcgaggggtcattgaagaaacttcggtttgctaatttttttcatccttttagtgttcaaaagttctagaaagactcctcgctgttttcagtttttaaacagtcaaatctccatctcccccagaaggtaacagtctggtgcagatccataaaaacgtgggaggaaggcgcgctggggagaggcctgtccctcttggaaggggccccacctctacatccgcaggaagagaaggaaccaaacagggctccagcacctctctcctgcaaacgagctccctttaaatgccaaatccagtcacacggcagttccttaaacacaggtacatttctgagtaccaggccagctctaagaggaaacaaaccatgagttgagagaaaaggactatgacggccatctggtcactttccacgtgatccatcatacttccaggaatcgggagctgctggacttggagtggaaaggctcagaccacatccgccggaggtcgccctttaaataggccatcgtgaggagtggcaataaagtaaatggcaccaaatagagaagggcgggctgggcggcccggtgaatgcgagacgccacagtagcagtgagcaggcctacaaagtatccgatgagggtgcagtgaaagtaggagaccttctgcatgcgcccggagatgttggcaggtccaggggccccacaggagtccccactggcttgctttttgtagttgtcatagcgaaggacaaagcatagtaggagaccaggcataacgatgtctccgatgcccaacatggagaagtggctgccagtggagcttgggaagaccagttttccaggcagagacaggcgaggaacatcacgcccaacattgggccccaggtggagcttccgggatagaacgtcaaggggattgtcagccggctgagtggccaccttcaccatgacgttgctattgaagatgtaggctgagaaaaatacccaaaagacatcatagatgagaagccctgagagaagcaggcaggagaccttgaggctcggcaggcggacaaaggcgatcatggcgacacagaggcccatggccagtgcatccatgagaagccaatggccagtgagaacccagatgaggacgagcatgacagacagagagaatgacagcaactcagcagcagtgaaacgtccacagcaaccaaaggaaatcttgttctgaggtgagcagggtcttgttaaatactggcacatcgggaggagaagaaaagcaaaagctatcgttgcaagaactgctgtacatattgtaaaaactacttgaactgagtcaaagaagaagaacattactaaaagagagacagatgctccaattggaaggaacagagcctgggtagagtcaattgtttggatgctattattggtgctgttgccattgaaagacccagaagaactattactgtctttctccttatcttgattttcaaagtccatattaagggacctgaaactaccatagactataagaagaatggaaatcagaaatgtagacacttgactggaatccaccagggaataggcccacgagtaggtctgctccgccatggcgctgcctctcgtgggctccgctgcaggctgtggccgggcccggcggcggcgggctcgctcgggccgtagctgaaggcgcggccggggtccggtgcttgcttgcttgctcgctcgctggctcgctggctgcacggcgggccgggaaggcggctggcggggagaggccgggctccgaagcggccccgctccctgggccccggggcggggcgggctccgctctcggcctccctcacccgcggcggcggcggcggctccgctgcagctccaaacccaacatggcggcggcggcggcgcggagaacaagggggccctggggcgggcgaacggcaagacgggcccgcgctcactgcgcgcggggccgcgggagcgccgcgctcgggcggcggcggcggcggccgggggacatggccggcgggcggaggcggcggcgactgaggggggcgctaggcgatgaggcgaggccactcgatcacacccgccgaggggag

SEQ ID NO: 8640 - RNA, 1853 nt, Homo sapiens
  source 1..1853: mol_type = other RNA
aaatatatatatatatgtacgtatgtataaaaaccgtgcccttgttcactgccaacacaacatctgggtggacatgaactcattacaacaaattcttatgtggatgttgtaagaagtcactcaatgtctgtggatttaataagtcacttcacaccacagaaaatatttaataaatccaaaaaaaggaaagaagaatataacgacagaagagcttctgtctcagttctctgaaactgagtcccctataggaaactggtcccaaagttctcgaggggtcattgaagaaacttcggtttgctaatttttttcatccttttagtgttcaaaagttctagaaagactcctcgctgttttcagtttttaaacagtcaaatctccatctcccccagaaggtaacagtctggtgcagatccataaaaacgtgggaggaaggcgcgctggggagaggcctgtccctcttggaaggggccccacctctacatccgcaggaagagaaggaaccaaacagggctccagcacctctctcctgcaaacgagctccctttaaatgccaaatccagtcacacggcagttccttaaacacaggtacatttctgagtaccaggccagctctaagaggaaacaaaccatgagttgagagaaaaggactatgacggccatctggtcactttccacgtgatccatcatacttccaggaatcgggagctgctggacttggagtggaaaggctcagaccacatccgccggaggtcgccctttaaataggccatcgtgaggagtggcaataaagtaaatggcaccaaatagagaagggcgggctgggcggcccggtgaatgcgagacgccacagtagcagtgagcaggcctacaaagtatccgatgagggtgcagtgaaagtaggagaccttctgcatgcgcccggagatgttggcaggtccaggggccccacaggagtccccactggcttgctttttgtagttgtcatagcgaaggacaaagcatagtaggagaccaggcataacgatgtctccgatgcccaacatggagaagtggctgccagtggagcttgggaagaccagttttccaggcagagacaggcgaggaacatcacgcccaacattgggccccaggtggagcttccgggatagaacgtcaaggggattgtcagccggctgagtggccaccttcaccatgacgttgctattgaagatgtaggctgagaaaaatacccaaaagacatcatagatgagaagccctgagagaagcaggcaggagaccttgaggctcggcaggcggacaaaggcgatcatggcgacacagaggcccatggccagtgcatccatgagaagccaatggccagtgagaacccagatgaggacgagcatgacagacagagagaatgacagcaactcagcagcagtgaaacgtccacagcaaccaaaggaaatcttgttctgaggtgagcagggtcttgttaaatactggcacatcgggaggagaagaaaagcaaaagctatcgttgcaagaactgctgtacatattgtaaaaactacttgaactgagtcaaagaagaagaacattactaaaagagagacagatgctccaattggaaggaacagagcctgggtagagtcaattgtttggatgctattattggtgctgttgccattgaaagacccagaagaactattactgtctttctccttatcttgattttcaaagtccatattaagggacctgaaactaccatagactataagaagaatggaaatcagaaatgtagacacttgactggaatccaccagggaataggcccttgaaaagacacctccacacatggcaaagtttatcct

SEQ ID NO: 8641 - RNA, 122 nt, Homo sapiens
  source 1..122: mol_type = other RNA
aaatctctgcaggcaaatgtgataccgaactctagaatctaaatctccagatgggtggaaagagccgctgcttagaggaacagctgagaagccatgccttctgcgtacacttcactcaggaa

SEQ ID NO: 8642 - RNA, 5684 nt, Homo sapiens
  source 1..5684: mol_type = other RNA
aaatgtcacctttttgagaggaagagtctgaatccattccatggagttcacatcaaagatatcaactgcattttcactgtacaccgagagatatggtgcattgtaacaacaagaggaaggatttgctggccacatcaattcctgttgtctagatcttcggccctggcagtcagtgtatatcccaatgctgttaaaacacagcagatattctttactggagatctcaactgcgcagatagcatccattggttgatgtgcaataaatgatagtgtatggtcatttgaatggagcatactgtatggatttccttctccattcaaggggtatcttagaaatcctgactggaatcccacacagagttgttcactgaagattgccatccactggacattatatgggacttgaatttctttaaattttctgtgacgggtcttgctctgaaatagttcataacagaggacctgccttttcatagccacacacaggcatgtgagagctccatggcgcacctttccagaagttacggtttgacaccctttagtttctgacagcttgtaaaaatcggtctctcgcccatccaatgctgacataggaaaaagtcgtacatgacgatttcgtcctgagatcacagcaacaagctgatcatttggaatgagttcaatctgatgaatcttcttattgtcaccaactctaataatttcatctttggtgacatgtacaacaaataacccttcttcgtttcccaaagcaattctttcatgatctatgattgcggctgcctgggttgttttaatgaggggtagagtgctgtcataagcctctttgggaacatagactgagcggtctctgaatttgtttttcttcaaaatcttgtgcaattcactcagcactcccacccacttattcttctcattctcagtgtctgctagcatcaggattgaacatttgttattagatgctgagagctgggaagctgtgaccctaaatatacagggtatatctttccgacttgcatggataacatcagaagccaagactgaactcacagaaaattcttcatccctcatgtcaatcacttgactaatgacaacactgggctgagatgcttttccttcagcaatatcgtacagaaagagtttgaagtcacacactatagccagtgctctctgccaccctttcttcactccagctggcttaggaatcctgacatgaccttcatatgctgttcctattcctttctgaggatctatacccaggggaccttttgtctgttcaggaggaactggacaagtggttggagctttgtttacacaagttatatggcatgagaatccacacacttcacatgaacagccctgtcttattaaacccaccatcaaggaggtacactgatgacacttggtaggagtagtaaaagattttacaaaaaactggtgagtcttgcgcttaggtggaaagccagttgaaccaggacatccttttttccttaaggttggtgtgtgaactgaaagtggagtggagtctacagtacgtctgcctttgctagccttttcagatctaagctcttcagtgtcctttatcagctgttcgatttctgagagtagttccaagttcttcttctctgaatcttttagtttacattctgttatgatattagatgctttaactttattcaactcttcttggatggcctgtttggctcttatttctgcatccagagccgactgcaactccagtctagctgacatatccagtttcgcaaaacgacgcattttccagggcatatctgttgctcgtgtacccaagctggaatttcttaatgcctccaattcttcagtcattttagaagctaaggcctgaagataccctcgtgcatccttttcatcgctgacccactgaattatttctgtgatttgggcttcccaatgtgcaactgattctttcttgtctgctagatctttaacctcttcttctaactgctggttgtgtatacttaagttctcatacaaagtagtaagcttatcaagttcactcgtcagctttttattttcttcagttaacaacactttttctcgttcatattgttgtttgaactcactttcaaattcctccctttcactttgactttctcttctggttttttccaatttgtcttttaaaatcataatttctttgttgagagcaagttgctgaccttctgaatcatgcagttctttcttaagattttttatttcatttgcatgtattccttctcttttagataattcttcttcataaaagatacttttcttttccaaatcagtctttagtttggttatctcttgctgatgttctatgctgcatactcctggtgagtaactaatttgtttttgcttcagtccctccaattcattttccagttgcttagaatagtgctcactctgttcacgtagcttcctgtctttagatgcttcagcagctagagcttctgtatgaacttccagctcttttttggctctttctgttctgcgcagttcttgccttaagctttcaactttttgcatcaccaggtccacctcttcttccttatctcggacatggcgagcaagtttctgtttttgggtgtgcaattctgttagccgctcattgatctccatgaattcctgcatggccagtttcctctgacagtgtgcgtctttcagctctttggattggttttttaatcgctcactagcctggactagttccttatttagatcttctctttcttgttgtaacgttttgatttgtttttcataagccttgatttgtctaaaagcatcatctagttcttgcctcacagcattagcttcttcaagttgctgttccaaatgacttgattctgttacttgttttcttagtttttcaatttcttcttttaagttttttatttctaaatctttgcttgctgttagtggaccatcaacagttgaatactgcagagcttggacagtctgtgttgactcttgaagttttctactgagttcaagtttttcttgctcaaggcgcttaattcttctttcataagcttcagttgctaagttgttgtctagagtcctctgaacattaacatcaagatccagtgaggtgggaccagccgtaactcttaaacagctccgatcagaaagtacacagctactagtatatgtaaaaccaacaaatggcagatggtggccagaaaatgcagtatgtgttggtgggggcatcgtttcagaattttttaaacaatcatcatctacatcaaaattcgatgtatctgttgggctactaacttctggaatataaggtgcttcacagttccgaatattatcccaatcaattccactgaaaaatgggtgtttcttaaagtcttctattccattttgaccaagtcgatgttctctgctacaaatgagccttcgaataagatccttagcattttcagacacatcagtcacttgggctggaaactgaaacctctctttgtggttcatgatttttccgtatgtctccaccagcgattctgcataaaatggtgtttctccgtaaagcatttcatacatacagacccccaaagaccaccagtcacattcaggtccatatctcccttttccatcttccatggcttgaaggatttcaggagagatataatctggagttcctacagccactgaggactgaaccgttccatcttccatcagcttcagacaagaaccaaaatctgctaaccgaatatgtccattcatatccatcagtatattgtcaggtttaatgtctctgtgtacataatgtagctgatgaactgagtcaattgctatcaccatctcagccaagtaaaatctagccatatcttcaggcaatctatcttcaaatttgctgagtagagtaagcaaatccccaccaacataataatccataaccaggtataagttattgtcatcctggaaagcatagtgcaaggttgtaatccatttattgtctccattcactaatacatccctttcttcacgaaaacatgctgtctcagctcttttcagcatttcccatttattcaatattttcatggcaaacactttatctgcattttttagttttactacagcaacctccccaaaagctcctcgaccaatcacctttaatatttcaaagtcttctctatgtaatcgcatttgtttcactttagaagtaaatggtttagcccattctaggtattcgagaatgttcttctctcttctcaatggagaattattgcattcatcataaaggcagatgagtatatccagtaatgtctccacactgaagcactgcccattggtctgagcgggcccgtccaaaataaactgctccaactgcctcaaacgcacttctccagacatgtttgcttcgatttctgctggttttcctttaaattattatgatgacttttactattatctgaacctaaattttaaaaggtatggttttaaaaataaaccacttgttattcaaacaactgtcatgcaatgctggtgctgaattaaacatccaacacaccagtaacctcacttaactgaagcgtcttcaatttcacccatatacatatattttgagggtaaattaccataaaatatatacttaatgcatttttaaaagaatacaattaagtcgtatatttaaataaaataataattaaaagtacaacgaactagagagtcaacacttctttaaaaaaaaaaaaaaaaactcttctccttcattcaaaattcaactcgtgcaacgtaatcctgaaacgaatccggttgcatcattaatgaataaagtccgatttgcatcagcaattcacttcccgggaagaagaaaaacagaaaagggaggaaaaaaacagaatgcatagaagggggagggaaaaccaaaaatgttgctgcaaatcctcccaaccaccacttggataatgcatcagcggcaatttctccagcgggaaagggagggggcgaggtccctgaagcagcccctcggctcggagcacgccaagtcttgcccggaggcggcttttcgtttctcctcccgaggtccttctttctttaaggctttgcagtcagtcctattttcaacggattccggtgaaaactcttcattttcctcccggcttcaccctagggcctgaccggcggcgcggccgggggtggaaggcgggctgcgggcggcactggcaccgggctccggagaagcggctacttggccgcccgagcccactccatgtcggtggtcgctcgtgggccgagccgcgccgcgccgcgccgggcagagagcccggtctccccgacacccgcaccgggccgccgcgccggaggctcccgacgccccaggcgggggggtgcttctctgaattcaaaggacacaagcagcagcagctgcggcggcggcgcgggcggctctggcagctacttctcccccttcttcacacccctgggctaagggcatctttccacagcgaggagggaggcggcccggcgcaggaggaggggtcgcttccgcggctgaggagactagaggctgcggcagcccggctcccaaccactcccttcctctcccttccagccctcccccgccttccctctcctctcgcgctcgcgccctgggctcagcgaggctcctccagtcccgccgcacagaggcggaggcttgcggacgagtctggatccaatat

SEQ ID NO: 8643 - RNA, 5489 nt, Homo sapiens
  source 1..5489: mol_type = other RNA
aaatgtcacctttttgagaggaagagtctgaatccattccatggagttcacatcaaagatatcaactgcattttcactgtacaccgagagatatggtgcattgtaacaacaagaggaaggatttgctggccacatcaattcctgttgtctagatcttcggccctggcagtcagtgtatatcccaatgctgttaaaacacagcagatattctttactggagatctcaactgcgcagatagcatccattggttgatgtgcaataaatgatagtgtatggtcatttgaatggagcatactgtatggatttccttctccattcaaggggtatcttagaaatcctgactggaatcccacacagagttgttcactgaagattgccatccactggacattatatgggacttgaatttctttaaattttctgtgacgggtcttgctctgaaatagttcataacagaggacctgccttttcatagccacacacaggcatgtgagagctccatggcgcacctttccagaagttacggtttgacaccctttagtttctgacagcttgtaaaaatcggtctctcgcccatccaatgctgacataggaaaaagtcgtacatgacgatttcgtcctgagatcacagcaacaagctgatcatttggaatgagttcaatctgatgaatcttcttattgtcaccaactctaataatttcatctttggtgacatgtacaacaaataacccttcttcgtttcccaaagcaattctttcatgatctatgattgcggctgcctgggttgttttaatgaggggtagagtgctgtcataagcctctttgggaacatagactgagcggtctctgaatttgtttttcttcaaaatcttgtgcaattcactcagcactcccacccacttattcttctcattctcagtgtctgctagcatcaggattgaacatttgttattagatgctgagagctgggaagctgtgaccctaaatatacagggtatatctttccgacttgcatggataacatcagaagccaagactgaactcacagaaaattcttcatccctcatgtcaatcacttgactaatgacaacactgggctgagatgcttttccttcagcaatatcgtacagaaagagtttgaagtcacacactatagccagtgctctctgccaccctttcttcactccagctggcttaggaatcctgacatgaccttcatatgctgttcctattcctttctgaggatctatacccaggggaccttttgtctgttcaggaggaactggacaagtggttggagctttgtttacacaagttatatggcatgagaatccacacacttcacatgaacagccctgtcttattaaacccaccatcaaggaggtacactgatgacacttggtaggagtagtaaaagattttacaaaaaactggtgagtcttgcgcttaggtggaaagccagttgaaccaggacatccttttttccttaaggttggtgtgtgaactgaaagtggagtggagtctacagtacgtctgcctttgctagctggagtacaggatggagagcggtcatccaaaaaatcaatcagtgaagatgaggaagaagaaaaggaatcttcaaattgatccagagcatcggtaggcgtattcaaaaatgccaagaaagaatgctgtgagtcttggtgctctatacccttttcagatctaagctcttcagtgtcctttatcagctgttcgatttctgagagtagttccaagttcttcttctctgaatcttttagtttacattctgttatgatattagatgctttaactttattcaactcttcttggatggcctgtttggctcttatttctgcatccagagccgactgcaactccagtctagctgacatatccagtttcgcaaaacgacgcattttccagggcatatctgttgctcgtgtacccaagctggaatttcttaatgcctccaattcttcagtcattttagaagctaaggcctgaagataccctcgtgcatccttttcatcgctgacccactgaattatttctgtgatttgggcttcccaatgtgcaactgattctttcttgtctgctagatctttaacctcttcttctaactgctggttgtgtatacttaagttctcatacaaagtagtaagcttatcaagttcactcgtcagctttttattttcttcagttaacaacactttttctcgttcatattgttgtttgaactcactttcaaattcctccctttcactttgactttctcttctggttttttccaatttgtcttttaaaatcataatttctttgttgagagcaagttgctgaccttctgaatcatgcagttctttcttaagattttttatttcatttgcatgtattccttctcttttagataattcttcttcataaaagatacttttcttttccaaatcagtctttagtttggttatctcttgctgatgttctatgctgcatactcctggtgagtaactaatttgtttttgcttcagtccctccaattcattttccagttgcttagaatagtgctcactctgttcacgtagcttcctgtctttagatgcttcagcagctagagcttctgtatgaacttccagctcttttttggctctttctgttctgcgcagttcttgccttaagctttcaactttttgcatcaccaggtccacctcttcttccttatctcggacatggcgagcaagtttctgtttttgggtgtgcaattctgttagccgctcattgatctccatgaattcctgcatggccagtttcctctgacagtgtgcgtctttcagctctttggattggttttttaatcgctcactagcctggactagttccttatttagatcttctctttcttgttgtaacgttttgatttgtttttcataagccttgatttgtctaaaagcatcatctagttcttgcctcacagcattagcttcttcaagttgctgttccaaatgacttgattctgttacttgttttcttagtttttcaatttcttcttttaagttttttatttctaaatctttgcttgctgttagtggaccatcaacagttgaatactgcagagcttggacagtctgtgttgactcttgaagttttctactgagttcaagtttttcttgctcaaggcgcttaattcttctttcataagcttcagttgctaagttgttgtctagagtcctctgaacattaacatcaagatccagtgaggtgggaccagccgtaactcttaaacagctccgatcagaaagtacacagctactagtatatgtaaaaccaacaaatggcagatggtggccagaaaatgcagtatgtgttggtgggggcatcgtttcagaattttttaaacaatcatcatctacatcaaaattcgatgtatctgttgggctactaacttctggaatataaggtgcttcacagttccgaatattatcccaatcaattccactgaaaaatgggtgtttcttaaagtcttctattccattttgaccaagtcgatgttctctgctacaaatgagccttcgaataagatccttagcattttcagacacatcagtcacttgggctggaaactgaaacctctctttgtggttcatgatttttccgtatgtctccaccagcgattctgcataaaatggtgtttctccgtaaagcatttcatacatacagacccccaaagaccaccagtcacattcaggtccatatctcccttttccatcttccatggcttgaaggatttcaggagagatataatctggagttcctacagccactgaggactgaaccgttccatcttccatcagcttcagacaagaaccaaaatctgctaaccgaatatgtccattcatatccatcagtatattgtcaggtttaatgtctctgtgtacataatgtagctgatgaactgagtcaattgctatcaccatctcagccaagtaaaatctagccatatcttcaggcaatctatcttcaaatttgctgagtagagtaagcaaatccccaccaacataataatccataaccaggtataagttattgtcatcctggaaagcatagtgcaaggttgtaatccatttattgtctccattcactaatacatccctttcttcacgaaaacatgctgtctcagctcttttcagcatttcccatttattcaatattttcatggcaaacactttatctgcattttttagttttactacagcaacctccccaaaagctcctcgaccaatcacctttaatatttcaaagtcttctctatgtaatcgcatttgtttcactttagaagtaaatggtttagcccattctaggtattcgagaatgttcttctctcttctcaatggagaattattgcattcatcataaaggcagatgagtatatccagtaatgtctccacactgaagcactgcccattggtctgagcgggcccgtccaaaataaactgctccaactgcctcaaacgcacttctccagacatgtttgcttcgatttctgctggttttcctttaaattattatgatgacttttactattatctgaacctaaattttaaaaggtatggttttaaaaataaaccacttgttattcaaacaactgtcatgcaatgctggtgctgaattaaacatccaacacaccagtaacctcacttaactgaagcgtcttcaatttcacccatatacatatattttgagggtaaattaccataaaatatatacttaatgcatttttaaaagaatacaattaagtcgtatatttaaataaaataataattaaaagtacaacgaactagagagtcaacacttctttaaaaaaaaaaaaaaaaactcttctccttcattcaaaattcaactcgtgcaacgtaatcctgaaacgaatccggttgcatcattaatgaataaagtccgatttgcatcagcaattcacttcccgggaagaagaaaaacagaaaagggaggaaaaaaacagaatgcatagaagggggagggaaaaccaaaaatgttgctgcaaatcctcccaaccaccacttggataatgcatcagcggcaatttctccagcgggaaagggagggggcgaggtccctgaagcagcccctcggctcggagcacgccaagtcttgcccggaggcggcttttcgtttctcctcccgaggtccttctttctttaaggctttgcagtcagtcctattttcaacggattccggtgaaaactcttcattttcctcccggcttcaccctagggcctgaccggcggcgcggccgggggtggaaggcgggctgcgggcggcactggcaccgggctccggagaagcggctacttggccgcccgagcccactccatgtcggtggtcgctcgtgggccgagccgcgccgcgccgcgccgggcagagagcccggtctccccgacacccgcaccgggccgccgcgccggaggctcccgacgcccca

SEQ ID NO: 8644 - RNA, 5624 nt, Homo sapiens
  source 1..5624: mol_type = other RNA
aaatgtcacctttttgagaggaagagtctgaatccattccatggagttcacatcaaagatatcaactgcattttcactgtacaccgagagatatggtgcattgtaacaacaagaggaaggatttgctggccacatcaattcctgttgtctagatcttcggccctggcagtcagtgtatatcccaatgctgttaaaacacagcagatattctttactggagatctcaactgcgcagatagcatccattggttgatgtgcaataaatgatagtgtatggtcatttgaatggagcatactgtatggatttccttctccattcaaggggtatcttagaaatcctgactggaatcccacacagagttgttcactgaagattgccatccactggacattatatgggacttgaatttctttaaattttctgtgacgggtcttgctctgaaatagttcataacagaggacctgccttttcatagccacacacaggcatgtgagagctccatggcgcacctttccagaagttacggtttgacaccctttagtttctgacagcttgtaaaaatcggtctctcgcccatccaatgctgacataggaaaaagtcgtacatgacgatttcgtcctgagatcacagcaacaagctgatcatttggaatgagttcaatctgatgaatcttcttattgtcaccaactctaataatttcatctttggtgacatgtacaacaaataacccttcttcgtttcccaaagcaattctttcatgatctatgattgcggctgcctgggttgttttaatgaggggtagagtgctgtcataagcctctttgggaacatagactgagcggtctctgaatttgtttttcttcaaaatcttgtgcaattcactcagcactcccacccacttattcttctcattctcagtgtctgctagcatcaggattgaacatttgttattagatgctgagagctgggaagctgtgaccctaaatatacagggtatatctttccgacttgcatggataacatcagaagccaagactgaactcacagaaaattcttcatccctcatgtcaatcacttgactaatgacaacactgggctgagatgcttttccttcagcaatatcgtacagaaagagtttgaagtcacacactatagccagtgctctctgccaccctttcttcactccagctggcttaggaatcctgacatgaccttcatatgctgttcctattcctttctgaggatctatacccaggggaccttttgtctgttcaggaggaactggacaagtggttggagctttgtttacacaagttatatggcatgagaatccacacacttcacatgaacagccctgtcttattaaacccaccatcaaggaggtacactgatgacacttggtaggagtagtaaaagattttacaaaaaactggtgagtcttgcgcttaggtggaaagccagttgaaccaggacatccttttttccttaaggttggtgtgtgaactgaaagtggagtggagtctacagtacgtctgcctttgctagctggagtacaggatggagagcgttcaaattgatccagagcatcggtaggcgtattcaaaaatgccaagaaagaatgctgtgagtcttggtgctctatacccttttcagatctaagctcttcagtgtcctttatcagctgttcgatttctgagagtagttccaagttcttcttctctgaatcttttagtttacattctgttatgatattagatgctttaactttattcaactcttcttggatggcctgtttggctcttatttctgcatccagagccgactgcaactccagtctagctgacatatccagtttcgcaaaacgacgcattttccagggcatatctgttgctcgtgtacccaagctggaatttcttaatgcctccaattcttcagtcattttagaagctaaggcctgaagataccctcgtgcatccttttcatcgctgacccactgaattatttctgtgatttgggcttcccaatgtgcaactgattctttcttgtctgctagatctttaacctcttcttctaactgctggttgtgtatacttaagttctcatacaaagtagtaagcttatcaagttcactcgtcagctttttattttcttcagttaacaacactttttctcgttcatattgttgtttgaactcactttcaaattcctccctttcactttgactttctcttctggttttttccaatttgtcttttaaaatcataatttctttgttgagagcaagttgctgaccttctgaatcatgcagttctttcttaagattttttatttcatttgcatgtattccttctcttttagataattcttcttcataaaagatacttttcttttccaaatcagtctttagtttggttatctcttgctgatgttctatgctgcatactcctggtgagtaactaatttgtttttgcttcagtccctccaattcattttccagttgcttagaatagtgctcactctgttcacgtagcttcctgtctttagatgcttcagcagctagagcttctgtatgaacttccagctcttttttggctctttctgttctgcgcagttcttgccttaagctttcaactttttgcatcaccaggtccacctcttcttccttatctcggacatggcgagcaagtttctgtttttgggtgtgcaattctgttagccgctcattgatctccatgaattcctgcatggccagtttcctctgacagtgtgcgtctttcagctctttggattggttttttaatcgctcactagcctggactagttccttatttagatcttctctttcttgttgtaacgttttgatttgtttttcataagccttgatttgtctaaaagcatcatctagttcttgcctcacagcattagcttcttcaagttgctgttccaaatgacttgattctgttacttgttttcttagtttttcaatttcttcttttaagttttttatttctaaatctttgcttgctgttagtggaccatcaacagttgaatactgcagagcttggacagtctgtgttgactcttgaagttttctactgagttcaagtttttcttgctcaaggcgcttaattcttctttcataagcttcagttgctaagttgttgtctagagtcctctgaacattaacatcaagatccagtgaggtgggaccagccgtaactcttaaacagctccgatcagaaagtacacagctactagtatatgtaaaaccaacaaatggcagatggtggccagaaaatgcagtatgtgttggtgggggcatcgtttcagaattttttaaacaatcatcatctacatcaaaattcgatgtatctgttgggctactaacttctggaatataaggtgcttcacagttccgaatattatcccaatcaattccactgaaaaatgggtgtttcttaaagtcttctattccattttgaccaagtcgatgttctctgctacaaatgagccttcgaataagatccttagcattttcagacacatcagtcacttgggctggaaactgaaacctctctttgtggttcatgatttttccgtatgtctccaccagcgattctgcataaaatggtgtttctccgtaaagcatttcatacatacagacccccaaagaccaccagtcacattcaggtccatatctcccttttccatcttccatggcttgaaggatttcaggagagatataatctggagttcctacagccactgaggactgaaccgttccatcttccatcagcttcagacaagaaccaaaatctgctaaccgaatatgtccattcatatccatcagtatattgtcaggtttaatgtctctgtgtacataatgtagctgatgaactgagtcaattgctatcaccatctcagccaagtaaaatctagccatatcttcaggcaatctatcttcaaatttgctgagtagagtaagcaaatccccaccaacataataatccataaccaggtataagttattgtcatcctggaaagcatagtgcaaggttgtaatccatttattgtctccattcactaatacatccctttcttcacgaaaacatgctgtctcagctcttttcagcatttcccatttattcaatattttcatggcaaacactttatctgcattttttagttttactacagcaacctccccaaaagctcctcgaccaatcacctttaatatttcaaagtcttctctatgtaatcgcatttgtttcactttagaagtaaatggtttagcccattctaggtattcgagaatgttcttctctcttctcaatggagaattattgcattcatcataaaggcagatgagtatatccagtaatgtctccacactgaagcactgcccattggtctgagcgggcccgtccaaaataaactgctccaactgcctcaaacgcacttctccagacatgtttgcttcgatttctgctggttttcctttaaattattatgatgacttttactattatctgaacctaaattttaaaaggtatggttttaaaaataaaccacttgttattcaaacaactgtcatgcaatgctggtgctgaattaaacatccaacacaccagtaacctcacttaactgaagcgtcttcaatttcacccatatacatatattttgagggtaaattaccataaaatatatacttaatgcatttttaaaagaatacaattaagtcgtatatttaaataaaataataattaaaagtacaacgaactagagagtcaacacttctttaaaaaaaaaaaaaaaaactcttctccttcattcaaaattcaactcgtgcaacgtaatcctgaaacgaatccggttgcatcattaatgaataaagtccgatttgcatcagcaattcacttcccgggaagaagaaaaacagaaaagggaggaaaaaaacagaatgcatagaagggggagggaaaaccaaaaatgttgctgcaaatcctcccaaccaccacttggataatgcatcagcggcaatttctccagcgggaaagggagggggcgaggtccctgaagcagcccctcggctcggagcacgccaagtcttgcccggaggcggcttttcgtttctcctcccgaggtccttctttctttaaggctttgcagtcagtcctattttcaacggattccggtgaaaactcttcattttcctcccggcttcaccctagggcctgaccggcggcgcggccgggggtggaaggcgggctgcgggcggcactggcaccgggctccggagaagcggctacttggccgcccgagcccactccatgtcggtggtcgctcgtgggccgagccgcgccgcgccgcgccgggcagagagcccggtctccccgacacccgcaccgggccgccgcgccggaggctcccgacgccccaggcgggggggtgcttctctgaattcaaaggacacaagcagcagcagctgcggcggcggcgcgggcggctctggcagctacttctcccccttcttcacacccctgggctaagggcatctttccacagcgaggagggaggcggcccggcgcaggaggaggggtcgcttccgcggctgaggagact

SEQ ID NO: 8645 - RNA, 5783 nt, Homo sapiens
  source 1..5783: mol_type = other RNA
aaatgtcacctttttgagaggaagagtctgaatccattccatggagttcacatcaaagatatcaactgcattttcactgtacaccgagagatatggtgcattgtaacaacaagaggaaggatttgctggccacatcaattcctgttgtctagatcttcggccctggcagtcagtgtatatcccaatgctgttaaaacacagcagatattctttactggagatctcaactgcgcagatagcatccattggttgatgtgcaataaatgatagtgtatggtcatttgaatggagcatactgtatggatttccttctccattcaaggggtatcttagaaatcctgactggaatcccacacagagttgttcactgaagattgccatccactggacattatatgggacttgaatttctttaaattttctgtgacgggtcttgctctgaaatagttcataacagaggacctgccttttcatagccacacacaggcatgtgagagctccatggcgcacctttccagaagttacggtttgacaccctttagtttctgacagcttgtaaaaatcggtctctcgcccatccaatgctgacataggaaaaagtcgtacatgacgatttcgtcctgagatcacagcaacaagctgatcatttggaatgagttcaatctgatgaatcttcttattgtcaccaactctaataatttcatctttggtgacatgtacaacaaataacccttcttcgtttcccaaagcaattctttcatgatctatgattgcggctgcctgggttgttttaatgaggggtagagtgctgtcataagcctctttgggaacatagactgagcggtctctgaatttgtttttcttcaaaatcttgtgcaattcactcagcactcccacccacttattcttctcattctcagtgtctgctagcatcaggattgaacatttgttattagatgctgagagctgggaagctgtgaccctaaatatacagggtatatctttccgacttgcatggataacatcagaagccaagactgaactcacagaaaattcttcatccctcatgtcaatcacttgactaatgacaacactgggctgagatgcttttccttcagcaatatcgtacagaaagagtttgaagtcacacactatagccagtgctctctgccaccctttcttcactccagctggcttaggaatcctgacatgaccttcatatgctgttcctattcctttctgaggatctatacccaggggaccttttgtctgttcaggaggaactggacaagtggttggagctttgtttacacaagttatatggcatgagaatccacacacttcacatgaacagccctgtcttattaaacccaccatcaaggaggtacactgatgacacttggtaggagtagtaaaagattttacaaaaaactggtgagtcttgcgcttaggtggaaagccagttgaaccaggacatccttttttccttaaggttggtgtgtgaactgaaagtggagtggagtctacagtacgtctgcctttgctagctggagtacaggatggagagcgttcaaattgatccagagcatcggtaggcgtattcaaaaatgccaagaaagaatgctgtgagtcttggtgctctatacccttttcagatctaagctcttcagtgtcctttatcagctgttcgatttctgagagtagttccaagttcttcttctctgaatcttttagtttacattctgttatgatattagatgctttaactttattcaactcttcttggatggcctgtttggctcttatttctgcatccagagccgactgcaactccagtctagctgacatatccagtttcgcaaaacgacgcattttccagggcatatctgttgctcgtgtacccaagctggaatttcttaatgcctccaattcttcagtcattttagaagctaaggcctgaagataccctcgtgcatccttttcatcgctgacccactgaattatttctgtgatttgggcttcccaatgtgcaactgattctttcttgtctgctagatctttaacctcttcttctaactgctggttgtgtatacttaagttctcatacaaagtagtaagcttatcaagttcactcgtcagctttttattttcttcagttaacaacactttttctcgttcatattgttgtttgaactcactttcaaattcctccctttcactttgactttctcttctggttttttccaatttgtcttttaaaatcataatttctttgttgagagcaagttgctgaccttctgaatcatgcagttctttcttaagattttttatttcatttgcatgtattccttctcttttagataattcttcttcataaaagatacttttcttttccaaatcagtctttagtttggttatctcttgctgatgttctatgctgcatactcctggtgagtaactaatttgtttttgcttcagtccctccaattcattttccagttgcttagaatagtgctcactctgttcacgtagcttcctgtctttagatgcttcagcagctagagcttctgtatgaacttccagctcttttttggctctttctgttctgcgcagttcttgccttaagctttcaactttttgcatcaccaggtccacctcttcttccttatctcggacatggcgagcaagtttctgtttttgggtgtgcaattctgttagccgctcattgatctccatgaattcctgcatggccagtttcctctgacagtgtgcgtctttcagctctttggattggttttttaatcgctcactagcctggactagttccttatttagatcttctctttcttgttgtaacgttttgatttgtttttcataagccttgatttgtctaaaagcatcatctagttcttgcctcacagcattagcttcttcaagttgctgttccaaatgacttgattctgttacttgttttcttagtttttcaatttcttcttttaagttttttatttctaaatctttgcttgctgttagtggaccatcaacagttgaatactgcagagcttggacagtctgtgttgactcttgaagttttctactgagttcaagtttttcttgctcaaggcgcttaattcttctttcataagcttcagttgctaagttgttgtctagagtcctctgaacattaacatcaagatccagtgaggtgggaccagccgtaactcttaaacagctccgatcagaaagtacacagctactagtatatgtaaaaccaacaaatggcagatggtggccagaaaatgcagtatgtgttggtgggggcatcgtttcagaattttttaaacaatcatcatctacatcaaaattcgatgtatctgttgggctactaacttctggaatataaggtgcttcacagttccgaatattatcccaatcaattccactgaaaaatgggtgtttcttaaagtcttctattccattttgaccaagtcgatgttctctgctacaaatgagccttcgaataagatccttagcattttcagacacatcagtcacttgggctggaaactgaaacctctctttgtggttcatgatttttccgtatgtctccaccagcgattctgcataaaatggtgtttctccgtaaagcatttcatacatacagacccccaaagaccaccagtcacattcaggtccatatctcccttttccatcttccatggcttgaaggatttcaggagagatataatctggagttcctacagccactgaggactgaaccgttccatcttccatcagcttcagacaagaaccaaaatctgctaaccgaatatgtccattcatatccatcagtatattgtcaggtttaatgtctctgtgtacataatgtagctgatgaactgagtcaattgctatcaccatctcagccaagtaaaatctagccatatcttcaggcaatctatcttcaaatttgctgagtagagtaagcaaatccccaccaacataataatccataaccaggtataagttattgtcatcctggaaagcatagtgcaaggttgtaatccatttattgtctccattcactaatacatccctttcttcacgaaaacatgctgtctcagctcttttcagcatttcccatttattcaatattttcatggcaaacactttatctgcattttttagttttactacagcaacctccccaaaagctcctcgaccaatcacctttaatatttcaaagtcttctctatgtaatcgcatttgtttcactttagaagtaaatggtttagcccattctaggtattcgagaatgttcttctctcttctcaatggagaattattgcattcatcataaaggcagatgagtatatccagtaatgtctccacactgaagcactgcccattggtctgagcgggcccgtccaaaataaactgctccaactgcctcaaacgcacttctccagacatgtttgcttcgatttctgctggttttcctttaaattattatgatgacttttactattatctgaacctaaattttaaaaggtatggttttaaaaataaaccacttgttattcaaacaactgtcatgcaatgctggtgctgaattaaacatccaacacaccagtaacctcacttaactgaagcgtcttcaatttcacccatatacatatattttgagggtaaattaccataaaatatatacttaatgcatttttaaaagaatacaattaagtcgtatatttaaataaaataataattaaaagtacaacgaactagagagtcaacacttctttaaaaaaaaaaaaaaaaactcttctccttcattcaaaattcaactcgtgcaacgtaatcctgaaacgaatccggttgcatcattaatgaataaagtccgatttgcatcagcaattcacttcccgggaagaagaaaaacagaaaagggaggaaaaaaacagaatgcatagaagggggagggaaaaccaaaaatgttgctgcaaatcctcccaaccaccacttggataatgcatcagcggcaatttctccagcgggaaagggagggggcgaggtccctgaagcagcccctcggctcggagcacgccaagtcttgcccggaggcggcttttcgtttctcctcccgaggtccttctttctttaaggctttgcagtcagtcctattttcaacggattccggtgaaaactcttcattttcctcccggcttcaccctagggcctgaccggcggcgcggccgggggtggaaggcgggctgcgggcggcactggcaccgggctccggagaagcggctacttggccgcccgagcccactccatgtcggtggtcgctcgtgggccgagccgcgccgcgccgcgccgggcagagagcccggtctccccgacacccgcaccgggccgccgcgccggaggctcccgacgccccaggcgggggggtgcttctctgaattcaaaggacacaagcagcagcagctgcggcggcggcgcgggcggctctggcagctacttctcccccttcttcacacccctgggctaagggcatctttccacagcgaggagggaggcggcccggcgcaggaggaggggtcgcttccgcggctgaggagactagaggctgcggcagcccggctcccaaccactcccttcctctcccttccagccctcccccgccttccctctcctctcgcgctcgcgccctgggctcagcgaggctcctccagtcccgccgcacagaggcggaggcttgcggacgagtctggatccaatat

SEQ ID NO: 8646 - RNA, 5854 nt, Homo sapiens
  source 1..5854: mol_type = other RNA
aaatgtcacctttttgagaggaagagtctgaatccattccatggagttcacatcaaagatatcaactgcattttcactgtacaccgagagatatggtgcattgtaacaacaagaggaaggatttgctggccacatcaattcctgttgtctagatcttcggccctggcagtcagtgtatatcccaatgctgttaaaacacagcagatattctttactggagatctcaactgcgcagatagcatccattggttgatgtgcaataaatgatagtgtatggtcatttgaatggagcatactgtatggatttccttctccattcaaggggtatcttagaaatcctgactggaatcccacacagagttgttcactgaagattgccatccactggacattatatgggacttgaatttctttaaattttctgtgacgggtcttgctctgaaatagttcataacagaggacctgccttttcatagccacacacaggcatgtgagagctccatggcgcacctttccagaagttacggtttgacaccctttagtttctgacagcttgtaaaaatcggtctctcgcccatccaatgctgacataggaaaaagtcgtacatgacgatttcgtcctgagatcacagcaacaagctgatcatttggaatgagttcaatctgatgaatcttcttattgtcaccaactctaataatttcatctttggtgacatgtacaacaaataacccttcttcgtttcccaaagcaattctttcatgatctatgattgcggctgcctgggttgttttaatgaggggtagagtgctgtcataagcctctttgggaacatagactgagcggtctctgaatttgtttttcttcaaaatcttgtgcaattcactcagcactcccacccacttattcttctcattctcagtgtctgctagcatcaggattgaacatttgttattagatgctgagagctgggaagctgtgaccctaaatatacagggtatatctttccgacttgcatggataacatcagaagccaagactgaactcacagaaaattcttcatccctcatgtcaatcacttgactaatgacaacactgggctgagatgcttttccttcagcaatatcgtacagaaagagtttgaagtcacacactatagccagtgctctctgccaccctttcttcactccagctggcttaggaatcctgacatgaccttcatatgctgttcctattcctttctgaggatctatacccaggggaccttttgtctgttcaggaggaactggacaagtggttggagctttgtttacacaagttatatggcatgagaatccacacacttcacatgaacagccctgtcttattaaacccaccatcaaggaggtacactgatgacacttggtaggagtagtaaaagattttacaaaaaactggtgagtcttgcgcttaggtggaaagccagttgaaccaggacatccttttttccttaaggttggtgtgtgaactgaaagtggagtggagtctacagtcttaactggctcagcttcactagatgtggaaggagatgtggaccgtgactggatgtgaaacttgacgctcgggttccatacatatgtgttctcaacgggatcagtacgtctgcctttgctagctggagtacaggatggagagcggtcatccaaaaaatcaatcagtgaagatgaggaagaagaaaaggaatcttcaaattgatccagagcatcggtaggcgtattcaaaaatgccaagaaagaatgctgtgagtcttggtgctctatacccttttcagatctaagctcttcagtgtcctttatcagctgttcgatttctgagagtagttccaagttcttcttctctgaatcttttagtttacattctgttatgatattagatgctttaactttattcaactcttcttggatggcctgtttggctcttatttctgcatccagagccgactgcaactccagtctagctgacatatccagtttcgcaaaacgacgcattttccagggcatatctgttgctcgtgtacccaagctggaatttcttaatgcctccaattcttcagtcattttagaagctaaggcctgaagataccctcgtgcatccttttcatcgctgacccactgaattatttctgtgatttgggcttcccaatgtgcaactgattctttcttgtctgctagatctttaacctcttcttctaactgctggttgtgtatacttaagttctcatacaaagtagtaagcttatcaagttcactcgtcagctttttattttcttcagttaacaacactttttctcgttcatattgttgtttgaactcactttcaaattcctccctttcactttgactttctcttctggttttttccaatttgtcttttaaaatcataatttctttgttgagagcaagttgctgaccttctgaatcatgcagttctttcttaagattttttatttcatttgcatgtattccttctcttttagataattcttcttcataaaagatacttttcttttccaaatcagtctttagtttggttatctcttgctgatgttctatgctgcatactcctggtgagtaactaatttgtttttgcttcagtccctccaattcattttccagttgcttagaatagtgctcactctgttcacgtagcttcctgtctttagatgcttcagcagctagagcttctgtatgaacttccagctcttttttggctctttctgttctgcgcagttcttgccttaagctttcaactttttgcatcaccaggtccacctcttcttccttatctcggacatggcgagcaagtttctgtttttgggtgtgcaattctgttagccgctcattgatctccatgaattcctgcatggccagtttcctctgacagtgtgcgtctttcagctctttggattggttttttaatcgctcactagcctggactagttccttatttagatcttctctttcttgttgtaacgttttgatttgtttttcataagccttgatttgtctaaaagcatcatctagttcttgcctcacagcattagcttcttcaagttgctgttccaaatgacttgattctgttacttgttttcttagtttttcaatttcttcttttaagttttttatttctaaatctttgcttgctgttagtggaccatcaacagttgaatactgcagagcttggacagtctgtgttgactcttgaagttttctactgagttcaagtttttcttgctcaaggcgcttaattcttctttcataagcttcagttgctaagttgttgtctagagtcctctgaacattaacatcaagatccagtgaggtgggaccagccgtaactcttaaacagctccgatcagaaagtacacagctactagtatatgtaaaaccaacaaatggcagatggtggccagaaaatgcagtatgtgttggtgggggcatcgtttcagaattttttaaacaatcatcatctacatcaaaattcgatgtatctgttgggctactaacttctggaatataaggtgcttcacagttccgaatattatcccaatcaattccactgaaaaatgggtgtttcttaaagtcttctattccattttgaccaagtcgatgttctctgctacaaatgagccttcgaataagatccttagcattttcagacacatcagtcacttgggctggaaactgaaacctctctttgtggttcatgatttttccgtatgtctccaccagcgattctgcataaaatggtgtttctccgtaaagcatttcatacatacagacccccaaagaccaccagtcacattcaggtccatatctcccttttccatcttccatggcttgaaggatttcaggagagatataatctggagttcctacagccactgaggactgaaccgttccatcttccatcagcttcagacaagaaccaaaatctgctaaccgaatatgtccattcatatccatcagtatattgtcaggtttaatgtctctgtgtacataatgtagctgatgaactgagtcaattgctatcaccatctcagccaagtaaaatctagccatatcttcaggcaatctatcttcaaatttgctgagtagagtaagcaaatccccaccaacataataatccataaccaggtataagttattgtcatcctggaaagcatagtgcaaggttgtaatccatttattgtctccattcactaatacatccctttcttcacgaaaacatgctgtctcagctcttttcagcatttcccatttattcaatattttcatggcaaacactttatctgcattttttagttttactacagcaaccccattctaggtattcgagaatgttcttctctcttctcaatggagaattattgcattcatcataaaggcagatgagtatatccagtaatgtctccacactgaagcactgcccattggtctgagcgggcccgtccaaaataaactgctccaactgcctcaaacgcacttctccagacatgtttgcttcgatttctgctggttttcctttaaattattatgatgacttttactattatctgaacctaaattttaaaaggtatggttttaaaaataaaccacttgttattcaaacaactgtcatgcaatgctggtgctgaattaaacatccaacacaccagtaacctcacttaactgaagcgtcttcaatttcacccatatacatatattttgagggtaaattaccataaaatatatacttaatgcatttttaaaagaatacaattaagtcgtatatttaaataaaataataattaaaagtacaacgaactagagagtcaacacttctttaaaaaaaaaaaaaaaaactcttctccttcattcaaaattcaactcgtgcaacgtaatcctgaaacgaatccggttgcatcattaatgaataaagtccgatttgcatcagcaattcacttcccgggaagaagaaaaacagaaaagggaggaaaaaaacagaatgcatagaagggggagggaaaaccaaaaatgttgctgcaaatcctcccaaccaccacttggataatgcatcagcggcaatttctccagcgggaaagggagggggcgaggtccctgaagcagcccctcggctcggagcacgccaagtcttgcccggaggcggcttttcgtttctcctcccgaggtccttctttctttaaggctttgcagtcagtcctattttcaacggattccggtgaaaactcttcattttcctcccggcttcaccctagggcctgaccggcggcgcggccgggggtggaaggcgggctgcgggcggcactggcaccgggctccggagaagcggctacttggccgcccgagcccactccatgtcggtggtcgctcgtgggccgagccgcgccgcgccgcgccgggcagagagcccggtctccccgacacccgcaccgggccgccgcgccggaggctcccgacgccccaggcgggggggtgcttctctgaattcaaaggacacaagcagcagcagctgcggcggcggcgcgggcggctctggcagctacttctcccccttcttcacacccctgggctaagggcatctttccacagcgaggagggaggcggcccggcgcaggaggaggggtcgcttccgcggctgaggagactagaggctgcggcagcccggctcccaaccactcccttcctctcccttccagccctcccccgccttccctctcctctcgcgctcgcgccctgggctcagcgaggctcctccagtcccgccgcacagaggcggaggcttgcggacgagtctggatccaatatggcggcctgg

SEQ ID NO: 8647 - RNA, 5594 nt, Homo sapiens
  source 1..5594: mol_type = other RNA
aaatgtcacctttttgagaggaagagtctgaatccattccatggagttcacatcaaagatatcaactgcattttcactgtacaccgagagatatggtgcattgtaacaacaagaggaaggatttgctggccacatcaattcctgttgtctagatcttcggccctggcagtcagtgtatatcccaatgctgttaaaacacagcagatattctttactggagatctcaactgcgcagatagcatccattggttgatgtgcaataaatgatagtgtatggtcatttgaatggagcatactgtatggatttccttctccattcaaggggtatcttagaaatcctgactggaatcccacacagagttgttcactgaagattgccatccactggacattatatgggacttgaatttctttaaattttctgtgacgggtcttgctctgaaatagttcataacagaggacctgccttttcatagccacacacaggcatgtgagagctccatggcgcacctttccagaagttacggtttgacaccctttagtttctgacagcttgtaaaaatcggtctctcgcccatccaatgctgacataggaaaaagtcgtacatgacgatttcgtcctgagatcacagcaacaagctgatcatttggaatgagttcaatctgatgaatcttcttattgtcaccaactctaataatttcatctttggtgacatgtacaacaaataacccttcttcgtttcccaaagcaattctttcatgatctatgattgcggctgcctgggttgttttaatgaggggtagagtgctgtcataagcctctttgggaacatagactgagcggtctctgaatttgtttttcttcaaaatcttgtgcaattcactcagcactcccacccacttattcttctcattctcagtgtctgctagcatcaggattgaacatttgttattagatgctgagagctgggaagctgtgaccctaaatatacagggtatatctttccgacttgcatggataacatcagaagccaagactgaactcacagaaaattcttcatccctcatgtcaatcacttgactaatgacaacactgggctgagatgcttttccttcagcaatatcgtacagaaagagtttgaagtcacacactatagccagtgctctctgccaccctttcttcactccagctggcttaggaatcctgacatgaccttcatatgctgttcctattcctttctgaggatctatacccaggggaccttttgtctgttcaggaggaactggacaagtggttggagctttgtttacacaagttatatggcatgagaatccacacacttcacatgaacagccctgtcttattaaacccaccatcaaggaggtacactgatgacacttggtaggagtagtaaaagattttacaaaaaactggtgagtcttgcgcttaggtggaaagccagttgaaccaggacatccttttttccttaaggttggtgtgtgaactgaaagtggagtggagtctacagtcttaactggctcagcttcactagatgtggaaggagatgtggaccgtgactggatgtgaaacttgacgctcgggttccatacatatgtgttctcaacgggatcagtacgtctgcctttgctagctggagtacaggatggagagcggtcatccaaaaaatcaatcagtgaagatgaggaagaagaaaaggaatcttcaaattgatccagagcatcggtaggcgtattcaaaaatgccaagaaagaatgctgtgagtcttggtgctctatacccttttcagatctaagctcttcagtgtcctttatcagctgttcgatttctgagagtagttccaagttcttcttctctgaatcttttagtttacattctgttatgatattagatgctttaactttattcaactcttcttggatggcctgtttggctcttatttctgcatccagagccgactgcaactccagtctagctgacatatccagtttcgcaaaacgacgcattttccagggcatatctgttgctcgtgtacccaagctggaatttcttaatgcctccaattcttcagtcattttagaagctaaggcctgaagataccctcgtgcatccttttcatcgctgacccactgaattatttctgtgatttgggcttcccaatgtgcaactgattctttcttgtctgctagatctttaacctcttcttctaactgctggttgtgtatacttaagttctcatacaaagtagtaagcttatcaagttcactcgtcagctttttattttcttcagttaacaacactttttctcgttcatattgttgtttgaactcactttcaaattcctccctttcactttgactttctcttctggttttttccaatttgtcttttaaaatcataatttctttgttgagagcaagttgctgaccttctgaatcatgcagttctttcttaagattttttatttcatttgcatgtattccttctcttttagataattcttcttcataaaagatacttttcttttccaaatcagtctttagtttggttatctcttgctgatgttctatgctgcatactcctggtgagtaactaatttgtttttgcttcagtccctccaattcattttccagttgcttagaatagtgctcactctgttcacgtagcttcctgtctttagatgcttcagcagctagagcttctgtatgaacttccagctcttttttggctctttctgttctgcgcagttcttgccttaagctttcaactttttgcatcaccaggtccacctcttcttccttatctcggacatggcgagcaagtttctgtttttgggtgtgcaattctgttagccgctcattgatctccatgaattcctgcatggccagtttcctctgacagtgtgcgtctttcagctctttggattggttttttaatcgctcactagcctggactagttccttatttagatcttctctttcttgttgtaacgttttgatttgtttttcataagccttgatttgtctaaaagcatcatctagttcttgcctcacagcattagcttcttcaagttgctgttccaaatgacttgattctgttacttgttttcttagtttttcaatttcttcttttaagttttttatttctaaatctttgcttgctgttagtggaccatcaacagttgaatactgcagagcttggacagtctgtgttgactcttgaagttttctactgagttcaagtttttcttgctcaaggcgcttaattcttctttcataagcttcagttgctaagttgttgtctagagtcctctgaacattaacatcaagatccagtgaggtgggaccagccgtaactcttaaacagctccgatcagaaagtacacagctactagtatatgtaaaaccaacaaatggcagatggtggccagaaaatgcagtatgtgttggtgggggcatcgtttcagaattttttaaacaatcatcatctacatcaaaattcgatgtatctgttgggctactaacttctggaatataaggtgcttcacagttccgaatattatcccaatcaattccactgaaaaatgggtgtttcttaaagtcttctattccattttgaccaagtcgatgttctctgctacaaatgagccttcgaataagatccttagcattttcagacacatcagtcacttgggctggaaactgaaacctctctttgtggttcatgatttttccgtatgtctccaccagcgattctgcataaaatggtgtttctccgtaaagcatttcatacatacagacccccaaagaccaccagtcacattcaggtccatatctcccttttccatcttccatggcttgaaggatttcaggagagatataatctggagttcctacagccactgaggactgaaccgttccatcttccatcagcttcagacaagaaccaaaatctgctaaccgaatatgtccattcatatccatcagtatattgtcaggtttaatgtctctgtgtacataatgtagctgatgaactgagtcaattgctatcaccatctcagccaagtaaaatctagccatatcttcaggcaatctatcttcaaatttgctgagtagagtaagcaaatccccaccaacataataatccataaccaggtataagttattgtcatcctggaaagcatagtgcaaggttgtaatccatttattgtctccattcactaatacatccctttcttcacgaaaacatgctgtctcagctcttttcagcatttcccatttattcaatattttcatggcaaacactttatctgcattttttagttttactacagcaacctccccaaaagctcctcgaccaatcacctttaatatttcaaagtcttctctatgtaatcgcatttgtttcactttagaagtaaatggtttagcccattctaggtattcgagaatgttcttctctcttctcaatggagaattattgcattcatcataaaggcagatgagtatatccagtaatgtctccacactgaagcactgcccattggtctgagcgggcccgtccaaaataaactgctccaactgcctcaaacgcacttctccagacatgtttgcttcgatttctgctggttttcctttaaattattatgatgacttttactattatctgaacctaaattttaaaaggtatggttttaaaaataaaccacttgttattcaaacaactgtcatgcaatgctggtgctgaattaaacatccaacacaccagtaacctcacttaactgaagcgtcttcaatttcacccatatacatatattttgagggtaaattaccataaaatatatacttaatgcatttttaaaagaatacaattaagtcgtatatttaaataaaataataattaaaagtacaacgaactagagagtcaacacttctttaaaaaaaaaaaaaaaaactcttctccttcattcaaaattcaactcgtgcaacgtaatcctgaaacgaatccggttgcatcattaatgaataaagtccgatttgcatcagcaattcacttcccgggaagaagaaaaacagaaaagggaggaaaaaaacagaatgcatagaagggggagggaaaaccaaaaatgttgctgcaaatcctcccaaccaccacttggataatgcatcagcggcaatttctccagcgggaaagggagggggcgaggtccctgaagcagcccctcggctcggagcacgccaagtcttgcccggaggcggcttttcgtttctcctcccgaggtccttctttctttaaggctttgcagtcagtcctattttcaacggattccggtgaaaactcttcattttcctcccggcttcaccctagggcctgaccggcggcgcggccgggggtggaaggcgggctgcgggcggcactggcaccgggctccggagaagcggctacttggccgcccgagcccactccatgtcggtggtcgctcgtgggccgagccgcgccgcgccgcgccgggcagagagcccggtctccccgacacccgcaccgggccgccgcgccggaggctcccgacgcccca

SEQ ID NO: 8648 - RNA, 5936 nt, Homo sapiens
  source 1..5936: mol_type = other RNA
aaatgtcacctttttgagaggaagagtctgaatccattccatggagttcacatcaaagatatcaactgcattttcactgtacaccgagagatatggtgcattgtaacaacaagaggaaggatttgctggccacatcaattcctgttgtctagatcttcggccctggcagtcagtgtatatcccaatgctgttaaaacacagcagatattctttactggagatctcaactgcgcagatagcatccattggttgatgtgcaataaatgatagtgtatggtcatttgaatggagcatactgtatggatttccttctccattcaaggggtatcttagaaatcctgactggaatcccacacagagttgttcactgaagattgccatccactggacattatatgggacttgaatttctttaaattttctgtgacgggtcttgctctgaaatagttcataacagaggacctgccttttcatagccacacacaggcatgtgagagctccatggcgcacctttccagaagttacggtttgacaccctttagtttctgacagcttgtaaaaatcggtctctcgcccatccaatgctgacataggaaaaagtcgtacatgacgatttcgtcctgagatcacagcaacaagctgatcatttggaatgagttcaatctgatgaatcttcttattgtcaccaactctaataatttcatctttggtgacatgtacaacaaataacccttcttcgtttcccaaagcaattctttcatgatctatgattgcggctgcctgggttgttttaatgaggggtagagtgctgtcataagcctctttgggaacatagactgagcggtctctgaatttgtttttcttcaaaatcttgtgcaattcactcagcactcccacccacttattcttctcattctcagtgtctgctagcatcaggattgaacatttgttattagatgctgagagctgggaagctgtgaccctaaatatacagggtatatctttccgacttgcatggataacatcagaagccaagactgaactcacagaaaattcttcatccctcatgtcaatcacttgactaatgacaacactgggctgagatgcttttccttcagcaatatcgtacagaaagagtttgaagtcacacactatagccagtgctctctgccaccctttcttcactccagctggcttaggaatcctgacatgaccttcatatgctgttcctattcctttctgaggatctatacccaggggaccttttgtctgttcaggaggaactggacaagtggttggagctttgtttacacaagttatatggcatgagaatccacacacttcacatgaacagccctgtcttattaaacccaccatcaaggaggtacactgatgacacttggtaggagtagtaaaagattttacaaaaaactggtgagtcttgcgcttaggtggaaagccagttgaaccaggacatccttttttccttaaggttggtgtgtgaactgaaagtggagtggagtctacagtcttaactggctcagcttcactagatgtggaaggagatgtggaccgtgactggatgtgaaacttgacgctcgggttccatacatatgtgttctcaacgggatcagtacgtctgcctttgctagctggagtacaggatggagagcggtcatccaaaaaatcaatcagtgaagatgaggaagaagaaaaggaatcttcaaattgatccagagcatcggtaggcgtattcaaaaatgccaagaaagaatgctgtgagtcttggtgctctatacccttttcagatctaagctcttcagtgtcctttatcagctgttcgatttctgagagtagttccaagttcttcttctctgaatcttttagtttacattctgttatgatattagatgctttaactttattcaactcttcttggatggcctgtttggctcttatttctgcatccagagccgactgcaactccagtctagctgacatatccagtttcgcaaaacgacgcattttccagggcatatctgttgctcgtgtacccaagctggaatttcttaatgcctccaattcttcagtcattttagaagctaaggcctgaagataccctcgtgcatccttttcatcgctgacccactgaattatttctgtgatttgggcttcccaatgtgcaactgattctttcttgtctgctagatctttaacctcttcttctaactgctggttgtgtatacttaagttctcatacaaagtagtaagcttatcaagttcactcgtcagctttttattttcttcagttaacaacactttttctcgttcatattgttgtttgaactcactttcaaattcctccctttcactttgactttctcttctggttttttccaatttgtcttttaaaatcataatttctttgttgagagcaagttgctgaccttctgaatcatgcagttctttcttaagattttttatttcatttgcatgtattccttctcttttagataattcttcttcataaaagatacttttcttttccaaatcagtctttagtttggttatctcttgctgatgttctatgctgcatactcctggtgagtaactaatttgtttttgcttcagtccctccaattcattttccagttgcttagaatagtgctcactctgttcacgtagcttcctgtctttagatgcttcagcagctagagcttctgtatgaacttccagctcttttttggctctttctgttctgcgcagttcttgccttaagctttcaactttttgcatcaccaggtccacctcttcttccttatctcggacatggcgagcaagtttctgtttttgggtgtgcaattctgttagccgctcattgatctccatgaattcctgcatggccagtttcctctgacagtgtgcgtctttcagctctttggattggttttttaatcgctcactagcctggactagttccttatttagatcttctctttcttgttgtaacgttttgatttgtttttcataagccttgatttgtctaaaagcatcatctagttcttgcctcacagcattagcttcttcaagttgctgttccaaatgacttgattctgttacttgttttcttagtttttcaatttcttcttttaagttttttatttctaaatctttgcttgctgttagtggaccatcaacagttgaatactgcagagcttggacagtctgtgttgactcttgaagttttctactgagttcaagtttttcttgctcaaggcgcttaattcttctttcataagcttcagttgctaagttgttgtctagagtcctctgaacattaacatcaagatccagtgaggtgggaccagccgtaactcttaaacagctccgatcagaaagtacacagctactagtatatgtaaaaccaacaaatggcagatggtggccagaaaatgcagtatgtgttggtgggggcatcgtttcagaattttttaaacaatcatcatctacatcaaaattcgatgtatctgttgggctactaacttctggaatataaggtgcttcacagttccgaatattatcccaatcaattccactgaaaaatgggtgtttcttaaagtcttctattccattttgaccaagtcgatgttctctgctacaaatgagccttcgaataagatccttagcattttcagacacatcagtcacttgggctggaaactgaaacctctctttgtggttcatgatttttccgtatgtctccaccagcgattctgcataaaatggtgtttctccgtaaagcatttcatacatacagacccccaaagaccaccagtcacattcaggtccatatctcccttttccatcttccatggcttgaaggatttcaggagagatataatctggagttcctacagccactgaggactgaaccgttccatcttccatcagcttcagacaagaaccaaaatctgctaaccgaatatgtccattcatatccatcagtatattgtcaggtttaatgtctctgtgtacataatgtagctgatgaactgagtcaattgctatcaccatctcagccaagtaaaatctagccatatcttcaggcaatctatcttcaaatttgctgagtagagtaagcaaatccccaccaacataataatccataaccaggtataagttattgtcatcctggaaagcatagtgcaaggttgtaatccatttattgtctccattcactaatacatccctttcttcacgaaaacatgctgtctcagctcttttcagcatttcccatttattcaatattttcatggcaaacactttatctgcattttttagttttactacagcaacctccccaaaagctcctcgaccaatcacctttaatatttcaaagtcttctctatgtaatcgcatttgtttcactttagaagtaaatggtttagcccattctaggtattcgagaatgttcttctctcttctcaatggagaattattgcattcatcataaaggcagatgagtatatccagtaatgtctccacactgaagcactgcccattggtctgagcgggcccgtccaaaataaactgctccaactgcctcaaacgcacttctccagacatgtttgcttcgatttctgctggttttcctttaaattattatgatgacttttactattatctgaacctaaattttaaaaggtatggttttaaaaataaaccacttgttattcaaacaactgtcatgcaatgctggtgctgaattaaacatccaacacaccagtaacctcacttaactgaagcgtcttcaatttcacccatatacatatattttgagggtaaattaccataaaatatatacttaatgcatttttaaaagaatacaattaagtcgtatatttaaataaaataataattaaaagtacaacgaactagagagtcaacacttctttaaaaaaaaaaaaaaaaactcttctccttcattcaaaattcaactcgtgcaacgtaatcctgaaacgaatccggttgcatcattaatgaataaagtccgatttgcatcagcaattcacttcccgggaagaagaaaaacagaaaagggaggaaaaaaacagaatgcatagaagggggagggaaaaccaaaaatgttgctgcaaatcctcccaaccaccacttggataatgcatcagcggcaatttctccagcgggaaagggagggggcgaggtccctgaagcagcccctcggctcggagcacgccaagtcttgcccggaggcggcttttcgtttctcctcccgaggtccttctttctttaaggctttgcagtcagtcctattttcaacggattccggtgaaaactcttcattttcctcccggcttcaccctagggcctgaccggcggcgcggccgggggtggaaggcgggctgcgggcggcactggcaccgggctccggagaagcggctacttggccgcccgagcccactccatgtcggtggtcgctcgtgggccgagccgcgccgcgccgcgccgggcagagagcccggtctccccgacacccgcaccgggccgccgcgccggaggctcccgacgccccaggcgggggggtgcttctctgaattcaaaggacacaagcagcagcagctgcggcggcggcgcgggcggctctggcagctacttctcccccttcttcacacccctgggctaagggcatctttccacagcgaggagggaggcggcccggcgcaggaggaggggtcgcttccgcggctgaggagactagaggctgcggcagcccggctcccaaccactcccttcctctcccttccagccctcccccgccttccctctcctctcgcgctcgcgccctgggctcagcgaggctcctccagtcccgccgcacagaggcggaggcttgcggacgagtctggatccaatat

SEQ ID NO: 8649 - RNA, 6104 nt, Homo sapiens
  source 1..6104: mol_type = other RNA
aaatgtcacctttttgagaggaagagtctgaatccattccatggagttcacatcaaagatatcaactgcattttcactgtacaccgagagatatggtgcattgtaacaacaagaggaaggatttgctggccacatcaattcctgttgtctagatcttcggccctggcagtcagtgtatatcccaatgctgttaaaacacagcagatattctttactggagatctcaactgcgcagatagcatccattggttgatgtgcaataaatgatagtgtatggtcatttgaatggagcatactgtatggatttccttctccattcaaggggtatcttagaaatcctgactggaatcccacacagagttgttcactgaagattgccatccactggacattatatgggacttgaatttctttaaattttctgtgacgggtcttgctctgaaatagttcataacagaggacctgccttttcatagccacacacaggcatgtgagagctccatggcgcacctttccagaagttacggtttgacaccctttagtttctgacagcttgtaaaaatcggtctctcgcccatccaatgctgacataggaaaaagtcgtacatgacgatttcgtcctgagatcacagcaacaagctgatcatttggaatgagttcaatctgatgaatcttcttattgtcaccaactctaataatttcatctttggtgacatgtacaacaaataacccttcttcgtttcccaaagcaattctttcatgatctatgattgcggctgcctgggttgttttaatgaggggtagagtgctgtcataagcctctttgggaacatagactgagcggtctctgaatttgtttttcttcaaaatcttgtgcaattcactcagcactcccacccacttattcttctcattctcagtgtctgctagcatcaggattgaacatttgttattagatgctgagagctgggaagctgtgaccctaaatatacagggtatatctttccgacttgcatggataacatcagaagccaagactgaactcacagaaaattcttcatccctcatgtcaatcacttgactaatgacaacactgggctgagatgcttttccttcagcaatatcgtacagaaagagtttgaagtcacacactatagccagtgctctctgccaccctttcttcactccagctggcttaggaatcctgacatgaccttcatatgctgttcctattcctttctgaggatctatacccaggggaccttttgtctgttcaggaggaactggacaagtggttggagctttgtttacacaagttatatggcatgagaatccacacacttcacatgaacagccctgtcttattaaacccaccatcaaggaggtacactgatgacacttggtaggagtagtaaaagattttacaaaaaactggtgagtcttgcgcttaggtggaaagccagttgaaccaggacatccttttttccttaaggttggtgtgtgaactgaaagtggagtggagtctacagtcttaactggctcagcttcactagatgtggaaggagatgtggaccgtgactggatgtgaaacttgacgctcgggttccatacatatgtgttctcaacgggatcagtacgtctgcctttgctagctggagtacaggatggagagcggtcatccaaaaaatcaatcagtgaagatgaggaagaagaaaaggaatcttcaaattgatccagagcatcggtaggcgtattcaaaaatgccaagaaagaatgctgtgagtcttggtgctctatacccttttcagatctaagctcttcagtgtcctttatcagctgttcgatttctgagagtagttccaagttcttcttctctgaatcttttagtttacattctgttatgatattagatgctttaactttattcaactcttcttggatggcctgtttggctcttatttctgcatccagagccgactgcaactccagtctagctgacatatccagtttcgcaaaacgacgcattttccagggcatatctgttgctcgtgtacccaagctggaatttcttaatgcctccaattcttcagtcattttagaagctaaggcctgaagataccctcgtgcatccttttcatcgctgacccactgaattatttctgtgatttgggcttcccaatgtgcaactgattctttcttgtctgctagatctttaacctcttcttctaactgctggttgtgtatacttaagttctcatacaaagtagtaagcttatcaagttcactcgtcagctttttattttcttcagttaacaacactttttctcgttcatattgttgtttgaactcactttcaaattcctccctttcactttgactttctcttctggttttttccaatttgtcttttaaaatcataatttctttgttgagagcaagttgctgaccttctgaatcatgcagttctttcttaagattttttatttcatttgcatgtattccttctcttttagataattcttcttcataaaagatacttttcttttccaaatcagtctttagtttggttatctcttgctgatgttctatgctgcatactcctggtgagtaactaatttgtttttgcttcagtccctccaattcattttccagttgcttagaatagtgctcactctgttcacgtagcttcctgtctttagatgcttcagcagctagagcttctgtatgaacttccagctcttttttggctctttctgttctgcgcagttcttgccttaagctttcaactttttgcatcaccaggtccacctcttcttccttatctcggacatggcgagcaagtttctgtttttgggtgtgcaattctgttagccgctcattgatctccatgaattcctgcatggccagtttcctctgacagtgtgcgtctttcagctctttggattggttttttaatcgctcactagcctggactagttccttatttagatcttctctttcttgttgtaacgttttgatttgtttttcataagccttgatttgtctaaaagcatcatctagttcttgcctcacagcattagcttcttcaagttgctgttccaaatgacttgattctgttacttgttttcttagtttttcaatttcttcttttaagttttttatttctaaatctttgcttgctgttagtggaccatcaacagttgaatactgcagagcttggacagtctgtgttgactcttgaagttttctactgagttcaagtttttcttgctcaaggcgcttaattcttctttcataagcttcagttgctaagttgttgtctagagtcctctgaacattaacatcaagatccagtgaggtgggaccagccgtaactcttaaacagctccgatcagaaagtacacagctactagtatatgtaaaaccaacaaatggcagatggtggccagaaaatgcagtatgtgttggtgggggcatcgtttcagaattttttaaacaatcatcatctacatcaaaattcgatgtatctgttgggctactaacttctggaatataaggtgcttcacagttccgaatattatcccaatcaattccactgaaaaatgggtgtttcttaaagtcttctattccattttgaccaagtcgatgttctctgctacaaatgagccttcgaataagatccttagcattttcagacacatcagtcacttgggctggaaactgaaacctctctttgtggttcatgatttttccgtatgtctccaccagcgattctgcataaaatggtgtttctccgtaaagcatttcatacatacagacccccaaagaccaccagtcacattcaggtccatatctcccttttccatcttccatggcttgaaggatttcaggagagatataatctggagttcctacagccactgaggactgaaccgttccatcttccatcagcttcagacaagaaccaaaatctgctaaccgaatatgtccattcatatccatcagtatattgtcaggtttaatgtctctgtgtacataatgtagctgatgaactgagtcaattgctatcaccatctcagccaagtaaaatctagccatatcttcaggcaatctatcttcaaatttgctgagtagagtaagcaaatccccaccaacataataatccataaccaggtataagttattgtcatcctggaaagcatagtgcaaggttgtaatccatttattgtctccattcactaatacatccctttcttcacgaaaacatgctgtctcagctcttttcagcatttcccatttattcaatattttcatggcaaacactttatctgcattttttagttttactacagcaacctgaagcaggggtagcaggccaaagcagcaagctttcacaacaagctctgaagcccagaagccttgaagctgccggagcaaggctggagcaggcagaagcggtgagccaccaggaaactgttgacaggcaacacccagggcgtaagttaaaggttttcctccccaaaagctcctcgaccaatcacctttaatatttcaaagtcttctctatgtaatcgcatttgtttcactttagaagtaaatggtttagcccattctaggtattcgagaatgttcttctctcttctcaatggagaattattgcattcatcataaaggcagatgagtatatccagtaatgtctccacactgaagcactgcccattggtctgagcgggcccgtccaaaataaactgctccaactgcctcaaacgcacttctccagacatgtttgcttcgatttctgctggttttcctttaaattattatgatgacttttactattatctgaacctaaattttaaaaggtatggttttaaaaataaaccacttgttattcaaacaactgtcatgcaatgctggtgctgaattaaacatccaacacaccagtaacctcacttaactgaagcgtcttcaatttcacccatatacatatattttgagggtaaattaccataaaatatatacttaatgcatttttaaaagaatacaattaagtcgtatatttaaataaaataataattaaaagtacaacgaactagagagtcaacacttctttaaaaaaaaaaaaaaaaactcttctccttcattcaaaattcaactcgtgcaacgtaatcctgaaacgaatccggttgcatcattaatgaataaagtccgatttgcatcagcaattcacttcccgggaagaagaaaaacagaaaagggaggaaaaaaacagaatgcatagaagggggagggaaaaccaaaaatgttgctgcaaatcctcccaaccaccacttggataatgcatcagcggcaatttctccagcgggaaagggagggggcgaggtccctgaagcagcccctcggctcggagcacgccaagtcttgcccggaggcggcttttcgtttctcctcccgaggtccttctttctttaaggctttgcagtcagtcctattttcaacggattccggtgaaaactcttcattttcctcccggcttcaccctagggcctgaccggcggcgcggccgggggtggaaggcgggctgcgggcggcactggcaccgggctccggagaagcggctacttggccgcccgagcccactccatgtcggtggtcgctcgtgggccgagccgcgccgcgccgcgccgggcagagagcccggtctccccgacacccgcaccgggccgccgcgccggaggctcccgacgccccaggcgggggggtgcttctctgaattcaaaggacacaagcagcagcagctgcggcggcggcgcgggcggctctggcagctacttctcccccttcttcacacccctgggctaagggcatctttccacagcgaggagggaggcggcccggcgcaggaggaggggtcgcttccgcggctgaggagactagaggctgcggcagcccggctcccaaccactcccttcctctcccttccagccctcccccgccttccctctcctctcgcgctcgcgccctgggctcagcgaggctcctccagtcccgccgcacagaggcggaggcttgcggacgagtctggatccaatatggcggcctgg

SEQ ID NO: 8650 - RNA, 5438 nt, Homo sapiens
  source 1..5438: mol_type = other RNA
aaatgtcacctttttgagaggaagagtctgaatccattccatggagttcacatcaaagatatcaactgcattttcactgtacaccgagagatatggtgcattgtaacaacaagaggaaggatttgctggccacatcaattcctgttgtctagatcttcggccctggcagtcagtgtatatcccaatgctgttaaaacacagcagatattctttactggagatctcaactgcgcagatagcatccattggttgatgtgcaataaatgatagtgtatggtcatttgaatggagcatactgtatggatttccttctccattcaaggggtatcttagaaatcctgactggaatcccacacagagttgttcactgaagattgccatccactggacattatatgggacttgaatttctttaaattttctgtgacgggtcttgctctgaaatagttcataacagaggacctgccttttcatagccacacacaggcatgtgagagctccatggcgcacctttccagaagttacggtttgacaccctttagtttctgacagcttgtaaaaatcggtctctcgcccatccaatgctgacataggaaaaagtcgtacatgacgatttcgtcctgagatcacagcaacaagctgatcatttggaatgagttcaatctgatgaatcttcttattgtcaccaactctaataatttcatctttggtgacatgtacaacaaataacccttcttcgtttcccaaagcaattctttcatgatctatgattgcggctgcctgggttgttttaatgaggggtagagtgctgtcataagcctctttgggaacatagactgagcggtctctgaatttgtttttcttcaaaatcttgtgcaattcactcagcactcccacccacttattcttctcattctcagtgtctgctagcatcaggattgaacatttgttattagatgctgagagctgggaagctgtgaccctaaatatacagggtatatctttccgacttgcatggataacatcagaagccaagactgaactcacagaaaattcttcatccctcatgtcaatcacttgactaatgacaacactgggctgagatgcttttccttcagcaatatcgtacagaaagagtttgaagtcacacactatagccagtgctctctgccaccctttcttcactccagctggcttaggaatcctgacatgaccttcatatgctgttcctattcctttctgaggatctatacccaggggaccttttgtctgttcaggaggaactggacaagtggttggagctttgtttacacaagttatatggcatgagaatccacacacttcacatgaacagccctgtcttattaaacccaccatcaaggaggtacactgatgacacttggtaggagtagtaaaagattttacaaaaaactggtgagtcttgcgcttaggtggaaagccagttgaaccaggacatccttttttccttaaggttggtgtgtgaactgaaagtggagtggagtctacagtcttaactggctcagcttcactagatgtggaaggagatgtggaccgtgactggatgtgaaacttgacgctcgggttccatacatatgtgttctcaacgggatcagtacgtctgcctttgctagctggagtacaggatggagagcggtcatccaaaaaatcaatcagtgaagatgaggaagaagaaaaggaatcttcaaattgatccagagcatcggtaggcgtattcaaaaatgccaagaaagaatgctgtgagtcttggtgctctatacccttttcagatctaagctcttcagtgtcctttatcagctgttcgatttctgagagtagttccaagttcttcttctctgaatcttttagtttacattctgttatgatattagatgctttaactttattcaactcttcttggatggcctgtttggctcttatttctgcatccagagccgactgcaactccagtctagctgacatatccagtttcgcaaaacgacgcattttccagggcatatctgttgctcgtgtacccaagctggaatttcttaatgcctccaattcttcagtcattttagaagctaaggcctgaagataccctcgtgcatccttttcatcgctgacccactgaattatttctgtgatttgggcttcccaatgtgcaactgattctttcttgtctgctagatctttaacctcttcttctaactgctggttgtgtatacttaagttctcatacaaagtagtaagcttatcaagttcactcgtcagctttttattttcttcagttaacaacactttttctcgttcatattgttgtttgaactcactttcaaattcctccctttcactttgactttctcttctggttttttccaatttgtcttttaaaatcataatttctttgttgagagcaagttgctgaccttctgaatcatgcagttctttcttaagattttttatttcatttgcatgtattccttctcttttagataattcttcttcataaaagatacttttcttttccaaatcagtctttagtttggttatctcttgctgatgttctatgctgcatactcctggtgagtaactaatttgtttttgcttcagtccctccaattcattttccagttgcttagaatagtgctcactctgttcacgtagcttcctgtctttagatgcttcagcagctagagcttctgtatgaacttccagcttatttagatcttctctttcttgttgtaacgttttgatttgtttttcataagccttgatttgtctaaaagcatcatctagttcttgcctcacagcattagcttcttcaagttgctgttccaaatgacttgattctgttacttgttttcttagtttttcaatttcttcttttaagttttttatttctaaatctttgcttgctgttagtggaccatcaacagttgaatactgcagagcttggacagtctgtgttgactcttgaagttttctactgagttcaagtttttcttgctcaaggcgcttaattcttctttcataagcttcagttgctaagttgttgtctagagtcctctgaacattaacatcaagatccagtgaggtgggaccagccgtaactcttaaacagctccgatcagaaagtacacagctactagtatatgtaaaaccaacaaatggcagatggtggccagaaaatgcagtatgtgttggtgggggcatcgtttcagaattttttaaacaatcatcatctacatcaaaattcgatgtatctgttgggctactaacttctggaatataaggtgcttcacagttccgaatattatcccaatcaattccactgaaaaatgggtgtttcttaaagtcttctattccattttgaccaagtcgatgttctctgctacaaatgagccttcgaataagatccttagcattttcagacacatcagtcacttgggctggaaactgaaacctctctttgtggttcatgatttttccgtatgtctccaccagcgattctgcataaaatggtgtttctccgtaaagcatttcatacatacagacccccaaagaccaccagtcacattcaggtccatatctcccttttccatcttccatggcttgaaggatttcaggagagatataatctggagttcctacagccactgaggactgaaccgttccatcttccatcagcttcagacaagaaccaaaatctgctaaccgaatatgtccattcatatccatcagtatattgtcaggtttaatgtctctgtgtacataatgtagctgatgaactgagtcaattgctatcaccatctcagccaagtaaaatctagccatatcttcaggcaatctatcttcaaatttgctgagtagagtaagcaaatccccaccaacataataatccataaccaggtataagttattgtcatcctggaaagcatagtgcaaggttgtaatccatttattgtctccattcactaatacatccctttcttcacgaaaacatgctgtctcagctcttttcagcatttcccatttattcaatattttcatggcaaacactttatctgcattttttagttttactacagcaacctccccaaaagctcctcgaccaatcacctttaatatttcaaagtcttctctatgtaatcgcatttgtttcactttagaagtaaatggtttagcccattctaggtattcgagaatgttcttctctcttctcaatggagaattattgcattcatcataaaggcagatgagtatatccagtaatgtctccacactgaagcactgcccattggtctgagcgggcccgtccaaaataaactgctccaactgcctcaaacgcacttctccagacatgtttgcttcgatttctgctggttttcctttaaattattatgatgacttttactattatctgaacctaaattttaaaaggtatggttttaaaaataaaccacttgttattcaaacaactgtcatgcaatgctggtgctgaattaaacatccaacacaccagtaacctcacttaactgaagcgtcttcaatttcacccatatacatatattttgagggtaaattaccataaaatatatacttaatgcatttttaaaagaatacaattaagtcgtatatttaaataaaataataattaaaagtacaacgaactagagagtcaacacttctttaaaaaaaaaaaaaaaaactcttctccttcattcaaaattcaactcgtgcaacgtaatcctgaaacgaatccggttgcatcattaatgaataaagtccgatttgcatcagcaattcacttcccgggaagaagaaaaacagaaaagggaggaaaaaaacagaatgcatagaagggggagggaaaaccaaaaatgttgctgcaaatcctcccaaccaccacttggataatgcatcagcggcaatttctccagcgggaaagggagggggcgaggtccctgaagcagcccctcggctcggagcacgccaagtcttgcccggaggcggcttttcgtttctcctcccgaggtccttctttctttaaggctttgcagtcagtcctattttcaacggattccggtgaaaactcttcattttcctcccggcttcaccctagggcctgaccggcggcgcggccgggggtggaaggcgggctgcgggcggcactggcaccgggctccggagaagcggctacttggccgcccgagcccactccatgtcggtggtcgctcgtgggccgagccgcgccgcgccgcgccgggcagagagcccggtctccccgacacccgcaccgggccgccgcgccggaggctcccgacgccccaggcgggggggtgcttctctgaattcaaaggacacaagcagcagcagctgcggcggcggcgcgggcggctctggcagctacttctccc

SEQ ID NO: 8651 - RNA, 5546 nt, Homo sapiens
  source 1..5546: mol_type = other RNA
aaatgtcacctttttgagaggaagagtctgaatccattccatggagttcacatcaaagatatcaactgcattttcactgtacaccgagagatatggtgcattgtaacaacaagaggaaggatttgctggccacatcaattcctgttgtctagatcttcggccctggcagtcagtgtatatcccaatgctgttaaaacacagcagatattctttactggagatctcaactgcgcagatagcatccattggttgatgtgcaataaatgatagtgtatggtcatttgaatggagcatactgtatggatttccttctccattcaaggggtatcttagaaatcctgactggaatcccacacagagttgttcactgaagattgccatccactggacattatatgggacttgaatttctttaaattttctgtgacgggtcttgctctgaaatagttcataacagaggacctgccttttcatagccacacacaggcatgtgagagctccatggcgcacctttccagaagttacggtttgacaccctttagtttctgacagcttgtaaaaatcggtctctcgcccatccaatgctgacataggaaaaagtcgtacatgacgatttcgtcctgagatcacagcaacaagctgatcatttggaatgagttcaatctgatgaatcttcttattgtcaccaactctaataatttcatctttggtgacatgtacaacaaataacccttcttcgtttcccaaagcaattctttcatgatctatgattgcggctgcctgggttgttttaatgaggggtagagtgctgtcataagcctctttgggaacatagactgagcggtctctgaatttgtttttcttcaaaatcttgtgcaattcactcagcactcccacccacttattcttctcattctcagtgtctgctagcatcaggattgaacatttgttattagatgctgagagctgggaagctgtgaccctaaatatacagggtatatctttccgacttgcatggataacatcagaagccaagactgaactcacagaaaattcttcatccctcatgtcaatcacttgactaatgacaacactgggctgagatgcttttccttcagcaatatcgtacagaaagagtttgaagtcacacactatagccagtgctctctgccaccctttcttcactccagctggcttaggaatcctgacatgaccttcatatgctgttcctattcctttctgaggatctatacccaggggaccttttgtctgttcaggaggaactggacaagtggttggagctttgtttacacaagttatatggcatgagaatccacacacttcacatgaacagccctgtcttattaaacccaccatcaaggaggtacactgatgacacttggtaggagtagtaaaagattttacaaaaaactggtgagtcttgcgcttaggtggaaagccagttgaaccaggacatccttttttccttaaggttggtgtgtgaactgaaagtggagtggagtctacagtcttaactggctcagcttcactagatgtggaaggagatgtggaccgtgactggatgtgaaacttgacgctcgggttccatacatatgtgttctcaacgggatcagtacgtctgcctttgctagctggagtacaggatggagagcgttcaaattgatccagagcatcggtaggcgtattcaaaaatgccaagaaagaatgctgtgagtcttggtgctctatacccttttcagatctaagctcttcagtgtcctttatcagctgttcgatttctgagagtagttccaagttcttcttctctgaatcttttagtttacattctgttatgatattagatgctttaactttattcaactcttcttggatggcctgtttggctcttatttctgcatccagagccgactgcaactccagtctagctgacatatccagtttcgcaaaacgacgcattttccagggcatatctgttgctcgtgtacccaagctggaatttcttaatgcctccaattcttcagtcattttagaagctaaggcctgaagataccctcgtgcatccttttcatcgctgacccactgaattatttctgtgatttgggcttcccaatgtgcaactgattctttcttgtctgctagatctttaacctcttcttctaactgctggttgtgtatacttaagttctcatacaaagtagtaagcttatcaagttcactcgtcagctttttattttcttcagttaacaacactttttctcgttcatattgttgtttgaactcactttcaaattcctccctttcactttgactttctcttctggttttttccaatttgtcttttaaaatcataatttctttgttgagagcaagttgctgaccttctgaatcatgcagttctttcttaagattttttatttcatttgcatgtattccttctcttttagataattcttcttcataaaagatacttttcttttccaaatcagtctttagtttggttatctcttgctgatgttctatgctgcatactcctggtgagtaactaatttgtttttgcttcagtccctccaattcattttccagttgcttagaatagtgctcactctgttcacgtagcttcctgtctttagatgcttcagcagctagagcttctgtatgaacttccagctcttttttggctctttctgttctgcgcagttcttgccttaagctttcaactttttgcatcaccaggtccacctcttcttccttatctcggacatggcgagcaagtttctgtttttgggtgtgcaattctgttagccgctcattgatctccatgaattcctgcatggccagtttcctctgacagtgtgcgtctttcagctctttggattggttttttaatcgctcactagcctggactagttccttatttagatcttctctttcttgttgtaacgttttgatttgtttttcataagccttgatttgtctaaaagcatcatctagttcttgcctcacagcattagcttcttcaagttgctgttccaaatgacttgattctgttacttgttttcttagtttttcaatttcttcttttaagttttttatttctaaatctttgcttgctgttagtggaccatcaacagttgaatactgcagagcttggacagtctgtgttgactcttgaagttttctactgagttcaagtttttcttgctcaaggcgcttaattcttctttcataagcttcagttgctaagttgttgtctagagtcctctgaacattaacatcaagatccagtgaggtgggaccagccgtaactcttaaacagctccgatcagaaagtacacagctactagtatatgtaaaaccaacaaatggcagatggtggccagaaaatgcagtatgtgttggtgggggcatcgtttcagaattttttaaacaatcatcatctacatcaaaattcgatgtatctgttgggctactaacttctggaatataaggtgcttcacagttccgaatattatcccaatcaattccactgaaaaatgggtgtttcttaaagtcttctattccattttgaccaagtcgatgttctctgctacaaatgagccttcgaataagatccttagcattttcagacacatcagtcacttgggctggaaactgaaacctctctttgtggttcatgatttttccgtatgtctccaccagcgattctgcataaaatggtgtttctccgtaaagcatttcatacatacagacccccaaagaccaccagtcacattcaggtccatatctcccttttccatcttccatggcttgaaggatttcaggagagatataatctggagttcctacagccactgaggactgaaccgttccatcttccatcagcttcagacaagaaccaaaatctgctaaccgaatatgtccattcatatccatcagtatattgtcaggtttaatgtctctgtgtacataatgtagctgatgaactgagtcaattgctatcaccatctcagccaagtaaaatctagccatatcttcaggcaatctatcttcaaatttgctgagtagagtaagcaaatccccaccaacataataatccataaccaggtataagttattgtcatcctggaaagcatagtgcaaggttgtaatccatttattgtctccattcactaatacatccctttcttcacgaaaacatgctgtctcagctcttttcagcatttcccatttattcaatattttcatggcaaacactttatctgcattttttagttttactacagcaacctccccaaaagctcctcgaccaatcacctttaatatttcaaagtcttctctatgtaatcgcatttgtttcactttagaagtaaatggtttagcccattctaggtattcgagaatgttcttctctcttctcaatggagaattattgcattcatcataaaggcagatgagtatatccagtaatgtctccacactgaagcactgcccattggtctgagcgggcccgtccaaaataaactgctccaactgcctcaaacgcacttctccagacatgtttgcttcgatttctgctggttttcctttaaattattatgatgacttttactattatctgaacctaaattttaaaaggtatggttttaaaaataaaccacttgttattcaaacaactgtcatgcaatgctggtgctgaattaaacatccaacacaccagtaacctcacttaactgaagcgtcttcaatttcacccatatacatatattttgagggtaaattaccataaaatatatacttaatgcatttttaaaagaatacaattaagtcgtatatttaaataaaataataattaaaagtacaacgaactagagagtcaacacttctttaaaaaaaaaaaaaaaaactcttctccttcattcaaaattcaactcgtgcaacgtaatcctgaaacgaatccggttgcatcattaatgaataaagtccgatttgcatcagcaattcacttcccgggaagaagaaaaacagaaaagggaggaaaaaaacagaatgcatagaagggggagggaaaaccaaaaatgttgctgcaaatcctcccaaccaccacttggataatgcatcagcggcaatttctccagcgggaaagggagggggcgaggtccctgaagcagcccctcggctcggagcacgccaagtcttgcccggaggcggcttttcgtttctcctcccgaggtccttctttctttaaggctttgcagtcagtcctattttcaacggattccggtgaaaactcttcattttcctcccggcttcaccctagggcctgaccggcggcgcggccgggggtggaaggcgggctgcgggcggcactggcaccgggctccggagaagcggctacttggccgcccgagcccactccatgtcggtggtcgctcgtgggccgagccgcgccgcgccgcgccgggcagagagcccggtctccccgacacccgcaccgggccgccgcgccggaggctcccgacgcccca

SEQ ID NO: 8652 - RNA, 5555 nt, Homo sapiens
  source 1..5555: mol_type = other RNA
aaatgtcacctttttgagaggaagagtctgaatccattccatggagttcacatcaaagatatcaactgcattttcactgtacaccgagagatatggtgcattgtaacaacaagaggaaggatttgctggccacatcaattcctgttgtctagatcttcggccctggcagtcagtgtatatcccaatgctgttaaaacacagcagatattctttactggagatctcaactgcgcagatagcatccattggttgatgtgcaataaatgatagtgtatggtcatttgaatggagcatactgtatggatttccttctccattcaaggggtatcttagaaatcctgactggaatcccacacagagttgttcactgaagattgccatccactggacattatatgggacttgaatttctttaaattttctgtgacgggtcttgctctgaaatagttcataacagaggacctgccttttcatagccacacacaggcatgtgagagctccatggcgcacctttccagaagttacggtttgacaccctttagtttctgacagcttgtaaaaatcggtctctcgcccatccaatgctgacataggaaaaagtcgtacatgacgatttcgtcctgagatcacagcaacaagctgatcatttggaatgagttcaatctgatgaatcttcttattgtcaccaactctaataatttcatctttggtgacatgtacaacaaataacccttcttcgtttcccaaagcaattctttcatgatctatgattgcggctgcctgggttgttttaatgaggggtagagtgctgtcataagcctctttgggaacatagactgagcggtctctgaatttgtttttcttcaaaatcttgtgcaattcactcagcactcccacccacttattcttctcattctcagtgtctgctagcatcaggattgaacatttgttattagatgctgagagctgggaagctgtgaccctaaatatacagggtatatctttccgacttgcatggataacatcagaagccaagactgaactcacagaaaattcttcatccctcatgtcaatcacttgactaatgacaacactgggctgagatgcttttccttcagcaatatcgtacagaaagagtttgaagtcacacactatagccagtgctctctgccaccctttcttcactccagctggcttaggaatcctgacatgaccttcatatgctgttcctattcctttctgaggatctatacccaggggaccttttgtctgttcaggaggaactggacaagtggttggagctttgtttacacaagttatatggcatgagaatccacacacttcacatgaacagccctgtcttattaaacccaccatcaaggaggtacactgatgacacttggtaggagtagtaaaagattttacaaaaaactggtgagtcttgcgcttaggtggaaagccagttgaaccaggacatccttttttccttaaggttggtgtgtgaactgaaagtggagtggagtctacagtcttaactggctcagcttcactagatgtggaaggagatgtggaccgtgactggatgtgaaacttgacgctcgggttccatacatatgtgttctcaacgggatcagtgtcatccaaaaaatcaatcagtgaagatgaggaagaagaaaaggaatcttcaaattgatccagagcatcggtaggcgtattcaaaaatgccaagaaagaatgctgtgagtcttggtgctctatacccttttcagatctaagctcttcagtgtcctttatcagctgttcgatttctgagagtagttccaagttcttcttctctgaatcttttagtttacattctgttatgatattagatgctttaactttattcaactcttcttggatggcctgtttggctcttatttctgcatccagagccgactgcaactccagtctagctgacatatccagtttcgcaaaacgacgcattttccagggcatatctgttgctcgtgtacccaagctggaatttcttaatgcctccaattcttcagtcattttagaagctaaggcctgaagataccctcgtgcatccttttcatcgctgacccactgaattatttctgtgatttgggcttcccaatgtgcaactgattctttcttgtctgctagatctttaacctcttcttctaactgctggttgtgtatacttaagttctcatacaaagtagtaagcttatcaagttcactcgtcagctttttattttcttcagttaacaacactttttctcgttcatattgttgtttgaactcactttcaaattcctccctttcactttgactttctcttctggttttttccaatttgtcttttaaaatcataatttctttgttgagagcaagttgctgaccttctgaatcatgcagttctttcttaagattttttatttcatttgcatgtattccttctcttttagataattcttcttcataaaagatacttttcttttccaaatcagtctttagtttggttatctcttgctgatgttctatgctgcatactcctggtgagtaactaatttgtttttgcttcagtccctccaattcattttccagttgcttagaatagtgctcactctgttcacgtagcttcctgtctttagatgcttcagcagctagagcttctgtatgaacttccagctcttttttggctctttctgttctgcgcagttcttgccttaagctttcaactttttgcatcaccaggtccacctcttcttccttatctcggacatggcgagcaagtttctgtttttgggtgtgcaattctgttagccgctcattgatctccatgaattcctgcatggccagtttcctctgacagtgtgcgtctttcagctctttggattggttttttaatcgctcactagcctggactagttccttatttagatcttctctttcttgttgtaacgttttgatttgtttttcataagccttgatttgtctaaaagcatcatctagttcttgcctcacagcattagcttcttcaagttgctgttccaaatgacttgattctgttacttgttttcttagtttttcaatttcttcttttaagttttttatttctaaatctttgcttgctgttagtggaccatcaacagttgaatactgcagagcttggacagtctgtgttgactcttgaagttttctactgagttcaagtttttcttgctcaaggcgcttaattcttctttcataagcttcagttgctaagttgttgtctagagtcctctgaacattaacatcaagatccagtgaggtgggaccagccgtaactcttaaacagctccgatcagaaagtacacagctactagtatatgtaaaaccaacaaatggcagatggtggccagaaaatgcagtatgtgttggtgggggcatcgtttcagaattttttaaacaatcatcatctacatcaaaattcgatgtatctgttgggctactaacttctggaatataaggtgcttcacagttccgaatattatcccaatcaattccactgaaaaatgggtgtttcttaaagtcttctattccattttgaccaagtcgatgttctctgctacaaatgagccttcgaataagatccttagcattttcagacacatcagtcacttgggctggaaactgaaacctctctttgtggttcatgatttttccgtatgtctccaccagcgattctgcataaaatggtgtttctccgtaaagcatttcatacatacagacccccaaagaccaccagtcacattcaggtccatatctcccttttccatcttccatggcttgaaggatttcaggagagatataatctggagttcctacagccactgaggactgaaccgttccatcttccatcagcttcagacaagaaccaaaatctgctaaccgaatatgtccattcatatccatcagtatattgtcaggtttaatgtctctgtgtacataatgtagctgatgaactgagtcaattgctatcaccatctcagccaagtaaaatctagccatatcttcaggcaatctatcttcaaatttgctgagtagagtaagcaaatccccaccaacataataatccataaccaggtataagttattgtcatcctggaaagcatagtgcaaggttgtaatccatttattgtctccattcactaatacatccctttcttcacgaaaacatgctgtctcagctcttttcagcatttcccatttattcaatattttcatggcaaacactttatctgcattttttagttttactacagcaacctccccaaaagctcctcgaccaatcacctttaatatttcaaagtcttctctatgtaatcgcatttgtttcactttagaagtaaatggtttagcccattctaggtattcgagaatgttcttctctcttctcaatggagaattattgcattcatcataaaggcagatgagtatatccagtaatgtctccacactgaagcactgcccattggtctgagcgggcccgtccaaaataaactgctccaactgcctcaaacgcacttctccagacatgtttgcttcgatttctgctggttttcctttaaattattatgatgacttttactattatctgaacctaaattttaaaaggtatggttttaaaaataaaccacttgttattcaaacaactgtcatgcaatgctggtgctgaattaaacatccaacacaccagtaacctcacttaactgaagcgtcttcaatttcacccatatacatatattttgagggtaaattaccataaaatatatacttaatgcatttttaaaagaatacaattaagtcgtatatttaaataaaataataattaaaagtacaacgaactagagagtcaacacttctttaaaaaaaaaaaaaaaaactcttctccttcattcaaaattcaactcgtgcaacgtaatcctgaaacgaatccggttgcatcattaatgaataaagtccgatttgcatcagcaattcacttcccgggaagaagaaaaacagaaaagggaggaaaaaaacagaatgcatagaagggggagggaaaaccaaaaatgttgctgcaaatcctcccaaccaccacttggataatgcatcagcggcaatttctccagcgggaaagggagggggcgaggtccctgaagcagcccctcggctcggagcacgccaagtcttgcccggaggcggcttttcgtttctcctcccgaggtccttctttctttaaggctttgcagtcagtcctattttcaacggattccggtgaaaactcttcattttcctcccggcttcaccctagggcctgaccggcggcgcggccgggggtggaaggcgggctgcgggcggcactggcaccgggctccggagaagcggctacttggccgcccgagcccactccatgtcggtggtcgctcgtgggccgagccgcgccgcgccgcgccgggcagagagcccggtctccccgacacccgcaccgggccgccgcgccggaggctcccgacgcccca

SEQ ID NO: 8653 - RNA, 5507 nt, Homo sapiens
  source 1..5507: mol_type = other RNA
aaatgtcacctttttgagaggaagagtctgaatccattccatggagttcacatcaaagatatcaactgcattttcactgtacaccgagagatatggtgcattgtaacaacaagaggaaggatttgctggccacatcaattcctgttgtctagatcttcggccctggcagtcagtgtatatcccaatgctgttaaaacacagcagatattctttactggagatctcaactgcgcagatagcatccattggttgatgtgcaataaatgatagtgtatggtcatttgaatggagcatactgtatggatttccttctccattcaaggggtatcttagaaatcctgactggaatcccacacagagttgttcactgaagattgccatccactggacattatatgggacttgaatttctttaaattttctgtgacgggtcttgctctgaaatagttcataacagaggacctgccttttcatagccacacacaggcatgtgagagctccatggcgcacctttccagaagttacggtttgacaccctttagtttctgacagcttgtaaaaatcggtctctcgcccatccaatgctgacataggaaaaagtcgtacatgacgatttcgtcctgagatcacagcaacaagctgatcatttggaatgagttcaatctgatgaatcttcttattgtcaccaactctaataatttcatctttggtgacatgtacaacaaataacccttcttcgtttcccaaagcaattctttcatgatctatgattgcggctgcctgggttgttttaatgaggggtagagtgctgtcataagcctctttgggaacatagactgagcggtctctgaatttgtttttcttcaaaatcttgtgcaattcactcagcactcccacccacttattcttctcattctcagtgtctgctagcatcaggattgaacatttgttattagatgctgagagctgggaagctgtgaccctaaatatacagggtatatctttccgacttgcatggataacatcagaagccaagactgaactcacagaaaattcttcatccctcatgtcaatcacttgactaatgacaacactgggctgagatgcttttccttcagcaatatcgtacagaaagagtttgaagtcacacactatagccagtgctctctgccaccctttcttcactccagctggcttaggaatcctgacatgaccttcatatgctgttcctattcctttctgaggatctatacccaggggaccttttgtctgttcaggaggaactggacaagtggttggagctttgtttacacaagttatatggcatgagaatccacacacttcacatgaacagccctgtcttattaaacccaccatcaaggaggtacactgatgacacttggtaggagtagtaaaagattttacaaaaaactggtgagtcttgcgcttaggtggaaagccagttgaaccaggacatccttttttccttaaggttggtgtgtgaactgaaagtggagtggagtctacagtcttaactggctcagcttcactagatgtggaaggagatgtggaccgtgactggatgtgaaacttgacgctcgggttccatacatatgtgttctcaacgggatcagtttcaaattgatccagagcatcggtaggcgtattcaaaaatgccaagaaagaatgctgtgagtcttggtgctctatacccttttcagatctaagctcttcagtgtcctttatcagctgttcgatttctgagagtagttccaagttcttcttctctgaatcttttagtttacattctgttatgatattagatgctttaactttattcaactcttcttggatggcctgtttggctcttatttctgcatccagagccgactgcaactccagtctagctgacatatccagtttcgcaaaacgacgcattttccagggcatatctgttgctcgtgtacccaagctggaatttcttaatgcctccaattcttcagtcattttagaagctaaggcctgaagataccctcgtgcatccttttcatcgctgacccactgaattatttctgtgatttgggcttcccaatgtgcaactgattctttcttgtctgctagatctttaacctcttcttctaactgctggttgtgtatacttaagttctcatacaaagtagtaagcttatcaagttcactcgtcagctttttattttcttcagttaacaacactttttctcgttcatattgttgtttgaactcactttcaaattcctccctttcactttgactttctcttctggttttttccaatttgtcttttaaaatcataatttctttgttgagagcaagttgctgaccttctgaatcatgcagttctttcttaagattttttatttcatttgcatgtattccttctcttttagataattcttcttcataaaagatacttttcttttccaaatcagtctttagtttggttatctcttgctgatgttctatgctgcatactcctggtgagtaactaatttgtttttgcttcagtccctccaattcattttccagttgcttagaatagtgctcactctgttcacgtagcttcctgtctttagatgcttcagcagctagagcttctgtatgaacttccagctcttttttggctctttctgttctgcgcagttcttgccttaagctttcaactttttgcatcaccaggtccacctcttcttccttatctcggacatggcgagcaagtttctgtttttgggtgtgcaattctgttagccgctcattgatctccatgaattcctgcatggccagtttcctctgacagtgtgcgtctttcagctctttggattggttttttaatcgctcactagcctggactagttccttatttagatcttctctttcttgttgtaacgttttgatttgtttttcataagccttgatttgtctaaaagcatcatctagttcttgcctcacagcattagcttcttcaagttgctgttccaaatgacttgattctgttacttgttttcttagtttttcaatttcttcttttaagttttttatttctaaatctttgcttgctgttagtggaccatcaacagttgaatactgcagagcttggacagtctgtgttgactcttgaagttttctactgagttcaagtttttcttgctcaaggcgcttaattcttctttcataagcttcagttgctaagttgttgtctagagtcctctgaacattaacatcaagatccagtgaggtgggaccagccgtaactcttaaacagctccgatcagaaagtacacagctactagtatatgtaaaaccaacaaatggcagatggtggccagaaaatgcagtatgtgttggtgggggcatcgtttcagaattttttaaacaatcatcatctacatcaaaattcgatgtatctgttgggctactaacttctggaatataaggtgcttcacagttccgaatattatcccaatcaattccactgaaaaatgggtgtttcttaaagtcttctattccattttgaccaagtcgatgttctctgctacaaatgagccttcgaataagatccttagcattttcagacacatcagtcacttgggctggaaactgaaacctctctttgtggttcatgatttttccgtatgtctccaccagcgattctgcataaaatggtgtttctccgtaaagcatttcatacatacagacccccaaagaccaccagtcacattcaggtccatatctcccttttccatcttccatggcttgaaggatttcaggagagatataatctggagttcctacagccactgaggactgaaccgttccatcttccatcagcttcagacaagaaccaaaatctgctaaccgaatatgtccattcatatccatcagtatattgtcaggtttaatgtctctgtgtacataatgtagctgatgaactgagtcaattgctatcaccatctcagccaagtaaaatctagccatatcttcaggcaatctatcttcaaatttgctgagtagagtaagcaaatccccaccaacataataatccataaccaggtataagttattgtcatcctggaaagcatagtgcaaggttgtaatccatttattgtctccattcactaatacatccctttcttcacgaaaacatgctgtctcagctcttttcagcatttcccatttattcaatattttcatggcaaacactttatctgcattttttagttttactacagcaacctccccaaaagctcctcgaccaatcacctttaatatttcaaagtcttctctatgtaatcgcatttgtttcactttagaagtaaatggtttagcccattctaggtattcgagaatgttcttctctcttctcaatggagaattattgcattcatcataaaggcagatgagtatatccagtaatgtctccacactgaagcactgcccattggtctgagcgggcccgtccaaaataaactgctccaactgcctcaaacgcacttctccagacatgtttgcttcgatttctgctggttttcctttaaattattatgatgacttttactattatctgaacctaaattttaaaaggtatggttttaaaaataaaccacttgttattcaaacaactgtcatgcaatgctggtgctgaattaaacatccaacacaccagtaacctcacttaactgaagcgtcttcaatttcacccatatacatatattttgagggtaaattaccataaaatatatacttaatgcatttttaaaagaatacaattaagtcgtatatttaaataaaataataattaaaagtacaacgaactagagagtcaacacttctttaaaaaaaaaaaaaaaaactcttctccttcattcaaaattcaactcgtgcaacgtaatcctgaaacgaatccggttgcatcattaatgaataaagtccgatttgcatcagcaattcacttcccgggaagaagaaaaacagaaaagggaggaaaaaaacagaatgcatagaagggggagggaaaaccaaaaatgttgctgcaaatcctcccaaccaccacttggataatgcatcagcggcaatttctccagcgggaaagggagggggcgaggtccctgaagcagcccctcggctcggagcacgccaagtcttgcccggaggcggcttttcgtttctcctcccgaggtccttctttctttaaggctttgcagtcagtcctattttcaacggattccggtgaaaactcttcattttcctcccggcttcaccctagggcctgaccggcggcgcggccgggggtggaaggcgggctgcgggcggcactggcaccgggctccggagaagcggctacttggccgcccgagcccactccatgtcggtggtcgctcgtgggccgagccgcgccgcgccgcgccgggcagagagcccggtctccccgacacccgcaccgggccgccgcgccggaggctcccgacgcccca

SEQ ID NO: 8654 - RNA, 6017 nt, Homo sapiens
  source 1..6017: mol_type = other RNA
aaatgtcacctttttgagaggaagagtctgaatccattccatggagttcacatcaaagatatcaactgcattttcactgtacaccgagagatatggtgcattgtaacaacaagaggaaggatttgctggccacatcaattcctgttgtctagatcttcggccctggcagtcagtgtatatcccaatgctgttaaaacacagcagatattctttactggagatctcaactgcgcagatagcatccattggttgatgtgcaataaatgatagtgtatggtcatttgaatggagcatactgtatggatttccttctccattcaaggggtatcttagaaatcctgactggaatcccacacagagttgttcactgaagattgccatccactggacattatatgggacttgaatttctttaaattttctgtgacgggtcttgctctgaaatagttcataacagaggacctgccttttcatagccacacacaggcatgtgagagctccatggcgcacctttccagaagttacggtttgacaccctttagtttctgacagcttgtaaaaatcggtctctcgcccatccaatgctgacataggaaaaagtcgtacatgacgatttcgtcctgagatcacagcaacaagctgatcatttggaatgagttcaatctgatgaatcttcttattgtcaccaactctaataatttcatctttggtgacatgtacaacaaataacccttcttcgtttcccaaagcaattctttcatgatctatgattgcggctgcctgggttgttttaatgaggggtagagtgctgtcataagcctctttgggaacatagactgagcggtctctgaatttgtttttcttcaaaatcttgtgcaattcactcagcactcccacccacttattcttctcattctcagtgtctgctagcatcaggattgaacatttgttattagatgctgagagctgggaagctgtgaccctaaatatacagggtatatctttccgacttgcatggataacatcagaagccaagactgaactcacagaaaattcttcatccctcatgtcaatcacttgactaatgacaacactgggctgagatgcttttccttcagcaatatcgtacagaaagagtttgaagtcacacactatagccagtgctctctgccaccctttcttcactccagctggcttaggaatcctgacatgaccttcatatgctgttcctattcctttctgaggatctatacccaggggaccttttgtctgttcaggaggaactggacaagtggttggagctttgtttacacaagttatatggcatgagaatccacacacttcacatgaacagccctgtcttattaaacccaccatcaaggaggtacactgatgacacttggtaggagtagtaaaagattttacaaaaaactggtgagtcttgcgcttaggtggaaagccagttgaaccaggacatccttttttccttaaggttggtgtgtgaactgaaagtggagtggagtctacagtcttaactggctcagcttcactagatgtggaaggagatgtggaccgtgactggatgtgaaacttgacgctcgggttccatacatatgtgttctcaacgggatcagtttcaaattgatccagagcatcggtaggcgtattcaaaaatgccaagaaagaatgctgtgagtcttggtgctctatacccttttcagatctaagctcttcagtgtcctttatcagctgttcgatttctgagagtagttccaagttcttcttctctgaatcttttagtttacattctgttatgatattagatgctttaactttattcaactcttcttggatggcctgtttggctcttatttctgcatccagagccgactgcaactccagtctagctgacatatccagtttcgcaaaacgacgcattttccagggcatatctgttgctcgtgtacccaagctggaatttcttaatgcctccaattcttcagtcattttagaagctaaggcctgaagataccctcgtgcatccttttcatcgctgacccactgaattatttctgtgatttgggcttcccaatgtgcaactgattctttcttgtctgctagatctttaacctcttcttctaactgctggttgtgtatacttaagttctcatacaaagtagtaagcttatcaagttcactcgtcagctttttattttcttcagttaacaacactttttctcgttcatattgttgtttgaactcactttcaaattcctccctttcactttgactttctcttctggttttttccaatttgtcttttaaaatcataatttctttgttgagagcaagttgctgaccttctgaatcatgcagttctttcttaagattttttatttcatttgcatgtattccttctcttttagataattcttcttcataaaagatacttttcttttccaaatcagtctttagtttggttatctcttgctgatgttctatgctgcatactcctggtgagtaactaatttgtttttgcttcagtccctccaattcattttccagttgcttagaatagtgctcactctgttcacgtagcttcctgtctttagatgcttcagcagctagagcttctgtatgaacttccagctcttttttggctctttctgttctgcgcagttcttgccttaagctttcaactttttgcatcaccaggtccacctcttcttccttatctcggacatggcgagcaagtttctgtttttgggtgtgcaattctgttagccgctcattgatctccatgaattcctgcatggccagtttcctctgacagtgtgcgtctttcagctctttggattggttttttaatcgctcactagcctggactagttccttatttagatcttctctttcttgttgtaacgttttgatttgtttttcataagccttgatttgtctaaaagcatcatctagttcttgcctcacagcattagcttcttcaagttgctgttccaaatgacttgattctgttacttgttttcttagtttttcaatttcttcttttaagttttttatttctaaatctttgcttgctgttagtggaccatcaacagttgaatactgcagagcttggacagtctgtgttgactcttgaagttttctactgagttcaagtttttcttgctcaaggcgcttaattcttctttcataagcttcagttgctaagttgttgtctagagtcctctgaacattaacatcaagatccagtgaggtgggaccagccgtaactcttaaacagctccgatcagaaagtacacagctactagtatatgtaaaaccaacaaatggcagatggtggccagaaaatgcagtatgtgttggtgggggcatcgtttcagaattttttaaacaatcatcatctacatcaaaattcgatgtatctgttgggctactaacttctggaatataaggtgcttcacagttccgaatattatcccaatcaattccactgaaaaatgggtgtttcttaaagtcttctattccattttgaccaagtcgatgttctctgctacaaatgagccttcgaataagatccttagcattttcagacacatcagtcacttgggctggaaactgaaacctctctttgtggttcatgatttttccgtatgtctccaccagcgattctgcataaaatggtgtttctccgtaaagcatttcatacatacagacccccaaagaccaccagtcacattcaggtccatatctcccttttccatcttccatggcttgaaggatttcaggagagatataatctggagttcctacagccactgaggactgaaccgttccatcttccatcagcttcagacaagaaccaaaatctgctaaccgaatatgtccattcatatccatcagtatattgtcaggtttaatgtctctgtgtacataatgtagctgatgaactgagtcaattgctatcaccatctcagccaagtaaaatctagccatatcttcaggcaatctatcttcaaatttgctgagtagagtaagcaaatccccaccaacataataatccataaccaggtataagttattgtcatcctggaaagcatagtgcaaggttgtaatccatttattgtctccattcactaatacatccctttcttcacgaaaacatgctgtctcagctcttttcagcatttcccatttattcaatattttcatggcaaacactttatctgcattttttagttttactacagcaacctgaagcaggggtagcaggccaaagcagcaagctttcacaacaagctctgaagcccagaagccttgaagctgccggagcaaggctggagcaggcagaagcggtgagccaccaggaaactgttgacaggcaacacccagggcgtaagttaaaggttttcctccccaaaagctcctcgaccaatcacctttaatatttcaaagtcttctctatgtaatcgcatttgtttcactttagaagtaaatggtttagcccattctaggtattcgagaatgttcttctctcttctcaatggagaattattgcattcatcataaaggcagatgagtatatccagtaatgtctccacactgaagcactgcccattggtctgagcgggcccgtccaaaataaactgctccaactgcctcaaacgcacttctccagacatgtttgcttcgatttctgctggttttcctttaaattattatgatgacttttactattatctgaacctaaattttaaaaggtatggttttaaaaataaaccacttgttattcaaacaactgtcatgcaatgctggtgctgaattaaacatccaacacaccagtaacctcacttaactgaagcgtcttcaatttcacccatatacatatattttgagggtaaattaccataaaatatatacttaatgcatttttaaaagaatacaattaagtcgtatatttaaataaaataataattaaaagtacaacgaactagagagtcaacacttctttaaaaaaaaaaaaaaaaactcttctccttcattcaaaattcaactcgtgcaacgtaatcctgaaacgaatccggttgcatcattaatgaataaagtccgatttgcatcagcaattcacttcccgggaagaagaaaaacagaaaagggaggaaaaaaacagaatgcatagaagggggagggaaaaccaaaaatgttgctgcaaatcctcccaaccaccacttggataatgcatcagcggcaatttctccagcgggaaagggagggggcgaggtccctgaagcagcccctcggctcggagcacgccaagtcttgcccggaggcggcttttcgtttctcctcccgaggtccttctttctttaaggctttgcagtcagtcctattttcaacggattccggtgaaaactcttcattttcctcccggcttcaccctagggcctgaccggcggcgcggccgggggtggaaggcgggctgcgggcggcactggcaccgggctccggagaagcggctacttggccgcccgagcccactccatgtcggtggtcgctcgtgggccgagccgcgccgcgccgcgccgggcagagagcccggtctccccgacacccgcaccgggccgccgcgccggaggctcccgacgccccaggcgggggggtgcttctctgaattcaaaggacacaagcagcagcagctgcggcggcggcgcgggcggctctggcagctacttctcccccttcttcacacccctgggctaagggcatctttccacagcgaggagggaggcggcccggcgcaggaggaggggtcgcttccgcggctgaggagactagaggctgcggcagcccggctcccaaccactcccttcctctcccttccagccctcccccgccttccctctcctctcgcgctcgcgccctgggctcagcgaggctcctccagtcccgccgcacagaggcggaggcttgcggacgagtctggatccaatatggcggcctgg

SEQ ID NO: 8655 - RNA, 5450 nt, Homo sapiens
  source 1..5450: mol_type = other RNA
aaatgtcacctttttgagaggaagagtctgaatccattccatggagttcacatcaaagatatcaactgcattttcactgtacaccgagagatatggtgcattgtaacaacaagaggaaggatttgctggccacatcaattcctgttgtctagatcttcggccctggcagtcagtgtatatcccaatgctgttaaaacacagcagatattctttactggagatctcaactgcgcagatagcatccattggttgatgtgcaataaatgatagtgtatggtcatttgaatggagcatactgtatggatttccttctccattcaaggggtatcttagaaatcctgactggaatcccacacagagttgttcactgaagattgccatccactggacattatatgggacttgaatttctttaaattttctgtgacgggtcttgctctgaaatagttcataacagaggacctgccttttcatagccacacacaggcatgtgagagctccatggcgcacctttccagaagttacggtttgacaccctttagtttctgacagcttgtaaaaatcggtctctcgcccatccaatgctgacataggaaaaagtcgtacatgacgatttcgtcctgagatcacagcaacaagctgatcatttggaatgagttcaatctgatgaatcttcttattgtcaccaactctaataatttcatctttggtgacatgtacaacaaataacccttcttcgtttcccaaagcaattctttcatgatctatgattgcggctgcctgggttgttttaatgaggggtagagtgctgtcataagcctctttgggaacatagactgagcggtctctgaatttgtttttcttcaaaatcttgtgcaattcactcagcactcccacccacttattcttctcattctcagtgtctgctagcatcaggattgaacatttgttattagatgctgagagctgggaagctgtgaccctaaatatacagggtatatctttccgacttgcatggataacatcagaagccaagactgaactcacagaaaattcttcatccctcatgtcaatcacttgactaatgacaacactgggctgagatgcttttccttcagcaatatcgtacagaaagagtttgaagtcacacactatagccagtgctctctgccaccctttcttcactccagctggcttaggaatcctgacatgaccttcatatgctgttcctattcctttctgaggatctatacccaggggaccttttgtctgttcaggaggaactggacaagtggttggagctttgtttacacaagttatatggcatgagaatccacacacttcacatgaacagccctgtcttattaaacccaccatcaaggaggtacactgatgacacttggtaggagtagtaaaagattttacaaaaaactggtgagtcttgcgcttaggtggaaagccagttgaaccaggacatccttttttccttaaggttggtgtgtgaactgaaagtggagtggagtctacagtgtcatccaaaaaatcaatcagtgaagatgaggaagaagaaaaggaatcttcaaattgatccagagcatcggtaggcgtattcaaaaatgccaagaaagaatgctgtgagtcttggtgctctatacccttttcagatctaagctcttcagtgtcctttatcagctgttcgatttctgagagtagttccaagttcttcttctctgaatcttttagtttacattctgttatgatattagatgctttaactttattcaactcttcttggatggcctgtttggctcttatttctgcatccagagccgactgcaactccagtctagctgacatatccagtttcgcaaaacgacgcattttccagggcatatctgttgctcgtgtacccaagctggaatttcttaatgcctccaattcttcagtcattttagaagctaaggcctgaagataccctcgtgcatccttttcatcgctgacccactgaattatttctgtgatttgggcttcccaatgtgcaactgattctttcttgtctgctagatctttaacctcttcttctaactgctggttgtgtatacttaagttctcatacaaagtagtaagcttatcaagttcactcgtcagctttttattttcttcagttaacaacactttttctcgttcatattgttgtttgaactcactttcaaattcctccctttcactttgactttctcttctggttttttccaatttgtcttttaaaatcataatttctttgttgagagcaagttgctgaccttctgaatcatgcagttctttcttaagattttttatttcatttgcatgtattccttctcttttagataattcttcttcataaaagatacttttcttttccaaatcagtctttagtttggttatctcttgctgatgttctatgctgcatactcctggtgagtaactaatttgtttttgcttcagtccctccaattcattttccagttgcttagaatagtgctcactctgttcacgtagcttcctgtctttagatgcttcagcagctagagcttctgtatgaacttccagctcttttttggctctttctgttctgcgcagttcttgccttaagctttcaactttttgcatcaccaggtccacctcttcttccttatctcggacatggcgagcaagtttctgtttttgggtgtgcaattctgttagccgctcattgatctccatgaattcctgcatggccagtttcctctgacagtgtgcgtctttcagctctttggattggttttttaatcgctcactagcctggactagttccttatttagatcttctctttcttgttgtaacgttttgatttgtttttcataagccttgatttgtctaaaagcatcatctagttcttgcctcacagcattagcttcttcaagttgctgttccaaatgacttgattctgttacttgttttcttagtttttcaatttcttcttttaagttttttatttctaaatctttgcttgctgttagtggaccatcaacagttgaatactgcagagcttggacagtctgtgttgactcttgaagttttctactgagttcaagtttttcttgctcaaggcgcttaattcttctttcataagcttcagttgctaagttgttgtctagagtcctctgaacattaacatcaagatccagtgaggtgggaccagccgtaactcttaaacagctccgatcagaaagtacacagctactagtatatgtaaaaccaacaaatggcagatggtggccagaaaatgcagtatgtgttggtgggggcatcgtttcagaattttttaaacaatcatcatctacatcaaaattcgatgtatctgttgggctactaacttctggaatataaggtgcttcacagttccgaatattatcccaatcaattccactgaaaaatgggtgtttcttaaagtcttctattccattttgaccaagtcgatgttctctgctacaaatgagccttcgaataagatccttagcattttcagacacatcagtcacttgggctggaaactgaaacctctctttgtggttcatgatttttccgtatgtctccaccagcgattctgcataaaatggtgtttctccgtaaagcatttcatacatacagacccccaaagaccaccagtcacattcaggtccatatctcccttttccatcttccatggcttgaaggatttcaggagagatataatctggagttcctacagccactgaggactgaaccgttccatcttccatcagcttcagacaagaaccaaaatctgctaaccgaatatgtccattcatatccatcagtatattgtcaggtttaatgtctctgtgtacataatgtagctgatgaactgagtcaattgctatcaccatctcagccaagtaaaatctagccatatcttcaggcaatctatcttcaaatttgctgagtagagtaagcaaatccccaccaacataataatccataaccaggtataagttattgtcatcctggaaagcatagtgcaaggttgtaatccatttattgtctccattcactaatacatccctttcttcacgaaaacatgctgtctcagctcttttcagcatttcccatttattcaatattttcatggcaaacactttatctgcattttttagttttactacagcaacctccccaaaagctcctcgaccaatcacctttaatatttcaaagtcttctctatgtaatcgcatttgtttcactttagaagtaaatggtttagcccattctaggtattcgagaatgttcttctctcttctcaatggagaattattgcattcatcataaaggcagatgagtatatccagtaatgtctccacactgaagcactgcccattggtctgagcgggcccgtccaaaataaactgctccaactgcctcaaacgcacttctccagacatgtttgcttcgatttctgctggttttcctttaaattattatgatgacttttactattatctgaacctaaattttaaaaggtatggttttaaaaataaaccacttgttattcaaacaactgtcatgcaatgctggtgctgaattaaacatccaacacaccagtaacctcacttaactgaagcgtcttcaatttcacccatatacatatattttgagggtaaattaccataaaatatatacttaatgcatttttaaaagaatacaattaagtcgtatatttaaataaaataataattaaaagtacaacgaactagagagtcaacacttctttaaaaaaaaaaaaaaaaactcttctccttcattcaaaattcaactcgtgcaacgtaatcctgaaacgaatccggttgcatcattaatgaataaagtccgatttgcatcagcaattcacttcccgggaagaagaaaaacagaaaagggaggaaaaaaacagaatgcatagaagggggagggaaaaccaaaaatgttgctgcaaatcctcccaaccaccacttggataatgcatcagcggcaatttctccagcgggaaagggagggggcgaggtccctgaagcagcccctcggctcggagcacgccaagtcttgcccggaggcggcttttcgtttctcctcccgaggtccttctttctttaaggctttgcagtcagtcctattttcaacggattccggtgaaaactcttcattttcctcccggcttcaccctagggcctgaccggcggcgcggccgggggtggaaggcgggctgcgggcggcactggcaccgggctccggagaagcggctacttggccgcccgagcccactccatgtcggtggtcgctcgtgggccgagccgcgccgcgccgcgccgggcagagagcccggtctccccgacacccgcaccgggccgccgcgccggaggctcccgacgcccca

SEQ ID NO: 8656 - RNA, 5402 nt, Homo sapiens
  source 1..5402: mol_type = other RNA
aaatgtcacctttttgagaggaagagtctgaatccattccatggagttcacatcaaagatatcaactgcattttcactgtacaccgagagatatggtgcattgtaacaacaagaggaaggatttgctggccacatcaattcctgttgtctagatcttcggccctggcagtcagtgtatatcccaatgctgttaaaacacagcagatattctttactggagatctcaactgcgcagatagcatccattggttgatgtgcaataaatgatagtgtatggtcatttgaatggagcatactgtatggatttccttctccattcaaggggtatcttagaaatcctgactggaatcccacacagagttgttcactgaagattgccatccactggacattatatgggacttgaatttctttaaattttctgtgacgggtcttgctctgaaatagttcataacagaggacctgccttttcatagccacacacaggcatgtgagagctccatggcgcacctttccagaagttacggtttgacaccctttagtttctgacagcttgtaaaaatcggtctctcgcccatccaatgctgacataggaaaaagtcgtacatgacgatttcgtcctgagatcacagcaacaagctgatcatttggaatgagttcaatctgatgaatcttcttattgtcaccaactctaataatttcatctttggtgacatgtacaacaaataacccttcttcgtttcccaaagcaattctttcatgatctatgattgcggctgcctgggttgttttaatgaggggtagagtgctgtcataagcctctttgggaacatagactgagcggtctctgaatttgtttttcttcaaaatcttgtgcaattcactcagcactcccacccacttattcttctcattctcagtgtctgctagcatcaggattgaacatttgttattagatgctgagagctgggaagctgtgaccctaaatatacagggtatatctttccgacttgcatggataacatcagaagccaagactgaactcacagaaaattcttcatccctcatgtcaatcacttgactaatgacaacactgggctgagatgcttttccttcagcaatatcgtacagaaagagtttgaagtcacacactatagccagtgctctctgccaccctttcttcactccagctggcttaggaatcctgacatgaccttcatatgctgttcctattcctttctgaggatctatacccaggggaccttttgtctgttcaggaggaactggacaagtggttggagctttgtttacacaagttatatggcatgagaatccacacacttcacatgaacagccctgtcttattaaacccaccatcaaggaggtacactgatgacacttggtaggagtagtaaaagattttacaaaaaactggtgagtcttgcgcttaggtggaaagccagttgaaccaggacatccttttttccttaaggttggtgtgtgaactgaaagtggagtggagtctacagtttcaaattgatccagagcatcggtaggcgtattcaaaaatgccaagaaagaatgctgtgagtcttggtgctctatacccttttcagatctaagctcttcagtgtcctttatcagctgttcgatttctgagagtagttccaagttcttcttctctgaatcttttagtttacattctgttatgatattagatgctttaactttattcaactcttcttggatggcctgtttggctcttatttctgcatccagagccgactgcaactccagtctagctgacatatccagtttcgcaaaacgacgcattttccagggcatatctgttgctcgtgtacccaagctggaatttcttaatgcctccaattcttcagtcattttagaagctaaggcctgaagataccctcgtgcatccttttcatcgctgacccactgaattatttctgtgatttgggcttcccaatgtgcaactgattctttcttgtctgctagatctttaacctcttcttctaactgctggttgtgtatacttaagttctcatacaaagtagtaagcttatcaagttcactcgtcagctttttattttcttcagttaacaacactttttctcgttcatattgttgtttgaactcactttcaaattcctccctttcactttgactttctcttctggttttttccaatttgtcttttaaaatcataatttctttgttgagagcaagttgctgaccttctgaatcatgcagttctttcttaagattttttatttcatttgcatgtattccttctcttttagataattcttcttcataaaagatacttttcttttccaaatcagtctttagtttggttatctcttgctgatgttctatgctgcatactcctggtgagtaactaatttgtttttgcttcagtccctccaattcattttccagttgcttagaatagtgctcactctgttcacgtagcttcctgtctttagatgcttcagcagctagagcttctgtatgaacttccagctcttttttggctctttctgttctgcgcagttcttgccttaagctttcaactttttgcatcaccaggtccacctcttcttccttatctcggacatggcgagcaagtttctgtttttgggtgtgcaattctgttagccgctcattgatctccatgaattcctgcatggccagtttcctctgacagtgtgcgtctttcagctctttggattggttttttaatcgctcactagcctggactagttccttatttagatcttctctttcttgttgtaacgttttgatttgtttttcataagccttgatttgtctaaaagcatcatctagttcttgcctcacagcattagcttcttcaagttgctgttccaaatgacttgattctgttacttgttttcttagtttttcaatttcttcttttaagttttttatttctaaatctttgcttgctgttagtggaccatcaacagttgaatactgcagagcttggacagtctgtgttgactcttgaagttttctactgagttcaagtttttcttgctcaaggcgcttaattcttctttcataagcttcagttgctaagttgttgtctagagtcctctgaacattaacatcaagatccagtgaggtgggaccagccgtaactcttaaacagctccgatcagaaagtacacagctactagtatatgtaaaaccaacaaatggcagatggtggccagaaaatgcagtatgtgttggtgggggcatcgtttcagaattttttaaacaatcatcatctacatcaaaattcgatgtatctgttgggctactaacttctggaatataaggtgcttcacagttccgaatattatcccaatcaattccactgaaaaatgggtgtttcttaaagtcttctattccattttgaccaagtcgatgttctctgctacaaatgagccttcgaataagatccttagcattttcagacacatcagtcacttgggctggaaactgaaacctctctttgtggttcatgatttttccgtatgtctccaccagcgattctgcataaaatggtgtttctccgtaaagcatttcatacatacagacccccaaagaccaccagtcacattcaggtccatatctcccttttccatcttccatggcttgaaggatttcaggagagatataatctggagttcctacagccactgaggactgaaccgttccatcttccatcagcttcagacaagaaccaaaatctgctaaccgaatatgtccattcatatccatcagtatattgtcaggtttaatgtctctgtgtacataatgtagctgatgaactgagtcaattgctatcaccatctcagccaagtaaaatctagccatatcttcaggcaatctatcttcaaatttgctgagtagagtaagcaaatccccaccaacataataatccataaccaggtataagttattgtcatcctggaaagcatagtgcaaggttgtaatccatttattgtctccattcactaatacatccctttcttcacgaaaacatgctgtctcagctcttttcagcatttcccatttattcaatattttcatggcaaacactttatctgcattttttagttttactacagcaacctccccaaaagctcctcgaccaatcacctttaatatttcaaagtcttctctatgtaatcgcatttgtttcactttagaagtaaatggtttagcccattctaggtattcgagaatgttcttctctcttctcaatggagaattattgcattcatcataaaggcagatgagtatatccagtaatgtctccacactgaagcactgcccattggtctgagcgggcccgtccaaaataaactgctccaactgcctcaaacgcacttctccagacatgtttgcttcgatttctgctggttttcctttaaattattatgatgacttttactattatctgaacctaaattttaaaaggtatggttttaaaaataaaccacttgttattcaaacaactgtcatgcaatgctggtgctgaattaaacatccaacacaccagtaacctcacttaactgaagcgtcttcaatttcacccatatacatatattttgagggtaaattaccataaaatatatacttaatgcatttttaaaagaatacaattaagtcgtatatttaaataaaataataattaaaagtacaacgaactagagagtcaacacttctttaaaaaaaaaaaaaaaaactcttctccttcattcaaaattcaactcgtgcaacgtaatcctgaaacgaatccggttgcatcattaatgaataaagtccgatttgcatcagcaattcacttcccgggaagaagaaaaacagaaaagggaggaaaaaaacagaatgcatagaagggggagggaaaaccaaaaatgttgctgcaaatcctcccaaccaccacttggataatgcatcagcggcaatttctccagcgggaaagggagggggcgaggtccctgaagcagcccctcggctcggagcacgccaagtcttgcccggaggcggcttttcgtttctcctcccgaggtccttctttctttaaggctttgcagtcagtcctattttcaacggattccggtgaaaactcttcattttcctcccggcttcaccctagggcctgaccggcggcgcggccgggggtggaaggcgggctgcgggcggcactggcaccgggctccggagaagcggctacttggccgcccgagcccactccatgtcggtggtcgctcgtgggccgagccgcgccgcgccgcgccgggcagagagcccggtctccccgacacccgcaccgggccgccgcgccggaggctcccgacgcccca

SEQ ID NO: 8657 - RNA, 5744 nt, Homo sapiens
  source 1..5744: mol_type = other RNA
aaatgtcacctttttgagaggaagagtctgaatccattccatggagttcacatcaaagatatcaactgcattttcactgtacaccgagagatatggtgcattgtaacaacaagaggaaggatttgctggccacatcaattcctgttgtctagatcttcggccctggcagtcagtgtatatcccaatgctgttaaaacacagcagatattctttactggagatctcaactgcgcagatagcatccattggttgatgtgcaataaatgatagtgtatggtcatttgaatggagcatactgtatggatttccttctccattcaaggggtatcttagaaatcctgactggaatcccacacagagttgttcactgaagattgccatccactggacattatatgggacttgaatttctttaaattttctgtgacgggtcttgctctgaaatagttcataacagaggacctgccttttcatagccacacacaggcatgtgagagctccatggcgcacctttccagaagttacggtttgacaccctttagtttctgacagcttgtaaaaatcggtctctcgcccatccaatgctgacataggaaaaagtcgtacatgacgatttcgtcctgagatcacagcaacaagctgatcatttggaatgagttcaatctgatgaatcttcttattgtcaccaactctaataatttcatctttggtgacatgtacaacaaataacccttcttcgtttcccaaagcaattctttcatgatctatgattgcggctgcctgggttgttttaatgaggggtagagtgctgtcataagcctctttgggaacatagactgagcggtctctgaatttgtttttcttcaaaatcttgtgcaattcactcagcactcccacccacttattcttctcattctcagtgtctgctagcatcaggattgaacatttgttattagatgctgagagctgggaagctgtgaccctaaatatacagggtatatctttccgacttgcatggataacatcagaagccaagactgaactcacagaaaattcttcatccctcatgtcaatcacttgactaatgacaacactgggctgagatgcttttccttcagcaatatcgtacagaaagagtttgaagtcacacactatagccagtgctctctgccaccctttcttcactccagctggcttaggaatcctgacatgaccttcatatgctgttcctattcctttctgaggatctatacccaggggaccttttgtctgttcaggaggaactggacaagtggttggagctttgtttacacaagttatatggcatgagaatccacacacttcacatgaacagccctgtcttattaaacccaccatcaaggaggtacactgatgacacttggtaggagtagtaaaagattttacaaaaaactggtgagtcttgcgcttaggtggaaagccagttgaaccaggacatccttttttccttaaggttggtgtgtgaactgaaagtggagtggagtctacagtttcaaattgatccagagcatcggtaggcgtattcaaaaatgccaagaaagaatgctgtgagtcttggtgctctatacccttttcagatctaagctcttcagtgtcctttatcagctgttcgatttctgagagtagttccaagttcttcttctctgaatcttttagtttacattctgttatgatattagatgctttaactttattcaactcttcttggatggcctgtttggctcttatttctgcatccagagccgactgcaactccagtctagctgacatatccagtttcgcaaaacgacgcattttccagggcatatctgttgctcgtgtacccaagctggaatttcttaatgcctccaattcttcagtcattttagaagctaaggcctgaagataccctcgtgcatccttttcatcgctgacccactgaattatttctgtgatttgggcttcccaatgtgcaactgattctttcttgtctgctagatctttaacctcttcttctaactgctggttgtgtatacttaagttctcatacaaagtagtaagcttatcaagttcactcgtcagctttttattttcttcagttaacaacactttttctcgttcatattgttgtttgaactcactttcaaattcctccctttcactttgactttctcttctggttttttccaatttgtcttttaaaatcataatttctttgttgagagcaagttgctgaccttctgaatcatgcagttctttcttaagattttttatttcatttgcatgtattccttctcttttagataattcttcttcataaaagatacttttcttttccaaatcagtctttagtttggttatctcttgctgatgttctatgctgcatactcctggtgagtaactaatttgtttttgcttcagtccctccaattcattttccagttgcttagaatagtgctcactctgttcacgtagcttcctgtctttagatgcttcagcagctagagcttctgtatgaacttccagctcttttttggctctttctgttctgcgcagttcttgccttaagctttcaactttttgcatcaccaggtccacctcttcttccttatctcggacatggcgagcaagtttctgtttttgggtgtgcaattctgttagccgctcattgatctccatgaattcctgcatggccagtttcctctgacagtgtgcgtctttcagctctttggattggttttttaatcgctcactagcctggactagttccttatttagatcttctctttcttgttgtaacgttttgatttgtttttcataagccttgatttgtctaaaagcatcatctagttcttgcctcacagcattagcttcttcaagttgctgttccaaatgacttgattctgttacttgttttcttagtttttcaatttcttcttttaagttttttatttctaaatctttgcttgctgttagtggaccatcaacagttgaatactgcagagcttggacagtctgtgttgactcttgaagttttctactgagttcaagtttttcttgctcaaggcgcttaattcttctttcataagcttcagttgctaagttgttgtctagagtcctctgaacattaacatcaagatccagtgaggtgggaccagccgtaactcttaaacagctccgatcagaaagtacacagctactagtatatgtaaaaccaacaaatggcagatggtggccagaaaatgcagtatgtgttggtgggggcatcgtttcagaattttttaaacaatcatcatctacatcaaaattcgatgtatctgttgggctactaacttctggaatataaggtgcttcacagttccgaatattatcccaatcaattccactgaaaaatgggtgtttcttaaagtcttctattccattttgaccaagtcgatgttctctgctacaaatgagccttcgaataagatccttagcattttcagacacatcagtcacttgggctggaaactgaaacctctctttgtggttcatgatttttccgtatgtctccaccagcgattctgcataaaatggtgtttctccgtaaagcatttcatacatacagacccccaaagaccaccagtcacattcaggtccatatctcccttttccatcttccatggcttgaaggatttcaggagagatataatctggagttcctacagccactgaggactgaaccgttccatcttccatcagcttcagacaagaaccaaaatctgctaaccgaatatgtccattcatatccatcagtatattgtcaggtttaatgtctctgtgtacataatgtagctgatgaactgagtcaattgctatcaccatctcagccaagtaaaatctagccatatcttcaggcaatctatcttcaaatttgctgagtagagtaagcaaatccccaccaacataataatccataaccaggtataagttattgtcatcctggaaagcatagtgcaaggttgtaatccatttattgtctccattcactaatacatccctttcttcacgaaaacatgctgtctcagctcttttcagcatttcccatttattcaatattttcatggcaaacactttatctgcattttttagttttactacagcaacctccccaaaagctcctcgaccaatcacctttaatatttcaaagtcttctctatgtaatcgcatttgtttcactttagaagtaaatggtttagcccattctaggtattcgagaatgttcttctctcttctcaatggagaattattgcattcatcataaaggcagatgagtatatccagtaatgtctccacactgaagcactgcccattggtctgagcgggcccgtccaaaataaactgctccaactgcctcaaacgcacttctccagacatgtttgcttcgatttctgctggttttcctttaaattattatgatgacttttactattatctgaacctaaattttaaaaggtatggttttaaaaataaaccacttgttattcaaacaactgtcatgcaatgctggtgctgaattaaacatccaacacaccagtaacctcacttaactgaagcgtcttcaatttcacccatatacatatattttgagggtaaattaccataaaatatatacttaatgcatttttaaaagaatacaattaagtcgtatatttaaataaaataataattaaaagtacaacgaactagagagtcaacacttctttaaaaaaaaaaaaaaaaactcttctccttcattcaaaattcaactcgtgcaacgtaatcctgaaacgaatccggttgcatcattaatgaataaagtccgatttgcatcagcaattcacttcccgggaagaagaaaaacagaaaagggaggaaaaaaacagaatgcatagaagggggagggaaaaccaaaaatgttgctgcaaatcctcccaaccaccacttggataatgcatcagcggcaatttctccagcgggaaagggagggggcgaggtccctgaagcagcccctcggctcggagcacgccaagtcttgcccggaggcggcttttcgtttctcctcccgaggtccttctttctttaaggctttgcagtcagtcctattttcaacggattccggtgaaaactcttcattttcctcccggcttcaccctagggcctgaccggcggcgcggccgggggtggaaggcgggctgcgggcggcactggcaccgggctccggagaagcggctacttggccgcccgagcccactccatgtcggtggtcgctcgtgggccgagccgcgccgcgccgcgccgggcagagagcccggtctccccgacacccgcaccgggccgccgcgccggaggctcccgacgccccaggcgggggggtgcttctctgaattcaaaggacacaagcagcagcagctgcggcggcggcgcgggcggctctggcagctacttctcccccttcttcacacccctgggctaagggcatctttccacagcgaggagggaggcggcccggcgcaggaggaggggtcgcttccgcggctgaggagactagaggctgcggcagcccggctcccaaccactcccttcctctcccttccagccctcccccgccttccctctcctctcgcgctcgcgccctgggctcagcgaggctcctccagtcccgccgcacagaggcggaggcttgcggacgagtctggatccaatat

SEQ ID NO: 8658 - RNA, 5501 nt, Homo sapiens
  source 1..5501: mol_type = other RNA
aaatgtcacctttttgagaggaagagtctgaatccattccatggagttcacatcaaagatatcaactgcattttcactgtacaccgagagatatggtgcattgtaacaacaagaggaaggatttgctggccacatcaattcctgttgtctagatcttcggccctggcagtcagtgtatatcccaatgctgttaaaacacagcagatattctttactggagatctcaactgcgcagatagcatccattggttgatgtgcaataaatgatagtgtatggtcatttgaatggagcatactgtatggatttccttctccattcaaggggtatcttagaaatcctgactggaatcccacacagagttgttcactgaagattgccatccactggacattatatgggacttgaatttctttaaattttctgtgacgggtcttgctctgaaatagttcataacagaggacctgccttttcatagccacacacaggcatgtgagagctccatggcgcacctttccagaagttacggtttgacaccctttagtttctgacagcttgtaaaaatcggtctctcgcccatccaatgctgacataggaaaaagtcgtacatgacgatttcgtcctgagatcacagcaacaagctgatcatttggaatgagttcaatctgatgaatcttcttattgtcaccaactctaataatttcatctttggtgacatgtacaacaaataacccttcttcgtttcccaaagcaattctttcatgatctatgattgcggctgcctgggttgttttaatgaggggtagagtgctgtcataagcctctttgggaacatagactgagcggtctctgaatttgtttttcttcaaaatcttgtgcaattcactcagcactcccacccacttattcttctcattctcagtgtctgctagcatcaggattgaacatttgttattagatgctgagagctgggaagctgtgaccctaaatatacagggtatatctttccgacttgcatggataacatcagaagccaagactgaactcacagaaaattcttcatccctcatgtcaatcacttgactaatgacaacactgggctgagatgcttttccttcagcaatatcgtacagaaagagtttgaagtcacacactatagccagtgctctctgccaccctttcttcactccagctggcttaggaatcctgacatgaccttcatatgctgttcctattcctttctgaggatctatacccaggggaccttttgtctgttcaggaggaactggacaagtggttggagctttgtttacacaagttatatggcatgagaatccacacacttcacatgaacagccctgtcttattaaacccaccatcaaggaggtacactgatgacacttggtaggagtagtaaaagattttacaaaaaactggtgagtcttgcgcttaggtggaaagccagttgaaccaggacatccttttttccttaaggttggtgtgtgaactgaaagtggagtggagtctacagtttcaaattgatccagagcatcggtaggcgtattcaaaaatgccaagaaagaatgctgtgagtcttggtgctctatacccttttcagatctaagctcttcagtgtcctttatcagctgttcgatttctgagagtagttccaagttcttcttctctgaatcttttagtttacattctgttatgatattagatgctttaactttattcaactcttcttggatggcctgtttggctcttatttctgcatccagagccgactgcaactccagtctagctgacatatccagtttcgcaaaacgacgcattttccagggcatatctgttgctcgtgtacccaagctggaatttcttaatgcctccaattcttcagtcattttagaagctaaggcctgaagataccctcgtgcatccttttcatcgctgacccactgaattatttctgtgatttgggcttcccaatgtgcaactgattctttcttgtctgctagatctttaacctcttcttctaactgctggttgtgtatacttaagttctcatacaaagtagtaagcttatcaagttcactcgtcagctttttattttcttcagttaacaacactttttctcgttcatattgttgtttgaactcactttcaaattcctccctttcactttgactttctcttctggttttttccaatttgtcttttaaaatcataatttctttgttgagagcaagttgctgaccttctgaatcatgcagttctttcttaagattttttatttcatttgcatgtattccttctcttttagataattcttcttcataaaagatacttttcttttccaaatcagtctttagtttggttatctcttgctgatgttctatgctgcatactcctggtgagtaactaatttgtttttgcttcagtccctccaattcattttccagttgcttagaatagtgctcactctgttcacgtagcttcctgtctttagatgcttcagcagctagagcttctgtatgaacttccagcttatttagatcttctctttcttgttgtaacgttttgatttgtttttcataagccttgatttgtctaaaagcatcatctagttcttgcctcacagcattagcttcttcaagttgctgttccaaatgacttgattctgttacttgttttcttagtttttcaatttcttcttttaagttttttatttctaaatctttgcttgctgttagtggaccatcaacagttgaatactgcagagcttggacagtctgtgttgactcttgaagttttctactgagttcaagtttttcttgctcaaggcgcttaattcttctttcataagcttcagttgctaagttgttgtctagagtcctctgaacattaacatcaagatccagtgaggtgggaccagccgtaactcttaaacagctccgatcagaaagtacacagctactagtatatgtaaaaccaacaaatggcagatggtggccagaaaatgcagtatgtgttggtgggggcatcgtttcagaattttttaaacaatcatcatctacatcaaaattcgatgtatctgttgggctactaacttctggaatataaggtgcttcacagttccgaatattatcccaatcaattccactgaaaaatgggtgtttcttaaagtcttctattccattttgaccaagtcgatgttctctgctacaaatgagccttcgaataagatccttagcattttcagacacatcagtcacttgggctggaaactgaaacctctctttgtggttcatgatttttccgtatgtctccaccagcgattctgcataaaatggtgtttctccgtaaagcatttcatacatacagacccccaaagaccaccagtcacattcaggtccatatctcccttttccatcttccatggcttgaaggatttcaggagagatataatctggagttcctacagccactgaggactgaaccgttccatcttccatcagcttcagacaagaaccaaaatctgctaaccgaatatgtccattcatatccatcagtatattgtcaggtttaatgtctctgtgtacataatgtagctgatgaactgagtcaattgctatcaccatctcagccaagtaaaatctagccatatcttcaggcaatctatcttcaaatttgctgagtagagtaagcaaatccccaccaacataataatccataaccaggtataagttattgtcatcctggaaagcatagtgcaaggttgtaatccatttattgtctccattcactaatacatccctttcttcacgaaaacatgctgtctcagctcttttcagcatttcccatttattcaatattttcatggcaaacactttatctgcattttttagttttactacagcaacctccccaaaagctcctcgaccaatcacctttaatatttcaaagtcttctctatgtaatcgcatttgtttcactttagaagtaaatggtttagcccattctaggtattcgagaatgttcttctctcttctcaatggagaattattgcattcatcataaaggcagatgagtatatccagtaatgtctccacactgaagcactgcccattggtctgagcgggcccgtccaaaataaactgctccaactgcctcaaacgcacttctccagacatgtttgcttcgatttctgctggttttcctttaaattattatgatgacttttactattatctgaacctaaattttaaaaggtatggttttaaaaataaaccacttgttattcaaacaactgtcatgcaatgctggtgctgaattaaacatccaacacaccagtaacctcacttaactgaagcgtcttcaatttcacccatatacatatattttgagggtaaattaccataaaatatatacttaatgcatttttaaaagaatacaattaagtcgtatatttaaataaaataataattaaaagtacaacgaactagagagtcaacacttctttaaaaaaaaaaaaaaaaactcttctccttcattcaaaattcaactcgtgcaacgtaatcctgaaacgaatccggttgcatcattaatgaataaagtccgatttgcatcagcaattcacttcccgggaagaagaaaaacagaaaagggaggaaaaaaacagaatgcatagaagggggagggaaaaccaaaaatgttgctgcaaatcctcccaaccaccacttggataatgcatcagcggcaatttctccagcgggaaagggagggggcgaggtccctgaagcagcccctcggctcggagcacgccaagtcttgcccggaggcggcttttcgtttctcctcccgaggtccttctttctttaaggctttgcagtcagtcctattttcaacggattccggtgaaaactcttcattttcctcccggcttcaccctagggcctgaccggcggcgcggccgggggtggaaggcgggctgcgggcggcactggcaccgggctccggagaagcggctacttggccgcccgagcccactccatgtcggtggtcgctcgtgggccgagccgcgccgcgccgcgccgggcagagagcccggtctccccgacacccgcaccgggccgccgcgccggaggctcccgacgccccaggcgggggggtgcttctctgaattcaaaggacacaagcagcagcagctgcggcggcggcgcgggcggctctggcagctacttctcccccttcttcacacccctgggctaagggcatctttccacagcgaggagggaggcggcccggcgcaggaggaggggtcgcttccgcggctgaggagactagaggctgcggcagcccggctcccaaccactcccttcctctcccttccagccctcccccgccttccctctcctctcgcgctcgcgccctgggctcagcgaggctcctccagtcccgccgcacagaggcggaggcttgcggacgagtctggatccaatat

SEQ ID NO: 8659 - RNA, 5660 nt, Homo sapiens
  source 1..5660: mol_type = other RNA
aaatgtcacctttttgagaggaagagtctgaatccattccatggagttcacatcaaagatatcaactgcattttcactgtacaccgagagatatggtgcattgtaacaacaagaggaaggatttgctggccacatcaattcctgttgtctagatcttcggccctggcagtcagtgtatatcccaatgctgttaaaacacagcagatattctttactggagatctcaactgcgcagatagcatccattggttgatgtgcaataaatgatagtgtatggtcatttgaatggagcatactgtatggatttccttctccattcaaggggtatcttagaaatcctgactggaatcccacacagagttgttcactgaagattgccatccactggacattatatgggacttgaatttctttaaattttctgtgacgggtcttgctctgaaatagttcataacagaggacctgccttttcatagccacacacaggcatgtgagagctccatggcgcacctttccagaagttacggtttgacaccctttagtttctgacagcttgtaaaaatcggtctctcgcccatccaatgctgacataggaaaaagtcgtacatgacgatttcgtcctgagatcacagcaacaagctgatcatttggaatgagttcaatctgatgaatcttcttattgtcaccaactctaataatttcatctttggtgacatgtacaacaaataacccttcttcgtttcccaaagcaattctttcatgatctatgattgcggctgcctgggttgttttaatgaggggtagagtgctgtcataagcctctttgggaacatagactgagcggtctctgaatttgtttttcttcaaaatcttgtgcaattcactcagcactcccacccacttattcttctcattctcagtgtctgctagcatcaggattgaacatttgttattagatgctgagagctgggaagctgtgaccctaaatatacagggtatatctttccgacttgcatggataacatcagaagccaagactgaactcacagaaaattcttcatccctcatgtcaatcacttgactaatgacaacactgggctgagatgcttttccttcagcaatatcgtacagaaagagtttgaagtcacacactatagccagtgctctctgccaccctttcttcactccagctggcttaggaatcctgacatgaccttcatatgctgttcctattcctttctgaggatctatacccaggggaccttttgtctgttcaggaggaactggacaagtggttggagctttgtttacacaagttatatggcatgagaatccacacacttcacatgaacagccctgtcttattaaacccaccatcaaggaggtacactgatgacacttggtaggagtagtaaaagattttacaaaaaactggtgagtcttgcgttcaaattgatccagagcatcggtaggcgtattcaaaaatgccaagaaagaatgctgtgagtcttggtgctctatacccttttcagatctaagctcttcagtgtcctttatcagctgttcgatttctgagagtagttccaagttcttcttctctgaatcttttagtttacattctgttatgatattagatgctttaactttattcaactcttcttggatggcctgtttggctcttatttctgcatccagagccgactgcaactccagtctagctgacatatccagtttcgcaaaacgacgcattttccagggcatatctgttgctcgtgtacccaagctggaatttcttaatgcctccaattcttcagtcattttagaagctaaggcctgaagataccctcgtgcatccttttcatcgctgacccactgaattatttctgtgatttgggcttcccaatgtgcaactgattctttcttgtctgctagatctttaacctcttcttctaactgctggttgtgtatacttaagttctcatacaaagtagtaagcttatcaagttcactcgtcagctttttattttcttcagttaacaacactttttctcgttcatattgttgtttgaactcactttcaaattcctccctttcactttgactttctcttctggttttttccaatttgtcttttaaaatcataatttctttgttgagagcaagttgctgaccttctgaatcatgcagttctttcttaagattttttatttcatttgcatgtattccttctcttttagataattcttcttcataaaagatacttttcttttccaaatcagtctttagtttggttatctcttgctgatgttctatgctgcatactcctggtgagtaactaatttgtttttgcttcagtccctccaattcattttccagttgcttagaatagtgctcactctgttcacgtagcttcctgtctttagatgcttcagcagctagagcttctgtatgaacttccagctcttttttggctctttctgttctgcgcagttcttgccttaagctttcaactttttgcatcaccaggtccacctcttcttccttatctcggacatggcgagcaagtttctgtttttgggtgtgcaattctgttagccgctcattgatctccatgaattcctgcatggccagtttcctctgacagtgtgcgtctttcagctctttggattggttttttaatcgctcactagcctggactagttccttatttagatcttctctttcttgttgtaacgttttgatttgtttttcataagccttgatttgtctaaaagcatcatctagttcttgcctcacagcattagcttcttcaagttgctgttccaaatgacttgattctgttacttgttttcttagtttttcaatttcttcttttaagttttttatttctaaatctttgcttgctgttagtggaccatcaacagttgaatactgcagagcttggacagtctgtgttgactcttgaagttttctactgagttcaagtttttcttgctcaaggcgcttaattcttctttcataagcttcagttgctaagttgttgtctagagtcctctgaacattaacatcaagatccagtgaggtgggaccagccgtaactcttaaacagctccgatcagaaagtacacagctactagtatatgtaaaaccaacaaatggcagatggtggccagaaaatgcagtatgtgttggtgggggcatcgtttcagaattttttaaacaatcatcatctacatcaaaattcgatgtatctgttgggctactaacttctggaatataaggtgcttcacagttccgaatattatcccaatcaattccactgaaaaatgggtgtttcttaaagtcttctattccattttgaccaagtcgatgttctctgctacaaatgagccttcgaataagatccttagcattttcagacacatcagtcacttgggctggaaactgaaacctctctttgtggttcatgatttttccgtatgtctccaccagcgattctgcataaaatggtgtttctccgtaaagcatttcatacatacagacccccaaagaccaccagtcacattcaggtccatatctcccttttccatcttccatggcttgaaggatttcaggagagatataatctggagttcctacagccactgaggactgaaccgttccatcttccatcagcttcagacaagaaccaaaatctgctaaccgaatatgtccattcatatccatcagtatattgtcaggtttaatgtctctgtgtacataatgtagctgatgaactgagtcaattgctatcaccatctcagccaagtaaaatctagccatatcttcaggcaatctatcttcaaatttgctgagtagagtaagcaaatccccaccaacataataatccataaccaggtataagttattgtcatcctggaaagcatagtgcaaggttgtaatccatttattgtctccattcactaatacatccctttcttcacgaaaacatgctgtctcagctcttttcagcatttcccatttattcaatattttcatggcaaacactttatctgcattttttagttttactacagcaacctccccaaaagctcctcgaccaatcacctttaatatttcaaagtcttctctatgtaatcgcatttgtttcactttagaagtaaatggtttagcccattctaggtattcgagaatgttcttctctcttctcaatggagaattattgcattcatcataaaggcagatgagtatatccagtaatgtctccacactgaagcactgcccattggtctgagcgggcccgtccaaaataaactgctccaactgcctcaaacgcacttctccagacatgtttgcttcgatttctgctggttttcctttaaattattatgatgacttttactattatctgaacctaaattttaaaaggtatggttttaaaaataaaccacttgttattcaaacaactgtcatgcaatgctggtgctgaattaaacatccaacacaccagtaacctcacttaactgaagcgtcttcaatttcacccatatacatatattttgagggtaaattaccataaaatatatacttaatgcatttttaaaagaatacaattaagtcgtatatttaaataaaataataattaaaagtacaacgaactagagagtcaacacttctttaaaaaaaaaaaaaaaaactcttctccttcattcaaaattcaactcgtgcaacgtaatcctgaaacgaatccggttgcatcattaatgaataaagtccgatttgcatcagcaattcacttcccgggaagaagaaaaacagaaaagggaggaaaaaaacagaatgcatagaagggggagggaaaaccaaaaatgttgctgcaaatcctcccaaccaccacttggataatgcatcagcggcaatttctccagcgggaaagggagggggcgaggtccctgaagcagcccctcggctcggagcacgccaagtcttgcccggaggcggcttttcgtttctcctcccgaggtccttctttctttaaggctttgcagtcagtcctattttcaacggattccggtgaaaactcttcattttcctcccggcttcaccctagggcctgaccggcggcgcggccgggggtggaaggcgggctgcgggcggcactggcaccgggctccggagaagcggctacttggccgcccgagcccactccatgtcggtggtcgctcgtgggccgagccgcgccgcgccgcgccgggcagagagcccggtctccccgacacccgcaccgggccgccgcgccggaggctcccgacgccccaggcgggggggtgcttctctgaattcaaaggacacaagcagcagcagctgcggcggcggcgcgggcggctctggcagctacttctcccccttcttcacacccctgggctaagggcatctttccacagcgaggagggaggcggcccggcgcaggaggaggggtcgcttccgcggctgaggagactagaggctgcggcagcccggctcccaaccactcccttcctctcccttccagccctcccccgccttccctctcctctcgcgctcgcgccctgggctcagcgaggctcctccagtcccgccgcacagaggcggaggcttgcggacgagtctggatccaatat

SEQ ID NO: 8660 - RNA, 47 nt, Homo sapiens
  source 1..47: mol_type = other RNA
aacaacaaaatcactagtcttccacacagaactaggccaacatccaa

SEQ ID NO: 8661 - RNA, 54 nt, Homo sapiens
  source 1..54: mol_type = other RNA
aacaacaaaatcactagtcttccacacagcactagaccacagccactctaatct

SEQ ID NO: 8662 - RNA, 55 nt, Homo sapiens
  source 1..55: mol_type = other RNA
aacaacaaaatcactagtcttccagatggggccagccggtccactctgtatccag

SEQ ID NO: 8663 - RNA, 68 nt, Homo sapiens
  source 1..68: mol_type = other RNA
aacaatatcctggtgctgagtgatgactcaggcgactccagcatcagtgattttgttgaagagggcag

SEQ ID NO: 8664 - RNA, 28 nt, Homo sapiens
  source 1..28: mol_type = other RNA
aacatcacagcaagtctgtgctgcttcc

SEQ ID NO: 8665 - RNA, 52 nt, Homo sapiens
  source 1..52: mol_type = other RNA
aacatcactgcaagtcttaacagccgcccgcccaaggcacaggggacagggc

SEQ ID NO: 8666 - RNA, 386 nt, Homo sapiens
  source 1..386: mol_type = other RNA
aaccactttctttgctcatccataaaaagtaactactcatatgttcaagttttttcatgacactgaagtaattcagtcacatcttcaggctctatttattcccttgctatttccatcacatctgcagttacttcctccactaacatcttgaacccctcaaagtcactcatgagggctggaatcaacttcttccaaattcctgttaatgtcaatattctgatctcctcccatgaatcacaaatgttcttaagggcatctagaatggtcaatcctttccaggtttttcaattactttgcacacatccatcaatctatggcagctatagccttataagatgtaattctgaaataataagatttgaaagtcaaaattactccttgatcca

SEQ ID NO: 8667 - RNA, 2401 nt, Homo sapiens
  source 1..2401: mol_type = other RNA
aaccactttctttgctcatccataagaagcaactcccaatttgttcaagttttatcatgagatttcagcaattcagatacatcttcaggatccacttccaattctggttctcttgctatttccaccacacctgcagttactttctctactgaagtcttgaacccctcaaagtcattcatgagggttggaatgaacttcttccaaactcctgttaatgtttatattttgacctcttcctgtgaatcataaatgttccctttggcatctagaattgtgaatccttttcagaagattttaactgacttttcccagatccaccagaagaattacaatctatgtcagctatggtcttacaaaatgtatttcttaaataataaggcttgaagttgaaattatgcttgatccatggactgcagacagatcttgtgttagcaggcatgaaaacaagatcaatttctttgtatatgtctatcagaactcttgggcaaccaagtgtattgtcaatgagcagcaatattctgaaaggaattatttttttccaagcattagatctcagcaatgggcttaaaatattcagtaaaccatgctttcaacagatgtgctgtcatccaggcttttgtccatctataaagcatggtagagtagagttagcataattgtcaagggcaataggattagcagaatggtaaatgatcattggcttcaacttaaagtcaccacctgcattagaccctaacaggagagttcatctccattgaaaatctgtttagtgttgcaacctgcaagaataactttagcctgatctgaataatttgctatagcttctatatcagcacttgctgctttacattgcattttttatgctgtggaaacagcttctttccttaaacttcatgaacctctgctatgtcaaacttttcttctgcaacttcttgacctctctctaccttgatagaattgaagagaagtagggccttgctctggattaggctttggcttaggaggatgttgtggttgatttgatcttttattgacaactaaaactttctccatattagtaataagattgtttcacttttttattatttgtgtgtttactggaatagcccttttaattttattccagaaattttcctttgtattcataacttggctgtttggtgcaggaggctcagttttcagtctactttggcttttggcataccttcctcaaaactaaacttaatcctttctagatttttattcaaagtgagagatgtgcaacgctttctttttcttgaacactttcttgaacacttgagaccattgcagggttattaattggcctaatttcaacattgttatgtctcagggattacagaggcccaaggagagggagatgagggaatggttggttggtatagcaatcagaatatatacaacctttattaattaagtttgctgtataatatgggcaccattaatgggacccaaaaacacaacaataacatcaaagatcacttatcacaaatcactataaaaaataataatgcaaacgtttgaaaattataagaattaccaaaatatgtcacagagacacaaagtgagcatacattggtgggaaaaatgatgctgatgaacttgcttgacacaaagtcaaatttgaagcccagggatcagtggaatttgaaatacaggagtcaaaatccagcctgccacctgttttgtaaagccagtgagctaagaatggattttgtatttttaaaagattgaaaagaagactaattatcttcgttttttgccactataataaaatagcatagactgagtaacttataatgaacaggaatttatttggctcatggttctggaggctgggaagcccaaaatcaagagccacatctggcgagggccttcttactgtatcataacatggaggaaatgaggaagacatcacactgagagggagcaagagacagccaaactcgcttttatgacaaacctactcttgtgataataaatgcactccaatgatagcaacattaatccattcatgaaggcagagccctcattacctaatcactttttaaaggtcccacttctcaacacttttgcaatggggattaaatttccaacacatgaacttcagaggacgcattcaaaccatagtactaatttttcatgacacacaaaattgttttaaattaaatttttactgtccataagtaagtttttgttggagttcagtcatactcatttgcttattatctgtggtcatttctgcactgctacaacacaaataagtagttgctacagagactctacggcctgcaaagtttaaaatatttattatctagatctctgctgagaaagttcactgatccttgctctaggctatatatttagaagtagaatttctatg

SEQ ID NO: 8668 - RNA, 9771 nt, Homo sapiens
  source 1..9771: mol_type = other RNA
aacccagtgggctatggaaatgaccaccttctggaaaagcctctgtgagaaaagaagggaagccaagggaaagcttgtctccaattactctctcatttattctttgcattgtttattggctgtttgaggaatcttgagccaagtcctagtcattatttttgcccatcctcgaacttgaaacagtcttcatggtctggcctgcattgtgctaatctgtattgttaagaatacactacagacagacattgccagcattgagggtggaggtgagactcactttagaaaaggtgatcaggcaatacctaatgaagtgacattccagcagacttaactgaaggaaggcagtgagccttgggatacatgtgagggaaggagggtgtggaattcctggcccagaaacagcaagtgcaaaggctctgaagcaggattgcccttggtacgttcaaaggaaagtgaggcagctgtgtggctgtagaggagtgagaaagggggagagttacaggaggtgatgtaagaagagctttggaggcctagattacctacaggtagggcattgttcgacttttattctgaataaaatgttgggatttgagcaggggagtgacatgatgtggcttagatttagaaaagatcgctctagctactctgtttagaagaggctctaggggtcaagtatggaagcaggaagatcagttgtgaggccattgcaccaatccaagcaagagatgatagcagctttgactactatgttagcagtagagacagtgagaagcggctgaattctggataatccgtatcttgaaggtagagcacaccagattggctgatggatttgatgtgaggtttatgaaaaagagaggaatctagaatgacttcctatttttagcctgtgcaactggaaaaaaaaaggagctgagatgaggaaaccatgggaggaaaatcaagtttgcctttgaacatgttgtatctgataatgcctattggacaagcaaaatgggaatttggaaaagacagcaacgtatgccttaaggggaatttatatgagaaggtacccaagttatactagtttacttgaagggatacattacatatttggttagaccttccattctaaaacaatgagaaactgaaatttataaatggttcttggtgtttgttatgactgtaaacctaataatacttggactcctgcattgtcatgtatttattatgtatattttaccaatctaccctcaaaaagatatgtttacaataaagatgattttgcaatgaaatcattaaacaaacactttttaaaacatgagctatctacaaagacttgtacatgcatgttcatagcaactttattcatacttcccaacttggaaacaatgaaaatacctacacagaaaaaaatgataaattgtggtatacacaaaaaatggaatactggcagggcacagtgcctcacacttgtaatcctagcactttgggaggccgaggagggtggattgctttgagcccaggagttcgagaccagcctggacaacatggcaaaaccccatctgtactaaaaaaaataacaaaaacaaactaggtatggtggcatacgcctgtagagtcttagctactcgggaggctgaggttagaggatggcttgagcctgggagacagaaattgcagtgagccgagatgatgccactgcactccagcctgagttgacagagccagactctgtctcaaaaaaaaaaaaataaaaaataaatttaaaaagcacacacacacacacaaaaccaaaagaaatggactactacacagcaactgaaaagaaagaactgctgagtcatgcaacaacatggacaaatgtcaaaacgttatactgagttttaaaagccaaacaaaaagattatatatgtacgattccattcaaataaagttcaagaatagccaaaaactgaactatggtcatagaaatgaaaaagtagttttagcagagggaaggaatatttgccggaaaggagcacaatggtattttctggggcaatgaaaatgttttgatgattgttaacatggacaaagaaaagtgtcaaaactcactgagttgaacacttaagatatatgcatttcgttgcatgtaaactatctataaaactcacaacaaaatatgagcaaactgaagggttacttcaagccctaccgaaagggtgatatacagaaaaacctaggctgaaagtaattaatctaagcaccgagtttggctctgagtttcccagcaaccaaggcaaaagggaagcaaatgaattctttagatgtactacctaatattaacatgtatcctatgtgaaaaaaattttcctaacactaaattttaaaatacttagataagaagtactagatatgacataatgcttttaacagcactttacaaaagctgaagaaacatttctggctcatttttatttctatcaatcctcaacaaaagtcaagagaataatatcatgccatggttatacaaagacatttctatggggagctaaaggaaggcactcataattttttagagtgtcagctagctgcagggctagaatctagggactcattccagagacatgaaggattctcaaatttcacaggctcatcttcctggatgcctcagcagtgtttctgacagaacttgggttatcagataattaggggttaaataaagtgtaatgttccctggagttgattaaaactagataagttgtagctgttacactagtatttggctaattatgttttaagaaatgttctaagaacttgccgtattcatacccaaatggaaaactattcctgcatcttagtctgaaggcttaatggatatatttatccctgacattctgaaagctcttctctctcctttcatgcttcccagcaggggcataattggcaaatcaagaagggcagtaattttttgtgcaggactcccggacttttaagacatttagcatcctgcctggcctcatctactaaatacaaatggcatcctctagtcctgtgacaatcaaaaatcccccctacattttaaaatgtagtgccaatcccttttgataatcactgggccttaaaagaatgttggtatgttttaaatgtggaaaaccatctggcccaaaaatactatcctagaagaaggtggcattatggaagaagacataatcttggcttgaaacatttgtggatatatatacacttctgtcatatgaaaatcttaatatggcccccacagaacattttacttaaaatgaggctctaactttgaacaacaagcccatcaagatgaaatagcctcaaagtataacccttactagctgaactccatttcatggagttaatccatgaaatgtagctcattcattcaacaaacattaatttccatctgaataatgaagattgtctgcccaaaaaaaccccctttggttttagtgaagtagataccgtatttcctttttttctagctatagttaccagatgtttattccttccttcagtgtcaagaaaacctattatgtgccaaatactgaggacacagtatgagcattttgctaatagtctagaggaggacttcatgaagacaggtgatgaagtatcatgaaaggtatgagaaatagagagctatggtggcatctctgaggaaacttttagtctgagatctgaaagatgagtaagagttaacttttctttgtggagggcagggggtagagtggggacagagacaactgtttcaggcagggctgcaagcttatatgaggccaaaactaaaaggctaggatgcaaacagagaaatggtgagagaagtctagtgagggcaggattttagggcttgaaaaaaggattttctcttaagtgcagcaggacaccatcactgaatcttatattcaaggcaactcactcagacccatggggatgagatctgaggagaaagtcagacaactggttgggaaatataatacccagaataaaaatgacagtgggcaagactagggtggtacgggaaggaatcattcattcattcaataaataagagctgcaactatgtgtcaggtgccctactaacgtattgagcagtctagtggtggaaatctattaaccaaacaagcaacaaggacaaaatataaaatattaattatattcaagtcacaaaaaagagacagatgatgctatgagactgagaaacaagagaagcctttcctaatggttcaggaaaatcttctcttgaggaagggtcacctgaactaaattctgaaggttgagtggaagctaactgaagggtgtcgggtgaggagatggaaataatcttcaggaagtaagaatagcatttaccaagaaacagtaagtcaggcaatgtggtaggacactaggagcaaagaggggtgtgattaagatgaagctggagagtgggttgggactggactgtgcagcattaagtattttggtctttatcctaagaaccaggggaagccaggaaagtgttttaagctggggtgtgacaatgaaaccatcaagttcgtgttttggaaagattgttgtggcttacgggtgggtgtggggaagcagagagaaccactagagcagaacagcaggaagctgctaggaggtggaggacacagtgactgtgaagactgtggggtttctggcttgggtttcttaaatatcctccatttgcgacggggataagaccacactgtttggaaagaagaaggcgtttgcatctgcttagtcactagggcaagaactaggtcattttgtgtcacacattattgtatcgcacgttaaactgttggggaatgggactgaggaaggaggatggtagaagggcgggaacatttactttttaccttcaaaaactgtattatttgatatttttacaatgaaaatataaacacaaatgcaagcttaaaaatcagatacagaagtcccatcaaattattttaagtgggaggaagctaggattatcttgttttataccacttaggtctcaattttgacccctaagcccactcccactcatcctgcttctcagaaccaatctgcaataggtggctggaagattaaaagtgtggaatctacaacccatacatgtgtgctatcaggaaataatttatggcctcaaaattcagtaaatatttcaaaaaaaatcttaaattgtgcttaattttttcagtaagataaaagcctaaaatgatcaatagagagctgagactaaatcatgcttcttcctcaaaaaagcattagccacaaagactcagaaagaagaacgctagcaataactttggacaagatattgaacgaactgatggctgtgtagctttgtggaaatgaagaaatgttctttttctaaatagatacacatgaagtccttatctaggaacctaagtcccaaagagttaaacatgcaaagattagtgtgcaatagagtaggatttatataactctgggcaacaaactctttgctaggtggaagagaagatgtctagtaaactactaaatgttcacttagcagaatcttagagattctgcccatattaattcataaccacattcaaacatagaatctagaccttttctattcaataatccatttgccttttcatttgcattattaatcagcctttaagttttacactcctacttctattattcgagataaacaacatttaggacactgtgtacatttttttttcttgcttctcactaatatgggtgtggaatctaaaaagggatacagggaaagcagaagtgaacaattacacattacaaaacaagatcagtgtttgcttgctaacatatagcagtgataggtttcaaaaaaggcactgtcaacaactgtacagagctgtatgaagcattttcatgcctattattttaattctcagccacctcttaagccagattctccagattctcactcctgcatcacaaaagagcaatcacggccaacaacttgtcaagatttatatagtctcatcttgacttctgtactttttttttaaaccaatgcaataggggcagaatgtgttgcaaagcagcaaactagagctatcttagataaataaataaatacacacacacacacatatgatggggtgcattatggaacttgctatggtttgaatgtttgtgtccccccagaattcatgttgaaatccttacccccaaggtgacagtattaggaaatggggcctttgagaggtgttaggtcatgagagtggaacccccatgaatggaactagtgtccttgtaagaggaacccagagtcatctgtgatataaggtcacagagagaagagagctttctgtgaggaaggaggacctcatcagacactgaatctgcaggtgacttgatcttgaactttccagcttctggaactgtgagaaacaagcttctgttgtttaaagccactcagtctatggtattttgttatagtagcccgaatggactaagacagaactcaagaagagggaaggatagctgagtctccctggaacccactgggagacctggcagtcctctctgcatgtctgattctctgtcatcttctcatccacatccctcaccctctggtttttccatgccacaccaagaccacagtttccagcatggcacaagggttcaaagggcacattattcattcagccctagaatgaataatgagcctgaaatctcagttggagttccaaaattcctgggacatgactaagcttaggtgagaggggtactctctactcaattgactctaaaggaaattatcagaatagtactggaaatgaagtaaaatcatgggtaccatgttagaccaatctggccaaatcaatgattgcaaatgttgtgaagaattatcaaatgttttactaagatgattatacaaaaacctttaaaaattcaaatgaaagaattacatttagtaaagtgtaagtttgggtccctgggagtctggaggttgcctgccatactggactgtgatgaaagcatattcctactgcatgaagccagtgagatgttgggattattattgcagttcagctaccctgatactgcattactactataatcaacaggaaaacaaactaataagctccttccaaaatgcaaaacttcaatagtggcccatggtctacagaatgaagtcctcaagatgacatacatggtcttcttccatgacctaatcccatgcacttcacattctgaaagtctcattgactctcctaaatgttttccaaagaacctagacctgtttttctccctcacactactgatcccaatgtattgtaatgagttgtttgctgtccctctcttttcctagattgtgagtctccacgacggcagtggctttttttcttctttgcagatatatcttcaacacaatatcatatgttgggcatataaaagatgctgaatgaataatgtgctcctaaatgttcacagctccctgaaaattcatgtaattttagagcctggaaagtaggaaaaaccaattctcattttattgaaacatattgtcttctaaaattgttaattcctgaatacccaactcactgacttaaagttctgacaatattactgaaatgaaatgaaaagccatgagtaaataatatccttttgaattagaattggtttctagactaaatcctttaagagttggaagctttaaaaactctgacctcctaaagtcagaattgaaattttttgtcttaggaacttgaggtgaaatgaatcataggtattttattaaatgggggtggattctgaattatttcagagaggaagcaaccttagaaacataaaaatcatcattattaactcaaaatgttccacttgtgaggcgggcattctcagagaagcacagttattttacgttccttggaaactttaggctttgattgcctttccatcaaaaataaaagcattttatattaaacaacatcattcaaggttgaggcttaaatgttactttaatagtatccacaaagaatctggtttagttattaaaatgacttatttttatttaaagaaaaaatctgtgattttactcattgtatatatagaagtgaatttttaaaaaatagtttcttcttttatgtggattctcttaagatttgaagaaccaaactattctttggttttattatacgggaaaaacaacacgcagtctagttaaacaactttgtgatatttatattccattgcacagatatgggttatacaaattagtaacacaagttatttcttaaattccaaacattttctaaaatattattacagcagatgcctaggatattaaaacataaaggtggaaatcattctctaaatagttaaatatatttgacactgaaaatactgcacattttaattagaggaaaattaaaatgtgtgctcaaatgcactaacaaactaggtagcagggcaactaacaactacaaataagtcactgtggtccatttttacgtatgcatatatatgattattctctagataatccgtcttcttgaaaatgctaataaaacataaaaatccagataaatgatttaaagaaattgtaattcttcctactacctaaggtgacatgtactattatctatgacttcatacagttactaattcaaatataaaagacaccacacttcgaaagaaaaaaattttaaggtaatggttttaattgaattaatgagatgaaaagatagtaaagccctgtttgctacttacatgaaagaagactttaaaaaataatcactgcacaaaatgtaaagggtggggttatgctgtgatattaattttcctcaataatgtttttcttgactgttcaagaacaaattaaagtttccacggcaaatttgttttcaaaatgccgaattgcgaaacaattgctggcttcacgtttctgaatacctttaatagtttctctgcgttgcagtttgtaagtttccttgtcatgacacagtcgataaataaagaaacccaggtgatcaatgttttcaatgcgatcagtaataaccatgtgctcatgaatcagataggactgaggcaaataggttccagccttgatgttaataagtaactccagtaggtttctgggtggcataacaatggaagtgttcagagggatcacatagcacttatccaggttaagatctaaataggctgtaagtttcttgttaaagtcatgaacaatgttggcaggatcactatctgcaaactctgggacaggcacactgataaattcaacttcttcttcttcaaagattttaatattttcttcaattgtctggtagagagcagctggggcatctgcagagggctcatttaagatgacatcatctttgatgtactttattccacagtagtacacgtcatctggttgaagtgcaaaatatttgtacaagtatgctcctcctagaataacacctgcaagcataaatgctagtccaaagcacatgcaccaacaccaggctcttctttggccaactggtaccacatcatctgggtccttgcagtccaccgcgacggcgtcgggggggatgatgagcgcctcctcgccgctcttgggctcgtccttcttggcctccttctgggccagagcggagttgaacgtcaccttcaccatggcgcggcctggggcgccctcgaagggcggcggcgggctcggggcgcgggctgcgggctcccggctgcgattgcagcctctacggccgggctccgggagcggctccgggcggctgaagaggttcgggaagctccgcggcggcagaggcggctact

SEQ ID NO: 8669 - RNA, 773 nt, Homo sapiens
  source 1..773: mol_type = other RNA
aacccagtgggctatggaaatgtgtggaagatggcatttctatttctcagtggggctcttacctattactcatcaaccttgtaggcagaattgactgatgcagcctacacagtatttaattacataaatgggacaccacctatgtgcccaacatgggatttgataggaaggatttgaaggggttagagacagggagaccaaataggagtctgcccagccacccagctttcgggtaatgtgcgtctggtcttcagggccaacaatagagagaatgtgaaattaagttgatgatggaaatgaaagaaggaggaattgaaagcttctcaactaagaaaccagaagacaagcaacaagagagcatctcatgaaatcacacaacagggtaactgagtgggtatttcctgtgagcagttataaagttagattgtggacgggtacggtggctcatgccactttgggaggccgaggcgcgccgatcacctgaggtcgggagttggagaccagcctgaccaacatggagaaaccccttctctactgataatacaaaaaaattagccaggcgtggtgacgcatgcctgtaatcccagctactcaggaggctgaggcaggagaatcgcttgaactcaggaggcggaggttgcggtgagctgagatcaggccattgcactccagcctggtcaacaagagtgaaactccgtctcaaaaaaaaaaaaaagattcaagtccagattttgctaaagatgataatttgggggttttcagcatggactatg

SEQ ID NO: 8670 - RNA, 5279 nt, Homo sapiens
  source 1..5279: mol_type = other RNA
aaccttggcccctctccccagaggagcccctggcactcatcctgtgaaccagagccctatcgctgatcagcaccaaatggctgaggatttcctggggctgatagaggggctcagacccttggttctcagacgtgagctgggaagagctggccatggcctgcgccatccctggatttccacactggtggctgcaccctggctaactctttagggctccaatctcaccatgagcttgaggaataagctctacattgcagagcctcctaggtctgctcagtcttatccagatcatatcccctgcagctgctccagaccggcctgtacaatctcactgtatgtccacagccggggctggatagcacctcttcaggcaggagcagtgggtgctgccaggcctgctgctcaggccccctccggacagacgctggggggctgtaaacctgccttaattgaaatatgcaacagggaggcccccaaggagcgatgtctttgctgtgctgccagtcccacctccctgctctgagcgaggggctgtgaatcaagctgcagtcaacttctgacctcgagctactgcgagggaccaagcaatggagtgtttgtgacccaggggtggctcccagttggatggaggtgtcttctttggccatcccactcaaagcccctgtgccctggaaatcactggacatctgggttgaggccacactgaccacaaggcatgtccagtgccttcagtttgtcaagtgctttcacagtcaccatctcgtcggagctccacagcagctggtgaggtaggtgaagactaccagacccattatacagaggaggtagataggctcagagaggcaaacggacttgccaaggtcacacagctgctagctagcagagccaggcacagcctggaaatcactaattcttgggggcagagtagcacaggctttgtggctttggggcaggtactgaactactttgaacctcagtcatctcatttgaaaaatggggataggtgggggcacagtggctcacgcctgtaatcccgggactttgggaggctgaggctgacgaatcacttgaggtcaggagttcagaccagcctgcccaacatggtgaaaccccgtctctactaaaaatacaaaaattagctaggcgtggtgacgcatgcctgtagtcccagttgctctggaggctgaagtgggagaattgcttgaacctggcaggtggaggttgcagtgagccaagatcgccccactgcactccagcctgggtgacagagcgagactccatctcaaaaataaaaaaaataaaaataaaaaaagaaagaaagaaaaagaaaaatggggtaataatacttcctgtctcatcaggttattgtggtgattaaatgagatgctgctataaaaagtattcggcatagaagtagcatagagacctgctcaataaatgtgagcaatataattgtcattattatcccaaggatattcagctgctgtccctgtgctggccatgccccagatgaagccctggtacctctaggctgtaacctcatctttgttcaggacctgctgagatgggctcaggggctgggtgtggagacatcgggacggagtggggaccactgggctcctttccaaggctgcccacctggtgaaggtggccaggagcctgtctacggccctaatttttagccccatggaagtggctgcctacttcctcgcacagatctcaggtctgcttagggccacgccaggactggctgaggctttgccctgaggttttggtcttggtctcagaatcaggctgagaatgggagctgaaaggattgggggtggtccagaccctccaatcaaacccctgcccagcccaggcgatccttcaggctctgtggatgcccagcatcccagcacggaggcctgcgccatgggagcagcttgccattcccctatgtcccaggcaaccctaagatggaagggggtgaggcaggactgtgtatagccgagtaagtctgccttggagtagaaggatggtgggtgcaagtgacgcagggcctggccagactgatgccacccccaggccctgagtcctgcagtctccagaccaccccgactgtgaaccctggcctaaagggacaccactccctttagagcccgcctcctgcaggggagtcccctctaggacatggccctggccatcagccagactccaccacagagttcaggggctagcaaaaggaggatcagacctcccatcagttttacatactttcagatacccccttcaggagccccgcaatgagaacggaggaagggcagtcctgcccacacctcctgggacctaggaggccaatgggcatcttcatgtctaagaggagctctgtgaaagctttggggcctgtggggccagatccttagcatttttaaattttattatgacttcatttgtttaaatatatatatatatatatatatatatatatttatttatagctctatgtgcccaccgcccccggccccctccccggcccctagtttttccccctggctttctgtctagtggctgtgtagggcagaaccgtctgcgtgctcttgtctgacactgtctgggtgctgctgttcctcgtgacccttcgagtctgttcaggggccaaggtagagcctgagtggcggctggtcagtggagagcgccgtgacttgtagggggctggggagggcttgtgggggcctgcatgggcctctgtatgggcaggctcagggggcaagcccacttcttcctcctccacctcctgctcaccgtccccctcctcatcgtcacagcacagagcatggtagagcactttgtcactgaaccgcaccctctcccgtgtccctggggtccgctggggcagctggctcttcaccgtggggccagcaccaaaggcctcctcactggaggagtctggggtctccactcgtggcccattggggatgggcgtgccaccattcatgaggcggtagtcagggccagcccctggccgagtcgactcgggaccatccacggagtccgagggggtagagacgtccaggaaggagcagaactcccagagtggccgtggtccagtcgtccggctccagttcaaagtcgaagtccgaggttagcttatcgatctggctcaccacctccctcagctccttggccacctccttgagctcgcgaaggatgccctcaagctgcccgatgaccatcttcatgcgctgtcgaatccgctcccgctcaccaccactgctggggtcgtcactgggctgcccgaggtccggggcgccccgaatgttcatcgtttaccacgtggccgcaggcctgcccatactccccccagctgggcacacactgcgtctgcctccacggagcccccctcggctgggcagagctccacattttaacggccccccagcccaccctggccctgggcggccctcaaccagcccctgccccctgccacccagcctcctctgcctctgggtggagagtgggacacccagagggagacagagtctagcagagggggtcaaggtgaggacacaggagaggagggggagggaccttgggtcccaggagtggcctccaggtcttgaagtgcctgtgggtgtgcagagctgatctctgcctgagcttgaacacagaggcagggggatgactctgcagggactaagggtaagagatgcccttgggatgggggaaggcagcagggatcccctcacaactcctaggcagttgcaaaggcagaggtctctggatgcaactgacacctgcagagggatggtggccagggtcttccagatgtggaaggggctccggatatgggcagctctggggagggagctggattggaagagggcagccccctgcggagagagcgagcctggcgtcagccctcccaggctgcagcaccagccggcaatgccgctgcctccctcctctcgccagcctgcacccttcctcgctggggatttttttttctttgtggggaggggtggtggaggcagacggtttacagcacagcccctcctcgagggtgggggcaccggccttccctccaagcagcgtcgggggccaagccccaagacggagttggggggcccccaaggctccctagggcgggcttctctctctggacccttcggccccgggcctcagggaggtcctccgagccgtgaccggagacatctgggcggtgggagggggcggggcctccgcgctccagggaagggggcaggaaaaatctttctcaagcctctccaggctcggggtcgggaatgagcgagggtccggcagatttggggctccgaggccacaggtgaccggggcgcggggaggccgaggagacgccgggcaggtcccagcgcgtgagccaaagtcggagggctgggagggcgccgggatcccctcagcccacgcccggcattccccgggctctgcaccgtccgggattcgctctgtccagtccagatcggccgggtccgtgttccgctggggtctgccctgccctaccccgcccggagtgagctggcaccgccgggcgcccgggacgcgctcagcccggacccagaacgtccgtgccccggcacccgcggcgtccggagcggccgcgagggtctgctcagcccagccccgcggtcggccctgggcgagaccgctcccacggctcagttcacgttccgaaaggtccggaatccaccgggtccccgaggaggggcgatgtcagccgcggggacccggtccccgccgggcccagccgagagcgcgcgaagccgggggccccggccgggctgggttcggcggcccgggcgcaggcgggagcagcgccgggcggaggagaggagaggaggcgagaagaggcgaggggaggaggcgcggcgaggggaagggaggggagggggcgagcggcgggccgggccgggccggggcgcactaggctcgcagcctccgctcggctccgctacctcccgtccgttcgctctcggctccccgcctcagcagcccccgggcgccgggtcgccgccggtggggcaaacaggcgccgggtcggggctgggcctcccttcaccgcctcgccctgccctgccccgccgggctcccggggcctgggcccgctccccaagcgccgcggcgccgcgccgcccgcgccccggccgcccccggcccgccccgccgccccccgccggactggccgcccgggcgggcgctggctcccttaaaggccgcccggctcgcttggctccgcttgcctcggcgctgtcagggaaggggcc

SEQ ID NO: 8671 - RNA, 5118 nt, Homo sapiens
  source 1..5118: mol_type = other RNA
aaccttggcccctctccccagaggagcccctggcactcatcctgtgaaccagagccctatcgctgatcagcaccaaatggctgaggatttcctggggctgatagaggggctcagacccttggttctcagacgtgagctgggaagagctggccatggcctgcgccatccctggatttccacactggtggctgcaccctggctaactctttagggctccaatctcaccatgagcttgaggaataagctctacattgcagagcctcctaggtctgctcagtcttatccagatcatatcccctgcagctgctccagaccggcctgtacaatctcactgtatgtccacagccggggctggatagcacctcttcaggcaggagcagtgggtgctgccaggcctgctgctcaggccccctccggacagacgctggggggctgtaaacctgccttaattgaaatatgcaacagggaggcccccaaggagcgatgtctttgctgtgctgccagtcccacctccctgctctgagcgaggggctgtgaatcaagctgcagtcaacttctgacctcgagctactgcgagggaccaagcaatggagtgtttgtgacccaggggtggctcccagttggatggaggtgtcttctttggccatcccactcaaagcccctgtgccctggaaatcactggacatctgggttgaggccacactgaccacaaggcatgtccagtgccttcagtttgtcaagtgctttcacagtcaccatctcgtcggagctccacagcagctggtgaggtaggtgaagactaccagacccattatacagaggaggtagataggctcagagaggcaaacggacttgccaaggtcacacagctgctagctagcagagccaggcacagcctggaaatcactaattcttgggggcagagtagcacaggctttgtggctttggggcaggtactgaactactttgaacctcagtcatctcatttgaaaaatggggataggtgggggcacagtggctcacgcctgtaatcccgggactttgggaggctgaggctgacgaatcacttgaggtcaggagttcagaccagcctgcccaacatggtgaaaccccgtctctactaaaaatacaaaaattagctaggcgtggtgacgcatgcctgtagtcccagttgctctggaggctgaagtgggagaattgcttgaacctggcaggtggaggttgcagtgagccaagatcgccccactgcactccagcctgggtgacagagcgagactccatctcaaaaataaaaaaaataaaaataaaaaaagaaagaaagaaaaagaaaaatggggtaataatacttcctgtctcatcaggttattgtggtgattaaatgagatgctgctataaaaagtattcggcatagaagtagcatagagacctgctcaataaatgtgagcaatataattgtcattattatcccaaggatattcagctgctgtccctgtgctggccatgccccagatgaagccctggtacctctaggctgtaacctcatctttgttcaggacctgctgagatgggctcaggggctgggtgtggagacatcgggacggagtggggaccactgggctcctttccaaggctgcccacctggtgaaggtggccaggagcctgtctacggccctaatttttagccccatggaagtggctgcctacttcctcgcacagatctcaggtctgcttagggccacgccaggactggctgaggctttgccctgaggttttggtcttggtctcagaatcaggctgagaatgggagctgaaaggattgggggtggtccagaccctccaatcaaacccctgcccagcccaggcgatccttcaggctctgtggatgcccagcatcccagcacggaggcctgcgccatgggagcagcttgccattcccctatgtcccaggcaaccctaagatggaagggggtgaggcaggactgtgtatagccgagtaagtctgccttggagtagaaggatggtgggtgcaagtgacgcagggcctggccagactgatgccacccccaggccctgagtcctgcagtctccagaccaccccgactgtgaaccctggcctaaagggacaccactccctttagagcccgcctcctgcaggggagtcccctctaggacatggccctggccatcagccagactccaccacagagttcaggggctagcaaaaggaggatcagacctcccatcagttttacatactttcagatacccccttcaggagccccgcaatgagaacggaggaagggcagtcctgcccacacctcctgggacctaggaggccaatgggcatcttcatgtctaagaggagctctgtgaaagctttggggcctgtggggccagatccttagcatttttaaattttattatgacttcatttgtttaaatatatatatatatatatatatatatatatttatttatagctctatgtgcccaccgcccccggccccctccccggcccctagtttttccccctggctttctgtctagtggctgtgtagggcagaaccgtctgcgtgctcttgtctgacactgtctgggtgctgctgttcctcgtgacccttcgagtctgttcaggggccaaggtagagcctgagtggcggctggtcagtggagagcgccgtgacttgtagggggctggggagggcttgtgggggcctgcatgggcctctgtatgggcaggctcagggggcaagcccacttcttcctcctccacctcctgctcaccgtccccctcctcatcgtcacagcacagagcatggtagagcactttgtcactgaaccgcaccctctcccgtgtccctggggtccgctggggcagctggctcttcaccgtggggccagcaccaaaggcctcctcactggaggagtctggggtctccactcgtggcccattggggatgggcgtgccaccattcatgaggcggtagtcagggccagcccctggccgagtcgactcgggaccatccacggagtccgagggggtagagacgtccaggaaggagcagaactcccagctgtagtggccgtggtccagtcgtccggctccagttcaaagtcgaagtccgaggttagcttatcgatctggctcaccacctccctcagctccttggccacctccttgagctcgcgaaggatgccctcaagctgcccgatgaccatcttcatgcgctgtcgaatccgctcccgctcaccaccactgctggggtcgtcactgggctgcccgaggtccggggcgccccgaatgttcatcgtttaccacgtggccgcaggcctgcccatactccccccagctgggcacacactgcgtctgcctccacggagcccccctcggctgggcagagctccacattttaacggccccccagcccaccctggccctgggcggccctcaaccagcccctgccccctgccacccagcctcctctgcctctgggtggagagtgggacacccagagggagacagagtctagcagagggggtcaaggtgaggacacaggagaggagggggagggaccttgggtcccaggagtggcctccaggtcttgaagtgcctgtgggtgtgcagagctgatctctgcctgagcttgaacacagaggcagggggatgactctgcagggactaagggtaagagatgcccttgggatgggggaaggcagcagggatcccctcacaactcctaggcagttgcaaaggcagaggtctctggatgcaactgacacctgcagagggatggtggccagggtcttccagatgtggaaggggctccggatatgggcagctctggggagggagctggattggaagagggcagcccccgagggtgggggcaccggccttccctccaagcagcgtcgggggccaagccccaagacggagttggggggcccccaaggctccctagggcgggcttctctctctggacccttcggccccgggcctcagggaggtcctccgagccgtgaccggagacatctgggcggtgggagggggcggggcctccgcgctccagggaagggggcaggaaaaatctttctcaagcctctccaggctcggggtcgggaatgagcgagggtccggcagatttggggctccgaggccacaggtgaccggggcgcggggaggccgaggagacgccgggcaggtcccagcgcgtgagccaaagtcggagggctgggagggcgccgggatcccctcagcccacgcccggcattccccgggctctgcaccgtccgggattcgctctgtccagtccagatcggccgggtccgtgttccgctggggtctgccctgccctaccccgcccggagtgagctggcaccgccgggcgcccgggacgcgctcagcccggacccagaacgtccgtgccccggcacccgcggcgtccggagcggccgcgagggtctgctcagcccagccccgcggtcggccctgggcgagaccgctcccacggctcagttcacgttccgaaaggtccggaatccaccgggtccccgaggaggggcgatgtcagccgcggggacccggtccccgccgggcccagccgagagcgcgcgaagccgggggccccggccgggctgggttcggcggcccgggcgcaggcgggagcagcgccgggcggaggagaggagaggaggcgagaagaggcgaggggaggaggcgcggcgaggggaagggaggggagggggcgagcggcgggccgggccgggccggggcgcactaggctcgcagcctccgctcggctccgctacctcccgtccgttcgctctcggctccccgcctcagcagcccccgggcgccgggtcgccgccggtggggcaaacaggcgccgggtcggggctgggcctcccttcaccgcctcgccctgccctgccccgccgggctcccggggcctgggcccgctccccaagcgccgcggcgccgcgccgcccgcgccccggccgcccccggcccgccccgccgccccccgccggactggccgcccgggcgggcgctggctcccttaaaggccgcccggctcgcttggctccgcttgcctcggcgctgtcagggaaggggcc

SEQ ID NO: 8672 - RNA, 3628 nt, Homo sapiens
  source 1..3628: mol_type = other RNA
aaccttggcccctctccccagaggagcccctggcactcatcctgtgaaccagagccctatcgctgatcagcaccaaatggctgaggatttcctggggctgatagaggggctcagacccttggttctcagacgtgagctgggaagagctggccatggcctgcgccatccctggatttccacactggtggctgcaccctggctaactctttagggctccaatctcaccatgagcttgaggaataagctctacattgcagagcctcctaggtctgctcagtcttatccagatcatatcccctgcagctgctccagaccggcctgtacaatctcactgtatgtccacagccggggctggatagcacctcttcaggcaggagcagtgggtgctgccaggcctgctgctcaggccccctccggacagacgctggggggctgtaaacctgccttaattgaaatatgcaacagggaggcccccaaggagcgatgtctttgctgtgctgccagtcccacctccctgctctgagcgaggggctgtgaatcaagctgcagtcaacttctgacctcgagctactgcgagggaccaagcaatggagtgtttgtgacccaggggtggctcccagttggatggaggtgtcttctttggccatcccactcaaagcccctgtgccctggaaatcactggacatctgggttgaggccacactgaccacaaggcatgtccagtgccttcagtttgtcaagtgctttcacagtcaccatctcgtcggagctccacagcagctggtgaggtaggtgaagactaccagacccattatacagaggaggtagataggctcagagaggcaaacggacttgccaaggtcacacagctgctagctagcagagccaggcacagcctggaaatcactaattcttgggggcagagtagcacaggctttgtggctttggggcaggtactgaactactttgaacctcagtcatctcatttgaaaaatggggataggtgggggcacagtggctcacgcctgtaatcccgggactttgggaggctgaggctgacgaatcacttgaggtcaggagttcagaccagcctgcccaacatggtgaaaccccgtctctactaaaaatacaaaaattagctaggcgtggtgacgcatgcctgtagtcccagttgctctggaggctgaagtgggagaattgcttgaacctggcaggtggaggttgcagtgagccaagatcgccccactgcactccagcctgggtgacagagcgagactccatctcaaaaataaaaaaaataaaaataaaaaaagaaagaaagaaaaagaaaaatggggtaataatacttcctgtctcatcaggttattgtggtgattaaatgagatgctgctataaaaagtattcggcatagaagtagcatagagacctgctcaataaatgtgagcaatataattgtcattattatcccaaggatattcagctgctgtccctgtgctggccatgccccagatgaagccctggtacctctaggctgtaacctcatctttgttcaggacctgctgagatgggctcaggggctgggtgtggagacatcgggacggagtggggaccactgggctcctttccaaggctgcccacctggtgaaggtggccaggagcctgtctacggccctaatttttagccccatggaagtggctgcctacttcctcgcacagatctcaggtctgcttagggccacgccaggactggctgaggctttgccctgaggttttggtcttggtctcagaatcaggctgagaatgggagctgaaaggattgggggtggtccagaccctccaatcaaacccctgcccagcccaggcgatccttcaggctctgtggatgcccagcatcccagcacggaggcctgcgccatgggagcagcttgccattcccctatgtcccaggcaaccctaagatggaagggggtgaggcaggactgtgtatagccgagtaagtctgccttggagtagaaggatggtgggtgcaagtgacgcagggcctggccagactgatgccacccccaggccctgagtcctgcagtctccagaccaccccgactgtgaaccctggcctaaagggacaccactccctttagagcccgcctcctgcaggggagtcccctctaggacatggccctggccatcagccagactccaccacagagttcaggggctagcaaaaggaggatcagacctcccatcagttttacatactttcagatacccccttcaggagccccgcaatgagaacggaggaagggcagtcctgcccacacctcctgggacctaggaggccaatgggcatcttcatgtctaagaggagctctgtgaaagctttggggcctgtggggccagatccttagcatttttaaattttattatgacttcatttgtttaaatatatatatatatatatatatatatatatttatttatagctctatgtgcccaccgcccccggccccctccccggcccctagtttttccccctggctttctgtctagtggctgtgtagggcagaaccgtctgcgtgctcttgtctgacactgtctgggtgctgctgttcctcgtgacccttcgagtctgttcaggggccaaggtagagcctgagtggcggctggtcagtggagagcgccgtgacttgtagggggctggggagggcttgtgggggcctgcatgggcctctgtatgggcaggctcagggggcaagcccacttcttcctcctccacctcctgctcaccgtccccctcctcatcgtcacagcacagagcatggtagagcactttgtcactgaaccgcaccctctcccgtgtccctggggtccgctggggcagctggctcttcaccgtggggccagcaccaaaggcctcctcactggaggagtctggggtctccactcgtggcccattggggatgggcgtgccaccattcatgaggcggtagtcagggccagcccctggccgagtcgactcgggaccatccacggagtccgagggggtagagacgtccaggaaggagcagaactcccagctgtctgagaggatatcggctgtcatgaagtccaggtggcccaggtcaaaggggccacccatgcccgccttgtcactgctagaggtgctgctcacagtggccgtggtccagtcgtccggctccagttcaaagtcgaagtccgaggttagcttatcgatctggctcaccacctccctcagctccttggccacctccttgagctcgcgaaggatgccctcaagctgcccgatgaccatcttcatgcgctgtcgaatccgctcccgctcaccaccactgctggggtcgtcactgggcgagggtgggggcaccggccttccctccaagcagcgtcgggggccaagccccaagacggagttggggggcccccaaggctccctagggcgggcttctctctctggacccttcggccccgggcctcagggaggtcctccgagccgtgaccggagacatctgggcggtgggagggggcggggcctccgcgctccagggaagggggcaggaaaaatctttctcaagcctctccaggctcggggtcgggaatgagcgagggtccg

SEQ ID NO: 8673 - RNA, 5209 nt, Homo sapiens
  source 1..5209: mol_type = other RNA
aaccttggcccctctccccagaggagcccctggcactcatcctgtgaaccagagccctatcgctgatcagcaccaaatggctgaggatttcctggggctgatagaggggctcagacccttggttctcagacgtgagctgggaagagctggccatggcctgcgccatccctggatttccacactggtggctgcaccctggctaactctttagggctccaatctcaccatgagcttgaggaataagctctacattgcagagcctcctaggtctgctcagtcttatccagatcatatcccctgcagctgctccagaccggcctgtacaatctcactgtatgtccacagccggggctggatagcacctcttcaggcaggagcagtgggtgctgccaggcctgctgctcaggccccctccggacagacgctggggggctgtaaacctgccttaattgaaatatgcaacagggaggcccccaaggagcgatgtctttgctgtgctgccagtcccacctccctgctctgagcgaggggctgtgaatcaagctgcagtcaacttctgacctcgagctactgcgagggaccaagcaatggagtgtttgtgacccaggggtggctcccagttggatggaggtgtcttctttggccatcccactcaaagcccctgtgccctggaaatcactggacatctgggttgaggccacactgaccacaaggcatgtccagtgccttcagtttgtcaagtgctttcacagtcaccatctcgtcggagctccacagcagctggtgaggtaggtgaagactaccagacccattatacagaggaggtagataggctcagagaggcaaacggacttgccaaggtcacacagctgctagctagcagagccaggcacagcctggaaatcactaattcttgggggcagagtagcacaggctttgtggctttggggcaggtactgaactactttgaacctcagtcatctcatttgaaaaatggggataggtgggggcacagtggctcacgcctgtaatcccgggactttgggaggctgaggctgacgaatcacttgaggtcaggagttcagaccagcctgcccaacatggtgaaaccccgtctctactaaaaatacaaaaattagctaggcgtggtgacgcatgcctgtagtcccagttgctctggaggctgaagtgggagaattgcttgaacctggcaggtggaggttgcagtgagccaagatcgccccactgcactccagcctgggtgacagagcgagactccatctcaaaaataaaaaaaataaaaataaaaaaagaaagaaagaaaaagaaaaatggggtaataatacttcctgtctcatcaggttattgtggtgattaaatgagatgctgctataaaaagtattcggcatagaagtagcatagagacctgctcaataaatgtgagcaatataattgtcattattatcccaaggatattcagctgctgtccctgtgctggccatgccccagatgaagccctggtacctctaggctgtaacctcatctttgttcaggacctgctgagatgggctcaggggctgggtgtggagacatcgggacggagtggggaccactgggctcctttccaaggctgcccacctggtgaaggtggccaggagcctgtctacggccctaatttttagccccatggaagtggctgcctacttcctcgcacagatctcaggtctgcttagggccacgccaggactggctgaggctttgccctgaggttttggtcttggtctcagaatcaggctgagaatgggagctgaaaggattgggggtggtccagaccctccaatcaaacccctgcccagcccaggcgatccttcaggctctgtggatgcccagcatcccagcacggaggcctgcgccatgggagcagcttgccattcccctatgtcccaggcaaccctaagatggaagggggtgaggcaggactgtgtatagccgagtaagtctgccttggagtagaaggatggtgggtgcaagtgacgcagggcctggccagactgatgccacccccaggccctgagtcctgcagtctccagaccaccccgactgtgaaccctggcctaaagggacaccactccctttagagcccgcctcctgcaggggagtcccctctaggacatggccctggccatcagccagactccaccacagagttcaggggctagcaaaaggaggatcagacctcccatcagttttacatactttcagatacccccttcaggagccccgcaatgagaacggaggaagggcagtcctgcccacacctcctgggacctaggaggccaatgggcatcttcatgtctaagaggagctctgtgaaagctttggggcctgtggggccagatccttagcatttttaaattttattatgacttcatttgtttaaatatatatatatatatatatatatatatatttatttatagctctatgtgcccaccgcccccggccccctccccggcccctagtttttccccctggctttctgtctagtggctgtgtagggcagaaccgtctgcgtgctcttgtctgacactgtctgggtgctgctgttcctcgtgacccttcgagtctgttcaggggccaaggtagagcctgagtggcggctggtcagtggagagcgccgtgacttgtagggggctggggagggcttgtgggggcctgcatgggcctctgtatgggcaggctcagggggcaagcccacttcttcctcctccacctcctgctcaccgtccccctcctcatcgtcacagcacagagcatggtagagcactttgtcactgaaccgcaccctctcccgtgtccctggggtccgctggggcagctggctcttcaccgtggggccagcaccaaaggcctcctcactggaggagtctggggtctccactcgtggcccattggggatgggcgtgccaccattcatgaggcggtagtcagggccagcccctggccgagtcgactcgggaccatccacggagtccgagggggtagagacgtccaggaaggagcagaactcccagctgtctgagaggatatcggctgtcatgaagtccaggtggcccaggtcaaaggggccacccatgcccgccttgtcactgctagaggtgctgctcacagtggccgtggtccagtcgtccggctccagttcaaagtcgaagtccgaggttagcttatcgatctggctcaccacctccctcagctccttggccacctccttgagctcgcgaaggatgccctcaagctgcccgatgaccatcttcatgcgctgtcgaatccgctcccgctcaccaccactgctggggtcgtcactgggctgcccgaggtccggggcgccccgaatgttcatcgtttaccacgtggccgcaggcctgcccatactccccccagctgggcacacactgcgtctgcctccacggagcccccctcggctgggcagagctccacattttaacggccccccagcccaccctggccctgggcggccctcaaccagcccctgccccctgccacccagcctcctctgcctctgggtggagagtgggacacccagagggagacagagtctagcagagggggtcaaggtgaggacacaggagaggagggggagggaccttgggtcccaggagtggcctccaggtcttgaagtgcctgtgggtgtgcagagctgatctctgcctgagcttgaacacagaggcagggggatgactctgcagggactaagggtaagagatgcccttgggatgggggaaggcagcagggatcccctcacaactcctaggcagttgcaaaggcagaggtctctggatgcaactgacacctgcagagggatggtggccagggtcttccagatgtggaaggggctccggatatgggcagctctggggagggagctggattggaagagggcagcccccgagggtgggggcaccggccttccctccaagcagcgtcgggggccaagccccaagacggagttggggggcccccaaggctccctagggcgggcttctctctctggacccttcggccccgggcctcagggaggtcctccgagccgtgaccggagacatctgggcggtgggagggggcggggcctccgcgctccagggaagggggcaggaaaaatctttctcaagcctctccaggctcggggtcgggaatgagcgagggtccggcagatttggggctccgaggccacaggtgaccggggcgcggggaggccgaggagacgccgggcaggtcccagcgcgtgagccaaagtcggagggctgggagggcgccgggatcccctcagcccacgcccggcattccccgggctctgcaccgtccgggattcgctctgtccagtccagatcggccgggtccgtgttccgctggggtctgccctgccctaccccgcccggagtgagctggcaccgccgggcgcccgggacgcgctcagcccggacccagaacgtccgtgccccggcacccgcggcgtccggagcggccgcgagggtctgctcagcccagccccgcggtcggccctgggcgagaccgctcccacggctcagttcacgttccgaaaggtccggaatccaccgggtccccgaggaggggcgatgtcagccgcggggacccggtccccgccgggcccagccgagagcgcgcgaagccgggggccccggccgggctgggttcggcggcccgggcgcaggcgggagcagcgccgggcggaggagaggagaggaggcgagaagaggcgaggggaggaggcgcggcgaggggaagggaggggagggggcgagcggcgggccgggccgggccggggcgcactaggctcgcagcctccgctcggctccgctacctcccgtccgttcgctctcggctccccgcctcagcagcccccgggcgccgggtcgccgccggtggggcaaacaggcgccgggtcggggctgggcctcccttcaccgcctcgccctgccctgccccgccgggctcccggggcctgggcccgctccccaagcgccgcggcgccgcgccgcccgcgccccggccgcccccggcccgccccgccgccccccgccggactggccgcccgggcgggcgctggctcccttaaaggccgcccggctcgcttggctccgcttgcctcggcgctgtcagggaaggggcc

SEQ ID NO: 8674 - RNA, 5374 nt, Homo sapiens
  source 1..5374: mol_type = other RNA
aaccttggcccctctccccagaggagcccctggcactcatcctgtgaaccagagccctatcgctgatcagcaccaaatggctgaggatttcctggggctgatagaggggctcagacccttggttctcagacgtgagctgggaagagctggccatggcctgcgccatccctggatttccacactggtggctgcaccctggctaactctttagggctccaatctcaccatgagcttgaggaataagctctacattgcagagcctcctaggtctgctcagtcttatccagatcatatcccctgcagctgctccagaccggcctgtacaatctcactgtatgtccacagccggggctggatagcacctcttcaggcaggagcagtgggtgctgccaggcctgctgctcaggccccctccggacagacgctggggggctgtaaacctgccttaattgaaatatgcaacagggaggcccccaaggagcgatgtctttgctgtgctgccagtcccacctccctgctctgagcgaggggctgtgaatcaagctgcagtcaacttctgacctcgagctactgcgagggaccaagcaatggagtgtttgtgacccaggggtggctcccagttggatggaggtgtcttctttggccatcccactcaaagcccctgtgccctggaaatcactggacatctgggttgaggccacactgaccacaaggcatgtccagtgccttcagtttgtcaagtgctttcacagtcaccatctcgtcggagctccacagcagctggtgaggtaggtgaagactaccagacccattatacagaggaggtagataggctcagagaggcaaacggacttgccaaggtcacacagctgctagctagcagagccaggcacagcctggaaatcactaattcttgggggcagagtagcacaggctttgtggctttggggcaggtactgaactactttgaacctcagtcatctcatttgaaaaatggggataggtgggggcacagtggctcacgcctgtaatcccgggactttgggaggctgaggctgacgaatcacttgaggtcaggagttcagaccagcctgcccaacatggtgaaaccccgtctctactaaaaatacaaaaattagctaggcgtggtgacgcatgcctgtagtcccagttgctctggaggctgaagtgggagaattgcttgaacctggcaggtggaggttgcagtgagccaagatcgccccactgcactccagcctgggtgacagagcgagactccatctcaaaaataaaaaaaataaaaataaaaaaagaaagaaagaaaaagaaaaatggggtaataatacttcctgtctcatcaggttattgtggtgattaaatgagatgctgctataaaaagtattcggcatagaagtagcatagagacctgctcaataaatgtgagcaatataattgtcattattatcccaaggatattcagctgctgtccctgtgctggccatgccccagatgaagccctggtacctctaggctgtaacctcatctttgttcaggacctgctgagatgggctcaggggctgggtgtggagacatcgggacggagtggggaccactgggctcctttccaaggctgcccacctggtgaaggtggccaggagcctgtctacggccctaatttttagccccatggaagtggctgcctacttcctcgcacagatctcaggtctgcttagggccacgccaggactggctgaggctttgccctgaggttttggtcttggtctcagaatcaggctgagaatgggagctgaaaggattgggggtggtccagaccctccaatcaaacccctgcccagcccaggcgatccttcaggctctgtggatgcccagcatcccagcacggaggcctgcgccatgggagcagcttgccattcccctatgtcccaggcaaccctaagatggaagggggtgaggcaggactgtgtatagccgagtaagtctgccttggagtagaaggatggtgggtgcaagtgacgcagggcctggccagactgatgccacccccaggccctgagtcctgcagtctccagaccaccccgactgtgaaccctggcctaaagggacaccactccctttagagcccgcctcctgcaggggagtcccctctaggacatggccctggccatcagccagactccaccacagagttcaggggctagcaaaaggaggatcagacctcccatcagttttacatactttcagatacccccttcaggagccccgcaatgagaacggaggaagggcagtcctgcccacacctcctgggacctaggaggccaatgggcatcttcatgtctaagaggagctctgtgaaagctttggggcctgtggggccagatccttagcatttttaaattttattatgacttcatttgtttaaatatatatatatatatatatatatatatatttatttatagctctatgtgcccaccgcccccggccccctccccggcccctagtttttccccctggctttctgtctagtggctgtgtagggcagaaccgtctgcgtgctcttgtctgacactgtctgggtgctgctgttcctcgtgacccttcgagtctgttcaggggccaaggtagagcctgagtggcggctggtcagtggagagcgccgtgacttgtagggggctggggagggcttgtgggggcctgcatgggcctctgtatgggcaggctcagggggcaagcccacttcttcctcctccacctcctgctcaccgtccccctcctcatcgtcacagcacagagcatggtagagcactttgtcactgaaccgcaccctctcccgtgtccctggggtccgctggggcagctggctcttcaccgtggggccagcaccaaaggcctcctcactggaggagtctggggtctccactcgtggcccattggggatgggcgtgccaccattcatgaggcggtagtcagggccagcccctggccgagtcgactcgggaccatccacggagtccgagggggtagagacgtccaggaaggagcagaactcccagctgtctgagaggatatcggctgtcatgaagtccaggtggcccaggtcaaaggggccacccatgcccgccttgtcactgctagaggtgctgctcacagtggccgtggtccagtcgtccggctccagttcaaagtcgaagtccgaggttagcttatcgatctggctcaccacctccctcagctccttggccacctccttgagctcgcgaaggatgccctcaagctgcccgatgaccatcttcatgcgctgtcgaatccgctcccgctcaccaccactgctggggtcgtcactgggctgcccgaggtccggggcgccccgaatgttcatcgtttaccacgtggccgcaggcctgcccatactccccccagctgggcacacactgcgtctgcctccacggagcccccctcggctgggcagagctccacattttaacggccccccagcccaccctggccctgggcggccctcaaccagcccctgccccctgccacccagcctcctctgcctctgggtggagagtgggacacccagagggagacagagtctagcagagggggtcaaggtgaggacacaggagaggagggggagggaccttgggtcccaggagtggcctccaggtcttgaagtgcctgtgggtgtgcagagctgatctctgcctgagcttgaacacagaggcagggggatgactctgcagggactaagggtaagagatgcccttgggatgggggaaggcagcagggatcccctcacaactcctaggcagttgcaaaggcagaggtctctggatgcaactgacacctgcagagggatggtggccagggtcttccagatgtggaaggggctccggatatgggcagctctggggagggagctggattggaagagggcagccccctgcggagagagcgagcctggcgtcagccctcccaggctgcagcaccagccggcaatgccgctgcctccctcctctcgccagcctgcacccttcctcgctggggatttttttttctttgtggggaggggtggtggaggcagacggtttacagcacagcccctcctcgagggtgggggcaccggccttccctccaagcagcgtcgggggccaagccccaagacggagttggggggcccccaaggctccctagggcgggcttctctctctggacccttcggccccgggcctcagggaggtcctccgagccgtgaccggagacatctgggcggtgggagggggcggggcctccgcgctccagggaagggggcaggaaaaatctttctcaagcctctccaggctcggggtcgggaatgagcgagggtccggcagatttggggctccgaggccacaggtgaccggggcgcggggaggccgaggagacgccgggcaggtcccagcgcgtgagccaaagtcggagggctgggagggcgccgggatcccctcagcccacgcccggcattccccgggctctgcaccgtccgggattcgctctgtccagtccagatcggccgggtccgtgttccgctggggtctgccctgccctaccccgcccggagtgagctggcaccgccgggcgcccgggacgcgctcagcccggacccagaacgtccgtgccccggcacccgcggcgtccggagcggccgcgagggtctgctcagcccagccccgcggtcggccctgggcgagaccgctcccacggctcagttcacgttccgaaaggtccggaatccaccgggtccccgaggaggggcgatgtcagccgcggggacccggtccccgccgggcccagccgagagcgcgcgaagccgggggccccggccgggctgggttcggcggcccgggcgcaggcgggagcagcgccgggcggaggagaggagaggaggcgagaagaggcgaggggaggaggcgcggcgaggggaagggaggggagggggcgagcggcgggccgggccgggccggggcgcactaggctcgcagcctccgctcggctccgctacctcccgtccgttcgctctcggctccccgcctcagcagcccccgggcgccgggtcgccgccggtggggcaaacaggcgccgggtcggggctgggcctcccttcaccgcctcgccctgccctgccccgccgggctcccggggcctgggcccgctccccaagcgccgcggcgccgcgccgcccgcgccccggccgcccccggcccgccccgccgccccccgccggactggccgcccgggcgggcgctggctcccttaaaggccgcccggctcgcttggctccgcttgcctcggcgctgtcagggaaggggcc

SEQ ID NO: 8675 - RNA, 51 nt, Homo sapiens
  source 1..51: mol_type = other RNA
aaccttggcccctctccccagcgccgcccggccacgaggcccgcgcgcggg

SEQ ID NO: 8676 - RNA, 1958 nt, Homo sapiens
  source 1..1958: mol_type = other RNA
aaccttggcccctctccccaggacgtcagggggtggggcccataaataaatggaagctggttttggtttttggtagcttgtctcagattccctctttggccttctgccaccacactctccaccctgtggtcttgttccgtccccgcccccatctagccccacctttgagaactgggggcagagcgaggctccaggttctgggctctccctgggagttggggtgatgaccatgggcagaggggatgggactgaagctgggcgctcaagagtcggggaagtagagggaggcagagtcaggtcacaggccccaagaaccccaggtggaaggagggctgagtggcagcgcctttatttgtgggggccttcaaggtagggtcgtggggggcagcggggaggaagagccgagaaactgtgtgaccggggcctcaggtggtgggcattgggggctcctcttgcagatgcccattggcatcaccggtgcagccattggtggcagcgggtaccggtcctttcttgttcaacatagggtaggtggcagccacgggtccaactcgcttgaggctgggccctgggcgctccattttgtgttccaggagcatgtggttctgtggcgggagccccacgcaggccctgaggatgttctcgatgcagctgcgctggcggaaaagcgcattgaccaccgggctgccgggcggcactagtggcgccttgaagaggaagctgagcagggacagcacggggtggaaggtctgcggctcggggtccatgtcagtgcagaagctcacgcgctggcacagctcggtcagcagcgctaggtccagcatgatgggtgcggccagcagcgagtcctcacacgtgttgtgcagcaccagtgtgttggttccgcccagcatcagctccgaggtatactcatccagcgcgcgcttgctgtcacccacgtacggcacatacttgatgaccacgcagtggtcaggctcttcgccgggcgtatagagcactgggttgctctgcaccatgtcgtccaccacgttgctcttggacacctccttagagcggaactgcaatggcgccgataggttctccccatcgttgttgcccaggtggttgtaactcacgatggacatggtcttgaggccggagccaatgaggaagtccacaagcacggacttgactttggtctggcctgacttgaagtcatctccgcccacaaaaacccggtgctgccacgcgagctcaagagctccgggcaccagggtgttctgcggagacccattgaggaaggcacagccctccaggatgctggccacggcgaagagcgtggagggcgacacctccagaccgagctcaatggtgcgcagcaggttctcggctgtgtcgttgaggcctggaatcacctcacagaagcgctccgtgttcgccgtccacagcactatgactttgtccagccccgcgctagaccggaagtctcggatgtccctgcggatctgctccagcatcgaacacgaggtcgttgggcgccaccatgggcagcaccgcgctgaagggtacgaacacctcctggccctcggcgtccaggcccaggctcacggtgcccgcctgagtcagcgagccgtagtagttggcctccttgcggccgctgcgcgtgggccaggacaaacgcagtcgattggccagcaccgcggcggtgagtgtggagccgttgttcccgccccagccgacaagcatgaccccgagccggggcacctgccgggcggtccggaaggtgaagcgcgtggacgtggggtgcaccttgagaacgccaccctcgcggctgacgcgcgtcgtccggtactcgtattgcgcctcgatggcctcggggccgtagaccacgtccgggctctcgacgaagaactgggcggcggcctccatcgcggcgggcggcgcagagtcgactcaggcagcggcggcggacagcgcgg

SEQ ID NO: 8677 - RNA, 2024 nt, Homo sapiens
  source 1..2024: mol_type = other RNA
aaccttggcccctctccccaggacgtcagggggtggggcccataaataaatggaagctggttttggtttttggtagcttgtctcagattccctctttggccttctgccaccacactctccaccctgtggtcttgttccgtccccgcccccatctagccccacctttgagaactgggggcagagcgaggctccaggttctgggctctccctgggagttggggtgatgaccatgggcagaggggatgggactgaagctgggcgctcaagagtcggggaagtagagggaggcagagtcaggtcacaggccccaagaaccccaggtggaaggagggctgagtggcagcgcctttatttgtgggggccttcaaggtagggtcgtggggggcagcggggaggaagagccgagaaactgtgtgaccggggcctcaggtggtgggcattgggggctcctcttgcagatgcccattggcatcaccggtgcagccattggtggcagcgggtaccggtcctttcttgttcaacatagggtaggtggcagccacgggtccaactcgcttgaggctgggccctgggcgctccattttgtgttccaggagcatgtggttctgtggcgggagccccacgcaggccctgaggatgttctcgatgcagctgcgctggcggaaaagcgcattgaccaccgggctgccgggcggcactagtggcgccttgaagaggaagctgagcagggacagcacggggtggaaggtctgcggctcggggtccatgtcagtgcagaagctcacgcgctggcacagctcggtcagcagcgctaggtccagcatgatgggtgcggccagcagcgagtcctcacacgtgttgtgcagcaccagtgtgttggttccgcccagcatcagctccgaggtatactcatccagcgcgcgcttgctgtcacccacgtacggcacatacttgatgaccacgcagtggtcaggctcttcgccgggcgtatagagcactgggttgctctgcaccatgtcgtccaccacgttgctcttggacacctccttagagcggaactgcaatggcgccgataggttctccccatcgttgttgcccaggtggttgtaactcacgatggacatggtcttgaggccggagccaatgaggaagtccacaagcacggacttgactttggtctggcctgacttgaagtcatctccgcccacaaaaacccggtgctgccacgcgagctcaagagctccgggcaccagggtgttctgcggagacccattgaggaaggcacagccctccaggatgctggccacggcgaagagcgtggagggcgacacctccagaccgagctcaatggtgcgcagcaggttctcggctgtgtcgttgaggcctggaatcacctcacagaagcgctccgtgttcgccgtccacagcactatgactttgtccagccccgcgctagaccggaagtctcggatgtccctgcggatctgctccagctgctgcgcacgcgagcctgggatgaggttgtccgcgcgcgcgctctggttggccgcgatgaattcggggatgtaaacagaaggccggggccgcagggcctccatgtgcggccacagttgctcctgcagcccccagtccagcaccttcgcgcgccgcatcgcctcggccaggttcagcgacgagatgtcccagccatcgaacacgaggtcgttgggcgccaccatgggcagcaccgcgctgaagggtacgaacacctcctggccctcggcgtccaggcccaggctcacggtgcccgcctgagtcagcgagccgtagtagttggcctcctgggggtcagcagacacggcgaggtgacgggtgggagtggtgaaagggccgcgacccggcctgggccccacctagactctcaagccccgccccactttcgggcatttttcagttccaggctcacagccaggacggaagccgctgcccccaggcccctcccctgagacctccggcaccttaagctccgcccctgtaagactccc

SEQ ID NO: 8678 - RNA, 1990 nt, Homo sapiens
  source 1..1990: mol_type = other RNA
aaccttggcccctctccccaggacgtcagggggtggggcccataaataaatggaagctggttttggtttttggtagcttgtctcagattccctctttggccttctgccaccacactctccaccctgtggtcttgttccgtccccgcccccatctagccccacctttgagaactgggggcagagcgaggctccaggttctgggctctccctgggagttggggtgatgaccatgggcagaggggatgggactgaagctgggcgctcaagagtcggggaagtagagggaggcagagtcaggtcacaggccccaagaaccccaggtggaaggagggctgagtggcagcgcctttatttgtgggggccttcaaggtagggtcgtggggggcagcggggaggaagagccgagaaactgtgtgaccggggcctcaggtggtgggcattgggggctcctcttgcagatgcccattggcatcaccggtgcagccattggtggcagcgggtaccggtcctttcttgttcaacatagggtaggtggcagccacgggtccaactcgcttgaggctgggccctgggcgctccattttgtgttccaggagcatgtggttctgtggcgggagccccacgcaggccctgaggatgttctcgatgcagctgcgctggcggaaaagcgcattgaccaccgggctgccgggcggcactagtggcgccttgaagaggaagctgagcagggacagcacggggtggaaggtctgcggctcggggtccatgtcagtgcagaagctcacgcgctggcacagctcggtcagcagcgctaggtccagcatgatgggtgcggccagcagcgagtcctcacacgtgttgtgcagcaccagtgtgttggttccgcccagcatcagctccgaggtatactcatccagcgcgcgcttgctgtcacccacgtacggcacatacttgatgaccacgcagtggtcaggctcttcgccgggcgtatagagcactgggttgctctgcaccatgtcgtccaccacgttgctcttggacacctccttagagcggaactgcaatggcgccgataggttctccccatcgttgttgcccaggtggttgtaactcacgatggacatggtcttgaggccggagccaatgaggaagtccacaagcacggacttgactttggtctggcctgacttgaagtcatctccgcccacaaaaacccggtgctgccacgcgagctcaagagctccgggcaccagggtgttctgcggagacccattgaggaaggcacagccctccaggatgctggccacggcgaagagcgtggagggcgacacctccagaccgagctcaatggtgcgcagcaggttctcggctgtgtcgttgaggcctggaatcacctcacagaagcgctccgtgttcgccgtccacagcactatgactttgtccagccccgcgctagaccggaagtctcggatgtccctgcggatctgctccagctgctgcgcacgcgagcctgggatgaggttgtccgcgcgcgcgctctggttggccgcgatgaattcggggatgtaaacagaaggccggggccgcagggcctccatgtgcggccacagttgctcctgcagcccccagtccagcaccttcgcgcgccgcatcgcctcggccaggttcagcgacgagatgtcccagccatcgaacacgaggtcgttgggcgccaccatgggcagcaccgcgctgaagggtacgaacacctcctggccctcggcgtccaggcccaggctcacggtgcccgcctgagtcagcgagccgtagtagttggcctccttgagaacgccaccctcgcggctgacgcgcgtcgtccggtactcgtattgcgcctcgatggcctcggggccgtagaccacgtccgggctctcgacgaagaactgggcggcggcctccatcgcggcgggcggcgcagagtcgactcaggcagcggcggcggacagcgcgg

SEQ ID NO: 8679 - RNA, 2152 nt, Homo sapiens
  source 1..2152: mol_type = other RNA
aaccttggcccctctccccaggacgtcagggggtggggcccataaataaatggaagctggttttggtttttggtagcttgtctcagattccctctttggccttctgccaccacactctccaccctgtggtcttgttccgtccccgcccccatctagccccacctttgagaactgggggcagagcgaggctccaggttctgggctctccctgggagttggggtgatgaccatgggcagaggggatgggactgaagctgggcgctcaagagtcggggaagtagagggaggcagagtcaggtcacaggccccaagaaccccaggtggaaggagggctgagtggcagcgcctttatttgtgggggccttcaaggtagggtcgtggggggcagcggggaggaagagccgagaaactgtgtgaccggggcctcaggtggtgggcattgggggctcctcttgcagatgcccattggcatcaccggtgcagccattggtggcagcgggtaccggtcctttcttgttcaacatagggtaggtggcagccacgggtccaactcgcttgaggctgggccctgggcgctccattttgtgttccaggagcatgtggttctgtggcgggagccccacgcaggccctgaggatgttctcgatgcagctgcgctggcggaaaagcgcattgaccaccgggctgccgggcggcactagtggcgccttgaagaggaagctgagcagggacagcacggggtggaaggtctgcggctcggggtccatgtcagtgcagaagctcacgcgctggcacagctcggtcagcagcgctaggtccagcatgatgggtgcggccagcagcgagtcctcacacgtgttgtgcagcaccagtgtgttggttccgcccagcatcagctccgaggtatactcatccagcgcgcgcttgctgtcacccacgtacggcacatacttgatgaccacgcagtggtcaggctcttcgccgggcgtatagagcactgggttgctctgcaccatgtcgtccaccacgttgctcttggacacctccttagagcggaactgcaatggcgccgataggttctccccatcgttgttgcccaggtggttgtaactcacgatggacatggtcttgaggccggagccaatgaggaagtccacaagcacggacttgactttggtctggcctgacttgaagtcatctccgcccacaaaaacccggtgctgccacgcgagctcaagagctccgggcaccagggtgttctgcggagacccattgaggaaggcacagccctccaggatgctggccacggcgaagagcgtggagggcgacacctccagaccgagctcaatggtgcgcagcaggttctcggctgtgtcgttgaggcctggaatcacctcacagaagcgctccgtgttcgccgtccacagcactatgactttgtccagccccgcgctagaccggaagtctcggatgtccctgcggatctgctccagctgctgcgcacgcgagcctgggatgaggttgtccgcgcgcgcgctctggttggccgcgatgaattcggggatgtaaacagaaggccggggccgcagggcctccatgtgcggccacagttgctcctgcagcccccagtccagcaccttcgcgcgccgcatcgcctcggccaggttcagcgacgagatgtcccagccatcgaacacgaggtcgttgggcgccaccatgggcagcaccgcgctgaagggtacgaacacctcctggccctcggcgtccaggcccaggctcacggtgcccgcctgagtcagcgagccgtagtagttggcctccttgcggccgctgcgcgtgggccaggacaaacgcagtcgattggccagcaccgcggcggtgagtgtggagccgttgttcccgccccagccgacaagcatgaccccgagccggggcacctgccgggcggtccggaaggtgaagcgcgtggacgtggggtgcaccttgagaacgccaccctcgcggctgacgcgcgtcgtccggtactcgtattgcgcctcgatggcctcggggccgtagaccacgtccgggctctcgacgaagaactgggcggcggcctccatcgcggcgggcggcgcagagtcgactcaggcagcggcggcggacagcgcgg

SEQ ID NO: 8680 - RNA, 1961 nt, Homo sapiens
  source 1..1961: mol_type = other RNA
aaccttggcccctctccccaggacgtcagggggtggggcccataaataaatggaagctggttttggtttttggtagcttgtctcagattccctctttggccttctgccaccacactctccaccctgtggtcttgttccgtccccgcccccatctagccccacctttgagaactgggggcagagcgaggctccaggttctgggctctccctgggagttggggtgatgaccatgggcagaggggatgggactgaagctgggcgctcaagagtcggggaagtagagggaggcagagtcaggtcacaggccccaagaaccccaggtggaaggagggctgagtggcagcgcctttatttgtgggggccttcaaggtagggtcgtggggggcagcggggaggaagagccgagaaactgtgtgaccggggcctcaggtggtgggcattgggggctcctcttgcagatgcccattggcatcaccggtgcagccattggtggcagcgggtaccggtcctttcttgttcaacatagggtaggtggcagccacgggtccaactcgcttgaggctgggccctgggcgctccattttgtgttccaggagcatgtggttctgtggcgggagccccacgcaggccctgaggatgttctcgatgcagctgcgctggcggaaaagcgcattgaccaccgggctgccgggcggcactagtggcgccttgaagaggaagctgagcagggacagcacggggtggaaggtctgcggctcggggtccatgtcagtgcagaagctcacgcgctggcacagctcggtcagcagcgctaggtccagcatgatgggtgcggccagcagcgagtcctcacacgtgttgtgcagcaccagtgtgttggttccgcccagcatcagctccgaggtatactcatccagcgcgcgcttgctgtcacccacgtacggcacatacttgatgaccacgcagtggtcaggctcttcgccgggcgtatagagcactgggttgctctgcaccatgtcgtccaccacgttgctcttggacacctccttagagcggaactgcaatggcgccgataggttctccccatcgttgttgcccaggtggttgtaactcacgatggacatggtcttgaggccggagccaatgaggaagtccacaagcacggacttgactttggtctggcctgacttgaagtcatctccgcccacaaaaacccggtgctgccacgcgagctcaagagctccgggcaccagggtgttctgcggagacccattgaggaaggcacagccctccaggatgctggccacggcgaagagcgtggagggcgacacctccagaccgagctcaatggtgcgcagcaggttctcggctgtgtcgttgaggcctggaatcacctcacagaagcgctccgtgttcgccgtccacagcactatgactttgtccagccccgcgctagaccggaagtctcggatgtccctgcggatctgctccagctgctgcgcacgcgagcctgggatgaggttgtccgcgcgcgcgctctggttggccgcgatgaattcggggatgtaaacagaaggccggggccgcagggcctccatgtgcggccacagttgctcctgcagcccccagtccagcaccttcgcgcgccgcatcgcctcggccaggttcagcgacgagatgtcccagccttgagaacgccaccctcgcggctgacgcgcgtcgtccggtactcgtattgcgcctcgatggcctcggggccgtagaccacgtccgggctctcgacgaagaactgggcggcggcctccatcgcggcgggctgggggcccggggtgagcagggggtcagcggggactctaagcggccggggccaagccagcctgggtccccacggaggccgtccctgccccgaaccgcactcaccggcgcagagtcgactcaggcagcggcggcggacagcgcgg

SEQ ID NO: 8681 - RNA, 1738 nt, Homo sapiens
  source 1..1738: mol_type = other RNA
aaccttggcccctctccccagggactgcaggcccgccttccctcccggacgaggttgcgcaatcccgcaggcgatcatcagctcttctctgggggccatctttatcccggggtgggactggaacgggctgtgtgtacctcttcccaactccacattctgggatgttctgttggggtttcagggcagccagggtgggggcacagacaccacagaaaggggcaagtccacccgacacgcagcccccagcgcagcactgcccaggaccgccatgaagggcggcaagcccccagccacagatgtgcgtttcctggcctgcaggtgtctgaagaaacgcgaggccacacccagcgcagccactgctggcctccagctgaggaagctctgagagtggctcgcaggccccacgatccctggccagacccaataacagagtctgtgtccccaaccccagcatggccggctgaatccttcctgtcgcaggccccacgctccctggctggacccaataaccaagtctgtgcccccaaccccagcatggccggctgaatcctttcctgtctcacgaacacacccataaggcaagcggggctcccgacacagcctgaatttccagcttccagaacacactgtctctcctcccacgcgctgtgctgtgatttaagggactcactgaaggcaggcaccgcgtgctcctaagggtgcagcgtcttaactctgctgcgtgtggcgcttacgctcgagcccagcacgcagccgtgctccttacccccctcatagtagtgctgcgtggactcctcgaaggaccggtcgtagctctgctccgtgtaggatgactgctggtaggcgtaatcgccatggccgtcggggtagtactgctggcccatgggctccgcggcgccctggctgtggctgtactgctcgccatagtactcctcctggcccaggtactgctgggaagagccttgctgggagggccggtagggcgccatgggccgctgccccatcatgctgctcccctggctgccctgccccatcatggcgatggacgactggccctggtagtgctggctgccgccctgcgccgagctgtagtgcgacgtggccgcctgctgctgcatcatggagactgggttggactgcatgttgatgttggtccgagacacgtagttgccgatggtgccttgcccctgcatggggacgccctgcgaggcgggtcccgcgtggctgtagccgggcccagagatgctcatggaggtggtgggcagcgtgttaggcgccgtctgctgcatggacacgtggctcggcccgttgccaatctggccctgcaggagggaggagggtggcaggcccgtgctgatggcgtcactcaggctgccctgagagtgcaggccctggctggagccgctctgagtcagggctccagggcccaggttcatgttctgcgtgggcggggcaggaagcagggactgcatgttctggttggagtctgcgatcgtggccaggtataccaggttccggtgcaggatctgctggtactgcgtgcactcggccgtcttgcccttgctctggtactccaggatgcactggatcaggtggtggttctcgtccagcatcttctggatggtttgctgcgtaacctcccctttgcctcttggccgggcagacgcgaaggccacggacatggtggcggcgcggggctcagcccgtggtcatcgaggtggatactccggctgcgctg

SEQ ID NO: 8682 - RNA, 3240 nt, Homo sapiens
  source 1..3240: mol_type = other RNA
aaccttggcccctctccccaggtggaatcaaggctaatcgcctgccctgatggccctatcgggtgagtctggaatcatcctgatcatttttctggaggctgcatgtaccttcttcctctgcttcctcccctgttccagtgggggccagtagaatctggggctctagggaggggtccgtgtgggagctccaggcaggtctttctgttttggtttctccaaagtctaaaccctggggagcttcaaacatccaccccctccagcgactgatgtgcggggtccggctggcctgtgtcctgagtatctgggtccttagcccctgggggaccctcaggcgaggccacggttgacaaccccctgcctgatgtgttgatcggtcagtgagctcctggtctgcacacgggccggccacatcctggacttccccgtgaattctccagcagggcagccgtgtggtgggatgctgtcaccgctgtctgctttgtctcatcgtctgttccatttctcttgcttcttacttcaactgtggattcttacagggcagaactgcacgagtcatctttgcaccttgtctagtgtccagagccagttcttgtggggaagctgagtgctctgtaactcccgtgtctcagctcccttgcgtggcccctagaggcagacgtgggaggaatgccgcagcctcggagaaccaggtctggcattcttggtgctggtcccagggtcccgaggcctgctttccacagtcacgctgtagagacggctccttgtggagacaccttctgtgtgcaggcacgaggtttctcctctgccccaggcttcggtgcggagtgtctggggggacagagccaccagatgtgaacgctgtgctagtcgccctctctggtctctcccttggcgtggccagactccccggtgcatctggacatcgtggcgggcaactgccatttacagacacgggaggacgttttgcatgacccgccttctgtgtgttttcccactctttgcaaacccattgcttttcagctcggagagttgctttccagttgtgccagctccgtggctgaggaggcggtttctttcccgttgtgccggctccgtggccgaggaggcggtttctttccggttctgccggctccgtggccgaggaggcggtttctttcgggttctgccggctccgtggccgaggaggcggtttctttcgggttctgccggctccgtggccgaggaggcggtttctttcgggttctgccggctccgtggccgaggaggcggtttctttcgggttctgccggctccgtggctgaggaggcggtttctttccggccgcgctggctccgtggctgaggaggcggtttctttcgggttctgccggctccgtggctgaggaggcggtttctttcgggttctgccggctccgtggccgaggaggcggtttctttcgggttctgccggctccgtggctgaggaggcggtttctttccggccgcgctggctccgtggccgaggaggcggtttctttcgggttctgccggctccgtggctgaggaggcggtttctttccggccgcgctggctccgtggctgaggaggcggtttctttccggccgcgccggctccgtggctgaggaggcggtttcttttgggttctgccggctccgtggctgaggaggcggtttctttccggccgcgccggctccatggctgaggaggcggtttctttccggccgcgccggctccatggctgaggaggcggtttctttccggccgcgccggctccatggctgaggaggcggtttctttcgggttctgccggctccgtggctgaggaggcggtttctttctggttctgccggctccgtggctgaggaggcggtttctttcgggttctgccggctccgtggctgaggaggcggtttctttccggccgcgccggctccatggctgaggaggcggtttctttccggccgcgccggctctgtggccgaggaggtggtttctttcccgttgtgccggctccgtggctgaggaggcggtttctttaaggtcttttctgtgctgatgttttagctttactgagattttgttgcttatcacacaattcaccattgaagtgtcctgggctgatctgatgccgatggcctccgagtcaaatgctctctaaaggaaattctcagaagatctccggggaaaagcacacataatttatagaattagaaagcaaaggatttgtaagacatcacaaggaattcagttaccagttaggactggtcacctccaaacttaagtacaaagaacttatttacttcttccaaggaaatttatttgggggattttttatgtggccatgatgatgctgtcagtggccgaagctgcattctggcaactccagatcctgggtgactttgcctagctctgcccggcctggtgttgcaggaaatacgctaattccaggcacggaagctgggagtgcatccggtctggggagactttgcctttctaagaggctctcagtgctgttgatggtgcacattcgacctttgagacttggagaaatcagattgcagaaatgatgcagagcacctgagcagaaccaatctggcgtgagacacacacgcacacacacacacaatcaggcgcacccacccacacatatacacacacaggtacacagtcgtgcacccatccacatacgtgcagtcatgcacacagccctgcacacagacctacacatacacatgcgtgcacacagacatgcacacacacagtaggggccctaagcaggcgtccttagcctttctgctctgagctctgcagcatcagaacctgctgccataactgagccaagtgaactcctgaagcaggagcatccccgggcgtggcaggggagcgcccaccaccaagattctgctgctgtgctcgggggcagttgtgccttttctgtttttctttctttctatatttccaggaaatcatgacattaaaaatgactttttcttatgacgaatattcattgtaggatatttagtgaaaattcacacaataaaaactgtgattcgtttgtgctctccgagtttctgggtttccttgcatttttctggcagcttctattctctctgggtgcttccgatgcacacatcgcagatcccaggatgatcttcctgcctggcacggctgcctcctccacgccacccctcattacctgtggtctaggaagaccaccagttcccattccaagctgcccaaa

SEQ ID NO: 8683 - RNA, 4675 nt, Homo sapiens
  source 1..4675: mol_type = other RNA
aaccttggcccctctccccaggtggaatcaaggctaatcgcctgccctgatggccctatcgggtgagtctggaatcatcctgatcatttttctggaggctgcatgtaccttcttcctctgcttcctcccctgttccagtgggggccagtagaatctggggctctagggaggggtccgtgtgggagctccaggcaggtctttctgttttggtttctccaaagtctaaaccctggggagcttcaaacatccaccccctccagcgactgatgtgcggggtccggctggcctgtgtcctgagtatctgggtccttagcccctgggggaccctcaggcgaggccacggttgacaaccccctgcctgatgtgttgatcggtcagtgagctcctggtctgcacacgggccggccacatcctggacttccccgtgaattctccagcagggcagccgtgtggtgggatgctgtcaccgctgtctgctttgtctcatcgtctgttccatttctcttgcttcttacttcaactgtggattcttacagggcagaactgcacgagtcatctttgcaccttgtctagtgtccagagccagttcttgtggggaagctgagtgctctgtaactcccgtgtctcagctcccttgcgtggcccctagaggcagacgtgggaggaatgccgcagcctcggagaaccaggtctggcattcttggtgctggtcccagggtcccgaggcctgctttccacagtcacgctgtagagacggctccttgtggagacaccttctgtgtgcaggcacgaggtttctcctctgccccaggcttcggtgcggagtgtctggggggacagagccaccagatgtgaacgctgtgctagtcgccctctctggtctctcccttggcgtggccagactccccggtgcatctggacatcgtggcgggcaactgccatttacagacacgggaggacgttttgcatgacccgccttctgtgtgttttcccactctttgcaaacccattgcttttcagctcggagagttgctttccagttgtgccagctccgtggctgaggaggcggtttctttcccgttgtgccggctccgtggccgaggaggcggtttctttccggttctgccggctccgtggccgaggaggcggtttctttcgggttctgccggctccgtggccgaggaggcggtttctttcgggttctgccggctccgtggccgaggaggcggtttctttcgggttctgccggctccgtggccgaggaggcggtttctttcgggttctgccggctccgtggctgaggaggcggtttctttccggccgcgctggctccgtggctgaggaggcggtttctttcgggttctgccggctccgtggctgaggaggcggtttctttcgggttctgccggctccgtggccgaggaggcggtttctttcgggttctgccggctccgtggctgaggaggcggtttctttccggccgcgctggctccgtggccgaggaggcggtttctttcgggttctgccggctccgtggctgaggaggcggtttctttccggccgcgctggctccgtggctgaggaggcggtttctttccggccgcgccggctccgtggctgaggaggcggtttcttttgggttctgccggctccgtggctgaggaggcggtttctttccggccgcgccggctccatggctgaggaggcggtttctttccggccgcgccggctccatggctgaggaggcggtttctttccggccgcgccggctccatggctgaggaggcggtttctttcgggttctgccggctccgtggctgaggaggcggtttctttctggttctgccggctccgtggctgaggaggcggtttctttcgggttctgccggctccgtggctgaggaggcggtttctttccggccgcgccggctccatggctgaggaggcggtttctttccggccgcgccggctctgtggccgaggaggtggtttctttcccgttgtgccggctccgtggctgaggaggcggtttctttaaggtcttttctgtgctgatgttttagctttactgagattttgttgcttatcacacaattcaccattgaagtgtcctgggctgatctgatgccgatggcctccgagtcaaatgctctctaaaggaaattctcagaagatctccggggaaaagcacacataatttatagaattagaaagcaaaggatttgtaagacatcacaaggaattcagttaccagttaggactggtcacctccaaacttaagtacaaagaacttatttacttcttccaaggaaatttatttgggggattttttatgtggccatgatgatgctgtcagtggccgaagctgcattctggcaactccagatcctgggtgactttgcctagctctgcccggcctggtgttgcaggaaatacgctaattccaggcacggaagctgggagtgcatccggtctggggagactttgcctttctaagaggctctcagtgctgttgatggtgcacattcgacctttgagacttggagaaatcagattgcagaaatgatgcagagcacctgagcagaaccaatctggcgtgagacacacacgcacacacacacacaatcaggcgcacccacccacacatatacacacacaggtacacagtcgtgcacccatccacatacgtgcagtcatgcacacagccctgcacacagacctacacatacacatgcgtgcacacagacatgcacacacacagtaggggccctaagcaggcgtccttagcctttctgctctgagctctgcagcatcagaacctgctgccataactgagccaagtgaactcctgaagcaggagcatccccgggcgtggcaggggagcgcccaccaccaagattctgctgctgtgctcgggggcagttgtgccttttctgtttttctttctttctatatttccaggaaatcatgacattaaaaatgactttttcttatgacgaatattcattgtaggatatttagtgaaaattcacacaataaaaactgtgattcgtttgtgctctccgagtttctgggtttccttgcatttttctggcagcttctattctctctgggtgcttccgatgcacacatcgcagatcccaggatgatcttcctgcctggcacggctgcctcctccacgccacccctcattacctgtggtctaggaagaccaccagttcccattccaagctgcccaaatagctgcgaaatatctgctggaacagtgtctggtatatcgcggatgtttagtaagtcttgagaggctcactgagtgaacagtgttaattttcatggtttaaaactttatataaatggtaccatactcgctgccgtacttgctgtcgtactcgctgccgtactgtgcacttgcatttttgctccgcgttctgtttttggcatttatccacattgatccatgtagctctcatttattttaactgccatgtggtatttcgctgtatatgcccatttctttatcgcttctccccgtgttggatattcagggtgtgtccggtgctttggacacacagtgttgtgaggaatattctgtacgcatcttctagcacatgcatacttcttgtggtagtttctctctcacagtggatggcctattagaatgactagggaattcttagctattagtttgttcccagaagttctggttcaattgatctggtctgggttcagtgctgcagaaatgttttttcttttaaagacattcctggatgactttaacgacagccggggttgagaaccacggctcctggctcgaaggagcagatctatgtttgtgttcttgggcatatctagaaagagatatgctttctttctggcttgtcatctacttgcttcaattttcctaaaggttgctttcaaagtggtggcaccatgcgtgatcccagcggtgaatgcagattcccacgttttcattaacattctttaagttgtttgacccttggggttttctgataggatgagggtgaaacgcatcctcttgttcccacagcgttcccctaattccgggggctgagtttattgatcgttcaagcatcttcttttgtgacgggaccgctgatgtccttgactcaaagatgttaaaaatacgtttagaaggatctttattttttcctgctgctgtacgaggcaccctttctggccccgtgtttccttgcccttctttccagcagcagattttactcagaacaacttcagtgctgtggacacaaagacgcaggccttggagaggcgggtcagccctgcctcggggctgctgagtgaggtgccagatgcgtttgttcctcatttactcatttgcgtttgttcctcatttactcgttcctcgcagactgggttgtaacaccatgtaccaccctctgaacccagagatcaagggctggctggccctgtagccccaaggagctccgtcaccggccaatggggaggcgaacccgtggtgacccactcagcggcaccgccaagggctgagcgtggcgccagcggcggaaggcccggggtcaccgtcccaggccggggctccgaccccgagtccgcagggtcctctccaggcaccttccatctggggtctggcttccactcccggccgcggcgtcctgatttccagaaaccaggcggc

SEQ ID NO: 8684 - RNA, 29 nt, Homo sapiens
  source 1..29: mol_type = other RNA
aacgccattatcacactaaatagctactg

SEQ ID NO: 8685 - RNA, 3883 nt, Homo sapiens
  source 1..3883: mol_type = other RNA
aacggcaatgacttttgtaccataagctgtttccatctaggacctatttctgtgggatggtctgagggtgaagctaaggagagaaggcatatgtgaatttattttgtttatctgaacatctgtgtttggccggccccacccctacaatgtaagctaaaatgctgtataataggtttatgtatgtacctatactgccaaaggtcatggttgaatcctgtgactaggtagagtttacctgtcaattggctaaatcagagacccatatgtttcatagtcaaggagattctgcagcataaatggctggcccagggaccactggcctgtatgcatcactgccctgctcataaacctcatggctccccactggcaaatgttgagtccaccttcctcaacctgtattcaaggcctgccatcatcttcttcctgccagactggccttcaggtcctgtgccttggcaggtgagcttttcccctgcctcccttctctctctctctctctctctcttcctccttccctccctgtctccctttcttcctccctttaaagagcaccagacactgttttaagtgctggggacacagtcactaagtgtggtggacaagacacaggaggctttagcttacgttgtagaggtggagacaaaagaaaacagatattcaaataaacaagataaattcagataagtgctatgaatacaataaaacaagatgatgtgctacagcaggggttcccccaccgcccatgctcctcaacgttagattctcaaaggatgtgaaccctattgcgaattgcacactccttatgagaatctaattcctgatgatctgaggtggtacagtttcatcttcaaaccatccacttcctgccctcccatccgtggagacattgtctttcatgaaactggttcctggtgctagagagctttgtgggtaggagtgaggctgaattctccctacccccatggccttcacaggtaaatgctgcccattggtcaaagcctgcccacatgtcacctcttccaggaagcctgcctgccttctcagcttggcagtgttctctcccaccactggactccagagcactttattccgctcccttgcagggtgtggagtggcttgcagcacagtccatggtcatccttgctgctgggctgtaagttcctcagagggcaaagagcagccggggcccatccccagggtcacctgctgagaagaggccacttttctcccaaggtaatcctgttggacaggaacacctcacactcttctaaacctttacagactttgctctgatgagaggcctaagaagagtgtcatgccccttccttggcttggggaagtctggacctgtgtgtaggggcgtggggtgaggtggggtcggtgtgcattgtgccagggtgtatggctcagagcatgtgtgcagtgaggtgtttgtgaggtgtctgtgactgtggtcctagaactgtgggcataggatgtgtgagagaacaagtgagtgcgtatgtgaatgtggtggtgaggtgcgtgcagggtggctggtttgtgtagtgtctttgtgtgtttggatgttgagtggtgggctggtggtggtgggggtgtgtgtgtatctgtggtacagcccgtggggttgggggacagggaagggtggagcagcagtggcctgggctctggggggccagcatctgtggtattagggctcagaaaatgatacccacaaagatggcactttgacatgctgaattgaagaagcagcctccaggtctctctgacctacctcccacaaaagcccctgtctctcccaaagcacaggatgaggctgtcttctgaagctcccatatcgaactggaaactggactcccaagcaggagcagaattgccttcgatccctctcctgaaatttcattaatcagaggagatgaaaactcctaccacagaggaagagactgatcacgaaacaccacatctagagcccaaactgtgtctcaaactattgtttgttctctggtcccattcagtttccaaaaagaatcattcacaagataatgcctgcctcctggctccattcatcccccaccataaaagtatttatgcctgtaacaccttgtctctttccactataaagaagggtttacaagcacctggacctctctgggttatcgggtaatcattctcccgccatacccctgtgctatgcatgttaaataacatccgtttacctcttttttctattgatctgctttttgtcagctcactttctgcaaaccttcagagggtgaagggggaagctttccttctttgcccctacactggcaactgggacttcactttccagctgctagctggggccttagagaggaccccacaactggaagccatcacagctcttcccccaccctgctggcctgtgggggatgctgttgcctcttcagctcccctctgactgtggtccctctgtttcgaagccctagcctcaagcctcatccccactctctttcctactaccaagagcagacaccaaaatatttctgcgtttcctctggaaaaatcctgggaggtctgtttatggctgtagcaaagcggcacacatctgtgcacagttgagctgggacagctggaaactcaggcactggagtttgctggaattcggagcacgttggtgtacacagtgcctgccccccacctacccacccaacgtgcctccccatctctgcacgagtgtcccaccagagtcagttcttgcttctatgaataacccttccctggcccctgcacaaacacacccacatacgcagacacactcctgcacacagccgatttcagtaggacacacagagacagagaaagggacacgtggcacacagatatgccagcacattctgagaacaaactcaagcatggttcctcaggtctagaggcccacagacacacacaggcaccctcccgcttcaccagggcacacccttgacctgtcacccaccagtaacacctacatacaccagcagacacgcaggacaacgcatgctgactcggcacacccacatataaacatgcaacccacacagaaggtgtgattcacctccagccacgtacagaaacccactcccagccagtcggggcccgccacctaacctcaggcgaggactaccctcccctgggagacctggggactcctgagcctgggaatgtccctgttctttcccattgcctgccctgtccctgaccctggctcccctctcaactctaccatgtgctgtctctgtcaggcaggccagggaacctgagttcccccagtcctgacctgcctcttccttcccttctgttcctgtaccccacatctttccagaggcctagaaagctctagggctaattatctcatggccctccctgctgccaggaactcctctgcccagtggctgacaccccttctgcctccctcaatccttcagggctgctcttggatctgaagtctcttcttcctcagccccaggccccccagattcccacaaggctccctgatggggaaagaaatgtactcttcaggacagattggggaggagcaggcagatgaagggagacaggaagaaggggagagagaaagtggaaagaaacaaaatgaacagatatttcctaaggcctaggaaggaaggaggggcagattgagtgcagctgtaggatgcccagggtagcaggtgtctgtggggagcagggacagagctgggccacctcagacccccttgctttgctgggcacccattttaagggcttacttggcccacatgaggacaaggcctctctagcaatttatcccaaactcctgatcttctcaggccagaccgggattctccagggctcttggagtggggagttctaggcctcctcttta

SEQ ID NO: 8686 - RNA, 8997 nt, Homo sapiens
  source 1..8997: mol_type = other RNA
aactccaaacactcaaaactcagttatgcttcactaacaaagacccatttacaacagcatcaaaaacataaaatactcaagaataaacttgaccaaggaggcaaaagacttgtacaatgacaactgtaacacattgctgaaaaaattaaagacggcacaaatacatggaaagacacctggggttcacagactgtaatgtttgttattgttagtatgtccacattacccaaagcgatctacaaattcaatgcaagcccaatcttcatgccattttccacaaaaacaaacaaaccatcctaaaattcatttgaaatcttaaggacccccaaatagccaaaacaatttgggaaagaacaaagctggaggcctcacacttcctcatttcaaaaacatactacaggaaacgtagtgtaatcctgattacaaaacattactggagtaatcaaaatagcatggtactggcataaagacaaacatatagaccaaagaaacagagcagacagccagaaataaacatgcatgtatatggtcaaatgatctttgacaagagtgcaaagaatacatgatgtggaaaggatagtctcttcaacagatggggctgggaaaactggatattcgcatgcaaaagaatgaagatggaccctttaccatacataaaaatcaaaatggttaaaagacttaaacataagacctgaaactataaaactcctagaataggagaaaagcttcatgacattggatttggccatggtttcttgggtatgaccagaaaagcacaggaaacaaaagaaaaaatagaaaaattaaacttcaccaaaattaaaaccttctttcaaagggcattaggaatagaatgaaaaggcaacccacacagaatggaagaaagtatttgcaaatcatttatctgaaaagttctttatatattctggatatattaagaacttctacaactaaacaacaacgccaacaaaaccaattaaaaaatgggcaaaggacttcaataaacatttctccaaagaagagatacaaatggtcaataagcacataaaaagacagttaacatcactaatcactagggaaatgcaaaacaaaactagaataagatgccacttcaaacccattaggatgtctattataaaaaagaaatagaaaataagtgttagcaagggcggggatactgaaacccttgtacatagctggtgggaatttaaaatagtgtagttgcacttcctcaagaagttaaatatagaatcatcataagatccagcaattctatttctaggcatatacttaaaagaacagaaagcaccactgattatagcaatgttattcttgatagccaaaatggtgcaaacaacttaaatgttcactggcagataaaaggataaacaaaatgtggtatacaagtaaaatggaatattattcagccttaaaaaggaattaaattctgatatgtgctacaacacggccgaaccttgaaaacataatgctaagtggaataagccaaacacaacagggcaaatattgtatgattccattcataccaagtaattagaacagtcaaatttgtacagacaggaagtagaacagtggttaccaggagcctgaggaggagaaaatggggagttactgtttaaggagtacagagtttcagtttgggatgatgaaaaagttctggagatggatagtggtgatgactgcacaaaatgtgcatctatctaaatgctattgagctgtataaccaaaaagtgtttaaatggttcattttaagctatatgtatcttactacattaaaaaataattctaaaataaataaaatgactttattgaccaaaaccttgccttgtcctgtgacatgaaaaaaatttatacacgctcattaagaggaaacattatttaaagcaaggacttcattttaaagtaaaatgtgtcacagtgctcttcataaaagcaatcctataatgaatcaaaagacgtttaaagccttttgataatctgacttaatccaaaagtgaatttaaatatttgggtgatgggccagactgaatgtcctgcaggcaattatacagacttaactactgaaatcaagactttgataaatattatccaacagagtttgggctgctctctgtagctagtacatggtatttagaaagttcatattggataaaggacttatatccagaataaaaaggactacaacacagtatcagcaaactccaattttaaatggacaaaaaatctgaataaacatttcactaagatacatgaatggctgaagagcacataaaagatgctttgacattattcgccatcaggaaaatcaaagttaaaaccacaaaggaatatcatttcaaacgctaggatgggcataatttttaaaaaacagacaacaatgactggcaagactgtagagaaatgggaagccccacacattactagtcagaatgtaaaataatgcggtcactttggaaaacaatttggcagtttcctaaaaaagttaaatgaaaatttaccgtatgacctagcaactcccctcaggcatctgcctaagaaaaatgaaaacatgtccacacaaagacttgtacactaacgttcaaaacacttgcataccaatgttcaaagcagcattattcctaacaggcaaaaactggaaaaacctcaaatgttcttcaactagtgaatgcacgaagcatccacataatgtaatattatttatgataaaaaggaataaagtactagtatgttacaacatggatgaacttaaaacacattaatgaaaaaaacacagaaagatcacatataacataaaatgtacagaaaaagacaactctagagacacaaagtcgactgagtagtgggtgcctgggattagaggttggacgggagattaactgtaaactggaataacggatcttgctgggatgatgttctaaaaaatggattatggtaatggttgcacaactcagcatatttactaaaactcactgaattgtacacttgaaatggttttaatgatatgtaatttgtacctcaataaattcctttaaaaaaaaagtttatactccagattcccaatggatactgggataaaacattgttatgaatgttagggagtctaagagtaatcatcttggaacaagcctcttctgaagacttttacgttatttcttcaactttctataaattatatttttcagaaaacaaaacttacaacaagttttctgtcttttcagaaaaaaacttaaaaccattatgaatgattctcataataaacattcctttcatggctaggatgtgattcgttggtctgcttagcaataactatgcggaccaatttatcacacggcaatatttaaactgcaggcttggggttggggaggcaccaaaaaccttctcccagaggtagcatttcacacctacatacattagtcacagtaaatgttcctgagtctaagattagcattaaggatcgctttacttccataagtgaagagttttctggtttagctctctttttataggaggtgcccacaatttcaactttaggaacttatttctagaccactgttgagtccatggggttcctccagaaccctatgacctgaagccaaaacctcactcattcagggccttaagttcctttttcagttggaaattattattcagactccaccaatgaaatttataaggaataatccaccaatacccgtatattccattcctctgaggtctaatttcacaaaagaaaacttaactgaaaattttttctgtatcaattctacattcattccctgaactttacttgctatcagtgcagtctctttagattttagggtatctattctccaaatggtaggggttataatagaacattcatacagtgggaaagtcaggtgacatacatgagagaactagctaagtcagaaagttgattccccatcaaaaggtggcagctgctacccaggaccagctgagtgctttacataaataaaagcccagtgttgttagcccttataattttttttaagacaagctttgtttttagtatgaaatgccctaattttagatagtggcaacaatgtatacacacacacacacacacacacacatgcacacacacccaagcaaattgttataacagcttttaactgttgccacacagaatgtttacactccaattgcaaaaaaatgtacttgctacaggcaaaattgttttaaagtagaatttttgcaaaccaaaatccatccagaatagctctgtcttcagcacatttccttacccccagcccccatctattttcctaggactgttactctcacggctgagatggctcaggtgcaagctctctggcttctcagtcctgttggccaatgcccaaaagaaaaagagttcccttgtccgattaaaatactccctcaaggaaaagtcgtttgaacttcactgacccattcctagttacagcatttgagggattcctgcacgaagttttcaaaaagtatactgcattctcactaagctagaagtccagcatcctaggaaccaggcttgatggagtgtacccgtaatgtcagctactcaggaaagtgagatggaaggatcacttgagcccaggagttcaagaccagtctgggcaacatagtgagactccatcccaaaaaagaaaaattgaaaaaaaaaaaagaaaaaaaaaagaaaagaagtccagcatcctgaatagtggtattgtattttttactagagaaacttgaaagtaatgacaaataaaaaaaaataacttatgtccacagcttcagagattatcaggataccaataaaaaactaaaaaaccaaaaaaggcaaaaatcattaatcccatcccttcattctgctggtgacgaaaataaaattctgaaaggtcaaatgacttgtccaaggtgtatacagcaagttggttggcaaactgggacagaatccaagttatgtgactgcagtcaagttctctccatcacactacatggtagtagaagaaatcagagagaaatcccctgaagaaaagagcttttccaattcgtctggcctcagaatcattttgcattcttccctttccagtgactttaccaactaattactgtttaccagtcgttgccatccttgaaaagaagagggatgaatgggcaaaaggatatttttcctaactgccaatttacgaaagctgcagctactgatcaatactgtaagtttacatcccagggtttcagtaactgacaatttgaattaaattccccccactttaatgtagttccaggattactctgcagagtgaaatccccgatgtctaatgaggcctgaattacttttaaatgtcttctcacattcgttacattcatattctctccttccggtatgaatttttaggtgttctacaaggattgagcttcgactaaaggttgcaccacaatagttacactcatagggtttctctcctgtatgaattcggtggtgctcattaagagatgaactctgactgaaggacttcccacattctttacatttataaggttttacaccagtatgaattctctgatgacgacttagcagtgaatgggttgggaaggctttctcacactggttacatttgtagggtttttctcctgaatgaagtctttgatgataaatcacagacgtaaaatggctaaaagtcattccgcaatcattacacaaatatggtttttctccagtgtgaattctctgatgccgggtaaggcatgaattctgcctaaaggcttttccacattcgccacatttatagggtttctctccagtatgaattctctgatgtttggaaagggatgagctatgactgaaggattttccacaattgctacatgtatagggtttttctccagtatgaattcgctgatgttgaataagagatgaactgtcactaaagggtctcccacagtctttacatttataaggtttttctccagtatgaattctctgatgtttaatgaggtgagcacttagggtgaaacctttcccacagtcatcacatttgaagggtttctctccactatgagttctatgatgtggtgtgagcgatgaactatcactaaaagcttttccacattcattacacatatagggtttttctccagtgtgaattctccgatgtttggtgagtgaggcgctatagccaaaggcttttccacacttactacatttatgagttttttctccactctcatttccctcatctttatttaaggctgcttcttgacatgaatctttccgacatttctcacacataggggtttttctcctagaaagagttgatcttctaataaagattatcccacacttactgcatttttgggacctatcccccaaatgaatcttctgacgtttctgatgttcagtaagagctgaagagtgactcaggactttcccaccatcattagatttccgtgacttttctccggcggttttctccttgcggttcagaacaaggtctgaatgaaaactgaagggtttcttgctttcattatacctccgagatttcttcctcaagtagactctcagatgtttaattaagtctgaagtttctttgaaattatgtccaaaggggcttttatctgggtcaaatttcttacccctactgccactcccaagagttttgttttgtgcgactcttccttttgaatttccctgattaccgtgatcctcctctgagctgccacaatattgctgggattcttccatcaagccatgatcatcatccctgaggcacctttctattattttatctaaagctgattcatctagtcgggagctttttgagacttcttccagcagccatggcaattcaacccactttagctgggaaatcaactctaattttgaaactggaaagtccagaaattctaggttcctgaggttttccagtagcacttccttatatagctccttttgaaaaggctccagcttcttccactctcctcttgaaaagttcacagctacatccttcaatgttatagattcacaggactcagtattgggacaaacagtgaccattttatcctcttttgagttctcctcttgggaaacagtagaatcttgagagactggatctttttcttcaagcatctgggtcaaatcttctattagggtcaccacttcctcactactctcaggatgttgtgactttacccaaatcctgatctccccaggcaaaatggtcaggaactgctcaaacaccagaagctctaaaatctgttctttcgtgtgaatgtctggtctcagccactgattgcagagctcccagagttgactcagagctttcctgggtccagctacttctgagtaacaaaaccacctaaacctctgtctgaaagactctgcatcagcagcatttcctcttaaaatagcttcttgttccccagaagtaaccactcttgggacctcattttgttcagtcgaggccagagtttgaggttctggtgagatggctgtcatcttgttcaagggcactacagcttgcattgtgtctcaggggcaggaatccagtcccttcacactctagttgagtatcagtacagtccaccaacaggcactatacacagccaggaatatcaaaggttccaggaatccagtttacagtcctgcagaaacagcaaaggcctagaaaagccctgctcaattaaaaggataactttctttctttttttttttgagacggagtttcgctcttggtgcccaggctggagtgaagtggtgcgatctcggctcactgcaacctctgccccggctgggttcaagtgattctcctacctcagcctcttgagtagctgggattataggcgcccaccaccatgcctggctaatttttgtatttttagtagagacggggtttcgccatgttggccaggctagtcttgaactcctgacttcaggcgatccacccacctcagcctcccaaagtgtcaggattacaggcgtgagccactgtgcccagccataattttctttatagtcaaaaaccagggagctacttaagggttaaggaaacagttgctttagattgaatactcctcctaaacaaaatgttatcagaaaaggttcacaaggggacccagtcacaaagctatttaacaactcctaccctttcttaatgaaagggcacacatttctcactagttgctcaactcagaagcccaatttaatatttgactttcaaatttctcttcctccttacttctcccatcaatcgccaagttctggcgattttatttcctaagaacctctccattctatccttctgaaactgcctaagtacagggttcttcactccagtctcacactgtggccaaaaaattccttctaacatgcaaaatatgatcttatcactccccggcttacagtccctcaccagccaccgaactgtctctcgataaagttcacatgcagggaccatggcattgtgatctagagacactgtctgatgacctcacctcttgagctctagctacccgattgacactacagccataaattagtatctcctctctctctacatactctcctagcctttgcaccaaggctattccctctcctcggaatgttgctttctttctcctaccaaacttttattcgtctttaaagcctgactcctttcaactgtcacttctggtgtgatgctctgcttgatcccaaagcactcctttgcacacagactgccctgtgttgcattcattcattcattctataagtgacggagcaactacaatgagctggaacgagaccaggggccatgagctgcggggccaggcgtggacaggcctgaaagggtcctcacgctcacagagggtccaggaaatgacaatacagccggagcgggactacaatgcgacaagtgaaggatgtgacagcctcgcattgcaactaccataccaataacaacccacttccgagtacagcgcccggcacacagcagcatgacgtcatttattcctctg

SEQ ID NO: 8687 - RNA, 7737 nt, Homo sapiens
  source 1..7737: mol_type = other RNA
aactccaaacactcaaaactcagttatgcttcactaacaaagacccatttacaacagcatcaaaaacataaaatactcaagaataaacttgaccaaggaggcaaaagacttgtacaatgacaactgtaacacattgctgaaaaaattaaagacggcacaaatacatggaaagacacctggggttcacagactgtaatgtttgttattgttagtatgtccacattacccaaagcgatctacaaattcaatgcaagcccaatcttcatgccattttccacaaaaacaaacaaaccatcctaaaattcatttgaaatcttaaggacccccaaatagccaaaacaatttgggaaagaacaaagctggaggcctcacacttcctcatttcaaaaacatactacaggaaacgtagtgtaatcctgattacaaaacattactggagtaatcaaaatagcatggtactggcataaagacaaacatatagaccaaagaaacagagcagacagccagaaataaacatgcatgtatatggtcaaatgatctttgacaagagtgcaaagaatacatgatgtggaaaggatagtctcttcaacagatggggctgggaaaactggatattcgcatgcaaaagaatgaagatggaccctttaccatacataaaaatcaaaatggttaaaagacttaaacataagacctgaaactataaaactcctagaataggagaaaagcttcatgacattggatttggccatggtttcttgggtatgaccagaaaagcacaggaaacaaaagaaaaaatagaaaaattaaacttcaccaaaattaaaaccttctttcaaagggcattaggaatagaatgaaaaggcaacccacacagaatggaagaaagtatttgcaaatcatttatctgaaaagttctttatatattctggatatattaagaacttctacaactaaacaacaacgccaacaaaaccaattaaaaaatgggcaaaggacttcaataaacatttctccaaagaagagatacaaatggtcaataagcacataaaaagacagttaacatcactaatcactagggaaatgcaaaacaaaactagaataagatgccacttcaaacccattaggatgtctattataaaaaagaaatagaaaataagtgttagcaagggcggggatactgaaacccttgtacatagctggtgggaatttaaaatagtgtagttgcacttcctcaagaagttaaatatagaatcatcataagatccagcaattctatttctaggcatatacttaaaagaacagaaagcaccactgattatagcaatgttattcttgatagccaaaatggtgcaaacaacttaaatgttcactggcagataaaaggataaacaaaatgtggtatacaagtaaaatggaatattattcagccttaaaaaggaattaaattctgatatgtgctacaacacggccgaaccttgaaaacataatgctaagtggaataagccaaacacaacagggcaaatattgtatgattccattcataccaagtaattagaacagtcaaatttgtacagacaggaagtagaacagtggttaccaggagcctgaggaggagaaaatggggagttactgtttaaggagtacagagtttcagtttgggatgatgaaaaagttctggagatggatagtggtgatgactgcacaaaatgtgcatctatctaaatgctattgagctgtataaccaaaaagtgtttaaatggttcattttaagctatatgtatcttactacattaaaaaataattctaaaataaataaaatgactttattgaccaaaaccttgccttgtcctgtgacatgaaaaaaatttatacacgctcattaagaggaaacattatttaaagcaaggacttcattttaaagtaaaatgtgtcacagtgctcttcataaaagcaatcctataatgaatcaaaagacgtttaaagccttttgataatctgacttaatccaaaagtgaatttaaatatttgggtgatgggccagactgaatgtcctgcaggcaattatacagacttaactactgaaatcaagactttgataaatattatccaacagagtttgggctgctctctgtagctagtacatggtatttagaaagttcatattggataaaggacttatatccagaataaaaaggactacaacacagtatcagcaaactccaattttaaatggacaaaaaatctgaataaacatttcactaagatacatgaatggctgaagagcacataaaagatgctttgacattattcgccatcaggaaaatcaaagttaaaaccacaaaggaatatcatttcaaacgctaggatgggcataatttttaaaaaacagacaacaatgactggcaagactgtagagaaatgggaagccccacacattactagtcagaatgtaaaataatgcggtcactttggaaaacaatttggcagtttcctaaaaaagttaaatgaaaatttaccgtatgacctagcaactcccctcaggcatctgcctaagaaaaatgaaaacatgtccacacaaagacttgtacactaacgttcaaaacacttgcataccaatgttcaaagcagcattattcctaacaggcaaaaactggaaaaacctcaaatgttcttcaactagtgaatgcacgaagcatccacataatgtaatattatttatgataaaaaggaataaagtactagtatgttacaacatggatgaacttaaaacacattaatgaaaaaaacacagaaagatcacatataacataaaatgtacagaaaaagacaactctagagacacaaagtcgactgagtagtgggtgcctgggattagaggttggacgggagattaactgtaaactggaataacggatcttgctgggatgatgttctaaaaaatggattatggtaatggttgcacaactcagcatatttactaaaactcactgaattgtacacttgaaatggttttaatgatatgtaatttgtacctcaataaattcctttaaaaaaaaagtttatactccagattcccaatggatactgggataaaacattgttatgaatgttagggagtctaagagtaatcatcttggaacaagcctcttctgaagacttttacgttatttcttcaactttctataaattatatttttcagaaaacaaaacttacaacaagttttctgtcttttcagaaaaaaacttaaaaccattatgaatgattctcataataaacattcctttcatggctaggatgtgattcgttggtctgcttagcaataactatgcggaccaatttatcacacggcaatatttaaactgcaggcttggggttggggaggcaccaaaaaccttctcccagaggtagcatttcacacctacatacattagtcacagtaaatgttcctgagtctaagattagcattaaggatcgctttacttccataagtgaagagttttctggtttagctctctttttataggaggtgcccacaatttcaactttaggaacttatttctagaccactgttgagtccatggggttcctccagaaccctatgacctgaagccaaaacctcactcattcagggccttaagttcctttttcagttggaaattattattcagactccaccaatgaaatttataaggaataatccaccaatacccgtatattccattcctctgaggtctaatttcacaaaagaaaacttaactgaaaattttttctgtatcaattctacattcattccctgaactttacttgctatcagtgcagtctctttagattttagggtatctattctccaaatggtaggggttataatagaacattcatacagtgggaaagtcaggtgacatacatgagagaactagctaagtcagaaagttgattccccatcaaaaggtggcagctgctacccaggaccagctgagtgctttacataaataaaagcccagtgttgttagcccttataattttttttaagacaagctttgtttttagtatgaaatgccctaattttagatagtggcaacaatgtatacacacacacacacacacacacacatgcacacacacccaagcaaattgttataacagcttttaactgttgccacacagaatgtttacactccaattgcaaaaaaatgtacttgctacaggcaaaattgttttaaagtagaatttttgcaaaccaaaatccatccagaatagctctgtcttcagcacatttccttacccccagcccccatctattttcctaggactgttactctcacggctgagatggctcaggtgcaagctctctggcttctcagtcctgttggccaatgcccaaaagaaaaagagttcccttgtccgattaaaatactccctcaaggaaaagtcgtttgaacttcactgacccattcctagttacagcatttgagggattcctgcacgaagttttcaaaaagtatactgcattctcactaagctagaagtccagcatcctaggaaccaggcttgatggagtgtacccgtaatgtcagctactcaggaaagtgagatggaaggatcacttgagcccaggagttcaagaccagtctgggcaacatagtgagactccatcccaaaaaagaaaaattgaaaaaaaaaaaagaaaaaaaaaagaaaagaagtccagcatcctgaatagtggtattgtattttttactagagaaacttgaaagtaatgacaaataaaaaaaaataacttatgtccacagcttcagagattatcaggataccaataaaaaactaaaaaaccaaaaaaggcaaaaatcattaatcccatcccttcattctgctggtgacgaaaataaaattctgaaaggtcaaatgacttgtccaaggtgtatacagcaagttggttggcaaactgggacagaatccaagttatgtgactgcagtcaagttctctccatcacactacatggtagtagaagaaatcagagagaaatcccctgaagaaaagagcttttccaattcgtctggcctcagaatcattttgcattcttccctttccagtgactttaccaactaattactgtttaccagtcgttgccatccttgaaaagaagagggatgaatgggcaaaaggatatttttcctaactgccaatttacgaaagctgcagctactgatcaatactgtaagtttacatcccagggtttcagtaactgacaatttgaattaaattccccccactttaatgtagttccaggattactctgcagagtgaaatccccgatgtctaatgaggcctgaattacttttaaatgtcttctcacattcgttacattcatattctctccttccggtatgaatttttaggtgttctacaaggattgagcttcgactaaaggttgcaccacaatagttacactcatagggtttctctcctgtatgaattcggtggtgctcattaagagatgaactctgactgaaggacttcccacattctttacatttataaggttttacaccagtatgaattctctgatgacgacttagcagtgaatgggttgggaaggctttctcacactggttacatttgtagggtttttctcctgaatgaagtctttgatgataaatcacagacgtaaaatggctaaaagtcattccgcaatcattacacaaatatggtttttctccagtgtgaattctctgatgccgggtaaggcatgaattctgcctaaaggcttttccacattcgccacatttatagggtttctctccagtatgaattctctgatgtttggaaagggatgagctatgactgaaggattttccacaattgctacatgtatagggtttttctccagtatgaattcgctgatgttgaataagagatgaactgtcactaaagggtctcccacagtctttacatttataaggtttttctccagtatgaattctctgatgtttaatgaggtgagcacttagggtgaaacctttcccacagtcatcacatttgaagggtttctctccactatgagttctatgatgtggtgtgagcgatgaactatcactaaaagcttttccacattcattacacatatagggtttttctccagtgtgaattctccgatgtttggtgagtgaggcgctatagccaaaggcttttccacacttactacatttatgagttttttctccactctcatttccctcatctttatttaaggctgcttcttgacatgaatctttccgacatttctcacacataggggtttttctcctagaaagagttgatcttctaataaagattatcccacacttactgcatttttgggacctatcccccaaatgaatcttctgacgtttctgatgttcagtaagagctgaagagtgactcaggactttcccaccatcattagatttccgtgacttttctccggcggttttctccttgcggttcagaacaaggtctgaatgaaaactgaagggtttcttgctttcattatacctccgagatttcttcctcaagtagactctcagatgtttaattaagtctgaagtttctttgaaattatgtccaaaggggcttttatctgggtcaaatttcttacccctactgccactcccaagagttttgttttgtgcgactcttccttttgaatttccctgattaccgtgatcctcctctgagctgccacaatattgctgggattcttccatcaagccatgatcatcatccctgaggcacctttctattattttatctaaagctgattcatctagtcgggagctttttgagacttcttccagcagccatggcaattcaacccactttagctgggaaatcaactctaattttgaaactggaaagtccagaaattctaggttcctgaggttttccagtagcacttccttatatagctccttttgaaaaggctccagcttcttccactctcctcttgaaaagttcacagctacatccttcaatgttatagattcacaggactcagtattgggacaaacagtgaccattttatcctcttttgagttctcctcttgggaaacagtagaatcttgagagactggatctttttcttcaagcatctgggtcaaatcttctattagggtcaccacttcctcactactctcaggatgttgtgactttacccaaatcctgatctccccaggcaaaatggtcaggaactgctcaaacaccagaagctctaaaatctgttctttcgtgtgaatgtctggtctcagccactgattgcagagctcccagagttgactcagagctttcctgggtccagctacttctgagtaacaaaaccacctaaacctctgtctgaaagactctgcatcagcagcatttcctcttaaaatagcttcttgttccccagaagtaaccactcttgggacctcattttgttcagtcgaggccagagtttgaggttctggtgagatggctgtcatcttgttcaagggcactacagcttgcattgtgtctcaggggcaggaatccagtcccttcacactctagttgagtatcagtacagtccaccaacaggcactatacacagccaggaatatcaaaggttccaggaatccagtttacagtcctgcagaaactgcatcagcatccgcaaacagcaccaacgccaccgcaaagagcttccagaagcttgtcccgcagcgagtgcgcgcgcaagcct

SEQ ID NO: 8688 - RNA, 7970 nt, Homo sapiens
  source 1..7970: mol_type = other RNA
aactccaaacactcaaaactcagttatgcttcactaacaaagacccatttacaacagcatcaaaaacataaaatactcaagaataaacttgaccaaggaggcaaaagacttgtacaatgacaactgtaacacattgctgaaaaaattaaagacggcacaaatacatggaaagacacctggggttcacagactgtaatgtttgttattgttagtatgtccacattacccaaagcgatctacaaattcaatgcaagcccaatcttcatgccattttccacaaaaacaaacaaaccatcctaaaattcatttgaaatcttaaggacccccaaatagccaaaacaatttgggaaagaacaaagctggaggcctcacacttcctcatttcaaaaacatactacaggaaacgtagtgtaatcctgattacaaaacattactggagtaatcaaaatagcatggtactggcataaagacaaacatatagaccaaagaaacagagcagacagccagaaataaacatgcatgtatatggtcaaatgatctttgacaagagtgcaaagaatacatgatgtggaaaggatagtctcttcaacagatggggctgggaaaactggatattcgcatgcaaaagaatgaagatggaccctttaccatacataaaaatcaaaatggttaaaagacttaaacataagacctgaaactataaaactcctagaataggagaaaagcttcatgacattggatttggccatggtttcttgggtatgaccagaaaagcacaggaaacaaaagaaaaaatagaaaaattaaacttcaccaaaattaaaaccttctttcaaagggcattaggaatagaatgaaaaggcaacccacacagaatggaagaaagtatttgcaaatcatttatctgaaaagttctttatatattctggatatattaagaacttctacaactaaacaacaacgccaacaaaaccaattaaaaaatgggcaaaggacttcaataaacatttctccaaagaagagatacaaatggtcaataagcacataaaaagacagttaacatcactaatcactagggaaatgcaaaacaaaactagaataagatgccacttcaaacccattaggatgtctattataaaaaagaaatagaaaataagtgttagcaagggcggggatactgaaacccttgtacatagctggtgggaatttaaaatagtgtagttgcacttcctcaagaagttaaatatagaatcatcataagatccagcaattctatttctaggcatatacttaaaagaacagaaagcaccactgattatagcaatgttattcttgatagccaaaatggtgcaaacaacttaaatgttcactggcagataaaaggataaacaaaatgtggtatacaagtaaaatggaatattattcagccttaaaaaggaattaaattctgatatgtgctacaacacggccgaaccttgaaaacataatgctaagtggaataagccaaacacaacagggcaaatattgtatgattccattcataccaagtaattagaacagtcaaatttgtacagacaggaagtagaacagtggttaccaggagcctgaggaggagaaaatggggagttactgtttaaggagtacagagtttcagtttgggatgatgaaaaagttctggagatggatagtggtgatgactgcacaaaatgtgcatctatctaaatgctattgagctgtataaccaaaaagtgtttaaatggttcattttaagctatatgtatcttactacattaaaaaataattctaaaataaataaaatgactttattgaccaaaaccttgccttgtcctgtgacatgaaaaaaatttatacacgctcattaagaggaaacattatttaaagcaaggacttcattttaaagtaaaatgtgtcacagtgctcttcataaaagcaatcctataatgaatcaaaagacgtttaaagccttttgataatctgacttaatccaaaagtgaatttaaatatttgggtgatgggccagactgaatgtcctgcaggcaattatacagacttaactactgaaatcaagactttgataaatattatccaacagagtttgggctgctctctgtagctagtacatggtatttagaaagttcatattggataaaggacttatatccagaataaaaaggactacaacacagtatcagcaaactccaattttaaatggacaaaaaatctgaataaacatttcactaagatacatgaatggctgaagagcacataaaagatgctttgacattattcgccatcaggaaaatcaaagttaaaaccacaaaggaatatcatttcaaacgctaggatgggcataatttttaaaaaacagacaacaatgactggcaagactgtagagaaatgggaagccccacacattactagtcagaatgtaaaataatgcggtcactttggaaaacaatttggcagtttcctaaaaaagttaaatgaaaatttaccgtatgacctagcaactcccctcaggcatctgcctaagaaaaatgaaaacatgtccacacaaagacttgtacactaacgttcaaaacacttgcataccaatgttcaaagcagcattattcctaacaggcaaaaactggaaaaacctcaaatgttcttcaactagtgaatgcacgaagcatccacataatgtaatattatttatgataaaaaggaataaagtactagtatgttacaacatggatgaacttaaaacacattaatgaaaaaaacacagaaagatcacatataacataaaatgtacagaaaaagacaactctagagacacaaagtcgactgagtagtgggtgcctgggattagaggttggacgggagattaactgtaaactggaataacggatcttgctgggatgatgttctaaaaaatggattatggtaatggttgcacaactcagcatatttactaaaactcactgaattgtacacttgaaatggttttaatgatatgtaatttgtacctcaataaattcctttaaaaaaaaagtttatactccagattcccaatggatactgggataaaacattgttatgaatgttagggagtctaagagtaatcatcttggaacaagcctcttctgaagacttttacgttatttcttcaactttctataaattatatttttcagaaaacaaaacttacaacaagttttctgtcttttcagaaaaaaacttaaaaccattatgaatgattctcataataaacattcctttcatggctaggatgtgattcgttggtctgcttagcaataactatgcggaccaatttatcacacggcaatatttaaactgcaggcttggggttggggaggcaccaaaaaccttctcccagaggtagcatttcacacctacatacattagtcacagtaaatgttcctgagtctaagattagcattaaggatcgctttacttccataagtgaagagttttctggtttagctctctttttataggaggtgcccacaatttcaactttaggaacttatttctagaccactgttgagtccatggggttcctccagaaccctatgacctgaagccaaaacctcactcattcagggccttaagttcctttttcagttggaaattattattcagactccaccaatgaaatttataaggaataatccaccaatacccgtatattccattcctctgaggtctaatttcacaaaagaaaacttaactgaaaattttttctgtatcaattctacattcattccctgaactttacttgctatcagtgcagtctctttagattttagggtatctattctccaaatggtaggggttataatagaacattcatacagtgggaaagtcaggtgacatacatgagagaactagctaagtcagaaagttgattccccatcaaaaggtggcagctgctacccaggaccagctgagtgctttacataaataaaagcccagtgttgttagcccttataattttttttaagacaagctttgtttttagtatgaaatgccctaattttagatagtggcaacaatgtatacacacacacacacacacacacacatgcacacacacccaagcaaattgttataacagcttttaactgttgccacacagaatgtttacactccaattgcaaaaaaatgtacttgctacaggcaaaattgttttaaagtagaatttttgcaaaccaaaatccatccagaatagctctgtcttcagcacatttccttacccccagcccccatctattttcctaggactgttactctcacggctgagatggctcaggtgcaagctctctggcttctcagtcctgttggccaatgcccaaaagaaaaagagttcccttgtccgattaaaatactccctcaaggaaaagtcgtttgaacttcactgacccattcctagttacagcatttgagggattcctgcacgaagttttcaaaaagtatactgcattctcactaagctagaagtccagcatcctaggaaccaggcttgatggagtgtacccgtaatgtcagctactcaggaaagtgagatggaaggatcacttgagcccaggagttcaagaccagtctgggcaacatagtgagactccatcccaaaaaagaaaaattgaaaaaaaaaaaagaaaaaaaaaagaaaagaagtccagcatcctgaatagtggtattgtattttttactagagaaacttgaaagtaatgacaaataaaaaaaaataacttatgtccacagcttcagagattatcaggataccaataaaaaactaaaaaaccaaaaaaggcaaaaatcattaatcccatcccttcattctgctggtgacgaaaataaaattctgaaaggtcaaatgacttgtccaaggtgtatacagcaagttggttggcaaactgggacagaatccaagttatgtgactgcagtcaagttctctccatcacactacatggtagtagaagaaatcagagagaaatcccctgaagaaaagagcttttccaattcgtctggcctcagaatcattttgcattcttccctttccagtgactttaccaactaattactgtttaccagtcgttgccatccttgaaaagaagagggatgaatgggcaaaaggatatttttcctaactgccaatttacgaaagctgcagctactgatcaatactgtaagtttacatcccagggtttcagtaactgacaatttgaattaaattccccccactttaatgtagttccaggattactctgcagagtgaaatccccgatgtctaatgaggcctgaattacttttaaatgtcttctcacattcgttacattcatattctctccttccggtatgaatttttaggtgttctacaaggattgagcttcgactaaaggttgcaccacaatagttacactcatagggtttctctcctgtatgaattcggtggtgctcattaagagatgaactctgactgaaggacttcccacattctttacatttataaggttttacaccagtatgaattctctgatgacgacttagcagtgaatgggttgggaaggctttctcacactggttacatttgtagggtttttctcctgaatgaagtctttgatgataaatcacagacgtaaaatggctaaaagtcattccgcaatcattacacaaatatggtttttctccagtgtgaattctctgatgccgggtaaggcatgaattctgcctaaaggcttttccacattcgccacatttatagggtttctctccagtatgaattctctgatgtttggaaagggatgagctatgactgaaggattttccacaattgctacatgtatagggtttttctccagtatgaattcgctgatgttgaataagagatgaactgtcactaaagggtctcccacagtctttacatttataaggtttttctccagtatgaattctctgatgtttaatgaggtgagcacttagggtgaaacctttcccacagtcatcacatttgaagggtttctctccactatgagttctatgatgtggtgtgagcgatgaactatcactaaaagcttttccacattcattacacatatagggtttttctccagtgtgaattctccgatgtttggtgagtgaggcgctatagccaaaggcttttccacacttactacatttatgagttttttctccactctcatttccctcatctttatttaaggctgcttcttgacatgaatctttccgacatttctcacacataggggtttttctcctagaaagagttgatcttctaataaagattatcccacacttactgcatttttgggacctatcccccaaatgaatcttctgacgtttctgatgttcagtaagagctgaagagtgactcaggactttcccaccatcattagatttccgtgacttttctccggcggttttctccttgcggttcagaacaaggtctgaatgaaaactgaagggtttcttgctttcattatacctccgagatttcttcctcaagtagactctcagatgtttaattaagtctgaagtttctttgaaattatgtccaaaggggcttttatctgggtcaaatttcttacccctactgccactcccaagagttttgttttgtgcgactcttccttttgaatttccctgattaccgtgatcctcctctgagctgccacaatattgctgggattcttccatcaagccatgatcatcatccctgaggcacctttctattattttatctaaagctgattcatctagtcgggagctttttgagacttcttccagcagccatggcaattcaacccactttagctgggaaatcaactctaattttgaaactggaaagtccagaaattctaggttcctgaggttttccagtagcacttccttatatagctccttttgaaaaggctccagcttcttccactctcctcttgaaaagttcacagctacatccttcaatgttatagattcacaggactcagtattgggacaaacagtgaccattttatcctcttttgagttctcctcttgggaaacagtagaatcttgagagactggatctttttcttcaagcatctgggtcaaatcttctattagggtcaccacttcctcactactctcaggatgttgtgactttacccaaatcctgatctccccaggcaaaatggtcaggaactgctcaaacaccagaagctctaaaatctgttctttcgtgtgaatgtctggtctcagccactgattgcagagctcccagagttgactcagagctttcctgggtccagctacttctgagtaacaaaaccacctaaacctctgtctgaaagactctgcatcagcagcatttcctcttaaaatagcttcttgttccccagaagtaaccactcttgggacctcattttgttcagtcgaggccagagtttgaggttctggtgagatggctgtcatcttgttcaagggcactacagcttgcattgtgtctcaggggcaggaatccagtcccttcacactctagttgagtatcagtacagtccaccaacaggcactatacacagccaggaatatcaaaggttccaggaatccagtttacagtcctgcagaaactggcgccgtgctgagcacctggggctccgcgatgactaagacactcggctccgtctacagggagtttacataggaggcccggtgaaaatgtgacgcagccagaggatctcaaccagagggaagaaaaaaggagagatttcaccccccagcggtcctctggcaatgtctggacacatttttggttagctcgactaggacgagaggtggtactgttatctgcatcagcatccgcaaacagcaccaacgccaccgcaaagagcttccagaagcttgtcccgcagcgagtgcgcgcgcaagcctgcgggaaccactgcgc

SEQ ID NO: 8689 - RNA, 7856 nt, Homo sapiens
  source 1..7856: mol_type = other RNA
aactccaaacactcaaaactcagttatgcttcactaacaaagacccatttacaacagcatcaaaaacataaaatactcaagaataaacttgaccaaggaggcaaaagacttgtacaatgacaactgtaacacattgctgaaaaaattaaagacggcacaaatacatggaaagacacctggggttcacagactgtaatgtttgttattgttagtatgtccacattacccaaagcgatctacaaattcaatgcaagcccaatcttcatgccattttccacaaaaacaaacaaaccatcctaaaattcatttgaaatcttaaggacccccaaatagccaaaacaatttgggaaagaacaaagctggaggcctcacacttcctcatttcaaaaacatactacaggaaacgtagtgtaatcctgattacaaaacattactggagtaatcaaaatagcatggtactggcataaagacaaacatatagaccaaagaaacagagcagacagccagaaataaacatgcatgtatatggtcaaatgatctttgacaagagtgcaaagaatacatgatgtggaaaggatagtctcttcaacagatggggctgggaaaactggatattcgcatgcaaaagaatgaagatggaccctttaccatacataaaaatcaaaatggttaaaagacttaaacataagacctgaaactataaaactcctagaataggagaaaagcttcatgacattggatttggccatggtttcttgggtatgaccagaaaagcacaggaaacaaaagaaaaaatagaaaaattaaacttcaccaaaattaaaaccttctttcaaagggcattaggaatagaatgaaaaggcaacccacacagaatggaagaaagtatttgcaaatcatttatctgaaaagttctttatatattctggatatattaagaacttctacaactaaacaacaacgccaacaaaaccaattaaaaaatgggcaaaggacttcaataaacatttctccaaagaagagatacaaatggtcaataagcacataaaaagacagttaacatcactaatcactagggaaatgcaaaacaaaactagaataagatgccacttcaaacccattaggatgtctattataaaaaagaaatagaaaataagtgttagcaagggcggggatactgaaacccttgtacatagctggtgggaatttaaaatagtgtagttgcacttcctcaagaagttaaatatagaatcatcataagatccagcaattctatttctaggcatatacttaaaagaacagaaagcaccactgattatagcaatgttattcttgatagccaaaatggtgcaaacaacttaaatgttcactggcagataaaaggataaacaaaatgtggtatacaagtaaaatggaatattattcagccttaaaaaggaattaaattctgatatgtgctacaacacggccgaaccttgaaaacataatgctaagtggaataagccaaacacaacagggcaaatattgtatgattccattcataccaagtaattagaacagtcaaatttgtacagacaggaagtagaacagtggttaccaggagcctgaggaggagaaaatggggagttactgtttaaggagtacagagtttcagtttgggatgatgaaaaagttctggagatggatagtggtgatgactgcacaaaatgtgcatctatctaaatgctattgagctgtataaccaaaaagtgtttaaatggttcattttaagctatatgtatcttactacattaaaaaataattctaaaataaataaaatgactttattgaccaaaaccttgccttgtcctgtgacatgaaaaaaatttatacacgctcattaagaggaaacattatttaaagcaaggacttcattttaaagtaaaatgtgtcacagtgctcttcataaaagcaatcctataatgaatcaaaagacgtttaaagccttttgataatctgacttaatccaaaagtgaatttaaatatttgggtgatgggccagactgaatgtcctgcaggcaattatacagacttaactactgaaatcaagactttgataaatattatccaacagagtttgggctgctctctgtagctagtacatggtatttagaaagttcatattggataaaggacttatatccagaataaaaaggactacaacacagtatcagcaaactccaattttaaatggacaaaaaatctgaataaacatttcactaagatacatgaatggctgaagagcacataaaagatgctttgacattattcgccatcaggaaaatcaaagttaaaaccacaaaggaatatcatttcaaacgctaggatgggcataatttttaaaaaacagacaacaatgactggcaagactgtagagaaatgggaagccccacacattactagtcagaatgtaaaataatgcggtcactttggaaaacaatttggcagtttcctaaaaaagttaaatgaaaatttaccgtatgacctagcaactcccctcaggcatctgcctaagaaaaatgaaaacatgtccacacaaagacttgtacactaacgttcaaaacacttgcataccaatgttcaaagcagcattattcctaacaggcaaaaactggaaaaacctcaaatgttcttcaactagtgaatgcacgaagcatccacataatgtaatattatttatgataaaaaggaataaagtactagtatgttacaacatggatgaacttaaaacacattaatgaaaaaaacacagaaagatcacatataacataaaatgtacagaaaaagacaactctagagacacaaagtcgactgagtagtgggtgcctgggattagaggttggacgggagattaactgtaaactggaataacggatcttgctgggatgatgttctaaaaaatggattatggtaatggttgcacaactcagcatatttactaaaactcactgaattgtacacttgaaatggttttaatgatatgtaatttgtacctcaataaattcctttaaaaaaaaagtttatactccagattcccaatggatactgggataaaacattgttatgaatgttagggagtctaagagtaatcatcttggaacaagcctcttctgaagacttttacgttatttcttcaactttctataaattatatttttcagaaaacaaaacttacaacaagttttctgtcttttcagaaaaaaacttaaaaccattatgaatgattctcataataaacattcctttcatggctaggatgtgattcgttggtctgcttagcaataactatgcggaccaatttatcacacggcaatatttaaactgcaggcttggggttggggaggcaccaaaaaccttctcccagaggtagcatttcacacctacatacattagtcacagtaaatgttcctgagtctaagattagcattaaggatcgctttacttccataagtgaagagttttctggtttagctctctttttataggaggtgcccacaatttcaactttaggaacttatttctagaccactgttgagtccatggggttcctccagaaccctatgacctgaagccaaaacctcactcattcagggccttaagttcctttttcagttggaaattattattcagactccaccaatgaaatttataaggaataatccaccaatacccgtatattccattcctctgaggtctaatttcacaaaagaaaacttaactgaaaattttttctgtatcaattctacattcattccctgaactttacttgctatcagtgcagtctctttagattttagggtatctattctccaaatggtaggggttataatagaacattcatacagtgggaaagtcaggtgacatacatgagagaactagctaagtcagaaagttgattccccatcaaaaggtggcagctgctacccaggaccagctgagtgctttacataaataaaagcccagtgttgttagcccttataattttttttaagacaagctttgtttttagtatgaaatgccctaattttagatagtggcaacaatgtatacacacacacacacacacacacacatgcacacacacccaagcaaattgttataacagcttttaactgttgccacacagaatgtttacactccaattgcaaaaaaatgtacttgctacaggcaaaattgttttaaagtagaatttttgcaaaccaaaatccatccagaatagctctgtcttcagcacatttccttacccccagcccccatctattttcctaggactgttactctcacggctgagatggctcaggtgcaagctctctggcttctcagtcctgttggccaatgcccaaaagaaaaagagttcccttgtccgattaaaatactccctcaaggaaaagtcgtttgaacttcactgacccattcctagttacagcatttgagggattcctgcacgaagttttcaaaaagtatactgcattctcactaagctagaagtccagcatcctaggaaccaggcttgatggagtgtacccgtaatgtcagctactcaggaaagtgagatggaaggatcacttgagcccaggagttcaagaccagtctgggcaacatagtgagactccatcccaaaaaagaaaaattgaaaaaaaaaaaagaaaaaaaaaagaaaagaagtccagcatcctgaatagtggtattgtattttttactagagaaacttgaaagtaatgacaaataaaaaaaaataacttatgtccacagcttcagagattatcaggataccaataaaaaactaaaaaaccaaaaaaggcaaaaatcattaatcccatcccttcattctgctggtgacgaaaataaaattctgaaaggtcaaatgacttgtccaaggtgtatacagcaagttggttggcaaactgggacagaatccaagttatgtgactgcagtcaagttctctccatcacactacatggtagtagaagaaatcagagagaaatcccctgaagaaaagagcttttccaattcgtctggcctcagaatcattttgcattcttccctttccagtgactttaccaactaattactgtttaccagtcgttgccatccttgaaaagaagagggatgaatgggcaaaaggatatttttcctaactgccaatttacgaaagctgcagctactgatcaatactgtaagtttacatcccagggtttcagtaactgacaatttgaattaaattccccccactttaatgtagttccaggattactctgcagagtgaaatccccgatgtctaatgaggcctgaattacttttaaatgtcttctcacattcgttacattcatattctctccttccggtatgaatttttaggtgttctacaaggattgagcttcgactaaaggttgcaccacaatagttacactcatagggtttctctcctgtatgaattcggtggtgctcattaagagatgaactctgactgaaggacttcccacattctttacatttataaggttttacaccagtatgaattctctgatgacgacttagcagtgaatgggttgggaaggctttctcacactggttacatttgtagggtttttctcctgaatgaagtctttgatgataaatcacagacgtaaaatggctaaaagtcattccgcaatcattacacaaatatggtttttctccagtgtgaattctctgatgccgggtaaggcatgaattctgcctaaaggcttttccacattcgccacatttatagggtttctctccagtatgaattctctgatgtttggaaagggatgagctatgactgaaggattttccacaattgctacatgtatagggtttttctccagtatgaattcgctgatgttgaataagagatgaactgtcactaaagggtctcccacagtctttacatttataaggtttttctccagtatgaattctctgatgtttaatgaggtgagcacttagggtgaaacctttcccacagtcatcacatttgaagggtttctctccactatgagttctatgatgtggtgtgagcgatgaactatcactaaaagcttttccacattcattacacatatagggtttttctccagtgtgaattctccgatgtttggtgagtgaggcgctatagccaaaggcttttccacacttactacatttatgagttttttctccactctcatttccctcatctttatttaaggctgcttcttgacatgaatctttccgacatttctcacacataggggtttttctcctagaaagagttgatcttctaataaagattatcccacacttactgcatttttgggacctatcccccaaatgaatcttctgacgtttctgatgttcagtaagagctgaagagtgactcaggactttcccaccatcattagatttccgtgacttttctccggcggttttctccttgcggttcagaacaaggtctgaatgaaaactgaagggtttcttgctttcattatacctccgagatttcttcctcaagtagactctcagatgtttaattaagtctgaagtttctttgaaattatgtccaaaggggcttttatctgggtcaaatttcttacccctactgccactcccaagagttttgttttgtgcgactcttccttttgaatttccctgattaccgtgatcctcctctgagctgccacaatattgctgggattcttccatcaagccatgatcatcatccctgaggcacctttctattattttatctaaagctgattcatctagtcgggagctttttgagacttcttccagcagccatggcaattcaacccactttagctgggaaatcaactctaattttgaaactggaaagtccagaaattctaggttcctgaggttttccagtagcacttccttatatagctccttttgaaaaggctccagcttcttccactctcctcttgaaaagttcacagctacatccttcaatgttatagattcacaggactcagtattgggacaaacagtgaccattttatcctcttttgagttctcctcttgggaaacagtagaatcttgagagactggatctttttcttcaagcatctgggtcaaatcttctattagggtcaccacttcctcactactctcaggatgttgtgactttacccaaatcctgatctccccaggcaaaatggtcaggaactgctcaaacaccagaagctctaaaatctgttctttcgtgtgaatgtctggtctcagccactgattgcagagctcccagagttgactcagagctttcctgggtccagctacttctgagtaacaaaaccacctaaacctctgtctgaaagactctgcatcagcagcatttcctcttaaaatagcttcttgttccccagaagtaaccactcttgggacctcattttgttcagtcgaggccagagtttgaggttctggtgagatggctgtcatcttgttcaagggcactacagcttgcattgtgtctcaggggcaggaatccagtcccttcacactctagttgagtatcagtacagtccaccaacaggcactatacacagccaggaatatcaaaggttccaggaatccagtttacagtcctgcagaaactggcgccgtgctgagcacctggggctccgcgatgactaagacactcggctccgtctacagggagtttacataggaggcccggtgaaaatgtgacgcagccagaggatctgcatcagcatccgcaaacagcaccaacgccaccgcaaagagcttccagaagcttgtcccgcagcgagtgcgcgcgcaagcctgcgggaaccac

SEQ ID NO: 8690 - RNA, 2782 nt, Homo sapiens
  source 1..2782: mol_type = other RNA
aactctagcctgagcaacagagcaagactccatctcaaaaaaaagtgcaagataatgaatttggggtaaataattcacagtcaagagctctgagcacttggattcaaaaagagagcatgagggacattaaatatggttctccctggaaatgttggtccactgtactgatgtgggctgagagagccaaccaaatccaagtggggttttgtcaggaacggtattggaaactctgaactagataaataattcaaaggatattagctaaagtgatcagggaccaggacaggaaggtactgttacaaacggagagaataaaagggcaaactgaaataatagatcctggaatagcacagacactgacctctgaccacagaccaaaagttagggcctagttgtatttcttagaaatacaaagaaaacaagtttagaatcatagaaaacactgttaacacattagcctgggaggtggtactggcactgaatatacacatacccataaagtcggatatgttcattaatcccagagttgactgataaaatgctgattaaagcaaaggtaggctatatgaggcagccacaccctcccaaaacatgtccccagagaccgggtggccttctttcttaaggctgtaatttatgcacagttaggagttactctctcatcctattaatatttaggatggctctcagctggctgattggagctaacacagaataggatcatacagattctgacatggtcccattttgcgttgttgaattatacatggaaagcaaaaccaggtttttttttttctctctttttcaggggaggtgggtgcagataagggtgggcagggcactgtatagggaggaaaaaaatactgatattgatgggtcttgggattgcaataagtcagtttaccatttaagaggaaaatttaaatattcagtggaatgaggcactcaaagggttgaaatgcgatttttctttggtttccagggacctgtccctgggctctcactccaaggttaagttccaaaactatactttttggctcacagggctctctgtgatgctctggtgccagctgtgtactcttgagtggttaggcagcagttcacattagatgtgtaaaattaattaaacctaaatctctaggctcaagtccaggatgtccccagactagttcagaaactaagtgctctctcctccccttaaaaaggtgttggcaaatgcaggtctccaaggaagtacgtggcctcaatgggagatgcccagagactgcaacaggtgaaaggtggcccccaaggcccagcccgtctctatgttgttcactttctttgtgagctgtaagactgtgctgtctgcaaagccaaagccatcctttaacagggctgtgatgtagctgagatccatgcacaggaaaggactgcctgaggtgaagttttccaagttatcacacacttccctggcttttctttcaaaatcttcaacttttaaaataccccccttttcataatcaatcatgtctgtgtcaacagctcggtcataatagtaagagaaagcatagaaggaacctctctggacctcctctggctggtgaagttttcctcgtaccaccctcagcacttcggcatagcagggctcaaagcccacctccccttcttggttgccaccatactggtatttcacacccccaaagatccactctgcttccaaccatctcggtaaacaggcactccggaaagtgtgcccatcagtcccttctgtctccagggctcccagggttgctagtcttgcagctttcaatccaaatcccaggtaactatgtgtatagagcttataagtgctgttaaacatctcaaaggaagtgaggtagcccctaggagtttgttccagagttttctcaaactggggcaggaacgtgatttgggtggaggctccccctaggtccaaggtccccacagtctcctgtctgtggccatgcagctgacctgtcagaaaattcacagtaacccaagctaatatgccttcgtcggatccatccatgatgctaacactgccctttggtaccaggaaaggtgacttcctgaagatctcctttacctcaaagagcagagccttggctttgtgttctggcagtaagcgtagtcctgctgttgcctttaggaccactggggtctttttccagtgacttcgggggattgagtctttggccacctctaagagcccttgaacggtctcagcaccctgcttaggttgatctacaaaagcagaaagtcctggcttcacagaatcaaaaacttccccttctagaattggaagctgtcctggcattttctgcacaaaggtgtaaacatgaattcgagttccagtgctccctgcatcaaacataattccatacaaggtgctggcgctgacattgatggggcacatggaagacaggaagataccctcaaaccaagtctgctggttcctgtgggagacagcgctgcaaacacaggataccaccagcatgaaaaagactgtgccccaagaagtggccattcttttcccaagatgtggctgggtggaggcttttgttgcagaagcaatcctgctcgcacacctgcagaggcaattttttctttccttctgaattttctccttggttcctttattatatcactttttcaacctaacagcaccataatgatcttgtctgtatgaggattcagccaagacactccacatttctttgttgaccaggaacaaggaaaacgcgcgcgcgccacccttgcgcggcagcccgccgccctc

SEQ ID NO: 8691 - RNA, 2806 nt, Homo sapiens
  source 1..2806: mol_type = other RNA
aactctagcctgagcaacagagcaagactccatctcaaaaaaaagtgcaagataatgaatttggggtaaataattcacagtcaagagctctgagcacttggattcaaaaagagagcatgagggacattaaatatggttctccctggaaatgttggtccactgtactgatgtgggctgagagagccaaccaaatccaagtggggttttgtcaggaacggtattggaaactctgaactagataaataattcaaaggatattagctaaagtgatcagggaccaggacaggaaggtactgttacaaacggagagaataaaagggcaaactgaaataatagatcctggaatagcacagacactgacctctgaccacagaccaaaagttagggcctagttgtatttcttagaaatacaaagaaaacaagtttagaatcatagaaaacactgttaacacattagcctgggaggtggtactggcactgaatatacacatacccataaagtcggatatgttcattaatcccagagttgactgataaaatgctgattaaagcaaaggtaggctatatgaggcagccacaccctcccaaaacatgtccccagagaccgggtggccttctttcttaaggctgtaatttatgcacagttaggagttactctctcatcctattaatatttaggatggctctcagctggctgattggagctaacacagaataggatcatacagattctgacatggtcccattttgcgttgttgaattatacatggaaagcaaaaccaggtttttttttttctctctttttcaggggaggtgggtgcagataagggtgggcagggcactgtatagggaggaaaaaaatactgatattgatgggtcttgggattgcaataagtcagtttaccatttaagaggaaaatttaaatattcagtggaatgaggcactcaaagggttgaaatgcgatttttctttggtttccagggacctgtccctgggctctcactccaaggttaagttccaaaactatactttttggctcacagggctctctgtgatgctctggtgccagctgtgtactcttgagtggttaggcagcagttcacattagatgtgtaaaattaattaaacctaaatctctaggctcaagtccaggatgtccccagactagttcagaaactaagtgctctctcctccccttaaaaaggtgttggcaaatgcaggtctccaaggaagtacgtggcctcaatgggagatgcccagagactgcaacaggtgaaaggtggcccccaaggcccagcccgtctctatgttgttcactttctttgtgagctgtaagactgtgctgtctgcaaagccaaagccatcctttaacagggctgtgatgtagctgagatccatgcacaggaaaggactgcctgaggtgaagttttccaagttatcacacacttccctggcttttctttcaaaatcttcaacttttaaaataccccccttttcataatcaatcatgtctgtgtcaacagctcggtcataatagtaagagaaagcatagaaggaacctctctggacctcctctggctggtgaagttttcctcgtaccaccctcagcacttcggcatagcagggctcaaagcccacctccccttcttggttgccaccatactggtatttcacacccccaaagatccactctgcttccaaccatctcggtaaacaggcactccggaaagtgtgcccatcagtcccttctgtctccagggctcccagggttgctagtcttgcagctttcaatccaaatcccaggtaactatgtgtatagagcttataagtgctgttaaacatctcaaaggaagtgaggtagcccctaggagtttgttccagagttttctcaaactggggcaggaacgtgatttgggtggaggctccccctaggtccaaggtccccacagtctcctgtctgtggccatgcagctgacctgtcagaaaattcacagtaacccaagctaatatgccttcgtcggatccatccatgatgctaacactgccctttggtaccaggaaaggtgacttcctgaagatctcctttacctcaaagagcagagccttggctttgtgttctggcagtaagcgtagtcctgctgttgcctttaggaccactggggtctttttccagtgacttcgggggattgagtctttggccacctctaagagcccttgaacggtctcagcaccctgcttaggttgatctacaaaagcagaaagtcctggcttcacagaatcaaaaacttccccttctagaattggaagctgtcctggcattttctgcacaaaggtgtaaacatgaattcgagttccagtgctccctgcatcaaacataattccatacaaggtgctggcgctgacattgatggggcacatggaagacaggaagataccctcaaaccaagtctgctggttcctgtgggagacagcgctgcaaacacaggataccaccagcatgaaaaagactgtgccccaagaagtggccattcttttcccaagatgtggctgggtggaggcttttgttgcagaagcaatcctgctcgcacacctgcagaggcaattttttctttccttctgaattttctccttggttcctttattatatcactttttcaaccttacatctggatacaagtcctacctaacagcaccataatgatcttgtctgtatgaggattcagccaagacactccacatttctttgttgaccaggaacaaggaaaacgcgcgcgcgccacccttgcgcggcagcccgccgccctc

SEQ ID NO: 8692 - RNA, 3582 nt, Homo sapiens
  source 1..3582: mol_type = other RNA
aactctagcctgagcaacagagcaagactccatctcaaaaaaaagtgcaagataatgaatttggggtaaataattcacagtcaagagctctgagcacttggattcaaaaagagagcatgagggacattaaatatggttctccctggaaatgttggtccactgtactgatgtgggctgagagagccaaccaaatccaagtggggttttgtcaggaacggtattggaaactctgaactagataaataattcaaaggatattagctaaagtgatcagggaccaggacaggaaggtactgttacaaacggagagaataaaagggcaaactgaaataatagatcctggaatagcacagacactgacctctgaccacagaccaaaagttagggcctagttgtatttcttagaaatacaaagaaaacaagtttagaatcatagaaaacactgttaacacattagcctgggaggtggtactggcactgaatatacacatacccataaagtcggatatgttcattaatcccagagttgactgataaaatgctgattaaagcaaaggtaggctatatgaggcagccacaccctcccaaaacatgtccccagagaccgggtggccttctttcttaaggctgtaatttatgcacagttaggagttactctctcatcctattaatatttaggatggctctcagctggctgattggagctaacacagaataggatcatacagattctgacatggtcccattttgcgttgttgaattatacatggaaagcaaaaccaggtttttttttttctctctttttcaggggaggtgggtgcagataagggtgggcagggcactgtatagggaggaaaaaaatactgatattgatgggtcttgggattgcaataagtcagtttaccatttaagaggaaaatttaaatattcagtggaatgaggcactcaaagggttgaaatgcgatttttctttggtttccagggacctgtccctgggctctcactccaaggttaagttccaaaactatactttttggctcacagggctctctgtgatgctctggtgccagctgtgtactcttgagtggttaggcagcagttcacattagatgtgtaaaattaattaaacctaaatctctaggctcaagtccaggatgtccccagactagttcagaaactaagtgctctctcctccccttaaaaaggtgttggcaaatgcaggtctccaaggaagtacgtggcctcaatgggagatgcccagagactgcaacaggtgaaaggtggcccccaaggcccagcccgtctctatgttgttcactttctttgtgagctgtaagactgtgctgtctgcaaagccaaagccatcctttaacagggctgtgatgtagctgagatccatgcacaggaaaggactgcctgaggtgaagttttccaagttatcacacacttccctggcttttctttcaaaatcttcaacttttaaaataccccccttttcataatcaatcatgtctgtgtcaacagctcggtcataatagtaagagaaagcatagaaggaacctctctggacctcctctggctggtgaagttttcctcgtaccaccctcagcacttcggcatagcagggctcaaagcccacctccccttcttggttgccaccatactggtatttcacacccccaaagatccactctgcttccaaccatctcggtaaacaggcactccggaaagtgtgcccatcagtcccttctgtctccagggctcccagggttgctagtcttgcagctttcaatccaaatcccaggtaactatgtgtatagagcttataagtgctgttaaacatctcaaaggaagtgaggtagcccctaggagtttgttccagagttttctcaaactggggcaggaacgtgatttgggtggaggctccccctaggtccaaggtccccacagtctcctgtctgtggccatgcagctgacctgtcagaaaattcacagtaacccaagctaatatgccttcgtcggatccatccatgatgctaacactgccctttggtaccaggaaaggtgacttcctgaagatctcctttacctcaaagagcagagccttggctttgtgttctggcagtaagcgtagtcctgctgttgcctttaggaccactggggtctttttccagtgacttcgggggattgagtctttggccacctctaagagcccttgaacggtctcagcaccctgcttaggttgatctacaaaagcagaaagtcctggcttcacagaatcaaaaacttccccttctagaattggaagctgtcctggcattttctgcacaaaggtgtaaacatgaattcgagttccagtgctccctgcatcaaacataattccatacaaggtgctggcgctgacattgatggggcacatggaagacaggaagataccctcaaaccaagtctgctggttcctgtgggagacagcgctgcaaacacaggataccaccagcatgaaaaagactgtgccccaagaagtggccattcttttcccaagatgtggctgggtggaggcttttgttgcagaagcaatcctgctcgcacacctgcagaggcaattttttctttccttctgaattttctccttggttcctttattatatcactttttcaaccttacatctggatacaagtcctacctaacagcaccataatgatcttgtctgtatgaggattcagccaagacactccacatttctttgttgaccaggaacaaggaaaacttccttaatgactcactgactgactctcattgaaaaatgagaatacttgtgagtacactccttttcagaggtgtattcgggatttcaggagtcggggaggcaagttgaagagcttccaactttatgcaactttcaggaaagaaggctgcggaccggtattagcaaatggaaatccggggggcggtcgtgggcaggaagtatcggccacacaggacctagtgaggccgaggaccctgctcccgacctcggtggcagcactcccctccccgcccggctccctggcgtgccgctgctcttcggaggctggcagcctcgccctcaaccaccgccctcgggaaagtcctcgactgcctatcaaaaaacatttggcctgggacgtccgctggctgcactatcccttacagaatcagcaagggtgaaaagccaggaaagagatgcaacccaaaggagtaaggcagtgccgggagcggcagaagcggagcgggggcgagggcaaggtagccgcggccacgctggctgcggcatggagacacgggaggaacgggacccgcgggcggcacgggaaagggctgcggctcagaccactgcggcgggacgggcggatcagcggggatctaagtctcctgaggcaagggcgccccgaccgcagcgactcctgacacacccaggccgcaggacgaagcgctaccgcctggggctgccagctcccgcctcccgcccgcagagcccgggccccacgtagaggatccggcgccgccgacactcgcacactcaccgcgcgcgcgccacccttgcgcggcagcccgccgccctc

SEQ ID NO: 8693 - RNA, 2903 nt, Homo sapiens
  source 1..2903: mol_type = other RNA
aactctagcctgagcaacagagcaagactccatctcaaaaaaaagtgcaagataatgaatttggggtaaataattcacagtcaagagctctgagcacttggattcaaaaagagagcatgagggacattaaatatggttctccctggaaatgttggtccactgtactgatgtgggctgagagagccaaccaaatccaagtggggttttgtcaggaacggtattggaaactctgaactagataaataattcaaaggatattagctaaagtgatcagggaccaggacaggaaggtactgttacaaacggagagaataaaagggcaaactgaaataatagatcctggaatagcacagacactgacctctgaccacagaccaaaagttagggcctagttgtatttcttagaaatacaaagaaaacaagtttagaatcatagaaaacactgttaacacattagcctgggaggtggtactggcactgaatatacacatacccataaagtcggatatgttcattaatcccagagttgactgataaaatgctgattaaagcaaaggtaggctatatgaggcagccacaccctcccaaaacatgtccccagagaccgggtggccttctttcttaaggctgtaatttatgcacagttaggagttactctctcatcctattaatatttaggatggctctcagctggctgattggagctaacacagaataggatcatacagattctgacatggtcccattttgcgttgttgaattatacatggaaagcaaaaccaggtttttttttttctctctttttcaggggaggtgggtgcagataagggtgggcagggcactgtatagggaggaaaaaaatactgatattgatgggtcttgggattgcaataagtcagtttaccatttaagaggaaaatttaaatattcagtggaatgaggcactcaaagggttgaaatgcgatttttctttggtttccagggacctgtccctgggctctcactccaaggttaagttccaaaactatactttttggctcacagggctctctgtgatgctctggtgccagctgtgtactcttgagtggttaggcagcagttcacattagatgtgtaaaattaattaaacctaaatctctaggctcaagtccaggatgtccccagactagttcagaaactaagtgctctctcctccccttaaaaaggtgttggcaaatgcaggtctccaaggaagtacgtggcctcaatgggagatgcccagagactgcaacaggtgaaaggtggcccccaaggcccagcccgtctctatgttgttcactttctttgtgagctgtaagactgtgctgtctgcaaagccaaagccatcctttaacagggctgtgatgtagctgagatccatgcacaggaaaggactgcctgaggtgaagttttccaagttatcacacacttccctggcttttctttcaaaatcttcaacttttaaaataccccccttttcataatcaatcatgtctgtgtcaacagctcggtcataatagtaagagaaagcatagaaggaacctctctggacctcctctggctggtgaagttttcctcgtaccaccctcagcacttcggcatagcagggctcaaagcccacctccccttcttggttgccaccatactggtatttcacacccccaaagatccactctgcttccaaccatctcggtaaacaggcactccggaaagtgtgcccatcagtcccttctgtctccagggctcccagggttgctagtcttgcagctttcaatccaaatcccaggtaactatgtgtatagagcttataagtgctgttaaacatctcaaaggaagtgaggtagcccctaggagtttgttccagagttttctcaaactggggcaggaacgtgatttgggtggaggctccccctaggtccaaggtccccacagtctcctgtctgtggccatgcagctgacctgtcagaaaattcacagtaacccaagctaatatgccttcgtcggatccatccatgatgctaacactgccctttggtaccaggaaaggtgacttcctgaagatctcctttacctcaaagagcagagccttggctttgtgttctggcagtaagcgtagtcctgctgttgcctttaggaccactggggtctttttccagtgacttcgggggattgagtctttggccacctctaagagcccttgaacggtctcagcaccctgcttaggttgatctacaaaagcagaaagtcctggcttcacagaatcaaaaacttccccttctagaattggaagctgtcctggcattttctgcacaaaggtgtaaacatgaattcgagttccagtgctccctgcatcaaacataattccatacaaggtgctggcgctgacattgatggggcacatggaagacaggaagataccctcaaaccaagtctgctggttcctgtgggagacagcgctgcaaacacaggataccaccagcatgaaaaagactgtgccccaagaagtggccattcttttcccaagatgtggctgggtggaggcttttgttgcagaagcaatcctgctcgcacacctgcagaggctccaagatggctcactcaatggttggcaagttgatgccagctgtgggcaggaagtctcagtagctccccgtgtagatcctccatagggctgcttgaatgtctttataacccagtggctggcaattttttctttccttctgaattttctccttggttcctttattatatcactttttcaacctaacagcaccataatgatcttgtctgtatgaggattcagccaagacactccacatttctttgttgaccaggaacaaggaaaacgcgcgcgcgccacccttgcgcggcagcccgccgccctc

SEQ ID NO: 8694 - RNA, 2718 nt, Homo sapiens
  source 1..2718: mol_type = other RNA
aactctagcctgagcaacagagcaagactccatctcaaaaaaaagtgcaagataatgaatttggggtaaataattcacagtcaagagctctgagcacttggattcaaaaagagagcatgagggacattaaatatggttctccctggaaatgttggtccactgtactgatgtgggctgagagagccaaccaaatccaagtggggttttgtcaggaacggtattggaaactctgaactagataaataattcaaaggatattagctaaagtgatcagggaccaggacaggaaggtactgttacaaacggagagaataaaagggcaaactgaaataatagatcctggaatagcacagacactgacctctgaccacagaccaaaagttagggcctagttgtatttcttagaaatacaaagaaaacaagtttagaatcatagaaaacactgttaacacattagcctgggaggtggtactggcactgaatatacacatacccataaagtcggatatgttcattaatcccagagttgactgataaaatgctgattaaagcaaaggtaggctatatgaggcagccacaccctcccaaaacatgtccccagagaccgggtggccttctttcttaaggctgtaatttatgcacagttaggagttactctctcatcctattaatatttaggatggctctcagctggctgattggagctaacacagaataggatcatacagattctgacatggtcccattttgcgttgttgaattatacatggaaagcaaaaccaggtttttttttttctctctttttcaggggaggtgggtgcagataagggtgggcagggcactgtatagggaggaaaaaaatactgatattgatgggtcttgggattgcaataagtcagtttaccatttaagaggaaaatttaaatattcagtggaatgaggcactcaaagggttgaaatgcgatttttctttggtttccagggacctgtccctgggctctcactccaaggttaagttccaaaactatactttttggctcacagggctctctgtgatgctctggtgccagctgtgtactcttgagtggttaggcagcagttcacattagatgtgtaaaattaattaaacctaaatctctaggctcaagtccaggatgtccccagactagttcagaaactaagtgctctctcctccccttaaaaaggtgttggcaaatgcaggtctccaaggaagtacgtggcctcaatgggagatgcccagagactgcaacaggtgaaaggtggcccccaaggcccagcccgtctctatgttgttcactttctttgtgagctgtaagactgtgctgtctgcaaagccaaagccatcctttaacagggctgtgatgtagctgagatccatgcacaggaaaggactgcctgaggtgaagttttccaagttatcacacacttccctggcttttctttcaaaatcttcaacttttaaaataccccccttttcataatcaatcatgtctgtgtcaacagctcggtcataatagtaagagaaagcatagaaggaacctctctggacctcctctggctggtgaagttttcctcgtaccaccctcagcacttcggcatagcagggctcaaagcccacctccccttcttggttgccaccatactggtatttcacacccccaaagatccactctgcttccaaccatctcggtaaacaggcactccggaaagtgtgcccatcagtcccttctgtctccagggctcccagggttgctagtcttgcagctttcaatccaaatcccaggtaactatgtgtatagagcttataagtgctgttaaacatctcaaaggaagtgaggtagcccctaggagtttgttccagagttttctcaaactggggcaggaacgtgatttgggtggaggctccccctaggtccaaggtccccacagtctcctgtctgtggccatgcagctgacctgtcagaaaattcacagtaacccaagctaatatgccttcgtcggatccatccatgatgctaacactgccctttggtaccaggaaaggtgacttcctgaagatctcctttacctcaaagagcagagccttggctttgtgttctggcagtaagcgtagtcctgctgttgcctttaggaccactggggtctttttccagtgacttcgggggattgagtctttggccacctctaagagcccttgaacggtctcagcaccctgcttaggttgatctacaaaagcagaaagtcctggcttcacagaatcaaaaacttccccttctagaattggaagctgtcctggcattttctgcacaaaggtgtaaacatgaattcgagttccagtgctccctgcatcaaacataattccatacaaggtgctggcgctgacattgatggggcacatggaagacaggaagataccctcaaaccaagtctgctggttcctgtgggagacagcgctgcaaacacaggataccaccagcatgaaaaagactgtgccccaagaagtggccattcttttcccaagatgtggctgggtggaggcttttgttgcagaagcaatcctgctcgcacacctgcagaggctgcttgtgtctgccggttccctgagtccttgctttcgctgcaggttgccttttgctctttgctcctgtttcagctcttcttaatcaagcgagcctcatgaaccgcattcacctttgt

SEQ ID NO: 8695 - RNA, 2923 nt, Homo sapiens
  source 1..2923: mol_type = other RNA
aactctagcctgagcaacagagcaagactccatctcaaaaaaaagtgcaagataatgaatttggggtaaataattcacagtcaagagctctgagcacttggattcaaaaagagagcatgagggacattaaatatggttctccctggaaatgttggtccactgtactgatgtgggctgagagagccaaccaaatccaagtggggttttgtcaggaacggtattggaaactctgaactagataaataattcaaaggatattagctaaagtgatcagggaccaggacaggaaggtactgttacaaacggagagaataaaagggcaaactgaaataatagatcctggaatagcacagacactgacctctgaccacagaccaaaagttagggcctagttgtatttcttagaaatacaaagaaaacaagtttagaatcatagaaaacactgttaacacattagcctgggaggtggtactggcactgaatatacacatacccataaagtcggatatgttcattaatcccagagttgactgataaaatgctgattaaagcaaaggtaggctatatgaggcagccacaccctcccaaaacatgtccccagagaccgggtggccttctttcttaaggctgtaatttatgcacagttaggagttactctctcatcctattaatatttaggatggctctcagctggctgattggagctaacacagaataggatcatacagattctgacatggtcccattttgcgttgttgaattatacatggaaagcaaaaccaggtttttttttttctctctttttcaggggaggtgggtgcagataagggtgggcagggcactgtatagggaggaaaaaaatactgatattgatgggtcttgggattgcaataagtcagtttaccatttaagaggaaaatttaaatattcagtggaatgaggcactcaaagggttgaaatgcgatttttctttggtttccagggacctgtccctgggctctcactccaaggttaagttccaaaactatactttttggctcacagggctctctgtgatgctctggtgccagctgtgtactcttgagtggttaggcagcagttcacattagatgtgtaaaattaattaaacctaaatctctaggctcaagtccaggatgtccccagactagttcagaaactaagtgctctctcctccccttaaaaaggtgttggcaaatgcaggtctccaaggaagtacgtggcctcaatgggagatgcccagagactgcaacaggtgaaaggtggcccccaaggcccagcccgtctctatgttgttcactttctttgtgagctgtaagactgtgctgtctgcaaagccaaagccatcctttaacagggctgtgatgtagctgagatccatgcacaggaaaggactgcctgaggtgaagttttccaagttatcacacacttccctggcttttctttcaaaatcttcaacttttaaaataccccccttttcataatcaatcatgtctgtgtcaacagctcggtcataatagtaagagaaagcatagaaggaacctctctggacctcctctggctggtgaagttttcctcgtaccaccctcagcacttcggcatagcagggctcaaagcccacctccccttcttggttgccaccatactggtatttcacacccccaaagatccactctgcttccaaccatctcggtaaacaggcactccggaaagtgtgcccatcagtcccttctgtctccagggctcccagggttgctagtcttgcagctttcaatccaaatcccaggtaactatgtgtatagagcttataagtgctgttaaacatctcaaaggaagtgaggtagcccctaggagtttgttccagagttttctcaaactggggcaggaacgtgatttgggtggaggctccccctaggtccaaggtccccacagtctcctgtctgtggccatgcagctgacctgtcagaaaattcacagtaacccaagctaatatgccttcgtcggatccatccatgatgctaacactgccctttggtaccaggaaaggtgacttcctgaagatctcctttacctcaaagagcagagccttggctttgtgttctggcagtaagcgtagtcctgctgttgcctttaggaccactggggtctttttccagtgacttcgggggattgagtctttggccacctctaagagcccttgaacggtctcagcaccctgcttaggttgatctacaaaagcagaaagtcctggcttcacagaatcaaaaacttccccttctagaattggaagctgtcctggcattttctgcacaaaggtgtaaacatgaattcgagttccagtgctccctgcatcaaacataattccatacaaggtgctggcgctgacattgatggggcacatggaagacaggaagataccctcaaaccaagtctgctggttcctgtgggagacagcgctgcaaacacaggataccaccagcatgaaaaagactgtgccccaagaagtggccattcttttcccaagatgtggctgggtggaggcttttgttgcagaagcaatcctgctcgcacacctgcagaggctgtagtctcagctactcgggagggtgaggcaggaggatcgcttgagcccaggagtttgaagctgccgtgagctgtgattgcaccactgtactccagcctcggtgacagagtgagaccaattttttctttccttctgaattttctccttggttcctttattatatcactttttcaaccttacatctggatacaagtcctacctaacagcaccataatgatcttgtctgtatgaggattcagccaagacactccacatttctttgttgaccaggaacaaggaaaacgcgcgcgcgccacccttgcgcggcagcccgccgccctc

SEQ ID NO: 8696 - RNA, 2933 nt, Homo sapiens
  source 1..2933: mol_type = other RNA
aactctagcctgagcaacagagcaagactccatctcaaaaaaaagtgcaagataatgaatttggggtaaataattcacagtcaagagctctgagcacttggattcaaaaagagagcatgagggacattaaatatggttctccctggaaatgttggtccactgtactgatgtgggctgagagagccaaccaaatccaagtggggttttgtcaggaacggtattggaaactctgaactagataaataattcaaaggatattagctaaagtgatcagggaccaggacaggaaggtactgttacaaacggagagaataaaagggcaaactgaaataatagatcctggaatagcacagacactgacctctgaccacagaccaaaagttagggcctagttgtatttcttagaaatacaaagaaaacaagtttagaatcatagaaaacactgttaacacattagcctgggaggtggtactggcactgaatatacacatacccataaagtcggatatgttcattaatcccagagttgactgataaaatgctgattaaagcaaaggtaggctatatgaggcagccacaccctcccaaaacatgtccccagagaccgggtggccttctttcttaaggctgtaatttatgcacagttaggagttactctctcatcctattaatatttaggatggctctcagctggctgattggagctaacacagaataggatcatacagattctgacatggtcccattttgcgttgttgaattatacatggaaagcaaaaccaggtttttttttttctctctttttcaggggaggtgggtgcagataagggtgggcagggcactgtatagggaggaaaaaaatactgatattgatgggtcttgggattgcaataagtcagtttaccatttaagaggaaaatttaaatattcagtggaatgaggcactcaaagggttgaaatgcgatttttctttggtttccagggacctgtccctgggctctcactccaaggttaagttccaaaactatactttttggctcacagggctctctgtgatgctctggtgccagctgtgtactcttgagtggttaggcagcagttcacattagatgtgtaaaattaattaaacctaaatctctaggctcaagtccaggatgtccccagactagttcagaaactaagtgctctctcctccccttaaaaaggtgttggcaaatgcaggtctccaaggaagtacgtggcctcaatgggagatgcccagagactgcaacaggtgaaaggtggcccccaaggcccagcccgtctctatgttgttcactttctttgtgagctgtaagactgtgctgtctgcaaagccaaagccatcctttaacagggctgtgatgtagctgagatccatgcacaggaaaggactgcctgaggtgaagttttccaagttatcacacacttccctggcttttctttcaaaatcttcaacttttaaaataccccccttttcataatcaatcatgtctgtgtcaacagctcggtcataatagtaagagaaagcatagaaggaacctctctggacctcctctggctggtgaagttttcctcgtaccaccctcagcacttcggcatagcagggctcaaagcccacctccccttcttggttgccaccatactggtatttcacacccccaaagatccactctgcttccaaccatctcggtaaacaggcactccggaaagtgtgcccatcagtcccttctgtctccagggctcccagggttgctagtcttgcagctttcaatccaaatcccaggtaactatgtgtatagagcttataagtgctgttaaacatctcaaaggaagtgaggtagcccctaggagtttgttccagagttttctcaaactggggcaggaacgtgatttgggtggaggctccccctaggtccaaggtccccacagtctcctgtctgtggccatgcagctgacctgtcagaaaattcacagtaacccaagctaatatgccttcgtcggatccatccatgatgctaacactgccctttggtaccaggaaaggtgacttcctgaagatctcctttacctcaaagagcagagccttggctttgtgttctggcagtaagcgtagtcctgctgttgcctttaggaccactggggtctttttccagtgacttcgggggattgagtctttggccacctctaagagcccttgaacggtctcagcaccctgcttaggttgatctacaaaagcagaaagtcctggcttcacagaatcaaaaacttccccttctagaattggaagctgtcctggcattttctgcacaaaggtgtaaacatgaattcgagttccagtgctccctgcatcaaacataattccatacaaggtgctggcgctgacattgatggggcacatggaagacaggaagataccctcaaaccaagtctgctggttcctgtgggagacagcgctgcaaacacaggataccaccagcatgaaaaagactgtgccccaagaagtggccattcttttcccaagatgtggctgggtggaggcttttgttgcagaagcaatcctgctcgcacacctgcagaggtggagaaaacagggctgggcacagtggctcttgtctgtaatcttagcactttggaaggtcgaggcaggaggattacttgaggtcaggatttcaagaccaccttgggcaacacagtgaagctctgtctcaattttttctttccttctgaattttctccttggttcctttattatatcactttttcaaccttacatctggatacaagtcctacctaacagcaccataatgatcttgtctgtatgaggattcagccaagacactccacatttctttgttgaccaggaacaaggaaaacgcgcgcgcgccacccttgcgcggcagcccgccgccctc

SEQ ID NO: 8697 - RNA, 3050 nt, Homo sapiens
  source 1..3050: mol_type = other RNA
aactctagcctgagcaacagagcaagactccatctcaaaaaaaagtgcaagataatgaatttggggtaaataattcacagtcaagagctctgagcacttggattcaaaaagagagcatgagggacattaaatatggttctccctggaaatgttggtccactgtactgatgtgggctgagagagccaaccaaatccaagtggggttttgtcaggaacggtattggaaactctgaactagataaataattcaaaggatattagctaaagtgatcagggaccaggacaggaaggtactgttacaaacggagagaataaaagggcaaactgaaataatagatcctggaatagcacagacactgacctctgaccacagaccaaaagttagggcctagttgtatttcttagaaatacaaagaaaacaagtttagaatcatagaaaacactgttaacacattagcctgggaggtggtactggcactgaatatacacatacccataaagtcggatatgttcattaatcccagagttgactgataaaatgctgattaaagcaaaggtaggctatatgaggcagccacaccctcccaaaacatgtccccagagaccgggtggccttctttcttaaggctgtaatttatgcacagttaggagttactctctcatcctattaatatttaggatggctctcagctggctgattggagctaacacagaataggatcatacagattctgacatggtcccattttgcgttgttgaattatacatggaaagcaaaaccaggtttttttttttctctctttttcaggggaggtgggtgcagataagggtgggcagggcactgtatagggaggaaaaaaatactgatattgatgggtcttgggattgcaataagtcagtttaccatttaagaggaaaatttaaatattcagtggaatgaggcactcaaagggttgaaatgcgatttttctttggtttccagggacctgtccctgggctctcactccaaggttaagttccaaaactatactttttggctcacagggctctctgtgatgctctggtgccagctgtgtactcttgagtggttaggcagcagttcacattagatgtgtaaaattaattaaacctaaatctctaggctcaagtccaggatgtccccagactagttcagaaactaagtgctctctcctccccttaaaaaggtgttggcaaatgcaggtctccaaggaagtacgtggcctcaatgggagatgcccagagactgcaacaggtgaaaggtggcccccaaggcccagcccgtctctatgttgttcactttctttgtgagctgtaagactgtgctgtctgcaaagccaaagccatcctttaacagggctgtgatgtagctgagatccatgcacaggaaaggactgcctgaggtgaagttttccaagttatcacacacttccctggcttttctttcaaaatcttcaacttttaaaataccccccttttcataatcaatcatgtctgtgtcaacagctcggtcataatagtaagagaaagcatagaaggaacctctctggacctcctctggctggtgaagttttcctcgtaccaccctcagcacttcggcatagcagggctcaaagcccacctccccttcttggttgccaccatactggtatttcacacccccaaagatccactctgcttccaaccatctcggtaaacaggcactccggaaagtgtgcccatcagtcccttctgtctccagggctcccagggttgctagtcttgcagctttcaatccaaatcccaggtaactatgtgtatagagcttataagtgctgttaaacatctcaaaggaagtgaggtagcccctaggagtttgttccagagttttctcaaactggggcaggaacgtgatttgggtggaggctccccctaggtccaaggtccccacagtctcctgtctgtggccatgcagctgacctgtcagaaaattcacagtaacccaagctaatatgccttcgtcggatccatccatgatgctaacactgccctttggtaccaggaaaggtgacttcctgaagatctcctttacctcaaagagcagagccttggctttgtgttctggcagtaagcgtagtcctgctgttgcctttaggaccactggggtctttttccagtgacttcgggggattgagtctttggccacctctaagagcccttgaacggtctcagcaccctgcttaggttgatctacaaaagcagaaagtcctggcttcacagaatcaaaaacttccccttctagaattggaagctgtcctggcattttctgcacaaaggtgtaaacatgaattcgagttccagtgctccctgcatcaaacataattccatacaaggtgctggcgctgacattgatggggcacatggaagacaggaagataccctcaaaccaagtctgctggttcctgtgggagacagcgctgcaaacacaggataccaccagcatgaaaaagactgtgccccaagaagtggccattcttttcccaagatgtggctgggtggaggcttttgttgcagaagcaatcctgctcgcacacctgcagaggtggagaaaacagggctgggcacagtggctcttgtctgtaatcttagcactttggaaggtcgaggcaggaggattacttgaggtcaggatttcaagaccaccttgggcaacacagtgaagctctgtctctgtagtctcagctactcgggagggtgaggcaggaggatcgcttgagcccaggagtttgaagctgccgtgagctgtgattgcaccactgtactccagcctcggtgacagagtgagaccaattttttctttccttctgaattttctccttggttcctttattatatcactttttcaaccttacatctggatacaagtcctacctaacagcaccataatgatcttgtctgtatgaggattcagccaagacactccacatttctttgttgaccaggaacaaggaaaacgcgcgcgcgccacccttgcgcggcagcccgccgccctc

SEQ ID NO: 8698 - RNA, 2665 nt, Homo sapiens
  source 1..2665: mol_type = other RNA
aactctagcctgagcaacagagcaagactccatctcaaaaaaaagtgcaagataatgaatttggggtaaataattcacagtcaagagctctgagcacttggattcaaaaagagagcatgagggacattaaatatggttctccctggaaatgttggtccactgtactgatgtgggctgagagagccaaccaaatccaagtggggttttgtcaggaacggtattggaaactctgaactagataaataattcaaaggatattagctaaagtgatcagggaccaggacaggaaggtactgttacaaacggagagaataaaagggcaaactgaaataatagatcctggaatagcacagacactgacctctgaccacagaccaaaagttagggcctagttgtatttcttagaaatacaaagaaaacaagtttagaatcatagaaaacactgttaacacattagcctgggaggtggtactggcactgaatatacacatacccataaagtcggatatgttcattaatcccagagttgactgataaaatgctgattaaagcaaaggtaggctatatgaggcagccacaccctcccaaaacatgtccccagagaccgggtggccttctttcttaaggctgtaatttatgcacagttaggagttactctctcatcctattaatatttaggatggctctcagctggctgattggagctaacacagaataggatcatacagattctgacatggtcccattttgcgttgttgaattatacatggaaagcaaaaccaggtttttttttttctctctttttcaggggaggtgggtgcagataagggtgggcagggcactgtatagggaggaaaaaaatactgatattgatgggtcttgggattgcaataagtcagtttaccatttaagaggaaaatttaaatattcagtggaatgaggcactcaaagggttgaaatgcgatttttctttggtttccagggacctgtccctgggctctcactccaaggttaagttccaaaactatactttttggctcacagggctctctgtgatgctctggtgccagctgtgtactcttgagtggttaggcagcagttcacattagatgtgtaaaattaattaaacctaaatctctaggctcaagtccaggatgtccccagactagttcagaaactaagtgctctctcctccccttaaaaaggtgttggcaaatgcaggtctccaaggaagtacgtggcctcaatgggagatgcccagagactgcaacaggtgaaaggtggcccccaaggcccagcccgtctctatgttgttcactttctttgtgagctgtaagactgtgctgtctgcaaagccaaagccatcctttaacagggctgtgatgtagctgagatccatgcacaggaaaggactgcctgaggtgaagttttccaagttatcacacacttccctggcttttctttcaaaatcttcaacttttaaaataccccccttttcataatcttcttggttgccaccatactggtatttcacacccccaaagatccactctgcttccaaccatctcggtaaacaggcactccggaaagtgtgcccatcagtcccttctgtctccagggctcccagggttgctagtcttgcagctttcaatccaaatcccaggtaactatgtgtatagagcttataagtgctgttaaacatctcaaaggaagtgaggtagcccctaggagtttgttccagagttttctcaaactggggcaggaacgtgatttgggtggaggctccccctaggtccaaggtccccacagtctcctgtctgtggccatgcagctgacctgtcagaaaattcacagtaacccaagctaatatgccttcgtcggatccatccatgatgctaacactgccctttggtaccaggaaaggtgacttcctgaagatctcctttacctcaaagagcagagccttggctttgtgttctggcagtaagcgtagtcctgctgttgcctttaggaccactggggtctttttccagtgacttcgggggattgagtctttggccacctctaagagcccttgaacggtctcagcaccctgcttaggttgatctacaaaagcagaaagtcctggcttcacagaatcaaaaacttccccttctagaattggaagctgtcctggcattttctgcacaaaggtgtaaacatgaattcgagttccagtgctccctgcatcaaacataattccatacaaggtgctggcgctgacattgatggggcacatggaagacaggaagataccctcaaaccaagtctgctggttcctgtgggagacagcgctgcaaacacaggataccaccagcatgaaaaagactgtgccccaagaagtggccattcttttcccaagatgtggctgggtggaggcttttgttgcagaagcaatcctgctcgcacacctgcagaggcaattttttctttccttctgaattttctccttggttcctttattatatcactttttcaaccttacatctggatacaagtcctacctaacagcaccataatgatcttgtctgtatgaggattcagccaagacactccacatttctttgttgaccaggaacaaggaaaacgcgcgcgcgccacccttgcgcggcagcccgccgccctc

SEQ ID NO: 8699 - RNA, 2577 nt, Homo sapiens
  source 1..2577: mol_type = other RNA
aactctagcctgagcaacagagcaagactccatctcaaaaaaaagtgcaagataatgaatttggggtaaataattcacagtcaagagctctgagcacttggattcaaaaagagagcatgagggacattaaatatggttctccctggaaatgttggtccactgtactgatgtgggctgagagagccaaccaaatccaagtggggttttgtcaggaacggtattggaaactctgaactagataaataattcaaaggatattagctaaagtgatcagggaccaggacaggaaggtactgttacaaacggagagaataaaagggcaaactgaaataatagatcctggaatagcacagacactgacctctgaccacagaccaaaagttagggcctagttgtatttcttagaaatacaaagaaaacaagtttagaatcatagaaaacactgttaacacattagcctgggaggtggtactggcactgaatatacacatacccataaagtcggatatgttcattaatcccagagttgactgataaaatgctgattaaagcaaaggtaggctatatgaggcagccacaccctcccaaaacatgtccccagagaccgggtggccttctttcttaaggctgtaatttatgcacagttaggagttactctctcatcctattaatatttaggatggctctcagctggctgattggagctaacacagaataggatcatacagattctgacatggtcccattttgcgttgttgaattatacatggaaagcaaaaccaggtttttttttttctctctttttcaggggaggtgggtgcagataagggtgggcagggcactgtatagggaggaaaaaaatactgatattgatgggtcttgggattgcaataagtcagtttaccatttaagaggaaaatttaaatattcagtggaatgaggcactcaaagggttgaaatgcgatttttctttggtttccagggacctgtccctgggctctcactccaaggttaagttccaaaactatactttttggctcacagggctctctgtgatgctctggtgccagctgtgtactcttgagtggttaggcagcagttcacattagatgtgtaaaattaattaaacctaaatctctaggctcaagtccaggatgtccccagactagttcagaaactaagtgctctctcctccccttaaaaaggtgttggcaaatgcaggtctccaaggaagtacgtggcctcaatgggagatgcccagagactgcaacaggtgaaaggtggcccccaaggcccagcccgtctctatgttgttcactttctttgtgagctgtaagactgtgctgtctgcaaagccaaagccatcctttaacagggctgtgatgtagctgagatccatgcacaggaaaggactgcctgaggtgaagttttccaagttatcacacacttccctggcttttctttcaaaatcttcaacttttaaaataccccccttttcataatcttcttggttgccaccatactggtatttcacacccccaaagatccactctgcttccaaccatctcggtaaacaggcactccggaaagtgtgcccatcagtcccttctgtctccagggctcccagggttgctagtcttgcagctttcaatccaaatcccaggtaactatgtgtatagagcttataagtgctgttaaacatctcaaaggaagtgaggtagcccctaggagtttgttccagagttttctcaaactggggcaggaacgtgatttgggtggaggctccccctaggtccaaggtccccacagtctcctgtctgtggccatgcagctgacctgtcagaaaattcacagtaacccaagctaatatgccttcgtcggatccatccatgatgctaacactgccctttggtaccaggaaaggtgacttcctgaagatctcctttacctcaaagagcagagccttggctttgtgttctggcagtaagcgtagtcctgctgttgcctttaggaccactggggtctttttccagtgacttcgggggattgagtctttggccacctctaagagcccttgaacggtctcagcaccctgcttaggttgatctacaaaagcagaaagtcctggcttcacagaatcaaaaacttccccttctagaattggaagctgtcctggcattttctgcacaaaggtgtaaacatgaattcgagttccagtgctccctgcatcaaacataattccatacaaggtgctggcgctgacattgatggggcacatggaagacaggaagataccctcaaaccaagtctgctggttcctgtgggagacagcgctgcaaacacaggataccaccagcatgaaaaagactgtgccccaagaagtggccattcttttcccaagatgtggctgggtggaggcttttgttgcagaagcaatcctgctcgcacacctgcagaggctgcttgtgtctgccggttccctgagtccttgctttcgctgcaggttgccttttgctctttgctcctgtttcagctcttcttaatcaagcgagcctcatgaaccgcattcacctttgt

SEQ ID NO: 8700 - RNA, 914 nt, Homo sapiens
  source 1..914: mol_type = other RNA
aactctagcctgagcaacagagtgagatcctgtctcaaaagacaataaaatttactttagtgagagtttgctgatggcaaattctctcagtttttatcagtgaaaggttctcatcttttcattgttattgaacaggggtttagctggtatcgtagtcagggttcttcagagaaacaggaccaattggatgtgggtggatatatgggtagatagatagacatagattgattgatacagatagatagatctgtatcggtagacagagaaatatagctctatcatctatctatctatcatctatctatatggagattaattttaaggagttgattcatgaaattatggaggctggcaagtcccacgattttccgtatgggaatcagggaataagaatccgagtagaggaggggcagggagtgctaatagcaggacaacagcaactgcagagagaagacggtcaggccggtgagggaagggaggagaacgggtgtcccggacaggttcttcttgcagtcctactcgatcccagaggaggcaggacgaggccttgagctccctggccagtgtcccgggcctgggcaggagggtgatgctggtgacgtgtaggagtgaatccgtgagtgagtcgtggcggtggggcgccagcaccagttccccgaaagtgagagcccgggaacagccagagatcagaagaggcgtgggactgcagccttgaaaggcgctaatgagaggagcctgccactgtagagggtatagcttggtggaagagcctctgcctacacgccaagaggttcctgcttcaagtccaggtgtctcctatggtttacgtttttatccagcaagagtattttgttttcttcctctcccacccctcaaaagccagcctgtaaggctgtaatgtcttatttgtctgt

SEQ ID NO: 8701 - RNA, 4998 nt, Homo sapiens
  source 1..4998: mol_type = other RNA
aactctagcctgagcaacaggagtcagaccctgtctcaaaaaaaaaaaaaaaaaggtgtcaaatcttattaagtgaggatactttgtttcaaaataggcctataaacagaaggttcactttgaatttgaaaagtcccttagcagacgtaaataagaactaaaccctgctttcacatgctagaaaattctagaattgcttcaattccacttatatacataaatatatatggatatataatatggctctgccaagtattggtaactgatttttcttccttactgaaatctaagatagttgcccttccagctgagttagcagggggagtattccagaccaagactcgcactgtacagctcctgccgattttgcactatttttaatgcagttgagtcttcagatttgtgactaggctgacagctttgtcttgtgttcccgccttaattttttgagaaaaatcccttcaagactattttagggtcaagtcttttgtagtcagtcctggtgggcagtcactatgagacaggcctgacagaggggtgctgtgagaacagagcgagattcggtgagaatagctcagctggaaactcactgtgcggcgctcctgatactgcccactcgaggctctaaagggattgccattgccagttcactcccaggagtagaagtgatctctgtcttaagatctactctcaaaaaaaaaaaattatatatatatatatatatatatttcgtggcaatttttttttttttttttttgagacagggtctccctctgtcacccaggctggagtgcaatggactgcagccttgatctccccaggctcaggtgatcctcccacctcagcctcccaggtagctggaactacaggcctgcaccaccacgcctggctaatttttgtatcttttgtaggacagggtttccatgttgcccagcctggagtcaaactcatgggctcaagtggttcgcccacctcggcctcccaaagtgctgggattacaggcgtgagccaccacatctggccttgttttggttttttatgtttttgttacctggtaatctcttttaaaaatacatttaatagaatttcactggcagataatgagttgctgaaggctgccttctttgcctcttacttcctactctccagcttccaaacccctctattgggagtgggggattctaggctgaccaggaggaaagaagctgacactaacactggttccctggttcctatgaaaccaagcttatcctgcctgtactaaatcttactaaagctgtaactgagtctctaagaataacttcagactgcctcagaacacagacatcagtgtgttctctaggtacttgtccaagcatttctgaaacagctaagctcaacttatagtaaaattgcaccaatatcaaaattatggattattcgaggtcttactagcaaaaaccagtcttggtaacactgaatgcagtcttcctaatgacttagtaaatacaggatgtgctacccaaagtgaacatattttcaaaaagaaaatatatttaatatcatatcacaaggtaattgtttaaaacgttactgcaataatgaaacatgattatttaattgctggcttccatagtatgctgttactcattttacatattcaccgtgtatccaaaactggaaatttcacatcttttaaaaggtgagttaaagttgtcatttcagaggtgcccttcttcatgtcctatttatgttccacttggaataagaactaatatttttactgtttctttttcaccctgcccaccatataaattttccaataagaaaatatttttaaaagagctctcaagtgtaaaagaattctttcttgctataaataattatccctaaatatttctctttaaggagagttcacaaactgggtcttgttcaaggggcgtactcatcaaggctatacagtgtggccccagagctgacacactggggtgcatagctactcatccatccataaaacagcacactgcacacatccacagcccaaagtatccctgactacttgtggtgactgatggggcaattgtggctgctacttatgaggttgtacaagatggaaactgcatccacattgccccagggaaacactgtggctgtcacccacacccacaggagagaaccccattcctgcaaacacggcctttctccagcacccacgctggccccatgggacaacaggtttaaggaagagcagctccagaagcagcgagatttgtatctcccacagtcctgcatgaaaatgatcacacgctcatacacacataccccaaattattggcaggctctgtgaatacaaatcgagagggacaaatctgtgtgcagctggcagcaaggtcagggagagaacatgactcacatcccagcttaaccacagtccctctggcctttgacagaataagcatcatatgatatgatcagtccccacaggcctgggaggtaagtacgcaattgccacaggggttttcaatcttacaatggagtggtccggaaaacagcaaaggtcaactctcagagggaagggtagtgtgtgccacacaagaagggttagcccacttctgtaagcgtgtcacttcctctcccctttctgattcgcagcccttccaagtcagatttccaccattcattccaaaacctttaagatgtttcacaaaggggaggaaggaagaaggaaagtaagaaagaccacactgagatcctatgaggccattgagtgtggaaacgctgcattcaaatgtgccctctgctaacaagggaaactatggcttcctcacaccgactcctgagagttgggaaggtggagggaaggatggtacatgaccaagcctgccatcaccaaatgagggaccacacagcagaaagatgaagcccaggctcctgacacactggagttcacgcttcagcctgtgacctctgtgggccagttcacctcagggccaggcgtcactgagactgtgggttctgggagccctctttgcttttactgtcctctgccgggctgcactcggaccccgtgatggaggacttgcacccgcgaagcacgtgggcattcagcatctccagcagcaggtcatacactgggaccacatttttgcacttcatgttgagcagatgttccatgcccttgttactcgcatgcctgacgtgggacaggagcatcaggaggttagccaggcgcatggattgctgctgggaggagatgccgctcttggcaatcacccaaaccaaagcatcggtcacggcgttcagcaagtgagccagcttccggctgctgtcagcatcctgggtcgctgtgaccagagggtacatactggaattgagcaggatcatggccttgacacagagatattctttgtgttggagttttaactctcgaaaccttgaagtagttgccaggagcatgtcaaagatttccagaattccttctacgcatttcccctcatccctgtccagaacaagatctggagcaaagatgagcttgccggggtggtcaattgagcgccacatcagccccatcattaacacctccatccaacagctctccaagagccgcacttggtcgaacaggctgagctccacaaagccgggaatcttcttggcccagctgatcatgtgtaccaactccttgtcggccaacttggtcagggacatcatcatggaggcctcggtgaagggcgcactggggcggctgatcagcacatggggcggctcagcctccaggagggtgagcactagctgctcggggctcagggcgtccagcagcagctcccgcactcggggcgcgtggccgccacttctcttggccttgccggcacagtgcagctgctcgtcggcacttctctgtctccgcacaaggcggtacccacatctctctctccgggagccacacttcaccattcccacttcgtaacacttccgaagtcggcaggcctggcagctcttgcgccggtttttatcgattgtacactgatttgtagctggacaaatataatcattatgtccttgaatgcttcttttaaaaaaggccttacatccttcacacgaccagactccatagtgatatcccgatgcgtaatcgctgcagacagcgcagaagtgagcatccctctttgaacctggaccagtaacagggctggcgcaacggttcccactaaccttccttttcagtgtctctctgtttacaggtaaggtgtgttctagcgatcttgcttcacaccagggactcttttgaggttccgcatacagatgtgataactggcgatggaccactaaaggagaaaggtgcccaggtgttggccacaacacatttgggcttgtggtctgccgaccaggcccaccttccaagttagtgacattgctgggaatgctgtaattcatcacagcagggctatagaatgtcatggctggatattcatggtggctgtctacataggaggaaggtatgtatatggagccgtgctccaggggtaagatggattgactgcagttgtaggaggaaggagaattaaggctagatggtgagttttttatatccatgtcttgagataacagctgagaaaacaccttgcaagaagaggcacaaaggtcattataatgttctcaaagattcgtgggcaagtataatggcttgcagataaacacaccggccttgccttctctaaaatgcggacacgtgcttttcccgcattagggggggtctcccggcgcgcgccccgccgccacctgttgaggaaagcgagcgcacctcctgcagctcaggctccgggcgccagccctgccccgcagccccagagcccgtcgcagctcgggtggtccctccccggcccagcgctcgccgcctgctcttcgccctgcaagtttcaagaggcagttatttctcgcagcctccgcgcttgcaactgcctcctggcgggggagtgggtgtccaaaaagccagcagctggagaaactgaaaagatcacaagc

SEQ ID NO: 8702 - RNA, 1011 nt, Homo sapiens
  source 1..1011: mol_type = other RNA
aactgtttgcagaggaaactgatgcccagcactgctggctgcacggtgaagcactccatagtatgattattgctatcacccttgtgtcatcctcctggcccctcgaggtgtgggggtttactccagagccagacacacctgggttgcagctctgcttccatccccctctgacccagggcaggcccctcgccacctctgagcttcagtttccccacctgcagaacagggttgtttaggggtgttcagatcgcaggagcagatgtccctggtgcccaagacccaggaggtggcagaagcaggcgggtcacatgtgcaggaggggttgcacttccagggtcgtggcactgtccctgcaataacctccaccctggccttctctgataccaggggtctcaggtccccatctggcctgcaccagccatgagcctctctgggcctcagtttacccatcaggctggggtaggcccaagcaaaaagggagttcttgaggggtgaaccaccctggtcacagcagtcatgcagctcaggagagttggccgtctggttggggtcagggttgggggtcaggggtcaggtaccttggtcacagccacggcactagcatgaccgcacagctccacgagctgctgccgcccaaagcgataatcctccagcagctcccgctccagggcggctgcctccgcggtgcccttcaccccaaggtgaagtcacagctcctaaaacactcttccctagactgagtctggacatcggctgaggggacacgtgccctgctaggtgggcagtgggcaggagctgttggacgcatctggttcacagtgaggtcaacagccttgcctggggtcccatgtcacaaaggctgaggaggatgaggtgagagtcacagccacggcgccagttctagatcccaaactcaccaacctctggcaaacaggccctgcgttccaaatctgctctagccatgactgccttccccaggcctgtttcctcctctggacaagggaggtggta

SEQ ID NO: 8703 - RNA, 457 nt, Homo sapiens
  source 1..457: mol_type = other RNA
aactgtttgcagaggaaactgatgcccagcactgctggctgcacggtgaagcactccatagtatgattattgctatcacccttgtgtcatcctcctggcccctcgaggtgtgggggtttactccagagccagacacacctgggttgcagctctgcttccatccccctctgacccagggcaggcccctcgccacctctgagcttcagtttccccaccttggtcacagccacggcactagcatgaccgcacagctccacgagctgctgccgcccaaagcgataatcctccagcagctcccgctccagggcggctgcctccgcggtgcaacctctggcaaacaggccctgcgttccaaatctgctctagccatgactgccttccccaggcctgtttcctcctctggacaagggaggtggtagcatttgagctaagctccgctcttcccatgtcggcaagt

SEQ ID NO: 8704 - RNA, 1060 nt, Homo sapiens
  source 1..1060: mol_type = other RNA
aactgtttgcagaggaaactgatgcccagcactgctggctgcacggtgaagcactccatagtatgattattgctatcacccttgtgtcatcctcctggcccctcgaggtgtgggggtttactccagagccagacacacctgggttgcagctctgcttccatccccctctgacccagggcaggcccctcgccacctctgagcttcagtttccccaccttggtcacagccacggcactagcatgaccgcacagctccacgagctgctgccgcccaaagcgataatcctccagcagctcccgctccagggcggctgcctccgcggtgccccgagtagcgtctgcagccttgagctggggatgccctcagtttcaccgtgcgacgcgcgggttgaatcgaggcctggcgggccgcggtgtgggagccaaagcccgaggcgcgggcgccctctggtggcagaagatgcgctggccgcgcgttggttctactgctccaaagcgtgggacacggaaccggacctagacgtccccagctcccaaggcggagggaaccaagaaaggggaatggagcatgaaggacttcgatgggggcgatgggctgatttcaggcagtgggagccacggaacaagcttcaggacgctgaaaggggtggacaggactgggggcatctggggtccatgggtttttaaggctgcagtgtttgatggcacactcagcggggaggccttggggcctggggctatgagaccctttggtgaccgattttcaggggcagtgacataattagattatttgtggccaggccgggcgcggtgcctcacatccgtaatcccagcacttcaggaggatgaggcgggtggatcacttgaggtcaggagttccagaccagcctgcccaacatggtgaaaccctgtttctactaaaaatacaaaaaattagccaggcatggtggtgggtgcctgcagtacgagctactcaggaggctaaggcttgaacctggagaatcgcttgaacccgggtggcagaggttgcagtgagccgagatcgtgccactgcactccag

SEQ ID NO: 8705 - RNA, 648 nt, Homo sapiens
  source 1..648: mol_type = other RNA
aactgtttgcagaggaaactgatgcccagcactgctggctgcacggtgaagcactccatagtatgattattgctatcacccttgtgtcatcctcctggcccctcgaggtgtgggggtttactccagagccagacacacctgggttgcagctctgcttccatccccctctgacccagggcaggcccctcgccacctctgagcttcagtttccccaccttggtcacagccacggcactagcatgaccgcacagctccacgagctgctgccgcccaaagcgataatcctccagcagctcccgctccagggcggctgcctccgcggtgcccttcaccccaaggtgaagtcacagctcctaaaacactcttccctagactgagtctggacatcggctgaggggacacgtgccctgctaggtgggcagtgggcaggagctgttggacgcatctggttcacagtgaggtcaacagccttgcctggggtcccatgtcacaaaggctgaggaggatgaggtgagagtcacagccacggcgccagttctagatcccaaactcaccaacctctggcaaacaggccctgcgttccaaatctgctctagccatgactgccttccccaggcctgtttcctcctctggacaagggaggtggta

SEQ ID NO: 8706 - RNA, 937 nt, Homo sapiens
  source 1..937: mol_type = other RNA
aactgtttgcagaggaaactgatgcccagcactgctggctgcacggtgaagcactccatagtatgattattgctatcacccttgtgtcatcctcctggcccctcgaggtgtgggggtttactccagagccagacacacctgggttgcagctctgcttccatccccctctgacccagggcaggcccctcgccacctctgagcttcagtttccccaccttggtcacagccacggcactagcatgaccgcacagctccacgagctgctgccgcccaaagcgataatcctccagcagctcccgctccagggcggctgcctccgcggtgctctggcaaacaggccctgcgttccaaatctgctctagccatgactgccttccccaggcctgtttcctcctctggacaagggaggtggtagcatttgagctaagctccgctcttcccatgtcggcaagtgggggctgcagctccaaggccctgggagagatggagagtgggggtgggccacggttggggttcggtgggggagcgaccagcgctgctgatgaatcattcatgaggggcgggctgccccggaggcagtttccccagcaacgcagcttagtgtctccagcaagatgccaggagggtctcggattcccgggattcccaggcccgtcttggccatatccctgcctccggttccccaccgtggtcatgcctctgccgttgaacctccatcccggctgtgcccgtctccagtccccggaccccattctgtcccagctatgaccctgcctccggtcctacgggctgctcctggccccatgggaaccatgcccgtctccagcttccctctccccagctgacctgaggaaatgccgctcttcgggcgcctccgacgggtctgggccggctgcgctgctcatggccgaggtgagcccgggcgccgggcgctgcc

SEQ ID NO: 8707 - RNA, 8443 nt, Homo sapiens
  source 1..8443: mol_type = other RNA
aagacgggaggaaagaagggaggctgggatcacctcccgccccttctagcatctctactgagagtgacaactccaggctgtccacccccatcctgagccttccacactcttctccgtgccactaacactcagtatctgacgcctgcagtgcgaagcctccagagtccccagactgacctgggcactccacccttgctggttctactttacttggacacacgggtaccttaaggcttgtcacactccaacacctttgtgtgtgtgtgtctttatttctttctaggttataaactcaggcagaggcctcatacattcacttctctatcccaccatcccagtacagggccagccacatattaactaatgcacaaatgaggccaagaaactggctagaaatcccaagaaactgtgccaagtatatgcagctgcacctgggaatacacgaaagcatgacatcacgagcacagcctcctccaccacaccttccctttctcctccttccctgctggcctcagacagctatgcatggctgcatgaaggaagatctaaatctggacttgttttatcctccccttcccttcttctcacctttattctgcctccaccttcttctttctttgtcttcccccactggcttctctgtcatttcccacagtgggttcccccaatccctgtggtcctcatgtcctgttcttgttctctttgtgctggatctcacatcctacagcatccaggaccatcctccatggctgatgccacagcctgccaattcccaaattcttcacgtttgtttgacttcctacttagctgtaaaaccaaagcccagggaggagtcccaaggtgcacaacacagagccaatctgcgtgtgtacagagatgcagatccgtttttaatcaatgtaagtatatgcgtatatgtatatacatatgcaattcacattcacaagtcctggtataaagttgcaatttttctggctgctataaaatgtgccagttttaaaactgtgcatttgttgcttgcaaacttataaatatgtataaaccccattataaataaattatggctggcagatggcatttaagctgccagcaatggttgcatggagttataaatgcttattaattctccacttttaaattcacagcacggaccctgggatctgtgacatgaagtggtgtgaaagcataattataaattagaggggggaaagccatcaataagagacaggtaagggctggaaactctcactagtgagtggttctcaaagtcaagacttcagagcagctgcaccagcatcacctcgagattttttgaaatgcaaattcccgggccccactccagacctagggagtcaggaacttggcggggccaggggggtggaagggcctgcaatctttgtctgaaccagctcacagggtggttctgatgcctgccttccactcgaagtctgcttgtcacgaacgcctgtctcagctcagggacatccccggcttaggaagtatgctcaggtgtgtgcagggccagtcagaaattgtttccagaaacagcctttcataagtgatagacttggtgaataaataccccagctgtctccccgccttgctgggtgaactctggggtgtcagctctgtctctcggggttccccggtgggattcagctccagttgtgcacatgacggtaacttacttgataatgcacgccttccccgtcagcttccttctctccctacttccgggatcttcactcaaataaactacataacctcaagtcctctctcagggtctccttctggaggaaccccaactaagaggaagtagaaacactgtctctcccatctgaatgactcaggcttttatgcattttgagatggagcacagatgtagaacccctggagggaagcactgcttgccatttccgtggggcagggggctagctttacgtgcaggcccaggactgtgagtcctgtgctcttttctaagttgatccccaggcccttgcatggctccagtttcctcttctgaaaagcagggccccctactgggctgtcttaccaagctcccttccctgtgatcctgtgtggagctgacagttctaggttggcactatgtccaggagtgggtttgtcctcttcatctttcttagagccagctttgaaagttccatgggagaacctgagtattactctgaaacccactgcaaggtctgtctgagtcctgcaatgacctctttgcaatctttccacaatcttcccactcactcccaatcctactgtcaccgtccacagaaagggatttatggacagcacacaaagttgggccagcgagagagaaccaatgggcacgctgggaatgcacaattttagaaaatcattgcgcttatatgtttcatatatttgtcaatccccagcacgccctcaagctgggaacatgtatagccctgcagtgtagagcacgccaaggctcagagaaatccagcaacccgcctgagtccacgccgttctgggtgtgccagggtggaggctggatggaggtatctactcgtggcccgcattgcctctgccctggaaaggcctatagtccgaggcttctgcccagctcagcccaacagaaaagaaatgtgtgactgccttcaggtagcagccagtttggaggaaatgaggacccagacgtccatcttcaagcattgcttatagaaagaagctacccaagtgtcggacgctactgaaaaggaaagctttattttgggagctgggggccaccttcagaatcccagcaccagacatggaggttgggctggacacacatgtccactgttcccctggcacatgggccctttagggtccacccttccctaggcctgtccttccttttaagttaggactttacctacacacacggcttgtcatttcccgtctttattagaaattacccacaacttcctccacctccaggaggccctaaagaaggccatatatggcccaatcaggcctttgtccattatcccaacatcatagatggcctgacaaaatagctgctcgctcatcaaggctgagcggacgcccagtctttgggtgcttcaaatataaaaaacagcaacagtggtgtcttaagcacaggattaaagattgagtcatttgactgcggtgtttttcacctccccacccgattctccggttagctactcagaggcagccttggaggtcaagaatcaaagctgacttaaaccacaatgagcacccccatgagaggcccagccggcctccgtgggacagagatgtcatttgaagcacagctgattcattcgtggggttaggggaggtgggtgggggtctctagggccactcggtaagggcagaggggccgttttaggactgctggcccccaccttgtactcccagaagacatagagtttggggttaagtgttgggggtgcccattggagggacagcagggcccaggtgcactctgcaggaccagggtggcccagcacagcagcagcgactgtgccctggaagcctgaggccctggaacgcaaggcctaatgccattcccgctgcgttcattgttcagcttccctgccctgcccaggcagagatgtggcctgagaaagtgtggggaagaggggcccaggctagacagggaggagcctccattgcttttgccttggaatcctgagctcaaagcacaggctggcacacagcagggctcacgaaatgctgagtgagcagaagagctctgcagccagatgacaacatggcctccaggaaggtgtggcaccagccccagcctcactttccccatgtgtctgtgaggctcacaggaatggcccaccacacagtgctggagggaagagttgggataactaatgtgtgctctaacccactttacaaatgggagggaacaaagattagaaaatcgctgccatctgctatgtctgaagcctgctcacttcactggcactattctagtgtaaccaatatataatctgagcttaaaaatgtatattttgaattaatattaaaaagaaaaaattcgactccaatactttaaattttctaaattgattctcatgcaaaaaatatatatattttctatcaccatcgaactagacactgacttcacagcaagagctactaaagctgcaggttaccattcaagtccccccaagagaaaaataaagtaaatcaaatgttacagcattcacagctcctaacttgcatttcctactttgctattgtccctgaatgttataatagcattttgacctttcacaagtggggaatgcatgaatgtagaaagaaggtcatttcgcacatttttctatgtggtgcacattcatgcacaggtgggtcagagctgtgtgtgtctctccagggctcccagcctcccagaggacagatgtgcagggcagctctcagagcacccaagtctatgctgtcttggggcaggagcctgatgcagctgctgccagcaaccccgtggagccgtctgcttctggatcactaagcagagtatccacatgatgcctgaagccaaaaccatttcagaaaacagcagtgcagtctacagtagtgtcagactctccagagtttcaatccactgcagaacattctagaacactgacttcactgtcatctcaaattcactggaccctcaaaggcaaagactccctagaaggccatgtatgaaggctggggcctgccctgactcatcctcactggttagctctaacctgtccttccatctggccacacgcacaccccaaggcagaaatggggctcataccattggcattagaacttagcagtattattatctgccagatttttcagtctcctcataactctccttacaggatcagatttatcactatccaactctaagcgtgtttagtgtgtctttctgttctgctgacccataccctacagggtgctgtaccctgtggggtctcaccagaacaagagccacgctgccagcaagcaaatggatccatctattctttaaagggcatctgtgaaaatcacagggcaatctcagcccagatagtatttgaaaggtataaacattgccagctttctaacaccaaatgactcctcaggaaatgacagtattttacctggaagaaagggagtcaagacaaagagtgggggcaggcacatgctcttccctgcagcaacggagaaaccttgttgttgggacagcaggcctttcccccatccctcatgccagaggcagtacctcaaatggattccagtgactcctgggtttctggcacatgcagccccagaagcctcaatacctgagtcttcgggactgagctctgggatgggtgcctgctcttgctgtcacacaggcttctcccctattgtataaggcgggcgggggactttactagcaattaccataagcagcctgtagtcaaccgctgactagagggagacacaaaccaggaatttgccccgaccacccttctacaaatacccattttagcattagatacatgagaacagggaagcacttgtcaatcaaaatcttggttggtgaagcttattttgtgccattttggcatgaaatgaattcccaagtactcctcgcacaactggggtcaagggtggcggggccctgtgctcagcaggacccggagaagctggagtgccacctgttctttagtgaagctgcagcgagttgtgtagacaccccaggcacgtggagtgcagtgcagggagcacaggaggtgtcccagggaggccaagggaggatgcccgctcccaccagcaagcacagccatgcctcagaaccagtatctcatagctttcagtgcagggctaggcatgctctgagcagcatgccttgcgattccctcacaattctgtgtttctattcccctccagttgtgcttattaggtaaaactgcaggctacaccttcctagtggcatttcccggtgggatgggtcagttgaattaaatttttgcctggacaactacagttaaacttatttttttttttcattaaaaacatacagcacagaacattagtcttacatctttcttagtcttaaaaaatataaatatagagggataatttgtacaggatgtataggtatgtacacctttaatatgcatatgagaaattcagaaccaagtttatgaaacttgaccttaaaggaagccttccttttgaagcttttgaagaaggctctgagccacaggcagctgtcccagttccagcagccccgattctagtccactccaggtcctcctgacctggtgcgcagtgctgggagcagtgctggccaggtcactgcttcctctccactggctgctggagacacagctcactccctgcagagacaatgggcaggctgctttctaggtggtggttgatgaggtggctgatactgtcaaagactctgtcctttgtccggatcgtgccttctgggtccacgagcagcaggtgcttggcctggccattgtgcatgcccgtgaggacaaaggagcccgggttggtggtgctcttcctgaccaggaagtctccgtctttctccagcagcccctctgcctccttcctgctcatctctccttggtaccaagtctcggcttgcagttcctccagcatcttggcatctggggctctaggtgacacagggctgatgcactccacggaggctgccttgcttaacacgggccccaagggctggttcttgagagcatcttcaaaaggtttcatgtcaaagaggtctttccttgggctgctctcagcactgctgaccgcagccggccaggcctgtggtgggatctgctgagtgttgacgtaggtgggtgcttctcccgtgggggccacgtgcagtttcccttctggcgtgctgtagatgtccgaggacccttgccttaaaggtgtttgctgccagtcttcgccaaaagtgtctcctaagtgtcttccctggtaataagtctgctcttttcctgcaaactgggctgtgtcaggagcatggggtctgggtttcagtctagtatcaagaaagccccctggaggaggcatcttgcttgggatgctgttgtagtatgggtggtctgagccatctccctcctcttccgtccatggctcatccagactctgcattcgatcatggagagcgggaatcttggtaggacactgtaaatattgcttaaaccggagctcaaaggcttgtccgatggagccgatgacatcctgggccagcccatcacagcattccaaaatgtgacaagctctgcgattaacagggtccttagccacatatgcaacatagtcagttgtgtccgggtctcccccagaggcgaaggagatggaccgcatgtggtgattcgctatgatctgtttggagtccggagttcgcaggttcagactggccgtggagatggtcagagagatgctcattcccgcaaactggaggttgctctttcccaagatgctggacagcattttgcttggaggctttctcttcttgaaggctcccttcgcaccaggcacagcttcacagacgcggctgatggcttccctggtaatttgtgttcttgtactgaagtcaagagacctcattgagcgcagaacttcaatgcaccccaagtacttgaccacgtaggtgactccgggccccagcacctggtcgctggcgtgcggcgccccccgagggggcctgggcagcggctcgtcgccgggccggcccttcctggcggcgctcatggccggggcgcggggcgccgagggcgcactgccgtccggggcggccaggctgggcgcgctgcagctgcccgagagccgcgcgcccgcccgctcccgggcggccgacgacaggccgcggaggcccgagctggagagtttcaggtgggacaccttgtggagcaggtggcccaggctgccgggcccatcgtcgggcgccttgcgcagcgcctcgccggacaccaagtagggagccgccgccggggtcgcgcgcgccgccgaaaccttgcctccgccgccgctcaccgacaggctgtggagaaggtcatcgaccgatgtcaccgagtcattcctgaagcggttatacttggtgcgtggaagcatgcccctccgtgggctcgctgcatccgcccgggcgctgctggtgccggccccggcgcgggctgccgcgcatagcaggcgagccactgtccccggagcgggacggagagtgggggccccgggacagccttctggagaacgagagcagagcaagaggatggtgccctcccaccgttaaaagccagcacagcggcggccgcgcagccccggcccgggagaccgctgcttggggttgcacgtttgctttgcaaaagtcatagttgcctctgatggagcgcccagctgcttggggctgctcacagcaaaagcatgactcactctgagaggagacccttctcaacaaaggctcggtgagcactgc

SEQ ID NO: 8708 - RNA, 925 nt, Homo sapiens
  source 1..925: mol_type = other RNA
aagacgggaggaaagaagggagggagaaagggagggagaaagggagggagggagggagtgagggggaaagagggaggggggcgggctcagcagcgagccccgggaggtggggaaaatgggttggggggccgggctcccgtccccatctccgcgggaaaatggagaaatcggcacaaagcttttgggggaaaggtcagccgctcccggggccggactagaggccagcccccaggagggggaggggaggagacagggccgggaaattcgcgctcctctgtgaggtggtcgccgcggcgcgctctcggcgcgggggagatggatgccgcctgccttcctccctgcgtggccgggctgcagctcgggacgcagggcgggctccggccccctccctctctccttgcttggctgcctgctccccccggcggcgggcccgcctgcccgcccgccctcctcgttccttctccccgcctcctggaggagatggcgggccccctgggcaggggcacccggggtgttgctcgtgcggctaacgccgagcgctgctctccgtgagcccgggctcgagctggggttccgctgggctgcgctcggacttgggctcccgcggcggtgctgaagggacagctcccggcggtcgcggagctgcacggggccaggcgggggttctcctggctgggtttgatttgcggggccggcgggcactggctccggtgcctctgcgccccgcactccgctcctcgcttcgggcaggcggtgggcgctgccggccgagacgggggctgcggaggtcgggcggggaggcgggggtggcgggtccgggcgcggcgaggtgaggccagcgaggccggtgaggcgaggcgcggagcggccgctgccgccgccgccgcgacgctgctgccgcccgggctgctgctccgcttgctgc

SEQ ID NO: 8709 - RNA, 954 nt, Homo sapiens
  source 1..954: mol_type = other RNA
aagacgggaggaaagaagggagggagaaagggagggagaaagggagggagggagggagtgagggggaaagagggaggggggcgggctcagcagcgagccccgggaggtggggaaaatgggttggggggccgggctcccgtccccatctccgcgggaaaatggagaaatcggcacaaagcttttgggggaaaggtcagccgctcccggggccggactagaggccagcccccaggagggggaggggaggagacagggccgggaaattcgcgctcctctgtgaggtggtcgccgcggcgcgctctcggcgcgggggagatggatgccgcctgccttcctccctgcgtggccgggctgcagctcgggacgcagggcgggctccggccccctccctctctccttgcttggctgcctgctccccccggcggcgggcccgcctgcccgcccgccctcctcgttccttctccccgcctcctggaggagatggcgggccccctgggcaggggcacccggggtgttgctcgtgcggctaacgccgagcgctgctctccgtgagcccgggctcgagctggggttccgctgggctgcgctcggacttgggctcccgcggcggtgctgaagggacagctcccggcggtcgcggagctgcacggggccaggcgggggttctcctggctgggtttgatttgcggggccggcgggcactggctccggtgcctctgcgccccgcactccgctcctcgcttcgggcaggcggtgggcgctgccggccgagacgggggctgcggaggtcgggcggggaggcgggggtggcgggtccgggcgcggcgaggtgaggccagcgaggccggtgaggcgaggcgcggagcggccgctgccgccgccgccgcgacgctgctgccgcccgggctgctgctccgcttgctgctcgcccgtcgcctgctcgttcgcgcggtc

SEQ ID NO: 8710 - RNA, 192 nt, Homo sapiens
  source 1..192: mol_type = other RNA
aagactgagaggagggaggagaaatgacagcagaggcttggccaggggctggggcgccggggccggtgccaggctgagcttcagaagggctgcaagaacaggggcttggatagggcaggaaaaggacgtcaagccagttcctgttcctgagaggacagagattgtggcgccgctacaagctctgagcaaagc

SEQ ID NO: 8711 - RNA, 193 nt, Homo sapiens
  source 1..193: mol_type = other RNA
aagactgagaggagggaggagaaatgacagcagaggcttggccaggggctggggcgccggggccggtgccaggctgagcttcagaagggctgcaagaacaggggcttggatagggcaggaaaaggacgtcaagccagttcctgttcctgagaggacagagattgtggcgccgctacaagctctgagcaaagcc

SEQ ID NO: 8712 - RNA, 121 nt, Homo sapiens
  source 1..121: mol_type = other RNA
aagagaactgaaagtggagcctcaccagggacctgcccccctccacccaggagcccatctgcctgctgtgctgaccaaggcacccaggctgcttgtaccaatgggcacctgcaggccagca

SEQ ID NO: 8713 - RNA, 239 nt, Homo sapiens
  source 1..239: mol_type = other RNA
aagagaggagcagtggtgctgtggacaggattcagagagcctgtgagttgagatccatgcgcaggactctcccacacacttaacccctgccaacccaaccccacacttaccagctctcaggtctgtgggtcggaggccgggctgcttagtcttcccggaaggtcttgggtttccttggtctacccagcagcagccaggagtctccctcgcaggcagtctgtttctgactggagatctct

SEQ ID NO: 8714 - RNA, 241 nt, Homo sapiens
  source 1..241: mol_type = other RNA
aagagaggagcagtggtgctgtggacaggattcagagagcctgtgagttgagatccatgcgcatgactctcccacacacttagcccctgccaacccagccccacacttaccagccctcaggtctgtgggtcggaggccgcgctgcttagtctttccggagggtcctgggtttccttggtctacaaagcagcagccaggaatctccctcgcaggcagtctctttctgactggagatctctgt

SEQ ID NO: 8715 - RNA, 8307 nt, Homo sapiens
  source 1..8307: mol_type = other RNA
aagccctgtctcctcccatctggccttctcgccagccaaccccgacacgagcatcccagctcgctccagcttcagctccatctcttcagacttcttgcgaagctcctccttctgtgccagcttctcatcatactgtttctttagcatctccagtttctcagctacctcccgcagcttctcctgggcctcagcgagcgcggcttgcttctcccgaagctgagccaaggcagcgttcattcggattcgcttgggctccaccacccgatatagccgcccatacagctccatggcccgcacccacatgcagagggacttggcagccagggagacgcggccgatgatatcaggctggaagtcaggctgggcgcagtaggccccaatcttcttcagaaccttatctgagatattgtctttatcaaagttgatcagtgacttgatgaagttctgttcccctagctgcctcttggcctctgcccatgtgggctcgttgcctcgaagaatcataactgcctgcatcactatctccacttgggctgggggccgtccataagacttgatctctcctatatccttcttgttcagagactccagggcccgcatggcctcttccagggcgggcagtgcctcttctagatctttctgggcattgtcagccagtgcctgacacttgatttcctcaactgcaatcttttcactgttggctgttacggccttctgctgctcatctgcctcccgcttctgctgcacaatgatgaccaggtactcctcacactgcttctggaactcagccaccttcttcttggcatcctccagctccaacgacatcacttgcaccttttccctagtttcgtcgatcttgaacaagcctgtccgcagtttattggcttgggccagcagctcctgccgtttttctcccagcaacttcttatatccagacaggagttccaggtatttggtgggtgtgacatagttgtgtctccgcagttccaacagcatcttctgggaatactgagctactgaccagtgcatagtgacaaagatctgggccaccttcctgtggatattctcctgagttcccaggtctactcctatgaggcacttctcagccacctcgagcagggcctcttggggccactctgagaaccagttgatggttgtgcagttcaccaaggctgggtactggcggatccagttcctgaagggatcccccatggggctgaggcagagcacgatgtgcaggttgttctgcacgcgttcaatgaggtaggcgaagaggctgtccgatgactcaggcacctgctccacccgggcctggtctatgatatgcgactggatctcttcaaattcatcaggcttgtagagattgggcacctcgcctgagctgaggatgttgttgatgtcctctaggaaggactcatcagctatttgggtgtccacaaaaatgaaggacgtggtcttgagctccaccccagcctggcgatacagacgcttgatatcatctcggaactcctgcttccgataatgtttggtgacctcgatctggaaggtggtgtagtcgcagatggatgaagccaggcgggccagactctggcgtccgctgcccccgatacccaccaggagcatgttgccccgaggctgtccaatgacccgcacgatccgtgtgatgtgttcaatagcctctcggaagagcactagctgcatgggcacgacagagggtgacaggttatactcatttagagctgtctccatgactgtcttcagcactgtcagatccgtgaggtcttcatacaccttgggctccttcaggaaatccccaaagataggaggacgcttgctgggacagagatgatgaaatgtgaggtcaaagaaggagccgagcttgtcgcttatgatgcccatgaaggcttctgtgtctgccgcatcaaccagccggtcagagaagactctgaaacattcatggatccagagccgtgtgatgctggacttggtatcatggaagtccttgttggctctaagcatgccctggaacaccttggagatgtctcgaaggttgaagaggtaatgcatcttggtgggcgtgggcaggaagcgctgtaccacggtgttgtacatgtccagggtggcctctgtcaccacgttcccaatgggcttcacctcttcctcaaagtcctgaagcttctgattgatcatggtgccgaatatgcggatgatctgggactttgtggggaaggtcatgttgataatgttgaagcgactccgtagccttggggagatgacagtccgtccacccccaggggggcccatggcagccatcaggaacatttctcgaatgtacttgatggtctgcttcgtacggtcataccagaagccatagtcaatccagaggcggatcagctccaggggtggctgggacccaaacatgtccttagcgggcatatttaggtcatccataaaggtgatcatgcttttgcccccgaatggcacgtagacacccttggttcgcttctcaaccctgctctcaatgatgctctgcacgttattggatgtggtctgtgcggacatgttgacaacgagcaccgaccactggctggagggcagggactgcagaacgctctgggcgatggaggtcttcccagtccccacgggacccaccagcagaatgggattctggttggccaccaagctgctcaccaggtagttgtagcgaacagtgtcgacggtgggcaccatgatcttatagaagggggcgtttggagggtagcgccaactcttagggagcttgtcctcaaatgatgtccaactccgtattttggggtccacaaaatactcatataccgtgtccttattgggaaaggagccctcgatctctcggaggtagctgtcgatcctcttccggccctcctcatccacagaggcacacacagaccagatcatgctgaacacaaatgtcatctctaccatggtgacatagttctcgccgtcagctgggttcaccccattctctggcgtggccagggcagagtacagcttgcagagggaggtgataccgctgtactcgggcaggggcaccagctccttgcagttgtccttcttaaaggccagcatcttgttgatgagcttttcgaacatgcgttgaaggggctccacctcagcctttggcctcttctccagccatgactgaacatagggcttccagcccaggtcagcgtagtcagtgtagaccatcccgcagcgggatacagtggccggagaggccattgccaggtcctccacttcaaacaggagagacacctgctcgggcatcgcgatgcgctcgccgttgatgagggtcaacaccttgttatcgtccatgacggagttcatgttctcgatccacagtgtgtccacggggccatcgaacaggatccacttctcgtcgggtttctcatctgcacatgccgtccgcatgacactggacaagatgccatctgtccattcattggtgctgaggtcatattccccatacagttcccctagggacaatgccttggggttcaaagggaactctctaacaatgttgaagttagggtctccggcgcggcacagagaggacagggaggcctgtagaatgcgccatgaggcagtcttgccgctgcccgtgcagcccacgatcatggtggagtggcgggagttcttggtttcatacaactggaaaaccttggtgagggtgaacggcgtgctttgcaggcccatgtctcgaatctcctgctcaacggtctcccgcagcttgccatagtcaatgacaggcagctcaatgttgggaaacagatcttgcacgatggcattgaacaggggtgcatcaactgaagtgagcttggcgatgttcatatctctcattgagagcagcagaacctcttcatcagtcagatccggctgtaggcggcgcttcttgccagcatagcgcagaagggaggtgagggcacgcaggccaaagtcatagtggtcctgtctggacagctgctgcacagccagtgagtagagtgtgtacaccttcttggccagaatcttgcagttgccaaagccctctccaaagagaatgatttctgcaatgagggtggagtcaggcaccaccatggcaattgggcggaacatggatttaagattttcgggaagctctgtgcggccagcatagccaggattcatggtaatgaagatcccacaggaccacaccagatttatttcaaagccatcaaaatggaaatgggtgaggccggcagccagggcagacaggatgcacaggatctggtgggccaccactgacagcacctcgatgttgatgcggttaaactcatcaaagcagccccaagctccagtctgggccagacctgagtacattcggcccatggacttgtagtccaggccctcagagcagttgaccacaatgacatatatgcccagggccttgcccaggtccttgacggtctcggtcttgcctgtgcctgcagggcctttgggggagccccctcggtgcaggtgcaatgccgtggtcagtgtcatgtaacacctgtccgtcaggggggtgatgacgagccggcccgagttacccaagtactcataattatactgaaattgcgtgttggtctggcggatgacacagtcatcaagatccttctcccagtagaaccgaagttggctgagccagtcaaaggaattgacatccatgaggccactcttgtaaagcttctccaacacatcccgggcatgaatttctatcgtcaccagagccacaattttaagccgcatgatcttggtcaagttccccctgatggcttctgaatacttattcaggattgacacctggttcttcttcatgaccttgaggattttcttgtctgcccgctccttcgctgtcagcaggcacttggtgacatcagccgtccactggatctgactggcagtgatcaccacctggccagcccactccttcacccatttgtccctcttgttgaggaacttcctgagggccaggtggcagttccggagaaggtcccgcagggtcaccctcatggtctgttccacatcgccaagccaggactccacagggccttctaaaaatactgagtggaggaagtcaatgtactcgccgtcgcccgagaacatccccacagcttcccatttgctgctgggccctccaaccttctggattctcagcaacttgatgttgtcaaagcattttttgaggtgtggctgcacagcctctgggtttcgggactggcccagaatctccagcaggtcatcattggacaagaagtagaagcgggggaaaatatgtcgcttggtctctaaatacatatccagagatttctgaatatcttccaggattgtattcatttctatcaatgtgtccaggaggcctgggtgatgggtgctccggagagcattgttgtccttgttcatcctgtccatgatggctttccagttgctgttgacctggtcaaataaggtcgattcattgggcagctgcttgcggatgtcttctcctaggaagatattctctaagtacatccactgacgctgcactgtgagaatcatctcaataacctccaaaatgagggagaggcagcgttcccagtggtccacatccttctcaaaggccttgacaaagcgtgatgccttcatggtagacagagctacctggttatcttccagtgcctggaatacttcttctgtacctctgagccgatgatggcccttatccttgtagggtactatgtcgagctgagtcacatcccaggtcttggcaatgttttgtaaagccacttctatagccagctctttagttgctgaagcagagatctccccaattttctccacatgctgatccatcccaagctccacaatctgctccaaggtgaagctttcagattcctgatcaaactcccgctggatctcatcccggacctggtcccagtgcctctctctaagggcagggttccgcaggtctgagatgagaggcatggtcctcttgaactgctctatttttgagcgagtggtttcaataatttcccagtttcggtccttatactctttggctaattttgtgaggcgacgaaacagcccgtgggccgtggtctccatggtttccgtctgcaggatcaggaaccggccagtcttccactcattccagttctcctcccagtctcgtgcgatctcccagatttgctggagggcatcgagctccttctccaggttctgaaggtccttggagggtggctgctcgatcttgaagatgcccaggttggctcggagactattttcctcttcccgcatggccatcagcatggcccgcacttgtgtaatctggtctaaggcagacatgtatcccacgttgctggtgaaatggcctttgaattcgaaatcttccagaagtgtatgtgctttcttcttgaagtcatctgccgagtggatcaggcctgtcttgaatttctccttgtgtttcttcagcatttgcttactgtccagcagagtttgttggaagacaacccactccccgttgagactgtccagcatctccaggacactgtcctcgactggcacctcgtacttttcaagaatggcaaattgctcgtgtatgggagggatctgagtctccacgttggccaagtcgtgcttcagggcatccacgagctgcaagctgacccccagttcctccagtgtctgcggagggcggctgattttctctgcgttctccttcaggtaggtgtgcagctccaggaggcgcccagcagccatctccctgagcagagtcgcgaacttgttctgccattcattgcagtgctgcaccagggagaacttgaggtgcgaacagtccagcagcacaaactggatgttggtgactgtctcctccttctgcacgttattagcaacttccgtgtagcgggcaatgtcggcaacaaaagaagagacaggagggttgaggcgctggtagcgatgaatgaaggagtccttgttgatctcccagatctcccggtacatgtcccaggtcttgaggtagttctgcagcaggcttgcgttgttagtcatgccgctgctgatttgggtctggatcttcttgatgtcctcatcttgctccacaactgtttggatgggttcacgatgtaacttgcgcttggtgagaatgtcagggaggtggcagaagacagagatggtggaaaagaggtggttgccaatgtcattgaccacacctgccaaagtctgcagagtgggtgagaattccacctgtgccacacttccttgcagatcattcttcaaaatgacaaggacttggaagagtgggtttgggctggtctttccatccccgttgatagccttggatagttctagcagtgaccacttcacattcaggcgcagggcatcctccatcatgcggtccagccgaatcatgtacagcatccactgctgctgaatctcaggaccatcattcttgaagacctcataggagttggtcatgatggtcaccacatcctggtgcaggttcatcaatttctgctgtacagctgcccgatgctctctttggtcctcttcaaattccaggtccctgtatacccgtttgccactaatgcgtaccagcagcttctctgacatctcttgggctcgccagccaatggtcagagtggatgccttgaactcattcacaatcatctgcaccttgctggcatgtatacggcactccgtgatgaagaaggcactggcccccttcaaggcccagtgcagtttcttgagtcccgggtggatcttcttatccaggagccgaatacgctctttgaatagggcctgctcatctggggacagcatggcaataatcctattgtagtctctagcaacgagtagcagattttcacgcagaatgcgcaggtcctcggctcgctcagctacgttcaccacgtaatggggcgtctcaaacagcagccgctcccagtagtcaatttccgcaaagagaatcagaagggacctccaaggcaagtgtggctcaagtgtgatgataaatggcaactgacgcttggccttaaagttgagctgaagaggacatgctcccgcgaagaaagccatgctccacgctccaggcaattgttgccatctggaaatgtgggcccagtgtggatgcattttctgatttttcaagagaggccagaaattggtttttcatgtaaaatctcctgaattttaagtgctaacaacaattcacctgaaaaataattattcagtgggcatgtgggagaggctctaggactcctggcaatccttgacttgggcagtagtttgcaaggg

SEQ ID NO: 8716 - RNA, 8290 nt, Homo sapiens
  source 1..8290: mol_type = other RNA
aagccctgtctcctcccatctggccttctcgccagccaaccccgacacgagcatcccagctcgctccagcttcagctccatctcttcagacttcttgcgaagctcctccttctgtgccagcttctcatcatactgtttctttagcatctccagtttctcagctacctcccgcagcttctcctgggcctcagcgagcgcggcttgcttctcccgaagctgagccaaggcagcgttcattcggattcgcttgggctccaccacccgatatagccgcccatacagctccatggcccgcacccacatgcagagggacttggcagccagggagacgcggccgatgatatcaggctggaagtcaggctgggcgcagtaggccccaatcttcttcagaaccttatctgagatattgtctttatcaaagttgatcagtgacttgatgaagttctgttcccctagctgcctcttggcctctgcccatgtgggctcgttgcctcgaagaatcataactgcctgcatcactatctccacttgggctgggggccgtccataagacttgatctctcctatatccttcttgttcagagactccagggcccgcatggcctcttccagggcgggcagtgcctcttctagatctttctgggcattgtcagccagtgcctgacacttgatttcctcaactgcaatcttttcactgttggctgttacggccttctgctgctcatctgcctcccgcttctgctgcacaatgatgaccaggtactcctcacactgcttctggaactcagccaccttcttcttggcatcctccagctccaacgacatcacttgcaccttttccctagtttcgtcgatcttgaacaagcctgtccgcagtttattggcttgggccagcagctcctgccgtttttctcccagcaacttcttatatccagacaggagttccaggtatttggtgggtgtgacatagttgtgtctccgcagttccaacagcatcttctgggaatactgagctactgaccagtgcatagtgacaaagatctgggccaccttcctgtggatattctcctgagttcccaggtctactcctatgaggcacttctcagccacctcgagcagggcctcttggggccactctgagaaccagttgatggttgtgcagttcaccaaggctgggtactggcggatccagttcctgaagggatcccccatggggctgaggcagagcacgatgtgcaggttgttctgcacgcgttcaatgaggtaggcgaagaggctgtccgatgactcaggcacctgctccacccgggcctggtctatgatatgcgactggatctcttcaaattcatcaggcttgtagagattgggcacctcgcctgagctgaggatgttgttgatgtcctctaggaaggactcatcagctatttgggtgtccacaaaaatgaaggacgtggtcttgagctccaccccagcctggcgatacagacgcttgatatcatctcggaactcctgcttccgataatgtttggtgacctcgatctggaaggtggtgtagtcgcagatggatgaagccaggcgggccagactctggcgtccgctgcccccgatacccaccaggagcatgttgccccgaggctgtccaatgacccgcacgatccgtgtgatgtgttcaatagcctctcggaagagcactagctgcatgggcacgacagagggtgacaggttatactcatttagagctgtctccatgactgtcttcagcactgtcagatccgtgaggtcttcatacaccttgggctccttcaggaaatccccaaagataggaggacgcttgctgggacagagatgatgaaatgtgaggtcaaagaaggagccgagcttgtcgcttatgatgcccatgaaggcttctgtgtctgccgcatcaaccagccggtcagagaagactctgaaacattcatggatccagagccgtgtgatgctggacttggtatcatggaagtccttgttggctctaagcatgccctggaacaccttggagatgtctcgaaggttgaagaggtaatgcatcttggtgggcgtgggcaggaagcgctgtaccacggtgttgtacatgtccagggtggcctctgtcaccacgttcccaatgggcttcacctcttcctcaaagtcctgaagcttctgattgatcatggtgccgaatatgcggatgatctgggactttgtggggaaggtcatgttgataatgttgaagcgactccgtagccttggggagatgacagtccgtccacccccaggggggcccatggcagccatcaggaacatttctcgaatgtacttgatggtctgcttcgtacggtcataccagaagccatagtcaatccagaggcggatcagctccaggggtggctgggacccaaacatgtccttagcgggcatatttaggtcatccataaaggtgatcatgcttttgcccccgaatggcacgtagacacccttggttcgcttctcaaccctgctctcaatgatgctctgcacgttattggatgtggtctgtgcggacatgttgacaacgagcaccgaccactggctggagggcagggactgcagaacgctctgggcgatggaggtcttcccagtccccacgggacccaccagcagaatgggattctggttggccaccaagctgctcaccaggtagttgtagcgaacagtgtcgacggtgggcaccatgatcttatagaagggggcgtttggagggtagcgccaactcttagggagcttgtcctcaaatgatgtccaactccgtattttggggtccacaaaatactcatataccgtgtccttattgggaaaggagccctcgatctctcggaggtagctgtcgatcctcttccggccctcctcatccacagaggcacacacagaccagatcatgctgaacacaaatgtcatctctaccatggtgacatagttctcgccgtcagctgggttcaccccattctctggcgtggccagggcagagtacagcttgcagagggaggtgataccgctgtactcgggcaggggcaccagctccttgcagttgtccttcttaaaggccagcatcttgttgatgagcttttcgaacatgcgttgaaggggctccacctcagcctttggcctcttctccagccatgactgaacatagggcttccagcccaggtcagcgtagtcagtgtagaccatcccgcagcgggatacagtggccggagaggccattgccaggtcctccacttcaaacaggagagacacctgctcgggcatcgcgatgcgctcgccgttgatgagggtcaacaccttgttatcgtccatgacggagttcatgttctcgatccacagtgtgtccacggggccatcgaacaggatccacttctcgtcgggtttctcatctgcacatgccgtccgcatgacactggacaagatgccatctgtccattcattggtgctgaggtcatattccccatacagttcccctagggacaatgccttggggttcaaagggaactctctaacaatgttgaagttagggtctccggcgcggcacagagaggacagggaggcctgtagaatgcgccatgaggcagtcttgccgctgcccgtgcagcccacgatcatggtggagtggcgggagttcttggtttcatacaactggaaaaccttggtgagggtgaacggcgtgctttgcaggcccatgtctcgaatctcctgctcaacggtctcccgcagcttgccatagtcaatgacaggcagctcaatgttgggaaacagatcttgcacgatggcattgaacaggggtgcatcaactgaagtgagcttggcgatgttcatatctctcattgagagcagcagaacctcttcatcagtcagatccggctgtaggcggcgcttcttgccagcatagcgcagaagggaggtgagggcacgcaggccaaagtcatagtggtcctgtctggacagctgctgcacagccagtgagtagagtgtgtacaccttcttggccagaatcttgcagttgccaaagccctctccaaagagaatgatttctgcaatgagggtggagtcaggcaccaccatggcaattgggcggaacatggatttaagattttcgggaagctctgtgcggccagcatagccaggattcatggtaatgaagatcccacaggaccacaccagatttatttcaaagccatcaaaatggaaatgggtgaggccggcagccagggcagacaggatgcacaggatctggtgggccaccactgacagcacctcgatgttgatgcggttaaactcatcaaagcagccccaagctccagtctgggccagacctgagtacattcggcccatggacttgtagtccaggccctcagagcagttgaccacaatgacatatatgcccagggccttgcccaggtccttgacggtctcggtcttgcctgtgcctgcagggcctttgggggagccccctcggtgcaggtgcaatgccgtggtcagtgtcatgtaacacctgtccgtcaggggggtgatgacgagccggcccgagttacccaagtactcataattatactgaaattgcgtgttggtctggcggatgacacagtcatcaagatccttctcccagtagaaccgaagttggctgagccagtcaaaggaattgacatccatgaggccactcttgtaaagcttctccaacacatcccgggcatgaatttctatcgtcaccagagccacaattttaagccgcatgatcttggtcaagttccccctgatggcttctgaatacttattcaggattgacacctggttcttcttcatgaccttgaggattttcttgtctgcccgctccttcgctgtcagcaggcacttggtgacatcagccgtccactggatctgactggcagtgatcaccacctggccagcccactccttcacccatttgtccctcttgttgaggaacttcctgagggccaggtggcagttccggagaaggtcccgcagggtcaccctcatggtctgttccacatcgccaagccaggactccacagggccttctaaaaatactgagtggaggaagtcaatgtactcgccgtcgcccgagaacatccccacagcttcccatttgctgctgggccctccaaccttctggattctcagcaacttgatgttgtcaaagcattttttgaggtgtggctgcacagcctctgggtttcgggactggcccagaatctccagcaggtcatcattggacaagaagtagaagcgggggaaaatatgtcgcttggtctctaaatacatatccagagatttctgaatatcttccaggattgtattcatttctatcaatgtgtccaggaggcctgggtgatgggtgctccggagagcattgttgtccttgttcatcctgtccatgatggctttccagttgctgttgacctggtcaaataaggtcgattcattgggcagctgcttgcggatgtcttctcctaggaagatattctctaagtacatccactgacgctgcactgtgagaatcatctcaataacctccaaaatgagggagaggcagcgttcccagtggtccacatccttctcaaaggccttgacaaagcgtgatgccttcatggtagacagagctacctggttatcttccagtgcctggaatacttcttctgtacctctgagccgatgatggcccttatccttgtagggtactatgtcgagctgagtcacatcccaggtcttggcaatgttttgtaaagccacttctatagccagctctttagttgctgaagcagagatctccccaattttctccacatgctgatccatcccaagctccacaatctgctccaaggtgaagctttcagattcctgatcaaactcccgctggatctcatcccggacctggtcccagtgcctctctctaagggcagggttccgcaggtctgagatgagaggcatggtcctcttgaactgctctatttttgagcgagtggtttcaataatttcccagtttcggtccttatactctttggctaattttgtgaggcgacgaaacagcccgtgggccgtggtctccatggtttccgtctgcaggatcaggaaccggccagtcttccactcattccagttctcctcccagtctcgtgcgatctcccagatttgctggagggcatcgagctccttctccaggttctgaaggtccttggagggtggctgctcgatcttgaagatgcccaggttggctcggagactattttcctcttcccgcatggccatcagcatggcccgcacttgtgtaatctggtctaaggcagacatgtatcccacgttgctggtgaaatggcctttgaattcgaaatcttccagaagtgtatgtgctttcttcttgaagtcatctgccgagtggatcaggcctgtcttgaatttctccttgtgtttcttcagcatttgcttactgtccagcagagtttgttggaagacaacccactccccgttgagactgtccagcatctccaggacactgtcctcgactggcacctcgtacttttcaagaatggcaaattgctcgtgtatgggagggatctgagtctccacgttggccaagtcgtgcttcagggcatccacgagctgcaagctgacccccagttcctccagtgtctgcggagggcggctgattttctctgcgttctccttcaggtaggtgtgcagctccaggaggcgcccagcagccatctccctgagcagagtcgcgaacttgttctgccattcattgcagtgctgcaccagggagaacttgaggtgcgaacagtccagcagcacaaactggatgttggtgactgtctcctccttctgcacgttattagcaacttccgtgtagcgggcaatgtcggcaacaaaagaagagacaggagggttgaggcgctggtagcgatgaatgaaggagtccttgttgatctcccagatctcccggtacatgtcccaggtcttgaggtagttctgcagcaggcttgcgttgttagtcatgccgctgctgatttgggtctggatcttcttgatgtcctcatcttgctccacaactgtttggatgggttcacgatgtaacttgcgcttggtgagaatgtcagggaggtggcagaagacagagatggtggaaaagaggtggttgccaatgtcattgaccacacctgccaaagtctgcagagtgggtgagaattccacctgtgccacacttccttgcagatcattcttcaaaatgacaaggacttggaagagtgggtttgggctggtctttccatccccgttgatagccttggatagttctagcagtgaccacttcacattcaggcgcagggcatcctccatcatgcggtccagccgaatcatgtacagcatccactgctgctgaatctcaggaccatcattcttgaagacctcataggagttggtcatgatggtcaccacatcctggtgcaggttcatcaatttctgctgtacagctgcccgatgctctctttggtcctcttcaaattccaggtccctgtatacccgtttgccactaatgcgtaccagcagcttctctgacatctcttgggctcgccagccaatggtcagagtggatgccttgaactcattcacaatcatctgcaccttgctggcatgtatacggcactccgtgatgaagaaggcactggcccccttcaaggcccagtgcagtttcttgagtcccgggtggatcttcttatccaggagccgaatacgctctttgaatagggcctgctcatctggggacagcatggcaataatcctattgtagtctctagcaacgagtagcagattttcacgcagaatgcgcaggtcctcggctcgctcagctacgttcaccacgtaatggggcgtctcaaacagcagccgctcccagtagtcaatttccgcaaagagaatcagaagggacttgtcaaagttgacatccagcatgcccgccttctcctggctgattcgcagcaatggggtatccaaccgccgaatgcaatccttgtccagacttgatgtccactcttggaaggtttttcgaaccagctcatcaatggcctggaccatctgctgataggtgtgcacactctcctttccagtcccaatacggggcaggaaatgagcaccagcaaggcactcactgaactggacctgccactcccctcaccgacataggtgctggtcctgaagactctttggggaacctctcaggagccatccc

SEQ ID NO: 8717 - RNA, 8604 nt, Homo sapiens
  source 1..8604: mol_type = other RNA
aagccctgtctcctcccatctggccttctcgccagccaaccccgacacgagcatcccagctcgctccagcttcagctccatctcttcagacttcttgcgaagctcctccttctgtgccagcttctcatcatactgtttctttagcatctccagtttctcagctacctcccgcagcttctcctgggcctcagcgagcgcggcttgcttctcccgaagctgagccaaggcagcgttcattcggattcgcttgggctccaccacccgatatagccgcccatacagctccatggcccgcacccacatgcagagggacttggcagccagggagacgcggccgatgatatcaggctggaagtcaggctgggcgcagtaggccccaatcttcttcagaaccttatctgagatattgtctttatcaaagttgatcagtgacttgatgaagttctgttcccctagctgcctcttggcctctgcccatgtgggctcgttgcctcgaagaatcataactgcctgcatcactatctccacttgggctgggggccgtccataagacttgatctctcctatatccttcttgttcagagactccagggcccgcatggcctcttccagggcgggcagtgcctcttctagatctttctgggcattgtcagccagtgcctgacacttgatttcctcaactgcaatcttttcactgttggctgttacggccttctgctgctcatctgcctcccgcttctgctgcacaatgatgaccaggtactcctcacactgcttctggaactcagccaccttcttcttggcatcctccagctccaacgacatcacttgcaccttttccctagtttcgtcgatcttgaacaagcctgtccgcagtttattggcttgggccagcagctcctgccgtttttctcccagcaacttcttatatccagacaggagttccaggtatttggtgggtgtgacatagttgtgtctccgcagttccaacagcatcttctgggaatactgagctactgaccagtgcatagtgacaaagatctgggccaccttcctgtggatattctcctgagttcccaggtctactcctatgaggcacttctcagccacctcgagcagggcctcttggggccactctgagaaccagttgatggttgtgcagttcaccaaggctgggtactggcggatccagttcctgaagggatcccccatggggctgaggcagagcacgatgtgcaggttgttctgcacgcgttcaatgaggtaggcgaagaggctgtccgatgactcaggcacctgctccacccgggcctggtctatgatatgcgactggatctcttcaaattcatcaggcttgtagagattgggcacctcgcctgagctgaggatgttgttgatgtcctctaggaaggactcatcagctatttgggtgtccacaaaaatgaaggacgtggtcttgagctccaccccagcctggcgatacagacgcttgatatcatctcggaactcctgcttccgataatgtttggtgacctcgatctggaaggtggtgtagtcgcagatggatgaagccaggcgggccagactctggcgtccgctgcccccgatacccaccaggagcatgttgccccgaggctgtccaatgacccgcacgatccgtgtgatgtgttcaatagcctctcggaagagcactagctgcatgggcacgacagagggtgacaggttatactcatttagagctgtctccatgactgtcttcagcactgtcagatccgtgaggtcttcatacaccttgggctccttcaggaaatccccaaagataggaggacgcttgctgggacagagatgatgaaatgtgaggtcaaagaaggagccgagcttgtcgcttatgatgcccatgaaggcttctgtgtctgccgcatcaaccagccggtcagagaagactctgaaacattcatggatccagagccgtgtgatgctggacttggtatcatggaagtccttgttggctctaagcatgccctggaacaccttggagatgtctcgaaggttgaagaggtaatgcatcttggtgggcgtgggcaggaagcgctgtaccacggtgttgtacatgtccagggtggcctctgtcaccacgttcccaatgggcttcacctcttcctcaaagtcctgaagcttctgattgatcatggtgccgaatatgcggatgatctgggactttgtggggaaggtcatgttgataatgttgaagcgactccgtagccttggggagatgacagtccgtccacccccaggggggcccatggcagccatcaggaacatttctcgaatgtacttgatggtctgcttcgtacggtcataccagaagccatagtcaatccagaggcggatcagctccaggggtggctgggacccaaacatgtccttagcgggcatatttaggtcatccataaaggtgatcatgcttttgcccccgaatggcacgtagacacccttggttcgcttctcaaccctgctctcaatgatgctctgcacgttattggatgtggtctgtgcggacatgttgacaacgagcaccgaccactggctggagggcagggactgcagaacgctctgggcgatggaggtcttcccagtccccacgggacccaccagcagaatgggattctggttggccaccaagctgctcaccaggtagttgtagcgaacagtgtcgacggtgggcaccatgatcttatagaagggggcgtttggagggtagcgccaactcttagggagcttgtcctcaaatgatgtccaactccgtattttggggtccacaaaatactcatataccgtgtccttattgggaaaggagccctcgatctctcggaggtagctgtcgatcctcttccggccctcctcatccacagaggcacacacagaccagatcatgctgaacacaaatgtcatctctaccatggtgacatagttctcgccgtcagctgggttcaccccattctctggcgtggccagggcagagtacagcttgcagagggaggtgataccgctgtactcgggcaggggcaccagctccttgcagttgtccttcttaaaggccagcatcttgttgatgagcttttcgaacatgcgttgaaggggctccacctcagcctttggcctcttctccagccatgactgaacatagggcttccagcccaggtcagcgtagtcagtgtagaccatcccgcagcgggatacagtggccggagaggccattgccaggtcctccacttcaaacaggagagacacctgctcgggcatcgcgatgcgctcgccgttgatgagggtcaacaccttgttatcgtccatgacggagttcatgttctcgatccacagtgtgtccacggggccatcgaacaggatccacttctcgtcgggtttctcatctgcacatgccgtccgcatgacactggacaagatgccatctgtccattcattggtgctgaggtcatattccccatacagttcccctagggacaatgccttggggttcaaagggaactctctaacaatgttgaagttagggtctccggcgcggcacagagaggacagggaggcctgtagaatgcgccatgaggcagtcttgccgctgcccgtgcagcccacgatcatggtggagtggcgggagttcttggtttcatacaactggaaaaccttggtgagggtgaacggcgtgctttgcaggcccatgtctcgaatctcctgctcaacggtctcccgcagcttgccatagtcaatgacaggcagctcaatgttgggaaacagatcttgcacgatggcattgaacaggggtgcatcaactgaagtgagcttggcgatgttcatatctctcattgagagcagcagaacctcttcatcagtcagatccggctgtaggcggcgcttcttgccagcatagcgcagaagggaggtgagggcacgcaggccaaagtcatagtggtcctgtctggacagctgctgcacagccagtgagtagagtgtgtacaccttcttggccagaatcttgcagttgccaaagccctctccaaagagaatgatttctgcaatgagggtggagtcaggcaccaccatggcaattgggcggaacatggatttaagattttcgggaagctctgtgcggccagcatagccaggattcatggtaatgaagatcccacaggaccacaccagatttatttcaaagccatcaaaatggaaatgggtgaggccggcagccagggcagacaggatgcacaggatctggtgggccaccactgacagcacctcgatgttgatgcggttaaactcatcaaagcagccccaagctccagtctgggccagacctgagtacattcggcccatggacttgtagtccaggccctcagagcagttgaccacaatgacatatatgcccagggccttgcccaggtccttgacggtctcggtcttgcctgtgcctgcagggcctttgggggagccccctcggtgcaggtgcaatgccgtggtcagtgtcatgtaacacctgtccgtcaggggggtgatgacgagccggcccgagttacccaagtactcataattatactgaaattgcgtgttggtctggcggatgacacagtcatcaagatccttctcccagtagaaccgaagttggctgagccagtcaaaggaattgacatccatgaggccactcttgtaaagcttctccaacacatcccgggcatgaatttctatcgtcaccagagccacaattttaagccgcatgatcttggtcaagttccccctgatggcttctgaatacttattcaggattgacacctggttcttcttcatgaccttgaggattttcttgtctgcccgctccttcgctgtcagcaggcacttggtgacatcagccgtccactggatctgactggcagtgatcaccacctggccagcccactccttcacccatttgtccctcttgttgaggaacttcctgagggccaggtggcagttccggagaaggtcccgcagggtcaccctcatggtctgttccacatcgccaagccaggactccacagggccttctaaaaatactgagtggaggaagtcaatgtactcgccgtcgcccgagaacatccccacagcttcccatttgctgctgggccctccaaccttctggattctcagcaacttgatgttgtcaaagcattttttgaggtgtggctgcacagcctctgggtttcgggactggcccagaatctccagcaggtcatcattggacaagaagtagaagcgggggaaaatatgtcgcttggtctctaaatacatatccagagatttctgaatatcttccaggattgtattcatttctatcaatgtgtccaggaggcctgggtgatgggtgctccggagagcattgttgtccttgttcatcctgtccatgatggctttccagttgctgttgacctggtcaaataaggtcgattcattgggcagctgcttgcggatgtcttctcctaggaagatattctctaagtacatccactgacgctgcactgtgagaatcatctcaataacctccaaaatgagggagaggcagcgttcccagtggtccacatccttctcaaaggccttgacaaagcgtgatgccttcatggtagacagagctacctggttatcttccagtgcctggaatacttcttctgtacctctgagccgatgatggcccttatccttgtagggtactatgtcgagctgagtcacatcccaggtcttggcaatgttttgtaaagccacttctatagccagctctttagttgctgaagcagagatctccccaattttctccacatgctgatccatcccaagctccacaatctgctccaaggtgaagctttcagattcctgatcaaactcccgctggatctcatcccggacctggtcccagtgcctctctctaagggcagggttccgcaggtctgagatgagaggcatggtcctcttgaactgctctatttttgagcgagtggtttcaataatttcccagtttcggtccttatactctttggctaattttgtgaggcgacgaaacagcccgtgggccgtggtctccatggtttccgtctgcaggatcaggaaccggccagtcttccactcattccagttctcctcccagtctcgtgcgatctcccagatttgctggagggcatcgagctccttctccaggttctgaaggtccttggagggtggctgctcgatcttgaagatgcccaggttggctcggagactattttcctcttcccgcatggccatcagcatggcccgcacttgtgtaatctggtctaaggcagacatgtatcccacgttgctggtgaaatggcctttgaattcgaaatcttccagaagtgtatgtgctttcttcttgaagtcatctgccgagtggatcaggcctgtcttgaatttctccttgtgtttcttcagcatttgcttactgtccagcagagtttgttggaagacaacccactccccgttgagactgtccagcatctccaggacactgtcctcgactggcacctcgtacttttcaagaatggcaaattgctcgtgtatgggagggatctgagtctccacgttggccaagtcgtgcttcagggcatccacgagctgcaagctgacccccagttcctccagtgtctgcggagggcggctgattttctctgcgttctccttcaggtaggtgtgcagctccaggaggcgcccagcagccatctccctgagcagagtcgcgaacttgttctgccattcattgcagtgctgcaccagggagaacttgaggtgcgaacagtccagcagcacaaactggatgttggtgactgtctcctccttctgcacgttattagcaacttccgtgtagcgggcaatgtcggcaacaaaagaagagacaggagggttgaggcgctggtagcgatgaatgaaggagtccttgttgatctcccagatctcccggtacatgtcccaggtcttgaggtagttctgcagcaggcttgcgttgttagtcatgccgctgctgatttgggtctggatcttcttgatgtcctcatcttgctccacaactgtttggatgggttcacgatgtaacttgcgcttggtgagaatgtcagggaggtggcagaagacagagatggtggaaaagaggtggttgccaatgtcattgaccacacctgccaaagtctgcagagtgggtgagaattccacctgtgccacacttccttgcagatcattcttcaaaatgacaaggacttggaagagtgggtttgggctggtctttccatccccgttgatagccttggatagttctagcagtgaccacttcacattcaggcgcagggcatcctccatcatgcggtccagccgaatcatgtacagcatccactgctgctgaatctcaggaccatcattcttgaagacctcataggagttggtcatgatggtcaccacatcctggtgcaggttcatcaatttctgctgtacagctgcccgatgctctctttggtcctcttcaaattccaggtccctgtatacccgtttgccactaatgcgtaccagcagcttctctgacatctcttgggctcgccagccaatggtcagagtggatgccttgaactcattcacaatcatctgcaccttgctggcatgtatacggcactccgtgatgaagaaggcactggcccccttcaaggcccagtgcagtttcttgagtcccgggtggatcttcttatccaggagccgaatacgctctttgaatagggcctgctcatctggggacagcatggcaataatcctattgtagtctctagcaacgagtagcagattttcacgcagaatgcgcaggtcctcggctcgctcagctacgttcaccacgtaatggggcgtctcaaacagcagccgctcccagtagtcaatttccgcaaagagaatcagaagggacttgtcaaagttgacatccagcatgcccgccttctcctggctgattcgcagcaatggggtatccaaccgccgaatgcaatccttgtccagacttgatgtccactcttggaaggtttttcgaaccagctcatcaatggcctggaccatctgctgataggtgtgcacactctcctttccagtcccaatacggggcaggaaatgagcaccagcaaggcaggtcatgactctgtcgatgcgacgccggaggatgtgcacccagcgcgcctttccggaatactgggccacgtagggctccaggtctggccatttcttgttccgttcacggttcaccagggccagctcgctattgaacagcatgtagagatccaccgccttcttgtcataagtccgcttgatagcctcgcgggaggcaagcctgtggaaggtgtccagcagaagcacgccgtgcggcacgtcccgcaccaactcgaaggctgaggtgatcaggttctgggtcatcacctccaggtccttgattccggcacggaacctacatgaatccatttaatcctcaaaacaatgctgtgagatgggctctatctctaaccgtattgcatagaggaggaagtggagaca

SEQ ID NO: 8718 - RNA, 10371 nt, Homo sapiens
  source 1..10371: mol_type = other RNA
aagccctgtctcctcccatctggccttctcgccagccaaccccgacacgagcatcccagctcgctccagcttcagctccatctcttcagacttcttgcgaagctcctccttctgtgccagcttctcatcatactgtttctttagcatctccagtttctcagctacctcccgcagcttctcctgggcctcagcgagcgcggcttgcttctcccgaagctgagccaaggcagcgttcattcggattcgcttgggctccaccacccgatatagccgcccatacagctccatggcccgcacccacatgcagagggacttggcagccagggagacgcggccgatgatatcaggctggaagtcaggctgggcgcagtaggccccaatcttcttcagaaccttatctgagatattgtctttatcaaagttgatcagtgacttgatgaagttctgttcccctagctgcctcttggcctctgcccatgtgggctcgttgcctcgaagaatcataactgcctgcatcactatctccacttgggctgggggccgtccataagacttgatctctcctatatccttcttgttcagagactccagggcccgcatggcctcttccagggcgggcagtgcctcttctagatctttctgggcattgtcagccagtgcctgacacttgatttcctcaactgcaatcttttcactgttggctgttacggccttctgctgctcatctgcctcccgcttctgctgcacaatgatgaccaggtactcctcacactgcttctggaactcagccaccttcttcttggcatcctccagctccaacgacatcacttgcaccttttccctagtttcgtcgatcttgaacaagcctgtccgcagtttattggcttgggccagcagctcctgccgtttttctcccagcaacttcttatatccagacaggagttccaggtatttggtgggtgtgacatagttgtgtctccgcagttccaacagcatcttctgggaatactgagctactgaccagtgcatagtgacaaagatctgggccaccttcctgtggatattctcctgagttcccaggtctactcctatgaggcacttctcagccacctcgagcagggcctcttggggccactctgagaaccagttgatggttgtgcagttcaccaaggctgggtactggcggatccagttcctgaagggatcccccatggggctgaggcagagcacgatgtgcaggttgttctgcacgcgttcaatgaggtaggcgaagaggctgtccgatgactcaggcacctgctccacccgggcctggtctatgatatgcgactggatctcttcaaattcatcaggcttgtagagattgggcacctcgcctgagctgaggatgttgttgatgtcctctaggaaggactcatcagctatttgggtgtccacaaaaatgaaggacgtggtcttgagctccaccccagcctggcgatacagacgcttgatatcatctcggaactcctgcttccgataatgtttggtgacctcgatctggaaggtggtgtagtcgcagatggatgaagccaggcgggccagactctggcgtccgctgcccccgatacccaccaggagcatgttgccccgaggctgtccaatgacccgcacgatccgtgtgatgtgttcaatagcctctcggaagagcactagctgcatgggcacgacagagggtgacaggttatactcatttagagctgtctccatgactgtcttcagcactgtcagatccgtgaggtcttcatacaccttgggctccttcaggaaatccccaaagataggaggacgcttgctgggacagagatgatgaaatgtgaggtcaaagaaggagccgagcttgtcgcttatgatgcccatgaaggcttctgtgtctgccgcatcaaccagccggtcagagaagactctgaaacattcatggatccagagccgtgtgatgctggacttggtatcatggaagtccttgttggctctaagcatgccctggaacaccttggagatgtctcgaaggttgaagaggtaatgcatcttggtgggcgtgggcaggaagcgctgtaccacggtgttgtacatgtccagggtggcctctgtcaccacgttcccaatgggcttcacctcttcctcaaagtcctgaagcttctgattgatcatggtgccgaatatgcggatgatctgggactttgtggggaaggtcatgttgataatgttgaagcgactccgtagccttggggagatgacagtccgtccacccccaggggggcccatggcagccatcaggaacatttctcgaatgtacttgatggtctgcttcgtacggtcataccagaagccatagtcaatccagaggcggatcagctccaggggtggctgggacccaaacatgtccttagcgggcatatttaggtcatccataaaggtgatcatgcttttgcccccgaatggcacgtagacacccttggttcgcttctcaaccctgctctcaatgatgctctgcacgttattggatgtggtctgtgcggacatgttgacaacgagcaccgaccactggctggagggcagggactgcagaacgctctgggcgatggaggtcttcccagtccccacgggacccaccagcagaatgggattctggttggccaccaagctgctcaccaggtagttgtagcgaacagtgtcgacggtgggcaccatgatcttatagaagggggcgtttggagggtagcgccaactcttagggagcttgtcctcaaatgatgtccaactccgtattttggggtccacaaaatactcatataccgtgtccttattgggaaaggagccctcgatctctcggaggtagctgtcgatcctcttccggccctcctcatccacagaggcacacacagaccagatcatgctgaacacaaatgtcatctctaccatggtgacatagttctcgccgtcagctgggttcaccccattctctggcgtggccagggcagagtacagcttgcagagggaggtgataccgctgtactcgggcaggggcaccagctccttgcagttgtccttcttaaaggccagcatcttgttgatgagcttttcgaacatgcgttgaaggggctccacctcagcctttggcctcttctccagccatgactgaacatagggcttccagcccaggtcagcgtagtcagtgtagaccatcccgcagcgggatacagtggccggagaggccattgccaggtcctccacttcaaacaggagagacacctgctcgggcatcgcgatgcgctcgccgttgatgagggtcaacaccttgttatcgtccatgacggagttcatgttctcgatccacagtgtgtccacggggccatcgaacaggatccacttctcgtcgggtttctcatctgcacatgccgtccgcatgacactggacaagatgccatctgtccattcattggtgctgaggtcatattccccatacagttcccctagggacaatgccttggggttcaaagggaactctctaacaatgttgaagttagggtctccggcgcggcacagagaggacagggaggcctgtagaatgcgccatgaggcagtcttgccgctgcccgtgcagcccacgatcatggtggagtggcgggagttcttggtttcatacaactggaaaaccttggtgagggtgaacggcgtgctttgcaggcccatgtctcgaatctcctgctcaacggtctcccgcagcttgccatagtcaatgacaggcagctcaatgttgggaaacagatcttgcacgatggcattgaacaggggtgcatcaactgaagtgagcttggcgatgttcatatctctcattgagagcagcagaacctcttcatcagtcagatccggctgtaggcggcgcttcttgccagcatagcgcagaagggaggtgagggcacgcaggccaaagtcatagtggtcctgtctggacagctgctgcacagccagtgagtagagtgtgtacaccttcttggccagaatcttgcagttgccaaagccctctccaaagagaatgatttctgcaatgagggtggagtcaggcaccaccatggcaattgggcggaacatggatttaagattttcgggaagctctgtgcggccagcatagccaggattcatggtaatgaagatcccacaggaccacaccagatttatttcaaagccatcaaaatggaaatgggtgaggccggcagccagggcagacaggatgcacaggatctggtgggccaccactgacagcacctcgatgttgatgcggttaaactcatcaaagcagccccaagctccagtctgggccagacctgagtacattcggcccatggacttgtagtccaggccctcagagcagttgaccacaatgacatatatgcccagggccttgcccaggtccttgacggtctcggtcttgcctgtgcctgcagggcctttgggggagccccctcggtgcaggtgcaatgccgtggtcagtgtcatgtaacacctgtccgtcaggggggtgatgacgagccggcccgagttacccaagtactcataattatactgaaattgcgtgttggtctggcggatgacacagtcatcaagatccttctcccagtagaaccgaagttggctgagccagtcaaaggaattgacatccatgaggccactcttgtaaagcttctccaacacatcccgggcatgaatttctatcgtcaccagagccacaattttaagccgcatgatcttggtcaagttccccctgatggcttctgaatacttattcaggattgacacctggttcttcttcatgaccttgaggattttcttgtctgcccgctccttcgctgtcagcaggcacttggtgacatcagccgtccactggatctgactggcagtgatcaccacctggccagcccactccttcacccatttgtccctcttgttgaggaacttcctgagggccaggtggcagttccggagaaggtcccgcagggtcaccctcatggtctgttccacatcgccaagccaggactccacagggccttctaaaaatactgagtggaggaagtcaatgtactcgccgtcgcccgagaacatccccacagcttcccatttgctgctgggccctccaaccttctggattctcagcaacttgatgttgtcaaagcattttttgaggtgtggctgcacagcctctgggtttcgggactggcccagaatctccagcaggtcatcattggacaagaagtagaagcgggggaaaatatgtcgcttggtctctaaatacatatccagagatttctgaatatcttccaggattgtattcatttctatcaatgtgtccaggaggcctgggtgatgggtgctccggagagcattgttgtccttgttcatcctgtccatgatggctttccagttgctgttgacctggtcaaataaggtcgattcattgggcagctgcttgcggatgtcttctcctaggaagatattctctaagtacatccactgacgctgcactgtgagaatcatctcaataacctccaaaatgagggagaggcagcgttcccagtggtccacatccttctcaaaggccttgacaaagcgtgatgccttcatggtagacagagctacctggttatcttccagtgcctggaatacttcttctgtacctctgagccgatgatggcccttatccttgtagggtactatgtcgagctgagtcacatcccaggtcttggcaatgttttgtaaagccacttctatagccagctctttagttgctgaagcagagatctccccaattttctccacatgctgatccatcccaagctccacaatctgctccaaggtgaagctttcagattcctgatcaaactcccgctggatctcatcccggacctggtcccagtgcctctctctaagggcagggttccgcaggtctgagatgagaggcatggtcctcttgaactgctctatttttgagcgagtggtttcaataatttcccagtttcggtccttatactctttggctaattttgtgaggcgacgaaacagcccgtgggccgtggtctccatggtttccgtctgcaggatcaggaaccggccagtcttccactcattccagttctcctcccagtctcgtgcgatctcccagatttgctggagggcatcgagctccttctccaggttctgaaggtccttggagggtggctgctcgatcttgaagatgcccaggttggctcggagactattttcctcttcccgcatggccatcagcatggcccgcacttgtgtaatctggtctaaggcagacatgtatcccacgttgctggtgaaatggcctttgaattcgaaatcttccagaagtgtatgtgctttcttcttgaagtcatctgccgagtggatcaggcctgtcttgaatttctccttgtgtttcttcagcatttgcttactgtccagcagagtttgttggaagacaacccactccccgttgagactgtccagcatctccaggacactgtcctcgactggcacctcgtacttttcaagaatggcaaattgctcgtgtatgggagggatctgagtctccacgttggccaagtcgtgcttcagggcatccacgagctgcaagctgacccccagttcctccagtgtctgcggagggcggctgattttctctgcgttctccttcaggtaggtgtgcagctccaggaggcgcccagcagccatctccctgagcagagtcgcgaacttgttctgccattcattgcagtgctgcaccagggagaacttgaggtgcgaacagtccagcagcacaaactggatgttggtgactgtctcctccttctgcacgttattagcaacttccgtgtagcgggcaatgtcggcaacaaaagaagagacaggagggttgaggcgctggtagcgatgaatgaaggagtccttgttgatctcccagatctcccggtacatgtcccaggtcttgaggtagttctgcagcaggcttgcgttgttagtcatgccgctgctgatttgggtctggatcttcttgatgtcctcatcttgctccacaactgtttggatgggttcacgatgtaacttgcgcttggtgagaatgtcagggaggtggcagaagacagagatggtggaaaagaggtggttgccaatgtcattgaccacacctgccaaagtctgcagagtgggtgagaattccacctgtgccacacttccttgcagatcattcttcaaaatgacaaggacttggaagagtgggtttgggctggtctttccatccccgttgatagccttggatagttctagcagtgaccacttcacattcaggcgcagggcatcctccatcatgcggtccagccgaatcatgtacagcatccactgctgctgaatctcaggaccatcattcttgaagacctcataggagttggtcatgatggtcaccacatcctggtgcaggttcatcaatttctgctgtacagctgcccgatgctctctttggtcctcttcaaattccaggtccctgtatacccgtttgccactaatgcgtaccagcagcttctctgacatctcttgggctcgccagccaatggtcagagtggatgccttgaactcattcacaatcatctgcaccttgctggcatgtatacggcactccgtgatgaagaaggcactggcccccttcaaggcccagtgcagtttcttgagtcccgggtggatcttcttatccaggagccgaatacgctctttgaatagggcctgctcatctggggacagcatggcaataatcctattgtagtctctagcaacgagtagcagattttcacgcagaatgcgcaggtcctcggctcgctcagctacgttcaccacgtaatggggcgtctcaaacagcagccgctcccagtagtcaatttccgcaaagagaatcagaagggacttgtcaaagttgacatccagcatgcccgccttctcctggctgattcgcagcaatggggtatccaaccgccgaatgcaatccttgtccagacttgatgtccactcttggaaggtttttcgaaccagctcatcaatggcctggaccatctgctgataggtgtgcacactctcctttccagtcccaatacggggcaggaaatgagcaccagcaaggcaggtcatgactctgtcgatgcgacgccggaggatgtgcacccagcgcgcctttccggaatactgggccacgtagggctccaggtctggccatttcttgttccgttcacggttcaccagggccagctcgctattgaacagcatgtagagatccaccgccttcttgtcataagtccgcttgatagcctcgcgggaggcaagcctgtggaaggtgtccagcagaagcacgccgtgcggcacgtcccgcaccaactcgaaggctgaggtgatcaggttctgggtcatcacctccaggtccttgattccggcacggaacttattgtagtcttcatgccaacaggtgttcttgacatccaggatacccccgcgaacggctcgcagcgtgtgcagatttttatgaaagatgtcctcaatctccagcaagttccgtgttatctgtggcccctgggcaccaaagaagcaaggaaggggaccctgcttgccatcttcccagcgggcgaagtgatactgacagtcacatacctcaataaggtccttgcagcgctgcacaaaggcatcaacctgagcaaagatgctggtctgatctaggacccagccccgactggagaactggatgtgcatctgcacagcctgtacgtagtgatctttccaagcgtgacaacagagaatgcagccttgcaggtcctccttgctggaagagacatatccctcaaagatccggtccagggagatggcgtggcagcataagcggatgatctcattgctcatctttcggaagagcgaggtcagtctctcccgagtgttgtagtggggagagttgacccagatgatgcggatgagactgatcagcttagggagcttgctagagatgtccttgggcttcatgaaagccaactcctggtaaggttccttcaggattgacaaaaaggtcaggtttgactgtgcttgacgagagccatcctggatctgctgtgccagtttcataaagggcgccaagtaggacgacttggcaaggtgcaggatggattcaacgtgcttcactcccttcttcaccagctgcttactgatgccagacaggtccatgcatcggttgcgccagaactcaatctcctccagaggacctaaattttctcctgtctccacagtctcctgggcactgagcatctcctttatctgccgggtccagtggatcatggaggtctctagccgttgcaccagctctttgtcctttatcaccatctcaggcttcatgttcatggcctctgcagggatgtagaggaccgtgtgcccctccagtttgtaccgagtgtctgtcaggcaggccaagaacttgtgcagatgagaagcaaaatgatttctaatgctctcaggccagcctgtgtttgcaaagatctgaggggcaaagactccaccgagcagccgaagcagggccgggatataggggccccgcaccgtcccaaactgcacagttgcctcgaagttctcccaggtgatgggaactggtgcttggcgaatgaagtagacaagctggttctgggtctgtacaggcatgcccagctctagcttcagcccaaaacaagggtcaatgaagatggtgaggatggattctgtagggtcctgggcaaagtgttccagaatggcatcatgctcctgtgtccacactgcatccgccagtcctgtcagcgcagctcgggaaaggaagaggggcttcacatctgcctcgggctccactgattcttcactctgtgcttgaggtccctccaaccgtggctcaggctcctccttggggagctcagcctgcagctctggctcactgacagccggggcattcccctgctcctgtgtggccacagcagcccgagtggcccgccctgaccagcttgcctgggagcttcctcggccactcaatcgctgcttcttctcagctttgctggacatcgtgcaggcaaaacctgggtctatcgctttgaagtcctgaggggcaggaacactgttttgtgtgtactgaggtctcttagcagagttggctgaggaactctgtgctaatggttaagatcagtcaggatcatttatttgactcaaaatgcccttgccacgctgaccctcccctccctagaccgaccgatgggccactctaagaagttgcccctcgcagccctctcgggccgg

SEQ ID NO: 8719 - RNA, 10222 nt, Homo sapiens
  source 1..10222: mol_type = other RNA
aagccctgtctcctcccatctggccttctcgccagccaaccccgacacgagcatcccagctcgctccagcttcagctccatctcttcagacttcttgcgaagctcctccttctgtgccagcttctcatcatactgtttctttagcatctccagtttctcagctacctcccgcagcttctcctgggcctcagcgagcgcggcttgcttctcccgaagctgagccaaggcagcgttcattcggattcgcttgggctccaccacccgatatagccgcccatacagctccatggcccgcacccacatgcagagggacttggcagccagggagacgcggccgatgatatcaggctggaagtcaggctgggcgcagtaggccccaatcttcttcagaaccttatctgagatattgtctttatcaaagttgatcagtgacttgatgaagttctgttcccctagctgcctcttggcctctgcccatgtgggctcgttgcctcgaagaatcataactgcctgcatcactatctccacttgggctgggggccgtccataagacttgatctctcctatatccttcttgttcagagactccagggcccgcatggcctcttccagggcgggcagtgcctcttctagatctttctgggcattgtcagccagtgcctgacacttgatttcctcaactgcaatcttttcactgttggctgttacggccttctgctgctcatctgcctcccgcttctgctgcacaatgatgaccaggtactcctcacactgcttctggaactcagccaccttcttcttggcatcctccagctccaacgacatcacttgcaccttttccctagtttcgtcgatcttgaacaagcctgtccgcagtttattggcttgggccagcagctcctgccgtttttctcccagcaacttcttatatccagacaggagttccaggtatttggtgggtgtgacatagttgtgtctccgcagttccaacagcatcttctgggaatactgagctactgaccagtgcatagtgacaaagatctgggccaccttcctgtggatattctcctgagttcccaggtctactcctatgaggcacttctcagccacctcgagcagggcctcttggggccactctgagaaccagttgatggttgtgcagttcaccaaggctgggtactggcggatccagttcctgaagggatcccccatggggctgaggcagagcacgatgtgcaggttgttctgcacgcgttcaatgaggtaggcgaagaggctgtccgatgactcaggcacctgctccacccgggcctggtctatgatatgcgactggatctcttcaaattcatcaggcttgtagagattgggcacctcgcctgagctgaggatgttgttgatgtcctctaggaaggactcatcagctatttgggtgtccacaaaaatgaaggacgtggtcttgagctccaccccagcctggcgatacagacgcttgatatcatctcggaactcctgcttccgataatgtttggtgacctcgatctggaaggtggtgtagtcgcagatggatgaagccaggcgggccagactctggcgtccgctgcccccgatacccaccaggagcatgttgccccgaggctgtccaatgacccgcacgatccgtgtgatgtgttcaatagcctctcggaagagcactagctgcatgggcacgacagagggtgacaggttatactcatttagagctgtctccatgactgtcttcagcactgtcagatccgtgaggtcttcatacaccttgggctccttcaggaaatccccaaagataggaggacgcttgctgggacagagatgatgaaatgtgaggtcaaagaaggagccgagcttgtcgcttatgatgcccatgaaggcttctgtgtctgccgcatcaaccagccggtcagagaagactctgaaacattcatggatccagagccgtgtgatgctggacttggtatcatggaagtccttgttggctctaagcatgccctggaacaccttggagatgtctcgaaggttgaagaggtaatgcatcttggtgggcgtgggcaggaagcgctgtaccacggtgttgtacatgtccagggtggcctctgtcaccacgttcccaatgggcttcacctcttcctcaaagtcctgaagcttctgattgatcatggtgccgaatatgcggatgatctgggactttgtggggaaggtcatgttgataatgttgaagcgactccgtagccttggggagatgacagtccgtccacccccaggggggcccatggcagccatcaggaacatttctcgaatgtacttgatggtctgcttcgtacggtcataccagaagccatagtcaatccagaggcggatcagctccaggggtggctgggacccaaacatgtccttagcgggcatatttaggtcatccataaaggtgatcatgcttttgcccccgaatggcacgtagacacccttggttcgcttctcaaccctgctctcaatgatgctctgcacgttattggatgtggtctgtgcggacatgttgacaacgagcaccgaccactggctggagggcagggactgcagaacgctctgggcgatggaggtcttcccagtccccacgggacccaccagcagaatgggattctggttggccaccaagctgctcaccaggtagttgtagcgaacagtgtcgacggtgggcaccatgatcttatagaagggggcgtttggagggtagcgccaactcttagggagcttgtcctcaaatgatgtccaactccgtattttggggtccacaaaatactcatataccgtgtccttattgggaaaggagccctcgatctctcggaggtagctgtcgatcctcttccggccctcctcatccacagaggcacacacagaccagatcatgctgaacacaaatgtcatctctaccatggtgacatagttctcgccgtcagctgggttcaccccattctctggcgtggccagggcagagtacagcttgcagagggaggtgataccgctgtactcgggcaggggcaccagctccttgcagttgtccttcttaaaggccagcatcttgttgatgagcttttcgaacatgcgttgaaggggctccacctcagcctttggcctcttctccagccatgactgaacatagggcttccagcccaggtcagcgtagtcagtgtagaccatcccgcagcgggatacagtggccggagaggccattgccaggtcctccacttcaaacaggagagacacctgctcgggcatcgcgatgcgctcgccgttgatgagggtcaacaccttgttatcgtccatgacggagttcatgttctcgatccacagtgtgtccacggggccatcgaacaggatccacttctcgtcgggtttctcatctgcacatgccgtccgcatgacactggacaagatgccatctgtccattcattggtgctgaggtcatattccccatacagttcccctagggacaatgccttggggttcaaagggaactctctaacaatgttgaagttagggtctccggcgcggcacagagaggacagggaggcctgtagaatgcgccatgaggcagtcttgccgctgcccgtgcagcccacgatcatggtggagtggcgggagttcttggtttcatacaactggaaaaccttggtgagggtgaacggcgtgctttgcaggcccatgtctcgaatctcctgctcaacggtctcccgcagcttgccatagtcaatgacaggcagctcaatgttgggaaacagatcttgcacgatggcattgaacaggggtgcatcaactgaagtgagcttggcgatgttcatatctctcattgagagcagcagaacctcttcatcagtcagatccggctgtaggcggcgcttcttgccagcatagcgcagaagggaggtgagggcacgcaggccaaagtcatagtggtcctgtctggacagctgctgcacagccagtgagtagagtgtgtacaccttcttggccagaatcttgcagttgccaaagccctctccaaagagaatgatttctgcaatgagggtggagtcaggcaccaccatggcaattgggcggaacatggatttaagattttcgggaagctctgtgcggccagcatagccaggattcatggtaatgaagatcccacaggaccacaccagatttatttcaaagccatcaaaatggaaatgggtgaggccggcagccagggcagacaggatgcacaggatctggtgggccaccactgacagcacctcgatgttgatgcggttaaactcatcaaagcagccccaagctccagtctgggccagacctgagtacattcggcccatggacttgtagtccaggccctcagagcagttgaccacaatgacatatatgcccagggccttgcccaggtccttgacggtctcggtcttgcctgtgcctgcagggcctttgggggagccccctcggtgcaggtgcaatgccgtggtcagtgtcatgtaacacctgtccgtcaggggggtgatgacgagccggcccgagttacccaagtactcataattatactgaaattgcgtgttggtctggcggatgacacagtcatcaagatccttctcccagtagaaccgaagttggctgagccagtcaaaggaattgacatccatgaggccactcttgtaaagcttctccaacacatcccgggcatgaatttctatcgtcaccagagccacaattttaagccgcatgatcttggtcaagttccccctgatggcttctgaatacttattcaggattgacacctggttcttcttcatgaccttgaggattttcttgtctgcccgctccttcgctgtcagcaggcacttggtgacatcagccgtccactggatctgactggcagtgatcaccacctggccagcccactccttcacccatttgtccctcttgttgaggaacttcctgagggccaggtggcagttccggagaaggtcccgcagggtcaccctcatggtctgttccacatcgccaagccaggactccacagggccttctaaaaatactgagtggaggaagtcaatgtactcgccgtcgcccgagaacatccccacagcttcccatttgctgctgggccctccaaccttctggattctcagcaacttgatgttgtcaaagcattttttgaggtgtggctgcacagcctctgggtttcgggactggcccagaatctccagcaggtcatcattggacaagaagtagaagcgggggaaaatatgtcgcttggtctctaaatacatatccagagatttctgaatatcttccaggattgtattcatttctatcaatgtgtccaggaggcctgggtgatgggtgctccggagagcattgttgtccttgttcatcctgtccatgatggctttccagttgctgttgacctggtcaaataaggtcgattcattgggcagctgcttgcggatgtcttctcctaggaagatattctctaagtacatccactgacgctgcactgtgagaatcatctcaataacctccaaaatgagggagaggcagcgttcccagtggtccacatccttctcaaaggccttgacaaagcgtgatgccttcatggtagacagagctacctggttatcttccagtgcctggaatacttcttctgtacctctgagccgatgatggcccttatccttgtagggtactatgtcgagctgagtcacatcccaggtcttggcaatgttttgtaaagccacttctatagccagctctttagttgctgaagcagagatctccccaattttctccacatgctgatccatcccaagctccacaatctgctccaaggtgaagctttcagattcctgatcaaactcccgctggatctcatcccggacctggtcccagtgcctctctctaagggcagggttccgcaggtctgagatgagaggcatggtcctcttgaactgctctatttttgagcgagtggtttcaataatttcccagtttcggtccttatactctttggctaattttgtgaggcgacgaaacagcccgtgggccgtggtctccatggtttccgtctgcaggatcaggaaccggccagtcttccactcattccagttctcctcccagtctcgtgcgatctcccagatttgctggagggcatcgagctccttctccaggttctgaaggtccttggagggtggctgctcgatcttgaagatgcccaggttggctcggagactattttcctcttcccgcatggccatcagcatggcccgcacttgtgtaatctggtctaaggcagacatgtatcccacgttgctggtgaaatggcctttgaattcgaaatcttccagaagtgtatgtgctttcttcttgaagtcatctgccgagtggatcaggcctgtcttgaatttctccttgtgtttcttcagcatttgcttactgtccagcagagtttgttggaagacaacccactccccgttgagactgtccagcatctccaggacactgtcctcgactggcacctcgtacttttcaagaatggcaaattgctcgtgtatgggagggatctgagtctccacgttggccaagtcgtgcttcagggcatccacgagctgcaagctgacccccagttcctccagtgtctgcggagggcggctgattttctctgcgttctccttcaggtaggtgtgcagctccaggaggcgcccagcagccatctccctgagcagagtcgcgaacttgttctgccattcattgcagtgctgcaccagggagaacttgaggtgcgaacagtccagcagcacaaactggatgttggtgactgtctcctccttctgcacgttattagcaacttccgtgtagcgggcaatgtcggcaacaaaagaagagacaggagggttgaggcgctggtagcgatgaatgaaggagtccttgttgatctcccagatctcccggtacatgtcccaggtcttgaggtagttctgcagcaggcttgcgttgttagtcatgccgctgctgatttgggtctggatcttcttgatgtcctcatcttgctccacaactgtttggatgggttcacgatgtaacttgcgcttggtgagaatgtcagggaggtggcagaagacagagatggtggaaaagaggtggttgccaatgtcattgaccacacctgccaaagtctgcagagtgggtgagaattccacctgtgccacacttccttgcagatcattcttcaaaatgacaaggacttggaagagtgggtttgggctggtctttccatccccgttgatagccttggatagttctagcagtgaccacttcacattcaggcgcagggcatcctccatcatgcggtccagccgaatcatgtacagcatccactgctgctgaatctcaggaccatcattcttgaagacctcataggagttggtcatgatggtcaccacatcctggtgcaggttcatcaatttctgctgtacagctgcccgatgctctctttggtcctcttcaaattccaggtccctgtatacccgtttgccactaatgcgtaccagcagcttctctgacatctcttgggctcgccagccaatggtcagagtggatgccttgaactcattcacaatcatctgcaccttgctggcatgtatacggcactccgtgatgaagaaggcactggcccccttcaaggcccagtgcagtttcttgagtcccgggtggatcttcttatccaggagccgaatacgctctttgaatagggcctgctcatctggggacagcatggcaataatcctattgtagtctctagcaacgagtagcagattttcacgcagaatgcgcaggtcctcggctcgctcagctacgttcaccacgtaatggggcgtctcaaacagcagccgctcccagtagtcaatttccgcaaagagaatcagaagggacttgtcaaagttgacatccagcatgcccgccttctcctggctgattcgcagcaatggggtatccaaccgccgaatgcaatccttgtccagacttgatgtccactcttggaaggtttttcgaaccagctcatcaatggcctggaccatctgctgataggtgtgcacactctcctttccagtcccaatacggggcaggaaatgagcaccagcaaggcaggtcatgactctgtcgatgcgacgccggaggatgtgcacccagcgcgcctttccggaatactgggccacgtagggctccaggtctggccatttcttgttccgttcacggttcaccagggccagctcgctattgaacagcatgtagagatccaccgccttcttgtcataagtccgcttgatagcctcgcgggaggcaagcctgtggaaggtgtccagcagaagcacgccgtgcggcacgtcccgcaccaactcgaaggctgaggtgatcaggttctgggtcatcacctccaggtccttgattccggcacggaacttattgtagtcttcatgccaacaggtgttcttgacatccaggatacccccgcgaacggctcgcagcgtgtgcagatttttatgaaagatgtcctcaatctccagcaagttccgtgttatctgtggcccctgggcaccaaagaagcaaggaaggggaccctgcttgccatcttcccagcgggcgaagtgatactgacagtcacatacctcaataaggtccttgcagcgctgcacaaaggcatcaacctgagcaaagatgctggtctgatctaggacccagccccgactggagaactggatgtgcatctgcacagcctgtacgtagtgatctttccaagcgtgacaacagagaatgcagccttgcaggtcctccttgctggaagagacatatccctcaaagatccggtccagggagatggcgtggcagcataagcggatgatctcattgctcatctttcggaagagcgaggtcagtctctcccgagtgttgtagtggggagagttgacccagatgatgcggatgagactgatcagcttagggagcttgctagagatgtccttgggcttcatgaaagccaactcctggtaaggttccttcaggattgacaaaaaggtcaggtttgactgtgcttgacgagagccatcctggatctgctgtgccagtttcataaagggcgccaagtaggacgacttggcaaggtgcaggatggattcaacgtgcttcactcccttcttcaccagctgcttactgatgccagacaggtccatgcatcggttgcgccagaactcaatctcctccagaggacctaaattttctcctgtctccacagtctcctgggcactgagcatctcctttatctgccgggtccagtggatcatggaggtctctagccgttgcaccagctctttgtcctttatcaccatctcaggcttcatgttcatggcctctgcagggatgtagaggaccgtgtgcccctccagtttgtaccgagtgtctgtcaggcaggccaagaacttgtgcagatgagaagcaaaatgatttctaatgctctcaggccagcctgtgtttgcaaagatctgaggggcaaagactccaccgagcagccgaagcagggccgggatataggggccccgcaccgtcccaaactgcacagttgcctcgaagttctcccaggtgatgggaactggtgcttggcgaatgaagtagacaagctggttctgggtctgtacaggcatgcccagctctagcttcagcccaaaacaagggtcaatgaagatggtgaggatggattctgtagggtcctgggcaaagtgttccagaatggcatcatgctcctgtgtccacactgcatccgccagtcctgtcagcgcagctcgggaaaggaagaggggcttcacatctgcctcgggctccactgattcttcactctgtgcttgaggtccctccaaccgtggctcaggctcctccttggggagctcagcctgcagctctggctcactgacagccggggcattcccctgctcctgtgtggccacagcagcccgagtggcccgccctgaccagcttgcctgggagcttcctcggccactcaatcgctgcttcttctcagctttgctggacatcgtgcaggcaaaaccttgccacgctgaccctcccctccctagaccgaccgatgggccactctaagaagttgcccctcgcagc

SEQ ID NO: 8720 - RNA, 10964 nt, Homo sapiens
  source 1..10964: mol_type = other RNA
aagccctgtctcctcccatctggccttctcgccagccaaccccgacacgagcatcccagctcgctccagcttcagctccatctcttcagacttcttgcgaagctcctccttctgtgccagcttctcatcatactgtttctttagcatctccagtttctcagctacctcccgcagcttctcctgggcctcagcgagcgcggcttgcttctcccgaagctgagccaaggcagcgttcattcggattcgcttgggctccaccacccgatatagccgcccatacagctccatggcccgcacccacatgcagagggacttggcagccagggagacgcggccgatgatatcaggctggaagtcaggctgggcgcagtaggccccaatcttcttcagaaccttatctgagatattgtctttatcaaagttgatcagtgacttgatgaagttctgttcccctagctgcctcttggcctctgcccatgtgggctcgttgcctcgaagaatcataactgcctgcatcactatctccacttgggctgggggccgtccataagacttgatctctcctatatccttcttgttcagagactccagggcccgcatggcctcttccagggcgggcagtgcctcttctagatctttctgggcattgtcagccagtgcctgacacttgatttcctcaactgcaatcttttcactgttggctgttacggccttctgctgctcatctgcctcccgcttctgctgcacaatgatgaccaggtactcctcacactgcttctggaactcagccaccttcttcttggcatcctccagctccaacgacatcacttgcaccttttccctagtttcgtcgatcttgaacaagcctgtccgcagtttattggcttgggccagcagctcctgccgtttttctcccagcaacttcttatatccagacaggagttccaggtatttggtgggtgtgacatagttgtgtctccgcagttccaacagcatcttctgggaatactgagctactgaccagtgcatagtgacaaagatctgggccaccttcctgtggatattctcctgagttcccaggtctactcctatgaggcacttctcagccacctcgagcagggcctcttggggccactctgagaaccagttgatggttgtgcagttcaccaaggctgggtactggcggatccagttcctgaagggatcccccatggggctgaggcagagcacgatgtgcaggttgttctgcacgcgttcaatgaggtaggcgaagaggctgtccgatgactcaggcacctgctccacccgggcctggtctatgatatgcgactggatctcttcaaattcatcaggcttgtagagattgggcacctcgcctgagctgaggatgttgttgatgtcctctaggaaggactcatcagctatttgggtgtccacaaaaatgaaggacgtggtcttgagctccaccccagcctggcgatacagacgcttgatatcatctcggaactcctgcttccgataatgtttggtgacctcgatctggaaggtggtgtagtcgcagatggatgaagccaggcgggccagactctggcgtccgctgcccccgatacccaccaggagcatgttgccccgaggctgtccaatgacccgcacgatccgtgtgatgtgttcaatagcctctcggaagagcactagctgcatgggcacgacagagggtgacaggttatactcatttagagctgtctccatgactgtcttcagcactgtcagatccgtgaggtcttcatacaccttgggctccttcaggaaatccccaaagataggaggacgcttgctgggacagagatgatgaaatgtgaggtcaaagaaggagccgagcttgtcgcttatgatgcccatgaaggcttctgtgtctgccgcatcaaccagccggtcagagaagactctgaaacattcatggatccagagccgtgtgatgctggacttggtatcatggaagtccttgttggctctaagcatgccctggaacaccttggagatgtctcgaaggttgaagaggtaatgcatcttggtgggcgtgggcaggaagcgctgtaccacggtgttgtacatgtccagggtggcctctgtcaccacgttcccaatgggcttcacctcttcctcaaagtcctgaagcttctgattgatcatggtgccgaatatgcggatgatctgggactttgtggggaaggtcatgttgataatgttgaagcgactccgtagccttggggagatgacagtccgtccacccccaggggggcccatggcagccatcaggaacatttctcgaatgtacttgatggtctgcttcgtacggtcataccagaagccatagtcaatccagaggcggatcagctccaggggtggctgggacccaaacatgtccttagcgggcatatttaggtcatccataaaggtgatcatgcttttgcccccgaatggcacgtagacacccttggttcgcttctcaaccctgctctcaatgatgctctgcacgttattggatgtggtctgtgcggacatgttgacaacgagcaccgaccactggctggagggcagggactgcagaacgctctgggcgatggaggtcttcccagtccccacgggacccaccagcagaatgggattctggttggccaccaagctgctcaccaggtagttgtagcgaacagtgtcgacggtgggcaccatgatcttatagaagggggcgtttggagggtagcgccaactcttagggagcttgtcctcaaatgatgtccaactccgtattttggggtccacaaaatactcatataccgtgtccttattgggaaaggagccctcgatctctcggaggtagctgtcgatcctcttccggccctcctcatccacagaggcacacacagaccagatcatgctgaacacaaatgtcatctctaccatggtgacatagttctcgccgtcagctgggttcaccccattctctggcgtggccagggcagagtacagcttgcagagggaggtgataccgctgtactcgggcaggggcaccagctccttgcagttgtccttcttaaaggccagcatcttgttgatgagcttttcgaacatgcgttgaaggggctccacctcagcctttggcctcttctccagccatgactgaacatagggcttccagcccaggtcagcgtagtcagtgtagaccatcccgcagcgggatacagtggccggagaggccattgccaggtcctccacttcaaacaggagagacacctgctcgggcatcgcgatgcgctcgccgttgatgagggtcaacaccttgttatcgtccatgacggagttcatgttctcgatccacagtgtgtccacggggccatcgaacaggatccacttctcgtcgggtttctcatctgcacatgccgtccgcatgacactggacaagatgccatctgtccattcattggtgctgaggtcatattccccatacagttcccctagggacaatgccttggggttcaaagggaactctctaacaatgttgaagttagggtctccggcgcggcacagagaggacagggaggcctgtagaatgcgccatgaggcagtcttgccgctgcccgtgcagcccacgatcatggtggagtggcgggagttcttggtttcatacaactggaaaaccttggtgagggtgaacggcgtgctttgcaggcccatgtctcgaatctcctgctcaacggtctcccgcagcttgccatagtcaatgacaggcagctcaatgttgggaaacagatcttgcacgatggcattgaacaggggtgcatcaactgaagtgagcttggcgatgttcatatctctcattgagagcagcagaacctcttcatcagtcagatccggctgtaggcggcgcttcttgccagcatagcgcagaagggaggtgagggcacgcaggccaaagtcatagtggtcctgtctggacagctgctgcacagccagtgagtagagtgtgtacaccttcttggccagaatcttgcagttgccaaagccctctccaaagagaatgatttctgcaatgagggtggagtcaggcaccaccatggcaattgggcggaacatggatttaagattttcgggaagctctgtgcggccagcatagccaggattcatggtaatgaagatcccacaggaccacaccagatttatttcaaagccatcaaaatggaaatgggtgaggccggcagccagggcagacaggatgcacaggatctggtgggccaccactgacagcacctcgatgttgatgcggttaaactcatcaaagcagccccaagctccagtctgggccagacctgagtacattcggcccatggacttgtagtccaggccctcagagcagttgaccacaatgacatatatgcccagggccttgcccaggtccttgacggtctcggtcttgcctgtgcctgcagggcctttgggggagccccctcggtgcaggtgcaatgccgtggtcagtgtcatgtaacacctgtccgtcaggggggtgatgacgagccggcccgagttacccaagtactcataattatactgaaattgcgtgttggtctggcggatgacacagtcatcaagatccttctcccagtagaaccgaagttggctgagccagtcaaaggaattgacatccatgaggccactcttgtaaagcttctccaacacatcccgggcatgaatttctatcgtcaccagagccacaattttaagccgcatgatcttggtcaagttccccctgatggcttctgaatacttattcaggattgacacctggttcttcttcatgaccttgaggattttcttgtctgcccgctccttcgctgtcagcaggcacttggtgacatcagccgtccactggatctgactggcagtgatcaccacctggccagcccactccttcacccatttgtccctcttgttgaggaacttcctgagggccaggtggcagttccggagaaggtcccgcagggtcaccctcatggtctgttccacatcgccaagccaggactccacagggccttctaaaaatactgagtggaggaagtcaatgtactcgccgtcgcccgagaacatccccacagcttcccatttgctgctgggccctccaaccttctggattctcagcaacttgatgttgtcaaagcattttttgaggtgtggctgcacagcctctgggtttcgggactggcccagaatctccagcaggtcatcattggacaagaagtagaagcgggggaaaatatgtcgcttggtctctaaatacatatccagagatttctgaatatcttccaggattgtattcatttctatcaatgtgtccaggaggcctgggtgatgggtgctccggagagcattgttgtccttgttcatcctgtccatgatggctttccagttgctgttgacctggtcaaataaggtcgattcattgggcagctgcttgcggatgtcttctcctaggaagatattctctaagtacatccactgacgctgcactgtgagaatcatctcaataacctccaaaatgagggagaggcagcgttcccagtggtccacatccttctcaaaggccttgacaaagcgtgatgccttcatggtagacagagctacctggttatcttccagtgcctggaatacttcttctgtacctctgagccgatgatggcccttatccttgtagggtactatgtcgagctgagtcacatcccaggtcttggcaatgttttgtaaagccacttctatagccagctctttagttgctgaagcagagatctccccaattttctccacatgctgatccatcccaagctccacaatctgctccaaggtgaagctttcagattcctgatcaaactcccgctggatctcatcccggacctggtcccagtgcctctctctaagggcagggttccgcaggtctgagatgagaggcatggtcctcttgaactgctctatttttgagcgagtggtttcaataatttcccagtttcggtccttatactctttggctaattttgtgaggcgacgaaacagcccgtgggccgtggtctccatggtttccgtctgcaggatcaggaaccggccagtcttccactcattccagttctcctcccagtctcgtgcgatctcccagatttgctggagggcatcgagctccttctccaggttctgaaggtccttggagggtggctgctcgatcttgaagatgcccaggttggctcggagactattttcctcttcccgcatggccatcagcatggcccgcacttgtgtaatctggtctaaggcagacatgtatcccacgttgctggtgaaatggcctttgaattcgaaatcttccagaagtgtatgtgctttcttcttgaagtcatctgccgagtggatcaggcctgtcttgaatttctccttgtgtttcttcagcatttgcttactgtccagcagagtttgttggaagacaacccactccccgttgagactgtccagcatctccaggacactgtcctcgactggcacctcgtacttttcaagaatggcaaattgctcgtgtatgggagggatctgagtctccacgttggccaagtcgtgcttcagggcatccacgagctgcaagctgacccccagttcctccagtgtctgcggagggcggctgattttctctgcgttctccttcaggtaggtgtgcagctccaggaggcgcccagcagccatctccctgagcagagtcgcgaacttgttctgccattcattgcagtgctgcaccagggagaacttgaggtgcgaacagtccagcagcacaaactggatgttggtgactgtctcctccttctgcacgttattagcaacttccgtgtagcgggcaatgtcggcaacaaaagaagagacaggagggttgaggcgctggtagcgatgaatgaaggagtccttgttgatctcccagatctcccggtacatgtcccaggtcttgaggtagttctgcagcaggcttgcgttgttagtcatgccgctgctgatttgggtctggatcttcttgatgtcctcatcttgctccacaactgtttggatgggttcacgatgtaacttgcgcttggtgagaatgtcagggaggtggcagaagacagagatggtggaaaagaggtggttgccaatgtcattgaccacacctgccaaagtctgcagagtgggtgagaattccacctgtgccacacttccttgcagatcattcttcaaaatgacaaggacttggaagagtgggtttgggctggtctttccatccccgttgatagccttggatagttctagcagtgaccacttcacattcaggcgcagggcatcctccatcatgcggtccagccgaatcatgtacagcatccactgctgctgaatctcaggaccatcattcttgaagacctcataggagttggtcatgatggtcaccacatcctggtgcaggttcatcaatttctgctgtacagctgcccgatgctctctttggtcctcttcaaattccaggtccctgtatacccgtttgccactaatgcgtaccagcagcttctctgacatctcttgggctcgccagccaatggtcagagtggatgccttgaactcattcacaatcatctgcaccttgctggcatgtatacggcactccgtgatgaagaaggcactggcccccttcaaggcccagtgcagtttcttgagtcccgggtggatcttcttatccaggagccgaatacgctctttgaatagggcctgctcatctggggacagcatggcaataatcctattgtagtctctagcaacgagtagcagattttcacgcagaatgcgcaggtcctcggctcgctcagctacgttcaccacgtaatggggcgtctcaaacagcagccgctcccagtagtcaatttccgcaaagagaatcagaagggacttgtcaaagttgacatccagcatgcccgccttctcctggctgattcgcagcaatggggtatccaaccgccgaatgcaatccttgtccagacttgatgtccactcttggaaggtttttcgaaccagctcatcaatggcctggaccatctgctgataggtgtgcacactctcctttccagtcccaatacggggcaggaaatgagcaccagcaaggcaggtcatgactctgtcgatgcgacgccggaggatgtgcacccagcgcgcctttccggaatactgggccacgtagggctccaggtctggccatttcttgttccgttcacggttcaccagggccagctcgctattgaacagcatgtagagatccaccgccttcttgtcataagtccgcttgatagcctcgcgggaggcaagcctgtggaaggtgtccagcagaagcacgccgtgcggcacgtcccgcaccaactcgaaggctgaggtgatcaggttctgggtcatcacctccaggtccttgattccggcacggaacttattgtagtcttcatgccaacaggtgttcttgacatccaggatacccccgcgaacggctcgcagcgtgtgcagatttttatgaaagatgtcctcaatctccagcaagttccgtgttatctgtggcccctgggcaccaaagaagcaaggaaggggaccctgcttgccatcttcccagcgggcgaagtgatactgacagtcacatacctttcggaagagcgaggtcagtctctcccgagtgttgtagtggggagagttgacccagatgatgcggatgagactgatcagcttagggagcttgctagagatgtccttgggcttcatgaaagccaactcctggtaaggttccttcaggattgacaaaaaggtcaggtttgactgtgcttgacgagagccatcctggatctgctgtgccagtttcataaagggcgccaagtaggacgacttggcaaggtgcaggatggattcaacgtgcttcactcccttcttcaccagctgcttactgatgccagacaggtccatgcatcggttgcgccagaactcaatctcctccagaggacctaaattttctcctgtctccacagtctcctgggcactgagcatctcctttatctgccgggtccagtggatcatggaggtctctagccgttgcaccagctctttgtcctttatcaccatctcaggcttcatgttcatggcctctgcagggatgtagaggaccgtgtgcccctccagtttgtaccgagtgtctgtcaggcaggccaagaacttgtgcagatgagaagcaaaatgatttctaatgctctcaggccagcctgtgtttgcaaagatctgaggggcaaagactccaccgagcagccgaagcagggccgggatataggggccccgcaccgtcccaaactgcacagttgcctcgaagttctcccaggtgatgggaactggtgcttggcgaatgaagtagacaagctggttctgggtctgtacaggcatgcccagctctagcttcagcccaaaacaagggtcaatgaagatggtgaggatggattctgtagggtcctgggcaaagtgttccagaatggcatcatgctcctgtgtccacactgcatccgccagtcctgtcagcgcagctcgggaaaggaagaggggcttcacatctgcctcgggctccactgattcttcactctgtgcttgaggtccctccaaccgtggctcaggctcctccttggggagctcagcctgcagctctggctcactgacagccggggcattcccctgctcctgtgtggccacagcagcccgagtggcccgccctgaccagcttgcctgggagcttcctcggccactcaatcgctgcttcttctcagctttgctggacatcgtgcaggcaaaacctgggtctatcgctttgaagtcctgaggggcaggaacactgttttgtgtgtactgaggtctcttagcagagttggctgaggaactctgtgctaatggttaagatcagtcaggatcatttatttgactcaaaatgccctgagaacagattggaagaaagaaggacaaaagtcatccaatcataaatttcaaattgtgtcatgaggaaaaagcaattggggcacgaggaaggtcacagtggtgcctctctcagaaaggtaggatggcaggaagcggggatctcggacaggtgctcagaatcccaggcgcaaagtctgaggcgctgggcactctcttttcattaggctgcagcctaacggcacctgtggctctccttcctcatccccacaggctgccacaggcattgatctcaggttatgaatttcaaacttgaaggatttgtactttgctccaaggaaaaacgttctgttaggccagcaaatcaataaaaccaactacagcaaggaggcttcctccatcagtctccagagaagcatcaagctgcgctttcctgcctcaaactagagcctgaggcgcatgcaccgtggggttcaccacgcgatcccacaccgcaggccccaggaggaactgctctgctaagtcggggctcactctagtactaggaaataccgcaggggccagcagtatttatcctgcagtataaatccagcagtatttatccagcagtatttataccagcagctggtatccttaaactggttaccagcaggcaaatttcccctcagaatggctcttcccccccagctgtcacaactgccccttctcctccccctcccccacacaaatattccttgctccctctccctccacaactgcctcttctccccaacaactgtcccttcctaccccgacactactgccccttctccccagcactccttccctccttccctctgcccccgacacacaccttgccacgctgaccctcccctccctagaccgaccgatgggccactctaagaagttgcccctcgcagccctctcgggccggcgtctgc

SEQ ID NO: 8721 - RNA, 10125 nt, Homo sapiens
  source 1..10125: mol_type = other RNA
aagccctgtctcctcccatctggccttctcgccagccaaccccgacacgagcatcccagctcgctccagcttcagctccatctcttcagacttcttgcgaagctcctccttctgtgccagcttctcatcatactgtttctttagcatctccagtttctcagctacctcccgcagcttctcctgggcctcagcgagcgcggcttgcttctcccgaagctgagccaaggcagcgttcattcggattcgcttgggctccaccacccgatatagccgcccatacagctccatggcccgcacccacatgcagagggacttggcagccagggagacgcggccgatgatatcaggctggaagtcaggctgggcgcagtaggccccaatcttcttcagaaccttatctgagatattgtctttatcaaagttgatcagtgacttgatgaagttctgttcccctagctgcctcttggcctctgcccatgtgggctcgttgcctcgaagaatcataactgcctgcatcactatctccacttgggctgggggccgtccataagacttgatctctcctatatccttcttgttcagagactccagggcccgcatggcctcttccagggcgggcagtgcctcttctagatctttctgggcattgtcagccagtgcctgacacttgatttcctcaactgcaatcttttcactgttggctgttacggccttctgctgctcatctgcctcccgcttctgctgcacaatgatgaccaggtactcctcacactgcttctggaactcagccaccttcttcttggcatcctccagctccaacgacatcacttgcaccttttccctagtttcgtcgatcttgaacaagcctgtccgcagtttattggcttgggccagcagctcctgccgtttttctcccagcaacttcttatatccagacaggagttccaggtatttggtgggtgtgacatagttgtgtctccgcagttccaacagcatcttctgggaatactgagctactgaccagtgcatagtgacaaagatctgggccaccttcctgtggatattctcctgagttcccaggtctactcctatgaggcacttctcagccacctcgagcagggcctcttggggccactctgagaaccagttgatggttgtgcagttcaccaaggctgggtactggcggatccagttcctgaagggatcccccatggggctgaggcagagcacgatgtgcaggttgttctgcacgcgttcaatgaggtaggcgaagaggctgtccgatgactcaggcacctgctccacccgggcctggtctatgatatgcgactggatctcttcaaattcatcaggcttgtagagattgggcacctcgcctgagctgaggatgttgttgatgtcctctaggaaggactcatcagctatttgggtgtccacaaaaatgaaggacgtggtcttgagctccaccccagcctggcgatacagacgcttgatatcatctcggaactcctgcttccgataatgtttggtgacctcgatctggaaggtggtgtagtcgcagatggatgaagccaggcgggccagactctggcgtccgctgcccccgatacccaccaggagcatgttgccccgaggctgtccaatgacccgcacgatccgtgtgatgtgttcaatagcctctcggaagagcactagctgcatgggcacgacagagggtgacaggttatactcatttagagctgtctccatgactgtcttcagcactgtcagatccgtgaggtcttcatacaccttgggctccttcaggaaatccccaaagataggaggacgcttgctgggacagagatgatgaaatgtgaggtcaaagaaggagccgagcttgtcgcttatgatgcccatgaaggcttctgtgtctgccgcatcaaccagccggtcagagaagactctgaaacattcatggatccagagccgtgtgatgctggacttggtatcatggaagtccttgttggctctaagcatgccctggaacaccttggagatgtctcgaaggttgaagaggtaatgcatcttggtgggcgtgggcaggaagcgctgtaccacggtgttgtacatgtccagggtggcctctgtcaccacgttcccaatgggcttcacctcttcctcaaagtcctgaagcttctgattgatcatggtgccgaatatgcggatgatctgggactttgtggggaaggtcatgttgataatgttgaagcgactccgtagccttggggagatgacagtccgtccacccccaggggggcccatggcagccatcaggaacatttctcgaatgtacttgatggtctgcttcgtacggtcataccagaagccatagtcaatccagaggcggatcagctccaggggtggctgggacccaaacatgtccttagcgggcatatttaggtcatccataaaggtgatcatgcttttgcccccgaatggcacgtagacacccttggttcgcttctcaaccctgctctcaatgatgctctgcacgttattggatgtggtctgtgcggacatgttgacaacgagcaccgaccactggctggagggcagggactgcagaacgctctgggcgatggaggtcttcccagtccccacgggacccaccagcagaatgggattctggttggccaccaagctgctcaccaggtagttgtagcgaacagtgtcgacggtgggcaccatgatcttatagaagggggcgtttggagggtagcgccaactcttagggagcttgtcctcaaatgatgtccaactccgtattttggggtccacaaaatactcatataccgtgtccttattgggaaaggagccctcgatctctcggaggtagctgtcgatcctcttccggccctcctcatccacagaggcacacacagaccagatcatgctgaacacaaatgtcatctctaccatggtgacatagttctcgccgtcagctgggttcaccccattctctggcgtggccagggcagagtacagcttgcagagggaggtgataccgctgtactcgggcaggggcaccagctccttgcagttgtccttcttaaaggccagcatcttgttgatgagcttttcgaacatgcgttgaaggggctccacctcagcctttggcctcttctccagccatgactgaacatagggcttccagcccaggtcagcgtagtcagtgtagaccatcccgcagcgggatacagtggccggagaggccattgccaggtcctccacttcaaacaggagagacacctgctcgggcatcgcgatgcgctcgccgttgatgagggtcaacaccttgttatcgtccatgacggagttcatgttctcgatccacagtgtgtccacggggccatcgaacaggatccacttctcgtcgggtttctcatctgcacatgccgtccgcatgacactggacaagatgccatctgtccattcattggtgctgaggtcatattccccatacagttcccctagggacaatgccttggggttcaaagggaactctctaacaatgttgaagttagggtctccggcgcggcacagagaggacagggaggcctgtagaatgcgccatgaggcagtcttgccgctgcccgtgcagcccacgatcatggtggagtggcgggagttcttggtttcatacaactggaaaaccttggtgagggtgaacggcgtgctttgcaggcccatgtctcgaatctcctgctcaacggtctcccgcagcttgccatagtcaatgacaggcagctcaatgttgggaaacagatcttgcacgatggcattgaacaggggtgcatcaactgaagtgagcttggcgatgttcatatctctcattgagagcagcagaacctcttcatcagtcagatccggctgtaggcggcgcttcttgccagcatagcgcagaagggaggtgagggcacgcaggccaaagtcatagtggtcctgtctggacagctgctgcacagccagtgagtagagtgtgtacaccttcttggccagaatcttgcagttgccaaagccctctccaaagagaatgatttctgcaatgagggtggagtcaggcaccaccatggcaattgggcggaacatggatttaagattttcgggaagctctgtgcggccagcatagccaggattcatggtaatgaagatcccacaggaccacaccagatttatttcaaagccatcaaaatggaaatgggtgaggccggcagccagggcagacaggatgcacaggatctggtgggccaccactgacagcacctcgatgttgatgcggttaaactcatcaaagcagccccaagctccagtctgggccagacctgagtacattcggcccatggacttgtagtccaggccctcagagcagttgaccacaatgacatatatgcccagggccttgcccaggtccttgacggtctcggtcttgcctgtgcctgcagggcctttgggggagccccctcggtgcaggtgcaatgccgtggtcagtgtcatgtaacacctgtccgtcaggggggtgatgacgagccggcccgagttacccaagtactcataattatactgaaattgcgtgttggtctggcggatgacacagtcatcaagatccttctcccagtagaaccgaagttggctgagccagtcaaaggaattgacatccatgaggccactcttgtaaagcttctccaacacatcccgggcatgaatttctatcgtcaccagagccacaattttaagccgcatgatcttggtcaagttccccctgatggcttctgaatacttattcaggattgacacctggttcttcttcatgaccttgaggattttcttgtctgcccgctccttcgctgtcagcaggcacttggtgacatcagccgtccactggatctgactggcagtgatcaccacctggccagcccactccttcacccatttgtccctcttgttgaggaacttcctgagggccaggtggcagttccggagaaggtcccgcagggtcaccctcatggtctgttccacatcgccaagccaggactccacagggccttctaaaaatactgagtggaggaagtcaatgtactcgccgtcgcccgagaacatccccacagcttcccatttgctgctgggccctccaaccttctggattctcagcaacttgatgttgtcaaagcattttttgaggtgtggctgcacagcctctgggtttcgggactggcccagaatctccagcaggtcatcattggacaagaagtagaagcgggggaaaatatgtcgcttggtctctaaatacatatccagagatttctgaatatcttccaggattgtattcatttctatcaatgtgtccaggaggcctgggtgatgggtgctccggagagcattgttgtccttgttcatcctgtccatgatggctttccagttgctgttgacctggtcaaataaggtcgattcattgggcagctgcttgcggatgtcttctcctaggaagatattctctaagtacatccactgacgctgcactgtgagaatcatctcaataacctccaaaatgagggagaggcagcgttcccagtggtccacatccttctcaaaggccttgacaaagcgtgatgccttcatggtagacagagctacctggttatcttccagtgcctggaatacttcttctgtacctctgagccgatgatggcccttatccttgtagggtactatgtcgagctgagtcacatcccaggtcttggcaatgttttgtaaagccacttctatagccagctctttagttgctgaagcagagatctccccaattttctccacatgctgatccatcccaagctccacaatctgctccaaggtgaagctttcagattcctgatcaaactcccgctggatctcatcccggacctggtcccagtgcctctctctaagggcagggttccgcaggtctgagatgagaggcatggtcctcttgaactgctctatttttgagcgagtggtttcaataatttcccagtttcggtccttatactctttggctaattttgtgaggcgacgaaacagcccgtgggccgtggtctccatggtttccgtctgcaggatcaggaaccggccagtcttccactcattccagttctcctcccagtctcgtgcgatctcccagatttgctggagggcatcgagctccttctccaggttctgaaggtccttggagggtggctgctcgatcttgaagatgcccaggttggctcggagactattttcctcttcccgcatggccatcagcatggcccgcacttgtgtaatctggtctaaggcagacatgtatcccacgttgctggtgaaatggcctttgaattcgaaatcttccagaagtgtatgtgctttcttcttgaagtcatctgccgagtggatcaggcctgtcttgaatttctccttgtgtttcttcagcatttgcttactgtccagcagagtttgttggaagacaacccactccccgttgagactgtccagcatctccaggacactgtcctcgactggcacctcgtacttttcaagaatggcaaattgctcgtgtatgggagggatctgagtctccacgttggccaagtcgtgcttcagggcatccacgagctgcaagctgacccccagttcctccagtgtctgcggagggcggctgattttctctgcgttctccttcaggtaggtgtgcagctccaggaggcgcccagcagccatctccctgagcagagtcgcgaacttgttctgccattcattgcagtgctgcaccagggagaacttgaggtgcgaacagtccagcagcacaaactggatgttggtgactgtctcctccttctgcacgttattagcaacttccgtgtagcgggcaatgtcggcaacaaaagaagagacaggagggttgaggcgctggtagcgatgaatgaaggagtccttgttgatctcccagatctcccggtacatgtcccaggtcttgaggtagttctgcagcaggcttgcgttgttagtcatgccgctgctgatttgggtctggatcttcttgatgtcctcatcttgctccacaactgtttggatgggttcacgatgtaacttgcgcttggtgagaatgtcagggaggtggcagaagacagagatggtggaaaagaggtggttgccaatgtcattgaccacacctgccaaagtctgcagagtgggtgagaattccacctgtgccacacttccttgcagatcattcttcaaaatgacaaggacttggaagagtgggtttgggctggtctttccatccccgttgatagccttggatagttctagcagtgaccacttcacattcaggcgcagggcatcctccatcatgcggtccagccgaatcatgtacagcatccactgctgctgaatctcaggaccatcattcttgaagacctcataggagttggtcatgatggtcaccacatcctggtgcaggttcatcaatttctgctgtacagctgcccgatgctctctttggtcctcttcaaattccaggtccctgtatacccgtttgccactaatgcgtaccagcagcttctctgacatctcttgggctcgccagccaatggtcagagtggatgccttgaactcattcacaatcatctgcaccttgctggcatgtatacggcactccgtgatgaagaaggcactggcccccttcaaggcccagtgcagtttcttgagtcccgggtggatcttcttatccaggagccgaatacgctctttgaatagggcctgctcatctggggacagcatggcaataatcctattgtagtctctagcaacgagtagcagattttcacgcagaatgcgcaggtcctcggctcgctcagctacgttcaccacgtaatggggcgtctcaaacagcagccgctcccagtagtcaatttccgcaaagagaatcagaagggacttgtcaaagttgacatccagcatgcccgccttctcctggctgattcgcagcaatggggtatccaaccgccgaatgcaatccttgtccagacttgatgtccactcttggaaggtttttcgaaccagctcatcaatggcctggaccatctgctgataggtgtgcacactctcctttccagtcccaatacggggcaggaaatgagcaccagcaaggcaggtcatgactctgtcgatgcgacgccggaggatgtgcacccagcgcgcctttccggaatactgggccacgtagggctccaggtctggccatttcttgttccgttcacggttcaccagggccagctcgctattgaacagcatgtagagatccaccgccttcttgtcataagtccgcttgatagcctcgcgggaggcaagcctgtggaaggtgtccagcagaagcacgccgtgcggcacgtcccgcaccaactcgaaggctgaggtgatcaggttctgggtcatcacctccaggtccttgattccggcacggaacttattgtagtcttcatgccaacaggtgttcttgacatccaggatacccccgcgaacggctcgcagcgtgtgcagatttttatgaaagatgtcctcaatctccagcaagttccgtgttatctgtggcccctgggcaccaaagaagcaaggaaggggaccctgcttgccatcttcccagcgggcgaagtgatactgacagtcacatacctttcggaagagcgaggtcagtctctcccgagtgttgtagtggggagagttgacccagatgatgcggatgagactgatcagcttagggagcttgctagagatgtccttgggcttcatgaaagccaactcctggtaaggttccttcaggattgacaaaaaggtcaggtttgactgtgcttgacgagagccatcctggatctgctgtgccagtttcataaagggcgccaagtaggacgacttggcaaggtgcaggatggattcaacgtgcttcactcccttcttcaccagctgcttactgatgccagacaggtccatgcatcggttgcgccagaactcaatctcctccagaggacctaaattttctcctgtctccacagtctcctgggcactgagcatctcctttatctgccgggtccagtggatcatggaggtctctagccgttgcaccagctctttgtcctttatcaccatctcaggcttcatgttcatggcctctgcagggatgtagaggaccgtgtgcccctccagtttgtaccgagtgtctgtcaggcaggccaagaacttgtgcagatgagaagcaaaatgatttctaatgctctcaggccagcctgtgtttgcaaagatctgaggggcaaagactccaccgagcagccgaagcagggccgggatataggggccccgcaccgtcccaaactgcacagttgcctcgaagttctcccaggtgatgggaactggtgcttggcgaatgaagtagacaagctggttctgggtctgtacaggcatgcccagctctagcttcagcccaaaacaagggtcaatgaagatggtgaggatggattctgtagggtcctgggcaaagtgttccagaatggcatcatgctcctgtgtccacactgcatccgccagtcctgtcagcgcagctcgggaaaggaagaggggcttcacatctgcctcgggctccactgattcttcactctgtgcttgaggtccctccaaccgtggctcaggctcctccttggggagctcagcctgcagctctggctcactgacagccggggcattcccctgctcctgtgtggccacagcagcccgagtggcccgccctgaccagcttgcctgggagcttcctcggccactcaatcgctgcttcttctcagctttgctggacatcgtgcaggcaaaacctgggtctatcgctttgaagtcctgaggggcaggaacactgttttgtgtgtactgaggtctcttagcagagttggctgaggaactctgtgctaatggttaagatcagtcaggatcatttatttgactcaaaatgcccttgccacgctgaccctcccctccctagaccgaccgatgggccactctaagaagttgcccctcgcagccctctcgggccgg

SEQ ID NO: 8722 - RNA, 9976 nt, Homo sapiens
  source 1..9976: mol_type = other RNA
aagccctgtctcctcccatctggccttctcgccagccaaccccgacacgagcatcccagctcgctccagcttcagctccatctcttcagacttcttgcgaagctcctccttctgtgccagcttctcatcatactgtttctttagcatctccagtttctcagctacctcccgcagcttctcctgggcctcagcgagcgcggcttgcttctcccgaagctgagccaaggcagcgttcattcggattcgcttgggctccaccacccgatatagccgcccatacagctccatggcccgcacccacatgcagagggacttggcagccagggagacgcggccgatgatatcaggctggaagtcaggctgggcgcagtaggccccaatcttcttcagaaccttatctgagatattgtctttatcaaagttgatcagtgacttgatgaagttctgttcccctagctgcctcttggcctctgcccatgtgggctcgttgcctcgaagaatcataactgcctgcatcactatctccacttgggctgggggccgtccataagacttgatctctcctatatccttcttgttcagagactccagggcccgcatggcctcttccagggcgggcagtgcctcttctagatctttctgggcattgtcagccagtgcctgacacttgatttcctcaactgcaatcttttcactgttggctgttacggccttctgctgctcatctgcctcccgcttctgctgcacaatgatgaccaggtactcctcacactgcttctggaactcagccaccttcttcttggcatcctccagctccaacgacatcacttgcaccttttccctagtttcgtcgatcttgaacaagcctgtccgcagtttattggcttgggccagcagctcctgccgtttttctcccagcaacttcttatatccagacaggagttccaggtatttggtgggtgtgacatagttgtgtctccgcagttccaacagcatcttctgggaatactgagctactgaccagtgcatagtgacaaagatctgggccaccttcctgtggatattctcctgagttcccaggtctactcctatgaggcacttctcagccacctcgagcagggcctcttggggccactctgagaaccagttgatggttgtgcagttcaccaaggctgggtactggcggatccagttcctgaagggatcccccatggggctgaggcagagcacgatgtgcaggttgttctgcacgcgttcaatgaggtaggcgaagaggctgtccgatgactcaggcacctgctccacccgggcctggtctatgatatgcgactggatctcttcaaattcatcaggcttgtagagattgggcacctcgcctgagctgaggatgttgttgatgtcctctaggaaggactcatcagctatttgggtgtccacaaaaatgaaggacgtggtcttgagctccaccccagcctggcgatacagacgcttgatatcatctcggaactcctgcttccgataatgtttggtgacctcgatctggaaggtggtgtagtcgcagatggatgaagccaggcgggccagactctggcgtccgctgcccccgatacccaccaggagcatgttgccccgaggctgtccaatgacccgcacgatccgtgtgatgtgttcaatagcctctcggaagagcactagctgcatgggcacgacagagggtgacaggttatactcatttagagctgtctccatgactgtcttcagcactgtcagatccgtgaggtcttcatacaccttgggctccttcaggaaatccccaaagataggaggacgcttgctgggacagagatgatgaaatgtgaggtcaaagaaggagccgagcttgtcgcttatgatgcccatgaaggcttctgtgtctgccgcatcaaccagccggtcagagaagactctgaaacattcatggatccagagccgtgtgatgctggacttggtatcatggaagtccttgttggctctaagcatgccctggaacaccttggagatgtctcgaaggttgaagaggtaatgcatcttggtgggcgtgggcaggaagcgctgtaccacggtgttgtacatgtccagggtggcctctgtcaccacgttcccaatgggcttcacctcttcctcaaagtcctgaagcttctgattgatcatggtgccgaatatgcggatgatctgggactttgtggggaaggtcatgttgataatgttgaagcgactccgtagccttggggagatgacagtccgtccacccccaggggggcccatggcagccatcaggaacatttctcgaatgtacttgatggtctgcttcgtacggtcataccagaagccatagtcaatccagaggcggatcagctccaggggtggctgggacccaaacatgtccttagcgggcatatttaggtcatccataaaggtgatcatgcttttgcccccgaatggcacgtagacacccttggttcgcttctcaaccctgctctcaatgatgctctgcacgttattggatgtggtctgtgcggacatgttgacaacgagcaccgaccactggctggagggcagggactgcagaacgctctgggcgatggaggtcttcccagtccccacgggacccaccagcagaatgggattctggttggccaccaagctgctcaccaggtagttgtagcgaacagtgtcgacggtgggcaccatgatcttatagaagggggcgtttggagggtagcgccaactcttagggagcttgtcctcaaatgatgtccaactccgtattttggggtccacaaaatactcatataccgtgtccttattgggaaaggagccctcgatctctcggaggtagctgtcgatcctcttccggccctcctcatccacagaggcacacacagaccagatcatgctgaacacaaatgtcatctctaccatggtgacatagttctcgccgtcagctgggttcaccccattctctggcgtggccagggcagagtacagcttgcagagggaggtgataccgctgtactcgggcaggggcaccagctccttgcagttgtccttcttaaaggccagcatcttgttgatgagcttttcgaacatgcgttgaaggggctccacctcagcctttggcctcttctccagccatgactgaacatagggcttccagcccaggtcagcgtagtcagtgtagaccatcccgcagcgggatacagtggccggagaggccattgccaggtcctccacttcaaacaggagagacacctgctcgggcatcgcgatgcgctcgccgttgatgagggtcaacaccttgttatcgtccatgacggagttcatgttctcgatccacagtgtgtccacggggccatcgaacaggatccacttctcgtcgggtttctcatctgcacatgccgtccgcatgacactggacaagatgccatctgtccattcattggtgctgaggtcatattccccatacagttcccctagggacaatgccttggggttcaaagggaactctctaacaatgttgaagttagggtctccggcgcggcacagagaggacagggaggcctgtagaatgcgccatgaggcagtcttgccgctgcccgtgcagcccacgatcatggtggagtggcgggagttcttggtttcatacaactggaaaaccttggtgagggtgaacggcgtgctttgcaggcccatgtctcgaatctcctgctcaacggtctcccgcagcttgccatagtcaatgacaggcagctcaatgttgggaaacagatcttgcacgatggcattgaacaggggtgcatcaactgaagtgagcttggcgatgttcatatctctcattgagagcagcagaacctcttcatcagtcagatccggctgtaggcggcgcttcttgccagcatagcgcagaagggaggtgagggcacgcaggccaaagtcatagtggtcctgtctggacagctgctgcacagccagtgagtagagtgtgtacaccttcttggccagaatcttgcagttgccaaagccctctccaaagagaatgatttctgcaatgagggtggagtcaggcaccaccatggcaattgggcggaacatggatttaagattttcgggaagctctgtgcggccagcatagccaggattcatggtaatgaagatcccacaggaccacaccagatttatttcaaagccatcaaaatggaaatgggtgaggccggcagccagggcagacaggatgcacaggatctggtgggccaccactgacagcacctcgatgttgatgcggttaaactcatcaaagcagccccaagctccagtctgggccagacctgagtacattcggcccatggacttgtagtccaggccctcagagcagttgaccacaatgacatatatgcccagggccttgcccaggtccttgacggtctcggtcttgcctgtgcctgcagggcctttgggggagccccctcggtgcaggtgcaatgccgtggtcagtgtcatgtaacacctgtccgtcaggggggtgatgacgagccggcccgagttacccaagtactcataattatactgaaattgcgtgttggtctggcggatgacacagtcatcaagatccttctcccagtagaaccgaagttggctgagccagtcaaaggaattgacatccatgaggccactcttgtaaagcttctccaacacatcccgggcatgaatttctatcgtcaccagagccacaattttaagccgcatgatcttggtcaagttccccctgatggcttctgaatacttattcaggattgacacctggttcttcttcatgaccttgaggattttcttgtctgcccgctccttcgctgtcagcaggcacttggtgacatcagccgtccactggatctgactggcagtgatcaccacctggccagcccactccttcacccatttgtccctcttgttgaggaacttcctgagggccaggtggcagttccggagaaggtcccgcagggtcaccctcatggtctgttccacatcgccaagccaggactccacagggccttctaaaaatactgagtggaggaagtcaatgtactcgccgtcgcccgagaacatccccacagcttcccatttgctgctgggccctccaaccttctggattctcagcaacttgatgttgtcaaagcattttttgaggtgtggctgcacagcctctgggtttcgggactggcccagaatctccagcaggtcatcattggacaagaagtagaagcgggggaaaatatgtcgcttggtctctaaatacatatccagagatttctgaatatcttccaggattgtattcatttctatcaatgtgtccaggaggcctgggtgatgggtgctccggagagcattgttgtccttgttcatcctgtccatgatggctttccagttgctgttgacctggtcaaataaggtcgattcattgggcagctgcttgcggatgtcttctcctaggaagatattctctaagtacatccactgacgctgcactgtgagaatcatctcaataacctccaaaatgagggagaggcagcgttcccagtggtccacatccttctcaaaggccttgacaaagcgtgatgccttcatggtagacagagctacctggttatcttccagtgcctggaatacttcttctgtacctctgagccgatgatggcccttatccttgtagggtactatgtcgagctgagtcacatcccaggtcttggcaatgttttgtaaagccacttctatagccagctctttagttgctgaagcagagatctccccaattttctccacatgctgatccatcccaagctccacaatctgctccaaggtgaagctttcagattcctgatcaaactcccgctggatctcatcccggacctggtcccagtgcctctctctaagggcagggttccgcaggtctgagatgagaggcatggtcctcttgaactgctctatttttgagcgagtggtttcaataatttcccagtttcggtccttatactctttggctaattttgtgaggcgacgaaacagcccgtgggccgtggtctccatggtttccgtctgcaggatcaggaaccggccagtcttccactcattccagttctcctcccagtctcgtgcgatctcccagatttgctggagggcatcgagctccttctccaggttctgaaggtccttggagggtggctgctcgatcttgaagatgcccaggttggctcggagactattttcctcttcccgcatggccatcagcatggcccgcacttgtgtaatctggtctaaggcagacatgtatcccacgttgctggtgaaatggcctttgaattcgaaatcttccagaagtgtatgtgctttcttcttgaagtcatctgccgagtggatcaggcctgtcttgaatttctccttgtgtttcttcagcatttgcttactgtccagcagagtttgttggaagacaacccactccccgttgagactgtccagcatctccaggacactgtcctcgactggcacctcgtacttttcaagaatggcaaattgctcgtgtatgggagggatctgagtctccacgttggccaagtcgtgcttcagggcatccacgagctgcaagctgacccccagttcctccagtgtctgcggagggcggctgattttctctgcgttctccttcaggtaggtgtgcagctccaggaggcgcccagcagccatctccctgagcagagtcgcgaacttgttctgccattcattgcagtgctgcaccagggagaacttgaggtgcgaacagtccagcagcacaaactggatgttggtgactgtctcctccttctgcacgttattagcaacttccgtgtagcgggcaatgtcggcaacaaaagaagagacaggagggttgaggcgctggtagcgatgaatgaaggagtccttgttgatctcccagatctcccggtacatgtcccaggtcttgaggtagttctgcagcaggcttgcgttgttagtcatgccgctgctgatttgggtctggatcttcttgatgtcctcatcttgctccacaactgtttggatgggttcacgatgtaacttgcgcttggtgagaatgtcagggaggtggcagaagacagagatggtggaaaagaggtggttgccaatgtcattgaccacacctgccaaagtctgcagagtgggtgagaattccacctgtgccacacttccttgcagatcattcttcaaaatgacaaggacttggaagagtgggtttgggctggtctttccatccccgttgatagccttggatagttctagcagtgaccacttcacattcaggcgcagggcatcctccatcatgcggtccagccgaatcatgtacagcatccactgctgctgaatctcaggaccatcattcttgaagacctcataggagttggtcatgatggtcaccacatcctggtgcaggttcatcaatttctgctgtacagctgcccgatgctctctttggtcctcttcaaattccaggtccctgtatacccgtttgccactaatgcgtaccagcagcttctctgacatctcttgggctcgccagccaatggtcagagtggatgccttgaactcattcacaatcatctgcaccttgctggcatgtatacggcactccgtgatgaagaaggcactggcccccttcaaggcccagtgcagtttcttgagtcccgggtggatcttcttatccaggagccgaatacgctctttgaatagggcctgctcatctggggacagcatggcaataatcctattgtagtctctagcaacgagtagcagattttcacgcagaatgcgcaggtcctcggctcgctcagctacgttcaccacgtaatggggcgtctcaaacagcagccgctcccagtagtcaatttccgcaaagagaatcagaagggacttgtcaaagttgacatccagcatgcccgccttctcctggctgattcgcagcaatggggtatccaaccgccgaatgcaatccttgtccagacttgatgtccactcttggaaggtttttcgaaccagctcatcaatggcctggaccatctgctgataggtgtgcacactctcctttccagtcccaatacggggcaggaaatgagcaccagcaaggcaggtcatgactctgtcgatgcgacgccggaggatgtgcacccagcgcgcctttccggaatactgggccacgtagggctccaggtctggccatttcttgttccgttcacggttcaccagggccagctcgctattgaacagcatgtagagatccaccgccttcttgtcataagtccgcttgatagcctcgcgggaggcaagcctgtggaaggtgtccagcagaagcacgccgtgcggcacgtcccgcaccaactcgaaggctgaggtgatcaggttctgggtcatcacctccaggtccttgattccggcacggaacttattgtagtcttcatgccaacaggtgttcttgacatccaggatacccccgcgaacggctcgcagcgtgtgcagatttttatgaaagatgtcctcaatctccagcaagttccgtgttatctgtggcccctgggcaccaaagaagcaaggaaggggaccctgcttgccatcttcccagcgggcgaagtgatactgacagtcacatacctttcggaagagcgaggtcagtctctcccgagtgttgtagtggggagagttgacccagatgatgcggatgagactgatcagcttagggagcttgctagagatgtccttgggcttcatgaaagccaactcctggtaaggttccttcaggattgacaaaaaggtcaggtttgactgtgcttgacgagagccatcctggatctgctgtgccagtttcataaagggcgccaagtaggacgacttggcaaggtgcaggatggattcaacgtgcttcactcccttcttcaccagctgcttactgatgccagacaggtccatgcatcggttgcgccagaactcaatctcctccagaggacctaaattttctcctgtctccacagtctcctgggcactgagcatctcctttatctgccgggtccagtggatcatggaggtctctagccgttgcaccagctctttgtcctttatcaccatctcaggcttcatgttcatggcctctgcagggatgtagaggaccgtgtgcccctccagtttgtaccgagtgtctgtcaggcaggccaagaacttgtgcagatgagaagcaaaatgatttctaatgctctcaggccagcctgtgtttgcaaagatctgaggggcaaagactccaccgagcagccgaagcagggccgggatataggggccccgcaccgtcccaaactgcacagttgcctcgaagttctcccaggtgatgggaactggtgcttggcgaatgaagtagacaagctggttctgggtctgtacaggcatgcccagctctagcttcagcccaaaacaagggtcaatgaagatggtgaggatggattctgtagggtcctgggcaaagtgttccagaatggcatcatgctcctgtgtccacactgcatccgccagtcctgtcagcgcagctcgggaaaggaagaggggcttcacatctgcctcgggctccactgattcttcactctgtgcttgaggtccctccaaccgtggctcaggctcctccttggggagctcagcctgcagctctggctcactgacagccggggcattcccctgctcctgtgtggccacagcagcccgagtggcccgccctgaccagcttgcctgggagcttcctcggccactcaatcgctgcttcttctcagctttgctggacatcgtgcaggcaaaaccttgccacgctgaccctcccctccctagaccgaccgatgggccactctaagaagttgcccctcgcagc

SEQ ID NO: 8723 - RNA, 10033 nt, Homo sapiens
  source 1..10033: mol_type = other RNA
aagccctgtctcctcccatctggccttctcgccagccaaccccgacacgagcatcccagctcgctccagcttcagctccatctcttcagacttcttgcgaagctcctccttctgtgccagcttctcatcatactgtttctttagcatctccagtttctcagctacctcccgcagcttctcctgggcctcagcgagcgcggcttgcttctcccgaagctgagccaaggcagcgttcattcggattcgcttgggctccaccacccgatatagccgcccatacagctccatggcccgcacccacatgcagagggacttggcagccagggagacgcggccgatgatatcaggctggaagtcaggctgggcgcagtaggccccaatcttcttcagaaccttatctgagatattgtctttatcaaagttgatcagtgacttgatgaagttctgttcccctagctgcctcttggcctctgcccatgtgggctcgttgcctcgaagaatcataactgcctgcatcactatctccacttgggctgggggccgtccataagacttgatctctcctatatccttcttgttcagagactccagggcccgcatggcctcttccagggcgggcagtgcctcttctagatctttctgggcattgtcagccagtgcctgacacttgatttcctcaactgcaatcttttcactgttggctgttacggccttctgctgctcatctgcctcccgcttctgctgcacaatgatgaccaggtactcctcacactgcttctggaactcagccaccttcttcttggcatcctccagctccaacgacatcacttgcaccttttccctagtttcgtcgatcttgaacaagcctgtccgcagtttattggcttgggccagcagctcctgccgtttttctcccagcaacttcttatatccagacaggagttccaggtatttggtgggtgtgacatagttgtgtctccgcagttccaacagcatcttctgggaatactgagctactgaccagtgcatagtgacaaagatctgggccaccttcctgtggatattctcctgagttcccaggtctactcctatgaggcacttctcagccacctcgagcagggcctcttggggccactctgagaaccagttgatggttgtgcagttcaccaaggctgggtactggcggatccagttcctgaagggatcccccatggggctgaggcagagcacgatgtgcaggttgttctgcacgcgttcaatgaggtaggcgaagaggctgtccgatgactcaggcacctgctccacccgggcctggtctatgatatgcgactggatctcttcaaattcatcaggcttgtagagattgggcacctcgcctgagctgaggatgttgttgatgtcctctaggaaggactcatcagctatttgggtgtccacaaaaatgaaggacgtggtcttgagctccaccccagcctggcgatacagacgcttgatatcatctcggaactcctgcttccgataatgtttggtgacctcgatctggaaggtggtgtagtcgcagatggatgaagccaggcgggccagactctggcgtccgctgcccccgatacccaccaggagcatgttgccccgaggctgtccaatgacccgcacgatccgtgtgatgtgttcaatagcctctcggaagagcactagctgcatgggcacgacagagggtgacaggttatactcatttagagctgtctccatgactgtcttcagcactgtcagatccgtgaggtcttcatacaccttgggctccttcaggaaatccccaaagataggaggacgcttgctgggacagagatgatgaaatgtgaggtcaaagaaggagccgagcttgtcgcttatgatgcccatgaaggcttctgtgtctgccgcatcaaccagccggtcagagaagactctgaaacattcatggatccagagccgtgtgatgctggacttggtatcatggaagtccttgttggctctaagcatgccctggaacactgtggggaaggtcatgttgataatgttgaagcgactccgtagccttggggagatgacagtccgtccacccccaggggggcccatggcagccatcaggaacatttctcgaatgtacttgatggtctgcttcgtacggtcataccagaagccatagtcaatccagaggcggatcagctccaggggtggctgggacccaaacatgtccttagcgggcatatttaggtcatccataaaggtgatcatgcttttgcccccgaatggcacgtagacacccttggttcgcttctcaaccctgctctcaatgatgctctgcacgttattggatgtggtctgtgcggacatgttgacaacgagcaccgaccactggctggagggcagggactgcagaacgctctgggcgatggaggtcttcccagtccccacgggacccaccagcagaatgggattctggttggccaccaagctgctcaccaggtagttgtagcgaacagtgtcgacggtgggcaccatgatcttatagaagggggcgtttggagggtagcgccaactcttagggagcttgtcctcaaatgatgtccaactccgtattttggggtccacaaaatactcatataccgtgtccttattgggaaaggagccctcgatctctcggaggtagctgtcgatcctcttccggccctcctcatccacagaggcacacacagaccagatcatgctgaacacaaatgtcatctctaccatggtgacatagttctcgccgtcagctgggttcaccccattctctggcgtggccagggcagagtacagcttgcagagggaggtgataccgctgtactcgggcaggggcaccagctccttgcagttgtccttcttaaaggccagcatcttgttgatgagcttttcgaacatgcgttgaaggggctccacctcagcctttggcctcttctccagccatgactgaacatagggcttccagcccaggtcagcgtagtcagtgtagaccatcccgcagcgggatacagtggccggagaggccattgccaggtcctccacttcaaacaggagagacacctgctcgggcatcgcgatgcgctcgccgttgatgagggtcaacaccttgttatcgtccatgacggagttcatgttctcgatccacagtgtgtccacggggccatcgaacaggatccacttctcgtcgggtttctcatctgcacatgccgtccgcatgacactggacaagatgccatctgtccattcattggtgctgaggtcatattccccatacagttcccctagggacaatgccttggggttcaaagggaactctctaacaatgttgaagttagggtctccggcgcggcacagagaggacagggaggcctgtagaatgcgccatgaggcagtcttgccgctgcccgtgcagcccacgatcatggtggagtggcgggagttcttggtttcatacaactggaaaaccttggtgagggtgaacggcgtgctttgcaggcccatgtctcgaatctcctgctcaacggtctcccgcagcttgccatagtcaatgacaggcagctcaatgttgggaaacagatcttgcacgatggcattgaacaggggtgcatcaactgaagtgagcttggcgatgttcatatctctcattgagagcagcagaacctcttcatcagtcagatccggctgtaggcggcgcttcttgccagcatagcgcagaagggaggtgagggcacgcaggccaaagtcatagtggtcctgtctggacagctgctgcacagccagtgagtagagtgtgtacaccttcttggccagaatcttgcagttgccaaagccctctccaaagagaatgatttctgcaatgagggtggagtcaggcaccaccatggcaattgggcggaacatggatttaagattttcgggaagctctgtgcggccagcatagccaggattcatggtaatgaagatcccacaggaccacaccagatttatttcaaagccatcaaaatggaaatgggtgaggccggcagccagggcagacaggatgcacaggatctggtgggccaccactgacagcacctcgatgttgatgcggttaaactcatcaaagcagccccaagctccagtctgggccagacctgagtacattcggcccatggacttgtagtccaggccctcagagcagttgaccacaatgacatatatgcccagggccttgcccaggtccttgacggtctcggtcttgcctgtgcctgcagggcctttgggggagccccctcggtgcaggtgcaatgccgtggtcagtgtcatgtaacacctgtccgtcaggggggtgatgacgagccggcccgagttacccaagtactcataattatactgaaattgcgtgttggtctggcggatgacacagtcatcaagatccttctcccagtagaaccgaagttggctgagccagtcaaaggaattgacatccatgaggccactcttgtaaagcttctccaacacatcccgggcatgaatttctatcgtcaccagagccacaattttaagccgcatgatcttggtcaagttccccctgatggcttctgaatacttattcaggattgacacctggttcttcttcatgaccttgaggattttcttgtctgcccgctccttcgctgtcagcaggcacttggtgacatcagccgtccactggatctgactggcagtgatcaccacctggccagcccactccttcacccatttgtccctcttgttgaggaacttcctgagggccaggtggcagttccggagaaggtcccgcagggtcaccctcatggtctgttccacatcgccaagccaggactccacagggccttctaaaaatactgagtggaggaagtcaatgtactcgccgtcgcccgagaacatccccacagcttcccatttgctgctgggccctccaaccttctggattctcagcaacttgatgttgtcaaagcattttttgaggtgtggctgcacagcctctgggtttcgggactggcccagaatctccagcaggtcatcattggacaagaagtagaagcgggggaaaatatgtcgcttggtctctaaatacatatccagagatttctgaatatcttccaggattgtattcatttctatcaatgtgtccaggaggcctgggtgatgggtgctccggagagcattgttgtccttgttcatcctgtccatgatggctttccagttgctgttgacctggtcaaataaggtcgattcattgggcagctgcttgcggatgtcttctcctaggaagatattctctaagtacatccactgacgctgcactgtgagaatcatctcaataacctccaaaatgagggagaggcagcgttcccagtggtccacatccttctcaaaggccttgacaaagcgtgatgccttcatggtagacagagctacctggttatcttccagtgcctggaatacttcttctgtacctctgagccgatgatggcccttatccttgtagggtactatgtcgagctgagtcacatcccaggtcttggcaatgttttgtaaagccacttctatagccagctctttagttgctgaagcagagatctccccaattttctccacatgctgatccatcccaagctccacaatctgctccaaggtgaagctttcagattcctgatcaaactcccgctggatctcatcccggacctggtcccagtgcctctctctaagggcagggttccgcaggtctgagatgagaggcatggtcctcttgaactgctctatttttgagcgagtggtttcaataatttcccagtttcggtccttatactctttggctaattttgtgaggcgacgaaacagcccgtgggccgtggtctccatggtttccgtctgcaggatcaggaaccggccagtcttccactcattccagttctcctcccagtctcgtgcgatctcccagatttgctggagggcatcgagctccttctccaggttctgaaggtccttggagggtggctgctcgatcttgaagatgcccaggttggctcggagactattttcctcttcccgcatggccatcagcatggcccgcacttgtgtaatctggtctaaggcagacatgtatcccacgttgctggtgaaatggcctttgaattcgaaatcttccagaagtgtatgtgctttcttcttgaagtcatctgccgagtggatcaggcctgtcttgaatttctccttgtgtttcttcagcatttgcttactgtccagcagagtttgttggaagacaacccactccccgttgagactgtccagcatctccaggacactgtcctcgactggcacctcgtacttttcaagaatggcaaattgctcgtgtatgggagggatctgagtctccacgttggccaagtcgtgcttcagggcatccacgagctgcaagctgacccccagttcctccagtgtctgcggagggcggctgattttctctgcgttctccttcaggtaggtgtgcagctccaggaggcgcccagcagccatctccctgagcagagtcgcgaacttgttctgccattcattgcagtgctgcaccagggagaacttgaggtgcgaacagtccagcagcacaaactggatgttggtgactgtctcctccttctgcacgttattagcaacttccgtgtagcgggcaatgtcggcaacaaaagaagagacaggagggttgaggcgctggtagcgatgaatgaaggagtccttgttgatctcccagatctcccggtacatgtcccaggtcttgaggtagttctgcagcaggcttgcgttgttagtcatgccgctgctgatttgggtctggatcttcttgatgtcctcatcttgctccacaactgtttggatgggttcacgatgtaacttgcgcttggtgagaatgtcagggaggtggcagaagacagagatggtggaaaagaggtggttgccaatgtcattgaccacacctgccaaagtctgcagagtgggtgagaattccacctgtgccacacttccttgcagatcattcttcaaaatgacaaggacttggaagagtgggtttgggctggtctttccatccccgttgatagccttggatagttctagcagtgaccacttcacattcaggcgcagggcatcctccatcatgcggtccagccgaatcatgtacagcatccactgctgctgaatctcaggaccatcattcttgaagacctcataggagttggtcatgatggtcaccacatcctggtgcaggttcatcaatttctgctgtacagctgcccgatgctctctttggtcctcttcaaattccaggtccctgtatacccgtttgccactaatgcgtaccagcagcttctctgacatctcttgggctcgccagccaatggtcagagtggatgccttgaactcattcacaatcatctgcaccttgctggcatgtatacggcactccgtgatgaagaaggcactggcccccttcaaggcccagtgcagtttcttgagtcccgggtggatcttcttatccaggagccgaatacgctctttgaatagggcctgctcatctggggacagcatggcaataatcctattgtagtctctagcaacgagtagcagattttcacgcagaatgcgcaggtcctcggctcgctcagctacgttcaccacgtaatggggcgtctcaaacagcagccgctcccagtagtcaatttccgcaaagagaatcagaagggacttgtcaaagttgacatccagcatgcccgccttctcctggctgattcgcagcaatggggtatccaaccgccgaatgcaatccttgtccagacttgatgtccactcttggaaggtttttcgaaccagctcatcaatggcctggaccatctgctgataggtgtgcacactctcctttccagtcccaatacggggcaggaaatgagcaccagcaaggcaggtcatgactctgtcgatgcgacgccggaggatgtgcacccagcgcgcctttccggaatactgggccacgtagggctccaggtctggccatttcttgttccgttcacggttcaccagggccagctcgctattgaacagcatgtagagatccaccgccttcttgtcataagtccgcttgatagcctcgcgggaggcaagcctgtggaaggtgtccagcagaagcacgccgtgcggcacgtcccgcaccaactcgaaggctgaggtgatcaggttctgggtcatcacctccaggtccttgattccggcacggaacttattgtagtcttcatgccaacaggtgttcttgacatccaggatacccccgcgaacggctcgcagcgtgtgcagatttttatgaaagatgtcctcaatctccagcaagttccgtgttatctgtggcccctgggcaccaaagaagcaaggaaggggaccctgcttgccatcttcccagcgggcgaagtgatactgacagtcacatacctcaataaggtccttgcagcgctgcacaaaggcatcaacctgagcaaagatgctggtctgatctaggacccagccccgactggagaactggatgtgcatctgcacagcctgtacgtagtgatctttccaagcgtgacaacagagaatgcagccttgcaggtcctccttgctggaagagacatatccctcaaagatccggtccagggagatggcgtggcagcataagcggatgatctcattgctcatctttcggaagagcgaggtcagtctctcccgagtgttgtagtggggagagttgacccagatgatgcggatgagactgatcagcttagggagcttgctagagatgtccttgggcttcatgaaagccaactcctggtaaggttccttcaggattgacaaaaaggtcaggtttgactgtgcttgacgagagccatcctggatctgctgtgccagtttcataaagggcgccaagtaggacgacttggcaaggtgcaggatggattcaacgtgcttcactcccttcttcaccagctgcttactgatgccagacaggtccatgcatcggttgcgccagaactcaatctcctccagaggacctaaattttctcctgtctccacagtctcctgggcactgagcatctcctttatctgccgggtccagtggatcatggaggtctctagccgttgcaccagctctttgtcctttatcaccatctcaggcttcatgttcatggcctctgcagggatgtagaggaccgtgtgcccctccagtttgtaccgagtgtctgtcaggcaggccaagaacttgtgcagatgagaagcaaaatgatttctaatgctctcaggccagcctgtgtttgcaaagatctgaggggcaaagactccaccgagcagccgaagcagggccgggatataggggccccgcaccgtcccaaactgcacagttgcctcgaagttctcccaggtgatgggaactggtgcttggcgaatgaagtagacaagctggttctgggtctgtacaggcatgcccagctctagcttcagcccaaaacaagggtcaatgaagatggtgaggatggattctgtagggtcctgggcaaagtgttccagaatggcatcatgctcctgtgtccacactgcatccgccagtcctgtcagcgcagctcgggaaaggaagaggggcttcacatctgcctcgggctccactgattcttcactctgtgcttgaggtccctccaaccgtggctcaggctcctccttggggagctcagcctgcagctctggctcactgacagccggggcattcccctgctcctgtgtggccacagcagcccgagtggcccgccctgaccagcttgcctgggagcttcctcggccactcaatcgctgcttcttctcagctttgctggacatcgtgcaggcaaaaccttgccacgctgaccctcccctccctagaccgaccgatgggccactctaagaagttgcccctcgcagc

SEQ ID NO: 8724 - RNA, 7512 nt, Homo sapiens
  source 1..7512: mol_type = other RNA
aagcctctgtccccaccccagaaggaaacgaatgccttcaagccaatgtggcctgaagtcccacgacaaaaggttcatgtcagctttgcctccctgtgaacaaactaaagttaaggcagaaatggaatgagagaaaaatgaaagaaaaaaaactagaaacattttcaacagacaaaacaagcctatcccaactgaaaccaaacacggtttttaagagaaactggaaatgtcgctatttgacgccagaacctgaatttgagccagtagctgctggtttctagatcaaactatcagcatctcttcctgctccctctgcggcctgggtcctggatggactttgtgtccgccgacccagtgtggtctctgtcctacaattcttgggatgggaccagcacaatggcagaagagacctccagtgtctgagagaaaaggatcggaagaggccacgtcctggcaggaagcagggccgacagagggcagacaccccagaacacccgccctcagcctgggagaaagtgcgttacggctgcagcctggaaacgagggcaggctctctccaggacggttccgctcagaagggcctggcctcctgagaagcagcccccacacagcatgctttctgaatgcactgtgggtgggactccagttcccacttccaggatgaagagtgggactcaaatggtttaccagtgcaatgtggggtcaccatgcagacctgcccctagggtaaaatacaggctgcccccaacacctgtcttaactccaggatctcccttgctcaaaagtggcctcaatctgtggcaagaaagatggggccgtcctcaccacaagatccaagtgacaatgcgcatgagaaggcagccttctaacacatccctttggcaggcatatgtcctgggtcacttgtgtgctgagttatttgtatggaatcattttcttagatgatgaaattttcggagtattaaaaaagacattcatccagaacaatcaagtgtgtgtacacagaaatctagaaggaaatctacaatggacacaggcccatgcgctttccatcccgtggaaacagaacagtgacactggagaacagaaagtgaacattcacctcctgcactccctgtgcaaaatggaagaggtctgatggagcagatgtctgtgctgctggcagagcacaggctaggagcagacacaagtgaaacgccaggcagaaaacagagtctgtaacatcgtccctgcaaaccctggatgctcgctgctgtgaccaggcctcggtccaagcctctgtccatgtggaacgcccctttgctccctttaattaaagggataattatatataactttttattaaaaaatcaactctgtattctgtcaatagttggtaggaattcacaattagtgacatggctggaaaaaatagatcacaatagtagtttatggaagaaaaaaaggctgttctaaaattatttatttacagacgtaaaaagccatgctgcagaactttctccaattatgaagatttcctacaatgtattaaaataaaagatttttttttttaaaaattatagctcttggattccaaattcctatgcccccgatctgcaagcctcgtgggctctggagcactcgtggcggagtgtgtcagtgtgtctgcacgcacagtgaagggtgtgaactggattctagcacctactgagaaatcaaggaaaagaaaactaaagccaaaccccaagattgcagggaagctttctggatgttcagtccagtccaggactcactaagtttctgggggactgtcatgcagggagatccaaaccagtctcaggaaatcctctcgacaaacgaacactactatgtggatacatttttagttgtgggtttttaaatatataaagaaatctttagaagatattctttttgcttttgcagctcctattttatgtaaaaagtcctgtttctccccccaagaactggggtttccacagccagcgttaacaaataaataacttataactgcttgtcaccttctttcttcagtcgactgtaataatcttcctgacttggtaggtggccaccatgcatgtgggggtgtccatgcagccactgctgctccatggccagtctctgcagctcggccgactgggcatgcatggcctgcagctggtgggctgctgacatggggggtgggatggccccaggcaggtcacgggggtagggggtgccgaaaactgggtggcgaagcatctcgtgctcgtgtgggggctgtccaagcagagggttggggagagtgccaggcgggtaggggaagcgagccaggtggggaccggcagtcagggggtcgaccagcgggtgaacggggcctgctgaaccttggtggagggggtcctgctggtggaggtggaggtgggagtgaatgtgagagtgctggtgatggtgcggagtcacgttgaacatctgcagtcgggccaggggatcgctggtcagcgatgccatgcgctctgcgtggatacgctcggctgccagtctgtcagggtagctcatctcgggccgcagctgggggcccgccagggccagtctctccctctccaaggggttcaggcccgggtggaaagaagcaaaagggtggggcccggcggtcggggggatggtgagggcgctgtgccgggcaaagtgctccatggggttggcggctgggtgcagggggtccagctctgggggcttcacctcgaagcccggcttcatcctctcccgcagctcccgctctcggatctcccgctctcggatctcccgctcccggagctcccgctcgcggatggtggggtcgacgttgtagaggccaggcatgtggtaggccagcagggggtccgtggggttaaggggcatgtagaaggggtggttgcggttggtgggcgacatgacgtggggccgggcgtactcgctcagagtccgaagggcaggtgtgtcgggcccgatgtaggggggcacagcagcaatggtggttggtggtggctcgaaggatggccgcatgtggccaggaccactgagctgtgggtcactgaggcgaccttcatgcgctgagctggacgccttagccgcccgctctgcctcgcgctcccgctctcgctcccgctcccgctccttctccttctccttctcccgctctcgctcctctcgggctttctgctcagcctcgcgcttggccttctcaatggcctcctccctcttcttggccagcttggacccggccagaggcatgaagtacaggtctgtccgggcacacgagttgtagccccggtccaggtgtttgtagaacctagctgactggctggcgtgactgggggtgtccaccacagtgggctccggggacgggctccttggtgggggaggggggctctcaggctcctcagcgtcgtccagagcctcctccttgatctggacggtggggagtgggcaggacgacccccccgctatgctgcctcctgaagccgccgcaccagagcagggtggctgggccgaggtgccaggtcccgccggtggggtagaggtggaggggcaggtcggaggggtgatgggaggagggcctccagggacaaaggggtgctgagcaaacgggggttggggggccacctggtggaggcctgtaggggggtgggaggcagggggcgggggcaggttctggctctgggtcagcccggggggctgggcgggcgaggagggcaatggctggctctgaggcatgagttgcaggggtggggggtgagccgacggggggtgatgtgtggacagggagctcaggggcttcagggctggagggggaggcaggttggcattcatggagaagggtgagggccccgagaggtggggagggtgcttgtgggcctgtggcgccggcagctgggggatgggagtggtaggcgggggcttgatgtggggcatggccaagggcgctggtggcaggggctgctcccgtggaggctgttgggactgcagcgctgactgagaggctggcagctgcagggaggtgtgagggtacgctgctgctggggaggtccccagaggggcctggccttgggaggcctggggagggaggccaaagggctgtggggggcctgggtgctgcagcaggggcccagcctgcaggctgtgagggccgggtgggccctgaccgtgcagtgggggctgggcatgagagggtgcagaaggctggcccgccgacccagtcagaggctgcagcgggggatgtggcgagggatgcggcgggggatgcggtgagggcggccgctgggggtgcaaggccggtgcctgttggatgtgggtgtggggaacaggcgctgtgggagcctgtggctggttaggggcctgggaggccgtgggggagccctgtgggggaactgcagtggcagagggcgtgggccctggcgtgggcagctgaggggtccctggaggagctgaggagggagctggggtgaccccagtgggagcctgcaaggctgggggctgggcctgcagcatctgctgctgggctgacgagtccgagtcactctcattgtcctgggggctggggatgctcggggacgtgctgcgattgtcctggtcgatgtctttggggtcactgctaccctcatcgttgacgctgcgactgtctgaactctctccctcaccttcagatggcgagttgggcctgctgatctcctgcgtttttgtcttcttggagctggtcctgtcagcctcctccgtatcagaggccaccttctcccgctggcgtttgttactcttaagaggggaagaggcttcctccttcaccttcttggccgacttcttcactgtctctgctttactgtcattgctggaggtactggcagcgctgggggagttccggccgctggagcggatgtcttcattgatgggtgaggtgcgaccatcagggctggctggctgcttcttccgaccactgcgtagtgtcgacatcgagccccgactccgccgtgtcctcatgctatgcttcccactgagcccatcatcctcttccttgacgggtttgaacataaacggtggcgggtccacgggcttctcaatgggcgggagctcaccgtatttcttgaagtggatgcgacagtcggtgcaaagcaggatgttctcccggcctccgtggtgccaatctttggaggtggtggtgaagcagtggcggcaggcgtaccccttcagctcctgctcactgtcctcactgtcgaagtcatcttcactggctgaacttaggtccaagaattcactggacgggggtctggagggtgtgttgacgggtgtggacgcggtgcgagtcttaatcctcctgaacacggcctgcctgcggtgcctacgatgggctcgggagctggctgcttcgggggtcttcttccaatagtaatagaaggtgatcagctcccctgtttccttattgggaagcagctcctttctaattctgaagaagttcttcccgtactgcctgagtcccttaacgaagcgtttcacttcgtcctcggtccagcacttctcgatgagcttgggcacaggcttcttcaccaggcgctgcagggctttgccagcatcgtaaccgctttcatgcagtgtgttcagtgcattcagagtggtgtcatcccgagaggctgcgacacagccgtcctctgtagagcctccatcacacattcctgcaaatgccgccatgctccttgctgccctcaagtacataaggaggtcacagtcgttaactccaggcatccagaccagttcctcatgttgggtcactgtatcaccatctggagaaggaaatggttgcagatctggaagtttggcctgatgactaggaccgacacgaatctccccctgggtactgttcagcctccttgtctcagggttatatcctaatatgtagaaaaatgaatccactcgggctttaaactctctagcagcaaatatgtcagaaaaatgggagatgttacacttccctctaagggcagcagcatggtaagtgtcaacgtaatcagaaatgaagagctctcggttcttgataactgggtctgtaatgacaagttctcttccagagtcattttcattatgtcgatcctgaaccaaatgctgatacacagaatctggaacctcagattgacggtagtaccatttgacgttcatgaggagatggtccctcttactccctacaggccctctcccggcttcagaaagatgctgtggtggctgtgatgccaccggcagagagcatgctggggggtcacacaaagcaggagttggagatctgcaacaggcctgggagttgtggaccagtttgaagtcttgaatgctacagatgaaatacggtgtgtttggcctccgactctcgatatacacacagtctcctggtctgtagaccacatcatcttcagtgatgtaggatgttatctcaccggtatctgtcctttcataacgagacttttttttcggtggtttcttcttattcttcttcgtggactcctctgcggtggcactattgttgtcattgtcctcgtcttcactgtgatcactctcagcataatttttggctcctccttccaaggtacagctccggcgtggccttgaattctcactctctcttgctttgtctcttttctctctctctcggtcccggtctcggtcccggtccttctctttgtctttgtctttgtctttgtccgctgtcatgattcgccacgtgccttcttctgtcctctcacggctaggcctccgtgaaaggtagacagtaagcctgggcttcagtcttctgaatttctcactcaattccagggaaaatccaaccactccaacaaccccaacgtttcaaaaatgctctaattcaatgtaatacaaataagaggtcttccatccagaattatatcaaatggccacaattcctttctcagtaacaccataaacaggctgaagctctccacaaatcttctctgtaagtggatcccacggtggttgtgacccggtgctgagcgcacatacagttactcctagacaatcacctccttcccctaaagcgctacaccatcaatagtgaggtgttcgcggcccagctccggggaaagtggcggggatggggcgggaggccgcgcggaggctgcggggccgcggggcgcagggccgagaggggcggcccgcggggaggcgacgcggaggggctgagggggcttccctgccgtgacctttcctgcgacttgaacctaggctccctcctcctcggtcgggcagatctttcagaagcaggagcccaggatcatgtctggttttgttttccgagggcgagggggctccctgaggatgatggtgatttttttttttttttaatcctcaactaggagagaaaatgaggcagagacaatgtggggagcgagagaggggaaaaggacgggggaggaggcggggaccgaggcccagcggggcgagcgtctcggggtgtgcgggaggctgaggaggctccggagcgcggagggttgctcgcgagcgtct

SEQ ID NO: 8725 - RNA, 7327 nt, Homo sapiens
  source 1..7327: mol_type = other RNA
aagcctctgtccccaccccagaaggaaacgaatgccttcaagccaatgtggcctgaagtcccacgacaaaaggttcatgtcagctttgcctccctgtgaacaaactaaagttaaggcagaaatggaatgagagaaaaatgaaagaaaaaaaactagaaacattttcaacagacaaaacaagcctatcccaactgaaaccaaacacggtttttaagagaaactggaaatgtcgctatttgacgccagaacctgaatttgagccagtagctgctggtttctagatcaaactatcagcatctcttcctgctccctctgcggcctgggtcctggatggactttgtgtccgccgacccagtgtggtctctgtcctacaattcttgggatgggaccagcacaatggcagaagagacctccagtgtctgagagaaaaggatcggaagaggccacgtcctggcaggaagcagggccgacagagggcagacaccccagaacacccgccctcagcctgggagaaagtgcgttacggctgcagcctggaaacgagggcaggctctctccaggacggttccgctcagaagggcctggcctcctgagaagcagcccccacacagcatgctttctgaatgcactgtgggtgggactccagttcccacttccaggatgaagagtgggactcaaatggtttaccagtgcaatgtggggtcaccatgcagacctgcccctagggtaaaatacaggctgcccccaacacctgtcttaactccaggatctcccttgctcaaaagtggcctcaatctgtggcaagaaagatggggccgtcctcaccacaagatccaagtgacaatgcgcatgagaaggcagccttctaacacatccctttggcaggcatatgtcctgggtcacttgtgtgctgagttatttgtatggaatcattttcttagatgatgaaattttcggagtattaaaaaagacattcatccagaacaatcaagtgtgtgtacacagaaatctagaaggaaatctacaatggacacaggcccatgcgctttccatcccgtggaaacagaacagtgacactggagaacagaaagtgaacattcacctcctgcactccctgtgcaaaatggaagaggtctgatggagcagatgtctgtgctgctggcagagcacaggctaggagcagacacaagtgaaacgccaggcagaaaacagagtctgtaacatcgtccctgcaaaccctggatgctcgctgctgtgaccaggcctcggtccaagcctctgtccatgtggaacgcccctttgctccctttaattaaagggataattatatataactttttattaaaaaatcaactctgtattctgtcaatagttggtaggaattcacaattagtgacatggctggaaaaaatagatcacaatagtagtttatggaagaaaaaaaggctgttctaaaattatttatttacagacgtaaaaagccatgctgcagaactttctccaattatgaagatttcctacaatgtattaaaataaaagatttttttttttaaaaattatagctcttggattccaaattcctatgcccccgatctgcaagcctcgtgggctctggagcactcgtggcggagtgtgtcagtgtgtctgcacgcacagtgaagggtgtgaactggattctagcacctactgagaaatcaaggaaaagaaaactaaagccaaaccccaagattgcagggaagctttctggatgttcagtccagtccaggactcactaagtttctgggggactgtcatgcagggagatccaaaccagtctcaggaaatcctctcgacaaacgaacactactatgtggatacatttttagttgtgggtttttaaatatataaagaaatctttagaagatattctttttgcttttgcagctcctattttatgtaaaaagtcctgtttctccccccaagaactggggtttccacagccagcgttaacaaataaataacttataactgcttgtcaccttctttcttcagtcgactgtaataatcttcctgacttggtaggtggccaccatgcatgtgggggtgtccatgcagccactgctgctccatggccagtctctgcagctcggccgactgggcatgcatggcctgcagctggtgggctgctgacatggggggtgggatggccccaggcaggtcacgggggtagggggtgccgaaaactgggtggcgaagcatctcgtgctcgtgtgggggctgtccaagcagagggttggggagagtgccaggcgggtaggggaagcgagccaggtggggaccggcagtcagggggtcgaccagcgggtgaacggggcctgctgaaccttggtggagggggtcctgctggtggaggtggaggtgggagtgaatgtgagagtgctggtgatggtgcggagtcacgttgaacatctgcagtcgggccaggggatcgctggtcagcgatgccatgcgctctgcgtggatacgctcggctgccagtctgtcagggtagctcatctcgggccgcagctgggggcccgccagggccagtctctccctctccaaggggttcaggcccgggtggaaagaagcaaaagggtggggcccggcggtcggggggatggtgagggcgctgtgccgggcaaagtgctccatggggttggcggctgggtgcagggggtccagctctgggggcttcacctcgaagcccggcttcatcctctcccgcagctcccgctctcggatctcccgctctcggatctcccgctcccggagctcccgctcgcggatggtggggtcgacgttgtagaggccaggcatgtggtaggccagcagggggtccgtggggttaaggggcatgtagaaggggtggttgcggttggtgggcgacatgacgtggggccgggcgtactcgctcagagtccgaagggcaggtgtgtcgggcccgatgtaggggggcacagcagcaatggtggttggtggtggctcgaaggatggccgcatgtggccaggaccactgagctgtgggtcactgaggcgaccttcatgcgctgagctggacgccttagccgcccgctctgcctcgcgctcccgctctcgctcccgctcccgctccttctccttctccttctcccgctctcgctcctctcgggctttctgctcagcctcgcgcttggccttctcaatggcctcctccctcttcttggccagcttggacccggccagaggcatgaagtacaggtctgtccgggcacacgagttgtagccccggtccaggtgtttgtagaacctagctgactggctggcgtgactgggggtgtccaccacagtgggctccggggacgggctccttggtgggggaggggggctctcaggctcctcagcgtcgtccagagcctcctccttgatctggacggtggggagtgggcaggacgacccccccgctatgctgcctcctgaagccgccgcaccagagcagggtggctgggccgaggtgccaggtcccgccggtggggtagaggtggaggggcaggtcggaggggtgatgggaggagggcctccagggacaaaggggtgctgagcaaacgggggttggggggccacctggtggaggcctgtaggggggtgggaggcagggggcgggggcaggttctggctctgggtcagcccggggggctgggcgggcgaggagggcaatggctggctctgaggcatgagttgcaggggtggggggtgagccgacggggggtgatgtgtggacagggagctcaggggcttcagggctggagggggaggcaggttggcattcatggagaagggtgagggccccgagaggtggggagggtgcttgtgggcctgtggcgccggcagctgggggatgggagtggtaggcgggggcttgatgtggggcatggccaagggcgctggtggcaggggctgctcccgtggaggctgttgggactgcagcgctgactgagaggctggcagctgcagggaggtgtgagggtacgctgctgctggggaggtccccagaggggcctggccttgggaggcctggggagggaggccaaagggctgtggggggcctgggtgctgcagcaggggcccagcctgcaggctgtgagggccgggtgggccctgaccgtgcagtgggggctgggcatgagagggtgcagaaggctggcccgccgacccagtcagaggctgcagcgggggatgtggcgagggatgcggcgggggatgcggtgagggcggccgctgggggtgcaaggccggtgcctgttggatgtgggtgtggggaacaggcgctgtgggagcctgtggctggttaggggcctgggaggccgtgggggagccctgtgggggaactgcagtggcagagggcgtgggccctggcgtgggcagctgaggggtccctggaggagctgaggagggagctggggtgaccccagtgggagcctgcaaggctgggggctgggcctgcagcatctgctgctgggctgacgagtccgagtcactctcattgtcctgggggctggggatgctcggggacgtgctgcgattgtcctggtcgatgtctttggggtcactgctaccctcatcgttgacgctgcgactgtctgaactctctccctcaccttcagatggcgagttgggcctgctgatctcctgcgtttttgtcttcttggagctggtcctgtcagcctcctccgtatcagaggccaccttctcccgctggcgtttgttactcttaagaggggaagaggcttcctccttcaccttcttggccgacttcttcactgtctctgctttactgtcattgctggaggtactggcagcgctgggggagttccggccgctggagcggatgtcttcattgatgggtgaggtgcgaccatcagggctggctggctgcttcttccgaccactgcgtagtgtcgacatcgagccccgactccgccgtgtcctcatgctatgcttcccactgagcccatcatcctcttccttgacgggtttgaacataaacggtggcgggtccacgggcttctcaatgggcgggagctcaccgtatttcttgaagtggatgcgacagtcggtgcaaagcaggatgttctcccggcctccgtggtgccaatctttggaggtggtggtgaagcagtggcggcaggcgtaccccttcagctcctgctcactgtcctcactgtcgaagtcatcttcactggctgaacttaggtccaagaattcactggacgggggtctggagggtgtgttgacgggtgtggacgcggtgcgagtcttaatcctcctgaacacggcctgcctgcggtgcctacgatgggctcgggagctggctgcttcgggggtcttcttccaatagtaatagaaggtgatcagctcccctgtttccttattgggaagcagctcctttctaattctgaagaagttcttcccgtactgcctgagtcccttaacgaagcgtttcacttcgtcctcggtccagcacttctcgatgagcttgggcacaggcttcttcaccaggcgctgcagggctttgccagcatcgtaaccgctttcatgcagtgtgttcagtgcattcagagtggtgtcatcccgagaggctgcgacacagccgtcctctgtagagcctccatcacacattcctgcaaatgccgccatgctccttgctgccctcaagtacataaggaggtcacagtcgttaactccaggcatccagaccagttcctcatgttgggtcactgtatcaccatctggagaaggaaatggttgcagatctggaagtttggcctgatgactaggaccgacacgaatctccccctgggtactgttcagcctccttgtctcagggttatatcctaatatgtagaaaaatgaatccactcgggctttaaactctctagcagcaaatatgtcagaaaaatgggagatgttacacttccctctaagggcagcagcatggtaagtgtcaacgtaatcagaaatgaagagctctcggttcttgataactgggtctgtaatgacaagttctcttccagagtcattttcattatgtcgatcctgaaccaaatgctgatacacagaatctggaacctcagattgacggtagtaccatttgacgttcatgaggagatggtccctcttactccctacaggccctctcccggcttcagaaagatgctgtggtggctgtgatgccaccggcagagagcatgctggggggtcacacaaagcaggagttggagatctgcaacaggcctgggagttgtggaccagtttgaagtcttgaatgctacagatgaaatacggtgtgtttggcctccgactctcgatatacacacagtctcctggtctgtagaccacatcatcttcagtgatgtaggatgttatctcaccggtatctgtcctttcataacgagacttttttttcggtggtttcttcttattcttcttcgtggactcctctgcggtggcactattgttgtcattgtcctcgtcttcactgtgatcactctcagcataatttttggctcctccttccaaggtacagctccggcgtggccttgaattctcactctctcttgctttgtctcttttctctctctctcggtcccggtctcggtcccggtccttctctttgtctttgtctttgtctttgtccgctgtcatgattcgccacgtgccttcttctgtcctctcacggctaggcctccgtgaaaggtagacagtaagcctgggcttcagtcttctgaatttctcactcaattccagggaaaatccaaccactccaacaaccccaacgtttcaaaaatgcttcccctaaagcgctacaccatcaatagtgaggtgttcgcggcccagctccggggaaagtggcggggatggggcgggaggccgcgcggaggctgcggggccgcggggcgcagggccgagaggggcggcccgcggggaggcgacgcggaggggctgagggggcttccctgccgtgacctttcctgcgacttgaacctaggctccctcctcctcggtcgggcagatctttcagaagcaggagcccaggatcatgtctggttttgttttccgagggcgagggggctccctgaggatgatggtgatttttttttttttttaatcctcaactaggagagaaaatgaggcagagacaatgtggggagcgagagaggggaaaaggacgggggaggaggcggggaccgaggcccagcggggcgagcgtctcggggtgtgcgggaggctgaggaggctccggagcgcggagggttgctcgcgagcgtct

SEQ ID NO: 8726 - RNA, 5771 nt, Homo sapiens
  source 1..5771: mol_type = other RNA
aagcctctgtccccaccccagaaggaaacgaatgccttcaagccaatgtggcctgaagtcccacgacaaaaggttcatgtcagctttgcctccctgtgaacaaactaaagttaaggcagaaatggaatgagagaaaaatgaaagaaaaaaaactagaaacattttcaacagacaaaacaagcctatcccaactgaaaccaaacacggtttttaagagaaactggaaatgtcgctatttgacgccagaacctgaatttgagccagtagctgctggtttctagatcaaactatcagcatctcttcctgctccctctgcggcctgggtcctggatggactttgtgtccgccgacccagtgtggtctctgtcctacaattcttgggatgggaccagcacaatggcagaagagacctccagtgtctgagagaaaaggatcggaagaggccacgtcctggcaggaagcagggccgacagagggcagacaccccagaacacccgccctcagcctgggagaaagtgcgttacggctgcagcctggaaacgagggcaggctctctccaggacggttccgctcagaagggcctggcctcctgagaagcagcccccacacagcatgctttctgaatgcactgtgggtgggactccagttcccacttccaggatgaagagtgggactcaaatggtttaccagtgcaatgtggggtcaccatgcagacctgcccctagggtaaaatacaggctgcccccaacacctgtcttaactccaggatctcccttgctcaaaagtggcctcaatctgtggcaagaaagatggggccgtcctcaccacaagatccaagtgacaatgcgcatgagaaggcagccttctaacacatccctttggcaggcatatgtcctgggtcacttgtgtgctgagttatttgtatggaatcattttcttagatgatgaaattttcggagtattaaaaaagacattcatccagaacaatcaagtgtgtgtacacagaaatctagaaggaaatctacaatggacacaggcccatgcgctttccatcccgtggaaacagaacagtgacactggagaacagaaagtgaacattcacctcctgcactccctgtgcaaaatggaagaggtctgatggagcagatgtctgtgctgctggcagagcacaggctaggagcagacacaagtgaaacgccaggcagaaaacagagtctgtaacatcgtccctgcaaaccctggatgctcgctgctgtgaccaggcctcggtccaagcctctgtccatgtggaacgcccctttgctccctttaattaaagggataattatatataactttttattaaaaaatcaactctgtattctgtcaatagttggtaggaattcacaattagtgacatggctggaaaaaatagatcacaatagtagtttatggaagaaaaaaaggctgttctaaaattatttatttacagacgtaaaaagccatgctgcagaactttctccaattatgaagatttcctacaatgtattaaaataaaagatttttttttttaaaaattatagctcttggattccaaattcctatgcccccgatctgcaagcctcgtgggctctggagcactcgtggcggagtgtgtcagtgtgtctgcacgcacagtgaagggtgtgaactggattctagcacctactgagaaatcaaggaaaagaaaactaaagccaaaccccaagattgcagggaagctttctggatgttcagtccagtccaggactcactaagtttctgggggactgtcatgcagggagatccaaaccagtctcaggaaatcctctcgacaaacgaacactactatgtggatacatttttagttgtgggtttttaaatatataaagaaatctttagaagatattctttttgcttttgcagctcctattttatgtaaaaagtcctgtttctccccccaagaactggggtttccacagccagcgttaacaaataaataacttataactgcttgtcaccttctttcttcagtcgactgtaataatcttcctgacttggtaggtggccaccatgcatgtgggggtgtccatgcagccactgctgctccatggccagtctctgcagctcggccgactgggcatgcatggcctgcagctggtgggctgctgacatggggggtgggatggccccaggcaggtcacgggggtagggggtgccgaaaactgggtggcgaagcatctcgtgctcgtgtgggggctgtccaagcagagggttggggagagtgccaggcgggtaggggaagcgagccaggtggggaccggcagtcagggggtcgaccagcgggtgaacggggcctgctgaaccttggtggagggggtcctgctggtggaggtggaggtgggagtgaatgtgagagtgctggtgatggtgcggagtcacgttgaacatctgcagtcgggccaggggatcgctggtcagcgatgccatgcgctctgcgtggatacgctcggctgccagtctgtcagggtagctcatctcgggccgcagctgggggcccgccagggccagtctctccctctccaaggggttcaggcccgggtggaaagaagcaaaagggtggggcccggcggtcggggggatggtgagggcgctgtgccgggcaaagtgctccatggggttggcggctgggtgcagggggtccagctctgggggcttcacctcgaagcccggcttcatcctctcccgcagctcccgctctcggatctcccgctctcggatctcccgctcccggagctcccgctcgcggatggtggggtcgacgttgtagaggccaggcatgtggtaggccagcagggggtccgtggggttaaggggcatgtagaaggggtggttgcggttggtgggcgacatgacgtggggccgggcgtactcgctcagagtccgaagggcaggtgtgtcgggcccgatgtaggggggcacagcagcaatggtggttggtggtggctcgaaggatggccgcatgtggccaggaccactgagctgtgggtcactgaggcgaccttcatgcgctgagctggacgccttagccgcccgctctgcctcgcgctcccgctctcgctcccgctcccgctccttctccttctccttctcccgctctcgctcctctcgggctttctgctcagcctcgcgcttggccttctcaatggcctcctccctcttcttggccagcttggacccggccagaggcatgaagtacaggtctgtccgggcacacgagttgtagccccggtccaggtgtttgtagaacctagctgactggctggcgtgactgggggtgtccaccacagtgggctccggggacgggctccttggtgggggaggggggctctcaggctcctcagcgtcgtccagagcctcctccttgatctggacggtggggagtgggcaggacgacccccccgctatgctgcctcctgaagccgccgcaccagagcagggtggctgggccgaggtgccaggtcccgccggtggggtagaggtggaggggcaggtcggaggggtgatgggaggagggcctccagggacaaaggggtgctgagcaaacgggggttggggggccacctggtggaggcctgtaggggggtgggaggcagggggcgggggcaggttctggctctgggtcagcccggggggctgggcgggcgaggagggcaatggctggctctgaggcatgagttgcaggggtggggggtgagccgacggggggtgatgtgtggacagggagctcaggggcttcagggctggagggggaggcaggttggcattcatggagaagggtgagggccccgagaggtggggagggtgcttgtgggcctgtggcgccggcagctgggggatgggagtggtaggcgggggcttgatgtggggcatggccaagggcgctggtggcaggggctgctcccgtggaggctgttgggactgcagcgctgactgagaggctggcagctgcagggaggtgtgagggtacgctgctgctggggaggtccccagaggggcctggccttgggaggcctggggagggaggccaaagggctgtggggggcctgggtgctgcagcaggggcccagcctgcaggctgtgagggccgggtgggccctgaccgtgcagtgggggctgggcatgagagggtgcagaaggctggcccgccgacccagtcagaggctgcagcgggggatgtggcgagggatgcggcgggggatgcggtgagggcggccgctgggggtgcaaggccggtgcctgttggatgtgggtgtggggaacaggcgctgtgggagcctgtggctggttaggggcctgggaggccgtgggggagccctgtgggggaactgcagtggcagagggcgtgggccctggcgtgggcagctgaggggtccctggaggagctgaggagggagctggggtgaccccagtgggagcctgcaaggctgggggctgggcctgcagcatctgctgctgggctgacgagtccgagtcactctcattgtcctgggggctggggatgctcggggacgtgctgcgattgtcctggtcgatgtctttggggtcactgctaccctcatcgttgacgctgcgactgtctgaactctctccctcaccttcagatggcgagttgggcctgctgatctcctgcgtttttgtcttcttggagctggtcctgtcagcctcctccgtatcagaggccaccttctcccgctggcgtttgttactcttaagaggggaagaggcttcctccttcaccttcttggccgacttcttcactgtctctgctttactgtcattgctggaggtactggcagcgctgggggagttccggccgctggagcggatgtcttcattgatgggtgaggtgcgaccatcagggctggctggctgcttcttccgaccactgcgtagtgtcgacatcgagccccgactccgccgtgtcctcatgctatgcttcccactgagcccatcatcctcttccttgacgggtttgaacataaacggtggcgggtccacgggcttctcaatgggcgggagctcaccgtatttcttgaagtggatgcgacagtcggtgcaaagcaggatgttctcccggcctccgtggtgccaatctttggaggtggtggtgaagcagtggcggcaggcgtaccccttcagctcctgctcactgtcctcactgtcgaagtcatcttcactggctgaacttaggtccaagaattcactggacgggggtctggagggtgtgttgacgggtgtggacgcggtgcgagtcttaatcctcctgaacacggcctgcctgcggtgcctacgatgggctcgggagctggctgcttcgggggtcttcttccaatagtaatagaaggtgatcagctcccctgtttccttattgggaagcagctcctttctaattctgaagaagttcttcccgtactgcctgagtcccttaacgaagcgtttctcggggctcccagcctggtcccgggcggccgaccccagcagccacaggtaagcgcccggggtccggggcggcaagaggccgtcgcctgtcactgggctccggctccacaaagcgcagggcggaggcggccgcgggtggctcggcgtgtgaccgcggcggggccgcgcggcgcggggcccggggggcgcggggctggggccgccgctgacgggggaggaggcaggagcgcggcgcgcagagcccggcgcggccgcgggcggctgcaaaaggc

SEQ ID NO: 8727 - RNA, 2294 nt, Homo sapiens
  source 1..2294: mol_type = other RNA
aagcctctgtccccaccccagtgcccccctccccccagcctcgttaaaaatcgctgcgtaaagtcaggttaactgcggcgggtcccccctcccccctcccacctaagatgcaaactaaaagcccccgtccctcccctgcccccctccccccaccccgggggccattctggttccgtgtacagcactgtgctacctcgcccctctttccctaataagggggggtgggcgagttcctggtgacctcctctccccccaaaatctgtccaacggggcggacgggcccttgaaagaggccagagttggggttctgaggggggaagagggacgtcaatgaggaggagagccagaaaatggaagacttagaggtttggggggggtgtcgacccccgctactgcccctccctccctcgacggggcctcgaggggggagaggcgggcacaggtgcggagatggcgtgggggaattccctccaccctagggtccccattctggccgtctggtgtgcgcctagggcgggatgcacccaagggcttgggacgaacgggtgaagggaggaaaggagagaaagagttaaaggaggaggaagacgaaaaagaagccaaggatagctgagaaagcaagaagatcctttagacaagagccccctaaaaggcaggtaaccttcaggaagcagaaaagagcccagccggtgagaaagaatgggaccttccagggaagtaggggagatggggagggaagggccaggttaaccgtacccgtggcttccagcccccttccctacgccaccccggggctgcgggtggagcaagccggccctcccactgcaccggaggacccagcaggtcaggaggtgagattaggcagggaaaaaggaagcccaggttagaagggagaagaggatggtcggtattcccgacggctgcccgaacctgctctccagcccagcgcccctgcggtgaggtccgaggttggggagctctggggagctgggcgcttgcaccgcctctggctgctcccagctcagagcaggtggagaacgagggaggagctaattttcttggagaggaggggccagaggaaaggggcgggccaacgaaggggaggagtcatttgggagtgagagggaccaatgaaaaggagaggtcgggaaaagagggcgcggccattgaaataagggagtctgtgggcggagccattgggaggagggcggggcctaaagctggcgcagcctcctccgggtgggagcgaggagtcccgaggacggaagggggcgctgcattgcagggagacccccctaagacgaggaggaggaggaggcagggggagctccgaggggcgggcctcagcagggcgaggtggagatgtgcaggtggtccgggtacttgatggcgggagggtagttctgcgtcatttggatggacacgtcgctggagatgtcggaggggctccggccgcggcgccacgcctcgggctgcaggaactggcccgagtagtcggagcagtcgctgagacgcgggcggtagaaggccgggtgtggacggtacatctcctcctccgcgtagcgcttggtgaacaggtacacggacatcacgccggccccccgatagtatgaagaagatgccagagacaaaagccagaatggtcctctgcgggcggatgtggccgatgttgctgatgacgaaggccgtgaacacgaggaagaggctgaccatggggaagggggtggccgtgcgcactgtcttcagaatattctccgtgttttccgtcaccaaattgatctccggttcaagaaaatattctgaggccacacagcgacctttctcccgacctgcaaagaagcagactcgccagaggccggcgtgcagggccatcttgacctcggtggtctggttctgcggtagcactgtgccttcttccatgtacagccagtagtcagtgctgaccgcgatgcctaccaggagcaggccacacgcaccaaacacgctgctcagcagggtcagggcgcggctgctgcagtgactcatcctcagaggcagggggcgccctgcggggcctcgctcagggctgggcggacgctccgggccgcgggccccgcagccgcatgaccggccccgaggcttcccccggccgccgccgccgccaccggggtcgccggtgcccgcgccccccgcccccgccccggagcccggcgtcccggccccctcccggcctcccaccccccaccccccgcggccgcggcctcactcggcggacggagccgggagcaggaaccggcggccgctcattggctact

SEQ ID NO: 8728 - RNA, 2440 nt, Homo sapiens
  source 1..2440: mol_type = other RNA
aagcctctgtccccaccccagtgcccccctccccccagcctcgttaaaaatcgctgcgtaaagtcaggttaactgcggcgggtcccccctcccccctcccacctaagatgcaaactaaaagcccccgtccctcccctgcccccctccccccaccccgggggccattctggttccgtgtacagcactgtgctacctcgcccctctttccctaataagggggggtgggcgagttcctggtgacctcctctccccccaaaatctgtccaacggggcggacgggcccttgaaagaggccagagttggggttctgaggggggaagagggacgtcaatgaggaggagagccagaaaatggaagacttagaggtttggggggggtgtcgacccccgctactgcccctccctccctcgacggggcctcgaggggggagaggcgggcacaggtgcggagatggcgtgggggaattccctccaccctagggtccccattctggccgtctggtgtgcgcctagggcgggatgcacccaagggcttgggacgaacgggtgaagggaggaaaggagagaaagagttaaaggaggaggaagacgaaaaagaagccaaggatagctgagaaagcaagaagatcctttagacaagagccccctaaaaggcaggtaaccttcaggaagcagaaaagagcccagccggtgagaaagaatgggaccttccagggaagtaggggagatggggagggaagggccaggttaaccgtacccgtggcttccagcccccttccctacgccaccccggggctgcgggtggagcaagccggccctcccactgcaccggaggacccagcaggtcaggaggtgagattaggcagggaaaaaggaagcccaggttagaagggagaagaggatggtcggtattcccgacggctgcccgaacctgctctccagcccagcgcccctgcggtgaggtccgaggttggggagctctggggagctgggcgcttgcaccgcctctggctgctcccagctcagagcaggtggagaacgagggaggagctaattttcttggagaggaggggccagaggaaaggggcgggccaacgaaggggaggagtcatttgggagtgagagggaccaatgaaaaggagaggtcgggaaaagagggcgcggccattgaaataagggagtctgtgggcggagccattgggaggagggcggggcctaaagctggcgcagcctcctccgggtgggagcgaggagtcccgaggacggaagggggcgctgcattgcagggagacccccctaagacgaggaggaggaggaggcagggggagctccgaggggcgggcctcagcagggcgaggtggagatgtgcaggtggtccgggtacttgatggcgggagggtagttctgcgtcatttggatggacacgtcgctggagatgtcggaggggctccggccgcggcgccacgcctcgggctgcaggaactggcccgagtagtcggagcagtcgctgagacgcgggcggtagaaggccgggtgtggacggtacatctcctcctccgcgtagcgcttggtgaacaggtacacggacatcacgccggccccctctttgagtaggaaggaggaagcggcgaaggcaaaagaccacccgtagcgataatgaaaatactgctcagagctgctgggcctgttcatgacctcgtcgttgatgctggagatgtaaagaaccaagcccaccaccaaggagaggcccgatagtatgaagaagatgccagagacaaaagccagaatggtcctctgcgggcggatgtggccgatgttgctgatgacgaaggccgtgaacacgaggaagaggctgaccatggggaagggggtggccgtgcgcactgtcttcagaatattctccgtgttttccgtcaccaaattgatctccggttcaagaaaatattctgaggccacacagcgacctttctcccgacctgcaaagaagcagactcgccagaggccggcgtgcagggccatcttgacctcggtggtctggttctgcggtagcactgtgccttcttccatgtacagccagtagtcagtgctgaccgcgatgcctaccaggagcaggccacacgcaccaaacacgctgctcagcagggtcagggcgcggctgctgcagtgactcatcctcagaggcagggggcgccctgcggggcctcgctcagggctgggcggacgctccgggccgcgggccccgcagccgcatgaccggccccgaggcttcccccggccgccgccgccgccaccggggtcgccggtgcccgcgccccccgcccccgccccggagcccggcgtcccggccccctcccggcctcccaccccccaccccccgcggccgcggcctcactcggcggacggagccgggagcaggaaccggcggccgctcattggctact

SEQ ID NO: 8729 - RNA, 35 nt, Homo sapiens
  source 1..35: mol_type = other RNA
aagcctgcccggctcctcgggcggactcggagtgc

SEQ ID NO: 8730 - RNA, 4633 nt, Homo sapiens
  source 1..4633: mol_type = other RNA
aagcctgcccggctcctcggggttcgcgggggctccgtccccgccggcttcctgcctcgccgccttccggggtttctgtggctcatcctctctgggaccctgggtcagctccacttccttcctcttctcgcctcggccccgccggcctctgaagccggggccccgcggcggaggctgctcgtcctcctcggactccgaggcgaagtcgtactcgcggagcctgcggtcctcagctccgggccggggcctccccgccgccagggagccgcacctgcccgcccgccgccccagccgccggtggcgcctgttcttctgctgcacgatcttcagaatgagctccttgccccaggcgccgccccgagccttcctcttcctggggtccttcctggggggcagccggcggcgccgggagctgcgggtctcctcggggagggcggcggctctcgggacccggggcgcggggtctgcgcggctcccgggggcctgcgttctagggcgccggggacggggtgggggccgctccccgagaccgtcgttcctccggggcctcaggccggaggctctgccgccgccgcccgaccccgacccctctgctgcgccgcccgagtccagatccttccggaacagcttcaactgcttccccctcctctgctgcctgccctggctgggcgcatccgcctcggtgggggccagacccagggaacgcgttttgggcctgcctcgggctgggcagcccctgtccccagggcggggggtttgggggtccggcgtggctgctgggagcgggggcggagctttgctctctggagtcacccccgccttgctcttaagggggtgtccggagctgggacctctggggccggaaggctcctcgtccgcgaagacgtcgatgaagctgctgtcgatctccgggttgtccgactggtactccatgccgttgagcgcctctgtgatgaggctgtccagcttggcgtcatcctccatgtccaggtccgaggcagggagcgggaagggggtggcggccaggctgggcaggaagcctgtcctcagggggtcgtctttgccctcggcctgggcgtccccagctaacaggaaggtcttcgcgtggctgagcaagcccgcgtgtgcgtcggcagggactctgggggcagcggggggcgaggggagcccaggggggcctggagaccgctggtggccatccttggccctggccaggagcaggccacagaactgccggtgggccaggaaggccgccaggctgctgtagttgcggtcacactgcctgcaggtcagcagcacgtccagctggtccaggctggcgctgctgagggagaagtggtgtgtggggtacggaggcggcgcacgggggaagccctgcagccctccccgacccacctcggggccctcgtgggggaatggggtctcctccaggcactggaaggcaccctcggctcccagcccatctgcgggaaaagggaaggccttggctggctctggctggtagtgggtggggagggagtgggggggctccggggacgggaaggggctgcccgtctcctgggggtgagtgggtgggtggaagaaggccgagggcccgagggggccggggagctggctttcctctgagctggggttggctgggctgctggacatcggcgacagggaagagcaggtgctgccggccgtgttggtggccggtgacggcagtggggactcgctgggggaggctcccactaccctcggtgggggcaggctgggtgtcccgtggggtgaaacctggggctgggccaccccgaagaacaggggctgagccccagggtctgtcattccgttgtaggtgaacagtgctggggagccgccctggctgcttctcacggctggcagcttctctctgggtcccggtgtcttgccagcagtgcccagggctccttggctgcccccctgccactcggggccccccgcggggaaaggcagccggctcagcatctccattccgtggggacttggccgggcggtcgggagcacttggggccaaggcaggggggcactctgggggaggcagagccgctggcctgggctgggctggccgttaaagaacatactcctggtggcagccagggggcccccaggaggtgtggggtaaggggctgctgtggggtcccacagctggggcagcctggcgggtgggggccctggggcggccagctcggtgtccggaggccccgggctggtgtccaccccactggctctgtacgcctgccctggaaagtgcctctggggtagggagctagggggccctctcgtgctccccagcccatcctgggctgaaggtggtctttcgggaaggattttggtcaggctcttgtgtaaactgtcagagaagggtctcggggccgagtgagcagctccaggggaagagagggcaccactgaggtcgctgtggcggttcaggccacctggctggccctggtagcagggcaggggtgagggcgcaggctgggtgggcagcgggtaggcagggcccgtgcccacggcctcctccggccacgctccctggggctgatggaaggcaaacaccagtggcccattggtgaatgcgtgcccagccacatccgcagggaagggttttgtgctggccccatgcagtgccgggaaggggaactggaaggaaactcccctggggctgccgccgggcctgctgcctttgggaataggttccggctcggcggggggaaccccgaaattagcacctgggaagctattctcagcagcgggaggccaggagtcggccccactggcctggtattcgggataggaaccgggctggagggggctggtgcccctgctctgggggggccccggggctgggggcctgggggtggcgcttggtgaggtatagttggtggaggtaaagctggagggtggctcctggaagcacctgtggaagccaagctcttcggcggcgggttgggcctcagtccttgggaggcccggcctgagtggagctccagtcccagggccctggggggtgtccacctcagggagctgggcagcctccagctgtgggttctctggtgtctcgtccagggtgggcttggtcctcgagctggcgatgcccagaatgtagcgctgtggggggctgccctctgccctgcccgccagccttgagggagcctgcaaggggcttctccccggtggggtctgggggctgcccctcttcccaggggtgctgctcggggcctggcctctcagggatgggggcttgagctccccgtccctggcctgccttggctgggcctcggggagctccatggcctgggcctggccgccagcctccctggcacccttggtggtcctggtagctggggtgttgtcctccagtggcggctgggaggggtgccccgggctgctggcaacttggcggggctgcaggtctccagtcatggtggggggcggcgctcctcgggggcgctccccaggcatggcccctccgtcctggcgctaggacgacgcagctgtccgaggggggccctggggagtgggctggacggccatcctcagccctcgatgggccccagggaagcctgcgctcatggtcctgagtggagcctggaaggaaaggtcaggggtgagtggggcagaggggctgggtggccctcgcctagacagggagcttctaggctctccatgcgggtgtggccgggccagaagcagaagaggctgcgtgcagccatcacagaagctccgcgcttagaagggatgctcggctcagcccctacctagaagcaggaagggagagggcatcccgccagatggaacagggacccttccctgtcttagggagaagaggggcggtggagcgcagagattgagtggagggggagggagggggagctttctggggtgtgaggaggccgcttacaggctcagagcagtcctcggccaggctgtggagaggacaggcacctgtgtggggcacaagctctcagcctgcaggaactgccccagggcagggtcctggcagcgtccaggagggcccaggtggatgcttacacctgccatggggagggccttgaggcaggaggctgcgttgcaggacataggggactgaggcagcagaggctcaacctgaacctctcagggcctgggcggctggttccaagcggggactcccctgccgtcagccagggtctccctgccaccaggccttacagggtaacctccagatcctgccgtcagccagggtctccctgccaccaggccttacagggtaacctccagatcctgctccaggaagcccccagcctccagacggtgccggctcccattctggcacatgccagatgtagcaggagccgcttgcccagaggagcctggccccttgctcacccagggctggcttcacactcatcatgtctgttctcatgtcatgacatacgggactgtcctctgtgcggacaggactcagacccgagccattggctgtggccacgaggtgcgcaggccgctccgtgtgggggccccttctgacttgcccagcagggaccgggcgtcctttacacagcagagtgaggcagggctcagcccttgcaggcattgtccttgccactgacccctgggtcctcatggcagg

SEQ ID NO: 8731 - RNA, 3970 nt, Homo sapiens
  source 1..3970: mol_type = other RNA
aagcctgcccggctcctcggggttcgcgggggctccgtccccgccggcttcctgcctcgccgccttccggggtttctgtggctcatcctctctgggaccctgggtcagctccacttccttcctcttctcgcctcggccccgccggcctctgaagccggggccccgcggcggaggctgctcgtcctcctcggactccgaggcgaagtcgtactcgcggagcctgcggtcctcagctccgggccggggcctccccgccgccagggagccgcacctgcccgcccgccgccccagccgccggtggcgcctgttcttctgctgcacgatcttcagaatgagctccttgccccaggcgccgccccgagccttcctcttcctggggtccttcctggggggcagccggcggcgccgggagctgcgggtctcctcggggagggcggcggctctcgggacccggggcgcggggtctgcgcggctcccgggggcctgcgttctagggcgccggggacggggtgggggccgctccccgagaccgtcgttcctccggggcctcaggccggaggctctgccgccgccgcccgaccccgacccctctgctgcgccgcccgagtccagatccttccggaacagcttcaactgcttccccctcctctgctgcctgccctggctgggcgcatccgcctcggtgggggccagacccagggaacgcgttttgggcctgcctcgggctgggcagcccctgtccccagggcggggggtttgggggtccggcgtggctgctgggagcgggggcggagctttgctctctggagtcacccccgccttgctcttaagggggtgtccggagctgggacctctggggccggaaggctcctcgtccgcgaagacgtcgatgaagctgctgtcgatctccgggttgtccgactggtactccatgccgttgagcgcctctgtgatgaggctgtccagcttggcgtcatcctccatgtccaggtccgaggcagggagcgggaagggggtggcggccaggctgggcaggaagcctgtcctcagggggtcgtctttgccctcggcctgggcgtccccagctaacaggaaggtcttcgcgtggctgagcaagcccgcgtgtgcgtcggcagggactctgggggcagcggggggcgaggggagcccaggggggcctggagaccgctggtggccatccttggccctggccaggagcaggccacagaactgccggtgggccaggaaggccgccaggctgctgtagttgcggtcacactgcctgcaggtcagcagcacgtccagctggtccaggctggcgctgctgagggagaagtggtgtgtggggtacggaggcggcgcacgggggaagccctgcagccctccccgacccacctcggggccctcgtgggggaatggggtctcctccaggcactggaaggcaccctcggctcccagcccatctgcgggaaaagggaaggccttggctggctctggctggtagtgggtggggagggagtgggggggctccggggacgggaaggggctgcccgtctcctgggggtgagtgggtgggtggaagaaggccgagggcccgagggggccggggagctggctttcctctgagctggggttggctgggctgctggacatcggcgacagggaagagcaggtgctgccggccgtgttggtggccggtgacggcagtggggactcgctgggggaggctcccactaccctcggtgggggcaggctgggtgtcccgtggggtgaaacctggggctgggccaccccgaagaacaggggctgagccccagggtctgtcattccgttgtaggtgaacagtgctggggagccgccctggctgcttctcacggctggcagcttctctctgggtcccggtgtcttgccagcagtgcccagggctccttggctgcccccctgccactcggggccccccgcggggaaaggcagccggctcagcatctccattccgtggggacttggccgggcggtcgggagcacttggggccaaggcaggggggcactctgggggaggcagagccgctggcctgggctgggctggccgttaaagaacatactcctggtggcagccagggggcccccaggaggtgtggggtaaggggctgctgtggggtcccacagctggggcagcctggcgggtgggggccctggggcggccagctcggtgtccggaggccccgggctggtgtccaccccactggctctgtacgcctgccctggaaagtgcctctggggtagggagctagggggccctctcgtgctccccagcccatcctgggctgaaggtggtctttcgggaaggattttggtcaggctcttgtgtaaactgtcagagaagggtctcggggccgagtgagcagctccaggggaagagagggcaccactgaggtcgctgtggcggttcaggccacctggctggccctggtagcagggcaggggtgagggcgcaggctgggtgggcagcgggtaggcagggcccgtgcccacggcctcctccggccacgctccctggggctgatggaaggcaaacaccagtggcccattggtgaatgcgtgcccagccacatccgcagggaagggttttgtgctggccccatgcagtgccgggaaggggaactggaaggaaactcccctggggctgccgccgggcctgctgcctttgggaataggttccggctcggcggggggaaccccgaaattagcacctgggaagctattctcagcagcgggaggccaggagtcggccccactggcctggtattcgggataggaaccgggctggagggggctggtgcccctgctctgggggggccccggggctgggggcctgggggtggcgcttggtgaggtatagttggtggaggtaaagctggagggtggctcctggaagcacctgtggaagccaagctcttcggcggcgggttgggcctcagtccttgggaggcccggcctgagtggagctccagtcccagggccctggggggtgtccacctcagggagctgggcagcctccagctgtgggttctctggtgtctcgtccagggtgggcttggtcctcgagctggcgatgcccagaatgtagcgctgtggggggctgccctctgccctgcccgccagccttgagggagcctgcaaggggcttctccccggtggggtctgggggctgcccctcttcccaggggtgctgctcggggcctggcctctcagggatgggggcttgagctccccgtccctggcctgccttggctgggcctcggggagctccatggcctgggcctggccgccagcctccctggcacccttggtggtcctggtagctggggtgttgtcctccagtggcggctgggaggggtgccccgggctgctggcaacttggcggggctgcaggtctccagtcatggtggggggcggcgctcctcgggggcgctccccaggcatggcccctccgtcctggcgctaggacgacgcagctgtccgaggggggccctggggagtgggctggacggccatcctcagccctcgatgggccccagggaagcctgcgctcatggtcctgagtggagcctggggagtcgggggcccctcagctgggtcgccgcacaacttcctgaggaatgagaatttcttggctccgctccgaggcccgctccgcccgccacgccggccgccgccaacgagctcccggcccgcgccgccccagcgctctgcagcggaggcgccgtcctcatcccgaccgcaggcccgcccgggccgcccgcccgccgggcaccgagccgctctgccgcgcgctgcgcctcggggcggggtgggaggagagggagcagccgccaccctgcccaggtcgccgcgggccagccctgcagccagctccagccctgggccgggtgctgggaaggccggacgccggccggcggccgcggggtct

SEQ ID NO: 8732 - RNA, 68 nt, Homo sapiens
  source 1..68: mol_type = other RNA
aagcgaccatgatgtaacttcagacttttggagagtctgtgaagttacatcatggtcgcttcctagag

SEQ ID NO: 8733 - RNA, 9674 nt, Homo sapiens
  source 1..9674: mol_type = other RNA
aagctcaggtttgagaactgctgacctagaatagtggttctcaaggctggctgcacattagaaacatctggagaatttgtgaaatcctaatattcaggtcacatctcagaccacctgactcagaatgtcaaggggtggggtcgcacgagtatttcttaaagctcttcagacgactctagcgtgcaccaaggcatagactgcctgccttagggtaatgactcccaaccatgtgagacagaaccacttaatgagatctttcaaaatagggataccaggccctatccccaggcctgctgaatcagatcctccgggaagtaaaggacctggcttggggattattttataaagacttccaggtgattcctatgtacacacaaggttgcaaatggcaattctagagaaaacagaacttttaccccaaagctgagcagatcatttagttgaaggaaatgagagatttgttgccatgggaaccatcttcaactgaagagagagtcactgatttctggcttttgtggccaacagctaagtcatggaagtgtatgtttttgcttttggtttttttcctttgaaataaaaaaaaaaaaaaagaaaggttctcagaagagactgtgcaggggaaaatacctaaagacttctaaaagatcagcaaggctattgtctctcaggacatgctggccaggacagtggagcccaggtggcagagcaaggccaggtctgcactctccctcagcaaggggccaaggtctcaggaagccaggggccaacgaccagcccaggacaactgcccaaggcaaaaacaaaaacaaaaatcagatttctgctttagggacacccaaaacagttaatgtcatttgagagctgcttgcacctaagtgattctaaaaagtctctggtatactatactaagtgaaataagccagtcatcagaaagacaaatattatatgattctacttatatgagggacctagagcagtaaaattcatagagaaagaaagtagaattgcgattgccaggggctggggaagggggaagtgaagacttgtcatttaatgggtttaaagttttcattttgcaagatgagaagagttccagagacagaatatacaacagtgtgaatgtacttaccattactgaactgtacacttaaaaatggttaagatgataaattctatgttatgtgtattttaccataattacaaatgaaaaagaaatctttgtttgtgttaaagcaaaaccaattttgtaaatgttagattcccgagcacttgacttttgttgctaggtacatagtgggttatatattatatttgtatgtacagaaaaggcagaagttgggttgtgtgccaaattcttcttttcattcttttcctactcaaggctccagtctgaatttcaagccatacatggccactcaactggtggcaacttctgaaccacaagcagttgtatgctcagggaacagatagggcctcacacatgctgattcccaggcgccacctctcccccaggttctcagtccatagttttaacaagcacccaggtgattctgatgcaggccatcagaaggccatcctacagggcatcctaataaacccatgtgatcttcaaagggtagactgtagatctatactgtagatctatactgtaggtctatccagtctaccctttgaagatcacactgtagatctatccagtctaccctttgaagatcacactggtttattaggatgccccgtaggatggaatcagcctccacagactggcctcgtttgactagacctctaaacaatagcacaaggcacaccctggccactggtgcacccctcgcctggcctcacctgacccctgagccacagttagcctcttcccagagggtgctctggttacagggaggagactaggtcagggcgtgtgttgagctcagagaagcagcaccttttttcccccaggaaacaaccccatgctcctggtcttccccttcgcatctggagcagacatcctgcaaagctcagctcacctgtttcccagccaaagcattcagcatgttcctctagttttttaaacaccattgataaatccctcttacattgcttcccaggctgcacctcagccacagtgatgtaagagcctgacatgtttgtgtggctttgaggaagggaagaagtagacaacaagaaacacagaaaatgtctctcccttctttcatttaaactagaggaaaaaggattggctagccagcaaaaagcagatgagcaggattataatgagggaaaacaaaaagaggctagccaagcccataagcccccactagacagacatttcagcctcctgagccccgagctcccctggacaggcaggaggagtctctgccttcctgggatgtgctaggtaaaaaaatcaatagaggactctcctcagctgacaatttccccaaggtgttactcagtttattagcggggtatcctgaactgctggagtcccccaggaaccagagacctcattactgtagtaaacatgtgttgagtggccatggcatgtgcttccccgccagtgctggcaatacaaaatgagcttagatatcgtgtcttcccttggggagaaggcaaaccttctatcaaggacacacgggcccttatgctgtgtgctgtgaggatgtcctaatggagtcggtgatggttgcagcagaagcacagaggagagagtgcccagcccaggtctctagaggggaggatgcagggggccattacctgacttctgcaaaagtggccagataaaaggaaggagagaggaacttaggagtgtgagggccattccaggtgtttgaacagagtgtgcaaaggtgcctggaatagtatgggatagggcagggaggtggcaggaggatctctgggaaggtgagtaagccagcttgggacattccctgcatgacttggtaaagaacctgaagtttatgatacaggtaggcaatgggccccacaaaaggtatttttggaaggttattctctgaaagcaaaaagatccatcagatggtctgggttagggcagtagcagaggggttgcagggagggaatgacttaaagggatgtttatgagttggaattgacaagatacagtgaacaaatagacataaagagtgaaggagaaggaagaggcaaaggtgatccaagttttgggccaaggcaacctgtgcttgctagtgtctagtttgtgctgggcactgtgctaggcattgtgcaacactatttcacttagctttgcaacagctgttgtggttggtatcctgtcctcatttcagatgatgagtccagagcctccaggggcttctggagctccctcaatttcacacagctacgaagtagtaggaggagactctgagttcagattgttcttttaactataccagttgaggacatgttgaggtctgagatgctgtgcagacacagacatgcaggaggccacagtgagcatgcttccaatgctcctagggaggactggcctgcaggtagaggggttaagatgccagggcagaagatacttaaggctttgaatagatgagatttctgcaggaatgctcctaggaagagaagagaaccctgaggaagcttcacggaagatgaatccacaaaggaacctgagaaggagcattcagagagacaggaggaaagtcagggaagaatagttagaaaacagaagaggagaggactttagaaagaccagagagactgtgcatagtggctcacacctgtaatcccagcactttgggaggccaaggcaggaggattgcttgagctcaggagttcgagactagcctcgtcaacatagcaaaaccccgtttctacaaaaaaaaaaaaattttcaaattagctgggagcaatggcacgtgcctgtggtcctagctacttgggaagctgaggtgggaggatcacttgaacccaggtgtcgaggctgcagtgagccatatttatatcaccaccctctagcctgggtgacagagggagactctgtctcaaacaaacaaacaaaaaagaccagagaggccaaccttgtcaaatgttacacggatgtcaaggatgatatctgagaagtatctgctgctttgctcattacactttttatgctgccaaccttcagaattcggaattgactttggtcatcccctcctccacctctcccagataactgtccctgagactggatttgatagtgttcagcacaaccagctcccacgtacgtttgtgggattcgtcatttaacgtctgtatacacacacaccagaccacaaactcccggagggcagggacgacgttttgttcatcactagctccccggcacctggcaccatgcctggcacaacatgagcactcaataaatataatttattcaccaattcactcactaaattggccagcactctactctgcctcagttgtttctaagcactgctctgcttcctccctgctctcagcaaagtcaagggcgatgagcacatgctgtctctgggcaccaggtgattagtgggcagagctgccgcagcagcattgctgaaatggtctcagacgctgcctctgaccttgagccacctttctttgtgcttggctaagcactgagtcatttacttgtttttgctgcctttcaagcctggagcagtgggtttagcacaaaggaagacatgatggttgttttgtttacgggaatcgatttcccttgaataataattcaatgggtagtctgcactgcatggtggcgtggtgacagggctgtggaggaacatggcagaaggcttccagagtcaacaccaggtctctctgagcctttgaaaaaatgtttttcttataaacactggctgcagcagaaaaactatatcctgaaagtcaggagactggtgagtcccagttgagccacaagctggccatgtagccctgggcaagtcattcgtgttgtcacttaacatgtgctatctctgggcatctttcctcaccttaaaaatgtgacgatggcctcagttcccctccagtgccactgtgggtaagtcgctactgctgtaggcggcagggttagggagaggcacctataagcacaggctgcttcccggacgatgacagcctcctagagcatttgtccctggaggagggccccgtactatcctgcaggggcatcttggtcaggatccctcatgttctggtgtcactgtctgggaagctaagacagaggtttggagcacagactttggggctctacagatctgggtgcagttccctccattgggtgccgttccctccattgggtgcctgaccaagggcaagtcctggaattgctttaagcctctgtctcctcatctgtacaatgggagcctccttacccaaaggggtctcatgatgattacaggagataatatagggaaagtgcttaacgtagcttgataaatgctagctagtataatgagaaatattaattatggtttagatccattcatcatgaatgtccccccaaaataaggacattgtacagacgctgaagatttttacaaagcttctagttgtagagatgaggaaactgagacattgagggagaggaaggactggccctaagacccacaggcaggaatatggccagcagccaggtgtcccaactcctctgtgggctggatcccgatgctccaatcctcagctcctacgagggccctggctggggcagattccaacctgcaacaccctcagctgtgggaatcctgatgtctgtgtcaccagggagcctcccccaaacactgcccatctggaacataactagtacccagagggcttccagtagagggctctgtccacagcaggcactcagtagagccccaggcatgacttgacccagtcacatctttgctctgggcctgtttcctaaagtggaacaaaatggtctttaagaaccttctagtttttatattccatggtttcaagaactgggttcaattaaccatgcagtggctagaaatctcaggtaactggaatctttcccagaaattccctccctgggagaaataggcagagctcaagcaagtaataaccatccactgtcctttgcagttcttcctggtttagcaggtgtttgggatcatttcatccccttggctactcccctacattcctgaccagcagactgagactcagagccacctgaggttttcccaaccaggaccagagctcagaatgcaggtgagagtcagcactgagaacagtgttgtgcacagggcacaggttccacaacaacccccccacaggaagcccaagccaagacacaaaagtttggccaagaacggagccctggatcaggagcctggaggcctgggataaagcctgcactctccacgtccctgactggctcagccggggggcctgtcaaatgaggtgattggatagcagatcccactccctgatagactcttacagctcctaaccctcccagagcacccagcacgtgggactgggtctataatctctgggccctgcacccccagaagacacagataatgcctttgtttatccttatgtcttcctaagtccaaccacagaccaaagcagaataggctttccagaaatgtttaaggggaggaagaaaagaggaagggagggaaggagaaaggggaggaggcagggagaaaggaaggagggagggagacaggttgccaggcaggtaggctgaagtcctcctcccagcactaacatcctatgattccacaaagctaagttctaaggcagttagttcaccaacagtgtctcttagacaccatcccatttatggtggaaacaccacagggagaagcaaagggaattaatttcagatgtgaaatgatatgtgaacccctctctgcctaagcccagctgactgccccaagcccaggccctggggtctgctgtgagaagtcccgccttcacagcggaagcctcagtgatgctggtgtcggaggccacaactcgtttctctctgctaagctcaccacctgacatgtcagtgctttccagcccagagcctatggttccgactgaggaacacgatacagcaggattctgcaggattcagagacatgagaggaagaggtctttataaataactcctggtttaaatggagctgaaaataggaagacaaaagaggaagccaattgctaagcacttattgagtcaataacattggcttggaagccatagtgcaagtggctggtttggtttatttccttctcatcaaaagagctaacgcaggattgaacctgggggcaccaagaccgcatgtgtgtccgaggatgtgtctgaaaggatgtggtgcttctcagatgatgatgtctcgactaagacataacccaggccttgggttagatctctcggtgtcacagaagaacctgtcgggtggtgtggcttggctgttaagtccctggacctcttgagatcactttcttcactggaaggtctagtcactgggttggcttctaagctctgagatttagatagcaattcatagctaagtcttcgatataaaacacaggaaccaaaagtgtgaataaaatcttgactgtgctcaagtgtcctgtgaagtgtcctgtctccactctcaattccattctctgtagggtcttccttcagctgcaacaagggcctgcagtttgtgctctctctcggatgacaaaattgggtggaaatgtgctttattcacttgccgtccccagggcccctgatcttggggtgtggcccagcagcatgctagccagggcaggtggacgcactgggcggatgcaccggtgggggccaggccaggaggctcagcacagagctgactctgccccggttcctaaccctgcctccctaccccaggatccaagtacagagctgaacaatggagggagagacagcctgaacgccaggaccccacgctgcccggttcggggctcccagttccaccaggagggacagcaggagagggggcgccgcttgccgggcagcctggctggcagccatcagcagcagctgcaggtgcccgtgtgcacgcggaggatgcctcggctgtgcaagtgcaggaagttgaagatctcagagggcatggcgtggaagccgggacgcggcttgacgttgtcatagtagtggtgagtgatgtagaggcccgaggggttcatggggaaggcccagaagccaaagaggtgcacctcctcacagagctccagcgccgcagtgaccagaatgaggccggtgctgatgcgcttggcgcgcacccccaggctgagccagtagcgcgacacgttgaccaggtactgcggatggaagtagtagacagcttgcggcgattcgaagtcgtccagcacgtacttgacgcggatggacacgtcggtgttgcgcgtgttgtagaaggcaggcagcagcaccgacgcgttctcgtacacctgcagcacgcgatagaacggccgccgccacttctccagcttgtggaacctctctgtgatgatgctggggttcacagtgaccacatccgtcttcacccccacatccatggtgtacttctctgagatggggggcaggttgcaccggaagacgaagtcggcgctgttgatctccctcccgcagcggctgttcttcaagatgcctccgttgcccactacagcacacttcttaaactgggaccggtagtagggcatgtccttgggaaacatgcggaagatctcctggttgatgtggtagatgccactggtgtccacctcatacttgagctttgtccccaggggagtgttcttctgggtggtgaagagaaaggcaggggcgttgcagcacctggacagagtagacttgaactggttggcctcagagatgttcatcgcccatttgcacatctggaggctcttccacctgtcgaacagctctgactgcttcaccatggacagcaccttcacttccaatatttcgtgcctcagctccaggcatcttgtggagttatattcaaaaggcccctcataaaattcaaagtacctcttaatgtagttcctgccatacaggatctgttgcagcaaggtcaccaaggcaaaggcgcagatgaagatgaagagcaaagttcggctccccaacaaatcccggttggccgaggggtccgcgtagcgcatcctggctaccgggcgccgcgggcgcggggtacggggcggccaggcaatgactcgcggggttccggggccccggggggcgcgcggccgacttggcgcctcacggtgcggtcaggcaggcgggggacttcgaggggcaaagtttctggttggcgcggccggagctgggggcatccaagcgtcgcaggcgctggggcggcaagcaggacagggccggtggcagggagctctgccgcggccaggggccttccccacccccgggtacctttacctccaggcgccggtgccgggtagccgccgatttccccgcggaggggagacgccaggtgccacgagccggaggcggcccctcccgccgaggtggcggccaatggggagcaagacccgggctccgtcccctgtgcgccccagcgcgccgcgcatcgacccctccagtccggcgccggatcgcggttgcccagcgcgctgtgccctgccgggggcgggccacgtttgatctccgggcccgcagcaagggatcgcgaaggttggcctccggttctgccgat

SEQ ID NO: 8734 - RNA, 9782 nt, Homo sapiens
  source 1..9782: mol_type = other RNA
aagctcaggtttgagaactgctgacctagaatagtggttctcaaggctggctgcacattagaaacatctggagaatttgtgaaatcctaatattcaggtcacatctcagaccacctgactcagaatgtcaaggggtggggtcgcacgagtatttcttaaagctcttcagacgactctagcgtgcaccaaggcatagactgcctgccttagggtaatgactcccaaccatgtgagacagaaccacttaatgagatctttcaaaatagggataccaggccctatccccaggcctgctgaatcagatcctccgggaagtaaaggacctggcttggggattattttataaagacttccaggtgattcctatgtacacacaaggttgcaaatggcaattctagagaaaacagaacttttaccccaaagctgagcagatcatttagttgaaggaaatgagagatttgttgccatgggaaccatcttcaactgaagagagagtcactgatttctggcttttgtggccaacagctaagtcatggaagtgtatgtttttgcttttggtttttttcctttgaaataaaaaaaaaaaaaaagaaaggttctcagaagagactgtgcaggggaaaatacctaaagacttctaaaagatcagcaaggctattgtctctcaggacatgctggccaggacagtggagcccaggtggcagagcaaggccaggtctgcactctccctcagcaaggggccaaggtctcaggaagccaggggccaacgaccagcccaggacaactgcccaaggcaaaaacaaaaacaaaaatcagatttctgctttagggacacccaaaacagttaatgtcatttgagagctgcttgcacctaagtgattctaaaaagtctctggtatactatactaagtgaaataagccagtcatcagaaagacaaatattatatgattctacttatatgagggacctagagcagtaaaattcatagagaaagaaagtagaattgcgattgccaggggctggggaagggggaagtgaagacttgtcatttaatgggtttaaagttttcattttgcaagatgagaagagttccagagacagaatatacaacagtgtgaatgtacttaccattactgaactgtacacttaaaaatggttaagatgataaattctatgttatgtgtattttaccataattacaaatgaaaaagaaatctttgtttgtgttaaagcaaaaccaattttgtaaatgttagattcccgagcacttgacttttgttgctaggtacatagtgggttatatattatatttgtatgtacagaaaaggcagaagttgggttgtgtgccaaattcttcttttcattcttttcctactcaaggctccagtctgaatttcaagccatacatggccactcaactggtggcaacttctgaaccacaagcagttgtatgctcagggaacagatagggcctcacacatgctgattcccaggcgccacctctcccccaggttctcagtccatagttttaacaagcacccaggtgattctgatgcaggccatcagaaggccatcctacagggcatcctaataaacccatgtgatcttcaaagggtagactgtagatctatactgtagatctatactgtaggtctatccagtctaccctttgaagatcacactgtagatctatccagtctaccctttgaagatcacactggtttattaggatgccccgtaggatggaatcagcctccacagactggcctcgtttgactagacctctaaacaatagcacaaggcacaccctggccactggtgcacccctcgcctggcctcacctgacccctgagccacagttagcctcttcccagagggtgctctggttacagggaggagactaggtcagggcgtgtgttgagctcagagaagcagcaccttttttcccccaggaaacaaccccatgctcctggtcttccccttcgcatctggagcagacatcctgcaaagctcagctcacctgtttcccagccaaagcattcagcatgttcctctagttttttaaacaccattgataaatccctcttacattgcttcccaggctgcacctcagccacagtgatgtaagagcctgacatgtttgtgtggctttgaggaagggaagaagtagacaacaagaaacacagaaaatgtctctcccttctttcatttaaactagaggaaaaaggattggctagccagcaaaaagcagatgagcaggattataatgagggaaaacaaaaagaggctagccaagcccataagcccccactagacagacatttcagcctcctgagccccgagctcccctggacaggcaggaggagtctctgccttcctgggatgtgctaggtaaaaaaatcaatagaggactctcctcagctgacaatttccccaaggtgttactcagtttattagcggggtatcctgaactgctggagtcccccaggaaccagagacctcattactgtagtaaacatgtgttgagtggccatggcatgtgcttccccgccagtgctggcaatacaaaatgagcttagatatcgtgtcttcccttggggagaaggcaaaccttctatcaaggacacacgggcccttatgctgtgtgctgtgaggatgtcctaatggagtcggtgatggttgcagcagaagcacagaggagagagtgcccagcccaggtctctagaggggaggatgcagggggccattacctgacttctgcaaaagtggccagataaaaggaaggagagaggaacttaggagtgtgagggccattccaggtgtttgaacagagtgtgcaaaggtgcctggaatagtatgggatagggcagggaggtggcaggaggatctctgggaaggtgagtaagccagcttgggacattccctgcatgacttggtaaagaacctgaagtttatgatacaggtaggcaatgggccccacaaaaggtatttttggaaggttattctctgaaagcaaaaagatccatcagatggtctgggttagggcagtagcagaggggttgcagggagggaatgacttaaagggatgtttatgagttggaattgacaagatacagtgaacaaatagacataaagagtgaaggagaaggaagaggcaaaggtgatccaagttttgggccaaggcaacctgtgcttgctagtgtctagtttgtgctgggcactgtgctaggcattgtgcaacactatttcacttagctttgcaacagctgttgtggttggtatcctgtcctcatttcagatgatgagtccagagcctccaggggcttctggagctccctcaatttcacacagctacgaagtagtaggaggagactctgagttcagattgttcttttaactataccagttgaggacatgttgaggtctgagatgctgtgcagacacagacatgcaggaggccacagtgagcatgcttccaatgctcctagggaggactggcctgcaggtagaggggttaagatgccagggcagaagatacttaaggctttgaatagatgagatttctgcaggaatgctcctaggaagagaagagaaccctgaggaagcttcacggaagatgaatccacaaaggaacctgagaaggagcattcagagagacaggaggaaagtcagggaagaatagttagaaaacagaagaggagaggactttagaaagaccagagagactgtgcatagtggctcacacctgtaatcccagcactttgggaggccaaggcaggaggattgcttgagctcaggagttcgagactagcctcgtcaacatagcaaaaccccgtttctacaaaaaaaaaaaaattttcaaattagctgggagcaatggcacgtgcctgtggtcctagctacttgggaagctgaggtgggaggatcacttgaacccaggtgtcgaggctgcagtgagccatatttatatcaccaccctctagcctgggtgacagagggagactctgtctcaaacaaacaaacaaaaaagaccagagaggccaaccttgtcaaatgttacacggatgtcaaggatgatatctgagaagtatctgctgctttgctcattacactttttatgctgccaaccttcagaattcggaattgactttggtcatcccctcctccacctctcccagataactgtccctgagactggatttgatagtgttcagcacaaccagctcccacgtacgtttgtgggattcgtcatttaacgtctgtatacacacacaccagaccacaaactcccggagggcagggacgacgttttgttcatcactagctccccggcacctggcaccatgcctggcacaacatgagcactcaataaatataatttattcaccaattcactcactaaattggccagcactctactctgcctcagttgtttctaagcactgctctgcttcctccctgctctcagcaaagtcaagggcgatgagcacatgctgtctctgggcaccaggtgattagtgggcagagctgccgcagcagcattgctgaaatggtctcagacgctgcctctgaccttgagccacctttctttgtgcttggctaagcactgagtcatttacttgtttttgctgcctttcaagcctggagcagtgggtttagcacaaaggaagacatgatggttgttttgtttacgggaatcgatttcccttgaataataattcaatgggtagtctgcactgcatggtggcgtggtgacagggctgtggaggaacatggcagaaggcttccagagtcaacaccaggtctctctgagcctttgaaaaaatgtttttcttataaacactggctgcagcagaaaaactatatcctgaaagtcaggagactggtgagtcccagttgagccacaagctggccatgtagccctgggcaagtcattcgtgttgtcacttaacatgtgctatctctgggcatctttcctcaccttaaaaatgtgacgatggcctcagttcccctccagtgccactgtgggtaagtcgctactgctgtaggcggcagggttagggagaggcacctataagcacaggctgcttcccggacgatgacagcctcctagagcatttgtccctggaggagggccccgtactatcctgcaggggcatcttggtcaggatccctcatgttctggtgtcactgtctgggaagctaagacagaggtttggagcacagactttggggctctacagatctgggtgcagttccctccattgggtgccgttccctccattgggtgcctgaccaagggcaagtcctggaattgctttaagcctctgtctcctcatctgtacaatgggagcctccttacccaaaggggtctcatgatgattacaggagataatatagggaaagtgcttaacgtagcttgataaatgctagctagtataatgagaaatattaattatggtttagatccattcatcatgaatgtccccccaaaataaggacattgtacagacgctgaagatttttacaaagcttctagttgtagagatgaggaaactgagacattgagggagaggaaggactggccctaagacccacaggcaggaatatggccagcagccaggtgtcccaactcctctgtgggctggatcccgatgctccaatcctcagctcctacgagggccctggctggggcagattccaacctgcaacaccctcagctgtgggaatcctgatgtctgtgtcaccagggagcctcccccaaacactgcccatctggaacataactagtacccagagggcttccagtagagggctctgtccacagcaggcactcagtagagccccaggcatgacttgacccagtcacatctttgctctgggcctgtttcctaaagtggaacaaaatggtctttaagaaccttctagtttttatattccatggtttcaagaactgggttcaattaaccatgcagtggctagaaatctcaggtaactggaatctttcccagaaattccctccctgggagaaataggcagagctcaagcaagtaataaccatccactgtcctttgcagttcttcctggtttagcaggtgtttgggatcatttcatccccttggctactcccctacattcctgaccagcagactgagactcagagccacctgaggttttcccaaccaggaccagagctcagaatgcaggtgagagtcagcactgagaacagtgttgtgcacagggcacaggttccacaacaacccccccacaggaagcccaagccaagacacaaaagtttggccaagaacggagccctggatcaggagcctggaggcctgggataaagcctgcactctccacgtccctgactggctcagccggggggcctgtcaaatgaggtgattggatagcagatcccactccctgatagactcttacagctcctaaccctcccagagcacccagcacgtgggactgggtctataatctctgggccctgcacccccagaagacacagataatgcctttgtttatccttatgtcttcctaagtccaaccacagaccaaagcagaataggctttccagaaatgtttaaggggaggaagaaaagaggaagggagggaaggagaaaggggaggaggcagggagaaaggaaggagggagggagacaggttgccaggcaggtaggctgaagtcctcctcccagcactaacatcctatgattccacaaagctaagttctaaggcagttagttcaccaacagtgtctcttagacaccatcccatttatggtggaaacaccacagggagaagcaaagggaattaatttcagatgtgaaatgatatgtgaacccctctctgcctaagcccagctgactgccccaagcccaggccctggggtctgctgtgagaagtcccgccttcacagcggaagcctcagtgatgctggtgtcggaggccacaactcgtttctctctgctaagctcaccacctgacatgtcagtgctttccagcccagagcctatggttccgactgaggaacacgatacagcaggattctgcaggattcagagacatgagaggaagaggtctttataaataactcctggtttaaatggagctgaaaataggaagacaaaagaggaagccaattgctaagcacttattgagtcaataacattggcttggaagccatagtgcaagtggctggtttggtttatttccttctcatcaaaagagctaacgcaggattgaacctgggggcaccaagaccgcatgtgtgtccgaggatgtgtctgaaaggatgtggtgcttctcagatgatgatgtctcgactaagacataacccaggccttgggttagatctctcggtgtcacagaagaacctgtcgggtggtgtggcttggctgttaagtccctggacctcttgagatcactttcttcactggaaggtctagtcactgggttggcttctaagctctgagatttagatagcaattcatagctaagtcttcgatataaaacacaggaaccaaaagtgtgaataaaatcttgactgtgctcaagtgtcctgtgaagtgtcctgtctccactctcaattccattctctgtagggtcttccttcagctgcaacaagggcctgcagtttgtgctctctctcggatgacaaaattgggtggaaatgtgctttattcacttgccgtccccagggcccctgatcttggggtgtggcccagcagcatgctagccagggcaggtggacgcactgggcggatgcaccggtgggggccaggccaggaggctcagcacagagctgactctgccccggttcctaaccctgcctccctaccccaggatccaagtacagagctgaacaatggagggagagacagcctgaacgccaggaccccacgctgcccggttcggggctcccagttccaccaggagggacagcaggagagggggcgccgcttgccgggcagcctggctggcagccatcagcagcagctgcaggtgcccgtgtgcacgcggaggatgcctcggctgtgcaagtgcaggaagttgaagatctcagagggcatggcgtggaagccgggacgcggcttgacgttgtcatagtagtggtgagtgatgtagaggcccgaggggttcatggggaaggcccagaagccaaagaggtgcacctcctcacagagctccagcgccgcagtgaccagaatgaggccggtgctgatgcgcttggcgcgcacccccaggctgagccagtagcgcgacacgttgaccaggtactgcggatggaagtagtagacagcttgcggcgattcgaagtcgtccagcacgtacttgacgcggatggacacgtcggtgttgcgcgtgttgtagaaggcaggcagcagcaccgacgcgttctcgtacacctgcagcacgcgatagaacggccgccgccacttctccagcttgtggaacctctctgtgatgatgctggggttcacagtgaccacatccgtcttcacccccacatccatggtgtacttctctgagatggggggcaggttgcaccggaagacgaagtcggcgctgttgatctccctcccgcagcggctgttcttcaagatgcctccgttgcccactacagcacacttcttaaactgggaccggtagtagggcatgtccttgggaaacatgcggaagatctcctggttgatgtggtagatgccactggtgtccacctcatacttgagctttgtccccaggggagtgttcttctgggtggtgaagagaaaggcaggggcgttgcagcacctggacagagtagacttgaactggttggcctcagagatgttcatcgcccatttgcacatctggaggctcttccacctgtcgaacagctctgactgcttcaccatggacagcaccttcacttccaatatttcgtgcctcagctccaggcatcttgtggagttatattcaaaaggcccctcataaaattcaaagtacctggagctggagtcactgccgctctgcactgctggatcatccgtgacattaaagagccccgtccaattggtcagctggtcaccactctgccaaccaaactggaggcctctcttaatgtagttcctgccatacaggatctgttgcagcaaggtcaccaaggcaaaggcgcagatgaagatgaagagcaaagttcggctccccaacaaatcccggttggccgaggggtccgcgtagcgcatcctggctaccgggcgccgcgggcgcggggtacggggcggccaggcaatgactcgcggggttccggggccccggggggcgcgcggccgacttggcgcctcacggtgcggtcaggcaggcgggggacttcgaggggcaaagtttctggttggcgcggccggagctgggggcatccaagcgtcgcaggcgctggggcggcaagcaggacagggccggtggcagggagctctgccgcggccaggggccttccccacccccgggtacctttacctccaggcgccggtgccgggtagccgccgatttccccgcggaggggagacgccaggtgccacgagccggaggcggcccctcccgccgaggtggcggccaatggggagcaagacccgggctccgtcccctgtgcgccccagcgcgccgcgcatcgacccctccagtccggcgccggatcgcggttgcccagcgcgctgtgccctgccgggggcgggccacgtttgatctccgggcccgcagcaagggatcgcgaaggttggcctccggttctgccgat

SEQ ID NO: 8735 - RNA, 9581 nt, Homo sapiens
  source 1..9581: mol_type = other RNA
aagctcaggtttgagaactgctgacctagaatagtggttctcaaggctggctgcacattagaaacatctggagaatttgtgaaatcctaatattcaggtcacatctcagaccacctgactcagaatgtcaaggggtggggtcgcacgagtatttcttaaagctcttcagacgactctagcgtgcaccaaggcatagactgcctgccttagggtaatgactcccaaccatgtgagacagaaccacttaatgagatctttcaaaatagggataccaggccctatccccaggcctgctgaatcagatcctccgggaagtaaaggacctggcttggggattattttataaagacttccaggtgattcctatgtacacacaaggttgcaaatggcaattctagagaaaacagaacttttaccccaaagctgagcagatcatttagttgaaggaaatgagagatttgttgccatgggaaccatcttcaactgaagagagagtcactgatttctggcttttgtggccaacagctaagtcatggaagtgtatgtttttgcttttggtttttttcctttgaaataaaaaaaaaaaaaaagaaaggttctcagaagagactgtgcaggggaaaatacctaaagacttctaaaagatcagcaaggctattgtctctcaggacatgctggccaggacagtggagcccaggtggcagagcaaggccaggtctgcactctccctcagcaaggggccaaggtctcaggaagccaggggccaacgaccagcccaggacaactgcccaaggcaaaaacaaaaacaaaaatcagatttctgctttagggacacccaaaacagttaatgtcatttgagagctgcttgcacctaagtgattctaaaaagtctctggtatactatactaagtgaaataagccagtcatcagaaagacaaatattatatgattctacttatatgagggacctagagcagtaaaattcatagagaaagaaagtagaattgcgattgccaggggctggggaagggggaagtgaagacttgtcatttaatgggtttaaagttttcattttgcaagatgagaagagttccagagacagaatatacaacagtgtgaatgtacttaccattactgaactgtacacttaaaaatggttaagatgataaattctatgttatgtgtattttaccataattacaaatgaaaaagaaatctttgtttgtgttaaagcaaaaccaattttgtaaatgttagattcccgagcacttgacttttgttgctaggtacatagtgggttatatattatatttgtatgtacagaaaaggcagaagttgggttgtgtgccaaattcttcttttcattcttttcctactcaaggctccagtctgaatttcaagccatacatggccactcaactggtggcaacttctgaaccacaagcagttgtatgctcagggaacagatagggcctcacacatgctgattcccaggcgccacctctcccccaggttctcagtccatagttttaacaagcacccaggtgattctgatgcaggccatcagaaggccatcctacagggcatcctaataaacccatgtgatcttcaaagggtagactgtagatctatactgtagatctatactgtaggtctatccagtctaccctttgaagatcacactgtagatctatccagtctaccctttgaagatcacactggtttattaggatgccccgtaggatggaatcagcctccacagactggcctcgtttgactagacctctaaacaatagcacaaggcacaccctggccactggtgcacccctcgcctggcctcacctgacccctgagccacagttagcctcttcccagagggtgctctggttacagggaggagactaggtcagggcgtgtgttgagctcagagaagcagcaccttttttcccccaggaaacaaccccatgctcctggtcttccccttcgcatctggagcagacatcctgcaaagctcagctcacctgtttcccagccaaagcattcagcatgttcctctagttttttaaacaccattgataaatccctcttacattgcttcccaggctgcacctcagccacagtgatgtaagagcctgacatgtttgtgtggctttgaggaagggaagaagtagacaacaagaaacacagaaaatgtctctcccttctttcatttaaactagaggaaaaaggattggctagccagcaaaaagcagatgagcaggattataatgagggaaaacaaaaagaggctagccaagcccataagcccccactagacagacatttcagcctcctgagccccgagctcccctggacaggcaggaggagtctctgccttcctgggatgtgctaggtaaaaaaatcaatagaggactctcctcagctgacaatttccccaaggtgttactcagtttattagcggggtatcctgaactgctggagtcccccaggaaccagagacctcattactgtagtaaacatgtgttgagtggccatggcatgtgcttccccgccagtgctggcaatacaaaatgagcttagatatcgtgtcttcccttggggagaaggcaaaccttctatcaaggacacacgggcccttatgctgtgtgctgtgaggatgtcctaatggagtcggtgatggttgcagcagaagcacagaggagagagtgcccagcccaggtctctagaggggaggatgcagggggccattacctgacttctgcaaaagtggccagataaaaggaaggagagaggaacttaggagtgtgagggccattccaggtgtttgaacagagtgtgcaaaggtgcctggaatagtatgggatagggcagggaggtggcaggaggatctctgggaaggtgagtaagccagcttgggacattccctgcatgacttggtaaagaacctgaagtttatgatacaggtaggcaatgggccccacaaaaggtatttttggaaggttattctctgaaagcaaaaagatccatcagatggtctgggttagggcagtagcagaggggttgcagggagggaatgacttaaagggatgtttatgagttggaattgacaagatacagtgaacaaatagacataaagagtgaaggagaaggaagaggcaaaggtgatccaagttttgggccaaggcaacctgtgcttgctagtgtctagtttgtgctgggcactgtgctaggcattgtgcaacactatttcacttagctttgcaacagctgttgtggttggtatcctgtcctcatttcagatgatgagtccagagcctccaggggcttctggagctccctcaatttcacacagctacgaagtagtaggaggagactctgagttcagattgttcttttaactataccagttgaggacatgttgaggtctgagatgctgtgcagacacagacatgcaggaggccacagtgagcatgcttccaatgctcctagggaggactggcctgcaggtagaggggttaagatgccagggcagaagatacttaaggctttgaatagatgagatttctgcaggaatgctcctaggaagagaagagaaccctgaggaagcttcacggaagatgaatccacaaaggaacctgagaaggagcattcagagagacaggaggaaagtcagggaagaatagttagaaaacagaagaggagaggactttagaaagaccagagagactgtgcatagtggctcacacctgtaatcccagcactttgggaggccaaggcaggaggattgcttgagctcaggagttcgagactagcctcgtcaacatagcaaaaccccgtttctacaaaaaaaaaaaaattttcaaattagctgggagcaatggcacgtgcctgtggtcctagctacttgggaagctgaggtgggaggatcacttgaacccaggtgtcgaggctgcagtgagccatatttatatcaccaccctctagcctgggtgacagagggagactctgtctcaaacaaacaaacaaaaaagaccagagaggccaaccttgtcaaatgttacacggatgtcaaggatgatatctgagaagtatctgctgctttgctcattacactttttatgctgccaaccttcagaattcggaattgactttggtcatcccctcctccacctctcccagataactgtccctgagactggatttgatagtgttcagcacaaccagctcccacgtacgtttgtgggattcgtcatttaacgtctgtatacacacacaccagaccacaaactcccggagggcagggacgacgttttgttcatcactagctccccggcacctggcaccatgcctggcacaacatgagcactcaataaatataatttattcaccaattcactcactaaattggccagcactctactctgcctcagttgtttctaagcactgctctgcttcctccctgctctcagcaaagtcaagggcgatgagcacatgctgtctctgggcaccaggtgattagtgggcagagctgccgcagcagcattgctgaaatggtctcagacgctgcctctgaccttgagccacctttctttgtgcttggctaagcactgagtcatttacttgtttttgctgcctttcaagcctggagcagtgggtttagcacaaaggaagacatgatggttgttttgtttacgggaatcgatttcccttgaataataattcaatgggtagtctgcactgcatggtggcgtggtgacagggctgtggaggaacatggcagaaggcttccagagtcaacaccaggtctctctgagcctttgaaaaaatgtttttcttataaacactggctgcagcagaaaaactatatcctgaaagtcaggagactggtgagtcccagttgagccacaagctggccatgtagccctgggcaagtcattcgtgttgtcacttaacatgtgctatctctgggcatctttcctcaccttaaaaatgtgacgatggcctcagttcccctccagtgccactgtgggtaagtcgctactgctgtaggcggcagggttagggagaggcacctataagcacaggctgcttcccggacgatgacagcctcctagagcatttgtccctggaggagggccccgtactatcctgcaggggcatcttggtcaggatccctcatgttctggtgtcactgtctgggaagctaagacagaggtttggagcacagactttggggctctacagatctgggtgcagttccctccattgggtgccgttccctccattgggtgcctgaccaagggcaagtcctggaattgctttaagcctctgtctcctcatctgtacaatgggagcctccttacccaaaggggtctcatgatgattacaggagataatatagggaaagtgcttaacgtagcttgataaatgctagctagtataatgagaaatattaattatggtttagatccattcatcatgaatgtccccccaaaataaggacattgtacagacgctgaagatttttacaaagcttctagttgtagagatgaggaaactgagacattgagggagaggaaggactggccctaagacccacaggcaggaatatggccagcagccaggtgtcccaactcctctgtgggctggatcccgatgctccaatcctcagctcctacgagggccctggctggggcagattccaacctgcaacaccctcagctgtgggaatcctgatgtctgtgtcaccagggagcctcccccaaacactgcccatctggaacataactagtacccagagggcttccagtagagggctctgtccacagcaggcactcagtagagccccaggcatgacttgacccagtcacatctttgctctgggcctgtttcctaaagtggaacaaaatggtctttaagaaccttctagtttttatattccatggtttcaagaactgggttcaattaaccatgcagtggctagaaatctcaggtaactggaatctttcccagaaattccctccctgggagaaataggcagagctcaagcaagtaataaccatccactgtcctttgcagttcttcctggtttagcaggtgtttgggatcatttcatccccttggctactcccctacattcctgaccagcagactgagactcagagccacctgaggttttcccaaccaggaccagagctcagaatgcaggtgagagtcagcactgagaacagtgttgtgcacagggcacaggttccacaacaacccccccacaggaagcccaagccaagacacaaaagtttggccaagaacggagccctggatcaggagcctggaggcctgggataaagcctgcactctccacgtccctgactggctcagccggggggcctgtcaaatgaggtgattggatagcagatcccactccctgatagactcttacagctcctaaccctcccagagcacccagcacgtgggactgggtctataatctctgggccctgcacccccagaagacacagataatgcctttgtttatccttatgtcttcctaagtccaaccacagaccaaagcagaataggctttccagaaatgtttaaggggaggaagaaaagaggaagggagggaaggagaaaggggaggaggcagggagaaaggaaggagggagggagacaggttgccaggcaggtaggctgaagtcctcctcccagcactaacatcctatgattccacaaagctaagttctaaggcagttagttcaccaacagtgtctcttagacaccatcccatttatggtggaaacaccacagggagaagcaaagggaattaatttcagatgtgaaatgatatgtgaacccctctctgcctaagcccagctgactgccccaagcccaggccctggggtctgctgtgagaagtcccgccttcacagcggaagcctcagtgatgctggtgtcggaggccacaactcgtttctctctgctaagctcaccacctgacatgtcagtgctttccagcccagagcctatggttccgactgaggaacacgatacagcaggattctgcaggattcagagacatgagaggaagaggtctttataaataactcctggtttaaatggagctgaaaataggaagacaaaagaggaagccaattgctaagcacttattgagtcaataacattggcttggaagccatagtgcaagtggctggtttggtttatttccttctcatcaaaagagctaacgcaggattgaacctgggggcaccaagaccgcatgtgtgtccgaggatgtgtctgaaaggatgtggtgcttctcagatgatgatgtctcgactaagacataacccaggccttgggttagatctctcggtgtcacagaagaacctgtcgggtggtgtggcttggctgttaagtccctggacctcttgagatcactttcttcactggaaggtctagtcactgggttggcttctaagctctgagatttagatagcaattcatagctaagtcttcgatataaaacacaggaaccaaaagtgtgaataaaatcttgactgtgctcaagtgtcctgtgaagtgtcctgtctccactctcaattccattctctgtagggtcttccttcagctgcaacaagggcctgcagtttgtgctctctctcggatgacaaaattgggtggaaatgtgctttattcacttgccgtccccagggcccctgatcttggggtgtggcccagcagcatgctagccagggcaggtggacgcactgggcggatgcaccggtgggggccaggccaggaggctcagcacagagctgactctgccccggttcctaaccctgcctccctaccccaggatccaagtacagagctgaacaatggagggagagacagcctgaacgccaggaccccacgctgcccggttcggggctcccagttccaccaggagggacagcaggagagggggcgccgcttgccgggcagcctggctggcagccatcagcagcagctgcaggtgcccgtgtgcacgcggaggatgcctcggctgtgcaagtgcaggaagttgaagatctcagagggcatggcgtggaagccgggacgcggcttgacgttgtcatagtagtggtgagtgatgtagaggcccgaggggttcatggggaaggcccagaagccaaagaggtgcacctcctcacagagctccagcgccgcagtgaccagaatgaggccggtgctgatgcgcttggcgcgcacccccaggctgagccagtagcgcgacacgttgaccaggtactgcggatggaagtagtagacagcttgcggcgattcgaagtcgtccagcacgtacttgacgcggatggacacgtcggtgttgcgcgtgttgtagaaggcaggcagcagcaccgacgcgttctcgtacacctgcagcacgcgatagaacggccgccgccacttctccagcttgtggaacctctctgtgatgatgctggggttcacagtgaccacatccgtcttcacccccacatccatggtgtacttctctgagatggggggcaggttgcaccggaagacgaagtcggcgctgttgatctccctcccgcagcggctgttcttcaagatgcctccgttgcccactacagcacacttcttaaactgggaccggtagtagggcatgtccttgggaaacatgcggaagatctcctggttgatgtggtagatgccactggtgtccacctcatacttgagctttgtccccaggggagtgttcttctgggtggtgaagagaaaggcaggggcgttgcagcacctggacagagtagacttgaactggttggcctcagagatgttcatcgcccatttgcacatctggaggctcttccacctgtcgaacagctctgactgcttcaccctcttaatgtagttcctgccatacaggatctgttgcagcaaggtcaccaaggcaaaggcgcagatgaagatgaagagcaaagttcggctccccaacaaatcccggttggccgaggggtccgcgtagcgcatcctggctaccgggcgccgcgggcgcggggtacggggcggccaggcaatgactcgcggggttccggggccccggggggcgcgcggccgacttggcgcctcacggtgcggtcaggcaggcgggggacttcgaggggcaaagtttctggttggcgcggccggagctgggggcatccaagcgtcgcaggcgctggggcggcaagcaggacagggccggtggcagggagctctgccgcggccaggggccttccccacccccgggtacctttacctccaggcgccggtgccgggtagccgccgatttccccgcggaggggagacgccaggtgccacgagccggaggcggcccctcccgccgaggtggcggccaatggggagcaagacccgggctccgtcccctgtgcgccccagcgcgccgcgcatcgacccctccagtccggcgccggatcgcggttgcccagcgcgctgtgccctgccgggggcgggccacgtttgatctccgggcccgcagcaagggatcgcgaaggttggcctccggttctgccgat

SEQ ID NO: 8736 - RNA, 687 nt, Homo sapiens
  source 1..687: mol_type = other RNA
aagctcaggtttgagaactgctgacttacacaaagcccctggcacagggctgggtggggtacccccggcctgggtcccatagggacagtcaggactgttctggtcctgattccaattcagcagcacaggactggcctcccaccagagcccagggacaatggcaagtgacaagagccgcggaggcagcttgggaggtggcgatgacagaggatagaatcgacccagaaaagcaaactttgatttcctaaaaatatccctgagttaggagagtctcccccaacggcccctcccaattcaaatccatgaaaagccagatgcaaggcacccagccaggattgagatcaggcaattagaccatttcagacaagcttgcaagctctcagacgcacagacatttcagccgtacaaagaaaatgtgcactttgtggatacaatgacagcaaatcgttttccctttttgtccctcttcttcgtccctcctggtatccatgcccttgcggaatctccttcccttgggtgtgggctggacccctctctctctcgccggctctgagggtgactcttcctgccatagctgctttacaaagaggcttctgcagcaggaaactgagggcagtccttgatcaacagccagcaaagaaagttctgttagtcccagctactcgggaggctgaggtaggaggattg

SEQ ID NO: 8737 - RNA, 1582 nt, Homo sapiens
  source 1..1582: mol_type = other RNA
aagctcaggtttgagaactgctgacttacacaaagcccctggcacagggctgggtggggtacccccggcctgggtcccatagggacagtcaggactgttctggtcctgattccaattcagcagcacaggactggcctcccaccagagcccagggacaatggcaagtgacaagagccgcggaggcagcttgggaggtggcgatgacagaggatagaatcgacccagaaaagcaaactttgatttcctaaaaatatccctgagttaggagagtctcccccaacggcccctcccaattcaaatccatgaaaagccagatgcaaggcacccagccaggattgagatcaggcaattagaccatttcagacaagcttgcaagctctcagacgcacagacatttcagccgtacaaagaaaatgtgcactttgtggatacaatgacagcaaatcgttttccctttttgtccctcttcttcgtccctcctggtatccatgcccttgcggaatctccttcccttgggtgtgggctggacccctctctctctcgccggctctgagggtgactcttcctgccatagctgctttacaaagaggcttctgcagcaggaaactgagggcagtccttgatcaacagccagcaaagaaagtttcccgttttaattaatccacatgcaatttcagcagcagaaatgcaccatcactccggccaggaagcagcaggtacaggcatcttattactcggcatttgatagcccggctctcacttggttgttaacagccttcacaagaagaaacctcaatctgcaccgaaatgatgagaccggtgcagagggagacatcccggagcctggacgccttcaggcctcgtttcctccccagcccatcctcagcgcagagtgggggagagaagtcctgcttgcctcatgttggacagcagccgcccttgcatgtggaagttacacacactcactcacagggaccagcgcagggagaaacagaattggctacctccacctcaatgctccccttccgctcacgggcacctgccactgctctgtccagtcctgccctccacggtgccttgagggcctgtgtggtacagccgagtacaccaggacccagcgaagaggtgcctccctcaacactgtcacatagctacgaaggggtcaaactgagaccccaggtctgttcactgctggtgctcgacccccagtgggtccatggatgctaaactggggagggtcatgaggctgagggagggaatccctccgccaactcccactacacaaaacacaggaaagagacagaggatgccgagtccaggaagagagactccatgtacctaccagggggctgtgggtgcccctgggaaagcaggctgcctggcagatggcacagagtaaagaggacagggcccacggtggtgacacaaggaatgtgaatggctttgataggcagtctgggagctaaggaaaattggatgaatggagttcaaggggtcatggtcttaagaaaaatggtcttttggctgggtgtggtggctcatgcctataatcccagcactttgggaagccgaggtgggcgga

SEQ ID NO: 8738 - RNA, 29 nt, Homo sapiens
  source 1..29: mol_type = other RNA
aagctcaggtttgagaactgctgatcaga

SEQ ID NO: 8739 - RNA, 221 nt, Homo sapiens
  source 1..221: mol_type = other RNA
aagctgccagttgaagaactgtgttaaaaagttacttggggccagacgcagtggctcacacctgtaatcccagccgagatcagtctgcttggctgtggcttgctcgtgggtgccagcaccctgcctcccttccagtgccaggtcagcaggactgaacctgggttccaggctagtccaaaagcagagggtccctaaagtcacatagacccatttagtatcct

SEQ ID NO: 8740 - RNA, 968 nt, Homo sapiens
  source 1..968: mol_type = other RNA
aagctgccagttgaagaactgttgggtggagctgacaatgaggtcttgggagatggggaacggcccatggctgtggacatgccggctcctgcaggagagggaggctgagtctgttcctcggacaccttactccctttgggtccagccttttctttggttgatttttttcttttctgagctccaggagttgcctctgctccttcagttttgacagtgctgcttgtggagggtgcaggtgaagtagcatccacttccttcttcctctttcttgatagggctggtccttttacttttaacttttcttttttaagagtttcagccaggtcttcaagcgttggtatatcttcgaaaatttttattagtttgcccaaaccagcatcacctcggaacttttcttccatcaagtcagcaatctgaattttgtcatactcttctctcatttttaaattaagttttaaatcgttgctcagtaaggacttaaccattctaaaatgataatcattgatgacctctaatccttttagtagaacaatgttcttgtatttttttcccatctttacagacataagtgagcctcactggaaattttttcaacagtagtccagatcttgagatcttcagaaatgcaggaatcaatgcttatttgtgtgaggggggagataaatcagtaaagttcccagaaacggaaccgcaggatgttgtaatctccagaaacgctaagaaaatgaagtatctcaatgattagattcacgaatgctcagattttctgcattattcctggataaacaaacgtggatagtggactctcaacatgacagcatcgaagacttgaaaatcctggaaaatgcactgaacttccggtagtgtgaggagtctgtttaatcctctgctcagcagtgtatttttctctgttaaggacagtgggtgccctttagcgtgctgtaaccccaggatgtcaaataaatggc

SEQ ID NO: 8741 - RNA, 829 nt, Homo sapiens
  source 1..829: mol_type = other RNA
aagctgccagttgaagaactgttgggtggagctgacaatgaggtcttgggagatggggaacggcccatggctgtggacatgccggctcctgcaggagagggaggctgagtctgttcctcggacaccttactccctttgggtccagccttttctttggttgatttttttcttttctgagctccaggagttgcctctgctccttcagttttgacagtgctgcttgtggagggtgcaggtgaagtagcatccacttccttcttcctctttcttgatagggctggtccttttacttttaacttttcttttttaagagtttcagccaggtcttcaagcgttggtatatcttcgaaaatttttattagtttgcccaaaccagcatcacctcggaacttttcttccatcaagtcagcaatctgaattttgtcatactcttctctcatttttaaattaagttttaaatcgttgctcagtaaggacttaaccattctaaaatgataatcattgatgacctctaatccttttagtagaacaatgttcttgtatttttttcccatctttacagacataagtgagcctcactggaaattttttcaacagtagtccagatcttgagatcttcagaaatgcaggaatcaatgcttatttgtgtgaggggggagataaatcagtaaagttcccagaaacggaaccgcaggatgttgtaatctccagaaacgctaagaaaatgaagtatctgcaaagataacaaggaaaaaaggccttggttgagtcacttagttagctgactagtgctggcttgctcctattctgctattgccccagagaaaat

SEQ ID NO: 8742 - RNA, 1153 nt, Homo sapiens
  source 1..1153: mol_type = other RNA
aagctgccagttgaagaactgttgggtggagctgacaatgaggtcttgggagatggggaacggcccatggctgtggacatgccggctcctgcaggagagggaggctgagtctgttcctcggacaccttactccctttgggtccagccttttctttggttgatttttttcttttctgagctccaggagttgcctctgctccttcagttttgacagtgctgcttgtggagggtgcaggtgaagtagcatccacttccttcttcctctttcttgatagggctggtccttttacttttaacttttcttttttaagagtttcagccaggtcttcaagcgttggtatatcttcgaaaatttttattagtttgcccaaaccagcatcacctcggaacttttcttccatcaagtcagcaatctgaattttgtcatactcttctctcatttttaaattaagttttaaatcgttgctcagtaaggacttaaccattctaaaatgataatcattgatgacctctaatccttttagtagaacaatgttcttgtatttttttcccatctttacagacataagtgagcctcactggaaattttttcaacagtagtccagatcttgagatcttcagaaatgcaggaatcaatgcttatttgtgtgaggggggagataaatcagtaaagttcccagaaacggaaccgcaggatgttgtaatctccagaaacgctaagaaaatgaagtatcttgcttcattttgaatgttgaatcacttttggtggtataatcttacatagtttggatcccttataagctgaaaagtcgtgagatggagagtaaatataaggagatactcttgctaaccagcctggataacatcaccgatgaggaactggataggtttaagtgctttcttccagatgagtttaatattgccacaggcaaactgcatactctaaacagcacgagtagccaacttgatttaaaacgctggcatggtgtctgcagtgaggaagaccgtatttttcagaagctgaattatatgcttgtggcaaaatgtcttcgggaagagcaggaaacaggtatatgtgggagtccctcatctgcccggtccgtttctcagtcaagacttggtctttcctttcatggcatttctgggaatgcat

SEQ ID NO: 8743 - RNA, 1907 nt, Homo sapiens
  source 1..1907: mol_type = other RNA
aaggaaccagaaaatgagaagtaccatttatagttcacaagaaatgcaacatggaccccaatagaagtagatatcataactgatacttcctttgtttatgaccgcagacatgctaaaatgctaaagtaatgcttgcaaagaatatgaatgacaaatgttatccatcagctttttggtttaaaatgattgccaatgactagcagctttaatggtaacagtagggaggaagaacccttcaatacctaacaatgctgcagtctgctcctaagtggctttagttagagtcccttgttttaagggcaatactgcattgattctaaaggcatatgcagcaaaatgagcagggggagaaaaactggaagaaacataaaagttatatggttaatgtctttaaagtctaaaaatttaaactattgtttaaaaaacctaacatagttcagttactggcccacattgtaagcaaatatctgtgtgtgggatgggagccttcactttggagtggttttggtgactctgtttacattaaaaaggacagaagagtgttttgttgcattgacaaggtcccattcttttctatggagtatgatccttgttgtccgtgcgtctcttgaatttgagatctttccttttgatgaaaacactaattttgctggtttttgagcaggaaaggtggtatttctccagtctttgtagatgaaggtcccgtgacattataacccctcatttctccctttaagagaggatggctttagagtgctgaataccaatgaagttgatcagcgctgaaagaccttcttacagctgctccacacaagtctttgtcttcacataatctagaaatagcctctaggttctgtgctctttctttgctaagaggagcaaatagaaaattcaggtggtcatctgctaaggagcgatggtcaaggtagtgtttggcataaacactagcaggaacattaatattaaactgaagaagctccgaaaaatgcctttccatttcattcatgtcctcaactgtaatgtccttgaggatctggcagtagtccacattccatacagcctgatcatcccaaaccttggaggcaagaagagtggctcccagaacaatccttttctagttagtggggcaaatgtcgatttcagcataagttaaaagcctttctaagtaaaccagagttactgttgcacattcagctgttagctgtgcagcactaaaaagagtatgaacaaatctgtaaataaatttgtgctcaggatcatgcttaaactattcctgtggaactttttctcgtgtgaggggatgtgatctctcatcaaaaatatccagggatctgtttgcatctctgttctttatgtggtaatatatttctaaggtcacattttactgtggttctaaggttaggctggctgactgttctgtcacctagaaatattgttgagcatgagctatactttttagtaagctgccctggagatagatgatttaagtggttgctcttcctcttgtctcgcacatcggtttgagatttgctcaggaaacttgtgcttgcccttggatggtcagaagggtttgactccaaagctaaatcttagggcatctcgtggtcgctgatgtgctgcaggtggtggccctcgcccgctgcgaaatccaactggtaggctccacagaagcgggcgctaccgccaccgcatccccgggtgccgcctcgtagatgtcggttgcgcagtacagctctggcaccacgcaccggcccagcttgaggctggtactggggggacacgcaataggtcagcgtgttccccatggggcgtctctgctcctctgggccggggctggcgccttctctagccccctactcgccgccctcagcagccgcccctcccccaacaatggcgcagcccaggct

SEQ ID NO: 8744 - RNA, 37 nt, Homo sapiens
  source 1..37: mol_type = other RNA
aaggaaccagaaaatgagaagttaaatctgaagtcca

SEQ ID NO: 8745 - RNA, 35 nt, Homo sapiens
  source 1..35: mol_type = other RNA
aaggaaccagaaaatgagaagttgagtaggaactc

SEQ ID NO: 8746 - RNA, 544 nt, Homo sapiens
  source 1..544: mol_type = other RNA
aaggagatgctcaggcagatggagcacagcagctcgtccttgaggccccgcgagcttagcagccaccgcttcggtccagcgcagcctctcaacccggaaccagccgaatccgagctgccggtggccgcggctgcctccccgcccccgtgggcgggacccaagcaactccgcccccgcagcgggcgggggaggggcggggccaccagccggttgaccccgccccacccccaccatcctccagctcccagggaagcgaagcccagctgttccttcggggtgtgtacttggaactgcatccaggtctcgcttagggtccccgcggcgaggcggagcagctaatttgagagcacaacaaataaacaaggagcatctttctggatcatcgatttgaagatgtagaaaaaatcatattttgtattaaaacgaacaagaatatatttggaatacaacttctgcataaaatataaagataaaactcttgaaatgccctgcttgcttagagcgagttcaaggccctcacactcctaagccctggggtcccatt

SEQ ID NO: 8747 - RNA, 599 nt, Homo sapiens
  source 1..599: mol_type = other RNA
aaggagatgctcaggcagatggagcacagcagctcgtccttgaggccccgcgagcttagcagccaccgcttcggtccagcgcagcctctcaacccggaaccagccgaatccgagctgccggtggccgcggctgcctccccgcccccgtgggcgggacccaagcaactccgcccccgcagcgggcgggggaggggcggggccaccagccggttgaccccgccccacccccaccatcctccagctcccagggaagcgaagcccagctgttccttcggggtgtgtacttggaactgcatccaggtctcgcttagggtccccgcggcgaggcggagcagctaatttgagagcacaacaaataaacaaggagcatctttctggatcatcgatttgaagatgtagaaaaaatcatattttgtattaaaacgaacaagaatatatttggaatacaacttctgcataaaatataaagataaaactcttgaaatgccctgcttgcttagagcgagttcaaggccctcacactcctaagccctggggtcccatttcctcttcactttcttaaggagtgcttggggagaagtttggaaagccctggctaa

SEQ ID NO: 8748 - RNA, 2826 nt, Homo sapiens
  source 1..2826: mol_type = other RNA
aaggagatgctcaggcagatggagcacagcagctcgtccttgaggccccgcgagcttagcagccaccgcttcggtccagcgcagcctctcaacccggaaccagccgaatccgagctgccggtggccgcggctgcctccccgcccccgtgggcgggacccaagcaactccgcccccgcagcgggcgggggaggggcggggccaccagccggttgaccccgccccacccccaccatcctccagctcccagggaagcgaagcccagctgttccttcggggtgtgtacttggaactgcatccaggtctcgcttagggtccccgcggcgaggcggagcagctaatttgagagcacaacaaataaacaaggagcatctttctggatcatcgatttgaagatgtagaaaaaatcatattttgtattaaaacgaacaagaatatatttggaatacaacttctgcataaaatataaagataaaactcttgaaatgccctgcttgcttagagcgagttcaaggccctcacactcctaagccctggggtcccatttcctcttcactttcttaaggagtgcttggggagaagtttggaaagccctggctaacatctggccccggaggctgcctccattggcaaacaattctggagtgctgtatttgtgtgtgtgtgtgtgtgtgtgtgtgtgtgtgtgtaaggcggtgaggggtggagcaggagagagggagaaaaagtaataggagaacttgtcttgtgtgccagatggagaggggataagggatttctaggcagaggagacagcctgtgcaaaagcatagaggcgtgaaaggggagggcgcagtgaaggaagtgctagtaattctgtactgttgggggtggggtggagaaggagcctgggtgggctggagggcattgtgggtcatggtaaagaatttcttgaaggcatggggctttcaggcaagggaatgacctggtccgattgggtttcaggaagtcttggagataatcattataccatctgcaaggtgaagaagacagggagcttttccaatgtgtctgcggatgcacagcactcagcacacagtaaaggtgtgtagctgaataaccgcatcaacgccctgggttgcaggaggaaggaaagactgggcacccctaaggtgctgttgtcatcgtgcctgcaggaggtgagacccgaactggggcctcagcagtgggtaaggagagaagactagggtattgcaagtacagacacggtgacatttggtgatggttggatacgggggtgagggaaatgagccatagagggtggctaccagtttctgcctcctccagaaatatcttcattggtgttaaactttattgaggtacagtttatgaaaaagctctcagtttagttctctatggttaacactttctccatcacaccctcatctggcccagaatctccatcattgcgagaaaaatagttggttgctcatgcaacagcagtttctcaacattttcttatgggcagagccctgattttggtcaggtggcccccttccccaagtgacccaaggaaggctgaccccagcccatttccaggagtgagtcttgtttggtccaagtccattatggtggtctcatggagtgagtcttgtttggtccaagtccattatggtggtctcattcctcttgccagtgacggtttgggcaggtccagcctgaaaaactaaaggggaagcctatggcagagaggggttttcaggaaatggtctctttactttgcaaaacagtctgccccctttgctgggatatgtttggtggcaatgcttggaattgcaacagccatcttgctcccagtctgaggatgcagcaaatacagaagggagggcaaggccaagagagtcctagggaagagaagcttttattctgatgcagagtctggacttcaggatatgtgagatggtccatcttattgcataagccagtttaacagtagtgcattgtcactttgcaacccagagaatcccaactgatatactgacgtgcacccctaatgagggggtggggaaagtgaacagggcagagtctaaattattgaagcatttgaaatgaaatgaaaaaaaaaaaggcttgatgatggatgaaacagtgacttcattattcaacatgtatttactgatgctgactccaagcaggtctttgtgaggaggtggaataaactatgctccttgctcccaaggagctggcagtctagagggcaaaatcaatgagaaattcttatcaggcacagtagggcttgctaagcattctcacatatattattggatttcagtcccaaagcagccttaactagtttatattattatccccgttttatagaggaagataccaaggctcaaataaaggagatgtgatggaaattgctagctgtccactaaacttcatcctcctgttcttctatgtagtagagtagcagtcggaggaatggctggtccactagagatcatacatcccagctgttcttgcagccgagtgagacttggtgactaaaatctttctaatagaacataaatagaaatagaccttaaggcatgaagcttttgctctcccatgctccattttctcttctcttgagttggaacatagatgtaccagggacacagcttcaataatgcttcaaaagggctgatggagcaaagatatgggaggatcctgggttcctgaatgactgcatgaagtacagccaccctgacatggactacagagtgagaagtaaacttattttctaagagccattgtattttgggtcttttgttgcagcagcccagctttctccatactattttgca

SEQ ID NO: 8749 - RNA, 667 nt, Homo sapiens
  source 1..667: mol_type = other RNA
aaggagatgctcaggcagatggagcacagcagctcgtccttgaggctgcacgccatggcgccaggggcagcagagaggggggcccgaggggcaggggggcggctgagagagcgcggcgctgtcggaggcagcaccgagggctgggcgcggggacgaggcccgcacaggcaggggtaggagctaccggagaagggagggggtgctgtccggaaggagggtaacgcgaggaaggggtgcgcggctgagactccgtgggacgccagcccgggagggcagtctagaggtagtgggcagctcaaggcgatgggcgctgggaggaggctgtgagcggctgagggacggagatcctgacggggaggttctagggggcggggcagtcctaagggataggagctgggagaaggggatcccggagcggggtggagcccttaagggggtcgaaatcccggggtgggggcggtgcggggagggcgagaagctggggatggggaatcctgggggagggggcagccaggccgagccgtacattggctgtgaccggcagagaagaggaggggtgccggcccgctcagctgccggatcccggccccaaaccctggcccagcgcgaccccttacccccgcgagcttagcagccaccgcttcggtccagcgcagcctctcaaccc

SEQ ID NO: 8750 - RNA, 1242 nt, Homo sapiens
  source 1..1242: mol_type = other RNA
aaggagcttacaatctagctgggaagagcattctattattttatatttatttttcaagactaggtctcgctctgctgcccaggctagagtgtagaggcacaaacacagctaactgcagcctctgcctcctgggctcagccttccaagtagctgggaacatgggcgcacaccaccatgcctgactaatttttttttgtagagacctggtttcactatgttgcccagactggtcttgaactcctgggcttcagtaatcctcccacctcggcctctcaaggtgctgggattacaggagtgagacactgagcccagcctctgtcattttaaaagctaaaaagtatgaaagtacttgatatgaaattaaggtaaaataaataaaatgcaatagttaacttttaatttgacggaagacatgcagtacagacacacacaattaactctcaaataatttttcttttgtttagactaaataaatgttagggccatcacaaagcactcaccttgaaaggggtgaagataaattggggggcagaatgggaataccagcttaaaaaaacaaagatagactttcttacctctagcattgctcttttcagagatgggttctcgctctcccgagtaactaagactacaggcgtgcaccaccatgccctgttaaatttttttgaagagataggggtctggctatgttgcccaggctgatctcgaactcctgggctcaaccaatcagcccacctcagcttcccaaagcactgggattatgggtatgagccactgcatctggcctgtcaaataatttctataaggcaataatgctaccagaattcacataggctgagacagtatctgaagcactacaggttacaaaaaaatgttattaataatcccaaactggggatttcaggtcaagaaactgtgtcttttgtaaataggaaggcacagggaagttagatgttggaatgcagaatcactatatgcagactattcccacagaacaattccatgaagagacaaagaatggagccaagaggggcagccgtggactttgagaagggctggtccacagacacgaagacaggacccctgcatccctcttgtccctgctattgccactgtaccccacagcaattcttgagcagacccagctttctgtgttgacagacaggtttgtttcctcatctgccaaaagaagatggtggtgcccatgagccacctgcgttacacaaatgtttcaaaggttaa

SEQ ID NO: 8751 - RNA, 1163 nt, Homo sapiens
  source 1..1163: mol_type = other RNA
aaggagcttacaatctagctggggagacacaactaatgcacacttaaacaatcagtacaattagcgattaccacaatattgaccacaactgcatgagaccagggaaaagcaagatcagtgaggggcaaggggggttcagagaaagtgttttagtaaaggtgggattcatttacttttactgcttgaatagttccaaatcaagtgacacattattttggagtagggtgggcttgggaggcagtgaggaggaaaggggaatcgagagagcaaatgcagcgaggctggaatgcaagtgccctgggcaagggacagcgagagggccccactgtatttcttaaccaccctccttcctcaactgtgccctccagtcccgccacacaggcacgcggttggtgctgcaccaagattcagggcgtcggctggcgatgtcagaatgtccattctgctggctggtgcggtgttttgatttccatggtggggcctgctggcatggccctggcttcggggctgggatggtgctgtcccgactttgtccagatcagaatgcggtgcctatgcccagatctcaggggtctgctccccctatcccccctcctctctcgaccctgccccttagtgggaccggtgcaaaggggttgggaagggatctggtatcttcgtcattgtcggtactgcttctccgggggtctactggcccctcactgaccttgccaagtgctcctctggcgagggaacacaggggaccccacattcctgcgcggcactggctcccgtgctggccgagatgcacaggagcacctgatgatacggccgcccagggctgggagctggggcctcagttgggggctcgctgcctgcgctcccccaacacctgccgcccggtccgcgacaccgtgtatgccagcttctgcagggagtacctgaacacctcacttctcgcaatgggctgtgtccctggaggatttcgaaaagcgaatcctacccagtaaatgcagcattccaggaacacctgcagcagcacgcggaagatgtaccagccgatgatgagcagttcagccgaggccgccgccactgccgccatggttccaagaatggtaggtgggtggtcgagaaagagggtttgccgagatccgctggtctcggagtccgctgttgggcgcact

SEQ ID NO: 8752 - RNA, 1082 nt, Homo sapiens
  source 1..1082: mol_type = other RNA
aaggagcttacaatctagctggggagacacaactaatgcacacttaaacaatcagtacaattagcgattaccacaatattgaccacaactgcatgagaccagggaaaagcaagatcagtgaggggcaaggggggttcagagaaagtgttttagtaaaggtgggattcatttacttttactgcttgaatagttccaaatcaagtgacacattattttggagtagggtgggcttgggaggcagtgaggaggaaaggggaatcgagagagcaaatgcagcgaggctggaatgcaagtgccctgggcaagggacagcgagagggccccactgtatttcttaaccaccctccttcctcaactgtgccctccagtcccgccacacaggcacgcggttggtgctgcaccaagattcagggcgtcggctggcgatgtcagaatgtccattctgctggctggtgcggtgttttgatttccatggtggggcctgctggcatggccctggcttcggggctgggatggtgctgtcccgactttgtccagatcagaatgcggtgcctatgcccagatctcaggggtctgctccccctatcccccctcctctctcgaccctgccccttagtgggaccggtgcaaaggggttgggaagggatctggtatcttcgtcattgtcggtactgcttctccgggggtctactggcccctcactgaccttgccaagtgctcctctggcgagggaacacaggggaccccacattcctgcgcggcactggctcccgtgctggccgagatgcacaggagcacctgatgatacggccgcccagggctgggagctggggcctcagttgggggctcgctgcctgcgctcccccaacacctgccgcccggtccgcgacaccgtgtatgccagcttctgcagggagtacctgaacacctgcagcagcacgcggaagatgtaccagccgatgatgagcagttcagccgaggccgccgccactgccgccatggttccaagaatggtaggtgggtggtcgagaaagagggtttgccgagatccgctggtctcggagtccgctgttgggcgcact

SEQ ID NO: 8753 - RNA, 1158 nt, Homo sapiens
  source 1..1158: mol_type = other RNA
aaggagcttacaatctagctggggagacacaactaatgcacacttaaacaatcagtacaattagcgattaccacaatattgaccacaactgcatgagaccagggaaaagcaagatcagtgaggggcaaggggggttcagagaaagtgttttagtaaaggtgggattcatttacttttactgcttgaatagttccaaatcaagtgacacattattttggagtagggtgggcttgggaggcagtgaggaggaaaggggaatcgagagagcaaatgcagcgaggctggaatgcaagtgccctgggcaagggacagcgagagggccccactgtatttcttaaccaccctccttcctcaactgtgccctccagtcccgccacacaggcacgcggttggtgctgcaccaagattcagggcgtcggctggcgatgtcagaatgtccattctgctggctggtgcggtgttttgatttccatggtggggcctgctggcatggccctggcttcggggctgggatggtgctgtcccgactttgtccagatcagaatgcggtgcctatgcccagatctcaggggtctgctccccctatcccccctcctctctcgaccctgccccttagtgggaccggtgcaaaggggttgggaagggatctggtatcttcgtcattgtcggtactgcttctccgggggtctactggcccctcactgaccttgccaagtgctcctctggcgagggaacacaggggaccccacattcctgcgcggcactggctcccgtgctggccgagatgcacaggagcacctgatgatacggccgcccagggctgggagctggggcctcagttgggggctcgctgcctgcgctcccccaacacctgccgcccggtccgcgacaccgtgtatgccagcttctgcagggagtacctgaacacttctcgcaatgggctgtgtccctggaggatttcgaaaagcgaatcctacccagtaaatgcagcattccaggaacacctgcagcagcacgcggaagatgtaccagccgatgatgagcagttcagccgaggccgccgccactgccgccatggttccaagaatggtaggtgggtggtcgagaaagagggtttgccgagatccgctggtctcggagtccgctgttgggcgcact

SEQ ID NO: 8754 - RNA, 5629 nt, Homo sapiens
  source 1..5629: mol_type = other RNA
aaggcagggcccccgctccccgcccttaggaagctgtctgccaattcctccacatgctagggaaagacgccaatccctaaatttccctgggaaatacctagcaggtatcatatttgtcaaggggtaattctctttttctgatctagggagaagtagtctaggtcctcacgccttccccattttcatccccaaaagaagatcctattaccccaagtttctcaggagctttcacagtctgacatccaaaagttaaatcaacttcacagggcccttcctataccctcgaataagtctccaacacccagttctctctctgcctatggatgaaggtgccgggctgcctctaagaagattggctcgagtgcagattcaaaaataaaaagttcacagtcaatgaaaagtgctctcattacattacatacataaattatctgtttgattggttctacatttccaacagacatcattttgataggctgtattctcgtagagaagaatgaaaagccatgtgactagtcacatcacaccccattagtctgagataaggtgatttctctgtcacagagatccatcagcagcaactagtaaagagaatcaatcttcacttttttcctccacagaaatagtccctttcctgcccaggcaggcaaattctcaaaatgatcctaggagagaaagggttaatggcaggtggtaggactgatacagaacagctgctttcttcccagtacccctgggaattccaatgcaggttaaatgtgaaacttaacactgatagtggctaccagtttatccagagccagcccctgatggctctcacactttttggctccgagttcaaccccacacagctatggtttagaaatgtagacgcagggctgggcatggtggctgaggcctgtaatcacagcactttgggaggcagaggagggtggatcacctgaggtcaagagttcaacaccagcctggccaacatggtgaaaccccgtctctaaaaaaaaaaaataaaacttagccgggcataatggcaggtgcctgtaatcccagctactcgggaggctgagacaggagaatggcttgaacccagggacagaggctgcagtgacccgagaccccaccattgcactccagcctgagcgactgagcaagactccgtctcaaaacaaacaaacaaaaaaaaaacgaacaaacaaaaagaaatgtagaggcagaatgcctctagcaagtccctaccccaaccctgcacagcctcctcccacactgtgcccagtggggcagtcatagtgctgtgtcgaactcctccgggggctcggtccgatcctcttcatggggctcaggctcgagccggctgtcctggtgctgtttcatttgttccttcacttcttcttccaggtcatgaggcacaacaaactggtcctctggttccatctgagtgggggcagcaaaatagccagttttcctcttgggcacttctgtggccacttcaatgaggttcaggctgtcctctaggggcacaatagagccattggagagtttcttcccatagaggcaggaggtggagggagacttctgtaactccatcctgtccttgctcattggcaggagcatgccactattcacactgttctgtcttcggatcccaaaacacgaccctctagcatgttcctcagaacacagggtaggagaactctctatgagagggggtgagttctccagatccctccccctgcagcagtggatgtctacttccacctctaccttgctgccattggttatgaccccctcaacgggctggtcatcatcactgtccaggccgttgtcagactggttactggagaaggtagcagaagaaggctggcgctgaaacagcccagaggtgggtgttgggtggaggctgcagcgccgctctggcctcggaagcaaggcagtgtccaggcccccagcattatgctcatcagaagcagtggaccccacttcactgctcacctctgaggtggacatctcactgctgaactcagaggcaatcccactgctagaggatggagtggctggcttaggggcatccttgatagtggtggttgaagcaaatcccacaggacctgggagggtgagcccattcatttcacaagtgcagccttcctcaccaatattcaaataaactaccatcgcccctacattgtcctgacagccatagctctgcgctaatgtgcacagcttcttagcagctgctaatgggtcttgtacgtgacgtacagcattgacagcttctgtgtaggacaagtgttcccacaatgctttgtttcccagaatcagcaactcatcttgaatggtcagcggagtggaagatatgtggggcttggggaggatccaagggtagaggtatgtacagcccagcatccgggtacagcaggttaccccattcactttgttgtcctctgtgatgatggctttttggtccttcaccctttgagcctcctctgggtcctgctccaggctgaagactttagagaggggcactggcttcccacctcggcacaggactgcttggcacgtgccaacattggctacagtcaagctaaagctacttgctggatcggcagtgtcagggcggatgtagcacaggagagcggaggagcccaacttctggccagccattcctaatttcctgtgagataccaagaaggtgttagccatgaaaactgtgtcattagttgactgctgtacctcttctaaaagcacatctgccatcgtacactgcagcaggcgcgggagctcctcatttcggtctccatcaaacatgccatacacagctcccaccccctctgcaaagctatccatagcaagtgctgagacacacagcttatttctctgccctgccatctcagccagtccatggctccagaaggttgacgtaactgtagaatctgtggttggcaaaggtttctgatcaattttcagggttgtgatatggctaaatatgtccagtgtcttgtgttccagaaccagatttgtatttccagtcaggtcaaggtcttgtaatgtagcaggcaaagcctctggaatcaggatttctgtcaagtcgttgcaacttaggtctacaaactggatctgaggcaactgcagtatttctgggaaaatgctgatgttgttggagtgtgcaacaagggtgtgcagccttttacagtttgctatggttgtgggaatggttttaagcttgttgccacttaggttcagttcctccaattgctccaatttatttagtttgcttgcaggaaaggtctgtaactgattgtttgcaaggtgcaagattcgcaggtgcaggtgccctaccaggacaggtatgcactgatccgtcaggagattgttggtcagataaagcagctgcagcatactcaaactctcctctccagtgcaggcggatggtaaagactccagactatttgcagatgcattcaagtatctgagatttaaggccttggagaagagggtgtctggcagcctcgtgagtgcattatgctgaagatccagcacctcgagggggatgtgctctaccagtgttggaaggttttgcacatgattgtgtcccagcatcagttttctaagactcaagctactcagaattctcacgggaacctctgtgagaagattatagctcacatctaatacttctatcttctttgcttcacaggcccagtcagggacacactctagcaggtttcgggagagatccaagaaagtgagcaggctgggtactggatagacgttcactgctgtcagcctgttggaactggcatagagggtccgaagggaaaagccactgagtgttagctccctcagctgattccgcccacagtgcagctgttccaagctgcataaggagctaagatccaagtcagtcagtcggttgtcccgcagatccacgtgggtgatgtgtttatttccctccagattttcaataaccatggttttcaaatggttcatccttaaatccacatgcttgatatggttcatcctattcagcacccctaagttcaggacttccaggcaatttcctgccataaccactctatctaacatagtgagtttctcataaacctcaggaatttgactaaagttgttgaaggaaattcccaaggaggaaagctgttgtagatttcccaattcttcaggtaaagtagtcagaaagttgccatcaagacagagggtttgaagatttagcagattgccaatttgacttggtaggtcatgaaatccattacaggaaaggttgagctcagtcagggtagagatctcgcataacaatataggaaacaacccaagtttattatgggacaagttcaggcccttcagttgagaaaatttgtagagtgtatcgaggcctccgggtctttctaactgcatgaagttgtgtcgcaagttgaggtaggtaatatcttgactatagaagagatgctcaggaacctcctcgaggctgtaacacgagagatccacggtactgattcgctgggacaccaccttggatgcttgccgttgccatcgctggtactcggccaaagtctcgaagctgacatgataggtctgagcttgggctcctgctgagctgaaagcaagggagtattgccgtcgcttcacttcttctatctttccaccaaccagaggcaaaatgtgcatctttccagtttgacaatccttcactgaggaaacgataaggcaggtaccacagaggacaactaggcgctcagcccacttatgcagctgggtctttcccttgcgtacattatagatgccagacaataggattcgatccaaacgatccatgtggcatggtttttcaccataaaatcgaatcatacagccgaggtcaggatttgtagcctcctcctgtatgcgcacaggatcatcaaatcccagcctggataagtaatcataaacgatctgaagaggtcgttcagtaggttccagtctcctgaccaggtctccatgaagctgtaaataaagactttctcttccctctccagcacatatttctgatgctggtgtctctacagtgcaaaggacgagatgtaagtcagaggaagaggaggaggaggaagaggaagaggaggtggtggtggttgtagtggcagtggtagtgtctgctccataaaggtaaacacagcctctctttacatcttctcttagccagtctctttctcgagaaccaaacctacttctcctattcaaacaatttctgctcccattgcgtttcatatttctcttggcaaggccttttctcttccttatcagagatgcgtgcgaccttcttaagcaaattcaacccaacctcgtacaaaacgtccgctcacctcccagccatgttttaattcccttgcctcctcctggagcaaaattatcagaattcggtgctctgcttcaagcagtaatatggcctgtgacccggtttatgatttatttgcaaggctgattcagaaaaaaacttttaaaagttaacttcttttcttttctttgttttgtttttcttttcgttctcgcagtgatagtagttttgttgccaatgggccaaatttggagtcagccagcctgtttccagatctcccctctgcccttctttagatctatacccctgtgc

SEQ ID NO: 8755 - RNA, 5775 nt, Homo sapiens
  source 1..5775: mol_type = other RNA
aaggcagggcccccgctccccgcccttaggaagctgtctgccaattcctccacatgctagggaaagacgccaatccctaaatttccctgggaaatacctagcaggtatcatatttgtcaaggggtaattctctttttctgatctagggagaagtagtctaggtcctcacgccttccccattttcatccccaaaagaagatcctattaccccaagtttctcaggagctttcacagtctgacatccaaaagttaaatcaacttcacagggcccttcctataccctcgaataagtctccaacacccagttctctctctgcctatggatgaaggtgccgggctgcctctaagaagattggctcgagtgcagattcaaaaataaaaagttcacagtcaatgaaaagtgctctcattacattacatacataaattatctgtttgattggttctacatttccaacagacatcattttgataggctgtattctcgtagagaagaatgaaaagccatgtgactagtcacatcacaccccattagtctgagataaggtgatttctctgtcacagagatccatcagcagcaactagtaaagagaatcaatcttcacttttttcctccacagaaatagtccctttcctgcccaggcaggcaaattctcaaaatgatcctaggagagaaagggttaatggcaggtggtaggactgatacagaacagctgctttcttcccagtacccctgggaattccaatgcaggttaaatgtgaaacttaacactgatagtggctaccagtttatccagagccagcccctgatggctctcacactttttggctccgagttcaaccccacacagctatggtttagaaatgtagacgcagggctgggcatggtggctgaggcctgtaatcacagcactttgggaggcagaggagggtggatcacctgaggtcaagagttcaacaccagcctggccaacatggtgaaaccccgtctctaaaaaaaaaaaataaaacttagccgggcataatggcaggtgcctgtaatcccagctactcgggaggctgagacaggagaatggcttgaacccagggacagaggctgcagtgacccgagaccccaccattgcactccagcctgagcgactgagcaagactccgtctcaaaacaaacaaacaaaaaaaaaacgaacaaacaaaaagaaatgtagaggcagaatgcctctagcaagtccctaccccaaccctgcacagcctcctcccacactgtgcccagtggggcagtcatagtgctgtgtcgaactcctccgggggctcggtccgatcctcttcatggggctcaggctcgagccggctgtcctggtgctgtttcatttgttccttcacttcttcttccaggtcatgaggcacaacaaactggtcctctggttccatctgagtgggggcagcaaaatagccagttttcctcttgggcacttctgtggccacttcaatgaggttcaggctgtcctctaggggcacaatagagccattggagagtttcttcccatagaggcaggaggtggagggagacttctgtaactccatcctgtccttgctcattggcaggagcatgccactattcacactgttctgtcttcggatcccaaaacacgaccctctagcatgttcctcagaacacagggtaggagaactctctatgagagggggtgagttctccagatccctccccctgcagcagtggatgtctacttccacctctaccttgctgccattggttatgaccccctcaacgggctggtcatcatcactgtccaggccgttgtcagactggttactggagaaggtagcagaagaaggctggcgctgaaacagcccagaggtgggtgttgggtggaggctgcagcgccgctctggcctcggaagcaaggcagtgtccaggcccccagcattatgctcatcagaagcagtggaccccacttcactgctcacctctgaggtggacatctcactgctgaactcagaggcaatcccactgctagaggatggagtggctggcttaggggcatccttgatagtggtggttgaagcaaatcccacaggacctgggagggtgagcccattcatttcacaagtgcagccttcctcaccaatattcaaataaactaccatcgcccctacattgtcctgacagccatagctctgcgctaatgtgcacagcttcttagcagctgctaatgggtcttgtacgtgacgtacagcattgacagcttctgtgtaggacaagtgttcccacaatgctttgtttcccagaatcagcaactcatcttgaatggtcagcggagtggaagatatgtggggcttggggaggatccaagggtagaggtatgtacagcccagcatccgggtacagcaggttaccccattcactttgttgtcctctgtgatgatggctttttggtccttcaccctttgagcctcctctgggtcctgctccaggctgaagactttagagaggggcactggcttcccacctcggcacaggactgcttggcacgtgccaacattggctacagtcaagctaaagctacttgctggatcggcagtgtcagggcggatgtagcacaggagagcggaggagcccaacttctggccagccattcctaatttcctgtgagataccaagaaggtgttagccatgaaaactgtgtcattagttgactgctgtacctcttctaaaagcacatctgccatcgtacactgcagcaggcgcgggagctcctcatttcggtctccatcaaacatgccatacacagctcccaccccctctgcaaagctatccatagcaagtgctgagacacacagcttatttctctgccctgccatctcagccagtccatggctccagaaggttgacgtaactgtagaatctgtggttggcaaaggtttctgatcaattttcagggttgtgatatggctaaatatgtccagtgtcttgtgttccagaaccagatttgtatttccagtcaggtcaaggtcttgtaatgtagcaggcaaagcctctggaatcaggatttctgtcaagtcgttgcaacttaggtctacaaactggatctgaggcaactgcagtatttctgggaaaatgctgatgttgttggagtgtgcaacaagggtgtgcagccttttacagtttgctatggttgtgggaatggttttaagcttgttgccacttaggttcagttcctccaattgctccaatttatttagtttgtttaaggccttggagaagagggtgtctggcagcctcgtgagtgcattatgctgaagatccagcacctcgagggggatgtgctctaccagtgttggaaggttttgcacatgattgtgtcccagcatcagttttctaagactcaagctactcagaattctcacgggaacctctgtgagaagattatagctcacatctaatacttctatcttctttgcttcacaggcccagtcagggacacactctagcaggtttcgggagagatccaagaaagtgagcaggctgggtactggatagacgttcactgctgtcagcctgttggaactggcatagagggtccgaagggaaaagccactgagtgttagctccctcagctgattccgcccacagtgcagctgttccaagctgcataaggagctaagatccaagtcagtcagtcggttgtcccgcagatccacgtgggtgatgtgtttatttccctccagattttcaataaccatggttttcaaatggttcatccttaaatccacatgcttgatatggttcatcctattcagcacccctaagttcaggacttccaggcaatttcctgccataaccactctatctaacatagtgagtttctcataaacctcaggaatttgactaaagttgttgaaggaaattcccaaggaggaaagctgttgtagatttcccaattcttcaggtaaagtagtcagaaagttgccatcaagacagagggtttgaagatttagcagattgccaatttgacttggtaggtcatgaaatccattacaggaaaggttgagctcagtcagggtagagatctcgcataacaatataggaaacaacccaagtttattatgggacaagttcaggcccttcagttgagaaaatttgtagagtgtatcgaggcctccgggtctttctaactgcatgaagttgtgtcgcaagttgaggtaggtaatatcttgactatagaagagatgctcaggaacctcctcgaggctgtaacacgagagatccacggtactgattcgctgggacaccaccttggatgcttgccgttgccatcgctggtactcggccaaagtctcgaagctgacatgataggtctgagcttgggctcctgctgagctgaaagcaagggagtattgccgtcgcttcacttcttctatctttccaccaaccagaggcaaaatgtgcatctttccagtttgacaatccttcactgaggaaacgataaggcaggtaccacagaggacaactaggcgctcagcccacttatgcagctgggtctttcccttgcgtacattatagatgccagacaataggattcgatccaaacgatccatgtggcatggtttttcaccataaaatcgaatcatacagccgaggtcaggatttgtagcctcctcctgtatgcgcacaggatcatcaaatcccagcctggataagtaatcataaacgatctgaagaggtcgttcagtaggttccagtctcctgaccaggtctccatgaagctgtaaataaagactttctcttccctctccagcacatatttctgatgctggtgtctctacagtgcaaaggacgagatgtaagtcagaggaagaggaggaggaggaagaggaagaggaggtggtggtggttgtagtggcagtggtagtgtctgctccataaaggtaaacacagcctctctttacatcttctcttagccagtctctttctcgagaaccaaacctacttctcctattcaaacaatttctgctcccattgcgtttcatatttctctaaaaaatatcaagagaaagaaatcgttagctagaacatctgactgaattagacatttcagtcctcaccccacctctctctactttatattccccaacattctgctcaagtatcccctccttttgtggagcacttcacatctatcatgctcattcgtaataactcagataacttaattttctttactgctgtctgtgtttccatccatcatcttcgttgacctctcttttccttgtgttttcagaaacgtgtcaagaataacgaaacagcgggttgcagtggctcaggcctgtaatcccagcactttggggggccaaggtaagaggactgcttgaggccaggagttcaagactagcctaggtaagatggcaacatcccatctctacaaaagaaatttttttttatatattagccaggcatggtggcacacgcctgtaatcctagctacctgggaggcagaggtgtgaagattgcttgaacctgggaggcagaggtttcagtgagccaagacagcgccactgcactccggcctgggtgacagagcaagactccatctcaaaaaaaaagaaactttaggctgggcaaggtggctcacacctgtaatcccaacactttaggaggcccaggtgagggatcatttgaggtcaagaattcgagaccagcttggccaacatggtaaagccccatctccactaaaaatacaaaaaaaaaaaaaaaac

SEQ ID NO: 8756 - RNA, 296 nt, Homo sapiens
  source 1..296: mol_type = other RNA
aaggcctttctgaaccttcagataccccatctgatcactaggaagaccacgtgggagagtggtcaggtcagcatggtgaatcaatcatctctcctggaaaagcaagtccccatgcaggtccatctatgggtggctccaaagcatcttcccggcacccagcaaacagccagttcattcatccgctggggacctacaatcctgtgagctagggctgtctgtgcacacgtctgtctcaaatggcagtagcacttagtgttaccctaggaggcagtttgttctggcctttcagggacaga

SEQ ID NO: 8757 - RNA, 2173 nt, Homo sapiens
  source 1..2173: mol_type = other RNA
aagggaagatggtgaccacataggagggacagcggcctttccaacaggggacccttgccagccatggtgagtagatggaatctgtgcccatcctctgcaagcccctagcaaacgtgtgaccaggaaagagtctgagatcatgtcacatttcctgagatgagcacgtaggtagaagctccttcctttaagctttagttcttactggggatggaaattccatccaacaaatgttgatatagcttgcttccttctaaggggatttccagcaggtggaaattgaattgtgagggaacaagtaaatcttcccagagtgtctgaagtcacatcgcagccttagcttttagccggggctttgtccctcccttctaggacagtctccatgacctcagctgaaaatgggacaaagtggggacctgtgagtccttacacttgcagttttcacagggctgctcagctttgagcttggccactcccatcctcagggtgtcccaatctgagatccaggaaatcaggaagactaagaggctggtgtcatggcccagggcagagcctacctgaatcatagctgaaccagcaaatgggggtgggggaagatgaaggctgagttctccagttcccttcattggcttccaggtgtgcaggtggcttgggattgaggactcagatcttctcaggccccgagggcatcgatgccagcagggctgagcaccagtgcctgaaggatgtcggagagggagaccacgcccaagagatgctgggtctcgtccactagcaccagcctgtgtacctgctcccgagcaatcctgtcgatcacttcccccaagctctcgtggggctggcaggaaaggactccctccagacatagtgtcctctgcctcagggcttctcccacactcatgtccaggtggttgtaggtttgctgggcagccaggtgaatcacatcaaagcgggaatagaggcccacgacctgaccacattcgttgaccacaggcagtgcagacacacgccggtccacaaagatgtccagtgcagtcaggatgggtgctgtctccagcaccacagccaagtctcggaatgtgccgatgcccaaatcttggatagtgcggtagaggaaggagggccggggcagcagggaaccaaagatgtgcaggaacttgagcaggcgtttgtgtgtgaggatgtggagtacgttgcctgacaccgggtcaagaacaggcaggcgatggatccggttcttgatgagggtgtagacagcttcaaacaggctatcattaggagagatggagaccagaggcttgaagcagccttgcaggtagatctccctccaggtctcaatcttatgttgttcaatctcatagatctggaccaggggggacctgtagtagcgatgcagcaccaggatgaagtcagtgatggtcagcatccccacaaagctctgcttcttgctgtcccatagaggggctgcccgcacaccgttggccaccagagcaaagaaggccttcttgatctccagcatggtgtcgaagatgactagcttggagctagttgccatggcatcgtagcaggtgtgctcctgcatgaagcgcatgtagatctgggcgccgggtttccgcagttcgtcatcccagcccagcttgggaaatggggcctgcggggacaggcacagggcaggcctctcttccagcaggccttctagctcacactcccaggcctctgtggctgggaactccgtggccagctccacatcatctgtgctggagcctgcagctgaggctgtacagtcagaggggaggcagtcccaccctgttggtggagtgcccaccccggcaggatcagcttgagccaagggtgtggtcttggggaatgtggcctccagcccggtggactcagcagctggcctggaccggggaccttccccctgacctggtggctccccttcctccaccgacttctgccttgtccatctcaaggctttggccctccgtttcccacggattctttctgagctgctggtcacagctggtgatggccatgagctgctgttttcttgctctaggaagctcatctcttgatgctcagaacccccaaggctgctccaggaaggggtcctgcgcagtgcgtgctccagcccgggctccatgtggccagccccagaccaactgagagcaagtgt

SEQ ID NO: 8758 - RNA, 103 nt, Homo sapiens
  source 1..103: mol_type = other RNA
aagggacagggagggtcgtggctccgcgctccggcggcgccagccgctctgccctgcgctgttggaggacagcggtccgagcgccgtggatcccaagcgctct

SEQ ID NO: 8759 - RNA, 2567 nt, Homo sapiens
  source 1..2567: mol_type = other RNA
aagggaggaggagcggaggggccctgagaagcaaagctgaggccctgaggactgagaaaagaaaagttgtaggaagcacaggaagctggggaccggctggaggccctggaggccgaacgttcccgggacttgtaggggtacttgagtgtggtgtccagctgcttgaagctctccttcagtgagtggcactggtagtactccaccaactccaggaggctgtcgaatttcttggcctctgtgatgtggatccagttgtccttctccaccaccttgatgtgcttcacctcatcattgaacttgatgcttattgcaaagcgctcagcctcggcaggccgctccctgatcaggtaggtcccgctggcgtgggacttgagcaggttgtccgtctgctgcctctccatgttacctgcaaaccaggggtatgcagtgtagtcgatctcccgggatggcggccggctgatgggcggccttccatccacagggcagggcttcacagatgagctggggaaataccctgacttcctggtttgtaccagacgaccctcccaccacggagactcagggtcgcccctcagcagctcaagcacgtcgcccgtctggaaggtcagcacaggcttcccgggaggggctgggttgccatggtaattctgcatggccaccatcttgggacctggtcccgctccggaggcgtccagatctgcaggagaagtgaacttgcagggaggtatcacttccaggcactccttgtgtgccccgacgccacacttggtacacatgtatccctggtagaaggtgcccctgaggaacattttgcaggctttgcagttggtggtcttgtcaaacgtgtacatctggaaactgtggtggttggcattggctttgtctggcttgatgtttgacatggccatctcaaactgctccatccacttcctcttcatatcttctgttttgcagaaaaactggaagccctgctttccttgaaggtgaattaggtagaagccgtaggaccacattttcccgtgagaccacagccctcctccaagcaccgcagggtgggacgggagaggaaagcctgcttgcttcttgacgtccttgttgttcatggggtcgtcggtcatcttgtggaacagcagctcgatgatctccttgagctcgtagctgtagcccttccgcttgcagacgatgaccaccttgtcaaacaggaacaagtacctgtcctgcttggtgtggttgactatggaccggactttcagttccccgtcaatctttggtcttccaaattcctccagtttcacttgcaaattttctatagaactctgaaattcgctgattttcctcaaggtctccttgtcccgtttaacttcattgatgtacatcgccaagtcctgcatggcttccagtgcttctttgagctgctgcctctcaggccgttccgcagaatggctcagaagctccttcaagagcaggtggtatttgagcaccctctgcatggggaccaccagcaggtcttgcagcttaaattttccatcctggaccttcagtgtgcactcctcgactttctgcctgaagtcctcccggctggccaggagctggttcagtgtgttctgggcgtgctccatgtggctgcagtactccccgtagatcagaagcctttccttgaaatcgaggaagaccttggccagcgtgctgccccccaccatcacggacacgtcgatggccctcaggaagctgtgatgcaccttgatcaggtcctccaggttaatgaagacagctgccatgtccgccgggctcagcaccagccgcagggggctcatgtagttcttctcaatgtcctccagggtgcggtagtacttggcctcggtctcctggatctccagcaggcagcagttcctcttgtcatcttcagtcatgcccattttcatgggctgctgcacctccaccttgatgatgtcctcgtagatgtcgtcccctccatcctcacacgggacgcagtcgtagatgtcctcccccaggtcatgctcgtcggccagctcctccaggctgcggtagacgtcatcgtcattctctgtggtctcctctgagggaaaaggcctgatccctttgttctgcgcgatgctgtgcagggagagcctcgacaccgcggagatgacctttccaaagtctcgcacatcgaagaggtcaaaggggtcaaacagctcgctgttccttaatccaaatttatcgtggcagactttcaggaaggtgcgtatgttcttcaaacacagaaactgggacatctgcggccggaagttgatgtccttgaggtcgatggagccgggggagaggttgtgcagcagctggcacagaaggaccccgtcgcgcagcgcctgcgccaggtcgaagaccacggccgagggccacaccacccggtggttgggcggcaggaccttgcaatcgatgagccagcggccgcactgccgccactgctccatggcgcccgcgggcccgaccggctcagggcagtgctcgagccaaagtgcagcggccgcggggcatcccgcccgcgcgcgcgcggggctcagggccgg

SEQ ID NO: 8760 - RNA, 2582 nt, Homo sapiens
  source 1..2582: mol_type = other RNA
aagggaggaggagcggaggggccctgagaagcaaagctgaggccctgaggactgagaaaagaaaagttgtaggaagcacaggaagctggggaccggctggaggccctggaggccgaacgttcccgggacttgtaggggtacttgagtgtggtgtccagctgcttgaagctctccttcagtgagtggcactggtagtactccaccaactccaggaggctgtcgaatttcttggcctctgtgatgtggatccagttgtccttctccaccaccttgatgtgcttcacctcatcattgaacttgatgcttattgcaaagcgctcagcctcggcaggccgctccctgatcaggtaggtcccgctggcgtgggacttgagcaggttgtccgtctgctgcctctccatgttacctgcaaaccaggggtatgcagtgtagtcgatctcccgggatggcggccggctgatgggcggccttccatccacagggcagggcttcacagatgagctggggaaataccctgacttcctggtttgtaccagacgaccctcccaccacggagactcagggtcgcccctcagcagctcaagcacgtcgcccgtctggaaggtcagcacaggcttcccgggaggggctgggttgccatggtaattctgcatggccaccatcttgggacctggtcccgctccggaggcgtccagatctgcaggagaagtgaacttgcagggaggtatcacttccaggcactccttgtgtgccccgacgccacacttggtacacatgtatccctggtagaaggtgcccctgaggaacattttgcaggctttgcagttggtggtcttgtcaaacgtgtacatctggaaactgtggtggttggcattggctttgtctggcttgatgtttgacatggccatctcaaactgctccatccacttcctcttcatatcttctgttttgcagaaaaactggaagccctgctttccttgaaggtgaattaggtagaagccgtaggaccacattttcccgtgagaccacagccctcctccaagcaccgcagggtgggacgggagaggaaagcctgcttgcttcttgacgtccttgttgttcatggggtcgtcggtcatcttgtggaacagcagctcgatgatctccttgagctcgtagctgtagcccttccgcttgcagacgatgaccaccttgtcaaacaggaacaagtacctgtcctgcttggtgtggttgactatggaccggactttcagttccccgtcaatctttggtcttccaaattcctccagtttcacttgcaaattttctatagaactctgaaattcgctgattttcctcaaggtctccttgtcccgtttaacttcattgatgtacatcgccaagtcctgcatggcttccagtgcttctttgagctgctgcctctcaggccgttccgcagaatggctcagaagctccttcaagagcaggtggtatttgagcaccctctgcatggggaccaccagcaggtcttgcagcttaaattttccatcctggaccttcagtgtgcactcctcgactttctgcctgaagtcctcccggctggccaggagctggttcagtgtgttctgggcgtgctccatgtggctgcagtactccccgtagatcagaagcctttccttgaaatcgaggaagaccttggccagcgtgctgccccccaccatcacggacacgtcgatggccctcaggaagctgtgatgcaccttgatcaggtcctccaggttaatgaagacagctgccatgtccgccgggctcagcaccagccgcagggggctcatgtagttcttctcaatgtcctccagggtgcggtagtacttggcctcggtctcctggatctccagcaggcagcagttcctcttgtcatcttcagtcatgcccattttctgcatgtatctaatcatgggctgctgcacctccaccttgatgatgtcctcgtagatgtcgtcccctccatcctcacacgggacgcagtcgtagatgtcctcccccaggtcatgctcgtcggccagctcctccaggctgcggtagacgtcatcgtcattctctgtggtctcctctgagggaaaaggcctgatccctttgttctgcgcgatgctgtgcagggagagcctcgacaccgcggagatgacctttccaaagtctcgcacatcgaagaggtcaaaggggtcaaacagctcgctgttccttaatccaaatttatcgtggcagactttcaggaaggtgcgtatgttcttcaaacacagaaactgggacatctgcggccggaagttgatgtccttgaggtcgatggagccgggggagaggttgtgcagcagctggcacagaaggaccccgtcgcgcagcgcctgcgccaggtcgaagaccacggccgagggccacaccacccggtggttgggcggcaggaccttgcaatcgatgagccagcggccgcactgccgccactgctccatggcgcccgcgggcccgaccggctcagggcagtgctcgagccaaagtgcagcggccgcggggcatcccgcccgcgcgcgcgcggggctcagggccgg

SEQ ID NO: 8761 - RNA, 2478 nt, Homo sapiens
  source 1..2478: mol_type = other RNA
aagggaggaggagcggaggggccctgagaagcaaagctgaggccctgaggactgagaaaagaaaagttgtaggaagcacaggaagctggggaccggctggaggccctggaggccgaacgttcccgggacttgtaggggtacttgagtgtggtgtccagctgcttgaagctctccttcagtgagtggcactggtagtactccaccaactccaggaggctgtcgaatttcttggcctctgtgatgtggatccagttgtccttctccaccaccttgatgtgcttcacctcatcattgaacttgatgcttattgcaaagcgctcagcctcggcaggccgctccctgatcaggtaggtcccgctggcgtgggacttgagcaggttgtccgtctgctgcctctccatgttacctgcaaaccaggggtatgcagtgtagtcgatctcccgggatggcggccggctgatgggcggccttccatccacagggcagggcttcacagatgagctggggaaataccctgacttcctggtttgtaccagacgaccctcccaccacggagactcagggtcgcccctcagcagctcaagcacgtcgcccgtctggaaggtcagcacaggcttcccgggaggggctgggttgccatggtaattctgcatggccaccatcttgggacctggtcccgctccggaggcgtccagatctgcaggagaagtgaacttgcagggaggtatcacttccaggcactccttgtgtgccccgacgccacacttggtacacatgtatccctggtagaaggtgcccctgaggaacattttgcaggctttgcagttggtggtcttgtcaaacgtgtacatctggaaactgtggtggttggcattggctttgtctggcttgatgtttgacatggccatctcaaactgctccatccacttcctcttcatatcttctgttttgcagaaaaactggaagccctgctttccttgaaggtgaattaggtagaagccgtaggaccacattttcccgtgagacttcttgacgtccttgttgttcatggggtcgtcggtcatcttgtggaacagcagctcgatgatctccttgagctcgtagctgtagcccttccgcttgcagacgatgaccaccttgtcaaacaggaacaagtacctgtcctgcttggtgtggttgactatggaccggactttcagttccccgtcaatctttggtcttccaaattcctccagtttcacttgcaaattttctatagaactctgaaattcgctgattttcctcaaggtctccttgtcccgtttaacttcattgatgtacatcgccaagtcctgcatggcttccagtgcttctttgagctgctgcctctcaggccgttccgcagaatggctcagaagctccttcaagagcaggtggtatttgagcaccctctgcatggggaccaccagcaggtcttgcagcttaaattttccatcctggaccttcagtgtgcactcctcgactttctgcctgaagtcctcccggctggccaggagctggttcagtgtgttctgggcgtgctccatgtggctgcagtactccccgtagatcagaagcctttccttgaaatcgaggaagaccttggccagcgtgctgccccccaccatcacggacacgtcgatggccctcaggaagctgtgatgcaccttgatcaggtcctccaggttaatgaagacagctgccatgtccgccgggctcagcaccagccgcagggggctcatgtagttcttctcaatgtcctccagggtgcggtagtacttggcctcggtctcctggatctccagcaggcagcagttcctcttgtcatcttcagtcatgcccattttctgcatgtatctaatcatgggctgctgcacctccaccttgatgatgtcctcgtagatgtcgtcccctccatcctcacacgggacgcagtcgtagatgtcctcccccaggtcatgctcgtcggccagctcctccaggctgcggtagacgtcatcgtcattctctgtggtctcctctgagggaaaaggcctgatccctttgttctgcgcgatgctgtgcagggagagcctcgacaccgcggagatgacctttccaaagtctcgcacatcgaagaggtcaaaggggtcaaacagctcgctgttccttaatccaaatttatcgtggcagactttcaggaaggtgcgtatgttcttcaaacacagaaactgggacatctgcggccggaagttgatgtccttgaggtcgatggagccgggggagaggttgtgcagcagctggcacagaaggaccccgtcgcgcagcgcctgcgccaggtcgaagaccacggccgagggccacaccacccggtggttgggcggcaggaccttgcaatcgatgagccagcggccgcactgccgccactgctccatggcgcccgcgggcccgaccggctcagggcagtgctcgagccaaagt

SEQ ID NO: 8762 - RNA, 2498 nt, Homo sapiens
  source 1..2498: mol_type = other RNA
aagggaggaggagcggaggggccctgagaagcaaagctgaggccctgaggactgagaaaagaaaagttgtaggaagcacaggaagctggggaccggctggaggccctggaggccgaacgttcccgggacttgtaggggtacttgagtgtggtgtccagctgcttgaagctctccttcagtgagtggcactggtagtactccaccaactccaggaggctgtcgaatttcttggcctctgtgatgtggatccagttgtccttctccaccaccttgatgtgcttcacctcatcattgaacttgatgcttattgcaaagcgctcagcctcggcaggccgctccctgatcaggtaggtcccgctggcgtgggacttgagcaggttgtccgtctgctgcctctccatgttacctgcaaaccaggggtatgcagtgtagtcgatctcccgggatggcggccggctgatgggcggccttccatccacagggcagggcttcacagatgagctggggaaataccctgacttcctggtttgtaccagacgaccctcccaccacggagactcagggtcgcccctcagcagctcaagcacgtcgcccgtctggaaggtcagcacaggcttcccgggaggggctgggttgccatggtaattctgcatggccaccatcttgggacctggtcccgctccggaggcgtccagatctgcaggagaagtgaacttgcagggaggtatcacttccaggcactccttgtgtgccccgacgccacacttggtacacatgtatccctggtagaaggtgcccctgaggaacattttgcaggctttgcagttggtggtcttgtcaaacgtgtacatctggaaactgtggtggttggcattggctttgtctggcttgatgtttgacatggccatctcaaactgctccatccacttcctcttcatatcttctgttttgcagaaaaactggaagccctgctttccttgaaggtgaattaggtagaagccgtaggaccacttcttgacgtccttgttgttcatggggtcgtcggtcatcttgtggaacagcagctcgatgatctccttgagctcgtagctgtagcccttccgcttgcagacgatgaccaccttgtcaaacaggaacaagtacctgtcctgcttggtgtggttgactatggaccggactttcagttccccgtcaatctttggtcttccaaattcctccagtttcacttgcaaattttctatagaactctgaaattcgctgattttcctcaaggtctccttgtcccgtttaacttcattgatgtacatcgccaagtcctgcatggcttccagtgcttctttgagctgctgcctctcaggccgttccgcagaatggctcagaagctccttcaagagcaggtggtatttgagcaccctctgcatggggaccaccagcaggtcttgcagcttaaattttccatcctggaccttcagtgtgcactcctcgactttctgcctgaagtcctcccggctggccaggagctggttcagtgtgttctgggcgtgctccatgtggctgcagtactccccgtagatcagaagcctttccttgaaatcgaggaagaccttggccagcgtgctgccccccaccatcacggacacgtcgatggccctcaggaagctgtgatgcaccttgatcaggtcctccaggttaatgaagacagctgccatgtccgccgggctcagcaccagccgcagggggctcatgtagttcttctcaatgtcctccagggtgcggtagtacttggcctcggtctcctggatctccagcaggcagcagttcctcttgtcatcttcagtcatgcccattttcatgggctgctgcacctccaccttgatgatgtcctcgtagatgtcgtcccctccatcctcacacgggacgcagtcgtagatgtcctcccccaggtcatgctcgtcggccagctcctccaggctgcggtagacgtcatcgtcattctctgtggtctcctctgagggaaaaggcctgatccctttgttctgcgcgatgctgtgcagggagagcctcgacaccgcggagatgacctttccaaagtctcgcacatcgaagaggtcaaaggggtcaaacagctcgctgttccttaatccaaatttatcgtggcagactttcaggaaggtgcgtatgttcttcaaacacagaaactgggacatctgcggccggaagttgatgtccttgaggtcgatggagccgggggagaggttgtgcagcagctggcacagaaggaccccgtcgcgcagcgcctgcgccaggtcgaagaccacggccgagggccacaccacccggtggttgggcggcaggaccttgcaatcgatgagccagcggccgcactgccgccactgctccatggcgcccgcgggcccgaccggctcagggcagtgctcgagccaaagtgcagcggccgcggggcatcccgcccgcgcgcgcgcggggctcagggccgg

SEQ ID NO: 8763 - RNA, 2513 nt, Homo sapiens
  source 1..2513: mol_type = other RNA
aagggaggaggagcggaggggccctgagaagcaaagctgaggccctgaggactgagaaaagaaaagttgtaggaagcacaggaagctggggaccggctggaggccctggaggccgaacgttcccgggacttgtaggggtacttgagtgtggtgtccagctgcttgaagctctccttcagtgagtggcactggtagtactccaccaactccaggaggctgtcgaatttcttggcctctgtgatgtggatccagttgtccttctccaccaccttgatgtgcttcacctcatcattgaacttgatgcttattgcaaagcgctcagcctcggcaggccgctccctgatcaggtaggtcccgctggcgtgggacttgagcaggttgtccgtctgctgcctctccatgttacctgcaaaccaggggtatgcagtgtagtcgatctcccgggatggcggccggctgatgggcggccttccatccacagggcagggcttcacagatgagctggggaaataccctgacttcctggtttgtaccagacgaccctcccaccacggagactcagggtcgcccctcagcagctcaagcacgtcgcccgtctggaaggtcagcacaggcttcccgggaggggctgggttgccatggtaattctgcatggccaccatcttgggacctggtcccgctccggaggcgtccagatctgcaggagaagtgaacttgcagggaggtatcacttccaggcactccttgtgtgccccgacgccacacttggtacacatgtatccctggtagaaggtgcccctgaggaacattttgcaggctttgcagttggtggtcttgtcaaacgtgtacatctggaaactgtggtggttggcattggctttgtctggcttgatgtttgacatggccatctcaaactgctccatccacttcctcttcatatcttctgttttgcagaaaaactggaagccctgctttccttgaaggtgaattaggtagaagccgtaggaccacttcttgacgtccttgttgttcatggggtcgtcggtcatcttgtggaacagcagctcgatgatctccttgagctcgtagctgtagcccttccgcttgcagacgatgaccaccttgtcaaacaggaacaagtacctgtcctgcttggtgtggttgactatggaccggactttcagttccccgtcaatctttggtcttccaaattcctccagtttcacttgcaaattttctatagaactctgaaattcgctgattttcctcaaggtctccttgtcccgtttaacttcattgatgtacatcgccaagtcctgcatggcttccagtgcttctttgagctgctgcctctcaggccgttccgcagaatggctcagaagctccttcaagagcaggtggtatttgagcaccctctgcatggggaccaccagcaggtcttgcagcttaaattttccatcctggaccttcagtgtgcactcctcgactttctgcctgaagtcctcccggctggccaggagctggttcagtgtgttctgggcgtgctccatgtggctgcagtactccccgtagatcagaagcctttccttgaaatcgaggaagaccttggccagcgtgctgccccccaccatcacggacacgtcgatggccctcaggaagctgtgatgcaccttgatcaggtcctccaggttaatgaagacagctgccatgtccgccgggctcagcaccagccgcagggggctcatgtagttcttctcaatgtcctccagggtgcggtagtacttggcctcggtctcctggatctccagcaggcagcagttcctcttgtcatcttcagtcatgcccattttctgcatgtatctaatcatgggctgctgcacctccaccttgatgatgtcctcgtagatgtcgtcccctccatcctcacacgggacgcagtcgtagatgtcctcccccaggtcatgctcgtcggccagctcctccaggctgcggtagacgtcatcgtcattctctgtggtctcctctgagggaaaaggcctgatccctttgttctgcgcgatgctgtgcagggagagcctcgacaccgcggagatgacctttccaaagtctcgcacatcgaagaggtcaaaggggtcaaacagctcgctgttccttaatccaaatttatcgtggcagactttcaggaaggtgcgtatgttcttcaaacacagaaactgggacatctgcggccggaagttgatgtccttgaggtcgatggagccgggggagaggttgtgcagcagctggcacagaaggaccccgtcgcgcagcgcctgcgccaggtcgaagaccacggccgagggccacaccacccggtggttgggcggcaggaccttgcaatcgatgagccagcggccgcactgccgccactgctccatggcgcccgcgggcccgaccggctcagggcagtgctcgagccaaagtgcagcggccgcggggcatcccgcccgcgcgcgcgcggggctcagggccgg

SEQ ID NO: 8764 - RNA, 245 nt, Homo sapiens
  source 1..245: mol_type = other RNA
aagggcttcctctctgcaggaccaaatctccccatcctgggaggcccccatccagcatcacattctccaggaagctgtccctgcctgccctgtcttcctctgagtcctcccgaccagtttcacagctcagtaacagaattgaatcctgtccatgccctgccttgcagtgaatcatgaggcctgggaccagcaattgactcctgcctgcctcccccagcatggctggcacagaggatcatgcacgc

SEQ ID NO: 8765 - RNA, 32 nt, Homo sapiens
  source 1..32: mol_type = other RNA
aagggcttcctctctgcaggaccggcctgaat

SEQ ID NO: 8766 - RNA, 5381 nt, Homo sapiens
  source 1..5381: mol_type = other RNA
aaggggctgggggagcacacgaggggtgagacctgccatgatgctctgccctaaaccagcttggtcctcaggcctctgagtactagtttccatatcagccgcttcctgggtttgatgctgatattggcaatgaagctgtatccaggatccaaatccacaggatccaaatccacagaatgttgccatgcagcacccagagaacacgtcgccactctgcgtcctcagctccagatctctacaggggtgtcacctggagacttctggggagcaggcctggatcctgcacagtgaggccagagacccggccacctgggaaccagccactggccccacctttgcctgaggccccacccacctcccactaggtatgggaggggcctcaagtctttcttgctgctccagctctctgggttccttacaaaataaaaccccaaagaggaattcaaaattccacagcccctcataacatggcccagcggtgtccttaactttggtccatgagaacgttcagagtaaggcagcctgtgtgtttacaacattgccggatctgacaactttcagattgttttatcgcaggttagaggagtgaggagatacgagtactcagtaaaagaaagtcagttatctatatgaagtcagtttttatatgtataaaacgtacacgtatttataatgtgtgtgtgtgtgtgtgttggcctgaacaagaccatcagtgtgatcacggccaggtcctcaccaaggcttatggcacagcaggttagaatatgaagttgggacgcacaagtatgaatcccaactaccttctttctcgtctgcataatgggtataatataattaccataagtatgatagttgttgtgaggattaaattagataatacatgtaaaatattcagaccagcagaaagaaacagtagcaggcatgtcccagggcctcctgcatgggaacagccactgacaaatacatgtaaaatactcagaacagtgtctcttaagctcccaagacatccagtattgacagtccagttattgttactgtttcttcgtggtaggtactcatagccatggtgtcgggttctgtacacatccaggaatagtgggacacgtttcatctcagcacaggcataatggttcccttgagccccaggcaagtccccgctcctggcatcatcagctttctaaggctgctgggatccctgagggtcagctcccaggctgagcgtccctgactgcaatcttcctcgtgcctccttcaccaggccaggtccggggcaagaacaaggcagggccacgcacacgtacatacagggaggagtcccccatcggtcctgcagggcacagagtctctccaggtccccgggggttggttcctgtccctgggggtagggatatcatcccagggtcccccagagccagatcgcaatgggctccttttggtctctggattgcagtgtggaatcttccgacgtgaactgcatgcaatgcctgcatcccagacagcatcagggaaggtggctaagaggcagtggcagaatgcactcaggatacacattccagatcccagggtctggtctctgtcagggttggggtccttcacactgttggcaggaagggtgacctctggagccctgagcctgtagtcaagaagtctgactgtgatgaggccgccatgctctgaggaagcccaagccacatgcagaggctgttgtggccaacagcctgggctgaggtcgcaccaacagccagcatcatgtgggggaaacatgagagatgacatcttcagatggttccagctgttgggtccctctcagctgtggagtctttgcagtggaggcctcagactttacaggatggaagcaagtcagccctcctgtgctctgtgcaacttccagacctgcagaaccaggagtatgggaagatggctgtggtaagccgctaagttttggggtgctttgttagaaaacagcagtaactggaacagatggcccagggagagattcagaaaactgtgccaaccaacattctgctcttttcactttcacggatgctgccgggacccaggaggccacaggtcttttgaagagctgtcccctctttagcaggtaatgactcaggctcaggggatgtgggagctgcctctggcagggcagccccctctgcctggtgtgcagggaaccaaagtttgcagcttgtgcaaggcagacctggcctcttcttctcaggcctgaggaaggtgctgctggccaagactgactgtccgtgctggctgagctctggggcggattggccagtcctgctggtgtttccaggcctgatggatgaacagggcctccagagtcatgggtgactacagcaccggctccttgtcaggcccaaacgaaaaccactgctgctgtggcctagcgaccttagagaggagacacaccttgcctttgccacttgtttctggcctgggctctgcactcctctccatcggctactctgactcatcgggagtagacaaagggacagaagtttccaggaaaagggaaagagactgcaggcaggtcctgtggctgtggaagtgggtctggggagccttgacaaggccccccgctccagaggcccacatggccagcagcagccaggccataagcagtcagcagctgccatcattgcctatcagactatctgtttccaaggaagaggctccaggaagccacaacacagacgcctttattctccctgctgagatgccagccagggactaaagggcaggagagaggcctccgaggtatgggtttgcctcccagaatgtgcagccggaaatgaccttgaccttctcccatccccattgtgcacatgggaaaggaaggcccagggaagcggccgatccaaaatgtgtcgttgccagggcaacccggccgcagcgcttgcaagcctgggaaaaagttgttgttcatcacgggggtggacgtttgtcttgttttgatttttcaaaagcctgaaccaactcagctttttaacatgctgctccaggacacggtgctacttgcagacagcctgaggagcagatgcaggcagagctgatggtgttcagacaccctcgccgattccaaaacatccctgctcggctcctgcctcacttctcggcagacagccctgtcctgtctatacccaagacccaagggtcaggccgattcctgtccatttccctcaatcagcaactttggtgtaggaatgaagttaaaagatccgagttcactgtccgcaatatgatgcagttgccctattttctcttccctgaaaagttaggaaactttgacattaaggaagtcgtttgtcatgatttctcattgtcacacaagtttaaccactgtcacatcagaccaaaaggcagcgctgatccagctgtgtgtggcatgactccagacttcttggtgaggaatggagatccttacggcagaattcaagcttcccttgttgcaaaagaaagcaaattccccctccggagaggccttctcagcattggccccagctggaggctctgtccatttaactcctaagcatctcacttgggcatccagtgagatgagcagggaccacagccatctcctaactccccagtctccattgtggggtccaggcctaggtggctcccaggtcctgattcagcttcacagggctgcggtgccctcctcaagccccgctgcttcacccagcctgactagcacggcctccaatccccctgtgcctgccccttctctcaggcacctccagtctgaaggacggtggggcagctcactagtgtgcacctgcaggaggactcagtgagaggagggagacagggcagccaggcactgctgtgctgtgcccaccctgcctactggacaggccgagggcaggccatgggcacccatgctcaggttttaagaagagagagatcattcagagtggaccgagccattcccaccagccattctacatcggcgcccgagaggcagtgcctcttgcgtgtggaggagcacacatgagaactccctggagcactcccaactgtagatcacggcagtcgcagagagccttaggaggcagagggtctacagagctggcaggggaccctcggagtccatgactgtcgctgtgactgggccccgcttccaggctgtgtccgacaaggccaggagggcagcctccacctcaagcctacatcatgcacgctggccccagggggtttctgtgtggaacaccagctgagtacatgaggatgagatggcacaaactgcaagatagaatagcggggaatagtacaaattaaataagccatgaggtgagatcacctcaagaagactggtgagcctaagctttggctccatgatcctgcccctaagttcttaaaaaatgcagaaaaggtgtttaagaaaataagttaattcctggcagtgctggggaaaggtggttgcgacagatcttgcattttccaagatggctaccacaagacctttcatcccacatggcttttctaccaaggggctcagacgctcctcctatccagagttggggtctctccttcctctcctggaaccctggtgggccagtgactacacaaaagtgatgccacgtgactagctgggtcagaaaggccgattccatttctgcctggccctctgggcgagcttattattgacactcagactccatgctatgagacagcccaagccacatggaggtgacacaggcaggtgttccatctgatgcccggataagcagcgcccaaccagtctggctgcaggcccataaaaggagggcatcggaacaggacctgcgcagccaaacccatcaaccctcaggagccatgagaaatgagaataaaatggttgttttaagccattacctttaagagtgattccttactcagcaacagataaccagaacaggatactttcagtggtccagaagttatgaagcagctgggattagtgagaatcaggaaaccatagctccaaattctggaaatggtggctgcttccagttcagtgggagcaggtacaagcgagagaacagggctgcaagtgaccgttaggtgctaagggcctgcatccagaagaccacccgggcccagcctacctggcgacgcattcttgcctctcacctgcaattgctgagggtaaatagatacatcacttacagatgcgtcaacaggaaacctccccctctaagatgagcgcttaacgaagacactacaaacagctgaggaaaacccacagcgagagagagtcaccaaactcaacagctaaaccacctaaagaaagtgagttcttattacaaagaaatggagattttaaaagaagtatgttggtcgggcatggtggctcacacctgtaatcccggcactttgggagg

SEQ ID NO: 8767 - RNA, 5387 nt, Homo sapiens
  source 1..5387: mol_type = other RNA
aaggggctgggggagcacacgaggggtgagacctgccatgatgctctgccctaaaccagcttggtcctcaggcctctgagtactagtttccatatcagccgcttcctgggtttgatgctgatattggcaatgaagctgtatccaggatccaaatccacaggatccaaatccacagaatgttgccatgcagcacccagagaacacgtcgccactctgcgtcctcagctccagatctctacaggggtgtcacctggagacttctggggagcaggcctggatcctgcacagtgaggccagagacccggccacctgggaaccagccactggccccacctttgcctgaggccccacccacctcccactaggtatgggaggggcctcaagtctttcttgctgctccagctctctgggttccttacaaaataaaaccccaaagaggaattcaaaattccacagcccctcataacatggcccagcggtgtccttaactttggtccatgagaacgttcagagtaaggcagcctgtgtgtttacaacattgccggatctgacaactttcagattgttttatcgcaggttagaggagtgaggagatacgagtactcagtaaaagaaagtcagttatctatatgaagtcagtttttatatgtataaaacgtacacgtatttataatgtgtgtgtgtgtgtgtgttggcctgaacaagaccatcagtgtgatcacggccaggtcctcaccaaggcttatggcacagcaggttagaatatgaagttgggacgcacaagtatgaatcccaactaccttctttctcgtctgcataatgggtataatataattaccataagtatgatagttgttgtgaggattaaattagataatacatgtaaaatattcagaccagcagaaagaaacagtagcaggcatgtcccagggcctcctgcatgggaacagccactgacaaatacatgtaaaatactcagaacagtgtctcttaagctcccaagacatccagtattgacagtccagttattgttactgtttcttcgtggtaggtactcatagccatggtgtcgggttctgtacacatccaggaatagtgggacacgtttcatctcagcacaggcataatggttcccttgagccccaggcaagtccccgctcctggcatcatcagctttctaaggctgctgggatccctggatctgagggtcagctcccaggctgagcgtccctgactgcaatcttcctcgtgcctccttcaccaggccaggtccggggcaagaacaaggcagggccacgcacacgtacatacagggaggagtcccccatcggtcctgcagggcacagagtctctccaggtccccgggggttggttcctgtccctgggggtagggatatcatcccagggtcccccagagccagatcgcaatgggctccttttggtctctggattgcagtgtggaatcttccgacgtgaactgcatgcaatgcctgcatcccagacagcatcagggaaggtggctaagaggcagtggcagaatgcactcaggatacacattccagatcccagggtctggtctctgtcagggttggggtccttcacactgttggcaggaagggtgacctctggagccctgagcctgtagtcaagaagtctgactgtgatgaggccgccatgctctgaggaagcccaagccacatgcagaggctgttgtggccaacagcctgggctgaggtcgcaccaacagccagcatcatgtgggggaaacatgagagatgacatcttcagatggttccagctgttgggtccctctcagctgtggagtctttgcagtggaggcctcagactttacaggatggaagcaagtcagccctcctgtgctctgtgcaacttccagacctgcagaaccaggagtatgggaagatggctgtggtaagccgctaagttttggggtgctttgttagaaaacagcagtaactggaacagatggcccagggagagattcagaaaactgtgccaaccaacattctgctcttttcactttcacggatgctgccgggacccaggaggccacaggtcttttgaagagctgtcccctctttagcaggtaatgactcaggctcaggggatgtgggagctgcctctggcagggcagccccctctgcctggtgtgcagggaaccaaagtttgcagcttgtgcaaggcagacctggcctcttcttctcaggcctgaggaaggtgctgctggccaagactgactgtccgtgctggctgagctctggggcggattggccagtcctgctggtgtttccaggcctgatggatgaacagggcctccagagtcatgggtgactacagcaccggctccttgtcaggcccaaacgaaaaccactgctgctgtggcctagcgaccttagagaggagacacaccttgcctttgccacttgtttctggcctgggctctgcactcctctccatcggctactctgactcatcgggagtagacaaagggacagaagtttccaggaaaagggaaagagactgcaggcaggtcctgtggctgtggaagtgggtctggggagccttgacaaggccccccgctccagaggcccacatggccagcagcagccaggccataagcagtcagcagctgccatcattgcctatcagactatctgtttccaaggaagaggctccaggaagccacaacacagacgcctttattctccctgctgagatgccagccagggactaaagggcaggagagaggcctccgaggtatgggtttgcctcccagaatgtgcagccggaaatgaccttgaccttctcccatccccattgtgcacatgggaaaggaaggcccagggaagcggccgatccaaaatgtgtcgttgccagggcaacccggccgcagcgcttgcaagcctgggaaaaagttgttgttcatcacgggggtggacgtttgtcttgttttgatttttcaaaagcctgaaccaactcagctttttaacatgctgctccaggacacggtgctacttgcagacagcctgaggagcagatgcaggcagagctgatggtgttcagacaccctcgccgattccaaaacatccctgctcggctcctgcctcacttctcggcagacagccctgtcctgtctatacccaagacccaagggtcaggccgattcctgtccatttccctcaatcagcaactttggtgtaggaatgaagttaaaagatccgagttcactgtccgcaatatgatgcagttgccctattttctcttccctgaaaagttaggaaactttgacattaaggaagtcgtttgtcatgatttctcattgtcacacaagtttaaccactgtcacatcagaccaaaaggcagcgctgatccagctgtgtgtggcatgactccagacttcttggtgaggaatggagatccttacggcagaattcaagcttcccttgttgcaaaagaaagcaaattccccctccggagaggccttctcagcattggccccagctggaggctctgtccatttaactcctaagcatctcacttgggcatccagtgagatgagcagggaccacagccatctcctaactccccagtctccattgtggggtccaggcctaggtggctcccaggtcctgattcagcttcacagggctgcggtgccctcctcaagccccgctgcttcacccagcctgactagcacggcctccaatccccctgtgcctgccccttctctcaggcacctccagtctgaaggacggtggggcagctcactagtgtgcacctgcaggaggactcagtgagaggagggagacagggcagccaggcactgctgtgctgtgcccaccctgcctactggacaggccgagggcaggccatgggcacccatgctcaggttttaagaagagagagatcattcagagtggaccgagccattcccaccagccattctacatcggcgcccgagaggcagtgcctcttgcgtgtggaggagcacacatgagaactccctggagcactcccaactgtagatcacggcagtcgcagagagccttaggaggcagagggtctacagagctggcaggggaccctcggagtccatgactgtcgctgtgactgggccccgcttccaggctgtgtccgacaaggccaggagggcagcctccacctcaagcctacatcatgcacgctggccccagggggtttctgtgtggaacaccagctgagtacatgaggatgagatggcacaaactgcaagatagaatagcggggaatagtacaaattaaataagccatgaggtgagatcacctcaagaagactggtgagcctaagctttggctccatgatcctgcccctaagttcttaaaaaatgcagaaaaggtgtttaagaaaataagttaattcctggcagtgctggggaaaggtggttgcgacagatcttgcattttccaagatggctaccacaagacctttcatcccacatggcttttctaccaaggggctcagacgctcctcctatccagagttggggtctctccttcctctcctggaaccctggtgggccagtgactacacaaaagtgatgccacgtgactagctgggtcagaaaggccgattccatttctgcctggccctctgggcgagcttattattgacactcagactccatgctatgagacagcccaagccacatggaggtgacacaggcaggtgttccatctgatgcccggataagcagcgcccaaccagtctggctgcaggcccataaaaggagggcatcggaacaggacctgcgcagccaaacccatcaaccctcaggagccatgagaaatgagaataaaatggttgttttaagccattacctttaagagtgattccttactcagcaacagataaccagaacaggatactttcagtggtccagaagttatgaagcagctgggattagtgagaatcaggaaaccatagctccaaattctggaaatggtggctgcttccagttcagtgggagcaggtacaagcgagagaacagggctgcaagtgaccgttaggtgctaagggcctgcatccagaagaccacccgggcccagcctacctggcgacgcattcttgcctctcacctgcaattgctgagggtaaatagatacatcacttacagatgcgtcaacaggaaacctccccctctaagatgagcgcttaacgaagacactacaaacagctgaggaaaacccacagcgagagagagtcaccaaactcaacagctaaaccacctaaagaaagtgagttcttattacaaagaaatggagattttaaaagaagtatgttggtcgggcatggtggctcacacctgtaatcccggcactttgggagg

SEQ ID NO: 8768 - RNA, 3567 nt, Homo sapiens
  source 1..3567: mol_type = other RNA
aaggggctgggggagcacacgaggggtgagacctgccatgatgctctgccctaaaccagcttggtcctcaggcctctgagtactagtttccatatcagccgcttcctgggtttgatgctgatattggcaatgaagctgtatccaggatccaaatccacaggatccaaatccacagaatgttgccatgcagcacccagagaacacgtcgccactctgcgtcctcagctccagatctctacaggggtgtcacctggagacttctggggagcaggcctggatcctgcacagtgaggccagagacccggccacctgggaaccagccactggccccacctttgcctgaggccccacccacctcccactaggtatgggaggggcctcaagtctttcttgctgctccagctctctgggttccttacaaaataaaaccccaaagaggaattcaaaattccacagcccctcataacatggcccagcggtgtccttaactttggtccatgagaacgttcagagtaaggcagcctgtgtgtttacaacattgccggatctgacaactttcagattgttttatcgcaggttagaggagtgaggagatacgagtactcagtaaaagaaagtcagttatctatatgaagtcagtttttatatgtataaaacgtacacgtatttataatgtgtgtgtgtgtgtgtgttggcctgaacaagaccatcagtgtgatcacggccaggtcctcaccaaggcttatggcacagcaggttagaatatgaagttgggacgcacaagtatgaatcccaactaccttctttctcgtctgcataatgggtataatataattaccataagtatgatagttgttgtgaggattaaattagataatacatgtaaaatattcagaccagcagaaagaaacagtagcaggcatgtcccagggcctcctgcatgggaacagccactgacaaatacatgtaaaatactcagaacagtgtctcttaagctcccaagacatccagtattgacagtccagttattgttactgtttcttcgtggtaggtactcatagccatggtgtcgggttctgtacacatccaggaatagtgggacacgtttcatctcagcacaggcataatggttcccttgagccccaggcaagtccccgctcctggcatcatcagctttctaaggctgctgggatccctggatctgagggtcagctcccaggctgagcgtccctgactgcaatcttcctcgtgcctccttcaccaggccaggtccggggcaagaacaaggcagggccacgcacacgtacatacagggaggagtcccccatcggtcctgcagggcacagagtctctccaggtccccgggggttggttcctgtccctgggggtagggatatcatcccagggtcccccagagccagatcgcaatgggctccttttggtctctggattgcagtgtggaatcttccgacgtgaactgcatgcaatgcctgcatcccagacagcatcagggaaggtggctaagaggcagtggcagaatgcactcaggatacacattccagatcccagggtctggtctctgtcagggttggggtccttcacactgttggcaggaagggtgacctcttcccagacggcctccgattcagttctcaagacccggggccttgtcccctcctttgagaagctgcccctcagtggggggcagctccctggcttttccgggctcctccgcccacaggattcaggcacggctcagccagctctggtttcatccaccctgaggggcctgtctgtgcataggcgccctcactaaatgcacaagaagcctttactggtgttgctttgttaaaatgtgactgtcatcatccaattccagtttgcccatctacaaaacaggtataagaagagacagaaggcctagcatacccaaaggtctaggccggtgtgcttggtaaatgagtattattattacttctggatggtcgcaaaatacatgaactcttctcttcacccttcttcagtttcatttaaaaaaaaaaaaaacaggtatgaaatgaaccttagagtcatttatgaccatggccccacagcgaggctacgcagcttgggaccaggcccgtaccagagcgcaggagaacacgacacaaagtgttattgaggccaccgctggcgagagcccccagccagggcaccacctcctgcacgaccagagggaataaagcctgctctgtgcagggcctcctgggcagggtgtctgccccctccaaggccgccagcgcgaagcctgcattcttgcacgcgcacccacgttcacacccagccgggacgtggcactcaccgccctggccggggcctgagccaggactgcagatagagacctggagcctgtttgccttggctgccttctttccctaaagtcctggggatggatttcgatacgctttcttagagcatgttgtcctggacagtgagctacgggtctccactccattgccctgcacagccagcctcctgagctcccccagctccccacaaggaggctttctgccctgccccctcactggcatgaggcccagctccctgctctgccctgactccagctttgttctgcagacctcttcccacccccaccacagccgacgcggtgtctaggctgcggagctgcactctgttcctggctctgccctgggaggtgccccggggcggtctggggtgggcccagcattcagcaaggtccctgcaactttggcctctgcccggtgacctctggcgggtgtagaagagctcatgcttcattgagggggtggggggcaccctgaggaccctgtcaacgtcagctgaaccacaggcatctcgatagatgtaagctgggatgagggctcagcaggctgagacaggcctccagaagagggttgagtaggaagcgatttcttccagaattagttcagcaaacacatgtcatccacttggagcaggagccaggtggagtcacagggccaccaagatgaaggagactgagcccttccctgtgccaggctagtgccacggggatgctggtgggctgggagcccatccttatggaacactctgcctggtggggggggtggcaggcagggggcagtgcacagatgcttgccatgcccccactgctgtcatgttaagcagcaccgagaaaagggcgggggcaccaggtcctgcctctgaaggaggccttggtggcctcaaggagaaggcagctccctgctgctcgccctgcaagaagctggcagaagcagaggcagcccatgtggtccaggtgacacgcagccttacttggtgccacaggccctgcctctgggtggcacattcctttctttgctgcagggatggtagatatggctctgcggagtcagagctgcacttctttaggagtagccccggcctttctaagagatttgctgccctgaggcgcactggtggaaagtgactgcccgcctggtgtgggtgcagatgagtccagtgcctactctgtgtctctcttggaatgtgtgaaatggaaggatgtgacacatccctgtctccttc

SEQ ID NO: 8769 - RNA, 31 nt, Homo sapiens
  source 1..31: mol_type = other RNA
aagggggaaggaaacatggagacaaagtatg

SEQ ID NO: 8770 - RNA, 14680 nt, Homo sapiens
  source 1..14680: mol_type = other RNA
aaggtattgttcagacttatgagcagacaggaactgccagagggcaatggtgtgttttaactggcatctgtttaaggcctttaacacgtgaatcgtctgatcacccatttgcaggatgtcttgagtatacacattcagctgcatgtttggatccccaccagctgtgctcagaaaccccagagtgacttctacgacagacagcacttcacaggcatcgctgtaggactgcagctgtccactgatggcactaatgaccgagctggggagggagtcctgtgccattttgttcttgatgtccataaagagatgttcatagttccagtcgtgtctgtacaccagagtgggtattcccttgaggctcagccggggcttgccctggaggaagcggctgacgatctgccgctgaatcttctccagatcgaactcctgcacggtctctctgccctcctccacctggtactggcagttggagagaatcagtggagtcaggtcccgctccacttcataactgatgacatgcagttcagtgacctcggcggcatccacggaatagctgttgttttccttggagagtttttccacggcgtagacaatttcattgtgtaggcgaatcaagtagctgacgagagcggtagcacagaggcccaggccccgtcggcgtggcaagaggatctcaaactcagtgtccagatccaagtcagtgctgcagtagtctttgggtaggttgatctcaccgttcgtctcaagcgatctcctcagtttgttccatgtggacagaaagactgtgatcctgttgtgaagcagctgcctcaacccatctgagctgtgcttgctgaggaagcctctgatggagctgtattcaacttgctggacgttctggaactgcttcactagatccctttgcaaggccaaaatctcaggcaggaactttaccagcctcagctctgcttccttctgcaggaaatgccagaggatgggcactctttctttgccatttttctgttccacaatgtgctggaggtactcaactgtaattcttttcctgcagctccaaatcttagagcaatggaccacacttttccggggcaggtggggcaggaaggtcactgggtcaccatatattattttggccacagggttagagctgatacgcttatcttggctgatgagattattcatggtgggaagggttttatctagatgctccagttcaggagaaatcacagctgcgatttccttttcccagttgttcctcatttctttagttgacaattctgtgtcaaaatttaaaagccttctgctagagagctggtgctgctcttggagaagcctgcgcaggacgaggtggaccacgccgatggtctcgtcggcactgtgtcccagcatcttggccaactgctccaggtccttcaggatgtgctgctgcagaaagccttttggatccctcactggaggcttaatgatgtttatcagagcctgggaactctgggacgctcccagaagcagagccaagtgagtgagtagccggataaggaggaagaccactgggggcagccctcggtcacatgtcaccacgtctctccgctgcgggttgcccagcacgtggccggtctgcgttctgtctgccttgtctttgaccagatgaaagccgtcccgaggtttgtggtcaatgcctccaatcggcgcatggcagtcaatgcagatgctctgttccatcggcctgccacactctcccacggagcaaggatggccgttgggacaagtgtaccagtggactcgctccagacccttccacctccgagcttgagccagcaagtcttcaggcatggttggaagaaaagcatgcgccatggtggctggggagaaggccagattctttaggggctccaagagttcattctgtccacacagaaggacggctgcagcatgaatggccatttctgtcaccgttccatcaaggttgctgtcactaggccccgccctcaacaatggcacagaattgtccacgagcgatgttgcaaaacggctgatatcaggaggtgaaaggatcttgcattcgccaatgaatttgctcacagcttcacattgctctggcgtggggtggaggcttgcattgtgggatctgtacaaaatagccacctctctaaacagtgttaacaggaagtaggctgactgctggctttggggggtcttgcaggccttcagagcagtcttaatgcccagtggcttgcactcgaggacagctttggccacagcatcacggagagccttgtattcatcgccgtacaccaggtacctatccatctggcctgggtggtcctgccgcagcccctgctgcttgacaacgtccttgggaaacacccactggtgcgggcggccgggcttggagaggccctgcacgaactccatcccccgctggctgctgagcttccgcaccaggtacacccggtgccagtcgttctccacccggatacagaactgcttgacttgctgcaggtagcactgcttctccttggccatctctgggcctccctcaggctccgagaggaaatctgcagctctgtcgaggcagaggcggatccgggccacctcttgcaggtattcaaccgaggcctcgttggcaggctctcggccccggcttgctggagaatatgccttaaggaaacgaccttcctcttctaggtggttcagttcatcatttctggagtaagcactggtcttctcaagtattgaatcctccaggcagttgatgaagagcatgtacagttcagttttatcttcagttatgaatgctttcttttttaacagggtcaaatattcctgaatataatcttttacatcatgaaagctgtacttcaaaagcagtttcagtatcactgagcggatgacaggagtcttatccacaacatcattgaatggagagagagattttgtgtgttcacagtgtctctgggcagcatctcttaagcgccccttttggacgaagaggagagagagcaggctctcaatcacttccttctcaggcggagcgttgtccttgaagcaaatggtggacaccaggtctacgaagaaactgttgcacatctgccggaagcgggcatgcttttcaatggcttccctgtgcgcttgggaaacagctggagagaattcgtctggcaaggcagttaaacagtaggggcatatcatctgctctgaggcaaaccaggccctgaggcagcgcaggcagtgcacgtggtcgcagggcagacagacggggtcctttgcatctcccaggcagatggagcacggctgaatcccaaacctgctgagggtcttgctggctgtctccttgcattcacagagagtgcgcatcacggcctcaaaaggcccgtgcgtcttcacgtcagagttctctcgaagacacttgtctagtaagaagacgtgctcggtcaccagcccctgtaactcggggacgcggctctcggttcctaggagcacgtgctccacgaagagtgcggtggagaaaatccgactccactgggctctgacttccctgatgacagcctgggccaggctcccgctgccttgcatgtgctcatcggagcagatgagctccagcggcatggaaagattcttcaccaactgtagccacgcctggggactgggcttcagggtgtttcttgtcagcatctccgtgcaggccattgcggcaaatgcgtccagggtcatctcacatccagccagctcatggttccaacgggcttccatcaggctgtggagaacctgagggtagatggtcaggattctggaaaagttctgcagacggcttctgaaacgctggtaggcaaggtgcacccacggtaaggaaacctcttcctcgggcgcttctgacgccgctttcagtttcctagtgcaggaccacagagccatctgcagaaactttaattcctcctccgttgacacacgcatggtcaagagaatgaaatccttcaagtaacactgaagaagttcctgctgcggctctccatggagctgggcaagaaacctgcccagaggagtctgctgaaagatgtccacgaacttcttgggcagtccttctgcgtctgtgatgtactgagcctggacccacagctcctccagatagtccttgattttccagctgaaagggacgttgttggaagcgttctcggaaaggttcatgtggttctgcaccacgatgtaggccatctcacctttatgtctttcattattcatcacaagaggaatgttcagaagcatcgtgtcactgaaaataaacatccaaagatctcttgcccagggcggagtatctggcctggtcagtaactctaggttgccgtctctgtcgatgaatgatatcatgctcgccagcagaggggtgacagcaccttggacccgcttccagagggtgtgcctgaatgtgcccgcctcctggagagcgtcctggttgcaggcttcccttgccaaccactccagagggtgaaactggctctcttcttgcttctttaaaaagacactgaggcgcatcttggatacccgcaagaaagaggcgtggcacgcgtcatcctcattcaagaggcccaggaggagcaccaccctccgcatattgcgcgtgcagctctcgttctggtctctgagcatgcccacggcgctctgcacacagcttctcagcagcctggtggtgtccaggatcgacacatcactgcctccgagttcagaggtttcctttcccaccttctcagaactttctgtttccatggcctcctctgccacctctgccacctcccctgatgtgctggcctccgtctccatcgcctcctcatggccgtcttccgcccggtgttccaagcccagctcaggcaagtctccgggcgcgaacagctggctgatggtgacatgctgcagcctggtcacatcagaaaccatgagggtggatctccggaggtcatcgatgtggacagactgccacagccctccgtggaagcccacataggctgttcctcttcccacccgggacagttttgtgatgaaatagacgaagatacggtcctcattttctcgtattttgttgatttcatttataacagaatacttagctgaggcaatgagctgggcgctacggattccatcttcaaaatctgtctgaaaaatgaggattttacatttggctgtattcgttaaacagtttcggacttctttgaggaatgagtactcggtgtcaaactgctgcagccacaggagtgtgggtttcggagccctgcctgtgacctctgattctaaaatttcacagtcgtgacttgttagcagcctggagaaagtggtgatctctgtgaagatggcgtggcgctccaggtctgccgtgtgcaggtgtgcctgaaggaaatctgcaaaggagttgtgcctctgtctgtgaaagtactcctgcgacagccactccgctgcgaacccgcccagcgagtaggcgctcagccggaccacggcatcgggcgtagcgcagttcagcaggatcgatttggcctcctcagacaccttctggtgaagttcctccgtcaaggcccggggaccctgcctctctatgacctgcagcaccacagacgcgcaggcgtccgagtggtagccgatgaagacgtcagaggggctgtatttgtgcctcttctggaaatgatgtgctttgacattgatgaacttctccacccacgcacagagctcctccacgatgctcttctgccatttctccagcaccgtgttgatatccagatagtgcttctccagccggttaatgagggggatgggaaagtgtttgtacacgacgtctttctcttcaatgacaatcaggcggaagttggggtgaacccgacatttgacgcggtgggtccccagaccgaggtccacgtacttctggccgccgaggtggacgtagtactggttgagtgcgtcgtagaggctctcgtagaggttctgcaggttgagaagcaacaccatcttgcctgtttccatgcagatcttcacacgattgatgtttctgcagagctgggtgtactcttggtccttggggaaaccagaaccaaaaataatctccggctgctggtccccctcgaagaatgtctgctgcaggatctgcagtgccacgtagtttttggtcagcacgagtaagtagcgggactcagcatcttcctgctctccacccggcaccttctgagaaggcccaaagatgttctgtttgatcagctgcatggggctgacttcctctgagcacttggcctcgggcaaattggccagaaagatgtccaaagcttggatgtcatccttgccactgaagttcctaaggacagcctgtgcaatgtcttgcggggaaggctttctatttgaagcctttgctgcagcaaagaccattttgatgaggctgtagtagtcacgaagcccgaagaattccttgtcctggcgcttacacaccgtttcgtaggctttggcaaaggacgcaaagtacccttggactcggtcctggacgaggatgtctgaggagcagatgcccttggcgctctctatgagctctgtctcgttggggctgccacgtgacacaaaaatgccccggttcatcttggcagggtcaagggcccagttggagatgcccacgaagccgacctttttgtggggggcgggatcgtcttcaatgcatccgtcttccagcagcgggtgcagagtcttcaggggcattttgggtgagtcttccgccagccccacctcatctaacaccaccacagagacgtactgctgcaggtccttcccctgctgaaagcgggcgcactgccggaaggtgctgatgatgccctgtggggtggagtgcgggctgcactggaaggacaccaggtggacctgcttcaggctgcggaagagatctgagtaggcagccgggccctgcatggcgtctgccacgatggtcttggcgagagacttggagctgccgggcttccccaccaggaagaggggaatcttcagctcgatgcagacgaccatcatgaagacgttctccttcaaggccaagttcttggcgatggttttcctcagaggtacgccgtccagaaaaagatcctgtgcccgtgttatttcatccagaagcagcctgctgtcgtcatacggtttcggaaagaacctggcgatggctttccgatatgagtctttcttttctaaagaggcatggtaacacaccccgatggccagcatcaacgaccagaggacgggatctctctcggtgtgatttttgctgacgctggacttggagagaaaggcattcagctgcgctaagagcatcgcgctgtgctcgtggaaccacctgaaaactttcacacagcgctccacgtccctgaggctgacaaagctgcactcatcttctgttttcctcatgaaaccctgagaggcgcagaggacttctgtgatcacgcgagtcccgttttcatctaggctgatggactcaaccagtctctggacaatctgctggatgtagagcttttcagcaacgtcactcagttgtccaaagtcccacaccagaggaatcaggctcgggggcagagcatggacccggtataccagctgcctcagaggaatggagcccagcctgtcggccgtctcctccatactaaccctgtagcccaaaccagctgactccaaacggcagatcatctcctcagagtgcttccggtatggattgcaggcagctataatatgcaggccagagtcctcagccagaggctggccatccaccatatgatcacacaggacttctttgatacagcttatagcttccgttgtgttggcttcatcaaaaaacaagatggtgtccaactgatgttggtccttattggcgaaggccacattttcagcctccctgactctggagtagatcatgtctgcagttgttcctccgtgcaccttgaccagctttatggtgtcagcattggtaccaccacgccgcaggtcgctaaggaatttaataagcctggttttcccacagccagtttctcccatgatgataaccgggatcccacaccggaaccgcatctcgatggcaaggattttaagcatattgtcggttgtgagctcatacgttttgtcggggtcggtggcctgggggatccctaaggtcaggcagagcctctcaagtttcttgtgtctgggcagtttatcaaagtcgacattgaagggcaccctctggagcagcaggccctggtacaggtccctggtcatgacgtctctcttgatgaccttcccagtcaagtgactgatggcatcgacactgccgttgatgttgggctgcagatggaagccgatgaatgtcatggttgtgtggtcgtcattgaagaaaacgtatgggtgaggctccgactcccacctcttccggagggagaagggcgctagatcttcttccctaaccccatccatggtgaccatgtgcttccccgggctttggtcagaggtgtggagtgatggtgtggcaaaatctcttgccataaagatcatgaaggtcaccacgaacttcttgaagcccctcagtgtgtcgccaataaaactcggattgcagaagagagaggcctcacaatctctgagctgataattcaggaaccgagcaaagttccgaagctctgaccaggatgggtttattaccccgcagtgaaacaggaaatgctggaggcattcctccggggtgccttcgacagagccttcttgatactgaaacgtgtctaggtcttggttttgattgaatcgtcttaaatactggtaaggtctttggaaagtttcgctgcagaactcccacagatccatcccaggctctgtgtcactcctcagggcactcagctccatgtctatcacctctttgggaggcctgcaggtgacttttgggaagatgtcaagaaaactgaactggggtacacgtgtacgcagcgctgaagagctcctcgacggcactgacgtcctcctttccaggatttcaacgatatacaaatggcaggggttccgaagccacattttcccatttatatccattaagtattgtaaaatgaggagcttgaaaagaaacacccaaattccagtctgcactgaggaggtcacgtccaggtgaaagagcacggggaccttctgatactgcgcatccaggaagggcagcagggcgcccaggactcggctctcatccacctgagggtcgatcagtcgaattgttttcagaggcacatttttcacgtttaactgcatcttcattttgtcgtgcaacctcttcacgtacagagactttccaacacctgctcgctccgaggccacgatcccaacacacagccggtcattgaacacggctgccgccgacagggtctgcttcgggacccggtagtgacctgccaggtaggcttggatggcctcgaggggtgcctggggggtgacgaagaccttgtgctggctgaaggcagaggggaggtagcagtgctcccagtccccatcacagaccatgacgagctggtagtcttctcggtgctgctgcgtgcacagattgtggaaaagctcctccgcttggcgtgccacctcgtagctcagctgatctgcgaacagcaggctgtagaccttgtgccccagggagcccagggtcaggcagcggcgcagcaacagtgccacctcctcaaaggtggttgccggggtgcagagcagcacctcatcgtaagtgggcaggggctggcttggggtttgcatgtagacagccagggcggctggcaacacctcggagtggccacagacgacgaggttgggctggccgacctgcagacctctcgggagacaacgctccacgggagacccacccatccctgccaggtgagccagacagtggccaagggtctctaggtcgaggcagtcgggcaggaaggcaggaaggcacctcatggactgctccatgatgatcctcagcttgtccaccaggctgaactctgataagagcatcagcgggagctcttccatgactctcctcatgcggtacctggcggcctcactcccacaccccacagaggcccttaagacatccctcagggtgcagttgcttttgatgaaggatagcatcgttagggcggcatcactcgggggctgcttcctgagctcagtgctcaggtaaaccagctgctctgccgtgtagaagttcaggtaaaagtgctccattcgcttctgggtcacaaatctcttccagctgtcaaggaagtgctccatctgcctgcagagggctgccagcagctcagtgacatctccaccttctttaagctccgtcaccaggtccaagccaaagtccatttggagggacacaccctgcttgggggagcagtaggccatggcgatccacgtcctgaacagcatattcccagcagagtgcaggtcgatgaaggcctggctgagcctctgcacactgcagaagacctctgaaaacctctccacttccgtgttgttacgatccttcttgccagacatcagcatcaacttgttcaaaagctccttcacctcctctaaagagtactctcgtgactcctcgtggctgccagggctctcaggaaggatcaagtgcagaaccgtgtctggggaaatcttttggccacctttgggcgcctggatcacatagatgcctctttggttgatggccgtggccagggtcagggatgagcgttccacagacccatgactctcattcacagtcttcagccattccaagttcctggcggagtcacacagtttcctgggcaggtactggtccttatccagagccttccacagctttttcagatgcttcatgaatgcactgaagtccacgctggggtccagcttaaatagcagggatgcgtagccctgcacagcgtcatggaagcaggccacccggtccacatcaatgtcattctcccccgctgagatggaggccaggtccacaaacaccttcagctcattgatgcctccaagagcctcccggacccagcagatgaactcctttctcagggacagagcctgcagccccttgcaccgggcctcgctgatgtcctggagcagctttttggcctggatgagctcctggttgatctggtccagtgtttcacggcgaaagtcgtcgaagttatcagtaaaatttagtaaagtgttgagaacactgaagtcaccgttcagtcccaggctctctttgacctgcaagatgaccttggctgcgtggacagcctggtgcaggtgatggtattccttgatctgttcgactcggtccttgatccaatctctttggtcctggtggtccacggtgcacatgatcttaagttctgaatccaggtccgtgtatttattcacaaagtccttgaagatgacatcaatctctgcaagggtgacctctcctgactttagatcctggtgcaacttaatgaactttctgtaagaaggctgatacaaatagtcatacacctcttcaagctcaaggatgtgcctttctgattcttcttcgggctcactcagcaactctgcggcttcctggtcctccttaggctcactcagcggctctgcggcttcccgccagaagagctggaagatgtggctgtctctgagcaagtctatcttcccagccatttcttggacctgggagctcaggtggtaatgcgttgccctctgcgagttcgaggaggtggacagtctcactgtcacggtgtcatttaatcttttactgctgaggtcttgtgagtgtcttactgcaagcactccaaagtccacttgtatcagatgtttcacgttcccacacatcttcaggagactatcaacacatcttttctctttctttagaagtaacagttcctcccttctccaatccagtgcttcctccacagcacattgttcatcctggggtgaaagacttttttccctcagttgccagatgtcaagaaactgattcttgtgctttataatcagctccagttgtccaactaaaatcgtgccacttaggaggtcaccaacaactttcgtcaacacagagtcggcaacagctatcagcctcttggcatcctctgtgacatttgctagtattttctcgtcggttccacacaatctgaagacgtgcttgacatctgccaacgtgagcagatgctttaaaatgtcatcgaagttgtccgcggtcctaggccaggacttagtgatcacagcagacaagacgatgccaaatttccgcaaatcagagtaagagaacccctgaaggatactggtctgagactggcaggctgagctcacggcttcaatgatgcatttctcgaaggtcttggccacactgtcctctaagcctttggtgtcccagcaactattgcagtaggcagtgatctgggagaggggttcctcctttgtgagcctccattccatgtctcccagcaacgactccttccagccatgctccgcggggaattggatttccaccagccgcctccagacctcaatttccttgacgtatgtgaatgaggcacctgaagatgtgagcatgttctttgtaaaaacttctcggagccaccttttcgtagcagcaagggtcccttggaagactgtttggactgaattatttccagtttcatctctctgtcctgcagaatccaccagagatagaagtctaatcattctgcagacaatctcggcagataaggctggcagctcgtaaaacttaagtagctttgtgctgctgcagatggcttcatgcagtttcagacacacagtcaggtaggatggtgacaaggcctcctcgggaatcttgtcccggtaagtgtccaggagtcgcaacagcatttctaaaatgttctgaacgttctgaacatcctgaacatcctgcgtattcaagacttgctcaagtcccggaagccggtagtaaatccctgaaagacagtccaggatatgagcaggaaaacgacccaggtgctcaatgaagttttccatatacataaccaggtgactcagaggtagcagactaaaccaggaccggaagagaggctcgtctatgctcagcaaatgctgcttctctctcataaactgaagtagggaactcgtatctagcatttgttcccggaacggtgagaaggagagtccctccagagcggcccaggtgtcctcaggctgtctccaggcatccttgtgccgcggggccagctccatacagcagtgcaggacaggcagggcgcccagccaggtgtacgtccttgtgtccatgcatctttggcacaggttcaccaggtacagccgccagctctgaggtatcccaaggatgtggcttaggtcacggtgaaactcatctggtgagctggcatctgaggttaggaggtgacacaaccagtccaggctgccttctaataaaagctcaattttttccactacaaaaaggacaatcaggcctgttttcagtttactcctcactgggcagtccacaggcaaaaagtccgtgctttttccgtccggcaatggtaccacgtgttttttcagatgttgccacaggtatctcttcacctctttctccctgtactgcaaatcggtccacagctgtgcctgtccttcataaatcataggctgttgcaggacaaagcaaaactgctcgaactgggtgaagaagctgttcaggttgatggtgtcccaggtctgcaggatgctgaaggtgctgtccagcatgagcgcagcggcaatctgcttccccttcaccaggtccttcctcggcccgtctgtgatgtggttcatgactttctggagtctcccatgaggcttcatataaactatgtcatagtactgatgccagtctcctgagcccagaagtgaagattttatgaacagacagcggttgacgtactcgcccttcttctgctggtgcttgtaaatgaactcatactcaaaagattccccattataaatgacgtacttgtaaggaatgtatttatctaggtgcttcttggaaatgcagacaatgccttcaacaagaacgcggtcatgacccaagtctctggtgtagtgcagctcacagatattgctgtcccattttgactccccaaattcttctcctcctctgatgaagactttatggaggtcaggattgaatgggaaatgaagagagatgatggcgtggaagaacacggtgactcctccacccgggctcagcgtgcttgccttcacttcctggacatctgcttcctggtttttttgctccttctcgtttttcacagcagctgcacttctgttcttcccctctggcttcttgaggtcttcaggctccccttgttcattcttaccgactttttcttcagcagcagccatctcgtccttggtcttggtctcagcttccgctgaagtcggtttcctgactctctctccgctggaatgtgagcaccccgaaggccagagctttgtctgaatcatggctatatccccagcacttaaatatttgctgaataattaaatgaaagaggcgcagccgtgggcaggagagggcctcctggagccggcaggcaggaaggagacgcacctggcagtgtgttttgaaaggaggagtggttgctggtggctgtttcattctctgggtcttctctttcatttccttcccggcccctttaactgcattggctggctcagctacagcatcaactgccatagaggctgaggcccctgcctgttgctcggtggt

SEQ ID NO: 8771 - RNA, 15898 nt, Homo sapiens
  source 1..15898: mol_type = other RNA
aaggtattgttcagacttatgagcagacaggaactgccagagggcaatggtgtgttttaactggcatctgtttaaggcctttaacacgtgaatcgtctgatcacccatttgcaggatgtcttgagtatacacattcagctgcatgtttggatccccaccagctgtgctcagaaaccccagagtgacttctacgacagacagcacttcacaggcatcgctgtaggactgcagctgtccactgatggcactaatgaccgagctggggagggagtcctgtgccattttgttcttgatgtccataaagagatgttcatagttccagtcgtgtctgtacaccagagtgggtattcccttgaggctcagccggggcttgccctggaggaagcggctgacgatctgccgctgaatcttctccagatcgaactcctgcacggtctctctgccctcctccacctggtactggcagttggagagaatcagtggagtcaggtcccgctccacttcataactgatgacatgcagttcagtgacctcggcggcatccacggaatagctgttgttttccttggagagtttttccacggcgtagacaatttcattgtgtaggcgaatcaagtagctgacgagagcggtagcacagaggcccaggccccgtcggcgtggcaagaggatctcaaactcagtgtccagatccaagtcagtgctgcagtagtctttgggtaggttgatctcaccgttcgtctcaagcgatctcctcagtttgttccatgtggacagaaagactgtgatcctgttgtgaagcagctgcctcaacccatctgagctgtgcttgctgaggaagcctctgatggagctgtattcaacttgctggacgttctggaactgcttcactagatccctttgcaaggccaaaatctcaggcaggaactttaccagcctcagctctgcttccttctgcaggaaatgccagaggatgggcactctttctttgccatttttctgttccacaatgtgctggaggtactcaactgtaattcttttcctgcagctccaaatcttagagcaatggaccacacttttccggggcaggtggggcaggaaggtcactgggtcaccatatattattttggccacagggttagagctgatacgcttatcttggctgatgagattattcatggtgggaagggttttatctagatgctccagttcaggagaaatcacagctgcgatttccttttcccagttgttcctcatttctttagttgacaattctgtgtcaaaatttaaaagccttctgctagagagctggtgctgctcttggagaagcctgcgcaggacgaggtggaccacgccgatggtctcgtcggcactgtgtcccagcatcttggccaactgctccaggtccttcaggatgtgctgctgcagaaagccttttggatccctcactggaggcttaatgatgtttatcagagcctgggaactctgggacgctcccagaagcagagccaagtgagtgagtagccggataaggaggaagaccactgggggcagccctcggtcacatgtcaccacgtctctccgctgcgggttgcccagcacgtggccggtctgcgttctgtctgccttgtctttgaccagatgaaagccgtcccgaggtttgtggtcaatgcctccaatcggcgcatggcagtcaatgcagatgctctgttccatcggcctgccacactctcccacggagcaaggatggccgttgggacaagtgtaccagtggactcgctccagacccttccacctccgagcttgagccagcaagtcttcaggcatggttggaagaaaagcatgcgccatggtggctggggagaaggccagattctttaggggctccaagagttcattctgtccacacagaaggacggctgcagcatgaatggccatttctgtcaccgttccatcaaggttgctgtcactaggccccgccctcaacaatggcacagaattgtccacgagcgatgttgcaaaacggctgatatcaggaggtgaaaggatcttgcattcgccaatgaatttgctcacagcttcacattgctctggcgtggggtggaggcttgcattgtgggatctgtacaaaatagccacctctctaaacagtgttaacaggaagtaggctgactgctggctttggggggtcttgcaggccttcagagcagtcttaatgcccagtggcttgcactcgaggacagctttggccacagcatcacggagagccttgtattcatcgccgtacaccaggtacctatccatctggcctgggtggtcctgccgcagcccctgctgcttgacaacgtccttgggaaacacccactggtgcgggcggccgggcttggagaggccctgcacgaactccatcccccgctggctgctgagcttccgcaccaggtacacccggtgccagtcgttctccacccggatacagaactgcttgacttgctgcaggtagcactgcttctccttggccatctctgggcctccctcaggctccgagaggaaatctgcagctctgtcgaggcagaggcggatccgggccacctcttgcaggtattcaaccgaggcctcgttggcaggctctcggccccggcttgctggagaatatgccttaaggaaacgaccttcctcttctaggtggttcagttcatcatttctggagtaagcactggtcttctcaagtattgaatcctccaggcagttgatgaagagcatgtacagttcagttttatcttcagttatgaatgctttcttttttaacagggtcaaatattcctgaatataatcttttacatcatgaaagctgtacttcaaaagcagtttcagtatcactgagcggatgacaggagtcttatccacaacatcattgaatggagagagagattttgtgtgttcacagtgtctctgggcagcatctcttaagcgccccttttggacgaagaggagagagagcaggctctcaatcacttccttctcaggcggagcgttgtccttgaagcaaatggtggacaccaggtctacgaagaaactgttgcacatctgccggaagcgggcatgcttttcaatggcttccctgtgcgcttgggaaacagctggagagaattcgtctggcaaggcagttaaacagtaggggcatatcatctgctctgaggcaaaccaggccctgaggcagcgcaggcagtgcacgtggtcgcagggcagacagacggggtcctttgcatctcccaggcagatggagcacggctgaatcccaaacctgctgagggtcttgctggctgtctccttgcattcacagagagtgcgcatcacggcctcaaaaggcccgtgcgtcttcacgtcagagttctctcgaagacacttgtctagtaagaagacgtgctcggtcaccagcccctgtaactcggggacgcggctctcggttcctaggagcacgtgctccacgaagagtgcggtggagaaaatccgactccactgggctctgacttccctgatgacagcctgggccaggctcccgctgccttgcatgtgctcatcggagcagatgagctccagcggcatggaaagattcttcaccaactgtagccacgcctggggactgggcttcagggtgtttcttgtcagcatctccgtgcaggccattgcggcaaatgcgtccagggtcatctcacatccagccagctcatggttccaacgggcttccatcaggctgtggagaacctgagggtagatggtcaggattctggaaaagttctgcagacggcttctgaaacgctggtaggcaaggtgcacccacggtaaggaaacctcttcctcgggcgcttctgacgccgctttcagtttcctagtgcaggaccacagagccatctgcagaaactttaattcctcctccgttgacacacgcatggtcaagagaatgaaatccttcaagtaacactgaagaagttcctgctgcggctctccatggagctgggcaagaaacctgcccagaggagtctgctgaaagatgtccacgaacttcttgggcagtccttctgcgtctgtgatgtactgagcctggacccacagctcctccagatagtccttgattttccagctgaaagggacgttgttggaagcgttctcggaaaggttcatgtggttctgcaccacgatgtaggccatctcacctttatgtctttcattattcatcacaagaggaatgttcagaagcatcgtgtcactgaaaataaacatccaaagatctcttgcccagggcggagtatctggcctggtcagtaactctaggttgccgtctctgtcgatgaatgatatcatgctcgccagcagaggggtgacagcaccttggacccgcttccagagggtgtgcctgaatgtgcccgcctcctggagagcgtcctggttgcaggcttcccttgccaaccactccagagggtgaaactggctctcttcttgcttctttaaaaagacactgaggcgcatcttggatacccgcaagaaagaggcgtggcacgcgtcatcctcattcaagaggcccaggaggagcaccaccctccgcatattgcgcgtgcagctctcgttctggtctctgagcatgcccacggcgctctgcacacagcttctcagcagcctggtggtgtccaggatcgacacatcactgcctccgagttcagaggtttcctttcccaccttctcagaactttctgtttccatggcctcctctgccacctctgccacctcccctgatgtgctggcctccgtctccatcgcctcctcatggccgtcttccgcccggtgttccaagcccagctcaggcaagtctccgggcgcgaacagctggctgatggtgacatgctgcagcctggtcacatcagaaaccatgagggtggatctccggaggtcatcgatgtggacagactgccacagccctccgtggaagcccacataggctgttcctcttcccacccgggacagttttgtgatgaaatagacgaagatacggtcctcattttctcgtattttgttgatttcatttataacagaatacttagctgaggcaatgagctgggcgctacggattccatcttcaaaatctgtctgaaaaatgaggattttacatttggctgtattcgttaaacagtttcggacttctttgaggaatgagtactcggtgtcaaactgctgcagccacaggagtgtgggtttcggagccctgcctgtgacctctgattctaaaatttcacagtcgtgacttgttagcagcctggagaaagtggtgatctctgtgaagatggcgtggcgctccaggtctgccgtgtgcaggtgtgcctgaaggaaatctgcaaaggagttgtgcctctgtctgtgaaagtactcctgcgacagccactccgctgcgaacccgcccagcgagtaggcgctcagccggaccacggcatcgggcgtagcgcagttcagcaggatcgatttggcctcctcagacaccttctggtgaagttcctccgtcaaggcccggggaccctgcctctctatgacctgcagcaccacagacgcgcaggcgtccgagtggtagccgatgaagacgtcagaggggctgtatttgtgcctcttctggaaatgatgtgctttgacattgatgaacttctccacccacgcacagagctcctccacgatgctcttctgccatttctccagcaccgtgttgatatccagatagtgcttctccagccggttaatgagggggatgggaaagtgtttgtacacgacgtctttctcttcaatgacaatcaggcggaagttggggtgaacccgacatttgacgcggtgggtccccagaccgaggtccacgtacttctggccgccgaggtggacgtagtactggttgagtgcgtcgtagaggctctcgtagaggttctgcaggttgagaagcaacaccatcttgcctgtttccatgcagatcttcacacgattgatgtttctgcagagctgggtgtactcttggtccttggggaaaccagaaccaaaaataatctccggctgctggtccccctcgaagaatgtctgctgcaggatctgcagtgccacgtagtttttggtcagcacgagtaagtagcgggactcagcatcttcctgctctccacccggcaccttctgagaaggcccaaagatgttctgtttgatcagctgcatggggctgacttcctctgagcacttggcctcgggcaaattggccagaaagatgtccaaagcttggatgtcatccttgccactgaagttcctaaggacagcctgtgcaatgtcttgcggggaaggctttctatttgaagcctttgctgcagcaaagaccattttgatgaggctgtagtagtcacgaagcccgaagaattccttgtcctggcgcttacacaccgtttcgtaggctttggcaaaggacgcaaagtacccttggactcggtcctggacgaggatgtctgaggagcagatgcccttggcgctctctatgagctctgtctcgttggggctgccacgtgacacaaaaatgccccggttcatcttggcagggtcaagggcccagttggagatgcccacgaagccgacctttttgtggggggcgggatcgtcttcaatgcatccgtcttccagcagcgggtgcagagtcttcaggggcattttgggtgagtcttccgccagccccacctcatctaacaccaccacagagacgtactgctgcaggtccttcccctgctgaaagcgggcgcactgccggaaggtgctgatgatgccctgtggggtggagtgcgggctgcactggaaggacaccaggtggacctgcttcaggctgcggaagagatctgagtaggcagccgggccctgcatggcgtctgccacgatggtcttggcgagagacttggagctgccgggcttccccaccaggaagaggggaatcttcagctcgatgcagacgaccatcatgaagacgttctccttcaaggccaagttcttggcgatggttttcctcagaggtacgccgtccagaaaaagatcctgtgcccgtgttatttcatccagaagcagcctgctgtcgtcatacggtttcggaaagaacctggcgatggctttccgatatgagtctttcttttctaaagaggcatggtaacacaccccgatggccagcatcaacgaccagaggacgggatctctctcggtgtgatttttgctgacgctggacttggagagaaaggcattcagctgcgctaagagcatcgcgctgtgctcgtggaaccacctgaaaactttcacacagcgctccacgtccctgaggctgacaaagctgcactcatcttctgttttcctcatgaaaccctgagaggcgcagaggacttctgtgatcacgcgagtcccgttttcatctaggctgatggactcaaccagtctctggacaatctgctggatgtagagcttttcagcaacgtcactcagttgtccaaagtcccacaccagaggaatcaggctcgggggcagagcatggacccggtataccagctgcctcagaggaatggagcccagcctgtcggccgtctcctccatactaaccctgtagcccaaaccagctgactccaaacggcagatcatctcctcagagtgcttccggtatggattgcaggcagctataatatgcaggccagagtcctcagccagaggctggccatccaccatatgatcacacaggacttctttgatacagcttatagcttccgttgtgttggcttcatcaaaaaacaagatggtgtccaactgatgttggtccttattggcgaaggccacattttcagcctccctgactctggagtagatcatgtctgcagttgttcctccgtgcaccttgaccagctttatggtgtcagcattggtaccaccacgccgcaggtcgctaaggaatttaataagcctggttttcccacagccagtttctcccatgatgataaccgggatcccacaccggaaccgcatctcgatggcaaggattttaagcatattgtcggttgtgagctcatacgttttgtcggggtcggtggcctgggggatccctaaggtcaggcagagcctctcaagtttcttgtgtctgggcagtttatcaaagtcgacattgaagggcaccctctggagcagcaggccctggtacaggtccctggtcatgacgtctctcttgatgaccttcccagtcaagtgactgatggcatcgacactgccgttgatgttgggctgcagatggaagccgatgaatgtcatggttgtgtggtcgtcattgaagaaaacgtatgggtgaggctccgactcccacctcttccggagggagaagggcgctagatcttcttccctaaccccatccatggtgaccatgtgcttccccgggctttggtcagaggtgtggagtgatggtgtggcaaaatctcttgccataaagatcatgaaggtcaccacgaacttcttgaagcccctcagtgtgtcgccaataaaactcggattgcagaagagagaggcctcacaatctctgagctgataattcaggaaccgagcaaagttccgaagctctgaccaggatgggtttattaccccgcagtgaaacaggaaatgctggaggcattcctccggggtgccttcgacagagccttcttgatactgaaacgtgtctaggtcttggttttgattgaatcgtcttaaatactggtaaggtctttggaaagtttcgctgcagaactcccacagatccatcccaggctctgtgtcactcctcagggcactcagctccatgtctatcacctctttgggaggcctgcaggtgacttttgggaagatgtcaagaaaactgaactggggtacacgtgtacgcagcgctgaagagctcctcgacggcactgacgtcctcctttccaggatttcaacgatatacaaatggcaggggttccgaagccacattttcccatttatatccattaagtattgtaaaatgaggagcttgaaaagaaacacccaaattccagtctgcactgaggaggtcacgtccaggtgaaagagcacggggaccttctgatactgcgcatccaggaagggcagcagggcgcccaggactcggctctcatccacctgagggtcgatcagtcgaattgttttcagaggcacatttttcacgtttaactgcatcttcattttgtcgtgcaacctcttcacgtacagagactttccaacacctgctcgctccgaggccacgatcccaacacacagccggtcattgaacacggctgccgccgacagggtctgcttcgggacccggtagtgacctgccaggtaggcttggatggcctcgaggggtgcctggggggtgacgaagaccttgtgctggctgaaggcagaggggaggtagcagtgctcccagtccccatcacagaccatgacgagctggtagtcttctcggtgctgctgcgtgcacagattgtggaaaagctcctccgcttggcgtgccacctcgtagctcagctgatctgcgaacagcaggctgtagaccttgtgccccagggagcccagggtcaggcagcggcgcagcaacagtgccacctcctcaaaggtggttgccggggtgcagagcagcacctcatcgtaagtgggcaggggctggcttggggtttgcatgtagacagccagggcggctggcaacacctcggagtggccacagacgacgaggttgggctggccgacctgcagacctctcgggagacaacgctccacgggagacccacccatccctgccaggtgagccagacagtggccaagggtctctaggtcgaggcagtcgggcaggaaggcaggaaggcacctcatggactgctccatgatgatcctcagcttgtccaccaggctgaactctgataagagcatcagcgggagctcttccatgactctcctcatgcggtacctggcggcctcactcccacaccccacagaggcccttaagacatccctcagggtgcagttgcttttgatgaaggatagcatcgttagggcggcatcactcgggggctgcttcctgagctcagtgctcaggtaaaccagctgctctgccgtgtagaagttcaggtaaaagtgctccattcgcttctgggtcacaaatctcttccagctgtcaaggaagtgctccatctgcctgcagagggctgccagcagctcagtgacatctccaccttctttaagctccgtcaccaggtccaagccaaagtccatttggagggacacaccctgcttgggggagcagtaggccatggcgatccacgtcctgaacagcatattcccagcagagtgcaggtcgatgaaggcctggctgagcctctgcacactgcagaagacctctgaaaacctctccacttccgtgttgttacgatccttcttgccagacatcagcatcaacttgttcaaaagctccttcacctcctctaaagagtactctcgtgactcctcgtggctgccagggctctcaggaaggatcaagtgcagaaccgtgtctggggaaatcttttggccacctttgggcgcctggatcacatagatgcctctttggttgatggccgtggccagggtcagggatgagcgttccacagacccatgactctcattcacagtcttcagccattccaagttcctggcggagtcacacagtttcctgggcaggtactggtccttatccagagccttccacagctttttcagatgcttcatgaatgcactgaagtccacgctggggtccagcttaaatagcagggatgcgtagccctgcacagcgtcatggaagcaggccacccggtccacatcaatgtcattctcccccgctgagatggaggccaggtccacaaacaccttcagctcattgatgcctccaagagcctcccggacccagcagatgaactcctttctcagggacagagcctgcagccccttgcaccgggcctcgctgatgtcctggagcagctttttggcctggatgagctcctggttgatctggtccagtgtttcacggcgaaagtcgtcgaagttatcagtaaaatttagtaaagtgttgagaacactgaagtcaccgttcagtcccaggctctctttgacctgcaagatgaccttggctgcgtggacagcctggtgcaggtgatggtattccttgatctgttcgactcggtccttgatccaatctctttggtcctggtggtccacggtgcacatgatcttaagttctgaatccaggtccgtgtatttattcacaaagtccttgaagatgacatcaatctctgcaagggtgacctctcctgactttagatcctggtgcaacttaatgaactttctgtaagaaggctgatacaaatagtcatacacctcttcaagctcaaggatgtgcctttctgattcttcttcgggctcactcagcaactctgcggcttcctggtcctccttaggctcactcagcggctctgcggcttcccgccagaagagctggaagatgtggctgtctctgagcaagtctatcttcccagccatttcttggacctgggagctcaggtggtaatgcgttgccctctgcgagttcgaggaggtggacagtctcactgtcacggtgtcatttaatcttttactgctgaggtcttgtgagtgtcttactgcaagcactccaaagtccacttgtatcagatgtttcacgttcccacacatcttcaggagactatcaacacatcttttctctttctttagaagtaacagttcctcccttctccaatccagtgcttcctccacagcacattgttcatcctggggtgaaagacttttttccctcagttgccagatgtcaagaaactgattcttgtgctttataatcagctccagttgtccaactaaaatcgtgccacttaggaggtcaccaacaactttcgtcaacacagagtcggcaacagctatcagcctcttggcatcctctgtgacatttgctagtattttctcgtcggttccacacaatctgaagacgtgcttgacatctgccaacgtgagcagatgctttaaaatgtcatcgaagttgtccgcggtcctaggccaggacttagtgatcacagcagacaagacgatgccaaatttccgcaaatcagagtaagagaacccctgaaggatactggtctgagactggcaggctgagctcacggcttcaatgatgcatttctcgaaggtcttggccacactgtcctctaagcctttggtgtcccagcaactattgcagtaggcagtgatctgggagaggggttcctcctttgtgagcctccattccatgtctcccagcaacgactccttccagccatgctccgcggggaattggatttccaccagccgcctccagacctcaatttccttgacgtatgtgaatgaggcacctgaagatgtgagcatgttctttgtaaaaacttctcggagccaccttttcgtagcagcaagggtcccttggaagactgtttggactgaattatttccagtttcatctctctgtcctgcagaatccaccagagatagaagtctaatcattctgcagacaatctcggcagataaggctggcagctcgtaaaacttaagtagctttgtgctgctgcagatggcttcatgcagtttcagacacacagtcaggtaggatggtgacaaggcctcctcgggaatcttgtcccggtaagtgtccaggagtcgcaacagcatttctaaaatgttctgaacgttctgaacatcctgaacatcctgcgtattcaagacttgctcaagtcccggaagccggtagtaaatccctgaaagacagtccaggatatgagcaggaaaacgacccaggtgctcaatgaagttttccatatacataaccaggtgactcagaggtagcagactaaaccaggaccggaagagaggctcgtctatgctcagcaaatgctgcttctctctcataaactgaagtagggaactcgtatctagcatttgttcccggaacggtgagaaggagagtccctccagagcggcccaggtgtcctcaggctgtctccaggcatccttgtgccgcggggccagctccatacagcagtgcaggacaggcagggcgcccagccaggtgtacgtccttgtgtccatgcatctttggcacaggttcaccaggtacagccgccagctctgaggtatcccaaggatgtggcttaggtcacggtgaaactcatctggtgagctggcatctgaggttaggaggtgacacaaccagtccaggctgccttctaataaaagctcaattttttccactacaaaaaggacaatcaggcctgttttcagtttactcctcactgggcagtccacaggcaaaaagtccgtgctttttccgtccggcaatggtaccacgtgttttttcagatgttgccacaggtatctcttcacctctttctccctgtactgcaaatcggtccacagctgtgcctgtccttcataaatcataggctgttgcaggacaaagcaaaactgctcgaactgggtgaagaagctgttcaggttgatggtgtcccaggtctgcaggatgctgaaggtgctgtccagcatgagcgcagcggcaatctgcttccccttcaccaggtccttcctcggcccgtctgtgatgtggttcatgactttctggagtctcccatgaggcttcatataaactatgtcatagtactgatgccagtctcctgagcccagaagtgaagattttatgaacagacagcggttgacgtactcgcccttcttctgctggtgcttgtaaatgaactcatactcaaaagattccccattataaatgacgtacttgtaaggaatgtatttatctaggtgcttcttggaaatgcagacaatgccttcaacaagaacgcggtcatgacccaagtctctggtgtagtgcagctcacagatattgctgtcccattttgactccccaaattcttctcctcctctgatgaagactttatggaggtcaggattgaatgggaaatgaagagagatgatggcgtggaagaacacggtgactcctccacccgggctcagcgtgcttgccttcacttcctggacatctgcttcctggtttttttgctccttctcgtttttcacagcagctgcacttctgttcttcccctctggcttcttgaggtcttcaggctccccttgttcattcttaccgactttttcttcagcagcagccatctcgtccttggtcttggtctcagcttcctggcagtgtgttttgaaaggaggagtggttgctggtggctgtttcattctctgggtcttctctttcatttccttcccggcccctttaactgcattggctggctcagctacagcatcaactgccatagaggctgaggcccctgcctgttgctcggtggtctgcagttctgtcccgggctcagagctgcctccttttgactcaggcaacaggagctcctgggcagcatcttcagtcctagaatggccttcaccagcagaggtggggggaccggtcccctcctgggacaggcctctgcccccagaggggatggaagcgtcctggtcctccccttccgtgtggtcctggaattgcgggctgctctgagcctcacttcctgtggccactcctgcctctcccaaagcctgggcctgcagggggctgtcgccaacctcggtgggcgcggagaggccgtcaccctccagtggcgtggtggctgtgcctgggggctggctcggctggccagtggggccactctgctgggcttggctgtggggcagggctgtgtcctgaggccacgggtttgaaagcaaagtcaggtgacaggggctggcaggagaaaggggcaaggaagccagctctgaggaagcggacttgttccccttctttttcttcttccttttcttctttttgctctgctcacagtctgcagaaggcacgctggcggcctcaagcggggctgcatcctgcttccttctcttgctgggtatggcattagcagcttcccattcatcggatatgaggtctacagcagcatctaccaaaacctctgatgtagctccttcttggacggtccaggaggctttggaacagggctcctcggggttttcttgccaactgtctgagcccgggaacaagcacgggcccccttcctccttcagctcctgcccacactccatttcaccctccgaggccgacgccattgtggagttattgttctcagaatctgctatgggggctgcaggaggcagcctctctccgcactggctgcagaacttgggggtttcctccttggagacatgctggcacgaaggacactccatgggtcctgctgggactgccctgcagatccagaagcaagagcaggagtcgctggcagcctgctatatactacatgtcctgtcacgtgaccacggcttcagtttcattttcctggccttgagccccgcgctcgggcgacttcgccaagtcggaaggacgctgcgcggtgcggttcagacggggcgatgcctccctcgtaaaagttaggagtctgtttttgcaacttcacttttccgttgttgccattcgtacaggcgcaggattcccgggcggacctgcaggcccgggtccggctgtccccttccactacaccccccgtgccccggccacttcccgggggcagcactgccggggcgcaaagcctcctccgcgctctgcgctccggggatgtcgccggggtcccaggcgtgcccgctgcccccaccccgacccctcccgcagccggggaacagggtcagtgggcgccgcgggcggggctgg

SEQ ID NO: 8772 - RNA, 15611 nt, Homo sapiens
  source 1..15611: mol_type = other RNA
aaggtattgttcagacttatgagcagacaggaactgccagagggcaatggtgtgttttaactggcatctgtttaaggcctttaacacgtgaatcgtctgatcacccatttgcaggatgtcttgagtatacacattcagctgcatgtttggatccccaccagctgtgctcagaaaccccagagtgacttctacgacagacagcacttcacaggcatcgctgtaggactgcagctgtccactgatggcactaatgaccgagctggggagggagtcctgtgccattttgttcttgatgtccataaagagatgttcatagttccagtcgtgtctgtacaccagagtgggtattcccttgaggctcagccggggcttgccctggaggaagcggctgacgatctgccgctgaatcttctccagatcgaactcctgcacggtctctctgccctcctccacctggtactggcagttggagagaatcagtggagtcaggtcccgctccacttcataactgatgacatgcagttcagtgacctcggcggcatccacggaatagctgttgttttccttggagagtttttccacggcgtagacaatttcattgtgtaggcgaatcaagtagctgacgagagcggtagcacagaggcccaggccccgtcggcgtggcaagaggatctcaaactcagtgtccagatccaagtcagtgctgcagtagtctttgggtaggttgatctcaccgttcgtctcaagcgatctcctcagtttgttccatgtggacagaaagactgtgatcctgttgtgaagcagctgcctcaacccatctgagctgtgcttgctgaggaagcctctgatggagctgtattcaacttgctggacgttctggaactgcttcactagatccctttgcaaggccaaaatctcaggcaggaactttaccagcctcagctctgcttccttctgcaggaaatgccagaggatgggcactctttctttgccatttttctgttccacaatgtgctggaggtactcaactgtaattcttttcctgcagctccaaatcttagagcaatggaccacacttttccggggcaggtggggcaggaaggtcactgggtcaccatatattattttggccacagggttagagctgatacgcttatcttggctgatgagattattcatggtgggaagggttttatctagatgctccagttcaggagaaatcacagctgcgatttccttttcccagttgttcctcatttctttagttgacaattctgtgtcaaaatttaaaagccttctgctagagagctggtgctgctcttggagaagcctgcgcaggacgaggtggaccacgccgatggtctcgtcggcactgtgtcccagcatcttggccaactgctccaggtccttcaggatgtgctgctgcagaaagccttttggatccctcactggaggcttaatgatgtttatcagagcctgggaactctgggacgctcccagaagcagagccaagtgagtgagtagccggataaggaggaagaccactgggggcagccctcggtcacatgtcaccacgtctctccgctgcgggttgcccagcacgtggccggtctgcgttctgtctgccttgtctttgaccagatgaaagccgtcccgaggtttgtggtcaatgcctccaatcggcgcatggcagtcaatgcagatgctctgttccatcggcctgccacactctcccacggagcaaggatggccgttgggacaagtgtaccagtggactcgctccagacccttccacctccgagcttgagccagcaagtcttcaggcatggttggaagaaaagcatgcgccatggtggctggggagaaggccagattctttaggggctccaagagttcattctgtccacacagaaggacggctgcagcatgaatggccatttctgtcaccgttccatcaaggttgctgtcactaggccccgccctcaacaatggcacagaattgtccacgagcgatgttgcaaaacggctgatatcaggaggtgaaaggatcttgcattcgccaatgaatttgctcacagcttcacattgctctggcgtggggtggaggcttgcattgtgggatctgtacaaaatagccacctctctaaacagtgttaacaggaagtaggctgactgctggctttggggggtcttgcaggccttcagagcagtcttaatgcccagtggcttgcactcgaggacagctttggccacagcatcacggagagccttgtattcatcgccgtacaccaggtacctatccatctggcctgggtggtcctgccgcagcccctgctgcttgacaacgtccttgggaaacacccactggtgcgggcggccgggcttggagaggccctgcacgaactccatcccccgctggctgctgagcttccgcaccaggtacacccggtgccagtcgttctccacccggatacagaactgcttgacttgctgcaggtagcactgcttctccttggccatctctgggcctccctcaggctccgagaggaaatctgcagctctgtcgaggcagaggcggatccgggccacctcttgcaggtattcaaccgaggcctcgttggcaggctctcggccccggcttgctggagaatatgccttaaggaaacgaccttcctcttctaggtggttcagttcatcatttctggagtaagcactggtcttctcaagtattgaatcctccaggcagttgatgaagagcatgtacagttcagttttatcttcagttatgaatgctttcttttttaacagggtcaaatattcctgaatataatcttttacatcatgaaagctgtacttcaaaagcagtttcagtatcactgagcggatgacaggagtcttatccacaacatcattgaatggagagagagattttgtgtgttcacagtgtctctgggcagcatctcttaagcgccccttttggacgaagaggagagagagcaggctctcaatcacttccttctcaggcggagcgttgtccttgaagcaaatggtggacaccaggtctacgaagaaactgttgcacatctgccggaagcgggcatgcttttcaatggcttccctgtgcgcttgggaaacagctggagagaattcgtctggcaaggcagttaaacagtaggggcatatcatctgctctgaggcaaaccaggccctgaggcagcgcaggcagtgcacgtggtcgcagggcagacagacggggtcctttgcatctcccaggcagatggagcacggctgaatcccaaacctgctgagggtcttgctggctgtctccttgcattcacagagagtgcgcatcacggcctcaaaaggcccgtgcgtcttcacgtcagagttctctcgaagacacttgtctagtaagaagacgtgctcggtcaccagcccctgtaactcggggacgcggctctcggttcctaggagcacgtgctccacgaagagtgcggtggagaaaatccgactccactgggctctgacttccctgatgacagcctgggccaggctcccgctgccttgcatgtgctcatcggagcagatgagctccagcggcatggaaagattcttcaccaactgtagccacgcctggggactgggcttcagggtgtttcttgtcagcatctccgtgcaggccattgcggcaaatgcgtccagggtcatctcacatccagccagctcatggttccaacgggcttccatcaggctgtggagaacctgagggtagatggtcaggattctggaaaagttctgcagacggcttctgaaacgctggtaggcaaggtgcacccacggtaaggaaacctcttcctcgggcgcttctgacgccgctttcagtttcctagtgcaggaccacagagccatctgcagaaactttaattcctcctccgttgacacacgcatggtcaagagaatgaaatccttcaagtaacactgaagaagttcctgctgcggctctccatggagctgggcaagaaacctgcccagaggagtctgctgaaagatgtccacgaacttcttgggcagtccttctgcgtctgtgatgtactgagcctggacccacagctcctccagatagtccttgattttccagctgaaagggacgttgttggaagcgttctcggaaaggttcatgtggttctgcaccacgatgtaggccatctcacctttatgtctttcattattcatcacaagaggaatgttcagaagcatcgtgtcactgaaaataaacatccaaagatctcttgcccagggcggagtatctggcctggtcagtaactctaggttgccgtctctgtcgatgaatgatatcatgctcgccagcagaggggtgacagcaccttggacccgcttccagagggtgtgcctgaatgtgcccgcctcctggagagcgtcctggttgcaggcttcccttgccaaccactccagagggtgaaactggctctcttcttgcttctttaaaaagacactgaggcgcatcttggatacccgcaagaaagaggcgtggcacgcgtcatcctcattcaagaggcccaggaggagcaccaccctccgcatattgcgcgtgcagctctcgttctggtctctgagcatgcccacggcgctctgcacacagcttctcagcagcctggtggtgtccaggatcgacacatcactgcctccgagttcagaggtttcctttcccaccttctcagaactttctgtttccatggcctcctctgccacctctgccacctcccctgatgtgctggcctccgtctccatcgcctcctcatggccgtcttccgcccggtgttccaagcccagctcaggcaagtctccgggcgcgaacagctggctgatggtgacatgctgcagcctggtcacatcagaaaccatgagggtggatctccggaggtcatcgatgtggacagactgccacagccctccgtggaagcccacataggctgttcctcttcccacccgggacagttttgtgatgaaatagacgaagatacggtcctcattttctcgtattttgttgatttcatttataacagaatacttagctgaggcaatgagctgggcgctacggattccatcttcaaaatctgtctgaaaaatgaggattttacatttggctgtattcgttaaacagtttcggacttctttgaggaatgagtactcggtgtcaaactgctgcagccacaggagtgtgggtttcggagccctgcctgtgacctctgattctaaaatttcacagtcgtgacttgttagcagcctggagaaagtggtgatctctgtgaagatggcgtggcgctccaggtctgccgtgtgcaggtgtgcctgaaggaaatctgcaaaggagttgtgcctctgtctgtgaaagtactcctgcgacagccactccgctgcgaacccgcccagcgagtaggcgctcagccggaccacggcatcgggcgtagcgcagttcagcaggatcgatttggcctcctcagacaccttctggtgaagttcctccgtcaaggcccggggaccctgcctctctatgacctgcagcaccacagacgcgcaggcgtccgagtggtagccgatgaagacgtcagaggggctgtatttgtgcctcttctggaaatgatgtgctttgacattgatgaacttctccacccacgcacagagctcctccacgatgctcttctgccatttctccagcaccgtgttgatatccagatagtgcttctccagccggttaatgagggggatgggaaagtgtttgtacacgacgtctttctcttcaatgacaatcaggcggaagttggggtgaacccgacatttgacgcggtgggtccccagaccgaggtccacgtacttctggccgccgaggtggacgtagtactggttgagtgcgtcgtagaggctctcgtagaggttctgcaggttgagaagcaacaccatcttgcctgtttccatgcagatcttcacacgattgatgtttctgcagagctgggtgtactcttggtccttggggaaaccagaaccaaaaataatctccggctgctggtccccctcgaagaatgtctgctgcaggatctgcagtgccacgtagtttttggtcagcacgagtaagtagcgggactcagcatcttcctgctctccacccggcaccttctgagaaggcccaaagatgttctgtttgatcagctgcatggggctgacttcctctgagcacttggcctcgggcaaattggccagaaagatgtccaaagcttggatgtcatccttgccactgaagttcctaaggacagcctgtgcaatgtcttgcggggaaggctttctatttgaagcctttgctgcagcaaagaccattttgatgaggctgtagtagtcacgaagcccgaagaattccttgtcctggcgcttacacaccgtttcgtaggctttggcaaaggacgcaaagtacccttggactcggtcctggacgaggatgtctgaggagcagatgcccttggcgctctctatgagctctgtctcgttggggctgccacgtgacacaaaaatgccccggttcatcttggcagggtcaagggcccagttggagatgcccacgaagccgacctttttgtggggggcgggatcgtcttcaatgcatccgtcttccagcagcgggtgcagagtcttcaggggcattttgggtgagtcttccgccagccccacctcatctaacaccaccacagagacgtactgctgcaggtccttcccctgctgaaagcgggcgcactgccggaaggtgctgatgatgccctgtggggtggagtgcgggctgcactggaaggacaccaggtggacctgcttcaggctgcggaagagatctgagtaggcagccgggccctgcatggcgtctgccacgatggtcttggcgagagacttggagctgccgggcttccccaccaggaagaggggaatcttcagctcgatgcagacgaccatcatgaagacgttctccttcaaggccaagttcttggcgatggttttcctcagaggtacgccgtccagaaaaagatcctgtgcccgtgttatttcatccagaagcagcctgctgtcgtcatacggtttcggaaagaacctggcgatggctttccgatatgagtctttcttttctaaagaggcatggtaacacaccccgatggccagcatcaacgaccagaggacgggatctctctcggtgtgatttttgctgacgctggacttggagagaaaggcattcagctgcgctaagagcatcgcgctgtgctcgtggaaccacctgaaaactttcacacagcgctccacgtccctgaggctgacaaagctgcactcatcttctgttttcctcatgaaaccctgagaggcgcagaggacttctgtgatcacgcgagtcccgttttcatctaggctgatggactcaaccagtctctggacaatctgctggatgtagagcttttcagcaacgtcactcagttgtccaaagtcccacaccagaggaatcaggctcgggggcagagcatggacccggtataccagctgcctcagaggaatggagcccagcctgtcggccgtctcctccatactaaccctgtagcccaaaccagctgactccaaacggcagatcatctcctcagagtgcttccggtatggattgcaggcagctataatatgcaggccagagtcctcagccagaggctggccatccaccatatgatcacacaggacttctttgatacagcttatagcttccgttgtgttggcttcatcaaaaaacaagatggtgtccaactgatgttggtccttattggcgaaggccacattttcagcctccctgactctggagtagatcatgtctgcagttgttcctccgtgcaccttgaccagctttatggtgtcagcattggtaccaccacgccgcaggtcgctaaggaatttaataagcctggttttcccacagccagtttctcccatgatgataaccgggatcccacaccggaaccgcatctcgatggcaaggattttaagcatattgtcggttgtgagctcatacgttttgtcggggtcggtggcctgggggatccctaaggtcaggcagagcctctcaagtttcttgtgtctgggcagtttatcaaagtcgacattgaagggcaccctctggagcagcaggccctggtacaggtccctggtcatgacgtctctcttgatgaccttcccagtcaagtgactgatggcatcgacactgccgttgatgttgggctgcagatggaagccgatgaatgtcatggttgtgtggtcgtcattgaagaaaacgtatgggtgaggctccgactcccacctcttccggagggagaagggcgctagatcttcttccctaaccccatccatggtgaccatgtgcttccccgggctttggtcagaggtgtggagtgatggtgtggcaaaatctcttgccataaagatcatgaaggtcaccacgaacttcttgaagcccctcagtgtgtcgccaataaaactcggattgcagaagagagaggcctcacaatctctgagctgataattcaggaaccgagcaaagttccgaagctctgaccaggatgggtttattaccccgcagtgaaacaggaaatgctggaggcattcctccggggtgccttcgacagagccttcttgatactgaaacgtgtctaggtcttggttttgattgaatcgtcttaaatactggtaaggtctttggaaagtttcgctgcagaactcccacagatccatcccaggctctgtgtcactcctcagggcactcagctccatgtctatcacctctttgggaggcctgcaggtgacttttgggaagatgtcaagaaaactgaactggggtacacgtgtacgcagcgctgaagagctcctcgacggcactgacgtcctcctttccaggatttcaacgatatacaaatggcaggggttccgaagccacattttcccatttatatccattaagtattgtaaaatgaggagcttgaaaagaaacacccaaattccagtctgcactgaggaggtcacgtccaggtgaaagagcacggggaccttctgatactgcgcatccaggaagggcagcagggcgcccaggactcggctctcatccacctgagggtcgatcagtcgaattgttttcagaggcacatttttcacgtttaactgcatcttcattttgtcgtgcaacctcttcacgtacagagactttccaacacctgctcgctccgaggccacgatcccaacacacagccggtcattgaacacggctgccgccgacagggtctgcttcgggacccggtagtgacctgccaggtaggcttggatggcctcgaggggtgcctggggggtgacgaagaccttgtgctggctgaaggcagaggggaggtagcagtgctcccagtccccatcacagaccatgacgagctggtagtcttctcggtgctgctgcgtgcacagattgtggaaaagctcctccgcttggcgtgccacctcgtagctcagctgatctgcgaacagcaggctgtagaccttgtgccccagggagcccagggtcaggcagcggcgcagcaacagtgccacctcctcaaaggtggttgccggggtgcagagcagcacctcatcgtaagtgggcaggggctggcttggggtttgcatgtagacagccagggcggctggcaacacctcggagtggccacagacgacgaggttgggctggccgacctgcagacctctcgggagacaacgctccacgggagacccacccatccctgccaggtgagccagacagtggccaagggtctctaggtcgaggcagtcgggcaggaaggcaggaaggcacctcatggactgctccatgatgatcctcagcttgtccaccaggctgaactctgataagagcatcagcgggagctcttccatgactctcctcatgcggtacctggcggcctcactcccacaccccacagaggcccttaagacatccctcagggtgcagttgcttttgatgaaggatagcatcgttagggcggcatcactcgggggctgcttcctgagctcagtgctcaggtaaaccagctgctctgccgtgtagaagttcaggtaaaagtgctccattcgcttctgggtcacaaatctcttccagctgtcaaggaagtgctccatctgcctgcagagggctgccagcagctcagtgacatctccaccttctttaagctccgtcaccaggtccaagccaaagtccatttggagggacacaccctgcttgggggagcagtaggccatggcgatccacgtcctgaacagcatattcccagcagagtgcaggtcgatgaaggcctggctgagcctctgcacactgcagaagacctctgaaaacctctccacttccgtgttgttacgatccttcttgccagacatcagcatcaacttgttcaaaagctccttcacctcctctaaagagtactctcgtgactcctcgtggctgccagggctctcaggaaggatcaagtgcagaaccgtgtctggggaaatcttttggccacctttgggcgcctggatcacatagatgcctctttggttgatggccgtggccagggtcagggatgagcgttccacagacccatgactctcattcacagtcttcagccattccaagttcctggcggagtcacacagtttcctgggcaggtactggtccttatccagagccttccacagctttttcagatgcttcatgaatgcactgaagtccacgctggggtccagcttaaatagcagggatgcgtagccctgcacagcgtcatggaagcaggccacccggtccacatcaatgtcattctcccccgctgagatggaggccaggtccacaaacaccttcagctcattgatgcctccaagagcctcccggacccagcagatgaactcctttctcagggacagagcctgcagccccttgcaccgggcctcgctgatgtcctggagcagctttttggcctggatgagctcctggttgatctggtccagtgtttcacggcgaaagtcgtcgaagttatcagtaaaatttagtaaagtgttgagaacactgaagtcaccgttcagtcccaggctctctttgacctgcaagatgaccttggctgcgtggacagcctggtgcaggtgatggtattccttgatctgttcgactcggtccttgatccaatctctttggtcctggtggtccacggtgcacatgatcttaagttctgaatccaggtccgtgtatttattcacaaagtccttgaagatgacatcaatctctgcaagggtgacctctcctgactttagatcctggtgcaacttaatgaactttctgtaagaaggctgatacaaatagtcatacacctcttcaagctcaaggatgtgcctttctgattcttcttcgggctcactcagcaactctgcggcttcctggtcctccttaggctcactcagcggctctgcggcttcccgccagaagagctggaagatgtggctgtctctgagcaagtctatcttcccagccatttcttggacctgggagctcaggtggtaatgcgttgccctctgcgagttcgaggaggtggacagtctcactgtcacggtgtcatttaatcttttactgctgaggtcttgtgagtgtcttactgcaagcactccaaagtccacttgtatcagatgtttcacgttcccacacatcttcaggagactatcaacacatcttttctctttctttagaagtaacagttcctcccttctccaatccagtgcttcctccacagcacattgttcatcctggggtgaaagacttttttccctcagttgccagatgtcaagaaactgattcttgtgctttataatcagctccagttgtccaactaaaatcgtgccacttaggaggtcaccaacaactttcgtcaacacagagtcggcaacagctatcagcctcttggcatcctctgtgacatttgctagtattttctcgtcggttccacacaatctgaagacgtgcttgacatctgccaacgtgagcagatgctttaaaatgtcatcgaagttgtccgcggtcctaggccaggacttagtgatcacagcagacaagacgatgccaaatttccgcaaatcagagtaagagaacccctgaaggatactggtctgagactggcaggctgagctcacggcttcaatgatgcatttctcgaaggtcttggccacactgtcctctaagcctttggtgtcccagcaactattgcagtaggcagtgatctgggagaggggttcctcctttgtgagcctccattccatgtctcccagcaacgactccttccagccatgctccgcggggaattggatttccaccagccgcctccagacctcaatttccttgacgtatgtgaatgaggcacctgaagatgtgagcatgttctttgtaaaaacttctcggagccaccttttcgtagcagcaagggtcccttggaagactgtttggactgaattatttccagtttcatctctctgtcctgcagaatccaccagagatagaagtctaatcattctgcagacaatctcggcagataaggctggcagctcgtaaaacttaagtagctttgtgctgctgcagatggcttcatgcagtttcagacacacagtcaggtaggatggtgacaaggcctcctcgggaatcttgtcccggtaagtgtccaggagtcgcaacagcatttctaaaatgttctgaacgttctgaacatcctgaacatcctgcgtattcaagacttgctcaagtcccggaagccggtagtaaatccctgaaagacagtccaggatatgagcaggaaaacgacccaggtgctcaatgaagttttccatatacataaccaggtgactcagaggtagcagactaaaccaggaccggaagagaggctcgtctatgctcagcaaatgctgcttctctctcataaactgaagtagggaactcgtatctagcatttgttcccggaacggtgagaaggagagtccctccagagcggcccaggtgtcctcaggctgtctccaggcatccttgtgccgcggggccagctccatacagcagtgcaggacaggcagggcgcccagccaggtgtacgtccttgtgtccatgcatctttggcacaggttcaccaggtacagccgccagctctgaggtatcccaaggatgtggcttaggtcacggtgaaactcatctggtgagctggcatctgaggttaggaggtgacacaaccagtccaggctgccttctaataaaagctcaattttttccactacaaaaaggacaatcaggcctgttttcagtttactcctcactgggcagtccacaggcaaaaagtccgtgctttttccgtccggcaatggtaccacgtgttttttcagatgttgccacaggtatctcttcacctctttctccctgtactgcaaatcggtccacagctgtgcctgtccttcataaatcataggctgttgcaggacaaagcaaaactgctcgaactgggtgaagaagctgttcaggttgatggtgtcccaggtctgcaggatgctgaaggtgctgtccagcatgagcgcagcggcaatctgcttccccttcaccaggtccttcctcggcccgtctgtgatgtggttcatgactttctggagtctcccatgaggcttcatataaactatgtcatagtactgatgccagtctcctgagcccagaagtgaagattttatgaacagacagcggttgacgtactcgcccttcttctgctggtgcttgtaaatgaactcatactcaaaagattccccattataaatgacgtacttgtaaggaatgtatttatctaggtgcttcttggaaatgcagacaatgccttcaacaagaacgcggtcatgacccaagtctctggtgtagtgcagctcacagatattgctgtcccattttgactccccaaattcttctcctcctctgatgaagactttatggaggtcaggattgaatgggaaatgaagagagatgatggcgtggaagaacacggtgactcctccacccgggctcagcgtgcttgccttcacttcctggacatctgcttcctggtttttttgctccttctcgtttttcacagcagctgcacttctgttcttcccctctggcttcttgaggtcttcaggctccccttgttcattcttaccgactttttcttcagcagcagccatctcgtccttggtcttggtctcagcttcctggcagtgtgttttgaaaggaggagtggttgctggtggctgtttcattctctgggtcttctctttcatttccttcccggcccctttaactgcattggctggctcagctacagcatcaactgccatagaggctgaggcccctgcctgttgctcggtggtctgcagttctgtcccgggctcagagctgcctccttttgactcaggcaacaggagctcctgggcagcatcttcagtcctagaatggccttcaccagcagaggtggggggaccggtcccctcctgggacaggcctctgcccccagaggggatggaagcgtcctggtcctccccttccgtgtggtcctggaattgcgggctgctctgagcctcacttcctgtggccactcctgcctctcccaaagcctgggcctgcagggggctgtcgccaacctcggtgggcgcggagaggccgtcaccctccagtggcgtggtggctgtgcctgggggctggctcggctggccagtggggccactctgctgggcttggctgtggggcagggctgtgtcctgaggccacgggtttgaaagcaaagtcaggtgacaggggctggcaggagaaaggggcaaggaagccagctctgaggaagcggacttgttccccttctttttcttcttccttttcttctttttgctctgctcacagtctgcagaaggcacgctggcggcctcaagcggggctgcatcctgcttccttctcttgctgggtatggcattagcagcttcccattcatcggatatgaggtctacagcagcatctaccaaaacctctgatgtagctccttcttggacggtccaggaggctttggaacagggctcctcggggttttcttgccaactgtctgagcccgggaacaagcacgggcccccttcctccttcagctcctgcccacactccatttcaccctccgaggccgacgccattgtggagttattgttctcagaatctgctatgggggctgcaggaggcagcctctctccgcactggctgcagaacttgggggtttcctccttggagacatgctggcacgaaggacactccatgggtcctgctgggactgccctgcagatccagaagcaagagcaggagtcgctggcagcctgctatatactacatgtcctgtcacgtgaccacggcttcagtttcattttctgcggcccccgagctcgccgcctgccgcgcgctgtcgcccctcgggtcacggggccctgggccccgccctgcccgccgccgc

SEQ ID NO: 8773 - RNA, 15515 nt, Homo sapiens
  source 1..15515: mol_type = other RNA
aaggtattgttcagacttatgagcagacaggaactgccagagggcaatggtgtgttttaactggcatctgtttaaggcctttaacacgtgaatcgtctgatcacccatttgcaggatgtcttgagtatacacattcagctgcatgtttggatccccaccagctgtgctcagaaaccccagagtgacttctacgacagacagcacttcacaggcatcgctgtaggactgcagctgtccactgatggcactaatgaccgagctggggagggagtcctgtgccattttgttcttgatgtccataaagagatgttcatagttccagtcgtgtctgtacaccagagtgggtattcccttgaggctcagccggggcttgccctggaggaagcggctgacgatctgccgctgaatcttctccagatcgaactcctgcacggtctctctgccctcctccacctggtactggcagttggagagaatcagtggagtcaggtcccgctccacttcataactgatgacatgcagttcagtgacctcggcggcatccacggaatagctgttgttttccttggagagtttttccacggcgtagacaatttcattgtgtaggcgaatcaagtagctgacgagagcggtagcacagaggcccaggccccgtcggcgtggcaagaggatctcaaactcagtgtccagatccaagtcagtgctgcagtagtctttgggtaggttgatctcaccgttcgtctcaagcgatctcctcagtttgttccatgtggacagaaagactgtgatcctgttgtgaagcagctgcctcaacccatctgagctgtgcttgctgaggaagcctctgatggagctgtattcaacttgctggacgttctggaactgcttcactagatccctttgcaaggccaaaatctcaggcaggaactttaccagcctcagctctgcttccttctgcaggaaatgccagaggatgggcactctttctttgccatttttctgttccacaatgtgctggaggtactcaactgtaattcttttcctgcagctccaaatcttagagcaatggaccacacttttccggggcaggtggggcaggaaggtcactgggtcaccatatattattttggccacagggttagagctgatacgcttatcttggctgatgagattattcatggtgggaagggttttatctagatgctccagttcaggagaaatcacagctgcgatttccttttcccagttgttcctcatttctttagttgacaattctgtgtcaaaatttaaaagccttctgctagagagctggtgctgctcttggagaagcctgcgcaggacgaggtggaccacgccgatggtctcgtcggcactgtgtcccagcatcttggccaactgctccaggtccttcaggatgtgctgctgcagaaagccttttggatccctcactggaggcttaatgatgtttatcagagcctgggaactctgggacgctcccagaagcagagccaagtgagtgagtagccggataaggaggaagaccactgggggcagccctcggtcacatgtcaccacgtctctccgctgcgggttgcccagcacgtggccggtctgcgttctgtctgccttgtctttgaccagatgaaagccgtcccgaggtttgtggtcaatgcctccaatcggcgcatggcagtcaatgcagatgctctgttccatcggcctgccacactctcccacggagcaaggatggccgttgggacaagtgtaccagtggactcgctccagacccttccacctccgagcttgagccagcaagtcttcaggcatggttggaagaaaagcatgcgccatggtggctggggagaaggccagattctttaggggctccaagagttcattctgtccacacagaaggacggctgcagcatgaatggccatttctgtcaccgttccatcaaggttgctgtcactaggccccgccctcaacaatggcacagaattgtccacgagcgatgttgcaaaacggctgatatcaggaggtgaaaggatcttgcattcgccaatgaatttgctcacagcttcacattgctctggcgtggggtggaggcttgcattgtgggatctgtacaaaatagccacctctctaaacagtgttaacaggaagtaggctgactgctggctttggggggtcttgcaggccttcagagcagtcttaatgcccagtggcttgcactcgaggacagctttggccacagcatcacggagagccttgtattcatcgccgtacaccaggtacctatccatctggcctgggtggtcctgccgcagcccctgctgcttgacaacgtccttgggaaacacccactggtgcgggcggccgggcttggagaggccctgcacgaactccatcccccgctggctgctgagcttccgcaccaggtacacccggtgccagtcgttctccacccggatacagaactgcttgacttgctgcaggtagcactgcttctccttggccatctctgggcctccctcaggctccgagaggaaatctgcagctctgtcgaggcagaggcggatccgggccacctcttgcaggtattcaaccgaggcctcgttggcaggctctcggccccggcttgctggagaatatgccttaaggaaacgaccttcctcttctaggtggttcagttcatcatttctggagtaagcactggtcttctcaagtattgaatcctccaggcagttgatgaagagcatgtacagttcagttttatcttcagttatgaatgctttcttttttaacagggtcaaatattcctgaatataatcttttacatcatgaaagctgtacttcaaaagcagtttcagtatcactgagcggatgacaggagtcttatccacaacatcattgaatggagagagagattttgtgtgttcacagtgtctctgggcagcatctcttaagcgccccttttggacgaagaggagagagagcaggctctcaatcacttccttctcaggcggagcgttgtccttgaagcaaatggtggacaccaggtctacgaagaaactgttgcacatctgccggaagcgggcatgcttttcaatggcttccctgtgcgcttgggaaacagctggagagaattcgtctggcaaggcagttaaacagtaggggcatatcatctgctctgaggcaaaccaggccctgaggcagcgcaggcagtgcacgtggtcgcagggcagacagacggggtcctttgcatctcccaggcagatggagcacggctgaatcccaaacctgctgagggtcttgctggctgtctccttgcattcacagagagtgcgcatcacggcctcaaaaggcccgtgcgtcttcacgtcagagttctctcgaagacacttgtctagtaagaagacgtgctcggtcaccagcccctgtaactcggggacgcggctctcggttcctaggagcacgtgctccacgaagagtgcggtggagaaaatccgactccactgggctctgacttccctgatgacagcctgggccaggctcccgctgccttgcatgtgctcatcggagcagatgagctccagcggcatggaaagattcttcaccaactgtagccacgcctggggactgggcttcagggtgtttcttgtcagcatctccgtgcaggccattgcggcaaatgcgtccagggtcatctcacatccagccagctcatggttccaacgggcttccatcaggctgtggagaacctgagggtagatggtcaggattctggaaaagttctgcagacggcttctgaaacgctggtaggcaaggtgcacccacggtaaggaaacctcttcctcgggcgcttctgacgccgctttcagtttcctagtgcaggaccacagagccatctgcagaaactttaattcctcctccgttgacacacgcatggtcaagagaatgaaatccttcaagtaacactgaagaagttcctgctgcggctctccatggagctgggcaagaaacctgcccagaggagtctgctgaaagatgtccacgaacttcttgggcagtccttctgcgtctgtgatgtactgagcctggacccacagctcctccagatagtccttgattttccagctgaaagggacgttgttggaagcgttctcggaaaggttcatgtggttctgcaccacgatgtaggccatctcacctttatgtctttcattattcatcacaagaggaatgttcagaagcatcgtgtcactgaaaataaacatccaaagatctcttgcccagggcggagtatctggcctggtcagtaactctaggttgccgtctctgtcgatgaatgatatcatgctcgccagcagaggggtgacagcaccttggacccgcttccagagggtgtgcctgaatgtgcccgcctcctggagagcgtcctggttgcaggcttcccttgccaaccactccagagggtgaaactggctctcttcttgcttctttaaaaagacactgaggcgcatcttggatacccgcaagaaagaggcgtggcacgcgtcatcctcattcaagaggcccaggaggagcaccaccctccgcatattgcgcgtgcagctctcgttctggtctctgagcatgcccacggcgctctgcacacagcttctcagcagcctggtggtgtccaggatcgacacatcactgcctccgagttcagaggtttcctttcccaccttctcagaactttctgtttccatggcctcctctgccacctctgccacctcccctgatgtgctggcctccgtctccatcgcctcctcatggccgtcttccgcccggtgttccaagcccagctcaggcaagtctccgggcgcgaacagctggctgatggtgacatgctgcagcctggtcacatcagaaaccatgagggtggatctccggaggtcatcgatgtggacagactgccacagccctccgtggaagcccacataggctgttcctcttcccacccgggacagttttgtgatgaaatagacgaagatacggtcctcattttctcgtattttgttgatttcatttataacagaatacttagctgaggcaatgagctgggcgctacggattccatcttcaaaatctgtctgaaaaatgaggattttacatttggctgtattcgttaaacagtttcggacttctttgaggaatgagtactcggtgtcaaactgctgcagccacaggagtgtgggtttcggagccctgcctgtgacctctgattctaaaatttcacagtcgtgacttgttagcagcctggagaaagtggtgatctctgtgaagatggcgtggcgctccaggtctgccgtgtgcaggtgtgcctgaaggaaatctgcaaaggagttgtgcctctgtctgtgaaagtactcctgcgacagccactccgctgcgaacccgcccagcgagtaggcgctcagccggaccacggcatcgggcgtagcgcagttcagcaggatcgatttggcctcctcagacaccttctggtgaagttcctccgtcaaggcccggggaccctgcctctctatgacctgcagcaccacagacgcgcaggcgtccgagtggtagccgatgaagacgtcagaggggctgtatttgtgcctcttctggaaatgatgtgctttgacattgatgaacttctccacccacgcacagagctcctccacgatgctcttctgccatttctccagcaccgtgttgatatccagatagtgcttctccagccggttaatgagggggatgggaaagtgtttgtacacgacgtctttctcttcaatgacaatcaggcggaagttggggtgaacccgacatttgacgcggtgggtccccagaccgaggtccacgtacttctggccgccgaggtggacgtagtactggttgagtgcgtcgtagaggctctcgtagaggttctgcaggttgagaagcaacaccatcttgcctgtttccatgcagatcttcacacgattgatgtttctgcagagctgggtgtactcttggtccttggggaaaccagaaccaaaaataatctccggctgctggtccccctcgaagaatgtctgctgcaggatctgcagtgccacgtagtttttggtcagcacgagtaagtagcgggactcagcatcttcctgctctccacccggcaccttctgagaaggcccaaagatgttctgtttgatcagctgcatggggctgacttcctctgagcacttggcctcgggcaaattggccagaaagatgtccaaagcttggatgtcatccttgccactgaagttcctaaggacagcctgtgcaatgtcttgcggggaaggctttctatttgaagcctttgctgcagcaaagaccattttgatgaggctgtagtagtcacgaagcccgaagaattccttgtcctggcgcttacacaccgtttcgtaggctttggcaaaggacgcaaagtacccttggactcggtcctggacgaggatgtctgaggagcagatgcccttggcgctctctatgagctctgtctcgttggggctgccacgtgacacaaaaatgccccggttcatcttggcagggtcaagggcccagttggagatgcccacgaagccgacctttttgtggggggcgggatcgtcttcaatgcatccgtcttccagcagcgggtgcagagtcttcaggggcattttgggtgagtcttccgccagccccacctcatctaacaccaccacagagacgtactgctgcaggtccttcccctgctgaaagcgggcgcactgccggaaggtgctgatgatgccctgtggggtggagtgcgggctgcactggaaggacaccaggtggacctgcttcaggctgcggaagagatctgagtaggcagccgggccctgcatggcgtctgccacgatggtcttggcgagagacttggagctgccgggcttccccaccaggaagaggggaatcttcagctcgatgcagacgaccatcatgaagacgttctccttcaaggccaagttcttggcgatggttttcctcagaggtacgccgtccagaaaaagatcctgtgcccgtgttatttcatccagaagcagcctgctgtcgtcatacggtttcggaaagaacctggcgatggctttccgatatgagtctttcttttctaaagaggcatggtaacacaccccgatggccagcatcaacgaccagaggacgggatctctctcggtgtgatttttgctgacgctggacttggagagaaaggcattcagctgcgctaagagcatcgcgctgtgctcgtggaaccacctgaaaactttcacacagcgctccacgtccctgaggctgacaaagctgcactcatcttctgttttcctcatgaaaccctgagaggcgcagaggacttctgtgatcacgcgagtcccgttttcatctaggctgatggactcaaccagtctctggacaatctgctggatgtagagcttttcagcaacgtcactcagttgtccaaagtcccacaccagaggaatcaggctcgggggcagagcatggacccggtataccagctgcctcagaggaatggagcccagcctgtcggccgtctcctccatactaaccctgtagcccaaaccagctgactccaaacggcagatcatctcctcagagtgcttccggtatggattgcaggcagctataatatgcaggccagagtcctcagccagaggctggccatccaccatatgatcacacaggacttctttgatacagcttatagcttccgttgtgttggcttcatcaaaaaacaagatggtgtccaactgatgttggtccttattggcgaaggccacattttcagcctccctgactctggagtagatcatgtctgcagttgttcctccgtgcaccttgaccagctttatggtgtcagcattggtaccaccacgccgcaggtcgctaaggaatttaataagcctggttttcccacagccagtttctcccatgatgataaccgggatcccacaccggaaccgcatctcgatggcaaggattttaagcatattgtcggttgtgagctcatacgttttgtcggggtcggtggcctgggggatccctaaggtcaggcagagcctctcaagtttcttgtgtctgggcagtttatcaaagtcgacattgaagggcaccctctggagcagcaggccctggtacaggtccctggtcatgacgtctctcttgatgaccttcccagtcaagtgactgatggcatcgacactgccgttgatgttgggctgcagatggaagccgatgaatgtcatggttgtgtggtcgtcattgaagaaaacgtatgggtgaggctccgactcccacctcttccggagggagaagggcgctagatcttcttccctaaccccatccatggtgaccatgtgcttccccgggctttggtcagaggtgtggagtgatggtgtggcaaaatctcttgccataaagatcatgaaggtcaccacgaacttcttgaagcccctcagtgtgtcgccaataaaactcggattgcagaagagagaggcctcacaatctctgagctgataattcaggaaccgagcaaagttccgaagctctgaccaggatgggtttattaccccgcagtgaaacaggaaatgctggaggcattcctccggggtgccttcgacagagccttcttgatactgaaacgtgtctaggtcttggttttgattgaatcgtcttaaatactggtaaggtctttggaaagtttcgctgcagaactcccacagatccatcccaggctctgtgtcactcctcagggcactcagctccatgtctatcacctctttgggaggcctgcaggtgacttttgggaagatgtcaagaaaactgaactggggtacacgtgtacgcagcgctgaagagctcctcgacggcactgacgtcctcctttccaggatttcaacgatatacaaatggcaggggttccgaagccacattttcccatttatatccattaagtattgtaaaatgaggagcttgaaaagaaacacccaaattccagtctgcactgaggaggtcacgtccaggtgaaagagcacggggaccttctgatactgcgcatccaggaagggcagcagggcgcccaggactcggctctcatccacctgagggtcgatcagtcgaattgttttcagaggcacatttttcacgtttaactgcatcttcattttgtcgtgcaacctcttcacgtacagagactttccaacacctgctcgctccgaggccacgatcccaacacacagccggtcattgaacacggctgccgccgacagggtctgcttcgggacccggtagtgacctgccaggtaggcttggatggcctcgaggggtgcctggggggtgacgaagaccttgtgctggctgaaggcagaggggaggtagcagtgctcccagtccccatcacagaccatgacgagctggtagtcttctcggtgctgctgcgtgcacagattgtggaaaagctcctccgcttggcgtgccacctcgtagctcagctgatctgcgaacagcaggctgtagaccttgtgccccagggagcccagggtcaggcagcggcgcagcaacagtgccacctcctcaaaggtggttgccggggtgcagagcagcacctcatcgtaagtgggcaggggctggcttggggtttgcatgtagacagccagggcggctggcaacacctcggagtggccacagacgacgaggttgggctggccgacctgcagacctctcgggagacaacgctccacgggagacccacccatccctgccaggtgagccagacagtggccaagggtctctaggtcgaggcagtcgggcaggaaggcaggaaggcacctcatggactgctccatgatgatcctcagcttgtccaccaggctgaactctgataagagcatcagcgggagctcttccatgactctcctcatgcggtacctggcggcctcactcccacaccccacagaggcccttaagacatccctcagggtgcagttgcttttgatgaaggatagcatcgttagggcggcatcactcgggggctgcttcctgagctcagtgctcaggtaaaccagctgctctgccgtgtagaagttcaggtaaaagtgctccattcgcttctgggtcacaaatctcttccagctgtcaaggaagtgctccatctgcctgcagagggctgccagcagctcagtgacatctccaccttctttaagctccgtcaccaggtccaagccaaagtccatttggagggacacaccctgcttgggggagcagtaggccatggcgatccacgtcctgaacagcatattcccagcagagtgcaggtcgatgaaggcctggctgagcctctgcacactgcagaagacctctgaaaacctctccacttccgtgttgttacgatccttcttgccagacatcagcatcaacttgttcaaaagctccttcacctcctctaaagagtactctcgtgactcctcgtggctgccagggctctcaggaaggatcaagtgcagaaccgtgtctggggaaatcttttggccacctttgggcgcctggatcacatagatgcctctttggttgatggccgtggccagggtcagggatgagcgttccacagacccatgactctcattcacagtcttcagccattccaagttcctggcggagtcacacagtttcctgggcaggtactggtccttatccagagccttccacagctttttcagatgcttcatgaatgcactgaagtccacgctggggtccagcttaaatagcagggatgcgtagccctgcacagcgtcatggaagcaggccacccggtccacatcaatgtcattctcccccgctgagatggaggccaggtccacaaacaccttcagctcattgatgcctccaagagcctcccggacccagcagatgaactcctttctcagggacagagcctgcagccccttgcaccgggcctcgctgatgtcctggagcagctttttggcctggatgagctcctggttgatctggtccagtgtttcacggcgaaagtcgtcgaagttatcagtaaaatttagtaaagtgttgagaacactgaagtcaccgttcagtcccaggctctctttgacctgcaagatgaccttggctgcgtggacagcctggtgcaggtgatggtattccttgatctgttcgactcggtccttgatccaatctctttggtcctggtggtccacggtgcacatgatcttaagttctgaatccaggtccgtgtatttattcacaaagtccttgaagatgacatcaatctctgcaagggtgacctctcctgactttagatcctggtgcaacttaatgaactttctgtaagaaggctgatacaaatagtcatacacctcttcaagctcaaggatgtgcctttctgattcttcttcgggctcactcagcaactctgcggcttcctggtcctccttaggctcactcagcggctctgcggcttcccgccagaagagctggaagatgtggctgtctctgagcaagtctatcttcccagccatttcttggacctgggagctcaggtggtaatgcgttgccctctgcgagttcgaggaggtggacagtctcactgtcacggtgtcatttaatcttttactgctgaggtcttgtgagtgtcttactgcaagcactccaaagtccacttgtatcagatgtttcacgttcccacacatcttcaggagactatcaacacatcttttctctttctttagaagtaacagttcctcccttctccaatccagtgcttcctccacagcacattgttcatcctggggtgaaagacttttttccctcagttgccagatgtcaagaaactgattcttgtgctttataatcagctccagttgtccaactaaaatcgtgccacttaggaggtcaccaacaactttcgtcaacacagagtcggcaacagctatcagcctcttggcatcctctgtgacatttgctagtattttctcgtcggttccacacaatctgaagacgtgcttgacatctgccaacgtgagcagatgctttaaaatgtcatcgaagttgtccgcggtcctaggccaggacttagtgatcacagcagacaagacgatgccaaatttccgcaaatcagagtaagagaacccctgaaggatactggtctgagactggcaggctgagctcacggcttcaatgatgcatttctcgaaggtcttggccacactgtcctctaagcctttggtgtcccagcaactattgcagtaggcagtgatctgggagaggggttcctcctttgtgagcctccattccatgtctcccagcaacgactccttccagccatgctccgcggggaattggatttccaccagccgcctccagacctcaatttccttgacgtatgtgaatgaggcacctgaagatgtgagcatgttctttgtaaaaacttctcggagccaccttttcgtagcagcaagggtcccttggaagactgtttggactgaattatttccagtttcatctctctgtcctgcagaatccaccagagatagaagtctaatcattctgcagacaatctcggcagataaggctggcagctcgtaaaacttaagtagctttgtgctgctgcagatggcttcatgcagtttcagacacacagtcaggtaggatggtgacaaggcctcctcgggaatcttgtcccggtaagtgtccaggagtcgcaacagcatttctaaaatgttctgaacgttctgaacatcctgaacatcctgcgtattcaagacttgctcaagtcccggaagccggtagtaaatccctgaaagacagtccaggatatgagcaggaaaacgacccaggtgctcaatgaagttttccatatacataaccaggtgactcagaggtagcagactaaaccaggaccggaagagaggctcgtctatgctcagcaaatgctgcttctctctcataaactgaagtagggaactcgtatctagcatttgttcccggaacggtgagaaggagagtccctccagagcggcccaggtgtcctcaggctgtctccaggcatccttgtgccgcggggccagctccatacagcagtgcaggacaggcagggcgcccagccaggtgtacgtccttgtgtccatgcatctttggcacaggttcaccaggtacagccgccagctctgaggtatcccaaggatgtggcttaggtcacggtgaaactcatctggtgagctggcatctgaggttaggaggtgacacaaccagtccaggctgccttctaataaaagctcaattttttccactacaaaaaggacaatcaggcctgttttcagtttactcctcactgggcagtccacaggcaaaaagtccgtgctttttccgtccggcaatggtaccacgtgttttttcagatgttgccacaggtatctcttcacctctttctccctgtactgcaaatcggtccacagctgtgcctgtccttcataaatcataggctgttgcaggacaaagcaaaactgctcgaactgggtgaagaagctgttcaggttgatggtgtcccaggtctgcaggatgctgaaggtgctgtccagcatgagcgcagcggcaatctgcttccccttcaccaggtccttcctcggcccgtctgtgatgtggttcatgactttctggagtctcccatgaggcttcatataaactatgtcatagtactgatgccagtctcctgagcccagaagtgaagattttatgaacagacagcggttgacgtactcgcccttcttctgctggtgcttgtaaatgaactcatactcaaaagattccccattataaatgacgtacttgtaaggaatgtatttatctaggtgcttcttggaaatgcagacaatgccttcaacaagaacgcggtcatgacccaagtctctggtgtagtgcagctcacagatattgctgtcccattttgactccccaaattcttctcctcctctgatgaagactttatggaggtcaggattgaatgggaaatgaagagagatgatggcgtggaagaacacggtgactcctccacccgggctcagcgtgcttgccttcacttcctggacatctgcttcctggtttttttgctccttctcgtttttcacagcagctgcacttctgttcttcccctctggcttcttgaggtcttcaggctccccttgttcattcttaccgactttttcttcagcagcagccatctcgtccttggtcttggtctcagcttcctggcagtgtgttttgaaaggaggagtggttgctggtggctgtttcattctctgggtcttctctttcatttccttcccggcccctttaactgcattggctggctcagctacagcatcaactgccatagaggctgaggcccctgcctgttgctcggtggtctgcagttctgtcccgggctcagagctgcctccttttgactcaggcaacaggagctcctgggcagcatcttcagtcctagaatggccttcaccagcagaggtggggggaccggtcccctcctgggacaggcctctgcccccagaggggatggaagcgtcctggtcctccccttccgtgtggtcctggaattgcgggctgctctgagcctcacttcctgtggccactcctgcctctcccaaagcctgggcctgcagggggctgtcgccaacctcggtgggcgcggagaggccgtcaccctccagtggcgtggtggctgtgcctgggggctggctcggctggccagtggggccactctgctgggcttggctgtggggcagggctgtgtcctgaggccacgggtttgaaagcaaagtcaggtgacaggggctggcaggagaaaggggcaaggaagccagctctgaggaagcggacttgttccccttctttttcttcttccttttcttctttttgctctgctcacagtctgcagaaggcacgctggcggcctcaagcggggctgcatcctgcttccttctcttgctgggtatggcattagcagcttcccattcatcggatatgaggtctacagcagcatctaccaaaacctctgatgtagctccttcttggacggtccaggaggctttggaacagggctcctcggggttttcttgccaactgtctgagcccgggaacaagcacgggcccccttcctccttcagctcctgcccacactccatttcaccctccgaggccgacgccattgtggagttattgttctcagaatctgctatgggggctgcaggaggcagcctctctccgcactggctgcagaacttgggggtttcctccttggagacatgctggcacgaaggacactccatgggtcctgctgggactgccctgcggcccccgagctcgccgcctgccgcgcgctgtcgcccctcgggtcacggggccctgggccccgccctgcccg

SEQ ID NO: 8774 - RNA, 15432 nt, Homo sapiens
  source 1..15432: mol_type = other RNA
aaggtattgttcagacttatgagcagacaggaactgccagagggcaatggtgtgttttaactggcatctgtttaaggcctttaacacgtgaatcgtctgatcacccatttgcaggatgtcttgagtatacacattcagctgcatgtttggatccccaccagctgtgctcagaaaccccagagtgacttctacgacagacagcacttcacaggcatcgctgtaggactgcagctgtccactgatggcactaatgaccgagctggggagggagtcctgtgccattttgttcttgatgtccataaagagatgttcatagttccagtcgtgtctgtacaccagagtgggtattcccttgaggctcagccggggcttgccctggaggaagcggctgacgatctgccgctgaatcttctccagatcgaactcctgcacggtctctctgccctcctccacctggtactggcagttggagagaatcagtggagtcaggtcccgctccacttcataactgatgacatgcagttcagtgacctcggcggcatccacggaatagctgttgttttccttggagagtttttccacggcgtagacaatttcattgtgtaggcgaatcaagtagctgacgagagcggtagcacagaggcccaggccccgtcggcgtggcaagaggatctcaaactcagtgtccagatccaagtcagtgctgcagtagtctttgggtaggttgatctcaccgttcgtctcaagcgatctcctcagtttgttccatgtggacagaaagactgtgatcctgttgtgaagcagctgcctcaacccatctgagctgtgcttgctgaggaagcctctgatggagctgtattcaacttgctggacgttctggaactgcttcactagatccctttgcaaggccaaaatctcaggcaggaactttaccagcctcagctctgcttccttctgcaggaaatgccagaggatgggcactctttctttgccatttttctgttccacaatgtgctggaggtactcaactgtaattcttttcctgcagctccaaatcttagagcaatggaccacacttttccggggcaggtggggcaggaaggtcactgggtcaccatatattattttggccacagggttagagctgatacgcttatcttggctgatgagattattcatggtgggaagggttttatctagatgctccagttcaggagaaatcacagctgcgatttccttttcccagttgttcctcatttctttagttgacaattctgtgtcaaaatttaaaagccttctgctagagagctggtgctgctcttggagaagcctgcgcaggacgaggtggaccacgccgatggtctcgtcggcactgtgtcccagcatcttggccaactgctccaggtccttcaggatgtgctgctgcagaaagccttttggatccctcactggaggcttaatgatgtttatcagagcctgggaactctgggacgctcccagaagcagagccaagtgagtgagtagccggataaggaggaagaccactgggggcagccctcggtcacatgtcaccacgtctctccgctgcgggttgcccagcacgtggccggtctgcgttctgtctgccttgtctttgaccagatgaaagccgtcccgaggtttgtggtcaatgcctccaatcggcgcatggcagtcaatgcagatgctctgttccatcggcctgccacactctcccacggagcaaggatggccgttgggacaagtgtaccagtggactcgctccagacccttccacctccgagcttgagccagcaagtcttcaggcatggttggaagaaaagcatgcgccatggtggctggggagaaggccagattctttaggggctccaagagttcattctgtccacacagaaggacggctgcagcatgaatggccatttctgtcaccgttccatcaaggttgctgtcactaggccccgccctcaacaatggcacagaattgtccacgagcgatgttgcaaaacggctgatatcaggaggtgaaaggatcttgcattcgccaatgaatttgctcacagcttcacattgctctggcgtggggtggaggcttgcattgtgggatctgtacaaaatagccacctctctaaacagtgttaacaggaagtaggctgactgctggctttggggggtcttgcaggccttcagagcagtcttaatgcccagtggcttgcactcgaggacagctttggccacagcatcacggagagccttgtattcatcgccgtacaccaggtacctatccatctggcctgggtggtcctgccgcagcccctgctgcttgacaacgtccttgggaaacacccactggtgcgggcggccgggcttggagaggccctgcacgaactccatcccccgctggctgctgagcttccgcaccaggtacacccggtgccagtcgttctccacccggatacagaactgcttgacttgctgcaggtagcactgcttctccttggccatctctgggcctccctcaggctccgagaggaaatctgcagctctgtcgaggcagaggcggatccgggccacctcttgcaggtattcaaccgaggcctcgttggcaggctctcggccccggcttgctggagaatatgccttaaggaaacgaccttcctcttctaggtggttcagttcatcatttctggagtaagcactggtcttctcaagtattgaatcctccaggcagttgatgaagagcatgtacagttcagttttatcttcagttatgaatgctttcttttttaacagggtcaaatattcctgaatataatcttttacatcatgaaagctgtacttcaaaagcagtttcagtatcactgagcggatgacaggagtcttatccacaacatcattgaatggagagagagattttgtgtgttcacagtgtctctgggcagcatctcttaagcgccccttttggacgaagaggagagagagcaggctctcaatcacttccttctcaggcggagcgttgtccttgaagcaaatggtggacaccaggtctacgaagaaactgttgcacatctgccggaagcgggcatgcttttcaatggcttccctgtgcgcttgggaaacagctggagagaattcgtctggcaaggcagttaaacagtaggggcatatcatctgctctgaggcaaaccaggccctgaggcagcgcaggcagtgcacgtggtcgcagggcagacagacggggtcctttgcatctcccaggcagatggagcacggctgaatcccaaacctgctgagggtcttgctggctgtctccttgcattcacagagagtgcgcatcacggcctcaaaaggcccgtgcgtcttcacgtcagagttctctcgaagacacttgtctagtaagaagacgtgctcggtcaccagcccctgtaactcggggacgcggctctcggttcctaggagcacgtgctccacgaagagtgcggtggagaaaatccgactccactgggctctgacttccctgatgacagcctgggccaggctcccgctgccttgcatgtgctcatcggagcagatgagctccagcggcatggaaagattcttcaccaactgtagccacgcctggggactgggcttcagggtgtttcttgtcagcatctccgtgcaggccattgcggcaaatgcgtccagggtcatctcacatccagccagctcatggttccaacgggcttccatcaggctgtggagaacctgagggtagatggtcaggattctggaaaagttctgcagacggcttctgaaacgctggtaggcaaggtgcacccacggtaaggaaacctcttcctcgggcgcttctgacgccgctttcagtttcctagtgcaggaccacagagccatctgcagaaactttaattcctcctccgttgacacacgcatggtcaagagaatgaaatccttcaagtaacactgaagaagttcctgctgcggctctccatggagctgggcaagaaacctgcccagaggagtctgctgaaagatgtccacgaacttcttgggcagtccttctgcgtctgtgatgtactgagcctggacccacagctcctccagatagtccttgattttccagctgaaagggacgttgttggaagcgttctcggaaaggttcatgtggttctgcaccacgatgtaggccatctcacctttatgtctttcattattcatcacaagaggaatgttcagaagcatcgtgtcactgaaaataaacatccaaagatctcttgcccagggcggagtatctggcctggtcagtaactctaggttgccgtctctgtcgatgaatgatatcatgctcgccagcagaggggtgacagcaccttggacccgcttccagagggtgtgcctgaatgtgcccgcctcctggagagcgtcctggttgcaggcttcccttgccaaccactccagagggtgaaactggctctcttcttgcttctttaaaaagacactgaggcgcatcttggatacccgcaagaaagaggcgtggcacgcgtcatcctcattcaagaggcccaggaggagcaccaccctccgcatattgcgcgtgcagctctcgttctggtctctgagcatgcccacggcgctctgcacacagcttctcagcagcctggtggtgtccaggatcgacacatcactgcctccgagttcagaggtttcctttcccaccttctcagaactttctgtttccatggcctcctctgccacctctgccacctcccctgatgtgctggcctccgtctccatcgcctcctcatggccgtcttccgcccggtgttccaagcccagctcaggcaagtctccgggcgcgaacagctggctgatggtgacatgctgcagcctggtcacatcagaaaccatgagggtggatctccggaggtcatcgatgtggacagactgccacagccctccgtggaagcccacataggctgttcctcttcccacccgggacagttttgtgatgaaatagacgaagatacggtcctcattttctcgtattttgttgatttcatttataacagaatacttagctgaggcaatgagctgggcgctacggattccatcttcaaaatctgtctgaaaaatgaggattttacatttggctgtattcgttaaacagtttcggacttctttgaggaatgagtactcggtgtcaaactgctgcagccacaggagtgtgggtttcggagccctgcctgtgacctctgattctaaaatttcacagtcgtgacttgttagcagcctggagaaagtggtgatctctgtgaagatggcgtggcgctccaggtctgccgtgtgcaggtgtgcctgaaggaaatctgcaaaggagttgtgcctctgtctgtgaaagtactcctgcgacagccactccgctgcgaacccgcccagcgagtaggcgctcagccggaccacggcatcgggcgtagcgcagttcagcaggatcgatttggcctcctcagacaccttctggtgaagttcctccgtcaaggcccggggaccctgcctctctatgacctgcagcaccacagacgcgcaggcgtccgagtggtagccgatgaagacgtcagaggggctgtatttgtgcctcttctggaaatgatgtgctttgacattgatgaacttctccacccacgcacagagctcctccacgatgctcttctgccatttctccagcaccgtgttgatatccagatagtgcttctccagccggttaatgagggggatgggaaagtgtttgtacacgacgtctttctcttcaatgacaatcaggcggaagttggggtgaacccgacatttgacgcggtgggtccccagaccgaggtccacgtacttctggccgccgaggtggacgtagtactggttgagtgcgtcgtagaggctctcgtagaggttctgcaggttgagaagcaacaccatcttgcctgtttccatgcagatcttcacacgattgatgtttctgcagagctgggtgtactcttggtccttggggaaaccagaaccaaaaataatctccggctgctggtccccctcgaagaatgtctgctgcaggatctgcagtgccacgtagtttttggtcagcacgagtaagtagcgggactcagcatcttcctgctctccacccggcaccttctgagaaggcccaaagatgttctgtttgatcagctgcatggggctgacttcctctgagcacttggcctcgggcaaattggccagaaagatgtccaaagcttggatgtcatccttgccactgaagttcctaaggacagcctgtgcaatgtcttgcggggaaggctttctatttgaagcctttgctgcagcaaagaccattttgatgaggctgtagtagtcacgaagcccgaagaattccttgtcctggcgcttacacaccgtttcgtaggctttggcaaaggacgcaaagtacccttggactcggtcctggacgaggatgtctgaggagcagatgcccttggcgctctctatgagctctgtctcgttggggctgccacgtgacacaaaaatgccccggttcatcttggcagggtcaagggcccagttggagatgcccacgaagccgacctttttgtggggggcgggatcgtcttcaatgcatccgtcttccagcagcgggtgcagagtcttcaggggcattttgggtgagtcttccgccagccccacctcatctaacaccaccacagagacgtactgctgcaggtccttcccctgctgaaagcgggcgcactgccggaaggtgctgatgatgccctgtggggtggagtgcgggctgcactggaaggacaccaggtggacctgcttcaggctgcggaagagatctgagtaggcagccgggccctgcatggcgtctgccacgatggtcttggcgagagacttggagctgccgggcttccccaccaggaagaggggaatcttcagctcgatgcagacgaccatcatgaagacgttctccttcaaggccaagttcttggcgatggttttcctcagaggtacgccgtccagaaaaagatcctgtgcccgtgttatttcatccagaagcagcctgctgtcgtcatacggtttcggaaagaacctggcgatggctttccgatatgagtctttcttttctaaagaggcatggtaacacaccccgatggccagcatcaacgaccagaggacgggatctctctcggtgtgatttttgctgacgctggacttggagagaaaggcattcagctgcgctaagagcatcgcgctgtgctcgtggaaccacctgaaaactttcacacagcgctccacgtccctgaggctgacaaagctgcactcatcttctgttttcctcatgaaaccctgagaggcgcagaggacttctgtgatcacgcgagtcccgttttcatctaggctgatggactcaaccagtctctggacaatctgctggatgtagagcttttcagcaacgtcactcagttgtccaaagtcccacaccagaggaatcaggctcgggggcagagcatggacccggtataccagctgcctcagaggaatggagcccagcctgtcggccgtctcctccatactaaccctgtagcccaaaccagctgactccaaacggcagatcatctcctcagagtgcttccggtatggattgcaggcagctataatatgcaggccagagtcctcagccagaggctggccatccaccatatgatcacacaggacttctttgatacagcttatagcttccgttgtgttggcttcatcaaaaaacaagatggtgtccaactgatgttggtccttattggcgaaggccacattttcagcctccctgactctggagtagatcatgtctgcagttgttcctccgtgcaccttgaccagctttatggtgtcagcattggtaccaccacgccgcaggtcgctaaggaatttaataagcctggttttcccacagccagtttctcccatgatgataaccgggatcccacaccggaaccgcatctcgatggcaaggattttaagcatattgtcggttgtgagctcatacgttttgtcggggtcggtggcctgggggatccctaaggtcaggcagagcctctcaagtttcttgtgtctgggcagtttatcaaagtcgacattgaagggcaccctctggagcagcaggccctggtacaggtccctggtcatgacgtctctcttgatgaccttcccagtcaagtgactgatggcatcgacactgccgttgatgttgggctgcagatggaagccgatgaatgtcatggttgtgtggtcgtcattgaagaaaacgtatgggtgaggctccgactcccacctcttccggagggagaagggcgctagatcttcttccctaaccccatccatggtgaccatgtgcttccccgggctttggtcagaggtgtggagtgatggtgtggcaaaatctcttgccataaagatcatgaaggtcaccacgaacttcttgaagcccctcagtgtgtcgccaataaaactcggattgcagaagagagaggcctcacaatctctgagctgataattcaggaaccgagcaaagttccgaagctctgaccaggatgggtttattaccccgcagtgaaacaggaaatgctggaggcattcctccggggtgccttcgacagagccttcttgatactgaaacgtgtctaggtcttggttttgattgaatcgtcttaaatactggtaaggtctttggaaagtttcgctgcagaactcccacagatccatcccaggctctgtgtcactcctcagggcactcagctccatgtctatcacctctttgggaggcctgcaggtgacttttgggaagatgtcaagaaaactgaactggggtacacgtgtacgcagcgctgaagagctcctcgacggcactgacgtcctcctttccaggatttcaacgatatacaaatggcaggggttccgaagccacattttcccatttatatccattaagtattgtaaaatgaggagcttgaaaagaaacacccaaattccagtctgcactgaggaggtcacgtccaggtgaaagagcacggggaccttctgatactgcgcatccaggaagggcagcagggcgcccaggactcggctctcatccacctgagggtcgatcagtcgaattgttttcagaggcacatttttcacgtttaactgcatcttcattttgtcgtgcaacctcttcacgtacagagactttccaacacctgctcgctccgaggccacgatcccaacacacagccggtcattgaacacggctgccgccgacagggtctgcttcgggacccggtagtgacctgccaggtaggcttggatggcctcgaggggtgcctggggggtgacgaagaccttgtgctggctgaaggcagaggggaggtagcagtgctcccagtccccatcacagaccatgacgagctggtagtcttctcggtgctgctgcgtgcacagattgtggaaaagctcctccgcttggcgtgccacctcgtagctcagctgatctgcgaacagcaggctgtagaccttgtgccccagggagcccagggtcaggcagcggcgcagcaacagtgccacctcctcaaaggtggttgccggggtgcagagcagcacctcatcgtaagtgggcaggggctggcttggggtttgcatgtagacagccagggcggctggcaacacctcggagtggccacagacgacgaggttgggctggccgacctgcagacctctcgggagacaacgctccacgggagacccacccatccctgccaggtgagccagacagtggccaagggtctctaggtcgaggcagtcgggcaggaaggcaggaaggcacctcatggactgctccatgatgatcctcagcttgtccaccaggctgaactctgataagagcatcagcgggagctcttccatgactctcctcatgcggtacctggcggcctcactcccacaccccacagaggcccttaagacatccctcagggtgcagttgcttttgatgaaggatagcatcgttagggcggcatcactcgggggctgcttcctgagctcagtgctcaggtaaaccagctgctctgccgtgtagaagttcaggtaaaagtgctccattcgcttctgggtcacaaatctcttccagctgtcaaggaagtgctccatctgcctgcagagggctgccagcagctcagtgacatctccaccttctttaagctccgtcaccaggtccaagccaaagtccatttggagggacacaccctgcttgggggagcagtaggccatggcgatccacgtcctgaacagcatattcccagcagagtgcaggtcgatgaaggcctggctgagcctctgcacactgcagaagacctctgaaaacctctccacttccgtgttgttacgatccttcttgccagacatcagcatcaacttgttcaaaagctccttcacctcctctaaagagtactctcgtgactcctcgtggctgccagggctctcaggaaggatcaagtgcagaaccgtgtctggggaaatcttttggccacctttgggcgcctggatcacatagatgcctctttggttgatggccgtggccagggtcagggatgagcgttccacagacccatgactctcattcacagtcttcagccattccaagttcctggcggagtcacacagtttcctgggcaggtactggtccttatccagagccttccacagctttttcagatgcttcatgaatgcactgaagtccacgctggggtccagcttaaatagcagggatgcgtagccctgcacagcgtcatggaagcaggccacccggtccacatcaatgtcattctcccccgctgagatggaggccaggtccacaaacaccttcagctcattgatgcctccaagagcctcccggacccagcagatgaactcctttctcagggacagagcctgcagccccttgcaccgggcctcgctgatgtcctggagcagctttttggcctggatgagctcctggttgatctggtccagtgtttcacggcgaaagtcgtcgaagttatcagtaaaatttagtaaagtgttgagaacactgaagtcaccgttcagtcccaggctctctttgacctgcaagatgaccttggctgcgtggacagcctggtgcaggtgatggtattccttgatctgttcgactcggtccttgatccaatctctttggtcctggtggtccacggtgcacatgatcttaagttctgaatccaggtccgtgtatttattcacaaagtccttgaagatgacatcaatctctgcaagggtgacctctcctgactttagatcctggtgcaacttaatgaactttctgtaagaaggctgatacaaatagtcatacacctcttcaagctcaaggatgtgcctttctgattcttcttcgggctcactcagcaactctgcggcttcctggtcctccttaggctcactcagcggctctgcggcttcccgccagaagagctggaagatgtggctgtctctgagcaagtctatcttcccagccatttcttggacctgggagctcaggtggtaatgcgttgccctctgcgagttcgaggaggtggacagtctcactgtcacggtgtcatttaatcttttactgctgaggtcttgtgagtgtcttactgcaagcactccaaagtccacttgtatcagatgtttcacgttcccacacatcttcaggagactatcaacacatcttttctctttctttagaagtaacagttcctcccttctccaatccagtgcttcctccacagcacattgttcatcctggggtgaaagacttttttccctcagttgccagatgtcaagaaactgattcttgtgctttataatcagctccagttgtccaactaaaatcgtgccacttaggaggtcaccaacaactttcgtcaacacagagtcggcaacagctatcagcctcttggcatcctctgtgacatttgctagtattttctcgtcggttccacacaatctgaagacgtgcttgacatctgccaacgtgagcagatgctttaaaatgtcatcgaagttgtccgcggtcctaggccaggacttagtgatcacagcagacaagacgatgccaaatttccgcaaatcagagtaagagaacccctgaaggatactggtctgagactggcaggctgagctcacggcttcaatgatgcatttctcgaaggtcttggccacactgtcctctaagcctttggtgtcccagcaactattgcagtaggcagtgatctgggagaggggttcctcctttgtgagcctccattccatgtctcccagcaacgactccttccagccatgctccgcggggaattggatttccaccagccgcctccagacctcaatttccttgacgtatgtgaatgaggcacctgaagatgtgagcatgttctttgtaaaaacttctcggagccaccttttcgtagcagcaagggtcccttggaagactgtttggactgaattatttccagtttcatctctctgtcctgcagaatccaccagagatagaagtctaatcattctgcagacaatctcggcagataaggctggcagctcgtaaaacttaagtagctttgtgctgctgcagatggcttcatgcagtttcagacacacagtcaggtaggatggtgacaaggcctcctcgggaatcttgtcccggtaagtgtccaggagtcgcaacagcatttctaaaatgttctgaacgttctgaacatcctgaacatcctgcgtattcaagacttgctcaagtcccggaagccggtagtaaatccctgaaagacagtccaggatatgagcaggaaaacgacccaggtgctcaatgaagttttccatatacataaccaggtgactcagaggtagcagactaaaccaggaccggaagagaggctcgtctatgctcagcaaatgctgcttctctctcataaactgaagtagggaactcgtatctagcatttgttcccggaacggtgagaaggagagtccctccagagcggcccaggtgtcctcaggctgtctccaggcatccttgtgccgcggggccagctccatacagcagtgcaggacaggcagggcgcccagccaggtgtacgtccttgtgtccatgcatctttggcacaggttcaccaggtacagccgccagctctgaggtatcccaaggatgtggcttaggtcacggtgaaactcatctggtgagctggcatctgaggttaggaggtgacacaaccagtccaggctgccttctaataaaagctcaattttttccactacaaaaaggacaatcaggcctgttttcagtttactcctcactgggcagtccacaggcaaaaagtccgtgctttttccgtccggcaatggtaccacgtgttttttcagatgttgccacaggtatctcttcacctctttctccctgtactgcaaatcggtccacagctgtgcctgtccttcataaatcataggctgttgcaggacaaagcaaaactgctcgaactgggtgaagaagctgttcaggttgatggtgtcccaggtctgcaggatgctgaaggtgctgtccagcatgagcgcagcggcaatctgcttccccttcaccaggtccttcctcggcccgtctgtgatgtggttcatgactttctggagtctcccatgaggcttcatataaactatgtcatagtactgatgccagtctcctgagcccagaagtgaagattttatgaacagacagcggttgacgtactcgcccttcttctgctggtgcttgtaaatgaactcatactcaaaagattccccattataaatgacgtacttgtaaggaatgtatttatctaggtgcttcttggaaatgcagacaatgccttcaacaagaacgcggtcatgacccaagtctctggtgtagtgcagctcacagatattgctgtcccattttgactccccaaattcttctcctcctctgatgaagactttatggaggtcaggattgaatgggaaatgaagagagatgatggcgtggaagaacacggtgactcctccacccgggctcagcgtgcttgccttcacttcctggacatctgcttcctggtttttttgctccttctcgtttttcacagcagctgcacttctgttcttcccctctggcttcttgaggtcttcaggctccccttgttcattcttaccgactttttcttcagcagcagccatctcgtccttggtcttggtctcagcttcctggcagtgtgttttgaaaggaggagtggttgctggtggctgtttcattctctgggtcttctctttcatttccttcccggcccctttaactgcattggctggctcagctacagcatcaactgccatagaggctgaggcccctgcctgttgctcggtggtctgcagttctgtcccgggctcagagctgcctccttttgactcaggcaacaggagctcctgggcagcatcttcagtcctagaatggccttcaccagcagaggtggggggaccggtcccctcctgggacaggcctctgcccccagaggggatggaagcgtcctggtcctccccttccgtgtggtcctggaattgcgggctgctctgagcctcacttcctgtggccactcctgcctctcccaaagcctgggcctgcagggggctgtcgccaacctcggtgggcgcggagaggccgtcaccctccagtggcgtggtggctgtgcctgggggctggctcggctggccagtggggccactctgctgggcttggctgtggggcagggctgtgtcctgaggccacgggtttgaaagcaaagtcaggtgacaggggctggcaggagaaaggggcaaggaagccagctctgaggaagcggacttgttccccttctttttcttcttccttttcttctttttgctttcttggacggtccaggaggctttggaacagggctcctcggggttttcttgccaactgtctgagcccgggaacaagcacgggcccccttcctccttcagctcctgcccacactccatttcaccctccgaggccgacgccattgtggagttattgttctcagaatctgctatgggggctgcaggaggcagcctctctccgcactggctgcagaacttgggggtttcctccttggagacatgctggcacgaaggacactccatgggtcctgctgggactgccctgcagatccagaagcaagagcaggagtcgctggcagcctgctatatactacatgtcctgtcacgtgaccacggcttcagtttcattttctgcggcccccgagctcgccgcctgccgcgcgctgtcgcccctcgggtcac

SEQ ID NO: 8775 - RNA, 1115 nt, Homo sapiens
  source 1..1115: mol_type = other RNA
aagtcctgcttctgttgcagcactaagtgctctggagaggtctgtgtttgcgcctgcttctgcagctttggctgcacctgggtgtctgtggatggtatccgcggctgagtctgtgactgcacctgggcctggacctgcaggacccgtggctggaatcgtggcagcacttgggcttccagggcctcaggcagcaggtctggtgtctgtgtctgtttcggtactgtcatccgggcctgcggctgggccttcacctgtaactgccctggaggttccttctctgtgggctcttctgagctcctcaatctctttgctggcagctcggacgcctcacaaggctcaggctcaggtgctggagtgcgtttttccttggcgatgtcctctgggcagggcggtaaatcttggtcttctggtgtgtccatccggggctctgcggcttcctcagacccctctggggggtctgacttgtcttccacaggcattgtctgagaagaagaatcctttcgattgggggtggtagaggaggaggtccgggcctgtttctgggggttccgtcctgaaaggttgaactgggaagggttcatggggaccccaacaggaggaggtcccagcaaggactggcgagtggcctggggaaagaactgttgcaaatttggagtggccagttgtgggggtgtgaggctgggggctgcgaggcctggggatgccatgccatagcctcggaggttacccagtgttgctgtgggcatggtgagaccggcagtgtcatacgtggctggtggcattgcaaactggtccagtccggctgacagccatgggcaacggggcctgtggtggggactgctggagcagctgctggagctgcagtaactgctgctgctgcaattgctgctgctggagctgctgctgctgtaactgctggagctgctgctgctgttgctggagctgctgctgctgctgctggctgaacatggtggctcgcctccccgcgcgccctcaacgctcaagtcgcccccacggatgggccggccccgcagcccccacgcctcggccgggcggctccggcccgcgggctcccggcctccccgctgctactccggggcctgtgggctcgtaag

SEQ ID NO: 8776 - RNA, 1158 nt, Homo sapiens
  source 1..1158: mol_type = other RNA
aagtcctgcttctgttgcagcactaagtgctctggagaggtctgtgtttgcgcctgcttctgcagctttggctgcacctgggtgtctgtggatggtatccgcggctgagtctgtgactgcacctgggcctggacctgcaggacccgtggctggaatcgtggcagcacttgggcttccagggcctcaggcagcaggtctggtgtctgtgtctgtttcggtactgtcatccgggcctgcggctgggccttcacctgtaactgccctggaggttccttctctgtgggctcttctgagctcctcaatctctttgctggcagctcggacgcctcacaaggctcaggctcaggtgctggagtgcgtttttccttggcgatgtcctctgggcagggcggtaaatcttggtcttctggtgtgtccatccggggctctgcggcttcctcagacccctctggggggtctgacttgtcttccacaggcattgtctgagaagaagaatcctttcgattgggggtggtagaggaggaggtccgggcctgtttctgggggttccgtcctgaaaggttgaactgggaagggttcatggggaccccaacaggaggaggtcccagcaaggactggcgagtggcctggggaaagaactgttgcaaatttggagtggccagttgtgggggtgtgaggctgggggctgcgaggcctggggatgccatgccatagcctcggaggttacccagtgttgctgtgggcatggtgagaccggcagtgtcatacgtggctggtggcattgcaaactggtccagtccttgcaactgctgtaaaagcaaagctctctgcagcatggagccgttgaggagggaggctgagttggtgccctggagattcagaagcggctgctgtggctgctgcggggggagcccccggctgacagccatgggcaacggggcctgtggtggggactgctggagcagctgctggagctgcagtaactgctgctgctgcaattgctgctgctggagctgctgctgctgtaactgctggagctgctgctgctgttgctggagctgctgctgctgctgctggctgaacatggtggagccccttttcaataccgcaaccctctctgggcccccgggtgtcaataacatcggcacccgtccaacc

SEQ ID NO: 8777 - RNA, 1193 nt, Homo sapiens
  source 1..1193: mol_type = other RNA
aagtcctgcttctgttgcagcactaagtgctctggagaggtctgtgtttgcgcctgcttctgcagctttggctgcacctgggtgtctgtggatggtatccgcggctgagtctgtgactgcacctgggcctggacctgcaggacccgtggctggaatcgtggcagcacttgggcttccagggcctcaggcagcaggtctggtgtctgtgtctgtttcggtactgtcatccgggcctgcggctgggccttcacctgtaactgccctggaggttccttctctgtgggctcttctgagctcctcaatctctttgctggcagctcggacgcctcacaaggctcaggctcaggtgctggagtgcgtttttccttggcgatgtcctctgggcagggcggtaaatcttggtcttctggtgtgtccatccggggctctgcggcttcctcagacccctctggggggtctgacttgtcttccacaggcattgtctgagaagaagaatcctttcgattgggggtggtagaggaggaggtccgggcctgtttctgggggttccgtcctgaaaggttgaactgggaagggttcatggggaccccaacaggaggaggtcccagcaaggactggcgagtggcctggggaaagaactgttgcaaatttggagtggccagttgtgggggtgtgaggctgggggctgcgaggcctggggatgccatgccatagcctcggaggttacccagtgttgctgtgggcatggtgagaccggcagtgtcatacgtggctggtggcattgcaaactggtccagtccttgcaactgctgtaaaagcaaagctctctgcagcatggagccgttgaggagggaggctgagttggtgccctggagattcagaagcggctgctgtggctgctgcggggggagcccccggctgacagccatgggcaacggggcctgtggtggggactgctggagcagctgctggagctgcagtaactgctgctgctgcaattgctgctgctggagctgctgctgctgtaactgctggagctgctgctgctgttgctggagctgctgctgctgctgctggctgaacatggtggcctctgtcccgcgtcctccgcatcgcgaaggggaggctcggagaccaaggtccgtctgccgcccggaagggtcagccatcccgcggggcatcgagggggactt

SEQ ID NO: 8778 - RNA, 1251 nt, Homo sapiens
  source 1..1251: mol_type = other RNA
aagtcctgcttctgttgcagcactaagtgctctggagaggtctgtgtttgcgcctgcttctgcagctttggctgcacctgggtgtctgtggatggtatccgcggctgagtctgtgactgcacctgggcctggacctgcaggacccgtggctggaatcgtggcagcacttgggcttccagggcctcaggcagcaggtctggtgtctgtgtctgtttcggtactgtcatccgggcctgcggctgggccttcacctgtaactgccctggaggttccttctctgtgggctcttctgagctcctcaatctctttgctggcagctcggacgcctcacaaggctcaggctcaggtgctggagtgcgtttttccttggcgatgtcctctgggcagggcggtaaatcttggtcttctggtgtgtccatccggggctctgcggcttcctcagacccctctggggggtctgacttgtcttccacaggcattgtctgagaagaagaatcctttcgattgggggtggtagaggaggaggtccgggcctgtttctgggggttccgtcctgaaaggttgaactgggaagggttcatggggaccccaacaggaggaggtcccagcaaggactggcgagtggcctggggaaagaactgttgcaaatttggagtggccagttgtgggggtgtgaggctgggggctgcgaggcctggggatgccatgccatagcctcggaggttacccagtgttgctgtgggcatggtgagaccggcagtgtcatacgtggctggtggcattgcaaactggtccagtccttgcaactgctgtaaaagcaaagctctctgcagcatggagccgttgaggagggaggctgagttggtgccctggagattcagaagcggctgctgtggctgctgcggggggagcccccggctgacagccatgggcaacggggcctgtggtggggactgctggagcagctgctggagctgcagtaactgctgctgctgcaattgctgctgctggagctgctgctgctgtaactgctggagctgctgctgctgttgctggagctgctgctgctgctgctggctgaacatggtggcgtggtcctgagctccgtgggacggcttctctccaccaccgccacctcctcgcgccccactccgcccgctcccaccccgccagccgcctcctccgcagacacagccagctcgcaggcggagccccacgacccagccgcccccggccccgcacctcgcctcc

SEQ ID NO: 8779 - RNA, 1340 nt, Homo sapiens
  source 1..1340: mol_type = other RNA
aagtcctgcttctgttgcagcactaagtgctctggagaggtctgtgtttgcgcctgcttctgcagctttggctgcacctgggtgtctgtggatggtatccgcggctgagtctgtgactgcacctgggcctggacctgcaggacccgtggctggaatcgtggcagcacttgggcttccagggcctcaggcagcaggtctggtgtctgtgtctgtttcggtactgtcatccgggcctgcggctgggccttcacctgtaactgccctggaggttccttctctgtgggctcttctgagctcctcaatctctttgctggcagctcggacgcctcacaaggctcaggctcaggtgctggagtgcgtttttccttggcgatgtcctctgggcagggcggtaaatcttggtcttctggtgtgtccatccggggctctgcggcttcctcagacccctctggggggtctgacttgtcttccacaggcattgtctgagaagaagaatcctttcgattgggggtggtagaggaggaggtccgggcctgtttctgggggttccgtcctgaaaggttgaactgggaagggttcatggggaccccaacaggaggaggtcccagcaaggactggcgagtggcctggggaaagaactgttgcaaatttggagtggccagttgtgggggtgtgaggctgggggctgcgaggcctggggatgccatgccatagcctcggaggttacccagtgttgctgtgggcatggtgagaccggcagtgtcatacgtggctggtggcattgcaaactggtccagtccttgcaactgctgtaaaagcaaagctctctgcagcatggagccgttgaggagggaggctgagttggtgccctggagattcagaagcggctgctgtggctgctgcggggggagcccccggctgacagccatgggcaacggggcctgtggtggggactgctggagcagctgctggagctgcagtaactgctgctgctgcaattgctgctgctggagctgctgctgctgtaactgctggagctgctgctgctgttgctggagctgctgctgctgctgctggctgaacatggtggctccctgcggccgccgcggtcctgcgatcctggggccccgcgcggggctgcggtgagagggggcgcgcagttggcggatgtacattcattcgagggacccaggccaggcgagagggcggccaaggtcttacagtccgtcaggagtttgcccacggaggggtggagggagagtccccctccaagtcttttctcagtagatttggctaaggaaggagtaggtgaggagggtcgaggccaattatcaaaaaat

SEQ ID NO: 8780 - RNA, 1456 nt, Homo sapiens
  source 1..1456: mol_type = other RNA
aagtcctgcttctgttgcagcactaagtgctctggagaggtctgtgtttgcgcctgcttctgcagctttggctgcacctgggtgtctgtggatggtatccgcggctgagtctgtgactgcacctgggcctggacctgcaggacccgtggctggaatcgtggcagcacttgggcttccagggcctcaggcagcaggtctggtgtctgtgtctgtttcggtactgtcatccgggcctgcggctgggccttcacctgtaactgccctggaggttccttctctgtgggctcttctgagctcctcaatctctttgctggcagctcggacgcctcacaaggctcaggctcaggtgctggagtgcgtttttccttggcgatgtcctctgggcagggcggtaaatcttggtcttctggtgtgtccatccggggctctgcggcttcctcagacccctctggggggtctgacttgtcttccacaggcattgtctgagaagaagaatcctttcgattgggggtggtagaggaggaggtccgggcctgtttctgggggttccgtcctgaaaggttgaactgggaagggttcatggggaccccaacaggaggaggtcccagcaaggactggcgagtggcctggggaaagaactgttgcaaatttggagtggccagttgtgggggtgtgaggctgggggctgcgaggcctggggatgccatgccatagcctcggaggttacccagtgttgctgtgggcatggtgagaccggcagtgtcatacgtggctggtggcattgcaaactggtccagtccttgcaactgctgtaaaagcaaagctctctgcagcatggagccgttgaggagggaggctgagttggtgccctggagattcagaagcggctgctgtggctgctgcggggggagcccccggctgacagccatgggcaacggggcctgtggtggggactgctggagcagctgctggagctgcagtaactgctgctgctgcaattgctgctgctggagctgctgctgctgtaactgctggagctgctgctgctgttgctggagctgctgctgctgctgctggctgaacatggtggctccctgcggccgccgcggtcctgcgatcctggggccccgcgcggggctgcggtgagagggggcgcgcagttggcggatgtacattcattcgagggacccaggccaggcgagagggcggccaaggtcttacagtccgtcaggagtttgcccacggaggggtggagggagagtccccctccaagtcttttctcagtagatttggctaaggaaggagtaggtgaggagggtcgaggccaattatcaaaaaatagccctaggggccgggcgcttccgcctgtaatctcagtactctgggaggccgaggctggaggatcaagaccagcctgggcaaaatggcgaaatccctctctacaaaaaatacaaac

SEQ ID NO: 8781 - RNA, 1231 nt, Homo sapiens
  source 1..1231: mol_type = other RNA
aagtcctgcttctgttgcagcactaagtgctctggagaggtctgtgtttgcgcctgcttctgcagctttggctgcacctgggtgtctgtggatggtatccgcggctgagtctgtgactgcacctgggcctggacctgcaggacccgtggctggaatcgtggcagcacttgggcttccagggcctcaggcagcaggtctggtgtctgtgtctgtttcggtactgtcatccgggcctgcggctgggccttcacctgtaactgccctggaggttccttctctgtgggctcttctgagctcctcaatctctttgctggcagctcggacgcctcacaaggctcaggctcaggtgctggagtgcgtttttccttggcgatgtcctctgggcagggcggtaaatcttggtcttctggtgtgtccatccggggctctgcggcttcctcagacccctctggggggtctgacttgtcttccacaggcattgtctgagaagaagaatcctttcgattgggggtggtagaggaggaggtccgggcctgtttctgggggttccgtcctgaaaggttgaactgggaagggttcatggggaccccaacaggaggaggtcccagcaaggactggcgagtggcctggggaaagaactgttgcaaatttggagtggccagttgtgggggtgtgaggctgggggctgcgaggcctggggatgccatgccatagcctcggaggttacccagtgttgctgtgggcatggtgagaccggcagtgtcatacgtggctggtggcattgcaaactggtccagtccttgcaactgctgtaaaagcaaagctctctgcagcatggagccgttgaggagggaggctgagttggtgccctggagattcagaagcggctgctgtggctgctgcggggggagcccccggctgacagccatgggcaacggggcctgtggtggggactgctggagcagctgctggagctgcagtaactgctgctgctgcaattgctgctgctggagctgctgctgctgtaactgctggagctgctgctgctgttgctggagctgctgctgctgctgctggctgaacatggtggctcgcctccccgcgcgccctcaacgctcaagtcgcccccacggatgggccggccccgcagcccccacgcctcggccgggcggctccggcccgcgggctcccggcctccccgctgctactccggggcctgtgggctcgtaag

SEQ ID NO: 8782 - RNA, 1235 nt, Homo sapiens
  source 1..1235: mol_type = other RNA
aagtcctgcttctgttgcagcactaagtgctctggagaggtctgtgtttgcgcctgcttctgcagctttggctgcacctgggtgtctgtggatggtatccgcggctgagtctgtgactgcacctgggcctggacctgcaggacccgtggctggaatcgtggcagcacttgggcttccagggcctcaggcagcaggtctggtgtctgtgtctgtttcggtactgtcatccgggcctgcggctgggccttcacctgtaactgccctggaggttccttctctgtgggctcttctgagctcctcaatctctttgctggcagctcggacgcctcacaaggctcaggctcaggtgctggagtgcgtttttccttggcgatgtcctctgggcagggcggtaaatcttggtcttctggtgtgtccatccggggctctgcggcttcctcagacccctctggggggtctgacttgtcttccacaggcattgtctgagaagaagaatcctttcgattgggggtggtagaggaggaggtccgggcctgtttctgggggttccgtcctgaaaggttgaactgggaagggttcatggggaccccaacaggaggaggtcccagcaaggactggcgagtggcctggggaaagaactgttgcaaatttggagtggccagttgtgggggtgtgaggctgggggctgcgaggcctggggatgccatgccatagcctcggaggttacccagtgttgctgtgggcatggtgagaccggcagtgtcatacgtggctggtggcattgcaaactggtccagtccttgcaactgctgtaaaagcaaagctctctgcagcatggagccgttgaggagggaggctgagttggtgccctggagattcagaagcggctgctgtggctgctgcggggggagcccccggctgacagccatgggcaacggggcctgtggtggggactgctggagcagctgctggagctgcagtaactgctgctgctgcaattgctgctgctggagctgctgctgctgtaactgctggagctgctgctgctgttgctggagctgctgctgctgctgctggctgaacatggtggctcgcctccccgcgcgccctcaacgctcaagtcgcccccacggatgggccggccccgcagcccccacgcctcggccgggcggctccggcccgcgggctcccggcctccccgctgctactccggggcctgtgggctcgtaaggccc

SEQ ID NO: 8783 - RNA, 1127 nt, Homo sapiens
  source 1..1127: mol_type = other RNA
aagtcctgcttctgttgcagcactaagtgctctggagaggtctgtgtttgcgcctgcttctgcagctttggctgcacctgggtgtctgtggatggtatccgcggctgagtctgtgactgcacctgggcctggacctgcaggacccgtggctggaatcgtggcagcacttgggcttccagggcctcaggcagcaggtctggtgtctgtgtctgtttcggtactgtcatccgggcctgcggctgggccttcacctgtaactgccctggaggttccttctctgtgggctcttctgagctcctcaatctctttgctggcagctcggacgcctcacaaggctcaggctcaggtgctggagtgcgtttttccttggcgatgtcctctgggcagggcggtaaatcttggtcttctggtgtgtccatccggggctctgcggcttcctcagacccctctggggggtctgacttgtcttccacaggcattgtctgagaagaagaatcctttcgattgggggtggtagaggaggaggtccgggcctgtttctgggggttccgtcctgaaaggttgaactgggaagggttcatggggaccccaacaggaggaggtcccagcaaggactggcgagtggcctggggaaagaactgttgcaaatttggagtggccagttgtgggggtgtgaggctgggggctgcgaggcctggggatgccatgccatagcctcggaggttacccagtgttgctgtgggcatggtgagaccggcagtgtcatacgtggctggtggcattgcaaactggtccagtccttgcaactgctgtaaaagcaaagctctctgcagcatggagccgttgaggagggaggctgagttggtgccctggagattcagaagcggctgctgtggctgctgcggggggagcccccggctgacagccatgggcaacggggcctgtggtggggactgctggagcagctgctggagctgcagtaactgctgctgctgcaattgctgctgctggagctgctgctgctgtaactgctggagctgctgctgctgttgctggagctgctgctgctgctgctggctgaacatggtggctctgcggctcccgccgccatccgtgcgcagcgcggc

SEQ ID NO: 8784 - RNA, 1042 nt, Homo sapiens
  source 1..1042: mol_type = other RNA
aagtcctgcttctgttgcagcactaagtgctctggagaggtctgtgtttgcgcctgcttctgcagctttggctgcacctgggtgtctgtggatggtatccgcggctgagtctgtgactgcacctgggcctggacctgcaggacccgtggctggaatcgtggcagcacttgggcttccagggcctcaggcagcaggtctggtgtctgtgtctgtttcggtactgtcatccgggcctgcggctgggccttcacctgtaactgccctggaggttccttctctgtgggctcttctgagctcctcaatctctttgctggcagctcggacgcctcacaaggctcaggctcaggtgctggagtgcgtttttccttggcgatgtcctctgggcagggcggtaaatcttggtcttctggtgtgtccatccggggctctgcggcttcctcagacccctctggggggtctgacttgtcttccacaggcattgtctgagaagaagaatcctttcgattgggggtggtagaggaggaggtccgggcctgtttctgggggttccgtcctgaaaggttgaactgggaagggttcatggggaccccaacaggaggaggtcccagcaaggactggcgagtggcctggggaaagaactgttgcaaatttggagtggccagttgtgggggtgtgaggctgggggctgcgaggcctggggatgccatgccatagcctcggaggttaccttgcaactgctgtaaaagcaaagctctctgcagcatggagccgttgaggagggaggctgagttggtgccctggagattcagaagcggctgctgtggctgctgcggggggagcccccggctgacagccatgggcaacggggcctgtggtggggactgctggagcagctgctggagctgcagtaactgctgctgctgcaattgctgctgctggagctgctgctgctgtaactgctggagctgctgctgctgttgctggagctgctgctgctgctgctggctgaacatggtggcctctgtcccgcgtcctccgcatc

SEQ ID NO: 8785 - RNA, 1159 nt, Homo sapiens
  source 1..1159: mol_type = other RNA
aagtcctgcttctgttgcagcactaagtgctctggagaggtctgtgtttgcgcctgcttctgcagctttggctgcacctgggtgtctgtggatggtatccgcggctgagtctgtgactgcacctgggcctggacctgcaggacccgtggctggaatcgtggcagcacttgggcttccagggcctcaggcagcaggtctggtgtctgtgtctgtttcggtactgtcatccgggcctgcggctgggccttcacctgtaactgccctggaggttccttctctgtgggctcttctgagctcctcaatctctttgctggcagctcggacgcctcacaaggctcaggctcaggtgctggagtgcgtttttccttggcgatgtcctctgggcagggcggtaaatcttggtcttctggtgtgtccatccggggctctgcggcttcctcagacccctctggggggtctgacttgtcttccacaggcattgtctgagaagaagaatcctttcgattgggggtggtagaggaggaggtccgggcctgtttctgggggttccgtcctgaaaggttgaactgggaagggttcatggggaccccaacaggaggaggtcccagcaaggactggcgagtggcctggggaaagaactgttgcaaatttggagtggccagttgtgggggtgtgaggctgggggctgcgaggcctggggatgccatgccatagcctcggaggttaccttgcaactgctgtaaaagcaaagctctctgcagcatggagccgttgaggagggaggctgagttggtgccctggagattcagaagcggctgctgtggctgctgcggggggagcccccggctgacagccatgggcaacggggcctgtggtggggactgctggagcagctgctggagctgcagtaactgctgctgctgcaattgctgctgctggagctgctgctgctgtaactgctggagctgctgctgctgttgctggagctgctgctgctgctgctggctgaacatggtggctcgcctccccgcgcgccctcaacgctcaagtcgcccccacggatgggccggccccgcagcccccacgcctcggccgggcggctccggcccgcgggctcccggcctccccgctgctactccggggcctgtgggctcgtaag

SEQ ID NO: 8786 - RNA, 1178 nt, Homo sapiens
  source 1..1178: mol_type = other RNA
aagtcctgcttctgttgcagcactaagtgctctggagaggtctgtgtttgcgcctgcttctgcagctttggctgcacctgggtgtctgtggatggtatccgcggctgagtctgtgactgcacctgggcctggacctgcaggacccgtggctggaatcgtggcagcacttgggcttccagggcctcaggcagcaggtctggtgtctgtgtctgtttcggtactgtcatccgggcctgcggctgggccttcacctgtaactgccctggaggttccttctctgtgggctcttctgagctcctcaatctctttgctggcagctcggacgcctcacaaggctcaggctcaggtgctggagtgcgtttttccttggcgatgtcctctgggcagggcggtaaatcttggtcttctggtgtgtccatccggggctctgcggcttcctcagacccctctggggggtctgacttgtcttccacaggcattgtctttcgattgggggtggtagaggaggaggtccgggcctgtttctgggggttccgtcctgaaaggttgaactgggaagggttcatggggaccccaacaggaggaggtcccagcaaggactggcgagtggcctggggaaagaactgttgcaaatttggagtggccagttgtgggggtgtgaggctgggggctgcgaggcctggggatgccatgccatagcctcggaggttacccagtgttgctgtgggcatggtgagaccggcagtgtcatacgtggctggtggcattgcaaactggtccagtccttgcaactgctgtaaaagcaaagctctctgcagcatggagccgttgaggagggaggctgagttggtgccctggagattcagaagcggctgctgtggctgctgcggggggagcccccggctgacagccatgggcaacggggcctgtggtggggactgctggagcagctgctggagctgcagtaactgctgctgctgcaattgctgctgctggagctgctgctgctgtaactgctggagctgctgctgctgttgctggagctgctgctgctgctgctggctgaacatggtggcctctgtcccgcgtcctccgcatcgcgaaggggaggctcggagaccaaggtccgtctgccgcccggaagggtcagccatcccgcggggcatcgagggggactt

SEQ ID NO: 8787 - RNA, 1216 nt, Homo sapiens
  source 1..1216: mol_type = other RNA
aagtcctgcttctgttgcagcactaagtgctctggagaggtctgtgtttgcgcctgcttctgcagctttggctgcacctgggtgtctgtggatggtatccgcggctgagtctgtgactgcacctgggcctggacctgcaggacccgtggctggaatcgtggcagcacttgggcttccagggcctcaggcagcaggtctggtgtctgtgtctgtttcggtactgtcatccgggcctgcggctgggccttcacctgtaactgccctggaggttccttctctgtgggctcttctgagctcctcaatctctttgctggcagctcggacgcctcacaaggctcaggctcaggtgctggagtgcgtttttccttggcgatgtcctctgggcagggcggtaaatcttggtcttctggtgtgtccatccggggctctgcggcttcctcagacccctctggggggtctgacttgtcttccacaggcattgtctttcgattgggggtggtagaggaggaggtccgggcctgtttctgggggttccgtcctgaaaggttgaactgggaagggttcatggggaccccaacaggaggaggtcccagcaaggactggcgagtggcctggggaaagaactgttgcaaatttggagtggccagttgtgggggtgtgaggctgggggctgcgaggcctggggatgccatgccatagcctcggaggttacccagtgttgctgtgggcatggtgagaccggcagtgtcatacgtggctggtggcattgcaaactggtccagtccttgcaactgctgtaaaagcaaagctctctgcagcatggagccgttgaggagggaggctgagttggtgccctggagattcagaagcggctgctgtggctgctgcggggggagcccccggctgacagccatgggcaacggggcctgtggtggggactgctggagcagctgctggagctgcagtaactgctgctgctgcaattgctgctgctggagctgctgctgctgtaactgctggagctgctgctgctgttgctggagctgctgctgctgctgctggctgaacatggtggctcgcctccccgcgcgccctcaacgctcaagtcgcccccacggatgggccggccccgcagcccccacgcctcggccgggcggctccggcccgcgggctcccggcctccccgctgctactccggggcctgtgggctcgtaag

SEQ ID NO: 8788 - RNA, 1220 nt, Homo sapiens
  source 1..1220: mol_type = other RNA
aagtcctgcttctgttgcagcactaagtgctctggagaggtctgtgtttgcgcctgcttctgcagctttggctgcacctgggtgtctgtggatggtatccgcggctgagtctgtgactgcacctgggcctggacctgcaggacccgtggctggaatcgtggcagcacttgggcttccagggcctcaggcagcaggtctggtgtctgtgtctgtttcggtactgtcatccgggcctgcggctgggccttcacctgtaactgccctggaggttccttctctgtgggctcttctgagctcctcaatctctttgctggcagctcggacgcctcacaaggctcaggctcaggtgctggagtgcgtttttccttggcgatgtcctctgggcagggcggtaaatcttggtcttctggtgtgtccatccggggctctgcggcttcctcagacccctctggggggtctgacttgtcttccacaggcattgtctttcgattgggggtggtagaggaggaggtccgggcctgtttctgggggttccgtcctgaaaggttgaactgggaagggttcatggggaccccaacaggaggaggtcccagcaaggactggcgagtggcctggggaaagaactgttgcaaatttggagtggccagttgtgggggtgtgaggctgggggctgcgaggcctggggatgccatgccatagcctcggaggttacccagtgttgctgtgggcatggtgagaccggcagtgtcatacgtggctggtggcattgcaaactggtccagtccttgcaactgctgtaaaagcaaagctctctgcagcatggagccgttgaggagggaggctgagttggtgccctggagattcagaagcggctgctgtggctgctgcggggggagcccccggctgacagccatgggcaacggggcctgtggtggggactgctggagcagctgctggagctgcagtaactgctgctgctgcaattgctgctgctggagctgctgctgctgtaactgctggagctgctgctgctgttgctggagctgctgctgctgctgctggctgaacatggtggctcgcctccccgcgcgccctcaacgctcaagtcgcccccacggatgggccggccccgcagcccccacgcctcggccgggcggctccggcccgcgggctcccggcctccccgctgctactccggggcctgtgggctcgtaaggccc

SEQ ID NO: 8789 - RNA, 1027 nt, Homo sapiens
  source 1..1027: mol_type = other RNA
aagtcctgcttctgttgcagcactaagtgctctggagaggtctgtgtttgcgcctgcttctgcagctttggctgcacctgggtgtctgtggatggtatccgcggctgagtctgtgactgcacctgggcctggacctgcaggacccgtggctggaatcgtggcagcacttgggcttccagggcctcaggcagcaggtctggtgtctgtgtctgtttcggtactgtcatccgggcctgcggctgggccttcacctgtaactgccctggaggttccttctctgtgggctcttctgagctcctcaatctctttgctggcagctcggacgcctcacaaggctcaggctcaggtgctggagtgcgtttttccttggcgatgtcctctgggcagggcggtaaatcttggtcttctggtgtgtccatccggggctctgcggcttcctcagacccctctggggggtctgacttgtcttccacaggcattgtctttcgattgggggtggtagaggaggaggtccgggcctgtttctgggggttccgtcctgaaaggttgaactgggaagggttcatggggaccccaacaggaggaggtcccagcaaggactggcgagtggcctggggaaagaactgttgcaaatttggagtggccagttgtgggggtgtgaggctgggggctgcgaggcctggggatgccatgccatagcctcggaggttaccttgcaactgctgtaaaagcaaagctctctgcagcatggagccgttgaggagggaggctgagttggtgccctggagattcagaagcggctgctgtggctgctgcggggggagcccccggctgacagccatgggcaacggggcctgtggtggggactgctggagcagctgctggagctgcagtaactgctgctgctgcaattgctgctgctggagctgctgctgctgtaactgctggagctgctgctgctgttgctggagctgctgctgctgctgctggctgaacatggtggcctctgtcccgcgtcctccgcatc

SEQ ID NO: 8790 - RNA, 26 nt, Homo sapiens
  source 1..26: mol_type = other RNA
aagtgatctaaaggcctacatataaa

SEQ ID NO: 8791 - RNA, 26 nt, Homo sapiens
  source 1..26: mol_type = other RNA
aagtgcccccacagtttgagtgccac

SEQ ID NO: 8792 - RNA, 27 nt, Homo sapiens
  source 1..27: mol_type = other RNA
aagtgccgccatcttttgagtgttacc

SEQ ID NO: 8793 - RNA, 2995 nt, Homo sapiens
  source 1..2995: mol_type = other RNA
aagtgcctccttttagagtgttctggtccctcttcattattagattgggaatcaggttagtctggagtggtagagctcaaatccagcaccctagagcccagaggtcacaggaagggctgcataaagggggtacagtgggtgaccagtcaaggtggggagtgcttcatgcccaggggaagaccacaggagactgcagacagctggaatggtggtaatttgggggaacttgtacatgggtgaagcaagtatgtgtggatggggaattgtcaggtgtcagatacccagcgggggatggaggcatgtgattttatctccattctgctgggccatgtggggattatgaggctgcctgcttgcgagtgcactagggagagtggggtgggcccagtgctgtgctgggctcagctgtgtgtatgtgtttgcctttgcctctgcctgtacagaagctgtgtgctggtgggagagtaaaaagctcggtggattgcctttggagagtttgttaggggagactctccccatatgggaaacactccaagccagcaggccagtttcacactgtccaggctgcagttaactcccatcagtgccctgcttctcacccctcttgctcctggaaagggccggacagcagatgggaggctgggggactcttggggagaaggataaaaatgaagtacagaaaggttgatggttctctcactgctcctctcttccaagccagcccagcgtctactgggctggggctggggtctgaaggagtctggatgaaagtccttcccactcagagaagccattctcagacctccaatgggttctagggctgtgcccctccctctgctctggtccatgtgctaggctgtggaggtttgcaggccaggaggcggaggcagcccttctgaagacaaagggcaatgttggggggcgggcgaggaagagagaagggagttgggtggggggctggagcgcccccctccttcattctcacgggcctgggaaactggggctgagtgggacctcaatggctggtagcccctttaagggtgaattctcctcccgcctcgtaaattacgctggtccaccctctggccggcccgtgaggcagtgaccgtgaacgccagcggggaagggagaatcagaggcctcggctgtggctgtcagaaattctcccggccaatcagtgtggtgctccgtagccccatctacagcctcttgcactttctttctggagagccagctggggacctctggggtggctactgaacctgaggctgtgtcccctgggctctcaggtccctgcttgctgcatcaggcctgcagccaccgcaggcaacggaggagtggatggcagcacacctatgaacagacattcgcccggtgcgggcagcgggatcaggagagggctggggaccaggacactgttctggtcctagagggaacatgaggctgatagtccttgtccacagcccggccagccaaatgcccaagcttctgcccactgggtgtcctgggggacccagacccaagcagactctggttcttgctaatcattttctcacaaaccacacttcctccttggttccccacttcctccagccctaccagagacacctgactccctcagctctctccgctgaccctccaccctcctctctcttcccagcctcttctaaccccaggaactgtgaggttgaggtgccttggttccactggccctgctctttgctcctgacggcaaagagaattaagaccatggaagggaagtagaggaaggggacatctgggccgctgcttctccagatcctcagcggaggtgcagtgccccagtcctgcctcaaataaaccagcccgcagcacctcagccttcctgcccctgccaaccgcaggcagctgccggcttctgctctccctggctaggtttcttcccttctctctgggacctggcagggtgttttgggtgtgtatgggagggaaccacgaacaaaacagacaagaggatatccagggagggcctgccagagacgcctggcgttctaagtggggactgtgttctaggcggcgccctcttttgctctctgccagggacaggctcagtctggggctggcgcccgtgtcctgcaccttaaaagaaggagagagcttgctccctcaacagaagtcttttctttttcattctccggttctgaaaccagatcttgacctgctggtcactaagattcaagcggtctgagagttccctccggcgctggcgtgtgatgaactcgttgaccagaaactcgccctccagctctgccagttgcaacttcgaatagggcttgcgcttcttccgagagcggctgttgatcgggtaccagggcgcgccgctggccgagagcccgccgccggggttcaacggcgataccaagctgccggggtcgcctgcgccggcgcccttgttgccctcgttgagcagggacgaactggagtcggattccagcgactggcaggagggcgggtcgtgcggaggtcctgcgccgccgccgccgtcgccaccgccgccgcccgccgcgtagtcgtacttgaagccgagcgcaggcggccccgacggctccagcgggagcagcgctgccccgggcccggctcccgggtcgcgcccgcgctcctcacgcttcaggcccccgccgccaccctcggcgcacggctcgcggtagtaacccttgccgtcctccacgcgcgccagctcgcacgtgcggccgaagggagggttgagagacactgggctgccgaggtagggctgcgggtagccattgcacggctccgccgacggccaggacagggagcacacgttgtcgcggcgtgggtaggacagcgaaggcagcccgggaagctgcgccccggacgcgcggaagttggggaagtagaaggtgtctcccgtgtggatgtttaccagcggccccacaaacccgggattcaggagattatgctcgcccatttccgcggggcccgaccggcagcttct

SEQ ID NO: 8794 - RNA, 2598 nt, Homo sapiens
  source 1..2598: mol_type = other RNA
aagtgtgcagggcactggtgagcagtggcaactgccttgtgtctctctcaaggcggagggaggcagctgtgtccctcagcgagatcatcccctctgggctctgcacctccttcaggatctggggctcccgctgataggccacgcgaatccgaaacacaaatccatccttaaggacatccgtgtgcgtggcagtggcacggcactgcagaccatgctgttgtgtcaacagctctgccaggcgcagctggaaggcagctcggacccgctgcacggcctcagcgtcctgtggccactggccactgccctccaggtgacaaaccacggtcatgggctccacgtaggccggacagggcttatcgagccggggcagcagtgaggaccgctcccgcagagtctcatagaaggagaaggctggacggactggagttggtgggaacacctctgtgtagcgcagcactgggtgagctccctgaacagcagacacggtcagtgggagaccctctagcccccacagtaggcgactgaggtcgtcgtagcaacgtaccgccgctaccagggcctcctcacctgtgctggaggtctctttcaggccttggataagtgcatccagggggccccccacatagtggacacaggtttctgggatgtcagcatggagtgccaagaggtgggtgaccacctggtggggaataaggcgcttctgggacatagaggctgcctcccagaccacagcttcccgaatggctccgtcctggaaacgccgaagctccgagcgggatccccagaactggcggaatttagcagcctcaggctggtctgcctctggacccagctcaaggacgctggtcagtccctcaggccggagaaggagtcccagggtcagggtcccagagtctttgtgctttggtggatcttggctgatgtcccactctgggactgggggtcgagagtgagccagcaggttcagccgagcccccaggccctgctccaggagggtggtcagggggcccaaagcagctgagacatagtccccaccattgtcctgcagctctggccagagcttcagccggtggcacgctgcctgcaggcgactcagtggacggagacctgtcacccctaaactcactgcaggacatggtcaaaagcccggatcatgggtttgggagtcatcaacagcaggtggaacccgtcgtcagctctgctgtccagcaacatcatagacagccgtgcctcatgctgtacctggtggtaagtagaggcagtgacatcagcacagaggttgagatggcctgaggaatccaggaagacaacggagaaggcctggtggaagtcagccagggccggcaaagagggatctgagctgagacataaactgatcccgttgactgtcaggtctgtagtggccagaaactgcaagacacttctcaggacctggtagccactcatggtggtatggatcttgcgtgtagacacaaggaagacaaccagcatggagacaaggaacccagtaaacccaccctggcccttgtccagctcccgctgccgcagccagaccttcagaagtgccacgccatccttcaggccctgggctgaactcagaatggttgacagcagctgcaaatgggactcgagaactgtatcttgcaggacccatgtgttatagcggggggtaggaggctctgggctaccatcccctgcaggactctgccctcggtaccaggcagagcgcacattgttcttggttggcagcaagcggcacgggcggaagaagtcaggtggagggcacggatgcagacgtacagtgaccaggcgctcatcctttccacgcggccgcagcaacagtgagggtttcaggtggcagccatttgtgtaggagaagcaaacactgccaaagagggggtcctgggccaggtggtgagccaagtgggccaggtagagggcacgcttgcggaagtagcgctggttcagcccgtccttgtcctgtaggatttccctgggcatggtcagtgccacatccacattgatgtctggtcggatgcaggtgcccagaaggtagctgcccacaacagtaacctgggctgggggcaggaagcggaaacagcccttcacggcatagggcacttggtggaggggcactcgaaccccagctgggagccatgcctggtcagtgagctctgtctcagggactgagggcaccctcacaacccgctggttgacctcccgtaggaaggcatcaatccgatccttcttcttctctgacagccttacttcctttagtagctcctctacctgtaaacgaagcaagctggagtggaacaagatctcagtctcccgaaggcgattaagctcctcattggtaggctccttgtacagttctgccctgctgagcttcactggctgcaggaggcccttcgctggaggttcagccaatgtacgcttcctggaggatgctttcttcccctctttgcctgtgccttccagggctggttccatcacctctggctctccagtcgctccgcgaagctgctctccagctggcgccggccccatcactcagggtccagcactctcccgcacttcagattctagccgggtcta

SEQ ID NO: 8795 - RNA, 2612 nt, Homo sapiens
  source 1..2612: mol_type = other RNA
aagtgtgcagggcactggtgagcagtggcaactgccttgtgtctctctcaaggcggagggaggcagctgtgtccctcagcgagatcatcccctctgggctctgcacctccttcaggatctggggctcccgctgataggccacgcgaatccgaaacacaaatccatccttaaggacatccgtgtgcgtggcagtggcacggcactgcagaccatgctgttgtgtcaacagctctgccaggcgcagctggaaggcagctcggacccgctgcacggcctcagcgtcctgtggccactggccactgccctccaggtgacaaaccacggtcatgggctccacgtaggccggacagggcttatcgagccggggcagcagtgaggaccgctcccgcagagtctcatagaaggagaaggctggacggactggagttggtgggaacacctctgtgtagcgcagcactgggtgagctccctgaacagcagacacggtcagtgggagaccctctagcccccacagtaggcgactgaggtcgtcgtagcaacgtaccgccgctaccagggcctcctcacctgtgctggaggtctctttcaggccttggataagtgcatccagggggccccccacatagtggacacaggtttctgggatgtcagcatggagtgccaagaggtgggtgaccacctggtggggaataaggcgcttctgggacatagaggctgcctcccagaccacagcttcccgaatggctccgtcctggaaacgccgaagctccgagcgggatccccagaactggcggaatttagcagcctcaggctggtctgcctctggacccagctcaaggacgctggtcagtccctcaggccggagaaggagtcccagggtcagggtcccagagtctttgtgctttggtggatcttggctgatgtcccactctgggactgggggtcgagagtgagccagcaggttcagccgagcccccaggccctgctccaggagggtggtcagggggcccaaagcagctgagacatagtccccaccattgtcctgcagctctggccagagcttcagccggtggcacgctgcctgcaggcgactcagtggacggagatgcaggacatggtcaaaagcccggatcatgggtttgggagtcatcaacagcaggtggaacccgtcgtcagctctgctgtccagcaacatcatagacagccgtgcctcatgctgtacctggtggtaagtagaggcagtgacatcagcacagaggttgagatggcctgaggaatccaggaagacaacggagaaggcctggtggaagtcagccagggccggcaaagagggatctgagctgagacataaactgatcccgttgactgtcaggtctgtagtggccagaaactgcaagacacttctcaggacctggtagccactcatggtggtatggatcttgcgtgtagacacaaggaagacaaccagcatggagacaaggaacccagtaaacccaccctggcccttgtccagctcccgctgccgcagccagaccttcagaagtgccacgccatccttcaggccctgggctgaactcagaatggttgacagcagctgcaaatgggactcgagaactgtatcttgcaggacccatgtgttatagcggggggtaggaggctctgggctaccatcccctgcaggactctgccctcggtaccaggcagagcgcacattgttcttggttggcagcaagcggcacgggcggaagaagtcaggtggagggcacggatgcagacgtacagtgaccaggcgctcatcctttccacgcggccgcagcaacagtgagggtttcaggtggcagccatttgtgtaggagaagcaaacactgccaaagagggggtcctgggccaggtggtgagccaagtgggccaggtagagggcacgcttgcggaagtagcgctggttcagcccgtccttgtcctgtaggatttccctgggcatggtcagtgccacatccacattgatgtctggtcggatgcaggtgcccagaaggtagctgcccacaacagtaacctgggctgggggcaggaagcggaaacagcccttcacggcatagggcacttggtggaggggcactcgaaccccagctgggagccatgcctggtcagtgagctctgtctcagggactgagggcaccctcacaacccgctggttgacctcccgtaggaaggcatcaatccgatccttcttcttctctgacagccttacttcctttagtagctcctctacctgtaaacgaagcaagctggagtggaacaagatctcagtctcccgaaggcgattaagctcctcattggtaggctccttgtacagttctgccctgctgagcttcactggctgcaggaggcccttcgctggaggttcagccaatgtacgcttcctggaggatgctttcttcccctctttgcctgtgccttccagggctggttccatcacctctggctctccagtcgctccgcgaagctgctctccagctggcgccggccccatcactcagggtccagcactctcccgcacttcagattctagccgggtctatacctcatagcttcccacgtgggcggaaatgcct

SEQ ID NO: 8796 - RNA, 699 nt, Homo sapiens
  source 1..699: mol_type = other RNA
aagtgtgcagggcactggtgctgctccaaagctcatgaatgcctttgctgcctagcacctggagtcgttttcctggagggaaaggcgttcctccctgaaatgcaagacctcttgctgcttctccctcaagtcttccaaaagctgctgcctttccaccttctggtgctccagctcctcttccagctcttgaaggtgggatcgagaggacagcagagcctccctcaggctttccatctcctgggagtgctctccagagcaacagctttatcatgtattcgctggcgaagtttctcaagcaacgtttcatttgcttcaagggttttgtctgagttatctcgatactgtaggagctcccgaaattcctgaagcaactgctccttgtgactcagactatggtttaggtgctggacgttttgttcctgggttcgaatctcattgtatttttcagcctcccaggcacgaagctgttggctcttattctgcaattcttgtagctgctgcaaggcttttcgcaattcctgaattaaacatattacctccggaagatcccgcctctgcctccgcacgagcctttcaggtctagatgtctggtctaccgctctccggcttctttccccgcttttgcttttcccttcccccgctcccgccctccagccccacgacccgaccactgtccagctgagcccccgcggctccact

SEQ ID NO: 8797 - RNA, 6929 nt, Homo sapiens
  source 1..6929: mol_type = other RNA
aagtgtgcagggcactggtgctgctccgaagctcatgaatacctttgctgcctagcacctctgtgccttgggcttcaaggccagggaagctgcacgctgatctcacaagagacactatctttttgaccagcagcttgccctccgcaatctgctgtcttagggcactgtagtcatcaatgtggccaatgacatggcggccatgcttattggcaaaggagccatcagtagcatcaccctctagcttgggaggggtcttcattactggagaagtatccaaacccaagccatttgctctgttgattatgggcgtttctgagccaggagtagaggaagcagagctggggaagaccagagctggggaattcataccaacatcccggactggaggggacacagctgaatcttggaggagcagctgcttgtttccagggtcagtgctggctgggaagttctggttaatggaggaggggctgaggctggctttgccagcaccgctctccagctgctgttgcagctgcagtcgcagacaattgttcccctgaatgctctgctccagctgccctctcagagctcgtacctctgccaccaggtggctcaggtcactgctcaaagggatttggtgacaggcatccaggctgtaagctttcagccccttcttggaattgccataaagtgcctcgtagatttgtagctctgactggagggactcaaagagctgctgtttctcttcacactgttgctgcaggagaaccagcttgtgctgcagtctggagtcgttttcctggagggaaagacgttcctccctgaaatgcaagacctcttgctgcttctccctcaagtcttccaaaagctgctgcctttccaccttctggtgctccagctccttttccagctcttgaaggtgggatcgagaggacagcagagcctccctcaggctttctgtttcctgggagtgctctctggaaacatgactcagttgagcctgaagtcttcgattgtcttccctgaggactctgttctcattgcagagctgaggtatggactccaggccctgactgtagaagttagaagtggatccccttccacgagcagtagaggtcagccggtgttccagttgctcccgtaggcggtcattgatgcagatggattcctccaggcgctggcgcaggttccggatttcaccaagatgctcttccagcaggtcagcccctgtgggtttggagttaagctggtacacagaggagcctgaggataggtccccagatacactccctttctgaggcctcatcacatcccacttgccactgctgcccaggtacccaggctctaggattcttcccagttctatggtgccccttggaggagagtgaggctgggcagagttgaggtagtaggaagagtcggcttccaagtcgttgctcagcaatgtagctgtggaagcaggaggaacagtgctggcacctgaatgggcctggttggcctccttgggggtattctggggagttggcaagctgatggggttgctgttggattcggccttagccccctgagatgcactggttgatgatggtttagaagacaacacagcagaatgactcgaatgatggatggaatctgagtgactgggagaagctttcttctcttcatagtgtgtgtactcgctgactatgtccatgtcagagcaggcttccagttcatcagacaggaaagaggtgctgctgggagagcggtgggagtcagacaaggcatggctgctggagggtgtgagggaccgagcatccagcttggcctgcaggacttcaatcactttctccttctcctgcagctccctgctgagcctgagggccagtggctcaagtccagcttgatctttctcacttttatgatccttggtgctgagtttgctggtgagcctctctgtcagctggcttccctgggcgagttgctcccggaagctctgtcccaggtagtagtcaatgtcattgctccttaggagatcctcaaaagattttactgtatcttttgcatgccgggtgataagataacaaatacctctcccttctcgtattttttgccgtaggtaagacagttcccgggcctgatcctgaatcagggaatcatatttcccaggccacgaggctgatctcagctcctcagccagcttctcttctagtccattttttgggagctgggcctccagctgggatactctctggatgagactctccaggtcctttttggcctgaagccctggagagtagaaagccccagtgccatcagacagccacccctcatcctcatcagggacactatgaggtgaagacccctccaaggtgccaacagctctcagcttccggggtctttccagactagacgaataatcacttgtaactgagagggaccggacccggctcttgaggttttgaatgaccttgttggcattctgcagctgggccttcagatctttgatgtcctttcgtaggaccaagatgttttctgactttccatatacccggaactcttcctgcttccctagctggttctccaagggcttcctctcagaggaactagccagtgttgagccccggcgtccctgctcagagcacagcccctccatcaggaccatttccttgaggctgttgtgctcctcacactcaggactggtggtttcctcccgttcagcctcattctcgcttcggccacaagtctcatagcccaggtcctggaggtccacctggatctgcttgctgtcctgcttcaccaaggattcacctgtaagcataactctgtatttctccagctcgttagcctgagcaaagacagtggcttctgatagcagcagcttctcctggagatcttgatagcgttgtttgcattgtgacagctgggagcgcaggtgctgggtggaccctggtaggctaaacgctgactgaggcccagggtcacgaggctgggactggttatccaactcgcccttctccttgtcttcctcgatctcccatccatcagacattgcttctcccatctgctctttcagctccgcattctcaaggcaaaggctcagcatggtgttcctgatgtgggacactgaggagaatcctgcttcctcaatttgagcctttagctccttcagttcctcctcagctttcctcttctcttctaagtgctggtggaactcagccctcaggtggagcatttcttcctgaagacacctgttactgtcccctcccatcggagaaggaggggaaaaagatgggttctgggtctccacagttgccagacttttctccaaagccaccttgacaagttgctggtgactatggtgtgcagcctcctcctcaatactgtcagtgaactcagtgcttgtatcttcggtgtcatcccctgcagctgcacctccaatggcggccagggtctccagcctgtttaagcgctccaagcttcttccaagaacttcttctagccgactgcgtaacacctgagccccttccagttccacctgcagagttcggtctctctcagagctctctggatgggcatggaacttcaccagactgctatagagctgtctctctgcttgtaaggcctcattgagccgactccgttcatctactagtccttctagcatcagcagcaactgttgtcttcggtttcctgaaatttcttgaccctgggattctactgaagcaactttttcccgaagaagtaagacttcctgggtcaggcgttccatagctggtatgtcttcaggatcaaccagttgcatttgcaggtcctttatgagatcttctttaatctgtatgttcctggtcagagactccatatcagcagcctgcacctgcagctcttcttcctgcacagccatcatggactgtagagcagaaagttccatctgactttctctttcttttttagccatgagttcaagttcctctttggcattactcagttctttttccagccctgcaactgtgtccaagtctcctaatgtggatctgggtatgctgacatcctctttggcagtcaatgaagtgctatcatctctggaaggtatctgcattgaaccttgatcagtctgttttccaagacggccagtgggggtaacttcagcttgttggttagagatgggtgcttgggacatcagggagtctctccctcctaaatattggcgcagggcctgtaattctgaatttctttccattaaggcttgcaccaacttctctgcagcagcttggctttcctgctccctggtgctcacagactgaagcaggccttgaatctccatttcatgttccagcacttgtttatttcgatcacttagaaggtcctgcagcatcctttcctttcgctgtagacgctggcacagctcctctgctatctcactctgccctggtccaagtttgcagagcagtgttgcactaagatcctccacttctttgttcctatcatgaagagacgtctgtaactgctgaatgatactctcttgttccttctgccaacggctaaatttggtttccatttcttctttcagccactggaggttttgacaggtagtagataactgttccacttccaggcctttggccctcaggagactctccatactttgcatagtagcttcattggaggagaggacatcgcgcagtctctctaagtcatgatctcgctctctcacagcaagacgaagctggcgcagttctttttctttctcttctagagcagagaatttttcatctatagcccgctccagagcaacagctttatcatgtattcgctggcgaagtttctcaagcaacatttcatttgcttcaagggttttgtctgagttatctcgatactgtaggagctcccgaaattcctgaagcaactgctccttgtgactcagactatggtttaggtgctggatgttttgttcctgggttcgaatctcattgtatttttcagcctcccaggcacgaagctgttggctcttattctgcaattcttcttgtagctgctgcaaggcttttcgcaattcctggttatgtttccaagaagcctctttctgctgttcactctcgtgtgctgcagcctctacaaattgcacacattgtttggcatcagccagttggcgctctttctgtcgtaccaccctctggagcttctgtatttcaagttggctgcagaataaagcactctgaagatcaagcagagctacctgttgctgagctggagaagtaccctctgagctgtgaagttgtccaagctggctttggtgcagcatttctcgaagctttgccattgtgtcattttgaccttcaattacctggtacaactcctcagtctcacgttccctgcttttcagagtttccttgaggttctgaattgtaccatcttgcttttgagacgactcctgagcacactttagttcatagctcatttcattaagtttctcttgaagaatcttgttggtggcctctgtttgctggattttttcctggagttctgccaagtgggaatcagatacagactgctgagttatagtggtctcatgtgaattcagcttttgttgtttcagcaactcttcagtcatgggctgcacttccatgctagttggctcctccaacagatgtagcagttgttgtttctcccgagatagctgttctacaagcctctcctgggcagccaggctctgattcagttcttcaattctcttgtccctctgggccagggcctcagtgtattggtcgggcttgacctggtctcctggtacatcttcccagtttttggtgactcccttcagtttctctgagagctccaggttacactccttctctgcttccaccagagctgccatccgcgcagcttcattctttgctagcctggattcctcctgcagaagctggatcttattctccaagagctcataaacatgctccgtctcctgctgtcgctcctcaaactggcgtcggagctcagcttcattctgactgttgagattctccacatcagcccatgttttatccagatgctgtttcttgtcctggagttctcgtttcaagctctccacttcaaccttcagctcaatgttccgcttgtagatgtcctcccggctggcctcatacttctgttgcatgcgctcctccaggaagtagatgcgcagcttgaggctgaagttctccttcttcaggtcattgaggtgcttctcaaagtctcgaagagcctgggtctgtacctgagggggtttctcaaatgctctcaaggaatatgtctgcacaaacgggaccttttcaccacttctccagatctgtgactgcactggagggcctcgatctttagtgtcactaagaaaagctgctgtgtgactcgttctgggtaccatctccccatcatcctctgcaaaataatctctcatccagggtgtggccgccgcagctgcttcttcctcctcggccgctgctgcccagctcccggctggctccgggcgccgtctttcccggctcggggtctgccgtggggactgaggggttcgcgtcgcgtccccggaccggtaaggcgtgtagtgagcccggcgggacgcgcgacagcagcagccaaagtcgcatcggcggcggcagcaggacccgctgtctgtgcccttcatggatttcctgggcctggccaccccagtcctagctacggttcctgcttgttttcctggtgttttccgggactgccagggcgcatcctctgggcctggctgagcatccccgtcagttccctgggcctcctccgcggctgcctctgccacctgctccgcccagattgctttggtccttctcccgcagacacactcagctgcccttcatcctctgtcgtctccccattctctctccacccactgcctcattcccagatcccacgccgtttcttcctttctatccgctccaatgtcaccttctctttatttc

SEQ ID NO: 8798 - RNA, 6756 nt, Homo sapiens
  source 1..6756: mol_type = other RNA
aagtgtgcagggcactggtgctgctccgaagctcatgaatacctttgctgcctagcacctctgtgccttgggcttcaaggccagggaagctgcacgctgatctcacaagagacactatctttttgaccagcagcttgccctccgcaatctgctgtcttagggcactgtagtcatcaatgtggccaatgacatggcggccatgcttattggcaaaggagccatcagtagcatcaccctctagcttgggaggggtcttcattactggagaagtatccaaacccaagccatttgctctgttgattatgggcgtttctgagccaggagtagaggaagcagagctggggaagaccagagctggggaattcataccaacatcccggactggaggggacacagctgaatcttggaggagcagctgcttgtttccagggtcagtgctggctgggaagttctggttaatggaggaggggctgaggctggctttgccagcaccgctctccagctgctgttgcagctgcagtcgcagacaattgttcccctgaatgctctgctccagctgccctctcagagctcgtacctctgccaccaggtggctcaggtcactgctcaaagggatttggtgacaggcatccaggctgtaagctttcagccccttcttggaattgccataaagtgcctcgtagatttgtagctctgactggagggactcaaagagctgctgtttctcttcacactgttgctgcaggagaaccagcttgtgctgcagtctggagtcgttttcctggagggaaagacgttcctccctgaaatgcaagacctcttgctgcttctccctcaagtcttccaaaagctgctgcctttccaccttctggtgctccagctccttttccagctcttgaaggtgggatcgagaggacagcagagcctccctcaggctttctgtttcctgggagtgctctctggaaacatgactcagttgagcctgaagtcttcgattgtcttccctgaggactctgttctcattgcagagctgaggtatggactccaggccctgactgtagaagttagaagtggatccccttccacgagcagtagaggtcagccggtgttccagttgctcccgtaggcggtcattgatgcagatggattcctccaggcgctggcgcaggttccggatttcaccaagatgctcttccagcaggtcagcccctgtgggtttggagttaagctggtacacagaggagcctgaggataggtccccagatacactccctttctgaggcctcatcacatcccacttgccactgctgcccaggtacccaggctctaggattcttcccagttctatggtgccccttggaggagagtgaggctgggcagagttgaggtagtaggaagagtcggcttccaagtcgttgctcagcaatgtagctgtggaagcaggaggaacagtgctggcacctgaatgggcctggttggcctccttgggggtattctggggagttggcaagctgatggggttgctgttggattcggccttagccccctgagatgcactggttgatgatggtttagaagacaacacagcagaatgactcgaatgatggatggaatctgagtgactgggagaagctttcttctcttcatagtgtgtgtactcgctgactatgtccatgtcagagcaggcttccagttcatcagacaggaaagaggtgctgctgggagagcggtgggagtcagacaaggcatggctgctggagggtgtgagggaccgagcatccagcttggcctgcaggacttcaatcactttctccttctcctgcagctccctgctgagcctgagggccagtggctcaagtccagcttgatctttctcacttttatgatccttggtgctgagtttgctggtgagcctctctgtcagctggcttccctgggcgagttgctcccggaagctctgtcccaggtagtagtcaatgtcattgctccttaggagatcctcaaaagattttactgtatcttttgcatgccgggtgataagataacaaatacctctcccttctcgtattttttgccgtaggtaagacagttcccgggcctgatcctgaatcagggaatcatatttcccaggccacgaggctgatctcagctcctcagccagcttctcttctagtccattttttgggagctgggcctccagctgggatactctctggatgagactctccaggtcctttttggcctgaagccctggagagtagaaagccccagtgccatcagacagccacccctcatcctcatcagggacactatgaggtgaagacccctccaaggtgccaacagctctcagcttccggggtctttccagactagacgaataatcacttgtaactgagagggaccggacccggctcttgaggttttgaatgaccttgttggcattctgcagctgggccttcagatctttgatgtcctttcgtaggaccaagatgttttctgactttccatatacccggaactcttcctgcttccctagctggttctccaagggcttcctctcagaggaactagccagtgttgagccccggcgtccctgctcagagcacagcccctccatcaggaccatttccttgaggctgttgtgctcctcacactcaggactggtggtttcctcccgttcagcctcattctcgcttcggccacaagtctcatagcccaggtcctggaggtccacctggatctgcttgctgtcctgcttcaccaaggattcacctgtaagcataactctgtatttctccagctcgttagcctgagcaaagacagtggcttctgatagcagcagcttctcctggagatcttgatagcgttgtttgcattgtgacagctgggagcgcaggtgctgggtggaccctggtaggctaaacgctgactgaggcccagggtcacgaggctgggactggttatccaactcgcccttctccttgtcttcctcgatctcccatccatcagacattgcttctcccatctgctctttcagctccgcattctcaaggcaaaggctcagcatggtgttcctgatgtgggacactgaggagaatcctgcttcctcaatttgagcctttagctccttcagttcctcctcagctttcctcttctcttctaagtgctggtggaactcagccctcaggtggagcatttcttcctgaagacacctgttactgtcccctcccatcggagaaggaggggaaaaagatgggttctgggtctccacagttgccagacttttctccaaagccaccttgacaagttgctggtgactatggtgtgcagcctcctcctcaatactgtcagtgaactcagtgcttgtatcttcggtgtcatcccctgcagctgcacctccaatggcggccagggtctccagcctgtttaagcgctccaagcttcttccaagaacttcttctagccgactgcgtaacacctgagccccttccagttccacctgcagagttcggtctctctcagagctctctggatgggcatggaacttcaccagactgctatagagctgtctctctgcttgtaaggcctcattgagccgactccgttcatctactagtccttctagcatcagcagcaactgttgtcttcggtttcctgaaatttcttgaccctgggattctactgaagcaactttttcccgaagaagtaagacttcctgggtcaggcgttccatagctggtatgtcttcaggatcaaccagttgcatttgcaggtcctttatgagatcttctttaatctgtatgttcctggtcagagactccatatcagcagcctgcacctgcagctcttcttcctgcacagccatcatggactgtagagcagaaagttccatctgactttctctttcttttttagccatgagttcaagttcctctttggcattactcagttctttttccagccctgcaactgtgtccaagtctcctaatgtggatctgggtatgctgacatcctctttggcagtcaatgaagtgctatcatctctggaaggtatctgcattgaaccttgatcagtctgttttccaagacggccagtgggggtaacttcagcttgttggttagagatgggtgcttgggacatcagggagtctctccctcctaaatattggcgcagggcctgtaattctgaatttctttccattaaggcttgcaccaacttctctgcagcagcttggctttcctgctccctggtgctcacagactgaagcaggccttgaatctccatttcatgttccagcacttgtttatttcgatcacttagaaggtcctgcagcatcctttcctttcgctgtagacgctggcacagctcctctgctatctcactctgccctggtccaagtttgcagagcagtgttgcactaagatcctccacttctttgttcctatcatgaagagacgtctgtaactgctgaatgatactctcttgttccttctgccaacggctaaatttggtttccatttcttctttcagccactggaggttttgacaggtagtagataactgttccacttccaggcctttggccctcaggagactctccatactttgcatagtagcttcattggaggagaggacatcgcgcagtctctctaagtcatgatctcgctctctcacagcaagacgaagctggcgcagttctttttctttctcttctagagcagagaatttttcatctatagcccgctccagagcaacagctttatcatgtattcgctggcgaagtttctcaagcaacatttcatttgcttcaagggttttgtctgagttatctcgatactgtaggagctcccgaaattcctgaagcaactgctccttgtgactcagactatggtttaggtgctggatgttttgttcctgggttcgaatctcattgtatttttcagcctcccaggcacgaagctgttggctcttattctgcaattcttcttgtagctgctgcaaggcttttcgcaattcctggttatgtttccaagaagcctctttctgctgttcactctcgtgtgctgcagcctctacaaattgcacacattgtttggcatcagccagttggcgctctttctgtcgtaccaccctctggagcttctgtatttcaagttggctgcagaataaagcactctgaagatcaagcagagctacctgttgctgagctggagaagtaccctctgagctgtgaagttgtccaagctggctttggtgcagcatttctcgaagctttgccattgtgtcattttgaccttcaattacctggtacaactcctcagtctcacgttccctgcttttcagagtttccttgaggttctgaattgtaccatcttgcttttgagacgactcctgagcacactttagttcatagctcatttcattaagtttctcttgaagaatcttgttggtggcctctgtttgctggattttttcctggagttctgccaagtgggaatcagatacagactgctgagttatagtggtctcatgtgaattcagcttttgttgtttcagcaactcttcagtcatgggctgcacttccatgctagttggctcctccaacagatgtagcagttgttgtttctcccgagatagctgttctacaagcctctcctgggcagccaggctctgattcagttcttcaattctcttgtccctctgggccagggcctcagtgtattggtcgggcttgacctggtctcctggtacatcttcccagtttttggtgactcccttcagtttctctgagagctccaggttacactccttctctgcttccaccagagctgccatccgcgcagcttcattctttgctagcctggattcctcctgcagaagctggatcttattctccaagagctcataaacatgctccgtctcctgctgtcgctcctcaaactggcgtcggagctcagcttcattctgactgttgagattctccacatcagcccatgttttatccagatgctgtttcttgtcctggagttctcgtttcaagctctccacttcaaccttcagctcaatgttccgcttgtagatgtcctcccggctggcctcatacttctgttgcatgcgctcctccaggaagtagatgcgcagcttgaggctgaagttctccttcttcaggtcattgaggtgcttctcaaagtctcgaagagcctgggtctgtacctgagggggtttctcaaatgctctcaaggaatatgtctgcacaaacgggaccttttcaccacttctccagatctgtgactgcactggagggcctcgatctttagtgtcactaagaaaagctgctgtgtgactcgttctgggtaccatctccccatcatcctctgcaaaataatctctcgtccaggtctgctccattttccaggctctttccttagtctcaggacgctcctcacccgggaggggaagcagcctgggaaaatgagaagccttgcccacgaatctccagcgcaaaaggcagcagctttttcctccccagctcctttctgcgtcggcggcgaagagagagctctgctccctgcttttttagaaaatggatttgacgtggccgaacctgcggctagccgtgcgacccgcacaagggagggactgttctcagtaggaggctggactcagagcggcgcggcgcccggggctgtttcgtgagctggagccagcggctgcccgggccgcggtgcgcgcactctccaggctgagacacgact

SEQ ID NO: 8799 - RNA, 7437 nt, Homo sapiens
  source 1..7437: mol_type = other RNA
aagtgtgcagggcactggtgctgctccgaagctcatgaatacctttgctgcctagcacctctgtgccttgggcttcaaggccagggaagctgcacgctgatctcacaagagacactatctttttgaccagcagcttgccctccgcaatctgctgtcttagggcactgtagtcatcaatgtggccaatgacatggcggccatgcttattggcaaaggagccatcagtagcatcaccctctagcttgggaggggtcttcattactggagaagtatccaaacccaagccatttgctctgttgattatgggcgtttctgagccaggagtagaggaagcagagctggggaagaccagagctggggaattcataccaacatcccggactggaggggacacagctgaatcttggaggagcagctgcttgtttccagggtcagtgctggctgggaagttctggttaatggaggaggggctgaggctggctttgccagcaccgctctccagctgctgttgcagctgcagtcgcagacaattgttcccctgaatgctctgctccagctgccctctcagagctcgtacctctgccaccaggtggctcaggtcactgctcaaagggatttggtgacaggcatccaggctgtaagctttcagccccttcttggaattgccataaagtgcctcgtagatttgtagctctgactggagggactcaaagagctgctgtttctcttcacactgttgctgcaggagaaccagcttgtgctgcagtctggagtcgttttcctggagggaaagacgttcctccctgaaatgcaagacctcttgctgcttctccctcaagtcttccaaaagctgctgcctttccaccttctggtgctccagctccttttccagctcttgaaggtgggatcgagaggacagcagagcctccctcaggctttctgtttcctgggagtgctctctggaaacatgactcagttgagcctgaagtcttcgattgtcttccctgaggactctgttctcattgcagagctgaggtatggactccaggccctgactgtagaagttagaagtggatccccttccacgagcagtagaggtcagccggtgttccagttgctcccgtaggcggtcattgatgcagatggattcctccaggcgctggcgcaggttccggatttcaccaagatgctcttccagcaggtcagcccctgtgggtttggagttaagctggtacacagaggagcctgaggataggtccccagatacactccctttctgaggcctcatcacatcccacttgccactgctgcccaggtacccaggctctaggattcttcccagttctatggtgccccttggaggagagtgaggctgggcagagttgaggtagtaggaagagtcggcttccaagtcgttgctcagcaatgtagctgtggaagcaggaggaacagtgctggcacctgaatgggcctggttggcctccttgggggtattctggggagttggcaagctgatggggttgctgttggattcggccttagccccctgagatgcactggttgatgatggtttagaagacaacacagcagaatgactcgaatgatggatggaatctgagtgactgggagaagctttcttctcttcatagtgtgtgtactcgctgactatgtccatgtcagagcaggcttccagttcatcagacaggaaagaggtgctgctgggagagcggtgggagtcagacaaggcatggctgctggagggtgtgagggaccgagcatccagcttggcctgcaggacttcaatcactttctccttctcctgcagctccctgctgagcctgagggccagtggctcaagtccagcttgatctttctcacttttatgatccttggtgctgagtttgctggtgagcctctctgtcagctggcttccctgggcgagttgctcccggaagctctgtcccaggtagtagtcaatgtcattgctccttaggagatcctcaaaagattttactgtatcttttgcatgccgggtgataagataacaaatacctctcccttctcgtattttttgccgtaggtaagacagttcccgggcctgatcctgaatcagggaatcatatttcccaggccacgaggctgatctcagctcctcagccagcttctcttctagtccattttttgggagctgggcctccagctgggatactctctggatgagactctccaggtcctttttggcctgaagccctggagagtagaaagccccagtgccatcagacagccacccctcatcctcatcagggacactatgaggtgaagacccctccaaggtgccaacagctctcagcttccggggtctttccagactagacgaataatcacttgtaactgagagggaccggacccggctcttgaggttttgaatgaccttgttggcattctgcagctgggccttcagatctttgatgtcctttcgtaggaccaagatgttttctgactttccatatacccggaactcttcctgcttccctagctggttctccaagggcttcctctcagaggaactagccagtgttgagccccggcgtccctgctcagagcacagcccctccatcaggaccatttccttgaggctgttgtgctcctcacactcaggactggtggtttcctcccgttcagcctcattctcgcttcggccacaagtctcatagcccaggtcctggaggtccacctggatctgcttgctgtcctgcttcaccaaggattcacctgtaagcataactctgtatttctccagctcgttagcctgagcaaagacagtggcttctgatagcagcagcttctcctggagatcttgatagcgttgtttgcattgtgacagctgggagcgcaggtgctgggtggaccctggtaggctaaacgctgactgaggcccagggtcacgaggctgggactggttatccaattggtgggcatccactgtgaaggtagccccaaggtcaaggctctggggtctggggaaaggcctcacagtcacattcccctcctcttggtgttggtgcttcccaggggaaccaaccagttctgtgtttattctttcaatggtgctggtcagatgcacaaggagctctggagtaagtttactattcccttccttgctactcagcacaagttgttctttgaggaggttgatgatattgtgggcattcttcagttttccctggagctttctgaactcagcctgaaggctactctcactcagaccctctttggttaccacagtctcaaccatcacctcgcccttctccttgtcttcctcgatctcccatccatcagacattgcttctcccatctgctctttcagctccgcattctcaaggcaaaggctcagcatggtgttcctgatgtgggacactgaggagaatcctgcttcctcaatttgagcctttagctccttcagttcctcctcagctttcctcttctcttctaagtgctggtggaactcagccctcaggtggagcatttcttcctgaagacacctgttactgtcccctcccatcggagaaggaggggaaaaagatgggttctgggtctccacagttgccagacttttctccaaagccaccttgacaagttgctggtgactatggtgtgcagcctcctcctcaatactgtcagtgaactcagtgcttgtatcttcggtgtcatcccctgcagctgcacctccaatggcggccagggtctccagcctgtttaagcgctccaagcttcttccaagaacttcttctagccgactgcgtaacacctgagccccttccagttccacctgcagagttcggtctctctcagagctctctggatgggcatggaacttcaccagactgctatagagctgtctctctgcttgtaaggcctcattgagccgactccgttcatctactagtccttctagcatcagcagcaactgttgtcttcggtttcctgaaatttcttgaccctgggattctactgaagcaactttttcccgaagaagtaagacttcctgggtcaggcgttccatagctggtatgtcttcaggatcaaccagttgcatttgcaggtcctttatgagatcttctttaatctgtatgttcctggtcagagactccatatcagcagcctgcacctgcagctcttcttcctgcacagccatcatggactgtagagcagaaagttccatctgactttctctttcttttttagccatgagttcaagttcctctttggcattactcagttctttttccagccctgcaactgtgtccaagtctcctaatgtggatctgggtatgctgacatcctctttggcagtcaatgaagtgctatcatctctggaaggtatctgcattgaaccttgatcagtctgttttccaagacggccagtgggggtaacttcagcttgttggttagagatgggtgcttgggacatcagggagtctctccctcctaaatattggcgcagggcctgtaattctgaatttctttccattaaggcttgcaccaacttctctgcagcagcttggctttcctgctccctggtgctcacagactgaagcaggccttgaatctccatttcatgttccagcacttgtttatttcgatcacttagaaggtcctgcagcatcctttcctttcgctgtagacgctggcacagctcctctgctatctcactctgccctggtccaagtttgcagagcagtgttgcactaagatcctccacttctttgttcctatcatgaagagacgtctgtaactgctgaatgatactctcttgttccttctgccaacggctaaatttggtttccatttcttctttcagccactggaggttttgacaggtagtagataactgttccacttccaggcctttggccctcaggagactctccatactttgcatagtagcttcattggaggagaggacatcgcgcagtctctctaagtcatgatctcgctctctcacagcaagacgaagctggcgcagttctttttctttctcttctagagcagagaatttttcatctatagcccgctccagagcaacagctttatcatgtattcgctggcgaagtttctcaagcaacatttcatttgcttcaagggttttgtctgagttatctcgatactgtaggagctcccgaaattcctgaagcaactgctccttgtgactcagactatggtttaggtgctggatgttttgttcctgggttcgaatctcattgtatttttcagcctcccaggcacgaagctgttggctcttattctgcaattcttcttgtagctgctgcaaggcttttcgcaattcctggttatgtttccaagaagcctctttctgctgttcactctcgtgtgctgcagcctctacaaattgcacacattgtttggcatcagccagttggcgctctttctgtcgtaccaccctctggagcttctgtatttcaagttggctgcagaataaagcactctgaagatcaagcagagctacctgttgctgagctggagaagtaccctctgagctgtgaagttgtccaagctggctttggtgcagcatttctcgaagctttgccattgtgtcattttgaccttcaattacctggtacaactcctcagtctcacgttccctgcttttcagagtttccttgaggttctgaattgtaccatcttgcttttgagacgactcctgagcacactttagttcatagctcatttcattaagtttctcttgaagaatcttgttggtggcctctgtttgctggattttttcctggagttctgccaagtgggaatcagatacagactgctgagttatagtggtctcatgtgaattcagcttttgttgtttcagcaactcttcagtcatgggctggacccggagcggcaaataatcttcacagagatcatcccacagctcctgcaggtctgaaagctccaagggataactcacaggtgtcttgtaaaggggtttcaaagacctgttaaggaaaccggaactaactccatctgtcatgctagggccaggcttggctccaggtaggctggatttcactggaatcggaagcctgctccctcgggggctctggatgggcttataatcaagacctttaatcatgctaagagctaattccagcttgtgattacacccatgctgcggagcctgatcatctgaacaacagtcacactttccaagttcctttgcacttctctcagtctcctcatctttctgttgtggagggctagcctggacgcttgcatccaaagattccacagaggaaccaggcgtctcttcctccatgctttctccatctgggggtacctttgtgcttgctaagtcgggtggcccaacctcagacaacgctggttcttcagtgcaaatgctggtcgaccacctgctagaagggccgcaggagatacttctggccacctttcgaggtaccttacaaatggcttcatagtcagaatcagcaacccgcaaagcggcacaaccacggcatctcctgggtcggtttccagggccttctgaaccatggcagctgtgtggctcctggatctgatcctcattctccacccagcactcaaaccctgaataggcgaagtcctcctggagcagtgcagagtatctcgcatcgggtaagacggacatgtcaaccgtcccattccccgccttgatctccgcgccagagtcatcgttattcttccgatacatactggcaatgcagaacttgaggcgatccttctccagtagcagcttttgcaagcgctcaatagaaagcgcttcaatccgggcaataactgtgtcgaatcgatagattcgatcaagcatgaaagcacacttgctgcaagcgaactcggctttgccatcgcgggggacatccttgcccaagacgtgcgaaagcagaacctggagattgagcttggacgccgtgtggaagatccagcgccgctggtttccacacagctctcgggcacagatcctgcaaatctccttcatcttccctcctagcgggtggcaagcttcccgaggcggcggcggcggcggctactgggtgaccactcaatggctcttcgccgcgctctgtctcccgcctcggtggtctccggtcagcatggcacagcccagtggggtccccactctgcaggggcgcgcccctgccccgcgcgccgactccgggtaccagagccgtcagccccgcccctcgggcagggggcgggcgtggaaacgcctaagaggatgctgagtgacagaggcgcaggccgcgctccgaccctgccatgtctctccccagctgtctctcccgccagccgccgcgtcctcaacgtcctccccttttagcagactgggctcccggagcagcagcggccggccgcgcagacgcaaagcctcggggatggaggatc

SEQ ID NO: 8800 - RNA, 6926 nt, Homo sapiens
  source 1..6926: mol_type = other RNA
aagtgtgcagggcactggtgctgctccgaagctcatgaatacctttgctgcctagcacctctgtgccttgggcttcaaggccagggaagctgcacgctgatctcacaagagacactatctttttgaccagcagcttgccctccgcaatctgctgtcttagggcactgtagtcatcaatgtggccaatgacatggcggccatgcttattggcaaaggagccatcagtagcatcaccctctagcttgggaggggtcttcattactggagaagtatccaaacccaagccatttgctctgttgattatgggcgtttctgagccaggagtagaggaagcagagctggggaagaccagagctggggaattcataccaacatcccggactggaggggacacagctgaatcttggaggagcagctgcttgtttccagggtcagtgctggctgggaagttctggttaatggaggaggggctgaggctggctttgccagcaccgctctccagctgctgttgcagctgcagtcgcagacaattgttcccctgaatgctctgctccagctgccctctcagagctcgtacctctgccaccaggtggctcaggtcactgctcaaagggatttggtgacaggcatccaggctgtaagctttcagccccttcttggaattgccataaagtgcctcgtagatttgtagctctgactggagggactcaaagagctgctgtttctcttcacactgttgctgcaggagaaccagcttgtgctgcagtctggagtcgttttcctggagggaaagacgttcctccctgaaatgcaagacctcttgctgcttctccctcaagtcttccaaaagctgctgcctttccaccttctggtgctccagctccttttccagctcttgaaggtgggatcgagaggacagcagagcctccctcaggctttctgtttcctgggagtgctctctggaaacatgactcagttgagcctgaagtcttcgattgtcttccctgaggactctgttctcattgcagagctgaggtatggactccaggccctgactgtagaagttagaagtggatccccttccacgagcagtagaggtcagccggtgttccagttgctcccgtaggcggtcattgatgcagatggattcctccaggcgctggcgcaggttccggatttcaccaagatgctcttccagcaggtcagcccctgtgggtttggagttaagctggtacacagaggagcctgaggataggtccccagatacactccctttctgaggcctcatcacatcccacttgccactgctgcccaggtacccaggctctaggattcttcccagttctatggtgccccttggaggagagtgaggctgggcagagttgaggtagtaggaagagtcggcttccaagtcgttgctcagcaatgtagctgtggaagcaggaggaacagtgctggcacctgaatgggcctggttggcctccttgggggtattctggggagttggcaagctgatggggttgctgttggattcggccttagccccctgagatgcactggttgatgatggtttagaagacaacacagcagaatgactcgaatgatggatggaatctgagtgactgggagaagctttcttctcttcatagtgtgtgtactcgctgactatgtccatgtcagagcaggcttccagttcatcagacaggaaagaggtgctgctgggagagcggtgggagtcagacaaggcatggctgctggagggtgtgagggaccgagcatccagcttggcctgcaggacttcaatcactttctccttctcctgcagctccctgctgagcctgagggccagtggctcaagtccagcttgatctttctcacttttatgatccttggtgctgagtttgctggtgagcctctctgtcagctggcttccctgggcgagttgctcccggaagctctgtcccaggtagtagtcaatgtcattgctccttaggagatcctcaaaagattttactgtatcttttgcatgccgggtgataagataacaaatacctctcccttctcgtattttttgccgtaggtaagacagttcccgggcctgatcctgaatcagggaatcatatttcccaggccacgaggctgatctcagctcctcagccagcttctcttctagtccattttttgggagctgggcctccagctgggatactctctggatgagactctccaggtcctttttggcctgaagccctggagagtagaaagccccagtgccatcagacagccacccctcatcctcatcagggacactatgaggtgaagacccctccaaggtgccaacagctctcagcttccggggtctttccagactagacgaataatcacttgtaactgagagggaccggacccggctcttgaggttttgaatgaccttgttggcattctgcagctgggccttcagatctttgatgtcctttcgtaggaccaagatgttttctgactttccatatacccggaactcttcctgcttccctagctggttctccaagggcttcctctcagaggaactagccagtgttgagccccggcgtccctgctcagagcacagcccctccatcaggaccatttccttgaggctgttgtgctcctcacactcaggactggtggtttcctcccgttcagcctcattctcgcttcggccacaagtctcatagcccaggtcctggaggtccacctggatctgcttgctgtcctgcttcaccaaggattcactaagcataactctgtatttctccagctcgttagcctgagcaaagacagtggcttctgatagcagcagcttctcctggagatcttgatagcgttgtttgcattgtgacagctgggagcgcaggtgctgggtggaccctggtaggctaaacgctgactgaggcccagggtcacgaggctgggactggttatccaactcgcccttctccttgtcttcctcgatctcccatccatcagacattgcttctcccatctgctctttcagctccgcattctcaaggcaaaggctcagcatggtgttcctgatgtgggacactgaggagaatcctgcttcctcaatttgagcctttagctccttcagttcctcctcagctttcctcttctcttctaagtgctggtggaactcagccctcaggtggagcatttcttcctgaagacacctgttactgtcccctcccatcggagaaggaggggaaaaagatgggttctgggtctccacagttgccagacttttctccaaagccaccttgacaagttgctggtgactatggtgtgcagcctcctcctcaatactgtcagtgaactcagtgcttgtatcttcggtgtcatcccctgcagctgcacctccaatggcggccagggtctccagcctgtttaagcgctccaagcttcttccaagaacttcttctagccgactgcgtaacacctgagccccttccagttccacctgcagagttcggtctctctcagagctctctggatgggcatggaacttcaccagactgctatagagctgtctctctgcttgtaaggcctcattgagccgactccgttcatctactagtccttctagcatcagcagcaactgttgtcttcggtttcctgaaatttcttgaccctgggattctactgaagcaactttttcccgaagaagtaagacttcctgggtcaggcgttccatagctggtatgtcttcaggatcaaccagttgcatttgcaggtcctttatgagatcttctttaatctgtatgttcctggtcagagactccatatcagcagcctgcacctgcagctcttcttcctgcacagccatcatggactgtagagcagaaagttccatctgactttctctttcttttttagccatgagttcaagttcctctttggcattactcagttctttttccagccctgcaactgtgtccaagtctcctaatgtggatctgggtatgctgacatcctctttggcagtcaatgaagtgctatcatctctggaaggtatctgcattgaaccttgatcagtctgttttccaagacggccagtgggggtaacttcagcttgttggttagagatgggtgcttgggacatcagggagtctctccctcctaaatattggcgcagggcctgtaattctgaatttctttccattaaggcttgcaccaacttctctgcagcagcttggctttcctgctccctggtgctcacagactgaagcaggccttgaatctccatttcatgttccagcacttgtttatttcgatcacttagaaggtcctgcagcatcctttcctttcgctgtagacgctggcacagctcctctgctatctcactctgccctggtccaagtttgcagagcagtgttgcactaagatcctccacttctttgttcctatcatgaagagacgtctgtaactgctgaatgatactctcttgttccttctgccaacggctaaatttggtttccatttcttctttcagccactggaggttttgacaggtagtagataactgttccacttccaggcctttggccctcaggagactctccatactttgcatagtagcttcattggaggagaggacatcgcgcagtctctctaagtcatgatctcgctctctcacagcaagacgaagctggcgcagttctttttctttctcttctagagcagagaatttttcatctatagcccgctccagagcaacagctttatcatgtattcgctggcgaagtttctcaagcaacatttcatttgcttcaagggttttgtctgagttatctcgatactgtaggagctcccgaaattcctgaagcaactgctccttgtgactcagactatggtttaggtgctggatgttttgttcctgggttcgaatctcattgtatttttcagcctcccaggcacgaagctgttggctcttattctgcaattcttcttgtagctgctgcaaggcttttcgcaattcctggttatgtttccaagaagcctctttctgctgttcactctcgtgtgctgcagcctctacaaattgcacacattgtttggcatcagccagttggcgctctttctgtcgtaccaccctctggagcttctgtatttcaagttggctgcagaataaagcactctgaagatcaagcagagctacctgttgctgagctggagaagtaccctctgagctgtgaagttgtccaagctggctttggtgcagcatttctcgaagctttgccattgtgtcattttgaccttcaattacctggtacaactcctcagtctcacgttccctgcttttcagagtttccttgaggttctgaattgtaccatcttgcttttgagacgactcctgagcacactttagttcatagctcatttcattaagtttctcttgaagaatcttgttggtggcctctgtttgctggattttttcctggagttctgccaagtgggaatcagatacagactgctgagttatagtggtctcatgtgaattcagcttttgttgtttcagcaactcttcagtcatgggctgcacttccatgctagttggctcctccaacagatgtagcagttgttgtttctcccgagatagctgttctacaagcctctcctgggcagccaggctctgattcagttcttcaattctcttgtccctctgggccagggcctcagtgtattggtcgggcttgacctggtctcctggtacatcttcccagtttttggtgactcccttcagtttctctgagagctccaggttacactccttctctgcttccaccagagctgccatccgcgcagcttcattctttgctagcctggattcctcctgcagaagctggatcttattctccaagagctcataaacatgctccgtctcctgctgtcgctcctcaaactggcgtcggagctcagcttcattctgactgttgagattctccacatcagcccatgttttatccagatgctgtttcttgtcctggagttctcgtttcaagctctccacttcaaccttcagctcaatgttccgcttgtagatgtcctcccggctggcctcatacttctgttgcatgcgctcctccaggaagtagatgcgcagcttgaggctgaagttctccttcttcaggtcattgaggtgcttctcaaagtctcgaagagcctgggtctgtacctgagggggtttctcaaatgctctcaaggaatatgtctgcacaaacgggaccttttcaccacttctccagatctgtgactgcactggagggcctcgatctttagtgtcactaagaaaagctgctgtgtgactcgttctgggtaccatctccccatcatcctctgcaaaataatctctcatccagggtgtggccgccgcagctgcttcttcctcctcggccgctgctgcccagctcccggctggctccgggcgccgtctttcccggctcggggtctgccgtggggactgaggggttcgcgtcgcgtccccggaccggtaaggcgtgtagtgagcccggcgggacgcgcgacagcagcagccaaagtcgcatcggcggcggcagcaggacccgctgtctgtgcccttcatggatttcctgggcctggccaccccagtcctagctacggttcctgcttgttttcctggtgttttccgggactgccagggcgcatcctctgggcctggctgagcatccccgtcagttccctgggcctcctccgcggctgcctctgccacctgctccgcccagattgctttggtccttctcccgcagacacactcagctgcccttcatcctctgtcgtctccccattctctctccacccactgcctcattcccagatcccacgccgtttcttcctttctatccgctccaatgtcaccttctctttatttc

SEQ ID NO: 8801 - RNA, 6753 nt, Homo sapiens
  source 1..6753: mol_type = other RNA
aagtgtgcagggcactggtgctgctccgaagctcatgaatacctttgctgcctagcacctctgtgccttgggcttcaaggccagggaagctgcacgctgatctcacaagagacactatctttttgaccagcagcttgccctccgcaatctgctgtcttagggcactgtagtcatcaatgtggccaatgacatggcggccatgcttattggcaaaggagccatcagtagcatcaccctctagcttgggaggggtcttcattactggagaagtatccaaacccaagccatttgctctgttgattatgggcgtttctgagccaggagtagaggaagcagagctggggaagaccagagctggggaattcataccaacatcccggactggaggggacacagctgaatcttggaggagcagctgcttgtttccagggtcagtgctggctgggaagttctggttaatggaggaggggctgaggctggctttgccagcaccgctctccagctgctgttgcagctgcagtcgcagacaattgttcccctgaatgctctgctccagctgccctctcagagctcgtacctctgccaccaggtggctcaggtcactgctcaaagggatttggtgacaggcatccaggctgtaagctttcagccccttcttggaattgccataaagtgcctcgtagatttgtagctctgactggagggactcaaagagctgctgtttctcttcacactgttgctgcaggagaaccagcttgtgctgcagtctggagtcgttttcctggagggaaagacgttcctccctgaaatgcaagacctcttgctgcttctccctcaagtcttccaaaagctgctgcctttccaccttctggtgctccagctccttttccagctcttgaaggtgggatcgagaggacagcagagcctccctcaggctttctgtttcctgggagtgctctctggaaacatgactcagttgagcctgaagtcttcgattgtcttccctgaggactctgttctcattgcagagctgaggtatggactccaggccctgactgtagaagttagaagtggatccccttccacgagcagtagaggtcagccggtgttccagttgctcccgtaggcggtcattgatgcagatggattcctccaggcgctggcgcaggttccggatttcaccaagatgctcttccagcaggtcagcccctgtgggtttggagttaagctggtacacagaggagcctgaggataggtccccagatacactccctttctgaggcctcatcacatcccacttgccactgctgcccaggtacccaggctctaggattcttcccagttctatggtgccccttggaggagagtgaggctgggcagagttgaggtagtaggaagagtcggcttccaagtcgttgctcagcaatgtagctgtggaagcaggaggaacagtgctggcacctgaatgggcctggttggcctccttgggggtattctggggagttggcaagctgatggggttgctgttggattcggccttagccccctgagatgcactggttgatgatggtttagaagacaacacagcagaatgactcgaatgatggatggaatctgagtgactgggagaagctttcttctcttcatagtgtgtgtactcgctgactatgtccatgtcagagcaggcttccagttcatcagacaggaaagaggtgctgctgggagagcggtgggagtcagacaaggcatggctgctggagggtgtgagggaccgagcatccagcttggcctgcaggacttcaatcactttctccttctcctgcagctccctgctgagcctgagggccagtggctcaagtccagcttgatctttctcacttttatgatccttggtgctgagtttgctggtgagcctctctgtcagctggcttccctgggcgagttgctcccggaagctctgtcccaggtagtagtcaatgtcattgctccttaggagatcctcaaaagattttactgtatcttttgcatgccgggtgataagataacaaatacctctcccttctcgtattttttgccgtaggtaagacagttcccgggcctgatcctgaatcagggaatcatatttcccaggccacgaggctgatctcagctcctcagccagcttctcttctagtccattttttgggagctgggcctccagctgggatactctctggatgagactctccaggtcctttttggcctgaagccctggagagtagaaagccccagtgccatcagacagccacccctcatcctcatcagggacactatgaggtgaagacccctccaaggtgccaacagctctcagcttccggggtctttccagactagacgaataatcacttgtaactgagagggaccggacccggctcttgaggttttgaatgaccttgttggcattctgcagctgggccttcagatctttgatgtcctttcgtaggaccaagatgttttctgactttccatatacccggaactcttcctgcttccctagctggttctccaagggcttcctctcagaggaactagccagtgttgagccccggcgtccctgctcagagcacagcccctccatcaggaccatttccttgaggctgttgtgctcctcacactcaggactggtggtttcctcccgttcagcctcattctcgcttcggccacaagtctcatagcccaggtcctggaggtccacctggatctgcttgctgtcctgcttcaccaaggattcactaagcataactctgtatttctccagctcgttagcctgagcaaagacagtggcttctgatagcagcagcttctcctggagatcttgatagcgttgtttgcattgtgacagctgggagcgcaggtgctgggtggaccctggtaggctaaacgctgactgaggcccagggtcacgaggctgggactggttatccaactcgcccttctccttgtcttcctcgatctcccatccatcagacattgcttctcccatctgctctttcagctccgcattctcaaggcaaaggctcagcatggtgttcctgatgtgggacactgaggagaatcctgcttcctcaatttgagcctttagctccttcagttcctcctcagctttcctcttctcttctaagtgctggtggaactcagccctcaggtggagcatttcttcctgaagacacctgttactgtcccctcccatcggagaaggaggggaaaaagatgggttctgggtctccacagttgccagacttttctccaaagccaccttgacaagttgctggtgactatggtgtgcagcctcctcctcaatactgtcagtgaactcagtgcttgtatcttcggtgtcatcccctgcagctgcacctccaatggcggccagggtctccagcctgtttaagcgctccaagcttcttccaagaacttcttctagccgactgcgtaacacctgagccccttccagttccacctgcagagttcggtctctctcagagctctctggatgggcatggaacttcaccagactgctatagagctgtctctctgcttgtaaggcctcattgagccgactccgttcatctactagtccttctagcatcagcagcaactgttgtcttcggtttcctgaaatttcttgaccctgggattctactgaagcaactttttcccgaagaagtaagacttcctgggtcaggcgttccatagctggtatgtcttcaggatcaaccagttgcatttgcaggtcctttatgagatcttctttaatctgtatgttcctggtcagagactccatatcagcagcctgcacctgcagctcttcttcctgcacagccatcatggactgtagagcagaaagttccatctgactttctctttcttttttagccatgagttcaagttcctctttggcattactcagttctttttccagccctgcaactgtgtccaagtctcctaatgtggatctgggtatgctgacatcctctttggcagtcaatgaagtgctatcatctctggaaggtatctgcattgaaccttgatcagtctgttttccaagacggccagtgggggtaacttcagcttgttggttagagatgggtgcttgggacatcagggagtctctccctcctaaatattggcgcagggcctgtaattctgaatttctttccattaaggcttgcaccaacttctctgcagcagcttggctttcctgctccctggtgctcacagactgaagcaggccttgaatctccatttcatgttccagcacttgtttatttcgatcacttagaaggtcctgcagcatcctttcctttcgctgtagacgctggcacagctcctctgctatctcactctgccctggtccaagtttgcagagcagtgttgcactaagatcctccacttctttgttcctatcatgaagagacgtctgtaactgctgaatgatactctcttgttccttctgccaacggctaaatttggtttccatttcttctttcagccactggaggttttgacaggtagtagataactgttccacttccaggcctttggccctcaggagactctccatactttgcatagtagcttcattggaggagaggacatcgcgcagtctctctaagtcatgatctcgctctctcacagcaagacgaagctggcgcagttctttttctttctcttctagagcagagaatttttcatctatagcccgctccagagcaacagctttatcatgtattcgctggcgaagtttctcaagcaacatttcatttgcttcaagggttttgtctgagttatctcgatactgtaggagctcccgaaattcctgaagcaactgctccttgtgactcagactatggtttaggtgctggatgttttgttcctgggttcgaatctcattgtatttttcagcctcccaggcacgaagctgttggctcttattctgcaattcttcttgtagctgctgcaaggcttttcgcaattcctggttatgtttccaagaagcctctttctgctgttcactctcgtgtgctgcagcctctacaaattgcacacattgtttggcatcagccagttggcgctctttctgtcgtaccaccctctggagcttctgtatttcaagttggctgcagaataaagcactctgaagatcaagcagagctacctgttgctgagctggagaagtaccctctgagctgtgaagttgtccaagctggctttggtgcagcatttctcgaagctttgccattgtgtcattttgaccttcaattacctggtacaactcctcagtctcacgttccctgcttttcagagtttccttgaggttctgaattgtaccatcttgcttttgagacgactcctgagcacactttagttcatagctcatttcattaagtttctcttgaagaatcttgttggtggcctctgtttgctggattttttcctggagttctgccaagtgggaatcagatacagactgctgagttatagtggtctcatgtgaattcagcttttgttgtttcagcaactcttcagtcatgggctgcacttccatgctagttggctcctccaacagatgtagcagttgttgtttctcccgagatagctgttctacaagcctctcctgggcagccaggctctgattcagttcttcaattctcttgtccctctgggccagggcctcagtgtattggtcgggcttgacctggtctcctggtacatcttcccagtttttggtgactcccttcagtttctctgagagctccaggttacactccttctctgcttccaccagagctgccatccgcgcagcttcattctttgctagcctggattcctcctgcagaagctggatcttattctccaagagctcataaacatgctccgtctcctgctgtcgctcctcaaactggcgtcggagctcagcttcattctgactgttgagattctccacatcagcccatgttttatccagatgctgtttcttgtcctggagttctcgtttcaagctctccacttcaaccttcagctcaatgttccgcttgtagatgtcctcccggctggcctcatacttctgttgcatgcgctcctccaggaagtagatgcgcagcttgaggctgaagttctccttcttcaggtcattgaggtgcttctcaaagtctcgaagagcctgggtctgtacctgagggggtttctcaaatgctctcaaggaatatgtctgcacaaacgggaccttttcaccacttctccagatctgtgactgcactggagggcctcgatctttagtgtcactaagaaaagctgctgtgtgactcgttctgggtaccatctccccatcatcctctgcaaaataatctctcgtccaggtctgctccattttccaggctctttccttagtctcaggacgctcctcacccgggaggggaagcagcctgggaaaatgagaagccttgcccacgaatctccagcgcaaaaggcagcagctttttcctccccagctcctttctgcgtcggcggcgaagagagagctctgctccctgcttttttagaaaatggatttgacgtggccgaacctgcggctagccgtgcgacccgcacaagggagggactgttctcagtaggaggctggactcagagcggcgcggcgcccggggctgtttcgtgagctggagccagcggctgcccgggccgcggtgcgcgcactctccaggctgagacacgact

SEQ ID NO: 8802 - RNA, 7434 nt, Homo sapiens
  source 1..7434: mol_type = other RNA
aagtgtgcagggcactggtgctgctccgaagctcatgaatacctttgctgcctagcacctctgtgccttgggcttcaaggccagggaagctgcacgctgatctcacaagagacactatctttttgaccagcagcttgccctccgcaatctgctgtcttagggcactgtagtcatcaatgtggccaatgacatggcggccatgcttattggcaaaggagccatcagtagcatcaccctctagcttgggaggggtcttcattactggagaagtatccaaacccaagccatttgctctgttgattatgggcgtttctgagccaggagtagaggaagcagagctggggaagaccagagctggggaattcataccaacatcccggactggaggggacacagctgaatcttggaggagcagctgcttgtttccagggtcagtgctggctgggaagttctggttaatggaggaggggctgaggctggctttgccagcaccgctctccagctgctgttgcagctgcagtcgcagacaattgttcccctgaatgctctgctccagctgccctctcagagctcgtacctctgccaccaggtggctcaggtcactgctcaaagggatttggtgacaggcatccaggctgtaagctttcagccccttcttggaattgccataaagtgcctcgtagatttgtagctctgactggagggactcaaagagctgctgtttctcttcacactgttgctgcaggagaaccagcttgtgctgcagtctggagtcgttttcctggagggaaagacgttcctccctgaaatgcaagacctcttgctgcttctccctcaagtcttccaaaagctgctgcctttccaccttctggtgctccagctccttttccagctcttgaaggtgggatcgagaggacagcagagcctccctcaggctttctgtttcctgggagtgctctctggaaacatgactcagttgagcctgaagtcttcgattgtcttccctgaggactctgttctcattgcagagctgaggtatggactccaggccctgactgtagaagttagaagtggatccccttccacgagcagtagaggtcagccggtgttccagttgctcccgtaggcggtcattgatgcagatggattcctccaggcgctggcgcaggttccggatttcaccaagatgctcttccagcaggtcagcccctgtgggtttggagttaagctggtacacagaggagcctgaggataggtccccagatacactccctttctgaggcctcatcacatcccacttgccactgctgcccaggtacccaggctctaggattcttcccagttctatggtgccccttggaggagagtgaggctgggcagagttgaggtagtaggaagagtcggcttccaagtcgttgctcagcaatgtagctgtggaagcaggaggaacagtgctggcacctgaatgggcctggttggcctccttgggggtattctggggagttggcaagctgatggggttgctgttggattcggccttagccccctgagatgcactggttgatgatggtttagaagacaacacagcagaatgactcgaatgatggatggaatctgagtgactgggagaagctttcttctcttcatagtgtgtgtactcgctgactatgtccatgtcagagcaggcttccagttcatcagacaggaaagaggtgctgctgggagagcggtgggagtcagacaaggcatggctgctggagggtgtgagggaccgagcatccagcttggcctgcaggacttcaatcactttctccttctcctgcagctccctgctgagcctgagggccagtggctcaagtccagcttgatctttctcacttttatgatccttggtgctgagtttgctggtgagcctctctgtcagctggcttccctgggcgagttgctcccggaagctctgtcccaggtagtagtcaatgtcattgctccttaggagatcctcaaaagattttactgtatcttttgcatgccgggtgataagataacaaatacctctcccttctcgtattttttgccgtaggtaagacagttcccgggcctgatcctgaatcagggaatcatatttcccaggccacgaggctgatctcagctcctcagccagcttctcttctagtccattttttgggagctgggcctccagctgggatactctctggatgagactctccaggtcctttttggcctgaagccctggagagtagaaagccccagtgccatcagacagccacccctcatcctcatcagggacactatgaggtgaagacccctccaaggtgccaacagctctcagcttccggggtctttccagactagacgaataatcacttgtaactgagagggaccggacccggctcttgaggttttgaatgaccttgttggcattctgcagctgggccttcagatctttgatgtcctttcgtaggaccaagatgttttctgactttccatatacccggaactcttcctgcttccctagctggttctccaagggcttcctctcagaggaactagccagtgttgagccccggcgtccctgctcagagcacagcccctccatcaggaccatttccttgaggctgttgtgctcctcacactcaggactggtggtttcctcccgttcagcctcattctcgcttcggccacaagtctcatagcccaggtcctggaggtccacctggatctgcttgctgtcctgcttcaccaaggattcactaagcataactctgtatttctccagctcgttagcctgagcaaagacagtggcttctgatagcagcagcttctcctggagatcttgatagcgttgtttgcattgtgacagctgggagcgcaggtgctgggtggaccctggtaggctaaacgctgactgaggcccagggtcacgaggctgggactggttatccaattggtgggcatccactgtgaaggtagccccaaggtcaaggctctggggtctggggaaaggcctcacagtcacattcccctcctcttggtgttggtgcttcccaggggaaccaaccagttctgtgtttattctttcaatggtgctggtcagatgcacaaggagctctggagtaagtttactattcccttccttgctactcagcacaagttgttctttgaggaggttgatgatattgtgggcattcttcagttttccctggagctttctgaactcagcctgaaggctactctcactcagaccctctttggttaccacagtctcaaccatcacctcgcccttctccttgtcttcctcgatctcccatccatcagacattgcttctcccatctgctctttcagctccgcattctcaaggcaaaggctcagcatggtgttcctgatgtgggacactgaggagaatcctgcttcctcaatttgagcctttagctccttcagttcctcctcagctttcctcttctcttctaagtgctggtggaactcagccctcaggtggagcatttcttcctgaagacacctgttactgtcccctcccatcggagaaggaggggaaaaagatgggttctgggtctccacagttgccagacttttctccaaagccaccttgacaagttgctggtgactatggtgtgcagcctcctcctcaatactgtcagtgaactcagtgcttgtatcttcggtgtcatcccctgcagctgcacctccaatggcggccagggtctccagcctgtttaagcgctccaagcttcttccaagaacttcttctagccgactgcgtaacacctgagccccttccagttccacctgcagagttcggtctctctcagagctctctggatgggcatggaacttcaccagactgctatagagctgtctctctgcttgtaaggcctcattgagccgactccgttcatctactagtccttctagcatcagcagcaactgttgtcttcggtttcctgaaatttcttgaccctgggattctactgaagcaactttttcccgaagaagtaagacttcctgggtcaggcgttccatagctggtatgtcttcaggatcaaccagttgcatttgcaggtcctttatgagatcttctttaatctgtatgttcctggtcagagactccatatcagcagcctgcacctgcagctcttcttcctgcacagccatcatggactgtagagcagaaagttccatctgactttctctttcttttttagccatgagttcaagttcctctttggcattactcagttctttttccagccctgcaactgtgtccaagtctcctaatgtggatctgggtatgctgacatcctctttggcagtcaatgaagtgctatcatctctggaaggtatctgcattgaaccttgatcagtctgttttccaagacggccagtgggggtaacttcagcttgttggttagagatgggtgcttgggacatcagggagtctctccctcctaaatattggcgcagggcctgtaattctgaatttctttccattaaggcttgcaccaacttctctgcagcagcttggctttcctgctccctggtgctcacagactgaagcaggccttgaatctccatttcatgttccagcacttgtttatttcgatcacttagaaggtcctgcagcatcctttcctttcgctgtagacgctggcacagctcctctgctatctcactctgccctggtccaagtttgcagagcagtgttgcactaagatcctccacttctttgttcctatcatgaagagacgtctgtaactgctgaatgatactctcttgttccttctgccaacggctaaatttggtttccatttcttctttcagccactggaggttttgacaggtagtagataactgttccacttccaggcctttggccctcaggagactctccatactttgcatagtagcttcattggaggagaggacatcgcgcagtctctctaagtcatgatctcgctctctcacagcaagacgaagctggcgcagttctttttctttctcttctagagcagagaatttttcatctatagcccgctccagagcaacagctttatcatgtattcgctggcgaagtttctcaagcaacatttcatttgcttcaagggttttgtctgagttatctcgatactgtaggagctcccgaaattcctgaagcaactgctccttgtgactcagactatggtttaggtgctggatgttttgttcctgggttcgaatctcattgtatttttcagcctcccaggcacgaagctgttggctcttattctgcaattcttcttgtagctgctgcaaggcttttcgcaattcctggttatgtttccaagaagcctctttctgctgttcactctcgtgtgctgcagcctctacaaattgcacacattgtttggcatcagccagttggcgctctttctgtcgtaccaccctctggagcttctgtatttcaagttggctgcagaataaagcactctgaagatcaagcagagctacctgttgctgagctggagaagtaccctctgagctgtgaagttgtccaagctggctttggtgcagcatttctcgaagctttgccattgtgtcattttgaccttcaattacctggtacaactcctcagtctcacgttccctgcttttcagagtttccttgaggttctgaattgtaccatcttgcttttgagacgactcctgagcacactttagttcatagctcatttcattaagtttctcttgaagaatcttgttggtggcctctgtttgctggattttttcctggagttctgccaagtgggaatcagatacagactgctgagttatagtggtctcatgtgaattcagcttttgttgtttcagcaactcttcagtcatgggctggacccggagcggcaaataatcttcacagagatcatcccacagctcctgcaggtctgaaagctccaagggataactcacaggtgtcttgtaaaggggtttcaaagacctgttaaggaaaccggaactaactccatctgtcatgctagggccaggcttggctccaggtaggctggatttcactggaatcggaagcctgctccctcgggggctctggatgggcttataatcaagacctttaatcatgctaagagctaattccagcttgtgattacacccatgctgcggagcctgatcatctgaacaacagtcacactttccaagttcctttgcacttctctcagtctcctcatctttctgttgtggagggctagcctggacgcttgcatccaaagattccacagaggaaccaggcgtctcttcctccatgctttctccatctgggggtacctttgtgcttgctaagtcgggtggcccaacctcagacaacgctggttcttcagtgcaaatgctggtcgaccacctgctagaagggccgcaggagatacttctggccacctttcgaggtaccttacaaatggcttcatagtcagaatcagcaacccgcaaagcggcacaaccacggcatctcctgggtcggtttccagggccttctgaaccatggcagctgtgtggctcctggatctgatcctcattctccacccagcactcaaaccctgaataggcgaagtcctcctggagcagtgcagagtatctcgcatcgggtaagacggacatgtcaaccgtcccattccccgccttgatctccgcgccagagtcatcgttattcttccgatacatactggcaatgcagaacttgaggcgatccttctccagtagcagcttttgcaagcgctcaatagaaagcgcttcaatccgggcaataactgtgtcgaatcgatagattcgatcaagcatgaaagcacacttgctgcaagcgaactcggctttgccatcgcgggggacatccttgcccaagacgtgcgaaagcagaacctggagattgagcttggacgccgtgtggaagatccagcgccgctggtttccacacagctctcgggcacagatcctgcaaatctccttcatcttccctcctagcgggtggcaagcttcccgaggcggcggcggcggcggctactgggtgaccactcaatggctcttcgccgcgctctgtctcccgcctcggtggtctccggtcagcatggcacagcccagtggggtccccactctgcaggggcgcgcccctgccccgcgcgccgactccgggtaccagagccgtcagccccgcccctcgggcagggggcgggcgtggaaacgcctaagaggatgctgagtgacagaggcgcaggccgcgctccgaccctgccatgtctctccccagctgtctctcccgccagccgccgcgtcctcaacgtcctccccttttagcagactgggctcccggagcagcagcggccggccgcgcagacgcaaagcctcggggatggaggatc

SEQ ID NO: 8803 - RNA, 6942 nt, Homo sapiens
  source 1..6942: mol_type = other RNA
aagtgtgcagggcactggtgctgctccgaagctcatgaatacctttgctgcctagcacctctgtgccttgggcttcaaggccagggaagctgcacgctgatctcacaagagacactatctttttgaccagcagcttgccctccgcaatctgctgtcttagggcactgtagtcatcaatgtggccaatgacatggcggccatgcttattggcaaaggagccatcagtagcatcaccctctagcttgggaggggtcttcattactggagaagtatccaaacccaagccatttgctctgttgattatgggcgtttctgagccaggagtagaggaagcagagctggggaagaccagagctggggaattcataccaacatcccggactggaggggacacagctgaatcttggaggagcagctgcttgtttccagggtcagtgctggctgggaagttctggttaatggaggaggggctgaggctggctttgccagcaccgctctccagctgctgttgcagctgcagtcgcagacaattgttcccctgaatgctctgctccagctgccctctcagagctcgtacctctgccaccaggtggctcaggtcactgctcaaagggatttggtgacaggcatccaggctgtaagctttcagccccttcttggaattgccataaagtgcctcgtagatttgtagctctgactggagggactcaaagagctgctgtttctcttcacactgttgctgcaggagaaccagcttgtgctgcagtctggagtcgttttcctggagggaaagacgttcctccctgaaatgcaagacctcttgctgcttctccctcaagtcttccaaaagctgctgcctttccaccttctggtgctccagctccttttccagctcttgaaggtgggatcgagaggacagcagagcctccctcaggctttctgtttcctgggagtgctctctggaaacatgactcagttgagcctgaagtcttcgattgtcttccctgaggactctgttctcattgcagagctgaggtatggactccaggccctgactgtagaagttagaagtggatccccttccacgagcagtagaggtcagccggtgttccagttgctcccgtaggcggtcattgatgcagatggattcctccaggcgctggcgcaggttccggatttcaccaagatgctcttccagcaggtcagcccctgtgggtttggagttaagctggtacacagaggagcctgaggataggtccccagatacactccctttctgaggcctcatcacatcccacttgccactgctgcccaggtacccaggctctaggattcttcccagttctatggtgccccttggaggagagtgaggctgggcagagttgaggtagtaggaagagtcggcttccaagtcgttgctcagcaatgtagctgtggaagcaggaggaacagtgctggcactttctcccaactgcttctgcagcatctgtagctcctgctgagcctcagccaaggagaccactggtgtctcacagcagccaaggaggagagggccagtggggctgaaaggcaggaagctggatggagctgagggcaatggtgcctgaggaaggctagccagcttgggtatggagtgaaaatgaaagcctgaatgggcctggttggcctccttgggggtattctggggagttggcaagctgatggggttgctgttggattcggccttagccccctgagatgcactggttgatgatggtttagaagacaacacagcagaatgactcgaatgatggatggaatctgagtgactgggagaagctttcttctcttcatagtgtgtgtactcgctgactatgtccatgtcagagcaggcttccagttcatcagacaggaaagaggtgctgctgggagagcggtgggagtcagacaaggcatggctgctggagggtgtgagggaccgagcatccagcttggcctgcaggacttcaatcactttctccttctcctgcagctccctgctgagcctgagggccagtggctcaagtccagcttgatctttctcacttttatgatccttggtgctgagtttgctggtgagcctctctgtcagctggcttccctgggcgagttgctcccggaagctctgtcccaggtagtagtcaatgtcattgctccttaggagatcctcaaaagattttactgtatcttttgcatgccgggtgataagataacaaatacctctcccttctcgtattttttgccgtaggtaagacagttcccgggcctgatcctgaatcagggaatcatatttcccaggccacgaggctgatctcagctcctcagccagcttctcttctagtccattttttgggagctgggcctccagctgggatactctctggatgagactctccaggtcctttttggcctgaagccctggagagtagaaagccccagtgccatcagacagccacccctcatcctcatcagggacactatgaggtgaagacccctccaaggtgccaacagctctcagcttccggggtctttccagactagacgaataatcacttgtaactgagagggaccggacccggctcttgaggttttgaatgaccttgttggcattctgcagctgggccttcagatctttgatgtcctttcgtaggaccaagatgttttctgactttccatatacccggaactcttcctgcttccctagctggttctccaagggcttcctctcagaggaactagccagtgttgagccccggcgtccctgctcagagcacagcccctccatcaggaccatttccttgaggctgttgtgctcctcacactcaggactggtggtttcctcccgttcagcctcattctcgcttcggccacaagtctcatagcccaggtcctggaggtccacctggatctgcttgctgtcctgcttcaccaaggattcacctgtaagcataactctgtatttctccagctcgttagcctgagcaaagacagtggcttctgatagcagcagcttctcctggagatcttgatagcgttgtttgcattgtgacagctgggagcgcaggtgctgggtggaccctggtaggctaaacgctgactgaggcccagggtcacgaggctgggactggttatccaactcgcccttctccttgtcttcctcgatctcccatccatcagacattgcttctcccatctgctctttcagctccgcattctcaaggcaaaggctcagcatggtgttcctgatgtgggacactgaggagaatcctgcttcctcaatttgagcctttagctccttcagttcctcctcagctttcctcttctcttctaagtgctggtggaactcagccctcaggtggagcatttcttcctgaagacacctgttactgtcccctcccatcggagaaggaggggaaaaagatgggttctgggtctccacagttgccagacttttctccaaagccaccttgacaagttgctggtgactatggtgtgcagcctcctcctcaatactgtcagtgaactcagtgcttgtatcttcggtgtcatcccctgcagctgcacctccaatggcggccagggtctccagcctgtttaagcgctccaagcttcttccaagaacttcttctagccgactgcgtaacacctgagccccttccagttccacctgcagagttcggtctctctcagagctctctggatgggcatggaacttcaccagactgctatagagctgtctctctgcttgtaaggcctcattgagccgactccgttcatctactagtccttctagcatcagcagcaactgttgtcttcggtttcctgaaatttcttgaccctgggattctactgaagcaactttttcccgaagaagtaagacttcctgggtcaggcgttccatagctggtatgtcttcaggatcaaccagttgcatttgcaggtcctttatgagatcttctttaatctgtatgttcctggtcagagactccatatcagcagcctgcacctgcagctcttcttcctgcacagccatcatggactgtagagcagaaagttccatctgactttctctttcttttttagccatgagttcaagttcctctttggcattactcagttctttttccagccctgcaactgtgtccaagtctcctaatgtggatctgggtatgctgacatcctctttggcagtcaatgaagtgctatcatctctggaaggtatctgcattgaaccttgatcagtctgttttccaagacggccagtgggggtaacttcagcttgttggttagagatgggtgcttgggacatcagggagtctctccctcctaaatattggcgcagggcctgtaattctgaatttctttccattaaggcttgcaccaacttctctgcagcagcttggctttcctgctccctggtgctcacagactgaagcaggccttgaatctccatttcatgttccagcacttgtttatttcgatcacttagaaggtcctgcagcatcctttcctttcgctgtagacgctggcacagctcctctgctatctcactctgccctggtccaagtttgcagagcagtgttgcactaagatcctccacttctttgttcctatcatgaagagacgtctgtaactgctgaatgatactctcttgttccttctgccaacggctaaatttggtttccatttcttctttcagccactggaggttttgacaggtagtagataactgttccacttccaggcctttggccctcaggagactctccatactttgcatagtagcttcattggaggagaggacatcgcgcagtctctctaagtcatgatctcgctctctcacagcaagacgaagctggcgcagttctttttctttctcttctagagcagagaatttttcatctatagcccgctccagagcaacagctttatcatgtattcgctggcgaagtttctcaagcaacatttcatttgcttcaagggttttgtctgagttatctcgatactgtaggagctcccgaaattcctgaagcaactgctccttgtgactcagactatggtttaggtgctggatgttttgttcctgggttcgaatctcattgtatttttcagcctcccaggcacgaagctgttggctcttattctgcaattcttcttgtagctgctgcaaggcttttcgcaattcctggttatgtttccaagaagcctctttctgctgttcactctcgtgtgctgcagcctctacaaattgcacacattgtttggcatcagccagttggcgctctttctgtcgtaccaccctctggagcttctgtatttcaagttggctgcagaataaagcactctgaagatcaagcagagctacctgttgctgagctggagaagtaccctctgagctgtgaagttgtccaagctggctttggtgcagcatttctcgaagctttgccattgtgtcattttgaccttcaattacctggtacaactcctcagtctcacgttccctgcttttcagagtttccttgaggttctgaattgtaccatcttgcttttgagacgactcctgagcacactttagttcatagctcatttcattaagtttctcttgaagaatcttgttggtggcctctgtttgctggattttttcctggagttctgccaagtgggaatcagatacagactgctgagttatagtggtctcatgtgaattcagcttttgttgtttcagcaactcttcagtcatgggctgcacttccatgctagttggctcctccaacagatgtagcagttgttgtttctcccgagatagctgttctacaagcctctcctgggcagccaggctctgattcagttcttcaattctcttgtccctctgggccagggcctcagtgtattggtcgggcttgacctggtctcctggtacatcttcccagtttttggtgactcccttcagtttctctgagagctccaggttacactccttctctgcttccaccagagctgccatccgcgcagcttcattctttgctagcctggattcctcctgcagaagctggatcttattctccaagagctcataaacatgctccgtctcctgctgtcgctcctcaaactggcgtcggagctcagcttcattctgactgttgagattctccacatcagcccatgttttatccagatgctgtttcttgtcctggagttctcgtttcaagctctccacttcaaccttcagctcaatgttccgcttgtagatgtcctcccggctggcctcatacttctgttgcatgcgctcctccaggaagtagatgcgcagcttgaggctgaagttctccttcttcaggtcattgaggtgcttctcaaagtctcgaagagcctgggtctgtacctgagggggtttctcaaatgctctcaaggaatatgtctgcacaaacgggaccttttcaccacttctccagatctgtgactgcactggagggcctcgatctttagtgtcactaagaaaagctgctgtgtgactcgttctgggtaccatctccccatcatcctctgcaaaataatctctcgtccaggtctgctccattttccaggctctttccttagtctcaggacgctcctcacccgggaggggaagcagcctgggaaaatgagaagccttgcccacgaatctccagcgcaaaaggcagcagctttttcctccccagctcctttctgcgtcggcggcgaagagagagctctgctccctgcttttttagaaaatggatttgacgtggccgaacctgcggctagccgtgcgacccgcacaagggagggactgttctcagtaggaggctggactcagagcggcgcggcgcccggggctgtttcgtgagctggagccagcggctgcccgggccgcggtgcgcgcactctccaggctgagacacgact

SEQ ID NO: 8804 - RNA, 7293 nt, Homo sapiens
  source 1..7293: mol_type = other RNA
aagtgtgcagggcactggtgctgctccgaagctcatgaatacctttgctgcctagcacctctgtgccttgggcttcaaggccagggaagctgcacgctgatctcacaagagacactatctttttgaccagcagcttgccctccgcaatctgctgtcttagggcactgtagtcatcaatgtggccaatgacatggcggccatgcttattggcaaaggagccatcagtagcatcaccctctagcttgggaggggtcttcattactggagaagtatccaaacccaagccatttgctctgttgattatgggcgtttctgagccaggagtagaggaagcagagctggggaagaccagagctggggaattcataccaacatcccggactggaggggacacagctgaatcttggaggagcagctgcttgtttccagggtcagtgctggctgggaagttctggttaatggaggaggggctgaggctggctttgccagcaccgctctccagctgctgttgcagctgcagtcgcagacaattgttcccctgaatgctctgctccagctgccctctcagagctcgtacctctgccaccaggtggctcaggtcactgctcaaagggatttggtgacaggcatccaggctgtaagctttcagccccttcttggaattgccataaagtgcctcgtagatttgtagctctgactggagggactcaaagagctgctgtttctcttcacactgttgctgcaggagaaccagcttgtgctgcagtctggagtcgttttcctggagggaaagacgttcctccctgaaatgcaagacctcttgctgcttctccctcaagtcttccaaaagctgctgcctttccaccttctggtgctccagctccttttccagctcttgaaggtgggatcgagaggacagcagagcctccctcaggctttctgtttcctgggagtgctctctggaaacatgactcagttgagcctgaagtcttcgattgtcttccctgaggactctgttctcattgcagagctgaggtatggactccaggccctgactgtagaagttagaagtggatccccttccacgagcagtagaggtcagccggtgttccagttgctcccgtaggcggtcattgatgcagatggattcctccaggcgctggcgcaggttccggatttcaccaagatgctcttccagcaggtcagcccctgtgggtttggagttaagctggtacacagaggagcctgaggataggtccccagatacactccctttctgaggcctcatcacatcccacttgccactgctgcccaggtacccaggctctaggattcttcccagttctatggtgccccttggaggagagtgaggctgggcagagttgaggtagtaggaagagtcggcttccaagtcgttgctcagcaatgtagctgtggaagcaggaggaacagtgctggcactttctcccaactgcttctgcagcatctgtagctcctgctgagcctcagccaaggagaccactggtgtctcacagcagccaaggaggagagggccagtggggctgaaaggcaggaagctggatggagctgagggcaatggtgcctgaggaaggctagccagcttgggtatggagtgaaaatgaaagcctgaatgggcctggttggcctccttgggggtattctggggagttggcaagctgatggggttgctgttggattcggccttagccccctgagatgcactggttgatgatggtttagaagacaacacagcagaatgactcgaatgatggatggaatctgagtgactgggagaagctttcttctcttcatagtgtgtgtactcgctgactatgtccatgtcagagcaggcttccagttcatcagacaggaaagaggtgctgctgggagagcggtgggagtcagacaaggcatggctgctggagggtgtgagggaccgagcatccagcttggcctgcaggacttcaatcactttctccttctcctgcagctccctgctgagcctgagggccagtggctcaagtccagcttgatctttctcacttttatgatccttggtgctgagtttgctggtgagcctctctgtcagctggcttccctgggcgagttgctcccggaagctctgtcccaggtagtagtcaatgtcattgctccttaggagatcctcaaaagattttactgtatcttttgcatgccgggtgataagataacaaatacctctcccttctcgtattttttgccgtaggtaagacagttcccgggcctgatcctgaatcagggaatcatatttcccaggccacgaggctgatctcagctcctcagccagcttctcttctagtccattttttgggagctgggcctccagctgggatactctctggatgagactctccaggtcctttttggcctgaagccctggagagtagaaagccccagtgccatcagacagccacccctcatcctcatcagggacactatgaggtgaagacccctccaaggtgccaacagctctcagcttccggggtctttccagactagacgaataatcacttgtaactgagagggaccggacccggctcttgaggttttgaatgaccttgttggcattctgcagctgggccttcagatctttgatgtcctttcgtaggaccaagatgttttctgactttccatatacccggaactcttcctgcttccctagctggttctccaagggcttcctctcagaggaactagccagtgttgagccccggcgtccctgctcagagcacagcccctccatcaggaccatttccttgaggctgttgtgctcctcacactcaggactggtggtttcctcccgttcagcctcattctcgcttcggccacaagtctcatagcccaggtcctggaggtccacctggatctgcttgctgtcctgcttcaccaaggattcacctgtaagcataactctgtatttctccagctcgttagcctgagcaaagacagtggcttctgatagcagcagcttctcctggagatcttgatagcgttgtttgcattgtgacagctgggagcgcaggtgctgggtggaccctggtaggctaaacgctgactgaggcccagggtcacgaggctgggactggttatccaactcgcccttctccttgtcttcctcgatctcccatccatcagacattgcttctcccatctgctctttcagctccgcattctcaaggcaaaggctcagcatggtgttcctgatgtgggacactgaggagaatcctgcttcctcaatttgagcctttagctccttcagttcctcctcagctttcctcttctcttctaagtgctggtggaactcagccctcaggtggagcatttcttcctgaagacacctgttactgtcccctcccatcggagaaggaggggaaaaagatgggttctgggtctccacagttgccagacttttctccaaagccaccttgacaagttgctggtgactatggtgtgcagcctcctcctcaatactgtcagtgaactcagtgcttgtatcttcggtgtcatcccctgcagctgcacctccaatggcggccagggtctccagcctgtttaagcgctccaagcttcttccaagaacttcttctagccgactgcgtaacacctgagccccttccagttccacctgcagagttcggtctctctcagagctctctggatgggcatggaacttcaccagactgctatagagctgtctctctgcttgtaaggcctcattgagccgactccgttcatctactagtccttctagcatcagcagcaactgttgtcttcggtttcctgaaatttcttgaccctgggattctactgaagcaactttttcccgaagaagtaagacttcctgggtcaggcgttccatagctggtatgtcttcaggatcaaccagttgcatttgcaggtcctttatgagatcttctttaatctgtatgttcctggtcagagactccatatcagcagcctgcacctgcagctcttcttcctgcacagccatcatggactgtagagcagaaagttccatctgactttctctttcttttttagccatgagttcaagttcctctttggcattactcagttctttttccagccctgcaactgtgtccaagtctcctaatgtggatctgggtatgctgacatcctctttggcagtcaatgaagtgctatcatctctggaaggtatctgcattgaaccttgatcagtctgttttccaagacggccagtgggggtaacttcagcttgttggttagagatgggtgcttgggacatcagggagtctctccctcctaaatattggcgcagggcctgtaattctgaatttctttccattaaggcttgcaccaacttctctgcagcagcttggctttcctgctccctggtgctcacagactgaagcaggccttgaatctccatttcatgttccagcacttgtttatttcgatcacttagaaggtcctgcagcatcctttcctttcgctgtagacgctggcacagctcctctgctatctcactctgccctggtccaagtttgcagagcagtgttgcactaagatcctccacttctttgttcctatcatgaagagacgtctgtaactgctgaatgatactctcttgttccttctgccaacggctaaatttggtttccatttcttctttcagccactggaggttttgacaggtagtagataactgttccacttccaggcctttggccctcaggagactctccatactttgcatagtagcttcattggaggagaggacatcgcgcagtctctctaagtcatgatctcgctctctcacagcaagacgaagctggcgcagttctttttctttctcttctagagcagagaatttttcatctatagcccgctccagagcaacagctttatcatgtattcgctggcgaagtttctcaagcaacatttcatttgcttcaagggttttgtctgagttatctcgatactgtaggagctcccgaaattcctgaagcaactgctccttgtgactcagactatggtttaggtgctggatgttttgttcctgggttcgaatctcattgtatttttcagcctcccaggcacgaagctgttggctcttattctgcaattcttcttgtagctgctgcaaggcttttcgcaattcctggttatgtttccaagaagcctctttctgctgttcactctcgtgtgctgcagcctctacaaattgcacacattgtttggcatcagccagttggcgctctttctgtcgtaccaccctctggagcttctgtatttcaagttggctgcagaataaagcactctgaagatcaagcagagctacctgttgctgagctggagaagtaccctctgagctgtgaagttgtccaagctggctttggtgcagcatttctcgaagctttgccattgtgtcattttgaccttcaattacctggtacaactcctcagtctcacgttccctgcttttcagagtttccttgaggttctgaattgtaccatcttgcttttgagacgactcctgagcacactttagttcatagctcatttcattaagtttctcttgaagaatcttgttggtggcctctgtttgctggattttttcctggagttctgccaagtgggaatcagatacagactgctgagttatagtggtctcatgtgaattcagcttttgttgtttcagcaactcttcagtcatgggctggacccggagcggcaaataatcttcacagagatcatcccacagctcctgcaggtctgaaagctccaagggataactcacaggtgtcttgtaaaggggtttcaaagacctgttaaggaaaccggaactaactccatctgtcatgctagggccaggcttggctccaggtaggctggatttcactggaatcggaagcctgctccctcgggggctctggatgggcttataatcaagacctttaatcatgctaagagctaattccagcttgtgattacacccatgctgcggagcctgatcatctgaacaacagtcacactttccaagttcctttgcacttctctcagtctcctcatctttctgttgtggagggctagcctggacgcttgcatccaaagattccacagaggaaccaggcgtctcttcctccatgctttctccatctgggggtacctttgtgcttgctaagtcgggtggcccaacctcagacaacgctggttcttcagtgcaaatgctggtcgaccacctgctagaagggccgcaggagatacttctggccacctttcgaggtaccttacaaatggcttcatagtcagaatcagcaacccgcaaagcggcacaaccacggcatctcctgggtcggtttccagggccttctgaaccatggcagctgtgtggctcctggatctgatcctcattctccacccagcactcaaaccctgaataggcgaagtcctcctggagcagtgcagagtatctcgcatcgggtaagacggacatgtcaaccgtcccattccccgccttgatctccgcgccagagtcatcgttattcttccgatacatactggcaatgcagaacttgaggcgatccttctccagtagcagcttttgcaagcgctcaatagaaagcgcttcaatccgggcaataactgtgtcgaatcgatagattcgatcaagcatgaaagcacacttgctgcaagcgaactcggctttgccatcgcgggggacatccttgcccaagacgtgcgaaagcagaacctggagattgagcttggacgccgtgtggaagatccagcgccgctggtttccacacagctctcgggcacagatcctgcaaatctccttcatcttccctcctagcgggtggcaagcttcccgaggcggcggcggcggcggctactgggtgaccactcaatggctcttcgccgcgctctgtctcccgcctcggtggtctccggtcagcatggcacagcccagtggggtccccactctgcaggggcgcgcccctgccccgcgcgccgactccgggtaccagagccgtcagccccgcccctcgggcagggggcgggcgtggaaacgcctaagaggatgctgagtgacagaggcgcaggccgcgctccgaccctgccatgtctctccccagctgtctctcccgccagccgccgcgtcctcaacgtcctccccttttagcagactgggctcccggagcagcagcggccggccgcgcagacgcaaagcctcggggatggaggatc

SEQ ID NO: 8805 - RNA, 6815 nt, Homo sapiens
  source 1..6815: mol_type = other RNA
aagtgtgcagggcactggtgctgctccgaagctcatgaatacctttgctgcctagcacctctgtgccttgggcttcaaggccagggaagctgcacgctgatctcacaagagacactatctttttgaccagcagcttgccctccgcaatctgctgtcttagggcactgtagtcatcaatgtggccaatgacatggcggccatgcttattggcaaaggagccatcagtagcatcaccctctagcttgggaggggtcttcattactggagaagtatccaaacccaagccatttgctctgttgattatgggcgtttctgagccaggagtagaggaagcagagctggggaagaccagagctggggaattcataccaacatcccggactggaggggacacagctgaatcttggaggagcagctgcttgtttccagggtcagtgctggctgggaagttctggttaatggaggaggggctgaggctggctttgccagcaccgctctccagctgctgttgcagctgcagtcgcagacaattgttcccctgaatgctctgctccagctgccctctcagagctcgtacctctgccaccaggtggctcaggtcactgctcaaagggatttggtgacaggcatccaggctgtaagctttcagccccttcttggaattgccataaagtgcctcgtagatttgtagctctgactggagggactcaaagagctgctgtttctcttcacactgttgctgcaggagaaccagcttgtgctgcagtctggagtcgttttcctggagggaaagacgttcctccctgaaatgcaagacctcttgctgcttctccctcaagtcttccaaaagctgctgcctttccaccttctggtgctccagctccttttccagctcttgaaggtgggatcgagaggacagcagagcctccctcaggctttctgtttcctgggagtgctctctggaaacatgactcagttgagcctgaagtcttcgattgtcttccctgaggactctgttctcattgcagagctgaggtatggactccaggccctgactgtagaagttagaagtggatccccttccacgagcagtagaggtcagccggtgttccagttgctcccgtaggcggtcattgatgcagatggattcctccaggcgctggcgcaggttccggatttcaccaagatgctcttccagcaggtcagcccctgtgggtttggagttaagctggtacacagaggagcctgaggataggtccccagatacactccctttctgaggcctcatcacatcccacttgccactgctgcccaggtacccaggctctaggattcttcccagttctatggtgccccttggaggagagtgaggctgggcagagttgaggtagtaggaagagtcggcttccaagtcgttgctcagcaatgtagctgtggaagcaggaggaacagtgctggcactttctcccaactgcttctgcagcatctgtagctcctgctgagcctcagccaaggagaccactggtgtctcacagcagccaaggaggagagggccagtggggctgaaaggcaggaagctggatggagctgagggcaatggtgcctgaggaaggctagccagcttgggtatggagtgaaaatgaaagcctgaatgggcctggttggcctccttgggggtattctggggagttggcaagctgatggggttgctgttggattcggccttagccccctgagatgcactggttgatgatggtttagaagacaacacagcagaatgactcgaatgatggatggaatctgagtgactgggagaagctttcttctcttcatagtgtgtgtactcgctgactatgtccatgtcagagcaggcttccagttcatcagacaggaaagaggtgctgctgggagagcggtgggagtcagacaaggcatggctgctggagggtgtgagggaccgagcatccagcttggcctgcaggacttcaatcactttctccttctcctgcagctccctgctgagcctgagggccagtggctcaagtccagcttgatctttctcacttttatgatccttggtgctgagtttgctggtgagcctctctgtcagctggcttccctgggcgagttgctcccggaagctctgtcccaggtagtagtcaatgtcattgctccttaggagatcctcaaaagattttactgtatcttttgcatgccgggtgataagataacaaatacctctcccttctcgtattttttgccgtaggtaagacagttcccgggcctgatcctgaatcagggaatcatatttcccaggccacgaggctgatctcagctcctcagccagcttctcttctagtccattttttgggagctgggcctccagctgggatactctctggatgagactctccaggtcctttttggcctgaagccctggagagtagaaagccccagtgccatcagacagccacccctcatcctcatcagggacactatgaggtgaagacccctccaaggtgccaacagctctcagcttccggggtctttccagactagacgaataatcacttgtaactgagagggaccggacccggctcttgaggttttgaatgaccttgttggcattctgcagctgggccttcagatctttgatgtcctttcgtaggaccaagatgttttctgactttccatatacccggaactcttcctgcttccctagctggttctccaagggcttcctctcagaggaactagccagtgttgagccccggcgtccctgctcagagcacagcccctccatcaggaccatttccttgaggctgttgtgctcctcacactcaggactggtggtttcctcccgttcagcctcattctcgcttcggccacaagtctcatagcccaggtcctggaggtccacctggatctgcttgctgtcctgcttcaccaaggattcacctgtaagcataactctgtatttctccagctcgttagcctgagcaaagacagtggcttctgatagcagcagcttctcctggagatcttgatagcgttgtttgcattgtgacagctgggagcgcaggtgctgggtggaccctggtaggctaaacgctgactgaggcccagggtcacgaggctgggactggttatccaattggtgggcatccactgtgaaggtagccccaaggtcaaggctctggggtctggggaaaggcctcacagtcacattcccctcctcttggtgttggtgcttcccaggggaaccaaccagttctgtgtttattctttcaatggtgctggtcagatgcacaaggagctctggagtaagtttactattcccttccttgctactcagcacaagttgttctttgaggaggttgatgatattgtgggcattcttcagttttccctggagctttctgaactcagcctgaaggctactctcactcagaccctctttggttaccacagtctcaaccatcacctcgcccttctccttgtcttcctcgatctcccatccatcagacattgcttctcccatctgctctttcagctccgcattctcaaggcaaaggctcagcatggtgttcctgatgtgggacactgaggagaatcctgcttcctcaatttgagcctttagctccttcagttcctcctcagctttcctcttctcttctaagtgctggtggaactcagccctcaggtggagcatttcttcctgaagacacctgttactgtcccctcccatcggagaaggaggggaaaaagatgggttctgggtctccacagttgccagacttttctccaaagccaccttgacaagttgctggtgactatggtgtgcagcctcctcctcaatactgtcagtgaactcagtgcttgtatcttcggtgtcatcccctgcagctgcacctccaatggcggccagggtctccagcctgtttaagcgctccaagcttcttccaagaacttcttctagccgactgcgtaacacctgagccccttccagttccacctgcagagttcggtctctctcagagctctctggatgggcatggaacttcaccagactgctatagagctgtctctctgcttgtaaggcctcattgagccgactccgttcatctactagtccttctagcatcagcagcaactgttgtcttcggtttcctgaaatttcttgaccctgggattctactgaagcaactttttcccgaagaagtaagacttcctgggtcaggcgttccatagctggtatgtcttcaggatcaaccagttgcatttgcaggtcctttatgagatcttctttaatctgtatgttcctggtcagagactccatatcagcagcctgcacctgcagctcttcttcctgcacagccatcatggactgtagagcagaaagttccatctgactttctctttcttttttagccatgagttcaagttcctctttggcattactcagttctttttccagccctgcaactgtgtccaagtctcctaatgtggatctgggtatgctgacatcctctttggcagtcaatgaagtgctatcatctctggaaggtatctgcattgaaccttgatcagtctgttttccaagacggccagtgggggtaacttcagcttgttggttagagatgggtgcttgggacatcagggagtctctccctcctaaatattggcgcagggcctgtaattctgaatttctttccattaaggcttgcaccaacttctctgcagcagcttggctttcctgctccctggtgctcacagactgaagcaggccttgaatctccatttcatgttccagcacttgtttatttcgatcacttagaaggtcctgcagcatcctttcctttcgctgtagacgctggcacagctcctctgctatctcactctgccctggtccaagtttgcagagcagtgttgcactaagatcctccacttctttgttcctatcatgaagagacgtctgtaactgctgaatgatactctcttgttccttctgccaacggctaaatttggtttccatttcttctttcagccactggaggttttgacaggtagtagataactgttccacttccaggcctttggccctcaggagactctccatactttgcatagtagcttcattggaggagaggacatcgcgcagtctctctaagtcatgatctcgctctctcacagcaagacgaagctggcgcagttctttttctttctcttctagagcagagaatttttcatctatagcccgctccagagcaacagctttatcatgtattcgctggcgaagtttctcaagcaacatttcatttgcttcaagggttttgtctgagttatctcgatactgtaggagctcccgaaattcctgaagcaactgctccttgtgactcagactatggtttaggtgctggatgttttgttcctgggttcgaatctcattgtatttttcagcctcccaggcacgaagctgttggctcttattctgcaattcttcttgtagctgctgcaaggcttttcgcaattcctggttatgtttccaagaagcctctttctgctgttcactctcgtgtgctgcagcctctacaaattgcacacattgtttggcatcagccagttggcgctctttctgtcgtaccaccctctggagcttctgtatttcaagttggctgcagaataaagcactctgaagatcaagcagagctacctgttgctgagctggagaagtaccctctgagctgtgaagttgtccaagctggctttggtgcagcatttctcgaagctttgccattgtgtcattttgaccttcaattacctggtacaactcctcagtctcacgttccctgcttttcagagtttccttgaggttctgaattgtaccatcttgcttttgagacgactcctgagcacactttagttcatagctcatttcattaagtttctcttgaagaatcttgttggtggcctctgtttgctggattttttcctggagttctgccaagtgggaatcagatacagactgctgagttatagtggtctcatgtgaattcagcttttgttgtttcagcaactcttcagtcatgggctgcacttccatgctagttggctcctccaacagatgtagcagttgttgtttctcccgagatagctgttctacaagcctctcctgggcagccaggctctgattcagttcttcaattctcttgtccctctgggccagggcctcagtgtattggtcgggcttgacctggtctcctggtacatcttcccagtttttggtgactcccttcagtttctctgagagctccaggttacactccttctctgcttccaccagagctgccatccgcgcagcttcattctttgctagcctggattcctcctgcagaagctggatcttattctccaagagctcataaacatgctccgtctcctgctgtcgctcctcaaactggcgtcggagctcagcttcattctgactgttgagattctccacatcagcccatgttttatccagatgctgtttcttgtcctggagttctcgtttcaagctctccacttcaaccttcagctcaatgttccgcttgtagatgtcctcccggctggcctcatacttctgttgcatgcgctcctccaggaagtagatgcgcagcttgaggctgaagttctccttcttcaggtcattgaggtgctcagggagatatttgcggaatccctgacagaggaacatgctgcgtgaactcagacacaagtggtgtaacccgactccaagccaggactctgctgtcaccctcctggagcctcccagg

SEQ ID NO: 8806 - RNA, 6921 nt, Homo sapiens
  source 1..6921: mol_type = other RNA
aagtgtgcagggcactggtgctgctccgaagctcatgaatacctttgctgcctagcacctctgtgccttgggcttcaaggccagggaagctgcacgctgatctcacaagagacactatctttttgaccagcagcttgccctccgcaatctgctgtcttagggcactgtagtcatcaatgtggccaatgacatggcggccatgcttattggcaaaggagccatcagtagcatcaccctctagcttgggaggggtcttcattactggagaagtatccaaacccaagccatttgctctgttgattatgggcgtttctgagccaggagtagaggaagcagagctggggaagaccagagctggggaattcataccaacatcccggactggaggggacacagctgaatcttggaggagcagctgcttgtttccagggtcagtgctggctgggaagttctggttaatggaggaggggctgaggctggctttgccagcaccgctctccagctgctgttgcagctgcagtcgcagacaattgttcccctgaatgctctgctccagctgccctctcagagctcgtacctctgccaccaggtggctcaggtcactgctcaaagggatttggtgacaggcatccaggctgtaagctttcagccccttcttggaattgccataaagtgcctcgtagatttgtagctctgactggagggactcaaagagctgctgtttctcttcacactgttgctgcaggagaaccagcttgtgctgcagtctggagtcgttttcctggagggaaagacgttcctccctgaaatgcaagacctcttgctgcttctccctcaagtcttccaaaagctgctgcctttccaccttctggtgctccagctccttttccagctcttgaaggtgggatcgagaggacagcagagcctccctcaggctttctgtttcctgggagtgctctctggaaacatgactcagttgagcctgaagtcttcgattgtcttccctgaggactctgttctcattgcagagctgaggtatggactccaggccctgactgtagaagttagaagtggatccccttccacgagcagtagaggtcagccggtgttccagttgctcccgtaggcggtcattgatgcagatggattcctccaggcgctggcgcaggttccggatttcaccaagatgctcttccagcaggtcagcccctgtgggtttggagttaagctggtacacagaggagcctgaggataggtccccagatacactccctttctgaggcctcatcacatcccacttgccactgctgcccaggtacccaggctctaggattcttcccagttctatggtgccccttggaggagagtgaggctgggcagagttgaggtagtaggaagagtcggcttccaagtcgttgctcagcaatgtagctgtggaagcaggaggaacagtgctggcactttctcccaactgcttctgcagcatctgtagctcctgctgagcctcagccaaggagaccactggtgtctcacagcagccaaggaggagagggccagtggggctgaaaggcaggaagctggatggagctgagggcaatggtgcctgaggaaggctagccagcttgggtatggagtgaaaatgaaagcctgaatgggcctggttggcctccttgggggtattctggggagttggcaagctgatggggttgctgttggattcggccttagccccctgagatgcactggttgatgatggtttagaagacaacacagcagaatgactcgaatgatggatggaatctgagtgactgggagaagctttcttctcttcatagtgtgtgtactcgctgactatgtccatgtcagagcaggcttccagttcatcagacaggaaagaggtgctgctgggagagcggtgggagtcagacaaggcatggctgctggagggtgtgagggaccgagcatccagcttggcctgcaggacttcaatcactttctccttctcctgcagctccctgctgagcctgagggccagtggctcaagtccagcttgatctttctcacttttatgatccttggtgctgagtttgctggtgagcctctctgtcagctggcttccctgggcgagttgctcccggaagctctgtcccaggtagtagtcaatgtcattgctccttaggagatcctcaaaagattttactgtatcttttgcatgccgggtgataagataacaaatacctctcccttctcgtattttttgccgtaggtaagacagttcccgggcctgatcctgaatcagggaatcatatttcccaggccacgaggctgatctcagctcctcagccagcttctcttctagtccattttttgggagctgggcctccagctgggatactctctggatgagactctccaggtcctttttggcctgaagccctggagagtagaaagccccagtgccatcagacagccacccctcatcctcatcagggacactatgaggtgaagacccctccaaggtgccaacagctctcagcttccggggtctttccagactagacgaataatcacttgtaactgagagggaccggacccggctcttgaggttttgaatgaccttgttggcattctgcagctgggccttcagatctttgatgtcctttcgtaggaccaagatgttttctgactttccatatacccggaactcttcctgcttccctagctggttctccaagggcttcctctcagaggaactagccagtgttgagccccggcgtccctgctcagagcacagcccctccatcaggaccatttccttgaggctgttgtgctcctcacactcaggactggtggtttcctcccgttcagcctcattctcgcttcggccacaagtctcatagcccaggtcctggaggtccacctggatctgcttgctgtcctgcttcaccaaggattcacctgtaagcataactctgtatttctccagctcgttagcctgagcaaagacagtggcttctgatagcagcagcttctcctggagatcttgatagcgttgtttgcattgtgacagctgggagcgcaggtgctgggtggaccctggtaggctaaacgctgactgaggcccagggtcacgaggctgggactggttatccaattggtgggcatccactgtgaaggtagccccaaggtcaaggctctggggtctggggaaaggcctcacagtcacattcccctcctcttggtgttggtgcttcccaggggaaccaaccagttctgtgtttattctttcaatggtgctggtcagatgcacaaggagctctggagtaagtttactattcccttccttgctactcagcacaagttgttctttgaggaggttgatgatattgtgggcattcttcagttttccctggagctttctgaactcagcctgaaggctactctcactcagaccctctttggttaccacagtctcaaccatcacctcgcccttctccttgtcttcctcgatctcccatccatcagacattgcttctcccatctgctctttcagctccgcattctcaaggcaaaggctcagcatggtgttcctgatgtgggacactgaggagaatcctgcttcctcaatttgagcctttagctccttcagttcctcctcagctttcctcttctcttctaagtgctggtggaactcagccctcaggtggagcatttcttcctgaagacacctgttactgtcccctcccatcggagaaggaggggaaaaagatgggttctgggtctccacagttgccagacttttctccaaagccaccttgacaagttgctggtgactatggtgtgcagcctcctcctcaatactgtcagtgaactcagtgcttgtatcttcggtgtcatcccctgcagctgcacctccaatggcggccagggtctccagcctgtttaagcgctccaagcttcttccaagaacttcttctagccgactgcgtaacacctgagccccttccagttccacctgcagagttcggtctctctcagagctctctggatgggcatggaacttcaccagactgctatagagctgtctctctgcttgtaaggcctcattgagccgactccgttcatctactagtccttctagcatcagcagcaactgttgtcttcggtttcctgaaatttcttgaccctgggattctactgaagcaactttttcccgaagaagtaagacttcctgggtcaggcgttccatagctggtatgtcttcaggatcaaccagttgcatttgcaggtcctttatgagatcttctttaatctgtatgttcctggtcagagactccatatcagcagcctgcacctgcagctcttcttcctgcacagccatcatggactgtagagcagaaagttccatctgactttctctttcttttttagccatgagttcaagttcctctttggcattactcagttctttttccagccctgcaactgtgtccaagtctcctaatgtggatctgggtatgctgacatcctctttggcagtcaatgaagtgctatcatctctggaaggtatctgcattgaaccttgatcagtctgttttccaagacggccagtgggggtaacttcagcttgttggttagagatgggtgcttgggacatcagggagtctctccctcctaaatattggcgcagggcctgtaattctgaatttctttccattaaggcttgcaccaacttctctgcagcagcttggctttcctgctccctggtgctcacagactgaagcaggccttgaatctccatttcatgttccagcacttgtttatttcgatcacttagaaggtcctgcagcatcctttcctttcgctgtagacgctggcacagctcctctgctatctcactctgccctggtccaagtttgcagagcagtgttgcactaagatcctccacttctttgttcctatcatgaagagacgtctgtaactgctgaatgatactctcttgttccttctgccaacggctaaatttggtttccatttcttctttcagccactggaggttttgacaggtagtagataactgttccacttccaggcctttggccctcaggagactctccatactttgcatagtagcttcattggaggagaggacatcgcgcagtctctctaagtcatgatctcgctctctcacagcaagacgaagctggcgcagttctttttctttctcttctagagcagagaatttttcatctatagcccgctccagagcaacagctttatcatgtattcgctggcgaagtttctcaagcaacatttcatttgcttcaagggttttgtctgagttatctcgatactgtaggagctcccgaaattcctgaagcaactgctccttgtgactcagactatggtttaggtgctggatgttttgttcctgggttcgaatctcattgtatttttcagcctcccaggcacgaagctgttggctcttattctgcaattcttcttgtagctgctgcaaggcttttcgcaattcctggttatgtttccaagaagcctctttctgctgttcactctcgtgtgctgcagcctctacaaattgcacacattgtttggcatcagccagttggcgctctttctgtcgtaccaccctctggagcttctgtatttcaagttggctgcagaataaagcactctgaagatcaagcagagctacctgttgctgagctggagaagtaccctctgagctgtgaagttgtccaagctggctttggtgcagcatttctcgaagctttgccattgtgtcattttgaccttcaattacctggtacaactcctcagtctcacgttccctgcttttcagagtttccttgaggttctgaattgtaccatcttgcttttgagacgactcctgagcacactttagttcatagctcatttcattaagtttctcttgaagaatcttgttggtggcctctgtttgctggattttttcctggagttctgccaagtgggaatcagatacagactgctgagttatagtggtctcatgtgaattcagcttttgttgtttcagcaactcttcagtcatgggctgcacttccatgctagttggctcctccaacagatgtagcagttgttgtttctcccgagatagctgttctacaagcctctcctgggcagccaggctctgattcagttcttcaattctcttgtccctctgggccagggcctcagtgtattggtcgggcttgacctggtctcctggtacatcttcccagtttttggtgactcccttcagtttctctgagagctccaggttacactccttctctgcttccaccagagctgccatccgcgcagcttcattctttgctagcctggattcctcctgcagaagctggatcttattctccaagagctcataaacatgctccgtctcctgctgtcgctcctcaaactggcgtcggagctcagcttcattctgactgttgagattctccacatcagcccatgttttatccagatgctgtttcttgtcctggagttctcgtttcaagctctccacttcaaccttcagctcaatgttccgcttgtagatgtcctcccggctggcctcatacttctgttgcatgcgctcctccaggaagtagatgcgcagcttgaggctgaagttctccttcttcaggtcattgaggtgctgggacagagtgcgatatccattagacatgatgggcaacccatggggaggagcgtgcccgattgccccctcaacccaggaacatggtgcagctgcaccgcagcatgaagccagccggctgggacgctgctgaggctgcggaccgagaggctggggctacggcgacatggcccctattgctggagctctctccgggactcgggactgggctcactgctctgggt

SEQ ID NO: 8807 - RNA, 7374 nt, Homo sapiens
  source 1..7374: mol_type = other RNA
aagtgtgcagggcactggtgctgctccgaagctcatgaatacctttgctgcctagcacctctgtgccttgggcttcaaggccagggaagctgcacgctgatctcacaagagacactatctttttgaccagcagcttgccctccgcaatctgctgtcttagggcactgtagtcatcaatgtggccaatgacatggcggccatgcttattggcaaaggagccatcagtagcatcaccctctagcttgggaggggtcttcattactggagaagtatccaaacccaagccatttgctctgttgattatgggcgtttctgagccaggagtagaggaagcagagctggggaagaccagagctggggaattcataccaacatcccggactggaggggacacagctgaatcttggaggagcagctgcttgtttccagggtcagtgctggctgggaagttctggttaatggaggaggggctgaggctggctttgccagcaccgctctccagctgctgttgcagctgcagtcgcagacaattgttcccctgaatgctctgctccagctgccctctcagagctcgtacctctgccaccaggtggctcaggtcactgctcaaagggatttggtgacaggcatccaggctgtaagctttcagccccttcttggaattgccataaagtgcctcgtagatttgtagctctgactggagggactcaaagagctgctgtttctcttcacactgttgctgcaggagaaccagcttgtgctgcagtctggagtcgttttcctggagggaaagacgttcctccctgaaatgcaagacctcttgctgcttctccctcaagtcttccaaaagctgctgcctttccaccttctggtgctccagctccttttccagctcttgaaggtgggatcgagaggacagcagagcctccctcaggctttctgtttcctgggagtgctctctggaaacatgactcagttgagcctgaagtcttcgattgtcttccctgaggactctgttctcattgcagagctgaggtatggactccaggccctgactgtagaagttagaagtggatccccttccacgagcagtagaggtcagccggtgttccagttgctcccgtaggcggtcattgatgcagatggattcctccaggcgctggcgcaggttccggatttcaccaagatgctcttccagcaggtcagcccctgtgggtttggagttaagctggtacacagaggagcctgaggataggtccccagatacactccctttctgaggcctcatcacatcccacttgccactgctgcccaggtacccaggctctaggattcttcccagttctatggtgccccttggaggagagtgaggctgggcagagttgaggtagtaggaagagtcggcttccaagtcgttgctcagcaatgtagctgtggaagcaggaggaacagtgctggcactttctcccaactgcttctgcagcatctgtagctcctgctgagcctcagccaaggagaccactggtgtctcacagcagccaaggaggagagggccagtggggctgaaaggcaggaagctggatggagctgagggcaatggtgcctgaggaaggctagccagcttgggtatggagtgaaaatgaaagcctgaatgggcctggttggcctccttgggggtattctggggagttggcaagctgatggggttgctgttggattcggccttagccccctgagatgcactggttgatgatggtttagaagacaacacagcagaatgactcgaatgatggatggaatctgagtgactgggagaagctttcttctcttcatagtgtgtgtactcgctgactatgtccatgtcagagcaggcttccagttcatcagacaggaaagaggtgctgctgggagagcggtgggagtcagacaaggcatggctgctggagggtgtgagggaccgagcatccagcttggcctgcaggacttcaatcactttctccttctcctgcagctccctgctgagcctgagggccagtggctcaagtccagcttgatctttctcacttttatgatccttggtgctgagtttgctggtgagcctctctgtcagctggcttccctgggcgagttgctcccggaagctctgtcccaggtagtagtcaatgtcattgctccttaggagatcctcaaaagattttactgtatcttttgcatgccgggtgataagataacaaatacctctcccttctcgtattttttgccgtaggtaagacagttcccgggcctgatcctgaatcagggaatcatatttcccaggccacgaggctgatctcagctcctcagccagcttctcttctagtccattttttgggagctgggcctccagctgggatactctctggatgagactctccaggtcctttttggcctgaagccctggagagtagaaagccccagtgccatcagacagccacccctcatcctcatcagggacactatgaggtgaagacccctccaaggtgccaacagctctcagcttccggggtctttccagactagacgaataatcacttgtaactgagagggaccggacccggctcttgaggttttgaatgaccttgttggcattctgcagctgggccttcagatctttgatgtcctttcgtaggaccaagatgttttctgactttccatatacccggaactcttcctgcttccctagctggttctccaagggcttcctctcagaggaactagccagtgttgagccccggcgtccctgctcagagcacagcccctccatcaggaccatttccttgaggctgttgtgctcctcacactcaggactggtggtttcctcccgttcagcctcattctcgcttcggccacaagtctcatagcccaggtcctggaggtccacctggatctgcttgctgtcctgcttcaccaaggattcacctgtaagcataactctgtatttctccagctcgttagcctgagcaaagacagtggcttctgatagcagcagcttctcctggagatcttgatagcgttgtttgcattgtgacagctgggagcgcaggtgctgggtggaccctggtaggctaaacgctgactgaggcccagggtcacgaggctgggactggttatccaattggtgggcatccactgtgaaggtagccccaaggtcaaggctctggggtctggggaaaggcctcacagtcacattcccctcctcttggtgttggtgcttcccaggggaaccaaccagttctgtgtttattctttcaatggtgctggtcagatgcacaaggagctctggagtaagtttactattcccttccttgctactcagcacaagttgttctttgaggaggttgatgatattgtgggcattcttcagttttccctggagctttctgaactcagcctgaaggctactctcactcagaccctctttggttaccacagtctcaaccatcacctcgcccttctccttgtcttcctcgatctcccatccatcagacattgcttctcccatctgctctttcagctccgcattctcaaggcaaaggctcagcatggtgttcctgatgtgggacactgaggagaatcctgcttcctcaatttgagcctttagctccttcagttcctcctcagctttcctcttctcttctaagtgctggtggaactcagccctcaggtggagcatttcttcctgaagacacctgttactgtcccctcccatcggagaaggaggggaaaaagatgggttctgggtctccacagttgccagacttttctccaaagccaccttgacaagttgctggtgactatggtgtgcagcctcctcctcaatactgtcagtgaactcagtgcttgtatcttcggtgtcatcccctgcagctgcacctccaatggcggccagggtctccagcctgtttaagcgctccaagcttcttccaagaacttcttctagccgactgcgtaacacctgagccccttccagttccacctgcagagttcggtctctctcagagctctctggatgggcatggaacttcaccagactgctatagagctgtctctctgcttgtaaggcctcattgagccgactccgttcatctactagtccttctagcatcagcagcaactgttgtcttcggtttcctgaaatttcttgaccctgggattctactgaagcaactttttcccgaagaagtaagacttcctgggtcaggcgttccatagctggtatgtcttcaggatcaaccagttgcatttgcaggtcctttatgagatcttctttaatctgtatgttcctggtcagagactccatatcagcagcctgcacctgcagctcttcttcctgcacagccatcatggactgtagagcagaaagttccatctgactttctctttcttttttagccatgagttcaagttcctctttggcattactcagttctttttccagccctgcaactgtgtccaagtctcctaatgtggatctgggtatgctgacatcctctttggcagtcaatgaagtgctatcatctctggaaggtatctgcattgaaccttgatcagtctgttttccaagacggccagtgggggtaacttcagcttgttggttagagatgggtgcttgggacatcagggagtctctccctcctaaatattggcgcagggcctgtaattctgaatttctttccattaaggcttgcaccaacttctctgcagcagcttggctttcctgctccctggtgctcacagactgaagcaggccttgaatctccatttcatgttccagcacttgtttatttcgatcacttagaaggtcctgcagcatcctttcctttcgctgtagacgctggcacagctcctctgctatctcactctgccctggtccaagtttgcagagcagtgttgcactaagatcctccacttctttgttcctatcatgaagagacgtctgtaactgctgaatgatactctcttgttccttctgccaacggctaaatttggtttccatttcttctttcagccactggaggttttgacaggtagtagataactgttccacttccaggcctttggccctcaggagactctccatactttgcatagtagcttcattggaggagaggacatcgcgcagtctctctaagtcatgatctcgctctctcacagcaagacgaagctggcgcagttctttttctttctcttctagagcagagaatttttcatctatagcccgctccagagcaacagctttatcatgtattcgctggcgaagtttctcaagcaacatttcatttgcttcaagggttttgtctgagttatctcgatactgtaggagctcccgaaattcctgaagcaactgctccttgtgactcagactatggtttaggtgctggatgttttgttcctgggttcgaatctcattgtatttttcagcctcccaggcacgaagctgttggctcttattctgcaattcttcttgtagctgctgcaaggcttttcgcaattcctggttatgtttccaagaagcctctttctgctgttcactctcgtgtgctgcagcctctacaaattgcacacattgtttggcatcagccagttggcgctctttctgtcgtaccaccctctggagcttctgtatttcaagttggctgcagaataaagcactctgaagatcaagcagagctacctgttgctgagctggagaagtaccctctgagctgtgaagttgtccaagctggctttggtgcagcatttctcgaagctttgccattgtgtcattttgaccttcaattacctggtacaactcctcagtctcacgttccctgcttttcagagtttccttgaggttctgaattgtaccatcttgcttttgagacgactcctgagcacactttagttcatagctcatttcattaagtttctcttgaagaatcttgttggtggcctctgtttgctggattttttcctggagttctgccaagtgggaatcagatacagactgctgagttatagtggtctcatgtgaattcagcttttgttgtttcagcaactcttcagtcatgggctgcacttccatgctagttggctcctccaacagatgtagcagttgttgtttctcccgagatagctgttctacaagcctctcctgggcagccaggctctgattcagttcttcaattctcttgtccctctgggccagggcctcagtgtattggtcgggcttgacctggtctcctggtacatcttcccagtttttggtgactcccttcagtttctctgagagctccaggttacactccttctctgcttccaccagagctgccatccgcgcagcttcattctttgctagcctggattcctcctgcagaagctggatcttattctccaagagctcataaacatgctccgtctcctgctgtcgctcctcaaactggcgtcggagctcagcttcattctgactgttgagattctccacatcagcccatgttttatccagatgctgtttcttgtcctggagttctcgtttcaagctctccacttcaaccttcagctcaatgttccgcttgtagatgtcctcccggctggcctcatacttctgttgcatgcgctcctccaggaagtagatgcgcagcttgaggctgaagttctccttcttcaggtcattgaggtgcttctcaaagtctcgaagagcctgggtctgtacctgagggggtttctcaaatgctctcaaggaatatgtctgcacaaacgggaccttttcaccacttctccagatctgtgactgcactggagggcctcgatctttagtgtcactaagaaaagcagaaggagcccaagaaaaagcacccagatgcttcagtcaacttcttagaattcttcttttttttatgttcagaaaagatggaaattcatttctgctgtgtgactcgttctgggtaccatctccccatcatcctctgcaaaataatctctcatccagggtgtggccgccgcagctgcttcttcctcctcggccgctgctgcccagctcccggctggctccgggcgccgtctttcccggctcggggtctgccgtggggactgaggggttcgcgtcgcgtccccggaccggtaaggcgtgtagtgagcccggcgggacgcgcgacagcagcagccaaagtcgcatcggcggcggcagcaggacccgctgtctgtgcccttcatggatttcctgggcctggccaccccagtcctagctacggttcctgcttgttttcctggtgttttccgggactgccagggcgcatcctctgggcctggctgagcatccccgtcagttccctgggcctcctccgcggctgcctctgc

(The sequence listing continues in the following parts.)